European Patent Application EP 4 520 821 A1 - sequence listing, part 3

SEQ ID NO: 9729 - RNA, 3353 nt, Homo sapiens
  source 1..3353: mol_type = other RNA
atgcgaggatgctgacagtggaaacgacttcctccattcttacagcacattccaaacacttcttgggaacaaggttacatccagccttgggggtcttccatcctcaccagggcccctgcaggagggagcccaggcatccccaccaggttcatccttggagctgccctgcacacaccctgggccactggcagaggtcctctctccagagtctcccggacacagtgacctccttacatggtggactcttccccccgagaagcccccactgggggctgctgggggccagggtgggtggtggctgcaagggctgtggagagtctagaggtggtgggagaaagcacgcgaggcccgaggagggtgatgggggtcttcgaggggctggggtccatcatggaaagtgctgaagcttccgtcaggagggtgccaggcagaggaggccacctggacactatctgggccccagaggctgagaacgagcgctctggagtcacaggaggtggctgaggagcccctggggaagctagaggtagagtgggggctcctggaggggtcgaaggccctggtgagagtcgaggggaggccccaggctcccctgggaaagtggctgtcagccccaaagcgagtgagtgtggaccatgagctcctgccgggcttgtaggtaaagtctgtgttttcatcaagttcgttcttaaaaggagctggaggagatgaagcaccggcctcgagggtgatgctgtcgggggcccaggacaggagctacagttgacaggggcctcagtgtctccatgcaggctccgaccagctttgctgaatgccacatttccgtgaggggagagcccctgcttttcttccagaggagacagggaatctggacaggaagagcagcagtccccaggaagcagggcagggtcggcacaggcccgctggcagggaaccttctcacagctcacctctcccagctggcacgtgcaccgggtgcagggttcatcatccaaggtgaacacctggccattcgccaccttccttccctcgtagttgcagtctcggcacacggggcagcactccccgtcagggtggaaagggtaggtacaggtgatggggcagtccacgggggaacaggccactgagcccagcaggcagatgcagctcagacatgggtccagcacagacgggaaggtctcgttgttatagaagattctgcctgtgtaggtgcagcctgctgaacagtctgggcagcactgtccagggatccggatcgggtgagggcaggagtccacacagtctgtcctcttgcagctcaccgagccataggggtcaccaggcgaccagatctgtccaatcggaaactcaaccccgttgtcgtcaagagagcagcctgtcgagggtgtgggctcctggcaggtgaagcaacactgcccagggcccagccgccactcttctcgggggcaggccagctcagggcagggcatgaaggagcactccacctccccattctggcaaacacaggtggtacactcgtcaccacccccactgaacacagccccgtctgcgtaccaccggccgtggaaatagcatctcactggaacacaagtacagcaatccgtctgtgggggggtctgacaggggccagaaggacactcaggagagatgcaggacacgtttccagccagacagacacagacggtgcagttctcattgggaggtgaaaacacatccccttcagctcggacgacaccactgtgaaaacagcctgtgcacgatgggcagcacccaccatctctggagggaattgggtgggaacaagcagcttcacacctcaccttttcacaggtcaccttcccgtcctcgcaccagcactgggaacacccaggctctgtccagcgactccttgattcatgcatggctcccaggtgccagcagggagagggccctgctgccagtcggggggactcagggcccctgggtgaggaaggggtccccatcacctccccctgaaggagtgaggggggtctgaggttccccagcagggaggcagtaggcactggggtggccagcagggtggacagcagccacacaggggcagaaggggaggatgtgggtagtcgtggggtgggagatggcaggcgggtggtcctgactccggctgggggccctggagccccagaaggagggctatgtcctggggacagggcaggccggccggcctcaggaagcaacagaagcatcttggacgggtgttgccggggttgcaggatggcagatggggccagcacggctttcgggaaagcttcacaggacacgcggtcagctcggagcctgaagccaggtcggcatgtgcataggaagctgcccacggtgttgtggcaggaatggtgacagactcgcctctccaatggcctccgacactcgtttacatctacacaggagtgccggttgccatgaaggtggaagccagttcgacaggaacacttgtagctgccaatgctgtttttacatctctgctgacagggagtccctaggcattcgtcagtgtcttggcagctgtggcggtcggcagacagctgcatgcccggcccacactcgcacacaaacccaccttctgtgttcacacagtggccctcgcaggaggaggttacacattcgtcaatgtctgtacacctgatgccaacagctgtctccgtcatcgagaagcccacggggcacactcgggccacctcctgacagcctccatggttgcaggtaaggtcacagccgtactccccacatggtccatgggtttctgggcaggtggccccttgctctccatcctggcaggagcagacattgggagcgatgcagatgccactcccacagccgaaggagcagaggggcagggtgcagtgcccaccacccatagagggcgcccagccagggcagcagccactcccaaacccagagaggcagacgtgggggcccagtcggcgtctctcggccgcgaagtgcccgggcggcttcctcccggtgtagcctcgggctggtgcccccggcagcaggagcgcgacacaggcggcccgaaggagcagtccggcccacatgaccggcggcggcgggtcccccgggctgggctcggctcctgcgccgcgcgcgggagagggggctgccggccctcgcccctcctcctggcgccgtggggagcgaaccagcgatccccgaaatggcacgcagagctgagcaggggggcttgggacgccgagaggaggggccgagggccgcgaggggacgcggcggacgattgtggggagggtctctggcacctcgaagcgaaacacacaaaggcaacgccgcccgcctgctgatgcctctccgagaggcgc

SEQ ID NO: 9730 - RNA, 3357 nt, Homo sapiens
  source 1..3357: mol_type = other RNA
atgcgaggatgctgacagtggaaacgacttcctccattcttacagcacattccaaacacttcttgggaacaaggttacatccagccttgggggtcttccatcctcaccagggcccctgcaggagggagcccaggcatccccaccaggttcatccttggagctgccctgcacacaccctgggccactggcagaggtcctctctccagagtctcccggacacagtgacctccttacatggtggactcttccccccgagaagcccccactgggggctgctgggggccagggtgggtggtggctgcaagggctgtggagagtctagaggtggtgggagaaagcacgcgaggcccgaggagggtgatgggggtcttcgaggggctggggtccatcatggaaagtgctgaagcttccgtcaggagggtgccaggcagaggaggccacctggacactatctgggccccagaggctgagaacgagcgctctggagtcacaggaggtggctgaggagcccctggggaagctagaggtagagtgggggctcctggaggggtcgaaggccctggtgagagtcgaggggaggccccaggctcccctgggaaagtggctgtcagccccaaagcgagtgagtgtggaccatgagctcctgccgggcttgtaggtaaagtctgtgttttcatcaagttcgttcttaaaaggagctggaggagatgaagcaccggcctcgagggtgatgctgtcgggggcccaggacaggagctacagttgacaggggcctcagtgtctccatgcaggctccgaccagctttgctgaatgccacatttccgtgaggggagagcccctgcttttcttccagaggagacagggaatctggacaggaagagcagcagtccccaggaagcagggcagggtcggcacaggcccgctggcagggaaccttctcacagctcacctctcccagctggcacgtgcaccgggtgcagggttcatcatccaaggtgaacacctggccattcgccaccttccttccctcgtagttgcagtctcggcacacggggcagcactccccgtcagggtggaaagggtaggtacaggtgatggggcagtccacgggggaacaggccactgagcccagcaggcagatgcagctcagacatgggtccagcacagacgggaaggtctcgttgttatagaagattctgcctgtgtaggtgcagcctgctgaacagtctgggcagcactgtccagggatccggatcgggtgagggcaggagtccacacagtctgtcctcttgcagctcaccgagccatctgcaggggtcaccaggcgaccagatctgtccaatcggaaactcaaccccgttgtcgtcaagagagcagcctgtcgagggtgtgggctcctggcaggtgaagcaacactgcccagggcccagccgccactcttctcgggggcaggccagctcagggcagggcatgaaggagcactccacctccccattctggcaaacacaggtggtacactcgtcaccacccccactgaacacagccccgtctgcgtaccaccggccgtggaaatagcatctcactggaacacaagtacagcaatccgtctgtgggggggtctgacaggggccagaaggacactcaggagagatgcaggacacgtttccagccagacagacacagacggtgcagttctcattgggaggtgaaaacacatccccttcagctcggacgacaccactgtgaaaacagcctgtgcacgatgggcagcacccaccatctctggagggaattgggtgggaacaagcagcttcacacctcaccttttcacaggtcaccttcccgtcctcgcaccagcactgggaacacccaggctctgtccagcgactccttgattcatgcatggctcccaggtgccagcagggagagggccctgctgccagtcggggggactcagggcccctgggtgaggaaggggtccccatcacctccccctgaaggagtgaggggggtctgaggttccccagcagggaggcagtaggcactggggtggccagcagggtggacagcagccacacaggggcagaaggggaggatgtgggtagtcgtggggtgggagatggcaggcgggtggtcctgactccggctgggggccctggagccccagaaggagggctatgtcctggggacagggcaggccggccggcctcaggaagcaacagaagcatcttggacgggtgttgccggggttgcaggatggcagatggggccagcacggctttcgggaaagcttcacaggacacgcggtcagctcggagcctgaagccaggtcggcatgtgcataggaagctgcccacggtgttgtggcaggaatggtgacagactcgcctctccaatggcctccgacactcgtttacatctacacaggagtgccggttgccatgaaggtggaagccagttcgacaggaacacttgtagctgccaatgctgtttttacatctctgctgacagggagtccctaggcattcgtcagtgtcttggcagctgtggcggtcggcagacagctgcatgcccggcccacactcgcacacaaacccaccttctgtgttcacacagtggccctcgcaggaggaggttacacattcgtcaatgtctgtacacctgatgccaacagctgtctccgtcatcgagaagcccacggggcacactcgggccacctcctgacagcctccatggttgcaggtaaggtcacagccgtactccccacatggtccatgggtttctgggcaggtggccccttgctctccatcctggcaggagcagacattgggagcgatgcagatgccactcccacagccgaaggagcagaggggcagggtgcagtgcccaccacccatagagggcgcccagccagggcagcagccactcccaaacccagagaggcagacgtgggggcccagtcggcgtctctcggccgcgaagtgcccgggcggcttcctcccggtgtagcctcgggctggtgcccccggcagcaggagcgcgacacaggcggcccgaaggagcagtccggcccacatgaccggcggcggcgggtcccccgggctgggctcggctcctgcgccgcgcgcgggagagggggctgccggccctcgcccctcctcctggcgccgtggggagcgaaccagcgatccccgaaatggcacgcagagctgagcaggggggcttgggacgccgagaggaggggccgagggccgcgaggggacgcggcggacgattgtggggagggtctctggcacctcgaagcgaaacacacaaaggcaacgccgcccgcctgctgatgcctctccgagaggcgc

SEQ ID NO: 9731 - RNA, 3248 nt, Homo sapiens
  source 1..3248: mol_type = other RNA
atgcgaggatgctgacagtggaaacgacttcctccattcttacagcacattccaaacacttcttgggaacaaggttacatccagccttgggggtcttccatcctcaccagggcccctgcaggagggagcccaggcatccccaccaggttcatccttggagctgccctgcacacaccctgggccactggcagaggtcctctctccagagtctcccggacacagtgacctccttacatggtggactcttccccccgagaagcccccactgggggctgctgggggccagggtgggtggtggctgcaagggctgtggagagtctagaggtggtgggagaaagcacgcgaggcccgaggagggtgatgggggtcttcgaggggctggggtccatcatggaaagtgctgaagcttccgtcaggagggtgccaggcagaggaggccacctggacactatctgggccccagaggctgagaacgagcgctctggagtcacaggaggtggctgaggagcccctggggaagctagaggtagagtgggggctcctggaggggtcgaaggccctggtgagagtcgaggggaggccccaggctcccctgggaaagtggctgtcagccccaaagcgagtgagtgtggaccatgagctcctgccgggcttgtaggtaaagtctgtgttttcatcaagttcgttcttaaaaggagctggaggagatgaagcaccggcctcgagggtgatgctgtcgggggcccaggacaggagctacagttgacaggggcctcagtgtctccatgcaggctccgaccagctttgctgaatgccacatttccgtgaggggagagcccctgcttttcttccagaggagacagggaatctggacaggaagagcagcagtccccaggaagcagggcagggtcggcacaggcccgctggcagggaaccttctcacagctcacctctcccagctggcacgtgcaccgggtgcagggttcatcatccaaggtgaacacctggccattcgccaccttccttccctcgtagttgcagtctcggcacacggggcagcactccccgtcagggtggaaagggtaggtacaggtgatggggcagtccacgggggaacaggccactgagcccagcaggcagatgcagctcagacatgggtccagcacagacgggaaggtctcgttgttatagaagattctgcctgtgtaggtgcagcctgctgaacagtctgggcagcactgtccagggatccggatcgggtgagggcaggagtccacacagtctgtcctcttgcagctcaccgagccatctgcctggcagatgcataactcacaggggtcaccaggcgaccagatctgtccaatcggaaactcaaccccgttgtcgtcaagagagcagcctgtcgagggtgtgggctcctggcaggtgaagcaacactgcccagggcccagccgccactcttctcgggggcaggccagctcagggcagggcatgaaggagcactccacctccccattctggcaaacacaggtggtacactcgtcaccacccccactgaacacagccccgtctgcgtaccaccggccgtggaaatagcatctcactggaacacaagtacagcaatccgtctgtgggggggtctgacaggggccagaaggacactcaggagagatgcaggacacgtttccagccagacagacacagacggtgcagttctcattgggaggtgaaaacacatccccttcagctcggacgacaccactgtgaaaacagcctgtgcacgatgggcagcacccaccatctctggagggaattgggtgggaacaagcagcttcacacctcaccttttcacaggtcaccttcccgtcctcgcaccagcactgggaacacccaggctctgtccagcgactccttgattcatgcatggctcccaggtgccagcagggagagggccctgctgccagtcggggggactcagggcccctgggtgaggaaggggtccccatcacctccccctgaaggagtgaggggggtctgaggttccccagcagggaggcagtaggcactggggtggccagcagggtggacagcagccacacaggggcagaaggggaggatgtgggtagtcgtggggtgggagatggcaggcgggtggtcctgactccggctgggggccctggagccccagaaggagggctatgtcctggggacagggcaggccggccggcctcaggaagcaacagaagcatcttggacgggtgttgccggggttgcaggatggcagatggggccagcacggctttcgggaaagctacacaggagtgccggttgccatgaaggtggaagccagttcgacaggaacacttgtagctgccaatgctgtttttacatctctgctgacagggagtccctaggcattcgtcagtgtcttggcagctgtggcggtcggcagacagctgcatgcccggcccacactcgcacacaaacccaccttctgtgttcacacagtggccctcgcaggaggaggttacacattcgtcaatgtctgtacacctgatgccaacagctgtctccgtcatcgagaagcccacggggcacactcgggccacctcctgacagcctccatggttgcaggtaaggtcacagccgtactccccacatggtccatgggtttctgggcaggtggccccttgctctccatcctggcaggagcagacattgggagcgatgcagatgccactcccacagccgaaggagcagaggggcagggtgcagtgcccaccacccatagagggcgcccagccagggcagcagccactcccaaacccagagaggcagacgtgggggcccagtcggcgtctctcggccgcgaagtgcccgggcggcttcctcccggtgtagcctcgggctggtgcccccggcagcaggagcgcgacacaggcggcccgaaggagcagtccggcccacatgaccggcggcggcgggtcccccgggctgggctcggctcctgcgccgcgcgcgggagagggggctgccggccctcgcccctcctcctggcgccgtggggagcgaaccagcgatccccgaaatggcacgcagagctgagcaggggggcttgggacgccgagaggaggggccgagggccgcgaggggacgcggcggacgattgtggggagggtctctggcacctcgaagcgaaacacacaaaggcaacgccgcccgcctgctgatgcctctccgagaggcgc

SEQ ID NO: 9732 - RNA, 3161 nt, Homo sapiens
  source 1..3161: mol_type = other RNA
atgcgaggatgctgacagtggaaacgacttcctccattcttacagcacattccaaacacttcttgggaacaaggttacatccagccttgggggtcttccatcctcaccagggcccctgcaggagggagcccaggcatccccaccaggttcatccttggagctgccctgcacacaccctgggccactggcagaggtcctctctccagagtctcccggacacagtgacctccttacatggtggactcttccccccgagaagcccccactgggggctgctgggggccagggtgggtggtggctgcaagggctgtggagagtctagaggtggtgggagaaagcacgcgaggcccgaggagggtgatgggggtcttcgaggggctggggtccatcatggaaagtgctgaagcttccgtcaggagggtgccaggcagaggaggccacctggacactatctgggccccagaggctgagaacgagcgctctggagtcacaggaggtggctgaggagcccctggggaagctagaggtagagtgggggctcctggaggggtcgaaggccctggtgagagtcgaggggaggccccaggctcccctgggaaagtggctgtcagccccaaagcgagtgagtgtggaccatgagctcctgccgggcttgtaggtaaagtctgtgttttcatcaagttcgttcttaaaaggagctggaggagatgaagcaccggcctcgagggtgatgctgtcgggggcccaggacaggagctacagttgacaggggcctcagtgtctccatgcaggctccgaccagctttgctgaatgccacatttccgtgaggggagagcccctgcttttcttccagaggagacagggaatctggacaggaagagcagcagtccccaggaagcagggcagggtcggcacaggcccgctggcagggaaccttctcacagctcacctctcccagctggcacgtgcaccgggtgcagggttcatcatccaaggtgaacacctggccattcgccaccttccttccctcgtagttgcagtctcggcacacggggcagcactccccgtcagggtggaaagggtaggtacaggtgatggggcagtccacgggggaacaggccactgagcccagcaggcagatgcagctcagacatgggtccagcacagacgggaaggtctcgttgttatagaagattctgcctgtgtaggtgcagcctgctgaacagtctgggcagcactgtccagggatccggatcgggtgagggcaggagtccacacagtctgtcctcttgcagctcaccgagccatctgcctggcagatgcataactcacaggggtcaccaggcgaccagatctgtccaatcggaaactcaaccccgttgtcgtcaagagagcagcctgtcgagggtgtgggctcctggcaggtgaagcaacactgcccagggcccagccgccactcttctcgggggcaggccagctcagggcagggcatgaaggagcactccacctccccattctggcaaacacaggtggtacactcgtcaccacccccactgaacacagccccgtctgcgtaccaccggccgtggaaatagcatctcactggaacacaagtacagcaatccgtctgtgggggggtctgacaggggccagaaggacactcaggagagatgcaggacacgtttccagccagacagacacagacggtgcagttctcattgggaggtgaaaacacatccccttcagctcggacgacaccactgtgaaaacagcctgtgcacgatgggcagcacccaccatctctggagggaattgggtgggaacaagcagcttcacacctcaccttttcacaggtcaccttcccgtcctcgcaccagcactgggaacacccaggctctgtccagcgactccttgattcatgcatggctcccaggtgccagcagggagagggccctgctgccagtcggggggactcagggcccctgggtgaggaaggggtccccatcacctccccctgaaggagtgaggggggtctgaggttccccagcagggaggcagtaggcactggggtggccagcagggtggacagcagccacacaggggcagaaggggaggatgtgggtagtcgtggggtgggagatggcaggcgggtggtcctgactccggctgggggccctggagccccagaaggagggctatgtcctggggacagggcaggccggccggcctcaggaagcaacagaagcatcttggacgggtgttgccggggttgcaggatggcagatggggccagcacggctttcgggaaagcttcacaggacacgcggtcagctcggagcctgaagccaggtcggcatgtgcataggaagctgcccacggtgttgtggcaggaatggtgacagactcgcctctccaatggcctccgacactcgtttacatcaaggggagcaaaggcagccaagaaaatgggtgagcagagaggaatccttggggtgtatctacacaggagtgccggttgccatgaaggtggaagccagttcgacaggaacacttgtagctgccaatgctgtttttacatctctgctgacagggagtccctaggcattcgtcagtgtcttggcagctgtggcggtcggcagacagctgcatgcccggcccacactcgcacacaaacccaccttctgtgttcacacagtggccctcgcaggaggaggttacacattcgtcaatgtctgtacacctgatgccaacagctgtctccgtcatcgagaagcccacggggcacactcgggccacctcctgacagcctccatggttgcaggtaaggtcacagccgtactccccacatggtccatgggtttctgggcaggtggccccttgctctccatcctggcaggagcagacattgggagcgatgcagatgccactcccacagccgaaggagcagaggggcagggtgcagtgcccaccacccatagagggcgcccagccagggcagcagccactcccaaacccagagaggcagacgtgggggcccagtcggcgtctctcggccgcgaagtgcccgggcggcttcctcccggtgtagcctcgggctggtgcccccggcagcaggagcgcgacacaggcggcccgaaggagcagtccggcccacatgacc

SEQ ID NO: 9733 - RNA, 2970 nt, Homo sapiens
  source 1..2970: mol_type = other RNA
atgcgaggatgctgacagtggaaacgacttcctccattcttacagcacattccaaacacttcttgggaacaaggttacatccagccttgggggtcttccatcctcaccagggcccctgcaggagggagcccaggcatccccaccaggttcatccttggagctgccctgcacacaccctgggccactggcagaggtcctctctccagagtctcccggacacagtgacctccttacatggtggactcttccccccgagaagcccccactgggggctgctgggggccagggtgggtggtggctgcaagggctgtggagagtctagaggtggtgggagaaagcacgcgaggcccgaggagggtgatgggggtcttcgaggggctggggtccatcatggaaagtgctgaagcttccgtcaggagggtgccaggcagaggaggccacctggacactatctgggccccagaggctgagaacgagcgctctggagtcacaggaggtggctgaggagcccctggggaagctagaggtagagtgggggctcctggaggggtcgaaggccctggtgagagtcgaggggaggccccaggctcccctgggaaagtggctgtcagccccaaagcgagtgagtgtggaccatgagctcctgccgggcttgtaggtaaagtctgtgttttcatcaagttcgttcttaaaaggagctggaggagatgaagcaccggcctcgagggtgatgctgtcgggggcccaggacaggagctacagttgacaggggcctcagtgtctccatgcaggctccgaccagctttgctgaatgccacatttccgtgaggggagagcccctgcttttcttccagaggagacagggaatctggacaggaagagcagcagtccccaggaagcagggcagggtcggcacaggcccgctggcagggaaccttctcacagctcacctctcccagctggcacgtgcaccgggtgcagggttcatcatccaaggtgaacacctggccattcgccaccttccttccctcgtagttgcagtctcggcacacggggcagcactccccgtcagggtggaaagggtaggtacaggtgatggggcagtccacgggggaacaggccactgagcccagcaggcagatgcagctcagacatgggtccagcacagacgggaaggtctcgttgttatagaagattctgcctgtgtaggtgcagcctgctgaacagtctgggcagcactgtccagggatccggatcgggtgagggcaggagtccacacagtctgtcctcttgcagctcaccgagccatctgcctggcagatgcataactcacaggggtcaccaggcgaccagatctgtccaatcggaaactcaaccccgttgtcgtcaagagagcagcctgtcgagggtgtgggctcctggcaggtgaagcaacactgcccagggcccagccgccactcttctcgggggcaggccagctcagggcagggcatgaaggagcactccacctccccattctggcaaacacaggtggtacactcgtcaccacccccactgaacacagccccgtctgcgtaccaccggccgtggaaatagcatctcactggaacacaagtacagcaatccgtctgtgggggggtctgacaggggccagaaggacactcaggagagatgcaggacacgtttccagccagacagacacagacggtgcagttctcattgggaggtgaaaacacatccccttcagctcggacgacaccactgtgaaaacagcctgtgcacgatgggcagcacccaccatctctggagggaattgggtgggaacaagcagcttcacacctcaccttttcacaggtcaccttcccgtcctcgcaccagcactgggaacacccaggctctgtccagcgactccttgattcatgcatggctcccaggtgccagcagggagagggccctgctgccagtcggggggactcagggcccctgggtgaggaaggggtccccatcacctccccctgaaggagtgaggggggtctgaggttccccagcagggaggcagtaggcactggggtggccagcagggtggacagcagccacacaggggcagaaggggaggatgtgggtagtcgtggggtgggagatggcaggcgggtggtcctgactccggctgggggccctggagccccagaaggagggctatgtcctggggacagggcaggccggccggcctcaggaagcaacagaagcatcttggacgggtgttgccggggttgcaggatggcagatggggccagcacggctttcgggaaagcttcacaggacacgcggtcagctcggagcctgaagccaggtcggcatgtgcataggaagctgcccacggtgttgtggcaggaatggtgacagactcgcctctccaatggcctccgacactcgtttacatctacacaggagtgccggttgccatgaaggtggaagccagttcgacaggaacacttgtagctgccaatgctgtttttacatctctgctgacagggagtccctaggcattcgtcagtgtcttggcagctgtggcggtcggcagacagctgcatgcccggcccacactcgcacacaaacccaccttctgtgttcacacagtggccctcgcaggaggaggttacacattcgtcaatgtctgtacacctgatgccaacagctgtctccgtcatcgagaagcccacggggcacactcgggccacctcctgacagcctccatggttgcaggtaaggtcacagccgtactccccacatggtccatgggtttctgggcaggtggccccttgctctccatcctggcaggagcagacattgggagcgatgcagatgccactcccacagccgaaggagcagagggctctcggccgcgaagtgcccgggcggcttcctcccggtgtagcctcgggctggtgcccccggcagcaggagcgcgac

SEQ ID NO: 9734 - RNA, 3377 nt, Homo sapiens
  source 1..3377: mol_type = other RNA
atgcgaggatgctgacagtggaaacgacttcctccattcttacagcacattccaaacacttcttgggaacaaggttacatccagccttgggggtcttccatcctcaccagggcccctgcaggagggagcccaggcatccccaccaggttcatccttggagctgccctgcacacaccctgggccactggcagaggtcctctctccagagtctcccggacacagtgacctccttacatggtggactcttccccccgagaagcccccactgggggctgctgggggccagggtgggtggtggctgcaagggctgtggagagtctagaggtggtgggagaaagcacgcgaggcccgaggagggtgatgggggtcttcgaggggctggggtccatcatggaaagtgctgaagcttccgtcaggagggtgccaggcagaggaggccacctggacactatctgggccccagaggctgagaacgagcgctctggagtcacaggaggtggctgaggagcccctggggaagctagaggtagagtgggggctcctggaggggtcgaaggccctggtgagagtcgaggggaggccccaggctcccctgggaaagtggctgtcagccccaaagcgagtgagtgtggaccatgagctcctgccgggcttgtaggtaaagtctgtgttttcatcaagttcgttcttaaaaggagctggaggagatgaagcaccggcctcgagggtgatgctgtcgggggcccaggacaggagctacagttgacaggggcctcagtgtctccatgcaggctccgaccagctttgctgaatgccacatttccgtgaggggagagcccctgcttttcttccagaggagacagggaatctggacaggaagagcagcagtccccaggaagcagggcagggtcggcacaggcccgctggcagggaaccttctcacagctcacctctcccagctggcacgtgcaccgggtgcagggttcatcatccaaggtgaacacctggccattcgccaccttccttccctcgtagttgcagtctcggcacacggggcagcactccccgtcagggtggaaagggtaggtacaggtgatggggcagtccacgggggaacaggccactgagcccagcaggcagatgcagctcagacatgggtccagcacagacgggaaggtctcgttgttatagaagattctgcctgtgtaggtgcagcctgctgaacagtctgggcagcactgtccagggatccggatcgggtgagggcaggagtccacacagtctgtcctcttgcagctcaccgagccatctgcctggcagatgcataactcacaggggtcaccaggcgaccagatctgtccaatcggaaactcaaccccgttgtcgtcaagagagcagcctgtcgagggtgtgggctcctggcaggtgaagcaacactgcccagggcccagccgccactcttctcgggggcaggccagctcagggcagggcatgaaggagcactccacctccccattctggcaaacacaggtggtacactcgtcaccacccccactgaacacagccccgtctgcgtaccaccggccgtggaaatagcatctcactggaacacaagtacagcaatccgtctgtgggggggtctgacaggggccagaaggacactcaggagagatgcaggacacgtttccagccagacagacacagacggtgcagttctcattgggaggtgaaaacacatccccttcagctcggacgacaccactgtgaaaacagcctgtgcacgatgggcagcacccaccatctctggagggaattgggtgggaacaagcagcttcacacctcaccttttcacaggtcaccttcccgtcctcgcaccagcactgggaacacccaggctctgtccagcgactccttgattcatgcatggctcccaggtgccagcagggagagggccctgctgccagtcggggggactcagggcccctgggtgaggaaggggtccccatcacctccccctgaaggagtgaggggggtctgaggttccccagcagggaggcagtaggcactggggtggccagcagggtggacagcagccacacaggggcagaaggggaggatgtgggtagtcgtggggtgggagatggcaggcgggtggtcctgactccggctgggggccctggagccccagaaggagggctatgtcctggggacagggcaggccggccggcctcaggaagcaacagaagcatcttggacgggtgttgccggggttgcaggatggcagatggggccagcacggctttcgggaaagcttcacaggacacgcggtcagctcggagcctgaagccaggtcggcatgtgcataggaagctgcccacggtgttgtggcaggaatggtgacagactcgcctctccaatggcctccgacactcgtttacatctacacaggagtgccggttgccatgaaggtggaagccagttcgacaggaacacttgtagctgccaatgctgtttttacatctctgctgacagggagtccctaggcattcgtcagtgtcttggcagctgtggcggtcggcagacagctgcatgcccggcccacactcgcacacaaacccaccttctgtgttcacacagtggccctcgcaggaggaggttacacattcgtcaatgtctgtacacctgatgccaacagctgtctccgtcatcgagaagcccacggggcacactcgggccacctcctgacagcctccatggttgcaggtaaggtcacagccgtactccccacatggtccatgggtttctgggcaggtggccccttgctctccatcctggcaggagcagacattgggagcgatgcagatgccactcccacagccgaaggagcagaggggcagggtgcagtgcccaccacccatagagggcgcccagccagggcagcagccactcccaaacccagagaggcagacgtgggggcccagtcggcgtctctcggccgcgaagtgcccgggcggcttcctcccggtgtagcctcgggctggtgcccccggcagcaggagcgcgacacaggcggcccgaaggagcagtccggcccacatgaccggcggcggcgggtcccccgggctgggctcggctcctgcgccgcgcgcgggagagggggctgccggccctcgcccctcctcctggcgccgtggggagcgaaccagcgatccccgaaatggcacgcagagctgagcaggggggcttgggacgccgagaggaggggccgagggccgcgaggggacgcggcggacgattgtggggagggtctctggcacctcgaagcgaaacacacaaaggcaacgccgcccgcctgctgatgcctctccgagaggcgc

SEQ ID NO: 9735 - RNA, 3083 nt, Homo sapiens
  source 1..3083: mol_type = other RNA
atgcgaggatgctgacagtggaaacgacttcctccattcttacagcacattccaaacacttcttgggaacaaggttacatccagccttgggggtcttccatcctcaccagggcccctgcaggagggagcccaggcatccccaccaggttcatccttggagctgccctgcacacaccctgggccactggcagaggtcctctctccagagtctcccggacacagtgacctccttacatggtggactcttccccccgagaagcccccactgggggctgctgggggccagggtgggtggtggctgcaagggctgtggagagtctagaggtggtgggagaaagcacgcgaggcccgaggagggtgatgggggtcttcgaggggctggggtccatcatggaaagtgctgaagcttccgtcaggagggtgccaggcagaggaggccacctggacactatctgggccccagaggctgagaacgagcgctctggagtcacaggaggtggctgaggagcccctggggaagctagaggtagagtgggggctcctggaggggtcgaaggccctggtgagagtcgaggggaggccccaggctcccctgggaaagtggctgtcagccccaaagcgagtgagtgtggaccatgagctcctgccgggcttgtaggtaaagtctgtgttttcatcaagttcgttcttaaaaggagctggaggagatgaagcaccggcctcgagggtgatgctgtcgggggcccaggacaggagctacagttgacaggggcctcagtgtctccatgcaggctccgaccagctttgctgaatgccacatttccgtgaggggagagcccctgcttttcttccagaggagacagggaatctggacaggaagagcagcagtccccaggaagcagggcagggtcggcacaggcccgctggcagggaaccttctcacagctcacctctcccagctggcacgtgcaccgggtgcagggttcatcatccaaggtgaacacctggccattcgccaccttccttccctcgtagttgcagtctcggcacacggggcagcactccccgtcagggtggaaagggtaggtacaggtgatggggcagtccacgggggaacaggccactgagcccagcaggcagatgcagctcagacatgggtccagcacagacgggaaggtctcgttgttatagaagattctgcctgtgtaggtgcagcctgctgaacagtctgggcagcactgtccagggatccggatcgggtgagggcaggagtccacacagtctgtcctcttgcagctcaccgagccatctggaacacaagtacagcaatccgtctgtgggggggtctgacaggggccagaaggacactcaggagagatgcaggacacgtttccagccagacagacacagacggtgcagttctcattgggaggtgaaaacacatccccttcagctcggacgacaccactgtgaaaacagcctgtgcacgatgggcagcacccaccatctctggagggaattgggtgggaacaagcagcttcacacctcaccttttcacaggtcaccttcccgtcctcgcaccagcactgggaacacccaggctctgtccagcgactccttgattcatgcatggctcccaggtgccagcagggagagggccctgctgccagtcggggggactcagggcccctgggtgaggaaggggtccccatcacctccccctgaaggagtgaggggggtctgaggttccccagcagggaggcagtaggcactggggtggccagcagggtggacagcagccacacaggggcagaaggggaggatgtgggtagtcgtggggtgggagatggcaggcgggtggtcctgactccggctgggggccctggagccccagaaggagggctatgtcctggggacagggcaggccggccggcctcaggaagcaacagaagcatcttggacgggtgttgccggggttgcaggatggcagatggggccagcacggctttcgggaaagcttcacaggacacgcggtcagctcggagcctgaagccaggtcggcatgtgcataggaagctgcccacggtgttgtggcaggaatggtgacagactcgcctctccaatggcctccgacactcgtttacatctacacaggagtgccggttgccatgaaggtggaagccagttcgacaggaacacttgtagctgccaatgctgtttttacatctctgctgacagggagtccctaggcattcgtcagtgtcttggcagctgtggcggtcggcagacagctgcatgcccggcccacactcgcacacaaacccaccttctgtgttcacacagtggccctcgcaggaggaggttacacattcgtcaatgtctgtacacctgatgccaacagctgtctccgtcatcgagaagcccacggggcacactcgggccacctcctgacagcctccatggttgcaggtaaggtcacagccgtactccccacatggtccatgggtttctgggcaggtggccccttgctctccatcctggcaggagcagacattgggagcgatgcagatgccactcccacagccgaaggagcagaggggcagggtgcagtgcccaccacccatagagggcgcccagccagggcagcagccactcccaaacccagagaggcagacgtgggggcccagtcggcgtctctcggccgcgaagtgcccgggcggcttcctcccggtgtagcctcgggctggtgcccccggcagcaggagcgcgacacaggcggcccgaaggagcagtccggcccacatgaccggcggcggcgggtcccccgggctgggctcggctcctgcgccgcgcgcgggagagggggctgccggccctcgcccctcctcctggcgccgtggggagcgaaccagcgatccccgaaatggcacgcagagctgagcaggggggcttgggacgccgagaggaggggccgagggccgcgaggggacgcggcggacgattgtggggagggtctctggcacctcgaagcgaaacacacaaaggcaacgccgcccgcctgctgatgcctctccgagaggcgc

SEQ ID NO: 9736 - RNA, 3197 nt, Homo sapiens
  source 1..3197: mol_type = other RNA
atgcgaggatgctgacagtggaaacgacttcctccattcttacagcacattccaaacacttcttgggaacaaggttacatccagccttgggggtcttccatcctcaccagggcccctgcaggagggagcccaggcatccccaccaggttcatccttggagctgccctgcacacaccctgggccactggcagaggtcctctctccagagtctcccggacacagtgacctccttacatggtggactcttccccccgagaagcccccactgggggctgctgggggccagggtgggtggtggctgcaagggctgtggagagtctagaggtggtgggagaaagcacgcgaggcccgaggagggtgatgggggtcttcgaggggctggggtccatcatggaaagtgctgaagcttccgtcaggagggtgccaggcagaggaggccacctggacactatctgggccccagaggctgagaacgagcgctctggagtcacaggaggtggctgaggagcccctggggaagctagaggtagagtgggggctcctggaggggtcgaaggccctggtgagagtcgaggggaggccccaggctcccctgggaaagtggctgtcagccccaaagcgagtgagtgtggaccatgagctcctgccgggcttgtaggtaaagtctgtgttttcatcaagttcgttcttaaaaggagctggaggagatgaagcaccggcctcgagggtgatgctgtcgggggcccaggacaggagctacagttgacaggggcctcagtgtctccatgcaggctccgaccagctttgctgaatgccacatttccgtgaggggagagcccctgcttttcttccagaggagacagggaatctggacaggaagagcagcagtccccaggaagcagggcagggtcggcacaggcccgctggcagggaaccttctcacagctcacctctcccagctggcacgtgcaccgggtgcagggttcatcatccaaggtgaacacctggccattcgccaccttccttccctcgtagttgcagtctcggcacacggggcagcactccccgtcagggtggaaagggtaggtacaggtgatggggcagtccacgggggaacaggccactgagcccagctggcagatgcataactcacaggggtcaccaggcgaccagatctgtccaatcggaaactcaaccccgttgtcgtcaagagagcagcctgtcgagggtgtgggctcctggcaggtgaagcaacactgcccagggcccagccgccactcttctcgggggcaggccagctcagggcagggcatgaaggagcactccacctccccattctggcaaacacaggtggtacactcgtcaccacccccactgaacacagccccgtctgcgtaccaccggccgtggaaatagcatctcactggaacacaagtacagcaatccgtctgtgggggggtctgacaggggccagaaggacactcaggagagatgcaggacacgtttccagccagacagacacagacggtgcagttctcattgggaggtgaaaacacatccccttcagctcggacgacaccactgtgaaaacagcctgtgcacgatgggcagcacccaccatctctggagggaattgggtgggaacaagcagcttcacacctcaccttttcacaggtcaccttcccgtcctcgcaccagcactgggaacacccaggctctgtccagcgactccttgattcatgcatggctcccaggtgccagcagggagagggccctgctgccagtcggggggactcagggcccctgggtgaggaaggggtccccatcacctccccctgaaggagtgaggggggtctgaggttccccagcagggaggcagtaggcactggggtggccagcagggtggacagcagccacacaggggcagaaggggaggatgtgggtagtcgtggggtgggagatggcaggcgggtggtcctgactccggctgggggccctggagccccagaaggagggctatgtcctggggacagggcaggccggccggcctcaggaagcaacagaagcatcttggacgggtgttgccggggttgcaggatggcagatggggccagcacggctttcgggaaagcttcacaggacacgcggtcagctcggagcctgaagccaggtcggcatgtgcataggaagctgcccacggtgttgtggcaggaatggtgacagactcgcctctccaatggcctccgacactcgtttacatctacacaggagtgccggttgccatgaaggtggaagccagttcgacaggaacacttgtagctgccaatgctgtttttacatctctgctgacagggagtccctaggcattcgtcagtgtcttggcagctgtggcggtcggcagacagctgcatgcccggcccacactcgcacacaaacccaccttctgtgttcacacagtggccctcgcaggaggaggttacacattcgtcaatgtctgtacacctgatgccaacagctgtctccgtcatcgagaagcccacggggcacactcgggccacctcctgacagcctccatggttgcaggtaaggtcacagccgtactccccacatggtccatgggtttctgggcaggtggccccttgctctccatcctggcaggagcagacattgggagcgatgcagatgccactcccacagccgaaggagcagaggggcagggtgcagtgcccaccacccatagagggcgcccagccagggcagcagccactcccaaacccagagaggcagacgtgggggcccagtcggcgtctctcggccgcgaagtgcccgggcggcttcctcccggtgtagcctcgggctggtgcccccggcagcaggagcgcgacacaggcggcccgaaggagcagtccggcccacatgaccggcggcggcgggtcccccgggctgggctcggctcctgcgccgcgcgcgggagagggggctgccggccctcgcccctcctcctggcgccgtggggagcgaaccagcgatccccgaaatggcacgcagagctgagcaggggggcttgggacgccgagaggaggggccgagggccgcgaggggacgcggcggacgattgtggggagggtctctggcacctcgaagcgaaacacacaaaggcaacgccgcccgcctgctgatgcctctccgagaggcgc

SEQ ID NO: 9737 - RNA, 5669 nt, Homo sapiens
  source 1..5669: mol_type = other RNA
atggggtgagatggggaggagcagcacccaccgcgaaggtgtccacggccaaggtcgggcgcccgggccgcccaggcactgcggcggggacgagcggccaggaggcagctcagcgtggaactgtagccccgccgcccccgcccccccctgcctgggctttttagataaaatccaggacttcatggacatttcccgcatgggaccgtttcagagtcatttgctcatcccacgagtttttactgcgcatctacaatggggtgcacagtgtcccctcggcactggggagaggcagggaacaggtggagaagtctccctttttcctggagcttagacttcagaggagagaagaagaagatgagtaagcaactaagcaaacaagataattttagacagtgatgtgttctgtgaagaaaagaaatgggaagaatgtgacggagaggactgtgaggaacctactttccactgggatgcagggaggcccctctgccgaggggatgtaggtttaacaaaattaatgctaaaattctatattttcaatgtcaacaatattttgtgggaaacattgataccatttaaaaagatctgattatttagaatctgtggcagttttttttgtcgttgttgttactgtggttgtttgttgtttttattgtttttagattaggcaacagtttaaaaaatctgttcaacaggggttgtggaagaatgtgccgtttgggatagagcctagggaggaaaacaaatgttgttctcctgaagagcaaggaagggctaatgcagacagaagatgatgctaataaaatatcattaaggcttatttcgttacagctattatgaaaccagattttttttcttttaacttttttgagatggagtctcactctgttgcccagcggggagtacagtagcgctgtctcagctcactacagcctctgtctcccaggttcaagtgattttcctgcctcagcctcccgagtagctgggactacaggtgcacaccaccacacccggctaatttttgtatttttagtacagacagggtttcaccatgttggccaggctggtctcgaactcctgacctcaagtgatccacctgcctcagcctcccacagtactgggattatagatgtgagccaacgtgcctggccgaaactggtttattgaatgaactaagtccagaaagcgagggcttcatttttctctaaccattgccttacaacaaagttctgttggatctcctcccatcatcactcctgaatcttgggcagataccataaattttagtgacaaatctcactttagtcattgcacctctatttaagggattaaaatgtccaggccagtccaatttaacagcaatctcacacctcattcaaaaatctgcttggccttccttgcagtgaaatgacgaaggcatatagtcagtttctttactcttcctccattgtctctgtcttctctatattctagatgtccctatgccattgcaagggaagagggtattacacaaagaggagcagatcttcctgtagttaactattgaataaggcagacaggccagcatgatcctgccagctgctatggcagagtccaaatgctggctttttcatagggcacatctgtgagttattggagggccttgagtgtaccccacattgcacagttccatgatgcagggccacattatctggctgacctcttgcagcaacctccaccccaaacccctcttctgcctaaccccgtgtcctcttactgctatagtttctttgcacaacaggctaccctgttggctgatatcccgtcatgacaatgcaagcccagctactcttccatagtcaaagccatgtgaagaaattcacatccttttaccatgtcaataatgggagggcaggttgctatcagtgcttctcttctctcatcctgccattttgggtgctcaagccaacctttcacctcctgaattccccaggggggaagaactcatctattcattcaacaaatattcatcaagcacttgtatttgccaaacactatttaccagtctctgtgttcccagtgcccaccctcggactccagcaaacactcatcaagctcttccaagaattctcaagccacaccacatctgctgcactgaacctgtgtgctcctgttactctgcaagctttcagtcttggagtgggatgccaggctaccttctaccatgctgagtccctcacacttgtctgcaagaaattcaaagcaatctccctatggcctagaacctccgcttaatgactctttaatcacgcttttgactctagtcttctagagatggataatacggactgggagtcattggtctctttctgctcttttgataagtccagactggctgtgtctagtatcatgttggtgcagttactgtctttcgtcagctttgagcctttagccagaattctaagacaaccagaaaagtcccattcaatatccagctgcaaataaatttggccgagttttcttggaaagcaggtggatccacgtctttcacctcaacagcttatgattaagtccatatatccctttacatacatacactatcaagtcatgagtcctcattggttaattacatatttgtgtagcaggataaaaaattaaataagctattacacatatgtgaaacaaaagacttttttatatgccgtagctgatctaattttttccccaagccccagacttgaagagaatgatgacactgacccaaagaccaatatgattcacagggcactccgaggactggtgcatatgatgctgaagttgactgttcccttgctgccatgaagccatataaactcttgctcacaacagaatccatttgggaaagcagagtggagaggagctgaaaaactgagcatttactcaaaagagactgtttcaatttgaaacataatgattaaaccagaagagactgggctgtctctaactggcaggctaacctcaccgcctagctcagttccccagatgaaacattgtttttgttaagtctttcctgaaggcatgaggataatggaggcacctccagacagttacttacgactgtactattcaccatcatccaagtaaataatggtttcttaagttgaatttcctaaatttttttaagatttcacatcattgttttcagtgactagtgttaatttcatattaaaagcggctctaatgttagcccaaaagagcccacgtttgcttttctccttgggccactgcaaataagtccgctgcgtcatgagagccttcagcttgtggtacttgttgggaatgctgttctgtggaatgggttccagtaagatgaggattaagttattagatccttcatgaaagagattgtgatgggcaaaatagagttcgtaatggcaccactcactctggacaaagttgggagacaaaacaaagatggacttgtaactcttctcaatgcagttgatgatattttccacaatgctcttgccagggacaaagtttctctcatgaagacaaatctgtatatcttctttttctaggtaaggtaccaattcacttttcacccaggcagaatcatgttcactatatgaaataaaagcatgaaactggaggtttctttggagttcttctaagggtatgttcctggccctgcgccgagtctgggtccactggcacaccatcctgagataccagggcagatccaagtagatgcagagggaggtcacagtcacagccaacaccagcatggtggcaccgatggtgacgatcagcagagttatgttgcaggataattcagacatgtgaaagtcctttagtgggcttcctctataactttctgggtagtcacacttataagaatcaggccagccctctaacacttcacttgatacttggtctatatttttgacaaattctcttagctcacaggtacattggaatggattgtcccctgcttttattgacctcatcttctggcagctctggaagaaatcagccgatgggtgggaaactgaattgtgatcaatgatcaatacagaaaggctgctaaagctgccacatccaggaaggtcagttaaagaattgaaagcaacattgagttcttgcaaagcttccagttttacgacttgtttaggaacgctctttattttattgctgtgaagatcaagtaccttgatcctgggaggtaaacatctgaaaacagagtcagtaagcatatttgaagacaaatttaacaccactatactctcaacccaagtgcagttttctttatgtctaccagattccaaagaattccagctaacatccagtatttccaaagaaggcatatccttcgtcatgagacctactttgaaaaggtcttttaatccattcttttgtaagataagtgtctccaatttaactaacgtggaacatttttcaaaaatactatctgtgaaaacgttctgggtaaagttcaaaaacttgaatgtgcttggtgcatgaggacacagcatgtgtataaaaggtgtatctgaaatggttaacatcataatgttcatctcagaaaacacggtgtacaaagctgtctgtgaaaacagaaaaacttggttcgtgatatgttctattgtcaatgctttcaatgtcgttttagaataagtaaaatcttcttcacgaatgctttcaattattgttaaattgtaaatattgagatattccacaggtttgggccaaagaaattgaaagactctgaccaggcatttccaagtcgtttctatgtggttgagggtaaaattcagtaaggttgaacctctggtgagttctgataaaaatttaatgaaaacttgacagttgtcatcattcaatttaatattagtcagttgtaagcaccctaaagtattaactgatatgttcacttggatagcgaataaactagttgggtgaaaaacaaggtgaagggtttttgcattcagaatttgtagactttctgtctcattttcttttatataataatttcttaaatccagaaggatataacttagatgcaagtgagcaattggcagcaaatctaatttttgcagcttcatagcactcaatcccaagaaattcagttgtgataagttgccaaattccttacagatgggcagggccttgaaatcattgaatgagagatctaaatgcctgaaactcacaataggatggcaggatatcttttgcaactgattatgagataaatccaaatattctaaatcctggttgaacttgaaaacacttaaatcaagtagctggattctgttatgggaaagtctcaaaactgtcaactctgatagaaagctcatgtcagagacctgaagctcagcgatgtagttctgagacatatctaagactttggttttcagcggtaggtcttttggaacatgaataagacctctttttgacttgtctactgcaaattcatttccgtcggagaactggattctggttccaactattatgatcataaggcaaacaaaatggaagcttttaacaataggttctttgtctttggtcatgatgttgcagtggctatcctaaagggttgttcttcttcagagcatcttgatatgagtccaaattaatttggctaatgacaaagttggacatctccgtaagaatcacttctgctttcaggaggaagagaaaggctggcttcttgt

SEQ ID NO: 9738 - RNA, 5646 nt, Homo sapiens
  source 1..5646: mol_type = other RNA
atggggtgagatggggaggagcagcacccaccgcgaaggtgtccacggccaaggtcgggcgcccgggccgcccaggcactgcggcggggacgagcggccaggaggcagctcagcgtggaactgtagccccgccgcccccgcccccccctgcctgggctttttagataaaatccaggacttcatggacatttcccgcatgggaccgtttcagagtcatttgctcatcccacgagtttttactgcgcatctacaatggggtgcacagtgtcccctcggcactggggagaggcagggaacaggtggagaagtctccctttttcctggagcttagacttcagaggagagaagaagaagatgagtaagcaactaagcaaacaagataattttagacagtgatgtgttctgtgaagaaaagaaatgggaagaatgtgacggagaggactgtgaggaacctactttccactgggatgcagggaggcccctctgccgaggggatgtaggtttaacaaaattaatgctaaaattctatattttcaatgtcaacaatattttgtgggaaacattgataccatttaaaaagatctgattatttagaatctgtggcagttttttttgtcgttgttgttactgtggttgtttgttgtttttattgtttttagattaggcaacagtttaaaaaatctgttcaacaggggttgtggaagaatgtgccgtttgggatagagcctagggaggaaaacaaatgttgttctcctgaagagcaaggaagggctaatgcagacagaagatgatgctaataaaatatcattaaggcttatttcgttacagctattatgaaaccagattttttttcttttaacttttttgagatggagtctcactctgttgcccagcggggagtacagtagcgctgtctcagctcactacagcctctgtctcccaggttcaagtgattttcctgcctcagcctcccgagtagctgggactacaggtgcacaccaccacacccggctaatttttgtatttttagtacagacagggtttcaccatgttggccaggctggtctcgaactcctgacctcaagtgatccacctgcctcagcctcccacagtactgggattatagatgtgagccaacgtgcctggccgaaactggtttattgaatgaactaagtccagaaagcgagggcttcatttttctctaaccattgccttacaacaaagttctgttggatctcctcccatcatcactcctgaatcttgggcagataccataaattttagtgacaaatctcactttagtcattgcacctctatttaagggattaaaatgtccaggccagtccaatttaacagcaatctcacacctcattcaaaaatctgcttggccttccttgcagtgaaatgacgaaggcatatagtcagtttctttactcttcctccattgtctctgtcttctctatattctagatgtccctatgccattgcaagggaagagggtattacacaaagaggagcagatcttcctgtagttaactattgaataaggcagacaggccagcatgatcctgccagctgctatggcagagtccaaatgctggctttttcatagggcacatctgtgagttattggagggccttgagtgtaccccacattgcacagttccatgatgcagggccacattatctggctgacctcttgcagcaacctccaccccaaacccctcttctgcctaaccccgtgtcctcttactgctatagtttctttgcacaacaggctaccctgttggctgatatcccgtcatgacaatgcaagcccagctactcttccatagtcaaagccatgtgaagaaattcacatccttttaccatgtcaataatgggagggcaggttgctatcagtgcttctcttctctcatcctgccattttgggtgctcaagccaacctttcacctcctgaattccccaggggggaagaactcatctattcattcaacaaatattcatcaagcacttgtatttgccaaacactatttaccagtctctgtgttcccagtgcccaccctcggactccagcaaacactcatcaagctcttccaagaattctcaagccacaccacatctgctgcactgaacctgtgtgctcctgttactctgcaagctttcagtcttggagtgggatgccaggctaccttctaccatgctgagtccctcacacttgtctgcaagaaattcaaagcaatctccctatggcctagaacctccgcttaatgactctttaatcacgcttttgactctagtcttctagagatggataatacggactgggagtcattggtctctttctgctcttttgataagtccagactggctgtgtctagtatcatgttggtgcagttactgtctttcgtcagctttgagcctttagccagaattctaagacaaccagaaaagtcccattcaatatccagctgcaaataaatttggccgagttttcttggaaagcaggtggatccacgtctttcacctcaacagcttatgattaagtccatatatccctttacatacatacactatcaagtcatgagtcctcattggttaattacatatttgtgtagcaggataaaaaattaaataagctattacacatatgtgaaacaaaagacttttttatatgccgtagctgatctaattttttccccaagccccagacttgaagagaatgatgacactgacccaaagaccaatatgattcacagggcactccgaggactggtgcatatgatgctgaagttgactgttcccttgctgccatgaagccatataaactcttgctcacaacagaatccatttgggaaagcagagtggagaggagctgaaaaactgagcatttactcaaaagagactgtttcaatttgaaacataatgattaaaccagaagagactgggctgtctctaactggcaggctaacctcaccgcctagctcagttccccagatgaaacattgtttttgttaagtctttcctgaaggcatgaggataatggaggcacctccagacagttacttacgactgtactattcaccatcatccaagtaaataatggtttcttaagttgaatttcctaaatttttttaagatttcacatcattgttttcagtgactagtgttaatttcatattaaaagcggctctaatgttagcccaaaagagcccacgtttgcttttctccttgggccactgcaaataagtccgctgcgtcatgagagccttcagcttgtggtacttgttgggaatgctgttctgtggaatgggttccagtaagatgaggattaagttattagatccttcatgaaagagattgtgatgggcaaaatagagttcgtaatggcaccactcactctggacaaagttgggagacaaaacaaagatggacttgtaactcttctcaatgcagttgatgatattttccacaatgctcttgccagggacaaagtttctctcatgaagacaaatctgtatatcttctttttctaggtaaggtaccaattcacttttcacccaggcagaatcatgttcactatatgaaataaaagcatgaaactggaggtttctttggagttcttctaagggtatgttcctggccctgcgccgagtctgggtccactggcacaccatcctgagataccagggcagatccaagtagatgcagagggaggtcacagtcacagccaacaccagcatggtggcaccgatggtgacgatcagcagagttatgttgcaggataattcagacatgtgaaagtcctttagtgggcttcctctataactttctgggtagtcacacttataagaatcaggccagccctctaacacttcacttgatacttggtctatatttttgacaaattctcttagctcacaggtacattggaatggattgtcccctgcttttattgacctcatcttctggcagctctggaagaaatcagccgatgggtgggaaactgaattgtgatcaatgatcaatacagaaaggctgctaaagctgccacatccaggaaggtcagttaaagaattgaaagcaacattgagttcttgcaaagcttccagttttacgacttgtttaggaacgctctttattttattgctgtgaagatcaagtaccttgatcctgggaggtaaacatctgaaaacagagtcagtaagcatatttgaagacaaatttaacaccactatactctcaacccaagtgcagttttctttatgtctaccagattccaaagaattccagctaacatccagtatttccaaagaaggcatatccttcgtcatgagacctactttgaaaaggtcttttaatccattcttttgtaagataagtgtctccaatttaactaacgtggaacatttttcaaaaatactatctgtgaaaacgttctgggtaaagttcaaaaacttgaatgtgcttggtgcatgaggacacagcatgtgtataaaaggtgtatctgaaatggttaacatcataatgttcatctcagaaaacacggtgtacaaagctgtctgtgaaaacagaaaaacttggttcgtgatatgttctattgtcaatgctttcaatgtcgttttagaataagtaaaatcttcttcacgaatgctttcaattattgttaaattgtaaatattgagatattccacaggtttgggccaaagaaattgaaagactctgaccaggcatttccaagtcgtttctatgtggttgagggtaaaattcagtaaggttgaacctctggtgagttctgataaaaatttaatgaaaacttgacagttgtcatcattcaatttaatattagtcagttgtaagcaccctaaagtattaactgatatgttcacttggatagcgaataaactagttgggtgaaaaacaaggtgaagggtttttgcattcagaatttgtagactttctgtctcattttcttttatataataatttcttaaatccagaaggatataacttagatgcaagtgagcaattggcagcaaatctaatttttgcagcttcatagcactcaatcccaagaaattcagttgtgataagttgccaaattccttacagatgggcagggccttgaaatcattgaatgagagatctaaatgcctgaaactcacaataggatggcaggatatcttttgcaactgattatgagataaatccaaatattctaaatcctggttgaacttgaaaacacttaaatcaagtagctggattctgttatgggaaagtctcaaaactgtcaactctgatagaaagctcatgtcagagacctgaagctcagcgatgtagttctgagacatatctaagactttggttttcagcggtaggtcttttggaacatgaataagacctctttttgacttgtctactgcaaattcatttccgtcggagaactggattctggttccaactattatgatcataaggcaaacaaaatggaagcttttaacaataggttctttgtctttggtcatgatgttgcagtggctatcctaaagggttgttcttcttcagagcatcttgatatgagtccaaattcaagatctctttttcagaagaagagaaaataacttgtaaatgaacggaaatacaatt

SEQ ID NO: 9739 - RNA, 6032 nt, Homo sapiens
  source 1..6032: mol_type = other RNA
atggggtgagatggggaggagcagcacccaccgcgaaggtgtccacggccaaggtcgggcgcccgggccgcccaggcactgcggcggggacgagcggccaggaggcagctcagcgtggaactgtagccccgccgcccccgcccccccctgcctgggctttttagataaaatccaggacttcatggacatttcccgcatgggaccgtttcagagtcatttgctcatcccacgagtttttactgcgcatctacaatggggtgcacagtgtcccctcggcactggggagaggcagggaacaggtggagaagtctccctttttcctggagcttagacttcagaggagagaagaagaagatgagtaagcaactaagcaaacaagataattttagacagtgatgtgttctgtgaagaaaagaaatgggaagaatgtgacggagaggactgtgaggaacctactttccactgggatgcagggaggcccctctgccgaggggatgtaggtttaacaaaattaatgctaaaattctatattttcaatgtcaacaatattttgtgggaaacattgataccatttaaaaagatctgattatttagaatctgtggcagttttttttgtcgttgttgttactgtggttgtttgttgtttttattgtttttagattaggcaacagtttaaaaaatctgttcaacaggggttgtggaagaatgtgccgtttgggatagagcctagggaggaaaacaaatgttgttctcctgaagagcaaggaagggctaatgcagacagaagatgatgctaataaaatatcattaaggcttatttcgttacagctattatgaaaccagattttttttcttttaacttttttgagatggagtctcactctgttgcccagcggggagtacagtagcgctgtctcagctcactacagcctctgtctcccaggttcaagtgattttcctgcctcagcctcccgagtagctgggactacaggtgcacaccaccacacccggctaatttttgtatttttagtacagacagggtttcaccatgttggccaggctggtctcgaactcctgacctcaagtgatccacctgcctcagcctcccacagtactgggattatagatgtgagccaacgtgcctggccgaaactggtttattgaatgaactaagtccagaaagcgagggcttcatttttctctaaccattgccttacaacaaagttctgttggatctcctcccatcatcactcctgaatcttgggcagataccataaattttagtgacaaatctcactttagtcattgcacctctatttaagggattaaaatgtccaggccagtccaatttaacagcaatctcacacctcattcaaaaatctgcttggccttccttgcagtgaaatgacgaaggcatatagtcagtttctttactcttcctccattgtctctgtcttctctatattctagatgtccctatgccattgcaagggaagagggtattacacaaagaggagcagatcttcctgtagttaactattgaataaggcagacaggccagcatgatcctgccagctgctatggcagagtccaaatgctggctttttcatagggcacatctgtgagttattggagggccttgagtgtaccccacattgcacagttccatgatgcagggccacattatctggctgacctcttgcagcaacctccaccccaaacccctcttctgcctaaccccgtgtcctcttactgctatagtttctttgcacaacaggctaccctgttggctgatatcccgtcatgacaatgcaagcccagctactcttccatagtcaaagccatgtgaagaaattcacatccttttaccatgtcaataatgggagggcaggttgctatcagtgcttctcttctctcatcctgccattttgggtgctcaagccaacctttcacctcctgaattccccaggggggaagaactcatctattcattcaacaaatattcatcaagcacttgtatttgccaaacactatttaccagtctctgtgttcccagtgcccaccctcggactccagcaaacactcatcaagctcttccaagaattctcaagccacaccacatctgctgcactgaacctgtgtgctcctgttactctgcaagctttcagtcttggagtgggatgccaggctaccttctaccatgctgagtccctcacacttgtctgcaagaaattcaaagcaatctccctatggcctagaacctccgcttaatgactctttaatcacgcttttgactctagtcttctagagatggataatacggactgggagtcattggtctctttctgctcttttgataagtccagactggctgtgtctagtatcatgttggtgcagttactgtctttcgtcagctttgagcctttagccagaattctaagacaaccagaaaagtcccattcaatatccagctgcaaataaatttggccgagttttcttggaaagcaggtggatccacgtctttcacctcaacagcttatgattaagtccatatatccctttacatacatacactatcaagtcatgagtcctcattggttaattacatatttgtgtagcaggataaaaaattaaataagctattacacatatgtgaaacaaaagacttttttatatgccgtagctgatctaattttttccccaagccccagacttgaagagaatgatgacactgacccaaagaccaatatgattcacagggcactccgaggactggtgcatatgatgctgaagttgactgttcccttgctgccatgaagccatataaactcttgctcacaacagaatccatttgggaaagcagagtggagaggagctgaaaaactgagcatttactcaaaagagactgtttcaatttgaaacataatgattaaaccagaagagactgggctgtctctaactggcaggctaacctcaccgcctagctcagttccccagatgaaacattgtttttgttaagtctttcctgaaggcatgaggataatggaggcacctccagacagttacttacgactgtactattcaccatcatccaagtaaataatggtttcttaagttgaatttcctaaatttttttaagatttcacatcattgttttcagtgactagtgttaatttcatattaaaagcggctctaatgttagcccaaaagagcccacgtttgcttttctccttgggccactgcaaataagtccgctgcgtcatgagagccttcagcttgtggtacttgttgggaatgctgttctgtggaatgggttccagtaagatgaggattaagttattagatccttcatgaaagagattgtgatgggcaaaatagagttcgtaatggcaccactcactctggacaaagttgggagacaaaacaaagatggacttgtaactcttctcaatgcagttgatgatattttccacaatgctcttgccagggacaaagtttctctcatgaagacaaatctgtatatcttctttttctaggtaaggtaccaattcacttttcacccaggcagaatcatgttcactatatgaaataaaagcatgaaactggaggtttctttggagttcttctaagggtatgttcctggccctgcgccgagtctgggtccactggcacaccatcctgagataccagggcagatccaagtagatgcagagggaggtcacagtcacagccaacaccagcatggtggcaccgatggtgacgatcagcagagttatgttgcaggataattcagacatgtgaaagtcctttagtgggcttcctctataactttctgggtagtcacacttataagaatcaggccagccctctaacacttcacttgatacttggtctatatttttgacaaattctcttagctcacaggtacattggaatggattgtcccctgcttttattgacctcatcttctggcagctctggaagaaatcagccgatgggtgggaaactgaattgtgatcaatgatcaatacagaaaggctgctaaagctgccacatccaggaaggtcagttaaagaattgaaagcaacattgagttcttgcaaagcttccagttttacgacttgtttaggaacgctctttattttattgctgtgaagatcaagtaccttgatcctgggaggtaaacatctgaaaacagagtcagtaagcatatttgaagacaaatttaacaccactatactctcaacccaagtgcagttttctttatgtctaccagattccaaagaattccagctaacatccagtatttccaaagaaggcatatccttcgtcatgagacctactttgaaaaggtcttttaatccattcttttgtaagataagtgtctccaatttaactaacgtggaacatttttcaaaaatactatctgtgaaaacgttctgggtaaagttcaaaaacttgaatgtgcttggtgcatgaggacacagcatgtgtataaaaggtgtatctgaaatggttaacatcataatgttcatctcagaaaacacggtgtacaaagctgtctgtgaaaacagaaaaacttggttcgtgatatgttctattgtcaatgctttcaatgtcgttttagaataagtaaaatcttcttcacgaatgctttcaattattgttaaattgtaaatattgagatattccacaggtttgggccaaagaaattgaaagactctgaccaggcatttccaagtcgtttctatgtggttgagggtaaaattcagtaaggttgaacctctggtgagttctgataaaaatttaatgaaaacttgacagttgtcatcattcaatttaatattagtcagttgtaagcaccctaaagtattaactgatatgttcacttggatagcgaataaactagttgggtgaaaaacaaggtgaagggtttttgcattcagaatttgtagactttctgtctcattttcttttatataataatttcttaaatccagaaggatataacttagatgcaagtgagcaattggcagcaaatctaatttttgcagcttcatagcactcaatcccaagaaattcagttgtgataagttgccaaattccttacagatgggcagggccttgaaatcattgaatgagagatctaaatgcctgaaactcacaataggatggcaggatatcttttgcaactgattatgagataaatccaaatattctaaatcctggttgaacttgaaaacacttaaatcaagtagctggattctgttatgggaaagtctcaaaactgtcaactctgatagaaagctcatgtcagagacctgaagctcagcgatgtagttctgagacatatctaagactttggttttcagcggtaggtcttttggaacatgaataagacctctttttgacttgtctactgcaaattcatttccgtcggagaactggattctggttccaactattatgatcataaggcaaacaaaatggaagcttttaacaataggttctttgtctttggtcatgatgttgcagtggctatcctaaagggttgttcttcttcagagcatcttgatatgagtccaaattcgatatggacagcgactggaatactggtagcggtgttcatcaggaattgcagtttttatacacaatatatacaaagtatatatcggtcaaagtactagagagttgggcaacgataggagaagctactactttatactggttatatggtcaaaacaaatagttcacaatgaagatgtaacagataagaacagttatgcagcaagtaatattgcatcaaaatttacaaagtaaaaaatgttacaaaacacatggagacattgtgagtaaaagtatttagcatatttctctgggtcactgttagatcaagtagcaaaaaataaaaacatatatggaaatttgaatgagaaattaataaaggatttaatagagacataagctgtaccctacaaaaagagaacatcatatgtctaagtctctagagttcatagagcatttactaaaat

SEQ ID NO: 9740 - RNA, 5631 nt, Homo sapiens
  source 1..5631: mol_type = other RNA
atggggtgagatggggaggagcagcacccaccgcgaaggtgtccacggccaaggtcgggcgcccgggccgcccaggcactgcggcggggacgagcggccaggaggcagctcagcgtggaactgtagccccgccgcccccgcccccccctgcctgggctttttagataaaatccaggacttcatggacatttcccgcatgggaccgtttcagagtcatttgctcatcccacgagtttttactgcgcatctacaatggggtgcacagtgtcccctcggcactggggagaggcagggaacaggtggagaagtctccctttttcctggagcttagacttcagaggagagaagaagaagatgagtaagcaactaagcaaacaagataattttagacagtgatgtgttctgtgaagaaaagaaatgggaagaatgtgacggagaggactgtgaggaacctactttccactgggatgcagggaggcccctctgccgaggggatgtaggtttaacaaaattaatgctaaaattctatattttcaatgtcaacaatattttgtgggaaacattgataccatttaaaaagatctgattatttagaatctgtggcagttttttttgtcgttgttgttactgtggttgtttgttgtttttattgtttttagattaggcaacagtttaaaaaatctgttcaacaggggttgtggaagaatgtgccgtttgggatagagcctagggaggaaaacaaatgttgttctcctgaagagcaaggaagggctaatgcagacagaagatgatgctaataaaatatcattaaggcttatttcgttacagctattatgaaaccagattttttttcttttaacttttttgagatggagtctcactctgttgcccagcggggagtacagtagcgctgtctcagctcactacagcctctgtctcccaggttcaagtgattttcctgcctcagcctcccgagtagctgggactacaggtgcacaccaccacacccggctaatttttgtatttttagtacagacagggtttcaccatgttggccaggctggtctcgaactcctgacctcaagtgatccacctgcctcagcctcccacagtactgggattatagatgtgagccaacgtgcctggccgaaactggtttattgaatgaactaagtccagaaagcgagggcttcatttttctctaaccattgccttacaacaaagttctgttggatctcctcccatcatcactcctgaatcttgggcagataccataaattttagtgacaaatctcactttagtcattgcacctctatttaagggattaaaatgtccaggccagtccaatttaacagcaatctcacacctcattcaaaaatctgcttggccttccttgcagtgaaatgacgaaggcatatagtcagtttctttactcttcctccattgtctctgtcttctctatattctagatgtccctatgccattgcaagggaagagggtattacacaaagaggagcagatcttcctgtagttaactattgaataaggcagacaggccagcatgatcctgccagctgctatggcagagtccaaatgctggctttttcatagggcacatctgtgagttattggagggccttgagtgtaccccacattgcacagttccatgatgcagggccacattatctggctgacctcttgcagcaacctccaccccaaacccctcttctgcctaaccccgtgtcctcttactgctatagtttctttgcacaacaggctaccctgttggctgatatcccgtcatgacaatgcaagcccagctactcttccatagtcaaagccatgtgaagaaattcacatccttttaccatgtcaataatgggagggcaggttgctatcagtgcttctcttctctcatcctgccattttgggtgctcaagccaacctttcacctcctgaattccccaggggggaagaactcatctattcattcaacaaatattcatcaagcacttgtatttgccaaacactatttaccagtctctgtgttcccagtgcccaccctcggactccagcaaacactcatcaagctcttccaagaattctcaagccacaccacatctgctgcactgaacctgtgtgctcctgttactctgcaagctttcagtcttggagtgggatgccaggctaccttctaccatgctgagtccctcacacttgtctgcaagaaattcaaagcaatctccctatggcctagaacctccgcttaatgactctttaatcacgcttttgactctagtcttctagagatggataatacggactgggagtcattggtctctttctgctcttttgataagtccagactggctgtgtctagtatcatgttggtgcagttactgtctttcgtcagctttgagcctttagccagaattctaagacaaccagaaaagtcccattcaatatccagctgcaaataaatttggccgagttttcttggaaagcaggtggatccacgtctttcacctcaacagcttatgattaagtccatatatccctttacatacatacactatcaagtcatgagtcctcattggttaattacatatttgtgtagcaggataaaaaattaaataagctattacacatatgtgaaacaaaagacttttttatatgccgtagctgatctaattttttccccaagccccagacttgaagagaatgatgacactgacccaaagaccaatatgattcacagggcactccgaggactggtgcatatgatgctgaagttgactgttcccttgctgccatgaagccatataaactcttgctcacaacagaatccatttgggaaagcagagtggagaggagctgaaaaactgagcatttactcaaaagagactgtttcaatttgaaacataatgattaaaccagaagagactgggctgtctctaactggcaggctaacctcaccgcctagctcagttccccagatgaaacattgtttttgttaagtctttcctgaaggcatgaggataatggaggcacctccagacagttacttacgactgtactattcaccatcatccaagtaaataatggtttcttaagttgaatttcctaaatttttttaagatttcacatcattgttttcagtgactagtgttaatttcatattaaaagcggctctaatgttagcccaaaagagcccacgtttgcttttctccttgggccactgcaaataagtccgctgcgtcatgagagccttcagcttgtggtacttgttgggaatgctgttctgtggaatgggttccagtaagatgaggattaagttattagatccttcatgaaagagattgtgatgggcaaaatagagttcgtaatggcaccactcactctggacaaagttgggagacaaaacaaagatggacttgtaactcttctcaatgcagttgatgatattttccacaatgctcttgccagggacaaagtttctctcatgaagacaaatctgtatatcttctttttctaggtaaggtaccaattcacttttcacccaggcagaatcatgttcactatatgaaataaaagcatgaaactggaggtttctttggagttcttctaagggtatgttcctggccctgcgccgagtctgggtccactggcacaccatcctgagataccagggcagatccaagtagatgcagagggaggtcacagtcacagccaacaccagcatggtggcaccgatggtgacgatcagcagagttatgttgcaggataattcagacatgtgaaagtcctttagtgggcttcctctataactttctgggtagtcacacttataagaatcaggccagccctctaacacttcacttgatacttggtctatatttttgacaaattctcttagctcacaggtacattggaatggattgtcccctgcttttattgacctcatcttctggcagctctggaagaaatcagccgatgggtgggaaactgaattgtgatcaatgatcaatacagaaaggctgctaaagctgccacatccaggaaggtcagttaaagaattgaaagcaacattgagttcttgcaaagcttccagttttacgacttgtttaggaacgctctttattttattgctgtgaagatcaagtaccttgatcctgggaggtaaacatctgaaaacagagtcagtaagcatatttgaagacaaatttaacaccactatactctcaacccaagtgcagttttctttatgtctaccagattccaaagaattccagctaacatccagtatttccaaagaaggcatatccttcgtcatgagacctactttgaaaaggtcttttaatccattcttttgtaagataagtgtctccaatttaactaacgtggaacatttttcaaaaatactatctgtgaaaacgttctgggtaaagttcaaaaacttgaatgtgcttggtgcatgaggacacagcatgtgtataaaaggtgtatctgaaatggttaacatcataatgttcatctcagaaaacacggtgtacaaagctgtctgtgaaaacagaaaaacttggttcgtgatatgttctattgtcaatgctttcaatgtcgttttagaataagtaaaatcttcttcacgaatgctttcaattattgttaaattgtaaatattgagatattccacaggtttgggccaaagaaattgaaagactctgaccaggcatttccaagtcgtttctatgtggttgagggtaaaattcagtaaggttgaacctctggtgagttctgataaaaatttaatgaaaacttgacagttgtcatcattcaatttaatattagtcagttgtaagcaccctaaagtattaactgatatgttcacttggatagcgaataaactagttgggtgaaaaacaaggtgaagggtttttgcattcagaatttgtagactttctgtctcattttcttttatataataatttcttaaatccagaaggatataacttagatgcaagtgagcaattggcagcaaatctaatttttgcagcttcatagcactcaatcccaagaaattcagttgtgataagttgccaaattccttacagatgggcagggccttgaaatcattgaatgagagatctaaatgcctgaaactcacaataggatggcaggatatcttttgcaactgattatgagataaatccaaatattctaaatcctggttgaacttgaaaacacttaaatcaagtagctggattctgttatgggaaagtctcaaaactgtcaactctgatagaaagctcatgtcagagacctgaagctcagcgatgtagttctgagacatatctaagactttggttttcagcggtaggtcttttggaacatgaataagacctctttttgacttgtctactgcaaattcatttccgtcggagaactggattctggttccaactattatgatcataaggcaaacaaaatggaagcttttaacaataggttctttgtctttggtcatgatgttgcagtggctatcctaaagggttgttcttcttcagagcatcttgatatgagtccaaattctctgtaatcctagcactttgggaggccgaggtggatggatt

SEQ ID NO: 9741 - RNA, 6090 nt, Homo sapiens
  source 1..6090: mol_type = other RNA
atggggtgagatggggaggagcagcacccaccgcgaaggtgtccacggccaaggtcgggcgcccgggccgcccaggcactgcggcggggacgagcggccaggaggcagctcagcgtggaactgtagccccgccgcccccgcccccccctgcctgggctttttagataaaatccaggacttcatggacatttcccgcatgggaccgtttcagagtcatttgctcatcccacgagtttttactgcgcatctacaatggggtgcacagtgtcccctcggcactggggagaggcagggaacaggtggagaagtctccctttttcctggagcttagacttcagaggagagaagaagaagatgagtaagcaactaagcaaacaagataattttagacagtgatgtgttctgtgaagaaaagaaatgggaagaatgtgacggagaggactgtgaggaacctactttccactgggatgcagggaggcccctctgccgaggggatgtaggtttaacaaaattaatgctaaaattctatattttcaatgtcaacaatattttgtgggaaacattgataccatttaaaaagatctgattatttagaatctgtggcagttttttttgtcgttgttgttactgtggttgtttgttgtttttattgtttttagattaggcaacagtttaaaaaatctgttcaacaggggttgtggaagaatgtgccgtttgggatagagcctagggaggaaaacaaatgttgttctcctgaagagcaaggaagggctaatgcagacagaagatgatgctaataaaatatcattaaggcttatttcgttacagctattatgaaaccagattttttttcttttaacttttttgagatggagtctcactctgttgcccagcggggagtacagtagcgctgtctcagctcactacagcctctgtctcccaggttcaagtgattttcctgcctcagcctcccgagtagctgggactacaggtgcacaccaccacacccggctaatttttgtatttttagtacagacagggtttcaccatgttggccaggctggtctcgaactcctgacctcaagtgatccacctgcctcagcctcccacagtactgggattatagatgtgagccaacgtgcctggccgaaactggtttattgaatgaactaagtccagaaagcgagggcttcatttttctctaaccattgccttacaacaaagttctgttggatctcctcccatcatcactcctgaatcttgggcagataccataaattttagtgacaaatctcactttagtcattgcacctctatttaagggattaaaatgtccaggccagtccaatttaacagcaatctcacacctcattcaaaaatctgcttggccttccttgcagtgaaatgacgaaggcatatagtcagtttctttactcttcctccattgtctctgtcttctctatattctagatgtccctatgccattgcaagggaagagggtattacacaaagaggagcagatcttcctgtagttaactattgaataaggcagacaggccagcatgatcctgccagctgctatggcagagtccaaatgctggctttttcatagggcacatctgtgagttattggagggccttgagtgtaccccacattgcacagttccatgatgcagggccacattatctggctgacctcttgcagcaacctccaccccaaacccctcttctgcctaaccccgtgtcctcttactgctatagtttctttgcacaacaggctaccctgttggctgatatcccgtcatgacaatgcaagcccagctactcttccatagtcaaagccatgtgaagaaattcacatccttttaccatgtcaataatgggagggcaggttgctatcagtgcttctcttctctcatcctgccattttgggtgctcaagccaacctttcacctcctgaattccccaggggggaagaactcatctattcattcaacaaatattcatcaagcacttgtatttgccaaacactatttaccagtctctgtgttcccagtgcccaccctcggactccagcaaacactcatcaagctcttccaagaattctcaagccacaccacatctgctgcactgaacctgtgtgctcctgttactctgcaagctttcagtcttggagtgggatgccaggctaccttctaccatgctgagtccctcacacttgtctgcaagaaattcaaagcaatctccctatggcctagaacctccgcttaatgactctttaatcacgcttttgactctagtcttctagagatggataatacggactgggagtcattggtctctttctgctcttttgataagtccagactggctgtgtctagtatcatgttggtgcagttactgtctttcgtcagctttgagcctttagccagaattctaagacaaccagaaaagtcccattcaatatccagctgcaaataaatttggccgagttttcttggaaagcaggtggatccacgtctttcacctcaacagcttatgattaagtccatatatccctttacatacatacactatcaagtcatgagtcctcattggttaattacatatttgtgtagcaggataaaaaattaaataagctattacacatatgtgaaacaaaagacttttttatatgccgtagctgatctaattttttccccaagccccagacttgaagagaatgatgacactgacccaaagaccaatatgattcacagggcactccgaggactggtgcatatgatgctgaagttgactgttcccttgctgccatgaagccatataaactcttgctcacaacagaatccatttgggaaagcagagtggagaggagctgaaaaactgagcatttactcaaaagagactgtttcaatttgaaacataatgattaaaccagaagagactgggctgtctctaactggcaggctaacctcaccgcctagctcagttccccagatgaaacattgtttttgttaagtctttcctgaaggcatgaggataatggaggcacctccagacagttacttacgactgtactattcaccatcatccaagtaaataatggtttcttaagttgaatttcctaaatttttttaagatttcacatcattgttttcagtgactagtgttaatttcatattaaaagcggctctaatgttagcccaaaagagcccacgtttgcttttctccttgggccactgcaaataagtccgctgcgtcatgagagccttcagcttgtggtacttgttgggaatgctgttctgtggaatgggttccagtaagatgaggattaagttattagatccttcatgaaagagattgtgatgggcaaaatagagttcgtaatggcaccactcactctggacaaagttgggagacaaaacaaagatggacttgtaactcttctcaatgcagttgatgatattttccacaatgctcttgccagggacaaagtttctctcatgaagacaaatctgtatatcttctttttctaggtaaggtaccaattcacttttcacccaggcagaatcatgttcactatatgaaataaaagcatgaaactggaggtttctttggagttcttctaagggtatgttcctggccctgcgccgagtctgggtccactggcacaccatcctgagataccagggcagatccaagtagatgcagagggaggtcacagtcacagccaacaccagcatggtggcaccgatggtgacgatcagcagagttatgttgcaggataattcagacatgtgaaagtcctttagtgggcttcctctataactttctgggtagtcacacttataagaatcaggccagccctctaacacttcacttgatacttggtctatatttttgacaaattctcttagctcacaggtacattggaatggattgtcccctgcttttattgacctcatcttctggcagctctggaagaaatcagccgatgggtgggaaactgaattgtgatcaatgatcaatacagaaaggctgctaaagctgccacatccaggaaggtcagttaaagaattgaaagcaacattgagttcttgcaaagcttccagttttacgacttgtttaggaacgctctttattttattgctgtgaagatcaagtaccttgatcctgggaggtaaacatctgaaaacagagtcagtaagcatatttgaagacaaatttaacaccactatactctcaacccaagtgcagttttctttatgtctaccagattccaaagaattccagctaacatccagtatttccaaagaaggcatatccttcgtcatgagacctactttgaaaaggtcttttaatccattcttttgtaagataagtgtctccaatttaactaacgtggaacatttttcaaaaatactatctgtgaaaacgttctgggtaaagttcaaaaacttgaatgtgcttggtgcatgaggacacagcatgtgtataaaaggtgtatctgaaatggttaacatcataatgttcatctcagaaaacacggtgtacaaagctgtctgtgaaaacagaaaaacttggttcgtgatatgttctattgtcaatgctttcaatgtcgttttagaataagtaaaatcttcttcacgaatgctttcaattattgttaaattgtaaatattgagatattccacaggtttgggccaaagaaattgaaagactctgaccaggcatttccaagtcgtttctatgtggttgagggtaaaattcagtaaggttgaacctctggtgagttctgataaaaatttaatgaaaacttgacagttgtcatcattcaatttaatattagtcagttgtaagcaccctaaagtattaactgatatgttcacttggatagcgaataaactagttgggtgaaaaacaaggtgaagggtttttgcattcagaatttgtagactttctgtctcattttcttttatataataatttcttaaatccagaaggatataacttagatgcaagtgagcaattggcagcaaatctaatttttgcagcttcatagcactcaatcccaagaaattcagttgtgataagttgccaaattccttacagatgggcagggccttgaaatcattgaatgagagatctaaatgcctgaaactcacaataggatggcaggatatcttttgcaactgattatgagataaatccaaatattctaaatcctggttgaacttgaaaacacttaaatcaagtagctggattctgttatgggaaagtctcaaaactgtcaactctgatagaaagctcatgtcagagacctgaagctcagcgatgtagttctgagacatatctaagactttggttttcagcggtaggtcttttggaacatgaataagacctctttttgacttgtctactgcaaattcatttccgtcggagaactggattctggttccaactattatgatcataaggcaaacaaaatggaagcttttaacaataggttctttgtctttggtcatgatgttgcagtggctatcctaaagggttgttcttcttcagagcatcttgatatgagtccaaattctttctttggaagagtgaaaactctgagttggggaacttttattactgaatggcgtatggttaaaagctcttcactgatccatataacttctcccaactgcccatcagaacacccacagagacacacatacatttgaaaaatccacttggccactgaaaacaaagaagcacagaaatgtaatggcaggatccaggagcatcttcactcacaaaaatgtaactggaactgtgttagggcaaacctgccacactcaagctttgtctcaggaaaatagactccctgatgaaaggcagaaagaaatttgtcctctctctgtctctgattcaaacagtgaggatgagttccaactagtacttaatgagtagctaggcagtgtcccttttaccccaatggtactgacatgagtggatcagcatgctgagttttccttctacggactgccacactccattctccccaaactttacacttagtgatggacactaccaggtaagagctgg

SEQ ID NO: 9742 - RNA, 134 nt, Homo sapiens
  source 1..134: mol_type = other RNA
atggggtgagatggggaggagcagcctggttactttcaaacgagaaagaacggatatgttaagcgtggagggctcctaatggtagcggtttgattttcagtgagtttggcgcggtggagacgtcaccgcggtct

SEQ ID NO: 9743 - RNA, 3387 nt, Homo sapiens
  source 1..3387: mol_type = other RNA
atggtaccctggcatactgagtcttcgtctgactcaaatcagtcatttctctattaatgcttatgagcattcctgatgtaccatgtgctgtgctgagtgctgaggataccatgatgattaaaaataggcatgcttccatccctcactgagcttacagtttgtgggagaggctgacattaacaaaataatcacacaaaaatgtgttacaagctgatataagtgctgtcaaggagggatgcagggtcaggcatgtgacagaggaacttgacctggactggggtcagagaaggctctcaggaagagtcacttgagcctggagaacgaatagacaagatgggagagcctttccagacaggaggaacagcatgtgcaaaggcttcagggctggagggagcctggcacagtgcagaccaaaaggtcagggtgctggaacctagagagcaatggaagtgtgttttgggtgaggttagagagaggcaggcaaggtaggctttgtgggccacatgagcgagtttggatttaagcagggagataacttgattggatttgcatttgagaagcatattcttccatgaagccagcagggttgtaggtagcacaccttcctctgagagccacatcatcaccttgtctgcacctctggtttaggagcttcttttaatcagcttccttgaaagagtccggaagaaagtgagttttaggcttttcttcttggaggcagaaacagagtgggaacgagggttctcagcagacttttcttagagagagagaaagctgcgtccgtttgccaatttgtttagtcatcctgtattctgggcagattaggacgtagccaccgctgtccataaatccctcctggttggaggaattgcatcaccatgttttctcaagttaggaaactgtatgaaatttcatactgtcctgatcagccaccacctacagctaaaattatgacatggtttgatcatgatcagagaaatcatttccttttctggaggggtgatccttgccatgctggttctggggagcttgagaagctaaacttgacagggcagctgagactcttccggggccatctggcaagggtgatgccctgcacttggctcactgacgtcatctgggaaagcccggtggtggaagcgattcgctgtgcttgttggcaatagtgatgtgactatttcctgttcttcactggctgaaaggtgaaagcatgactcacgggaactgctttccccgggctgccaacatcacagcctttttgtaagctggaaataagtcagaggctgacaatttctttttcctaaatgtggacctacagaattaagaaagagctagcagtgttcctttggtgcctgttaaagttatttaaaggagcagaagcctattctgtgctcccagaagatgaaaaaaaagaaaaaataaagtaacaaaagccttttcaggattctgagcaaagagcctcctaaattaaaaaaataaataaataaaagtttttgaatgcaggggctggaagggaatggagaggtgagtgaagggttgctatcactggctgaaggccagacattgtactgggtgctgtgtgtacctgagtccatccctagtcctcagaaccttgtgaggatgatgttttccgttttatcagcagtgccatgagactcagaggttgagtttccccaagggtcatacaactagtaaatgttggagctgggatttgaaactagctgtttactaatctggcagcttacttaactacctaacttatctatctgattatttattaatacttaatgtacccaaccagcagcttatttaatctcttgtgccctaaatgtccttttctgccaaatggtgataaatcatagcaatttcacaggtggctgattaaatgagaaatgtgtggaagcagctagcactgtacctgacacctagcaggatcttggtgaattttagttcctcatttaatcctgtgtttagagacagaattgtcagtgtgaaagatgaaagaaggtcagattcaggtcttatacagaattatcctattgttgaatatgtaccttactgccaaatgataacagatcagggggcaagttcagttccttgtcttctcattactttgactcccaaaagttttattaatatttctgattctcaacaagaaaactatttgaatataaacacacttcaatgcttgccttctgtgatatttgaagtctagtcagtgtcagagctaatgggagattcagggacgccaccaaatcctggggtggccctcagccaagttctctgaagtttccagaacaaagattctcatggtttcttgtgtaccagagctctgagaaggttatgaattatgcagattcccagggccccactctctgagattctaattagggaggtgtagggtcgggtcctggaatctaaatttttttttttttttggagacagagtctcactttgttgcccaagctggagtgccatggagtgatctcagctcactgcaacttccgcctcccaggttcaagtgattctcctgccttagcctctagagtagctgggattacaggtgcctgtcaccatgcctggctaatttttgtatttctagtagagacagggtttcaccatgttgcccaggctggtctcgaactcctgacctcaggtgacccacctggctcagcctcccaaagtgctgggattacaggcgtgagtcaccacactcagaatctgaatttttaacttacacgtttggtgacaagaatgcaggtggtataaagatctcactctttgtaacattgtcctagaggttacatttataggtcatgaggacttgggataaaggagaactcattaagttggatctggatttctcaggctagtatagggtctaaagttgagaggagtgaggtggtgattacattaatctatgagaatgtatttttgttgagggagctgaataagataaaagagagaataacattaagatcaacgttggccttgctctttcaccaataaagaaatgacatcactaaaatatttggtgtgttcaactgggtacatggcttattcagctcaatttaatatatactaaggcaattgctgtgagtcatatgaaaatgattgtatcatcaggcctaaactcaggaaacttgaaactttcatgggggaaacaacatatttctaataatttataatataaagcagaatgacgtttctacagtaaaaggaatatataatgtggtagagaaagtaattcctcacaaggacatcaaggatggctttcaaaggaggtggcatttgaattcaactctaaagaataaataaggctggtcgtggtggctcacacctgtaatcccagcactttgggaggctgaggtgggtggatcacctgag

SEQ ID NO: 9744 - RNA, 162 nt, Homo sapiens
  source 1..162: mol_type = other RNA
atggtctcctgttctctgcagaccatactcttacctcctgttcttggttctccgacatcctacaccaaaagcccattggaaggaaacatctgagaacagcaccagctccccacagcgacaccgcccgcgccccaccatatagccagatcacggcttctcctt

SEQ ID NO: 9745 - RNA, 145 nt, Homo sapiens
  source 1..145: mol_type = other RNA
atggtctcctgttctctgcagaccatactcttacctcctgttcttggttctccgacatcctacaccaaaagcccattggaaggaaacatttgggacgccggagagtgcacgcaggtgccgggtgagggacggcgaatggatatcc

SEQ ID NO: 9746 - RNA, 2220 nt, Homo sapiens
  source 1..2220: mol_type = other RNA
atggtctcctgttctctgcagcacattgaagggaagtgaccatttcaagtgagggtgtcacttcctctgcttttttattccaggtacaacagactagcaagagagtggacacaaaaatatgctatgtaagtgccttggaggttttacatgagacactgtccaagagaagctggcagagaggtcttcccttaaaactttgggctgttggctgagccattcaaagagcatcatctgttcttcaaacaaatgttggtcacccactctctccagctgcagcatgttggtgccattttcagcaattacggctttgacagtgccacctctttgatgccaaatcagcaaccattgttgttatgatctgcagtcttcctggtgacactggaatctctctctctgccgcctcagtttgtctgctggtctcttggggggccaggccctgcacgtctctcctacccggcctcaaatggtgctgctgcccatgatggtaccacaccagggcctcagcctggcccctcaccacataccctttgccttttagaactcagtgccatcctgggtgcccagggcagagcaggctttgttcgcacctcatctgctgcagaaccacatcctgaggagtctcagcttatcctgcatgcccagcttgacctcgtggcacagcaggtgcaccagtggctggtagtagctggagggcagcaccgtctcgtcccgcagccgcacctccagctgcaaggagcccaggttgccctcgtcatgctgccggctcttggactggtcgggctgcagccggaaccagccctcctcctgctgcgccacccgcagtctctggacatcgatcaccactttgcccaggaagtcgtttcggctgacaaggtcccagtcccaggcctccacgcacagcgcctccacggccccctcctgcagctcaaattcaaacgtctcattccagcgtgggtagcatgacttcttcatgatctggcctccagcacagagcagcgtagctggcaggcccgggcccctgggcgcacttccagccgcaggtggatctcgccctgcacctcctcatcagggtcaacctccgtcaggtgggcccacccgctgaaacccttagggtgagaagctatggtgtcccttgtaaggcagacctttccgataacgtcgtcccggctgagggcatcctcatccatgacgtagaaagccacagcgtggaaggtgggcggcaggtgcacttggtactcctcaccccagaaggggcacagggtcttccacactgtggctgtccttgctgcaggcgagtgttgctggaccactttgtttcagccacgggtcctttgtcattcatcaccaggaacttcaccctgtaggggctcggtcctggtaggggatggttgcagccaatttttgttggttggcagtgggtatcattgccaacacggaggacatggagctggcctctggcctggtacagcacccggttggccctcagtgtgagatagtagcccctctgggagaagttggcaggagcagggatgtcctggtttgtccgtggggccgtgaagctctgggtggcgttgctgagggccaccaccagccagatggtatccaagtcagagatgttgtggctgctgaactggcctagaggctgctccagcgtgaaggtggacagggtgagcctccccgccagggtgtcgtttgagagctggggcacatagctgatgtgctctggggcagagttctgcaggctgtacagaaagcgtggctggggaggcctcaggaaactgacaatcacggcagaaggcgaaggggaagcaggcacgtccggaagcgctcctccagcagggacagctcactgatgaggtcggtgatggcgttggtaaaggcttcctgggggctgtagtccggcgtggtctgcactcggatgatgatcttgtgctccaaggggtgggggactttgtagccagcaaatagcacttgcgggtcctttaggtcacactgtgatttaatgatgtttcccagtgtgtggtcttctttgttgatggtgaataaacaggcattgggtaccttggtgtccttgttaatggtgatcttcttctcgccctcgaagagcaagaacgactcgaaggctggaggggcgttcacgctcccgcctccgttgcgtccagaccccaagtgtctgccgccgccgccaccagagccctaataagaggcctcttccggatt

SEQ ID NO: 9747 - RNA, 1413 nt, Homo sapiens
  source 1..1413: mol_type = other RNA
atggtctcctgttctctgcagcctgtgtttttgagcagcctgtgactaaagtcaccctcctattcgtgtttgccatattcctagcgtaacagaagccaaccacaatagtccaacaatgaagaatttaggcaaatagaaagttaaacactttctttctccctggacacgaatcccgtggtacacgcacagccagaagagcagcagggcgcacaggaacatggactgaaagaggtcatccagcatccctgggagccagctgttgaccaggaaggagagggggaagaacggatcattgtaaagtagcagcagaggcaggagaacagacatccacttctgctcgatgccccagtctctcatggaaaatttccggagggaatgcgcaaacaggcaagtgacgatgaaggtgagcaccacaaagaaaaaccggaaccagatttccaaccgggagaaggcagggttataagtcttccatgtgaagttcattcccttgatggggagcttcaggtgttcaaatcccactatcactgtatactgagtgtagttcaggtagccaaggtgagccacaataatctccgcacatttctgcaaatacacagaaagatttgcccctgcacatgtgagggtccttgtccggttgtgaactttgttatgaatgtacatcgtggttccatcttgagctacaccatcgactttaacagtcatgggaaagcttgtcttaatagaagtttcttttgattgatccaactcaacaacacatgtcagccatagttgctgattgtatgtagacagtggatttgaaagtatttgaattggctttagctttttgctattatttagtgaaaaattagccgcagaagtctggatcactttaggtcctctgatcccaacgaagatggtcaggccaaagcagatgaagaagacgacaaacacgaggacaaagtggcgcttggagagcgtgtagagccgcatgggcgccagcctgtagtagcggtcatccttgaagggcgtgaggtcctccttgagctcgcggtacgcttcccgcagccgccggcacaggtgcttgagctcgctgcagagcgggggctcaaaggcagggtactcggcgtccatgccgcgcagcctcccgggtcccggtcccgccgctccaccctttgtgtcgccgcctgcgccccctctcttctcccagcactggggatcgggctgctggcgcgctgggcgggaccgaggaggaggagcaggtgcgggggaggtggtgagggggcgcgcaggactcggacccagtgcgctcagggctccgccgcgagcacgcgaggagctggacacggcgcgggtgggggctgggggacccggccccccgccccgtgaagaggcctgagtgggggagggagccgcgcccatccgcctccgcgccca

SEQ ID NO: 9748 - RNA, 8196 nt, Homo sapiens
  source 1..8196: mol_type = other RNA
atgtataaatgtatacacacttcctatatgtatccacatatatatagtgtatatattatacatgtataggtgtgtatatgtgcatatatacacacatgcacataacaaaatcagatgctcattacaaatccagatgctcattacaaaaccagatgctacacaaacagcagcagaggaaacaaggttggactcttgcaacagatcacaaaaaataaaaacagctacttgcagtgactttggtcatttctgtatgttcataaagaatggattgtaacaaggaaaaaaaggaacagtgttagtgaaaaaggaaaaatgggcgaaaccatcttgatccgatgcgaatgcagtaatgttctatataccatttcatcagttatttcttttagtcatgttgatttgatttcagtttctggctatgaaaaacatttttaaactcgtcacccacaacaaactgaacaaaactactacagtgaaagcccttttcagtgaaagatgtcagaaacctcaaaacctttggcctgactcagaactaccatgtgaaaatcagtactctcttaatgtttgaaataaaaactgaaaaaaaaaacaaaaaaacaaaaaaccttttttgaagcaccttaacgtggccatccatttgagaagtgggtgccacttttttctttgagcaccttattgatgtgtttgctatctgctgtctttctgttacctgttggctgaatggctagctgttaacatatacatgtgcacagaagagatatctgggcatgtatgttctcaatgaagtttactgtggtgactgctgaaaggtgaacccatttcctgattttcccgccgcagtgttgtgataagattcgaagaaacctttttccctgcacagaaatgtttcttatcacattgtatcttagtatggaaaggaatatggtcccttttttgcaattgctactgtgtacacacacacacacacacacacacacacacacacacactgtatgtttagacctaaaatacacacacccacgcacacactgtatgtttatgtgacctaaaacatacacacatgcacacacacatacatatccattcattcattcattcaagtggtgtttccagtgtctgtgtgtcactgtttatgcagtttccatttcccagtgaattatgagtggagggcaacttttctaaccagattgtcttttcagaacaaagacctgggaattgaggaagagtttggaaagagggagaggcaaggaaagagagctttaaattgaaaggttaatttcctaagaggaacctgggctgaatgactgcagtgttataccctccaatctttgcaggtgggcatggaacactgcttgtatcactctgtgcacggtataaatccatatatccacaaaaacacacatccatccatcaacatatacatggtttgggatgagcaggtcaatagttttgagagggagtttgttcctttttttttctcattatactcttaaattgttgtcagttatcaaacaaacaaacagaaaaattgtttggaaaaaccttgcatacgccttttctatcaagtgctttaaaatatagactaaatacacacatcctgccagttttttcttacagtgacagtatccttacctgccatttaatattagcctcgtatttttctcacgtatatttacctgtgacttgtatttgttatttaaacaggaaaaaaaacattcaaaaaaagaaaaattaactgtagcgcttcattatactattatattattattattattgtgacattttggaatactgtgaagttttatctcttgcatatactttatacggaagtattacgccttaaaaatacgaaaataaattttacaaggtttctgttttgtgtggaagagtaattgatgttgctaagaatgatgtttgtttttttggggtttttgttgttttttttttaaatgttaccagcactttttttgtaagtttcactttccgaggtattgtacaagttcacactgtttgtgaagtttgaatatgaaggaataattaaaaaaaaaaaaactcttctcttggtttcctattgtgtcttctttatactgtagtttctgttttaggcagttctccacattctttcacacattgtattctatgtctaatctgagattatttatccaaactgaggactctacctacaaggccagaaaaactctgagtatattagtcttctcaatacaagaagtaggaactacagacaggattggtgatgtcgaagtcactttgaggaaatataaagcaaattggtgtattgtcttatacatattcaaacctcaaaaatgacaaggatcacttattgctctacaaattgattcacattttttccttttccacatgcaaatcacagtctgcctgctgtggaaataatcaatcccatattataacactatgcccacctattcttgtttccacccatctctgttatccatgaatctatcactgagtctcctttttaacttttgggtttctcagctccatatgcaaaaaaggaaagttcatggcacaaaacatgcccctctttaatgactttggagactcataagggactcctatttggcccatagattctttgttatagtgaccctggccataaagagctctctgatctcatcattcttacagaaagtgctaatatggtgaagaaaacttatatcttgtttgtccttggtgaagtcaacacaaattaaattcacaatgtcttctgtatttcagtcagcactgtgcaatgtatgaataaaagagaggaaattatttcagccatgagaaggcttaaaatctaacaactagacatgaagagaggtttgtataaaatcaagagctagattgtgccattcagactctcaatgccaagggagtttctaaactaacaggaagttgataatggctagagtgagtcaagaaagggtccaaagaataagcggtctagtttggggactcgcaagaacactaagctttgagttggagaagctgagtgtggacagacatttccaccagtgtgaggagcacaaaaatatccaggcatgagcttgggatggggagagtcatcaagagacctctagactgaaaggatgtcaataaattcctgagatttcaacattaccactgtgaatttaaatatttacttcttgcaactcaattgctgaacttctaagtcaacctgattgatagtctagaagtataaagaggaagaaaatattttcatgatgcataatttgtctctatatcatttctgtgaaccaacatcttcttaacaatgccagccagcttcacccaaagtcttggatctctctttgcactatccacacactcttaagttttcttctgtacctcagttgctccaagccagttttgttgcctccatgaaaacttctgtggcatcattagcattacctggtgcacgtgttcctggggcagaacacaataatattaacccagcatcttgcagctcacaaagcagtcagccacgttcctgcctcatcttcttaagaatcttagaaagatagtaatattaccattttataaatgaggaaatatttatgagtctttgataggttaagtggcttatccaaagtcgtgaaactaattgcagagctcagcacttggaccaagtttctaaattccctgtccactacactccatgattacttcttttttgatctctgtgaagtccatcagagttttagtcccagagaaggtgctcttcacagcctacatgaagtcagaatgaatatagtctatggtaagtcctgtgatgacagtctatttctgcataacccctatgagttgcaaatttcttgacaattttggccctatttacatgaactggaccacttagctgcctcagatttttttttttgaaaaaacctgaaataaataaatgtacagcctgctttgacctcatggtttgtctcgatcagaggatggatataggagagtagaggagaaccttcaagtttcttcctggtgatagccatttcaaatgcataacaactggcgagccatccaatgtcctataaacacagctgtctgtgttttctctatatgcaaggcaattactagaattggaatgtccaatatactagccaccagtcacatgttgctatttacatttaaatttgttaattacaatgaaataaaatttaaaattcagtttctttgtcacattagccaaatttcaagtgctcaacagccacatgcagctaatggctaccatactggatgggacagacatagagcatttccataattgcagaaagttctttggatagcattgtcctacactaccttatgcaaataaattacctcaaacattgagtatatcgttgtgacttccagaaagctcaggctcttgccacacaaaaagctcccctgtacctcttgacaggtgtgacttggagtaagtgtgggaaactaccagttacagctatgaagcagcacctgaaagaatcaggagactaaacaaaactcacaccccacaaatgacagccacactgcccattgccccctctctgtggggtgaggtgtgcccaccagaatgctgtcattggtggacctcacacccagcctccctgcctgtccagctcagcactgatggaatctgaatgaacctgagtgtatgacgactcatttctggggctcacagtggtgagaaatgaaaaggggaaaaggcaggaaataaaattgcatagtgaggtcctgttcactcatgaagaccatctatctcaaagctccatgactcaaagtttctcacgtttctttagtataattctcaggattatagatcagacttgtacgcccaggcttagaatgtggtcagggaatcagtaatgtattcctccttgaatgctcattcatagatttgtctattcgctcctcctgttagggaatccacgaggggacccagaaaagcctggcatcgcttcctgtcagcactgagtgttccccttcctcaatcttctctgtgatgcttccctacatatttcccaaaagacatcataagcaggaaaatcttcctcaaacactattttgaaagaaaaagaaatggagaccaatagacatagatagacaccctccctgggtatcagtttggcttgggtttagctactagagcagcacagtcacatagaaatatgagagccacatatgcaattttagactttccagtagccacgttaaaaagataaaaagaagcatgaaactaatgttaatattttatttcacccaatacatccaaaatattatcatttttgacacacaatataccaaaactactgaaatagtattcttattattcatattaaatctccagaatctagtgtgattttatgcttataccaattataacagcacatcttgatttaaactaaccccatcttaagtggttgatggccacatgtggaaagtggctacgtggtggatagcgcatgtctccaggaatccaactatgaaatggtcttctctggttctcagaggagaatctagttcagtgagttctatttaaaaaaatttttttcaaattgaatcccatttcagtaacctgacccatttctaacatctataggcccttttgtattttatcaccatcccaatagtgtttataaatgtttcccaattaccataattatgttaaataacacccaactctcagtccaacctctgccgaatatacacctcctccaaatcaaaacactactcccttttcgtcattacattttagttcacttccaatttgtgaattgtgttctatttccaacagatttgcactaattttgcaagaaaaatgctgtaaactgccacagcaaacaacaacatttttacgttcatctaatctttcttccaaaggacttggagctctggacagatttcagttcattcttcctatgtaacccatttggtagaaaagtgaaaaaataataataataaaaatcctaggagaaatagttgaattgtcttgttgctaaaacaattgtcaaccccagtctaagtcttaggaagcaggacaatgctttatttttaaccatgcgcaagacacaaccttgcttcacattctctttcagttccttggcccatgaaagaaaatcagtcaccagtaaatccaacctccccgctcattcctctgagagagatggtggaaggataaaagtcttctaagatccagcctgaatgcaattaaacagaaataagcggttcagttaccccaaccccagcacaaagtcgtcagggagtgaataaaagggttcgaagaagttagtttgaaggtgtttattttttaaaccctctatcactcccagcccccctttttcccctaggaagagtccctattttaaaaatccacattttctttttagtgggaaacgttcttttttcaaaggctcaagagtgtattgatgcagaaaaggtagatcaaggcccaaatgctacgacttggctccctgtgtgggcatgtgcgtttcctggggcttccccagcacacacggccggaagaggctacaggcctgtatcaggctgtctaatggatgagtatgtcacagcaaaaggaaacttgaaatgcctgcccagagaataaaatctgaagtttgctgactcccttggtgccagggccttctttgtgggactttcagctccaagaatttcctacaagttccctagacaaaactcctgctcctcccagactagcctcaacatccccttggtgctcccaggccacttcatcacagataagcctatgccaactacctcaccccaaactgtcgtctcttcctgaaggcctgtgtatgtctccttctctccttactataataccttttcatgacaacattgtctccccatttaactgtaagttcttgagggcagataccaagatttagtcactctcaaatctccccatagaggctgctaccaggacttacttataacctgcctttgaatgagtgaaagttactgaaaatgacgtgaaaaaatgagatgaggatggctctgcagtcatgccatcctcatcatcaaccacaaaaccttgtagcccaaaatgctggccattatgaggaatgtgtctctcagagacataggatctgctcaaactgccagatttaaaaccaggtcaagatattttttaattttgcatttatgatcaagatccacgttactcaccctaggcctgccataatgcaaaatggaatagaacgaaaaggccaaggaaatgaagatggagaagaggatgacatttattcactcaactgaacacacacacacatacacacacacacacacacgcagcactgatggagagtacagctgcttatatattcatctataatagcaaagacaaaagtgtatcttccagaagatgcctctggttgctaaccagtctctgtgaagaagctgcagttacccaggcttctgtaactcaggacattgaagtagtcatgcagctcggcacagtcctctccccgctgctctccacagagcccagcaggtgcagcttctgcctggacacagcttcctgggggtgagggagcactggggctccattcctcctgtccagctgattttctcctgaggtcaccttccacagaatggattctgagggctttcttctttctagtcaacgcgaccaccacgatgactgctgtgcagatgaccaccagcgtcgcggccatggctccaagcaatggaatctggaacctggcaccgtgctcagccactgagctttctaggacctccaggaagattctcccagtgtacgtcccatcagggtaggtgtgatagatgcagaagtactcccctgtatcgttcacggtcagcgactggagggtgaggcccaggccgggacctggggccactcgatccttgaaggatggggagatgtgccaccccaagtcagcattacaaatggccagaagctggtcctgctgctcccagttgacctgggtcacttgtgccgtggtggaggagaggtgacattgtaagatgatagagccacctttctctgcagaaatgttccccgttgtttctattgtgcctgtcatcattcctgaggcgaggggagcctgcctcagcccctgggcccagatcaggaggagacaccagcgcatgcttctgcccagagggcctacaggaagcagatgtggcctcttctgccactgaaagtagccgact

SEQ ID NO: 9749 - RNA, 9415 nt, Homo sapiens
  source 1..9415: mol_type = other RNA
atgtataaatgtatacacacttcctatatgtatccacatatatatagtgtatatattatacatgtataggtgtgtatatgtgcatatatacacacatgcacataacaaaatcagatgctcattacaaatccagatgctcattacaaaaccagatgctacacaaacagcagcagaggaaacaaggttggactcttgcaacagatcacaaaaaataaaaacagctacttgcagtgactttggtcatttctgtatgttcataaagaatggattgtaacaaggaaaaaaaggaacagtgttagtgaaaaaggaaaaatgggcgaaaccatcttgatccgatgcgaatgcagtaatgttctatataccatttcatcagttatttcttttagtcatgttgatttgatttcagtttctggctatgaaaaacatttttaaactcgtcacccacaacaaactgaacaaaactactacagtgaaagcccttttcagtgaaagatgtcagaaacctcaaaacctttggcctgactcagaactaccatgtgaaaatcagtactctcttaatgtttgaaataaaaactgaaaaaaaaaacaaaaaaacaaaaaaccttttttgaagcaccttaacgtggccatccatttgagaagtgggtgccacttttttctttgagcaccttattgatgtgtttgctatctgctgtctttctgttacctgttggctgaatggctagctgttaacatatacatgtgcacagaagagatatctgggcatgtatgttctcaatgaagtttactgtggtgactgctgaaaggtgaacccatttcctgattttcccgccgcagtgttgtgataagattcgaagaaacctttttccctgcacagaaatgtttcttatcacattgtatcttagtatggaaaggaatatggtcccttttttgcaattgctactgtgtacacacacacacacacacacacacacacacacacacactgtatgtttagacctaaaatacacacacccacgcacacactgtatgtttatgtgacctaaaacatacacacatgcacacacacatacatatccattcattcattcattcaagtggtgtttccagtgtctgtgtgtcactgtttatgcagtttccatttcccagtgaattatgagtggagggcaacttttctaaccagattgtcttttcagaacaaagacctgggaattgaggaagagtttggaaagagggagaggcaaggaaagagagctttaaattgaaaggttaatttcctaagaggaacctgggctgaatgactgcagtgttataccctccaatctttgcaggtgggcatggaacactgcttgtatcactctgtgcacggtataaatccatatatccacaaaaacacacatccatccatcaacatatacatggtttgggatgagcaggtcaatagttttgagagggagtttgttcctttttttttctcattatactcttaaattgttgtcagttatcaaacaaacaaacagaaaaattgtttggaaaaaccttgcatacgccttttctatcaagtgctttaaaatatagactaaatacacacatcctgccagttttttcttacagtgacagtatccttacctgccatttaatattagcctcgtatttttctcacgtatatttacctgtgacttgtatttgttatttaaacaggaaaaaaaacattcaaaaaaagaaaaattaactgtagcgcttcattatactattatattattattattattgtgacattttggaatactgtgaagttttatctcttgcatatactttatacggaagtattacgccttaaaaatacgaaaataaattttacaaggtttctgttttgtgtggaagagtaattgatgttgctaagaatgatgtttgtttttttggggtttttgttgttttttttttaaatgttaccagcactttttttgtaagtttcactttccgaggtattgtacaagttcacactgtttgtgaagtttgaatatgaaggaataattaaaaaaaaaaaaactcttctcttggtttcctattgtgtcttctttatactgtagtttctgttttaggcagttctccacattctttcacacattgtattctatgtctaatctgagattatttatccaaactgaggactctacctacaaggccagaaaaactctgagtatattagtcttctcaatacaagaagtaggaactacagacaggattggtgatgtcgaagtcactttgaggaaatataaagcaaattggtgtattgtcttatacatattcaaacctcaaaaatgacaaggatcacttattgctctacaaattgattcacattttttccttttccacatgcaaatcacagtctgcctgctgtggaaataatcaatcccatattataacactatgcccacctattcttgtttccacccatctctgttatccatgaatctatcactgagtctcctttttaacttttgggtttctcagctccatatgcaaaaaaggaaagttcatggcacaaaacatgcccctctttaatgactttggagactcataagggactcctatttggcccatagattctttgttatagtgaccctggccataaagagctctctgatctcatcattcttacagaaagtgctaatatggtgaagaaaacttatatcttgtttgtccttggtgaagtcaacacaaattaaattcacaatgtcttctgtatttcagtcagcactgtgcaatgtatgaataaaagagaggaaattatttcagccatgagaaggcttaaaatctaacaactagacatgaagagaggtttgtataaaatcaagagctagattgtgccattcagactctcaatgccaagggagtttctaaactaacaggaagttgataatggctagagtgagtcaagaaagggtccaaagaataagcggtctagtttggggactcgcaagaacactaagctttgagttggagaagctgagtgtggacagacatttccaccagtgtgaggagcacaaaaatatccaggcatgagcttgggatggggagagtcatcaagagacctctagactgaaaggatgtcaataaattcctgagatttcaacattaccactgtgaatttaaatatttacttcttgcaactcaattgctgaacttctaagtcaacctgattgatagtctagaagtataaagaggaagaaaatattttcatgatgcataatttgtctctatatcatttctgtgaaccaacatcttcttaacaatgccagccagcttcacccaaagtcttggatctctctttgcactatccacacactcttaagttttcttctgtacctgttaaaaacattgtggtgcgatttatatacaggctgtaataattgtaaatgacacatacgctactcatatggtacttcacagtttacaaagtttctccttaatatccttcatcttcacagttatactgtaaatattgtgatgtagctatgattgcactaatttataaaaacacaggttcagaaatatgtgtttttccaataaaaaacaataaactagtgcctgaggtcaggttttctgaaatccaataatatttataccataccattattctcaaacttgagtaatgtgtgtatgcccatatgaaggaaaaaaaatagtttcacagacctcctcaatgggaggcgataataataaaataattattcttattataatatctagtaataaattcataatatgcataattattttattatagacattcttaaataggctcaaacacaacgacaagtgaacttactatgcttatatcccttgtagaattataaaactacaagttactaattaagtacaagtaaaactataaaattagtaatgtctacaataacaatgagtgcatagaatgatgctttcctgaatctaagtcatggctcacaaagttaagtgtactgcacacacccttctgaatacaacatccctacactacagtgtgcaaagtaaagcaattatcgcttcactttcctgttagttcaatactgcaaagtcttccacttctccacccatctgggagtaaatgaatcatttataaattaagcttctgtgcctttaaataaacttgattataatcaagtttatatgtataaacacaaacatagaggctaaaaccaatgacaacactctgttttaagaaggctatcaacatccagatatagatgacttctttgaagattatcatttcacttaaaacacacaatgtttaaacgcttgcagagaacttgtggaccccaaggctgtatctgcaactcttagctttccttatatctcagtttttaagaacattgattgatagataatttcagatacctcagttgctccaagccagttttgttgcctccatgaaaacttctgtggcatcattagcattacctggtgcacgtgttcctggggcagaacacaataatattaacccagcatcttgcagctcacaaagcagtcagccacgttcctgcctcatcttcttaagaatcttagaaagatagtaatattaccattttataaatgaggaaatatttatgagtctttgataggttaagtggcttatccaaagtcgtgaaactaattgcagagctcagcacttggaccaagtttctaaattccctgtccactacactccatgattacttcttttttgatctctgtgaagtccatcagagttttagtcccagagaaggtgctcttcacagcctacatgaagtcagaatgaatatagtctatggtaagtcctgtgatgacagtctatttctgcataacccctatgagttgcaaatttcttgacaattttggccctatttacatgaactggaccacttagctgcctcagatttttttttttgaaaaaacctgaaataaataaatgtacagcctgctttgacctcatggtttgtctcgatcagaggatggatataggagagtagaggagaaccttcaagtttcttcctggtgatagccatttcaaatgcataacaactggcgagccatccaatgtcctataaacacagctgtctgtgttttctctatatgcaaggcaattactagaattggaatgtccaatatactagccaccagtcacatgttgctatttacatttaaatttgttaattacaatgaaataaaatttaaaattcagtttctttgtcacattagccaaatttcaagtgctcaacagccacatgcagctaatggctaccatactggatgggacagacatagagcatttccataattgcagaaagttctttggatagcattgtcctacactaccttatgcaaataaattacctcaaacattgagtatatcgttgtgacttccagaaagctcaggctcttgccacacaaaaagctcccctgtacctcttgacaggtgtgacttggagtaagtgtgggaaactaccagttacagctatgaagcagcacctgaaagaatcaggagactaaacaaaactcacaccccacaaatgacagccacactgcccattgccccctctctgtggggtgaggtgtgcccaccagaatgctgtcattggtggacctcacacccagcctccctgcctgtccagctcagcactgatggaatctgaatgaacctgagtgtatgacgactcatttctggggctcacagtggtgagaaatgaaaaggggaaaaggcaggaaataaaattgcatagtgaggtcctgttcactcatgaagaccatctatctcaaagctccatgactcaaagtttctcacgtttctttagtataattctcaggattatagatcagacttgtacgcccaggcttagaatgtggtcagggaatcagtaatgtattcctccttgaatgctcattcatagatttgtctattcgctcctcctgttagggaatccacgaggggacccagaaaagcctggcatcgcttcctgtcagcactgagtgttccccttcctcaatcttctctgtgatgcttccctacatatttcccaaaagacatcataagcaggaaaatcttcctcaaacactattttgaaagaaaaagaaatggagaccaatagacatagatagacaccctccctgggtatcagtttggcttgggtttagctactagagcagcacagtcacatagaaatatgagagccacatatgcaattttagactttccagtagccacgttaaaaagataaaaagaagcatgaaactaatgttaatattttatttcacccaatacatccaaaatattatcatttttgacacacaatataccaaaactactgaaatagtattcttattattcatattaaatctccagaatctagtgtgattttatgcttataccaattataacagcacatcttgatttaaactaaccccatcttaagtggttgatggccacatgtggaaagtggctacgtggtggatagcgcatgtctccaggaatccaactatgaaatggtcttctctggttctcagaggagaatctagttcagtgagttctatttaaaaaaatttttttcaaattgaatcccatttcagtaacctgacccatttctaacatctataggcccttttgtattttatcaccatcccaatagtgtttataaatgtttcccaattaccataattatgttaaataacacccaactctcagtccaacctctgccgaatatacacctcctccaaatcaaaacactactcccttttcgtcattacattttagttcacttccaatttgtgaattgtgttctatttccaacagatttgcactaattttgcaagaaaaatgctgtaaactgccacagcaaacaacaacatttttacgttcatctaatctttcttccaaaggacttggagctctggacagatttcagttcattcttcctatgtaacccatttggtagaaaagtgaaaaaataataataataaaaatcctaggagaaatagttgaattgtcttgttgctaaaacaattgtcaaccccagtctaagtcttaggaagcaggacaatgctttatttttaaccatgcgcaagacacaaccttgcttcacattctctttcagttccttggcccatgaaagaaaatcagtcaccagtaaatccaacctccccgctcattcctctgagagagatggtggaaggataaaagtcttctaagatccagcctgaatgcaattaaacagaaataagcggttcagttaccccaaccccagcacaaagtcgtcagggagtgaataaaagggttcgaagaagttagtttgaaggtgtttattttttaaaccctctatcactcccagcccccctttttcccctaggaagagtccctattttaaaaatccacattttctttttagtgggaaacgttcttttttcaaaggctcaagagtgtattgatgcagaaaaggtagatcaaggcccaaatgctacgacttggctccctgtgtgggcatgtgcgtttcctggggcttccccagcacacacggccggaagaggctacaggcctgtatcaggctgtctaatggatgagtatgtcacagcaaaaggaaacttgaaatgcctgcccagagaataaaatctgaagtttgctgactcccttggtgccagggccttctttgtgggactttcagctccaagaatttcctacaagttccctagacaaaactcctgctcctcccagactagcctcaacatccccttggtgctcccaggccacttcatcacagataagcctatgccaactacctcaccccaaactgtcgtctcttcctgaaggcctgtgtatgtctccttctctccttactataataccttttcatgacaacattgtctccccatttaactgtaagttcttgagggcagataccaagatttagtcactctcaaatctccccatagaggctgctaccaggacttacttataacctgcctttgaatgagtgaaagttactgaaaatgacgtgaaaaaatgagatgaggatggctctgcagtcatgccatcctcatcatcaaccacaaaaccttgtagcccaaaatgctggccattatgaggaatgtgtctctcagagacataggatctgctcaaactgccagatttaaaaccaggtcaagatattttttaattttgcatttatgatcaagatccacgttactcaccctaggcctgccataatgcaaaatggaatagaacgaaaaggccaaggaaatgaagatggagaagaggatgacatttattcactcaactgaacacacacacacatacacacacacacacacacgcagcactgatggagagtacagctgcttatatattcatctataatagcaaagacaaaagtgtatcttccagaagatgcctctggttgctaaccagtctctgtgaagaagctgcagttacccaggcttctgtaactcaggacattgaagtagtcatgcagctcggcacagtcctctccccgctgctctccacagagcccagcaggtgcagcttctgcctggacacagcttcctgggggtgagggagcactggggctccattcctcctgtccagctgattttctcctgaggtcaccttccacagaatggattctgagggctttcttctttctagtcaacgcgaccaccacgatgactgctgtgcagatgaccaccagcgtcgcggccatggctccaagcaatggaatctggaacctggcaccgtgctcagccactgagctttctaggacctccaggaagattctcccagtgtacgtcccatcagggtaggtgtgatagatgcagaagtactcccctgtatcgttcacggtcagcgactggagggtgaggcccaggccgggacctggggccactcgatccttgaaggatggggagatgtgccaccccaagtcagcattacaaatggccagaagctggtcctgctgctcccagttgacctgggtcacttgtgccgtggtggaggagaggtgacattgtaagatgatagagccacctttctctgcagaaatgttccccgttgtttctattgtgcctgtcatcattcctgaggcgaggggagcctgcctcagcccctgggcccagatcaggaggagacaccagcgcatgcttctgcccagagggcctacaggaagcagatgtggcctcttctgccactgaaagtagccgacttccacaagatcggtggcttgtacacgggaaacacaacctagggttctcccagagcacagaccaatctcccagcagtgtctttgggcttctgcttctccaaagtcttccctctggctcagaagtggtaggggagctccatggctgtcacagctgtctgatgcctcctgtctctgcctagaatcaagggcaacat

SEQ ID NO: 9750 - RNA, 746 nt, Homo sapiens
  source 1..746: mol_type = other RNA
atgtatgtgtgcatgtgcatgggtgtgtgcacgcacagagtcaatgactccttggaattctagacccgtgctgcactgtatggtaatctactagctgcatgtggctatttaaattacaatgaaataaaacagaatatttagctcttcagttgtactagctacgttttttcctcagcactttctgtgtagagagtaactgaggcccagagaagcgaagtaagtcgcctaaggtcccacagcaagtctgtggcaaccagagggcagaatccaagttttctgagaaattcaccaggctcctttcatctgggatttaaaaaatcctcaagagttcggtttagtaacaagaaaactgaaaacagatctcagagctggaagagttagggaggaggaaggggagaaccggattcagagaaggccaggactgaacccgagggtgggggctcaaatatccgtccctccctccacctgcttcagggaagggaggagtgggactcacacgctgtctccctggatgaacaactctggccgctcttttagcaaattcttcttgatccagatgagcaggttccggatgtcccagggttcctcctgtccaggcaaagtgactcgatgtttcttaataccgtcaaacaggagctccgcaccacctccgaactccacctccactgacaagggcgcagccatgttgaggaagccgagctcgcaggaaactcccctcaacttccggcgcgcccgcaaatttccgg

SEQ ID NO: 9751 - RNA, 3581 nt, Homo sapiens
  source 1..3581: mol_type = other RNA
atgtatgtgtgcatgtgcatgtgggcacatgtgtgcacacacggctaatgtgtgtgtaggggtggtagggcactgccctcggccaaggtgcctggaagcagcaaggcaggcacaggtggacccagagaccatctgagcatggccccagggtggctcaggtgactgggctggctggctgggacccggctgggcagcaaatggcttctacctgcacccagacctctgtgtgcgctgcactgcgtttccccgcgagccatgcctgtggacactgtgggcccctggccttgccgctgccaggagagttactggacacccagatggtgaggctgggttgggagaggctggggctgttgtggccagagtggggctctggaggcctactgatgggtttgaatcctgatactgcccccacctagctgagtgtcatgggcaatcaggttcttcaagcctcagttttttcatctgtaaaatggggcaatgtttgccctacaggattcaggaaaaagtgaagtgagatgatgctttgaggtgtccagcacagcaccgggcccacaacaggcgctggaaacagcagccactctggcctggcacctggggcaggcaagctggcctgggaaagacccaccccagaaagcagcccccagcactttcctccttcccccgacccgggaggaccctgggggctcatcacttgagtcagtgaggggcagccattcatttgtttctttattcaatccctcgcaccaatgcctctctggcccagcgctgtgtggggagctgggacatggggtcatgggactgccccaaccctctgggaactcataggctggcagggtgggaggaggcaggcttgtggctgtaactgtgggtaggagtttcacgggcatctcaggctggccctggacccctggaaggggggctgggtttgggggttaagtggagtcggtcagggatgagggtgggaaggggacagcaggcagaggatgtggcgggcaggtggctgaggcctggagggacatggggaggggccaggggccaggcttacagggcttctgggtaaagctgtggagctgagactctactgcttgtgtggagctaggagaggtcttgaccatggatggtggttagctctgagctctgggcaggtggacgggtgtggggggacaagtggcagtgcggagtcaagcagagggttggcaaggccagctcgttcccctgggcctgacccctctgctctccgaagccacgagggcagggcagggtgatggtgcactgggtcacctcctgccaatcaaactgtccttttccccttcagtattgaagggggccccttggactgtgagaggggcagggctcacctggaggggcagccctgggggagagtggggacctcagagggcagcctctgggcctctggaaatggaggtctttgctttcctcctgccttctccagagaacagaagaagtctcttcctctgaccgtcccatcgcaggttccccaggaggctaaaactgtgtggattttaggacagagttccccagcgtgccatgtgttgccttctttactgcctggttctgcacatcttggatggtgtcgggcagcggcaagctctgggtctcgggcagaagcagtgcggccaggccactcagcactggcaccgtcccatacaccagcaagggcagccaggggccatggacacccagcagccggaccagaggccccaggatggctcctccacgggctgccatctggcccaagcccactgccgtcatcctgagcacagtggggaagagctcgctgctgtagatggtgatgcaggtgaaggcagcccccaccccgcccagccccagcacggccaaggctgagcgcagagcccccatttcgtggggcaccagcgtgttggccagaatgcagagccctgccagcaacagggatgcggccagcgtggggcggcggcccaggtggctcagcagcagcagggcgcccatcttggctgggatgtccacgacaccaatgaacatttggagcaggaagatgttgctgcccagggcctgcaggtccagggccaggccgaagaaggtgaagccaaaggcgaaccagcacaacgtggagatacaggtccggaagcgcagtccgggcatgcggagcagggtgcccaggctggcaggaggctggcccatgctcagctcctcccgcatggctgaaagcaagacctcaggggtcagggtgtcctgcactgccccctttccgttgatggcagccaccctccacagctcctgcaggccccaatccagcctgcctgtggtgaggagccatcgtgccgactctgccagccaccaggagtacaaaaagcagaggaagaaggggaccgagaccaccagctgcagcagtgtccagtcccgcacaccgtaggccactgcagctgtcaggccatggccgaagctgaagcccagagagttcaaggtcatcaccaagggtcgggcccgtgccgccgtccactccatcactgcaaggagaccgagtggttcagccctggagcctgcatggagcccccctgcatggcgccaggtcagagacctacggagagtgcccgtgttcatcatgacgcctgccacggcaaaggccaacaggaagcggaacaggcagtacacggggaaggcaggggcgaaggcagctgccgtacccatcacagccatctgaaggtagctccaggttagcaccagcctgcgcccaaacctgtctgaggcagggccgcacgcagcagctcccaccagaatcccagccaggtagatggactgggccatgggcttcagagcatgagagtcacacacgaggttccacttggccacgattgtggaggtgaagatgctgcggtcatagacccagccatccacacacggctccgtgtcggcctcgctccagctggtggccgtggcattggggtccaagagctgccactgtggctggcggaagcggcggcactggtggggcctctggttggggcccggcgggatggaaatagccaggagggcctcaggactcaagctccctaggatgctggcctgagccgtgctgttgtccaggaggggtgcccagcagcggtggctgggcacggcggccgagaagttctccagcatgctctgggtacacagccacatgatggagaccatcagagccatcgtctggagaacctggaacctgcccaggccacccacgaggtccaggagttcagaaaatgccatggaacctactcaaggggcccagaagaggggcccacttcacaaaggctggcccagggcaaagaggccagggcaacgggcctgtttcccccacggtggtgcccacagtggcttctccagcccagcggctaggcttcacagactcggggccggaggctcaggctctctggtcatctgcctgctggtgtcacttggggtggctccaactgggccctgaggccgcgtgaggtgattccgagacctccagcatctccccagagaggcagctgctccagacctcccgggaaagctgaatttggaaagtagggaatgtggagactgaagactttaattttagactg

SEQ ID NO: 9752 - RNA, 3469 nt, Homo sapiens
  source 1..3469: mol_type = other RNA
atgtatgtgtgcatgtgcatgtgggcacatgtgtgcacacacggctaatgtgtgtgtaggggtggtagggcactgccctcggccaaggtgcctggaagcagcaaggcaggcacaggtggacccagagaccatctgagcatggccccagggtggctcaggtgactgggctggctggctgggacccggctgggcagcaaatggcttctacctgcacccagacctctgtgtgcgctgcactgcgtttccccgcgagccatgcctgtggacactgtgggcccctggccttgccgctgccaggagagttactggacacccagatggtgaggctgggttgggagaggctggggctgttgtggccagagtggggctctggaggcctactgatgggtttgaatcctgatactgcccccacctagctgagtgtcatgggcaatcaggttcttcaagcctcagttttttcatctgtaaaatggggcaatgtttgccctacaggattcaggaaaaagtgaagtgagatgatgctttgaggtgtccagcacagcaccgggcccacaacaggcgctggaaacagcagccactctggcctggcacctggggcaggcaagctggcctgggaaagacccaccccagaaagcagcccccagcactttcctccttcccccgacccgggaggaccctgggggctcatcacttgagtcagtgaggggcagccattcatttgtttctttattcaatccctcgcaccaatgcctctctggcccagcgctgtgtggggagctgggacatggggtcatgggactgccccaaccctctgggaactcataggctggcagggtgggaggaggcaggcttgtggctgtaactgtgggtaggagtttcacgggcatctcaggctggccctggacccctggaaggggggctgggtttgggggttaagtggagtcggtcagggatgagggtgggaaggggacagcaggcagaggatgtggcgggcaggtggctgaggcctggagggacatggggaggggccaggggccaggcttacagggcttctgggtaaagctgtggagctgagactctactgcttgtgtggagctaggagaggtcttgaccatggatggtggttagctctgagctctgggcaggtggacgggtgtggggggacaagtggcagtgcggagtcaagcagagggttggcaaggccagctcgttcccctgggcctgacccctctgctctccgaagccacgagggcagggcagggtgatggtgcactgggtcacctcctgccaatcaaactgtccttttccccttcagtattgaagggggccccttggactgtgagaggggcagggctcacctggaggggcagccctgggggagagtggggacctcagagggcagcctctgggcctctggaaatggaggtctttgctttcctcctgccttctccagagaacagaagaagtctcttcctctgaccgtcccatcgcaggttccccaggaggctaaaactgtgtggattttaggacagagttccccagcgtgccatgtgttgccttctttactgcctggttctgcacatcttggatggtgtcgggcagcggcaagctctgggtctcgggcagaagcagtgcggccaggccactcagcactggcaccgtcccatacaccagcaagggcagccaggggccatggacacccagcagccggaccagaggccccaggatggctcctccacgggctgccatctggcccaagcccactgccgtcatcctgagcacagtggggaagagctcgctgctgtagatggtgatgcaggtgaaggcagcccccaccccgcccagccccagcacggccaaggctgagcgcagagcccccatttcgtggggcaccagcgtgttggccagaatgcagagccctgccagcaacagggatgcggccagcgtggggcggcggcccaggtggctcagcagcagcagggcgcccatcttggctgggatgtccacgacaccaatgaacatttggagcaggaagatgttgctgcccagggcctgcaggtccagggccaggccgaagaaggtgaagccaaaggcgaaccagcacaacgtggagatacaggtccggaagcgcagtccgggcatgcggagcagggtgcccaggctggcaggaggctggcccatgctcagctcctcccgcatggctgaaagcaagacctcaggggtcagggtgtcctgcactgccccctttccgttgatggcagccaccctccacagctcctgcaggccccaatccagcctgcctgtggtgaggagccatcgtgccgactctgccagccaccaggagtacaaaaagcagaggaagaaggggaccgagaccaccagctgcagcagtgtccagtcccgcacaccgtaggccactgcagctgtcaggccatggccgaagctgaagcccagagagttcaaggtcatcaccaagggtcgggcccgtgccgccgtccactccatcactgcaaggagaccgagtggttcagccctggagcctgcatggagcccccctgcatggcgccaggtcagagacctacggagagtgcccgtgttcatcatgacgcctgccacggcaaaggccaacaggaagcggaacaggcagtacacggggaaggcaggggcgaaggcagctgccgtacccatcacagccatctgaaggtagctccaggttagcaccagcctgcgcccaaacctgtctgaggcagggccgcacgcagcagctcccaccagaatcccagccaggtagatggactgggccatgggcttcagagcatgagagtcacacacgaggttccacttggccacgattgtggaggtgaagatgctgcggtcatagacccagccatccacacacggctccgtgtcggcctcgctccagctggtggccgtggcattggggtccaagagctgccactgtggctggcggaagcggcggcactggtggggcctctggttggggcccggcgggatggaaatagccaggagggcctcaggactcaagctccctaggatgctggcctgagccgtgctgttgtccaggaggggtgcccagcagcggtggctgggcacggcggccgagaagttctccagcatgcttcaaggggcccagaagaggggcccacttcacaaaggctggcccagggcaaagaggccagggcaacgggcctgtttcccccacggtggtgcccacagtggcttctccagcccagcggctaggcttcacagactcggggccggaggctcaggctctctggtcatctgcctgctggtgtcacttggggtggctccaactgggccctgaggccgcgtgaggtgattccgagacctccagcatctccccagagaggcagctgctccagacctcccgggaaagctgaatttggaaagtagggaatgtggagactgaagactttaattttagact

SEQ ID NO: 9753 - RNA, 38 nt, Homo sapiens
  source 1..38: mol_type = other RNA
atgtatgtgtgcatgtgcatgtgtgactgaatctcact

SEQ ID NO: 9754 - RNA, 209 nt, Homo sapiens
  source 1..209: mol_type = other RNA
atgtcccacccccactcctgtcgcgctgtgatctcggctggggccccaccccccgaggacagagttggtggagaagggagtccccgtcttcaagcctcggggactgggagctctggcttttagcgcgggtccttgtgtaggcgagctcatatactacgatggggcaggggcgcgacggtctggcggctccggggcattgtctaagcggg

SEQ ID NO: 9755 - RNA, 71 nt, Homo sapiens
  source 1..71: mol_type = other RNA
atgtcccacccccactcctgtttgaatatttcaccagaaacaggagtggggggtgggacgtaaggaggatg

SEQ ID NO: 9756 - RNA, 43 nt, Homo sapiens
  source 1..43: mol_type = other RNA
atgtgattgacggctgactccagcctctccacaggcaagccct

SEQ ID NO: 9757 - RNA, 82 nt, Homo sapiens
  source 1..82: mol_type = other RNA
atgtgcctgagggagtaagacactatctgacaacaacagggctcttactccctcaggcactgcaccagccagcaaagcatca

SEQ ID NO: 9758 - RNA, 81 nt, Homo sapiens
  source 1..81: mol_type = other RNA
atgtgcctgagggagtaagacactatcttacaacaacaggactcttactccctcaggcactgcaccagccagcaaagcatc

SEQ ID NO: 9759 - RNA, 82 nt, Homo sapiens
  source 1..82: mol_type = other RNA
atgtgcctgagggagtaagacactatcttacaacaacagggctcttactccctcaggcactgcaccagccagcaaagcatca

SEQ ID NO: 9760 - RNA, 32 nt, Homo sapiens
  source 1..32: mol_type = other RNA
attaaggacatttgtgattgatgggaggagga

SEQ ID NO: 9761 - RNA, 16016 nt, Homo sapiens
  source 1..16016: mol_type = other RNA
attaaggacatttgtgattgatttttaggaggaagtaatggttctggagagaatcttactgcagaccatcaagtttgatttacaggtagaacatccataccagttcctactaaaatatgcaaagcaactcaaaggtaagaagaaagttttcagaagaattttttcattctgaaatcaagtctttataatttgatgacactcaaattacgcttctcaaaagcggaaaacaaagtttgatgtgtgaaataccaagggcatggcttgctcagtcaattcagcattgcagctgctaatgctgtttccttttatgtataaacaggctctgtcatccagttgccaagtgatgggagaggcaggaaaatgaggcagaattttttaaatggactaataaacttagccttggagccaggttttccatacatggtggttcagcgtaggtcatgaggaggaagaaggggtaggatgtggacccacatcattcatccttgtttcccacgcaaaagctctttgctgtgtatttgagtggtgctgaacacgtggtaggtttttaataaatacttgatgctgcctgtgaatttttctattgctattaatttacctttttgtccccatttctaggtgataaaaacaaaattcaaaagttggttcaaatggcatggacatttgtaaatgacaggtatacatgttcaaatgttgattaattacagtattttaaaataggcagagactttatggaccatttcatctaaacccctcattttgtgtcagaagaaactgacttgccctggcttgaggagccagttaatggcaaagctggggctgacgtccaggtcatctgcttcccggcagagggtttccttctgccctgccgtgtcatggtgttgtgaggtgctgaaattttatcaccagtctgaaacataagtccaaaacaatacactggagaattttgaaaactaattacttagagcccatttggttttgcaaaaatatacttcctggtatagttttagagccttaacactcttttgagaggccagggatctaatgaggggccgtggtgggaaacagaatgcctgtgaatggagttgctgccagccccatcccactgcagtcagtgaagcttctcttacatttgacttcctccataagatttcatttgaagaaacagttgagtggctaggatttcaacagtttaaataacataagtcattttcattggtgtagcaatttttggatgtgctagaattcttctgattctttaaggaatagagaaattactaactatggttaaagtaacttagtcgggtacctttagaagagtaaagacttgagtttatttatttatagtactttaattaaatttaggggagaataagcaaattaatggttagttatggcatctccatgcactggtttaatcataaatattagatcatattatctaacctttttttttcttgttgaactagtctctgcaccaccttgtcactgcagtgggaaccagagatcatagcagtagcagtgatgtatctcgcaggacgtttgtgcaaatttgaaatacaagaatggacctccaaacccatgtataggagatggtgggagcagtttgttcaagatgtcccggtcgacgttttggaaggtaccaggcatgctaagcgttctcgtgagggtgttccatgttgagatgattcttccatgtgtaccctgagtcccaagaatggattttcccagatagacatatgtgagcaatatttcagaagcatcattaattaaattatctaatagtttccactttgtccaaacacatacttttggtaaactaaaaatacacaccagtgttgcacacaacgaagatggggtgagttgtaaatgtgattcatgcttaggtcctcgtaggggtatcataactgattctttatccaggtaaaattttatttaaaataccaatttgtgtaaaatgtaattgttggctatcatttagacatctgccaccaaatcctggatctttactcacaaggaaaacaacagatgcctcatcacaccccccatcagctgcaacagcccccatctcttcagcctacaccacaagtgccgcaagtacagcagtcacagccgtctcaaagctccgaaccatcccagccccagcagaaggacccccagcaaccagcccagcagcagcagccagcccaacagcccaagaaaccctctccgcagcccagttctccccgacaggttaagcgagccgtggtgagtgggctaaagcaggccctgggtagagcaggctttccaggtggcggcaacacctgagcactgttcccatttctaagcgagcacagggaacaccggaagcagggggtgttcgccgaaactcgcagtccgactgcttgtcggtggggagcctgaaaacaaaggtgctccaaggacaggctgcctctgagaaccaggagggggctctctgcccggctccagccctgctgcctgtttcatccctgccagggttctgaagcctgtcggtgtcgttgccgtgtcctagcagtgtcgttgtgcatgctgcttctgtgcagctgcctgaccccaaacagtggaccgtttcctgcacccaagtggtcctgaaacttagtgtttactcagaactcaccattcaggaaagctagtcattctgtcttatttggtaaatggaaagaggaagggagcagaaatgatgatctggtaggtgccgtggtttgccctgaaagttcaggctagaaataatttttgtccgaggctgttcacagtgactgccgtcgctgattctggtggtacctggataatccatttttttctcatcatactcaggatcccagttaacaattgtgtattttcttttgtaacaggttgtttctcccaaagaagagaacaaagcagcaggtaatttcctgttctgatgtttttttagttttatgtgtttatatgcaaaactttaaattcttagccaacattgtttcttttcagatctaaattggccttaaatcttaactttagagctcatacaaaacttttccatcagcattgtctttctgttcatcacctgatcatagattctaaaattgtgctcttacgaagctatcagtacagaaaacattactggcaataaaaatgtactcagtaacatatataaaagtataattatggctgtaggagaactgttgctgcaattttatttttagagactatttacccccatcacagcagcaggagtcctctcccaagcaccaagccacagcagatgcgggggggcagtagggggtggtgtgctgcccggacagcaccagcccggcccagcccagctgcccttgcaggcaaggcctctttgaaacacacttgggttgaggtgctgtcacatgtctagaacccaaagttagttcatgtcaatattggaaataaacagaaggagtgagcaaaattggaacaattacaaaacagaaagttagaaatgttttgtcacagggtcagtccacctatcatactgaactctttgaaggcacagaccctattgactcatttgtctttctttgttacttggttcttagttccagtagttcctggttcttagaaccatgttctcggttcttagttccattcattaaactgctgtgaaatcttccagttatgatagagctactttttttttttttccagtatatttgagggaatgatgagttcagtacaggtgaattttttttttttttttgagacagagtttcactcttgttgcccaggctggagtgcagcggtgcaatcttaactcaccacaacctccgcctcctgggttcaagcaattctcctgcctcagcctcccgagtagctgggattacaggcatgcaccaccaggcctggctaattttgtatttttagtagagacagggtttctccatgttggtcaggcaggtgtcaaactcccgacctcaggtgatctgctcgccccagcctcccaaagtgctgcgattacaggcatgagccaccgtgcccagcctacaggtgaattttttaattagcttcaaattgaccgacattaaatgttagacacaagaacgggctacactccatgccacatgaaatgcaattgagttgacgtgcaggtctgtcagaggcaggaaacaaactatatatgaccttgaaggaagagttgcatttgagcagcgagagcagagggggaggatggagcaataagttggaagtacgcaagtgagcaaaggaattgagaatcaggggaaatggagaggagtctttctggaatgtgatgaattgaaaggcaatagcttctgataggatctaaaatgtgggttaggaccagatcacagagtttacctggaggactgtgagtttggcagaggcaagggaagccattggagatttagcaggggaatggcagagtctaaattcatttgagaaggagtcccctggcagcagtaaatagggcaagtggttaggaatggggagaatcttgctggcactcatgggaaacatggtggcctcagcatgctggctgcggggcaggaagggcagatccggaggaagctttatagaggaactcagctgcactgtgccatgccgaaggctactggctgcagagggctgcaagcactcgaaatgtgactgggtcaaattctgaagcactgacaatgcaaaatacacagagatttccaagaaaggagaacgtaagacatctcattagtaaagctttatattggttacatgttgaaataaaattttcgatctatcgggttaaataaattttatcctttttccttttatttccagagtcttgctctgttaatgcaggctggagtgctcctttttcttgttaaagtggttcctggcacacttgtaatcccagcactttgggaggccaaggcatgctttgagcccaggagttccaggccagactgggccacatagggtgaccccatcactacacaaaacttaaaaatcagctcggcgtggtggcgccacacctatggtcccagctacttgggagactcaggcagcaagatcacttgagcctggttggttgaagctgcagtgagccatgattacattactacactccagcctgggtgacagagcgagaccctgtctcaaaaaataaaatggctcctggaaagtttaaaattgtagatatgtggctctcagttatattgctgttggacagccctgatgtagacggctttagctaactattaccagctgtggaaaaaggcaggaggtgggtccctgaggtgagagtaatagcagttataggatacagaggcaaaaggtagagtgtgaggtgctgattggtgggtctagggatgggccatggttttggtggcaagatggacgctagaaatgtaggtttgtagttgtccacttagagaggggctttggactctgaggaagagggtgaagagagaggaagtccctggaacttaaattgagcctgtatttgagatggaggaaatccagagaaagaggccagtgatggcagaggagactcagatctgagtggtgtacaagccagaagaaagtacatttcaggaagaaaaagcctcagcatgcaaacagaaaaatagggttctttttcagttgtgatgtgcacgctgccttcttaaacggatgagattggacttcccttgggctgccttggagacctagtgctgtcattgtggattctggctgcgtgccgctgcctgaccccggaagggtgggctgtttcctccacctcaaggggtcctgactgctgggcttttgtgagcggcacattcttcctgccatcagtgtgtcaacctccagagctctgctgactccagttaatgtgctgcttctgacatgctgccaactggaagtcagtatttgggaaagagagaataaactatgtctaagaatgaaaagatagagattctcttgtggaaccctcaggggactcagtgacatgatgttgctactctggacccttctttgtgtcctctgtaccagggaggactccagataggtcatacatgctcatgaagacgttgctctgctggtctcacatggtcggaaggacttgagtgaagtggtcagcaaggaaacttaggtagacatggaaaatgggctgcctgtgggaagctcgcaggtcttttggagggaggtggcatttaatttgttaacaggattcatgcataatggtttagctgaaaccttcttcaagttcccttaaagccttggtcatctctgttgtttttctcccaaagaaatctctgccagtacatttttctttatgacatgcttattcatgtgaagaagtatgagtggttttctaatctgctttttctttgtagaaccaccaccacctaaaatccccaaaattgagaccactcatccaccgttgcctccagcccacccacctccaggtaagcatctgctgaagcagcttggccagctgtgcacatcgcctctgaatgttggacgcagcaggtcctgggaacttagaaaagggagactggggcccagattgacaatgtcagccacaggcaggaatctttgcaaaattgttcttgggctgggcacaatggcttgtgtttttgatcccagcactttgggaggcggaggcaggagaatcacctgaccccaggagttcgaggtcagcctgggcaacaaagtgagaccctgtctaaaaaattagccaggtgtggtagcacacacctgtagtcccaactacttaggagtctgagatgggaagatcatttgagccctgggcagtcaaggctgcagtgagctatgattgcaccaccgtactccagcctgggtgagagggagaccgtgtctcaaagttctgattttgaccaggtattttgagaatgttgtaaattgttaagtatatctgaatattttccgacctctcacatccagaaatgctaaactacacattgtattagaatcagttttaggaaagaaagccaaaccccgccttctgagatagaggcagggttactgtggctactaggctccggccgcccctacacctgcttcctattggcagtgtgtcgtcttagtgcattctgaagaataagcaattgtacagagagtaaatgaaagagtgaaaagttctcaacaagtagtacatggtaagctggaaagcctctctgataccgctggcaatagaggagaaaagctgtaaagtagatggcattctttacctgtggcaccatttcagaaggtgatgcgctagagaaggccagagtgacctgtgcttgctctccaaaaggtggtcgatactccggaggcttccaagcctctgtcagcagctcctccagcctgctacactcactgttggtcggtgcacgtggctcacactggggctgacagcactgtgtgcccgtaacagatgtgccacagattacatttctgttcctactcaatcatgatagtgtttgtgctttgggagaacagaggcgtcattttccactttggggccaaatcccaaaacccccaattcaatatgaaccttacttaaatgcctgtggttgctcatgaagcatttatggagcacctcctcgccaagtgcagttcccctggtccgagcctggggctgtgccttcactgaggagatgggtggtttatctggggagcctggggcagccacaggggtgctgctacctccagggcactgagtagctgctgtggaggcctcagagctctgctccctcccccattacagatagccaggagtaggcctgggacttgagtgggacctgggtgccagatacactgccaggaggccatggctgaagagagcagggcctgggaggcgcagtaaagctgggccgtgaggaagggagggaagtacgcttcctgggaggccctaggccatgggaagaggcattcaggtcagcagtgatgtttagggagcagtttggtggcagtgtgtgggacttggtcaggagcaagtgtacagagagggaatggggtgcccaggagagacccccacttgctgttccagctcagtcacacagcacaagggcaggcacactggtgacttgaagattcaggctacagggtcgagtgttggaaaagttgatttctgcaaggtggaggagcaggcctgtgggcccaggtggctgtggagtgacacacaggaggcattgaagggtgtcagcacttttctgcacctcttttttagtcagctcctagaaccacagggcatctggccctgacctggagccaaagccagttatctaaggccaggcacatatgaccttcctacccggtaggctggcggggtgctgatgtggcacaccagtggcacacctgttaccgacctgatgaaatcctgctcatgctcgctttggcaagatcaaacgggttgtgtgccaatggccacgtctacccaaccaggatgtcgtgctgtgccttgcctaacccaagtgcctggggaaccagaagcatcttcgtggctttgtcctctctatgttctctggaaccagaaatgttgctcctgtggtctgtctcctgggctgccttgggaaaggacactcattctgtgtgtttggctacctgtggtggggtgttgcgatgtcattttccagtggtctgacggtgacccgggatcacaggccaaaacatgttaaataaggctttggcagaagggggcgtgagggctcatgggttgggaggcgctgtgggaggggcctgaggctggttctgagcacgagtatcttgggcgtgctcaacacctagtgctgcctgtccctgctgcacacgcagcacgcacacacacgcagcacgcacagacatgcagcacgcacgcagcacgcacacgcacacacatgcacacactcctctcaaggaggctgctatctgagagcacacagtggggtttgatgtagcctctcttgagtagaatagaacctgaattgctgcttcgatgggtacaccgggaatgtcagagacttgtacagaattgttttaagtgccatcacattcatttgactaactctgaggttttctgcaaaatgccactgctgcagacaggagttcagtgtggccctgacccctggggtcagtttctgaaggcagaaaaacagaggagcccccacacgttttgcactaggaagagggggctggggccagggcacaagggggcttcgggtgctgccgagactgcctgtaggtggtgtggtcagggctgagggagggaaaaccccaggtcgtcgcagacagggtggagggccttcttgacagatggtggggagacatctggtggcatcaggacatggggcatgggcccatgcgttgggccacagaggaggcgggcagctgctccctgctcctctgtaaagatggccctgaagggccaggaggcactgaaaaagcaaccattgctggcggaggccgggcactgatgcgtctctctcctgcagaccggaagcctcccctcgctgctgccttaggtgaggctgagccgccgggccctgtggatgccactgacctccccaaagtccagattccccctccggcccacccggcccctgtgcaccagccaccgccgctgccacaccggcccccgcccccacccccctccagctacatgaccgggatgtccaccaccagctcctacatgtctggagagggctaccagagcctgcagtccatgatgaagaccgagggaccctcctacggtgccctgccccccgcctacggcccacctgcacacctgccctaccacccccatgtctacccgcccaacccgcccccgccacctgtgcctcctcccccagcctccttccccccacctgccatcccaccccctactcctggctaccccccacccccacccacctacaaccccaacttcccacccccacccccacgcctcccgcctacccacgcagtcccccctcatcctcctccagggttgggcctgccgccagccagctacccacctcctgccgtcccccctggaggacagcctcctgtgcccccgcccattcccccacccggcatgcctccagttggggggctggggcgggcagcctggatgagataacgtgagccttttttccctctttgtttttttaacaagattttctaatcgacttgcagagtagttgaagtgggtaagcagcagggtaccttgtataatgcacgacagttgcagtatgggaagaatggaccgggcccctgggataaaatcagagtggtcctcacacctagaggacggggacaaccagctttcagagtagcctcatcagtgcccttgcagtctgactgtgtacacttggttcagctaatgtctgagagtcctgcactgggttactttatactagtgaggacgttaaccagccatattggctcaataaatagcttcggtaaggagttaatttccttctagaaatcagtgcctatttttcctggaaactcaattttaaatagtccaattccatctgaagccaagctgttgtcattttcattcggtgacattctctcccatgacacccagaaggggcagaagaaccacatttttcatttatagatgtttgcatcctttgtattaaaattattttgaaggggttgcctcattggatggctttttttttttcctccagggagaaggggagaaatgtacttggaaattaatgtatgtttacatctctttgcaaattcctgtacatagagatatattttttaagtgtgaatgtaacaacatactgtgaattccatcttggttacaaatgagactccttcagtcagttatccaaataaaagcagttctgaaactatccctttctttgttatgggtggaaggtggggctccaggccttcgcagtctgtggcttataaaatgtgcagaggccctccttccagaccctggggacgcgggagaggcctggctgcagctcacagcagccacagccaaccccactgcctcccaaggcactctgggtggatccgcacagctgcctgccaagccagcctgcccccatcctgtgcctgccttggtttcctttggaggacctggttgagttccaaaccagtttgaaactttgaagccttgctgcgtagaacgcacacaggaacccgggggcttggatttgaaaccctttccacttctggcctgtgatgagacagaggcagctggaggagcagcggcctcactgtccaccttgaggggccacggctctgtctgtggaaggggccccgactgagcccccatctgcggtgcttgaggggccttggccctgtctctgcctgctgaccctgccacccacgacagaaacaagcactgagcacccagccaggaggctcacaaagaggcctttatttatctagctcaaagtagacactatcacaatcttgtttgttactccttttactaaaatagttcaaatcaatgtttttaccacactatcaaaaagttctatttcttcttgtctccccacgtcagagtggttgaatagaaggtagaaacaggccgggagtccacgggctcccagctctaaacggcgccagggcaggaaggggtggctccaggtctcactgtggcaccttctacagaaaatagacgtagctgccgggcccggggacagaaaccagacgttccagtccatctccaaaaagcagcacaaatactttgccccacagtatgaaaaatatacacctctaccgctctgcagtcatgcatttagttttaagaaaaaaaaaaaatcagtagtatgtatcttgtttcctcaagtttcaagaaaaaaaaaatgaaaggtcacttttttctctttaaacactgatgtgtagctagtaacttggataaaaaggtgccaccctacaaaatgtgctcagcatgttctgaggccaggatgggcttggccacctgggctggggcgaaaggagacctccatctgtcacagtggaaactgaagccgagtgccagtgccgcgtccggcttcaagatcaagagtcagagcctttgaaatggaaagggggcatctgaaagggcacccccactgggggctttcagagctaaggctccagaaggaagggggtcgccctgctagtgacggagctgggagtcaccctgagctacagcatgcccagatttcccctgtgggaagccccatctgaccttctacagcccacggctctgcaactgccacctgtactcaggtacatggcgtcgctgctgctggcttttaaaatcagctattagtttgagatgtgacagtcgccgacagggttctgtcctagaaagccatcccagtgccgtgttggctcaggggtcaccagctttgtgctgcctccgtaacagcaggagggttctcaaagcaatgttccactgatccctggatgccactgcagcattaaagacagggtcagtccccttgaggggaaaggtggcttcaaggctgttctctgggcctgtttgcaggagatccgcaggtaccaggagcccgtacttattgcttatttcagtggtggccacgccaacctgacccaaacatgatgcacacgggctcccagacttggctgccactcaaaatggacccacagcccttgggctactctgcggttctttggactgcaagacccagaggggcctctgctcagctgcccactcgggcaagaatcactgggtaccatgagcagcaggtgttcacccaacttcacgtgtacacccctagtgaccgggagcgcaccacctgaccgggcgacactccttcccaaagagcctcctggcaacacccacggcaggagcgccacaccatcccatcaccagcacccacttacccccctggggctaagatggggggcgtgagcctttcccctgagagcaaacgggcagcaagaactgctcagaatagagccgccagctagggagagggacagggcggccatctccctcctcttgcctgcatccccagccctgggcctgcatgagacctgctgggtaggaagacagcctctctgggctcttcaggtggggctgagcagcccctggaagagcacaggagtctgacgaggacctggtgaggtcctggacccaagagctagggctgcttacagtggcatgagcggatgtggggaagcggcctgtccccgtgctgcagctgtgggatcaaaatccctgtcatgtgccacacatcaccccctctaggccttactttcctcacacacacagttttctattgcactttacagtttatacatggtcatttacactgaagatctcacttgatgccagaatcctgtgaggagggccttatgctgcccattttactactgaggacacgggctcagagtggggaggcaactctccacccgcagcgactgcaaggcagcagaactcagctccacccggcccgccctcagccgtcggctgttggctcacgccccctcagtgaggacccctgccctgtggcgctggatgacctggagccataagcatggccgaaaaggaacctcagagacctgtttccaccaagagcccagacaggctgagtgaactgctaaaggtcacaccacaaactaaaggcagaacctggccagacacgctccttcccaaaaagaacagaactctcatctgcagcctacacagctctgtccacagggacccaagatgcagccaggccctgggggaggtcacagccaaccagagccccagctgtggcccagtgctgcccatcaggaaaatcacatgtggctcagcccagaaactctccccaggcccttcctgttactggcctgtcatgtaaaccacgaaaagggacgtgcctcaggcatggggcaggaggagcccaagaagggcatagcctggacagggtggcagggggacattgcagagactgggggggagggggatgacctccaaaagcaaggagcagcgggcatcgggtggctgagcacagatccccaggtgtgagggcaccctgacctccaaggctgagggtcacaggaagggcccagggcagcctccagccagccacagatgtggtgagtggccttgtccacatgccggggacccagtgcttggggggcctggggccaggccacggcatttgggcaagaagtggtgccacctgcgtcaagacccaggtagtggtggtctctgtccagtgtgggtggcagccggggagtagagggtttgatgagtggcccctccatcccaggcaggacagaggagcctggacagttcccaggctggatctcagaagcagcctgcagcctcttgctcatggagcccagggcccagagggggaatgaggcgtccgggccgctctgctgcaggaacagtcgcagcgtctcgtcttcccaggttgctggtgtatgaggcgggagatggcggcttgggccagtgcatcggacccatggcagctgggccagggcgggcagcgtcctatgtacagttcaccacagaggaagaagacaggggctgggctggaggtcctgcccgtgtctggggcctgaaactccccctggggacccccagcagggccagtccacgtccacagaagagtggccctacaaaggccccttgaactggttcccagacaggtgctgccgtatggagggcttggagctggctgcatctcccagctttctccagaccacgttgcacatctcgcgaacgatggccttctccttctcactcaggtcctcctcacagctgtcctggagctgccggtccagattctcgtgtacctccaggaccttcatggcatgcacgacagcctcgggcttctgtcctgcagggctgtagccagcagaggggggcgagggcagctcaggtgcggggcaggccgggccgttctgcagggagtcctggtaggagggcggcagggacgcaagctgggactccgagtggtagggcgagaagcctttccgcagcgtgcggaactctccggagcctgcctgctgtgcgaggagcttgtcaccctccagcagcctcactttgctctccagttgcctgatgtaggtggatgagggatcgtgcaggccgttggggatgctgcggtggtgcggcggcgccgacaagtcgtccagggaccgacgtgtggctcctgccttgccgtcgggggccttgtgcggcccggggggcagcagcgggggtgggacgtggtggtggtggtcggggctgccgccgctgcccgcgctggacgtactgctgccgtcgcccacgtcgcgggcccccgcgccgggcgcgccacccgacagcggcccgctcaggctggcctggctgtcgatggagctgcgggagccggcgccgcccccgccgccgccgccaccgcttgcggcccccgtcgccgccagtgccgcgcgctcctcgtccagcagcagcaccagctccttgagctccaggttctcgcgcagcagggcctcctggcgcgcctcgagctcgcgcagcttctgctgcgagcgggccacctcgtgccacacggcgccggccgcgtggcgcccgaagcgctgccactcgcgcgccagcttgcgccccttctgccggtcgtcgtcgaggaagcagcagagctcgcgcagctcctggttgtcgtcctgcagccgctggttcacgtccttgaggccgcggatctccagcaggtgctgctgcagccgccggttcacgtcgcgcatcaggccgccgtgctccagcatgaggcccaccttctcgccctcggcgcgccgcagccgccgcgccagctcctccttgctccagcgcagcagctcctcgtccggcacctggctcagctcctccgacgccgccgccgccgtcgccgcgggcttagccatggcggggccgtcaccgcggcatcgccctcgccctcgcccggccggcgcttccccgcgccggggctccgctgggccggtccgcgcgcgggcggggggcggccgggggcgcgtgcggcccgccccgcgccgcctggcgcgtcctctcgccgcgcccgccggggccgcccgggagcccgcgcgcctcggggttgacgagcggaggcggctgctgcgtcggcggccgcggtgccgggcgctctcagggttct

SEQ ID NO: 9762 - RNA, 1330 nt, Homo sapiens
  source 1..1330: mol_type = other RNA
attctgcatttttagcaagttcccaggtgatgctttgatgctgatagtccagggaccacactttgagaaccactgctttaaaccgttagtttataagttctttaaagagcaatgtaagcttagaatccagaacctacatggtacttactaaactctcttcagagctgtgttccaggggcattccttgagaaaatcatttttttttttaaactttcttcttttagcaacagtaatgcccaggcagctagagagtccttaatattcattgcttagcattttggttttgctgggcctggactgggagtattccctatttctcatcagaagggctgcaatctactgtgtatctccaagatgttctggatctaaactctcccaggataggatctatgcctctgggggaccaaagccacagctacatgtctttacccagtaagtctatctcatccaggaggaagtccatgtcctcccggctcacttgagggctgatcaccacctggcggaagaagttgacctttccccggtgcggctggtagcccagcatcaagcttcccttcttcatcatcctctccttaatggctggggccaccaaattaagttttgcccagaactcgggtccttcttccatctctctgaggctcggtggaatgtaccaaaagcaaatattggcatattcaggttccatcagtaacttgaatccttctcttttcttgatttcatctactaggtacctagataaagcaagagcacgattaactctttcttcaaggcctaatgtacccagggccttccaggtcatccagaacttgaatgcatctggtcttctgctacactggatagacttgtctcctgtgtcatagctcacatcatagaatttatcctgctggaagaggtaagatgccttggcagagtagcattttttaagaagatcagatttgtctttcacaaggagagcacagcactggatcccagccatcagcatcttgtgtgggttccaggccacagagtcagccctgtggatgccatgcagaagcttgcggtgcttcctcgacatcaaagctgagccaccccaagaagcatctacatgaagccagaggctgtgcctctcgcagatgtctgctatttcatccagagggtcaaaagctcccaacacagttgtaccagaagtggcacagacaagaaacggtgctgccccctcttttctggcttgccagacttgcttctccagttcctcaggtatcattttacctctctgcagatgtgaaaaggattaatcttggcgaaccagacagccccttttccttaatatcaggacaatatttgtatctag

SEQ ID NO: 9763 - RNA, 2028 nt, Homo sapiens
  source 1..2028: mol_type = other RNA
attctgcatttttagcaagttcccaggtgatgctttgatgctgatagtccagggaccacactttgagaaccactgctttaaaccgttagtttataagttctttaaagagcaatgtaagcttagaatccagaacctacatggtacttactaaactctcttcagagctgtgttccaggggcattccttgagaaaatcatttttttttttaaactttcttcttttagcaacagtaatgcccaggcagctagagagtccttaatattcattgcttagcattttggttttgctgggcctggactgggagtattccctatttctcatcagaagggctgcaatctactgtgtatctccaagatgttctggatctaaactctcccaggataggatctatgcctctgggggaccaaagccacagctacatgtctttacccagtaagtctatctcatccaggaggaagtccatgtcctcccggctcacttgagggctgatcaccacctggcggaagaagttgacctttccccggtgcggctggtagcccagcatcaagcttcccttcttcatcatcctctccttaatggctggggccaccaaattaagttttgcccagaactcgggtccttcttccatctctctgaggctcggtggaatgtaccaaaagcaaatattggcatattcaggttccatcagtaacttgaatccttctcttttcttgatttcatctactaggtacctagataaagcaagagcacgattaactctttcttcaaggcctaatgtacccagggccttccaggtcatccagaacttgaatgcatctggtcttctgctacactggatagacttgtctcctgtgtcatagctcacatcatagaatttatcctgctggaagaggtaagatgccttggcagagtagcattttttaagaagatcagatttgtctttcacaaggagagcacagcactggatcccagccatcagcatcttgtgtgggttccaggccacagagtcagccctgtggatgccatgcagaagcttgcggtgcttcctcgacatcaaagctgagccaccccaagaagcatctacatgaagccagaggctgtgcctctcgcagatgtctgctatttcatccagagggtcaaaagctcccaacacagttgtaccagaagtggcacagacaagaaacggtgctgccccctcttttctggcttgccagacttgcttctccagttcctcaggtatcattttacctcttccatctgtttccacaaagcaaacattctcagtgccaatcccaagaaaagaggctgccttcttcatagagtaatgacactctgcagatgtgaaaaggattaatcttggcgaaccagacagccccttttccttaatatcaggacaatatttgtatctagctaaattcattgcatacatattggacactgagccacctgggttaaatattccatccccttctttccagccaataaattcaatcattttcttcagaaccgcttcttccactaacagaaacactggggacacctcatacgtataaacacttggattcaatgcttcggtcataaatcgggccaccaaggagtaataatcaagtccagcatacaattggttgaaaaatcttgggtggttagttttgacactgtagtgtatgacatcccgacagagttccaatagtttatggggtggctcgcctgagtctctcatctccaaatcaagaagctgtttcagttgttcaggaggcctccattcacacaccttctcattgacatctgtagctttcaaaaccacctcttccattattagcctacaggcctcttcaacaaatttttctccagcttttgcatctgttgtaggaccattcagcacaaccccatccacaagaacagcattcttcttacttggaatcatctcttgttgatcaatatctccgtccacaggacactggcggtccgagtcgctgctcatctccgctcccccactccaggctgccccgggcgcggctcccgcagtct

SEQ ID NO: 9764 - RNA, 2426 nt, Homo sapiens
  source 1..2426: mol_type = other RNA
attctgcatttttagcaagttcccaggtgatgctttgatgctgatagtccagggaccacactttgagaaccactgctttaaaccgttagtttataagttctttaaagagcaatgtaagcttagaatccagaacctacatggtacttactaaactctcttcagagctgtgttccaggggcattccttgagaaaatcatttttttttttaaactttcttcttttagcaacagtaatgcccaggcagctagagagtccttaatattcattgcttagcattttggttttgctgggcctggactgggagtattccctatttctcatcagaagggctgcaatctactgtgtatctccaagatgttctggatctaaactctcccaggataggatctatgcctctgggggaccaaagccacagctacatgtctttacccagtaagtctatctcatccaggaggaagtccatgtcctcccggctcacttgagggctgatcaccacctggcggaagaagttgacctttccccggtgcggctggtagcccagcatcaagcttcccttcttcatcatcctctccttaatggctggggccaccaaattaagttttgcccagaactcgggtccttcttccatctctctgaggctcggtggaatgtaccaaaagcaaatattggcatattcaggttccatcagtaacttgaatccttctcttttcttgatttcatctactaggtacctagataaagcaagagcacgattaactctttcttcaaggcctaatgtacccagggccttccaggtcatccagaacttgaatgcatctggtcttctgctacactggatagacttgtctcctgtgtcatagctcacatcatagaatttatcctgctggaagaggtaagatgccttggcagagtagcattttttaagaagatcagatttgtctttcacaaggagagcacagcactggatcccagccatcagcatcttgtgtgggttccaggccacagagtcagccctgtggatgccatgcagaagcttgcggtgcttcctcgacatcaaagctgagccaccccaagaagcatctacatgaagccagaggctgtgcctctcgcagatgtctgctatttcatccagagggtcaaaagctcccaacacagttgtaccagaagtggcacagacaagaaacggtgctgccccctcttttctggcttgccagacttgcttctccagttcctcaggtatcattttacctcttccatctgtttccacaaagcaaacattctcagtgccaatcccaagaaaagaggctgccttcttcatagagtaatgacactctgcagatgtgaaaaggattaatcttggcgaaccagacagccccttttccttaatatcaggacaatatttgtatctagctaaattcattgcatacatattggacactgagccacctgggttaaatattccatccccttctttccagccaataaattcaatcattttcttcagaaccgcttcttccactaacagaaacactggggacacctcatacgtataaacacttggattcaatgcttcggtcataaatcgggccaccaaggagtaataatcaagtccagcatacaattggttgaaaaatcttgggtggttagttttgacactgtagtgtatgacatcccgacagagttccaatagtttatggggtggctcgcctgagtctctcatctccaaatcaagaagctgtttcagttgttcaggaggcctccattcacacaccttctcattgacatctgtagctttcaaaaccacctcttccattattagcctacaggcctcttcaacaaatttttctccagcttttgcatctgttgtaggaccattcagcacaaccccatccacaagaacagcattcttcttacttggaatcatctcttgttgatcaatatctcctcttgatgacagaaggcagttgtcacatcattgcaaagtggtaagcatactaggaagaaaggattctgaaaccaattttgcaatctatcatagtccagtctctgatcaaaattcatattcctctcatccacaaaatatcctcattcccatatgaggaccttccaaaatcttatctcattatagaattaggcttgaagtccagaatatcgtggtctgtgtcttgtctataggcagacaagactgttcagttatgttcttggtccagagacccctaaactaaaaacacaagttatcagatgtcgcacacaacatacaatagtcatgcaggccaggataatttctgcagacactctcacgaaagaataggaggcagagggtaatcactgtcttacagcagttctgaaatcccgctgggcacatacttcacatattaaataggatctgatttgccctctcgggtggtttcctaatccagtattct

SEQ ID NO: 9765 - RNA, 288 nt, Homo sapiens
  source 1..288: mol_type = other RNA
attcttcctgccctggctccatgggaacgccctctggctatcgtccttgtttggccactcaacttcctgggggaagccgtttcaagcagggctctccgggctccagcccgagcactccggggtcgccgcggggtgcgcgggtccgctgtatccagcacgcgtcgcagcagcgtgcgcggcgtggagtcgctgtcagggttgtggtcagccatcgtctcggccccgggccctcctaaccgcccagccagctgcaggctccgccttcccgccgccacagttaatgtaact

SEQ ID NO: 9766 - RNA, 665 nt, Homo sapiens
  source 1..665: mol_type = other RNA
attgaaacctctaagagtggaactccattaatgcttccaggtgcatcaaggtctactcctttgacttttgtccctgtagttccataaactcttccccctgtcttgatgttaagatttacaggtgctgtaccataaccatactgtggtgctcccgttttaatgtctcctatagtgacatgaacatcatcttcatcatcatcgctgtcactatcactatcatcttcggtctcagtcactttcggttttggtacaccattttcagcagtttcatcttcaattccagatggaggattagcactggcattttcttcttctggcctttcaacttcattttcatctaggtcctttgccaaatcactgtgcacatgcacgtcccatgggccgccatagagccactcttcctcctcatcccctccggtcccgccgctcagctccgacactaggcgctcgacctcgccggccgacatggccgccccgagcgcaacttaaacgcggcgatcaacagccccctccaaccccttccccagcctcgcagccccgaggcgcgagaagggcgcgaacccgccgacgaacgaacgaagaaagctcgagactccaatcccaggaaggcgacggcagcggcggcaaagatgaagcctccagcgcaggtccgtctgcgcatgcgc

SEQ ID NO: 9767 - RNA, 609 nt, Homo sapiens
  source 1..609: mol_type = other RNA
attgaaacctctaagagtggaactccattaatgcttccaggtgcatcaaggtctactcctttgacttttgtccctgtagttccataaactcttccccctgtcttgatgttaagatttacaggtgctgtaccataactcccatactgtggtgctcccgttttaatgtctcctatagtgacatgaacatcatcttcatcatcatcgctgtcactatcactatcatcttcggtctcagtcactttcattttcagcagtttcatcttcaattccagatggaggattagcactggcattttcttcttctggcctttcaacttcattttcatcgccatagagccactcttcctcctcatcccctccggtcccgccgctcagctccgacactaggcgctcgacctcgccggccgacatggccgccccgagcgcaacttaaacgcggcgatcaacagccccctccaaccccttccccagcctcgcagccccgaggcgcgagaagggcgcgaacccgccgacgaacgaacgaagaaagctcgagactccaatcccaggaaggcgacggcagcggcggcaaagatgaagcctccagcgcaggtccgtctgcgcatgcgc

SEQ ID NO: 9768 - RNA, 623 nt, Homo sapiens
  source 1..623: mol_type = other RNA
attgaaacctctaagagtggaactccattaatgcttccaggtgcatcaaggtctactcctttgacttttgtccctgtagttccataaactcttccccctgtcttgatgttaagatttacaggtgctgtaccataactcccatactgtggtgctcccgttttaatgtctcctatagtgacatgaacatcatcttcatcatcatcgctgtcactatcactatcatcttcggtctcagtcactttcggttttggtacaccattttcagcagtttcatcttcaattccagatggaggattagcactggcattttcttcttctggcctttcaacttcattttcatcgccatagagccactcttcctcctcatcccctccggtcccgccgctcagctccgacactaggcgctcgacctcgccggccgacatggccgccccgagcgcaacttaaacgcggcgatcaacagccccctccaaccccttccccagcctcgcagccccgaggcgcgagaagggcgcgaacccgccgacgaacgaacgaagaaagctcgagactccaatcccaggaaggcgacggcagcggcggcaaagatgaagcctccagcgcaggtccgtctgcgcatgcgc

SEQ ID NO: 9769 - RNA, 663 nt, Homo sapiens
  source 1..663: mol_type = other RNA
attgaaacctctaagagtggaactccattaatgcttccaggtgcatcaaggtctactcctttgacttttgtccctgtagttccataaactcttccccctgtcttgatgttaagatttacaggtgctgtaccataactcccatactgtggtgctcccgttttaatgtctcctatagtgacatgaacatcatcttcatcatcatcgctgtcactatcactatcatcttcggtctcagtcactttcggttttggtacaccattttcagcagtttcatcttcaattccagatggaggattagcactggcattttcttcttctggcctttcaacttcattttcatctaggtcctttgccaaatcactgtgcacatgcacgtcccatgggccgccatagagccactcttcctcctcatcccctccggtcccgccgctcagctccgacactaggcgctcgacctcgccggccgacatggccgccccgagcgcaacttaaacgcggcgatcaacagccccctccaaccccttccccagcctcgcagccccgaggcgcgagaagggcgcgaacccgccgacgaacgaacgaagaaagctcgagactccaatcccaggaaggcgacggcagcggcggcaaagatgaagcctccagcgcaggtccgtctgcgca

SEQ ID NO: 9770 - RNA, 668 nt, Homo sapiens
  source 1..668: mol_type = other RNA
attgaaacctctaagagtggaactccattaatgcttccaggtgcatcaaggtctactcctttgacttttgtccctgtagttccataaactcttccccctgtcttgatgttaagatttacaggtgctgtaccataactcccatactgtggtgctcccgttttaatgtctcctatagtgacatgaacatcatcttcatcatcatcgctgtcactatcactatcatcttcggtctcagtcactttcggttttggtacaccattttcagcagtttcatcttcaattccagatggaggattagcactggcattttcttcttctggcctttcaacttcattttcatctaggtcctttgccaaatcactgtgcacatgcacgtcccatgggccgccatagagccactcttcctcctcatcccctccggtcccgccgctcagctccgacactaggcgctcgacctcgccggccgacatggccgccccgagcgcaacttaaacgcggcgatcaacagccccctccaaccccttccccagcctcgcagccccgaggcgcgagaagggcgcgaacccgccgacgaacgaacgaagaaagctcgagactccaatcccaggaaggcgacggcagcggcggcaaagatgaagcctccagcgcaggtccgtctgcgcatgcgc

SEQ ID NO: 9771 - RNA, 1123 nt, Homo sapiens
  source 1..1123: mol_type = other RNA
attgtagaacctaagattggccttttgagatgtctttacctgcatttctgatgaccggatggccccacccagaccttcaactcttggctcagccggtcctggggagcccgcccagaagtggacttggtgcacaaggaccaatttccacaaccctgtgattgcatccccaaccaatcagcagcccccattccccagccccctgcccaccaaagtatcctttaaaaaccctagcctccaaattttcagattgatttgatttgagacaggagtggccaaccttgtgtcaattaagctctttctttattgcaatgccgtcgtctcagtgaattggttttgtctgtgcagtgggcaggaggaactcatcaggtgattacatcatcttgcttggcctcttagcgaagaccgcaccggaacttgcagggggcagatggaatgttgtccctggatgggcttcaaactctgcattgttgtccaagaaacaaagttaccaaccagaaagaggtggcaagggccccaaatctgttttcacttcaccatcactttacatcgagcctggtaggggaggctgggcaggggccggggggtgggagttgagttcacatggtccgcaggtgacacagccctggtgggtccaagcccctgacccacgaagcagtgatacttctcacaggtgcctatctccaccgggggttacctggcattttgaccggctggggcaggcagccggggtgggagactgtagaggtaagaggtggggcctggagccctgaggccccccagccctgcctggccacgctgactcagcagagctcagaacctactctccgctgacaaggcaagcgtgctcttcccagctggccgctctcagctgtctcttcaaaccctcccaggagggctgcggagagcagacacgggaaccacacctggcttcttacttggcatggagaagcaccatctggtggctttttccaggcgttttccatatttgctatgggacaccacgcttggttgaattcacaggagggccaatgcctctgggggcctggagtgacgtgctggttccaggagggagtcaggaataggagatctccatttctcgtgttaacacttccttgccaggccc

SEQ ID NO: 9772 - RNA, 2101 nt, Homo sapiens
  source 1..2101: mol_type = other RNA
attgtagaacctaagattggccttttgagatgtctttacctgcatttctgatgaccggatggccccacccagaccttcaactcttggctcagccggtcctggggagcccgcccagaagtggacttggtgcacaaggaccaatttccacaaccctgtgattgcatccccaaccaatcagcagcccccattccccagccccctgcccaccaaagtatcctttaaaaaccctagcctccaaattttcagattgatttgatttgagacaggagtggccaaccttgtgtcaattaagctctttctttattgcaatgccgtcgtctcagtgaattggttttgtctgtgcagtgggcaggaggaactcatcaggtgattacatcatcttgcttggcctcttagcgaagaccgcacctaaaccacatcaaacaagcaatgtgtggtgaagctctcataaagtaggtccagggagagggagaccgcacaggtggcctgcgtcagtgatttggctctgacacagacgctttttctcataagatcattcaggctccttaggctggtttcatatgtcgtggtctcttggttttcgtgtcaatgggatcagagattcacccgcaatttgcattttgaaattaaagttatcgttttgattttcttttgaacaatcttttttcccgaggcaccctgatcttcccccatagccgtgggcatgctataggagatcgattcagatctgagttgaatcctggctctgcccactccctggctgtgtaccattgggttggttatattgcaactccaaacctcaatgtcttcatcggtataataggccccacaatcccatctttgaagagtcggaacaagggtgaaatggctggcatagagcacacccttcccaactgtctgttcctttttttttggcaggggggtggtagttggacatcaaggactttatagccagcctgactctcctgtctcttctagcctcccgtctctcccggtcccgtgactcccagtgagacacatcaatgaaactcagactcgaatctctgtccagctcccagttcttacagaatcagatttggtcttgggagaatgatcgcagcaagggggctttagaatagttccttctcttcattctctgagagctttaaactcaaccttgagttagaaaatcacccctggccccttcctgggtggcagaatcactgctgtcaccagcatcattgcttcagcccatggctggagctgagtggcccagacctcagagggacgctgccctacaggagggcaggctggctgcctaaaaataggaggagactgggtttttggggagggcagcttaagcttgtttttctattatttatataattataaatagtgaccaattaccggaacttgcagggggcagatggaatgttgtccctggatgggcttcaaactctgcattgttgtccaagaaacaaagttaccaaccagaaagaggtggcaagggccccaaatctgttttcacttcaccatcactttacatcgagcctggtaggggaggctgggcaggggccggggggtgggagttgagttcacatggtccgcaggtgacacagccctggtgggtccaagcccctgacccacgaagcagtgatacttctcacaggtgcctatctccaccgggggttacctggcattttgaccggctggggcaggcagccggggtgggagactgtagaggtaagaggtggggcctggagccctgaggccccccagccctgcctggccacgctgactcagcagagctcagaacctactctccgctgacaaggcaagcgtgctcttcccagctggccgctctcagctgtctcttcaaaccctcccaggagggctgcggagagcagacacgggaaccacacctggcttcttacttggcatggagaagcaccatctggtggctttttccaggcgttttccatatttgctatgggacaccacgcttggttgaattcacaggagggccaatgcctctgggggcctggagtgacgtgctggttccaggagggagtcaggaataggagatctccatttctcgtgttaacacttccttgccaggccc

SEQ ID NO: 9773 - RNA, 2026 nt, Homo sapiens
  source 1..2026: mol_type = other RNA
attgtagaacctaagattggccttttgagatgtctttacctgcatttctgatgaccggatggccccacccagaccttcaactcttggctcagccggtcctggggagcccgcccagaagtggacttggtgcacaaggaccaatttccacaaccctgtgattgcatccccaaccaatcagcagcccccattccccagccccctgcccaccaaagtatcctttaaaaaccctagcctccaaattttcagattgatttgatttgagacaggagtggccaaccttgtgtcaattaagctctttctttattgcaatgccgtcgtctcagtgaattggttttgtctgtgcagtgggcaggaggaactcatcaggtgattacatcatcttgcttggcctcttagcgaagaccgcacctaaaccacatcaaacaagcaatgtgtggtgaagctctcataaagtaggtccagggagagggagaccgcacaggtggcctgcgtcagtgatttggctctgacacagacgctttttctcataagatcattcaggctccttaggctggtttcatatgtcgtggtctcttggttttcgtgtcaatgggatcagagattcacccgcaatttgcattttgaaattaaagttatcgttttgattttcttttgaacaatcttttttcccgaggcaccctgatcttcccccatagccgtgggcatgctataggagatcgattcagatctgagttgaatcctggctctgcccactccctggctgtgtaccattgggttggttatattgcaactccaaacctcaatgtcttcatcggtataataggccccacaatcccatctttgaagagtcggaacaagggtgaaatggctggcatagagcacacccttcccaactgtctgttcctttttttttggcaggggggtggtagttggacatcaaggactttatagccagcctgactctcctgtctcttctagcctcccgtctctcccggtcccgtgactcccagtgagacacatcaatgaaactcagactcgaatctctgtccagctcccagttcttacagaatcagatttggtcttgggagaatgatcgcagcaagggggctttagaatagttccttctcttcattctctgagagctttaaactcaaccttgagttagaaaatcacccctggccccttcctgggtggcagaatcactgctgtcaccagcatcattgcttcagcccatggctggagctgagtggcccagacctcagagggacgctgccctacaggagggcaggctggctgcctaaaaataggaggagactgggtttttggggagggcagcttaagcttgtttttctattatttatataattataaatagtgaccaattaccggaacttgcagggggcagatggaatgttgtccctggatgggcttcaaactctgcattgttgtccaagaaacaaagttaccaaccagaaagaggtggcaagggccccaaatctgttttcacttcaccatcactttacatcgagcctggtaggggaggctgggcaggggccggggggtgggagttgagttcacatggtccgcaggtgacacagccctggtgggtccaagcccctgacccacgaagcagtgatacttctcacaggtgcctatctccaccgggggttacctggcttcatgcaggaaaacaaggagtgggatgtgaacaaaaggcgggaggcttcccagctgccctttaagtagaagcttcatctgtgccaaggagaccatgtggttagtgggtaggggagaaaaatgctttgagggtttctgggtcccagctgcctgcacaggcgggtgaaagtcctgcaccaggtttgttgttttgacctgatataggacccttctaggggagaaaatctggagagaagttctccctccctccctcctttccataggagctgaacagctgaacttctactgaagccggggaactcaaggcagggctgacaagccccttgtaattggctagttctaccctctc

SEQ ID NO: 9774 - RNA, 751 nt, Homo sapiens
  source 1..751: mol_type = other RNA
attgtagaacctaagattggccttttgagatgtcttttcagggttttgcatttttgacaaccagtggctccacgtggacctgccaacccatcctgtggcccctcccagaggcagactcagcacatatgcagaaggaccattttccacactcctatgattgcatccccagccaatcagcagcactccattccctggactgccaaactatccttgaaaaaccacagcctctgaattttcagggtgactgatttgagtaataaaaccccagtctcctgttcagctggctctgcatgaattaactctttctcttttgcaattcccctgtcttgataaatcggctgtatctgggcagcaggtaaaatgagcctgttggttggttacataaacttttcagccattactgctcaccttctcccttctcaggctgctcttcagccttgtggaactcctggcagtttcccaaaaatgccaggttgtttcaaatgcacccacagagtcttggctccttcagttctgagtagattcttttaaaccttccctccctattcactctctggggtcttctggagttacctcccgcagcatagatggcatactttgcttccttcattgtttctccaagccatgatgatcatctgcatcaaatccccttgcaaaggtatcttgctcactggggacaggattagcaaacctgacacctctgcaaataattgtcttcctcccgtattcctcctgaaacggttcgctcctt

SEQ ID NO: 9775 - RNA, 2207 nt, Homo sapiens
  source 1..2207: mol_type = other RNA
attgtccctctcccttcccagaaggcactgggaggaggaaatctaccacccagcacatggcaagacccagggcctggccaggcagcgcacacaataagctgggcctgagccaggaggcaggcggggtgttgggggagacaggctgaacggccaggccactgcaacagtgagagacccggggagcccctctgctatctcagccaagaggaaggagagaccaaggcacagagccttaaaaaagacatcctctcccggcctcccatcccaaagccctggcccctaggccagtctagacagaaccaggaaagccaaaaacaaaaggcacctagtatgtaagttcatggggagaacgcaggcaggtgtgggaagctcccacctccaaccccgggccttggctactgggacagtgcgggctccagcagcttcaggacaccacccaccaggtgcaggctgccagtgactagcacatggatggcagcagcctcacggagtatgctggccccactgtgagccacagggtgggtgaggaggccctttgggggactaggtggctggaagatggggtctcggccttggctgatccattgcaaggcatgtgaaatgcagctgaagacgagggagctggcactgcaggtgtggggtgggtggggcgccagaagcagggatgcggacccaccgggctctgggctgggggcactccagaggtccgggctggcctgctcttcgtccaggtggttccagtgctgctggtgttccaggcagcggagcaggacctggtccagtgtcactgtgaagttctgttggtctgcgttgcctgtggatgacacctctgtcaggttagggcagaagacggcatagtcaaactggcagggctgcagcagcttcagcagggccgccgggtcccggtccccggtagcattgaagagcaagactcgaacctcggggccaccgctcggcctctcgcggccctgcagcgcctggcggaaccagcgcacgcaggcctgcgcgctgctggcggtgtgcgcaccgtccaggtaccaggtgaggggcccgcgccgcagcacctgcgtccggcccggccactccgtgttccgaagcccgagccgcatgtgggatgtgggctggaacacaggtgccaggggcagctgccacaggagccctggcctggatgcctttggctccccagcaccatggcggtcctgccgctgcagccagcagtgggccagctgcaaggccaaggcggcgttggaccgctggtgctccccctccaggcccagggtcagcggcggccccccttcctcgagggcctccagcatcggacacaggtatagaggacatgagatctgctgggctcggtccctcagcactgccaggggaccttcaggttggagcacagtgaaggcagggacaccttgcttaaagatgccccctttctgccatgcgatcttctccaccgtatcccccaggaggctggtgtggtcgatgccaagagaggagactccgcacaccacaggcttcctgatgatgttggtgcagtcataagccccgccaatgcccacctccaccactgccaggtccaccttctcttggaggaagacgtggaaggccatgagtgtcaggaagcggaagtaggggggcatggagacacagctgccatccttggtctcctccagccggtggtagaggcgccagaagtacttggtgaagagctcaggactgatgggctgcccattgatgcggatccgctcccgaacctaaagaatcccgtcttcaggccatagcttcggaggatacattccgtgaaggcacaggtggagcccttccccttcgtcccagtgacgtggatgatgttcagccggtccaagtcctccacctgcagcccactccgtgccaggtacagttccatggcttccaactgtgtctgagggtcaccccgctggcgcttcacctgctccaggtagccggcattggtctgcagggtattgagcatgcgcacggcatcctggtactccatgctcggctcctgcggcaccggccacgcgctcaagccccgccgcgccgcgacctgggtcgttatgccgcgcgcagacgccgctgccaggaatagagcggcgcgcaggtggctccgcgcccgcgacatagtcccggcgcccccggcagcgctctaggcccgggcgggagacgccccgccccgcccccagccaatc

SEQ ID NO: 9776 - RNA, 2245 nt, Homo sapiens
  source 1..2245: mol_type = other RNA
attgtccctctcccttcccagaaggcactgggaggaggaaatctaccacccagcacatggcaagacccagggcctggccaggcagcgcacacaataagctgggcctgagccaggaggcaggcggggtgttgggggagacaggctgaacggccaggccactgcaacagtgagagacccggggagcccctctgctatctcagccaagaggaaggagagaccaaggcacagagccttaaaaaagacatcctctcccggcctcccatcccaaagccctggcccctaggccagtctagacagaaccaggaaagccaaaaacaaaaggcacctagtatgtaagttcatggggagaacgcaggcaggtgtgggaagctcccacctccaaccccgggccttggctactgggacagtgcgggctccagcagcttcaggacaccacccaccaggtgcaggctgccagtgactagcacatggatggcagcagcctcacggagtatgctggccccactgtgagccacagggtgggtgaggaggccctttgggggactaggtggctggaagatggggtctcggccttggctgatccattgcaaggcatgtgaaatgcagctgaagacgagggagctggcactgcaggtgtggggtgggtggggcgccagaagcagggatgcggacccaccgggctctgggctgggggcactccagaggtccgggctggcctgctcttcgtccaggtggttccagtgctgctggtgttccaggcagcggagcaggacctggtccagtgtcactgtgaagttctgttggtctgcgttgcctgtggatgacacctctgtcaggttagggcagaagacggcatagtcaaactggcagggctgcagcagcttcagcagggccgccgggtcccggtccccggtagcattgaagagcaagactcgaacctcggggccaccgctcggcctctcgcggccctgcagcgcctggcggaaccagcgcacgcaggcctgcgcgctgctggcggtgtgcgcaccgtccaggtaccaggtgaggggcccgcgccgcagcacctgcgtccggcccggccactccgtgttccgaagcccgagccgcatgtgggatgtgggctggaacacaggtgccaggggcagctgccacaggagccctggcctggatgcctttggctccccagcaccatggcggtcctgccgctgcagccagcagtgggccagctgcaaggccaaggcggcgttggaccgctggtgctccccctccaggcccagggtcagcggcggccccccttcctcgagggcctccagcatcggacacaggtatagaggacatgagatctgctgggctcggtccctcagcactgccaggggaccttcaggttggagcacagtgaaggcagggacaccttgcttaaagatgccccctttctgccatgcgatcttctccaccgtatcccccaggaggctggtgtggtcgatgccaagagaggagactccgcacaccacaggcttcctgatgatgttggtgcagtcataagccccgccaatgcccacctccaccactgccaggtccaccttctcttggaggaagacgtggaaggccatgagtgtcaggaagcggaagtaggggggcatggagacacagctgccatccttggtctcctccagccggtggtagaggcgccagaagtacttggtgaagagctcaggactgatgggctgcccattgatgcggatccgctcccgaacctgcaccaggtggggagagctaaagaatcccgtcttcaggccatagcttcggaggatacattccgtgaaggcacaggtggagcccttccccttcgtcccagtgacgtggatgatgttcagccggtccaagtcctccacctgcagcccactccgtgccaggtacagttccatggcttccaactgtgtctgagggtcaccccgctggcgcttcacctgctccaggtagccggcattggtctgcagggtattgagcatgcgcacggcatccctctttccccactctcactgccggttcagactccgggatcactggaactccagaagcaccgctgagcctctgggcttctggatcctagctcctgtgccacttcccacttcccaacccggggcggggacgctatagtctccgaattcccagccccggcggcccgggcccaacttcctggtccctgtccccacccccagcctccaggatgttccgccccccgagt

SEQ ID NO: 9777 - RNA, 2202 nt, Homo sapiens
  source 1..2202: mol_type = other RNA
attgtccctctcccttcccagaaggcactgggaggaggaaatctaccacccagcacatggcaagacccagggcctggccaggcagcgcacacaataagctgggcctgagccaggaggcaggcggggtgttgggggagacaggctgaacggccaggccactgcaacagtgagagacccggggagcccctctgctatctcagccaagaggaaggagagaccaaggcacagagccttaaaaaagacatcctctcccggcctcccatcccaaagccctggcccctaggccagtctagacagaaccaggaaagccaaaaacaaaaggcacctagtatgtaagttcatggggagaacgcaggcaggtgtgggaagctcccacctccaaccccgggccttggctactgggacagtgcgggctccagcagcttcaggacaccacccaccaggtgcaggctgccagtgactagcacatggatggcagcagcctcacggagtatgctggccccactgtgagccacagggtgggtgaggaggccctttgggggactaggtggctggaagatggggtctcggccttggctgatccattgcaaggcatgtgaaatgcagctgaagacgagggagctggcactgcaggtgtggggtgggtggggcgccagaagcagggatgcggacccaccgggctctgggctgggggcactccagaggtccgggctggcctgctcttcgtccaggtggttccagtgctgctggtgttccaggcagcggagcaggacctggtccagtgtcactgtgaagttctgttggtctgcgttgcctgtggatgacacctctgtcaggttagggcagaagacggcatagtcaaactggcagggctgcagcagcttcagcagggccgccgggtcccggtccccggtagcattgaagagcaagactcgaacctcggggccaccgctcggcctctcgcggccctgcagcgcctggcggaaccagcgcacgcaggcctgcgcgctgctggcggtgtgcgcaccgtccaggtaccaggtgaggggcccgcgccgcagcacctgcgtccggcccggccactccgtgttccgaagcccgagccgcatgtgggatgtgggctggaacacaggtgccaggggcagctgccacaggagccctggcctggatgcctttggctccccagcaccatggcggtcctgccgctgcagccagcagtgggccagctgcaaggccaaggcggcgttggaccgctggtgctccccctccaggcccagggtcagcggcggccccccttcctcgagggcctccagcatcggacacaggtatagaggacatgagatctgctgggctcggtccctcagcactgccaggggaccttcaggttggagcacagtgaaggcagggacaccttgcttaaagatgccccctttctgccatgcgatcttctccaccgtatcccccaggaggctggtgtggtcgatgccaagagaggagactccgcacaccacaggcttcctgatgatgttggtgcagtcataagccccgccaatgcccacctccaccactgccaggtccaccttctcttggaggaagacgtggaaggccatgagtgtcaggaagcggaagtaggggggcatggagacacagctgccatccttggtctcctccagccggtggtagaggcgccagaagtacttggtgaagagctcaggactgatgggctgcccattgatgcggatccgctcccgaacctgcaccaggtggggagagctaaagaatcccgtcttcaggccatagcttcggaggatacattccgtgaaggcacaggtggagcccttccccttcgtcccagtgacgtggatgatgttcagccggtccaagtcctccacctgcagcccactccgtgccaggtacagttccatggcttccaactgtgtctgagggtcaccccgctggcgcttcacctgctccaggtagccggcattggtctgcagggtattgagcatgcgcacggcatcctggtactccatgctcggctcctgcggcaccggccacgcgctcaagccccgccgcgccgcgacctgggtcgttatgccgcgcgcagacgccgctgccaggaatagagcggcgcgcaggtggctccgcgcccgcgacatagtcccggcgcccccggcagcgctctaggcccgggcgggagac

SEQ ID NO: 9778 - RNA, 2148 nt, Homo sapiens
  source 1..2148: mol_type = other RNA
attgtccctctcccttcccagaaggcactgggaggaggaaatctaccacccagcacatggcaagacccagggcctggccaggcagcgcacacaataagctgggcctgagccaggaggcaggcggggtgttgggggagacaggctgaacggccaggccactgcaacagtgagagacccggggagcccctctgctatctcagccaagaggaaggagagaccaaggcacagagccttaaaaaagacatcctctcccggcctcccatcccaaagccctggcccctaggccagtctagacagaaccaggaaagccaaaaacaaaaggcacctagtatgtaagttcatggggagaacgcaggcaggtgtgggaagctcccacctccaaccccgggccttggctactgggacagtgcgggctccagcagcttcaggacaccacccaccaggtgcaggctgccagtgactagcacatggatggcagcagcctcacggagtatgctggccccactgtgagccacagggtgggtgaggaggccctttgggggactaggtggctggaagatggggtctcggccttggctgatccattgcaaggcatgtgaaatgcagctgaagacgagggagctggcactgcaggtgtggggtgggtggggcgccagaagcagggatgcggacccaccgggctctgggctgggggcactccagaggtccgggctggcctgctcttcgtccaggtggttccagtgctgctggtgttccaggcagcggagcaggacctggtccagtgtcactgtgaagttctgttggtctgcgttgcctgtggatgacacctctgtcaggttagggcagaagacggcatagtcaaactggcagggctgcagcagcttcagcagggccgccgggtcccggtccccggtagcattgaagagcaagactcgaacctcggggccaccgctcggcctctcgcggccctgcagcgcctggcggaaccagcgcacgcaggcctgcgcgctgctggcggtgtgcgcaccgtccaggtaccaggtgaggggcccgcgccgcagcacctgcgtccggcccggccactccgtgttccgaagcccgagccgcatgtgggatgtgggctggaacacaggtgccaggggcagctgccacaggagccctggcctggatgcctttggctccccagcaccatggcggtcctgccgctgcagccagcagtgggccagctgcaaggccaaggcggcgttggaccgctggtgctccccctccaggcccagggtcagcggcggccccccttcctcgagggcctccagcatcggacacaggtatagaggacatgagatctgctgggctcggtccctcagcactgccaggggaccttcaggttggagcacagtgaaggcagggacaccttgcttaaagatgccccctttctgccatgcgatcttctccaccgtatcccccaggaggctggtgtggtcgatgccaagagaggagactccgcacaccacaggcttcctgatgatgttggtgcagtcataagccccgccaatgcccacctccaccactgccaggtccaccttggtctcctccagccggtggtagaggcgccagaagtacttggtgaagagctcaggactgatgggctgcccattgatgcggatccgctcccgaacctgcaccaggtggggagagctaaagaatcccgtcttcaggccatagcttcggaggatacattccgtgaaggcacaggtggagcccttccccttcgtcccagtgacgtggatgatgttcagccggtccaagtcctccacctgcagcccactccgtgccaggtacagttccatggcttccaactgtgtctgagggtcaccccgctggcgcttcacctgctccaggtagccggcattggtctgcagggtattgagcatgcgcacggcatcctggtactccatgctcggctcctgcggcaccggccacgcgctcaagccccgccgcgccgcgacctgggtcgttatgccgcgcgcagacgccgctgccaggaatagagcggcgcgcaggtggctccgcgcccgcgacatagtcccggcgcccccggcagcgctctaggcccgggcgggagacgccccgccccgcccccagccaatc

SEQ ID NO: 9779 - RNA, 1859 nt, Homo sapiens
  source 1..1859: mol_type = other RNA
attgtccctctcccttcccagaaggcactgggaggaggaaatctaccacccagcacatggcaagacccagggcctggccaggcagcgcacacaataagctgggcctgagccaggaggcaggcggggtgttgggggagacaggctgaacggccaggccactgcaacagtgagagacccggggagcccctctgctatctcagccaagaggaaggagagaccaaggcacagagccttaaaaaagacatcctctcccggcctcccatcccaaagccctggcccctaggccagtctagacagaaccaggaaagccaaaaacaaaaggcacctagtatgtaagttcatggggagaacgcaggcaggtgtgggaagctcccacctccaaccccgggccttggctactgggacagtgcgggctccagcagcttcaggacaccacccaccaggtgcaggctgccagtgactagcacatggatggcagcagcctcacggagtatgctggccccactgtgagccacagggtgggtgaggaggccctttgggggactaggtggctggaagatggggtctcggccttggctgatccattgcaaggcatgtgaaatgcagctgaagacgagggagctggcactgcaggtgtggggtgggtggggcgccagaagcagggatgcggacccaccgggctctgggctgggggcactccagaggtccgggctggcctgctcttcgtccaggtggttccagtgctgctggtgttccaggcagcggagcaggacctggtccagtgtcactgtgaagttctgttggtctgcgttgcctgtggatgacacctctgtcaggttagggcagaagacggcatagtcaaactggcagggctgcagcagcttcagcagggccgccgggtcccggtccccggtagcattgaagagcaagactcgaacctcggggccaccgctcggcctctcgcggccctgcagcgcctggcggaaccagcgcacgcaggcctgcgcgctgctggcggtgtgcgcaccgtccaggtaccaggtgaggggcccgcgccgcagcacctgcgtccggcccggccactccgtgttccgaagcccgagccgcatgtgggatgtgggctggaacacaggtgccaggggcagctgccacaggagccctggcctggatgcctttggctccccagcaccatggcggtcctgccgctgcagccagcagtgggccagctgcaaggccaaggcggcgttggaccgctggtgctccccctccaggcccagggtcagcggcggccccccttcctcgagggcctccagcatcggacacaggtatagaggacatgagatctgctgggctcggtccctcagcactgccaggggaccttcaggttggagcacagtgaaggcagggacaccttgttgttccagtcacacagtgaagccaggatgaaaacgtagactcccaggccttccatgtctctcccttcccccagtctgcctggtcaccttaaagatgccccctttctgccatgcgatcttctccaccgtatcccccaggaggctggtgtggtcgatgccaagagaggagactccgcacaccacaggcttcctgatgatgttggtgcagtcataagccccgccaatgcccacctccaccactgccaggtccaccttctcttggaggaagacgtggaaggccatgagtgtcaggaagcggaagtaggggggcatggagacacagctgccatccttggtctcctccagccggtggtagaggcgccagaagtacttggtgaagagctcaggactgatgggctgcccattgatgcggatccgctcccgaacctaaagaatcccgtcttc

SEQ ID NO: 9780 - RNA, 2183 nt, Homo sapiens
  source 1..2183: mol_type = other RNA
attgtccctctcccttcccagaaggcactgggaggaggaaatctaccacccagcacatggcaagacccagggcctggccaggcagcgcacacaataagctgggcctgagccaggaggcaggcggggtgttgggggagacaggctgaacggccaggccactgcaacagtgagagacccggggagcccctctgctatctcagccaagaggaaggagagaccaaggcacagagccttaaaaaagacatcctctcccggcctcccatcccaaagccctggcccctaggccagtctagacagaaccaggaaagccaaaaacaaaaggcacctagtatgtaagttcatggggagaacgcaggcaggtgtgggaagctcccacctccaaccccgggccttggctactgggacagtgcgggctccagcagcttcaggacaccacccaccaggtgcaggctgccagtgactagcacatggatggcagcagcctcacggagtatgctggccccactgtgagccacagggtgggtgaggaggccctttgggggactaggtggctggaagatggggtctcggccttggctgatccattgcaaggcatgtgaaatgcagctgaagacgagggagctggcactgcaggtgtggggtgggtggggcgccagaagcagggatgcggacccaccgggctctgggctgggggcactccagaggtccgggctggcctgctcttcgtccaggtggttccagtgctgctggtgttccaggcagcggagcaggacctggtccagtgtcactgtgaagttctgttggtctgcgttgcctgtggatgacacctctgtcaggttagggcagaagacggcatagtcaaactggcagggctgcagcagcttcagcagggccgccgggtcccggtccccggtagcattgaagagcaagactcgaacctcggggccaccgctcggcctctcgcggccctgcagcgcctggcggaaccagcgcacgcaggcctgcgcgctgctggcggtgtgcgcaccgtccaggtaccaggtgaggggcccgcgccgcagcacctgcgtccggcccggccactccgtgttccgaagcccgagccgcatgtgggatgtgggctggaacacaggtgccaggggcagctgccacaggagccctggcctggatgcctttggctccccagcaccatggcggtcctgccgctgcagccagcagtgggccagctgcaaggccaaggcggcgttggaccgctggtgctccccctccaggcccagggtcagcggcggccccccttcctcgagggcctccagcatcggacacaggtatagaggacatgagatctgctgggctcggtccctcagcactgccaggggaccttcaggttggagcacagtgaaggcagggacaccttgttgttccagtcacacagtgaagccaggatgaaaacgtagactcccaggccttccatgtctctcccttcccccagtctgcctggtcaccttaaagatgccccctttctgccatgcgatcttctccaccgtatcccccaggaggctggtgtggtcgatgccaagagaggagactccgcacaccacaggcttcctgatgatgttggtgcagtcataagccccgccaatgcccacctccaccactgccaggtccaccttctcttggaggaagacgtggaaggccatgagtgtcaggaagcggaagtaggggggcatggagacacagctgccatccttggtctcctccagccggtggtagaggcgccagaagtacttggtgaagagctcaggactgatgggctgcccattgatgcggatccgctcccgaacctgcaccaggtggggagagctaaagaatcccgtcttcaggccatagcttcggaggatacattccgtgaaggcacaggtggagcccttccccttcgtcccagtgacgtggatgatgttcagccggtccaagtcctccacctgcagcccactccgtgccaggtacagttccatggcttccaactgtgtctgagggtcaccccgctggcgcttcacctgctccaggtagccggcattggtctgcagggtattgagcatgcgcacggcatcctggtactccatgctcggctcctgcggcaccggccacgcgctcaagccccgccgcgccgcgacctgggtcgttat

SEQ ID NO: 9781 - RNA, 2054 nt, Homo sapiens
  source 1..2054: mol_type = other RNA
attgtccctctcccttcccagaaggcactgggaggaggaaatctaccacccagcacatggcaagacccagggcctggccaggcagcgcacacaataagctgggcctgagccaggaggcaggcggggtgttgggggagacaggctgaacggccaggccactgcaacagtgagagacccggggagcccctctgctatctcagccaagaggaaggagagaccaaggcacagagccttaaaaaagacatcctctcccggcctcccatcccaaagccctggcccctaggccagtctagacagaaccaggaaagccaaaaacaaaaggcacctagtatgtaagttcatggggagaacgcaggcaggtgtgggaagctcccacctccaaccccgggccttggctactgggacagtgcgggctccagcagcttcaggacaccacccaccaggtgcaggctgccagtgactagcacatggatggcagcagcctcacggagtatgctggccccactgtgagccacagggtgggtgaggaggccctttgggggactaggtggctggaagatggggtctcggccttggctgatccattgcaaggcatgtgaaatgcagctgaagacgagggagctggcactgcaggtgtggggtgggtggggcgccagaagcagggatgcggacccaccgggctctgggctgggggcactccagaggtccgggctggcctgctcttcgtccaggtggttccagtgctgctggtgttccaggcagcggagcaggacctggtccagtgtcactgtgaagttctgttggtctgcgttgcctgtggatgacacctctgtcaggttagggcagaagacggcatagtcaaactggcagggctgcagcagcttcagcagggccgccgggtcccggtccccggtagcattgaagagcaagactcgaacctcggggccaccgctcggcctctcgcggccctgcagcgcctggcggaaccagcgcacgcaggcctgcgcgctgctggcggtgtgcgcaccgtccaggtaccaggtgaggggcccgcgccgcagcacctgcgtccggcccggccactccgtgttccgaagcccgagccgcatgtgggatgtgggctggaacacaggtgccaggggcagctgccacaggagccctggcctggatgcctttggctccccagcactgagatctgctgggctcggtccctcagcactgccaggggaccttcaggttggagcacagtgaaggcagggacaccttgcttaaagatgccccctttctgccatgcgatcttctccaccgtatcccccaggaggctggtgtggtcgatgccaagagaggagactccgcacaccacaggcttcctgatgatgttggtgcagtcataagccccgccaatgcccacctccaccactgccaggtccaccttctcttggaggaagacgtggaaggccatgagtgtcaggaagcggaagtaggggggcatggagacacagctgccatccttggtctcctccagccggtggtagaggcgccagaagtacttggtgaagagctcaggactgatgggctgcccattgatgcggatccgctcccgaacctgcaccaggtggggagagctaaagaatcccgtcttcaggccatagcttcggaggatacattccgtgaaggcacaggtggagcccttccccttcgtcccagtgacgtggatgatgttcagccggtccaagtcctccacctgcagcccactccgtgccaggtacagttccatggcttccaactgtgtctgagggtcaccccgctggcgcttcacctgctccaggtagccggcattggtctgcagggtattgagcatgcgcacggcatcctggtactccatgctcggctcctgcggcaccggccacgcgctcaagccccgccgcgccgcgacctgggtcgttatgccgcgcgcagacgccgctgccaggaatagagcggcgcgcaggtggctccgcgcccgcgacatagtcccggcgcccccggcagcgctctaggcccgggcgggagac

SEQ ID NO: 9782 - RNA, 522 nt, Homo sapiens
  source 1..522: mol_type = other RNA
attgtccctctcccttcccagaattgaccctctgcaccctctcctgggccctcttctcactacctccatctccaccatgccccaacagagcccctcccccaggcccctttggccgctctccacaccccacagctttctgtctgacctggtttcttagcctctctggacctcagcctccttatctgtaaaatgggaataaggatactacttcccttgtaacgcggtggtaaagtttaaataagctaaggaacacactgcatgtcctgcgggccctggcacaccagacatgctgacagacgctggctgctttcatcagctatgcaaccaaattctaaggggcccttcgtatgtgtcaggctgcgtgccaggaacctagaggtaccaccgtaccacagtacaagatgctgtgtctggcttcgaagagatttcagtcccggtgcctgcgggattgctggagagaacgcggcgatggagccgggcaggacccagataaagcttgaccccaggtaagtgagggcggcg

SEQ ID NO: 9783 - RNA, 1567 nt, Homo sapiens
  source 1..1567: mol_type = other RNA
attgtccctctcccttcccagaattgaccctctgcaccctctcctgggccctcttctcactacctccatctccaccatgccccaacagagcccctcccccaggcccctttggccgctctccacaccccacagctttctgtctgacctggtttcttagcctctctggacctcagcctccttatctgtaaaatgggaataaggatactacttcccttgtaacgcggtggtaaagtttaaataagctaaggaacacactgcatgtcctgcgggccctggcacaccagacatgctgacagacgctggctgctttcatcagctatgcaaccaaattctaaggggcccttcgtatgtgtcaggctgcgtgccaggaacctagaggtaccaccgtaccacagtacaagatgctgtgtctggcttcgaagagatttcagtctttgcgttttgtcgctctgtttcctgaagataacttggggtgctcctggtcgtccatctactgctttgattccttggatcccacccattctttcagcctgcgttttattttgttttcctgctgcatactgactacctctgaaatgttggatacaagtctgtgtctctgtagcacatttaacacgtttcccaggcaacaggaagctctcagtgtgcgttctgttgcagacgtgggcgtgtccttgggctgtgtagggcttcatttcagatgatctgaaccagagcggttgccaactgccagtgtccggagatgcctggtggccactctgtggttagtggcagtaggtggctgctacatctagttccagtgaacctcctgttgagagagtgcagctggtggtacaagccttcccttacacagcagctgtccccccagggaatatttggcagtgtcgggagacttccggttgccacactggaaggtgctactggcatctcgtggtcagaggccaggaaagctgctaaacttcctacagggcacgggaagagcccccacagaaaagattattcaggccaaagtgtcaatagtgctcaggttgagaaaccttgcctcacgcaatgaaaacggttctcacattgctttgcttcagaatgtgcaaacggaaaccccaaggctgttcagaacaggccattctgagtctgctagtccagcaagcctcgccgcaggcagagtggggaggatttggccagcgggccctcctgggacagggaagctgcgaggatgagttcggggacgccccaggcccaggggagcgaggtctggcaggattcaaggatcctggtggaagagcaggggacaattgagagggccgggcaggagaggtgaggcccgctgcgcgccgggctggcggaggagctgtgctttatcccgcagcgagaaggagctcgtgaaggctctgaggctgggagtggctggatgaaagtcgtgcttctcggccattcgttagtaatcaggatggactgcagaggaagaggcttaagaagcagggatgcggccggacaccgtggctcatgcctgtaatcccagcactttgggaggccgaggcaggcggatcatctgcggtcaagagttcaa

SEQ ID NO: 9784 - RNA, 5026 nt, Homo sapiens
  source 1..5026: mol_type = other RNA
attgtccctctcccttcccagggcttcctgccttctctactccaacttgtgtgtgccagacaagctaggtgagtgcagcccagggggaggagtctgcttggctccatggggcttttgtccctctctgatccaagagtcaaggcctgggatagtggggaccttggtgctagaggccagagagacagctgtcccagcatgtgaggagtggctgagcagcaggggcccccacagggttctcgcgtggccttggttctctgtgtatgagttatctatgctgcataagaacatcactacaaattagcaacttaaaacaacacacatttatgatctcccagtttctgtggatcaggagcccaagtgtggctttgttgggttctctgctcaaggtcccattaggctacaatcaagatgtcagctggggctgtggtctccccttcaggtatgaccaggaaagcagccacttctgaagctcacgttgttgctagccacactcaactccttgtggatgggatgattgagggccccagtttcttgctagttgggggctggaggcaaccccagtaccctgctacatgggcctcttcataggacagctcatagcctagcagctcactttttaaagctagcaagggatagactgctattccttgataatgttataatcttatgtcacatgatcacaaggtgtcacaggagtgacatccccttacctctgtattctattggttacaacaaggcacaggtcctgcacacactcaaggtgagatcacacaagggcatgcataccagcaggtgggggtcaagggagccattctagagtctgtctgctatagcccagaaggggccacattgtggcaccctcctggggtctcccaagccttgtcaagctggatttcctttggaataggcatctgccttgaagcaggcctctgtcagtgccactgaggtgtgactgccagtccccaggtgtgtggaaagaggcctttcactggctgagggccaccagccagttgtccaaatcacagcctggagcacagagccctcctagaacatagttggcaggccaagagagcaggccaagtgctctgagacacattcaggtataaggccaagaaccagggagcaaacccacacgtgcaaccctggagggcagagcttagtctgggatgatatcggcttctgagccaggtgttgccacgaagctttttgccagatggttactgaggagatatggagcatgaatgagggataggaagccacagggagcagccactgcaactgccagagcttggcttggccaagtgcagctcacacacaaagcagcccccagaagctcctgaaggccttgcagggctatgtggatccctatccccctgcagcatctgcagcaagcttttcacaagcttgggcagggaggcaggatgggtgtaggagatttctgcacagacagaatgctgaagtctaaggtgtcctttagatgggggaagtatgaggtcactaatcgaacagaaaagtaacttgtactgtacctgagatgaactttgctagctttccccaaagcaaagagggaagaggaagatatggctgagttcacagtgtggcagggacacaaatgtaggaaagaaaaaagtagagaagggtaggaaaaggagagaagtagagaagggtaggaaagtggtgcctcaagaccgggagagcattcggggcaccctggggtccattcagcatccagtgctccttcataccgctgagccatccctgaactccagcctagcatggccccatggacctccaccaggggagggtaccctgtggtcttggtcaggaaccatcaggtgagataagccagggtgttttgagaatccttctgacccagcattcatagcagaagagtgggaactgagttgccaaacctgggttcaaatcctgcatctgcaggacaggtgcccaggtggctcccaggatagggtgagttccagtggagctgcatccaagtcctggtctcagactggagtcaccttcctgccctccagctcaaatgctggtcctctcagccccatccaccaaccctgggcactgcatccccaggacaagcctgcccccacatgcttggacccaccctgcacaacagcccacaaaccacacagccttgtgcacccctaccctcgcccgcctgtctccccagcccgcacgcaggacctgtcccctcagccgcgggtcccctcccgccctccccgtcccctcagccccgggtcgcctcccgccctccccgtcccctcagccgcgggtcccctcccgccctccccgtcccctcagccgcgggtcccctcccaccctcccctcactcagccccggatcgcctcacatcctccccgtcccctcagtcgcaggtcccctcccgccctcccggtcccctcagccccgctcccctcccgccctcccctcactcagccccgggtcgcctcccgccctcccggtcccctcagccgcgggtcccctcccgccctccctgtcccctcagccgcgggtcccctcccaccctcccctcactcagccgcgggtcgcctcccgccctcccggtcccctcagccgcgggtcccctcccgcccttccctcactcagccgcgggtcgcctcccgccctccctgtcccctcagtcgcaggtcccctcccgccctcccggtcccctcagccccgctcccctcccgcgccgcccctgtccggcgccgtaggagctgccccctggcggtgggtgcgcggcgctgcgccttggtctgcgtttcctccgctggagtcccgggcgtgggctccgcgcctctcgcttcccccggcagcctcggggcgggaatttgggttccggagcgcggcagcccggcgcggggtgggaggtggagggttcgctccgcctgggaggcccgtctggtccccgccccgccccgccccaggttctcgcggacccggggctagctgaggcgctgccacggcggtcgcgcggcgcagtttcgcaggggcgggcgcatagaggcgggcccttggcaagaggatgaagggccgcccgcgcgggactcacacagaggcaccgggaagccacgagttttttttaggcctggcctgtgggccaggagtcagggaaggggcttcctggagggctccctggaggaggtggggctcagggggggctggactcggaaatcagagagcaggcgggcggtttgcgacgcccgggcggtcgcaggcggctcctggcgcagtgcggacccgggctgcttgcgggaggaagcggctgaagcccaggccggggtcagaggggagggcgcgtgcggggcggggtcgccgagagaaaaagaggcccccctcagccctgccaaacgcagtcctggcccggagcctgtccgtccaggccgacggcgtagcgcgaactccagtcccgctcaaagagctgccgcagctgctcctgcaccgtggcccccgcgggctgcgcgccagggctctgggtgaccaccaagcccacccccgccgtgctgctgaagtaatcctccgaccagttggaggtgcctatgtaggctgccttctccgtgaccatgaacttgctgtggttcaccctgctgaatgggatgttggaatggttccccaccggcacgatgaagactttcacgtccacagagacgttggccgcggggttgctgagcgcctgcagggaccgcaggtaggggaacatggtggggtccgtgttgagtccgcagccgaccagcaggcgcacgcgcacgcccttgccgaaggctgccgcccgcagcgcgttgtccagcaccggccagtacctcggggggtggctgaagcgcgtggtggggaaatactccatcacggaggcatagatgaactcctgggcgctccccatcaccgccagcagcgcctccaggtcccgggtgcggccctggggacagagtgctggtggcgacgctgagaagtaggcagtggtgggcaccccatcaaagaggccgtggaagggctggaaacggttgaagtgagatgagaagttctgaggccaggttttggggaggacagccttgggcacccccagtacccagtaggtctggaaggtcttctccaggtcttgggccaggtggctgcagttatagatgacagcgccaagctccttcacctgcgtcagagaccgccagtccatgttggcactgcccatgtatatgtgccgtccatccacaacccagaatttggagtgcaaaacacccctggtgagccgccccatgggcacctgtcgtacatgggcacctcgggcagccagaacctgcaggtcggtggatgtcctggccagtgtcgggctgctggtggccacagccagggaaatgttcctgcccagcagctgctgcagcttctgcagaagagcctctcccagctgggaagacgagtcgttgaccccgatgtcaggccctgtgagggaccagtagtatgaagccacgtggacgctctcctgggcagtgtccagcagctgcagccaggcctggcccagaggctgggcagaggggctgccggctgcagatggcaggtcctgggggatgctttccacaaggacaagctggcaggagtccctctgctgcctggcctctgcttccaggggctcccaagctgggctggagccatgctcccaggacctgggcacgtccttgggctgcacctggccccaggtgggaggacggggcacttgccacaggaggcagataagagccacggagcccagccacagcacagccagcgctcccaggacctgcaacgtgccagcctctctgtcccacgggcggcggggcggcatggagcatggccatgtgggggccactgctgctttccaaagaggcttcagcatctgcacagggcagcctggcatcaccagcagctccagctctctgggggtcctgccttggtgtctatcctgattccagccgcagactgcaggccctcagctcacggggcaggctcggtgctgcctgtgctccacaccaacctcctcttctct

SEQ ID NO: 9785 - RNA, 37 nt, Homo sapiens
  source 1..37: mol_type = other RNA
caaaaaccacagtttcttttgcaccaacctaataaaa

SEQ ID NO: 9786 - RNA, 37 nt, Homo sapiens
  source 1..37: mol_type = other RNA
caaaaaccacagtttcttttgcaccagactaataaag

SEQ ID NO: 9787 - RNA, 197 nt, Homo sapiens
  source 1..197: mol_type = other RNA
caaaaaccacagtttcttttgctttcttctttcctgcttgatcagaaccctggaccgggaccccccgacccaattcatcttcccaaatcttttgacactgaggtccctgtgtctagagctcagacatctcagctctgcgccaaatcgcagcttcagcaggatcccccagggcctcctgacaacgtcagggcccgagt

SEQ ID NO: 9788 - RNA, 232 nt, Homo sapiens
  source 1..232: mol_type = other RNA
caaaaaccacagtttcttttgctttcttctttcctgcttgatcagaaccctggaccgggaccccccgacccaattcatcttcccaaatcttttgacactgaggtccctgtgtctagagctcagacatctcagctctgcgccaaatcgcagcttcagcaggatcccccagggcctcctgacaacgtcagggcccgagtaagctccttctggtccaccgcctgaggcccaacct

SEQ ID NO: 9789 - RNA, 32 nt, Homo sapiens
  source 1..32: mol_type = other RNA
caaaaaccatagttacttttgcaccaatctaa

SEQ ID NO: 9790 - RNA, 58 nt, Homo sapiens
  source 1..58: mol_type = other RNA
caaaaaccgcaattacttttgcacaaacctaataggatgtaaacttcggagccatctg

SEQ ID NO: 9791 - RNA, 3004 nt, Homo sapiens
  source 1..3004: mol_type = other RNA
caaaaaccgcaattacttttgcacaaatctaattttaaaaattagagtatgtcggacagtgtcagtgctaaggaggaaaataaagtacaagtagtgaatagggactacggaatggtggtgcaggattttaaatagggtagccaggaaggggtttgcgaggaccacgtttgagcaaaccgaaaggtgagggagcgagctgtgcagatgtgggggtcggggaggacactgtcccagagacagaagagcaggttcaaaggccctgagacagaaacaatcgcctggtgatccccattttacagaagagagatctgaggctcagaaagatggagtcactcatccaaacttgcacagctgtaagtggcagagctgggattcgaatgccaggcccgataccaccaaaacctgcatttgtttctcattttctcatatttttcaattcagacactgaggatgtaggtgttggggcatcggcagagtgcttaagagctagacgtgatgtgaaccagacctgggttcaggttttgtggtgccacttacctccttgggtggctgacttgaactgtctgagcctcagtttccacatgctggtatttatcatatgcctcggctcctcaaactgcagcaaacaaactccatggaagagaaaaaaatgggactccagagacttgaaaccacggccacttgtcagatgcagcccccaactcagctgcaggagcttagccaaatttctagtcctctctgagcctcaatttccttatctataaaatgtggctctggatacctctcttgtagagttcttgtttagattacatgtgagcacttctataaaacactgaagacatgagctagccgttattctttataaacagtcatcaggagaattttgattttccacctcacagatttcccacaggaatgtgctgtcctgaaatgtgtctaaaggtcaacatttgaaaaacagaaagaatggaaaagaaagtcagcaaagtccagcatcatgacttggcagtgtccccagtggccaggtgcaaaggagcacccagagaggtgttttcagaccactgtaaatagtgtgagtgctatttaggacttacacacactcagacacatgcacacacacacaaatatagatacagccacacacatctgcagtttcactgccacacatagacactcacacatgcaagcacacacaaatatctagtcacacttctagacactcacacacatgaatacacacagttacacttacaatcttatgcacatgccaaactcataaacagatacatagacatacacttaactacagagctacatatacatgacagtcacacacatagttacatacacagtctcacacatacattcacacacatccacatctaccaacacacatgcatgcatgtaagtatacataaacacctgtacacctgcgcatacagctctacacacacttgcacacatgtacacatacacagtctcacatacatccatgtactgacacataggcacacatgggcacaaacatgcacaaccttacacacatgtctttacacacagaaccgcacacacataacagctatacatacatcccacagtcacatgtgcacacacaaaaacatacatgcatgcacttaggctatctcacatacacagctatgtacttcacacaggcacacacattataacaacatgttttcttttctttacagcccttattcattctctcagctatttactgaatgtttactgtgtgctagctaccgttaaaagtccttgagctaaatcattgaacaaaatgagcaaaaatatctgccctcatgaagcttagattctaatggaaggagagagaggcaaaaatagtaagtaagtatgttagcaggtagtgagtattagagacaatagtgcctagtaatgaggaggaggaagaaccaacttggaggtgggttgccgttttgagaaggtggtcaaggtaagcttcattgagaagttgacaaaaatatttagcaaggaaataaagtaggagagggagttatccatgtagatatctatgaaaaatcagtctgagaagaggaaacagcaagtgcagataccctaaaggcagagtgtgacttcaaggaacaggaagaaagcccttgtagttgacatgcagtgaataagggggtaaaggaacaggacatcaaaccagagatgaagagagtgtgtgaaaatcttaccagaccttgaataatgaggtaaaaactctgaagttaattttgcatgaaactgagattcaccggtaggttgtgagcagaggtgtgacatgatctgacctctgacttatcctttacagtatataaaatgaacttcattactttacatgttattatctgtgtcacttctgaacaggaatgaatctgtcatggtcacctctgtgtctacctgagagtaacactcagtcaatatttgttgactacttgataaggacagacatttccaaggagaaaagtgttctgaggtgctccagtttggatgtttgctctcaataaaactcatattgaaatttgagatggaaccttacaggaggtatttgagtcatgagggagaatccctcatgaataaattaatgccctccctagggagtgagtgagtcctaatcctattattccccacaagagctggttgttgcaaagagcctggcatctccccactatctctcttgcttcctctctcaccatgtcatccatgcacacgccagctccctttcaccttctaccatgaatagaagcatcccgaggcccttgccagctgcagatgcccaatcttgaaatttccagctatcagaatcatgggcctaataaacatttctgaaataaattacccagcctcagatatttctttatagcaatgaaaaatggactacaacaggaaattgttgccagggagtagggtattgctataaagatacctgaaaatatgacagcagctttggaactgggcaatggaaaaggttggaagagtttgg

SEQ ID NO: 9792 - RNA, 26 nt, Homo sapiens
  source 1..26: mol_type = other RNA
caaaaaccgcaattacttttgcacca

SEQ ID NO: 9793 - RNA, 43 nt, Homo sapiens
  source 1..43: mol_type = other RNA
caaaaaccgcaattacttttgcaccaaaccaacagcatcaatc

SEQ ID NO: 9794 - RNA, 58 nt, Homo sapiens
  source 1..58: mol_type = other RNA
caaaaaccgcaattacttttgcaccaaactaataggatgcaaacttcggagccatcta

SEQ ID NO: 9795 - RNA, 802 nt, Homo sapiens
  source 1..802: mol_type = other RNA
caaaaaccgcaattacttttgcaccaaatgaatatcatttctcagtcccaagccaatgcttctattttttgcaatgtttagttggacatctataacggccttccatgaggcagcctactgtctcccagagcatgataaggaagttccttgggttagatatctttctagcctgaaacataacaatttgcatttcagcccattgaattagacatttttctcttcagataatttctttggaaatgaaaatgttcctcaaagtgtagctacctattgggtcactgaagctttaatattagcaggtttgctggttcgctgtcttcaagaatagtggatattttgccacaaagggagaataggaagccagagtggaaagaggggaacaaaaacagggatagatacaagggaagaagatagacggtattagcatttactaccccatcattatatgtaccttgatttgttcctggagttgctgaaggatggctcagtttcccctttcttgtataattctttgattcagttgtagtctgacttttgaaagctgactgggtattggtgatggaaagcatatcctgaaattggagatagcaagactcttggtgaactgttgagtagactgggttgaattcagtgaaggatcaggcagcaggacacagcaaggccagccacggcacagcctcctcctccaccatctcaccaggctccctgccagggccggcgcagggcagcgcctgagctactagggagtctggtccggctgctgctccgccgccgccgccgccttctcacagccacaacaaca

SEQ ID NO: 9796 - RNA, 1651 nt, Homo sapiens
  source 1..1651: mol_type = other RNA
caaaaaccgcaattacttttgcaccaaatgaatatcatttctcagtcccaagccaatgcttctattttttgcaatgtttagttggacatctataacggccttccatgaggcagcctactgtctcccagagcatgataaggaagttccttgggttagatatctttctagcctgaaacataacaatttgcatttcagcccattgaattagacatttttctcttcagataatttctttggaaatgaaaatgttcctcaaagtgtagctacctattgggtcactgaagctttaatattagcaggtttgctggttcgctgtcttcaagaatagtggatattttgccacaaagggagaataggaagccagagtggaaagaggggaacaaaaacagggatagatacaagggaagaagatagacggtattagcatttactaccccatcattatatgtaccttgatttgttcctggagttgctgaaggatggctcagtttcccctttcttgtataattctttgattcagttgtagtctgacttttgaaagctgactgtagaaagaggaatatttagaaaaataggcaaagtgatgttatggtttaaaatcatcaagtgggaaatccaaaaccacggttctcaaccttagctactcatggaaaccacctgggaaatttttaaaaatactgatggatgggttccatgcccatagatttttaaaaaattcttccaaaggattctgacatcctaatcagggttgaaagctactgctccaaagagcttgacataatcaaatgaacatttatcaggtgttcacaaggtttaggaaggcccagcacaaagcaaaaccatagagacgttgagtactcttttgcttcagcattcagcatccaattccaactccatgcttttccttacttccaacttccatctttgccccgagcaacctgtgcagaaaaccatcagtttccctgctccactggacatctaaggactatggtggtgataaaaaatgagagtcatcaaaaaggtccaagtttagtgaagatgtgcaaagggaagcagcccttcccaaagaattcagtgaatgagccaagattctccagaaaccgctcagctttgcagtgataattttctgggtattggtgatggaaagcatatcctgaaattggagatagcaagactcttggtgaactgttgagtagactgggttgaattcagtgaaggatctaattattaccaggtcaggaagatgtcctgctgcacgctcaggcggtcactcctcctttccacaaggcccatgtccgcaccgttcgccccggggctcccatggcccccgacctccagtctccggcaacgatggaccctcacagacacggcagggagcgaagggcgcacactcacctcccaggcagcaggacacagcaaggccagccacggcacagcctcctcctccaccatctcaccaggctccctgccagggccggcgcagggcagcgcctgagctactagggagtctggtccggctgctgctccgccgccgccgccgccttctcacagccacaacaacactgcagcagcgaccacacagagcgcgctcccgacgccgagccgggcgacgagcggggacgcgctcgcacgctcgggcgctgaacccggt

SEQ ID NO: 9797 - RNA, 1746 nt, Homo sapiens
  source 1..1746: mol_type = other RNA
caaaaaccgcaattacttttgcaccaaatgaatatcatttctcagtcccaagccaatgcttctattttttgcaatgtttagttggacatctataacggccttccatgaggcagcctactgtctcccagagcatgataaggaagttccttgggttagatatctttctagcctgaaacataacaatttgcatttcagcccattgaattagacatttttctcttcagataatttctttggaaatgaaaatgttcctcaaagtgtagctacctattgggtcactgaagctttaatattagcaggtttgctggttcgctgtcttcaagaatagtggatattttgccacaaagggagaataggaagccagagtggaaagaggggaacaaaaacagggatagatacaagggaagaagatagacggtattagcatttactaccccatcattatatgtaccttgatttgttcctggagttgctgaaggatggctcagtttcccctttcttgtataattctttgattcagttgtagtctgacttttgaaagctgactgtagaaagaggaatatttagaaaaataggcaaagtgatgttatggtttaaaatcatcaagtgggaaatccaaaaccacggttctcaaccttagctactcatggaaaccacctgggaaatttttaaaaatactgatggatgggttccatgcccatagatttttaaaaaattcttccaaaggattctgacatcctaatcagggttgaaagctactgctccaaagagcttgacataatcaaatgaacatttatcaggtgttcacaaggtttaggaaggcccagcacaaagcaaaaccatagagacgttgagtactcttttgcttcagcattcagcatccaattccaactccatgcttttccttacttccaacttccatctttgccccgagcaacctgtgcagaaaaccatcagtttccctgctccactggacatctaaggactatggtggtgataaaaaatgagagtcatcaaaaaggtccaagtttagtgaagatgtgcaaagggaagcagcccttcccaaagaattcagtgaatgagccaagattctccagaaaccgctcagctttgcagtgataattttctgggtattggtgatggaaagcatatcctgaaattggagatagcaagactcttggtgaactgttgagtagactgggttgaattcagtgaaggatctgtaatcccagctacttgggaggctgaggggagaatcgattgaactcgggcagcagtggttgcagtagccgagattgcaccattgcactccagcctaattattaccaggtcaggaagatgtcctgctgcacgctcaggcggtcactcctcctttccacaaggcccatgtccgcaccgttcgccccggggctcccatggcccccgacctccagtctccggcaacgatggaccctcacagacacggcagggagcgaagggcgcacactcacctcccaggcagcaggacacagcaaggccagccacggcacagcctcctcctccaccatctcaccaggctccctgccagggccggcgcagggcagcgcctgagctactagggagtctggtccggctgctgctccgccgccgccgccgccttctcacagccacaacaacactgcagcagcgaccacacagagcgcgctcccgacgccgagccgggcgacgagcggggacgcgctcgcacgctcgggcgctgaacccggt

SEQ ID NO: 9798 - RNA, 2808 nt, Homo sapiens
  source 1..2808: mol_type = other RNA
caaaaaccgcaattacttttgcaccaaccaatataaattgtaacagatttgagacaaaatataaaatttttcaaattgagcagaatttatcaacccagaatctataatgtatgaaataaattaatagagaacccaacagatcatgttatgttgtaaatataacatctatctttaggttaaagtaacatagcaaaaatatatatttatgggtgcaagacacatacataatttgtaccaatctcacagaactaattcaattcaaaacaacaaaaaacttactctattatctaatggatgcaataaaaattaaccatttgaagataagttctcttgcacttcccctacttacgtttttcctggcacctgctatactgtgtatgtatttcttcaccgctttactgcctgactcccctactagatcataagttccaagagggcaagccctctgaaacactgctatgtctccagcacctagaacttggcatgtagtaggcatccaatacataagtgttaaatgagtgaatttaaaacacgtacatgccaggaatggtggctcaggcctgtaatcccagcactttgggaggccgaggcgggggatggcctgaggtcaggagttccagaccagcctggctaatatggtgaaaccccgactctactaaaaatacaaaaattagctcttcctttctctgccattgtggtgtgtgcttgactctgcttcttgccatgtcttctcataagacttccaggattaagtgattcctgaccgagaaattaaaacaaaatcgccccactccccagtggattcagatgaaaactggtaataaaatcaggtacaactccaaaaggagacattgaagaagaaccaagctagccctataaggaattgcacatgagagggcacacatatttatgctgtctgaaggtcacagtcatgttaccacatcaagctgaaaatgtcaccgctctctggagaattgtacatgttttattgggaatatattttttctttctgaatctgttatgaatgcattggttggctgggttcagtaataaatatgtgagacctttcattaaaaaaaaatacaaaaattagctgggcatggtggcgcacacctgtagtaccagctactctggaggctgaggcgggagaattgcttcaacccagaaggcggaggttgcagtgagctgagatcgcgccactgcactccagcctgtgtgacagagtgagactttgtctcaaaaaacaaacaaaacatgcacacatttaatcaatataaaatattatttctgcgaagtcacttcaagctgatactgcatactccatatatgctaaacttcacaaggtctttacctcatacctgactctctttcctgaccccctgcggggtaagtcaatgccctggggttgcttagccacttggtactaccagctttgggcaccaggtctgtttcagctcattggtgtatgccccggctggcttttcccatagggcagagttgcacaagttgtgggtgtgaagctgagaggtgagcagaggaggaagggaggtagacagtcctcatcccagtgtccctctgaactgccgcgtgtgttgctccagcttctcagcctccgcctggaggtgccccagcgcggcagggctggggtacgtgagcacggcattcttagtggccagcgctacgtccttgagcaggctgcagaggtgactgctgccacggaggatctcgttgcgcacgtccctctcctgggtctccatgcacagcgtgtccaccagcttctgtcccaccatgatgaccagcttgctctgagtgatgatctccgcgggctggctgctgctgaggctgccgtgaaatgcgctgatggctttgaagagcgccccaaagtagagccggcagtgttcagataagcggggtttcctctcaggagtctgttgactcgaaggctgaggtataagagggccaggattacttgcttggctgtctgggggatggagtcctgccttcttggggctggctggtatgtcatataactgctgcttctctggctccttcaggaccacggggccccggtgctgggtaggcacgtcatacacctgggaaggcagagtcggcagtgaggcccggacaggtctgggaagcgtgaggatggcctgttttggaaagctgagagtcttttcacagatgattctggcactggtgggagggtcggggaattcatagacttgggcagtagggggctggggcccctccgcccaactcctcatctgctcataaacggggcctggagtgggagggcggggtagagtgggcacctgataggtctcctctgagctggcaggagcttcttccaggcctctcaggaatggggggcacggcctgtctgcagcgacctccgtgaggatttggaggcggttggcaggggccaggccttgcctcccatggagcaaacacttccaccaaccctcgctttctggcacgtgttgctccagaatggtcaggatgtcccctctgctgaaagccagctcgtcagagcagtcagggcagttgtcataaagtgccctggccaggagtgccttgggcgcacagtccatgatgcctgttcccttcatgtcggtgatgtggagcagctcccctgagctctgcagctagtatctccagcttcagaggcagattgtgcaatgtcactgcatgcttctggctggttctcagaaactgaattctatggagctatctgacaacacatgggaaacgatcaaaaagactctcccagcaggcaaactttctggaaagcacgataagagtaaaatg

SEQ ID NO: 9799 - RNA, 3957 nt, Homo sapiens
  source 1..3957: mol_type = other RNA
caaaaaccgcaattacttttgcaccaaccaatataaattgtaacagatttgagacaaaatataaaatttttcaaattgagcagaatttatcaacccagaatctataatgtatgaaataaattaatagagaacccaacagatcatgttatgttgtaaatataacatctatctttaggttaaagtaacatagcaaaaatatatatttatgggtgcaagacacatacataatttgtaccaatctcacagaactaattcaattcaaaacaacaaaaaacttactctattatctaatggatgcaataaaaattaaccatttgaagataagttctcttgcacttcccctacttacgtttttcctggcacctgctatactgtgtatgtatttcttcaccgctttactgcctgactcccctactagatcataagttccaagagggcaagccctctgaaacactgctatgtctccagcacctagaacttggcatgtagtaggcatccaatacataagtgttaaatgagtgaatttaaaacacgtacatgccaggaatggtggctcaggcctgtaatcccagcactttgggaggccgaggcgggggatggcctgaggtcaggagttccagaccagcctggctaatatggtgaaaccccgactctactaaaaatacaaaaattagctcttcctttctctgccattgtggtgtgtgcttgactctgcttcttgccatgtcttctcataagacttccaggattaagtgattcctgaccgagaaattaaaacaaaatcgccccactccccagtggattcagatgaaaactggtaataaaatcaggtacaactccaaaaggagacattgaagaagaaccaagctagccctataaggaattgcacatgagagggcacacatatttatgctgtctgaaggtcacagtcatgttaccacatcaagctgaaaatgtcaccgctctctggagaattgtacatgttttattgggaatatattttttctttctgaatctgttatgaatgcattggttggctgggttcagtaataaatatgtgagacctttcattaaaaaaaaatacaaaaattagctgggcatggtggcgcacacctgtagtaccagctactctggaggctgaggcgggagaattgcttcaacccagaaggcggaggttgcagtgagctgagatcgcgccactgcactccagcctgtgtgacagagtgagactttgtctcaaaaaacaaacaaaacatgcacacatttaatcaatataaaatattatttctgcgaagtcacttcaagctgatactgcatactccatatatgctaaacttcacaaggtctttacctcatacctgactctctttcctgaccccctgcggggtaagtcaatgccctggggttgcttagccacttggtactaccagctttgggcaccaggtctgtttcagctcattggtgtatgccccggctggcttttcccatagggcagagttgcacaagttgtgggtgtgaagctgagaggtgagcagaggaggaagggaggtagacagtcctcatcccagtgtccctctgaactgccgcgtgtgttgctccagcttctcagcctccgcctggaggtgccccagcgcggcagggctggggtacgtgagcacggcattcttagtggccagcgctacgtccttgagcaggctgcagaggtgactgctgccacggaggatctcgttgcgcacgtccctctcctgggtctccatgcacagcgtgtccaccagcttctgtcccaccatgatgaccagcttgctctgagtgatgatctccgcgggctggctgctgctgaggctgccgtgaaatgcgctgatggctttgaagagcgccccaaagtagagccggcagtgttcagataagcggggtttcctctcaggagtctgttgactcgaaggctgaggtataagagggccaggattctgtccacagatatttgccctatttttctttaatagttcagaagagtgttcatcttccctttgcttagtggaaggggtactcttttggtgtgattcagtttctctttggggaggctggatgtatttttcacacttaaattctgcatttggggtcaactgcacagtctcttccttttcacagttccgcttaaaaaggagccttccattggcaatgacaatggaggcaaacctcttgatgtcttctggaagcatccgtgccaccatgacaaacctctcaaggtcatctgggctgttctggacactgtcagtcacaagaacttccagaggccaattgcgattatccaagctttcctttgtttcaagcaggatgcggtaggagttggagatggtctgcatctggtcccgaattctgttctgaaggttactgtcagtgaggttacaggcagtcccatggactcctcgggcaaaatccagaaattctcttacagattcttctatgtgatcagtggacctgtggattgcatcaatgttggcctccagatagtctcggaatctccacttcctgctgacaaagagcatcaggccagcgacagagctgaccaccttgtgctgcagagccatcactgtctccttggccacatccaggtccaaggagagctcctttgctgactcctccgaggaagagctggaggagtcgtcggtggatgtggtggagcacgaggaaacgatgctagctctgctgtcagaactggaacctgataatctgtccggttcaggagatggggaagttgtccgtctggagaaccatgaggaattatggcccgcggaattctctgacacctccttggctttctccagctccttcccagcctgagaaacactcgacgttgctttagggatgtcataaatattgggcttggtgttctgctgttccactcggggaatcagaaagcttgaaggaaccttgtagctgacatcttcatccaaaggaaatgtgcctctgggtacaagaaagccataagaaggaatttctggaaggctgagttttttctgcatgggcacattgttattcagttgtggagtgagggacctggatctgccacttggaggattgtagaaagtggagctggaactggggagagcgtggggccttgattcttccgcaaagctggtgagaggcgtgtttctgacgctggcctttcctggagacactggagtgtcataaatccattccgatttctgaggatttggtaatgtgctgtaaccgcctcttcttaaggtagtcactgatatcaggggaacaccctgcccacttgcttggctgtctgggggatggagtcctgccttcttggggctggctggtatgtcatataactgctgcttctctggctccttcaggaccacggggccccggtgctgggtaggcacgtcatacacctgggaaggcagagtcggcagtgaggcccggacaggtctgggaagcgtgaggatggcctgataggtctcctctgagctggcaggagcttcttccaggcctctcaggaatggggggcacggcctgtctgcagcgacctccgtgaggatttggaggcggttggcaggggccaggccttgcctcccatggagcaaacacttccaccaaccctcgctttctggcacgtgttgctccagaatggtcaggatgtcccctctgctgaaagccagctcgtcagagcagtcagggcagttgtcataaagtgccctggccaggagtgccttgggcgcacagtccatgatgcctgttcccttcatgtcggtgatgtggagcagctcccctgagctctgcagctagtatctccagcttcagaggcagattgtgcaatgtcactgcatgcttctggctggttctcagaaactgaattctatggagctatctgacaacacatgggaaacgatcaaaaagactctcccagcaggcaaactttctggaaagcacgataagagtaaaatg

SEQ ID NO: 9800 - RNA, 4119 nt, Homo sapiens
  source 1..4119: mol_type = other RNA
caaaaaccgcaattacttttgcaccaaccaatataaattgtaacagatttgagacaaaatataaaatttttcaaattgagcagaatttatcaacccagaatctataatgtatgaaataaattaatagagaacccaacagatcatgttatgttgtaaatataacatctatctttaggttaaagtaacatagcaaaaatatatatttatgggtgcaagacacatacataatttgtaccaatctcacagaactaattcaattcaaaacaacaaaaaacttactctattatctaatggatgcaataaaaattaaccatttgaagataagttctcttgcacttcccctacttacgtttttcctggcacctgctatactgtgtatgtatttcttcaccgctttactgcctgactcccctactagatcataagttccaagagggcaagccctctgaaacactgctatgtctccagcacctagaacttggcatgtagtaggcatccaatacataagtgttaaatgagtgaatttaaaacacgtacatgccaggaatggtggctcaggcctgtaatcccagcactttgggaggccgaggcgggggatggcctgaggtcaggagttccagaccagcctggctaatatggtgaaaccccgactctactaaaaatacaaaaattagctcttcctttctctgccattgtggtgtgtgcttgactctgcttcttgccatgtcttctcataagacttccaggattaagtgattcctgaccgagaaattaaaacaaaatcgccccactccccagtggattcagatgaaaactggtaataaaatcaggtacaactccaaaaggagacattgaagaagaaccaagctagccctataaggaattgcacatgagagggcacacatatttatgctgtctgaaggtcacagtcatgttaccacatcaagctgaaaatgtcaccgctctctggagaattgtacatgttttattgggaatatattttttctttctgaatctgttatgaatgcattggttggctgggttcagtaataaatatgtgagacctttcattaaaaaaaaatacaaaaattagctgggcatggtggcgcacacctgtagtaccagctactctggaggctgaggcgggagaattgcttcaacccagaaggcggaggttgcagtgagctgagatcgcgccactgcactccagcctgtgtgacagagtgagactttgtctcaaaaaacaaacaaaacatgcacacatttaatcaatataaaatattatttctgcgaagtcacttcaagctgatactgcatactccatatatgctaaacttcacaaggtctttacctcatacctgactctctttcctgaccccctgcggggtaagtcaatgccctggggttgcttagccacttggtactaccagctttgggcaccaggtctgtttcagctcattggtgtatgccccggctggcttttcccatagggcagagttgcacaagttgtgggtgtgaagctgagaggtgagcagaggaggaagggaggtagacagtcctcatcccagtgtccctctgaactgccgcgtgtgttgctccagcttctcagcctccgcctggaggtgccccagcgcggcagggctggggtacgtgagcacggcattcttagtggccagcgctacgtccttgagcaggctgcagaggtgactgctgccacggaggatctcgttgcgcacgtccctctcctgggtctccatgcacagcgtgtccaccagcttctgtcccaccatgatgaccagcttgctctgagtgatgatctccgcgggctggctgctgctgaggctgccgtgaaatgcgctgatggctttgaagagcgccccaaagtagagccggcagtgttcagataagcggggtttcctctcaggagtctgttgactcgaaggctgaggtataagagggccaggattctgtccacagatatttgccctatttttctttaatagttcagaagagtgttcatcttccctttgcttagtggaaggggtactcttttggtgtgattcagtttctctttggggaggctggatgtatttttcacacttaaattctgcatttggggtcaactgcacagtctcttccttttcacagttccgcttaaaaaggagccttccattggcaatgacaatggaggcaaacctcttgatgtcttctggaagcatccgtgccaccatgacaaacctctcaaggtcatctgggctgttctggacactgtcagtcacaagaacttccagaggccaattgcgattatccaagctttcctttgtttcaagcaggatgcggtaggagttggagatggtctgcatctggtcccgaattctgttctgaaggttactgtcagtgaggttacaggcagtcccatggactcctcgggcaaaatccagaaattctcttacagattcttctatgtgatcagtggacctgtggattgcatcaatgttggcctccagatagtctcggaatctccacttcctgctgacaaagagcatcaggccagcgacagagctgaccaccttgtgctgcagagccatcactgtctccttggccacatccaggtccaaggagagctcctttgctgactcctccgaggaagagctggaggagtcgtcggtggatgtggtggagcacgaggaaacgatgctagctctgctgtcagaactggaacctgataatctgtccggttcaggagatggggaagttgtccgtctggagaaccatgaggaattatggcccgcggaattctctgacacctccttggctttctccagctccttcccagcctgagaaacactcgacgttgctttagggatgtcataaatattgggcttggtgttctgctgttccactcggggaatcagaaagcttgaaggaaccttgtagctgacatcttcatccaaaggaaatgtgcctctgggtacaagaaagccataagaaggaatttctggaaggctgagttttttctgcatgggcacattgttattcagttgtggagtgagggacctggatctgccacttggaggattgtagaaagtggagctggaactggggagagcgtggggccttgattcttccgcaaagctggtgagaggcgtgtttctgacgctggcctttcctggagacactggagtgtcataaatccattccgatttctgaggatttggtaatgtgctgtaaccgcctcttcttaaggtagtcactgatatcaggggaacaccctgcccacttgcttggctgtctgggggatggagtcctgccttcttggggctggctggtatgtcatataactgctgcttctctggctccttcaggaccacggggccccggtgctgggtaggcacgtcatacacctgggaaggcagagtcggcagtgaggcccggacaggtctgggaagcgtgaggatggcctgttttggaaagctgagagtcttttcacagatgattctggcactggtgggagggtcggggaattcatagacttgggcagtagggggctggggcccctccgcccaactcctcatctgctcataaacggggcctggagtgggagggcggggtagagtgggcacctgataggtctcctctgagctggcaggagcttcttccaggcctctcaggaatggggggcacggcctgtctgcagcgacctccgtgaggatttggaggcggttggcaggggccaggccttgcctcccatggagcaaacacttccaccaaccctcgctttctggcacgtgttgctccagaatggtcaggatgtcccctctgctgaaagccagctcgtcagagcagtcagggcagttgtcataaagtgccctggccaggagtgccttgggcgcacagtccatgatgcctgttcccttcatgtcggtgatgtggagcagctcccctgagctctgcagctagtatctccagcttcagaggcagattgtgcaatgtcactgcatgcttctggctggttctcagaaactgaattctatggagctatctgacaacacatgggaaacgatcaaaaagactctcccagcaggcaaactttctggaaagcacgataagagtaaaatg

SEQ ID NO: 9801 - RNA, 4221 nt, Homo sapiens
  source 1..4221: mol_type = other RNA
caaaaaccgcaattacttttgcaccaaccaatataaattgtaacagatttgagacaaaatataaaatttttcaaattgagcagaatttatcaacccagaatctataatgtatgaaataaattaatagagaacccaacagatcatgttatgttgtaaatataacatctatctttaggttaaagtaacatagcaaaaatatatatttatgggtgcaagacacatacataatttgtaccaatctcacagaactaattcaattcaaaacaacaaaaaacttactctattatctaatggatgcaataaaaattaaccatttgaagataagttctcttgcacttcccctacttacgtttttcctggcacctgctatactgtgtatgtatttcttcaccgctttactgcctgactcccctactagatcataagttccaagagggcaagccctctgaaacactgctatgtctccagcacctagaacttggcatgtagtaggcatccaatacataagtgttaaatgagtgaatttaaaacacgtacatgccaggaatggtggctcaggcctgtaatcccagcactttgggaggccgaggcgggggatggcctgaggtcaggagttccagaccagcctggctaatatggtgaaaccccgactctactaaaaatacaaaaattagctcttcctttctctgccattgtggtgtgtgcttgactctgcttcttgccatgtcttctcataagacttccaggattaagtgattcctgaccgagaaattaaaacaaaatcgccccactccccagtggattcagatgaaaactggtaataaaatcaggtacaactccaaaaggagacattgaagaagaaccaagctagccctataaggaattgcacatgagagggcacacatatttatgctgtctgaaggtcacagtcatgttaccacatcaagctgaaaatgtcaccgctctctggagaattgtacatgttttattgggaatatattttttctttctgaatctgttatgaatgcattggttggctgggttcagtaataaatatgtgagacctttcattaaaaaaaaatacaaaaattagctgggcatggtggcgcacacctgtagtaccagctactctggaggctgaggcgggagaattgcttcaacccagaaggcggaggttgcagtgagctgagatcgcgccactgcactccagcctgtgtgacagagtgagactttgtctcaaaaaacaaacaaaacatgcacacatttaatcaatataaaatattatttctgcgaagtcacttcaagctgatactgcatactccatatatgctaaacttcacaaggtctttacctcatacctgactctctttcctgaccccctgcggggtaagtcaatgccctggggttgcttagccacttggtactaccagctttgggcaccaggtctgtttcagctcattggtgtatgccccggctggcttttcccatagggcagagttgcacaagttgtgggtgtgaagctgagaggtgagcagaggaggaagggaggtagacagtcctcatcccagtgtccctctgaactgccgcgtgtgttgctccagcttctcagcctccgcctggaggtgccccagcgcggcagggctggggtacgtgagcacggcattcttagtggccagcgctacgtccttgagcaggctgcagaggtgactgctgccacggaggatctcgttgcgcacgtccctctcctgggtctccatgcacagcgtgtccaccagcttctgtcccaccatgatgaccagcttgctctgagtgatgatctccgcgggctggctgctgctgaggctgccgtgaaatgcgctgatggctttgaagagcgccccaaagtagagccggcagtgttcagataagcggggtttcctctcaggagtctgttgactcgaaggctgaggtataagagggccaggattctgtccacagatatttgccctatttttctttaatagttcagaagagtgttcatcttccctttgcttagtggaaggggtactcttttggtgtgattcagtttctctttggggaggctggatgtatttttcacacttaaattctgcatttggggtcaactgcacagtctcttccttttcacagttccgcttaaaaaggagccttccattggcaatgacaatggaggcaaacctcttgatgtcttctggaagcatccgtgccaccatgacaaacctctcaaggtcatctgggctgttctggacactgtcagtcacaagaacttccagaggccaattgcgattatccaagctttcctttgtttcaagcaggatgcggtaggagttggagatggtctgcatctggtcccgaattctgttctgaaggttactgtcagtgaggttacaggcagtcccatggactcctcgggcaaaatccagaaattctcttacagattcttctatgtgatcagtggacctgtggattgcatcaatgttggcctccagatagtctcggaatctccacttcctgctgacaaagagcatcaggccagcgacagagctgaccaccttgtgctgcagagccatcactgtctccttggccacatccaggtccaaggagagctcctttgctgactcctccgaggaagagctggaggagtcgtcggtggatgtggtggagcacgaggaaacgatgctagctctgctgtcagaactggaacctgataatctgtccggttcaggagatggggaagttgtccgtctggagaaccatgaggaattatggcccgcggaattctctgacacctccttggctttctccagctccttcccagcctgagaaacactcgacgttgctttagggatgtcataaatattgggcttggtgttctgctgttccactcggggaatcagaaagcttgaaggaaccttgtagctgacatcttcatccaaaggaaatgtgcctctgggtacaagaaagccataagaaggaatttctggaaggctgagttttttctgcatgggcacattgttattcagttgtggagtgagggacctggatctgccacttggaggattgtagaaagtggagctggaactggggagagcgtggggccttgattcttccgcaaagctggtgagaggcgtgtttctgacgctggcctttcctggagacactggagtgtcataaatccattccgatttctgaggatttggtaatgtgctgtaaccgcctcttcttaaggtagtcactgatatcaggggaacaccctgcccacttgcttggctgtctgggggatggagtcctgccttcttggggctggctggtatgtcatataactgctgcttctctggctccttcaggaccacggggccccggtgctgggtaggcacgtcatacacctgggaaggcagagtcggcagtgaggcccggacaggtctgggaagcgtgaggatggcctgttttggaaagctgagagtcttttcacagatgattctggcactggtgggagggtcggggaattcatagacttgggcagtagggggctggggcccctccgcccaactcctcatctgctcataaacggggcctggagtgggagggcggggtagagtgggcacctgataggtctcctctgagctggcaggagcttcttccaggcctctcaggaatggggggcacggcctgtctgcagcgacctccgtgaggatttggaggcggttggcaggggccaggccttgcctcccatggagcaaacacttccaccaaccctcgctttctggcacgtgttgctccagaatggtcaggatgtcccctctgctgaaagccagctcgtcagagcagtcagggcagttgtcataaagtgccctggccaggagtgccttgggcgcacagtccatgatgcctgttcccttcatgtcggtgatgtggagcagctcccctgagctctgcagctagtatctccagcttcagaggcagattgtgcaatgtcactgcatgcttctggctggttctcagaaactgaattctatggagctatgtctcaatgcctgacgtctcactttgtctgtaagtagagactgtcactcatttgctatgtgaaaccacaaaagaagaagaagaagaaaaaaacaccactcttctgctttatagggcgaagttcctacttcgaagagctcagtgtatgaacacacagcattcttgtcctttgaactctgt

SEQ ID NO: 9802 - RNA, 30 nt, Homo sapiens
  source 1..30: mol_type = other RNA
caaaaaccgcaattacttttgcaccaacct

SEQ ID NO: 9803 - RNA, 218 nt, Homo sapiens
  source 1..218: mol_type = other RNA
caaaaaccgcaattacttttgcaccaacctaaaatataataaaaaagtgtcttctctttataacttttctgttgttttgcttaagttatcattgctattcctctgcaacctaaaaagaaatcattgaatatacatttaattttagaataatcactacacaaatgccctaaaagtgtatgtataacatccctgatgtctgcatttgtcctttgactggt

SEQ ID NO: 9804 - RNA, 1409 nt, Homo sapiens
  source 1..1409: mol_type = other RNA
caaaaaccgcaattacttttgcaccaacctaataataacaggagttatttgtagaattgacggattttagaagggtaaaaggaaaaaggaaagctaagaaatgtgaaataaagaaaaaagcagacaacttagttacacgccaagtccttaactgagcgagaagagaaataaattctggaatctgtctattaataattcttcctcacccacaagataaaaacagtagcttccaatctgagacacactcatgcaacttcctctgtgacagagtgctctgaacactatgtgagtgggaccatagtgttctcagtattgcactttctacggtaaatttggctaagaaacacttttgttcttttcctgtaagtcaaaagaaagtcctcctaaactaactaaaatctaaaatttgtctgactctaggagattttttttctccagacaaattcaaattaaatgataacatctcttaaggatttctcaccagtatcagataaaaatacattgaatccaagctatttgaatggacaatactcagttgcacatacacaccatcaactgcagggggcgccaatgccttttccctcaggcccttcagaaaaggcggtgcagctggaattttaatttcttcctgtctgttaagtgtgattattgatgaagtactgcgctcatcccagtacccaaattgaagcttctcgaacatatacgaaatggaactgggccttacaacaaaggcaaatctagttcccatgtttaaaatagtctccggggtccatttggagtgaggagtaaggaagggaagggacttatgcaggtctttccatgcggccttgatttagtccacggagtccaaagcccattctgaggcagggtctctaggttcttggtttacacctatatacaggcgagcgcgcccccgggccgcggaccgcgcgcacagcccgcactgccccacgccgcgggctagggacacccggcccgccaccatgacttccagcaagatagagatgcccggcgaggtgaaggccgaccccgccgccctcatggcgtcgctgcacctcctgccgtcgcccacgcccaatctcgaaattaagtacaccaaggtaagcggccgcccagcgcccgtcgtccacggagactttctagaaccttcttcggtttccccgatctcttcagcgggtgagggctgcgggacggggccggggtcgtcggggccagcctgtcatcccggcgcagcagagggaccccctgcctgtcttcgggactggggcgtttgaagccccgccgtggtctgaggacgccttggggacttaacccaacccgaagcgcagcgttgaggggcagccgtcaacggctcctgccccggactctgaggctggtttctgtccgattctcccggtcccgactgccgc

SEQ ID NO: 9805 - RNA, 38 nt, Homo sapiens
  source 1..38: mol_type = other RNA
caaaaaccgcaattacttttgcaccaacctaatacctt

SEQ ID NO: 9806 - RNA, 44 nt, Homo sapiens
  source 1..44: mol_type = other RNA
caaaaaccgcaattacttttgcaccaacctaatagatgccaatg

SEQ ID NO: 9807 - RNA, 58 nt, Homo sapiens
  source 1..58: mol_type = other RNA
caaaaaccgcaattacttttgcaccaacctaatagggtgcaaacttcagagccatctg

SEQ ID NO: 9808 - RNA, 40 nt, Homo sapiens
  source 1..40: mol_type = other RNA
caaaaaccgcaattacttttgcaccaacctaggaattggt

SEQ ID NO: 9809 - RNA, 4258 nt, Homo sapiens
  source 1..4258: mol_type = other RNA
caaaaaccgcaattacttttgcaccaacctatatatgcctatttaggcatgcttatttatgcatatttagccactcagcctatggctgagtggactatgtcagagaactgaacccaagttctagagagatctgtcccaagtcagcggacagccaatatacaaggaacctcgcagacagacatacagatgcagagataccccatcacatacatgttaaccagtttggacaatttgaatgaagcctgtggtcaccagggatatgggagcaattctaatcaggattgttagattatctctagaaggttgcttctgatagcttggacaagatgatggcggtgggggagaagcagggaattccttggcagtagggaggttgaatactttcctcattgtgctctagtaaactgaggaacttctagcagcaggagaaacatctgtcctttaaaagccatgtatcctgttcagaaaggcttggcattaatggagaccaaattgtcccactagaaaggacattgatgtcaagggggcatttggtgtcttttctggttctagtcctatgcaaaaaagcatatatcttaaaatatattaactacattttggcaaacaatagttcctgggaggttattatagtattatggtatgcccctatgggaaacttttctattttgtcaggattatagtttctaaaagttcctctccaagtatttaggttgctggcctggcttgtagagaacaacttgagttcaccatccttggtcatcacagaaggagagagcagggcacagttctgcttcggatgtcacagggccagggatttgtcccagatgttgtaagaaagattcaggggacacaggttcaagtacttcaggtctagcaaagtttctgaagactcttttggttgactagctcagggaagcacgagtgagggatgccttcctggaagatgacttattagcctccttcattcctttcaggctttccaggaggatgggctgatagaataccgctggagcttggggcaagggaggtgtggaaagcccctgttttaattctcctcctggccagacttatcagcatgttggactgtgccttgatgttcttctcctaaactgcagaggttctcacctatagctttcttgctctcttagtatctcttgcaacacacgcagcagggcttgagcaggagtggttaacacagcttcctttcttgattcccaaagatcttacttttcacatgactgccaccatggccaccattgctgatgttttatctacacattgtaaagcaggagtctcctattcaggtgttacctgtgtagtctctgtttcagagcctgcaatttgccctaccgtgagcatagttcaatctgtacagcagatgggtttggctgccttctatttagcttatccactagcacattcatggatgctgaattccagggccccactacccagccttctgaggcattctcttccccaagcacttgagaaagcactggaaagagaactgtgttagggttgagccccaaccttgccacatagcaagtcatatccaaccttgagacttttttccccatctgtaaaacaggattactgatgtttgatttacctcctgcacagggatgtgaaaagtcaaggagaatgatgcaaaaatactcatgaactatccggtgctgaacaaatagagggaagataatgatgctgctgacgaaactgatgaagaagaccacgatgatgataattgtgctttgctcgtaaagttacttgatttttgactgactgattagatgcagtttccctgaatggagctgcctaccgccttccttctagggcttatccagacaaccttgggtaagtcactcaactctctacgattaattcatctgtcaaatggggataataaaaaccaccaggcagtgttgctgtgagaattgaaagaagtgagtcaatagatataaaagtgcccagaggagtgcctggaccttatgaggaactttgtcagctctagttgaatttgaatttatataactctagagggaatggtgatgttccccaacttggatggggcagtagaaagagcacagactttatcttgctcatagtggcatgtgactttaacctctctgagccttagttgcctcatccgtaaaatgggaacaacagcgttcacctcaaaagatttgtgtgtgtgtgtgtcaaagggaatggtttgtgcagagagcttttcaaagtacctgacactggcaagggcttagtatttaatagctctctcaccctcatgcttaacgtgggtaagttgcttagaagaaaatgcaaagcctcatatggtcataactgtgctgcctttgtccccttttagctctgggtgctgccaggctgtgggtctgtggcccacagtgcactttcctggtgagaccctgtggcatgagcactgtggcaagaacagtcacatgattaggatcccaaggtgccaggactcttgctgccccagttgctgggcctcctgcctctctcttctgaagcaaaacttgagtgagaggcaggagcaagggcattgaaagtgtccatcctcagcctgctgcctgggacctcaccaactggtgacatttggtcatatgggggcagtcactgggaggtggtctcacctggtagctgctggtggaaggaggccaggggctgtcatagaggtgttcttactccctgtaggcagtggctggcattgctgagagctgacagttttggtgtcaggaggtgaggggtaggtttgagttctgtgccacaccccctctatacaagtaagtgaccaggaactgttcactcttctcaacacagcacactatgcatattctggcctctgccatgtgcagacacccttctttgcctacctgacaaagtagatatttcctgatgacccagttcacaaatcactctaatcttataattctcatggacattgctagatacagatgatggctcctcctctgggcctccataatgacgtgctcagagtcctgacatatagtcttaaagggaatagtttttggatctctctccttgaccagagggaagtgccttgagggcagggactgagtcagttcatctgatgttcccaattcctagcgtgccgcctggcccaaagcagatgctcatacaaaatgagtgtccccaccttgcttgaaccatgactgaggcagccaggtcaccatggaaccagagtgagcagtcagggagggcgtctggtggccagcagctgtggcggtcagcagcatggagggatgagaggcaggcatgtcagatctcttcctcttcactggccttgctccagcggtggcagcagttggcagtgatgcccaggaggaagttggtggccacagaagcaatggagaccacgaagcccacgaacgcaatgaataggtaatcatccagggtcagggtcaggtggcaggccttgaagctctcctcagtgagtgagaagagcggggcgccctcgacttcaggagggccccggcactcagccagctgagaatctgctgtacagcgctggatccggtttcgcagccacttcagcaggggttccatggtgcagccacacacccagggattgccaccgatctgcagggtcaccagccccggtaggccctcaagagcctccaggctgaggaaggccaggcccccataactgaggtccaggtctcggagctgcatgaggccctgaaaggcctggggatgcaccctccgcagccaggggttgtggctcaggtcgatgtggactagcccatgggcctcctggaacatgtcggctggcacatggctgaaattgttgtagctcaggtccaagtgtgccaagcgcttggcatggaggaagaggccccggggcagctccattaaggagttgttgtgcaaatccagcacctggagctccatgtagcatgtgaggtagccaggcggcactgctgtgatgcggttgtgggccaggctgaggtttcgggtgtccattggcaggtctgggggcacggagaatagccgctggctgctacaatccaccacctggttacggcatgtgcaaaggacggggcagctggtgccggcatccgagtgcatcaacccggctgccaagaggagggagatcagcagcattgctgggtggggtggcccgggccagggaagctgggcccaagtgtcacccatcttaggcagcaggcaacagcagtgctggagggagcccatgaggactgtgtccatggaatcgagagtctgt

SEQ ID NO: 9810 - RNA, 29 nt, Homo sapiens
  source 1..29: mol_type = other RNA
caaaaaccgcaattacttttgcaccaact

SEQ ID NO: 9811 - RNA, 1506 nt, Homo sapiens
  source 1..1506: mol_type = other RNA
caaaaaccgcaattacttttgcaccaacttaaatatataacctctctgagctcccattttctcatctaaaaaatgaaataataccaacctcacagcactgttggaagggttggggtaaagcaccaagtacgtgggtagcttatatcctacagaataattttcaccaacatgacccatgaccatgaagtttatggtttgactatctgtaggaagggtacaaaaatacatcatgcaacaaggtcattcatttggaaatgtaatgctttctgaaaaacttgagcattcacttttcttcacttgcctgttctaataagagaggtttggtgtggtgatttttcaatagaaaggatgttaccaatatataaataacataaaaggatcacatgagaattaaagtgaagtaacttaacatacaattttcattctaatcttatacaataatttttcttgactattgatagatcacaataaaggtatgctgatgatataagttattttaagactttggggaaaaaggcttccgtctctggcattgaccttattgtggaggaccctccaaaatcttcagctctgcaccagcaggtatgctgagtcatgtatgatgacataaaccacaaggagtcaaggagctaaaacaaccacagcgactggctcagatctcagatgtgcaagatgaatcctcaggatttttcacacactgaagaaacttgtcaggtctgtagatattcttgcaggaaaattgaatattccttttgcttataatcgattccagctcttttatggtgggatcctggcataagtctctggaatcttctcttccaccatgtatcacccaggcctctagtgtctgaaccttctctggttgcaaattatggacttccacactcccaaaagtgctgtttttgtcaaagattttactgcgggatccattgagcatcacatggaccacatcacaggcagcttctgcaaacctgcgggaaaccgttttccagaatactgaaacagggttgttgctgcagtcctttctccagtctgggcaagattgatagtttatttcttgttgcaaggtacggtctgagttcccaacttcattagtggctgatagtcttcttcagtaatgttgcaaggatgttttgaaataaatgcacccttgaaagcatcccatacactttggcagtctacatgtctcatctcaggatgaatttcagtgtacttgacgcatcgcgccaggacggtctcgggaaagcgcttggtggtgcccggaccgctccactgctggcgccacctcgggacgaccaccgcgagcaccacgacgaggatcaggaccaggatactgacgccaagacagagttgggctctcctagagagccggcagcagggtttgtccccggacaccgggctgaactcgcagttggccatagggctccaggcggggttggctgggcgaagatgaggccggcaggaggctaggcagcaagagagaggctggctgggttctgaaactgc

SEQ ID NO: 9812 - RNA, 1642 nt, Homo sapiens
  source 1..1642: mol_type = other RNA
caaaaaccgcaattacttttgcaccaacttaaatatataacctctctgagctcccattttctcatctaaaaaatgaaataataccaacctcacagcactgttggaagggttggggtaaagcaccaagtacgtgggtagcttatatcctacagaataattttcaccaacatgacccatgaccatgaagtttatggtttgactatctgtaggaagggtacaaaaatacatcatgcaacaaggtcattcatttggaaatgtaatgctttctgaaaaacttgagcattcacttttcttcacttgcctgttctaataagagaggtttggtgtggtgatttttcaatagaaaggatgttaccaatatataaataacataaaaggatcacatgagaattaaagtgaagtaacttaacatacaattttcattctaatcttatacaataatttttcttgactattgatagatcacaataaaggtatgctgatgatataagttattttaagactttggggaaaaaggcttccgtctctggcattgaccttattgtggaggaccctccaaaatcttcagctctgcaccagcaggtatgctgagtcatgtatgatgacataaaccacaaggagtcaaggagctaaaacaaccacagcgactggctcagatctcagatgtgcaagatgaatcctcaggatttttcacacactgaagaaacttgtcaggtctgtagatattcttgcaggaaaattgaatattccttttgcttataatcgattccagctcttttatggtgggatcctggcataagtctctggaatcttctcttccaccatgtatcacccaggcctctagtgtctgaaccttctctggttgcaaattatggacttccacactcccaaaagtgctgtttttgtcaaagattttactgcgggatccattgagcatcacatggaccacatcacaggcagcttctgcaaacctgcgggaaaccgttttccagaatactgaaacagggttgttgctgcagtcctttctccagtctgggcaagattgatagtttattttggaagtgttgaattcaccacaccatgtgaggtcatcagcaaggtagcctagcagcgtgtcctccagggtgaacatgtcccgctggacctgtgtgaactgatgggccagatcttttattctgctccaaagaagaatcttgttgcaaggtacggtctgagttcccaacttcattagtggctgatagtcttcttcagtaatgttgcaaggatgttttgaaataaatgcacccttgaaagcatcccatacactttggcagtctacatgtctcatctcaggatgaatttcagtgtacttgacgcatcgcgccaggacggtctcgggaaagcgcttggtggtgcccggaccgctccactgctggcgccacctcgggacgaccaccgcgagcaccacgacgaggatcaggaccaggatactgacgccaagacagagttgggctctcctagagagccggcagcagggtttgtccccggacaccgggctgaactcgcagttggccatagggctccaggcggggttggctgggcgaagatgaggccggcaggaggctaggcagcaagagagaggctggctgggttctgaaactgc

SEQ ID NO: 9813 - RNA, 2385 nt, Homo sapiens
  source 1..2385: mol_type = other RNA
caaaaaccgcaattacttttgcaccaatttaatattttagagtgtacttctacttatttaaaaaaagttaactgtaaaacagcctcaggcagatcctacagaaggtattccagaagaaggcattgttatcataggagatgacagctccatgcatattactgctcctggaaggctttccagtcagctaagatgtgaagctgtaaaacagtgatattgataatcctgactgccccgctgtctacacctggtttcaaaccatatggtgtcagtactaggctggactgcaccagcagtccaggcagcagtggcaccccaactagacatagctgtgtaccatgtcctattaggaatggaagaacaccctttctaacagtgaaggctcggggtctaggggtgccccaggccccatggccttatcttgcattaggactacaggttccaagacctcttgcaactctgctgctaagggacttatacttagcgtactccactgctctaagtaggtgccccacttcgctaaagtggatgtctgtgctgtcccagtctgggggggtcattgctcatgaacgcacccatcccactatggggtaagccatccacacgactgtaacccatccagccacgctcttatgaacctgaagggcagcatatatggttactaactgcttctttattaatgaacactggggctcagctcccttccatagctgggactaaaagctgactggcgcttccaagcactccatatactgccataggccctagccaactctattggtggttacatgcacatctagtttaaatgggcaccctggttaaccacccagagggcttatgtcatcagaagggctgtttcagcctcatcatcccaatcccaggcaagaggggtgttgtggcctccaaaccagcaaaagaactagaggttaacataacatcattaataagaaaatgatatataatggggctatacatatagccctgcagcaacactatgaaagtccattgtcgccctcccatgaaggcaaactgttcctggctctctggagcaatgctgattgagaagaatgcattggtcaagtccaccacacagtggcaccatcccagttctgttgtcaaacggtccatcaagtccatgacaggtggcacagctgccaagtcttgcaaaacatccacccccaagaatgtcctcaggcatgcaagagacatacacagtgcataagtggagagccaagcagctgatgcccaggtgcaaagacacaggtttcactttcactgaccagctttcatagctgtctatgcagccttccctggaaacttatccgggtccagggaccagtggattgccaagtccatatatggcctttggttgtctggtatcccctaccaagccgggcaccttggccagttctcttatcaaacagaaaatgctttatacttccaccaactgcagcaggtactctttgaactggaacactctggcaggaccaggttgcgcagcaacatccttctcccaaatgacttgcaccaagtctcatcccattctcattgccagttgttaggtttagggttcgggtccagcccatgctgaggtacaagggagtgggtcccttacagaagatgtcatcaacaaaccagaggcggagatgtcactacaagatttgcagctccattacttcaaaatgcacgattatgatggcaattatttgcttgatggtttagaaatctccacagccatcactcatatacagggaccaggattttactccagttctgccgactccagtactggatctcttaagctggatcctagcagatctgcacaggtacctactggaatgcttggctccatgatccatggctctgtcccttgctctaactgggaaatcacatcaggtttagaaacttggagtcctatagagaccaggtgtgtataattttccaatgtcacatccctgaacaaatctctctggccagggtccagctgtttccattcttcctgggtaaagtccactatcacatccttgaaagtcaccgcttcctgaaaactggctgatgagagtagattatgtcccccttggagaagggtggagtctggagaggacagatcttccatctcaggagctcatcccgttcctctggaacttgaacaccagggttcgccaggcagcgttccttcagctggtatctcggtctaggactcagatgtctaactccccttgcagggaatctgcaacacgctgaggttgtctaccctgagctcccctccccctatagcgatccacacactctgatcccgggtccggaagcgcattgaccgccaccagacctaacgcagggagccgaagcaactggacttccagcgcgccaacctctttccacgcctac

SEQ ID NO: 9814 - RNA, 2600 nt, Homo sapiens
  source 1..2600: mol_type = other RNA
caaaaaccgcaattacttttgcaccaatttaatattttagagtgtacttctacttatttaaaaaaagttaactgtaaaacagcctcaggcagatcctacagaaggtattccagaagaaggcattgttatcataggagatgacagctccatgcatattactgctcctggaaggctttccagtcagctaagatgtgaagctgtaaaacagtgatattgataatcctgactgccccgctgtctacacctggtttcaaaccatatggtgtcagtactaggctggactgcaccagcagtccaggcagcagtggcaccccaactagacatagctgtgtaccatgtcctattaggaatggaagaacaccctttctaacagtgaaggctcggggtctaggggtgccccaggccccatggccttatcttgcattaggactacaggttccaagacctcttgcaactctgctgctaagggacttatacttagcgtactccactgctctaagtaggtgccccacttcgctaaagtggatgtctgtgctgtcccagtctgggggggtcattgctcatgaacgcacccatcccactatggggtaagccatccacacgactgtaacccatccagccacgctcttatgaacctgaagggcagcatatatggttactaactgcttctttattaatgaacactggggctcagctcccttccatagctgggactaaaagctgactggcgcttccaagcactccatatactgccataggccctagccaactctattggtggttacatgcacatctagtttaaatgggcaccctggttaaccacccagagggcttatgtcatcagaagggctgtttcagcctcatcatcccaatcccaggcaagaggggtgttgtggcctccaaaccagcaaaagaactagaggttaacataacatcattaataagaaaatgatatataatggggctatacatatagccctgcagcaacactatgaaagtccattgtcgccctcccatgaaggcaaactgttcctggctctctggagcaatgctgattgagaagaatgcattggtcaagtccaccacacagtggcaccatcccagttctgttgtcaaacggtccatcaagtccatgacaggtggcacagctgccaagtcttgcaaaacatccacccccaagaatgtcctcaggcatgcaagagacatacacagtgcataagtggagagccaagcagctgatgcccaggtgcaaagacacaggtttcactttcactgaccagctttcatagctgtctatgcagccttccctggaaacttatccgggtccagggaccagtggattgccaagtccatatatggcctttggttgtctggtatcccctaccaagccgggcaccttggccagttctcttatcaaacagaaaatgctttatacttccaccaactgcagcaggtactctttgaactggaacactctggcaggaccaggttgcgcagcaacatccttctcccaaatgacttgcaccaagtctgtacaagagtgccaacattacttgcttaactcctacaacttagcaggggcacagacaacataggaagtgtgctccaccacagtagggggtctctggcccacccttggggcccaacagctgctcatgctctattttctggcagaccattgggtgaacctgtaacggaggttcttcctccctgtgtgcatccctcagggactgggcaggcacttcctcatcccattctcattgccagttgttaggtttagggttcgggtccagcccatgctgaggtacaagggagtgggtcccttacagaagatgtcatcaacaaaccagaggcggagatgtcactacaagatttgcagctccattacttcaaaatgcacgattatgatggcaattatttgcttgatggtttagaaatctccacagccatcactcatatacagggaccaggattttactccagttctgccgactccagtactggatctcttaagctggatcctagcagatctgcacaggtacctactggaatgcttggctccatgatccatggctctgtcccttgctctaactgggaaatcacatcaggtttagaaacttggagtcctatagagaccaggtgtgtataattttccaatgtcacatccctgaacaaatctctctggccagggtccagctgtttccattcttcctgggtaaagtccactatcacatccttgaaagtcaccgcttcctgaaaactggctgatgagagtagattatgtcccccttggagaagggtggagtctggagaggacagatcttccatctcaggagctcatcccgttcctctggaacttgaacaccagggttcgccaggcagcgttccttcagctggtatctcggtctaggactcagatgtctaactccccttgcagggaatctgcaacacgctgaggttgtctaccctgagctcccctccccctatagcgatccacacactctgatcccgggtccggaagcgcattgaccgccaccagacctaacgcagggagccgaagcaactggacttccagcgcgccaacctctttccacgcctac

SEQ ID NO: 9815 - RNA, 48 nt, Homo sapiens
  source 1..48: mol_type = other RNA
caaaaaccgcaattacttttgcaccagctaactattcactggctgccc

SEQ ID NO: 9816 - RNA, 29 nt, Homo sapiens
  source 1..29: mol_type = other RNA
caaaaaccgcaattacttttgcaccgacc

SEQ ID NO: 9817 - RNA, 44 nt, Homo sapiens
  source 1..44: mol_type = other RNA
caaaaaccgcaattacttttgcaccgacctaataacattctagg

SEQ ID NO: 9818 - RNA, 30 nt, Homo sapiens
  source 1..30: mol_type = other RNA
caaaaaccgcaattacttttgcactaacct

SEQ ID NO: 9819 - RNA, 6737 nt, Homo sapiens
  source 1..6737: mol_type = other RNA
caaaaaccgcaattacttttgcactaacctaatagttatatcctgaagaggcagaaactgataggtttgtctgtgtagtttttcagcttgtattattactaccactaacagcctctgttgaacccttcattactatgtaagcagccatatttaattctcagaacaatgtaatgagggagagcctatgaaaaaacaaagcctatgaaacagagcctatgaaaaaacattaaccaaggtcatcatccacaaaaatacaagttccagcactaactctgctttctctgtgatgcttctcctgcccattcatacttgtagggaataggagtagaggccaattatgtcgcttgagagtgctcttggaacagtggcaaattttctgtacgtgaaattagcttctcaacttttttgtacgtacggtactggttcttaaccttggctaccattggaattacccgggaaacattaaaacactcatcaggtcccaccctccagggattctgtataactcggctgggtgtagcctaagcatcaaaatgattatgcgcagccaaggttgaaagccaccaacactgacacatggatttaatattaaccacttggaacagaataccactgttaaaattgccgtggaaggttaaataatgggcagcccttgctattccaagtttggtttttttgttttttgtttttgagaccaagtcttgctctgtcacccaggctggagtgcagtggcacagtctcagctcactgcaacctctgcctcccgggttccagctattctcctgcctcagcctcctaggtagctgggactacaggcgtgtgccaccatgcccggctaattttgtatccttagtagagacagggtgtcaccatgttggccagggtggtcttgaactcctgacctcgtgatccacccacctcggcctcccaaagtgctgggattacaggcttgagccaccgtgcccggcctattgtaagttttaaacaacctcagaccagggaacttcctcacttggacatacacttcatagcaatttcttctcttaaaatagtggaaaatgaagctgtaaaagcacagtgaatgagaacactagcaagctatggcaatttgaaaaaatgtgattttaagagtcagtcttgcacctttatcatttaaatttggttatctcagcatgaaacttctgagactgacagcaagaattaaaacaccttttgtatatgcggaaactaccctgtagtctacctgctctcaaatttgagcacgcttgctgggccccaccaccaatttctgattctgtaggtctgggataggaccttagaatgtgtctatcacgtgacacttgtaagaaccactgttctagcacaagccaaaagaagtgacagcaaagactgacatccagaatcctctaattcagttctctctactcatctcactacctgtgctctgcttaggtgaatgtgtttgcagcatgtggaggaacaatccatgtattctttgtccctgcccaaacctaaagattgaggaggaactgacagcaatattgagagtgaggcaagagagaaaaaaaacctagcttcggagtcacatctggttttcaatgcgagcttcgtgcaagttggactgagttaggtgcctcacgtctggaaacctgtttcttcatgtgcatttgcgcaccctcattacattgttctgagaattaaatatggctgcttacatagcaaggaagggctcaacagaggccgttagtggtagtaataatacatgctgaaaaaaaacaactggtgaagaagatactgaattgtacctgagatttataccatttgctgttaaaaaaaaaaaaaaaaaaaaagccatactactcccaaatacctccgcgcaatgttttccagtcattaattcaacagcagaataggggataggacaaatgtccttatgctcatggaattaattttaacgccaggtagtttagcttctatgttaagtgctagagagcagcatccgttaaatctggtggctgcagcagagcacttccctaggaaccgactgcacacgcccaattcagaaggaagtgagcactgattcccggcagccaactcccgttcgcgcagccgctgccaccggcccttaagacgatgtgaccgccaattttgtaacagtgacgtcacccgacgtctgcaggccctgacagttggctctagcgggtgcgcagtctccctacccccggtaaggggctctaccggccctggacccaagatgggactcctacctccgaccacccggagcagcggcgccccagatccggccgtccgccctgcgcgtgcgcggcccgaccccgccgcggtctggctgtaagggcgctggaggggagctgggctgccccagccttcaatgctggagggacggccgcgtggggcttcagaaaggctaggcgccgaggagtgtaagcagcgtgtgcccatttaaagacaaaatcagtgtgtttttcaggtttgtacgaaatgaagttgtagaaagattaacaagggttacctgggaaaggcagattttcaacttagcgtttacatgttcacccagtgcattattttatttaaaaagaagaaaaatatatacttaacggctcctaatccagctctctttgcctggtctcccaagacacctatcattttgcccagcacataccttgccgctgtgccacactggagtccccggttaggttccctgtgcttagaccgccccctagtccctccaggaagcctttcccaaccctttcgcgttaactgcccgcctcatcatcacaaaggtaacttgagcttttatcagttttaattactccttttaatttgctcttcttccctatgtttaggcagaaacgagtctttttttaaccatattcatcacctggtgccagcaacagaagtgttccctaaaaattcctagaataaaccaacacgtgctgactagattctccatcttcataaacggtgatacaaactatgcacatcataactaccagcttcatgaggtcaagactaaatcaaaaattctcaaggacttttctaaaaatttttttagcataaactgtttcctctaacttaaacttctcttaagtgaacgtgtctttccactgggatgactgtctacatgctcaggaatcctgaattcatgactatgttcaactcccacgaccatttttaaatcatcaaaatggcagcaaatgtcattacctggaccaaaaagctgcaggttttgtggcaaatgggaaatgtgttatagaatatgactgggaaagagggatttcttagtgctgcccagaattaattcagcaaacactgaacattactacgtgccacatataggatcatactgcatttcaggtcaccatcaaaggtaaattacaaggctgggcgcagtggctcatgcctgtaatcccagcactttgggaggccagggcaggcggatcacctgaggtcaggagttcaagaccagcctggccaacatggcaaaacccccgctctactaaaaatacaaaaattagccaggcatgctggcatgcgcctgtagtcccagctacttgggaggctaaggcaggagaatcgcttgaacctgggaagtggaagttgcagttagctgagatggcaccactgcactccagcctgggcaacagagcaagactccatctcagaaaaataaaataaattttttaaaaaggtaaattacaagactgcaaaactttttaaaaaaaccttccccactagtttgtacctaataaatgctaacatttaaaagggggcacaaaaggcctgcagaaataagaactcacgttcttgaaagtactgcctagcatggtatcttcctcatcatcagaggtgctctatacatcttcagttgaaacgtgaaacagacatccatatgcaaaatattttcaagggttttgttggcttttacatgtttttctttagataactggtaatgatgcacattacaaaggagacttttctaaatctcaagtcctttgctaatttttctttggaacaacagcacattttcaatgccaaaccttctcctacaacatacaaaggggagatgccaaaactctgaattcttgtaacggatcctgcaactagttctatccagaagatggagacaatattccctggagttgactgaacatgtgagaaggcacagctcagaaggagaggaaggctgagggcagtgaaatgagaacctatgcatcacctggcctttttacatgttagtctatcctactatcccaggaattcacttctgctgtacttgagattcagggataataatgtgactcctcctcccacattctaagtaaatatgttaactagatgagcatttatgtacattttagaacaaagtctccagaaaggtataaagtttattaacatctttaaaaaaaaaaaaaaaaaaaaagatgggccgggcatggtggctcacgcctgtgatcccagcactttgggaggccaaggcgggtggatcctttgaggtcaggagtttgagaccagcctggccaacatggtgaaaccccatctctactaaaaatacaaaaaaattagccaggcatggtgtcgcacacctgtagtccccagctactcgggaggctgaggcaagagaatcgcttgaacctgggaggcggaggttgcagtgaaccaagatcgtgccgctgcactccagcctgggcaacaagcaaaactccatctcaaaaaaaaaaaaaaagatggaacagaacacagctactgaatatgatatagttccttatttacaagttttactatgggagggacattttcctcagcatttcaaataatcagaggagtagaatttttttctagaaatatcagtatttcactctccaggtcgaagattaatgaaaacattaagtgactgcaccagttagaagaagataaactaataccttaaaaatatataaaaaaagaaagggtagttgctacttaaacatgaattttcacaaaattattctgtgactaattcagacaatctatttgcttagaaaagctggcaaaaaaaaaaaaaagcacattacatgaatatgcttcatttaagtacatgctttcgagctgatttaaaaagaaaagttgaattatggtttccagagctttaggagtccatcttcactgtaggtagcaatcaggttctgatgagggtgatgtgcaataccaatcacatccttctcgtgcactgtcaaagttctctccagtttgccagtgactgtactgaaacagtagagcacaaagtcctcccctacacagtagatccattcaccacggggagagagggcacagcaaacaaagtccccaccttctcttttaccagaactgaagcttctgacaatctgcccctgcatgttcatgatgaccaccgtgtttgatctgttgcacaccacaaagtgctcagggtttttaggaagtagaatcacactgttgacggtaatatctgtccctgcggtgctgcccagggatttaaaggtatttgaacattctgtggtcttcatattccagatctttacagtgccatcagaggatgcactaataatgtaatgtccatcttgtgtaaatgttgcttcgttaacaaaggaggaatggccacgaaattccttcagggttttcccagattttaaaccatgaattctaattgtctggtcaaaagaagcactaaggatctgactgctatccttagaaaagcttagacaggtgacacccttactgtgtgccctctcaaatctccttaaacattgtccactctgaatcttccacaccttgatttttccatcttgggccccagttgctaacatttctgtatctctgctgaaacacatgcagaggacagcatcatccatcatcataaagttatcttgggcctggtacttaagatcctttctgatttttccagtagtaaagttccatacttcaatgaatccatcaacagacccagtgaccaaatactgaccatctggagaaaatcgagcacactccacatgtgatttctgaccaaacttaatatgcctgctcagttgtgtaggaaacttttcttcttccacatctttgacagctgccttgcctcgaaacaaatctatggtcataccaggaggaagcaatccctgatgctgctgccacttcagtgcctgtcccagcaatgccatgagacgagatggaggcaccacactgacttcgccagctaaggcctgggcaattgctgctcttctcttttctttgctacttccatctgggtatgcctcacgaggatcaaagtaagacctggccaaaaggttctccagatgaatatatcgctctggctgtgtttgttttaacatgatcatgggatcagtctgtctcaaaagtgacctggcagcacccaattcacggagctctatcaattccagaacaacctgttcatagaggtcaatgagggttttgtctggcaatttcagagactgtatagcctgcaacacagtatcccaatggccactgttaatgtcagccacaaaactctcaatgctgtccacagtattcagagacacagtagtctcctcctgcaaggtggctaacgcccgatgtaaactgttctccttcaagtactgcataataaggcggatcacatccgaagattcgatttcgatcgacatagccgtatctctccgggagcaggccccagctctccctcaaggccagtcgcgcaacacaccaacgac

SEQ ID NO: 9820 - RNA, 37 nt, Homo sapiens
  source 1..37: mol_type = other RNA
caaaaaccgcaattacttttgcactaatctaataact

SEQ ID NO: 9821 - RNA, 2612 nt, Homo sapiens
  source 1..2612: mol_type = other RNA
caaaaaccgcaattacttttgcatcaacctaatattattgacattatggtataattatcattttacagaagatgaaagtgaggctcagggtgaagtcacttaagtcccttgactggtacacgccacagccaacatctgaactaatgttctggttctctttcaaccttaccgctctcgtacctccagcgaggcatccttctgcctccaacagataaagtctgtgcaccttaaaatcgccacggcatgtcttcacactttattctttctctgttcttcatgtcaagagaggcagcatggtgcaatgaaaagggtgtcagaacacctagttccgtggtctggggcaaactcctctctctgggcctcagtttcctgttggcctccacgtggtgcagcctgaaggcttctcctgtgctctcattcaccacatcaaattggtgtcgataagccacacagatgagattgtcactctcttcagctggcccatccactaaggtcatcaccatgggagagtcagacagacagatctccctgatgtactggaattcttcaacaggtgactcagacaggggagataacaatgaggtgctggtgaccccgcttggcttgttgtgttttcttgtgatcagaagcagtttattccgaattgcaaccacaatcctcagctctctgctgtggtgagtgttaatagcatacaggtggcagccttttgttttctccaacttgttttctctgcagtcagacctgctcttcccagcctgcttcccctcaaggcccttttgcagagcacttagcctgaagacaaagaggcgagcatcttttcctttgtctgctctgagaaccagaaggtccagggtctcaagcacatgcatttgcttcactggcagagttctgtcaaacacgggcactgatggaaggtcatcatccactagcaagacgccagcatcagtggaaaccagcaaggcctggccccagggatctgcacacacggcttcatgagggaaattactgcagaaacactggggctcccacggctcttttttacagatccctgaagctgccaagcttgatggagcatcccctctcacaatggatttcagttttagtgcctgccctattctaacaaactccgcctggcgggcctcctctttcttccgcgctgacttgggtgactctggtaagacatcactaaaagatcgtctattaagcatgttcttatgcaaatctggcatcaaatcctggtgtaaagatctaatcaacatatccagggtacgccgacgtttctgggcaaatgttggggtttccaaagtggctttttcaccattaattaatttcactagcaaaaagtccctgaattcctggtggtctgtaaacactggtggagttggcaagggagggccaaagagtggtacgctctcttctgaaaatattttcagcctgtaattgtcattttgttgattgtatctcactaaggcaaaaatatgtgtaaagtgggagcggatcatggaaggcttaaaggcaggagaagattcctctccttcttggaacacaatggtgacgatatcgtttccaatgtggcgtttcctttccacctgctgtttgttctctttggaatatggcaacatggtggaaacatgaaacatgatctcatgcccttggtacacagtataaactgaatgtatccctgtggtatcatttttggtatccagaccgccacggtagcccgtccagccctttagagtgattgtgtcacccagaagatttaaaaatttttgaaaaggctcgcttccaatttcattgctgaacatctcatcatcagtgagctgcccatctttggcaaaaagaaccccaaacttgaaattcacagagccctcttgttcttcaagaaccagcaagtccttttgtatttcaggatgaaaaatttccctggggcctttctcaaatttgtccagattcatggcacttaagatggacttcacagaaagagtttttgtgggactgtagggaaggcatattttctgggtacctgtttttctccaaagaattgcacggtattgagggacacgttgattgttttggtcagaaagggtcacggacaagaagaaagggctcttctcggcatcgtttccaatgtagttctgatggacttgtcctaaaaaatatttgaaataccatctggtgtggtattctgggttctctaagtgcacgtctgttcttcgccaagtaccaggcagggcagttgcattctcatctgaagagccattttccactctgaatcttccagccctttggatggctccatcagcatcactggaaataagcagctccacagatccataatgtttcctactgaaatccccacgtctacagcctaggtcttccgagacagagttacaggttgacctgggactctagttcagggtctttcgttggccatgtctgaaggggctggatgccgaaggagagagacgactttgctttccatagaatggtttgtgctatctgactcccacaaggcaccttcgttaacgggtccatcagtgggcctggaggctgggcagctgtccttgggctctcgaagctgcaccccctgcgccgcagcgccgccctcttct

SEQ ID NO: 9822 - RNA, 4025 nt, Homo sapiens
  source 1..4025: mol_type = other RNA
caaaaaccgcaattacttttgcatcaacttaatagaacatctgtattcccaagatctactgcctgttctttttttgtgaaaaatgctttattgtcctacacagtttttaaagtaatagtttaagtatcaggaatatcaagatattaataatataaagcaacagtttaaaatcaataacaagaaaacatttcttcttctgtgtagctcaaattcatttcatggtggaaaacaactgacagccccagcagtctctatccttgagcctgcagtggccttcaatgaatggtaggtcataacttcacagaatccaagtaggaggctttgtgtattttgttcttagggatgtttgttttcttgtttgtttaaaagaatgaaaacatggcagcgtatctctcaaactgatccctaagtattataatcactgtggaatataacaggctgcaatcactgctgaaggatgtttagtaataaagacagcaaaactgcgagtaaaacctcaagattctagtggtctagcttcccacatactccaaagctcagcaaacttttgcccaagggccaagattggccaaatatttttgttgaataaaagccacgcccatttgttaaagtatcttctatggccgctctctaagatagcagagttgagtggttggaacagagatcacacggcttgcaaagccaaaaatatgtactatatagccccaaactacaaagccctttaaatctctaaaattgtgtaaagactgttggcttattttcagagctctgtcaactctctgtaaacgataataaagttaaaaagagttgctgcataacttcaatgggctaagatatttggagaggggtttgctgggaaaaggagacatctggacatctgcattacagcagctaaggtcatagctgacacctccgctaggtaactcggaggaaggacattgaacttgtggcaactctggaatttagtttaactctttcgtttaaaaatacagaaggggttagcctggatgacctttaagcttttgaaaattcatgatcgtttaaaatgacgtaactaaaaccgtaagcaaattcagaactacatgactgcgcaacatcatcataaacgtcccatagcacctgcctaaggagcaggaaagtaatatatttaagaaaaatgggaactgaactggttacacaagtgtatgtggaagtttcttgtactattgaaacttttcagtaaatctgaaataaagaaaacggtatgaaatagttaaaacaatttaaatgttagcacttaaaaggggaaacttcagtgaaccttcttcaacaagcgaagttaacacagcagcagccataagggatctgtaaaacataaaccacgtcgtgtgctcgctgaatggagcatgcctgaggctgcagacctccctcattccctctcatagtgcatcctaaagttccccgtacaaatgttacctttgagtttatcttacttgacggaaaccaacctaatatctaaagagagcaaagagagttaaaacacaaaagaagccaggagtggagagagggacaggagggacaggggagagggaaaaggagtggtaagagaaggaaaggatggagggggaggaatacaaatagaagagcctcgttaatcaacaaacgagataaacgtggtccaaatgattagaagtataactgtcttttgtgatcttttctttggcagaataggaagctgacttaaccaaaaatacttgactctcacacaatatatgtacatcccatatattttacatatacacatattccaaaaagagaggttatttttataaaatacaaacactaagcaaaaattatgctaactgaaaaagtgcctagagagccacatacatccacgttgttaaatatagaaactaactgtaatgagaatcattatctccagtttccaaggataccaggataagcactactcctaaattgcagttcattcagcaaagggcacagaataatttatattcagggtcatccctagctgagagcagatgtggaaggaggaccagggtaaatcaccttgtttcttctattccatttgctacctgatccagttcccagccctcgacccccacactctggtcccaaccttggccaatgttttatggaagaaatttggaaaatctgcttgtaaatggcaacttccaagagaaaaagaatcttcaaagggcagggcagtctgagatgtgattaatactgggggtagggtgggggctggtatttccatttgctttgtctgtgaaaaggaaaggagtctgggagtctggttttgtgtgtcagtcacactagtcgccatctttcccagtgcctataaggaaatttcaacttcccactcgaccaaggctatgcaaagcttgccactcataaactgccatggtctctagaatcaaattcagcttcaacttgttcttccttcttagactctagaatctagatctttcataacaattactttttgtttctacagcaataaaaatataaaagctactttctgaaaacctaggagatagtgcctctgaatcatttatttgtttattcaagaccacttactgttgttttcaatgtggcaggcattgcgccaggccaggcagacaggcattacgccaggcagacaggcattgcgccaggcaggcagggacaagaagtgatagataaggtatcaataacaggccacgccacttaggcagtttaaaaagaggcattcttcctcttagtcaaatcgtcacttactaaaatactgatgcggattttatggatactctagatttgtcttaaacttacagaaagtacatataaacatacgattcagatataataccaattttccatttagttccttccccatcacctgtctacccaatacaataataagatctgccatatagcacctcagctaggagcagacatccttctaacgggcagaagagctctctctgccttcaaatgcttcctcttaatggacaggagacactgtaccaagataagcgtcttagcttaatgtgataatacaggagaataggctattttgataatgaaggccttctaggatgtcccttctttgcaggttatattaatcgatactggtcactgtttttaagaggacgaaggaatgaaacacaacaaaggttcccaacagttacgtaacatatacagtctatctcaataaggcaagctattttaagattaacagttaatacaaaatttactacacgtcctttcctatatattttagatgacttgacgactgcatacctaaatgcatcctcatgataatgcctgtacagcctcatcttttcccaacaacagactcaaggttttttttttggactattaagcttgtttctaaatcccttcaagtaataacagcaaattttaaaactatatgaaataaaagtctcggttctcttacaacttacatcagtgattattttgatgtattattatgacactttctcacaaggcgcaacattttgaggtaagatggcttcagacaagattttatgtctgaatcttgaggctttgaaaatgctgagcttgtgaaggctcaatataataggccactatttcatcttttccctcgtcccacccaaagctagcacttggtagggcaaaaacagacactttgttaggtggagcaccaaacacagaaagcattcacaagtcactggcagaaaggtcattttctgttttaacatctttttctgataacccagatcagttttcataaaacccctgaaggtagaaaccagcttacattaagcgacatcattgtactccctacttgtgcataataatcaactttttaaaaaattttaatcttcagcattaaaagtatcctacccaccaattcaggaacctcgaactcggactggagccacttcgctctctggatgtaaaaacctcagacgatcacctctttttttctctccctactgttcaaacacctaaattatggtttagtgtgttgcacatgtcctcaaaaatactttctagta

SEQ ID NO: 9823 - RNA, 2386 nt, Homo sapiens
  source 1..2386: mol_type = other RNA
caaaaaccggcaattacttttgcaccaatttaatattttagagtgtacttctacttatttaaaaaaagttaactgtaaaacagcctcaggcagatcctacagaaggtattccagaagaaggcattgttatcataggagatgacagctccatgcatattactgctcctggaaggctttccagtcagctaagatgtgaagctgtaaaacagtgatattgataatcctgactgccccgctgtctacacctggtttcaaaccatatggtgtcagtactaggctggactgcaccagcagtccaggcagcagtggcaccccaactagacatagctgtgtaccatgtcctattaggaatggaagaacaccctttctaacagtgaaggctcggggtctaggggtgccccaggccccatggccttatcttgcattaggactacaggttccaagacctcttgcaactctgctgctaagggacttatacttagcgtactccactgctctaagtaggtgccccacttcgctaaagtggatgtctgtgctgtcccagtctgggggggtcattgctcatgaacgcacccatcccactatggggtaagccatccacacgactgtaacccatccagccacgctcttatgaacctgaagggcagcatatatggttactaactgcttctttattaatgaacactggggctcagctcccttccatagctgggactaaaagctgactggcgcttccaagcactccatatactgccataggccctagccaactctattggtggttacatgcacatctagtttaaatgggcaccctggttaaccacccagagggcttatgtcatcagaagggctgtttcagcctcatcatcccaatcccaggcaagaggggtgttgtggcctccaaaccagcaaaagaactagaggttaacataacatcattaataagaaaatgatatataatggggctatacatatagccctgcagcaacactatgaaagtccattgtcgccctcccatgaaggcaaactgttcctggctctctggagcaatgctgattgagaagaatgcattggtcaagtccaccacacagtggcaccatcccagttctgttgtcaaacggtccatcaagtccatgacaggtggcacagctgccaagtcttgcaaaacatccacccccaagaatgtcctcaggcatgcaagagacatacacagtgcataagtggagagccaagcagctgatgcccaggtgcaaagacacaggtttcactttcactgaccagctttcatagctgtctatgcagccttccctggaaacttatccgggtccagggaccagtggattgccaagtccatatatggcctttggttgtctggtatcccctaccaagccgggcaccttggccagttctcttatcaaacagaaaatgctttatacttccaccaactgcagcaggtactctttgaactggaacactctggcaggaccaggttgcgcagcaacatccttctcccaaatgacttgcaccaagtctcatcccattctcattgccagttgttaggtttagggttcgggtccagcccatgctgaggtacaagggagtgggtcccttacagaagatgtcatcaacaaaccagaggcggagatgtcactacaagatttgcagctccattacttcaaaatgcacgattatgatggcaattatttgcttgatggtttagaaatctccacagccatcactcatatacagggaccaggattttactccagttctgccgactccagtactggatctcttaagctggatcctagcagatctgcacaggtacctactggaatgcttggctccatgatccatggctctgtcccttgctctaactgggaaatcacatcaggtttagaaacttggagtcctatagagaccaggtgtgtataattttccaatgtcacatccctgaacaaatctctctggccagggtccagctgtttccattcttcctgggtaaagtccactatcacatccttgaaagtcaccgcttcctgaaaactggctgatgagagtagattatgtcccccttggagaagggtggagtctggagaggacagatcttccatctcaggagctcatcccgttcctctggaacttgaacaccagggttcgccaggcagcgttccttcagctggtatctcggtctaggactcagatgtctaactccccttgcagggaatctgcaacacgctgaggttgtctaccctgagctcccctccccctatagcgatccacacactctgatcccgggtccggaagcgcattgaccgccaccagacctaacgcagggagccgaagcaactggacttccagcgcgccaacctctttccacgcctac

SEQ ID NO: 9824 - RNA, 2601 nt, Homo sapiens
  source 1..2601: mol_type = other RNA
caaaaaccggcaattacttttgcaccaatttaatattttagagtgtacttctacttatttaaaaaaagttaactgtaaaacagcctcaggcagatcctacagaaggtattccagaagaaggcattgttatcataggagatgacagctccatgcatattactgctcctggaaggctttccagtcagctaagatgtgaagctgtaaaacagtgatattgataatcctgactgccccgctgtctacacctggtttcaaaccatatggtgtcagtactaggctggactgcaccagcagtccaggcagcagtggcaccccaactagacatagctgtgtaccatgtcctattaggaatggaagaacaccctttctaacagtgaaggctcggggtctaggggtgccccaggccccatggccttatcttgcattaggactacaggttccaagacctcttgcaactctgctgctaagggacttatacttagcgtactccactgctctaagtaggtgccccacttcgctaaagtggatgtctgtgctgtcccagtctgggggggtcattgctcatgaacgcacccatcccactatggggtaagccatccacacgactgtaacccatccagccacgctcttatgaacctgaagggcagcatatatggttactaactgcttctttattaatgaacactggggctcagctcccttccatagctgggactaaaagctgactggcgcttccaagcactccatatactgccataggccctagccaactctattggtggttacatgcacatctagtttaaatgggcaccctggttaaccacccagagggcttatgtcatcagaagggctgtttcagcctcatcatcccaatcccaggcaagaggggtgttgtggcctccaaaccagcaaaagaactagaggttaacataacatcattaataagaaaatgatatataatggggctatacatatagccctgcagcaacactatgaaagtccattgtcgccctcccatgaaggcaaactgttcctggctctctggagcaatgctgattgagaagaatgcattggtcaagtccaccacacagtggcaccatcccagttctgttgtcaaacggtccatcaagtccatgacaggtggcacagctgccaagtcttgcaaaacatccacccccaagaatgtcctcaggcatgcaagagacatacacagtgcataagtggagagccaagcagctgatgcccaggtgcaaagacacaggtttcactttcactgaccagctttcatagctgtctatgcagccttccctggaaacttatccgggtccagggaccagtggattgccaagtccatatatggcctttggttgtctggtatcccctaccaagccgggcaccttggccagttctcttatcaaacagaaaatgctttatacttccaccaactgcagcaggtactctttgaactggaacactctggcaggaccaggttgcgcagcaacatccttctcccaaatgacttgcaccaagtctgtacaagagtgccaacattacttgcttaactcctacaacttagcaggggcacagacaacataggaagtgtgctccaccacagtagggggtctctggcccacccttggggcccaacagctgctcatgctctattttctggcagaccattgggtgaacctgtaacggaggttcttcctccctgtgtgcatccctcagggactgggcaggcacttcctcatcccattctcattgccagttgttaggtttagggttcgggtccagcccatgctgaggtacaagggagtgggtcccttacagaagatgtcatcaacaaaccagaggcggagatgtcactacaagatttgcagctccattacttcaaaatgcacgattatgatggcaattatttgcttgatggtttagaaatctccacagccatcactcatatacagggaccaggattttactccagttctgccgactccagtactggatctcttaagctggatcctagcagatctgcacaggtacctactggaatgcttggctccatgatccatggctctgtcccttgctctaactgggaaatcacatcaggtttagaaacttggagtcctatagagaccaggtgtgtataattttccaatgtcacatccctgaacaaatctctctggccagggtccagctgtttccattcttcctgggtaaagtccactatcacatccttgaaagtcaccgcttcctgaaaactggctgatgagagtagattatgtcccccttggagaagggtggagtctggagaggacagatcttccatctcaggagctcatcccgttcctctggaacttgaacaccagggttcgccaggcagcgttccttcagctggtatctcggtctaggactcagatgtctaactccccttgcagggaatctgcaacacgctgaggttgtctaccctgagctcccctccccctatagcgatccacacactctgatcccgggtccggaagcgcattgaccgccaccagacctaacgcagggagccgaagcaactggacttccagcgcgccaacctctttccacgcctac

SEQ ID NO: 9825 - RNA, 43 nt, Homo sapiens
  source 1..43: mol_type = other RNA
caaaaactgcaattacttttgcaccaaaccaacagcatcaatc

SEQ ID NO: 9826 - RNA, 218 nt, Homo sapiens
  source 1..218: mol_type = other RNA
caaaaactgcaattacttttgcaccaacctaaaatataataaaaaagtgtcttctctttataacttttctgttgttttgcttaagttatcattgctattcctctgcaacctaaaaagaaatcattgaatatacatttaattttagaataatcactacacaaatgccctaaaagtgtatgtataacatccctgatgtctgcatttgtcctttgactggt

SEQ ID NO: 9827 - RNA, 38 nt, Homo sapiens
  source 1..38: mol_type = other RNA
caaaaactgcaattacttttgcaccaacctaatacctt

SEQ ID NO: 9828 - RNA, 1506 nt, Homo sapiens
  source 1..1506: mol_type = other RNA
caaaaactgcaattacttttgcaccaacttaaatatataacctctctgagctcccattttctcatctaaaaaatgaaataataccaacctcacagcactgttggaagggttggggtaaagcaccaagtacgtgggtagcttatatcctacagaataattttcaccaacatgacccatgaccatgaagtttatggtttgactatctgtaggaagggtacaaaaatacatcatgcaacaaggtcattcatttggaaatgtaatgctttctgaaaaacttgagcattcacttttcttcacttgcctgttctaataagagaggtttggtgtggtgatttttcaatagaaaggatgttaccaatatataaataacataaaaggatcacatgagaattaaagtgaagtaacttaacatacaattttcattctaatcttatacaataatttttcttgactattgatagatcacaataaaggtatgctgatgatataagttattttaagactttggggaaaaaggcttccgtctctggcattgaccttattgtggaggaccctccaaaatcttcagctctgcaccagcaggtatgctgagtcatgtatgatgacataaaccacaaggagtcaaggagctaaaacaaccacagcgactggctcagatctcagatgtgcaagatgaatcctcaggatttttcacacactgaagaaacttgtcaggtctgtagatattcttgcaggaaaattgaatattccttttgcttataatcgattccagctcttttatggtgggatcctggcataagtctctggaatcttctcttccaccatgtatcacccaggcctctagtgtctgaaccttctctggttgcaaattatggacttccacactcccaaaagtgctgtttttgtcaaagattttactgcgggatccattgagcatcacatggaccacatcacaggcagcttctgcaaacctgcgggaaaccgttttccagaatactgaaacagggttgttgctgcagtcctttctccagtctgggcaagattgatagtttatttcttgttgcaaggtacggtctgagttcccaacttcattagtggctgatagtcttcttcagtaatgttgcaaggatgttttgaaataaatgcacccttgaaagcatcccatacactttggcagtctacatgtctcatctcaggatgaatttcagtgtacttgacgcatcgcgccaggacggtctcgggaaagcgcttggtggtgcccggaccgctccactgctggcgccacctcgggacgaccaccgcgagcaccacgacgaggatcaggaccaggatactgacgccaagacagagttgggctctcctagagagccggcagcagggtttgtccccggacaccgggctgaactcgcagttggccatagggctccaggcggggttggctgggcgaagatgaggccggcaggaggctaggcagcaagagagaggctggctgggttctgaaactgc

SEQ ID NO: 9829 - RNA, 1642 nt, Homo sapiens
  source 1..1642: mol_type = other RNA
caaaaactgcaattacttttgcaccaacttaaatatataacctctctgagctcccattttctcatctaaaaaatgaaataataccaacctcacagcactgttggaagggttggggtaaagcaccaagtacgtgggtagcttatatcctacagaataattttcaccaacatgacccatgaccatgaagtttatggtttgactatctgtaggaagggtacaaaaatacatcatgcaacaaggtcattcatttggaaatgtaatgctttctgaaaaacttgagcattcacttttcttcacttgcctgttctaataagagaggtttggtgtggtgatttttcaatagaaaggatgttaccaatatataaataacataaaaggatcacatgagaattaaagtgaagtaacttaacatacaattttcattctaatcttatacaataatttttcttgactattgatagatcacaataaaggtatgctgatgatataagttattttaagactttggggaaaaaggcttccgtctctggcattgaccttattgtggaggaccctccaaaatcttcagctctgcaccagcaggtatgctgagtcatgtatgatgacataaaccacaaggagtcaaggagctaaaacaaccacagcgactggctcagatctcagatgtgcaagatgaatcctcaggatttttcacacactgaagaaacttgtcaggtctgtagatattcttgcaggaaaattgaatattccttttgcttataatcgattccagctcttttatggtgggatcctggcataagtctctggaatcttctcttccaccatgtatcacccaggcctctagtgtctgaaccttctctggttgcaaattatggacttccacactcccaaaagtgctgtttttgtcaaagattttactgcgggatccattgagcatcacatggaccacatcacaggcagcttctgcaaacctgcgggaaaccgttttccagaatactgaaacagggttgttgctgcagtcctttctccagtctgggcaagattgatagtttattttggaagtgttgaattcaccacaccatgtgaggtcatcagcaaggtagcctagcagcgtgtcctccagggtgaacatgtcccgctggacctgtgtgaactgatgggccagatcttttattctgctccaaagaagaatcttgttgcaaggtacggtctgagttcccaacttcattagtggctgatagtcttcttcagtaatgttgcaaggatgttttgaaataaatgcacccttgaaagcatcccatacactttggcagtctacatgtctcatctcaggatgaatttcagtgtacttgacgcatcgcgccaggacggtctcgggaaagcgcttggtggtgcccggaccgctccactgctggcgccacctcgggacgaccaccgcgagcaccacgacgaggatcaggaccaggatactgacgccaagacagagttgggctctcctagagagccggcagcagggtttgtccccggacaccgggctgaactcgcagttggccatagggctccaggcggggttggctgggcgaagatgaggccggcaggaggctaggcagcaagagagaggctggctgggttctgaaactgc

SEQ ID NO: 9830 - RNA, 30 nt, Homo sapiens
  source 1..30: mol_type = other RNA
caaaaactgcaattacttttgcactaacct

SEQ ID NO: 9831 - RNA, 37 nt, Homo sapiens
  source 1..37: mol_type = other RNA
caaaaactgcaattacttttgcactaatctaataact

SEQ ID NO: 9832 - RNA, 2612 nt, Homo sapiens
  source 1..2612: mol_type = other RNA
caaaaactgcaattacttttgcatcaacctaatattattgacattatggtataattatcattttacagaagatgaaagtgaggctcagggtgaagtcacttaagtcccttgactggtacacgccacagccaacatctgaactaatgttctggttctctttcaaccttaccgctctcgtacctccagcgaggcatccttctgcctccaacagataaagtctgtgcaccttaaaatcgccacggcatgtcttcacactttattctttctctgttcttcatgtcaagagaggcagcatggtgcaatgaaaagggtgtcagaacacctagttccgtggtctggggcaaactcctctctctgggcctcagtttcctgttggcctccacgtggtgcagcctgaaggcttctcctgtgctctcattcaccacatcaaattggtgtcgataagccacacagatgagattgtcactctcttcagctggcccatccactaaggtcatcaccatgggagagtcagacagacagatctccctgatgtactggaattcttcaacaggtgactcagacaggggagataacaatgaggtgctggtgaccccgcttggcttgttgtgttttcttgtgatcagaagcagtttattccgaattgcaaccacaatcctcagctctctgctgtggtgagtgttaatagcatacaggtggcagccttttgttttctccaacttgttttctctgcagtcagacctgctcttcccagcctgcttcccctcaaggcccttttgcagagcacttagcctgaagacaaagaggcgagcatcttttcctttgtctgctctgagaaccagaaggtccagggtctcaagcacatgcatttgcttcactggcagagttctgtcaaacacgggcactgatggaaggtcatcatccactagcaagacgccagcatcagtggaaaccagcaaggcctggccccagggatctgcacacacggcttcatgagggaaattactgcagaaacactggggctcccacggctcttttttacagatccctgaagctgccaagcttgatggagcatcccctctcacaatggatttcagttttagtgcctgccctattctaacaaactccgcctggcgggcctcctctttcttccgcgctgacttgggtgactctggtaagacatcactaaaagatcgtctattaagcatgttcttatgcaaatctggcatcaaatcctggtgtaaagatctaatcaacatatccagggtacgccgacgtttctgggcaaatgttggggtttccaaagtggctttttcaccattaattaatttcactagcaaaaagtccctgaattcctggtggtctgtaaacactggtggagttggcaagggagggccaaagagtggtacgctctcttctgaaaatattttcagcctgtaattgtcattttgttgattgtatctcactaaggcaaaaatatgtgtaaagtgggagcggatcatggaaggcttaaaggcaggagaagattcctctccttcttggaacacaatggtgacgatatcgtttccaatgtggcgtttcctttccacctgctgtttgttctctttggaatatggcaacatggtggaaacatgaaacatgatctcatgcccttggtacacagtataaactgaatgtatccctgtggtatcatttttggtatccagaccgccacggtagcccgtccagccctttagagtgattgtgtcacccagaagatttaaaaatttttgaaaaggctcgcttccaatttcattgctgaacatctcatcatcagtgagctgcccatctttggcaaaaagaaccccaaacttgaaattcacagagccctcttgttcttcaagaaccagcaagtccttttgtatttcaggatgaaaaatttccctggggcctttctcaaatttgtccagattcatggcacttaagatggacttcacagaaagagtttttgtgggactgtagggaaggcatattttctgggtacctgtttttctccaaagaattgcacggtattgagggacacgttgattgttttggtcagaaagggtcacggacaagaagaaagggctcttctcggcatcgtttccaatgtagttctgatggacttgtcctaaaaaatatttgaaataccatctggtgtggtattctgggttctctaagtgcacgtctgttcttcgccaagtaccaggcagggcagttgcattctcatctgaagagccattttccactctgaatcttccagccctttggatggctccatcagcatcactggaaataagcagctccacagatccataatgtttcctactgaaatccccacgtctacagcctaggtcttccgagacagagttacaggttgacctgggactctagttcagggtctttcgttggccatgtctgaaggggctggatgccgaaggagagagacgactttgctttccatagaatggtttgtgctatctgactcccacaaggcaccttcgttaacgggtccatcagtgggcctggaggctgggcagctgtccttgggctctcgaagctgcaccccctgcgccgcagcgccgccctcttct

SEQ ID NO: 9833 - RNA, 4025 nt, Homo sapiens
  source 1..4025: mol_type = other RNA
caaaaactgcaattacttttgcatcaacttaatagaacatctgtattcccaagatctactgcctgttctttttttgtgaaaaatgctttattgtcctacacagtttttaaagtaatagtttaagtatcaggaatatcaagatattaataatataaagcaacagtttaaaatcaataacaagaaaacatttcttcttctgtgtagctcaaattcatttcatggtggaaaacaactgacagccccagcagtctctatccttgagcctgcagtggccttcaatgaatggtaggtcataacttcacagaatccaagtaggaggctttgtgtattttgttcttagggatgtttgttttcttgtttgtttaaaagaatgaaaacatggcagcgtatctctcaaactgatccctaagtattataatcactgtggaatataacaggctgcaatcactgctgaaggatgtttagtaataaagacagcaaaactgcgagtaaaacctcaagattctagtggtctagcttcccacatactccaaagctcagcaaacttttgcccaagggccaagattggccaaatatttttgttgaataaaagccacgcccatttgttaaagtatcttctatggccgctctctaagatagcagagttgagtggttggaacagagatcacacggcttgcaaagccaaaaatatgtactatatagccccaaactacaaagccctttaaatctctaaaattgtgtaaagactgttggcttattttcagagctctgtcaactctctgtaaacgataataaagttaaaaagagttgctgcataacttcaatgggctaagatatttggagaggggtttgctgggaaaaggagacatctggacatctgcattacagcagctaaggtcatagctgacacctccgctaggtaactcggaggaaggacattgaacttgtggcaactctggaatttagtttaactctttcgtttaaaaatacagaaggggttagcctggatgacctttaagcttttgaaaattcatgatcgtttaaaatgacgtaactaaaaccgtaagcaaattcagaactacatgactgcgcaacatcatcataaacgtcccatagcacctgcctaaggagcaggaaagtaatatatttaagaaaaatgggaactgaactggttacacaagtgtatgtggaagtttcttgtactattgaaacttttcagtaaatctgaaataaagaaaacggtatgaaatagttaaaacaatttaaatgttagcacttaaaaggggaaacttcagtgaaccttcttcaacaagcgaagttaacacagcagcagccataagggatctgtaaaacataaaccacgtcgtgtgctcgctgaatggagcatgcctgaggctgcagacctccctcattccctctcatagtgcatcctaaagttccccgtacaaatgttacctttgagtttatcttacttgacggaaaccaacctaatatctaaagagagcaaagagagttaaaacacaaaagaagccaggagtggagagagggacaggagggacaggggagagggaaaaggagtggtaagagaaggaaaggatggagggggaggaatacaaatagaagagcctcgttaatcaacaaacgagataaacgtggtccaaatgattagaagtataactgtcttttgtgatcttttctttggcagaataggaagctgacttaaccaaaaatacttgactctcacacaatatatgtacatcccatatattttacatatacacatattccaaaaagagaggttatttttataaaatacaaacactaagcaaaaattatgctaactgaaaaagtgcctagagagccacatacatccacgttgttaaatatagaaactaactgtaatgagaatcattatctccagtttccaaggataccaggataagcactactcctaaattgcagttcattcagcaaagggcacagaataatttatattcagggtcatccctagctgagagcagatgtggaaggaggaccagggtaaatcaccttgtttcttctattccatttgctacctgatccagttcccagccctcgacccccacactctggtcccaaccttggccaatgttttatggaagaaatttggaaaatctgcttgtaaatggcaacttccaagagaaaaagaatcttcaaagggcagggcagtctgagatgtgattaatactgggggtagggtgggggctggtatttccatttgctttgtctgtgaaaaggaaaggagtctgggagtctggttttgtgtgtcagtcacactagtcgccatctttcccagtgcctataaggaaatttcaacttcccactcgaccaaggctatgcaaagcttgccactcataaactgccatggtctctagaatcaaattcagcttcaacttgttcttccttcttagactctagaatctagatctttcataacaattactttttgtttctacagcaataaaaatataaaagctactttctgaaaacctaggagatagtgcctctgaatcatttatttgtttattcaagaccacttactgttgttttcaatgtggcaggcattgcgccaggccaggcagacaggcattacgccaggcagacaggcattgcgccaggcaggcagggacaagaagtgatagataaggtatcaataacaggccacgccacttaggcagtttaaaaagaggcattcttcctcttagtcaaatcgtcacttactaaaatactgatgcggattttatggatactctagatttgtcttaaacttacagaaagtacatataaacatacgattcagatataataccaattttccatttagttccttccccatcacctgtctacccaatacaataataagatctgccatatagcacctcagctaggagcagacatccttctaacgggcagaagagctctctctgccttcaaatgcttcctcttaatggacaggagacactgtaccaagataagcgtcttagcttaatgtgataatacaggagaataggctattttgataatgaaggccttctaggatgtcccttctttgcaggttatattaatcgatactggtcactgtttttaagaggacgaaggaatgaaacacaacaaaggttcccaacagttacgtaacatatacagtctatctcaataaggcaagctattttaagattaacagttaatacaaaatttactacacgtcctttcctatatattttagatgacttgacgactgcatacctaaatgcatcctcatgataatgcctgtacagcctcatcttttcccaacaacagactcaaggttttttttttggactattaagcttgtttctaaatcccttcaagtaataacagcaaattttaaaactatatgaaataaaagtctcggttctcttacaacttacatcagtgattattttgatgtattattatgacactttctcacaaggcgcaacattttgaggtaagatggcttcagacaagattttatgtctgaatcttgaggctttgaaaatgctgagcttgtgaaggctcaatataataggccactatttcatcttttccctcgtcccacccaaagctagcacttggtagggcaaaaacagacactttgttaggtggagcaccaaacacagaaagcattcacaagtcactggcagaaaggtcattttctgttttaacatctttttctgataacccagatcagttttcataaaacccctgaaggtagaaaccagcttacattaagcgacatcattgtactccctacttgtgcataataatcaactttttaaaaaattttaatcttcagcattaaaagtatcctacccaccaattcaggaacctcgaactcggactggagccacttcgctctctggatgtaaaaacctcagacgatcacctctttttttctctccctactgttcaaacacctaaattatggtttagtgtgttgcacatgtcctcaaaaatactttctagta

SEQ ID NO: 9834 - RNA, 24149 nt, Homo sapiens
  source 1..24149: mol_type = other RNA
caaaaactgcagttacttttgccaacactgtttttcacttcaaagctatataatcctttgtcactcatttcggcacaggggattttaagggaagccactttattgatgaatgtaatgtgatgtttgctgtctgcagacaattctcttccatctttgaaccacttggctgagagttctggtgttccagtcactacacactctaatgcaaaaggatttccagtagtgacagtcatgggttcgggcttctctatgattcttgctggttctagtacagtcaagactgcagagcattctctcattccagcatcgtttttgatttggcatatatattttccagaattagatgcttctggactccccagctggagggttgcaatgttatcaatgaatgaaatcctggtattttcactctctctgatgacttcacctctatctttcagccagacaacagaaattggctggaagccctccactatggcccgtaactcaacagcatccccaataagggttgaggtgtcacttagctttttcacgaatcgtggaggttctttgaacttgacagagcaagaacacgtgtcacttcccacctcattagtagctttgcagtgatattccccgacatcggaggcttcaagattaaggatatgaagacttgtatcaaaatgttttgaagtgattttaaatttcttgctgtttctaacctgctttcgatctttaacccatactacttcaaatgggggagttcccgaaatttcacattggagaatcacatcagaacctttaagagctcctactggagaaggcttctgggtgaaaacaggaggtgctttcactgtcaacgctgtgctgcagctggcgtcaccaacaccattatgagcctcacaaatgtagtccccgctgtcttcagcactagcttcattgatcgtaagcaatgccacagaattaatgaatgacatgttgtatttccaactttcatgaagttcgctgtcatttcggaaccatgaaactttgatttctggggagccacttattttacattccagttgaatggattctccctgctttgcaacttttgaagcttctaatttcttaacaaactttggaggttcttttacactgagctgagctgagcacatgtctttgccaacatcattggttgcttggcaagtatattgaccagagtctcctttgcctactttaagaattctcaaatgaggagtgtttcccacacatgtgattgtatagtttcctccaggacggatctccttgttatcttttgaccaagtgattcgcatcggttgagcaccagtaacatgacactcaaaatcagcactttctccagcaataacatctatagatacaggcttgatgtcaaagaagggagatttcttgggttctcttgctgtgagtctagcactagaagatgctgttccaagtgggttggaagctgagcaagagtactggccagagtgactcaagtcagtttgcaaaatttttaaagttgccacattatctacaaatgaagtctgtagattttcatcgtctcttaaaagtactccatctctataccagcacacttggatgggtgcagagccatttaatcgacaagtgagtgtaacaggtaaccccacagtttgttcaatgtcctttaattgtcttgcaaaagaaggtgggagttggcgctcttgaattctgaacacagtcttagaagaagcagttcctatactattttctgctttgcatgtgtactctccactgtcattgatgttcactttattaaaaacaagtgtggccacattgtttgtaaagtaggtcctgtattcaggagttggccgtaatttggtatctcctttgtaccaagacactgtaatttctggtgtcccagcaacttggcattgtaaagaaaccgaatctccaactgctgcctccagaggttccagttccgtaacaaaataaggcggttctaatgtagataccagagctccacaaacatcccttcctgcctcattttcaatctcgcaggaatactgccctgcatctctttttgtgctattcagaatttccaggatacaagttttctctgttgtgactatgttacatttttcagaggtagttatgttaaaaccatcctttttccaagtgacagaaattggaagtgttccagtgtaggtgctctccagaattatggacttccctggttctacagaatgatcacttaatctcttcaaaaatgcagctggttctttcacaaagagacgggtagtgcaagatgcttggccagcgttgttagaaaccacacaggtgtattccccactctgagatatgtcaatattaaataattccagttctgccacagtgtcttcaaaatagatgttgcaccggtctcctttcactagttctctggcacctctgaaccagttgactttgaatggaggggttcctctaataacgcttgtgaaggttacatttttgcctggtagtacttccaaaggttcaggttctttcacaaaagagggtggttcttgtacagttagcactgcacgacattcatcagacccagcgacattagcagccacgcatgtgtaattgcccatatctgaggaatccagagaattcaactgcaatgtgcagacattatctgaaaatgtggtttggtactttgctccactgacaatcttggttttctcatgaaaccaggcaactgaaataggtgatgatccagctactttgcattccaagatgcaagaagcacctaacaccccaccagtatttttcagtcttcgtgtgaaagagggaggaactgctcggtctgaaacatcaaccacagctgtgcagctgcttttcccaacattattttgaacctggaaagtgtatgtgcctgcatcttgcctttcaactgagagaatccttaaggaagagattttgttgtagaagctaaatttgtgtttttggctgctggtcaacagctttccatccttgtaccattcaacagagagttccggagtgccagccaccttacactccagagtgcacgtttctcctacagtcaccgtcatcggtcctgccttctcaacaatgactgcgggctctaagaccatcagtgtggccatgttctccctcattccaccatcattcttgatttggcagatatactttccagcattagctggctctgcttttgcaaactgtagagttgcaacattttccacaaatgtaatcctgatgttttcactttctctaatcacttcttccttctctttaagccactggacaaaaataggctgggcgccttctatggatgcttgtaattcagcaggctctccggctacaacagtgaggctgttcagtttggagacaaatcttggtggttctttcaattttacagtacaaacacaagtatcacttcccacttcattctgtgctttgcagtggtattcaccgatgtctgaagtgtccacattgagaatgtgaatacttgtgtggaagtttttggatgcaatcttgtatttcttgctgcttctgagttgccgcttgtctttgtaccataccacctcaaacggtggtgttcccgaaagttcacattcaagactgacttcagcatttttaagggtttctactataggagggaagctgctaaaaacaggtggctcttttactataaccttggtactgcagcttgtgctgccagcgggattctgagcctcacaaatgaaatctccactgtcctcagtactgagattgttcatctgtatgacggccactgagtcaatgaaagtcattctgtacttatcactggctggaagttcatgttcatttcggaaccacacaactctgatttctggggatccagctatcttgcattcaagtcgtgaagagtcacctgctttcacaattttggaggcttctaatttctttacaaactttggtggttctgtcacaagcaacatcgtagtacaagagtcgctaccaacatcattggtaacatggcaagtatactgtccagtcttagaagcatccactgagtagagatttaagaagctagtcgacccttccaagccaatgaaacatttaggacctgagacaagttccacatcatccttaaaccattttattttaaatggtggtgttccttttagtattgccttaaattccactgtagaatcaggtatggcttgctgtcgcccaggtttcactaggaagcttggtggttctttcacagttaagatgccactgcatgcatcatctcctgctacatttgacactttgcatgtgtaatttgcagtatcttctaattccagattattaacttccagagacacagatctctcatggcacacaagtctgtattttgcacttgtagatatttcttttccatccttaaaccactgagcactaatgggaagtgaaccagacaccttgcactccatatgaatagaagagcccagaactttatccattttggttaattttttggtgaatgatggaggaatattttgatctagcactcttaagtaggcatcacagctactgcttccgaagtcattttccaccttgaaagtgtactgaccgctgtcctgcttcattactgactgaattctaaaactggccacgttattttcaaaactcattgaaaagtatctactgggaactatttgtttcccgtctttaagccatttcactttgagttctggtgttccagccacaacacattccaaggtcatgggatctttctccgtaacatcaactgatttagctttctctacgatttgagctggttcttgtactaaaaggaaagcataacacctctcaactcctgactcattcttggcttgacaggtatatctcccactgtgtccattatccacacttctgatttgaagtgtggccacactgtccacaaatgaaatatagacattatcatcttcatcaagaatctgatcatcctttagccaggttatagaaataggaggagaacctgccacggtactctgaaaggtggcagaacttttcaaaacagtagtggtattttctatcttcttaatgaatgatggtggttctttcagggcaactctagtactgcatgagcagctgccgccttcattggatacaatgcactggtattccccagtgtctgaagggtcacacttggttatatggaggttaaacacagacactctgtcggtcaatgtgtattttttgctgcttcgaatttccctgttattcttcagccaagtgacttcaaacggaggtgttcccgtaacttcacactccagctccacgtcactatattttactacctccacaggcttcagctctctgataaaggtggggggttctttcactttgagttcaatgctgcagctcgccgtgcctgcgtcatttcgagcttcacacacataagtcccactattttctaccctggcaccagaaatctggaaagtggctaaaccatcaatgaaggaaatgccatgtttctgaatggctgttatttcattcccgtctagataccaagacactcggattttaggagtgcctgttatttggcattcaaatgttgttgactgtccattcctcagcactaagactggactgggcttcttaatgaattgaggaggttcttttacaaagagagtggctttgctggttgctgtgccaacatcattgcttagttggcaaatgtaggttccagaatcggtagctttggctgcaaagagctctagactggtagaggtgtcatccttccaaactgagcgggctgctcctgagtgtaactctttgttatctttaaaccactttattgtcatgggtgcagtgccacccacaagagcctttaactgtacccttgtgttgggattgacatcttgtgactgtggcttttccacaaagtaagggggttctttgactgtcagatgcccactgcattggttgtgccctgccttatttgtggcagaacaagtgtatgtcccactgtctgtaccttccagctggctgatttccaagaaggcagtattgtcatgaaaagagaatttgtacttttcactagctgatatttcttggtcatctttgaaccactggatgcttatgggatgtgacccagccactatacattctaaatcaatgaaagaacctttaatgctgtccattttcttcagctttttggtgaatgaaggaggtatgataagatctaatacattaattctagccttgcagctgctcctcccaacatcattttggacctcgaaagtatattctccactatctttcttttctgtagaaataatcttcagtattgagactgtatcagtgacactgattttatattttgagcccagggtcagttcttggccatctttaaaccatttggctgtaatctccttagtccctgaaaatttaacctgcaaagtggctgggtctccttgggtgacatctatagacacagcttcctcggtgattgttgcaggttcttttactgagagtaatgcagaacatctttgtattcctgcatcatttttggcctgacagacatatttcccatcatgcttgacttcaatgccactgaggtacaaactggccacattgttctcaaaggtcattcttatattatcgtcttcagtgatttcatcgctgtcttttagccaagtcaccgtaattggcaaggagcccttcagagtggcctggaaggcagctgtgcctccccggagggagctggtactctcgatcttctttatgaaggatgggggttctcttaaagtcaccctggcactgcagatgctgctgcccacctcattggtcacccgacactggtattcgccagcatctgcagctacaaacttgaggatctgcaggctaaccagatgatcctgaatgaaagtcttatactttctaccacttcgcaggattgtgttatctttgaaccaagtgatctcaaagggaggagtgcctgccacctcagccagcaacatgacatcgtactcctttaagacttcaattggcttaaattccttggtaaaataaggtgactctttgactattacaatgctactgcagtggtcactgccagcctcattttgggcctcacacatatattcaccactgtcttcgatgccaacatctgtcagtcttagaactgcagtagactccacaaaagacattctgtgtttgctgctctccttaatttctctatcatttgcaaaccatgttattttaattggaggggtaccagttactttgcaggctagctgggtggcatctcccttctttaacagctgtgatggctctaacttttcaacaaatgtggcaggttcttttacaaacaagtttgcactgcattccacccctccagcgacattgctgactttacatgtgtacgtgcccgaatcagaggtttttactaaatagagttccagggaactctctaaagcttctttggtaatatagcagcttccaccagaaaccagctctttgttgcccttaaaccatctgattgtgagaggagtagatccttggaaagtgctcttcaggcagactgctgagccaggcagaacatcctttgagccgggtttagttacaaaactgggtggttcttgcacaatcagggctccactgctgtctttgcttcccacggaatttgtggctcgacaagtgaaattccctgcatcattcatgtctactctgatgatctccaaagaggctgtgccttccacaaatgctatcctgtatctgtcagaagcagctatttctttgccatccttaaaccaggacaccctcatggggagggagcctgcaattttgcagtccagtctgcaggtaccattaacaacactatccacgttgcgcaagggtttggtaaaaaatggagcaatgtctcgatctaatacagtgaatgtagtctcacaggagctgctgcccacttcattggaaatctcaaatgtgtattggccactgtcgtgcagctcagctgaataaaatttgagctgggcaacattgtttttaaaacttattcggtattttttactggcgaccaagggtctcccatctttgtaccatttgggcttcagttctggcgtgcctgccactgtgtactccagtgtggcgggatctcctgctgtcacctggatcagttctgctcgctcaatgattttggcaggttctttaactattaattccccaacagatgtttggcttccagcttcattttcagccaggcacgtgtatttgcctccaaaactaatctgaacatcagggattatcaagactgcaacaccattggaaaagctcattttgatttttccgtcttctctgatgacctcttgacctttcatccatgtgacagaaatgggctctgaccctctcacagcagcttgcagggtaacggtttgtcctcctagtgcaatcaaatcatctactttctttacaaaggttggaggttctttgagtaagtgggttgccatgcagccacacttgccgacttcattagcaacaacacattcatattcaccaacatctgcactattaaacgaaaagatctccagacacacaagagacttctgagaaaacaatctgtattttttactacttcgaatttgtttcttgtctttgaaccagctaatttcaaatggtccagtgcctgagacttcacactgaagtagagcatttgttcctctcactatgtctgcaggctcaagagttttgatgaaagaaggaggttctttgataactatttcagtactgcagctatcactgccgacgtcattcactgcttcacatgagtaactcccactgtcttcaacttttacatccgtaatatcaagtatagcctcagaattgacaaaatacattcggactgtgttactttcactgagttctttgttatttttaaaccaagtaacctggatcacaggtgagcctttcagcttgcaatggaggcgtgctgattcacctgggagcattaaataagagggatccaccttcttcacgaaggatggtggctctctgacagtgactgtggctgagcaggagctgcttccagcctcatttgaagctgtacagacataggttcctgaatctttcagtttggccaaaggaatctcaagtgttgctattttatcttcaaaacagatcttataatctttccctggggggagtttttgcccatctttgctccacgtaactgtgacttttctgtcttcatctacttggcactcaaggtggaccttcttattgatagcggactgcacaggctctaattctttaatgaaatgtggcttatcaatgatgatcaactctgcttggcagatgtctgctccaaacttgttggaagccttacaagaataaactcctctatcttgaatggtaaggtttgagagttctaaaatgtgtttgttttctgcgtcggaaatcctccagttaggtgaaggtgagagtgcagcaccatctttctgccaaatggtttctatcacaggagtccctgtcactgtgcagatgaacttggctgccttacccacaaaagttgtaagggacttaggtctggagagaaaggttggtggatatgcctctgtcacagttagtgtggctgtacagctgacactgccatactcattggaagctttgcatgtatactcgccgcagtcaaccacctgggttctcaggatttcaaggctggagatatactttgaagatcgaatagaacacttgtcactctcataaatttctcggccagctttaaaccactggaaccggacattgggagcactttggatctcacaggtgaatttggctaggtggcccagtgctacttccaggggttcgattttcctcttgatcactggggcagctctttttactacagtgagtttggctgaagttgctgtttttccgctgtcattcaaggcctcacagacatactctccttgatggtcttcggtatttactttgtcgatgactagcgtatatgtattttgatcttgtaaacacttgaacttttcatctgaaggcaccagtttattctcaaaataccaattcacctctttagcatttgttatggatgttgtgaggtgtacaatatcaccttcctcagaaacagtgtccactaaaggtgtatgtatcatggggccatcctctttgattaagccaccctcagcttcctgtatctttactgtagcaacctcctcagtaccactttcagaggaagactcctctttttcctctgatggtttcagactctcatcttgtttttcgtcagagacaacagctgaagcaacccctttagtgacaggtgtggcatccaaatatttaaccctactttgcacgttaaaataactgacctcttcagttgagatcagatatttagattcaacttctggttcagtaatgggttcaaccttctgtgaacctgaaaaagaatccatttcttcttgcaaacttgttttggctccttgctgaattctaggaccctcagctgttaggatgtctatttcctcatatataatagcacacaaagcatccctaagttccattttcaggttagccatttgaggatcaacatcttcaataatgatggttacttcttctgttacagactttgccgaagtaacaaggtacatgcacatgatgtgtctgggctcttgggtgatgtttacagcctcgacctccaccttttcaatatttcttagccactcagagaaaagacctggctgctcgctggccacggctgcttgcaaagcccggcagatttgaattttcaggtttaatctctgctcttctggaataccagaaagcaagctttccttagaaagaaggtcccttccctgtacctcctgcactttctttattgccacgggctctcttttagactcaatgatttggtctgggggcatcaccacgttgtcagaatgctcttctttgagcagtacctgcttttcttcaagtgctagtggaaatcttaaggacttgccttcctcaattctgaccgcagaatcttgccctgcattttccagtggatttgcactttctatcaaaattttacctccttctgtgcatgagtgttctgaagggactaggggctcatagtttacctgagagatcatgacatcaggactctggagactctccacgtgtccctcagctaagctctgactcaagatgagcgcactttgtgcctcttgcttttgaagagtcactctttgctctctgttggtgtcagatactgtcttttcttttggtgaaagtacttcctcagccacagaggttagataagaatgcattggaggttctattgaagactgtggataattcccttcaggttcagctaataaagttttcagaggctcaactgttaatgaattaatttgttctatggacatggcacttgggaagattttctcggtatctgatagaactgcctgtgtctcaggctcttcaggcattagaataccttctttggagaaggttttctgggactgtacaatctgcagctgtaggttgggagatggttccttgagaggctgaaagtgaatactgccattgatgcaaagaaattccctggtgctttcaggagtgagcttgtcttgctccaaaatggattgcaattcctgagctcccaaaggaagctgactgctcaattcattggctttagcaatatgctcataagatagttgctggttttcttctgtaattaaagcagctttcaaaatggtgtcttttacaaacgttgcaatttcctgctctgagtcaagtgcttcaactgcgggaccctttaagggtgtctgtggaaaatcctcaggagcctctggtgtggactttgctttgcagggggtatcagtcatgtctgtgtcttccagaagcacaagcagctctgctgcacaggtggactcacccaacatattctctgctttacagatatagaggccactgtcttccctctgagggtcattgacaatgaaagttccagagccattagggttatgaatgatagtgtaataaacactggtgcaaagctgcttgttttctttgaaccatgtaacagtaggggcaggctctccaaccactgtgtactcaaagatggcaggaagcccttgagcacagcgaattggttttaactccttaaggaagtgaggaggacaaggacctcccagcttttccagagattttgccactgctgattctgtttcagtgtctttgtgaccctctcctttggaattaatttttagataggcactacatattgtctttccatagtcattactggccatacatgtatactctccctcatcctccaatttggtgaacagaatgatcaggctatgatcatcaccgtcaaaaacaaatttgtagtcagcagaaggggttaatagcactccattaaagaaccactgaattttaggtttggggatgccaatgacagttacagacagtgtagccacatcccccatgcttatatcagcatttgacacttctttgatgaaaattgggccagtgccttccttttcggaatcaaatttagttgggtaaactggagattcagacaaaagttcaagtgtttcatttattttagataattgaagttcggcgctatgaagtccttcttcctcggcagacagaaaagaactagaaaactctttcatttccatctcaatctcttgttcaatcctctcatgcaaaattgattcaggagcaccttctacacttagtactgctgacgttgtcctctctccacagtcattgtgtacaatgcagctgtatagtccttggtctaccagctgaacattacatatggtaagaaactgaatatttccattttgtgattgtttcagtctctcggattcctctatctttgcaccttcgtgagtccaggttacatcaatgaaagaatcatcttttaaaacacagaggaattgagccgtgtcaccgcactttacagtgacgtcctgaagatgcaggaaaatcttgggcgcctcacccgtggactctttagcacattccttagatagctcagtgctttctgcaatttgtgaaagggatgcagtatggcacaactgtgtatcttgaacagatgcagctgtgtggatggaactttgagatacactttcaaaaacctgcacttcatattcatatgatgatccttgaaatgacttaatttccttttgagatattttgctctcctcctttgtgaaagaggaatctgccactgcctgggacttggtggactctcttacatctttcccagaactttgcctatctagggcttgcacttttggagtcactgtgagtgtagctgcacaagtggcttccccagcactattggctgctttgcaagagtactgcccagcatgctctgagtaagcatcaactataagcattaaagccatgcctgtggactcctcaaaatggaaaactacatcttttgttggtagaattagctgctggttatgaaaccattggatttctggcttgggaatgccagaaaccctcgcatgaaatctgactgtctccccgttgtgcaccctgaggcttgacagaggctggatgaagctgggcttttggccaaggggctccttcttaaatgaaactgataaagagacatgccattgggagtttgatgtattttcttcaaatttgctaaatccttccagactcaggttggctgtgcttgatacttggcctacagcattactagcaacaaacgtgtaagttccttcatcttctggataagcttcggcaatttccagttgataagtgtcttcaaattgagtcattctaaagaaccgagatggcttgattttcttgtctttgctgtaccacgacacttttagatctgttccagaaacccggcattgaaaacgggctggctgcccttcagaagtgacagtgtcctgaagcggggtgatgatggcaggtggataaacaggcatttcctgatcaggagacacaacttctggaacttccactgagagtgaagctgatgttgtggcaacaccatagtcattcttggcttcacaggtatagactgccgcatcctctgggaaggcttcaattagcaaaagcgtgtattcttgcccatcatgaagaaatttgcacttgaagccagtggaaagcagctgctcttccttgtaccaggaaattttgggctgtggtcttccggatatcacggcacagaagcgggcaggcttgccagactgcacagtgacaggctggagctcctgcagaacttggggcggttcaggagcattgacatagagagtgacagaactcctgttccttcctgccacaaaggtgtattctcctgcatcgctctgtctggtctcagagataaacattcggtggattcttctttccactacatatttgtgtcgttcttgaacttggaaattgatttcaatgccatctttataccagtgggcatcaacatcgtcttcattgacctcaaattcaacaacagcacgctgtttctcaatgacctgaacctcctttttaatacttcggatgcgaacatctctgccttctacaaagagttttgcagttgacacgttgcctcctgccaccactgtgtacttcccagcatcagacatccgggtggatgggatcagaaggcggtggacatatttctccttctgaatctttattctgtctgtgatctgcagttcctggtcatctttcatccactgtacagtgatgtcaggttcagaaacttcacattcaaacatggctcgcttcttctccagtaccttaatgtccttaatgtgtttcctaaattctatatgacgagcttccacataaagtgtggctgttgatgttgcttttccagccacaaaggtgtagtcagcagcatccccaaagtgaacattcctgatgttcagtgagtgtgtgagctttttggttctcatctggcacttgtcagttgatttgatttccacaccattctttaaccatttgtaagagatgccttcatagttcactgtcacctcaaaagtaatagtgtctttttcttcagcgttgatgtctttcagcatggaagtaatcatgattggggtgactgtcagggtggcactgacttggtcattgccacagacaaatgtgtattctgccgagtcctctgtgctggtgttcatgatgatcagctgatggagttttccctgcacaactatcttgaacttttcactcatctcaatttccacaccattcttcagccacatggaagggacattgaagtgggacacctcacactcaaaagaggcagttttggtctcaggcacctcgatatttttcatggtttttgtaatatgtaatgtctccacaaacagttttgctttgcattccaattgcccgaccacagctgtgtattccccagcatctgagggggagatgttctgcagcatcagcttgtggactttcctttctgagaccagtctgtgtttgtcacttggcttaatttccacactcttatggaaccattttactggaacagtgtcatgggaaacactaacttcaaaggcaacagtggcattttccaaggctgtcacatcctttggctttttaatgatcttgacagtctccacgtgcagtctggcactggctccaagccttccaagcctgaagccataaacagactcatccacgatggcacagtttttaatcctcagagagtaaattgttcctttgacagagatagcatacttttcattggattccagcacaactccatttttgatccactggacacctttgacattagggtgtgtaagctcgacagtgaaaacagcatcctgtgtttctgtcactgtgaggttcttcagagtcttcttaattttgacagcttcaactttgagtttggcagatgttttggaggtggccaccttgtaggtatattctccaatgtcatctaatttggtggcagcaatgataagtctccttttgtggccatcagactcacttctgatgttgttagtcagtggtaggtgtttgccatccctcaaccattcgcctttggaatctgggttggcaacttcacattcaaacacagcttcctgggattcagctacggtctgatctgtgagtggcttggagatggccccacctgccacagtaagttttccagatgtcatattttctcccgcgtaaaatgtgtattttccttcatcatctttcatcatatttagaactgtcaatttatatatttttccatgtgcttcaattttatatttagaactgggcttgatttccttgtccttaaaattccacaggacatcaattccagagtgggacagctcaacctcaaacaccacattttgagtttctgtacaggtaaggtcacgaagacctctgataattttaattttttctacagagagattacagttggtttcaactctgccaactatcagcttgtaaggtccttcgtctgaagcatgagttcggttaatgactagtcgctgtttagtacctttcacaatggcctgtacacggtcatcaggcttgatttgttcatcatttaagtaccacttaacagaagtcacatcagggactgacaccttacattcaagcacagccttggtgccttcaatcacattaacatcttttagaggtgttatcacgtccacactatagacagagacacgcccactggtggagaggccaagggctggaatggtgaaagagtaatttccagcatcttccttagtcatgtcttcaatgagcagcatatgagattgtttgtctatcacaatgtgaaccctgtcactgggctgcacttcttggccgtctttcatccagacgccttccacactttccaaggagactttaacttcaagctgaacaatgtcaccctcacagactttttggtcactaagtccttgtaggatagcaatggggcggggtttcatctttaatttacaggttgtctttttcccgtcgatgacaaagctgtattctccctggtcctccttggttacatccttgaccgtgaggttctgacgtccacgacgagatgtaattgtatatttgccattggatttaagctccacatcattatgataccattttccttctatattttctggggatacaatgcactctaattctcctgaatatgattctggaacttctatgtcctgaagttctttcacaaactcaacaactgcaccttcaacaataagtttagcagtcgttttgacattttcatcttccacaagtacacagctgtaatcttcagcatcagacgtatcaatggtcagtatggagaggaagtgaacctttctgtcagagtgcatcctgtatttatctccctcatgaacctccataccatctttataccatttcactttgacaaatggttctgaagtttcacattcaaaggttgccatagtgtctttttccttagcaacaacatcttgtaattcctgtgtgaaagtgatcaattgcttggcttggacaagtaagaatgcgtgactggaggtttctccagctatgttgatggcttttaccatgatgctggcagagtcctcagcagtcacatctcttatgaccaattcacaaacattgtcttcgggccagtaccagtagatccggtcagaccgttcaattttgacaccatttttgtaccattcacattcggggtctggtttccccacgactctgacccggaagtgtgcatcagatccttggcccactgtttggctctggattctttcgaagatttttggagcctccatactaggacttagttcaatcttgtcaggtttaaaagttggaatcgtgattttgccttcttcggcaagagctttcttttcctcttcagttaactctttggtccagtggagaagttcatcttttgtcttcctgaggagttcctcataggattcatccttctttcgagacttgagctccacagcggtaatggcttcataatagccctcttctgttctgcgcttgaatttactgcgcagctcttccgactcttcaggcactttttcatgggtaattctttcagcccttttcaacttcacaacttctttggtttcagtggtgtcaacaggtctatccactttttgtacttcaaactgaagctttcctggttcatgtacgtgaaactcaggccttggttcaggagctctcctaaggacagacctaaaatcttccctctgttgaatctcaagcttcactttatgctctatcacaccttcaggattttccgcggtgaccttcacttcacctgtgtcatatgatttgcagtccacgatgtccaggtaatggataccatcatagcgaactctgaaccttttgcttttgcggatgagctgtccattgaggtaccagttgactttgggctgagggtagcctgttaccctgcagcggaaccttgcagtctccccttcaagtactctaactggctctgggtacaagacaatgtctggcttttgcttttctttctgatctgttgttacacctgtaagtgcaccttcatgagccattctctctaattcttcaattctctgtaagcctttcctcccctcaggcaattgggattcttccacaagacttttctcatctttaacaataagggtagcagatgtgtgatctgttccatatttgttagtggctctgcaagtaatgataccactgtctctagaatatgcaacgccataatcaaggctgcagtacccaaattcattgatcatacggagcctgttggctgcttcaagtggctttccatcatggagccactccaccaccatcgttgggtcaccaatgggtgttagcctgcattcaaagtgggcaggcccaaagcgcttaagtcttaaggaagtgagttttttcttgaaaaatggtttctgttgtttctctttgtcatagagatcaccttcttcccattgctcttggccatatcgcaaatggaggggctccagttctggggctgcaatctcctttgctctatatgtcccccgtgggatgattaactttctctctggctcaggctctgcaaactcaacttcaacatttactttgcatcttgtagtgtctctgccagctttattaatagcagtcgcagtataccaggcagaatcttggctgacagtggaatcgattttaagggcagcttctcccttggttccttcaattctgattttgggatatttatgaggcacaatgatgtcactgtttttcaaccatacaatgtcagggttggggttacccgtagctctgactttcatttcaagtcgggaaccttcctttatattgacatttttcagtttttctacaaacatcggttttacctgatgttccacagcttccacagttaaaatcactgaaattgaagatctgcctgccctgttttgggcaaccacagtccattccccagaatcactgggtgtggcagggacaataattagtgattgagtaccatcttctttaatgactactttatgggtatagtcattgacaatttgctggccatcatgaaaccagaacgtctctggcataggtctaccaacaacctttaagtcaaatctggcagtttgcccttctaaacatttgaaagaaacaggttttaacacaaagactggtttatatagtctctcaagttgtgactcatctgtctcctccagcctacgtccaggggacattcttgcaggggacatccgtgcaggagacatccttgcaggtgacatccgtgcaggagacatgcgtataggagacctgctcactgaacgtggagagagagatctgattctgctcactggctctagtgtgggaatgtaagtcggagctccaagtggtgcagcaggctccacatacaatttccctgagcaaattgcatttcctttaatattgctggcaaatgcagtgtagattccttcatcttctggaagaacaacaggtatacgcagactagctctgccatcttgtagaaagtccatttggtatctttctccatgtttgatgcgcttgccatctttgtaccaagcaatctttggtaatggatatccagacatcttgcaatgaaaagtgacacccatcccctcaagaattctataattcttgattcttgaatcaaatcctgattcaacagcttcagattcagaaatgtcaactgccatcttttcttctccatcttcttcaagaagttcttctaatgtagtctttattattctatattcaatttctttaataagtctctcttcaaaggaagaaatatggaattcctgatcttctacataagttctgaccactacagtatctttggccattttcttcctaattaaggcttgttctttttcatactctttttcatactcagagtatacaaatccaggtgctgtttctccaactttaggttcttgaacaaatgcagtcacttgtgtctgataaagcatttcttgctgggacttcatcagtaactcataatcagcttcttcaagcaaggaagcagatgcagaagtttctccatgcttattgcgaacaacaatagtgtattctccagcatcatcagcaaaagtcatagaaatcaccagcttgcattcaccggtttgtttgttgtaactcactttgtatctgtatccagtggttagaggaacaccagattttttccagtatacatggggctttgggttgccgccaacttggcatccaaacaccacgctcccaccttccaccagtttctggaccactggttttgtaataaagtaaggcgcggcaggttctccaggccctgcttgttcctctgtgaggctagtatcagtcataaccacatctcttgactcaacaaagcgtttctcttctgtagtaaatttctcagtcacggctgtggtttccttttcaaattcttctgacacctgcacagccagatagcaggatgtgctgacggttccagcctcatttacagcactgcaagtaaatcgcccgctgtcttccgcaaatgcttcgcgaatcataagacgagcaattccactctggaaggttatctggaagtcaatggaactttcgatttggtagtcttccctgtaccatgtcactgtcggggatgggtatccagagatgtggcactccaaggtgacagattcaccttctatgacagtcacattttttaagcccgagaccaaagttggtggagtaacaggaatttcaacaggtgctggtactcttgctgtttctgttaccttggcttcgcgtccgtgcagtacttcaaagcgctcttcacggacggtggtgccagtgatgctcacccctacttcctttttcacctcaacgccagcttcactcttgtaagtatctggtgtgtcagcgaaggggaactgtggcaagggtgtgggctctgcccttactctagtctcactgggcttcacagtaggagccttcaccgatttggtgatcttctgagcagaagatgtggctgacaactctttttgtaatgtggcaatagcactaccggctattgatgcctcatatccatgttctgtcttaggaacagaaatttttgaaacagtaaagtgagggctagctgtgcgggggcgtttatccacatggactaatctttccgttgttagatctgtagttttcttgatctgtgatgatatgtgcattcccttttgatcagtagttttgatatgagtctcagaaggagcctggattactctaggcttgactgctttagggacaacgtggggttctgaggctggacgttggggaggctcagctacctttgcggcggaaatgcgttccttatatccgtactccaaagtggtctgctgagcataggattcttcaagatgcccaggctctctgggctctctgactcgggcctggtctactgcagcaacaactgttgctacagcttcagccttttttccaacgtccacctttccatgggtaacttggatttgttcttgtctagtagccatagtttctctagttctcagtattgtttcttgttctttggctttagcagtagcaactgctattgtagacaaggcagttttctcggcttcctttctcatcttctcctgagttatttgcacttgttctcttttggtagtaatgccttctctacctcttgatactaaatcttgttctttgactttgggtgtggcaactatgactttaggtacaactgttttcctagtttccttcattatcttttcataacttaggtgcatttgatcttgttgtgtggtagtttcttcttgagctcccgggactgtttctagttttgtggactttgcagtggcaactaccaccatggatgcagcagttatctcagtttcctgtcttattgcttcttgagttacttgtttctgtttcttagtaatttcttcagaaattctagtttcttgttctttggctttagctgcggaaattactacctttggtacaaatgttttttcagtttcttttcttatctgctcatgagttacgtgcatctgctcttgctttgtggtaattacttctttggttcttgattttaattcttgttccttggctttatcggcggccactactaccttagttacagcagtcttctccgcttcctttcttacctgttcttgagcaggttggatgtgcacagcagtcgtggttgtcctctgagcagtctgctctacagcgctgatcactggttctctcactctggccatatcaacggcagcaacaacagtcgcaacagctgcacttttgtcagcatcttgtttcacctctttagcaccagtggcaacagcctctgctgcgtagctagcactggccgacacactggcggcagcacccgcagcaccactgatggtcacttgctcctggacaccgtatctcccttcccatctctcttctgtcctgatctgagtagaggttgtcagcgttgtctctctcatctcagcctcagatgaggaggccacgtagccctcttgcttccaagggggaggcacttcaggacctgtggccacggtggatgcctgagtcttacgcatgagcaatggagacctaacagacctgatgggggatgtggagattcttgctgctggagacacggacctgaccggagatggggtcggtgcccgcacgtgtctgaccggggaaggggagtgtcttatgggcgatggggactgctgccgagccagctgtgctttggcagcaatagacggtggtgttggggatcttgactttggcttcggaggaatcctgggaggtgttttatgtggcagctgttgcccagcggcaccatctatgaccatctcaactgttgcaattgatctggcatcaaagtgggcttcaatcttcttttcaattcgggtttgtcttgattctgagatctgagcagtcgaaacaattgtctttgtctttttagcaggtacttcttcttcaccttgaaccagtaattcagcagtcgaagtagctcttccaacgctattggtggcatttactgaataggtccctgagtcctcagggtatgcttctgcaatcagtaagctgtagaggtcgccttcttgtgaaatttggaaatcaagggagctctggatttcggctccatcccggtagaacttcaccacaggtgtagggattccagtcactctcacttggagtctcacttggcttccttgtctcacggtcatgctctgcagtcgttgaacgaagttgggtggtgctgtctcagctttcacgagaagctcagcagtactagtcgcttgtccagatccattggtggctttcagggaatatcgtccactgttggctttagtcacggcggggatcgtcagtttagcgcggccatcgctaaaggagatctgcacgccgggcagagtggaagtggaaatcacctggccatccctaaaccagctcacctcaggaactggaaaaccactaatgtgagcctcaaaggttgcggtactaccctccagtaccacaacgctttgtaacggctgcgtaaacgtcggtgcttgagttgtcatctttctaggcactctgatttctcaagagtgcctaaaaagggtgggactaagcccaaggttgcttctgaaacgacgtcctatggagagttggtttttctgaccatctccgacatgaatcggtgagcctctaatcctaaaaacaaaactacacagtcaagactgtgtagttttgcttttctatgcaatccctacacccgaggcgaggctgggaatgcacgactgctc

SEQ ID NO: 9835 - RNA, 23201 nt, Homo sapiens
  source 1..23201: mol_type = other RNA
caaaaactgcagttacttttgccaacactgtttttcacttcaaagctatataatcctttgtcactcatttcggcacaggggattttaagggaagccactttattgatgaatgtaatgtgatgtttgctgtctgcagacaattctcttccatctttgaaccacttggctgagagttctggtgttccagtcactacacactctaatgcaaaaggatttccagtagtgacagtcatgggttcgggcttctctatgattcttgctggttctagtacagtcaagactgcagagcattctctcattccagcatcgtttttgatttggcatatatattttccagaattagatgcttctggactccccagctggagggttgcaatgttatcaatgaatgaaatcctggtattttcactctctctgatgacttcacctctatctttcagccagacaacagaaattggctggaagccctccactatggcccgtaactcaacagcatccccaataagggttgaggtgtcacttagctttttcacgaatcgtggaggttctttgaacttgacagagcaagaacacgtgtcacttcccacctcattagtagctttgcagtgatattccccgacatcggaggcttcaagattaaggatatgaagacttgtatcaaaatgttttgaagtgattttaaatttcttgctgtttctaacctgctttcgatctttaacccatactacttcaaatgggggagttcccgaaatttcacattggagaatcacatcagaacctttaagagctcctactggagaaggcttctgggtgaaaacaggaggtgctttcactgtcaacgctgtgctgcagctggcgtcaccaacaccattatgagcctcacaaatgtagtccccgctgtcttcagcactagcttcattgatcgtaagcaatgccacagaattaatgaatgacatgttgtatttccaactttcatgaagttcgctgtcatttcggaaccatgaaactttgatttctggggagccacttattttacattccagttgaatggattctccctgctttgcaacttttgaagcttctaatttcttaacaaactttggaggttcttttacactgagctgagctgagcacatgtctttgccaacatcattggttgcttggcaagtatattgaccagagtctcctttgcctactttaagaattctcaaatgaggagtgtttcccacacatgtgattgtatagtttcctccaggacggatctccttgttatcttttgaccaagtgattcgcatcggttgagcaccagtaacatgacactcaaaatcagcactttctccagcaataacatctatagatacaggcttgatgtcaaagaagggagatttcttgggttctcttgctgtgagtctagcactagaagatgctgttccaagtgggttggaagctgagcaagagtactggccagagtgactcaagtcagtttgcaaaatttttaaagttgccacattatctacaaatgaagtctgtagattttcatcgtctcttaaaagtactccatctctataccagcacacttggatgggtgcagagccatttaatcgacaagtgagtgtaacaggtaaccccacagtttgttcaatgtcctttaattgtcttgcaaaagaaggtgggagttggcgctcttgaattctgaacacagtcttagaagaagcagttcctatactattttctgctttgcatgtgtactctccactgtcattgatgttcactttattaaaaacaagtgtggccacattgtttgtaaagtaggtcctgtattcaggagttggccgtaatttggtatctcctttgtaccaagacactgtaatttctggtgtcccagcaacttggcattgtaaagaaaccgaatctccaactgctgcctccagaggttccagttccgtaacaaaataaggcggttctaatgtagataccagagctccacaaacatcccttcctgcctcattttcaatctcgcaggaatactgccctgcatctctttttgtgctattcagaatttccaggatacaagttttctctgttgtgactatgttacatttttcagaggtagttatgttaaaaccatcctttttccaagtgacagaaattggaagtgttccagtgtaggtgctctccagaattatggacttccctggttctacagaatgatcacttaatctcttcaaaaatgcagctggttctttcacaaagagacgggtagtgcaagatgcttggccagcgttgttagaaaccacacaggtgtattccccactctgagatatgtcaatattaaataattccagttctgccacagtgtcttcaaaatagatgttgcaccggtctcctttcactagttctctggcacctctgaaccagttgactttgaatggaggggttcctctaataacgcttgtgaaggttacatttttgcctggtagtacttccaaaggttcaggttctttcacaaaagagggtggttcttgtacagttagcactgcacgacattcatcagacccagcgacattagcagccacgcatgtgtaattgcccatatctgaggaatccagagaattcaactgcaatgtgcagacattatctgaaaatgtggtttggtactttgctccactgacaatcttggttttctcatgaaaccaggcaactgaaataggtgatgatccagctactttgcattccaagatgcaagaagcacctaacaccccaccagtatttttcagtcttcgtgtgaaagagggaggaactgctcggtctgaaacatcaaccacagctgtgcagctgcttttcccaacattattttgaacctggaaagtgtatgtgcctgcatcttgcctttcaactgagagaatccttaaggaagagattttgttgtagaagctaaatttgtgtttttggctgctggtcaacagctttccatccttgtaccattcaacagagagttccggagtgccagccaccttacactccagagtgcacgtttctcctacagtcaccgtcatcggtcctgccttctcaacaatgactgcgggctctaagaccatcagtgtggccatgttctccctcattccaccatcattcttgatttggcagatatactttccagcattagctggctctgcttttgcaaactgtagagttgcaacattttccacaaatgtaatcctgatgttttcactttctctaatcacttcttccttctctttaagccactggacaaaaataggctgggcgccttctatggatgcttgtaattcagcaggctctccggctacaacagtgaggctgttcagtttggagacaaatcttggtggttctttcaattttacagtacaaacacaagtatcacttcccacttcattctgtgctttgcagtggtattcaccgatgtctgaagtgtccacattgagaatgtgaatacttgtgtggaagtttttggatgcaatcttgtatttcttgctgcttctgagttgccgcttgtctttgtaccataccacctcaaacggtggtgttcccgaaagttcacattcaagactgacttcagcatttttaagggtttctactataggagggaagctgctaaaaacaggtggctcttttactataaccttggtactgcagcttgtgctgccagcgggattctgagcctcacaaatgaaatctccactgtcctcagtactgagattgttcatctgtatgacggccactgagtcaatgaaagtcattctgtacttatcactggctggaagttcatgttcatttcggaaccacacaactctgatttctggggatccagctatcttgcattcaagtcgtgaagagtcacctgctttcacaattttggaggcttctaatttctttacaaactttggtggttctgtcacaagcaacatcgtagtacaagagtcgctaccaacatcattggtaacatggcaagtatactgtccagtcttagaagcatccactgagtagagatttaagaagctagtcgacccttccaagccaatgaaacatttaggacctgagacaagttccacatcatccttaaaccattttattttaaatggtggtgttccttttagtattgccttaaattccactgtagaatcaggtatggcttgctgtcgcccaggtttcactaggaagcttggtggttctttcacagttaagatgccactgcatgcatcatctcctgctacatttgacactttgcatgtgtaatttgcagtatcttctaattccagattattaacttccagagacacagatctctcatggcacacaagtctgtattttgcacttgtagatatttcttttccatccttaaaccactgagcactaatgggaagtgaaccagacaccttgcactccatatgaatagaagagcccagaactttatccattttggttaattttttggtgaatgatggaggaatattttgatctagcactcttaagtaggcatcacagctactgcttccgaagtcattttccaccttgaaagtgtactgaccgctgtcctgcttcattactgactgaattctaaaactggccacgttattttcaaaactcattgaaaagtatctactgggaactatttgtttcccgtctttaagccatttcactttgagttctggtgttccagccacaacacattccaaggtcatgggatctttctccgtaacatcaactgatttagctttctctacgatttgagctggttcttgtactaaaaggaaagcataacacctctcaactcctgactcattcttggcttgacaggtatatctcccactgtgtccattatccacacttctgatttgaagtgtggccacactgtccacaaatgaaatatagacattatcatcttcatcaagaatctgatcatcctttagccaggttatagaaataggaggagaacctgccacggtactctgaaaggtggcagaacttttcaaaacagtagtggtattttctatcttcttaatgaatgatggtggttctttcagggcaactctagtactgcatgagcagctgccgccttcattggatacaatgcactggtattccccagtgtctgaagggtcacacttggttatatggaggttaaacacagacactctgtcggtcaatgtgtattttttgctgcttcgaatttccctgttattcttcagccaagtgacttcaaacggaggtgttcccgtaacttcacactccagctccacgtcactatattttactacctccacaggcttcagctctctgataaaggtggggggttctttcactttgagttcaatgctgcagctcgccgtgcctgcgtcatttcgagcttcacacacataagtcccactattttctaccctggcaccagaaatctggaaagtggctaaaccatcaatgaaggaaatgccatgtttctgaatggctgttatttcattcccgtctagataccaagacactcggattttaggagtgcctgttatttggcattcaaatgttgttgactgtccattcctcagcactaagactggactgggcttcttaatgaattgaggaggttcttttacaaagagagtggctttgctggttgctgtgccaacatcattgcttagttggcaaatgtaggttccagaatcggtagctttggctgcaaagagctctagactggtagaggtgtcatccttccaaactgagcgggctgctcctgagtgtaactctttgttatctttaaaccactttattgtcatgggtgcagtgccacccacaagagcctttaactgtacccttgtgttgggattgacatcttgtgactgtggcttttccacaaagtaagggggttctttgactgtcagatgcccactgcattggttgtgccctgccttatttgtggcagaacaagtgtatgtcccactgtctgtaccttccagctggctgatttccaagaaggcagtattgtcatgaaaagagaatttgtacttttcactagctgatatttcttggtcatctttgaaccactggatgcttatgggatgtgacccagccactatacattctaaatcaatgaaagaacctttaatgctgtccattttcttcagctttttggtgaatgaaggaggtatgataagatctaatacattaattctagccttgcagctgctcctcccaacatcattttggacctcgaaagtatattctccactatctttcttttctgtagaaataatcttcagtattgagactgtatcagtgacactgattttatattttgagcccagggtcagttcttggccatctttaaaccatttggctgtaatctccttagtccctgaaaatttaacctgcaaagtggctgggtctccttgggtgacatctatagacacagcttcctcggtgattgttgcaggttcttttactgagagtaatgcagaacatctttgtattcctgcatcatttttggcctgacagacatatttcccatcatgcttgacttcaatgccactgaggtacaaactggccacattgttctcaaaggtcattcttatattatcgtcttcagtgatttcatcgctgtcttttagccaagtcaccgtaattggcaaggagcccttcagagtggcctggaaggcagctgtgcctccccggagggagctggtactctcgatcttctttatgaaggatgggggttctcttaaagtcaccctggcactgcagatgctgctgcccacctcattggtcacccgacactggtattcgccagcatctgcagctacaaacttgaggatctgcaggctaaccagatgatcctgaatgaaagtcttatactttctaccacttcgcaggattgtgttatctttgaaccaagtgatctcaaagggaggagtgcctgccacctcagccagcaacatgacatcgtactcctttaagacttcaattggcttaaattccttggtaaaataaggtgactctttgactattacaatgctactgcagtggtcactgccagcctcattttgggcctcacacatatattcaccactgtcttcgatgccaacatctgtcagtcttagaactgcagtagactccacaaaagacattctgtgtttgctgctctccttaatttctctatcatttgcaaaccatgttattttaattggaggggtaccagttactttgcaggctagctgggtggcatctcccttctttaacagctgtgatggctctaacttttcaacaaatgtggcaggttcttttacaaacaagtttgcactgcattccacccctccagcgacattgctgactttacatgtgtacgtgcccgaatcagaggtttttactaaatagagttccagggaactctctaaagcttctttggtaatatagcagcttccaccagaaaccagctctttgttgcccttaaaccatctgattgtgagaggagtagatccttggaaagtgctcttcaggcagactgctgagccaggcagaacatcctttgagccgggtttagttacaaaactgggtggttcttgcacaatcagggctccactgctgtctttgcttcccacggaatttgtggctcgacaagtgaaattccctgcatcattcatgtctactctgatgatctccaaagaggctgtgccttccacaaatgctatcctgtatctgtcagaagcagctatttctttgccatccttaaaccaggacaccctcatggggagggagcctgcaattttgcagtccagtctgcaggtaccattaacaacactatccacgttgcgcaagggtttggtaaaaaatggagcaatgtctcgatctaatacagtgaatgtagtctcacaggagctgctgcccacttcattggaaatctcaaatgtgtattggccactgtcgtgcagctcagctgaataaaatttgagctgggcaacattgtttttaaaacttattcggtattttttactggcgaccaagggtctcccatctttgtaccatttgggcttcagttctggcgtgcctgccactgtgtactccagtgtggcgggatctcctgctgtcacctggatcagttctgctcgctcaatgattttggcaggttctttaactattaattccccaacagatgtttggcttccagcttcattttcagccaggcacgtgtatttgcctccaaaactaatctgaacatcagggattatcaagactgcaacaccattggaaaagctcattttgatttttccgtcttctctgatgacctcttgacctttcatccatgtgacagaaatgggctctgaccctctcacagcagcttgcagggtaacggtttgtcctcctagtgcaatcaaatcatctactttctttacaaaggttggaggttctttgagtaagtgggttgccatgcagccacacttgccgacttcattagcaacaacacattcatattcaccaacatctgcactattaaacgaaaagatctccagacacacaagagacttctgagaaaacaatctgtattttttactacttcgaatttgtttcttgtctttgaaccagctaatttcaaatggtccagtgcctgagacttcacactgaagtagagcatttgttcctctcactatgtctgcaggctcaagagttttgatgaaagaaggaggttctttgataactatttcagtactgcagctatcactgccgacgtcattcactgcttcacatgagtaactcccactgtcttcaacttttacatccgtaatatcaagtatagcctcagaattgacaaaatacattcggactgtgttactttcactgagttctttgttatttttaaaccaagtaacctggatcacaggtgagcctttcagcttgcaatggaggcgtgctgattcacctgggagcattaaataagagggatccaccttcttcacgaaggatggtggctctctgacagtgactgtggctgagcaggagctgcttccagcctcatttgaagctgtacagacataggttcctgaatctttcagtttggccaaaggaatctcaagtgttgctattttatcttcaaaacagatcttataatctttccctggggggagtttttgcccatctttgctccacgtaactgtgacttttctgtcttcatctacttggcactcaaggtggaccttcttattgatagcggactgcacaggctctaattctttaatgaaatgtggcttatcaatgatgatcaactctgcttggcagatgtctgctccaaacttgttggaagccttacaagaataaactcctctatcttgaatggtaaggtttgagagttctaaaatgtgtttgttttctgcgtcggaaatcctccagttaggtgaaggtgagagtgcagcaccatctttctgccaaatggtttctatcacaggagtccctgtcactgtgcagatgaacttggctgccttacccacaaaagttgtaagggacttaggtctggagagaaaggttggtggatatgcctctgtcacagttagtgtggctgtacagctgacactgccatactcattggaagctttgcatgtatactcgccgcagtcaaccacctgggttctcaggatttcaaggctggagatatactttgaagatcgaatagaacacttgtcactctcataaatttctcggccagctttaaaccactggaaccggacattgggagcactttggatctcacaggtgaatttggctaggtggcccagtgctacttccaggggttcgattttcctcttgatcactggggcagctctttttactacagtgagtttggctgaagttgctgtttttccgctgtcattcaaggcctcacagacatactctccttgatggtcttcggtatttactttgtcgatgactagcgtatatgtattttgatcttgtaaacacttgaacttttcatctgaaggcaccagtttattctcaaaataccaattcacctctttagcatttgttatggatgttgtgaggtgtacaatatcaccttcctcagaaacagtgtccactaaaggtgtatgtatcatggggccatcctctttgattaagccaccctcagcttcctgtatctttactgtagcaacctcctcagtaccactttcagaggaagactcctctttttcctctgatggtttcagactctcatcttgtttttcgtcagagacaacagctgaagcaacccctttagtgacaggtgtggcatccaaatatttaaccctactttgcacgttaaaataactgacctcttcagttgagatcagatatttagattcaacttctggttcagtaatgggttcaaccttctgtgaacctgaaaaagaatccatttcttcttgcaaacttgttttggctccttgctgaattctaggaccctcagctgttaggatgtctatttcctcatatataatagcacacaaagcatccctaagttccattttcaggttagccatttgaggatcaacatcttcaataatgatggttacttcttctgttacagactttgccgaagtaacaaggtacatgcacatgatgtgtctgggctcttgggtgatgtttacagcctcgacctccaccttttcaatatttcttagccactcagagaaaagacctggctgctcgctggccacggctgcttgcaaagcccggcagatttgaattttcaggtttaatctctgctcttctggaataccagaaagcaagctttccttagaaagaaggtcccttccctgtacctcctgcactttctttattgccacgggctctcttttagactcaatgatttggtctgggggcatcaccacgttgtcagaatgctcttctttgagcagtacctgcttttcttcaagtgctagtggaaatcttaaggacttgccttcctcaattctgaccgcagaatcttgccctgcattttccagtggatttgcactttctatcaaaattttacctccttctgtgcatgagtgttctgaagggactaggggctcatagtttacctgagagatcatgacatcaggactctggagactctccacgtgtccctcagctaagctctgactcaagatgagcgcactttgtgcctcttgcttttgaagagtcactctttgctctctgttggtgtcagatactgtcttttcttttggtgaaagtacttcctcagccacagaggttagataagaatgcattggaggttctattgaagactgtggataattcccttcaggttcagctaataaagttttcagaggctcaactgttaatgaattaatttgttctatggacatggcacttgggaagattttctcggtatctgatagaactgcctgtgtctcaggctcttcaggcattagaataccttctttggagaaggttttctgggactgtacaatctgcagctgtaggttgggagatggttccttgagaggctgaaagtgaatactgccattgatgcaaagaaattccctggtgctttcaggagtgagcttgtcttgctccaaaatggattgcaattcctgagctcccaaaggaagctgactgctcaattcattggctttagcaatatgctcataagatagttgctggttttcttctgtaattaaagcagctttcaaaatggtgtcttttacaaacgttgcaatttcctgctctgagtcaagtgcttcaactgcgggaccctttaagggtgtctgtggaaaatcctcaggagcctctggtgtggactttgctttgcagggggtatcagtcatgtctgtgtcttccagaagcacaagcagctctgctgcacaggtggactcacccaacatattctctgctttacagatatagaggccactgtcttccctctgagggtcattgacaatgaaagttccagagccattagggttatgaatgatagtgtaataaacactggtgcaaagctgcttgttttctttgaaccatgtaacagtaggggcaggctctccaaccactgtgtactcaaagatggcaggaagcccttgagcacagcgaattggttttaactccttaaggaagtgaggaggacaaggacctcccagcttttccagagattttgccactgctgattctgtttcagtgtctttgtgaccctctcctttggaattaatttttagataggcactacatattgtctttccatagtcattactggccatacatgtatactctccctcatcctccaatttggtgaacagaatgatcaggctatgatcatcaccgtcaaaaacaaatttgtagtcagcagaaggggttaatagcactccattaaagaaccactgaattttaggtttggggatgccaatgacagttacagacagtgtagccacatcccccatgcttatatcagcatttgacacttctttgatgaaaattgggccagtgccttccttttcggaatcaaatttagttgggtaaactggagattcagacaaaagttcaagtgtttcatttattttagataattgaagttcggcgctatgaagtccttcttcctcggcagacagaaaagaactagaaaactctttcatttccatctcaatctcttgttcaatcctctcatgcaaaattgattcaggagcttccagactcaggttggctgtgcttgatacttggcctacagcattactagcaacaaacgtgtaagttccttcatcttctggataagcttcggcaatttccagttgataagtgtcttcaaattgagtcattctaaagaaccgagatggcttgattttcttgtctttgctgtaccacgacacttttagatctgttccagaaacccggcattgaaaacgggctggctgcccttcagaagtgacagtgtcctgaagcggggtgatgatggcaggtggataaacaggcatttcctgatcaggagacacaacttctggaacttccactgagagtgaagctgatgttgtggcaacaccatagtcattcttggcttcacaggtatagactgccgcatcctctgggaaggcttcaattagcaaaagcgtgtattcttgcccatcatgaagaaatttgcacttgaagccagtggaaagcagctgctcttccttgtaccaggaaattttgggctgtggtcttccggatatcacggcacagaagcgggcaggcttgccagactgcacagtgacaggctggagctcctgcagaacttggggcggttcaggagcattgacatagagagtgacagaactcctgttccttcctgccacaaaggtgtattctcctgcatcgctctgtctggtctcagagataaacattcggtggattcttctttccactacatatttgtgtcgttcttgaacttggaaattgatttcaatgccatctttataccagtgggcatcaacatcgtcttcattgacctcaaattcaacaacagcacgctgtttctcaatgacctgaacctcctttttaatacttcggatgcgaacatctctgccttctacaaagagttttgcagttgacacgttgcctcctgccaccactgtgtacttcccagcatcagacatccgggtggatgggatcagaaggcggtggacatatttctccttctgaatctttattctgtctgtgatctgcagttcctggtcatctttcatccactgtacagtgatgtcaggttcagaaacttcacattcaaacatggctcgcttcttctccagtaccttaatgtccttaatgtgtttcctaaattctatatgacgagcttccacataaagtgtggctgttgatgttgcttttccagccacaaaggtgtagtcagcagcatccccaaagtgaacattcctgatgttcagtgagtgtgtgagctttttggttctcatctggcacttgtcagttgatttgatttccacaccattctttaaccatttgtaagagatgccttcatagttcactgtcacctcaaaagtaatagtgtctttttcttcagcgttgatgtctttcagcatggaagtaatcatgattggggtgactgtcagggtggcactgacttggtcattgccacagacaaatgtgtattctgccgagtcctctgtgctggtgttcatgatgatcagctgatggagttttccctgcacaactatcttgaacttttcactcatctcaatttccacaccattcttcagccacatggaagggacattgaagtgggacacctcacactcaaaagaggcagttttggtctcaggcacctcgatatttttcatggtttttgtaatatgtaatgtctccacaaacagttttgctttgcattccaattgcccgaccacagctgtgtattccccagcatctgagggggagatgttctgcagcatcagcttgtggactttcctttctgagaccagtctgtgtttgtcacttggcttaatttccacactcttatggaaccattttactggaacagtgtcatgggaaacactaacttcaaaggcaacagtggcattttccaaggctgtcacatcctttggctttttaatgatcttgacagtctccacgtgcagtctggcactggctccaagccttccaagcctgaagccataaacagactcatccacgatggcacagtttttaatcctcagagagtaaattgttcctttgacagagatagcatacttttcattggattccagcacaactccatttttgatccactggacacctttgacattagggtgtgtaagctcgacagtgaaaacagcatcctgtgtttctgtcactgtgaggttcttcagagtcttcttaattttgacagcttcaactttgagtttggcagatgttttggaggtggccaccttgtaggtatattctccaatgtcatctaatttggtggcagcaatgataagtctccttttgtggccatcagactcacttctgatgttgttagtcagtggtaggtgtttgccatccctcaaccattcgcctttggaatctgggttggcaacttcacattcaaacacagcttcctgggattcagctacggtctgatctgtgagtggcttggagatggccccacctgccacagtaagttttccagatgtcatattttctcccgcgtaaaatgtgtattttccttcatcatctttcatcatatttagaactgtcaatttatatatttttccatgtgcttcaattttatatttagaactgggcttgatttccttgtccttaaaattccacaggacatcaattccagagtgggacagctcaacctcaaacaccacattttgagtttctgtacaggtaaggtcacgaagacctctgataattttaattttttctacagagagattacagttggtttcaactctgccaactatcagcttgtaaggtccttcgtctgaagcatgagttcggttaatgactagtcgctgtttagtacctttcacaatggcctgtacacggtcatcaggcttgatttgttcatcatttaagtaccacttaacagaagtcacatcagggactgacaccttacattcaagcacagccttggtgccttcaatcacattaacatcttttagaggtgttatcacgtccacactatagacagagacacgcccactggtggagaggccaagggctggaatggtgaaagagtaatttccagcatcttccttagtcatgtcttcaatgagcagcatatgagattgtttgtctatcacaatgtgaaccctgtcactgggctgcacttcttggccgtctttcatccagacgccttccacactttccaaggagactttaacttcaagctgaacaatgtcaccctcacagactttttggtcactaagtccttgtaggatagcaatggggcggggtttcatctttaatttacaggttgtctttttcccgtcgatgacaaagctgtattctccctggtcctccttggttacatccttgaccgtgaggttctgacgtccacgacgagatgtaattgtatatttgccattggatttaagctccacatcattatgataccattttccttctatattttctggggatacaatgcactctaattctcctgaatatgattctggaacttctatgtcctgaagttctttcacaaactcaacaactgcaccttcaacaataagtttagcagtcgttttgacattttcatcttccacaagtacacagctgtaatcttcagcatcagacgtatcaatggtcagtatggagaggaagtgaacctttctgtcagagtgcatcctgtatttatctccctcatgaacctccataccatctttataccatttcactttgacaaatggttctgaagtttcacattcaaaggttgccatagtgtctttttccttagcaacaacatcttgtaattcctgtgtgaaagtgatcaattgcttggcttggacaagtaagaatgcgtgactggaggtttctccagctatgttgatggcttttaccatgatgctggcagagtcctcagcagtcacatctcttatgaccaattcacaaacattgtcttcgggccagtaccagtagatccggtcagaccgttcaattttgacaccatttttgtaccattcacattcggggtctggtttccccacgactctgacccggaagtgtgcatcagatccttggcccactgtttggctctggattctttcgaagatttttggagcctccatactaggacttagttcaatcttgtcaggtttaaaagttggaatcgtgattttgccttcttcggcaagagctttcttttcctcttcagttaactctttggtccagtggagaagttcatcttttgtcttcctgaggagttcctcataggattcatccttctttcgagacttgagctccacagcggtaatggcttcataatagccctcttctgttctgcgcttgaatttactgcgcagctcttccgactcttcaggcactttttcatgggtaattctttcagcccttttcaacttcacaacttctttggtttcagtggtgtcaacaggtctatccactttttgtacttcaaactgaagctttcctggttcatgtacgtgaaactcaggccttggttcaggagctctcctaaggacagacctaaaatcttccctctgttgaatctcaagcttcactttatgctctatcacaccttcaggattttccgcggtgaccttcacttcacctgtgtcatatgatttgcagtccacgatgtccaggtaatggataccatcatagcgaactctgaaccttttgcttttgcggatgagctgtccattgaggtaccagttgactttgggctgagggtagcctgttaccctgcagcggaaccttgcagtctccccttcaagtactctaactggctctgggtacaagacaatgtctggcttttgcttttctttctgatctgttgttacacctgtaagtgcaccttcatgagccattctctctaattcttcaattctctgtaagcctttcctcccctcaggcaattgggattcttccacaagacttttctcatctttaacaataagggtagcagatgtgtgatctgttccatatttgttagtggctctgcaagtaatgataccactgtctctagaatatgcaacgccataatcaaggctgcagtacccaaattcattgatcatacggagcctgttggctgcttcaagtggctttccatcatggagccactccaccaccatcgttgggtcaccaatgggtgttagcctgcattcaaagtgggcaggcccaaagcgcttaagtcttaaggaagtgagttttttcttgaaaaatggtttctgttgtttctctttgtcatagagatcaccttcttcccattgctcttggccatatcgcaaatggaggggctccagttctggggctgcaatctcctttgctctatatgtcccccgtgggatgattaactttctctctggctcaggctctgcaaactcaacttcaacatttactttgcatcttgtagtgtctctgccagctttattaatagcagtcgcagtataccaggcagaatcttggctgacagtggaatcgattttaagggcagcttctcccttggttccttcaattctgattttgggatatttatgaggcacaatgatgtcactgtttttcaaccatacaatgtcagggttggggttacccgtagctctgactttcatttcaagtcgggaaccttcctttatattgacatttttcagtttttctacaaacatcggttttacctgatgttccacagcttccacagttaaaatcactgaaattgaagatctgcctgccctgttttgggcaaccacagtccattccccagaatcactgggtgtggcagggacaataattagtgattgagtaccatcttctttaatgactactttatgggtatagtcattgacaatttgctggccatcatgaaaccagaacgtctctggcataggtctaccaacaacctttaagtcaaatctggcagtttgcccttctaaacatttgaaagaaacaggttttaacacaaagactggtttatatagtctctcaagttgtgactcatctgtctcctccagcctacgtccaggggacattcttgcaggggacatccgtgcaggagacatccttgcaggtgacatccgtgcaggagacatgcgtataggagacctgctcactgaacgtggagagagagatctgattctgctcactggctctagtgtgggaatgtaagtcggagctccaagtggtgcagcaggctccacatacaatttccctgagcaaattgcatttcctttaatattgctggcaaatgcagtgtagattccttcatcttctggaagaacaacaggtatacgcagactagctctgccatcttgtagaaagtccatttggtatctttctccatgtttgatgcgcttgccatctttgtaccaagcaatctttggtaatggatatccagacatcttgcaatgaaaagtgacacccatcccctcaagaattctataattcttgattcttgaatcaaatcctgattcaacagcttcagattcagaaatgtcaactgccatcttttcttctccatcttcttcaagaagttcttctaatgtagtctttattattctatattcaatttctttaataagtctctcttcaaaggaagaaatatggaattcctgatcttctacataagttctgaccactacagtatctttggccattttcttcctaattaaggcttgttctttttcatactctttttcatactcagagtatacaaatccaggtgctgtttctccaactttaggttcttgaacaaatgcagtcacttgtgtctgataaagcatttcttgctgggacttcatcagtaactcataatcagcttcttcaagcaaggaagcagatgcagaagtttctccatgcttattgcgaacaacaatagtgtattctccagcatcatcagcaaaagtcatagaaatcaccagcttgcattcaccggtttgtttgttgtaactcactttgtatctgtatccagtggttagaggaacaccagattttttccagtatacatggggctttgggttgccgccaacttggcatccaaacaccacgctcccaccttccaccagtttctggaccactggttttgtaataaagtaaggcgcggcaggttctccaggccctgcttgttcctctgtgaggctagtatcagtcataaccacatctcttgactcaacaaagcgtttctcttctgtagtaaatttctcagtcacggctgtggtttccttttcaaattcttctgacacctgcacagccagatagcaggatgtgctgacggttccagcctcatttacagcactgcaagtaaatcgcccgctgtcttccgcaaatgcttcgcgaatcataagacgagcaattccactctggaaggttatctggaagtcaatggaactttcgatttggtagtcttccctgtaccatgtcactgtcggggatgggtatccagagatgtggcactccaaggtgacagattcaccttctatgacagtcacattttttaagcccgagaccaaagttggtggagtaacaggaatttcaacaggtgctggtactcttgctgtttctgttaccttggcttcgcgtccgtgcagtacttcaaagcgctcttcacggacggtggtgccagtgatgctcacccctacttcctttttcacctcaacgccagcttcactcttgtaagtatctggtgtgtcagcgaaggggaactgtggcaagggtgtgggctctgcccttactctagtctcactgggcttcacagtaggagccttcaccgatttggtgatcttctgagcagaagatgtggctgacaactctttttgtaatgtggcaatagcactaccggctattgatgcctcatatccatgttctgtcttaggaacagaaatttttgaaacagtaaagtgagggctagctgtgcgggggcgtttatccacatggactaatctttccgttgttagatctgtagttttcttgatctgtgatgatatgtgcattcccttttgatcagtagttttgatatgagtctcagaaggagcctggattactctaggcttgactgctttagggacaacgtggggttctgaggctggacgttggggaggctcagctacctttgcggcggaaatgcgttccttatatccgtactccaaagtggtctgctgagcataggattcttcaagatgcccaggctctctgggctctctgactcgggcctggtctactgcagcaacaactgttgctacagcttcagccttttttccaacgtccacctttccatgggtaacttggatttgttcttgtctagtagccatagtttctctagttctcagtattgtttcttgttctttggctttagcagtagcaactgctattgtagacaaggcagttttctcggcttcctttctcatcttctcctgagttatttgcacttgttctcttttggtagtaatgccttctctacctcttgatactaaatcttgttctttgactttgggtgtggcaactatgactttaggtacaactgttttcctagtttccttcattatcttttcataacttaggtgcatttgatcttgttgtgtggtagtttcttcttgagctcccgggactgtttctagttttgtggactttgcagtggcaactaccaccatggatgcagcagttatctcagtttcctgtcttattgcttcttgagttacttgtttctgtttcttagtaatttcttcagaaattctagtttcttgttctttggctttagctgcggaaattactacctttggtacaaatgttttttcagtttcttttcttatctgctcatgagttacgtgcatctgctcttgctttgtggtaattacttctttggttcttgattttaattcttgttccttggctttatcggcggccactactaccttagttacagcagtcttctccgcttcctttcttacctgctgttcttgagcaggttggatgtgcacagcagtcgtggttgtcctctgagcagtctgctctacagcgctgatcactggttctctcactctggccatatcaacggcagcaacaacagtcgcaacagctgcacttttgtcagcatcttgtttcacctctttagcaccagtggcaacagcctctgctgcgtagctagcactggccgacacactggcggcagcacccgcagcaccactgatggtcacttgctcctggacaccgtatctcccttcccatctctcttctgtcctgatctgagtagaggttgtcagcgttgtctctctcatctcagcctcagatgaggaggccacgtagccctcttgcttccaagggggaggcacttcaggacctgtggccacggtggatgcctgagtcttacgcatgagcaatggagacctaacagacctgatgggggatgtggagattcttgctgctggagacacggacctgaccggagatggggtcggtgcccgcacgtgtctgaccggggaaggggagtgtcttatgggcgatggggactgctgccgagccagctgtgctttggcagcaatagacggtggtgttggggatcttgactttggcttcggaggaatcctgggaggtgttttatgtggcagctgttgcccagcggcaccatctatgaccatctcaactgttgcaattgatctggcatcaaagtgggcttcaatcttcttttcaattcgggtttgtcttgattctgagatctgagcagtcgaaacaattgtctttgtctttttagcaggtacttcttcttcaccttgaaccagtaattcagcagtcgaagtagctcttccaacgctattggtggcatttactgaataggtccctgagtcctcagggtatgcttctgcaatcagtaagctgtagaggtcgccttcttgtgaaatttggaaatcaagggagctctggatttcggctccatcccggtagaacttcaccacaggtgtagggattccagtcactctcacttggagtctcacttggcttccttgtctcacggtcatgctctgcagtcgttgaacgaagttgggtggtgctgtctcagctttcacgagaagctcagcagtactagtcgcttgtccagatccattggtggctttcagggaatatcgtccactgttggctttagtcacggcggggatcgtcagtttagcgcggccatcgctaaaggagatctgcacgccgggcagagtggaagtggaaatcacctggccatccctaaaccagctcacctcaggaactggaaaaccactaatgtgagcctcaaaggttgcggtactaccctccagtaccacaacgctttgtaacggctgcgtaaacgtcggtgcttgagttgtcatctttctaggcactctgatttctcaagagtgcctaaaaagggtgggactaagcccaaggttgcttctgaaacgacgtcctatggagagttggtttttctgaccatctccgacatgaatcggtgagcctctaatcctaaaaacaaaactacacagtcaagactgtgtagttttgcttttctatgcaatccctacacccgaggcgaggctgggaatgcacgactgctc

SEQ ID NO: 9836 - RNA, 23198 nt, Homo sapiens
  source 1..23198: mol_type = other RNA
caaaaactgcagttacttttgccaacactgtttttcacttcaaagctatataatcctttgtcactcatttcggcacaggggattttaagggaagccactttattgatgaatgtaatgtgatgtttgctgtctgcagacaattctcttccatctttgaaccacttggctgagagttctggtgttccagtcactacacactctaatgcaaaaggatttccagtagtgacagtcatgggttcgggcttctctatgattcttgctggttctagtacagtcaagactgcagagcattctctcattccagcatcgtttttgatttggcatatatattttccagaattagatgcttctggactccccagctggagggttgcaatgttatcaatgaatgaaatcctggtattttcactctctctgatgacttcacctctatctttcagccagacaacagaaattggctggaagccctccactatggcccgtaactcaacagcatccccaataagggttgaggtgtcacttagctttttcacgaatcgtggaggttctttgaacttgacagagcaagaacacgtgtcacttcccacctcattagtagctttgcagtgatattccccgacatcggaggcttcaagattaaggatatgaagacttgtatcaaaatgttttgaagtgattttaaatttcttgctgtttctaacctgctttcgatctttaacccatactacttcaaatgggggagttcccgaaatttcacattggagaatcacatcagaacctttaagagctcctactggagaaggcttctgggtgaaaacaggaggtgctttcactgtcaacgctgtgctgcagctggcgtcaccaacaccattatgagcctcacaaatgtagtccccgctgtcttcagcactagcttcattgatcgtaagcaatgccacagaattaatgaatgacatgttgtatttccaactttcatgaagttcgctgtcatttcggaaccatgaaactttgatttctggggagccacttattttacattccagttgaatggattctccctgctttgcaacttttgaagcttctaatttcttaacaaactttggaggttcttttacactgagctgagctgagcacatgtctttgccaacatcattggttgcttggcaagtatattgaccagagtctcctttgcctactttaagaattctcaaatgaggagtgtttcccacacatgtgattgtatagtttcctccaggacggatctccttgttatcttttgaccaagtgattcgcatcggttgagcaccagtaacatgacactcaaaatcagcactttctccagcaataacatctatagatacaggcttgatgtcaaagaagggagatttcttgggttctcttgctgtgagtctagcactagaagatgctgttccaagtgggttggaagctgagcaagagtactggccagagtgactcaagtcagtttgcaaaatttttaaagttgccacattatctacaaatgaagtctgtagattttcatcgtctcttaaaagtactccatctctataccagcacacttggatgggtgcagagccatttaatcgacaagtgagtgtaacaggtaaccccacagtttgttcaatgtcctttaattgtcttgcaaaagaaggtgggagttggcgctcttgaattctgaacacagtcttagaagaagcagttcctatactattttctgctttgcatgtgtactctccactgtcattgatgttcactttattaaaaacaagtgtggccacattgtttgtaaagtaggtcctgtattcaggagttggccgtaatttggtatctcctttgtaccaagacactgtaatttctggtgtcccagcaacttggcattgtaaagaaaccgaatctccaactgctgcctccagaggttccagttccgtaacaaaataaggcggttctaatgtagataccagagctccacaaacatcccttcctgcctcattttcaatctcgcaggaatactgccctgcatctctttttgtgctattcagaatttccaggatacaagttttctctgttgtgactatgttacatttttcagaggtagttatgttaaaaccatcctttttccaagtgacagaaattggaagtgttccagtgtaggtgctctccagaattatggacttccctggttctacagaatgatcacttaatctcttcaaaaatgcagctggttctttcacaaagagacgggtagtgcaagatgcttggccagcgttgttagaaaccacacaggtgtattccccactctgagatatgtcaatattaaataattccagttctgccacagtgtcttcaaaatagatgttgcaccggtctcctttcactagttctctggcacctctgaaccagttgactttgaatggaggggttcctctaataacgcttgtgaaggttacatttttgcctggtagtacttccaaaggttcaggttctttcacaaaagagggtggttcttgtacagttagcactgcacgacattcatcagacccagcgacattagcagccacgcatgtgtaattgcccatatctgaggaatccagagaattcaactgcaatgtgcagacattatctgaaaatgtggtttggtactttgctccactgacaatcttggttttctcatgaaaccaggcaactgaaataggtgatgatccagctactttgcattccaagatgcaagaagcacctaacaccccaccagtatttttcagtcttcgtgtgaaagagggaggaactgctcggtctgaaacatcaaccacagctgtgcagctgcttttcccaacattattttgaacctggaaagtgtatgtgcctgcatcttgcctttcaactgagagaatccttaaggaagagattttgttgtagaagctaaatttgtgtttttggctgctggtcaacagctttccatccttgtaccattcaacagagagttccggagtgccagccaccttacactccagagtgcacgtttctcctacagtcaccgtcatcggtcctgccttctcaacaatgactgcgggctctaagaccatcagtgtggccatgttctccctcattccaccatcattcttgatttggcagatatactttccagcattagctggctctgcttttgcaaactgtagagttgcaacattttccacaaatgtaatcctgatgttttcactttctctaatcacttcttccttctctttaagccactggacaaaaataggctgggcgccttctatggatgcttgtaattcagcaggctctccggctacaacagtgaggctgttcagtttggagacaaatcttggtggttctttcaattttacagtacaaacacaagtatcacttcccacttcattctgtgctttgcagtggtattcaccgatgtctgaagtgtccacattgagaatgtgaatacttgtgtggaagtttttggatgcaatcttgtatttcttgctgcttctgagttgccgcttgtctttgtaccataccacctcaaacggtggtgttcccgaaagttcacattcaagactgacttcagcatttttaagggtttctactataggagggaagctgctaaaaacaggtggctcttttactataaccttggtactgcagcttgtgctgccagcgggattctgagcctcacaaatgaaatctccactgtcctcagtactgagattgttcatctgtatgacggccactgagtcaatgaaagtcattctgtacttatcactggctggaagttcatgttcatttcggaaccacacaactctgatttctggggatccagctatcttgcattcaagtcgtgaagagtcacctgctttcacaattttggaggcttctaatttctttacaaactttggtggttctgtcacaagcaacatcgtagtacaagagtcgctaccaacatcattggtaacatggcaagtatactgtccagtcttagaagcatccactgagtagagatttaagaagctagtcgacccttccaagccaatgaaacatttaggacctgagacaagttccacatcatccttaaaccattttattttaaatggtggtgttccttttagtattgccttaaattccactgtagaatcaggtatggcttgctgtcgcccaggtttcactaggaagcttggtggttctttcacagttaagatgccactgcatgcatcatctcctgctacatttgacactttgcatgtgtaatttgcagtatcttctaattccagattattaacttccagagacacagatctctcatggcacacaagtctgtattttgcacttgtagatatttcttttccatccttaaaccactgagcactaatgggaagtgaaccagacaccttgcactccatatgaatagaagagcccagaactttatccattttggttaattttttggtgaatgatggaggaatattttgatctagcactcttaagtaggcatcacagctactgcttccgaagtcattttccaccttgaaagtgtactgaccgctgtcctgcttcattactgactgaattctaaaactggccacgttattttcaaaactcattgaaaagtatctactgggaactatttgtttcccgtctttaagccatttcactttgagttctggtgttccagccacaacacattccaaggtcatgggatctttctccgtaacatcaactgatttagctttctctacgatttgagctggttcttgtactaaaaggaaagcataacacctctcaactcctgactcattcttggcttgacaggtatatctcccactgtgtccattatccacacttctgatttgaagtgtggccacactgtccacaaatgaaatatagacattatcatcttcatcaagaatctgatcatcctttagccaggttatagaaataggaggagaacctgccacggtactctgaaaggtggcagaacttttcaaaacagtagtggtattttctatcttcttaatgaatgatggtggttctttcagggcaactctagtactgcatgagcagctgccgccttcattggatacaatgcactggtattccccagtgtctgaagggtcacacttggttatatggaggttaaacacagacactctgtcggtcaatgtgtattttttgctgcttcgaatttccctgttattcttcagccaagtgacttcaaacggaggtgttcccgtaacttcacactccagctccacgtcactatattttactacctccacaggcttcagctctctgataaaggtggggggttctttcactttgagttcaatgctgcagctcgccgtgcctgcgtcatttcgagcttcacacacataagtcccactattttctaccctggcaccagaaatctggaaagtggctaaaccatcaatgaaggaaatgccatgtttctgaatggctgttatttcattcccgtctagataccaagacactcggattttaggagtgcctgttatttggcattcaaatgttgttgactgtccattcctcagcactaagactggactgggcttcttaatgaattgaggaggttcttttacaaagagagtggctttgctggttgctgtgccaacatcattgcttagttggcaaatgtaggttccagaatcggtagctttggctgcaaagagctctagactggtagaggtgtcatccttccaaactgagcgggctgctcctgagtgtaactctttgttatctttaaaccactttattgtcatgggtgcagtgccacccacaagagcctttaactgtacccttgtgttgggattgacatcttgtgactgtggcttttccacaaagtaagggggttctttgactgtcagatgcccactgcattggttgtgccctgccttatttgtggcagaacaagtgtatgtcccactgtctgtaccttccagctggctgatttccaagaaggcagtattgtcatgaaaagagaatttgtacttttcactagctgatatttcttggtcatctttgaaccactggatgcttatgggatgtgacccagccactatacattctaaatcaatgaaagaacctttaatgctgtccattttcttcagctttttggtgaatgaaggaggtatgataagatctaatacattaattctagccttgcagctgctcctcccaacatcattttggacctcgaaagtatattctccactatctttcttttctgtagaaataatcttcagtattgagactgtatcagtgacactgattttatattttgagcccagggtcagttcttggccatctttaaaccatttggctgtaatctccttagtccctgaaaatttaacctgcaaagtggctgggtctccttgggtgacatctatagacacagcttcctcggtgattgttgcaggttcttttactgagagtaatgcagaacatctttgtattcctgcatcatttttggcctgacagacatatttcccatcatgcttgacttcaatgccactgaggtacaaactggccacattgttctcaaaggtcattcttatattatcgtcttcagtgatttcatcgctgtcttttagccaagtcaccgtaattggcaaggagcccttcagagtggcctggaaggcagctgtgcctccccggagggagctggtactctcgatcttctttatgaaggatgggggttctcttaaagtcaccctggcactgcagatgctgctgcccacctcattggtcacccgacactggtattcgccagcatctgcagctacaaacttgaggatctgcaggctaaccagatgatcctgaatgaaagtcttatactttctaccacttcgcaggattgtgttatctttgaaccaagtgatctcaaagggaggagtgcctgccacctcagccagcaacatgacatcgtactcctttaagacttcaattggcttaaattccttggtaaaataaggtgactctttgactattacaatgctactgcagtggtcactgccagcctcattttgggcctcacacatatattcaccactgtcttcgatgccaacatctgtcagtcttagaactgcagtagactccacaaaagacattctgtgtttgctgctctccttaatttctctatcatttgcaaaccatgttattttaattggaggggtaccagttactttgcaggctagctgggtggcatctcccttctttaacagctgtgatggctctaacttttcaacaaatgtggcaggttcttttacaaacaagtttgcactgcattccacccctccagcgacattgctgactttacatgtgtacgtgcccgaatcagaggtttttactaaatagagttccagggaactctctaaagcttctttggtaatatagcagcttccaccagaaaccagctctttgttgcccttaaaccatctgattgtgagaggagtagatccttggaaagtgctcttcaggcagactgctgagccaggcagaacatcctttgagccgggtttagttacaaaactgggtggttcttgcacaatcagggctccactgctgtctttgcttcccacggaatttgtggctcgacaagtgaaattccctgcatcattcatgtctactctgatgatctccaaagaggctgtgccttccacaaatgctatcctgtatctgtcagaagcagctatttctttgccatccttaaaccaggacaccctcatggggagggagcctgcaattttgcagtccagtctgcaggtaccattaacaacactatccacgttgcgcaagggtttggtaaaaaatggagcaatgtctcgatctaatacagtgaatgtagtctcacaggagctgctgcccacttcattggaaatctcaaatgtgtattggccactgtcgtgcagctcagctgaataaaatttgagctgggcaacattgtttttaaaacttattcggtattttttactggcgaccaagggtctcccatctttgtaccatttgggcttcagttctggcgtgcctgccactgtgtactccagtgtggcgggatctcctgctgtcacctggatcagttctgctcgctcaatgattttggcaggttctttaactattaattccccaacagatgtttggcttccagcttcattttcagccaggcacgtgtatttgcctccaaaactaatctgaacatcagggattatcaagactgcaacaccattggaaaagctcattttgatttttccgtcttctctgatgacctcttgacctttcatccatgtgacagaaatgggctctgaccctctcacagcagcttgcagggtaacggtttgtcctcctagtgcaatcaaatcatctactttctttacaaaggttggaggttctttgagtaagtgggttgccatgcagccacacttgccgacttcattagcaacaacacattcatattcaccaacatctgcactattaaacgaaaagatctccagacacacaagagacttctgagaaaacaatctgtattttttactacttcgaatttgtttcttgtctttgaaccagctaatttcaaatggtccagtgcctgagacttcacactgaagtagagcatttgttcctctcactatgtctgcaggctcaagagttttgatgaaagaaggaggttctttgataactatttcagtactgcagctatcactgccgacgtcattcactgcttcacatgagtaactcccactgtcttcaacttttacatccgtaatatcaagtatagcctcagaattgacaaaatacattcggactgtgttactttcactgagttctttgttatttttaaaccaagtaacctggatcacaggtgagcctttcagcttgcaatggaggcgtgctgattcacctgggagcattaaataagagggatccaccttcttcacgaaggatggtggctctctgacagtgactgtggctgagcaggagctgcttccagcctcatttgaagctgtacagacataggttcctgaatctttcagtttggccaaaggaatctcaagtgttgctattttatcttcaaaacagatcttataatctttccctggggggagtttttgcccatctttgctccacgtaactgtgacttttctgtcttcatctacttggcactcaaggtggaccttcttattgatagcggactgcacaggctctaattctttaatgaaatgtggcttatcaatgatgatcaactctgcttggcagatgtctgctccaaacttgttggaagccttacaagaataaactcctctatcttgaatggtaaggtttgagagttctaaaatgtgtttgttttctgcgtcggaaatcctccagttaggtgaaggtgagagtgcagcaccatctttctgccaaatggtttctatcacaggagtccctgtcactgtgcagatgaacttggctgccttacccacaaaagttgtaagggacttaggtctggagagaaaggttggtggatatgcctctgtcacagttagtgtggctgtacagctgacactgccatactcattggaagctttgcatgtatactcgccgcagtcaaccacctgggttctcaggatttcaaggctggagatatactttgaagatcgaatagaacacttgtcactctcataaatttctcggccagctttaaaccactggaaccggacattgggagcactttggatctcacaggtgaatttggctaggtggcccagtgctacttccaggggttcgattttcctcttgatcactggggcagctctttttactacagtgagtttggctgaagttgctgtttttccgctgtcattcaaggcctcacagacatactctccttgatggtcttcggtatttactttgtcgatgactagcgtatatgtattttgatcttgtaaacacttgaacttttcatctgaaggcaccagtttattctcaaaataccaattcacctctttagcatttgttatggatgttgtgaggtgtacaatatcaccttcctcagaaacagtgtccactaaaggtgtatgtatcatggggccatcctctttgattaagccaccctcagcttcctgtatctttactgtagcaacctcctcagtaccactttcagaggaagactcctctttttcctctgatggtttcagactctcatcttgtttttcgtcagagacaacagctgaagcaacccctttagtgacaggtgtggcatccaaatatttaaccctactttgcacgttaaaataactgacctcttcagttgagatcagatatttagattcaacttctggttcagtaatgggttcaaccttctgtgaacctgaaaaagaatccatttcttcttgcaaacttgttttggctccttgctgaattctaggaccctcagctgttaggatgtctatttcctcatatataatagcacacaaagcatccctaagttccattttcaggttagccatttgaggatcaacatcttcaataatgatggttacttcttctgttacagactttgccgaagtaacaaggtacatgcacatgatgtgtctgggctcttgggtgatgtttacagcctcgacctccaccttttcaatatttcttagccactcagagaaaagacctggctgctcgctggccacggctgcttgcaaagcccggcagatttgaattttcaggtttaatctctgctcttctggaataccagaaagcaagctttccttagaaagaaggtcccttccctgtacctcctgcactttctttattgccacgggctctcttttagactcaatgatttggtctgggggcatcaccacgttgtcagaatgctcttctttgagcagtacctgcttttcttcaagtgctagtggaaatcttaaggacttgccttcctcaattctgaccgcagaatcttgccctgcattttccagtggatttgcactttctatcaaaattttacctccttctgtgcatgagtgttctgaagggactaggggctcatagtttacctgagagatcatgacatcaggactctggagactctccacgtgtccctcagctaagctctgactcaagatgagcgcactttgtgcctcttgcttttgaagagtcactctttgctctctgttggtgtcagatactgtcttttcttttggtgaaagtacttcctcagccacagaggttagataagaatgcattggaggttctattgaagactgtggataattcccttcaggttcagctaataaagttttcagaggctcaactgttaatgaattaatttgttctatggacatggcacttgggaagattttctcggtatctgatagaactgcctgtgtctcaggctcttcaggcattagaataccttctttggagaaggttttctgggactgtacaatctgcagctgtaggttgggagatggttccttgagaggctgaaagtgaatactgccattgatgcaaagaaattccctggtgctttcaggagtgagcttgtcttgctccaaaatggattgcaattcctgagctcccaaaggaagctgactgctcaattcattggctttagcaatatgctcataagatagttgctggttttcttctgtaattaaagcagctttcaaaatggtgtcttttacaaacgttgcaatttcctgctctgagtcaagtgcttcaactgcgggaccctttaagggtgtctgtggaaaatcctcaggagcctctggtgtggactttgctttgcagggggtatcagtcatgtctgtgtcttccagaagcacaagcagctctgctgcacaggtggactcacccaacatattctctgctttacagatatagaggccactgtcttccctctgagggtcattgacaatgaaagttccagagccattagggttatgaatgatagtgtaataaacactggtgcaaagctgcttgttttctttgaaccatgtaacagtaggggcaggctctccaaccactgtgtactcaaagatggcaggaagcccttgagcacagcgaattggttttaactccttaaggaagtgaggaggacaaggacctcccagcttttccagagattttgccactgctgattctgtttcagtgtctttgtgaccctctcctttggaattaatttttagataggcactacatattgtctttccatagtcattactggccatacatgtatactctccctcatcctccaatttggtgaacagaatgatcaggctatgatcatcaccgtcaaaaacaaatttgtagtcagcagaaggggttaatagcactccattaaagaaccactgaattttaggtttggggatgccaatgacagttacagacagtgtagccacatcccccatgcttatatcagcatttgacacttctttgatgaaaattgggccagtgccttccttttcggaatcaaatttagttgggtaaactggagattcagacaaaagttcaagtgtttcatttattttagataattgaagttcggcgctatgaagtccttcttcctcggcagacagaaaagaactagaaaactctttcatttccatctcaatctcttgttcaatcctctcatgcaaaattgattcaggagcttccagactcaggttggctgtgcttgatacttggcctacagcattactagcaacaaacgtgtaagttccttcatcttctggataagcttcggcaatttccagttgataagtgtcttcaaattgagtcattctaaagaaccgagatggcttgattttcttgtctttgctgtaccacgacacttttagatctgttccagaaacccggcattgaaaacgggctggctgcccttcagaagtgacagtgtcctgaagcggggtgatgatggcaggtggataaacaggcatttcctgatcaggagacacaacttctggaacttccactgagagtgaagctgatgttgtggcaacaccatagtcattcttggcttcacaggtatagactgccgcatcctctgggaaggcttcaattagcaaaagcgtgtattcttgcccatcatgaagaaatttgcacttgaagccagtggaaagcagctgctcttccttgtaccaggaaattttgggctgtggtcttccggatatcacggcacagaagcgggcaggcttgccagactgcacagtgacaggctggagctcctgcagaacttggggcggttcaggagcattgacatagagagtgacagaactcctgttccttcctgccacaaaggtgtattctcctgcatcgctctgtctggtctcagagataaacattcggtggattcttctttccactacatatttgtgtcgttcttgaacttggaaattgatttcaatgccatctttataccagtgggcatcaacatcgtcttcattgacctcaaattcaacaacagcacgctgtttctcaatgacctgaacctcctttttaatacttcggatgcgaacatctctgccttctacaaagagttttgcagttgacacgttgcctcctgccaccactgtgtacttcccagcatcagacatccgggtggatgggatcagaaggcggtggacatatttctccttctgaatctttattctgtctgtgatctgcagttcctggtcatctttcatccactgtacagtgatgtcaggttcagaaacttcacattcaaacatggctcgcttcttctccagtaccttaatgtccttaatgtgtttcctaaattctatatgacgagcttccacataaagtgtggctgttgatgttgcttttccagccacaaaggtgtagtcagcagcatccccaaagtgaacattcctgatgttcagtgagtgtgtgagctttttggttctcatctggcacttgtcagttgatttgatttccacaccattctttaaccatttgtaagagatgccttcatagttcactgtcacctcaaaagtaatagtgtctttttcttcagcgttgatgtctttcagcatggaagtaatcatgattggggtgactgtcagggtggcactgacttggtcattgccacagacaaatgtgtattctgccgagtcctctgtgctggtgttcatgatgatcagctgatggagttttccctgcacaactatcttgaacttttcactcatctcaatttccacaccattcttcagccacatggaagggacattgaagtgggacacctcacactcaaaagaggcagttttggtctcaggcacctcgatatttttcatggtttttgtaatatgtaatgtctccacaaacagttttgctttgcattccaattgcccgaccacagctgtgtattccccagcatctgagggggagatgttctgcagcatcagcttgtggactttcctttctgagaccagtctgtgtttgtcacttggcttaatttccacactcttatggaaccattttactggaacagtgtcatgggaaacactaacttcaaaggcaacagtggcattttccaaggctgtcacatcctttggctttttaatgatcttgacagtctccacgtgcagtctggcactggctccaagccttccaagcctgaagccataaacagactcatccacgatggcacagtttttaatcctcagagagtaaattgttcctttgacagagatagcatacttttcattggattccagcacaactccatttttgatccactggacacctttgacattagggtgtgtaagctcgacagtgaaaacagcatcctgtgtttctgtcactgtgaggttcttcagagtcttcttaattttgacagcttcaactttgagtttggcagatgttttggaggtggccaccttgtaggtatattctccaatgtcatctaatttggtggcagcaatgataagtctccttttgtggccatcagactcacttctgatgttgttagtcagtggtaggtgtttgccatccctcaaccattcgcctttggaatctgggttggcaacttcacattcaaacacagcttcctgggattcagctacggtctgatctgtgagtggcttggagatggccccacctgccacagtaagttttccagatgtcatattttctcccgcgtaaaatgtgtattttccttcatcatctttcatcatatttagaactgtcaatttatatatttttccatgtgcttcaattttatatttagaactgggcttgatttccttgtccttaaaattccacaggacatcaattccagagtgggacagctcaacctcaaacaccacattttgagtttctgtacaggtaaggtcacgaagacctctgataattttaattttttctacagagagattacagttggtttcaactctgccaactatcagcttgtaaggtccttcgtctgaagcatgagttcggttaatgactagtcgctgtttagtacctttcacaatggcctgtacacggtcatcaggcttgatttgttcatcatttaagtaccacttaacagaagtcacatcagggactgacaccttacattcaagcacagccttggtgccttcaatcacattaacatcttttagaggtgttatcacgtccacactatagacagagacacgcccactggtggagaggccaagggctggaatggtgaaagagtaatttccagcatcttccttagtcatgtcttcaatgagcagcatatgagattgtttgtctatcacaatgtgaaccctgtcactgggctgcacttcttggccgtctttcatccagacgccttccacactttccaaggagactttaacttcaagctgaacaatgtcaccctcacagactttttggtcactaagtccttgtaggatagcaatggggcggggtttcatctttaatttacaggttgtctttttcccgtcgatgacaaagctgtattctccctggtcctccttggttacatccttgaccgtgaggttctgacgtccacgacgagatgtaattgtatatttgccattggatttaagctccacatcattatgataccattttccttctatattttctggggatacaatgcactctaattctcctgaatatgattctggaacttctatgtcctgaagttctttcacaaactcaacaactgcaccttcaacaataagtttagcagtcgttttgacattttcatcttccacaagtacacagctgtaatcttcagcatcagacgtatcaatggtcagtatggagaggaagtgaacctttctgtcagagtgcatcctgtatttatctccctcatgaacctccataccatctttataccatttcactttgacaaatggttctgaagtttcacattcaaaggttgccatagtgtctttttccttagcaacaacatcttgtaattcctgtgtgaaagtgatcaattgcttggcttggacaagtaagaatgcgtgactggaggtttctccagctatgttgatggcttttaccatgatgctggcagagtcctcagcagtcacatctcttatgaccaattcacaaacattgtcttcgggccagtaccagtagatccggtcagaccgttcaattttgacaccatttttgtaccattcacattcggggtctggtttccccacgactctgacccggaagtgtgcatcagatccttggcccactgtttggctctggattctttcgaagatttttggagcctccatactaggacttagttcaatcttgtcaggtttaaaagttggaatcgtgattttgccttcttcggcaagagctttcttttcctcttcagttaactctttggtccagtggagaagttcatcttttgtcttcctgaggagttcctcataggattcatccttctttcgagacttgagctccacagcggtaatggcttcataatagccctcttctgttctgcgcttgaatttactgcgcagctcttccgactcttcaggcactttttcatgggtaattctttcagcccttttcaacttcacaacttctttggtttcagtggtgtcaacaggtctatccactttttgtacttcaaactgaagctttcctggttcatgtacgtgaaactcaggccttggttcaggagctctcctaaggacagacctaaaatcttccctctgttgaatctcaagcttcactttatgctctatcacaccttcaggattttccgcggtgaccttcacttcacctgtgtcatatgatttgcagtccacgatgtccaggtaatggataccatcatagcgaactctgaaccttttgcttttgcggatgagctgtccattgaggtaccagttgactttgggctgagggtagcctgttaccctgcagcggaaccttgcagtctccccttcaagtactctaactggctctgggtacaagacaatgtctggcttttgcttttctttctgatctgttgttacacctgtaagtgcaccttcatgagccattctctctaattcttcaattctctgtaagcctttcctcccctcaggcaattgggattcttccacaagacttttctcatctttaacaataagggtagcagatgtgtgatctgttccatatttgttagtggctctgcaagtaatgataccactgtctctagaatatgcaacgccataatcaaggctgcagtacccaaattcattgatcatacggagcctgttggctgcttcaagtggctttccatcatggagccactccaccaccatcgttgggtcaccaatgggtgttagcctgcattcaaagtgggcaggcccaaagcgcttaagtcttaaggaagtgagttttttcttgaaaaatggtttctgttgtttctctttgtcatagagatcaccttcttcccattgctcttggccatatcgcaaatggaggggctccagttctggggctgcaatctcctttgctctatatgtcccccgtgggatgattaactttctctctggctcaggctctgcaaactcaacttcaacatttactttgcatcttgtagtgtctctgccagctttattaatagcagtcgcagtataccaggcagaatcttggctgacagtggaatcgattttaagggcagcttctcccttggttccttcaattctgattttgggatatttatgaggcacaatgatgtcactgtttttcaaccatacaatgtcagggttggggttacccgtagctctgactttcatttcaagtcgggaaccttcctttatattgacatttttcagtttttctacaaacatcggttttacctgatgttccacagcttccacagttaaaatcactgaaattgaagatctgcctgccctgttttgggcaaccacagtccattccccagaatcactgggtgtggcagggacaataattagtgattgagtaccatcttctttaatgactactttatgggtatagtcattgacaatttgctggccatcatgaaaccagaacgtctctggcataggtctaccaacaacctttaagtcaaatctggcagtttgcccttctaaacatttgaaagaaacaggttttaacacaaagactggtttatatagtctctcaagttgtgactcatctgtctcctccagcctacgtccaggggacattcttgcaggggacatccgtgcaggagacatccttgcaggtgacatccgtgcaggagacatgcgtataggagacctgctcactgaacgtggagagagagatctgattctgctcactggctctagtgtgggaatgtaagtcggagctccaagtggtgcagcaggctccacatacaatttccctgagcaaattgcatttcctttaatattgctggcaaatgcagtgtagattccttcatcttctggaagaacaacaggtatacgcagactagctctgccatcttgtagaaagtccatttggtatctttctccatgtttgatgcgcttgccatctttgtaccaagcaatctttggtaatggatatccagacatcttgcaatgaaaagtgacacccatcccctcaagaattctataattcttgattcttgaatcaaatcctgattcaacagcttcagattcagaaatgtcaactgccatcttttcttctccatcttcttcaagaagttcttctaatgtagtctttattattctatattcaatttctttaataagtctctcttcaaaggaagaaatatggaattcctgatcttctacataagttctgaccactacagtatctttggccattttcttcctaattaaggcttgttctttttcatactctttttcatactcagagtatacaaatccaggtgctgtttctccaactttaggttcttgaacaaatgcagtcacttgtgtctgataaagcatttcttgctgggacttcatcagtaactcataatcagcttcttcaagcaaggaagcagatgcagaagtttctccatgcttattgcgaacaacaatagtgtattctccagcatcatcagcaaaagtcatagaaatcaccagcttgcattcaccggtttgtttgttgtaactcactttgtatctgtatccagtggttagaggaacaccagattttttccagtatacatggggctttgggttgccgccaacttggcatccaaacaccacgctcccaccttccaccagtttctggaccactggttttgtaataaagtaaggcgcggcaggttctccaggccctgcttgttcctctgtgaggctagtatcagtcataaccacatctcttgactcaacaaagcgtttctcttctgtagtaaatttctcagtcacggctgtggtttccttttcaaattcttctgacacctgcacagccagatagcaggatgtgctgacggttccagcctcatttacagcactgcaagtaaatcgcccgctgtcttccgcaaatgcttcgcgaatcataagacgagcaattccactctggaaggttatctggaagtcaatggaactttcgatttggtagtcttccctgtaccatgtcactgtcggggatgggtatccagagatgtggcactccaaggtgacagattcaccttctatgacagtcacattttttaagcccgagaccaaagttggtggagtaacaggaatttcaacaggtgctggtactcttgctgtttctgttaccttggcttcgcgtccgtgcagtacttcaaagcgctcttcacggacggtggtgccagtgatgctcacccctacttcctttttcacctcaacgccagcttcactcttgtaagtatctggtgtgtcagcgaaggggaactgtggcaagggtgtgggctctgcccttactctagtctcactgggcttcacagtaggagccttcaccgatttggtgatcttctgagcagaagatgtggctgacaactctttttgtaatgtggcaatagcactaccggctattgatgcctcatatccatgttctgtcttaggaacagaaatttttgaaacagtaaagtgagggctagctgtgcgggggcgtttatccacatggactaatctttccgttgttagatctgtagttttcttgatctgtgatgatatgtgcattcccttttgatcagtagttttgatatgagtctcagaaggagcctggattactctaggcttgactgctttagggacaacgtggggttctgaggctggacgttggggaggctcagctacctttgcggcggaaatgcgttccttatatccgtactccaaagtggtctgctgagcataggattcttcaagatgcccaggctctctgggctctctgactcgggcctggtctactgcagcaacaactgttgctacagcttcagccttttttccaacgtccacctttccatgggtaacttggatttgttcttgtctagtagccatagtttctctagttctcagtattgtttcttgttctttggctttagcagtagcaactgctattgtagacaaggcagttttctcggcttcctttctcatcttctcctgagttatttgcacttgttctcttttggtagtaatgccttctctacctcttgatactaaatcttgttctttgactttgggtgtggcaactatgactttaggtacaactgttttcctagtttccttcattatcttttcataacttaggtgcatttgatcttgttgtgtggtagtttcttcttgagctcccgggactgtttctagttttgtggactttgcagtggcaactaccaccatggatgcagcagttatctcagtttcctgtcttattgcttcttgagttacttgtttctgtttcttagtaatttcttcagaaattctagtttcttgttctttggctttagctgcggaaattactacctttggtacaaatgttttttcagtttcttttcttatctgctcatgagttacgtgcatctgctcttgctttgtggtaattacttctttggttcttgattttaattcttgttccttggctttatcggcggccactactaccttagttacagcagtcttctccgcttcctttcttacctgttcttgagcaggttggatgtgcacagcagtcgtggttgtcctctgagcagtctgctctacagcgctgatcactggttctctcactctggccatatcaacggcagcaacaacagtcgcaacagctgcacttttgtcagcatcttgtttcacctctttagcaccagtggcaacagcctctgctgcgtagctagcactggccgacacactggcggcagcacccgcagcaccactgatggtcacttgctcctggacaccgtatctcccttcccatctctcttctgtcctgatctgagtagaggttgtcagcgttgtctctctcatctcagcctcagatgaggaggccacgtagccctcttgcttccaagggggaggcacttcaggacctgtggccacggtggatgcctgagtcttacgcatgagcaatggagacctaacagacctgatgggggatgtggagattcttgctgctggagacacggacctgaccggagatggggtcggtgcccgcacgtgtctgaccggggaaggggagtgtcttatgggcgatggggactgctgccgagccagctgtgctttggcagcaatagacggtggtgttggggatcttgactttggcttcggaggaatcctgggaggtgttttatgtggcagctgttgcccagcggcaccatctatgaccatctcaactgttgcaattgatctggcatcaaagtgggcttcaatcttcttttcaattcgggtttgtcttgattctgagatctgagcagtcgaaacaattgtctttgtctttttagcaggtacttcttcttcaccttgaaccagtaattcagcagtcgaagtagctcttccaacgctattggtggcatttactgaataggtccctgagtcctcagggtatgcttctgcaatcagtaagctgtagaggtcgccttcttgtgaaatttggaaatcaagggagctctggatttcggctccatcccggtagaacttcaccacaggtgtagggattccagtcactctcacttggagtctcacttggcttccttgtctcacggtcatgctctgcagtcgttgaacgaagttgggtggtgctgtctcagctttcacgagaagctcagcagtactagtcgcttgtccagatccattggtggctttcagggaatatcgtccactgttggctttagtcacggcggggatcgtcagtttagcgcggccatcgctaaaggagatctgcacgccgggcagagtggaagtggaaatcacctggccatccctaaaccagctcacctcaggaactggaaaaccactaatgtgagcctcaaaggttgcggtactaccctccagtaccacaacgctttgtaacggctgcgtaaacgtcggtgcttgagttgtcatctttctaggcactctgatttctcaagagtgcctaaaaagggtgggactaagcccaaggttgcttctgaaacgacgtcctatggagagttggtttttctgaccatctccgacatgaatcggtgagcctctaatcctaaaaacaaaactacacagtcaagactgtgtagttttgcttttctatgcaatccctacacccgaggcgaggctgggaatgcacgactgctc

SEQ ID NO: 9837 - RNA, 20420 nt, Homo sapiens
  source 1..20420: mol_type = other RNA
caaaaactgcagttacttttgccaacactgtttttcacttcaaagctatataatcctttgtcactcatttcggcacaggggattttaagggaagccactttattgatgaatgtaatgtgatgtttgctgtctgcagacaattctcttccatctttgaaccacttggctgagagttctggtgttccagtcactacacactctaatgcaaaaggatttccagtagtgacagtcatgggttcgggcttctctatgattcttgctggttctagtacagtcaagactgcagagcattctctcattccagcatcgtttttgatttggcatatatattttccagaattagatgcttctggactccccagctggagggttgcaatgttatcaatgaatgaaatcctggtattttcactctctctgatgacttcacctctatctttcagccagacaacagaaattggctggaagccctccactatggcccgtaactcaacagcatccccaataagggttgaggtgtcacttagctttttcacgaatcgtggaggttctttgaacttgacagagcaagaacacgtgtcacttcccacctcattagtagctttgcagtgatattccccgacatcggaggcttcaagattaaggatatgaagacttgtatcaaaatgttttgaagtgattttaaatttcttgctgtttctaacctgctttcgatctttaacccatactacttcaaatgggggagttcccgaaatttcacattggagaatcacatcagaacctttaagagctcctactggagaaggcttctgggtgaaaacaggaggtgctttcactgtcaacgctgtgctgcagctggcgtcaccaacaccattatgagcctcacaaatgtagtccccgctgtcttcagcactagcttcattgatcgtaagcaatgccacagaattaatgaatgacatgttgtatttccaactttcatgaagttcgctgtcatttcggaaccatgaaactttgatttctggggagccacttattttacattccagttgaatggattctccctgctttgcaacttttgaagcttctaatttcttaacaaactttggaggttcttttacactgagctgagctgagcacatgtctttgccaacatcattggttgcttggcaagtatattgaccagagtctcctttgcctactttaagaattctcaaatgaggagtgtttcccacacatgtgattgtatagtttcctccaggacggatctccttgttatcttttgaccaagtgattcgcatcggttgagcaccagtaacatgacactcaaaatcagcactttctccagcaataacatctatagatacaggcttgatgtcaaagaagggagatttcttgggttctcttgctgtgagtctagcactagaagatgctgttccaagtgggttggaagctgagcaagagtactggccagagtgactcaagtcagtttgcaaaatttttaaagttgccacattatctacaaatgaagtctgtagattttcatcgtctcttaaaagtactccatctctataccagcacacttggatgggtgcagagccatttaatcgacaagtgagtgtaacaggtaaccccacagtttgttcaatgtcctttaattgtcttgcaaaagaaggtgggagttggcgctcttgaattctgaacacagtcttagaagaagcagttcctatactattttctgctttgcatgtgtactctccactgtcattgatgttcactttattaaaaacaagtgtggccacattgtttgtaaagtaggtcctgtattcaggagttggccgtaatttggtatctcctttgtaccaagacactgtaatttctggtgtcccagcaacttggcattgtaaagaaaccgaatctccaactgctgcctccagaggttccagttccgtaacaaaataaggcggttctaatgtagataccagagctccacaaacatcccttcctgcctcattttcaatctcgcaggaatactgccctgcatctctttttgtgctattcagaatttccaggatacaagttttctctgttgtgactatgttacatttttcagaggtagttatgttaaaaccatcctttttccaagtgacagaaattggaagtgttccagtgtaggtgctctccagaattatggacttccctggttctacagaatgatcacttaatctcttcaaaaatgcagctggttctttcacaaagagacgggtagtgcaagatgcttggccagcgttgttagaaaccacacaggtgtattccccactctgagatatgtcaatattaaataattccagttctgccacagtgtcttcaaaatagatgttgcaccggtctcctttcactagttctctggcacctctgaaccagttgactttgaatggaggggttcctctaataacgcttgtgaaggttacatttttgcctggtagtacttccaaaggttcaggttctttcacaaaagagggtggttcttgtacagttagcactgcacgacattcatcagacccagcgacattagcagccacgcatgtgtaattgcccatatctgaggaatccagagaattcaactgcaatgtgcagacattatctgaaaatgtggtttggtactttgctccactgacaatcttggttttctcatgaaaccaggcaactgaaataggtgatgatccagctactttgcattccaagatgcaagaagcacctaacaccccaccagtatttttcagtcttcgtgtgaaagagggaggaactgctcggtctgaaacatcaaccacagctgtgcagctgcttttcccaacattattttgaacctggaaagtgtatgtgcctgcatcttgcctttcaactgagagaatccttaaggaagagattttgttgtagaagctaaatttgtgtttttggctgctggtcaacagctttccatccttgtaccattcaacagagagttccggagtgccagccaccttacactccagagtgcacgtttctcctacagtcaccgtcatcggtcctgccttctcaacaatgactgcgggctctaagaccatcagtgtggccatgttctccctcattccaccatcattcttgatttggcagatatactttccagcattagctggctctgcttttgcaaactgtagagttgcaacattttccacaaatgtaatcctgatgttttcactttctctaatcacttcttccttctctttaagccactggacaaaaataggctgggcgccttctatggatgcttgtaattcagcaggctctccggctacaacagtgaggctgttcagtttggagacaaatcttggtggttctttcaattttacagtacaaacacaagtatcacttcccacttcattctgtgctttgcagtggtattcaccgatgtctgaagtgtccacattgagaatgtgaatacttgtgtggaagtttttggatgcaatcttgtatttcttgctgcttctgagttgccgcttgtctttgtaccataccacctcaaacggtggtgttcccgaaagttcacattcaagactgacttcagcatttttaagggtttctactataggagggaagctgctaaaaacaggtggctcttttactataaccttggtactgcagcttgtgctgccagcgggattctgagcctcacaaatgaaatctccactgtcctcagtactgagattgttcatctgtatgacggccactgagtcaatgaaagtcattctgtacttatcactggctggaagttcatgttcatttcggaaccacacaactctgatttctggggatccagctatcttgcattcaagtcgtgaagagtcacctgctttcacaattttggaggcttctaatttctttacaaactttggtggttctgtcacaagcaacatcgtagtacaagagtcgctaccaacatcattggtaacatggcaagtatactgtccagtcttagaagcatccactgagtagagatttaagaagctagtcgacccttccaagccaatgaaacatttaggacctgagacaagttccacatcatccttaaaccattttattttaaatggtggtgttccttttagtattgccttaaattccactgtagaatcaggtatggcttgctgtcgcccaggtttcactaggaagcttggtggttctttcacagttaagatgccactgcatgcatcatctcctgctacatttgacactttgcatgtgtaatttgcagtatcttctaattccagattattaacttccagagacacagatctctcatggcacacaagtctgtattttgcacttgtagatatttcttttccatccttaaaccactgagcactaatgggaagtgaaccagacaccttgcactccatatgaatagaagagcccagaactttatccattttggttaattttttggtgaatgatggaggaatattttgatctagcactcttaagtaggcatcacagctactgcttccgaagtcattttccaccttgaaagtgtactgaccgctgtcctgcttcattactgactgaattctaaaactggccacgttattttcaaaactcattgaaaagtatctactgggaactatttgtttcccgtctttaagccatttcactttgagttctggtgttccagccacaacacattccaaggtcatgggatctttctccgtaacatcaactgatttagctttctctacgatttgagctggttcttgtactaaaaggaaagcataacacctctcaactcctgactcattcttggcttgacaggtatatctcccactgtgtccattatccacacttctgatttgaagtgtggccacactgtccacaaatgaaatatagacattatcatcttcatcaagaatctgatcatcctttagccaggttatagaaataggaggagaacctgccacggtactctgaaaggtggcagaacttttcaaaacagtagtggtattttctatcttcttaatgaatgatggtggttctttcagggcaactctagtactgcatgagcagctgccgccttcattggatacaatgcactggtattccccagtgtctgaagggtcacacttggttatatggaggttaaacacagacactctgtcggtcaatgtgtattttttgctgcttcgaatttccctgttattcttcagccaagtgacttcaaacggaggtgttcccgtaacttcacactccagctccacgtcactatattttactacctccacaggcttcagctctctgataaaggtggggggttctttcactttgagttcaatgctgcagctcgccgtgcctgcgtcatttcgagcttcacacacataagtcccactattttctaccctggcaccagaaatctggaaagtggctaaaccatcaatgaaggaaatgccatgtttctgaatggctgttatttcattcccgtctagataccaagacactcggattttaggagtgcctgttatttggcattcaaatgttgttgactgtccattcctcagcactaagactggactgggcttcttaatgaattgaggaggttcttttacaaagagagtggctttgctggttgctgtgccaacatcattgcttagttggcaaatgtaggttccagaatcggtagctttggctgcaaagagctctagactggtagaggtgtcatccttccaaactgagcgggctgctcctgagtgtaactctttgttatctttaaaccactttattgtcatgggtgcagtgccacccacaagagcctttaactgtacccttgtgttgggattgacatcttgtgactgtggcttttccacaaagtaagggggttctttgactgtcagatgcccactgcattggttgtgccctgccttatttgtggcagaacaagtgtatgtcccactgtctgtaccttccagctggctgatttccaagaaggcagtattgtcatgaaaagagaatttgtacttttcactagctgatatttcttggtcatctttgaaccactggatgcttatgggatgtgacccagccactatacattctaaatcaatgaaagaacctttaatgctgtccattttcttcagctttttggtgaatgaaggaggtatgataagatctaatacattaattctagccttgcagctgctcctcccaacatcattttggacctcgaaagtatattctccactatctttcttttctgtagaaataatcttcagtattgagactgtatcagtgacactgattttatattttgagcccagggtcagttcttggccatctttaaaccatttggctgtaatctccttagtccctgaaaatttaacctgcaaagtggctgggtctccttgggtgacatctatagacacagcttcctcggtgattgttgcaggttcttttactgagagtaatgcagaacatctttgtattcctgcatcatttttggcctgacagacatatttcccatcatgcttgacttcaatgccactgaggtacaaactggccacattgttctcaaaggtcattcttatattatcgtcttcagtgatttcatcgctgtcttttagccaagtcaccgtaattggcaaggagcccttcagagtggcctggaaggcagctgtgcctccccggagggagctggtactctcgatcttctttatgaaggatgggggttctcttaaagtcaccctggcactgcagatgctgctgcccacctcattggtcacccgacactggtattcgccagcatctgcagctacaaacttgaggatctgcaggctaaccagatgatcctgaatgaaagtcttatactttctaccacttcgcaggattgtgttatctttgaaccaagtgatctcaaagggaggagtgcctgccacctcagccagcaacatgacatcgtactcctttaagacttcaattggcttaaattccttggtaaaataaggtgactctttgactattacaatgctactgcagtggtcactgccagcctcattttgggcctcacacatatattcaccactgtcttcgatgccaacatctgtcagtcttagaactgcagtagactccacaaaagacattctgtgtttgctgctctccttaatttctctatcatttgcaaaccatgttattttaattggaggggtaccagttactttgcaggctagctgggtggcatctcccttctttaacagctgtgatggctctaacttttcaacaaatgtggcaggttcttttacaaacaagtttgcactgcattccacccctccagcgacattgctgactttacatgtgtacgtgcccgaatcagaggtttttactaaatagagttccagggaactctctaaagcttctttggtaatatagcagcttccaccagaaaccagctctttgttgcccttaaaccatctgattgtgagaggagtagatccttggaaagtgctcttcaggcagactgctgagccaggcagaacatcctttgagccgggtttagttacaaaactgggtggttcttgcacaatcagggctccactgctgtctttgcttcccacggaatttgtggctcgacaagtgaaattccctgcatcattcatgtctactctgatgatctccaaagaggctgtgccttccacaaatgctatcctgtatctgtcagaagcagctatttctttgccatccttaaaccaggacaccctcatggggagggagcctgcaattttgcagtccagtctgcaggtaccattaacaacactatccacgttgcgcaagggtttggtaaaaaatggagcaatgtctcgatctaatacagtgaatgtagtctcacaggagctgctgcccacttcattggaaatctcaaatgtgtattggccactgtcgtgcagctcagctgaataaaatttgagctgggcaacattgtttttaaaacttattcggtattttttactggcgaccaagggtctcccatctttgtaccatttgggcttcagttctggcgtgcctgccactgtgtactccagtgtggcgggatctcctgctgtcacctggatcagttctgctcgctcaatgattttggcaggttctttaactattaattccccaacagatgtttggcttccagcttcattttcagccaggcacgtgtatttgcctccaaaactaatctgaacatcagggattatcaagactgcaacaccattggaaaagctcattttgatttttccgtcttctctgatgacctcttgacctttcatccatgtgacagaaatgggctctgaccctctcacagcagcttgcagggtaacggtttgtcctcctagtgcaatcaaatcatctactttctttacaaaggttggaggttctttgagtaagtgggttgccatgcagccacacttgccgacttcattagcaacaacacattcatattcaccaacatctgcactattaaacgaaaagatctccagacacacaagagacttctgagaaaacaatctgtattttttactacttcgaatttgtttcttgtctttgaaccagctaatttcaaatggtccagtgcctgagacttcacactgaagtagagcatttgttcctctcactatgtctgcaggctcaagagttttgatgaaagaaggaggttctttgataactatttcagtactgcagctatcactgccgacgtcattcactgcttcacatgagtaactcccactgtcttcaacttttacatccgtaatatcaagtatagcctcagaattgacaaaatacattcggactgtgttactttcactgagttctttgttatttttaaaccaagtaacctggatcacaggtgagcctttcagcttgcaatggaggcgtgctgattcacctgggagcattaaataagagggatccaccttcttcacgaaggatggtggctctctgacagtgactgtggctgagcaggagctgcttccagcctcatttgaagctgtacagacataggttcctgaatctttcagtttggccaaaggaatctcaagtgttgctattttatcttcaaaacagatcttataatctttccctggggggagtttttgcccatctttgctccacgtaactgtgacttttctgtcttcatctacttggcactcaaggtggaccttcttattgatagcggactgcacaggctctaattctttaatgaaatgtggcttatcaatgatgatcaactctgcttggcagatgtctgctccaaacttgttggaagccttacaagaataaactcctctatcttgaatggtaaggtttgagagttctaaaatgtgtttgttttctgcgtcggaaatcctccagttaggtgaaggtgagagtgcagcaccatctttctgccaaatggtttctatcacaggagtccctgtcactgtgcagatgaacttggctgccttacccacaaaagttgtaagggacttaggtctggagagaaaggttggtggatatgcctctgtcacagttagtgtggctgtacagctgacactgccatactcattggaagctttgcatgtatactcgccgcagtcaaccacctgggttctcaggatttcaaggctggagatatactttgaagatcgaatagaacacttgtcactctcataaatttctcggccagctttaaaccactggaaccggacattgggagcactttggatctcacaggtgaatttggctaggtggcccagtgctacttccaggggttcgattttcctcttgatcactggggcagctttcatttccatctcaatctcttgttcaatcctctcatgcaaaattgattcaggagcttccagactcaggttggctgtgcttgatacttggcctacagcattactagcaacaaacgtgtaagttccttcatcttctggataagcttcggcaatttccagttgataagtgtcttcaaattgagtcattctaaagaaccgagatggcttgattttcttgtctttgctgtaccacgacacttttagatctgttccagaaacccggcattgaaaacgggctggctgcccttcagaagtgacagtgtcctgaagcggggtgatgatggcaggtggataaacaggcatttcctgatcaggagacacaacttctggaacttccactgagagtgaagctgatgttgtggcaacaccatagtcattcttggcttcacaggtatagactgccgcatcctctgggaaggcttcaattagcaaaagcgtgtattcttgcccatcatgaagaaatttgcacttgaagccagtggaaagcagctgctcttccttgtaccaggaaattttgggctgtggtcttccggatatcacggcacagaagcgggcaggcttgccagactgcacagtgacaggctggagctcctgcagaacttggggcggttcaggagcattgacatagagagtgacagaactcctgttccttcctgccacaaaggtgtattctcctgcatcgctctgtctggtctcagagataaacattcggtggattcttctttccactacatatttgtgtcgttcttgaacttggaaattgatttcaatgccatctttataccagtgggcatcaacatcgtcttcattgacctcaaattcaacaacagcacgctgtttctcaatgacctgaacctcctttttaatacttcggatgcgaacatctctgccttctacaaagagttttgcagttgacacgttgcctcctgccaccactgtgtacttcccagcatcagacatccgggtggatgggatcagaaggcggtggacatatttctccttctgaatctttattctgtctgtgatctgcagttcctggtcatctttcatccactgtacagtgatgtcaggttcagaaacttcacattcaaacatggctcgcttcttctccagtaccttaatgtccttaatgtgtttcctaaattctatatgacgagcttccacataaagtgtggctgttgatgttgcttttccagccacaaaggtgtagtcagcagcatccccaaagtgaacattcctgatgttcagtgagtgtgtgagctttttggttctcatctggcacttgtcagttgatttgatttccacaccattctttaaccatttgtaagagatgccttcatagttcactgtcacctcaaaagtaatagtgtctttttcttcagcgttgatgtctttcagcatggaagtaatcatgattggggtgactgtcagggtggcactgacttggtcattgccacagacaaatgtgtattctgccgagtcctctgtgctggtgttcatgatgatcagctgatggagttttccctgcacaactatcttgaacttttcactcatctcaatttccacaccattcttcagccacatggaagggacattgaagtgggacacctcacactcaaaagaggcagttttggtctcaggcacctcgatatttttcatggtttttgtaatatgtaatgtctccacaaacagttttgctttgcattccaattgcccgaccacagctgtgtattccccagcatctgagggggagatgttctgcagcatcagcttgtggactttcctttctgagaccagtctgtgtttgtcacttggcttaatttccacactcttatggaaccattttactggaacagtgtcatgggaaacactaacttcaaaggcaacagtggcattttccaaggctgtcacatcctttggctttttaatgatcttgacagtctccacgtgcagtctggcactggctccaagccttccaagcctgaagccataaacagactcatccacgatggcacagtttttaatcctcagagagtaaattgttcctttgacagagatagcatacttttcattggattccagcacaactccatttttgatccactggacacctttgacattagggtgtgtaagctcgacagtgaaaacagcatcctgtgtttctgtcactgtgaggttcttcagagtcttcttaattttgacagcttcaactttgagtttggcagatgttttggaggtggccaccttgtaggtatattctccaatgtcatctaatttggtggcagcaatgataagtctccttttgtggccatcagactcacttctgatgttgttagtcagtggtaggtgtttgccatccctcaaccattcgcctttggaatctgggttggcaacttcacattcaaacacagcttcctgggattcagctacggtctgatctgtgagtggcttggagatggccccacctgccacagtaagttttccagatgtcatattttctcccgcgtaaaatgtgtattttccttcatcatctttcatcatatttagaactgtcaatttatatatttttccatgtgcttcaattttatatttagaactgggcttgatttccttgtccttaaaattccacaggacatcaattccagagtgggacagctcaacctcaaacaccacattttgagtttctgtacaggtaaggtcacgaagacctctgataattttaattttttctacagagagattacagttggtttcaactctgccaactatcagcttgtaaggtccttcgtctgaagcatgagttcggttaatgactagtcgctgtttagtacctttcacaatggcctgtacacggtcatcaggcttgatttgttcatcatttaagtaccacttaacagaagtcacatcagggactgacaccttacattcaagcacagccttggtgccttcaatcacattaacatcttttagaggtgttatcacgtccacactatagacagagacacgcccactggtggagaggccaagggctggaatggtgaaagagtaatttccagcatcttccttagtcatgtcttcaatgagcagcatatgagattgtttgtctatcacaatgtgaaccctgtcactgggctgcacttcttggccgtctttcatccagacgccttccacactttccaaggagactttaacttcaagctgaacaatgtcaccctcacagactttttggtcactaagtccttgtaggatagcaatggggcggggtttcatctttaatttacaggttgtctttttcccgtcgatgacaaagctgtattctccctggtcctccttggttacatccttgaccgtgaggttctgacgtccacgacgagatgtaattgtatatttgccattggatttaagctccacatcattatgataccattttccttctatattttctggggatacaatgcactctaattctcctgaatatgattctggaacttctatgtcctgaagttctttcacaaactcaacaactgcaccttcaacaataagtttagcagtcgttttgacattttcatcttccacaagtacacagctgtaatcttcagcatcagacgtatcaatggtcagtatggagaggaagtgaacctttctgtcagagtgcatcctgtatttatctccctcatgaacctccataccatctttataccatttcactttgacaaatggttctgaagtttcacattcaaaggttgccatagtgtctttttccttagcaacaacatcttgtaattcctgtgtgaaagtgatcaattgcttggcttggacaagtaagaatgcgtgactggaggtttctccagctatgttgatggcttttaccatgatgctggcagagtcctcagcagtcacatctcttatgaccaattcacaaacattgtcttcgggccagtaccagtagatccggtcagaccgttcaattttgacaccatttttgtaccattcacattcggggtctggtttccccacgactctgacccggaagtgtgcatcagatccttggcccactgtttggctctggattctttcgaagatttttggagcctccatactaggacttagttcaatcttgtcaggtttaaaagttggaatcgtgattttgccttcttcggcaagagctttcttttcctcttcagttaactctttggtccagtggagaagttcatcttttgtcttcctgaggagttcctcataggattcatccttctttcgagacttgagctccacagcggtaatggcttcataatagccctcttctgttctgcgcttgaatttactgcgcagctcttccgactcttcaggcactttttcatgggtaattctttcagcccttttcaacttcacaacttctttggtttcagtggtgtcaacaggtctatccactttttgtacttcaaactgaagctttcctggttcatgtacgtgaaactcaggccttggttcaggagctctcctaaggacagacctaaaatcttccctctgttgaatctcaagcttcactttatgctctatcacaccttcaggattttccgcggtgaccttcacttcacctgtgtcatatgatttgcagtccacgatgtccaggtaatggataccatcatagcgaactctgaaccttttgcttttgcggatgagctgtccattgaggtaccagttgactttgggctgagggtagcctgttaccctgcagcggaaccttgcagtctccccttcaagtactctaactggctctgggtacaagacaatgtctggcttttgcttttctttctgatctgttgttacacctgtaagtgcaccttcatgagccattctctctaattcttcaattctctgtaagcctttcctcccctcaggcaattgggattcttccacaagacttttctcatctttaacaataagggtagcagatgtgtgatctgttccatatttgttagtggctctgcaagtaatgataccactgtctctagaatatgcaacgccataatcaaggctgcagtacccaaattcattgatcatacggagcctgttggctgcttcaagtggctttccatcatggagccactccaccaccatcgttgggtcaccaatgggtgttagcctgcattcaaagtgggcaggcccaaagcgcttaagtcttaaggaagtgagttttttcttgaaaaatggtttctgttgtttctctttgtcatagagatcaccttcttcccattgctcttggccatatcgcaaatggaggggctccagttctggggctgcaatctcctttgctctatatgtcccccgtgggatgattaactttctctctggctcaggctctgcaaactcaacttcaacatttactttgcatcttgtagtgtctctgccagctttattaatagcagtcgcagtataccaggcagaatcttggctgacagtggaatcgattttaagggcagcttctcccttggttccttcaattctgattttgggatatttatgaggcacaatgatgtcactgtttttcaaccatacaatgtcagggttggggttacccgtagctctgactttcatttcaagtcgggaaccttcctttatattgacatttttcagtttttctacaaacatcggttttacctgatgttccacagcttccacagttaaaatcactgaaattgaagatctgcctgccctgttttgggcaaccacagtccattccccagaatcactgggtgtggcagggacaataattagtgattgagtaccatcttctttaatgactactttatgggtatagtcattgacaatttgctggccatcatgaaaccagaacgtctctggcataggtctaccaacaacctttaagtcaaatctggcagtttgcccttctaaacatttgaaagaaacaggttttaacacaaagactggtttatatagtctctcaagttgtgactcatctgtctcctccagcctacgtccaggggacattcttgcaggggacatccgtgcaggagacatccttgcaggtgacatccgtgcaggagacatgcgtataggagacctgctcactgaacgtggagagagagatctgattctgctcactggctctagtgtgggaatgtaagtcggagctccaagtggtgcagcaggctccacatacaatttccctgagcaaattgcatttcctttaatattgctggcaaatgcagtgtagattccttcatcttctggaagaacaacaggtatacgcagactagctctgccatcttgtagaaagtccatttggtatctttctccatgtttgatgcgcttgccatctttgtaccaagcaatctttggtaatggatatccagacatcttgcaatgaaaagtgacacccatcccctcaagaattctataattcttgattcttgaatcaaatcctgattcaacagcttcagattcagaaatgtcaactgccatcttttcttctccatcttcttcaagaagttcttctaatgtagtctttattattctatattcaatttctttaataagtctctcttcaaaggaagaaatatggaattcctgatcttctacataagttctgaccactacagtatctttggccattttcttcctaattaaggcttgttctttttcatactctttttcatactcagagtatacaaatccaggtgctgtttctccaactttaggttcttgaacaaatgcagtcacttgtgtctgataaagcatttcttgctgggacttcatcagtaactcataatcagcttcttcaagcaaggaagcagatgcagaagtttctccatgcttattgcgaacaacaatagtgtattctccagcatcatcagcaaaagtcatagaaatcaccagcttgcattcaccggtttgtttgttgtaactcactttgtatctgtatccagtggttagaggaacaccagattttttccagtatacatggggctttgggttgccgccaacttggcatccaaacaccacgctcccaccttccaccagtttctggaccactggttttgtaataaagtaaggcgcggcaggttctccaggccctgcttgttcctctgtgaggctagtatcagtcataaccacatctcttgactcaacaaagcgtttctcttctgtagtaaatttctcagtcacggctgtggtttccttttcaaattcttctgacacctgcacagccagatagcaggatgtgctgacggttccagcctcatttacagcactgcaagtaaatcgcccgctgtcttccgcaaatgcttcgcgaatcataagacgagcaattccactctggaaggttatctggaagtcaatggaactttcgatttggtagtcttccctgtaccatgtcactgtcggggatgggtatccagagatgtggcactccaaggtgacagattcaccttctatgacagtcacattttttaagcccgagaccaaagttggtggagtaacaggaatttcaacaggtgctggtactcttgctgtttctgttaccttggcttcgcgtccgtgcagtacttcaaagcgctcttcacggacggtggtgccagtgatgctcacccctacttcctttttcacctcaacgccagcttcactcttgtaagtatctggtgtgtcagcgaaggggaactgtggcaagggtgtgggctctgcccttactctagtctcactgggcttcacagtaggagccttcaccgatttggtgatcttctgagcagaagatgtggctgacaactctttttgtaatgtggcaatagcactaccggctattgatgcctcatatccatgttctgtcttaggaacagaaatttttgaaacagtaaagtgagggctagctgtgcgggggcgtttatccacatggactaatctttccgttgttagatctgtagttttcttgatctgtgatgatatgtgcattcccttttgatcagtagttttgatatgagtctcagaaggagcctggattactctaggcttgactgctttagggacaacgtggggttctgaggctggacgttggggaggctcagctacctttgcggcggaaatgcgttccttatatccgtactccaaagtggtctgctgagcataggattcttcaagatgcccaggctctctgggctctctgactcgggcctggtctactgcagcaacaactgttgctacagcttcagccttttttccaacgtccacctttccatgggtaacttggatttgttcttgtctagtagccatagtttctctagttctcagtattgtttcttgttctttggctttagcagtagcaactgctattgtagacaaggcagttttctcggcttcctttctcatcttctcctgagttatttgcacttgttctcttttggtagtaatgccttctctacctcttgatactaaatcttgttctttgactttgggtgtggcaactatgactttaggtacaactgttttcctagtttccttcattatcttttcataacttaggtgcatttgatcttgttgtgtggtagtttcttcttgagctcccgggactgtttctagttttgtggactttgcagtggcaactaccaccatggatgcagcagttatctcagtttcctgtcttattgcttcttgagttacttgtttctgtttcttagtaatttcttcagaaattctagtttcttgttctttggctttagctgcggaaattactacctttggtacaaatgttttttcagtttcttttcttatctgctcatgagttacgtgcatctgctcttgctttgtggtaattacttctttggttcttgattttaattcttgttccttggctttatcggcggccactactaccttagttacagcagtcttctccgcttcctttcttacctgctgttcttgagcaggttggatgtgcacagcagtcgtggttgtcctctgagcagtctgctctacagcgctgatcactggttctctcactctggccatatcaacggcagcaacaacagtcgcaacagctgcacttttgtcagcatcttgtttcacctctttagcaccagtggcaacagcctctgctgcgtagctagcactggccgacacactggcggcagcacccgcagcaccactgatggtcacttgctcctggacaccgtatctcccttcccatctctcttctgtcctgatctgagtagaggttgtcagcgttgtctctctcatctcagcctcagatgaggaggccacgtagccctcttgcttccaagggggaggcacttcaggacctgtggccacggtggatgcctgagtcttacgcatgagcaatggagacctaacagacctgatgggggatgtggagattcttgctgctggagacacggacctgaccggagatggggtcggtgcccgcacgtgtctgaccggggaaggggagtgtcttatgggcgatggggactgctgccgagccagctgtgctttggcagcaatagacggtggtgttggggatcttgactttggcttcggaggaatcctgggaggtgttttatgtggcagctgttgcccagcggcaccatctatgaccatctcaactgttgcaattgatctggcatcaaagtgggcttcaatcttcttttcaattcgggtttgtcttgattctgagatctgagcagtcgaaacaattgtctttgtctttttagcaggtacttcttcttcaccttgaaccagtaattcagcagtcgaagtagctcttccaacgctattggtggcatttactgaataggtccctgagtcctcagggtatgcttctgcaatcagtaagctgtagaggtcgccttcttgtgaaatttggaaatcaagggagctctggatttcggctccatcccggtagaacttcaccacaggtgtagggattccagtcactctcacttggagtctcacttggcttccttgtctcacggtcatgctctgcagtcgttgaacgaagttgggtggtgctgtctcagctttcacgagaagctcagcagtactagtcgcttgtccagatccattggtggctttcagggaatatcgtccactgttggctttagtcacggcggggatcgtcagtttagcgcggccatcgctaaaggagatctgcacgccgggcagagtggaagtggaaatcacctggccatccctaaaccagctcacctcaggaactggaaaaccactaatgtgagcctcaaaggttgcggtactaccctccagtaccacaacgctttgtaacggctgcgtaaacgtcggtgcttgagttgtcatctttctaggcactctgatttctcaagagtgcctaaaaagggtgggactaagcccaaggttgcttctgaaacgacgtcctatggagagttggtttttctgaccatctccgacatgaatcggtgagcctctaatcctaaaaacaaaactacacagtcaagactgtgtagttttgcttttctatgcaatccctacacccgaggcgaggctgggaatgcacgactgctc

SEQ ID NO: 9838 - RNA, 20417 nt, Homo sapiens
  source 1..20417: mol_type = other RNA
caaaaactgcagttacttttgccaacactgtttttcacttcaaagctatataatcctttgtcactcatttcggcacaggggattttaagggaagccactttattgatgaatgtaatgtgatgtttgctgtctgcagacaattctcttccatctttgaaccacttggctgagagttctggtgttccagtcactacacactctaatgcaaaaggatttccagtagtgacagtcatgggttcgggcttctctatgattcttgctggttctagtacagtcaagactgcagagcattctctcattccagcatcgtttttgatttggcatatatattttccagaattagatgcttctggactccccagctggagggttgcaatgttatcaatgaatgaaatcctggtattttcactctctctgatgacttcacctctatctttcagccagacaacagaaattggctggaagccctccactatggcccgtaactcaacagcatccccaataagggttgaggtgtcacttagctttttcacgaatcgtggaggttctttgaacttgacagagcaagaacacgtgtcacttcccacctcattagtagctttgcagtgatattccccgacatcggaggcttcaagattaaggatatgaagacttgtatcaaaatgttttgaagtgattttaaatttcttgctgtttctaacctgctttcgatctttaacccatactacttcaaatgggggagttcccgaaatttcacattggagaatcacatcagaacctttaagagctcctactggagaaggcttctgggtgaaaacaggaggtgctttcactgtcaacgctgtgctgcagctggcgtcaccaacaccattatgagcctcacaaatgtagtccccgctgtcttcagcactagcttcattgatcgtaagcaatgccacagaattaatgaatgacatgttgtatttccaactttcatgaagttcgctgtcatttcggaaccatgaaactttgatttctggggagccacttattttacattccagttgaatggattctccctgctttgcaacttttgaagcttctaatttcttaacaaactttggaggttcttttacactgagctgagctgagcacatgtctttgccaacatcattggttgcttggcaagtatattgaccagagtctcctttgcctactttaagaattctcaaatgaggagtgtttcccacacatgtgattgtatagtttcctccaggacggatctccttgttatcttttgaccaagtgattcgcatcggttgagcaccagtaacatgacactcaaaatcagcactttctccagcaataacatctatagatacaggcttgatgtcaaagaagggagatttcttgggttctcttgctgtgagtctagcactagaagatgctgttccaagtgggttggaagctgagcaagagtactggccagagtgactcaagtcagtttgcaaaatttttaaagttgccacattatctacaaatgaagtctgtagattttcatcgtctcttaaaagtactccatctctataccagcacacttggatgggtgcagagccatttaatcgacaagtgagtgtaacaggtaaccccacagtttgttcaatgtcctttaattgtcttgcaaaagaaggtgggagttggcgctcttgaattctgaacacagtcttagaagaagcagttcctatactattttctgctttgcatgtgtactctccactgtcattgatgttcactttattaaaaacaagtgtggccacattgtttgtaaagtaggtcctgtattcaggagttggccgtaatttggtatctcctttgtaccaagacactgtaatttctggtgtcccagcaacttggcattgtaaagaaaccgaatctccaactgctgcctccagaggttccagttccgtaacaaaataaggcggttctaatgtagataccagagctccacaaacatcccttcctgcctcattttcaatctcgcaggaatactgccctgcatctctttttgtgctattcagaatttccaggatacaagttttctctgttgtgactatgttacatttttcagaggtagttatgttaaaaccatcctttttccaagtgacagaaattggaagtgttccagtgtaggtgctctccagaattatggacttccctggttctacagaatgatcacttaatctcttcaaaaatgcagctggttctttcacaaagagacgggtagtgcaagatgcttggccagcgttgttagaaaccacacaggtgtattccccactctgagatatgtcaatattaaataattccagttctgccacagtgtcttcaaaatagatgttgcaccggtctcctttcactagttctctggcacctctgaaccagttgactttgaatggaggggttcctctaataacgcttgtgaaggttacatttttgcctggtagtacttccaaaggttcaggttctttcacaaaagagggtggttcttgtacagttagcactgcacgacattcatcagacccagcgacattagcagccacgcatgtgtaattgcccatatctgaggaatccagagaattcaactgcaatgtgcagacattatctgaaaatgtggtttggtactttgctccactgacaatcttggttttctcatgaaaccaggcaactgaaataggtgatgatccagctactttgcattccaagatgcaagaagcacctaacaccccaccagtatttttcagtcttcgtgtgaaagagggaggaactgctcggtctgaaacatcaaccacagctgtgcagctgcttttcccaacattattttgaacctggaaagtgtatgtgcctgcatcttgcctttcaactgagagaatccttaaggaagagattttgttgtagaagctaaatttgtgtttttggctgctggtcaacagctttccatccttgtaccattcaacagagagttccggagtgccagccaccttacactccagagtgcacgtttctcctacagtcaccgtcatcggtcctgccttctcaacaatgactgcgggctctaagaccatcagtgtggccatgttctccctcattccaccatcattcttgatttggcagatatactttccagcattagctggctctgcttttgcaaactgtagagttgcaacattttccacaaatgtaatcctgatgttttcactttctctaatcacttcttccttctctttaagccactggacaaaaataggctgggcgccttctatggatgcttgtaattcagcaggctctccggctacaacagtgaggctgttcagtttggagacaaatcttggtggttctttcaattttacagtacaaacacaagtatcacttcccacttcattctgtgctttgcagtggtattcaccgatgtctgaagtgtccacattgagaatgtgaatacttgtgtggaagtttttggatgcaatcttgtatttcttgctgcttctgagttgccgcttgtctttgtaccataccacctcaaacggtggtgttcccgaaagttcacattcaagactgacttcagcatttttaagggtttctactataggagggaagctgctaaaaacaggtggctcttttactataaccttggtactgcagcttgtgctgccagcgggattctgagcctcacaaatgaaatctccactgtcctcagtactgagattgttcatctgtatgacggccactgagtcaatgaaagtcattctgtacttatcactggctggaagttcatgttcatttcggaaccacacaactctgatttctggggatccagctatcttgcattcaagtcgtgaagagtcacctgctttcacaattttggaggcttctaatttctttacaaactttggtggttctgtcacaagcaacatcgtagtacaagagtcgctaccaacatcattggtaacatggcaagtatactgtccagtcttagaagcatccactgagtagagatttaagaagctagtcgacccttccaagccaatgaaacatttaggacctgagacaagttccacatcatccttaaaccattttattttaaatggtggtgttccttttagtattgccttaaattccactgtagaatcaggtatggcttgctgtcgcccaggtttcactaggaagcttggtggttctttcacagttaagatgccactgcatgcatcatctcctgctacatttgacactttgcatgtgtaatttgcagtatcttctaattccagattattaacttccagagacacagatctctcatggcacacaagtctgtattttgcacttgtagatatttcttttccatccttaaaccactgagcactaatgggaagtgaaccagacaccttgcactccatatgaatagaagagcccagaactttatccattttggttaattttttggtgaatgatggaggaatattttgatctagcactcttaagtaggcatcacagctactgcttccgaagtcattttccaccttgaaagtgtactgaccgctgtcctgcttcattactgactgaattctaaaactggccacgttattttcaaaactcattgaaaagtatctactgggaactatttgtttcccgtctttaagccatttcactttgagttctggtgttccagccacaacacattccaaggtcatgggatctttctccgtaacatcaactgatttagctttctctacgatttgagctggttcttgtactaaaaggaaagcataacacctctcaactcctgactcattcttggcttgacaggtatatctcccactgtgtccattatccacacttctgatttgaagtgtggccacactgtccacaaatgaaatatagacattatcatcttcatcaagaatctgatcatcctttagccaggttatagaaataggaggagaacctgccacggtactctgaaaggtggcagaacttttcaaaacagtagtggtattttctatcttcttaatgaatgatggtggttctttcagggcaactctagtactgcatgagcagctgccgccttcattggatacaatgcactggtattccccagtgtctgaagggtcacacttggttatatggaggttaaacacagacactctgtcggtcaatgtgtattttttgctgcttcgaatttccctgttattcttcagccaagtgacttcaaacggaggtgttcccgtaacttcacactccagctccacgtcactatattttactacctccacaggcttcagctctctgataaaggtggggggttctttcactttgagttcaatgctgcagctcgccgtgcctgcgtcatttcgagcttcacacacataagtcccactattttctaccctggcaccagaaatctggaaagtggctaaaccatcaatgaaggaaatgccatgtttctgaatggctgttatttcattcccgtctagataccaagacactcggattttaggagtgcctgttatttggcattcaaatgttgttgactgtccattcctcagcactaagactggactgggcttcttaatgaattgaggaggttcttttacaaagagagtggctttgctggttgctgtgccaacatcattgcttagttggcaaatgtaggttccagaatcggtagctttggctgcaaagagctctagactggtagaggtgtcatccttccaaactgagcgggctgctcctgagtgtaactctttgttatctttaaaccactttattgtcatgggtgcagtgccacccacaagagcctttaactgtacccttgtgttgggattgacatcttgtgactgtggcttttccacaaagtaagggggttctttgactgtcagatgcccactgcattggttgtgccctgccttatttgtggcagaacaagtgtatgtcccactgtctgtaccttccagctggctgatttccaagaaggcagtattgtcatgaaaagagaatttgtacttttcactagctgatatttcttggtcatctttgaaccactggatgcttatgggatgtgacccagccactatacattctaaatcaatgaaagaacctttaatgctgtccattttcttcagctttttggtgaatgaaggaggtatgataagatctaatacattaattctagccttgcagctgctcctcccaacatcattttggacctcgaaagtatattctccactatctttcttttctgtagaaataatcttcagtattgagactgtatcagtgacactgattttatattttgagcccagggtcagttcttggccatctttaaaccatttggctgtaatctccttagtccctgaaaatttaacctgcaaagtggctgggtctccttgggtgacatctatagacacagcttcctcggtgattgttgcaggttcttttactgagagtaatgcagaacatctttgtattcctgcatcatttttggcctgacagacatatttcccatcatgcttgacttcaatgccactgaggtacaaactggccacattgttctcaaaggtcattcttatattatcgtcttcagtgatttcatcgctgtcttttagccaagtcaccgtaattggcaaggagcccttcagagtggcctggaaggcagctgtgcctccccggagggagctggtactctcgatcttctttatgaaggatgggggttctcttaaagtcaccctggcactgcagatgctgctgcccacctcattggtcacccgacactggtattcgccagcatctgcagctacaaacttgaggatctgcaggctaaccagatgatcctgaatgaaagtcttatactttctaccacttcgcaggattgtgttatctttgaaccaagtgatctcaaagggaggagtgcctgccacctcagccagcaacatgacatcgtactcctttaagacttcaattggcttaaattccttggtaaaataaggtgactctttgactattacaatgctactgcagtggtcactgccagcctcattttgggcctcacacatatattcaccactgtcttcgatgccaacatctgtcagtcttagaactgcagtagactccacaaaagacattctgtgtttgctgctctccttaatttctctatcatttgcaaaccatgttattttaattggaggggtaccagttactttgcaggctagctgggtggcatctcccttctttaacagctgtgatggctctaacttttcaacaaatgtggcaggttcttttacaaacaagtttgcactgcattccacccctccagcgacattgctgactttacatgtgtacgtgcccgaatcagaggtttttactaaatagagttccagggaactctctaaagcttctttggtaatatagcagcttccaccagaaaccagctctttgttgcccttaaaccatctgattgtgagaggagtagatccttggaaagtgctcttcaggcagactgctgagccaggcagaacatcctttgagccgggtttagttacaaaactgggtggttcttgcacaatcagggctccactgctgtctttgcttcccacggaatttgtggctcgacaagtgaaattccctgcatcattcatgtctactctgatgatctccaaagaggctgtgccttccacaaatgctatcctgtatctgtcagaagcagctatttctttgccatccttaaaccaggacaccctcatggggagggagcctgcaattttgcagtccagtctgcaggtaccattaacaacactatccacgttgcgcaagggtttggtaaaaaatggagcaatgtctcgatctaatacagtgaatgtagtctcacaggagctgctgcccacttcattggaaatctcaaatgtgtattggccactgtcgtgcagctcagctgaataaaatttgagctgggcaacattgtttttaaaacttattcggtattttttactggcgaccaagggtctcccatctttgtaccatttgggcttcagttctggcgtgcctgccactgtgtactccagtgtggcgggatctcctgctgtcacctggatcagttctgctcgctcaatgattttggcaggttctttaactattaattccccaacagatgtttggcttccagcttcattttcagccaggcacgtgtatttgcctccaaaactaatctgaacatcagggattatcaagactgcaacaccattggaaaagctcattttgatttttccgtcttctctgatgacctcttgacctttcatccatgtgacagaaatgggctctgaccctctcacagcagcttgcagggtaacggtttgtcctcctagtgcaatcaaatcatctactttctttacaaaggttggaggttctttgagtaagtgggttgccatgcagccacacttgccgacttcattagcaacaacacattcatattcaccaacatctgcactattaaacgaaaagatctccagacacacaagagacttctgagaaaacaatctgtattttttactacttcgaatttgtttcttgtctttgaaccagctaatttcaaatggtccagtgcctgagacttcacactgaagtagagcatttgttcctctcactatgtctgcaggctcaagagttttgatgaaagaaggaggttctttgataactatttcagtactgcagctatcactgccgacgtcattcactgcttcacatgagtaactcccactgtcttcaacttttacatccgtaatatcaagtatagcctcagaattgacaaaatacattcggactgtgttactttcactgagttctttgttatttttaaaccaagtaacctggatcacaggtgagcctttcagcttgcaatggaggcgtgctgattcacctgggagcattaaataagagggatccaccttcttcacgaaggatggtggctctctgacagtgactgtggctgagcaggagctgcttccagcctcatttgaagctgtacagacataggttcctgaatctttcagtttggccaaaggaatctcaagtgttgctattttatcttcaaaacagatcttataatctttccctggggggagtttttgcccatctttgctccacgtaactgtgacttttctgtcttcatctacttggcactcaaggtggaccttcttattgatagcggactgcacaggctctaattctttaatgaaatgtggcttatcaatgatgatcaactctgcttggcagatgtctgctccaaacttgttggaagccttacaagaataaactcctctatcttgaatggtaaggtttgagagttctaaaatgtgtttgttttctgcgtcggaaatcctccagttaggtgaaggtgagagtgcagcaccatctttctgccaaatggtttctatcacaggagtccctgtcactgtgcagatgaacttggctgccttacccacaaaagttgtaagggacttaggtctggagagaaaggttggtggatatgcctctgtcacagttagtgtggctgtacagctgacactgccatactcattggaagctttgcatgtatactcgccgcagtcaaccacctgggttctcaggatttcaaggctggagatatactttgaagatcgaatagaacacttgtcactctcataaatttctcggccagctttaaaccactggaaccggacattgggagcactttggatctcacaggtgaatttggctaggtggcccagtgctacttccaggggttcgattttcctcttgatcactggggcagctttcatttccatctcaatctcttgttcaatcctctcatgcaaaattgattcaggagcttccagactcaggttggctgtgcttgatacttggcctacagcattactagcaacaaacgtgtaagttccttcatcttctggataagcttcggcaatttccagttgataagtgtcttcaaattgagtcattctaaagaaccgagatggcttgattttcttgtctttgctgtaccacgacacttttagatctgttccagaaacccggcattgaaaacgggctggctgcccttcagaagtgacagtgtcctgaagcggggtgatgatggcaggtggataaacaggcatttcctgatcaggagacacaacttctggaacttccactgagagtgaagctgatgttgtggcaacaccatagtcattcttggcttcacaggtatagactgccgcatcctctgggaaggcttcaattagcaaaagcgtgtattcttgcccatcatgaagaaatttgcacttgaagccagtggaaagcagctgctcttccttgtaccaggaaattttgggctgtggtcttccggatatcacggcacagaagcgggcaggcttgccagactgcacagtgacaggctggagctcctgcagaacttggggcggttcaggagcattgacatagagagtgacagaactcctgttccttcctgccacaaaggtgtattctcctgcatcgctctgtctggtctcagagataaacattcggtggattcttctttccactacatatttgtgtcgttcttgaacttggaaattgatttcaatgccatctttataccagtgggcatcaacatcgtcttcattgacctcaaattcaacaacagcacgctgtttctcaatgacctgaacctcctttttaatacttcggatgcgaacatctctgccttctacaaagagttttgcagttgacacgttgcctcctgccaccactgtgtacttcccagcatcagacatccgggtggatgggatcagaaggcggtggacatatttctccttctgaatctttattctgtctgtgatctgcagttcctggtcatctttcatccactgtacagtgatgtcaggttcagaaacttcacattcaaacatggctcgcttcttctccagtaccttaatgtccttaatgtgtttcctaaattctatatgacgagcttccacataaagtgtggctgttgatgttgcttttccagccacaaaggtgtagtcagcagcatccccaaagtgaacattcctgatgttcagtgagtgtgtgagctttttggttctcatctggcacttgtcagttgatttgatttccacaccattctttaaccatttgtaagagatgccttcatagttcactgtcacctcaaaagtaatagtgtctttttcttcagcgttgatgtctttcagcatggaagtaatcatgattggggtgactgtcagggtggcactgacttggtcattgccacagacaaatgtgtattctgccgagtcctctgtgctggtgttcatgatgatcagctgatggagttttccctgcacaactatcttgaacttttcactcatctcaatttccacaccattcttcagccacatggaagggacattgaagtgggacacctcacactcaaaagaggcagttttggtctcaggcacctcgatatttttcatggtttttgtaatatgtaatgtctccacaaacagttttgctttgcattccaattgcccgaccacagctgtgtattccccagcatctgagggggagatgttctgcagcatcagcttgtggactttcctttctgagaccagtctgtgtttgtcacttggcttaatttccacactcttatggaaccattttactggaacagtgtcatgggaaacactaacttcaaaggcaacagtggcattttccaaggctgtcacatcctttggctttttaatgatcttgacagtctccacgtgcagtctggcactggctccaagccttccaagcctgaagccataaacagactcatccacgatggcacagtttttaatcctcagagagtaaattgttcctttgacagagatagcatacttttcattggattccagcacaactccatttttgatccactggacacctttgacattagggtgtgtaagctcgacagtgaaaacagcatcctgtgtttctgtcactgtgaggttcttcagagtcttcttaattttgacagcttcaactttgagtttggcagatgttttggaggtggccaccttgtaggtatattctccaatgtcatctaatttggtggcagcaatgataagtctccttttgtggccatcagactcacttctgatgttgttagtcagtggtaggtgtttgccatccctcaaccattcgcctttggaatctgggttggcaacttcacattcaaacacagcttcctgggattcagctacggtctgatctgtgagtggcttggagatggccccacctgccacagtaagttttccagatgtcatattttctcccgcgtaaaatgtgtattttccttcatcatctttcatcatatttagaactgtcaatttatatatttttccatgtgcttcaattttatatttagaactgggcttgatttccttgtccttaaaattccacaggacatcaattccagagtgggacagctcaacctcaaacaccacattttgagtttctgtacaggtaaggtcacgaagacctctgataattttaattttttctacagagagattacagttggtttcaactctgccaactatcagcttgtaaggtccttcgtctgaagcatgagttcggttaatgactagtcgctgtttagtacctttcacaatggcctgtacacggtcatcaggcttgatttgttcatcatttaagtaccacttaacagaagtcacatcagggactgacaccttacattcaagcacagccttggtgccttcaatcacattaacatcttttagaggtgttatcacgtccacactatagacagagacacgcccactggtggagaggccaagggctggaatggtgaaagagtaatttccagcatcttccttagtcatgtcttcaatgagcagcatatgagattgtttgtctatcacaatgtgaaccctgtcactgggctgcacttcttggccgtctttcatccagacgccttccacactttccaaggagactttaacttcaagctgaacaatgtcaccctcacagactttttggtcactaagtccttgtaggatagcaatggggcggggtttcatctttaatttacaggttgtctttttcccgtcgatgacaaagctgtattctccctggtcctccttggttacatccttgaccgtgaggttctgacgtccacgacgagatgtaattgtatatttgccattggatttaagctccacatcattatgataccattttccttctatattttctggggatacaatgcactctaattctcctgaatatgattctggaacttctatgtcctgaagttctttcacaaactcaacaactgcaccttcaacaataagtttagcagtcgttttgacattttcatcttccacaagtacacagctgtaatcttcagcatcagacgtatcaatggtcagtatggagaggaagtgaacctttctgtcagagtgcatcctgtatttatctccctcatgaacctccataccatctttataccatttcactttgacaaatggttctgaagtttcacattcaaaggttgccatagtgtctttttccttagcaacaacatcttgtaattcctgtgtgaaagtgatcaattgcttggcttggacaagtaagaatgcgtgactggaggtttctccagctatgttgatggcttttaccatgatgctggcagagtcctcagcagtcacatctcttatgaccaattcacaaacattgtcttcgggccagtaccagtagatccggtcagaccgttcaattttgacaccatttttgtaccattcacattcggggtctggtttccccacgactctgacccggaagtgtgcatcagatccttggcccactgtttggctctggattctttcgaagatttttggagcctccatactaggacttagttcaatcttgtcaggtttaaaagttggaatcgtgattttgccttcttcggcaagagctttcttttcctcttcagttaactctttggtccagtggagaagttcatcttttgtcttcctgaggagttcctcataggattcatccttctttcgagacttgagctccacagcggtaatggcttcataatagccctcttctgttctgcgcttgaatttactgcgcagctcttccgactcttcaggcactttttcatgggtaattctttcagcccttttcaacttcacaacttctttggtttcagtggtgtcaacaggtctatccactttttgtacttcaaactgaagctttcctggttcatgtacgtgaaactcaggccttggttcaggagctctcctaaggacagacctaaaatcttccctctgttgaatctcaagcttcactttatgctctatcacaccttcaggattttccgcggtgaccttcacttcacctgtgtcatatgatttgcagtccacgatgtccaggtaatggataccatcatagcgaactctgaaccttttgcttttgcggatgagctgtccattgaggtaccagttgactttgggctgagggtagcctgttaccctgcagcggaaccttgcagtctccccttcaagtactctaactggctctgggtacaagacaatgtctggcttttgcttttctttctgatctgttgttacacctgtaagtgcaccttcatgagccattctctctaattcttcaattctctgtaagcctttcctcccctcaggcaattgggattcttccacaagacttttctcatctttaacaataagggtagcagatgtgtgatctgttccatatttgttagtggctctgcaagtaatgataccactgtctctagaatatgcaacgccataatcaaggctgcagtacccaaattcattgatcatacggagcctgttggctgcttcaagtggctttccatcatggagccactccaccaccatcgttgggtcaccaatgggtgttagcctgcattcaaagtgggcaggcccaaagcgcttaagtcttaaggaagtgagttttttcttgaaaaatggtttctgttgtttctctttgtcatagagatcaccttcttcccattgctcttggccatatcgcaaatggaggggctccagttctggggctgcaatctcctttgctctatatgtcccccgtgggatgattaactttctctctggctcaggctctgcaaactcaacttcaacatttactttgcatcttgtagtgtctctgccagctttattaatagcagtcgcagtataccaggcagaatcttggctgacagtggaatcgattttaagggcagcttctcccttggttccttcaattctgattttgggatatttatgaggcacaatgatgtcactgtttttcaaccatacaatgtcagggttggggttacccgtagctctgactttcatttcaagtcgggaaccttcctttatattgacatttttcagtttttctacaaacatcggttttacctgatgttccacagcttccacagttaaaatcactgaaattgaagatctgcctgccctgttttgggcaaccacagtccattccccagaatcactgggtgtggcagggacaataattagtgattgagtaccatcttctttaatgactactttatgggtatagtcattgacaatttgctggccatcatgaaaccagaacgtctctggcataggtctaccaacaacctttaagtcaaatctggcagtttgcccttctaaacatttgaaagaaacaggttttaacacaaagactggtttatatagtctctcaagttgtgactcatctgtctcctccagcctacgtccaggggacattcttgcaggggacatccgtgcaggagacatccttgcaggtgacatccgtgcaggagacatgcgtataggagacctgctcactgaacgtggagagagagatctgattctgctcactggctctagtgtgggaatgtaagtcggagctccaagtggtgcagcaggctccacatacaatttccctgagcaaattgcatttcctttaatattgctggcaaatgcagtgtagattccttcatcttctggaagaacaacaggtatacgcagactagctctgccatcttgtagaaagtccatttggtatctttctccatgtttgatgcgcttgccatctttgtaccaagcaatctttggtaatggatatccagacatcttgcaatgaaaagtgacacccatcccctcaagaattctataattcttgattcttgaatcaaatcctgattcaacagcttcagattcagaaatgtcaactgccatcttttcttctccatcttcttcaagaagttcttctaatgtagtctttattattctatattcaatttctttaataagtctctcttcaaaggaagaaatatggaattcctgatcttctacataagttctgaccactacagtatctttggccattttcttcctaattaaggcttgttctttttcatactctttttcatactcagagtatacaaatccaggtgctgtttctccaactttaggttcttgaacaaatgcagtcacttgtgtctgataaagcatttcttgctgggacttcatcagtaactcataatcagcttcttcaagcaaggaagcagatgcagaagtttctccatgcttattgcgaacaacaatagtgtattctccagcatcatcagcaaaagtcatagaaatcaccagcttgcattcaccggtttgtttgttgtaactcactttgtatctgtatccagtggttagaggaacaccagattttttccagtatacatggggctttgggttgccgccaacttggcatccaaacaccacgctcccaccttccaccagtttctggaccactggttttgtaataaagtaaggcgcggcaggttctccaggccctgcttgttcctctgtgaggctagtatcagtcataaccacatctcttgactcaacaaagcgtttctcttctgtagtaaatttctcagtcacggctgtggtttccttttcaaattcttctgacacctgcacagccagatagcaggatgtgctgacggttccagcctcatttacagcactgcaagtaaatcgcccgctgtcttccgcaaatgcttcgcgaatcataagacgagcaattccactctggaaggttatctggaagtcaatggaactttcgatttggtagtcttccctgtaccatgtcactgtcggggatgggtatccagagatgtggcactccaaggtgacagattcaccttctatgacagtcacattttttaagcccgagaccaaagttggtggagtaacaggaatttcaacaggtgctggtactcttgctgtttctgttaccttggcttcgcgtccgtgcagtacttcaaagcgctcttcacggacggtggtgccagtgatgctcacccctacttcctttttcacctcaacgccagcttcactcttgtaagtatctggtgtgtcagcgaaggggaactgtggcaagggtgtgggctctgcccttactctagtctcactgggcttcacagtaggagccttcaccgatttggtgatcttctgagcagaagatgtggctgacaactctttttgtaatgtggcaatagcactaccggctattgatgcctcatatccatgttctgtcttaggaacagaaatttttgaaacagtaaagtgagggctagctgtgcgggggcgtttatccacatggactaatctttccgttgttagatctgtagttttcttgatctgtgatgatatgtgcattcccttttgatcagtagttttgatatgagtctcagaaggagcctggattactctaggcttgactgctttagggacaacgtggggttctgaggctggacgttggggaggctcagctacctttgcggcggaaatgcgttccttatatccgtactccaaagtggtctgctgagcataggattcttcaagatgcccaggctctctgggctctctgactcgggcctggtctactgcagcaacaactgttgctacagcttcagccttttttccaacgtccacctttccatgggtaacttggatttgttcttgtctagtagccatagtttctctagttctcagtattgtttcttgttctttggctttagcagtagcaactgctattgtagacaaggcagttttctcggcttcctttctcatcttctcctgagttatttgcacttgttctcttttggtagtaatgccttctctacctcttgatactaaatcttgttctttgactttgggtgtggcaactatgactttaggtacaactgttttcctagtttccttcattatcttttcataacttaggtgcatttgatcttgttgtgtggtagtttcttcttgagctcccgggactgtttctagttttgtggactttgcagtggcaactaccaccatggatgcagcagttatctcagtttcctgtcttattgcttcttgagttacttgtttctgtttcttagtaatttcttcagaaattctagtttcttgttctttggctttagctgcggaaattactacctttggtacaaatgttttttcagtttcttttcttatctgctcatgagttacgtgcatctgctcttgctttgtggtaattacttctttggttcttgattttaattcttgttccttggctttatcggcggccactactaccttagttacagcagtcttctccgcttcctttcttacctgttcttgagcaggttggatgtgcacagcagtcgtggttgtcctctgagcagtctgctctacagcgctgatcactggttctctcactctggccatatcaacggcagcaacaacagtcgcaacagctgcacttttgtcagcatcttgtttcacctctttagcaccagtggcaacagcctctgctgcgtagctagcactggccgacacactggcggcagcacccgcagcaccactgatggtcacttgctcctggacaccgtatctcccttcccatctctcttctgtcctgatctgagtagaggttgtcagcgttgtctctctcatctcagcctcagatgaggaggccacgtagccctcttgcttccaagggggaggcacttcaggacctgtggccacggtggatgcctgagtcttacgcatgagcaatggagacctaacagacctgatgggggatgtggagattcttgctgctggagacacggacctgaccggagatggggtcggtgcccgcacgtgtctgaccggggaaggggagtgtcttatgggcgatggggactgctgccgagccagctgtgctttggcagcaatagacggtggtgttggggatcttgactttggcttcggaggaatcctgggaggtgttttatgtggcagctgttgcccagcggcaccatctatgaccatctcaactgttgcaattgatctggcatcaaagtgggcttcaatcttcttttcaattcgggtttgtcttgattctgagatctgagcagtcgaaacaattgtctttgtctttttagcaggtacttcttcttcaccttgaaccagtaattcagcagtcgaagtagctcttccaacgctattggtggcatttactgaataggtccctgagtcctcagggtatgcttctgcaatcagtaagctgtagaggtcgccttcttgtgaaatttggaaatcaagggagctctggatttcggctccatcccggtagaacttcaccacaggtgtagggattccagtcactctcacttggagtctcacttggcttccttgtctcacggtcatgctctgcagtcgttgaacgaagttgggtggtgctgtctcagctttcacgagaagctcagcagtactagtcgcttgtccagatccattggtggctttcagggaatatcgtccactgttggctttagtcacggcggggatcgtcagtttagcgcggccatcgctaaaggagatctgcacgccgggcagagtggaagtggaaatcacctggccatccctaaaccagctcacctcaggaactggaaaaccactaatgtgagcctcaaaggttgcggtactaccctccagtaccacaacgctttgtaacggctgcgtaaacgtcggtgcttgagttgtcatctttctaggcactctgatttctcaagagtgcctaaaaagggtgggactaagcccaaggttgcttctgaaacgacgtcctatggagagttggtttttctgaccatctccgacatgaatcggtgagcctctaatcctaaaaacaaaactacacagtcaagactgtgtagttttgcttttctatgcaatccctacacccgaggcgaggctgggaatgcacgactgctc

SEQ ID NO: 9839 - RNA, 4733 nt, Homo sapiens
  source 1..4733: mol_type = other RNA
caaaaatctcaattacttttgcaccaacctaataattttaataatatatataacatttaattacagtgtagaactatcaatgttttcgcagtgtaatttgctgtaatatctattaaatcccatagacttgcagtctataaacatgtatacactctaagtaaaatattaaatgaaattaaattagctactcaattttcctcctacacataatcttctgtacatgccttcattatttgtatagtgttgtgacttccgaaaatatcaggcacattcatattaaaatattagatacaaaatgcattctaaactcaagtaatacttttgagtttatctgagcactgttgctaagttctaatatggagataaatatatacttacacaaaatattttcatatttaggaatatcataaatgaatcccttgatgacaggcttttcttaataataaaaagatacccatggcagaattcgaaagtaattacttgtattataattttttttttgagactcttgtcacccaggctggtgtgcaatggcgcaatctcagctcattgcaacctctgcctcccaggttcaagtgattctcctgcctcagcctcccaagtagctgagactacaggcgcgtgccaccacacccagctaatttttgtatttttagtacagacggtgtttcaccatgttggccaggctagtctcgaactcttggcctcaagtgatccgcctgccaaggcctccgaaactgttggcacttgaggcactgcgctgagccttgtattataatttttttaagttataagtcttgtaagcacctgcagcgttgattgatgaagagagagatgcattgttaaacaagatgccctcaggctttcctttaaggaataaagattaataggacactcagaaaagtaaacacataatgtaagtgtgaataaagtggtgtaattcagattctatgggaactcagaggacagacactcaaatgtctgatgaatgaaggcttgtgtccattttaatttatatattcagcagatcgatcacttttgaatacaatactcctcgatgaaaaagtatagtctgaagtaaccttaagattgtatgtattatttttcacaaatgcaaagttgaaatgattattcccagagggtgagcagggccacagaaaagaataaaacaggaaatttctaaaactgcattgagatacttgtttcttggagacttggtacccgttccaatgcttagcatttatcaagttattatggtttgccagaaaatgtgctcaaaggactctttaccctttaaccctcctaaccctattaatgtagtactagtattatgttcatcttttacatgtggaaacggggacccacagaggttatagaacctacctcaaattagaaagctggaaggcaagcttttaacaactgtgagtaaatcttcttttacagtgtgagaaaaatcctaaaacagagggaaagggagacagggtggcaaggggagaggtatttggtggagcgtagaataacacaacgtcaaattctcttttattttttttagatgggtgtcactctgttgcccagtctggagtgcagtggcatgatcatagctcactgtagccttgacctcctgggctcaagcaatcttcctgccccagcctcctaagtagctgggactatagttgcagatcaccatgcccagctaatttttgtattttttgtagaggtagaatctctccatgttgcccaggctggtctcagactcctggactccagtgatctacctgcctcaacctcccaaagtgctgggattacacgtgtgagccaccacagccggccatatgtcaaattcttaagcttcattcttaagccatatgtctcattcttaatgatttgttatcacagatcattgaagaaactggctacataaatcattactcttgcattatcagcctctcacaaatctctctagcatctgaaaattactatcaaatgaacagtgctgactgttcagagtgtcccaacagggtgaaagcaagttgcatgactctgtatctaattattttataacatcaatatatccatgatatagtatcacataagacactgatacattggctattatatttgtaagccgaacttttaattttaaacagggcttgtactttgattatttatcaaagtatcaaattccacaaataaaatattcttttactttgaaatctctgtcttcactttatggctttttattatgaaactttatcttggtattactgatgtaccttgacttcattatactaaacaacactcatattagtacttcagtactggcaatacagctaagccttaaactgagccaaatatctgttaaagtgaattgctttttatgctgaaatcaatttattgaataaaagtcccttgccacaatggaataaagaatataattccacctttgaaggaacccctaaaactacaattttcaaatttttaaaaagtataatccagccgggcgtggtggctcacacctgtaatcccagcactttggaaggccgaggtgggcagatcacctgaggtcaggagtttgagaccagcctggccaacatggtgaaacctcgtctctactaaaaatacaaaaattagccagcgtggtggcaggtgcctgtattcccagctacttgggaggctgaggcaggagaatcgcttgaacccgggagatacaggttgcagtgagctgagaacgcgccatcgcactccagcctaggggacaagagcgagacatcgtctcaaaaaaaaaaaaaaaagtataacctaaaaattattcaataatttcaagtgtgttttttaaaactaaatttaatcaatcaattcatataatgctatctatataaaagataaaaatcttattcttgggctaacttgatggaaaaggttcttagttttttaaagggctccgttgaagagtattcttagaaaaagcgtggtatacatcagtggtccccaacctttttggcaccagggactagttttgtggaagacaatttttccacagccagggttgggggtggggttgggttctgggatgaaactgtcccacctcagatcatcaggtattagattttcttaaagagcgaaagctagatcccttgcatacgcagttcacaatagggtttgggctcctatgaggatctaatgctgctgctgatctgacaggaggcggaatgcaggcgggaacgctcagtttgaggttcaccacgtgctgtgcggtctgcttgctaacagatcacggaccagtactgggaccatggtccaggggttggggacctcagtatacataactaactaaaattagctgctaacattttctagaaatacctgagagccaacttataagaatattactttacttaaatttagcaccatttgtatatgtaaaaaaaaaaactgatatgctagagttagtaaaaatggcttattctctacaatctagtcatttcctttatagtgcaaacacctacgccccaagaaaaaaagaaggattacaaatgtgcacacaggtatcacaaagaggccttactagatcccatttcctttttaaaatggagacatttcaaaggcagaaaaaatcctgattctggttaggtaattgaagtaaatgtaagagagagtcacgaggatatttttacacaggcccagtacgggtgtgatagtccccagggcaatgattaaaccaagtctaacaaaaacgaatggtaaatcttgcagcaggacgctcagggaattgagaagagggttttggggagtgaatgtaattcgaaggagagaaataaaactgaatatgtagactgggtatagccagcttgacttgtacacgttggggtgaccagccacacgcaccatttctatcgtgtcagaccacaggagaaagctccataagaataactctgcccggacatctcgccgggacatcattctcaggattccggagtcacaggagggctcctggggtcccatgaacacagactcctggctccgtgtcatggctcctgatggctgcgacacctgggtgctgttggttgcctggggagatgcagcgttttctggactttgcctcacttgctccgtcacagtttttatgtgttgcaaagaggttgaatggatgtgtccattttcactactcttttgactccctctaagaggatatatcctgagtttttcaataatatcaaccatgatcagggataacagaaccagagatacgggcaggtcaggtaacatatcaggtaagacatcagcggacccattaatgctcttttgaacctcagtcactgctatggaaaaggtgaggcagggcagtgtggtgaggaccacacacatcatcagaacaggtctccatcctttaatttttctgtaaatataacgtttcttgtgcaggataacttttacaggaacccagatcagtagagtcactaacgcaacataggcaatagaacaggagatgatcagccagtagtgtgtgttgtcagatctagcccttgttccttggtaggcggtggcaaactgttctgtgatcacgagtgtggggatggagaaagcggcaaactctaggagctcaaaaaccacgaacttaatgagccttccagaagccatcctgaggaaaagcaagctgccaagaacctgggactccctctttgactgtgggcagcatatggacccacagacactgaactgggatcaagttcctt

SEQ ID NO: 9840 - RNA, 5385 nt, Homo sapiens
  source 1..5385: mol_type = other RNA
caaaaatctcaattacttttgcaccaacctcatagcttttcttggttttctttttatctttcttcctttcccactttcattcctttcctccctttattcatttttattttgttacaatcaaatgtttagttttctgttgtttaaaaaccagatataccctcctgatctcttagatggaacaagaacctgtgtctcatggttttagccactaccttttatgttataaacacggaatgaaggacaagagggaagggatgccataccaatattgacctcagtgtaccatgttggtacaaaataataaataataatagctgcgagtcatggatttgtagaaaggatggaaggaaaaactttctgataagatagtacatgtatcactaatgtgtcattttcttttattataacttcctttggtctgtactcttgatggttttaaatgttatgaattcatgtaaactccaaatcatgtgaaggggcattccaaaattttgtttataaattactgacttgggactttatataattaaaacatccttaccaatgttgtttggggtcctaggataccctaaaaaatatcattcaacacacaaaaatgaatctaagatatatatttaatacttttagtacttgttactggcatttatacaattttctcagaaaaaaatattgagttttatctcagtatgccaaggagatttggctgtgattctgttagggactgagttggacggggttgtaggagtgagtcacctaaaaatcagaggcatgttaacactatttatgcatatggaaagttaccttttccatttacataaaaatatgcaagctggtaatttggcttactctctagcagctacattgattcctatattcatggggagggacaagtataaatgctttgaatttagaccctcaattgtctggttgtatgtatgaaccaatctcacatcctaaattatgtcatgtgttgcttacatgagattttacatggtcaggaaatcacaagtcattaaaaactgtagatccagaaagaatatattgaaaatgaaataaccctctacatccttggaaggtaaactatatgaaattctttctaaaataatgattttcaacaaagtagtggtggtaagttgcatgcttgccttgtcagaatcataaacaatgtgagagactgctttagttcttaatatctccttccaacccccaagacacactcagctgagaatcttctgtggtaagtcactgatactgatggaagcgtgccatattgctcaggagtactgggtagtgaaaattctctaatgatgggtttattaagagaagggtaatcaaatgacagaaatctatgttggaaaaccttgagatgtttcagaatttgtgctataaaactttatgtaacttgctgattttttaaaataataaaacaggaatagatacctgaaaacaagtcatgagtctcaaaagaaataatttttcttgacctgtagccagcgtgttcttggatgattaaaattcctatattagttgtgcttggagaaaaaaagatgagtaaggaaggatgggtgcttgaggctgatagcttaataaaaagcaaagactgaaaggaagacaaaaaagtcaacatatattgaatacctattgctaggtcagagacttccacatatatcatctgttttaaatttcacaattctccgtactgaagcttacagcatgttgttttctccagatgagtatgttgaggttcagcttaaataattttctcaaggcatggctaacatggtgtaatagtaaaatctggcctcatgattttgagacctgtgcagttacacaaggccacgttcttagatgggccccaaacttagatgggctctgctgtcactgtcttgaaattcttaaaaatttttgaacaaggagcccacattttcatttcatactgagttttacacattatatagccaatcctgctggtaggctgtgccactctttccatagataatctctaaagacacactgtgaaaactcttccctgtaaagcagatgtagagatagagagccccagggcagacacagccagaactttgtgttctggaatcaagatttaggcttgggggatgtggctccctcagaagaagaatcattgcctcgtatgattgtgtaagtagtttctgggtgctaatgtggcttgatgcattatatcagttttctatggttgtgtaacaaatttagtgacttgaaacaacacatgtttattacctcacagtttctgtgggtcaggaggttgggcgtggcctacctggatcagaggctcagggtgtcagtaggctgcaatcaaggtgttggctgggctgcatttttttctggagcttaggacctcttccaagatcatgtgattattggcagaactcagttccttggtattgcaggactcaggccctcagctactagaggccacccacagtttcctgacatgggctcctctctccataggcagtttacacatgattgcttctttaaggccagcaggagattctctgattctctctctatctctctccagtcttctgcctttggagaggattgcagcactaccttttaatgatcttcagacatatgctaaagaaatgtcatagtgaagaacagttgtacaagaataagcccgaaggtgtcttcatctcaggtgcgttagccaacacctccatgattgcactggttcagacagctccaggcaggcctcagaaacaagttatttacttatgacatccagatggcaagtttttctctgatcattttggaattacacagtctggatagaaagggagaaataattgttgagcactgtttggaaaggattaaagaaaagcctctgacattttatttatgtacatgcactcttcttttctcttaagaaaactaacaaaaagttaaaggcaacaaaattaagacataaaacccaccatggttttaatattggatgttatcatctcagttttaaatactatctggtaaaatgatgcttgaggccaattccagtgaataggaataacttttggaaggcagcgctactgttatccatgggaacagatggctcttactctccaaaaatctagatcaatttcattctcttcttgggctattgtaatagaataccatctgatcctttctgtatccagtatagttttctacaaatcgatcctccatacttctagcaagttccaaaaaacaaatcctttccttgttccctgttgcctgtagaattaatcccaaactaaggcaaatgtagctctttatcctttatgaccacatcttgacctcttcatggtacagctttattttctgacagtcagccatggaattcaatgtcttgacctttttgatcccctggctgttctctaaaagcttcatgttctttcttgtttctgtgacttgcttctgtatatgttgctctcagtacttgaaatgcacatctcttgctatgtgccagctttgctttaaccacttgacatgaattactttattaaattcctacaacaatgctctgaggtagataatacagtcaatgccttcactgccttgtgtcattgtgacttaactctgatttcagtcatctccatggccattcctgaggccactcctatgtgactgctaagattgtgttcagatagcacatcctctgggaaatctttctgactgctatgacctctgggcagagtgtgttgctatctactttgtgtagcaattacacccaatatatacgtttatcttgatgtctagtgctttgactgacaaatgcttctttgctgcctgtagtacactgtgaagagactgagagcagtctttagtatttatttattcacttaatttattgttattatttttgtatcacatggtataaagcacttagtgtctggtaggcactcagtaaatgttaaaaagaagaatcacagctaacataattgatcccttgctatatgccaggttcgttctaaccactttacatgaattactttattaagtccctacaacaatgcttttgaggtagacaacacagccaatgcttccagtgccctgtgtcactgtgacataactcatatttcagccatcactatggcagagagttttgtgtgagctcagacttgtgctgagtgtctcaccccatgcacaagtatcagtctgcctgttcaggccttctctaaagtgcaggaagtcactagatctttctaatgtcctggcacagaagtgaagtggatttaacattctcagggcaaccctcaaccacagatgcacaggagctggtgggtaaattctctagcttcccaccctttgaatggacaattctaagaggcattctgtacactcttggaagtctcagctgagtcaaacttccattgcttatagaagcaacttctgtaatttactcctattgtagctctgtctcactcttgtcattcgtaactccttccagagaattctcccaagccaaatacctgcatccaagatcttgtcatgttctattttggagaaacccaaatgaagataagtactactattatccccagtgtatttgaaacagaggcacagagaggctaagctaagttacttgcctaagactttacacctggaaagtgaaagagactagatttgaactcggataatctggctgcagagccagcccattcctgactatcactctatgctcaatgaggtttataacagatataggggtctcaaacagtctaatattacctacctgcccttataatgtttaaaacttgtcttggctggaaggttaagttttcatatctcttacctaggtttggaagcaagggcatactgcttctttagattttcaccctctttcaaatgaattcccacttttaagctccaaagtgttttcccctcccccaccggaagaagaacaatctaaaagagtgacagagcaaacattaaagtattgtaacttcccactttcaaaagctccatttttaaaatctcacattggagggctttgaatagaggcagtgtgaaaagtggaatgagcgtttagattatcattgaggaaaccagtgtcatctgaatcactaactaggttcatcaccttgggtggctttattccccaatctgggcctcagtttttcctattgtgtaagataaagagtttgagttaaagtggctgctcttactgtttttagagtcattaagaatcttctgaactctatgtatatcatctctattatttctcctcccactctaaatacacatccacatgtacatgtattcttccttgagtaatttcagatgctggtgtcatctctggatcctctggggttaaaaatccatggacacaatctctaaatcctattccagttccagcctcctatggtc

SEQ ID NO: 9841 - RNA, 37 nt, Homo sapiens
  source 1..37: mol_type = other RNA
caaaaatctcaattacttttgcaccaacttaatactt

SEQ ID NO: 9842 - RNA, 2385 nt, Homo sapiens
  source 1..2385: mol_type = other RNA
caaaactggcaattacttttgcaccaatttaatattttagagtgtacttctacttatttaaaaaaagttaactgtaaaacagcctcaggcagatcctacagaaggtattccagaagaaggcattgttatcataggagatgacagctccatgcatattactgctcctggaaggctttccagtcagctaagatgtgaagctgtaaaacagtgatattgataatcctgactgccccgctgtctacacctggtttcaaaccatatggtgtcagtactaggctggactgcaccagcagtccaggcagcagtggcaccccaactagacatagctgtgtaccatgtcctattaggaatggaagaacaccctttctaacagtgaaggctcggggtctaggggtgccccaggccccatggccttatcttgcattaggactacaggttccaagacctcttgcaactctgctgctaagggacttatacttagcgtactccactgctctaagtaggtgccccacttcgctaaagtggatgtctgtgctgtcccagtctgggggggtcattgctcatgaacgcacccatcccactatggggtaagccatccacacgactgtaacccatccagccacgctcttatgaacctgaagggcagcatatatggttactaactgcttctttattaatgaacactggggctcagctcccttccatagctgggactaaaagctgactggcgcttccaagcactccatatactgccataggccctagccaactctattggtggttacatgcacatctagtttaaatgggcaccctggttaaccacccagagggcttatgtcatcagaagggctgtttcagcctcatcatcccaatcccaggcaagaggggtgttgtggcctccaaaccagcaaaagaactagaggttaacataacatcattaataagaaaatgatatataatggggctatacatatagccctgcagcaacactatgaaagtccattgtcgccctcccatgaaggcaaactgttcctggctctctggagcaatgctgattgagaagaatgcattggtcaagtccaccacacagtggcaccatcccagttctgttgtcaaacggtccatcaagtccatgacaggtggcacagctgccaagtcttgcaaaacatccacccccaagaatgtcctcaggcatgcaagagacatacacagtgcataagtggagagccaagcagctgatgcccaggtgcaaagacacaggtttcactttcactgaccagctttcatagctgtctatgcagccttccctggaaacttatccgggtccagggaccagtggattgccaagtccatatatggcctttggttgtctggtatcccctaccaagccgggcaccttggccagttctcttatcaaacagaaaatgctttatacttccaccaactgcagcaggtactctttgaactggaacactctggcaggaccaggttgcgcagcaacatccttctcccaaatgacttgcaccaagtctcatcccattctcattgccagttgttaggtttagggttcgggtccagcccatgctgaggtacaagggagtgggtcccttacagaagatgtcatcaacaaaccagaggcggagatgtcactacaagatttgcagctccattacttcaaaatgcacgattatgatggcaattatttgcttgatggtttagaaatctccacagccatcactcatatacagggaccaggattttactccagttctgccgactccagtactggatctcttaagctggatcctagcagatctgcacaggtacctactggaatgcttggctccatgatccatggctctgtcccttgctctaactgggaaatcacatcaggtttagaaacttggagtcctatagagaccaggtgtgtataattttccaatgtcacatccctgaacaaatctctctggccagggtccagctgtttccattcttcctgggtaaagtccactatcacatccttgaaagtcaccgcttcctgaaaactggctgatgagagtagattatgtcccccttggagaagggtggagtctggagaggacagatcttccatctcaggagctcatcccgttcctctggaacttgaacaccagggttcgccaggcagcgttccttcagctggtatctcggtctaggactcagatgtctaactccccttgcagggaatctgcaacacgctgaggttgtctaccctgagctcccctccccctatagcgatccacacactctgatcccgggtccggaagcgcattgaccgccaccagacctaacgcagggagccgaagcaactggacttccagcgcgccaacctctttccacgcctac

SEQ ID NO: 9843 - RNA, 2600 nt, Homo sapiens
  source 1..2600: mol_type = other RNA
caaaactggcaattacttttgcaccaatttaatattttagagtgtacttctacttatttaaaaaaagttaactgtaaaacagcctcaggcagatcctacagaaggtattccagaagaaggcattgttatcataggagatgacagctccatgcatattactgctcctggaaggctttccagtcagctaagatgtgaagctgtaaaacagtgatattgataatcctgactgccccgctgtctacacctggtttcaaaccatatggtgtcagtactaggctggactgcaccagcagtccaggcagcagtggcaccccaactagacatagctgtgtaccatgtcctattaggaatggaagaacaccctttctaacagtgaaggctcggggtctaggggtgccccaggccccatggccttatcttgcattaggactacaggttccaagacctcttgcaactctgctgctaagggacttatacttagcgtactccactgctctaagtaggtgccccacttcgctaaagtggatgtctgtgctgtcccagtctgggggggtcattgctcatgaacgcacccatcccactatggggtaagccatccacacgactgtaacccatccagccacgctcttatgaacctgaagggcagcatatatggttactaactgcttctttattaatgaacactggggctcagctcccttccatagctgggactaaaagctgactggcgcttccaagcactccatatactgccataggccctagccaactctattggtggttacatgcacatctagtttaaatgggcaccctggttaaccacccagagggcttatgtcatcagaagggctgtttcagcctcatcatcccaatcccaggcaagaggggtgttgtggcctccaaaccagcaaaagaactagaggttaacataacatcattaataagaaaatgatatataatggggctatacatatagccctgcagcaacactatgaaagtccattgtcgccctcccatgaaggcaaactgttcctggctctctggagcaatgctgattgagaagaatgcattggtcaagtccaccacacagtggcaccatcccagttctgttgtcaaacggtccatcaagtccatgacaggtggcacagctgccaagtcttgcaaaacatccacccccaagaatgtcctcaggcatgcaagagacatacacagtgcataagtggagagccaagcagctgatgcccaggtgcaaagacacaggtttcactttcactgaccagctttcatagctgtctatgcagccttccctggaaacttatccgggtccagggaccagtggattgccaagtccatatatggcctttggttgtctggtatcccctaccaagccgggcaccttggccagttctcttatcaaacagaaaatgctttatacttccaccaactgcagcaggtactctttgaactggaacactctggcaggaccaggttgcgcagcaacatccttctcccaaatgacttgcaccaagtctgtacaagagtgccaacattacttgcttaactcctacaacttagcaggggcacagacaacataggaagtgtgctccaccacagtagggggtctctggcccacccttggggcccaacagctgctcatgctctattttctggcagaccattgggtgaacctgtaacggaggttcttcctccctgtgtgcatccctcagggactgggcaggcacttcctcatcccattctcattgccagttgttaggtttagggttcgggtccagcccatgctgaggtacaagggagtgggtcccttacagaagatgtcatcaacaaaccagaggcggagatgtcactacaagatttgcagctccattacttcaaaatgcacgattatgatggcaattatttgcttgatggtttagaaatctccacagccatcactcatatacagggaccaggattttactccagttctgccgactccagtactggatctcttaagctggatcctagcagatctgcacaggtacctactggaatgcttggctccatgatccatggctctgtcccttgctctaactgggaaatcacatcaggtttagaaacttggagtcctatagagaccaggtgtgtataattttccaatgtcacatccctgaacaaatctctctggccagggtccagctgtttccattcttcctgggtaaagtccactatcacatccttgaaagtcaccgcttcctgaaaactggctgatgagagtagattatgtcccccttggagaagggtggagtctggagaggacagatcttccatctcaggagctcatcccgttcctctggaacttgaacaccagggttcgccaggcagcgttccttcagctggtatctcggtctaggactcagatgtctaactccccttgcagggaatctgcaacacgctgaggttgtctaccctgagctcccctccccctatagcgatccacacactctgatcccgggtccggaagcgcattgaccgccaccagacctaacgcagggagccgaagcaactggacttccagcgcgccaacctctttccacgcctac

SEQ ID NO: 9844 - RNA, 4888 nt, Homo sapiens
  source 1..4888: mol_type = other RNA
caaaactggcaattacttttgctcttattttcctgttatatgaaattaacaacatacctgctgcaatataactcatttggtacaatttaggtgtttcgagaaattcaacccactaagatcattagcgtaattcatttttatgctacacattaaaatggtgccttcttacagtcactttggaaaactgtttgacagtaaatactaaaactgaaaatatacacaccctacaacctggcaattccattcttaggtttatactcaatggaaatgtatacactcaccaaaagacatgtataagaatgttctacacagtactattcataatagctcagaattgaaaaattctcaaaagactattaatgggagaatgaataacttttggatgtaatgaaaaatggataaacaaacggaagactatacagcaatgagaatgaatgaactacaaatacatgcaacaataagaatggatctcactttggcaggttgaataacggcctccaaagatagccagcgtatgaatccctggaacctgtgaatgtcacttatatggcaaaagagattctgcagatgtgattaaattaaggatcttgagatagggggattatccctgctttatgcaggtgagccctaaacttagaggcagggaaagatctgactacagaagagaagatgatataatgacaaaagcaagctttgatcatagagaggaaggggtcacaagcccataaatacaggccgtcactggaagccaaaaaagggaagaaaacattctccctcacaacctcaataaagagccaaccctgctgatactttgatttaggcctaatgaaactgatttttggacttctgatctccaggactataaaagaataaatctgtgttgttttaagtcactaagtttgtggtagtttgttacagtggcaacaagaaactaaaatattcacaaaaatgatgaatgaaaaaaagtgtattatgtatgattacatttacataaaataaaaaacaggcaaaactaatctatgattttagaagtcaggatagtaactttcagcaagaaagaagacagtgttaagatggggaaagaggagggcttctggggtacacataatgctctgtgttttgatctgaagactagtatgtgagtttgtttaatttgtgaaaacctttatttgtgtactgttttgtgtgtgtgtggtatatgcagttttaaaaactgatgccttttaaacacttactaatctgataatctgccgaaaaagaatatataacatatattcaaggggatggaaaaatacttactgaacaataattttatttctcaagaacgctgaagattttgtttctctcttcaaaagatttaaaaaattttaactggcaaaacataatagtgactcttaaatgctaaaaaaaaaaaaaaaaaaaaaaaaaaaagaaaaaacctaaaaataaaatattgcataagtaagctttgttatgcctcgatcttaggactgtaaattataaaaatacaagtaaaaccacattttttgaaataacagtaaacaaaaacaaaaggcaggtactacataccaaatgaccaaaatgtcttttgggcctaagattcttgaaaatagtaaaaatggtaataatagaaatctctctatagaacattaaatataaaaaccatttataaaacacatcacaattttattgcttgaagaatacagcatatgaaatcacaagaatgtcaaaatgaaaagtcactaggcttcaaacgtataatacattatcagatgcagtaaaatattaacctgaactctgcatcagaaaaaaaaaaaaaggtgtggaaaatatctaagttgtttacttaagaaacagatatacttaaaatagaaagtataaggatgttacagtacaaattagaaaagccaacacgtattaacttatcgttctagactagactacctttggtacttaaactttttaaaaaacaatttcttctatctcatccaaatgcacttcatgggtatgacatccatgaagtaacttcaacttaaaacattcagcaaaattaaccttttcacttcatgggggaagtatatttaataaatgtataacaatatttcccttttactaaaactgcaaaatatgatcattaagaaacctaacagttataaaactttacttacttagctctccaattaaaattggaatcctgggagccacaatctatttttgggcttggtgaatacataagtttaaaagatttggcaactgacataggaatttaattacttaatactatcttaagtgacttttcctttctgtttccaaaatatagacattatgccatttcttcaacatcctggattcctataaacactaccatactgtatttattagaaccaaattaaagcttctctaacaagcaggtagaaactatttatgttccatatacggctgataagttataacacaacttatgtttcatatagggctgatcagttaattcatatagggctgatcagttgtaacataacttcttaagcaaaactaatcttttttttaaagctatcactcaattatggagacaataatgtcatctcaaaaggtaatgttggactctaggccatctagttgggaaaatgtaaaagtaattctaaaaacaataagtaaactataactacaagttaaattaaaaatccctctctcatagcaagcatgctcattaactttcatttctttcccccagcaaaggtttgaatattcataaacctcagttaaaccaagagaaccaatgtaattgtttcaaaagtaccacctatatatttgaataatatgagtatggatggactaggtaagtaatactatcaacaattactgaattggagtgaaagagtaaaaatcatgacagacttccaaactgggcagtctttgaaatgtcatagtggagctcaaaatgaattatgctgtaataaaactatagtttttacctctacacaaaacagaaacaaaataaaaaaacataaccaccaaatttatacaaatactattaaacatactccttcctagtttttgaatgtcttgaagtttttctaaacaagtatattgatctgagcatatatatttattgcctatatatgtactcattttaaaagacaaattcagatactacagaactgaactctttcaccaacccaatccaatgtctactgattcacacagcaccccccccttaataatttaaaattcacaagttttagtttagttaaaagggcagaggaaatgcaaatgcagatttagagctttgtagaaatttcactgtatttttataaacttgaagttatctgtaacactgtttattgatcaaacgaaggactcgctgctatctaaaatttcataaacaccattaaaaattcaaaattgatattatactgaaccttaaattttcaatagttcaaagagacagtttttacatgtatagcacacaatagatgaaacttaatagcagacatccctagaataccaatgacaagtccaccaagatgcatacaaaattacagataagcatttctttcactgtttttgttgtgcagggaaaaacatttatagaagaaatagaaactcagctggtgaatttcagatatcatcatcatcttcttcatcctgagaagatcccgcctgattagatgcactggctgaggcagcagcaagctgggcttgttgggcagcttgctgcatttgaagccattcctgttgggccaattctgcttgttgctgtctagcttttgcaaataattcttgttgctgtctcaataactcttcttcaggaatgccaaggttttccaaacgagaactggcctttcttctttttaatgctactgttttacactcttgcaagacttcttttacttcactgatgtaagagccaaatcccaaactttctagtgcttgtatgacatgctctggtgagatggtcttcttttccgatttgttacaaatctcattggcttcagaagatataaggtgaatgaattcagtgcagcagttcaccaccagctctcgagcatcgttggccacccggacattaggaagagtctctttgatcattttattgatagcagctctggggatagtgagatcatcatcgttgccagacgaggaagccatagtaccttcctgtttctcgcgccccggcttttaaaaactccccagctctggtccactactccaccgagatttctcaaaaagtcgccctcggagagtgatcccggggggtgctttgcgaagagggtgcagaaaatgaacggaggagcagctggcttgagggctgggaacactcgcgtgtgtgagagatttaggatgagtttgggaagaaagtgggggcccgaggattctagagagagcacagcccaggctgaggaggggaaagcgcggtggtccggaaatttgagcggctggggaaccaccttcgtgtctcctcagaggggcgggcgctgtcgcctaactggtccccaacggcgtcggagcagaggcaagatccaggggcactggcctcgccgcggtaccgggcgggtacccagcgggctcggctctatagagcccgaggccccgctgccgctgccgccgccgccagcagccgttgccgccgcctcggccaaaccatccttcagacacccgcgccgccgcctcacaacatgtccgccgctgccgctgccgctgccgctgctggaacggcgacggccgcctgggaactaatatggacagagccaggcacagtgggagtcgcagtggctgccgccgtggccgcgtagcccgaacgcagatcgtggaagccgaagacgcggcaacggtggtccctccagatgccagggaaggtttgcaggaagccgctcccgacaccctttgc

SEQ ID NO: 9845 - RNA, 4939 nt, Homo sapiens
  source 1..4939: mol_type = other RNA
caaaagcaatcgcggtttttgccactgaaatggcgaaactgcatttacttttatatcaacctagtattataaaatatatacaaagcaagttgaggaaccaaacacaaaatacatgtctacaaacatgctttccaatgtactataaataaacctttacttaagatcttgaaatcaaaattagtttgtatagtattcagaatcaaacctaatgacaaagcaagatgaaataaccaacagcatcatcattatcagaatagtaactaacatttatataaaagattactatgtgtcagaaactaagggctttcatttcattcaattctcataacaacctataaagtaggtactatcattatatccattttacagatgagtgaatgaaggctagaatttgggtcaccggcccaacatgacccaactattagtagtaggtagagaagcgggtctccgaacctaggtaatctggctttggaatctgtgctcataaccactgtgctataatgtctctgatagcagctactaattaaaaaataaaaaatgtatgttttcctaactttaatcatcaccagataaggaatattcttggttcatttatgtctaaattttcaacatactttttccctttcaacctattaactatcctcaattttgagtcagctgattttatgtgattgtttccttccctcccacccccagtacactgcctttatgtggctgcatttgtattagtctctgcttagaaaaccaaaaatgtatgacatgattaaaccttgtttgttcaatataaaataagagttaaatactttccataactttgctctcttctcaggccttcaaagtcttgctcagtaaagtactgttgatgctgataatcagagtatcccaccaagagcacatgatgccttggactgcaatactgtcacagcagtgtcttcagttcttctctactgtgtataatgcagagcaaaatgggggtggtggtagaaattatggtagtaaatatatattttctagaaatatatccatttcgtggaaagataatattaagaccatatcaagccaaatatacaaatgagaaagtttcatttacctcaaaaaaatccaggctatacaaacagacaactgaaagccacataggaaatttccgaaacacaaaagaaaaagtctcacctacaagattatttacatgtttagggccagtattattaaaagacgtcatcccctaggtctagtagaaacatatagagaagtctatgctaacacacttggaaagaggactattgtccttccttgcacatgacaaaaaccaaatgaaccaaacccctagaaggtattaatgcacaaaggttttaataccttggctttaatgatttttcaaggttaagaaacaaattcaaattggttggagcttcaactcagtaattacaatcacaatgcatctctgaaaggccctgcatttggaggcagagtaatctgcaaagatgatagtttttacatatgtcctgttacctacaccaatataattactacattatcttataaagacaaacagttgcttcaaactctttaaaaaatatatatataatgagtttcccaaagactcgagtctatattcaaagatgagtaaaaaaaaatccattacttccctagggtcactttcttcctttactcctgcttaaatgcaaaagctgatagtttctgatttgtagaaaaatctaaaggtttctgctttttagacaaattcaggttctcttttgctttttcttcctggttttctgtttcatcactttcatcaaccacacgttttcgcttctttgcttcagttccttcacttgccgtttctcctttggctttgttagcccacacctttctttcttcagttgacaatactctaaatcgaatcattccttcttttattatgtctgcttcatctgaaaagtcaggattgtcagacaaaatattacttctattttcttctaaccacatctggaacccggtctttggcctttggttttcagtgttttgaggaggacatatagctggggtttcagataatacatttttaagattttcttctttcacttcctcagttttattagtttgagaatttcttttctggaaataggatgctgcagatgcctgcttaggcttcggctttggaatcagaggctttataatgggagacttttcattatttgtagttcgactaagtgcagtggatttcttggatgatttgcccatattgtctaaaatattagttgaacgtgctgaattcattgacatggctggttctttggaactggctgataccttaaagggatttactcgtccttggctgctaaaggtaactgacttagctgaaacatcagaggaatttgtacttttggaaaacgagttctgtccaggcttatgtatttctggtttttcttcatcatcagcttctccactgtcctcagcatcttcttcaacttgatttctgaaccttggttggctccactctgtagcagtattgctgtaaccagcattcagcttttttctgaaatcttcttcttcttcttcctcttccacctgggttgctgtcaattcggctgccttctctacagccagttcacttagtttttgagccagtattaatttccgagagcgagaagcatatttaatggctaaattcacagcattttgagtcattagatcagcaagttccacacaacggaattctcgctccagtttacaagaaagcgcaagcattttcattaaaagttcctgttgctcttttgttgcttgatttttagtgctctcttcatattcataaccatttttagctaaataatcaaggtggttgtgaaatataactgaacgccaaaattgctcctccatttgtcctttctctgttgcaatctgacagtaaggaagcttaaaggataatatagcaacagcagggcgtggaagggttgggggaaaccgagaacctttacaaggaatgcaccttagttgctggggattttcatggataccaaccacccagtagtgatcagattttcctttgcagtgctctcttgtattacatataggagtccacgtattaccaagtcctctgttaagcattcgaacaattccttctgaatccacgtaacaaggggtaccttcagctgaaaacccaatccatgcaaggtaggatttccttgtaagaggaagagggtcaccatgcaaaatttgttttttctttttccccagctctagcagttgaactccaaggcactgatccccatcaaatcctgtacctctgtgataaacaatgaaaagctgttctccatgtcctgccattgacaccacaggtccagcaaggctgaatacctctttttgaacccctccaatagtaaacaatcgaagaagcagggcactagtagcggcagcagcccatccttgaccgagacatatggcttcaatatcctcattctgaggcaagtctattatccactctttgcttgaatcccaagaactaaagtgcaggcagtgaagcttgcttgctagttcatcagtgctttcacatgccaacaaaatagcttcgtgggaaagatctgctattgtataattcaaagtgtttgataagtgtgttgcatggtgtatggaggtatcatggaactccacatctatggcattgtcttgctcatcattatagcagcgaataattccaatagagttccacaccatgaatctgtgagtgagatgcaacggtgtagaacctgactgaaatggcttttgccggggagttggcatgggtccatcataaaatggcctttgggatgttacaagtggtagattgtgaatgctgccttcttgaccatcttcctcctcctctttgagaagactagaaccagtttttagcattgaaatatcaactgagttttcatcatcttctaggatgtgacttcgctgtctaggacgacctgaagccatcatgaggtcttcatcatcctcatcatcatttataatcccttactgcttgatgtctttccactggggtcacaaacattctctagaagccctagatttccttccgcatcagtatacgatattcgaccacaagtaggatgccatgccagaccacaaattgcataacctttctcatgtttcaccctttccatgcagtctttggtttccacattccaaactatgattagaccattaatactacctgcagctaaatattgcccacagggagaccaggttactatattgagggtctgagagatgaaattatctgaaagatcaaattgatgactccaagattctcttctatatagcttaacagatttttccacaggaattgccagtaacttcccactttttggctgccaagcaagtctgcagattgattttgcatttatcacatcgttgcatttttgtagcagtggccaactaatagcacatgtctgatctgaaatttgccacactctgacagatccatcacaactagctgatgccagaaagatgtccttaggatcaaaggaaagacttaaaacaggggcatcatgtcctcgaaatgttttctgttggctgctatccatcacatccacaattttgactagaaaatcactagatccagcagcaattttagtaccatccccattaaagaccacatggtttgcatttgtagtgaagcgagtcaatataccatctggaactccttcaggaaatgtgtggacttgaatagtattattagaaactgcagtgaccagttttccactcttcaaagcacatgaatatgccttttctccaacattaatgaacttaggatcatcatcatccaagtcttcccaaatcctcacatcaccatcacttccacaagtcacaataaaaccgggtgaccgagcctccgccactgaggatccacaagagctgcttcccgcgcttcggctcgctcaccacactgcgcctg

SEQ ID NO: 9846 - RNA, 5137 nt, Homo sapiens
  source 1..5137: mol_type = other RNA
caaaagcaatcgcggtttttgccactgaaatggcgaaactgcatttacttttatatcaacctagtattataaaatatatacaaagcaagttgaggaaccaaacacaaaatacatgtctacaaacatgctttccaatgtactataaataaacctttacttaagatcttgaaatcaaaattagtttgtatagtattcagaatcaaacctaatgacaaagcaagatgaaataaccaacagcatcatcattatcagaatagtaactaacatttatataaaagattactatgtgtcagaaactaagggctttcatttcattcaattctcataacaacctataaagtaggtactatcattatatccattttacagatgagtgaatgaaggctagaatttgggtcaccggcccaacatgacccaactattagtagtaggtagagaagcgggtctccgaacctaggtaatctggctttggaatctgtgctcataaccactgtgctataatgtctctgatagcagctactaattaaaaaataaaaaatgtatgttttcctaactttaatcatcaccagataaggaatattcttggttcatttatgtctaaattttcaacatactttttccctttcaacctattaactatcctcaattttgagtcagctgattttatgtgattgtttccttccctcccacccccagtacactgcctttatgtggctgcatttgtattagtctctgcttagaaaaccaaaaatgtatgacatgattaaaccttgtttgttcaatataaaataagagttaaatactttccataactttgctctcttctcaggccttcaaagtcttgctcagtaaagtactgttgatgctgataatcagagtatcccaccaagagcacatgatgccttggactgcaatactgtcacagcagtgtcttcagttcttctctactgtgtataatgcagagcaaaatgggggtggtggtagaaattatggtagtaaatatatattttctagaaatatatccatttcgtggaaagataatattaagaccatatcaagccaaatatacaaatgagaaagtttcatttacctcaaaaaaatccaggctatacaaacagacaactgaaagccacataggaaatttccgaaacacaaaagaaaaagtctcacctacaagattatttacatgtttagggccagtattattaaaagacgtcatcccctaggtctagtagaaacatatagagaagtctatgctaacacacttggaaagaggactattgtccttccttgcacatgacaaaaaccaaatgaaccaaacccctagaaggtattaatgcacaaaggttttaataccttggctttaatgatttttcaaggttaagaaacaaattcaaattggttggagcttcaactcagtaattacaatcacaatgcatctctgaaaggccctgcatttggaggcagagtaatctgcaaagatgatagtttttacatatgtcctgttacctacaccaatataattactacattatcttataaagacaaacagttgcttcaaactctttaaaaaatatatatataatgagtttcccaaagactcgagtctatattcaaagatgagtaaaaaaaaatccattacttccctagggtcactttcttcctttactcctgcttaaatgcaaaagctgatagtttctgatttgtagaaaaatctaaaggtttctgctttttagacaaattcaggttctcttttgctttttcttcctggttttctgtttcatcactttcatcaaccacacgttttcgcttctttgcttcagttccttcacttgccgtttctcctttggctttgttagcccacacctttctttcttcagttgacaatactctaaatcgaatcattccttcttttattatgtctgcttcatctgaaaagtcaggattgtcagacaaaatattacttctattttcttctaaccacatctggaacccggtctttggcctttggttttcagtgttttgaggaggacatatagctggggtttcagataatacatttttaagattttcttctttcacttcctcagttttattagtttgagaatttcttttctggaaataggatgctgcagatgcctgcttaggcttcggctttggaatcagaggctttataatgggagacttttcattatttgtagttcgactaagtgcagtggatttcttggatgatttgcccatattgtctaaaatattagttgaacgtgctgaattcattgacatggctggttctttggaactggctgataccttaaagggatttactcgtccttggctgctaaaggtaactgacttagctgaaacatcagaggaatttgtacttttggaaaacgagttctgtccaggcttatgtatttctggtttttcttcatcatcagcttctccactgtcctcagcatcttcttcaacttgatttctgaaccttggttggctccactctgtagcagtattgctgtaaccagcattcagcttttttctgaaatcttcttcttcttcttcctcttccacctgggttgctgtcaattcggctgccttctctacagccagttcacttagtttttgagccagtattaatttccgagagcgagaagcatatttaatggctaaattcacagcattttgagtcattagatcagcaagttccacacaacggaattctcgctccagtttacaagaaagcgcaagcattttcattaaaagttcctgttgctcttttgttgcttgatttttagtgctctcttcatattcataaccatttttagctaaataatcaaggtggttgtgaaatataactgaacgccaaaattgctcctccatttgtcctttctctgttgcaatctgacagtaaggaagcttaaaggataatatagcaacagcagggcgtggaagggttgggggaaaccgagaacctttacaaggaatgcaccttagttgctggggattttcatggataccaaccacccagtagtgatcagattttcctttgcagtgctctcttgtattacatataggagtccacgtattaccaagtcctctgttaagcattcgaacaattccttctgaatccacgtaacaaggggtaccttcagctgaaaacccaatccatgcaaggtaggatttccttgtaagaggaagagggtcaccatgcaaaatttgttttttctttttccccagctctagcagttgaactccaaggcactgatccccatcaaatcctgtacctctgtgataaacaatgaaaagctgttctccatgtcctgccattgacaccacaggtccagcaaggctgaatacctctttttgaacccctccaatagtaaacaatcgaagaagcagggcactagtagcggcagcagcccatccttgaccgagacatatggcttcaatatcctcattctgaggcaagtctattatccactctttgcttgaatcccaagaactaaagtgcaggcagtgaagcttgcttgctagttcatcagtgctttcacatgccaacaaaatagcttcgtgggaaagatctgctattgtataattcaaagtgtttgataagtgtgttgcatggtgtatggaggtatcatggaactccacatctatggcattgtcttgctcatcattatagcagcgaataattccaatagagttccacaccatgaatctgtgagtgagatgcaacggtgtagaacctgactgaaatggcttttgccggggagttggcatgggtccatcataaaatggcctttgggatgttacaagtggtagattgtgaatgctgccttcttgaccatcttcctcctcctctttgagaagactagaaccagtttttagcattgaaatatcaactgagttttcatcatcttctaggatgtgacttcgctgtctaggacgacctgaagccatcatgaggtcttcatcatcctcatcatcatttataatcccttttgaaaaagaagggatctcaactgcattgtcatttagaaaatcaccagcattactcatatcatctccatcaaaaagatcattataatccttttccactctgctagataccttactgcttgatgtctttccactggggtcacaaacattctctagaagccctagatttccttccgcatcagtatacgatattcgaccacaagtaggatgccatgccagaccacaaattgcataacctttctcatgtttcaccctttccatgcagtctttggtttccacattccaaactatgattagaccattaatactacctgcagctaaatattgcccacagggagaccaggttactatattgagggtctgagagatgaaattatctgaaagatcaaattgatgactccaagattctcttctatatagcttaacagatttttccacaggaattgccagtaacttcccactttttggctgccaagcaagtctgcagattgattttgcatttatcacatcgttgcatttttgtagcagtggccaactaatagcacatgtctgatctgaaatttgccacactctgacagatccatcacaactagctgatgccagaaagatgtccttaggatcaaaggaaagacttaaaacaggggcatcatgtcctcgaaatgttttctgttggctgctatccatcacatccacaattttgactagaaaatcactagatccagcagcaattttagtaccatccccattaaagaccacatggtttgcatttgtagtgaagcgagtcaatataccatctggaactccttcaggaaatgtgtggacttgaatagtattattagaaactgcagtgaccagttttccactcttcaaagcacatgaatatgccttttctccaacattaatgaacttaggatcatcatcatccaagtcttcccaaatcctcacatcaccatcacttccacaagtcacaataaaactcccagaatcatcaaaacagacctccgtgtgtccctctgtatgcccatatctcattggcttccgtgtggcaggcatgttttcctttacctatccgggtgaccgagcctccgccactgaggatccacaagagctgcttcccgcgcttcggctcgctcaccacact

SEQ ID NO: 9847 - RNA, 4944 nt, Homo sapiens
  source 1..4944: mol_type = other RNA
caaaagcaatcgcggtttttgccactgaaatggcgaaactgcatttacttttatatcaacctagtattataaaatatatacaaagcaagttgaggaaccaaacacaaaatacatgtctacaaacatgctttccaatgtactataaataaacctttacttaagatcttgaaatcaaaattagtttgtatagtattcagaatcaaacctaatgacaaagcaagatgaaataaccaacagcatcatcattatcagaatagtaactaacatttatataaaagattactatgtgtcagaaactaagggctttcatttcattcaattctcataacaacctataaagtaggtactatcattatatccattttacagatgagtgaatgaaggctagaatttgggtcaccggcccaacatgacccaactattagtagtaggtagagaagcgggtctccgaacctaggtaatctggctttggaatctgtgctcataaccactgtgctataatgtctctgatagcagctactaattaaaaaataaaaaatgtatgttttcctaactttaatcatcaccagataaggaatattcttggttcatttatgtctaaattttcaacatactttttccctttcaacctattaactatcctcaattttgagtcagctgattttatgtgattgtttccttccctcccacccccagtacactgcctttatgtggctgcatttgtattagtctctgcttagaaaaccaaaaatgtatgacatgattaaaccttgtttgttcaatataaaataagagttaaatactttccataactttgctctcttctcaggccttcaaagtcttgctcagtaaagtactgttgatgctgataatcagagtatcccaccaagagcacatgatgccttggactgcaatactgtcacagcagtgtcttcagttcttctctactgtgtataatgcagagcaaaatgggggtggtggtagaaattatggtagtaaatatatattttctagaaatatatccatttcgtggaaagataatattaagaccatatcaagccaaatatacaaatgagaaagtttcatttacctcaaaaaaatccaggctatacaaacagacaactgaaagccacataggaaatttccgaaacacaaaagaaaaagtctcacctacaagattatttacatgtttagggccagtattattaaaagacgtcatcccctaggtctagtagaaacatatagagaagtctatgctaacacacttggaaagaggactattgtccttccttgcacatgacaaaaaccaaatgaaccaaacccctagaaggtattaatgcacaaaggttttaataccttggctttaatgatttttcaaggttaagaaacaaattcaaattggttggagcttcaactcagtaattacaatcacaatgcatctctgaaaggccctgcatttggaggcagagtaatctgcaaagatgatagtttttacatatgtcctgttacctacaccaatataattactacattatcttataaagacaaacagttgcttcaaactctttaaaaaatatatatataatgagtttcccaaagactcgagtctatattcaaagatgagtaaaaaaaaatccattacttccctagggtcactttcttcctttactcctgcttaaatgcaaaagctgatagtttctgatttgtagaaaaatctaaaggtttctgctttttagacaaattcaggttctcttttgctttttcttcctggttttctgtttcatcactttcatcaaccacacgttttcgcttctttgcttcagttccttcacttgccgtttctcctttggctttgttagcccacacctttctttcttcagttgacaatactctaaatcgaatcattccttcttttattatgtctgcttcatctgaaaagtcaggattgtcagacaaaatattacttctattttcttctaaccacatctggaacccggtctttggcctttggttttcagtgttttgaggaggacatatagctggggtttcagataatacatttttaagattttcttctttcacttcctcagttttattagtttgagaatttcttttctggaaataggatgctgcagatgcctgcttaggcttcggctttggaatcagaggctttataatgggagacttttcattatttgtagttcgactaagtgcagtggatttcttggatgatttgcccatattgtctaaaatattagttgaacgtgctgaattcattgacatggctggttctttggaactggctgataccttaaagggatttactcgtccttggctgctaaaggtaactgcacctgacttagctgaaacatcagaggaatttgtacttttggaaaacgagttctgtccaggcttatgtatttctggtttttcttcatcatcagcttctccactgtcctcagcatcttcttcaacttgatttctgaaccttggttggctccactctgtagcagtattgctgtaaccagcattcagcttttttctgaaatcttcttcttcttcttcctcttccacctgggttgctgtcaattcggctgccttctctacagccagttcacttagtttttgagccagtattaatttccgagagcgagaagcatatttaatggctaaattcacagcattttgagtcattagatcagcaagttccacacaacggaattctcgctccagtttacaagaaagcgcaagcattttcattaaaagttcctgttgctcttttgttgcttgatttttagtgctctcttcatattcataaccatttttagctaaataatcaaggtggttgtgaaatataactgaacgccaaaattgctcctccatttgtcctttctctgttgcaatctgacagtaaggaagcttaaaggataatatagcaacagcagggcgtggaagggttgggggaaaccgagaacctttacaaggaatgcaccttagttgctggggattttcatggataccaaccacccagtagtgatcagattttcctttgcagtgctctcttgtattacatataggagtccacgtattaccaagtcctctgttaagcattcgaacaattccttctgaatccacgtaacaaggggtaccttcagctgaaaacccaatccatgcaaggtaggatttccttgtaagaggaagagggtcaccatgcaaaatttgttttttctttttccccagctctagcagttgaactccaaggcactgatccccatcaaatcctgtacctctgtgataaacaatgaaaagctgttctccatgtcctgccattgacaccacaggtccagcaaggctgaatacctctttttgaacccctccaatagtaaacaatcgaagaagcagggcactagtagcggcagcagcccatccttgaccgagacatatggcttcaatatcctcattctgaggcaagtctattatccactctttgcttgaatcccaagaactaaagtgcaggcagtgaagcttgcttgctagttcatcagtgctttcacatgccaacaaaatagcttcgtgggaaagatctgctattgtataattcaaagtgtttgataagtgtgttgcatggtgtatggaggtatcatggaactccacatctatggcattgtcttgctcatcattatagcagcgaataattccaatagagttccacaccatgaatctgtgagtgagatgcaacggtgtagaacctgactgaaatggcttttgccggggagttggcatgggtccatcataaaatggcctttgggatgttacaagtggtagattgtgaatgctgccttcttgaccatcttcctcctcctctttgagaagactagaaccagtttttagcattgaaatatcaactgagttttcatcatcttctaggatgtgacttcgctgtctaggacgacctgaagccatcatgaggtcttcatcatcctcatcatcatttataatcccttactgcttgatgtctttccactggggtcacaaacattctctagaagccctagatttccttccgcatcagtatacgatattcgaccacaagtaggatgccatgccagaccacaaattgcataacctttctcatgtttcaccctttccatgcagtctttggtttccacattccaaactatgattagaccattaatactacctgcagctaaatattgcccacagggagaccaggttactatattgagggtctgagagatgaaattatctgaaagatcaaattgatgactccaagattctcttctatatagcttaacagatttttccacaggaattgccagtaacttcccactttttggctgccaagcaagtctgcagattgattttgcatttatcacatcgttgcatttttgtagcagtggccaactaatagcacatgtctgatctgaaatttgccacactctgacagatccatcacaactagctgatgccagaaagatgtccttaggatcaaaggaaagacttaaaacaggggcatcatgtcctcgaaatgttttctgttggctgctatccatcacatccacaattttgactagaaaatcactagatccagcagcaattttagtaccatccccattaaagaccacatggtttgcatttgtagtgaagcgagtcaatataccatctggaactccttcaggaaatgtgtggacttgaatagtattattagaaactgcagtgaccagttttccactcttcaaagcacatgaatatgccttttctccaacattaatgaacttaggatcatcatcatccaagtcttcccaaatcctcacatcaccatcacttccacaagtcacaataaaaccgggtgaccgagcctccgccactgaggatccacaagagctgcttcccgcgcttcggctcgctcaccacactgcgcct

SEQ ID NO: 9848 - RNA, 5050 nt, Homo sapiens
  source 1..5050: mol_type = other RNA
caaaagcaatcgcggtttttgccactgaaatggcgaaactgcatttacttttatatcaacctagtattataaaatatatacaaagcaagttgaggaaccaaacacaaaatacatgtctacaaacatgctttccaatgtactataaataaacctttacttaagatcttgaaatcaaaattagtttgtatagtattcagaatcaaacctaatgacaaagcaagatgaaataaccaacagcatcatcattatcagaatagtaactaacatttatataaaagattactatgtgtcagaaactaagggctttcatttcattcaattctcataacaacctataaagtaggtactatcattatatccattttacagatgagtgaatgaaggctagaatttgggtcaccggcccaacatgacccaactattagtagtaggtagagaagcgggtctccgaacctaggtaatctggctttggaatctgtgctcataaccactgtgctataatgtctctgatagcagctactaattaaaaaataaaaaatgtatgttttcctaactttaatcatcaccagataaggaatattcttggttcatttatgtctaaattttcaacatactttttccctttcaacctattaactatcctcaattttgagtcagctgattttatgtgattgtttccttccctcccacccccagtacactgcctttatgtggctgcatttgtattagtctctgcttagaaaaccaaaaatgtatgacatgattaaaccttgtttgttcaatataaaataagagttaaatactttccataactttgctctcttctcaggccttcaaagtcttgctcagtaaagtactgttgatgctgataatcagagtatcccaccaagagcacatgatgccttggactgcaatactgtcacagcagtgtcttcagttcttctctactgtgtataatgcagagcaaaatgggggtggtggtagaaattatggtagtaaatatatattttctagaaatatatccatttcgtggaaagataatattaagaccatatcaagccaaatatacaaatgagaaagtttcatttacctcaaaaaaatccaggctatacaaacagacaactgaaagccacataggaaatttccgaaacacaaaagaaaaagtctcacctacaagattatttacatgtttagggccagtattattaaaagacgtcatcccctaggtctagtagaaacatatagagaagtctatgctaacacacttggaaagaggactattgtccttccttgcacatgacaaaaaccaaatgaaccaaacccctagaaggtattaatgcacaaaggttttaataccttggctttaatgatttttcaaggttaagaaacaaattcaaattggttggagcttcaactcagtaattacaatcacaatgcatctctgaaaggccctgcatttggaggcagagtaatctgcaaagatgatagtttttacatatgtcctgttacctacaccaatataattactacattatcttataaagacaaacagttgcttcaaactctttaaaaaatatatatataatgagtttcccaaagactcgagtctatattcaaagatgagtaaaaaaaaatccattacttccctagggtcactttcttcctttactcctgcttaaatgcaaaagctgatagtttctgatttgtagaaaaatctaaaggtttctgctttttagacaaattcaggttctcttttgctttttcttcctggttttctgtttcatcactttcatcaaccacacgttttcgcttctttgcttcagttccttcacttgccgtttctcctttggctttgttagcccacacctttctttcttcagttgacaatactctaaatcgaatcattccttcttttattatgtctgcttcatctgaaaagtcaggattgtcagacaaaatattacttctattttcttctaaccacatctggaacccggtctttggcctttggttttcagtgttttgaggaggacatatagctggggtttcagataatacatttttaagattttcttctttcacttcctcagttttattagtttgagaatttcttttctggaaataggatgctgcagatgcctgcttaggcttcggctttggaatcagaggctttataatgggagacttttcattatttgtagttcgactaagtgcagtggatttcttggatgatttgcccatattgtctaaaatattagttgaacgtgctgaattcattgacatggctggttctttggaactggctgataccttaaagggatttactcgtccttggctgctaaaggtaactgcacctgacttagctgaaacatcagaggaatttgtacttttggaaaacgagttctgtccaggcttatgtatttctggtttttcttcatcatcagcttctccactgtcctcagcatcttcttcaacttgatttctgaaccttggttggctccactctgtagcagtattgctgtaaccagcattcagcttttttctgaaatcttcttcttcttcttcctcttccacctgggttgctgtcaattcggctgccttctctacagccagttcacttagtttttgagccagtattaatttccgagagcgagaagcatatttaatggctaaattcacagcattttgagtcattagatcagcaagttccacacaacggaattctcgctccagtttacaagaaagcgcaagcattttcattaaaagttcctgttgctcttttgttgcttgatttttagtgctctcttcatattcataaccatttttagctaaataatcaaggtggttgtgaaatataactgaacgccaaaattgctcctccatttgtcctttctctgttgcaatctgacagtaaggaagcttaaaggataatatagcaacagcagggcgtggaagggttgggggaaaccgagaacctttacaaggaatgcaccttagttgctggggattttcatggataccaaccacccagtagtgatcagattttcctttgcagtgctctcttgtattacatataggagtccacgtattaccaagtcctctgttaagcattcgaacaattccttctgaatccacgtaacaaggggtaccttcagctgaaaacccaatccatgcaaggtaggatttccttgtaagaggaagagggtcaccatgcaaaatttgttttttctttttccccagctctagcagttgaactccaaggcactgatccccatcaaatcctgtacctctgtgataaacaatgaaaagctgttctccatgtcctgccattgacaccacaggtccagcaaggctgaatacctctttttgaacccctccaatagtaaacaatcgaagaagcagggcactagtagcggcagcagcccatccttgaccgagacatatggcttcaatatcctcattctgaggcaagtctattatccactctttgcttgaatcccaagaactaaagtgcaggcagtgaagcttgcttgctagttcatcagtgctttcacatgccaacaaaatagcttcgtgggaaagatctgctattgtataattcaaagtgtttgataagtgtgttgcatggtgtatggaggtatcatggaactccacatctatggcattgtcttgctcatcattatagcagcgaataattccaatagagttccacaccatgaatctgtgagtgagatgcaacggtgtagaacctgactgaaatggcttttgccggggagttggcatgggtccatcataaaatggcctttgggatgttacaagtggtagattgtgaatgctgccttcttgaccatcttcctcctcctctttgagaagactagaaccagtttttagcattgaaatatcaactgagttttcatcatcttctaggatgtgacttcgctgtctaggacgacctgaagccatcatgaggtcttcatcatcctcatcatcatttataatcccttttgaaaaagaagggatctcaactgcattgtcatttagaaaatcaccagcattactcatatcatctccatcaaaaagatcattataatccttttccactctgctagataccttactgcttgatgtctttccactggggtcacaaacattctctagaagccctagatttccttccgcatcagtatacgatattcgaccacaagtaggatgccatgccagaccacaaattgcataacctttctcatgtttcaccctttccatgcagtctttggtttccacattccaaactatgattagaccattaatactacctgcagctaaatattgcccacagggagaccaggttactatattgagggtctgagagatgaaattatctgaaagatcaaattgatgactccaagattctcttctatatagcttaacagatttttccacaggaattgccagtaacttcccactttttggctgccaagcaagtctgcagattgattttgcatttatcacatcgttgcatttttgtagcagtggccaactaatagcacatgtctgatctgaaatttgccacactctgacagatccatcacaactagctgatgccagaaagatgtccttaggatcaaaggaaagacttaaaacaggggcatcatgtcctcgaaatgttttctgttggctgctatccatcacatccacaattttgactagaaaatcactagatccagcagcaattttagtaccatccccattaaagaccacatggtttgcatttgtagtgaagcgagtcaatataccatctggaactccttcaggaaatgtgtggacttgaatagtattattagaaactgcagtgaccagttttccactcttcaaagcacatgaatatgccttttctccaacattaatgaacttaggatcatcatcatccaagtcttcccaaatcctcacatcaccatcacttccacaagtcacaataaaaccgggtgaccgagcctccgccactgaggatccacaagagctgcttcccgcgcttcggctcgctcaccacact

SEQ ID NO: 9849 - RNA, 5143 nt, Homo sapiens
  source 1..5143: mol_type = other RNA
caaaagcaatcgcggtttttgccactgaaatggcgaaactgcatttacttttatatcaacctagtattataaaatatatacaaagcaagttgaggaaccaaacacaaaatacatgtctacaaacatgctttccaatgtactataaataaacctttacttaagatcttgaaatcaaaattagtttgtatagtattcagaatcaaacctaatgacaaagcaagatgaaataaccaacagcatcatcattatcagaatagtaactaacatttatataaaagattactatgtgtcagaaactaagggctttcatttcattcaattctcataacaacctataaagtaggtactatcattatatccattttacagatgagtgaatgaaggctagaatttgggtcaccggcccaacatgacccaactattagtagtaggtagagaagcgggtctccgaacctaggtaatctggctttggaatctgtgctcataaccactgtgctataatgtctctgatagcagctactaattaaaaaataaaaaatgtatgttttcctaactttaatcatcaccagataaggaatattcttggttcatttatgtctaaattttcaacatactttttccctttcaacctattaactatcctcaattttgagtcagctgattttatgtgattgtttccttccctcccacccccagtacactgcctttatgtggctgcatttgtattagtctctgcttagaaaaccaaaaatgtatgacatgattaaaccttgtttgttcaatataaaataagagttaaatactttccataactttgctctcttctcaggccttcaaagtcttgctcagtaaagtactgttgatgctgataatcagagtatcccaccaagagcacatgatgccttggactgcaatactgtcacagcagtgtcttcagttcttctctactgtgtataatgcagagcaaaatgggggtggtggtagaaattatggtagtaaatatatattttctagaaatatatccatttcgtggaaagataatattaagaccatatcaagccaaatatacaaatgagaaagtttcatttacctcaaaaaaatccaggctatacaaacagacaactgaaagccacataggaaatttccgaaacacaaaagaaaaagtctcacctacaagattatttacatgtttagggccagtattattaaaagacgtcatcccctaggtctagtagaaacatatagagaagtctatgctaacacacttggaaagaggactattgtccttccttgcacatgacaaaaaccaaatgaaccaaacccctagaaggtattaatgcacaaaggttttaataccttggctttaatgatttttcaaggttaagaaacaaattcaaattggttggagcttcaactcagtaattacaatcacaatgcatctctgaaaggccctgcatttggaggcagagtaatctgcaaagatgatagtttttacatatgtcctgttacctacaccaatataattactacattatcttataaagacaaacagttgcttcaaactctttaaaaaatatatatataatgagtttcccaaagactcgagtctatattcaaagatgagtaaaaaaaaatccattacttccctagggtcactttcttcctttactcctgcttaaatgcaaaagctgatagtttctgatttgtagaaaaatctaaaggtttctgctttttagacaaattcaggttctcttttgctttttcttcctggttttctgtttcatcactttcatcaaccacacgttttcgcttctttgcttcagttccttcacttgccgtttctcctttggctttgttagcccacacctttctttcttcagttgacaatactctaaatcgaatcattccttcttttattatgtctgcttcatctgaaaagtcaggattgtcagacaaaatattacttctattttcttctaaccacatctggaacccggtctttggcctttggttttcagtgttttgaggaggacatatagctggggtttcagataatacatttttaagattttcttctttcacttcctcagttttattagtttgagaatttcttttctggaaataggatgctgcagatgcctgcttaggcttcggctttggaatcagaggctttataatgggagacttttcattatttgtagttcgactaagtgcagtggatttcttggatgatttgcccatattgtctaaaatattagttgaacgtgctgaattcattgacatggctggttctttggaactggctgataccttaaagggatttactcgtccttggctgctaaaggtaactgcacctgacttagctgaaacatcagaggaatttgtacttttggaaaacgagttctgtccaggcttatgtatttctggtttttcttcatcatcagcttctccactgtcctcagcatcttcttcaacttgatttctgaaccttggttggctccactctgtagcagtattgctgtaaccagcattcagcttttttctgaaatcttcttcttcttcttcctcttccacctgggttgctgtcaattcggctgccttctctacagccagttcacttagtttttgagccagtattaatttccgagagcgagaagcatatttaatggctaaattcacagcattttgagtcattagatcagcaagttccacacaacggaattctcgctccagtttacaagaaagcgcaagcattttcattaaaagttcctgttgctcttttgttgcttgatttttagtgctctcttcatattcataaccatttttagctaaataatcaaggtggttgtgaaatataactgaacgccaaaattgctcctccatttgtcctttctctgttgcaatctgacagtaaggaagcttaaaggataatatagcaacagcagggcgtggaagggttgggggaaaccgagaacctttacaaggaatgcaccttagttgctggggattttcatggataccaaccacccagtagtgatcagattttcctttgcagtgctctcttgtattacatataggagtccacgtattaccaagtcctctgttaagcattcgaacaattccttctgaatccacgtaacaaggggtaccttcagctgaaaacccaatccatgcaaggtaggatttccttgtaagaggaagagggtcaccatgcaaaatttgttttttctttttccccagctctagcagttgaactccaaggcactgatccccatcaaatcctgtacctctgtgataaacaatgaaaagctgttctccatgtcctgccattgacaccacaggtccagcaaggctgaatacctctttttgaacccctccaatagtaaacaatcgaagaagcagggcactagtagcggcagcagcccatccttgaccgagacatatggcttcaatatcctcattctgaggcaagtctattatccactctttgcttgaatcccaagaactaaagtgcaggcagtgaagcttgcttgctagttcatcagtgctttcacatgccaacaaaatagcttcgtgggaaagatctgctattgtataattcaaagtgtttgataagtgtgttgcatggtgtatggaggtatcatggaactccacatctatggcattgtcttgctcatcattatagcagcgaataattccaatagagttccacaccatgaatctgtgagtgagatgcaacggtgtagaacctgactgaaatggcttttgccggggagttggcatgggtccatcataaaatggcctttgggatgttacaagtggtagattgtgaatgctgccttcttgaccatcttcctcctcctctttgagaagactagaaccagtttttagcattgaaatatcaactgagttttcatcatcttctaggatgtgacttcgctgtctaggacgacctgaagccatcatgaggtcttcatcatcctcatcatcatttataatcccttttgaaaaagaagggatctcaactgcattgtcatttagaaaatcaccagcattactcatatcatctccatcaaaaagatcattataatccttttccactctgctagataccttactgcttgatgtctttccactggggtcacaaacattctctagaagccctagatttccttccgcatcagtatacgatattcgaccacaagtaggatgccatgccagaccacaaattgcataacctttctcatgtttcaccctttccatgcagtctttggtttccacattccaaactatgattagaccattaatactacctgcagctaaatattgcccacagggagaccaggttactatattgagggtctgagagatgaaattatctgaaagatcaaattgatgactccaagattctcttctatatagcttaacagatttttccacaggaattgccagtaacttcccactttttggctgccaagcaagtctgcagattgattttgcatttatcacatcgttgcatttttgtagcagtggccaactaatagcacatgtctgatctgaaatttgccacactctgacagatccatcacaactagctgatgccagaaagatgtccttaggatcaaaggaaagacttaaaacaggggcatcatgtcctcgaaatgttttctgttggctgctatccatcacatccacaattttgactagaaaatcactagatccagcagcaattttagtaccatccccattaaagaccacatggtttgcatttgtagtgaagcgagtcaatataccatctggaactccttcaggaaatgtgtggacttgaatagtattattagaaactgcagtgaccagttttccactcttcaaagcacatgaatatgccttttctccaacattaatgaacttaggatcatcatcatccaagtcttcccaaatcctcacatcaccatcacttccacaagtcacaataaaactcccagaatcatcaaaacagacctccgtgtgtccctctgtatgcccatatctcattggcttccgtgtggcaggcatgttttcctttacctatccgggtgaccgagcctccgccactgaggatccacaagagctgcttcccgcgcttcggctcgctcaccacact

SEQ ID NO: 9850 - RNA, 2281 nt, Homo sapiens
  source 1..2281: mol_type = other RNA
caaaagtgattgtggtttttgccattacttttgcaccatcctactacaagtttggtctccagaatatattgtatatcggatgaaacacaggctgaacatcccttttccggcacccttggcctattgatcatgatcttctttcctggcatgcttggactcaacttcagaatgtttcttgatactgtgtttcaggcaactgccaccaatcaattggtgttggcacaatccagaggaccgctaccggtctccagtagatttcacctggtgtagagagatctgaggcgtattatcgctggcaaaacgcgatggggagttcccggctgggcaccagggtgcctgagtgtagcatctcaacaggctcattgtctgtggcctggatgtcgtatttgcggacaatccaacaaagagccaaatgcagttgaagctctgctaatcggcgaccaatgcacattctttttccaacgccaaatggaagatgcgcaaaaggattaattttttccttctcctgaagccaacgttcaggtctaaactgacttgaatcttcaaaattgtcttcactggatcccaacacctgggtatttagcatgagcactgttcctttgggtaaagcatattcacccagaactgttgccttgtcaagagtccgagttgtaaatggtacactcggcgtaagcctcatagattctttcagacaggcttttaaatacggcatattcctcaaatcttctgcccgtggcacctgattctcaggtaatacactttgaatttccttaagaagcttttgttgcacttggggattacgggataaattgtagagaatccacattagactgtttgctgtcgtttccaccgcagccagctggagctctgtgacagcagcatacaattctttctttgaaagccgattctggtgataaatgtcacaaaggaaatctgcactaggctgctgagaatacttctctaaccggttgtcgatacaagctttgactgatttgaaaatggtgtcccaggccagagtgtggtcctgccagaccttggtgttgaggctcttgtgcagctcgactggagtgaccatcatcctcccaaacgtgctcatcattgttttgatggccatgatgaagttcacagcttcatcccctgcattcttctggagaagcccaaatctcttctcatacaacacgaggcagatactttcaaacgaccatttgttcagttcgctgtacaagtcttcaacgtggcctctttcatcacagagctcatctattctgcccataaaatcggccaagacctcattgattttgttgtccagcttcatcacttcccctggtttcattagtttcttttgaaaggcactccggacccgctgccagtcttccccttccaggatcagcagcccgtagccttctttgcggtagtcgcgataggccttccacggtttgatctccagccgctgcgggtacgcgctctcggtgcggtacagcgcttccagcaggcatggcgagcccaggtgcaccgactcaaaggaacccaacttcatgcggaaaatcttgccatacttcttgtggtactccaccagggtgtcgtgctgtttcttgagaccccctttccagagaatctgcagcaggctgcccagcagtggccagctggtggggcccggcagggcggccgcgttctgagtctcgccaccagctgtcagcgggcagactggcacctctcgcggctgaggggacgtgtacgccgtagatgtcaccagtctcgggggctgcctcggactgcgcagctgctgcaggaaggcggcaagcgagcggctcttgctgatgggggagctcatggcagcgggggacaccggagcgcgggaaggcaggaggatggggtggggcgaggttggtacgaggtgctagtgggagtcggggcttaacgattctgggaaaaggaagcaaagagggccagctggtgtgatggagcggggtgaggcgggacaggcagcagaaaggacctcggcgaggatgctcgacgctgcaccacgcgacagcctcagagcattggtgcctccttgcactggccgcaggggctggaagagggtggccggtgtctggggacctcttgaaaagggaaagctgggagtcctcctgttggtccgcaaggctgacctctagggtctggctggagccacggggaggtgtcaaggagggtagatgagatgctgctggcgctgcgtttcctcctgtccctctccatgttcctatgcccagggaccatgcatttatggagacagagcatg

SEQ ID NO: 9851 - RNA, 635 nt, Homo sapiens
  source 1..635: mol_type = other RNA
caaagaattctccttttgggctctgacactgatgatgacttcagctctttgggaggccacagccaagctcgtaaagttctttctatgcagttcttggttaccctggagaagggcaagggtgagactctccaagggtgctacactgggtacatgacacttcactgtgaaggcttcgtccacagccacccaggcaggctgcagctccaggatcacttgctctggtggctaatacacagtgatgccaaggcttgtgtccttttgaatccctgcacaagagaagaagcactgcaggatggaattctctgtgacatcctccagaagaaactctttccactgaggccctttgcccacctgagttttctttaagaaggtctcaattccactgggtcctgggtctgggcaagtagtgctgcagttgaccactagggactgtccaaactccaccagggcctgacttggccaaatagaaacctcaaacaactcttccgggacccctgaaatatgaaccacatcggccaggcgcggtggctcacgcctgtaatcccagcactttgggaggccgaggcgggcggatcacaaggtcaagagatcaagaccatcctggccaacatgatgaaaccccgtctctattaaaa

SEQ ID NO: 9852 - RNA, 1961 nt, Homo sapiens
  source 1..1961: mol_type = other RNA
caaagaattctccttttgggcttcccttcttcaccttttagctgcttttgttacattcgaggattagatgtcacaaagcttaggcccctcttgtctaaggaccttggctgtcaagacttagaaatgcaattcccactgctaacctggcccccctgcagtttgaagtgagagctcagactgagggatgtggtctttgccagaggcaatatttgttatgatagataatgaagattccaaatgcccagtgtcctcttatttatcattcaaacctggctgattcaaagattttgctaataaggaatctttagggccagaagtacaatctatttggaatctcaggaaccccaccactaccaccctcactctcactccatgggagacgttattttaatgataaaagaagcctgtatttcaaatgttcacttaacttttactatttccttgtgtatttcaaaaacattagagaaacttttgaaagaatacaactgttttctgctgtaggactcattattatgcaatttgaggggtgggaggggacattttcaggtgtctgcgaatgactgcagattaatttcactgactgacaggctgcggtgggaagtcagctggagatctggagacagcagacctatgccctagttccagctcaatgcaattgtgggcaagtcatttaaccttgatttcttaaattgagaatggaatcacaccaattaattcggcctcaaagaaatgtgggaagtaggagggagccgtaaaacgattcccatttcctgcctcttctcattttgccctttttgttcacttaatgctgcccaaagccacctcagcttcacttgtggtcacaaggtgcaccgtatatcctgaatcccttcactgttacctccgaatcttgtaagtaaatactgtttgtcaggagggactgaacattgtcaaagtcctctggtttcaatttggacacagaggggaaacggtagtagtcctgtttaacaaggtctgccatgaattccttatcaaatgtcagttcatgattcccagcaatcactattttatattcatatggcaggtttcacttgctgatggagccacacagcaggttcagactgctaccttctcctctgaaactcatgcattagggtttcttccatgcttgcaatgggaaaccaggtctaaccagtcattaaacttcttaacctctgagggcagtcccagctcggtgaaatcgcctgtgtggagaaggatgtccccataaggcatctggataccatctgttctggagtgtgtgtctgagatgcagacaaaccgcgtgtggcccgctggttttggagtgtcatatgggatggggtcgaccatatgtacatgtggaggctggaatctgctctggttgatgttgtagtgcgtgaatgcctgggtggggtttgagctgtactcatccaccgttatggtaactttgccttgagaaggaatcccatgtgccatccttcctccctataggcatgagcaattcacaactttacagagcaaaagatggaagcaggcatggtgcgtttcagccaacctctgaatccaaggatctactcatcaataccgctgtgcatttctctgtagagaagaaatccggcggcaacggttacttttcctcggtactcgtcccccgtcgcctagcctcgaccccagcttgggtcgccgggtcgctccgcaggctgcgagcgcggagacccaggcagcggcggagagtgaggttggggcgcggggacggggtgagaaagagccccgagcgagagcggcgcgcgcgggcggccccgggggcggccgcggggcgcagccggagcacaaagctgcgcggtgccttcccctcgtcactgcacctggcctcgggccgccgcgggagcccggggatcgggccaacacaatgcacccaggcctaggccggggcggctcgaacacatcaccccgggactttc

SEQ ID NO: 9853 - RNA, 1562 nt, Homo sapiens
  source 1..1562: mol_type = other RNA
caaagactgcaattacttttgcgccaacctagtaccactacagacaaggaaacagatgcagagaggctaagttacaagggcacacagccataaactttggatctgtggagtgactgggcttcagagtcctcttcctgactgctgttcctatgtcttttgcaaagagaagtctttgacaggtatatgctttattaaaatcatgtttagaaagaaatgagagaatagaattagaaaaaggaatgactgtaggcttcgatgaaaatgacttttgtgactaggtgaaaattgtttggctgggtatcctggaaaattgtcttctgggaatatctatattccagggttcacttttgtcatagaattgtttcttggcccatttaagagagatactttgtttattaataaatcaaacgttttaattttagacatctgtgatcagttcttttaaagagactatatttatttaagtacttcccaagtttagtgcaggggtactacctaccatttattcaggatcatagaggataagttagggtcaaagaaaatagagactgccatgacagcggcttgcttgctttctccccaggaataatgcacaaataatttatagcagctgatatttttcggtgttaacagataataggggaatttgctgaaatttttatttggagcctcggatttaattttaggccactgggctaatttatttttaaatgtaaattaattccagtactttatttgtaaagtttacttgagatctaactgttctaagacatgctgttgcattacaaataagaattgctgcatttattttgatcccattgccagaggcaaaattagtcaaaatttaaaggtatgtagaaatacttttgtaatccttctaaactacattaaatttctggctgactggtggctcacacctgcagtctcagcactttgggaggctgaggttggcagatcaacatggtgaaagcaggtctctactaaaaaataccaaaaaaaattagccgggcgtggtggcgcatgctactcaggaggctgaggcgcgagaatctcttgaacctggaaggtggagtttgcagagagccgagatggtgtcactatactcaagcctgggctacagagtaagacactgtctcaaaaataaataaaattataatttcttagatttaaaaattagatttgttttccaaagacagggtagtagaatatgtagggtacttgtatagatagatatatgttacttaatgcagtactgtctggtgcagggtatcttcacgtggcataatagacccagagcttcaggtctaggctctgtaaagcgaaatgccaaactactgtgtgtgcatttctcgaaagaaaggtgatgtagttttatacaattttgaaacaagtccatgactcccaagggtttaaggaccaatggttcagtgagacatttacagattttgaagtcagaattcagtttgaattctatacacatttactagctatgcaaccttggacaagttacctaacatctgtgagcctcagtttctttacctgtaaaatgatatatttgcccc

SEQ ID NO: 9854 - RNA, 3805 nt, Homo sapiens
  source 1..3805: mol_type = other RNA
caaagcgcttccctttggagctggagtctgggtcccaggcatccagttgaagcacagaggtgcccacgggagcatcctcctggatggaggggtagaacacagcttgggacatctggggtgggttgtcattggcatccgtaacctcgatgtagacttcagttacagaagagaggggcacagaacccctgtccactgctaataccgtcaaccagtagtaagatgcaaattctcggtccaggggtgccagagtctgaatcattcctgtatcttggttgatgctgaaggctgcgagtccagtgccagcacgcaggaagtactggagctccccatccaagccactgtcatcgtcctgggcagccactacaatcacctgagttcccgaggggctgttctcctgcacctggccctggtgcacgaaggaggcaaagtggggagggtggagattctcattcacatccaggacgatcacctccacatggcagagagtcctgcgggctaggggcctcccaccatcactggcccacaggctcagattgtacccagctcgcctctcaaagtccagctctctctccagaatgagcgcccctgtcatcaggtccacccggaaggtcccatgggcgccatccatcagaacatatcgcacttcacctgcggggcccaggtcaggatcagaggcatccagaaatgtcaagacagtcccggggggcaggtcctctggaaccttcagcctgttgtgttctgtgatgcactggggagagttgtcgttgacatcctccaatgtgattatcaggtcagtgacagagaagagctggtggcctttgctgggctgatccctggcctccaccttgagtatgtaccgaggctctgattcgcggtccaggtgtcctgtaacaaccagttccccagtgagagggtggagggagaacttctctgtgggacttagcagggtgtagcgaaccctgccattgtcttccgagtcagcatctttggttgtcagctctgcaattgtggttccaacttctgtgtcctccgagatggttaactggtacccaccgggaggaaatctgggtgcgttgtcattccagtctttcacattcactgtcagcagcttccaggaggacttctggggtgtgcccaggtcatatactgttacattgaggatgtagaaattggtggcttcatagtccaagggagcagctacagtgagcagccctgtctccagctctatgtcaaagcagccctcctcattgccatctgcaatcacatagaccagtttgccattaaaaccagcatcagggtcagtggctgctaggcgggccaagggggtgttgatagggacactctcaaggacatcaatggattgggggaagtggtcctcaaactgtggggtgtaatgattaatctgatatgtgcttaaagaagtgaattcctcatcactggactcctggttctgaagcccaataaagtggaggatagtctttgtgaattgtgtcaatacccctgttttatcacatgttacaggaacttcaaaatgagggtccttcaccacagtaatattcaaagttgtgggtgaggcatagtttttgccatctgaggctgtaatcttcagggaataactggtgggttgaccagcagtaagattgataaaagggcgtttgagggatatcactccggagaaatgatttagatcaaaatactctagttcattgcctgatacaatctcgtattttaggttctgaagctcatccacatctatggctgacatagtcattatcgatttccctactggccagtcttggcggatagaccctgtacagttgacttcttcaaacataggctggttgtcattcaagttcctgagctgaagaaaaatggacacttccttctcccggcgaaaaggggatccccagtctgatgctcttacccggaaggtataaattcttttcatgagttcatagtccatgggtttggaggtggagatgatccccaggtaggggtcaatagaaaatggcaaagcttttggtccagcaatggaataggtgacatatccattttccccatgatcccggtcagtggcagtcacagccaaaacactggtgcctggagggatgttctcatccaaggtaccatcataggaagacctgttgaagaggggggcatggttgttgcagtccacaatgtcaatgaccaccacggtggaggcctggcccggtgaggttctgatgtgtagctgatagtgggctctgtcgtggaagtccatgagctttgtggtggtgatcaacccagttcgagcattaagtttaaatcctacattctctgaagatggctttagaacatactgcaggttggggaaggctggggtgactctcaccatcaccacgcggctgccaggaggggaaaactcactaagctgcactctgtaaacagccttctcgaatttgagggaagacagtttggaaggtggtaggtgaaagcccctgatctgggaataaaaataagggccgctcccactcctggcctggaggctgaggttgaacccatgaaggtactccatccagttgatgtctttgacagacaccaaactgaactcattgctccgggcataagacttgatggctttgaagtgctttccagggtcaccaccaacaacttccactgactccacttcagctcctgagctatttgcatcgaccagtacagtggcataggtggtaccatcattgctgtctggtggagtcaccaccaccgaagcaatggctgggggcttcctgagggcaggctccacatgaaccacaagtgcagccaggctgccaaacccattgccctcagagattttccgcatgcggtccacagctagcacctggagctcatgctttcctcgccaggtgacgttaagcttcccagccacagtgaccacaccgctggtgggatggatggcaaacatctctgaccttgtgttaaaggcataatagaactcagcattctggcctagatcagcatctgtggcagtcaccttgcagatggggctcttcaggggcatgtcctcagagatggtgactctgtacgaaggtggagagaagagaggcttcaggtcattctggtccaggatgtggaccaccacacgggtcaaagcttccaactccaaggtcttctctgtggcttggatgatgagggtgtagctgtctcgcacctctctgttcagaagagctgtgttgctgctctttgtccttattcttaggaagcagaagttgcccaccacatactcctcagttttaaatacattggccacatccccagagatgatccggtacctcactgcccactgtggctccgcgaggtagatgcccattttctcgaagctctccacataggtcttgggagaagaattttcatagatggtggcattgtaatgggagtgtgtgaagtgccaagcagaggaggagagaatcccttctagaggcttctcacaggtcgcacaatggagcaagaatatggcaaaacccagcagggcaatagtcatggtggaaaactcccgaaaccaggccaaggtgagttcagtcgcacttaggttagagtatgcaggaagctgagcatcaggctagctgacatcatggattcagtatcttcctgccagaagtctaacatgtactctatcgagagccctgggggaagaccctagtttgcctcttacagggacatggaacattgagcctctcaaggttcttcatcagcaagatggagacaatcactcctgctctgtctacccaacagaatggattcagaagggatcttggccaggtgtggt

SEQ ID NO: 9855 - RNA, 3716 nt, Homo sapiens
  source 1..3716: mol_type = other RNA
caaagcgcttccctttggagctggagtctgggtcccaggcatccagttgaagcacagaggtgcccacgggagcatcctcctggatggaggggtagaacacagcttgggacatctggggtgggttgtcattggcatccgtaacctcgatgtagacttcagttacagaagagaggggcacagaacccctgtccactgctaataccgtcaaccagtagtaagatgcaaattctcggtccaggggtgccagagtctgaatcattcctgtatcttggttgatgctgaaggctgcgagtccagtgccagcacgcaggaagtactggagctccccatccaagccactgtcatcgtcctgggcagccactacaatcacctgagttcccgaggggctgttctcctgcacctggccctggtgcacgaaggaggcaaagtggggagggtggagattctcattcacatccaggacgatcacctccacatggcagagagtcctgcgggctaggggcctcccaccatcactggcccacaggctcagattgtacccagctcgcctctcaaagtccagctctctctccagaatgagcgcccctgtcatcaggtccacccggaaggtcccatgggcgccatccatcagaacatatcgcacttcacctgcggggcccaggtcaggatcagaggcatccagaaatgtcaagacagtcccggggggcaggtcctctggaaccttcagcctgttgtgttctgtgatgcactggggagagttgtcgttgacatcctccaatgtgattatcaggtcagtgacagagaagagctggtggcctttgctgggctgatccctggcctccaccttgagtatgtaccgaggctctgattcgcggtccaggtgtcctgtaacaaccagttccccagtgagagggtggagggagaacttctctgtgggacttagcagggtgtagcgaaccctgccattgtcttccgagtcagcatctttggttgtcagctctgcaattgtggttccaacttctgtgtcctccgagatggttaactggtacccaccgggaggaaatctgggtgcgttgtcattccagtctttcacattcactgtcagcagcttccaggaggacttctggggtgtgcccaggtcatatactgttacattgaggatgtagaaattggtggcttcatagtccaagggagcagctacagtgagcagccctgtctccagctctatgtcaaagcagccctcctcattgccatctgcaatcacatagaccagtttgccattaaaaccagcatcagggtcagtggctgctaggcgggccaagggggtgttgatagggacactctcaaggacatcaatggattgggggaagtggtcctcaaactgtggggtgtaatgattaatctgatatgtgcttaaagaagtgaattcctcatcactggactcctggttctgaagcccaataaagtggaggatagtctttgtgaattgtgtcaatacccctgttttatcacatgttacaggaacttcaaaatgagggtccttcaccacagtaatattcaaagttgtgggtgaggcatagtttttgccatctgaggctgtaatcttcagggaataactggtgggttgaccagcagtaagattgataaaagggcgtttgagggatatcactccggagaaatgatttagatcaaaatactctagttcattgcctgatacaatctcgtattttaggttctgaagctcatccacatctatggctgacatagtcattatcgatttccctactggccagtcttggcggatagaccctgtacagttgacttcttcaaacataggctggttgtcattcaagttcctgagctgaagaaaaatggacacttccttctcccggcgaaaaggggatccccagtctgatgctcttacccggaaggtataaattcttttcatgagttcatagtccatgggtttggaggtggagatgatccccaggtaggggtcaatagaaaatggcaaagcttttggtccagcaatggaataggtgacatatccattttccccatgatcccggtcagtggcagtcacagccaaaacactggtgcctggagggatgttctcatccaaggtaccatcataggaagacctgttgaagaggggggcatggttgttgcagtccacaatgtcaatgaccaccacggtggaggcctggcccggtgaggttctgatgtgtagctgatagtgggctctgtcgtggaagtccatgagctttgtggtggtgatcaacccagttcgagcattaagtttaaatcctacattctctgaagatggctttagaacatactgcaggttggggaaggctggggtgactctcaccatcaccacgcggctgccaggaggggaaaactcactaagctgcactctgtaaacagccttctcgaatttgagggaagacagtttggaaggtggtaggtgaaagcccctgatctgggaataaaaataagggccgctcccactcctggcctggaggctgaggttgaacccatgaaggtactccatccagttgatgtctttgacagacaccaaactgaactcattgctccgggcataagacttgatggctttgaagtgctttccagggtcaccaccaacaacttccactgactccacttcagctcctgagctatttgcatcgaccagtacagtggcataggtggtaccatcattgctgtctggtggagtcaccaccaccgaagcaatggctgggggcttcctgagggcaggctccacatgaaccacaagtgcagccaggctgccaaacccattgccctcagagattttccgcatgcggtccacagctagcacctggagctcatgctttcctcgccaggtgacgttaagcttcccagccacagtgaccacaccgctggtgggatggatggcaaacatctctgaccttgtgttaaaggcataatagaactcagcattctggcctagatcagcatctgtggcagtcaccttgcagatggggctcttcaggggcatgtcctcagagatggtgactctgtacgaaggtggagagaagagaggcttcaggtcattctggtccaggatgtggaccaccacacgggtcaaagcttccaactccaaggtcttctctgtggcttggatgatgagggtgtagctgtctcgcacctctctgttcagaagagctgtgttgctgctctttgtccttattcttaggaagcagaagttgcccaccacatactcctcagttttaaatacattggccacatccccagagatgatccggtacctcactgcccactgtggctccgcgaggtagatgcccattttctcgaagctctccacataggtcttgggagaagaattttcatagatggtggcattgtaatgggagtgtgtgaagtgccaagcagaggaggagagaatcccttctagaggcttctcacaggtcgcacaatggagcaagaatatggcaaaacccagcagggcaatagtcatggtggaaaactcccgaaaccctctaattacaagaagcttatcacctctcccagcaatcagtttgagctcttagcaattctagctgatgttcagctgagcagcaactcttccacctaatgagcaacgatgtaaatgaggggacggagcagaggaccctctgaccaggcagcagatttcagggtgcccataaagtctg

SEQ ID NO: 9856 - RNA, 3872 nt, Homo sapiens
  source 1..3872: mol_type = other RNA
caaagcgcttccctttggagctggagtctgggtcccaggcatccagttgaagcacagaggtgcccacgggagcatcctcctggatggaggggtagaacacagcttgggacatctggggtgggttgtcattggcatccgtaacctcgatgtagacttcagttacagaagagaggggcacagaacccctgtccactgctaataccgtcaaccagtagtaagatgcaaattctcggtccaggggtgccagagtctgaatcattcctgtatcttggttgatgctgaaggctgcgagtccagtgccagcacgcaggaagtactggagctccccatccaagccactgtcatcgtcctgggcagccactacaatcacctgagttcccgaggggctgttctcctgcacctggccctggtgcacgaaggaggcaaagtggggagggtggagattctcattcacatccaggacgatcacctccacatggcagagagtcctgcgggctaggggcctcccaccatcactggcccacaggctcagattgtacccagctcgcctctcaaagtccagctctctctccagaatgagcgcccctgtcatcaggtccacccggaaggtcccatgggcgccatccatcagaacatatcgcacttcacctgcggggcccaggtcaggatcagaggcatccagaaatgtcaagacagtcccggggggcaggtcctctggaaccttcagcctgttgtgttctgtgatgcactggggagagttgtcgttgacatcctccaatgtgattatcaggtcagtgacagagaagagctggtggcctttgctgggctgatccctggcctccaccttgagtatgtaccgaggctctgattcgcggtccaggtgtcctgtaacaaccagttccccagtgagagggtggagggagaacttctctgtgggacttagcagggtgtagcgaaccctgccattgtcttccgagtcagcatctttggttgtcagctctgcaattgtggttccaacttctgtgtcctccgagatggttaactggtacccaccgggaggaaatctgggtgcgttgtcattccagtctttcacattcactgtcagcagcttccaggaggacttctggggtgtgcccaggtcatatactgttacattgaggatgtagaaattggtggcttcatagtccaagggagcagctacagtgagcagccctgtctccagctctatgtcaaagcagccctcctcattgccatctgcaatcacatagaccagtttgccattaaaaccagcatcagggtcagtggctgctaggcgggccaagggggtgttgatagggacactctcaaggacatcaatggattgggggaagtggtcctcaaactgtggggtgtaatgattaatctgatatgtgcttaaagaagtgaattcctcatcactggactcctggttctgaagcccaataaagtggaggatagtctttgtgaattgtgtcaatacccctgttttatcacatgttacaggaacttcaaaatgagggtccttcaccacagtaatattcaaagttgtgggtgaggcatagtttttgccatctgaggctgtaatcttcagggaataactggtgggttgaccagcagtaagattgataaaagggcgtttgagggatatcactccggagaaatgatttagatcaaaatactctagttcattgcctgatacaatctcgtattttaggttctgaagctcatccacatctatggctgacatagtcattatcgatttccctactggccagtcttggcggatagaccctgtacagttgacttcttcaaacataggctggttgtcattcaagttcctgagctgaagaaaaatggacacttccttctcccggcgaaaaggggatccccagtctgatgctcttacccggaaggtataaattcttttcatgagttcatagtccatgggtttggaggtggagatgatccccaggtaggggtcaatagaaaatggcaaagcttttggtccagcaatggaataggtgacatatccattttccccatgatcccggtcagtggcagtcacagccaaaacactggtgcctggagggatgttctcatccaaggtaccatcataggaagacctgttgaagaggggggcatggttgttgcagtccacaatgtcaatgaccaccacggtggaggcctggcccggtgaggttctgatgtgtagctgatagtgggctctgtcgtggaagtccatgagctttgtggtggtgatcaacccagttcgagcattaagtttaaatcctacattctctgaagatggctttagaacatactgcaggttggggaaggctggggtgactctcaccatcaccacgcggctgccaggaggggaaaactcactaagctgcactctgtaaacagccttctcgaatttgagggaagacagtttggaaggtggtaggtgaaagcccctgatctgggaataaaaataagggccgctcccactcctggcctggaggctgaggttgaacccatgaaggtactccatccagttgatgtctttgacagacaccaaactgaactcattgctccgggcataagacttgatggctttgaagtgctttccagggtcaccaccaacaacttccactgactccacttcagctcctgagctatttgcatcgaccagtacagtggcataggtggtaccatcattgctgtctggtggagtcaccaccaccgaagcaatggctgggggcttcctgagggcaggctccacatgaaccacaagtgcagccaggctgccaaacccattgccctcagagattttccgcatgcggtccacagctagcacctggagctcatgctttcctcgccaggtgacgttaagcttcccagccacagtgaccacaccgctggtgggatggatggcaaacatctctgaccttgtgttaaaggcataatagaactcagcattctggcctagatcagcatctgtggcagtcaccttgcagatggggctcttcaggggcatgtcctcagagatggtgactctgtacgaaggtggagagaagagaggcttcaggtcattctggtccaggatgtggaccaccacacgggtcaaagcttccaactccaaggtcttctctgtggcttggatgatgagggtgtagctgtctcgcacctctctgttcagaagagctgtgttgctgctctttgtccttattcttaggaagcagaagttgcccaccacatactcctcagttttaaatacattggccacatccccagagatgatccggtacctcactgcccactgtggctccgcgaggtagatgcccattttctcgaagctctccacataggtcttgggagaagaattttcatagatggtggcattgtaatgggagtgtgtgaagtgccaagcagaggaggagagaatcccttctagaggcttctcacaggtcgcacaatggagcaagaatatggcaaaacccagcagggcaatagtcatggtggaaaactcccgaaaccctgcttcataaggttgtacagattcatgagaccgattatgtgtgcatcacaaagcacggtgagtgatggctcactggggtgcaggacgccttggctttgatgcgttttatgaggtgcctctctgttctggctccccatataattccattacgcaccctctaattacaagaagcttatcacctctcccagcaatcagtttgagctcttagcaattctagctgatgttcagctgagcagcaactcttccacctaatgagcaacgatgtaaatgaggggacggagcagaggaccctctgaccaggcagcagatttcagggtgcccataaagtctg

SEQ ID NO: 9857 - RNA, 3874 nt, Homo sapiens
  source 1..3874: mol_type = other RNA
caaagcgcttccctttggagctggagtctgggtcccaggcatccagttgaagcacagaggtgcccacgggagcatcctcctggatggaggggtagaacacagcttgggacatctggggtgggttgtcattggcatccgtaacctcgatgtagacttcagttacagaagagaggggcacagaacccctgtccactgctaataccgtcaaccagtagtaagatgcaaattctcggtccaggggtgccagagtctgaatcattcctgtatcttggttgatgctgaaggctgcgagtccagtgccagcacgcaggaagtactggagctccccatccaagccactgtcatcgtcctgggcagccactacaatcacctgagttcccgaggggctgttctcctgcacctggccctggtgcacgaaggaggcaaagtggggagggtggagattctcattcacatccaggacgatcacctccacatggcagagagtcctgcgggctaggggcctcccaccatcactggcccacaggctcagattgtacccagctcgcctctcaaagtccagctctctctccagaatgagcgcccctgtcatcaggtccacccggaaggtcccatgggcgccatccatcagaacatatcgcacttcacctgcggggcccaggtcaggatcagaggcatccagaaatgtcaagacagtcccggggggcaggtcctctggaaccttcagcctgttgtgttctgtgatgcactggggagagttgtcgttgacatcctccaatgtgattatcaggtcagtgacagagaagagctggtggcctttgctgggctgatccctggcctccaccttgagtatgtaccgaggctctgattcgcggtccaggtgtcctgtaacaaccagttccccagtgagagggtggagggagaacttctctgtgggacttagcagggtgtagcgaaccctgccattgtcttccgagtcagcatctttggttgtcagctctgcaattgtggttccaacttctgtgtcctccgagatggttaactggtacccaccgggaggaaatctgggtgcgttgtcattccagtctttcacattcactgtcagcagcttccaggaggacttctggggtgtgcccaggtcatatactgttacattgaggatgtagaaattggtggcttcatagtccaagggagcagctacagtgagcagccctgtctccagctctatgtcaaagcagccctcctcattgccatctgcaatcacatagaccagtttgccattaaaaccagcatcagggtcagtggctgctaggcgggccaagggggtgttgatagggacactctcaaggacatcaatggattgggggaagtggtcctcaaactgtggggtgtaatgattaatctgatatgtgcttaaagaagtgaattcctcatcactggactcctggttctgaagcccaataaagtggaggatagtctttgtgaattgtgtcaatacccctgttttatcacatgttacaggaacttcaaaatgagggtccttcaccacagtaatattcaaagttgtgggtgaggcatagtttttgccatctgaggctgtaatcttcagggaataactggtgggttgaccagcagtaagattgataaaagggcgtttgagggatatcactccggagaaatgatttagatcaaaatactctagttcattgcctgatacaatctcgtattttaggttctgaagctcatccacatctatggctgacatagtcattatcgatttccctactggccagtcttggcggatagaccctgtacagttgacttcttcaaacataggctggttgtcattcaagttcctgagctgaagaaaaatggacacttccttctcccggcgaaaaggggatccccagtctgatgctcttacccggaaggtataaattcttttcatgagttcatagtccatgggtttggaggtggagatgatccccaggtaggggtcaatagaaaatggcaaagcttttggtccagcaatggaataggtgacatatccattttccccatgatcccggtcagtggcagtcacagccaaaacactggtgcctggagggatgttctcatccaaggtaccatcataggaagacctgttgaagaggggggcatggttgttgcagtccacaatgtcaatgaccaccacggtggaggcctggcccggtgaggttctgatgtgtagctgatagtgggctctgtcgtggaagtccatgagctttgtggtggtgatcaacccagttcgagcattaagtttaaatcctacattctctgaagatggctttagaacatactgcaggttggggaaggctggggtgactctcaccatcaccacgcggctgccaggaggggaaaactcactaagctgcactctgtaaacagccttctcgaatttgagggaagacagtttggaaggtggtaggtgaaagcccctgatctgggaataaaaataagggccgctcccactcctggcctggaggctgaggttgaacccatgaaggtactccatccagttgatgtctttgacagacaccaaactgaactcattgctccgggcataagacttgatggctttgaagtgctttccagggtcaccaccaacaacttccactgactccacttcagctcctgagctatttgcatcgaccagtacagtggcataggtggtaccatcattgctgtctggtggagtcaccaccaccgaagcaatggctgggggcttcctgagggcaggctccacatgaaccacaagtgcagccaggctgccaaacccattgccctcagagattttccgcatgcggtccacagctagcacctggagctcatgctttcctcgccaggtgacgttaagcttcccagccacagtgaccacaccgctggtgggatggatggcaaacatctctgaccttgtgttaaaggcataatagaactcagcattctggcctagatcagcatctgtggcagtcaccttgcagatggggctcttcaggggcatgtcctcagagatggtgactctgtacgaaggtggagagaagagaggcttcaggtcattctggtccaggatgtggaccaccacacgggtcaaagcttccaactccaaggtcttctctgtggcttggatgatgagggtgtagctgtctcgcacctctctgttcagaagagctgtgttgctgctctttgtccttattcttaggaagcagaagttgcccaccacatactcctcagttttaaatacattggccacatccccagagatgatccggtacctcactgcccactgtggctccgcgaggtagatgcccattttctcgaagctctccacataggtcttgggagaagaattttcatagatggtggcattgtaatgggagtgtgtgaagtgccaagcagaggaggagagaatcccttctagaggcttctcacaggtcgcacaatggagcaagaatatggcaaaacccagcagggcaatagtcatggtggaaaactcccgaaaccctgcttcataaggttgtacagattcatgagaccgattatgtgtgcatcacaaagcacggtgagtgatggctcactggggtgcaggacgccttggctttgatgcgttttatgaggtgcctctctgttctggctccccatataattccattacgcaccctctaattacaagaagcttatcacctctcccagcaatcagtttgagctcttagcaattctagctgatgttcagctgagcagcaactcttccacctgagcaattatccacttggctgattgccactcaagcctccaagtttggtccgattaggcattaaccagaggaagggtggcgggg

SEQ ID NO: 9858 - RNA, 3707 nt, Homo sapiens
  source 1..3707: mol_type = other RNA
caaagcgcttccctttggagctggagtctgggtcccaggcatccagttgaagcacagaggtgcccacgggagcatcctcctggatggaggggtagaacacagcttgggacatctggggtgggttgtcattggcatccgtaacctcgatgtagacttcagttacagaagagaggggcacagaacccctgtccactgctaataccgtcaaccagtagtaagatgcaaattctcggtccaggggtgccagagtctgaatcattcctgtatcttggttgatgctgaaggctgcgagtccagtgccagcacgcaggaagtactggagctccccatccaagccactgtcatcgtcctgggcagccactacaatcacctgagttcccgaggggctgttctcctgcacctggccctggtgcacgaaggaggcaaagtggggagggtggagattctcattcacatccaggacgatcacctccacatggcagagagtcctgcgggctaggggcctcccaccatcactggcccacaggctcagattgtacccagctcgcctctcaaagtccagctctctctccagaatgagcgcccctgtcatcaggtccacccggaaggtcccatgggcgccatccatcagaacatatcgcacttcacctgcggggcccaggtcaggatcagaggcatccagaaatgtcaagacagtcccggggggcaggtcctctggaaccttcagcctgttgtgttctgtgatgcactggggagagttgtcgttgacatcctccaatgtgattatcaggtcagtgacagagaagagctggtggcctttgctgggctgatccctggcctccaccttgagtatgtaccgaggctctgattcgcggtccaggtgtcctgtaacaaccagttccccagtgagagggtggagggagaacttctctgtgggacttagcagggtgtagcgaaccctgccattgtcttccgagtcagcatctttggttgtcagctctgcaattgtggttccaacttctgtgtcctccgagatggttaactggtacccaccgggaggaaatctgggtgcgttgtcattccagtctttcacattcactgtcagcagcttccaggaggacttctggggtgtgcccaggtcatatactgttacattgaggatgtagaaattggtggcttcatagtccaagggagcagctacagtgagcagccctgtctccagctctatgtcaaagcagccctcctcattgccatctgcaatcacatagaccagtttgccattaaaaccagcatcagggtcagtggctgctaggcgggccaagggggtgttgatagggacactctcaaggacatcaatggattgggggaagtggtcctcaaactgtggggtgtaatgattaatctgatatgtgcttaaagaagtgaattcctcatcactggactcctggttctgaagcccaataaagtggaggatagtctttgtgaattgtgtcaatacccctgttttatcacatgttacaggaacttcaaaatgagggtccttcaccacagtaatattcaaagttgtgggtgaggcatagtttttgccatctgaggctgtaatcttcagggaataactggtgggttgaccagcagtaagattgataaaagggcgtttgagggatatcactccggagaaatgatttagatcaaaatactctagttcattgcctgatacaatctcgtattttaggttctgaagctcatccacatctatggctgacatagtcattatcgatttccctactggccagtcttggcggatagaccctgtacagttgacttcttcaaacataggctggttgtcattcaagttcctgagctgaagaaaaatggacacttccttctcccggcgaaaaggggatccccagtctgatgctcttacccggaaggtataaattcttttcatgagttcatagtccatgggtttggaggtggagatgatccccaggtaggggtcaatagaaaatggcaaagcttttggtccagcaatggaataggtgacatatccattttccccatgatcccggtcagtggcagtcacagccaaaacactggtgcctggagggatgttctcatccaaggtaccatcataggaagacctgttgaagaggggggcatggttgttgcagtccacaatgtcaatgaccaccacggtggaggcctggcccggtgaggttctgatgtgtagctgatagtgggctctgtcgtggaagtccatgagctttgtggtggtgatcaacccagttcgagcattaagtttaaatcctacattctctgaagatggctttagaacatactgcaggttggggaaggctggggtgactctcaccatcaccacgcggctgccaggaggggaaaactcactaagctgcactctgtaaacagccttctcgaatttgagggaagacagtttggaaggtggtaggtgaaagcccctgatctgggaataaaaataagggccgctcccactcctggcctggaggctgaggttgaacccatgaaggtactccatccagttgatgtctttgacagacaccaaactgaactcattgctccgggcataagacttgatggctttgaagtgctttccagggtcaccaccaacaacttccactgactccacttcagctcctgagctatttgcatcgaccagtacagtggcataggtggtaccatcattgctgtctggtggagtcaccaccaccgaagcaatggctgggggcttcctgagggcaggctccacatgaaccacaagtgcagccaggctgccaaacccattgccctcagagattttccgcatgcggtccacagctagcacctggagctcatgctttcctcgccaggtgacgttaagcttcccagccacagtgaccacaccgctggtgggatggatggcaaacatctctgaccttgtgttaaaggcataatagaactcagcattctggcctagatcagcatctgtggcagtcaccttgcagatggggctcttcaggggcatgtcctcagagatggtgactctgtacgaaggtggagagaagagaggcttcaggtcattctggtccaggatgtggaccaccacacgggtcaaagcttccaactccaaggtcttctctgtggcttggatgatgagggtgtagctgtctcgcacctctctgttcagaagagctgtgttgctgctctttgtccttattcttaggaagcagaagttgcccaccacatactcctcagttttaaatacattggccacatccccagagatgatccggtacctcactgcccactgtggctccgcgaggtagatgcccattttctcgaagctctccacataggtcttgggagaagaattttcatagatggtggcattgtaatgggagtgtgtgaagtgccaagcagaggaggagagaatcccttctagaggcttctcacaggtcgcacaatggagcaagaatatggcaaaacccagcagggcaatagtcatggtggaaaactcccgaaaccctgtgcccttcaggtaggggagggtgccccagagcaggctgctgggctggcgcccctctcacgagggccaggctgacaggctcctgagggaggtgcagagactcggagcaggaaggcgcgcagcccgcagccggagaggctgctgagaaagttggagtaggtgtgtc

SEQ ID NO: 9859 - RNA, 4108 nt, Homo sapiens
  source 1..4108: mol_type = other RNA
caaagcgcttccctttggagctggagtctgggtcccaggcatccagttgaagcacagaggtgcccacgggagcatcctcctggatggaggggtagaacacagcttgggacatctggggtgggttgtcattggcatccgtaacctcgatgtagacttcagttacagaagagaggggcacagaacccctgtccactgctaataccgtcaaccagtagtaagatgcaaattctcggtccaggggtgccagagtctgaatcattcctgtatcttggttgatgctgaaggctgcgagtccagtgccagcacgcaggaagtactggagctccccatccaagccactgtcatcgtcctgggcagccactacaatcacctgagttcccgaggggctgttctcctgcacctggccctggtgcacgaaggaggcaaagtggggagggtggagattctcattcacatccaggacgatcacctccacatggcagagagtcctgcgggctaggggcctcccaccatcactggcccacaggctcagattgtacccagctcgcctctcaaagtccagctctctctccagaatgagcgcccctgtcatcaggtccacccggaaggtcccatgggcgccatccatcagaacatatcgcacttcacctgcggggcccaggtcaggatcagaggcatccagaaatgtcaagacagtcccggggggcaggtcctctggaaccttcagcctgttgtgttctgtgatgcactggggagagttgtcgttgacatcctccaatgtgattatcaggtcagtgacagagaagagctggtggcctttgctgggctgatccctggcctccaccttgagtatgtaccgaggctctgattcgcggtccaggtgtcctgtaacaaccagttccccagtgagagggtggagggagaacttctctgtgggacttagcagggtgtagcgaaccctgccattgtcttccgagtcagcatctttggttgtcagctctgcaattgtggttccaacttctgtgtcctccgagatggttaactggtacccaccgggaggaaatctgggtgcgttgtcattccagtctttcacattcactgtcagcagcttccaggaggacttctggggtgtgcccaggtcatatactgttacattgaggatgtagaaattggtggcttcatagtccaagggagcagctacagtgagcagccctgtctccagctctatgtcaaagcagccctcctcattgccatctgcaatcacatagaccagtttgccattaaaaccagcatcagggtcagtggctgctaggcgggccaagggggtgttgatagggacactctcaaggacatcaatggattgggggaagtggtcctcaaactgtggggtgtaatgattaatctgatatgtgcttaaagaagtgaattcctcatcactggactcctggttctgaagcccaataaagtggaggatagtctttgtgaattgtgtcaatacccctgttttatcacatgttacaggaacttcaaaatgagggtccttcaccacagtaatattcaaagttgtgggtgaggcatagtttttgccatctgaggctgtaatcttcagggaataactggtgggttgaccagcagtaagattgataaaagggcgtttgagggatatcactccggagaaatgatttagatcaaaatactctagttcattgcctgatacaatctcgtattttaggttctgaagctcatccacatctatggctgacatagtcattatcgatttccctactggccagtcttggcggatagaccctgtacagttgacttcttcaaacataggctggttgtcattcaagttcctgagctgaagaaaaatggacacttccttctcccggcgaaaaggggatccccagtctgatgctcttacccggaaggtataaattcttttcatgagttcatagtccatgggtttggaggtggagatgatccccaggtaggggtcaatagaaaatggcaaagcttttggtccagcaatggaataggtgacatatccattttccccatgatcccggtcagtggcagtcacagccaaaacactggtgcctggagggatgttctcatccaaggtaccatcataggaagacctgttgaagaggggggcatggttgttgcagtccacaatgtcaatgaccaccacggtggaggcctggcccggtgaggttctgatgtgtagctgatagtgggctctgtcgtggaagtccatgagctttgtggtggtgatcaacccagttcgagcattaagtttaaatcctacattctctgaagatggctttagaacatactgcaggttggggaaggctggggtgactctcaccatcaccacgcggctgccaggaggggaaaactcactaagctgcactctgtaaacagccttctcgaatttgagggaagacagtttggaaggtggtaggtgaaagcccctgatctgggaataaaaataagggccgctcccactcctggcctggaggctgaggttgaacccatgaaggtactccatccagttgatgtctttgacagacaccaaactgaactcattgctccgggcataagacttgatggctttgaagtgctttccagggtcaccaccaacaacttccactgactccacttcagctcctgagctatttgcatcgaccagtacagtggcataggtggtaccatcattgctgtctggtggagtcaccaccaccgaagcaatggctgggggcttcctgagggcaggctccacatgaaccacaagtgcagccaggctgccaaacccattgccctcagagattttccgcatgcggtccacagctagcacctggagctcatgctttcctcgccaggtgacgttaagcttcccagccacagtgaccacaccgctggtgggatggatggcaaacatctctgaccttgtgttaaaggcataatagaactcagcattctggcctagatcagcatctgtggcagtcaccttgcagatggggctcttcaggggcatgtcctcagagatggtgactctgtacgaaggtggagagaagagaggcttcaggtcattctggtccaggatgtggaccaccacacgggtcaaagcttccaactccaaggtcttctctgtggcttggatgatgagggtgtagctgtctcgcacctctctgttcagaagagctgtgttgctgctctttgtccttattcttaggaagcagaagttgcccaccacatactcctcagttttaaatacattggccacatccccagagatgatccggtacctcactgcccactgtggctccgcgaggtagatgcccattttctcgaagctctccacataggtcttgggagaagaattttcatagatggtggcattgtaatgggagtgtgtgaagtgccaagcagaggaggagagaatcccttctagaggcttctcacaggtcgcacaatggagcaagaatatggcaaaacccagcagggcaatagtcatggtggaaaactcccgaaaccctgtgcccttcaggtaggggagggtgccccagagcaggctgctgggctggcgcccctctcacgagggccaggctgacaggctcctgagggaggtgcagagactcggagcaggaaggcgcgcagcccgcagccggagaggctgctgagaaagttggagtaggtgtgtcccagcccaggaggaggaggaggaggaaaaaggaggtgggagaattgaggcggatcatcccctcctgccagctctctgtctcacggagagggagggaggaagccaactggtttgtggcccagaactcacggtggggaatcaagtcatggaaaatgaaaggagctgagaaatcaggcccatctccacctcccttcttggtttcaccgagggataaactgaggccctggacaggtagtgttgccccaggtcacacagtcacacagagaccacaagggaactagaaaaggtcacttggctgtcagaacagtagtgttctctccactcctccatgcttcagatctgagactgacaaccacagcacccctttccccagggctttggagacggacagatttggttcga

SEQ ID NO: 9860 - RNA, 66 nt, Homo sapiens
  source 1..66: mol_type = other RNA
caaaggtatttgtggtttttgccgttaaaagtatggcaaaatccgcaattacttttgcaccaacct

SEQ ID NO: 9861 - RNA, 1468 nt, Homo sapiens
  source 1..1468: mol_type = other RNA
caaagtgctcatagtgcaggtagagcccgatgcggtgggggtggccggccacgggcaggggtacccgggggcaggcaaaggcttcgtacacccggccctccttcaggccgatcagccacacgccgtgctcgggggacctgttcagcttgcccttacggctggctgtgcccttgatgacccccaggcgccagtcgctcttgctgcccaccaccacctcccagtagtggcggccgcaggagaagccgcggctggccaggacgcaggtgctgtagtcgaagcgctcaggctggctggctcgccgctgggccagaagcccgcactgcaccaccgtgttgcccttggagagctccaggagtgggtgggcagtggcagggtccaacttgagaggctccggggctggcaaaactttccggaagagccttttccacacggtcagcttgatgtcagcctggtggaggcctggcttgaaggagatggggctgaatgcgccttctaagggccgggcctgcggcatctctgctctggaggccatggagtggaaccggatgaacttgtggtggtcctcattgccgaactgttccagcacacactcggcttgggccagccgctcccgggttccctgggcctgctccagctgcatgtccagggaggccaccaggccacgggtgtgaccccctatcccctccaggcagcgggccttctcctcatccaccaggtggtgcagctcctggaactcgcggcggatcacccagctgaagacatccgactcattgacgattcgggtccggttgttcaccagtttggcgatgagctcatccacctttttctgctcctgcttcagctcagagatgagggctgcgagctcctccttcatgcggctgtagacggtggagacgggcgtgaccgggtggtgttggtgggagcccagcagaccgcagaggccacagatgagctcctggtccttctcgcagaaaaggctgagcgggttccggtggtgcacgcagaccttgggctccgggtccccagggagcctcagggcttcgatcaccctggccagggagacgttgggcagggagctgctgccgtccaccgcctgccggcacacggggcagcgcagctcggcatccaggtggcaggacagggaaaccaggcagcccttgcagtaagagtggccacactgcagcatcaggggctccttgaagacctccaggcagatgggacactgaagccggtcctccagctctggcaggctcacctgccaagccatccacactcactgcccgggccagcctccggcccctgtaagtgccccatcgtgctctctgtcgctccagttagatgccccatcctgccccgcgagctccaattacgtgccccacctaaccccccacgtccgtgcctcatcatgacccgcacgctatggttacatgccccgcctcgcgctaccgcgcgtgccccatcatgctct

SEQ ID NO: 9862 - RNA, 1396 nt, Homo sapiens
  source 1..1396: mol_type = other RNA
caaagtgctcatagtgcaggtagagcccgatgcggtgggggtggccggccacgggcaggggtacccgggggcaggcaaaggcttcgtacacccggccctccttcaggccgatcagccacacgccgtgctcgggggacctgttcagcttgcccttacggctggctgtgcccttgatgacccccaggcgccagtcgctcttgctgcccaccaccacctcccagtagtggcggccgcaggagaagccgcggctggccaggacgcaggtgctgtagtcgaagcgctcaggctggctggctcgccgctgggccagaagcccgcactgcaccaccgtgttgcccttggagagctccaggagtgggtgggcagtggcagggtccaacttgagaggctccggggctggcaaaactttccggaagagccttttccacacggtcagcttgatgtcagcctggtggaggcctggcttgaaggagatggggctgaatgcgccttctaagggccgggcctgcggcatctctgctctggaggccatggagtggaaccggatgaacttgtggtggtcctcattgccgaactgttccagcacacactcggcttgggccagccgctcccgggttccctgggcctgctccagctgcatgtccagggaggccaccaggccacgggtgtgaccccctatcccctccaggcagcgggccttctcctcatccaccaggtggtgcagctcctggaactcgcggcggatcacccagctgaagacatccgactcattgacgattcgggtccggttgttcaccagtttggcgatgagctcatccacctttttctgctcctgcttcagctcagagatgagggctgcgagctcctccttcatgcggctgtagacggtggagacgggcgtgaccgggtggtgttggtgggagcccagcagaccgcagaggccacagatgagctcctggtccttctcgcagaaaaggctgagcgggttccggtggtgcacgcagaccttgggctccgggtccccagggagcctcagggcttcgatcaccctggccagggagacgttgggcagggagctgctgccgtccaccgcctgccggcacacggggcagcgcagctcggcatccaggtggcaggacagggaaaccaggcagcccttgcagtaagagtggccacactgcagcatcaggggctccttgaagacctccaggcagatgggacactgaagccggtcctccagctctggcaggctcacctgccaagccatccacactcactgcccgggctggcttctcacaatccgctgggcctcccactacagcctcaagccagcatcactggctttccttcttcccagcagggaacagcaggcacagagtcagaagtgggaaatgca

SEQ ID NO: 9863 - RNA, 1021 nt, Homo sapiens
  source 1..1021: mol_type = other RNA
caaagtgctcatagtgcaggtagagcccgatgcggtgggggtggccggccacgggcaggggtacccgggggcaggcaaaggcttcgtacacccggccctccttcaggccgatcagccacacgccgtgctcgggggacctgttcagcttgcccttacggctggctgtgcccttgatgacccccaggcgccagtcgctcttgctgcccaccaccacctcccagtagtggcggccgcaggagaagccgcggctggccaggacgcaggtgctgtagtcgaagcgctcaggctggctggctcgccgctgggccagaagcccgcactgcaccaccgtgttgcccttggagagctccaggagtgggtgggcagtggcagggtccaacttgagaggctccggggctggcaaaactttccggaagagccttttccacacggtcagcttgatgtcagcctggtggaggcctggcttgaaggagatggggctgaatgcgccttctaagggccgggcctgcggcatctctgctctggaggccatggagtggaacttccggatgaacttgtggtggtcctcattgccgaactgttccagcacacactcggcttgggccagccgctcccgggttccctgggcctgctccagctgcatgtccagggaggccaccaggccacgggtgtgaccccctatcccctccaggcagcgggccttctcctcatccaccaggtggtgcagctcctggaactcgcggcggatcacccagctgaagacatccgactcattctgggacagggagggctggtcagacgattcgggtccggttgttcaccagtttggcgatgagctcatccacctttttctgctcctgcttcagctcagagatgagggctgcgagctcctcccagcctccggcccctgtaagtgccccatcgtgctctctgtcgctccagttagatgccccatcctgccccgcgagctccaattacgtgccccacctaaccccccacgtccgtgcctcatcatgacccg

SEQ ID NO: 9864 - RNA, 1471 nt, Homo sapiens
  source 1..1471: mol_type = other RNA
caaagtgctcatagtgcaggtagagcccgatgcggtgggggtggccggccacgggcaggggtacccgggggcaggcaaaggcttcgtacacccggccctccttcaggccgatcagccacacgccgtgctcgggggacctgttcagcttgcccttacggctggctgtgcccttgatgacccccaggcgccagtcgctcttgctgcccaccaccacctcccagtagtggcggccgcaggagaagccgcggctggccaggacgcaggtgctgtagtcgaagcgctcaggctggctggctcgccgctgggccagaagcccgcactgcaccaccgtgttgcccttggagagctccaggagtgggtgggcagtggcagggtccaacttgagaggctccggggctggcaaaactttccggaagagccttttccacacggtcagcttgatgtcagcctggtggaggcctggcttgaaggagatggggctgaatgcgccttctaagggccgggcctgcggcatctctgctctggaggccatggagtggaacttccggatgaacttgtggtggtcctcattgccgaactgttccagcacacactcggcttgggccagccgctcccgggttccctgggcctgctccagctgcatgtccagggaggccaccaggccacgggtgtgaccccctatcccctccaggcagcgggccttctcctcatccaccaggtggtgcagctcctggaactcgcggcggatcacccagctgaagacatccgactcattgacgattcgggtccggttgttcaccagtttggcgatgagctcatccacctttttctgctcctgcttcagctcagagatgagggctgcgagctcctccttcatgcggctgtagacggtggagacgggcgtgaccgggtggtgttggtgggagcccagcagaccgcagaggccacagatgagctcctggtccttctcgcagaaaaggctgagcgggttccggtggtgcacgcagaccttgggctccgggtccccagggagcctcagggcttcgatcaccctggccagggagacgttgggcagggagctgctgccgtccaccgcctgccggcacacggggcagcgcagctcggcatccaggtggcaggacagggaaaccaggcagcccttgcagtaagagtggccacactgcagcatcaggggctccttgaagacctccaggcagatgggacactgaagccggtcctccagctctggcaggctcacctgccaagccatccacactcactgcccgggccagcctccggcccctgtaagtgccccatcgtgctctctgtcgctccagttagatgccccatcctgccccgcgagctccaattacgtgccccacctaaccccccacgtccgtgcctcatcatgacccgcacgctatggttacatgccccgcctcgcgctaccgcgcgtgccccatcatgctct

SEQ ID NO: 9865 - RNA, 1399 nt, Homo sapiens
  source 1..1399: mol_type = other RNA
caaagtgctcatagtgcaggtagagcccgatgcggtgggggtggccggccacgggcaggggtacccgggggcaggcaaaggcttcgtacacccggccctccttcaggccgatcagccacacgccgtgctcgggggacctgttcagcttgcccttacggctggctgtgcccttgatgacccccaggcgccagtcgctcttgctgcccaccaccacctcccagtagtggcggccgcaggagaagccgcggctggccaggacgcaggtgctgtagtcgaagcgctcaggctggctggctcgccgctgggccagaagcccgcactgcaccaccgtgttgcccttggagagctccaggagtgggtgggcagtggcagggtccaacttgagaggctccggggctggcaaaactttccggaagagccttttccacacggtcagcttgatgtcagcctggtggaggcctggcttgaaggagatggggctgaatgcgccttctaagggccgggcctgcggcatctctgctctggaggccatggagtggaacttccggatgaacttgtggtggtcctcattgccgaactgttccagcacacactcggcttgggccagccgctcccgggttccctgggcctgctccagctgcatgtccagggaggccaccaggccacgggtgtgaccccctatcccctccaggcagcgggccttctcctcatccaccaggtggtgcagctcctggaactcgcggcggatcacccagctgaagacatccgactcattgacgattcgggtccggttgttcaccagtttggcgatgagctcatccacctttttctgctcctgcttcagctcagagatgagggctgcgagctcctccttcatgcggctgtagacggtggagacgggcgtgaccgggtggtgttggtgggagcccagcagaccgcagaggccacagatgagctcctggtccttctcgcagaaaaggctgagcgggttccggtggtgcacgcagaccttgggctccgggtccccagggagcctcagggcttcgatcaccctggccagggagacgttgggcagggagctgctgccgtccaccgcctgccggcacacggggcagcgcagctcggcatccaggtggcaggacagggaaaccaggcagcccttgcagtaagagtggccacactgcagcatcaggggctccttgaagacctccaggcagatgggacactgaagccggtcctccagctctggcaggctcacctgccaagccatccacactcactgcccgggctggcttctcacaatccgctgggcctcccactacagcctcaagccagcatcactggctttccttcttcccagcagggaacagcaggcacagagtcagaagtgggaaatgca

SEQ ID NO: 9866 - RNA, 4635 nt, Homo sapiens
  source 1..4635: mol_type = other RNA
caaagtgcttacagtgcaggtagaaactctgtaaccttaagcatgtaaactacatagaataaaactgtttccactgcatttctgtccttcaaagtggccaacctgattaagtcagccttaatcactgctgctgtcagtttcacgactaaaggtcatattgactaagtagtcatcagctgaccacctcgctgtatcagccagcaacgaggggaaggtgaagaaacatgataggccatatagaatctgccctatgtttacttttttaacccagataattatttttgtgtgcagtatctaagctcctgattgtgtaacctgggacttctggcaccttttgttccattcattttatgtataaaatgcatgccaaagcacactgtgccctctggtacccttgcttccaatcgccaaccatgctcatttccttcctttttttgtggtccctttttgtggtgatcattttaaaccacgtcatccaacaaatgttttatggtcaaccttagcttgttcataagccatagcaactgaaagattaaactcttaaatatgtgtctgggcagtggctattaaatagcaaaaaacaatcagattttagtattttattatttccttgtaaaatggctgaactaaattaaacccttgtttcccatttgttctataatttatagtgaaactgagaacaaaactatctttataaatgatagctaaaagtatttccagatatttaaacaatttaaaataaatttcttctgcagagatgcaaagcatctcaacactggaatgaacaaatgccttaaattcaatggagtaaacctttagaatgaagaggaactgtcatttcacccaagccgaagacaacagccttatgcacttgtgtgctctgtctttgctgcttctcgtgtttcaagcctttcctgtgggatcagcacagcaaagtgcaacttaccaaatggtttaatgactggttaattctttcttctcccaatggaaaagcaatggcaacacaacagtagactgctggcttgacaatcttaaacgtgagcctttgcacatgtaggtttatcatcatttgagtatacgactaagcaagtcaatgaactttttttttttttttagcagtttaatttggtcctgagaatgttgcagtctttattaccccttttgcattaatccacttttctaaccaccttttaagctttaatttttaacactatacaccaagtctttgaaatcagtgatctgttatttaactctaaagcatttgacacttcttgccttaacagttttaaaaaccacacacaaaaaaactctgtaagtaatacagtaggccaaaagtttcatcctatctatcttgcagtttacctatctgatctgatctctgtaattatagttctgtcatttaaaatatactatttaaatctaatttttacatttcaaaaattatcttcagtagtaactaagtatattttctgtggattctgagaatgttatttttcagaatgtgagaatatatatgtacatttataatcttgtgactttaaagtctgttttcagatacagtatgtaaatacttgtaaaaaaatttgtataattttgtgataatgtagtttcccaaaaaaattatttagaaggcattatgttattagtaaatgagagcactgtatagaactgttcctattttctgcacttgccattccagctgcctccactgtccatacccacctcattcatcctgtcacagaaggcaggaaaactgggaactttaccaaagtagcactcagcctgagaggcctgtataatcatgcttttcaaactaaattcacttaaaaattaaaaagcagaattgaatattttaagcagcctcagtacctttggccaatgctgttttcatggtggattatgaacattatataatctttgggaaaagtgaaagtagtacaatttttagaataatgacaactgcctcactgcatctctccactcacacagcaaccgtgtagccccctaagctgcagtaccatgactaaccatgatgtcaatttcatatgctgatcctcacaacagcagtgcacaaacatgccccaaatattttaacagaatttagctcttccttaagctgtcttttcatagtaaaaacaaaacaaaaacacccaatgttaaaaccacataataaacttacaaacttgaaaaattagacacttcagatagataggcaataaaacttcatattatgaaagcaatatattccaagtttcaaagatttgacaagttctgtagagtatctttcatcagtacatgaaaacttccaaactgcatgatcttctgccaggcaggactgggtgctattcgctggtttgaggtcgaatccatttcaaggcatgtcgtggtgggacattaatggtgggatggtagaatgtgcagtccggtcttgtacattgagtgttaaacctacaatgttttggatgatagaagggacattccatcttcttacaagcagggaagtaacggcagagctgactactggaaggtggtgctggtggtgcaactgctggttttggagacagtactggaattcttctactcacatgagtgaagggacaatctggtttagtacactttgcatcatatttacaatttgggtgaacaaacaaacatttttcagcaaatttacaattggggaaggctttgcagggtgagatggggtgatggtaggcacactcatccccatttttacaagcaggccagtacttgcagcgctccaaaagtttttctggtttctgtgccacactcagttcactcatctcagcatttgggtcctcaagctgcctgctcagcaagtgcaactgctgtgggtggaggagacctctgagtcccttgtttgaggctgcagtttggtttacgggtttcattccttcaaagcacatgtcctcctcttgatctgacatgtatcctggggggctggggacaccatccagcgtcactataaacttgggacttgcaggtttatctggttgtacaagatctcgtgtctgcataaggtgtcctgaaagtacccgaagggaatctgcagtcttcatccccgactcttggtttggtgccactactacttcctcagacagctttggcttcttcagaataaatgatcttgtgtctgcatggaccatggattccatgtcatagtaatcttgactcatctgcagagtttctgccattactgggtcgatttgcagtcgggataataattgcctctgttgagttccttgatttttttctacagaatctccttttgtttcctcttctttaatggggggacttattctgggggtcctactttgtccctggaccacttctgctagcaattcttcttgagaagttcgagttctgggagcaactggaagtgtctgtttctgtggaactgtagagtagttagttgtttttgttacggattcttgagcttcagatatagccttcaaaatcagattcttgttagcttgtttagaaggtggaagagaaggtctcctttcaggctttgcaggcacagacacactgctggagatgcttcctgttcgagacccgtaatcatcatcttcttcctcctcttctccatcatgattgaatttttttactttaacaactgaacttaccacaggcaactttctcttccgaaagttttcatcctccatactcattttctccgagttgtttctaaagaacggactatacgtttcttctaagctgttaagcacctctggttcacacaaacgtcctgtttcatatacccaactactctgcatatcaagctgcttggcagcatgaatactattctgctgctgttgaaattgcaacctgtttaaatgaacaccactatctgcatttctacttgcaggtggtcgataaatttcaatagaagggcgagaagaaccatatgtaagtgtcactgtaggttttttctgagataagggattctcctgcacaaagttgaggtcttcgtcaatgagatcatctggttctggcttaatatcaatcacatcttcagagggtgctggctccctcaaaggtttcactgttgacattagtcgggttgcagctccatcatcgtaagtctgtctgacatttgtggtttttgactcctgcgaacttgtagaaactctggaatctcttttttcaggtctcgcgctaggaatggcaagtggtggcactgcagcttcatgcctcctctcatctccccgactgaaattgctcttgtttgaaggcacgttactatcaaagatgttggtatcagaagacttcagactagagggttcagttgtaacagagcgaagtttatctaatacaccatgaagccatacggtgaatcgaattgtgttgttccctagaaacagggacagatcctctgtcatttggtcctgacttttcttgttggccaccatcaccataatgtaatcaggaagttcttcatcaacataagctcctaattcttgtaatttccccttaatggcactccggatcttgcggctgatctcggtgccgatctccatggctctgcggcgtgcgggaactcagcactgcgcggcgcttggcttacccggaggctgccgcggactcctaccccgcagccgggacaccaccgcctcc

SEQ ID NO: 9867 - RNA, 4560 nt, Homo sapiens
  source 1..4560: mol_type = other RNA
caaagtgcttacagtgcaggtagaaactctgtaaccttaagcatgtaaactacatagaataaaactgtttccactgcatttctgtccttcaaagtggccaacctgattaagtcagccttaatcactgctgctgtcagtttcacgactaaaggtcatattgactaagtagtcatcagctgaccacctcgctgtatcagccagcaacgaggggaaggtgaagaaacatgataggccatatagaatctgccctatgtttacttttttaacccagataattatttttgtgtgcagtatctaagctcctgattgtgtaacctgggacttctggcaccttttgttccattcattttatgtataaaatgcatgccaaagcacactgtgccctctggtacccttgcttccaatcgccaaccatgctcatttccttcctttttttgtggtccctttttgtggtgatcattttaaaccacgtcatccaacaaatgttttatggtcaaccttagcttgttcataagccatagcaactgaaagattaaactcttaaatatgtgtctgggcagtggctattaaatagcaaaaaacaatcagattttagtattttattatttccttgtaaaatggctgaactaaattaaacccttgtttcccatttgttctataatttatagtgaaactgagaacaaaactatctttataaatgatagctaaaagtatttccagatatttaaacaatttaaaataaatttcttctgcagagatgcaaagcatctcaacactggaatgaacaaatgccttaaattcaatggagtaaacctttagaatgaagaggaactgtcatttcacccaagccgaagacaacagccttatgcacttgtgtgctctgtctttgctgcttctcgtgtttcaagcctttcctgtgggatcagcacagcaaagtgcaacttaccaaatggtttaatgactggttaattctttcttctcccaatggaaaagcaatggcaacacaacagtagactgctggcttgacaatcttaaacgtgagcctttgcacatgtaggtttatcatcatttgagtatacgactaagcaagtcaatgaactttttttttttttttagcagtttaatttggtcctgagaatgttgcagtctttattaccccttttgcattaatccacttttctaaccaccttttaagctttaatttttaacactatacaccaagtctttgaaatcagtgatctgttatttaactctaaagcatttgacacttcttgccttaacagttttaaaaaccacacacaaaaaaactctgtaagtaatacagtaggccaaaagtttcatcctatctatcttgcagtttacctatctgatctgatctctgtaattatagttctgtcatttaaaatatactatttaaatctaatttttacatttcaaaaattatcttcagtagtaactaagtatattttctgtggattctgagaatgttatttttcagaatgtgagaatatatatgtacatttataatcttgtgactttaaagtctgttttcagatacagtatgtaaatacttgtaaaaaaatttgtataattttgtgataatgtagtttcccaaaaaaattatttagaaggcattatgttattagtaaatgagagcactgtatagaactgttcctattttctgcacttgccattccagctgcctccactgtccatacccacctcattcatcctgtcacagaaggcaggaaaactgggaactttaccaaagtagcactcagcctgagaggcctgtataatcatgcttttcaaactaaattcacttaaaaattaaaaagcagaattgaatattttaagcagcctcagtacctttggccaatgctgttttcatggtggattatgaacattatataatctttgggaaaagtgaaagtagtacaatttttagaataatgacaactgcctcactgcatctctccactcacacagcaaccgtgtagccccctaagctgcagtaccatgactaaccatgatgtcaatttcatatgctgatcctcacaacagcagtgcacaaacatgccccaaatattttaacagaatttagctcttccttaagctgtcttttcatagtaaaaacaaaacaaaaacacccaatgttaaaaccacataataaacttacaaacttgaaaaattagacacttcagatagataggcaataaaacttcatattatgaaagcaatatattccaagtttcaaagatttgacaagttctgtagagtatctttcatcagtacatgaaaacttccaaactgcatgatcttctgccaggcaggactgggtgctattcgctggtttgaggtcgaatccatttcaaggcatgtcgtggtgggacattaatggtgggatggtagaatgtgcagtccggtcttgtacattgagtgttaaacctacaatgttttggatgatagaagggacattccatcttcttacaagcagggaagtaacggcagagctgactactggaaggtggtgctggtggtgcaactgctggttttggagacagtactggaattcttctactcacatgagtgaagggacaatctggtttagtacactttgcatcatatttacaatttgggtgaacaaacaaacatttttcagcaaatttacaattggggaaggctttgcagggtgagatggggtgatggtaggcacactcatccccatttttacaagcaggccagtacttgcagcgctccaaaagtttttctggtttctgtgccacactcagttcactcatctcagcatttgggtcctcaagctgcctgctcagcaagtgcaactgctgtgggtggaggagacctctgagtcccttgtttgaggctgcagtttggtttacgggtttcattccttcaaagcacatgtcctcctcttgatctgacatgtatcctggggggctggggacaccatccagcgtcactataaacttgggacttgcaggtttatctggttgtacaagatctcgtgtctgcataaggtgtcctgaaagtacccgaagggaatctgcagtcttcatccccgactcttggtttggtgccactactacttcctcagacagctttggcttcttcagaataaatgatcttgtgtctgcatggaccatggattccatgtcatagtaatcttgatttttttctacagaatctccttttgtttcctcttctttaatggggggacttattctgggggtcctactttgtccctggaccacttctgctagcaattcttcttgagaagttcgagttctgggagcaactggaagtgtctgtttctgtggaactgtagagtagttagttgtttttgttacggattcttgagcttcagatatagccttcaaaatcagattcttgttagcttgtttagaaggtggaagagaaggtctcctttcaggctttgcaggcacagacacactgctggagatgcttcctgttcgagacccgtaatcatcatcttcttcctcctcttctccatcatgattgaatttttttactttaacaactgaacttaccacaggcaactttctcttccgaaagttttcatcctccatactcattttctccgagttgtttctaaagaacggactatacgtttcttctaagctgttaagcacctctggttcacacaaacgtcctgtttcatatacccaactactctgcatatcaagctgcttggcagcatgaatactattctgctgctgttgaaattgcaacctgtttaaatgaacaccactatctgcatttctacttgcaggtggtcgataaatttcaatagaagggcgagaagaaccatatgtaagtgtcactgtaggttttttctgagataagggattctcctgcacaaagttgaggtcttcgtcaatgagatcatctggttctggcttaatatcaatcacatcttcagagggtgctggctccctcaaaggtttcactgttgacattagtcgggttgcagctccatcatcgtaagtctgtctgacatttgtggtttttgactcctgcgaacttgtagaaactctggaatctcttttttcaggtctcgcgctaggaatggcaagtggtggcactgcagcttcatgcctcctctcatctccccgactgaaattgctcttgtttgaaggcacgttactatcaaagatgttggtatcagaagacttcagactagagggttcagttgtaacagagcgaagtttatctaatacaccatgaagccatacggtgaatcgaattgtgttgttccctagaaacagggacagatcctctgtcatttggtcctgacttttcttgttggccaccatcaccataatgtaatcaggaagttcttcatcaacataagctcctaattcttgtaatttccccttaatggcactccggatcttgcggctgatctcggtgccgatctccatggctctgcggcgtgcgggaactcagcactgcgcggcgcttggcttacccggaggctgccgcggactcctaccccgcagccgggacaccaccgcctcc

SEQ ID NO: 9868 - RNA, 4535 nt, Homo sapiens
  source 1..4535: mol_type = other RNA
caaagtgcttacagtgcaggtagaaactctgtaaccttaagcatgtaaactacatagaataaaactgtttccactgcatttctgtccttcaaagtggccaacctgattaagtcagccttaatcactgctgctgtcagtttcacgactaaaggtcatattgactaagtagtcatcagctgaccacctcgctgtatcagccagcaacgaggggaaggtgaagaaacatgataggccatatagaatctgccctatgtttacttttttaacccagataattatttttgtgtgcagtatctaagctcctgattgtgtaacctgggacttctggcaccttttgttccattcattttatgtataaaatgcatgccaaagcacactgtgccctctggtacccttgcttccaatcgccaaccatgctcatttccttcctttttttgtggtccctttttgtggtgatcattttaaaccacgtcatccaacaaatgttttatggtcaaccttagcttgttcataagccatagcaactgaaagattaaactcttaaatatgtgtctgggcagtggctattaaatagcaaaaaacaatcagattttagtattttattatttccttgtaaaatggctgaactaaattaaacccttgtttcccatttgttctataatttatagtgaaactgagaacaaaactatctttataaatgatagctaaaagtatttccagatatttaaacaatttaaaataaatttcttctgcagagatgcaaagcatctcaacactggaatgaacaaatgccttaaattcaatggagtaaacctttagaatgaagaggaactgtcatttcacccaagccgaagacaacagccttatgcacttgtgtgctctgtctttgctgcttctcgtgtttcaagcctttcctgtgggatcagcacagcaaagtgcaacttaccaaatggtttaatgactggttaattctttcttctcccaatggaaaagcaatggcaacacaacagtagactgctggcttgacaatcttaaacgtgagcctttgcacatgtaggtttatcatcatttgagtatacgactaagcaagtcaatgaactttttttttttttttagcagtttaatttggtcctgagaatgttgcagtctttattaccccttttgcattaatccacttttctaaccaccttttaagctttaatttttaacactatacaccaagtctttgaaatcagtgatctgttatttaactctaaagcatttgacacttcttgccttaacagttttaaaaaccacacacaaaaaaactctgtaagtaatacagtaggccaaaagtttcatcctatctatcttgcagtttacctatctgatctgatctctgtaattatagttctgtcatttaaaatatactatttaaatctaatttttacatttcaaaaattatcttcagtagtaactaagtatattttctgtggattctgagaatgttatttttcagaatgtgagaatatatatgtacatttataatcttgtgactttaaagtctgttttcagatacagtatgtaaatacttgtaaaaaaatttgtataattttgtgataatgtagtttcccaaaaaaattatttagaaggcattatgttattagtaaatgagagcactgtatagaactgttcctattttctgcacttgccattccagctgcctccactgtccatacccacctcattcatcctgtcacagaaggcaggaaaactgggaactttaccaaagtagcactcagcctgagaggcctgtataatcatgcttttcaaactaaattcacttaaaaattaaaaagcagaattgaatattttaagcagcctcagtacctttggccaatgctgttttcatggtggattatgaacattatataatctttgggaaaagtgaaagtagtacaatttttagaataatgacaactgcctcactgcatctctccactcacacagcaaccgtgtagccccctaagctgcagtaccatgactaaccatgatgtcaatttcatatgctgatcctcacaacagcagtgcacaaacatgccccaaatattttaacagaatttagctcttccttaagctgtcttttcatagtaaaaacaaaacaaaaacacccaatgttaaaaccacataataaacttacaaacttgaaaaattagacacttcagatagataggcaataaaacttcatattatgaaagcaatatattccaagtttcaaagatttgacaagttctgtagagtatctttcatcagtacatgaaaacttccaaactgcatgatcttctgccaggcaggactgggtgctattcgctggtttgaggtcgaatccatttcaaggcatgtcgtggtgggacattaatggtgggatggtagaatgtgcagtccggtcttgtacattgagtgttaaacctacaatgttttggatgatagaagggacattccatcttcttacaagcagggaagtaacggcagagctgactactggaaggtggtgctggtggtgcaactgctggttttggagacagtactggaattcttctactcacatgagtgaagggacaatctggtttagtacactttgcatcatatttacaatttgggtgaacaaacaaacatttttcagcaaatttacaattggggaaggctttgcagggtgagatggggtgatggtaggcacactcatccccatttttacaagcaggccagtacttgcagcgctccaaaagtttttctggtttctgtgccacactcagttcactcatctcagcgttagaaaagctaccatttgggtcctcaagctgcctgctcagcaagtgcaactgctgtgggtggaggagacctctgagtcccttgtttgaggctgcagtttggtttacgggtttcattccttcaaagcacatgtcctcctcttgatctgacatgtatcctggggggctggggacaccatccagcgtcactataaacttgggacttgcaggtttatctggttgtacaagatctcgtgtctgcataaggtgtcctgaaagtacccgaagggaatctgcagtcttcatccccgactcttggtttggtgccactactacttcctcagacagctttggcttcttcagaataaatgatcttgtgtctgcatggaccatggattccatgtcatagtaatcttgactcatctgcagagtttctgccattactgggtcgatttgcagtcgggataataattgcctctgttgagttccttgatttttttctacagaatctccttttgtttcctcttctttaatggggggacttattctgggggtcctactttgtccctggaccacttctgctagcaattcttcttgagaagttcgagttctgggagcaactggaagtgtctgtttctgtggaactgtagagtagttagttgtttttgttacggattcttgagcttcagatatagccttcaaaatcagattcttgttagcttgtttagaaggtggaagagaaggtctcctttcaggctttgcaggcacagacacactgctggagatgcttcctgttcgagacccgtaatcatcatcttcttcctcctcttctccatcatgattgaatttttttactttaacaactgaacttaccacaggcaactttctcttccgaaagttttcatcctccatactcattttctccgagttgtttctaaagaacggactatacgtttcttctaagctgttaagcacctctggttcacacaaacgtcctgtttcatatacccaactactctgcatatcaagctgcttggcagcatgaatactattctgctgctgttgaaattgcaacctgtttaaatgaacaccactatctgcatttctacttgcaggtggtcgataaatttcaatagaagggcgagaagaaccatatgtaagtgtcactgtaggttttttctgagataagggattctcctgcacaaagttgaggtcttcgtcaatgagatcatctggttctggcttaatatcaatcacatcttcagagggtgctggctccctcaaaggtttcactgttgacattagtcgggttgcagctccatcatcgtaagtctgtctgacatttgtggtttttgactcctgcgaacttgtagaaactctggaatctcttttttcaggtctcgcgctaggaatggcaagtggtggcactgcagcttcatgcctcctctcatctccccgactgaaattgctcttgtttgaaggcacgttactatcaaagatgttggtatcagaagacttcagactagagggttcagttgtaacagagcgaagtttatctaatacaccatgaagccaacataagctcctaattcttgtaatttccccttaatggcactccggatcttgcggctgatctcggtgccgatctccatggctctgcggcgtgcgggaactcagcactgcgcggcgcttggcttacccggaggctgccgcggactcctaccccgcagccgggacaccaccgcctcc

SEQ ID NO: 9869 - RNA, 4650 nt, Homo sapiens
  source 1..4650: mol_type = other RNA
caaagtgcttacagtgcaggtagaaactctgtaaccttaagcatgtaaactacatagaataaaactgtttccactgcatttctgtccttcaaagtggccaacctgattaagtcagccttaatcactgctgctgtcagtttcacgactaaaggtcatattgactaagtagtcatcagctgaccacctcgctgtatcagccagcaacgaggggaaggtgaagaaacatgataggccatatagaatctgccctatgtttacttttttaacccagataattatttttgtgtgcagtatctaagctcctgattgtgtaacctgggacttctggcaccttttgttccattcattttatgtataaaatgcatgccaaagcacactgtgccctctggtacccttgcttccaatcgccaaccatgctcatttccttcctttttttgtggtccctttttgtggtgatcattttaaaccacgtcatccaacaaatgttttatggtcaaccttagcttgttcataagccatagcaactgaaagattaaactcttaaatatgtgtctgggcagtggctattaaatagcaaaaaacaatcagattttagtattttattatttccttgtaaaatggctgaactaaattaaacccttgtttcccatttgttctataatttatagtgaaactgagaacaaaactatctttataaatgatagctaaaagtatttccagatatttaaacaatttaaaataaatttcttctgcagagatgcaaagcatctcaacactggaatgaacaaatgccttaaattcaatggagtaaacctttagaatgaagaggaactgtcatttcacccaagccgaagacaacagccttatgcacttgtgtgctctgtctttgctgcttctcgtgtttcaagcctttcctgtgggatcagcacagcaaagtgcaacttaccaaatggtttaatgactggttaattctttcttctcccaatggaaaagcaatggcaacacaacagtagactgctggcttgacaatcttaaacgtgagcctttgcacatgtaggtttatcatcatttgagtatacgactaagcaagtcaatgaactttttttttttttttagcagtttaatttggtcctgagaatgttgcagtctttattaccccttttgcattaatccacttttctaaccaccttttaagctttaatttttaacactatacaccaagtctttgaaatcagtgatctgttatttaactctaaagcatttgacacttcttgccttaacagttttaaaaaccacacacaaaaaaactctgtaagtaatacagtaggccaaaagtttcatcctatctatcttgcagtttacctatctgatctgatctctgtaattatagttctgtcatttaaaatatactatttaaatctaatttttacatttcaaaaattatcttcagtagtaactaagtatattttctgtggattctgagaatgttatttttcagaatgtgagaatatatatgtacatttataatcttgtgactttaaagtctgttttcagatacagtatgtaaatacttgtaaaaaaatttgtataattttgtgataatgtagtttcccaaaaaaattatttagaaggcattatgttattagtaaatgagagcactgtatagaactgttcctattttctgcacttgccattccagctgcctccactgtccatacccacctcattcatcctgtcacagaaggcaggaaaactgggaactttaccaaagtagcactcagcctgagaggcctgtataatcatgcttttcaaactaaattcacttaaaaattaaaaagcagaattgaatattttaagcagcctcagtacctttggccaatgctgttttcatggtggattatgaacattatataatctttgggaaaagtgaaagtagtacaatttttagaataatgacaactgcctcactgcatctctccactcacacagcaaccgtgtagccccctaagctgcagtaccatgactaaccatgatgtcaatttcatatgctgatcctcacaacagcagtgcacaaacatgccccaaatattttaacagaatttagctcttccttaagctgtcttttcatagtaaaaacaaaacaaaaacacccaatgttaaaaccacataataaacttacaaacttgaaaaattagacacttcagatagataggcaataaaacttcatattatgaaagcaatatattccaagtttcaaagatttgacaagttctgtagagtatctttcatcagtacatgaaaacttccaaactgcatgatcttctgccaggcaggactgggtgctattcgctggtttgaggtcgaatccatttcaaggcatgtcgtggtgggacattaatggtgggatggtagaatgtgcagtccggtcttgtacattgagtgttaaacctacaatgttttggatgatagaagggacattccatcttcttacaagcagggaagtaacggcagagctgactactggaaggtggtgctggtggtgcaactgctggttttggagacagtactggaattcttctactcacatgagtgaagggacaatctggtttagtacactttgcatcatatttacaatttgggtgaacaaacaaacatttttcagcaaatttacaattggggaaggctttgcagggtgagatggggtgatggtaggcacactcatccccatttttacaagcaggccagtacttgcagcgctccaaaagtttttctggtttctgtgccacactcagttcactcatctcagcgttagaaaagctaccatttgggtcctcaagctgcctgctcagcaagtgcaactgctgtgggtggaggagacctctgagtcccttgtttgaggctgcagtttggtttacgggtttcattccttcaaagcacatgtcctcctcttgatctgacatgtatcctggggggctggggacaccatccagcgtcactataaacttgggacttgcaggtttatctggttgtacaagatctcgtgtctgcataaggtgtcctgaaagtacccgaagggaatctgcagtcttcatccccgactcttggtttggtgccactactacttcctcagacagctttggcttcttcagaataaatgatcttgtgtctgcatggaccatggattccatgtcatagtaatcttgactcatctgcagagtttctgccattactgggtcgatttgcagtcgggataataattgcctctgttgagttccttgatttttttctacagaatctccttttgtttcctcttctttaatggggggacttattctgggggtcctactttgtccctggaccacttctgctagcaattcttcttgagaagttcgagttctgggagcaactggaagtgtctgtttctgtggaactgtagagtagttagttgtttttgttacggattcttgagcttcagatatagccttcaaaatcagattcttgttagcttgtttagaaggtggaagagaaggtctcctttcaggctttgcaggcacagacacactgctggagatgcttcctgttcgagacccgtaatcatcatcttcttcctcctcttctccatcatgattgaatttttttactttaacaactgaacttaccacaggcaactttctcttccgaaagttttcatcctccatactcattttctccgagttgtttctaaagaacggactatacgtttcttctaagctgttaagcacctctggttcacacaaacgtcctgtttcatatacccaactactctgcatatcaagctgcttggcagcatgaatactattctgctgctgttgaaattgcaacctgtttaaatgaacaccactatctgcatttctacttgcaggtggtcgataaatttcaatagaagggcgagaagaaccatatgtaagtgtcactgtaggttttttctgagataagggattctcctgcacaaagttgaggtcttcgtcaatgagatcatctggttctggcttaatatcaatcacatcttcagagggtgctggctccctcaaaggtttcactgttgacattagtcgggttgcagctccatcatcgtaagtctgtctgacatttgtggtttttgactcctgcgaacttgtagaaactctggaatctcttttttcaggtctcgcgctaggaatggcaagtggtggcactgcagcttcatgcctcctctcatctccccgactgaaattgctcttgtttgaaggcacgttactatcaaagatgttggtatcagaagacttcagactagagggttcagttgtaacagagcgaagtttatctaatacaccatgaagccatacggtgaatcgaattgtgttgttccctagaaacagggacagatcctctgtcatttggtcctgacttttcttgttggccaccatcaccataatgtaatcaggaagttcttcatcaacataagctcctaattcttgtaatttccccttaatggcactccggatcttgcggctgatctcggtgccgatctccatggctctgcggcgtgcgggaactcagcactgcgcggcgcttggcttacccggaggctgccgcggactcctaccccgcagccgggacaccaccgcctcc

SEQ ID NO: 9870 - RNA, 4831 nt, Homo sapiens
  source 1..4831: mol_type = other RNA
caaagtgcttacagtgcaggtagaaactctgtaaccttaagcatgtaaactacatagaataaaactgtttccactgcatttctgtccttcaaagtggccaacctgattaagtcagccttaatcactgctgctgtcagtttcacgactaaaggtcatattgactaagtagtcatcagctgaccacctcgctgtatcagccagcaacgaggggaaggtgaagaaacatgataggccatatagaatctgccctatgtttacttttttaacccagataattatttttgtgtgcagtatctaagctcctgattgtgtaacctgggacttctggcaccttttgttccattcattttatgtataaaatgcatgccaaagcacactgtgccctctggtacccttgcttccaatcgccaaccatgctcatttccttcctttttttgtggtccctttttgtggtgatcattttaaaccacgtcatccaacaaatgttttatggtcaaccttagcttgttcataagccatagcaactgaaagattaaactcttaaatatgtgtctgggcagtggctattaaatagcaaaaaacaatcagattttagtattttattatttccttgtaaaatggctgaactaaattaaacccttgtttcccatttgttctataatttatagtgaaactgagaacaaaactatctttataaatgatagctaaaagtatttccagatatttaaacaatttaaaataaatttcttctgcagagatgcaaagcatctcaacactggaatgaacaaatgccttaaattcaatggagtaaacctttagaatgaagaggaactgtcatttcacccaagccgaagacaacagccttatgcacttgtgtgctctgtctttgctgcttctcgtgtttcaagcctttcctgtgggatcagcacagcaaagtgcaacttaccaaatggtttaatgactggttaattctttcttctcccaatggaaaagcaatggcaacacaacagtagactgctggcttgacaatcttaaacgtgagcctttgcacatgtaggtttatcatcatttgagtatacgactaagcaagtcaatgaactttttttttttttttagcagtttaatttggtcctgagaatgttgcagtctttattaccccttttgcattaatccacttttctaaccaccttttaagctttaatttttaacactatacaccaagtctttgaaatcagtgatctgttatttaactctaaagcatttgacacttcttgccttaacagttttaaaaaccacacacaaaaaaactctgtaagtaatacagtaggccaaaagtttcatcctatctatcttgcagtttacctatctgatctgatctctgtaattatagttctgtcatttaaaatatactatttaaatctaatttttacatttcaaaaattatcttcagtagtaactaagtatattttctgtggattctgagaatgttatttttcagaatgtgagaatatatatgtacatttataatcttgtgactttaaagtctgttttcagatacagtatgtaaatacttgtaaaaaaatttgtataattttgtgataatgtagtttcccaaaaaaattatttagaaggcattatgttattagtaaatgagagcactgtatagaactgttcctattttctgcacttgccattccagctgcctccactgtccatacccacctcattcatcctgtcacagaaggcaggaaaactgggaactttaccaaagtagcactcagcctgagaggcctgtataatcatgcttttcaaactaaattcacttaaaaattaaaaagcagaattgaatattttaagcagcctcagtacctttggccaatgctgttttcatggtggattatgaacattatataatctttgggaaaagtgaaagtagtacaatttttagaataatgacaactgcctcactgcatctctccactcacacagcaaccgtgtagccccctaagctgcagtaccatgactaaccatgatgtcaatttcatatgctgatcctcacaacagcagtgcacaaacatgccccaaatattttaacagaatttagctcttccttaagctgtcttttcatagtaaaaacaaaacaaaaacacccaatgttaaaaccacataataaacttacaaacttgaaaaattagacacttcagatagataggcaataaaacttcatattatgaaagcaatatattccaagtttcaaagatttgacaagttctgtagagtatctttcatcagtacatgaaaacttccaaactgcatgatcttctgccaggcaggactgggtgctattcgctggtttgaggtcgaatccatttcaaggcatgtcgtggtgggacattaatggtgggatggtagaatgtgcagtccggtcttgtacattgagtgttaaacctacaatgttttggatgatagaagggacattccatcttcttacaagcagggaagtaacggcagagctgactactggaaggtggtgctggtggtgcaactgctggttttggagacagtactggaattcttctactcacatgagtgaagggacaatctggtttagtacactttgcatcatatttacaatttgggtgaacaaacaaacatttttcagcaaatttacaattggggaaggctttgcagggtgagatggggtgatggtaggcacactcatccccatttttacaagcaggccagtacttgcagcgctccaaaagtttttctggtttctgtgccacactcagttcactcatctcagcgttagaaaagctaccatttgggtcctcaagctgcctgctcagcaagtgcaactgctgtgggtggaggagacctctgagtcccttgtttgaggctgcagtttggtttacgggtttcattccttcaaagcacatgtcctcctcttgatctgacatgtatcctggggggctggggacaccatccagcgtcactataaacttgggacttgcaggtttatctggttgtacaagatctcgtgtctgcataaggtgtcctgaaagtacccgaagggaatctgcagtcttcatccccgactcttggtttggtgccactactacttcctcagacagctttggcttcttcagaataaatgatcttgtgtctgcatggaccatggattccatgtcatagtaatcttgactcatctgcagagtttctgccattactgggtcgatttgcagtcgggataataattgcctctgttgagttccttgatttttttctacagaatctccttttgtttcctcttctttaatggggggacttattctgggggtcctactttgtccctggaccacttctgctagcaattcttcttgagaagttcgagttctgggagcaactggaagtgtctgtttctgtggaactgtagagtagttagttgtttttgttacggattcttgagcttcagatatagccttcaaaatcagattcttgttagcttgtttagaaggtggaagagaaggtctcctttcaggctttgcaggcacagacacactgctggagatgcttcctgttcgagacccgtaatcatcatcttcttcctcctcttctccatcatgattgaatttttttactttaacaactgaacttaccacaggcaactttctcttccgaaagttttcatcctccatactcattttctccgagttgtttctaaagaacggactatacgtttcttctaagctgttaagcacctctggttcacacaaacgtcctgtttcatatacccaactactctgcatatcaagctgcttggcagcatgaatactattctgctgctgttgaaattgcaacctgtttaaatgaacaccactatctgcatttctacttgcaggtggtcgataaatttcaatagaagggcgagaagaaccatatgtaagtgtcactgtaggttttttctgagataagggattctcctgcacaaagttgaggtcttcgtcaatgagatcatctggttctggcttaatatcaatcacatcttcagagggtgctggctccctcaaaggtttcactgttgacattagtcgggttgcagctccatcatcgtaagtctgtctgacatttgtggtttttgactcctgcgaacttgtagaaactctggaatctcttttttcaggtctcgcgctaggaatggcaagtggtggcactgcagcttcatgcctcctctcatctccccgactgaaattgctcttgtttgaaggcacgttactatcaaagatgttggtatcagaagacttcagactagagggttcagttgtaacagagcgaagtttatctaatacaccatgaagccatacggtgaatcgaattgtgttgttccctagaaacagggacagatcctctgtcatttggtcctgacttttcttgttggccaccatcaccataatgtaatcaggaagttcttcatctatttaaaaggaaaggtagatcaaaactttgtttcctcaaaactttcttcttaaagttgatgtgcttgaaaatatagatgtagctctaagctttagagtcgcagagctctactggaattacattggacaagatggcttagctttaatttttttctcttcattccacaggtatttcaaatacaacataagctcctaattcttgtaatttccccttaatggcactccggatcttgcggctgatctcggtgccgatctccatggctctgcggcgtgcgggaactcagcactgcgcggcgcttggcttacccggaggctgccgcggactcctaccccgcagccgggacaccaccgcctcc

SEQ ID NO: 9871 - RNA, 4460 nt, Homo sapiens
  source 1..4460: mol_type = other RNA
caaagtgcttacagtgcaggtagaaactctgtaaccttaagcatgtaaactacatagaataaaactgtttccactgcatttctgtccttcaaagtggccaacctgattaagtcagccttaatcactgctgctgtcagtttcacgactaaaggtcatattgactaagtagtcatcagctgaccacctcgctgtatcagccagcaacgaggggaaggtgaagaaacatgataggccatatagaatctgccctatgtttacttttttaacccagataattatttttgtgtgcagtatctaagctcctgattgtgtaacctgggacttctggcaccttttgttccattcattttatgtataaaatgcatgccaaagcacactgtgccctctggtacccttgcttccaatcgccaaccatgctcatttccttcctttttttgtggtccctttttgtggtgatcattttaaaccacgtcatccaacaaatgttttatggtcaaccttagcttgttcataagccatagcaactgaaagattaaactcttaaatatgtgtctgggcagtggctattaaatagcaaaaaacaatcagattttagtattttattatttccttgtaaaatggctgaactaaattaaacccttgtttcccatttgttctataatttatagtgaaactgagaacaaaactatctttataaatgatagctaaaagtatttccagatatttaaacaatttaaaataaatttcttctgcagagatgcaaagcatctcaacactggaatgaacaaatgccttaaattcaatggagtaaacctttagaatgaagaggaactgtcatttcacccaagccgaagacaacagccttatgcacttgtgtgctctgtctttgctgcttctcgtgtttcaagcctttcctgtgggatcagcacagcaaagtgcaacttaccaaatggtttaatgactggttaattctttcttctcccaatggaaaagcaatggcaacacaacagtagactgctggcttgacaatcttaaacgtgagcctttgcacatgtaggtttatcatcatttgagtatacgactaagcaagtcaatgaactttttttttttttttagcagtttaatttggtcctgagaatgttgcagtctttattaccccttttgcattaatccacttttctaaccaccttttaagctttaatttttaacactatacaccaagtctttgaaatcagtgatctgttatttaactctaaagcatttgacacttcttgccttaacagttttaaaaaccacacacaaaaaaactctgtaagtaatacagtaggccaaaagtttcatcctatctatcttgcagtttacctatctgatctgatctctgtaattatagttctgtcatttaaaatatactatttaaatctaatttttacatttcaaaaattatcttcagtagtaactaagtatattttctgtggattctgagaatgttatttttcagaatgtgagaatatatatgtacatttataatcttgtgactttaaagtctgttttcagatacagtatgtaaatacttgtaaaaaaatttgtataattttgtgataatgtagtttcccaaaaaaattatttagaaggcattatgttattagtaaatgagagcactgtatagaactgttcctattttctgcacttgccattccagctgcctccactgtccatacccacctcattcatcctgtcacagaaggcaggaaaactgggaactttaccaaagtagcactcagcctgagaggcctgtataatcatgcttttcaaactaaattcacttaaaaattaaaaagcagaattgaatattttaagcagcctcagtacctttggccaatgctgttttcatggtggattatgaacattatataatctttgggaaaagtgaaagtagtacaatttttagaataatgacaactgcctcactgcatctctccactcacacagcaaccgtgtagccccctaagctgcagtaccatgactaaccatgatgtcaatttcatatgctgatcctcacaacagcagtgcacaaacatgccccaaatattttaacagaatttagctcttccttaagctgtcttttcatagtaaaaacaaaacaaaaacacccaatgttaaaaccacataataaacttacaaacttgaaaaattagacacttcagatagataggcaataaaacttcatattatgaaagcaatatattccaagtttcaaagatttgacaagttctgtagagtatctttcatcagtacatgaaaacttccaaactgcatgatcttctgccaggcaggactgggtgctattcgctggtttgaggtcgaatccatttcaaggcatgtcgtggtgggacattaatggtgggatggtagaatgtgcagtccggtcttgtacattgagtgttaaacctacaatgttttggatgatagaagggacattccatcttcttacaagcagggaagtaacggcagagctgactactggaaggtggtgctggtggtgcaactgctggttttggagacagtactggaattcttctactcacatgagtgaagggacaatctggtttagtacactttgcatcatatttacaatttgggtgaacaaacaaacatttttcagcaaatttacaattggggaaggctttgcagggtgagatggggtgatggtaggcacactcatccccatttttacaagcaggccagtacttgcagcgctccaaaagtttttctggtttctgtgccacactcagttcactcatctcagcgttagaaaagctaccatttgggtcctcaagctgcctgctcagcaagtgcaactgctgtgggtggaggagacctctgagtcccttgtttgaggctgcagtttggtttacgggtttcattccttcaaagcacatgtcctcctcttgatctgacatgtatcctggggggctggggacaccatccagcgtcactataaacttgggacttgcaggtttatctggttgtacaagatctcgtgtctgcataaggtgtcctgaaagtacccgaagggaatctgcagtcttcatccccgactcttggtttggtgccactactacttcctcagacagctttggcttcttcagaataaatgatcttgtgtctgcatggaccatggattccatgtcatagtaatcttgatttttttctacagaatctccttttgtttcctcttctttaatggggggacttattctgggggtcctactttgtccctggaccacttctgctagcaattcttcttgagaagttcgagttctgggagcaactggaagtgtctgtttctgtggaactgtagagtagttagttgtttttgttacggattcttgagcttcagatatagccttcaaaatcagattcttgttagcttgtttagaaggtggaagagaaggtctcctttcaggctttgcaggcacagacacactgctggagatgcttcctgttcgagacccgtaatcatcatcttcttcctcctcttctccatcatgattgaatttttttactttaacaactgaacttaccacaggcaactttctcttccgaaagttttcatcctccatactcattttctccgagttgtttctaaagaacggactatacgtttcttctaagctgttaagcacctctggttcacacaaacgtcctgtttcatatacccaactactctgcatatcaagctgcttggcagcatgaatactattctgctgctgttgaaattgcaacctgtttaaatgaacaccactatctgcatttctacttgcaggtggtcgataaatttcaatagaagggcgagaagaaccatatgtaagtgtcactgtaggttttttctgagataagggattctcctgcacaaagttgaggtcttcgtcaatgagatcatctggttctggcttaatatcaatcacatcttcagagggtgctggctccctcaaaggtttcactgttgacattagtcgggttgcagctccatcatcgtaagtctgtctgacatttgtggtttttgactcctgcgaacttgtagaaactctggaatctcttttttcaggtctcgcgctaggaatggcaagtggtggcactgcagcttcatgcctcctctcatctccccgactgaaattgctcttgtttgaaggcacgttactatcaaagatgttggtatcagaagacttcagactagagggttcagttgtaacagagcgaagtttatctaatacaccatgaagccaacataagctcctaattcttgtaatttccccttaatggcactccggatcttgcggctgatctcggtgccgatctccatggctctgcggcgtgcgggaactcagcactgcgcggcgcttggcttacccggaggctgccgcggactcctaccccgcagccgggacaccaccgcctcc

SEQ ID NO: 9872 - RNA, 4575 nt, Homo sapiens
  source 1..4575: mol_type = other RNA
caaagtgcttacagtgcaggtagaaactctgtaaccttaagcatgtaaactacatagaataaaactgtttccactgcatttctgtccttcaaagtggccaacctgattaagtcagccttaatcactgctgctgtcagtttcacgactaaaggtcatattgactaagtagtcatcagctgaccacctcgctgtatcagccagcaacgaggggaaggtgaagaaacatgataggccatatagaatctgccctatgtttacttttttaacccagataattatttttgtgtgcagtatctaagctcctgattgtgtaacctgggacttctggcaccttttgttccattcattttatgtataaaatgcatgccaaagcacactgtgccctctggtacccttgcttccaatcgccaaccatgctcatttccttcctttttttgtggtccctttttgtggtgatcattttaaaccacgtcatccaacaaatgttttatggtcaaccttagcttgttcataagccatagcaactgaaagattaaactcttaaatatgtgtctgggcagtggctattaaatagcaaaaaacaatcagattttagtattttattatttccttgtaaaatggctgaactaaattaaacccttgtttcccatttgttctataatttatagtgaaactgagaacaaaactatctttataaatgatagctaaaagtatttccagatatttaaacaatttaaaataaatttcttctgcagagatgcaaagcatctcaacactggaatgaacaaatgccttaaattcaatggagtaaacctttagaatgaagaggaactgtcatttcacccaagccgaagacaacagccttatgcacttgtgtgctctgtctttgctgcttctcgtgtttcaagcctttcctgtgggatcagcacagcaaagtgcaacttaccaaatggtttaatgactggttaattctttcttctcccaatggaaaagcaatggcaacacaacagtagactgctggcttgacaatcttaaacgtgagcctttgcacatgtaggtttatcatcatttgagtatacgactaagcaagtcaatgaactttttttttttttttagcagtttaatttggtcctgagaatgttgcagtctttattaccccttttgcattaatccacttttctaaccaccttttaagctttaatttttaacactatacaccaagtctttgaaatcagtgatctgttatttaactctaaagcatttgacacttcttgccttaacagttttaaaaaccacacacaaaaaaactctgtaagtaatacagtaggccaaaagtttcatcctatctatcttgcagtttacctatctgatctgatctctgtaattatagttctgtcatttaaaatatactatttaaatctaatttttacatttcaaaaattatcttcagtagtaactaagtatattttctgtggattctgagaatgttatttttcagaatgtgagaatatatatgtacatttataatcttgtgactttaaagtctgttttcagatacagtatgtaaatacttgtaaaaaaatttgtataattttgtgataatgtagtttcccaaaaaaattatttagaaggcattatgttattagtaaatgagagcactgtatagaactgttcctattttctgcacttgccattccagctgcctccactgtccatacccacctcattcatcctgtcacagaaggcaggaaaactgggaactttaccaaagtagcactcagcctgagaggcctgtataatcatgcttttcaaactaaattcacttaaaaattaaaaagcagaattgaatattttaagcagcctcagtacctttggccaatgctgttttcatggtggattatgaacattatataatctttgggaaaagtgaaagtagtacaatttttagaataatgacaactgcctcactgcatctctccactcacacagcaaccgtgtagccccctaagctgcagtaccatgactaaccatgatgtcaatttcatatgctgatcctcacaacagcagtgcacaaacatgccccaaatattttaacagaatttagctcttccttaagctgtcttttcatagtaaaaacaaaacaaaaacacccaatgttaaaaccacataataaacttacaaacttgaaaaattagacacttcagatagataggcaataaaacttcatattatgaaagcaatatattccaagtttcaaagatttgacaagttctgtagagtatctttcatcagtacatgaaaacttccaaactgcatgatcttctgccaggcaggactgggtgctattcgctggtttgaggtcgaatccatttcaaggcatgtcgtggtgggacattaatggtgggatggtagaatgtgcagtccggtcttgtacattgagtgttaaacctacaatgttttggatgatagaagggacattccatcttcttacaagcagggaagtaacggcagagctgactactggaaggtggtgctggtggtgcaactgctggttttggagacagtactggaattcttctactcacatgagtgaagggacaatctggtttagtacactttgcatcatatttacaatttgggtgaacaaacaaacatttttcagcaaatttacaattggggaaggctttgcagggtgagatggggtgatggtaggcacactcatccccatttttacaagcaggccagtacttgcagcgctccaaaagtttttctggtttctgtgccacactcagttcactcatctcagcgttagaaaagctaccatttgggtcctcaagctgcctgctcagcaagtgcaactgctgtgggtggaggagacctctgagtcccttgtttgaggctgcagtttggtttacgggtttcattccttcaaagcacatgtcctcctcttgatctgacatgtatcctggggggctggggacaccatccagcgtcactataaacttgggacttgcaggtttatctggttgtacaagatctcgtgtctgcataaggtgtcctgaaagtacccgaagggaatctgcagtcttcatccccgactcttggtttggtgccactactacttcctcagacagctttggcttcttcagaataaatgatcttgtgtctgcatggaccatggattccatgtcatagtaatcttgatttttttctacagaatctccttttgtttcctcttctttaatggggggacttattctgggggtcctactttgtccctggaccacttctgctagcaattcttcttgagaagttcgagttctgggagcaactggaagtgtctgtttctgtggaactgtagagtagttagttgtttttgttacggattcttgagcttcagatatagccttcaaaatcagattcttgttagcttgtttagaaggtggaagagaaggtctcctttcaggctttgcaggcacagacacactgctggagatgcttcctgttcgagacccgtaatcatcatcttcttcctcctcttctccatcatgattgaatttttttactttaacaactgaacttaccacaggcaactttctcttccgaaagttttcatcctccatactcattttctccgagttgtttctaaagaacggactatacgtttcttctaagctgttaagcacctctggttcacacaaacgtcctgtttcatatacccaactactctgcatatcaagctgcttggcagcatgaatactattctgctgctgttgaaattgcaacctgtttaaatgaacaccactatctgcatttctacttgcaggtggtcgataaatttcaatagaagggcgagaagaaccatatgtaagtgtcactgtaggttttttctgagataagggattctcctgcacaaagttgaggtcttcgtcaatgagatcatctggttctggcttaatatcaatcacatcttcagagggtgctggctccctcaaaggtttcactgttgacattagtcgggttgcagctccatcatcgtaagtctgtctgacatttgtggtttttgactcctgcgaacttgtagaaactctggaatctcttttttcaggtctcgcgctaggaatggcaagtggtggcactgcagcttcatgcctcctctcatctccccgactgaaattgctcttgtttgaaggcacgttactatcaaagatgttggtatcagaagacttcagactagagggttcagttgtaacagagcgaagtttatctaatacaccatgaagccatacggtgaatcgaattgtgttgttccctagaaacagggacagatcctctgtcatttggtcctgacttttcttgttggccaccatcaccataatgtaatcaggaagttcttcatcaacataagctcctaattcttgtaatttccccttaatggcactccggatcttgcggctgatctcggtgccgatctccatggctctgcggcgtgcgggaactcagcactgcgcggcgcttggcttacccggaggctgccgcggactcctaccccgcagccgggacaccaccgcctcc

SEQ ID NO: 9873 - RNA, 4756 nt, Homo sapiens
  source 1..4756: mol_type = other RNA
caaagtgcttacagtgcaggtagaaactctgtaaccttaagcatgtaaactacatagaataaaactgtttccactgcatttctgtccttcaaagtggccaacctgattaagtcagccttaatcactgctgctgtcagtttcacgactaaaggtcatattgactaagtagtcatcagctgaccacctcgctgtatcagccagcaacgaggggaaggtgaagaaacatgataggccatatagaatctgccctatgtttacttttttaacccagataattatttttgtgtgcagtatctaagctcctgattgtgtaacctgggacttctggcaccttttgttccattcattttatgtataaaatgcatgccaaagcacactgtgccctctggtacccttgcttccaatcgccaaccatgctcatttccttcctttttttgtggtccctttttgtggtgatcattttaaaccacgtcatccaacaaatgttttatggtcaaccttagcttgttcataagccatagcaactgaaagattaaactcttaaatatgtgtctgggcagtggctattaaatagcaaaaaacaatcagattttagtattttattatttccttgtaaaatggctgaactaaattaaacccttgtttcccatttgttctataatttatagtgaaactgagaacaaaactatctttataaatgatagctaaaagtatttccagatatttaaacaatttaaaataaatttcttctgcagagatgcaaagcatctcaacactggaatgaacaaatgccttaaattcaatggagtaaacctttagaatgaagaggaactgtcatttcacccaagccgaagacaacagccttatgcacttgtgtgctctgtctttgctgcttctcgtgtttcaagcctttcctgtgggatcagcacagcaaagtgcaacttaccaaatggtttaatgactggttaattctttcttctcccaatggaaaagcaatggcaacacaacagtagactgctggcttgacaatcttaaacgtgagcctttgcacatgtaggtttatcatcatttgagtatacgactaagcaagtcaatgaactttttttttttttttagcagtttaatttggtcctgagaatgttgcagtctttattaccccttttgcattaatccacttttctaaccaccttttaagctttaatttttaacactatacaccaagtctttgaaatcagtgatctgttatttaactctaaagcatttgacacttcttgccttaacagttttaaaaaccacacacaaaaaaactctgtaagtaatacagtaggccaaaagtttcatcctatctatcttgcagtttacctatctgatctgatctctgtaattatagttctgtcatttaaaatatactatttaaatctaatttttacatttcaaaaattatcttcagtagtaactaagtatattttctgtggattctgagaatgttatttttcagaatgtgagaatatatatgtacatttataatcttgtgactttaaagtctgttttcagatacagtatgtaaatacttgtaaaaaaatttgtataattttgtgataatgtagtttcccaaaaaaattatttagaaggcattatgttattagtaaatgagagcactgtatagaactgttcctattttctgcacttgccattccagctgcctccactgtccatacccacctcattcatcctgtcacagaaggcaggaaaactgggaactttaccaaagtagcactcagcctgagaggcctgtataatcatgcttttcaaactaaattcacttaaaaattaaaaagcagaattgaatattttaagcagcctcagtacctttggccaatgctgttttcatggtggattatgaacattatataatctttgggaaaagtgaaagtagtacaatttttagaataatgacaactgcctcactgcatctctccactcacacagcaaccgtgtagccccctaagctgcagtaccatgactaaccatgatgtcaatttcatatgctgatcctcacaacagcagtgcacaaacatgccccaaatattttaacagaatttagctcttccttaagctgtcttttcatagtaaaaacaaaacaaaaacacccaatgttaaaaccacataataaacttacaaacttgaaaaattagacacttcagatagataggcaataaaacttcatattatgaaagcaatatattccaagtttcaaagatttgacaagttctgtagagtatctttcatcagtacatgaaaacttccaaactgcatgatcttctgccaggcaggactgggtgctattcgctggtttgaggtcgaatccatttcaaggcatgtcgtggtgggacattaatggtgggatggtagaatgtgcagtccggtcttgtacattgagtgttaaacctacaatgttttggatgatagaagggacattccatcttcttacaagcagggaagtaacggcagagctgactactggaaggtggtgctggtggtgcaactgctggttttggagacagtactggaattcttctactcacatgagtgaagggacaatctggtttagtacactttgcatcatatttacaatttgggtgaacaaacaaacatttttcagcaaatttacaattggggaaggctttgcagggtgagatggggtgatggtaggcacactcatccccatttttacaagcaggccagtacttgcagcgctccaaaagtttttctggtttctgtgccacactcagttcactcatctcagcgttagaaaagctaccatttgggtcctcaagctgcctgctcagcaagtgcaactgctgtgggtggaggagacctctgagtcccttgtttgaggctgcagtttggtttacgggtttcattccttcaaagcacatgtcctcctcttgatctgacatgtatcctggggggctggggacaccatccagcgtcactataaacttgggacttgcaggtttatctggttgtacaagatctcgtgtctgcataaggtgtcctgaaagtacccgaagggaatctgcagtcttcatccccgactcttggtttggtgccactactacttcctcagacagctttggcttcttcagaataaatgatcttgtgtctgcatggaccatggattccatgtcatagtaatcttgatttttttctacagaatctccttttgtttcctcttctttaatggggggacttattctgggggtcctactttgtccctggaccacttctgctagcaattcttcttgagaagttcgagttctgggagcaactggaagtgtctgtttctgtggaactgtagagtagttagttgtttttgttacggattcttgagcttcagatatagccttcaaaatcagattcttgttagcttgtttagaaggtggaagagaaggtctcctttcaggctttgcaggcacagacacactgctggagatgcttcctgttcgagacccgtaatcatcatcttcttcctcctcttctccatcatgattgaatttttttactttaacaactgaacttaccacaggcaactttctcttccgaaagttttcatcctccatactcattttctccgagttgtttctaaagaacggactatacgtttcttctaagctgttaagcacctctggttcacacaaacgtcctgtttcatatacccaactactctgcatatcaagctgcttggcagcatgaatactattctgctgctgttgaaattgcaacctgtttaaatgaacaccactatctgcatttctacttgcaggtggtcgataaatttcaatagaagggcgagaagaaccatatgtaagtgtcactgtaggttttttctgagataagggattctcctgcacaaagttgaggtcttcgtcaatgagatcatctggttctggcttaatatcaatcacatcttcagagggtgctggctccctcaaaggtttcactgttgacattagtcgggttgcagctccatcatcgtaagtctgtctgacatttgtggtttttgactcctgcgaacttgtagaaactctggaatctcttttttcaggtctcgcgctaggaatggcaagtggtggcactgcagcttcatgcctcctctcatctccccgactgaaattgctcttgtttgaaggcacgttactatcaaagatgttggtatcagaagacttcagactagagggttcagttgtaacagagcgaagtttatctaatacaccatgaagccatacggtgaatcgaattgtgttgttccctagaaacagggacagatcctctgtcatttggtcctgacttttcttgttggccaccatcaccataatgtaatcaggaagttcttcatctatttaaaaggaaaggtagatcaaaactttgtttcctcaaaactttcttcttaaagttgatgtgcttgaaaatatagatgtagctctaagctttagagtcgcagagctctactggaattacattggacaagatggcttagctttaatttttttctcttcattccacaggtatttcaaatacaacataagctcctaattcttgtaatttccccttaatggcactccggatcttgcggctgatctcggtgccgatctccatggctctgcggcgtgcgggaactcagcactgcgcggcgcttggcttacccggaggctgccgcggactcctaccccgcagccgggacaccaccgcctcc

SEQ ID NO: 9874 - RNA, 4490 nt, Homo sapiens
  source 1..4490: mol_type = other RNA
caaagtgcttacagtgcaggtagaaactctgtaaccttaagcatgtaaactacatagaataaaactgtttccactgcatttctgtccttcaaagtggccaacctgattaagtcagccttaatcactgctgctgtcagtttcacgactaaaggtcatattgactaagtagtcatcagctgaccacctcgctgtatcagccagcaacgaggggaaggtgaagaaacatgataggccatatagaatctgccctatgtttacttttttaacccagataattatttttgtgtgcagtatctaagctcctgattgtgtaacctgggacttctggcaccttttgttccattcattttatgtataaaatgcatgccaaagcacactgtgccctctggtacccttgcttccaatcgccaaccatgctcatttccttcctttttttgtggtccctttttgtggtgatcattttaaaccacgtcatccaacaaatgttttatggtcaaccttagcttgttcataagccatagcaactgaaagattaaactcttaaatatgtgtctgggcagtggctattaaatagcaaaaaacaatcagattttagtattttattatttccttgtaaaatggctgaactaaattaaacccttgtttcccatttgttctataatttatagtgaaactgagaacaaaactatctttataaatgatagctaaaagtatttccagatatttaaacaatttaaaataaatttcttctgcagagatgcaaagcatctcaacactggaatgaacaaatgccttaaattcaatggagtaaacctttagaatgaagaggaactgtcatttcacccaagccgaagacaacagccttatgcacttgtgtgctctgtctttgctgcttctcgtgtttcaagcctttcctgtgggatcagcacagcaaagtgcaacttaccaaatggtttaatgactggttaattctttcttctcccaatggaaaagcaatggcaacacaacagtagactgctggcttgacaatcttaaacgtgagcctttgcacatgtaggtttatcatcatttgagtatacgactaagcaagtcaatgaactttttttttttttttagcagtttaatttggtcctgagaatgttgcagtctttattaccccttttgcattaatccacttttctaaccaccttttaagctttaatttttaacactatacaccaagtctttgaaatcagtgatctgttatttaactctaaagcatttgacacttcttgccttaacagttttaaaaaccacacacaaaaaaactctgtaagtaatacagtaggccaaaagtttcatcctatctatcttgcagtttacctatctgatctgatctctgtaattatagttctgtcatttaaaatatactatttaaatctaatttttacatttcaaaaattatcttcagtagtaactaagtatattttctgtggattctgagaatgttatttttcagaatgtgagaatatatatgtacatttataatcttgtgactttaaagtctgttttcagatacagtatgtaaatacttgtaaaaaaatttgtataattttgtgataatgtagtttcccaaaaaaattatttagaaggcattatgttattagtaaatgagagcactgtatagaactgttcctattttctgcacttgccattccagctgcctccactgtccatacccacctcattcatcctgtcacagaaggcaggaaaactgggaactttaccaaagtagcactcagcctgagaggcctgtataatcatgcttttcaaactaaattcacttaaaaattaaaaagcagaattgaatattttaagcagcctcagtacctttggccaatgctgttttcatggtggattatgaacattatataatctttgggaaaagtgaaagtagtacaatttttagaataatgacaactgcctcactgcatctctccactcacacagcaaccgtgtagccccctaagctgcagtaccatgactaaccatgatgtcaatttcatatgctgatcctcacaacagcagtgcacaaacatgccccaaatattttaacagaatttagctcttccttaagctgtcttttcatagtaaaaacaaaacaaaaacacccaatgttaaaaccacataataaacttacaaacttgaaaaattagacacttcagatagataggcaataaaacttcatattatgaaagcaatatattccaagtttcaaagatttgacaagttctgtagagtatctttcatcagtacatgaaaacttccaaactgcatgatcttctgccaggcaggactgggtgctattcgctggtttgaggtcgaatccatttcaaggcatgtcgtggtgggacattaatggtgggatggtagaatgtgcagtccggtcttgtacattgagtgttaaacctacaatgttttggatgatagaagggacattccatcttcttacaagcagggaagtaacggcagagctgactactggaaggtggtgctggtggtgcaactgctggttttggagacagtactggaattcttctactcacatgagtgaagggacaatctggtttagtacactttgcatcatatttacaatttgggtgaacaaacaaacatttttcagcaaatttacaattggggaaggctttgcagggtgagatggggtgatggtaggcacactcatccccatttttacaagcaggccagtacttgcagcgctccaaaagtttttctggtttctgtgccacactcagttcactcatctcagcgttagaaaagctaccatttgggtcctcaagctgcctgctcagcaagtgcaactgctgtgggtggaggagacctctgagtcccttgtttgaggctgcagtttggtttacgggtttcattccttcaaagcacatgtcctcctcttgatctgacatgtatcctggggggctggggacaccatccagcgtcactataaacttgggacttgcaggtttatctggttgtacaagatctcttgactcatctgcagagtttctgccattactgggtcgatttgcagtcgggataataattgcctctgttgagttccttgatttttttctacagaatctccttttgtttcctcttctttaatggggggacttattctgggggtcctactttgtccctggaccacttctgctagcaattcttcttgagaagttcgagttctgggagcaactggaagtgtctgtttctgtggaactgtagagtagttagttgtttttgttacggattcttgagcttcagatatagccttcaaaatcagattcttgttagcttgtttagaaggtggaagagaaggtctcctttcaggctttgcaggcacagacacactgctggagatgcttcctgttcgagacccgtaatcatcatcttcttcctcctcttctccatcatgattgaatttttttactttaacaactgaacttaccacaggcaactttctcttccgaaagttttcatcctccatactcattttctccgagttgtttctaaagaacggactatacgtttcttctaagctgttaagcacctctggttcacacaaacgtcctgtttcatatacccaactactctgcatatcaagctgcttggcagcatgaatactattctgctgctgttgaaattgcaacctgtttaaatgaacaccactatctgcatttctacttgcaggtggtcgataaatttcaatagaagggcgagaagaaccatatgtaagtgtcactgtaggttttttctgagataagggattctcctgcacaaagttgaggtcttcgtcaatgagatcatctggttctggcttaatatcaatcacatcttcagagggtgctggctccctcaaaggtttcactgttgacattagtcgggttgcagctccatcatcgtaagtctgtctgacatttgtggtttttgactcctgcgaacttgtagaaactctggaatctcttttttcaggtctcgcgctaggaatggcaagtggtggcactgcagcttcatgcctcctctcatctccccgactgaaattgctcttgtttgaaggcacgttactatcaaagatgttggtatcagaagacttcagactagagggttcagttgtaacagagcgaagtttatctaatacaccatgaagccatacggtgaatcgaattgtgttgttccctagaaacagggacagatcctctgtcatttggtcctgacttttcttgttggccaccatcaccataatgtaatcaggaagttcttcatcaacataagctcctaattcttgtaatttccccttaatggcactccggatcttgcggctgatctcggtgccgatctccatggctctgcggcgtgcgggaactcagcactgcgcggcgcttggcttacccggaggctgccgcggactcctaccccgcagccgggacaccaccgcctcc

SEQ ID NO: 9875 - RNA, 4026 nt, Homo sapiens
  source 1..4026: mol_type = other RNA
caaagtgcttacagtgcaggtagaaactctgtaaccttaagcatgtaaactacatagaataaaactgtttccactgcatttctgtccttcaaagtggccaacctgattaagtcagccttaatcactgctgctgtcagtttcacgactaaaggtcatattgactaagtagtcatcagctgaccacctcgctgtatcagccagcaacgaggggaaggtgaagaaacatgataggccatatagaatctgccctatgtttacttttttaacccagataattatttttgtgtgcagtatctaagctcctgattgtgtaacctgggacttctggcaccttttgttccattcattttatgtataaaatgcatgccaaagcacactgtgccctctggtacccttgcttccaatcgccaaccatgctcatttccttcctttttttgtggtccctttttgtggtgatcattttaaaccacgtcatccaacaaatgttttatggtcaaccttagcttgttcataagccatagcaactgaaagattaaactcttaaatatgtgtctgggcagtggctattaaatagcaaaaaacaatcagattttagtattttattatttccttgtaaaatggctgaactaaattaaacccttgtttcccatttgttctataatttatagtgaaactgagaacaaaactatctttataaatgatagctaaaagtatttccagatatttaaacaatttaaaataaatttcttctgcagagatgcaaagcatctcaacactggaatgaacaaatgccttaaattcaatggagtaaacctttagaatgaagaggaactgtcatttcacccaagccgaagacaacagccttatgcacttgtgtgctctgtctttgctgcttctcgtgtttcaagcctttcctgtgggatcagcacagcaaagtgcaacttaccaaatggtttaatgactggttaattctttcttctcccaatggaaaagcaatggcaacacaacagtagactgctggcttgacaatcttaaacgtgagcctttgcacatgtaggtttatcatcatttgagtatacgactaagcaagtcaatgaactttttttttttttttagcagtttaatttggtcctgagaatgttgcagtctttattaccccttttgcattaatccacttttctaaccaccttttaagctttaatttttaacactatacaccaagtctttgaaatcagtgatctgttatttaactctaaagcatttgacacttcttgccttaacagttttaaaaaccacacacaaaaaaactctgtaagtaatacagtaggccaaaagtttcatcctatctatcttgcagtttacctatctgatctgatctctgtaattatagttctgtcatttaaaatatactatttaaatctaatttttacatttcaaaaattatcttcagtagtaactaagtatattttctgtggattctgagaatgttatttttcagaatgtgagaatatatatgtacatttataatcttgtgactttaaagtctgttttcagatacagtatgtaaatacttgtaaaaaaatttgtataattttgtgataatgtagtttcccaaaaaaattatttagaaggcattatgttattagtaaatgagagcactgtatagaactgttcctattttctgcacttgccattccagctgcctccactgtccatacccacctcattcatcctgtcacagaaggcaggaaaactgggaactttaccaaagtagcactcagcctgagaggcctgtataatcatgcttttcaaactaaattcacttaaaaattaaaaagcagaattgaatattttaagcagcctcagtacctttggccaatgctgttttcatggtggattatgaacattatataatctttgggaaaagtgaaagtagtacaatttttagaataatgacaactgcctcactgcatctctccactcacacagcaaccgtgtagccccctaagctgcagtaccatgactaaccatgatgtcaatttcatatgctgatcctcacaacagcagtgcacaaacatgccccaaatattttaacagaatttagctcttccttaagctgtcttttcatagtaaaaacaaaacaaaaacacccaatgttaaaaccacataataaacttacaaacttgaaaaattagacacttcagatagataggcaataaaacttcatattatgaaagcaatatattccaagtttcaaagatttgacaagttctgtagagtatctttcatcagtacatgaaaacttccaaactgcatgatcttctgccaggcaggactgggtgctattcgctggtttgaggtcgaatccatttcaaggcatgtcgtggtgggacattaatggtgggatggtagaatgtgcagtccggtcttgtacattgagtgttaaacctacaatgttttggatgatagaagggacattccatcttcttacaagcagggaagtaacggcagagctgactactggaaggtggtgctggtggtgcaactgctggttttggagacagtactggaattcttctactcacatgagtgaagggacaatctggtttagtacactttgcatcatatttacaatttgggtgaacaaacaaacatttttcagcaaatttacaattggggaaggctttgcagggtgagatggggtgatggtaggcacactcatccccatttttacaagcaggccagtacttgcagcgctccaaaagtttttctggtttctgtgccacactcagttcactcatctcagctgtagagtagttagttgtttttgttacggattcttgagcttcagatatagccttcaaaatcagattcttgttagcttgtttagaaggtggaagagaaggtctcctttcaggctttgcaggcacagacacactgctggagatgcttcctgttcgagacccgtaatcatcatcttcttcctcctcttctccatcatgattgaatttttttactttaacaactgaacttaccacaggcaactttctcttccgaaagttttcatcctccatactcattttctccgagttgtttctaaagaacggactatacgtttcttctaagctgttaagcacctctggttcacacaaacgtcctgtttcatatacccaactactctgcatatcaagctgcttggcagcatgaatactattctgctgctgttgaaattgcaacctgtttaaatgaacaccactatctgcatttctacttgcaggtggtcgataaatttcaatagaagggcgagaagaaccatatgtaagtgtcactgtaggttttttctgagataagggattctcctgcacaaagttgaggtcttcgtcaatgagatcatctggttctggcttaatatcaatcacatcttcagagggtgctggctccctcaaaggtttcactgttgacattagtcgggttgcagctccatcatcgtaagtctgtctgacatttgtggtttttgactcctgcgaacttgtagaaactctggaatctcttttttcaggtctcgcgctaggaatggcaagtggtggcactgcagcttcatgcctcctctcatctccccgactgaaattgctcttgtttgaaggcacgttactatcaaagatgttggtatcagaagacttcagactagagggttcagttgtaacagagcgaagtttatctaatacaccatgaagccatacggtgaatcgaattgtgttgttccctagaaacagggacagatcctctgtcatttggtcctgacttttcttgttggccaccatcaccataatgtaatcaggaagttcttcatcaacataagctcctaattcttgtaatttccccttaatggcactccggatcttgcggctgatctcggtgccgatctccatggctctgcggcgtgcgggaactcagcactgcgcggcgcttggcttacccggaggctgccgcggactcctaccccgcagccgggacaccaccgcctcc

SEQ ID NO: 9876 - RNA, 4142 nt, Homo sapiens
  source 1..4142: mol_type = other RNA
caaagtgcttacagtgcaggtagaaactctgtaaccttaagcatgtaaactacatagaataaaactgtttccactgcatttctgtccttcaaagtggccaacctgattaagtcagccttaatcactgctgctgtcagtttcacgactaaaggtcatattgactaagtagtcatcagctgaccacctcgctgtatcagccagcaacgaggggaaggtgaagaaacatgataggccatatagaatctgccctatgtttacttttttaacccagataattatttttgtgtgcagtatctaagctcctgattgtgtaacctgggacttctggcaccttttgttccattcattttatgtataaaatgcatgccaaagcacactgtgccctctggtacccttgcttccaatcgccaaccatgctcatttccttcctttttttgtggtccctttttgtggtgatcattttaaaccacgtcatccaacaaatgttttatggtcaaccttagcttgttcataagccatagcaactgaaagattaaactcttaaatatgtgtctgggcagtggctattaaatagcaaaaaacaatcagattttagtattttattatttccttgtaaaatggctgaactaaattaaacccttgtttcccatttgttctataatttatagtgaaactgagaacaaaactatctttataaatgatagctaaaagtatttccagatatttaaacaatttaaaataaatttcttctgcagagatgcaaagcatctcaacactggaatgaacaaatgccttaaattcaatggagtaaacctttagaatgaagaggaactgtcatttcacccaagccgaagacaacagccttatgcacttgtgtgctctgtctttgctgcttctcgtgtttcaagcctttcctgtgggatcagcacagcaaagtgcaacttaccaaatggtttaatgactggttaattctttcttctcccaatggaaaagcaatggcaacacaacagtagactgctggcttgacaatcttaaacgtgagcctttgcacatgtaggtttatcatcatttgagtatacgactaagcaagtcaatgaactttttttttttttttagcagtttaatttggtcctgagaatgttgcagtctttattaccccttttgcattaatccacttttctaaccaccttttaagctttaatttttaacactatacaccaagtctttgaaatcagtgatctgttatttaactctaaagcatttgacacttcttgccttaacagttttaaaaaccacacacaaaaaaactctgtaagtaatacagtaggccaaaagtttcatcctatctatcttgcagtttacctatctgatctgatctctgtaattatagttctgtcatttaaaatatactatttaaatctaatttttacatttcaaaaattatcttcagtagtaactaagtatattttctgtggattctgagaatgttatttttcagaatgtgagaatatatatgtacatttataatcttgtgactttaaagtctgttttcagatacagtatgtaaatacttgtaaaaaaatttgtataattttgtgataatgtagtttcccaaaaaaattatttagaaggcattatgttattagtaaatgagagcactgtatagaactgttcctattttctgcacttgccattccagctgcctccactgtccatacccacctcattcatcctgtcacagaaggcaggaaaactgggaactttaccaaagtagcactcagcctgagaggcctgtataatcatgcttttcaaactaaattcacttaaaaattaaaaagcagaattgaatattttaagcagcctcagtacctttggccaatgctgttttcatggtggattatgaacattatataatctttgggaaaagtgaaagtagtacaatttttagaataatgacaactgcctcactgcatctctccactcacacagcaaccgtgtagccccctaagctgcagtaccatgactaaccatgatgtcaatttcatatgctgatcctcacaacagcagtgcacaaacatgccccaaatattttaacagaatttagctcttccttaagctgtcttttcatagtaaaaacaaaacaaaaacacccaatgttaaaaccacataataaacttacaaacttgaaaaattagacacttcagatagataggcaataaaacttcatattatgaaagcaatatattccaagtttcaaagatttgacaagttctgtagagtatctttcatcagtacatgaaaacttccaaactgcatgatcttctgccaggcaggactgggtgctattcgctggtttgaggtcgaatccatttcaaggcatgtcgtggtgggacattaatggtgggatggtagaatgtgcagtccggtcttgtacattgagtgttaaacctacaatgttttggatgatagaagggacattccatcttcttacaagcagggaagtaacggcagagctgactactggaaggtggtgctggtggtgcaactgctggttttggagacagtactggaattcttctactcacatgagtgaagggacaatctggtttagtacactttgcatcatatttacaatttgggtgaacaaacaaacatttttcagcaaatttacaattggggaaggctttgcagggtgagatggggtgatggtaggcacactcatccccatttttacaagcaggccagtacttgcagcgctccaaaagtttttctggtttctgtgccacactcagttcactcatctcagcttgactcatctgcagagtttctgccattactgggtcgatttgcagtcgggataataattgcctctgttgagttccttgatttttttctacagaatctccttttgtttcctcttctttaatggggggacttattctgggggtcctactttgtccctggaccacttctgctagcaattcttcttgagaagttcgagttctgggagcaactggaagtgtctgtttctgtggaactgtagagtagttagttgtttttgttacggattcttgagcttcagatatagccttcaaaatcagattcttgttagcttgtttagaaggtggaagagaaggtctcctttcaggctttgcaggcacagacacactgctggagatgcttcctgttcgagacccgtaatcatcatcttcttcctcctcttctccatcatgattgaatttttttactttaacaactgaacttaccacaggcaactttctcttccgaaagttttcatcctccatactcattttctccgagttgtttctaaagaacggactatacgtttcttctaagctgttaagcacctctggttcacacaaacgtcctgtttcatatacccaactactctgcatatcaagctgcttggcagcatgaatactattctgctgctgttgaaattgcaacctgtttaaatgaacaccactatctgcatttctacttgcaggtggtcgataaatttcaatagaagggcgagaagaaccatatgtaagtgtcactgtaggttttttctgagataagggattctcctgcacaaagttgaggtcttcgtcaatgagatcatctggttctggcttaatatcaatcacatcttcagagggtgctggctccctcaaaggtttcactgttgacattagtcgggttgcagctccatcatcgtaagtctgtctgacatttgtggtttttgactcctgcgaacttgtagaaactctggaatctcttttttcaggtctcgcgctaggaatggcaagtggtggcactgcagcttcatgcctcctctcatctccccgactgaaattgctcttgtttgaaggcacgttactatcaaagatgttggtatcagaagacttcagactagagggttcagttgtaacagagcgaagtttatctaatacaccatgaagccaacataagctcctaattcttgtaatttccccttaatggcactccggatcttgcggctgatctcggtgccgatctccatggctctgcggcgtgcgggaactcagcactgcgcggcgcttggcttacccggaggctgccgcggactcctaccccgcagccgggacaccaccgcctcc

SEQ ID NO: 9877 - RNA, 4257 nt, Homo sapiens
  source 1..4257: mol_type = other RNA
caaagtgcttacagtgcaggtagaaactctgtaaccttaagcatgtaaactacatagaataaaactgtttccactgcatttctgtccttcaaagtggccaacctgattaagtcagccttaatcactgctgctgtcagtttcacgactaaaggtcatattgactaagtagtcatcagctgaccacctcgctgtatcagccagcaacgaggggaaggtgaagaaacatgataggccatatagaatctgccctatgtttacttttttaacccagataattatttttgtgtgcagtatctaagctcctgattgtgtaacctgggacttctggcaccttttgttccattcattttatgtataaaatgcatgccaaagcacactgtgccctctggtacccttgcttccaatcgccaaccatgctcatttccttcctttttttgtggtccctttttgtggtgatcattttaaaccacgtcatccaacaaatgttttatggtcaaccttagcttgttcataagccatagcaactgaaagattaaactcttaaatatgtgtctgggcagtggctattaaatagcaaaaaacaatcagattttagtattttattatttccttgtaaaatggctgaactaaattaaacccttgtttcccatttgttctataatttatagtgaaactgagaacaaaactatctttataaatgatagctaaaagtatttccagatatttaaacaatttaaaataaatttcttctgcagagatgcaaagcatctcaacactggaatgaacaaatgccttaaattcaatggagtaaacctttagaatgaagaggaactgtcatttcacccaagccgaagacaacagccttatgcacttgtgtgctctgtctttgctgcttctcgtgtttcaagcctttcctgtgggatcagcacagcaaagtgcaacttaccaaatggtttaatgactggttaattctttcttctcccaatggaaaagcaatggcaacacaacagtagactgctggcttgacaatcttaaacgtgagcctttgcacatgtaggtttatcatcatttgagtatacgactaagcaagtcaatgaactttttttttttttttagcagtttaatttggtcctgagaatgttgcagtctttattaccccttttgcattaatccacttttctaaccaccttttaagctttaatttttaacactatacaccaagtctttgaaatcagtgatctgttatttaactctaaagcatttgacacttcttgccttaacagttttaaaaaccacacacaaaaaaactctgtaagtaatacagtaggccaaaagtttcatcctatctatcttgcagtttacctatctgatctgatctctgtaattatagttctgtcatttaaaatatactatttaaatctaatttttacatttcaaaaattatcttcagtagtaactaagtatattttctgtggattctgagaatgttatttttcagaatgtgagaatatatatgtacatttataatcttgtgactttaaagtctgttttcagatacagtatgtaaatacttgtaaaaaaatttgtataattttgtgataatgtagtttcccaaaaaaattatttagaaggcattatgttattagtaaatgagagcactgtatagaactgttcctattttctgcacttgccattccagctgcctccactgtccatacccacctcattcatcctgtcacagaaggcaggaaaactgggaactttaccaaagtagcactcagcctgagaggcctgtataatcatgcttttcaaactaaattcacttaaaaattaaaaagcagaattgaatattttaagcagcctcagtacctttggccaatgctgttttcatggtggattatgaacattatataatctttgggaaaagtgaaagtagtacaatttttagaataatgacaactgcctcactgcatctctccactcacacagcaaccgtgtagccccctaagctgcagtaccatgactaaccatgatgtcaatttcatatgctgatcctcacaacagcagtgcacaaacatgccccaaatattttaacagaatttagctcttccttaagctgtcttttcatagtaaaaacaaaacaaaaacacccaatgttaaaaccacataataaacttacaaacttgaaaaattagacacttcagatagataggcaataaaacttcatattatgaaagcaatatattccaagtttcaaagatttgacaagttctgtagagtatctttcatcagtacatgaaaacttccaaactgcatgatcttctgccaggcaggactgggtgctattcgctggtttgaggtcgaatccatttcaaggcatgtcgtggtgggacattaatggtgggatggtagaatgtgcagtccggtcttgtacattgagtgttaaacctacaatgttttggatgatagaagggacattccatcttcttacaagcagggaagtaacggcagagctgactactggaaggtggtgctggtggtgcaactgctggttttggagacagtactggaattcttctactcacatgagtgaagggacaatctggtttagtacactttgcatcatatttacaatttgggtgaacaaacaaacatttttcagcaaatttacaattggggaaggctttgcagggtgagatggggtgatggtaggcacactcatccccatttttacaagcaggccagtacttgcagcgctccaaaagtttttctggtttctgtgccacactcagttcactcatctcagcttgactcatctgcagagtttctgccattactgggtcgatttgcagtcgggataataattgcctctgttgagttccttgatttttttctacagaatctccttttgtttcctcttctttaatggggggacttattctgggggtcctactttgtccctggaccacttctgctagcaattcttcttgagaagttcgagttctgggagcaactggaagtgtctgtttctgtggaactgtagagtagttagttgtttttgttacggattcttgagcttcagatatagccttcaaaatcagattcttgttagcttgtttagaaggtggaagagaaggtctcctttcaggctttgcaggcacagacacactgctggagatgcttcctgttcgagacccgtaatcatcatcttcttcctcctcttctccatcatgattgaatttttttactttaacaactgaacttaccacaggcaactttctcttccgaaagttttcatcctccatactcattttctccgagttgtttctaaagaacggactatacgtttcttctaagctgttaagcacctctggttcacacaaacgtcctgtttcatatacccaactactctgcatatcaagctgcttggcagcatgaatactattctgctgctgttgaaattgcaacctgtttaaatgaacaccactatctgcatttctacttgcaggtggtcgataaatttcaatagaagggcgagaagaaccatatgtaagtgtcactgtaggttttttctgagataagggattctcctgcacaaagttgaggtcttcgtcaatgagatcatctggttctggcttaatatcaatcacatcttcagagggtgctggctccctcaaaggtttcactgttgacattagtcgggttgcagctccatcatcgtaagtctgtctgacatttgtggtttttgactcctgcgaacttgtagaaactctggaatctcttttttcaggtctcgcgctaggaatggcaagtggtggcactgcagcttcatgcctcctctcatctccccgactgaaattgctcttgtttgaaggcacgttactatcaaagatgttggtatcagaagacttcagactagagggttcagttgtaacagagcgaagtttatctaatacaccatgaagccatacggtgaatcgaattgtgttgttccctagaaacagggacagatcctctgtcatttggtcctgacttttcttgttggccaccatcaccataatgtaatcaggaagttcttcatcaacataagctcctaattcttgtaatttccccttaatggcactccggatcttgcggctgatctcggtgccgatctccatggctctgcggcgtgcgggaactcagcactgcgcggcgcttggcttacccggaggctgccgcggactcctaccccgcagccgggacaccaccgcctcc

SEQ ID NO: 9878 - RNA, 4233 nt, Homo sapiens
  source 1..4233: mol_type = other RNA
caaagtgcttacagtgcaggtagaaactctgtaaccttaagcatgtaaactacatagaataaaactgtttccactgcatttctgtccttcaaagtggccaacctgattaagtcagccttaatcactgctgctgtcagtttcacgactaaaggtcatattgactaagtagtcatcagctgaccacctcgctgtatcagccagcaacgaggggaaggtgaagaaacatgataggccatatagaatctgccctatgtttacttttttaacccagataattatttttgtgtgcagtatctaagctcctgattgtgtaacctgggacttctggcaccttttgttccattcattttatgtataaaatgcatgccaaagcacactgtgccctctggtacccttgcttccaatcgccaaccatgctcatttccttcctttttttgtggtccctttttgtggtgatcattttaaaccacgtcatccaacaaatgttttatggtcaaccttagcttgttcataagccatagcaactgaaagattaaactcttaaatatgtgtctgggcagtggctattaaatagcaaaaaacaatcagattttagtattttattatttccttgtaaaatggctgaactaaattaaacccttgtttcccatttgttctataatttatagtgaaactgagaacaaaactatctttataaatgatagctaaaagtatttccagatatttaaacaatttaaaataaatttcttctgcagagatgcaaagcatctcaacactggaatgaacaaatgccttaaattcaatggagtaaacctttagaatgaagaggaactgtcatttcacccaagccgaagacaacagccttatgcacttgtgtgctctgtctttgctgcttctcgtgtttcaagcctttcctgtgggatcagcacagcaaagtgcaacttaccaaatggtttaatgactggttaattctttcttctcccaatggaaaagcaatggcaacacaacagtagactgctggcttgacaatcttaaacgtgagcctttgcacatgtaggtttatcatcatttgagtatacgactaagcaagtcaatgaactttttttttttttttagcagtttaatttggtcctgagaatgttgcagtctttattaccccttttgcattaatccacttttctaaccaccttttaagctttaatttttaacactatacaccaagtctttgaaatcagtgatctgttatttaactctaaagcatttgacacttcttgccttaacagttttaaaaaccacacacaaaaaaactctgtaagtaatacagtaggccaaaagtttcatcctatctatcttgcagtttacctatctgatctgatctctgtaattatagttctgtcatttaaaatatactatttaaatctaatttttacatttcaaaaattatcttcagtagtaactaagtatattttctgtggattctgagaatgttatttttcagaatgtgagaatatatatgtacatttataatcttgtgactttaaagtctgttttcagatacagtatgtaaatacttgtaaaaaaatttgtataattttgtgataatgtagtttcccaaaaaaattatttagaaggcattatgttattagtaaatgagagcactgtatagaactgttcctattttctgcacttgccattccagctgcctccactgtccatacccacctcattcatcctgtcacagaaggcaggaaaactgggaactttaccaaagtagcactcagcctgagaggcctgtataatcatgcttttcaaactaaattcacttaaaaattaaaaagcagaattgaatattttaagcagcctcagtacctttggccaatgctgttttcatggtggattatgaacattatataatctttgggaaaagtgaaagtagtacaatttttagaataatgacaactgcctcactgcatctctccactcacacagcaaccgtgtagccccctaagctgcagtaccatgactaaccatgatgtcaatttcatatgctgatcctcacaacagcagtgcacaaacatgccccaaatattttaacagaatttagctcttccttaagctgtcttttcatagtaaaaacaaaacaaaaacacccaatgttaaaaccacataataaacttacaaacttgaaaaattagacacttcagatagataggcaataaaacttcatattatgaaagcaatatattccaagtttcaaagatttgacaagttctgtagagtatctttcatcagtacatgaaaacttccaaactgcatgatcttctgccaggcaggactgggtgctattcgctggtttgaggtcgaatccatttcaaggcatgtcgtggtgggacattaatggtgggatggtagaatgtgcagtccggtcttgtacattgagtgttaaacctacaatgttttggatgatagaagggacattccatcttcttacaagcagggaagtaacggcagagctgactactggaaggtggtgctggtggtgcaactgctggttttggagacagtactggaattcttctactcacatgagtgaagggacaatctggtttagtacactttgcatcatatttacaatttgggtgaacaaacaaacatttttcagcaaatttacaattggggaaggctttgcagggtgagatggggtgatggtaggcacactcatccccatttttacaagcaggccagtacttgcagcgctccaaaagtttttctggtttctgtgccacactcagttcactcatctcagcttgactcatctgcagagtttctgccattactgggtcgatttgcagtcgggataataattgcctctgttgagttccttgatttttttctacagaatctccttttgtttcctcttctttaatggggggacttattctgggggtcctactttgtccctggaccacttctgctagcaattcttcttgagaagttcgagttctgggagcaactggaagtgtctgtttctgtggaactgtagagtagttagttgtttttgttacggattcttgagcttcagatatagccttcaaaatcagattcttgttagcttgtttagaaggtggaagagaaggtctcctttcaggctttgcaggcacagacacactgctggagatgcttcctgttcgagacccgtaatcatcatcttcttcctcctcttctccatcatgattgaatttttttactttaacaactgaacttaccacaggcaactttctcttccgaaagttttcatcctccatactcattttctccgagttgtttctaaagaacggactatacgtttcttctaagctgttaagcacctctggttcacacaaacgtcctgtttcatatacccaactactctgcatatcaagctgcttggcagcatgaatactattctgctgctgttgaaattgcaacctgtttaaatgaacaccactatctgcatttctacttgcaggtggtcgataaatttcaatagaagggcgagaagaaccatatgtaagtgtcactgtaggttttttctgagataagggattctcctgcacaaagttgaggtcttcgtcaatgagatcatctggttctggcttaatatcaatcacatcttcagagggtgctggctccctcaaaggtttcactgttgacattagtcgggttgcagctccatcatcgtaagtctgtctgacatttgtggtttttgactcctgcgaacttgtagaaactctggaatctcttttttcaggtctcgcgctaggaatggcaagtggtggcactgcagcttcatgcctcctctcatctccccgactgaaattgctcttgtttgaaggcacgttactatcaaagatgttggtatcagaagacttcagactagagggttcagttgtaacagagcgaagtttatctaatacaccatgaagccatacggtgaatcgaattgtgttgttccctagaaacagggacagatcctctgtcatttggtcctgacttttcttgttggccaccatcaccataatgtaatcaggaagttcttcatcaacataagctcctaattcttgtaatttccccttaatggcactctcccgcagcggatccaaagcggcgccgtgcgccgcggtggtggctccagccgggcctgcgcctgtccttccatttcccggcggctacttcagccgcagccacgctccg

SEQ ID NO: 9879 - RNA, 4067 nt, Homo sapiens
  source 1..4067: mol_type = other RNA
caaagtgcttacagtgcaggtagaaactctgtaaccttaagcatgtaaactacatagaataaaactgtttccactgcatttctgtccttcaaagtggccaacctgattaagtcagccttaatcactgctgctgtcagtttcacgactaaaggtcatattgactaagtagtcatcagctgaccacctcgctgtatcagccagcaacgaggggaaggtgaagaaacatgataggccatatagaatctgccctatgtttacttttttaacccagataattatttttgtgtgcagtatctaagctcctgattgtgtaacctgggacttctggcaccttttgttccattcattttatgtataaaatgcatgccaaagcacactgtgccctctggtacccttgcttccaatcgccaaccatgctcatttccttcctttttttgtggtccctttttgtggtgatcattttaaaccacgtcatccaacaaatgttttatggtcaaccttagcttgttcataagccatagcaactgaaagattaaactcttaaatatgtgtctgggcagtggctattaaatagcaaaaaacaatcagattttagtattttattatttccttgtaaaatggctgaactaaattaaacccttgtttcccatttgttctataatttatagtgaaactgagaacaaaactatctttataaatgatagctaaaagtatttccagatatttaaacaatttaaaataaatttcttctgcagagatgcaaagcatctcaacactggaatgaacaaatgccttaaattcaatggagtaaacctttagaatgaagaggaactgtcatttcacccaagccgaagacaacagccttatgcacttgtgtgctctgtctttgctgcttctcgtgtttcaagcctttcctgtgggatcagcacagcaaagtgcaacttaccaaatggtttaatgactggttaattctttcttctcccaatggaaaagcaatggcaacacaacagtagactgctggcttgacaatcttaaacgtgagcctttgcacatgtaggtttatcatcatttgagtatacgactaagcaagtcaatgaactttttttttttttttagcagtttaatttggtcctgagaatgttgcagtctttattaccccttttgcattaatccacttttctaaccaccttttaagctttaatttttaacactatacaccaagtctttgaaatcagtgatctgttatttaactctaaagcatttgacacttcttgccttaacagttttaaaaaccacacacaaaaaaactctgtaagtaatacagtaggccaaaagtttcatcctatctatcttgcagtttacctatctgatctgatctctgtaattatagttctgtcatttaaaatatactatttaaatctaatttttacatttcaaaaattatcttcagtagtaactaagtatattttctgtggattctgagaatgttatttttcagaatgtgagaatatatatgtacatttataatcttgtgactttaaagtctgttttcagatacagtatgtaaatacttgtaaaaaaatttgtataattttgtgataatgtagtttcccaaaaaaattatttagaaggcattatgttattagtaaatgagagcactgtatagaactgttcctattttctgcacttgccattccagctgcctccactgtccatacccacctcattcatcctgtcacagaaggcaggaaaactgggaactttaccaaagtagcactcagcctgagaggcctgtataatcatgcttttcaaactaaattcacttaaaaattaaaaagcagaattgaatattttaagcagcctcagtacctttggccaatgctgttttcatggtggattatgaacattatataatctttgggaaaagtgaaagtagtacaatttttagaataatgacaactgcctcactgcatctctccactcacacagcaaccgtgtagccccctaagctgcagtaccatgactaaccatgatgtcaatttcatatgctgatcctcacaacagcagtgcacaaacatgccccaaatattttaacagaatttagctcttccttaagctgtcttttcatagtaaaaacaaaacaaaaacacccaatgttaaaaccacataataaacttacaaacttgaaaaattagacacttcagatagataggcaataaaacttcatattatgaaagcaatatattccaagtttcaaagatttgacaagttctgtagagtatctttcatcagtacatgaaaacttccaaactgcatgatcttctgccaggcaggactgggtgctattcgctggtttgaggtcgaatccatttcaaggcatgtcgtggtgggacattaatggtgggatggtagaatgtgcagtccggtcttgtacattgagtgttaaacctacaatgttttggatgatagaagggacattccatcttcttacaagcagggaagtaacggcagagctgactactggaaggtggtgctggtggtgcaactgctggttttggagacagtactggaattcttctactcacatgagtgaagggacaatctggtttagtacactttgcatcatatttacaatttgggtgaacaaacaaacatttttcagcaaatttacaattggggaaggctttgcagggtgagatggggtgatggtaggcacactcatccccatttttacaagcaggccagtacttgcagcgctccaaaagtttttctggtttctgtgccacactcagttcactcatctcagcttgatttttttctacagaatctccttttgtttcctcttctttaatggggggacttattctgggggtcctactttgtccctggaccacttctgctagcaattcttcttgagaagttcgagttctgggagcaactggaagtgtctgtttctgtggaactgtagagtagttagttgtttttgttacggattcttgagcttcagatatagccttcaaaatcagattcttgttagcttgtttagaaggtggaagagaaggtctcctttcaggctttgcaggcacagacacactgctggagatgcttcctgttcgagacccgtaatcatcatcttcttcctcctcttctccatcatgattgaatttttttactttaacaactgaacttaccacaggcaactttctcttccgaaagttttcatcctccatactcattttctccgagttgtttctaaagaacggactatacgtttcttctaagctgttaagcacctctggttcacacaaacgtcctgtttcatatacccaactactctgcatatcaagctgcttggcagcatgaatactattctgctgctgttgaaattgcaacctgtttaaatgaacaccactatctgcatttctacttgcaggtggtcgataaatttcaatagaagggcgagaagaaccatatgtaagtgtcactgtaggttttttctgagataagggattctcctgcacaaagttgaggtcttcgtcaatgagatcatctggttctggcttaatatcaatcacatcttcagagggtgctggctccctcaaaggtttcactgttgacattagtcgggttgcagctccatcatcgtaagtctgtctgacatttgtggtttttgactcctgcgaacttgtagaaactctggaatctcttttttcaggtctcgcgctaggaatggcaagtggtggcactgcagcttcatgcctcctctcatctccccgactgaaattgctcttgtttgaaggcacgttactatcaaagatgttggtatcagaagacttcagactagagggttcagttgtaacagagcgaagtttatctaatacaccatgaagccaacataagctcctaattcttgtaatttccccttaatggcactccggatcttgcggctgatctcggtgccgatctccatggctctgcggcgtgcgggaactcagcactgcgcggcgcttggcttacccggaggctgccgcggactcctaccccgcagccgggacaccaccgcctcc

SEQ ID NO: 9880 - RNA, 4182 nt, Homo sapiens
  source 1..4182: mol_type = other RNA
caaagtgcttacagtgcaggtagaaactctgtaaccttaagcatgtaaactacatagaataaaactgtttccactgcatttctgtccttcaaagtggccaacctgattaagtcagccttaatcactgctgctgtcagtttcacgactaaaggtcatattgactaagtagtcatcagctgaccacctcgctgtatcagccagcaacgaggggaaggtgaagaaacatgataggccatatagaatctgccctatgtttacttttttaacccagataattatttttgtgtgcagtatctaagctcctgattgtgtaacctgggacttctggcaccttttgttccattcattttatgtataaaatgcatgccaaagcacactgtgccctctggtacccttgcttccaatcgccaaccatgctcatttccttcctttttttgtggtccctttttgtggtgatcattttaaaccacgtcatccaacaaatgttttatggtcaaccttagcttgttcataagccatagcaactgaaagattaaactcttaaatatgtgtctgggcagtggctattaaatagcaaaaaacaatcagattttagtattttattatttccttgtaaaatggctgaactaaattaaacccttgtttcccatttgttctataatttatagtgaaactgagaacaaaactatctttataaatgatagctaaaagtatttccagatatttaaacaatttaaaataaatttcttctgcagagatgcaaagcatctcaacactggaatgaacaaatgccttaaattcaatggagtaaacctttagaatgaagaggaactgtcatttcacccaagccgaagacaacagccttatgcacttgtgtgctctgtctttgctgcttctcgtgtttcaagcctttcctgtgggatcagcacagcaaagtgcaacttaccaaatggtttaatgactggttaattctttcttctcccaatggaaaagcaatggcaacacaacagtagactgctggcttgacaatcttaaacgtgagcctttgcacatgtaggtttatcatcatttgagtatacgactaagcaagtcaatgaactttttttttttttttagcagtttaatttggtcctgagaatgttgcagtctttattaccccttttgcattaatccacttttctaaccaccttttaagctttaatttttaacactatacaccaagtctttgaaatcagtgatctgttatttaactctaaagcatttgacacttcttgccttaacagttttaaaaaccacacacaaaaaaactctgtaagtaatacagtaggccaaaagtttcatcctatctatcttgcagtttacctatctgatctgatctctgtaattatagttctgtcatttaaaatatactatttaaatctaatttttacatttcaaaaattatcttcagtagtaactaagtatattttctgtggattctgagaatgttatttttcagaatgtgagaatatatatgtacatttataatcttgtgactttaaagtctgttttcagatacagtatgtaaatacttgtaaaaaaatttgtataattttgtgataatgtagtttcccaaaaaaattatttagaaggcattatgttattagtaaatgagagcactgtatagaactgttcctattttctgcacttgccattccagctgcctccactgtccatacccacctcattcatcctgtcacagaaggcaggaaaactgggaactttaccaaagtagcactcagcctgagaggcctgtataatcatgcttttcaaactaaattcacttaaaaattaaaaagcagaattgaatattttaagcagcctcagtacctttggccaatgctgttttcatggtggattatgaacattatataatctttgggaaaagtgaaagtagtacaatttttagaataatgacaactgcctcactgcatctctccactcacacagcaaccgtgtagccccctaagctgcagtaccatgactaaccatgatgtcaatttcatatgctgatcctcacaacagcagtgcacaaacatgccccaaatattttaacagaatttagctcttccttaagctgtcttttcatagtaaaaacaaaacaaaaacacccaatgttaaaaccacataataaacttacaaacttgaaaaattagacacttcagatagataggcaataaaacttcatattatgaaagcaatatattccaagtttcaaagatttgacaagttctgtagagtatctttcatcagtacatgaaaacttccaaactgcatgatcttctgccaggcaggactgggtgctattcgctggtttgaggtcgaatccatttcaaggcatgtcgtggtgggacattaatggtgggatggtagaatgtgcagtccggtcttgtacattgagtgttaaacctacaatgttttggatgatagaagggacattccatcttcttacaagcagggaagtaacggcagagctgactactggaaggtggtgctggtggtgcaactgctggttttggagacagtactggaattcttctactcacatgagtgaagggacaatctggtttagtacactttgcatcatatttacaatttgggtgaacaaacaaacatttttcagcaaatttacaattggggaaggctttgcagggtgagatggggtgatggtaggcacactcatccccatttttacaagcaggccagtacttgcagcgctccaaaagtttttctggtttctgtgccacactcagttcactcatctcagcttgatttttttctacagaatctccttttgtttcctcttctttaatggggggacttattctgggggtcctactttgtccctggaccacttctgctagcaattcttcttgagaagttcgagttctgggagcaactggaagtgtctgtttctgtggaactgtagagtagttagttgtttttgttacggattcttgagcttcagatatagccttcaaaatcagattcttgttagcttgtttagaaggtggaagagaaggtctcctttcaggctttgcaggcacagacacactgctggagatgcttcctgttcgagacccgtaatcatcatcttcttcctcctcttctccatcatgattgaatttttttactttaacaactgaacttaccacaggcaactttctcttccgaaagttttcatcctccatactcattttctccgagttgtttctaaagaacggactatacgtttcttctaagctgttaagcacctctggttcacacaaacgtcctgtttcatatacccaactactctgcatatcaagctgcttggcagcatgaatactattctgctgctgttgaaattgcaacctgtttaaatgaacaccactatctgcatttctacttgcaggtggtcgataaatttcaatagaagggcgagaagaaccatatgtaagtgtcactgtaggttttttctgagataagggattctcctgcacaaagttgaggtcttcgtcaatgagatcatctggttctggcttaatatcaatcacatcttcagagggtgctggctccctcaaaggtttcactgttgacattagtcgggttgcagctccatcatcgtaagtctgtctgacatttgtggtttttgactcctgcgaacttgtagaaactctggaatctcttttttcaggtctcgcgctaggaatggcaagtggtggcactgcagcttcatgcctcctctcatctccccgactgaaattgctcttgtttgaaggcacgttactatcaaagatgttggtatcagaagacttcagactagagggttcagttgtaacagagcgaagtttatctaatacaccatgaagccatacggtgaatcgaattgtgttgttccctagaaacagggacagatcctctgtcatttggtcctgacttttcttgttggccaccatcaccataatgtaatcaggaagttcttcatcaacataagctcctaattcttgtaatttccccttaatggcactccggatcttgcggctgatctcggtgccgatctccatggctctgcggcgtgcgggaactcagcactgcgcggcgcttggcttacccggaggctgccgcggactcctaccccgcagccgggacaccaccgcctcc

SEQ ID NO: 9881 - RNA, 4632 nt, Homo sapiens
  source 1..4632: mol_type = other RNA
caaagtgcttacagtgcaggtagaaactctgtaaccttaagcatgtaaactacatagaataaaactgtttccactgcatttctgtccttcaaagtggccaacctgattaagtcagccttaatcactgctgctgtcagtttcacgactaaaggtcatattgactaagtagtcatcagctgaccacctcgctgtatcagccagcaacgaggggaaggtgaagaaacatgataggccatatagaatctgccctatgtttacttttttaacccagataattatttttgtgtgcagtatctaagctcctgattgtgtaacctgggacttctggcaccttttgttccattcattttatgtataaaatgcatgccaaagcacactgtgccctctggtacccttgcttccaatcgccaaccatgctcatttccttcctttttttgtggtccctttttgtggtgatcattttaaaccacgtcatccaacaaatgttttatggtcaaccttagcttgttcataagccatagcaactgaaagattaaactcttaaatatgtgtctgggcagtggctattaaatagcaaaaaacaatcagattttagtattttattatttccttgtaaaatggctgaactaaattaaacccttgtttcccatttgttctataatttatagtgaaactgagaacaaaactatctttataaatgatagctaaaagtatttccagatatttaaacaatttaaaataaatttcttctgcagagatgcaaagcatctcaacactggaatgaacaaatgccttaaattcaatggagtaaacctttagaatgaagaggaactgtcatttcacccaagccgaagacaacagccttatgcacttgtgtgctctgtctttgctgcttctcgtgtttcaagcctttcctgtgggatcagcacagcaaagtgcaacttaccaaatggtttaatgactggttaattctttcttctcccaatggaaaagcaatggcaacacaacagtagactgctggcttgacaatcttaaacgtgagcctttgcacatgtaggtttatcatcatttgagtatacgactaagcaagtcaatgaactttttttttttttttagcagtttaatttggtcctgagaatgttgcagtctttattaccccttttgcattaatccacttttctaaccaccttttaagctttaatttttaacactatacaccaagtctttgaaatcagtgatctgttatttaactctaaagcatttgacacttcttgccttaacagttttaaaaaccacacacaaaaaaactctgtaagtaatacagtaggccaaaagtttcatcctatctatcttgcagtttacctatctgatctgatctctgtaattatagttctgtcatttaaaatatactatttaaatctaatttttacatttcaaaaattatcttcagtagtaactaagtatattttctgtggattctgagaatgttatttttcagaatgtgagaatatatatgtacatttataatcttgtgactttaaagtctgttttcagatacagtatgtaaatacttgtaaaaaaatttgtataattttgtgataatgtagtttcccaaaaaaattatttagaaggcattatgttattagtaaatgagagcactgtatagaactgttcctattttctgcacttgccattccagctgcctccactgtccatacccacctcattcatcctgtcacagaaggcaggaaaactgggaactttaccaaagtagcactcagcctgagaggcctgtataatcatgcttttcaaactaaattcacttaaaaattaaaaagcagaattgaatattttaagcagcctcagtacctttggccaatgctgttttcatggtggattatgaacattatataatctttgggaaaagtgaaagtagtacaatttttagaataatgacaactgcctcactgcatctctccactcacacagcaaccgtgtagccccctaagctgcagtaccatgactaaccatgatgtcaatttcatatgctgatcctcacaacagcagtgcacaaacatgccccaaatattttaacagaatttagctcttccttaagctgtcttttcatagtaaaaacaaaacaaaaacacccaatgttaaaaccacataataaacttacaaacttgaaaaattagacacttcagatagataggcaataaaacttcatattatgaaagcaatatattccaagtttcaaagatttgacaagttctgtagagtatctttcatcagtacatgaaaacttccaaactgcatgatcttctgccaggcaggactgggtgctattcgctggtttgaggtcgaatccatttcaaggcatgtcgtggtgggacattaatggtgggatggtagaatgtgcagtccggtcttgtacattgagtgttaaacctacaatgttttggatgatagaagggacattccatcttcttacaagcagggaagtaacggcagagctgactactggaaggtggtgctggtggtgcaactggttttggagacagtactggaattcttctactcacatgagtgaagggacaatctggtttagtacactttgcatcatatttacaatttgggtgaacaaacaaacatttttcagcaaatttacaattggggaaggctttgcagggtgagatggggtgatggtaggcacactcatccccatttttacaagcaggccagtacttgcagcgctccaaaagtttttctggtttctgtgccacactcagttcactcatctcagcatttgggtcctcaagctgcctgctcagcaagtgcaactgctgtgggtggaggagacctctgagtcccttgtttgaggctgcagtttggtttacgggtttcattccttcaaagcacatgtcctcctcttgatctgacatgtatcctggggggctggggacaccatccagcgtcactataaacttgggacttgcaggtttatctggttgtacaagatctcgtgtctgcataaggtgtcctgaaagtacccgaagggaatctgcagtcttcatccccgactcttggtttggtgccactactacttcctcagacagctttggcttcttcagaataaatgatcttgtgtctgcatggaccatggattccatgtcatagtaatcttgactcatctgcagagtttctgccattactgggtcgatttgcagtcgggataataattgcctctgttgagttccttgatttttttctacagaatctccttttgtttcctcttctttaatggggggacttattctgggggtcctactttgtccctggaccacttctgctagcaattcttcttgagaagttcgagttctgggagcaactggaagtgtctgtttctgtggaactgtagagtagttagttgtttttgttacggattcttgagcttcagatatagccttcaaaatcagattcttgttagcttgtttagaaggtggaagagaaggtctcctttcaggctttgcaggcacagacacactgctggagatgcttcctgttcgagacccgtaatcatcatcttcttcctcctcttctccatcatgattgaatttttttactttaacaactgaacttaccacaggcaactttctcttccgaaagttttcatcctccatactcattttctccgagttgtttctaaagaacggactatacgtttcttctaagctgttaagcacctctggttcacacaaacgtcctgtttcatatacccaactactctgcatatcaagctgcttggcagcatgaatactattctgctgctgttgaaattgcaacctgtttaaatgaacaccactatctgcatttctacttgcaggtggtcgataaatttcaatagaagggcgagaagaaccatatgtaagtgtcactgtaggttttttctgagataagggattctcctgcacaaagttgaggtcttcgtcaatgagatcatctggttctggcttaatatcaatcacatcttcagagggtgctggctccctcaaaggtttcactgttgacattagtcgggttgcagctccatcatcgtaagtctgtctgacatttgtggtttttgactcctgcgaacttgtagaaactctggaatctcttttttcaggtctcgcgctaggaatggcaagtggtggcactgcagcttcatgcctcctctcatctccccgactgaaattgctcttgtttgaaggcacgttactatcaaagatgttggtatcagaagacttcagactagagggttcagttgtaacagagcgaagtttatctaatacaccatgaagccatacggtgaatcgaattgtgttgttccctagaaacagggacagatcctctgtcatttggtcctgacttttcttgttggccaccatcaccataatgtaatcaggaagttcttcatcaacataagctcctaattcttgtaatttccccttaatggcactccggatcttgcggctgatctcggtgccgatctccatggctctgcggcgtgcgggaactcagcactgcgcggcgcttggcttacccggaggctgccgcggactcctaccccgcagccgggacaccaccgcctcc

SEQ ID NO: 9882 - RNA, 4557 nt, Homo sapiens
  source 1..4557: mol_type = other RNA
caaagtgcttacagtgcaggtagaaactctgtaaccttaagcatgtaaactacatagaataaaactgtttccactgcatttctgtccttcaaagtggccaacctgattaagtcagccttaatcactgctgctgtcagtttcacgactaaaggtcatattgactaagtagtcatcagctgaccacctcgctgtatcagccagcaacgaggggaaggtgaagaaacatgataggccatatagaatctgccctatgtttacttttttaacccagataattatttttgtgtgcagtatctaagctcctgattgtgtaacctgggacttctggcaccttttgttccattcattttatgtataaaatgcatgccaaagcacactgtgccctctggtacccttgcttccaatcgccaaccatgctcatttccttcctttttttgtggtccctttttgtggtgatcattttaaaccacgtcatccaacaaatgttttatggtcaaccttagcttgttcataagccatagcaactgaaagattaaactcttaaatatgtgtctgggcagtggctattaaatagcaaaaaacaatcagattttagtattttattatttccttgtaaaatggctgaactaaattaaacccttgtttcccatttgttctataatttatagtgaaactgagaacaaaactatctttataaatgatagctaaaagtatttccagatatttaaacaatttaaaataaatttcttctgcagagatgcaaagcatctcaacactggaatgaacaaatgccttaaattcaatggagtaaacctttagaatgaagaggaactgtcatttcacccaagccgaagacaacagccttatgcacttgtgtgctctgtctttgctgcttctcgtgtttcaagcctttcctgtgggatcagcacagcaaagtgcaacttaccaaatggtttaatgactggttaattctttcttctcccaatggaaaagcaatggcaacacaacagtagactgctggcttgacaatcttaaacgtgagcctttgcacatgtaggtttatcatcatttgagtatacgactaagcaagtcaatgaactttttttttttttttagcagtttaatttggtcctgagaatgttgcagtctttattaccccttttgcattaatccacttttctaaccaccttttaagctttaatttttaacactatacaccaagtctttgaaatcagtgatctgttatttaactctaaagcatttgacacttcttgccttaacagttttaaaaaccacacacaaaaaaactctgtaagtaatacagtaggccaaaagtttcatcctatctatcttgcagtttacctatctgatctgatctctgtaattatagttctgtcatttaaaatatactatttaaatctaatttttacatttcaaaaattatcttcagtagtaactaagtatattttctgtggattctgagaatgttatttttcagaatgtgagaatatatatgtacatttataatcttgtgactttaaagtctgttttcagatacagtatgtaaatacttgtaaaaaaatttgtataattttgtgataatgtagtttcccaaaaaaattatttagaaggcattatgttattagtaaatgagagcactgtatagaactgttcctattttctgcacttgccattccagctgcctccactgtccatacccacctcattcatcctgtcacagaaggcaggaaaactgggaactttaccaaagtagcactcagcctgagaggcctgtataatcatgcttttcaaactaaattcacttaaaaattaaaaagcagaattgaatattttaagcagcctcagtacctttggccaatgctgttttcatggtggattatgaacattatataatctttgggaaaagtgaaagtagtacaatttttagaataatgacaactgcctcactgcatctctccactcacacagcaaccgtgtagccccctaagctgcagtaccatgactaaccatgatgtcaatttcatatgctgatcctcacaacagcagtgcacaaacatgccccaaatattttaacagaatttagctcttccttaagctgtcttttcatagtaaaaacaaaacaaaaacacccaatgttaaaaccacataataaacttacaaacttgaaaaattagacacttcagatagataggcaataaaacttcatattatgaaagcaatatattccaagtttcaaagatttgacaagttctgtagagtatctttcatcagtacatgaaaacttccaaactgcatgatcttctgccaggcaggactgggtgctattcgctggtttgaggtcgaatccatttcaaggcatgtcgtggtgggacattaatggtgggatggtagaatgtgcagtccggtcttgtacattgagtgttaaacctacaatgttttggatgatagaagggacattccatcttcttacaagcagggaagtaacggcagagctgactactggaaggtggtgctggtggtgcaactggttttggagacagtactggaattcttctactcacatgagtgaagggacaatctggtttagtacactttgcatcatatttacaatttgggtgaacaaacaaacatttttcagcaaatttacaattggggaaggctttgcagggtgagatggggtgatggtaggcacactcatccccatttttacaagcaggccagtacttgcagcgctccaaaagtttttctggtttctgtgccacactcagttcactcatctcagcatttgggtcctcaagctgcctgctcagcaagtgcaactgctgtgggtggaggagacctctgagtcccttgtttgaggctgcagtttggtttacgggtttcattccttcaaagcacatgtcctcctcttgatctgacatgtatcctggggggctggggacaccatccagcgtcactataaacttgggacttgcaggtttatctggttgtacaagatctcgtgtctgcataaggtgtcctgaaagtacccgaagggaatctgcagtcttcatccccgactcttggtttggtgccactactacttcctcagacagctttggcttcttcagaataaatgatcttgtgtctgcatggaccatggattccatgtcatagtaatcttgatttttttctacagaatctccttttgtttcctcttctttaatggggggacttattctgggggtcctactttgtccctggaccacttctgctagcaattcttcttgagaagttcgagttctgggagcaactggaagtgtctgtttctgtggaactgtagagtagttagttgtttttgttacggattcttgagcttcagatatagccttcaaaatcagattcttgttagcttgtttagaaggtggaagagaaggtctcctttcaggctttgcaggcacagacacactgctggagatgcttcctgttcgagacccgtaatcatcatcttcttcctcctcttctccatcatgattgaatttttttactttaacaactgaacttaccacaggcaactttctcttccgaaagttttcatcctccatactcattttctccgagttgtttctaaagaacggactatacgtttcttctaagctgttaagcacctctggttcacacaaacgtcctgtttcatatacccaactactctgcatatcaagctgcttggcagcatgaatactattctgctgctgttgaaattgcaacctgtttaaatgaacaccactatctgcatttctacttgcaggtggtcgataaatttcaatagaagggcgagaagaaccatatgtaagtgtcactgtaggttttttctgagataagggattctcctgcacaaagttgaggtcttcgtcaatgagatcatctggttctggcttaatatcaatcacatcttcagagggtgctggctccctcaaaggtttcactgttgacattagtcgggttgcagctccatcatcgtaagtctgtctgacatttgtggtttttgactcctgcgaacttgtagaaactctggaatctcttttttcaggtctcgcgctaggaatggcaagtggtggcactgcagcttcatgcctcctctcatctccccgactgaaattgctcttgtttgaaggcacgttactatcaaagatgttggtatcagaagacttcagactagagggttcagttgtaacagagcgaagtttatctaatacaccatgaagccatacggtgaatcgaattgtgttgttccctagaaacagggacagatcctctgtcatttggtcctgacttttcttgttggccaccatcaccataatgtaatcaggaagttcttcatcaacataagctcctaattcttgtaatttccccttaatggcactccggatcttgcggctgatctcggtgccgatctccatggctctgcggcgtgcgggaactcagcactgcgcggcgcttggcttacccggaggctgccgcggactcctaccccgcagccgggacaccaccgcctcc

SEQ ID NO: 9883 - RNA, 4532 nt, Homo sapiens
  source 1..4532: mol_type = other RNA
caaagtgcttacagtgcaggtagaaactctgtaaccttaagcatgtaaactacatagaataaaactgtttccactgcatttctgtccttcaaagtggccaacctgattaagtcagccttaatcactgctgctgtcagtttcacgactaaaggtcatattgactaagtagtcatcagctgaccacctcgctgtatcagccagcaacgaggggaaggtgaagaaacatgataggccatatagaatctgccctatgtttacttttttaacccagataattatttttgtgtgcagtatctaagctcctgattgtgtaacctgggacttctggcaccttttgttccattcattttatgtataaaatgcatgccaaagcacactgtgccctctggtacccttgcttccaatcgccaaccatgctcatttccttcctttttttgtggtccctttttgtggtgatcattttaaaccacgtcatccaacaaatgttttatggtcaaccttagcttgttcataagccatagcaactgaaagattaaactcttaaatatgtgtctgggcagtggctattaaatagcaaaaaacaatcagattttagtattttattatttccttgtaaaatggctgaactaaattaaacccttgtttcccatttgttctataatttatagtgaaactgagaacaaaactatctttataaatgatagctaaaagtatttccagatatttaaacaatttaaaataaatttcttctgcagagatgcaaagcatctcaacactggaatgaacaaatgccttaaattcaatggagtaaacctttagaatgaagaggaactgtcatttcacccaagccgaagacaacagccttatgcacttgtgtgctctgtctttgctgcttctcgtgtttcaagcctttcctgtgggatcagcacagcaaagtgcaacttaccaaatggtttaatgactggttaattctttcttctcccaatggaaaagcaatggcaacacaacagtagactgctggcttgacaatcttaaacgtgagcctttgcacatgtaggtttatcatcatttgagtatacgactaagcaagtcaatgaactttttttttttttttagcagtttaatttggtcctgagaatgttgcagtctttattaccccttttgcattaatccacttttctaaccaccttttaagctttaatttttaacactatacaccaagtctttgaaatcagtgatctgttatttaactctaaagcatttgacacttcttgccttaacagttttaaaaaccacacacaaaaaaactctgtaagtaatacagtaggccaaaagtttcatcctatctatcttgcagtttacctatctgatctgatctctgtaattatagttctgtcatttaaaatatactatttaaatctaatttttacatttcaaaaattatcttcagtagtaactaagtatattttctgtggattctgagaatgttatttttcagaatgtgagaatatatatgtacatttataatcttgtgactttaaagtctgttttcagatacagtatgtaaatacttgtaaaaaaatttgtataattttgtgataatgtagtttcccaaaaaaattatttagaaggcattatgttattagtaaatgagagcactgtatagaactgttcctattttctgcacttgccattccagctgcctccactgtccatacccacctcattcatcctgtcacagaaggcaggaaaactgggaactttaccaaagtagcactcagcctgagaggcctgtataatcatgcttttcaaactaaattcacttaaaaattaaaaagcagaattgaatattttaagcagcctcagtacctttggccaatgctgttttcatggtggattatgaacattatataatctttgggaaaagtgaaagtagtacaatttttagaataatgacaactgcctcactgcatctctccactcacacagcaaccgtgtagccccctaagctgcagtaccatgactaaccatgatgtcaatttcatatgctgatcctcacaacagcagtgcacaaacatgccccaaatattttaacagaatttagctcttccttaagctgtcttttcatagtaaaaacaaaacaaaaacacccaatgttaaaaccacataataaacttacaaacttgaaaaattagacacttcagatagataggcaataaaacttcatattatgaaagcaatatattccaagtttcaaagatttgacaagttctgtagagtatctttcatcagtacatgaaaacttccaaactgcatgatcttctgccaggcaggactgggtgctattcgctggtttgaggtcgaatccatttcaaggcatgtcgtggtgggacattaatggtgggatggtagaatgtgcagtccggtcttgtacattgagtgttaaacctacaatgttttggatgatagaagggacattccatcttcttacaagcagggaagtaacggcagagctgactactggaaggtggtgctggtggtgcaactggttttggagacagtactggaattcttctactcacatgagtgaagggacaatctggtttagtacactttgcatcatatttacaatttgggtgaacaaacaaacatttttcagcaaatttacaattggggaaggctttgcagggtgagatggggtgatggtaggcacactcatccccatttttacaagcaggccagtacttgcagcgctccaaaagtttttctggtttctgtgccacactcagttcactcatctcagcgttagaaaagctaccatttgggtcctcaagctgcctgctcagcaagtgcaactgctgtgggtggaggagacctctgagtcccttgtttgaggctgcagtttggtttacgggtttcattccttcaaagcacatgtcctcctcttgatctgacatgtatcctggggggctggggacaccatccagcgtcactataaacttgggacttgcaggtttatctggttgtacaagatctcgtgtctgcataaggtgtcctgaaagtacccgaagggaatctgcagtcttcatccccgactcttggtttggtgccactactacttcctcagacagctttggcttcttcagaataaatgatcttgtgtctgcatggaccatggattccatgtcatagtaatcttgactcatctgcagagtttctgccattactgggtcgatttgcagtcgggataataattgcctctgttgagttccttgatttttttctacagaatctccttttgtttcctcttctttaatggggggacttattctgggggtcctactttgtccctggaccacttctgctagcaattcttcttgagaagttcgagttctgggagcaactggaagtgtctgtttctgtggaactgtagagtagttagttgtttttgttacggattcttgagcttcagatatagccttcaaaatcagattcttgttagcttgtttagaaggtggaagagaaggtctcctttcaggctttgcaggcacagacacactgctggagatgcttcctgttcgagacccgtaatcatcatcttcttcctcctcttctccatcatgattgaatttttttactttaacaactgaacttaccacaggcaactttctcttccgaaagttttcatcctccatactcattttctccgagttgtttctaaagaacggactatacgtttcttctaagctgttaagcacctctggttcacacaaacgtcctgtttcatatacccaactactctgcatatcaagctgcttggcagcatgaatactattctgctgctgttgaaattgcaacctgtttaaatgaacaccactatctgcatttctacttgcaggtggtcgataaatttcaatagaagggcgagaagaaccatatgtaagtgtcactgtaggttttttctgagataagggattctcctgcacaaagttgaggtcttcgtcaatgagatcatctggttctggcttaatatcaatcacatcttcagagggtgctggctccctcaaaggtttcactgttgacattagtcgggttgcagctccatcatcgtaagtctgtctgacatttgtggtttttgactcctgcgaacttgtagaaactctggaatctcttttttcaggtctcgcgctaggaatggcaagtggtggcactgcagcttcatgcctcctctcatctccccgactgaaattgctcttgtttgaaggcacgttactatcaaagatgttggtatcagaagacttcagactagagggttcagttgtaacagagcgaagtttatctaatacaccatgaagccaacataagctcctaattcttgtaatttccccttaatggcactccggatcttgcggctgatctcggtgccgatctccatggctctgcggcgtgcgggaactcagcactgcgcggcgcttggcttacccggaggctgccgcggactcctaccccgcagccgggacaccaccgcctcc

SEQ ID NO: 9884 - RNA, 4647 nt, Homo sapiens
  source 1..4647: mol_type = other RNA
caaagtgcttacagtgcaggtagaaactctgtaaccttaagcatgtaaactacatagaataaaactgtttccactgcatttctgtccttcaaagtggccaacctgattaagtcagccttaatcactgctgctgtcagtttcacgactaaaggtcatattgactaagtagtcatcagctgaccacctcgctgtatcagccagcaacgaggggaaggtgaagaaacatgataggccatatagaatctgccctatgtttacttttttaacccagataattatttttgtgtgcagtatctaagctcctgattgtgtaacctgggacttctggcaccttttgttccattcattttatgtataaaatgcatgccaaagcacactgtgccctctggtacccttgcttccaatcgccaaccatgctcatttccttcctttttttgtggtccctttttgtggtgatcattttaaaccacgtcatccaacaaatgttttatggtcaaccttagcttgttcataagccatagcaactgaaagattaaactcttaaatatgtgtctgggcagtggctattaaatagcaaaaaacaatcagattttagtattttattatttccttgtaaaatggctgaactaaattaaacccttgtttcccatttgttctataatttatagtgaaactgagaacaaaactatctttataaatgatagctaaaagtatttccagatatttaaacaatttaaaataaatttcttctgcagagatgcaaagcatctcaacactggaatgaacaaatgccttaaattcaatggagtaaacctttagaatgaagaggaactgtcatttcacccaagccgaagacaacagccttatgcacttgtgtgctctgtctttgctgcttctcgtgtttcaagcctttcctgtgggatcagcacagcaaagtgcaacttaccaaatggtttaatgactggttaattctttcttctcccaatggaaaagcaatggcaacacaacagtagactgctggcttgacaatcttaaacgtgagcctttgcacatgtaggtttatcatcatttgagtatacgactaagcaagtcaatgaactttttttttttttttagcagtttaatttggtcctgagaatgttgcagtctttattaccccttttgcattaatccacttttctaaccaccttttaagctttaatttttaacactatacaccaagtctttgaaatcagtgatctgttatttaactctaaagcatttgacacttcttgccttaacagttttaaaaaccacacacaaaaaaactctgtaagtaatacagtaggccaaaagtttcatcctatctatcttgcagtttacctatctgatctgatctctgtaattatagttctgtcatttaaaatatactatttaaatctaatttttacatttcaaaaattatcttcagtagtaactaagtatattttctgtggattctgagaatgttatttttcagaatgtgagaatatatatgtacatttataatcttgtgactttaaagtctgttttcagatacagtatgtaaatacttgtaaaaaaatttgtataattttgtgataatgtagtttcccaaaaaaattatttagaaggcattatgttattagtaaatgagagcactgtatagaactgttcctattttctgcacttgccattccagctgcctccactgtccatacccacctcattcatcctgtcacagaaggcaggaaaactgggaactttaccaaagtagcactcagcctgagaggcctgtataatcatgcttttcaaactaaattcacttaaaaattaaaaagcagaattgaatattttaagcagcctcagtacctttggccaatgctgttttcatggtggattatgaacattatataatctttgggaaaagtgaaagtagtacaatttttagaataatgacaactgcctcactgcatctctccactcacacagcaaccgtgtagccccctaagctgcagtaccatgactaaccatgatgtcaatttcatatgctgatcctcacaacagcagtgcacaaacatgccccaaatattttaacagaatttagctcttccttaagctgtcttttcatagtaaaaacaaaacaaaaacacccaatgttaaaaccacataataaacttacaaacttgaaaaattagacacttcagatagataggcaataaaacttcatattatgaaagcaatatattccaagtttcaaagatttgacaagttctgtagagtatctttcatcagtacatgaaaacttccaaactgcatgatcttctgccaggcaggactgggtgctattcgctggtttgaggtcgaatccatttcaaggcatgtcgtggtgggacattaatggtgggatggtagaatgtgcagtccggtcttgtacattgagtgttaaacctacaatgttttggatgatagaagggacattccatcttcttacaagcagggaagtaacggcagagctgactactggaaggtggtgctggtggtgcaactggttttggagacagtactggaattcttctactcacatgagtgaagggacaatctggtttagtacactttgcatcatatttacaatttgggtgaacaaacaaacatttttcagcaaatttacaattggggaaggctttgcagggtgagatggggtgatggtaggcacactcatccccatttttacaagcaggccagtacttgcagcgctccaaaagtttttctggtttctgtgccacactcagttcactcatctcagcgttagaaaagctaccatttgggtcctcaagctgcctgctcagcaagtgcaactgctgtgggtggaggagacctctgagtcccttgtttgaggctgcagtttggtttacgggtttcattccttcaaagcacatgtcctcctcttgatctgacatgtatcctggggggctggggacaccatccagcgtcactataaacttgggacttgcaggtttatctggttgtacaagatctcgtgtctgcataaggtgtcctgaaagtacccgaagggaatctgcagtcttcatccccgactcttggtttggtgccactactacttcctcagacagctttggcttcttcagaataaatgatcttgtgtctgcatggaccatggattccatgtcatagtaatcttgactcatctgcagagtttctgccattactgggtcgatttgcagtcgggataataattgcctctgttgagttccttgatttttttctacagaatctccttttgtttcctcttctttaatggggggacttattctgggggtcctactttgtccctggaccacttctgctagcaattcttcttgagaagttcgagttctgggagcaactggaagtgtctgtttctgtggaactgtagagtagttagttgtttttgttacggattcttgagcttcagatatagccttcaaaatcagattcttgttagcttgtttagaaggtggaagagaaggtctcctttcaggctttgcaggcacagacacactgctggagatgcttcctgttcgagacccgtaatcatcatcttcttcctcctcttctccatcatgattgaatttttttactttaacaactgaacttaccacaggcaactttctcttccgaaagttttcatcctccatactcattttctccgagttgtttctaaagaacggactatacgtttcttctaagctgttaagcacctctggttcacacaaacgtcctgtttcatatacccaactactctgcatatcaagctgcttggcagcatgaatactattctgctgctgttgaaattgcaacctgtttaaatgaacaccactatctgcatttctacttgcaggtggtcgataaatttcaatagaagggcgagaagaaccatatgtaagtgtcactgtaggttttttctgagataagggattctcctgcacaaagttgaggtcttcgtcaatgagatcatctggttctggcttaatatcaatcacatcttcagagggtgctggctccctcaaaggtttcactgttgacattagtcgggttgcagctccatcatcgtaagtctgtctgacatttgtggtttttgactcctgcgaacttgtagaaactctggaatctcttttttcaggtctcgcgctaggaatggcaagtggtggcactgcagcttcatgcctcctctcatctccccgactgaaattgctcttgtttgaaggcacgttactatcaaagatgttggtatcagaagacttcagactagagggttcagttgtaacagagcgaagtttatctaatacaccatgaagccatacggtgaatcgaattgtgttgttccctagaaacagggacagatcctctgtcatttggtcctgacttttcttgttggccaccatcaccataatgtaatcaggaagttcttcatcaacataagctcctaattcttgtaatttccccttaatggcactccggatcttgcggctgatctcggtgccgatctccatggctctgcggcgtgcgggaactcagcactgcgcggcgcttggcttacccggaggctgccgcggactcctaccccgcagccgggacaccaccgcctcc

SEQ ID NO: 9885 - RNA, 4623 nt, Homo sapiens
  source 1..4623: mol_type = other RNA
caaagtgcttacagtgcaggtagaaactctgtaaccttaagcatgtaaactacatagaataaaactgtttccactgcatttctgtccttcaaagtggccaacctgattaagtcagccttaatcactgctgctgtcagtttcacgactaaaggtcatattgactaagtagtcatcagctgaccacctcgctgtatcagccagcaacgaggggaaggtgaagaaacatgataggccatatagaatctgccctatgtttacttttttaacccagataattatttttgtgtgcagtatctaagctcctgattgtgtaacctgggacttctggcaccttttgttccattcattttatgtataaaatgcatgccaaagcacactgtgccctctggtacccttgcttccaatcgccaaccatgctcatttccttcctttttttgtggtccctttttgtggtgatcattttaaaccacgtcatccaacaaatgttttatggtcaaccttagcttgttcataagccatagcaactgaaagattaaactcttaaatatgtgtctgggcagtggctattaaatagcaaaaaacaatcagattttagtattttattatttccttgtaaaatggctgaactaaattaaacccttgtttcccatttgttctataatttatagtgaaactgagaacaaaactatctttataaatgatagctaaaagtatttccagatatttaaacaatttaaaataaatttcttctgcagagatgcaaagcatctcaacactggaatgaacaaatgccttaaattcaatggagtaaacctttagaatgaagaggaactgtcatttcacccaagccgaagacaacagccttatgcacttgtgtgctctgtctttgctgcttctcgtgtttcaagcctttcctgtgggatcagcacagcaaagtgcaacttaccaaatggtttaatgactggttaattctttcttctcccaatggaaaagcaatggcaacacaacagtagactgctggcttgacaatcttaaacgtgagcctttgcacatgtaggtttatcatcatttgagtatacgactaagcaagtcaatgaactttttttttttttttagcagtttaatttggtcctgagaatgttgcagtctttattaccccttttgcattaatccacttttctaaccaccttttaagctttaatttttaacactatacaccaagtctttgaaatcagtgatctgttatttaactctaaagcatttgacacttcttgccttaacagttttaaaaaccacacacaaaaaaactctgtaagtaatacagtaggccaaaagtttcatcctatctatcttgcagtttacctatctgatctgatctctgtaattatagttctgtcatttaaaatatactatttaaatctaatttttacatttcaaaaattatcttcagtagtaactaagtatattttctgtggattctgagaatgttatttttcagaatgtgagaatatatatgtacatttataatcttgtgactttaaagtctgttttcagatacagtatgtaaatacttgtaaaaaaatttgtataattttgtgataatgtagtttcccaaaaaaattatttagaaggcattatgttattagtaaatgagagcactgtatagaactgttcctattttctgcacttgccattccagctgcctccactgtccatacccacctcattcatcctgtcacagaaggcaggaaaactgggaactttaccaaagtagcactcagcctgagaggcctgtataatcatgcttttcaaactaaattcacttaaaaattaaaaagcagaattgaatattttaagcagcctcagtacctttggccaatgctgttttcatggtggattatgaacattatataatctttgggaaaagtgaaagtagtacaatttttagaataatgacaactgcctcactgcatctctccactcacacagcaaccgtgtagccccctaagctgcagtaccatgactaaccatgatgtcaatttcatatgctgatcctcacaacagcagtgcacaaacatgccccaaatattttaacagaatttagctcttccttaagctgtcttttcatagtaaaaacaaaacaaaaacacccaatgttaaaaccacataataaacttacaaacttgaaaaattagacacttcagatagataggcaataaaacttcatattatgaaagcaatatattccaagtttcaaagatttgacaagttctgtagagtatctttcatcagtacatgaaaacttccaaactgcatgatcttctgccaggcaggactgggtgctattcgctggtttgaggtcgaatccatttcaaggcatgtcgtggtgggacattaatggtgggatggtagaatgtgcagtccggtcttgtacattgagtgttaaacctacaatgttttggatgatagaagggacattccatcttcttacaagcagggaagtaacggcagagctgactactggaaggtggtgctggtggtgcaactggttttggagacagtactggaattcttctactcacatgagtgaagggacaatctggtttagtacactttgcatcatatttacaatttgggtgaacaaacaaacatttttcagcaaatttacaattggggaaggctttgcagggtgagatggggtgatggtaggcacactcatccccatttttacaagcaggccagtacttgcagcgctccaaaagtttttctggtttctgtgccacactcagttcactcatctcagcgttagaaaagctaccatttgggtcctcaagctgcctgctcagcaagtgcaactgctgtgggtggaggagacctctgagtcccttgtttgaggctgcagtttggtttacgggtttcattccttcaaagcacatgtcctcctcttgatctgacatgtatcctggggggctggggacaccatccagcgtcactataaacttgggacttgcaggtttatctggttgtacaagatctcgtgtctgcataaggtgtcctgaaagtacccgaagggaatctgcagtcttcatccccgactcttggtttggtgccactactacttcctcagacagctttggcttcttcagaataaatgatcttgtgtctgcatggaccatggattccatgtcatagtaatcttgactcatctgcagagtttctgccattactgggtcgatttgcagtcgggataataattgcctctgttgagttccttgatttttttctacagaatctccttttgtttcctcttctttaatggggggacttattctgggggtcctactttgtccctggaccacttctgctagcaattcttcttgagaagttcgagttctgggagcaactggaagtgtctgtttctgtggaactgtagagtagttagttgtttttgttacggattcttgagcttcagatatagccttcaaaatcagattcttgttagcttgtttagaaggtggaagagaaggtctcctttcaggctttgcaggcacagacacactgctggagatgcttcctgttcgagacccgtaatcatcatcttcttcctcctcttctccatcatgattgaatttttttactttaacaactgaacttaccacaggcaactttctcttccgaaagttttcatcctccatactcattttctccgagttgtttctaaagaacggactatacgtttcttctaagctgttaagcacctctggttcacacaaacgtcctgtttcatatacccaactactctgcatatcaagctgcttggcagcatgaatactattctgctgctgttgaaattgcaacctgtttaaatgaacaccactatctgcatttctacttgcaggtggtcgataaatttcaatagaagggcgagaagaaccatatgtaagtgtcactgtaggttttttctgagataagggattctcctgcacaaagttgaggtcttcgtcaatgagatcatctggttctggcttaatatcaatcacatcttcagagggtgctggctccctcaaaggtttcactgttgacattagtcgggttgcagctccatcatcgtaagtctgtctgacatttgtggtttttgactcctgcgaacttgtagaaactctggaatctcttttttcaggtctcgcgctaggaatggcaagtggtggcactgcagcttcatgcctcctctcatctccccgactgaaattgctcttgtttgaaggcacgttactatcaaagatgttggtatcagaagacttcagactagagggttcagttgtaacagagcgaagtttatctaatacaccatgaagccatacggtgaatcgaattgtgttgttccctagaaacagggacagatcctctgtcatttggtcctgacttttcttgttggccaccatcaccataatgtaatcaggaagttcttcatcaacataagctcctaattcttgtaatttccccttaatggcactctcccgcagcggatccaaagcggcgccgtgcgccgcggtggtggctccagccgggcctgcgcctgtccttccatttcccggcggctacttcagccgcagccacgctccg

SEQ ID NO: 9886 - RNA, 4828 nt, Homo sapiens
  source 1..4828: mol_type = other RNA
caaagtgcttacagtgcaggtagaaactctgtaaccttaagcatgtaaactacatagaataaaactgtttccactgcatttctgtccttcaaagtggccaacctgattaagtcagccttaatcactgctgctgtcagtttcacgactaaaggtcatattgactaagtagtcatcagctgaccacctcgctgtatcagccagcaacgaggggaaggtgaagaaacatgataggccatatagaatctgccctatgtttacttttttaacccagataattatttttgtgtgcagtatctaagctcctgattgtgtaacctgggacttctggcaccttttgttccattcattttatgtataaaatgcatgccaaagcacactgtgccctctggtacccttgcttccaatcgccaaccatgctcatttccttcctttttttgtggtccctttttgtggtgatcattttaaaccacgtcatccaacaaatgttttatggtcaaccttagcttgttcataagccatagcaactgaaagattaaactcttaaatatgtgtctgggcagtggctattaaatagcaaaaaacaatcagattttagtattttattatttccttgtaaaatggctgaactaaattaaacccttgtttcccatttgttctataatttatagtgaaactgagaacaaaactatctttataaatgatagctaaaagtatttccagatatttaaacaatttaaaataaatttcttctgcagagatgcaaagcatctcaacactggaatgaacaaatgccttaaattcaatggagtaaacctttagaatgaagaggaactgtcatttcacccaagccgaagacaacagccttatgcacttgtgtgctctgtctttgctgcttctcgtgtttcaagcctttcctgtgggatcagcacagcaaagtgcaacttaccaaatggtttaatgactggttaattctttcttctcccaatggaaaagcaatggcaacacaacagtagactgctggcttgacaatcttaaacgtgagcctttgcacatgtaggtttatcatcatttgagtatacgactaagcaagtcaatgaactttttttttttttttagcagtttaatttggtcctgagaatgttgcagtctttattaccccttttgcattaatccacttttctaaccaccttttaagctttaatttttaacactatacaccaagtctttgaaatcagtgatctgttatttaactctaaagcatttgacacttcttgccttaacagttttaaaaaccacacacaaaaaaactctgtaagtaatacagtaggccaaaagtttcatcctatctatcttgcagtttacctatctgatctgatctctgtaattatagttctgtcatttaaaatatactatttaaatctaatttttacatttcaaaaattatcttcagtagtaactaagtatattttctgtggattctgagaatgttatttttcagaatgtgagaatatatatgtacatttataatcttgtgactttaaagtctgttttcagatacagtatgtaaatacttgtaaaaaaatttgtataattttgtgataatgtagtttcccaaaaaaattatttagaaggcattatgttattagtaaatgagagcactgtatagaactgttcctattttctgcacttgccattccagctgcctccactgtccatacccacctcattcatcctgtcacagaaggcaggaaaactgggaactttaccaaagtagcactcagcctgagaggcctgtataatcatgcttttcaaactaaattcacttaaaaattaaaaagcagaattgaatattttaagcagcctcagtacctttggccaatgctgttttcatggtggattatgaacattatataatctttgggaaaagtgaaagtagtacaatttttagaataatgacaactgcctcactgcatctctccactcacacagcaaccgtgtagccccctaagctgcagtaccatgactaaccatgatgtcaatttcatatgctgatcctcacaacagcagtgcacaaacatgccccaaatattttaacagaatttagctcttccttaagctgtcttttcatagtaaaaacaaaacaaaaacacccaatgttaaaaccacataataaacttacaaacttgaaaaattagacacttcagatagataggcaataaaacttcatattatgaaagcaatatattccaagtttcaaagatttgacaagttctgtagagtatctttcatcagtacatgaaaacttccaaactgcatgatcttctgccaggcaggactgggtgctattcgctggtttgaggtcgaatccatttcaaggcatgtcgtggtgggacattaatggtgggatggtagaatgtgcagtccggtcttgtacattgagtgttaaacctacaatgttttggatgatagaagggacattccatcttcttacaagcagggaagtaacggcagagctgactactggaaggtggtgctggtggtgcaactggttttggagacagtactggaattcttctactcacatgagtgaagggacaatctggtttagtacactttgcatcatatttacaatttgggtgaacaaacaaacatttttcagcaaatttacaattggggaaggctttgcagggtgagatggggtgatggtaggcacactcatccccatttttacaagcaggccagtacttgcagcgctccaaaagtttttctggtttctgtgccacactcagttcactcatctcagcgttagaaaagctaccatttgggtcctcaagctgcctgctcagcaagtgcaactgctgtgggtggaggagacctctgagtcccttgtttgaggctgcagtttggtttacgggtttcattccttcaaagcacatgtcctcctcttgatctgacatgtatcctggggggctggggacaccatccagcgtcactataaacttgggacttgcaggtttatctggttgtacaagatctcgtgtctgcataaggtgtcctgaaagtacccgaagggaatctgcagtcttcatccccgactcttggtttggtgccactactacttcctcagacagctttggcttcttcagaataaatgatcttgtgtctgcatggaccatggattccatgtcatagtaatcttgactcatctgcagagtttctgccattactgggtcgatttgcagtcgggataataattgcctctgttgagttccttgatttttttctacagaatctccttttgtttcctcttctttaatggggggacttattctgggggtcctactttgtccctggaccacttctgctagcaattcttcttgagaagttcgagttctgggagcaactggaagtgtctgtttctgtggaactgtagagtagttagttgtttttgttacggattcttgagcttcagatatagccttcaaaatcagattcttgttagcttgtttagaaggtggaagagaaggtctcctttcaggctttgcaggcacagacacactgctggagatgcttcctgttcgagacccgtaatcatcatcttcttcctcctcttctccatcatgattgaatttttttactttaacaactgaacttaccacaggcaactttctcttccgaaagttttcatcctccatactcattttctccgagttgtttctaaagaacggactatacgtttcttctaagctgttaagcacctctggttcacacaaacgtcctgtttcatatacccaactactctgcatatcaagctgcttggcagcatgaatactattctgctgctgttgaaattgcaacctgtttaaatgaacaccactatctgcatttctacttgcaggtggtcgataaatttcaatagaagggcgagaagaaccatatgtaagtgtcactgtaggttttttctgagataagggattctcctgcacaaagttgaggtcttcgtcaatgagatcatctggttctggcttaatatcaatcacatcttcagagggtgctggctccctcaaaggtttcactgttgacattagtcgggttgcagctccatcatcgtaagtctgtctgacatttgtggtttttgactcctgcgaacttgtagaaactctggaatctcttttttcaggtctcgcgctaggaatggcaagtggtggcactgcagcttcatgcctcctctcatctccccgactgaaattgctcttgtttgaaggcacgttactatcaaagatgttggtatcagaagacttcagactagagggttcagttgtaacagagcgaagtttatctaatacaccatgaagccatacggtgaatcgaattgtgttgttccctagaaacagggacagatcctctgtcatttggtcctgacttttcttgttggccaccatcaccataatgtaatcaggaagttcttcatctatttaaaaggaaaggtagatcaaaactttgtttcctcaaaactttcttcttaaagttgatgtgcttgaaaatatagatgtagctctaagctttagagtcgcagagctctactggaattacattggacaagatggcttagctttaatttttttctcttcattccacaggtatttcaaatacaacataagctcctaattcttgtaatttccccttaatggcactccggatcttgcggctgatctcggtgccgatctccatggctctgcggcgtgcgggaactcagcactgcgcggcgcttggcttacccggaggctgccgcggactcctaccccgcagccgggacaccaccgcctcc

SEQ ID NO: 9887 - RNA, 4457 nt, Homo sapiens
  source 1..4457: mol_type = other RNA
caaagtgcttacagtgcaggtagaaactctgtaaccttaagcatgtaaactacatagaataaaactgtttccactgcatttctgtccttcaaagtggccaacctgattaagtcagccttaatcactgctgctgtcagtttcacgactaaaggtcatattgactaagtagtcatcagctgaccacctcgctgtatcagccagcaacgaggggaaggtgaagaaacatgataggccatatagaatctgccctatgtttacttttttaacccagataattatttttgtgtgcagtatctaagctcctgattgtgtaacctgggacttctggcaccttttgttccattcattttatgtataaaatgcatgccaaagcacactgtgccctctggtacccttgcttccaatcgccaaccatgctcatttccttcctttttttgtggtccctttttgtggtgatcattttaaaccacgtcatccaacaaatgttttatggtcaaccttagcttgttcataagccatagcaactgaaagattaaactcttaaatatgtgtctgggcagtggctattaaatagcaaaaaacaatcagattttagtattttattatttccttgtaaaatggctgaactaaattaaacccttgtttcccatttgttctataatttatagtgaaactgagaacaaaactatctttataaatgatagctaaaagtatttccagatatttaaacaatttaaaataaatttcttctgcagagatgcaaagcatctcaacactggaatgaacaaatgccttaaattcaatggagtaaacctttagaatgaagaggaactgtcatttcacccaagccgaagacaacagccttatgcacttgtgtgctctgtctttgctgcttctcgtgtttcaagcctttcctgtgggatcagcacagcaaagtgcaacttaccaaatggtttaatgactggttaattctttcttctcccaatggaaaagcaatggcaacacaacagtagactgctggcttgacaatcttaaacgtgagcctttgcacatgtaggtttatcatcatttgagtatacgactaagcaagtcaatgaactttttttttttttttagcagtttaatttggtcctgagaatgttgcagtctttattaccccttttgcattaatccacttttctaaccaccttttaagctttaatttttaacactatacaccaagtctttgaaatcagtgatctgttatttaactctaaagcatttgacacttcttgccttaacagttttaaaaaccacacacaaaaaaactctgtaagtaatacagtaggccaaaagtttcatcctatctatcttgcagtttacctatctgatctgatctctgtaattatagttctgtcatttaaaatatactatttaaatctaatttttacatttcaaaaattatcttcagtagtaactaagtatattttctgtggattctgagaatgttatttttcagaatgtgagaatatatatgtacatttataatcttgtgactttaaagtctgttttcagatacagtatgtaaatacttgtaaaaaaatttgtataattttgtgataatgtagtttcccaaaaaaattatttagaaggcattatgttattagtaaatgagagcactgtatagaactgttcctattttctgcacttgccattccagctgcctccactgtccatacccacctcattcatcctgtcacagaaggcaggaaaactgggaactttaccaaagtagcactcagcctgagaggcctgtataatcatgcttttcaaactaaattcacttaaaaattaaaaagcagaattgaatattttaagcagcctcagtacctttggccaatgctgttttcatggtggattatgaacattatataatctttgggaaaagtgaaagtagtacaatttttagaataatgacaactgcctcactgcatctctccactcacacagcaaccgtgtagccccctaagctgcagtaccatgactaaccatgatgtcaatttcatatgctgatcctcacaacagcagtgcacaaacatgccccaaatattttaacagaatttagctcttccttaagctgtcttttcatagtaaaaacaaaacaaaaacacccaatgttaaaaccacataataaacttacaaacttgaaaaattagacacttcagatagataggcaataaaacttcatattatgaaagcaatatattccaagtttcaaagatttgacaagttctgtagagtatctttcatcagtacatgaaaacttccaaactgcatgatcttctgccaggcaggactgggtgctattcgctggtttgaggtcgaatccatttcaaggcatgtcgtggtgggacattaatggtgggatggtagaatgtgcagtccggtcttgtacattgagtgttaaacctacaatgttttggatgatagaagggacattccatcttcttacaagcagggaagtaacggcagagctgactactggaaggtggtgctggtggtgcaactggttttggagacagtactggaattcttctactcacatgagtgaagggacaatctggtttagtacactttgcatcatatttacaatttgggtgaacaaacaaacatttttcagcaaatttacaattggggaaggctttgcagggtgagatggggtgatggtaggcacactcatccccatttttacaagcaggccagtacttgcagcgctccaaaagtttttctggtttctgtgccacactcagttcactcatctcagcgttagaaaagctaccatttgggtcctcaagctgcctgctcagcaagtgcaactgctgtgggtggaggagacctctgagtcccttgtttgaggctgcagtttggtttacgggtttcattccttcaaagcacatgtcctcctcttgatctgacatgtatcctggggggctggggacaccatccagcgtcactataaacttgggacttgcaggtttatctggttgtacaagatctcgtgtctgcataaggtgtcctgaaagtacccgaagggaatctgcagtcttcatccccgactcttggtttggtgccactactacttcctcagacagctttggcttcttcagaataaatgatcttgtgtctgcatggaccatggattccatgtcatagtaatcttgatttttttctacagaatctccttttgtttcctcttctttaatggggggacttattctgggggtcctactttgtccctggaccacttctgctagcaattcttcttgagaagttcgagttctgggagcaactggaagtgtctgtttctgtggaactgtagagtagttagttgtttttgttacggattcttgagcttcagatatagccttcaaaatcagattcttgttagcttgtttagaaggtggaagagaaggtctcctttcaggctttgcaggcacagacacactgctggagatgcttcctgttcgagacccgtaatcatcatcttcttcctcctcttctccatcatgattgaatttttttactttaacaactgaacttaccacaggcaactttctcttccgaaagttttcatcctccatactcattttctccgagttgtttctaaagaacggactatacgtttcttctaagctgttaagcacctctggttcacacaaacgtcctgtttcatatacccaactactctgcatatcaagctgcttggcagcatgaatactattctgctgctgttgaaattgcaacctgtttaaatgaacaccactatctgcatttctacttgcaggtggtcgataaatttcaatagaagggcgagaagaaccatatgtaagtgtcactgtaggttttttctgagataagggattctcctgcacaaagttgaggtcttcgtcaatgagatcatctggttctggcttaatatcaatcacatcttcagagggtgctggctccctcaaaggtttcactgttgacattagtcgggttgcagctccatcatcgtaagtctgtctgacatttgtggtttttgactcctgcgaacttgtagaaactctggaatctcttttttcaggtctcgcgctaggaatggcaagtggtggcactgcagcttcatgcctcctctcatctccccgactgaaattgctcttgtttgaaggcacgttactatcaaagatgttggtatcagaagacttcagactagagggttcagttgtaacagagcgaagtttatctaatacaccatgaagccaacataagctcctaattcttgtaatttccccttaatggcactccggatcttgcggctgatctcggtgccgatctccatggctctgcggcgtgcgggaactcagcactgcgcggcgcttggcttacccggaggctgccgcggactcctaccccgcagccgggacaccaccgcctcc

SEQ ID NO: 9888 - RNA, 4572 nt, Homo sapiens
  source 1..4572: mol_type = other RNA
caaagtgcttacagtgcaggtagaaactctgtaaccttaagcatgtaaactacatagaataaaactgtttccactgcatttctgtccttcaaagtggccaacctgattaagtcagccttaatcactgctgctgtcagtttcacgactaaaggtcatattgactaagtagtcatcagctgaccacctcgctgtatcagccagcaacgaggggaaggtgaagaaacatgataggccatatagaatctgccctatgtttacttttttaacccagataattatttttgtgtgcagtatctaagctcctgattgtgtaacctgggacttctggcaccttttgttccattcattttatgtataaaatgcatgccaaagcacactgtgccctctggtacccttgcttccaatcgccaaccatgctcatttccttcctttttttgtggtccctttttgtggtgatcattttaaaccacgtcatccaacaaatgttttatggtcaaccttagcttgttcataagccatagcaactgaaagattaaactcttaaatatgtgtctgggcagtggctattaaatagcaaaaaacaatcagattttagtattttattatttccttgtaaaatggctgaactaaattaaacccttgtttcccatttgttctataatttatagtgaaactgagaacaaaactatctttataaatgatagctaaaagtatttccagatatttaaacaatttaaaataaatttcttctgcagagatgcaaagcatctcaacactggaatgaacaaatgccttaaattcaatggagtaaacctttagaatgaagaggaactgtcatttcacccaagccgaagacaacagccttatgcacttgtgtgctctgtctttgctgcttctcgtgtttcaagcctttcctgtgggatcagcacagcaaagtgcaacttaccaaatggtttaatgactggttaattctttcttctcccaatggaaaagcaatggcaacacaacagtagactgctggcttgacaatcttaaacgtgagcctttgcacatgtaggtttatcatcatttgagtatacgactaagcaagtcaatgaactttttttttttttttagcagtttaatttggtcctgagaatgttgcagtctttattaccccttttgcattaatccacttttctaaccaccttttaagctttaatttttaacactatacaccaagtctttgaaatcagtgatctgttatttaactctaaagcatttgacacttcttgccttaacagttttaaaaaccacacacaaaaaaactctgtaagtaatacagtaggccaaaagtttcatcctatctatcttgcagtttacctatctgatctgatctctgtaattatagttctgtcatttaaaatatactatttaaatctaatttttacatttcaaaaattatcttcagtagtaactaagtatattttctgtggattctgagaatgttatttttcagaatgtgagaatatatatgtacatttataatcttgtgactttaaagtctgttttcagatacagtatgtaaatacttgtaaaaaaatttgtataattttgtgataatgtagtttcccaaaaaaattatttagaaggcattatgttattagtaaatgagagcactgtatagaactgttcctattttctgcacttgccattccagctgcctccactgtccatacccacctcattcatcctgtcacagaaggcaggaaaactgggaactttaccaaagtagcactcagcctgagaggcctgtataatcatgcttttcaaactaaattcacttaaaaattaaaaagcagaattgaatattttaagcagcctcagtacctttggccaatgctgttttcatggtggattatgaacattatataatctttgggaaaagtgaaagtagtacaatttttagaataatgacaactgcctcactgcatctctccactcacacagcaaccgtgtagccccctaagctgcagtaccatgactaaccatgatgtcaatttcatatgctgatcctcacaacagcagtgcacaaacatgccccaaatattttaacagaatttagctcttccttaagctgtcttttcatagtaaaaacaaaacaaaaacacccaatgttaaaaccacataataaacttacaaacttgaaaaattagacacttcagatagataggcaataaaacttcatattatgaaagcaatatattccaagtttcaaagatttgacaagttctgtagagtatctttcatcagtacatgaaaacttccaaactgcatgatcttctgccaggcaggactgggtgctattcgctggtttgaggtcgaatccatttcaaggcatgtcgtggtgggacattaatggtgggatggtagaatgtgcagtccggtcttgtacattgagtgttaaacctacaatgttttggatgatagaagggacattccatcttcttacaagcagggaagtaacggcagagctgactactggaaggtggtgctggtggtgcaactggttttggagacagtactggaattcttctactcacatgagtgaagggacaatctggtttagtacactttgcatcatatttacaatttgggtgaacaaacaaacatttttcagcaaatttacaattggggaaggctttgcagggtgagatggggtgatggtaggcacactcatccccatttttacaagcaggccagtacttgcagcgctccaaaagtttttctggtttctgtgccacactcagttcactcatctcagcgttagaaaagctaccatttgggtcctcaagctgcctgctcagcaagtgcaactgctgtgggtggaggagacctctgagtcccttgtttgaggctgcagtttggtttacgggtttcattccttcaaagcacatgtcctcctcttgatctgacatgtatcctggggggctggggacaccatccagcgtcactataaacttgggacttgcaggtttatctggttgtacaagatctcgtgtctgcataaggtgtcctgaaagtacccgaagggaatctgcagtcttcatccccgactcttggtttggtgccactactacttcctcagacagctttggcttcttcagaataaatgatcttgtgtctgcatggaccatggattccatgtcatagtaatcttgatttttttctacagaatctccttttgtttcctcttctttaatggggggacttattctgggggtcctactttgtccctggaccacttctgctagcaattcttcttgagaagttcgagttctgggagcaactggaagtgtctgtttctgtggaactgtagagtagttagttgtttttgttacggattcttgagcttcagatatagccttcaaaatcagattcttgttagcttgtttagaaggtggaagagaaggtctcctttcaggctttgcaggcacagacacactgctggagatgcttcctgttcgagacccgtaatcatcatcttcttcctcctcttctccatcatgattgaatttttttactttaacaactgaacttaccacaggcaactttctcttccgaaagttttcatcctccatactcattttctccgagttgtttctaaagaacggactatacgtttcttctaagctgttaagcacctctggttcacacaaacgtcctgtttcatatacccaactactctgcatatcaagctgcttggcagcatgaatactattctgctgctgttgaaattgcaacctgtttaaatgaacaccactatctgcatttctacttgcaggtggtcgataaatttcaatagaagggcgagaagaaccatatgtaagtgtcactgtaggttttttctgagataagggattctcctgcacaaagttgaggtcttcgtcaatgagatcatctggttctggcttaatatcaatcacatcttcagagggtgctggctccctcaaaggtttcactgttgacattagtcgggttgcagctccatcatcgtaagtctgtctgacatttgtggtttttgactcctgcgaacttgtagaaactctggaatctcttttttcaggtctcgcgctaggaatggcaagtggtggcactgcagcttcatgcctcctctcatctccccgactgaaattgctcttgtttgaaggcacgttactatcaaagatgttggtatcagaagacttcagactagagggttcagttgtaacagagcgaagtttatctaatacaccatgaagccatacggtgaatcgaattgtgttgttccctagaaacagggacagatcctctgtcatttggtcctgacttttcttgttggccaccatcaccataatgtaatcaggaagttcttcatcaacataagctcctaattcttgtaatttccccttaatggcactccggatcttgcggctgatctcggtgccgatctccatggctctgcggcgtgcgggaactcagcactgcgcggcgcttggcttacccggaggctgccgcggactcctaccccgcagccgggacaccaccgcctcc

SEQ ID NO: 9889 - RNA, 4023 nt, Homo sapiens
  source 1..4023: mol_type = other RNA
caaagtgcttacagtgcaggtagaaactctgtaaccttaagcatgtaaactacatagaataaaactgtttccactgcatttctgtccttcaaagtggccaacctgattaagtcagccttaatcactgctgctgtcagtttcacgactaaaggtcatattgactaagtagtcatcagctgaccacctcgctgtatcagccagcaacgaggggaaggtgaagaaacatgataggccatatagaatctgccctatgtttacttttttaacccagataattatttttgtgtgcagtatctaagctcctgattgtgtaacctgggacttctggcaccttttgttccattcattttatgtataaaatgcatgccaaagcacactgtgccctctggtacccttgcttccaatcgccaaccatgctcatttccttcctttttttgtggtccctttttgtggtgatcattttaaaccacgtcatccaacaaatgttttatggtcaaccttagcttgttcataagccatagcaactgaaagattaaactcttaaatatgtgtctgggcagtggctattaaatagcaaaaaacaatcagattttagtattttattatttccttgtaaaatggctgaactaaattaaacccttgtttcccatttgttctataatttatagtgaaactgagaacaaaactatctttataaatgatagctaaaagtatttccagatatttaaacaatttaaaataaatttcttctgcagagatgcaaagcatctcaacactggaatgaacaaatgccttaaattcaatggagtaaacctttagaatgaagaggaactgtcatttcacccaagccgaagacaacagccttatgcacttgtgtgctctgtctttgctgcttctcgtgtttcaagcctttcctgtgggatcagcacagcaaagtgcaacttaccaaatggtttaatgactggttaattctttcttctcccaatggaaaagcaatggcaacacaacagtagactgctggcttgacaatcttaaacgtgagcctttgcacatgtaggtttatcatcatttgagtatacgactaagcaagtcaatgaactttttttttttttttagcagtttaatttggtcctgagaatgttgcagtctttattaccccttttgcattaatccacttttctaaccaccttttaagctttaatttttaacactatacaccaagtctttgaaatcagtgatctgttatttaactctaaagcatttgacacttcttgccttaacagttttaaaaaccacacacaaaaaaactctgtaagtaatacagtaggccaaaagtttcatcctatctatcttgcagtttacctatctgatctgatctctgtaattatagttctgtcatttaaaatatactatttaaatctaatttttacatttcaaaaattatcttcagtagtaactaagtatattttctgtggattctgagaatgttatttttcagaatgtgagaatatatatgtacatttataatcttgtgactttaaagtctgttttcagatacagtatgtaaatacttgtaaaaaaatttgtataattttgtgataatgtagtttcccaaaaaaattatttagaaggcattatgttattagtaaatgagagcactgtatagaactgttcctattttctgcacttgccattccagctgcctccactgtccatacccacctcattcatcctgtcacagaaggcaggaaaactgggaactttaccaaagtagcactcagcctgagaggcctgtataatcatgcttttcaaactaaattcacttaaaaattaaaaagcagaattgaatattttaagcagcctcagtacctttggccaatgctgttttcatggtggattatgaacattatataatctttgggaaaagtgaaagtagtacaatttttagaataatgacaactgcctcactgcatctctccactcacacagcaaccgtgtagccccctaagctgcagtaccatgactaaccatgatgtcaatttcatatgctgatcctcacaacagcagtgcacaaacatgccccaaatattttaacagaatttagctcttccttaagctgtcttttcatagtaaaaacaaaacaaaaacacccaatgttaaaaccacataataaacttacaaacttgaaaaattagacacttcagatagataggcaataaaacttcatattatgaaagcaatatattccaagtttcaaagatttgacaagttctgtagagtatctttcatcagtacatgaaaacttccaaactgcatgatcttctgccaggcaggactgggtgctattcgctggtttgaggtcgaatccatttcaaggcatgtcgtggtgggacattaatggtgggatggtagaatgtgcagtccggtcttgtacattgagtgttaaacctacaatgttttggatgatagaagggacattccatcttcttacaagcagggaagtaacggcagagctgactactggaaggtggtgctggtggtgcaactggttttggagacagtactggaattcttctactcacatgagtgaagggacaatctggtttagtacactttgcatcatatttacaatttgggtgaacaaacaaacatttttcagcaaatttacaattggggaaggctttgcagggtgagatggggtgatggtaggcacactcatccccatttttacaagcaggccagtacttgcagcgctccaaaagtttttctggtttctgtgccacactcagttcactcatctcagctgtagagtagttagttgtttttgttacggattcttgagcttcagatatagccttcaaaatcagattcttgttagcttgtttagaaggtggaagagaaggtctcctttcaggctttgcaggcacagacacactgctggagatgcttcctgttcgagacccgtaatcatcatcttcttcctcctcttctccatcatgattgaatttttttactttaacaactgaacttaccacaggcaactttctcttccgaaagttttcatcctccatactcattttctccgagttgtttctaaagaacggactatacgtttcttctaagctgttaagcacctctggttcacacaaacgtcctgtttcatatacccaactactctgcatatcaagctgcttggcagcatgaatactattctgctgctgttgaaattgcaacctgtttaaatgaacaccactatctgcatttctacttgcaggtggtcgataaatttcaatagaagggcgagaagaaccatatgtaagtgtcactgtaggttttttctgagataagggattctcctgcacaaagttgaggtcttcgtcaatgagatcatctggttctggcttaatatcaatcacatcttcagagggtgctggctccctcaaaggtttcactgttgacattagtcgggttgcagctccatcatcgtaagtctgtctgacatttgtggtttttgactcctgcgaacttgtagaaactctggaatctcttttttcaggtctcgcgctaggaatggcaagtggtggcactgcagcttcatgcctcctctcatctccccgactgaaattgctcttgtttgaaggcacgttactatcaaagatgttggtatcagaagacttcagactagagggttcagttgtaacagagcgaagtttatctaatacaccatgaagccatacggtgaatcgaattgtgttgttccctagaaacagggacagatcctctgtcatttggtcctgacttttcttgttggccaccatcaccataatgtaatcaggaagttcttcatcaacataagctcctaattcttgtaatttccccttaatggcactccggatcttgcggctgatctcggtgccgatctccatggctctgcggcgtgcgggaactcagcactgcgcggcgcttggcttacccggaggctgccgcggactcctaccccgcagccgggacaccaccgcctcc

SEQ ID NO: 9890 - RNA, 4139 nt, Homo sapiens
  source 1..4139: mol_type = other RNA
caaagtgcttacagtgcaggtagaaactctgtaaccttaagcatgtaaactacatagaataaaactgtttccactgcatttctgtccttcaaagtggccaacctgattaagtcagccttaatcactgctgctgtcagtttcacgactaaaggtcatattgactaagtagtcatcagctgaccacctcgctgtatcagccagcaacgaggggaaggtgaagaaacatgataggccatatagaatctgccctatgtttacttttttaacccagataattatttttgtgtgcagtatctaagctcctgattgtgtaacctgggacttctggcaccttttgttccattcattttatgtataaaatgcatgccaaagcacactgtgccctctggtacccttgcttccaatcgccaaccatgctcatttccttcctttttttgtggtccctttttgtggtgatcattttaaaccacgtcatccaacaaatgttttatggtcaaccttagcttgttcataagccatagcaactgaaagattaaactcttaaatatgtgtctgggcagtggctattaaatagcaaaaaacaatcagattttagtattttattatttccttgtaaaatggctgaactaaattaaacccttgtttcccatttgttctataatttatagtgaaactgagaacaaaactatctttataaatgatagctaaaagtatttccagatatttaaacaatttaaaataaatttcttctgcagagatgcaaagcatctcaacactggaatgaacaaatgccttaaattcaatggagtaaacctttagaatgaagaggaactgtcatttcacccaagccgaagacaacagccttatgcacttgtgtgctctgtctttgctgcttctcgtgtttcaagcctttcctgtgggatcagcacagcaaagtgcaacttaccaaatggtttaatgactggttaattctttcttctcccaatggaaaagcaatggcaacacaacagtagactgctggcttgacaatcttaaacgtgagcctttgcacatgtaggtttatcatcatttgagtatacgactaagcaagtcaatgaactttttttttttttttagcagtttaatttggtcctgagaatgttgcagtctttattaccccttttgcattaatccacttttctaaccaccttttaagctttaatttttaacactatacaccaagtctttgaaatcagtgatctgttatttaactctaaagcatttgacacttcttgccttaacagttttaaaaaccacacacaaaaaaactctgtaagtaatacagtaggccaaaagtttcatcctatctatcttgcagtttacctatctgatctgatctctgtaattatagttctgtcatttaaaatatactatttaaatctaatttttacatttcaaaaattatcttcagtagtaactaagtatattttctgtggattctgagaatgttatttttcagaatgtgagaatatatatgtacatttataatcttgtgactttaaagtctgttttcagatacagtatgtaaatacttgtaaaaaaatttgtataattttgtgataatgtagtttcccaaaaaaattatttagaaggcattatgttattagtaaatgagagcactgtatagaactgttcctattttctgcacttgccattccagctgcctccactgtccatacccacctcattcatcctgtcacagaaggcaggaaaactgggaactttaccaaagtagcactcagcctgagaggcctgtataatcatgcttttcaaactaaattcacttaaaaattaaaaagcagaattgaatattttaagcagcctcagtacctttggccaatgctgttttcatggtggattatgaacattatataatctttgggaaaagtgaaagtagtacaatttttagaataatgacaactgcctcactgcatctctccactcacacagcaaccgtgtagccccctaagctgcagtaccatgactaaccatgatgtcaatttcatatgctgatcctcacaacagcagtgcacaaacatgccccaaatattttaacagaatttagctcttccttaagctgtcttttcatagtaaaaacaaaacaaaaacacccaatgttaaaaccacataataaacttacaaacttgaaaaattagacacttcagatagataggcaataaaacttcatattatgaaagcaatatattccaagtttcaaagatttgacaagttctgtagagtatctttcatcagtacatgaaaacttccaaactgcatgatcttctgccaggcaggactgggtgctattcgctggtttgaggtcgaatccatttcaaggcatgtcgtggtgggacattaatggtgggatggtagaatgtgcagtccggtcttgtacattgagtgttaaacctacaatgttttggatgatagaagggacattccatcttcttacaagcagggaagtaacggcagagctgactactggaaggtggtgctggtggtgcaactggttttggagacagtactggaattcttctactcacatgagtgaagggacaatctggtttagtacactttgcatcatatttacaatttgggtgaacaaacaaacatttttcagcaaatttacaattggggaaggctttgcagggtgagatggggtgatggtaggcacactcatccccatttttacaagcaggccagtacttgcagcgctccaaaagtttttctggtttctgtgccacactcagttcactcatctcagcttgactcatctgcagagtttctgccattactgggtcgatttgcagtcgggataataattgcctctgttgagttccttgatttttttctacagaatctccttttgtttcctcttctttaatggggggacttattctgggggtcctactttgtccctggaccacttctgctagcaattcttcttgagaagttcgagttctgggagcaactggaagtgtctgtttctgtggaactgtagagtagttagttgtttttgttacggattcttgagcttcagatatagccttcaaaatcagattcttgttagcttgtttagaaggtggaagagaaggtctcctttcaggctttgcaggcacagacacactgctggagatgcttcctgttcgagacccgtaatcatcatcttcttcctcctcttctccatcatgattgaatttttttactttaacaactgaacttaccacaggcaactttctcttccgaaagttttcatcctccatactcattttctccgagttgtttctaaagaacggactatacgtttcttctaagctgttaagcacctctggttcacacaaacgtcctgtttcatatacccaactactctgcatatcaagctgcttggcagcatgaatactattctgctgctgttgaaattgcaacctgtttaaatgaacaccactatctgcatttctacttgcaggtggtcgataaatttcaatagaagggcgagaagaaccatatgtaagtgtcactgtaggttttttctgagataagggattctcctgcacaaagttgaggtcttcgtcaatgagatcatctggttctggcttaatatcaatcacatcttcagagggtgctggctccctcaaaggtttcactgttgacattagtcgggttgcagctccatcatcgtaagtctgtctgacatttgtggtttttgactcctgcgaacttgtagaaactctggaatctcttttttcaggtctcgcgctaggaatggcaagtggtggcactgcagcttcatgcctcctctcatctccccgactgaaattgctcttgtttgaaggcacgttactatcaaagatgttggtatcagaagacttcagactagagggttcagttgtaacagagcgaagtttatctaatacaccatgaagccaacataagctcctaattcttgtaatttccccttaatggcactccggatcttgcggctgatctcggtgccgatctccatggctctgcggcgtgcgggaactcagcactgcgcggcgcttggcttacccggaggctgccgcggactcctaccccgcagccgggacaccaccgcctcc

SEQ ID NO: 9891 - RNA, 3570 nt, Homo sapiens
  source 1..3570: mol_type = other RNA
caaagtgcttacagtgcaggtagaaactctgtaaccttaagcatgtaaactacatagaataaaactgtttccactgcatttctgtccttcaaagtggccaacctgattaagtcagccttaatcactgctgctgtcagtttcacgactaaaggtcatattgactaagtagtcatcagctgaccacctcgctgtatcagccagcaacgaggggaaggtgaagaaacatgataggccatatagaatctgccctatgtttacttttttaacccagataattatttttgtgtgcagtatctaagctcctgattgtgtaacctgggacttctggcaccttttgttccattcattttatgtataaaatgcatgccaaagcacactgtgccctctggtacccttgcttccaatcgccaaccatgctcatttccttcctttttttgtggtccctttttgtggtgatcattttaaaccacgtcatccaacaaatgttttatggtcaaccttagcttgttcataagccatagcaactgaaagattaaactcttaaatatgtgtctgggcagtggctattaaatagcaaaaaacaatcagattttagtattttattatttccttgtaaaatggctgaactaaattaaacccttgtttcccatttgttctataatttatagtgaaactgagaacaaaactatctttataaatgatagctaaaagtatttccagatatttaaacaatttaaaataaatttcttctgcagagatgcaaagcatctcaacactggaatgaacaaatgccttaaattcaatggagtaaacctttagaatgaagaggaactgtcatttcacccaagccgaagacaacagccttatgcacttgtgtgctctgtctttgctgcttctcgtgtttcaagcctttcctgtgggatcagcacagcaaagtgcaacttaccaaatggtttaatgactggttaattctttcttctcccaatggaaaagcaatggcaacacaacagtagactgctggcttgacaatcttaaacgtgagcctttgcacatgtaggtttatcatcatttgagtatacgactaagcaagtcaatgaactttttttttttttttagcagtttaatttggtcctgagaatgttgcagtctttattaccccttttgcattaatccacttttctaaccaccttttaagctttaatttttaacactatacaccaagtctttgaaatcagtgatctgttatttaactctaaagcatttgacacttcttgccttaacagttttaaaaaccacacacaaaaaaactctgtaagtaatacagtaggccaaaagtttcatcctatctatcttgcagtttacctatctgatctgatctctgtaattatagttctgtcatttaaaatatactatttaaatctaatttttacatttcaaaaattatcttcagtagtaactaagtatattttctgtggattctgagaatgttatttttcagaatgtgagaatatatatgtacatttataatcttgtgactttaaagtctgttttcagatacagtatgtaaatacttgtaaaaaaatttgtataattttgtgataatgtagtttcccaaaaaaattatttagaaggcattatgttattagtaaatgagagcactgtatagaactgttcctattttctgcacttgccattccagctgcctccactgtccatacccacctcattcatcctgtcacagaaggcaggaaaactgggaactttaccaaagtagcactcagcctgagaggcctgtataatcatgcttttcaaactaaattcacttaaaaattaaaaagcagaattgaatattttaagcagcctcagtacctttggccaatgctgttttcatggtggattatgaacattatataatctttgggaaaagtgaaagtagtacaatttttagaataatgacaactgcctcactgcatctctccactcacacagcaaccgtgtagccccctaagctgcagtaccatgactaaccatgatgtcaatttcatatgctgatcctcacaacagcagtgcacaaacatgccccaaatattttaacagaatttagctcttccttaagctgtcttttcatagtaaaaacaaaacaaaaacacccaatgttaaaaccacataataaacttacaaacttgaaaaattagacacttcagatagataggcaataaaacttcatattatgaaagcaatatattccaagtttcaaagatttgacaagttctgtagagtatctttcatcagtacatgaaaacttccaaactgcatgatcttctgccaggcaggactgggtgctattcgctggtttgaggtcgaatccatttcaaggcatgtcgtggtgggacattaatggtgggatggtagaatgtgcagtccggtcttgtacattgagtgttaaacctacaatgttttggatgatagaagggacattccatcttcttacaagcagggaagtaacggcagagctgactactggaaggtggtgctggtggtgcaactggttttggagacagtactggaattcttctactcacatgagtgaagggacaatctggtttagtacactttgcatcatatttacaatttgggtgaacaaacaaacatttttcagcaaatttacaattggggaaggctttgcagggtgagatggggtgatggtaggcacactcatccccatttttacaagcaggccagtacttgcagcgctccaaaagtttttctggtttctgtgccacactcagttcactcatctcagcttgactcatctgcagagtttctgccattactgggtcgatttgcagtcgggataataattgcctctgttgagttcctttctcaacgtttctaaggaagccgattatttttacatcagtagttcttgactgtgattcagtatcttcttcttgatcttcaaactgtctgttgcattcatatgttgttgaatattcattcattttaacctccaaagatgaaatttttgcttcattcttggacactctaacatttagatcaaaaagatttgcttccactgtcaaaatagctgctttcattcctttaatttcattgatatcagctgatattttccttaaaaggtgggaaatattgtctagctcattcagtgaacaagaggagcttgttatggaacctaagtccactggctccggtggaagaaaaattggtagaggtggtgatggaaactttgaagacattctcataaaggtgacaggaacctcaaagacattttcataaaattctctcccttaaaatctgataattttttcttcacagctcattaagttatttcatcgaaagtaaaagcagtgatcaaggctgttaccttaagacgtattaagagcaaataacatcttaaaacctgtaattcaaaagatggggttgtacatttctagagtcagaattcaaaactaaatgtgaaaaagctaaacgtaccagaccaattgctcttcgctacaactaagaagccctaatacgtagggccctacatcctctaagtaccatctgtat

SEQ ID NO: 9892 - RNA, 4064 nt, Homo sapiens
  source 1..4064: mol_type = other RNA
caaagtgcttacagtgcaggtagaaactctgtaaccttaagcatgtaaactacatagaataaaactgtttccactgcatttctgtccttcaaagtggccaacctgattaagtcagccttaatcactgctgctgtcagtttcacgactaaaggtcatattgactaagtagtcatcagctgaccacctcgctgtatcagccagcaacgaggggaaggtgaagaaacatgataggccatatagaatctgccctatgtttacttttttaacccagataattatttttgtgtgcagtatctaagctcctgattgtgtaacctgggacttctggcaccttttgttccattcattttatgtataaaatgcatgccaaagcacactgtgccctctggtacccttgcttccaatcgccaaccatgctcatttccttcctttttttgtggtccctttttgtggtgatcattttaaaccacgtcatccaacaaatgttttatggtcaaccttagcttgttcataagccatagcaactgaaagattaaactcttaaatatgtgtctgggcagtggctattaaatagcaaaaaacaatcagattttagtattttattatttccttgtaaaatggctgaactaaattaaacccttgtttcccatttgttctataatttatagtgaaactgagaacaaaactatctttataaatgatagctaaaagtatttccagatatttaaacaatttaaaataaatttcttctgcagagatgcaaagcatctcaacactggaatgaacaaatgccttaaattcaatggagtaaacctttagaatgaagaggaactgtcatttcacccaagccgaagacaacagccttatgcacttgtgtgctctgtctttgctgcttctcgtgtttcaagcctttcctgtgggatcagcacagcaaagtgcaacttaccaaatggtttaatgactggttaattctttcttctcccaatggaaaagcaatggcaacacaacagtagactgctggcttgacaatcttaaacgtgagcctttgcacatgtaggtttatcatcatttgagtatacgactaagcaagtcaatgaactttttttttttttttagcagtttaatttggtcctgagaatgttgcagtctttattaccccttttgcattaatccacttttctaaccaccttttaagctttaatttttaacactatacaccaagtctttgaaatcagtgatctgttatttaactctaaagcatttgacacttcttgccttaacagttttaaaaaccacacacaaaaaaactctgtaagtaatacagtaggccaaaagtttcatcctatctatcttgcagtttacctatctgatctgatctctgtaattatagttctgtcatttaaaatatactatttaaatctaatttttacatttcaaaaattatcttcagtagtaactaagtatattttctgtggattctgagaatgttatttttcagaatgtgagaatatatatgtacatttataatcttgtgactttaaagtctgttttcagatacagtatgtaaatacttgtaaaaaaatttgtataattttgtgataatgtagtttcccaaaaaaattatttagaaggcattatgttattagtaaatgagagcactgtatagaactgttcctattttctgcacttgccattccagctgcctccactgtccatacccacctcattcatcctgtcacagaaggcaggaaaactgggaactttaccaaagtagcactcagcctgagaggcctgtataatcatgcttttcaaactaaattcacttaaaaattaaaaagcagaattgaatattttaagcagcctcagtacctttggccaatgctgttttcatggtggattatgaacattatataatctttgggaaaagtgaaagtagtacaatttttagaataatgacaactgcctcactgcatctctccactcacacagcaaccgtgtagccccctaagctgcagtaccatgactaaccatgatgtcaatttcatatgctgatcctcacaacagcagtgcacaaacatgccccaaatattttaacagaatttagctcttccttaagctgtcttttcatagtaaaaacaaaacaaaaacacccaatgttaaaaccacataataaacttacaaacttgaaaaattagacacttcagatagataggcaataaaacttcatattatgaaagcaatatattccaagtttcaaagatttgacaagttctgtagagtatctttcatcagtacatgaaaacttccaaactgcatgatcttctgccaggcaggactgggtgctattcgctggtttgaggtcgaatccatttcaaggcatgtcgtggtgggacattaatggtgggatggtagaatgtgcagtccggtcttgtacattgagtgttaaacctacaatgttttggatgatagaagggacattccatcttcttacaagcagggaagtaacggcagagctgactactggaaggtggtgctggtggtgcaactggttttggagacagtactggaattcttctactcacatgagtgaagggacaatctggtttagtacactttgcatcatatttacaatttgggtgaacaaacaaacatttttcagcaaatttacaattggggaaggctttgcagggtgagatggggtgatggtaggcacactcatccccatttttacaagcaggccagtacttgcagcgctccaaaagtttttctggtttctgtgccacactcagttcactcatctcagcttgatttttttctacagaatctccttttgtttcctcttctttaatggggggacttattctgggggtcctactttgtccctggaccacttctgctagcaattcttcttgagaagttcgagttctgggagcaactggaagtgtctgtttctgtggaactgtagagtagttagttgtttttgttacggattcttgagcttcagatatagccttcaaaatcagattcttgttagcttgtttagaaggtggaagagaaggtctcctttcaggctttgcaggcacagacacactgctggagatgcttcctgttcgagacccgtaatcatcatcttcttcctcctcttctccatcatgattgaatttttttactttaacaactgaacttaccacaggcaactttctcttccgaaagttttcatcctccatactcattttctccgagttgtttctaaagaacggactatacgtttcttctaagctgttaagcacctctggttcacacaaacgtcctgtttcatatacccaactactctgcatatcaagctgcttggcagcatgaatactattctgctgctgttgaaattgcaacctgtttaaatgaacaccactatctgcatttctacttgcaggtggtcgataaatttcaatagaagggcgagaagaaccatatgtaagtgtcactgtaggttttttctgagataagggattctcctgcacaaagttgaggtcttcgtcaatgagatcatctggttctggcttaatatcaatcacatcttcagagggtgctggctccctcaaaggtttcactgttgacattagtcgggttgcagctccatcatcgtaagtctgtctgacatttgtggtttttgactcctgcgaacttgtagaaactctggaatctcttttttcaggtctcgcgctaggaatggcaagtggtggcactgcagcttcatgcctcctctcatctccccgactgaaattgctcttgtttgaaggcacgttactatcaaagatgttggtatcagaagacttcagactagagggttcagttgtaacagagcgaagtttatctaatacaccatgaagccaacataagctcctaattcttgtaatttccccttaatggcactccggatcttgcggctgatctcggtgccgatctccatggctctgcggcgtgcgggaactcagcactgcgcggcgcttggcttacccggaggctgccgcggactcctaccccgcagccgggacaccaccgcctcc

SEQ ID NO: 9893 - RNA, 4179 nt, Homo sapiens
  source 1..4179: mol_type = other RNA
caaagtgcttacagtgcaggtagaaactctgtaaccttaagcatgtaaactacatagaataaaactgtttccactgcatttctgtccttcaaagtggccaacctgattaagtcagccttaatcactgctgctgtcagtttcacgactaaaggtcatattgactaagtagtcatcagctgaccacctcgctgtatcagccagcaacgaggggaaggtgaagaaacatgataggccatatagaatctgccctatgtttacttttttaacccagataattatttttgtgtgcagtatctaagctcctgattgtgtaacctgggacttctggcaccttttgttccattcattttatgtataaaatgcatgccaaagcacactgtgccctctggtacccttgcttccaatcgccaaccatgctcatttccttcctttttttgtggtccctttttgtggtgatcattttaaaccacgtcatccaacaaatgttttatggtcaaccttagcttgttcataagccatagcaactgaaagattaaactcttaaatatgtgtctgggcagtggctattaaatagcaaaaaacaatcagattttagtattttattatttccttgtaaaatggctgaactaaattaaacccttgtttcccatttgttctataatttatagtgaaactgagaacaaaactatctttataaatgatagctaaaagtatttccagatatttaaacaatttaaaataaatttcttctgcagagatgcaaagcatctcaacactggaatgaacaaatgccttaaattcaatggagtaaacctttagaatgaagaggaactgtcatttcacccaagccgaagacaacagccttatgcacttgtgtgctctgtctttgctgcttctcgtgtttcaagcctttcctgtgggatcagcacagcaaagtgcaacttaccaaatggtttaatgactggttaattctttcttctcccaatggaaaagcaatggcaacacaacagtagactgctggcttgacaatcttaaacgtgagcctttgcacatgtaggtttatcatcatttgagtatacgactaagcaagtcaatgaactttttttttttttttagcagtttaatttggtcctgagaatgttgcagtctttattaccccttttgcattaatccacttttctaaccaccttttaagctttaatttttaacactatacaccaagtctttgaaatcagtgatctgttatttaactctaaagcatttgacacttcttgccttaacagttttaaaaaccacacacaaaaaaactctgtaagtaatacagtaggccaaaagtttcatcctatctatcttgcagtttacctatctgatctgatctctgtaattatagttctgtcatttaaaatatactatttaaatctaatttttacatttcaaaaattatcttcagtagtaactaagtatattttctgtggattctgagaatgttatttttcagaatgtgagaatatatatgtacatttataatcttgtgactttaaagtctgttttcagatacagtatgtaaatacttgtaaaaaaatttgtataattttgtgataatgtagtttcccaaaaaaattatttagaaggcattatgttattagtaaatgagagcactgtatagaactgttcctattttctgcacttgccattccagctgcctccactgtccatacccacctcattcatcctgtcacagaaggcaggaaaactgggaactttaccaaagtagcactcagcctgagaggcctgtataatcatgcttttcaaactaaattcacttaaaaattaaaaagcagaattgaatattttaagcagcctcagtacctttggccaatgctgttttcatggtggattatgaacattatataatctttgggaaaagtgaaagtagtacaatttttagaataatgacaactgcctcactgcatctctccactcacacagcaaccgtgtagccccctaagctgcagtaccatgactaaccatgatgtcaatttcatatgctgatcctcacaacagcagtgcacaaacatgccccaaatattttaacagaatttagctcttccttaagctgtcttttcatagtaaaaacaaaacaaaaacacccaatgttaaaaccacataataaacttacaaacttgaaaaattagacacttcagatagataggcaataaaacttcatattatgaaagcaatatattccaagtttcaaagatttgacaagttctgtagagtatctttcatcagtacatgaaaacttccaaactgcatgatcttctgccaggcaggactgggtgctattcgctggtttgaggtcgaatccatttcaaggcatgtcgtggtgggacattaatggtgggatggtagaatgtgcagtccggtcttgtacattgagtgttaaacctacaatgttttggatgatagaagggacattccatcttcttacaagcagggaagtaacggcagagctgactactggaaggtggtgctggtggtgcaactggttttggagacagtactggaattcttctactcacatgagtgaagggacaatctggtttagtacactttgcatcatatttacaatttgggtgaacaaacaaacatttttcagcaaatttacaattggggaaggctttgcagggtgagatggggtgatggtaggcacactcatccccatttttacaagcaggccagtacttgcagcgctccaaaagtttttctggtttctgtgccacactcagttcactcatctcagcttgatttttttctacagaatctccttttgtttcctcttctttaatggggggacttattctgggggtcctactttgtccctggaccacttctgctagcaattcttcttgagaagttcgagttctgggagcaactggaagtgtctgtttctgtggaactgtagagtagttagttgtttttgttacggattcttgagcttcagatatagccttcaaaatcagattcttgttagcttgtttagaaggtggaagagaaggtctcctttcaggctttgcaggcacagacacactgctggagatgcttcctgttcgagacccgtaatcatcatcttcttcctcctcttctccatcatgattgaatttttttactttaacaactgaacttaccacaggcaactttctcttccgaaagttttcatcctccatactcattttctccgagttgtttctaaagaacggactatacgtttcttctaagctgttaagcacctctggttcacacaaacgtcctgtttcatatacccaactactctgcatatcaagctgcttggcagcatgaatactattctgctgctgttgaaattgcaacctgtttaaatgaacaccactatctgcatttctacttgcaggtggtcgataaatttcaatagaagggcgagaagaaccatatgtaagtgtcactgtaggttttttctgagataagggattctcctgcacaaagttgaggtcttcgtcaatgagatcatctggttctggcttaatatcaatcacatcttcagagggtgctggctccctcaaaggtttcactgttgacattagtcgggttgcagctccatcatcgtaagtctgtctgacatttgtggtttttgactcctgcgaacttgtagaaactctggaatctcttttttcaggtctcgcgctaggaatggcaagtggtggcactgcagcttcatgcctcctctcatctccccgactgaaattgctcttgtttgaaggcacgttactatcaaagatgttggtatcagaagacttcagactagagggttcagttgtaacagagcgaagtttatctaatacaccatgaagccatacggtgaatcgaattgtgttgttccctagaaacagggacagatcctctgtcatttggtcctgacttttcttgttggccaccatcaccataatgtaatcaggaagttcttcatcaacataagctcctaattcttgtaatttccccttaatggcactccggatcttgcggctgatctcggtgccgatctccatggctctgcggcgtgcgggaactcagcactgcgcggcgcttggcttacccggaggctgccgcggactcctaccccgcagccgggacaccaccgcctcc

SEQ ID NO: 9894 - RNA, 4360 nt, Homo sapiens
  source 1..4360: mol_type = other RNA
caaagtgcttacagtgcaggtagaaactctgtaaccttaagcatgtaaactacatagaataaaactgtttccactgcatttctgtccttcaaagtggccaacctgattaagtcagccttaatcactgctgctgtcagtttcacgactaaaggtcatattgactaagtagtcatcagctgaccacctcgctgtatcagccagcaacgaggggaaggtgaagaaacatgataggccatatagaatctgccctatgtttacttttttaacccagataattatttttgtgtgcagtatctaagctcctgattgtgtaacctgggacttctggcaccttttgttccattcattttatgtataaaatgcatgccaaagcacactgtgccctctggtacccttgcttccaatcgccaaccatgctcatttccttcctttttttgtggtccctttttgtggtgatcattttaaaccacgtcatccaacaaatgttttatggtcaaccttagcttgttcataagccatagcaactgaaagattaaactcttaaatatgtgtctgggcagtggctattaaatagcaaaaaacaatcagattttagtattttattatttccttgtaaaatggctgaactaaattaaacccttgtttcccatttgttctataatttatagtgaaactgagaacaaaactatctttataaatgatagctaaaagtatttccagatatttaaacaatttaaaataaatttcttctgcagagatgcaaagcatctcaacactggaatgaacaaatgccttaaattcaatggagtaaacctttagaatgaagaggaactgtcatttcacccaagccgaagacaacagccttatgcacttgtgtgctctgtctttgctgcttctcgtgtttcaagcctttcctgtgggatcagcacagcaaagtgcaacttaccaaatggtttaatgactggttaattctttcttctcccaatggaaaagcaatggcaacacaacagtagactgctggcttgacaatcttaaacgtgagcctttgcacatgtaggtttatcatcatttgagtatacgactaagcaagtcaatgaactttttttttttttttagcagtttaatttggtcctgagaatgttgcagtctttattaccccttttgcattaatccacttttctaaccaccttttaagctttaatttttaacactatacaccaagtctttgaaatcagtgatctgttatttaactctaaagcatttgacacttcttgccttaacagttttaaaaaccacacacaaaaaaactctgtaagtaatacagtaggccaaaagtttcatcctatctatcttgcagtttacctatctgatctgatctctgtaattatagttctgtcatttaaaatatactatttaaatctaatttttacatttcaaaaattatcttcagtagtaactaagtatattttctgtggattctgagaatgttatttttcagaatgtgagaatatatatgtacatttataatcttgtgactttaaagtctgttttcagatacagtatgtaaatacttgtaaaaaaatttgtataattttgtgataatgtagtttcccaaaaaaattatttagaaggcattatgttattagtaaatgagagcactgtatagaactgttcctattttctgcacttgccattccagctgcctccactgtccatacccacctcattcatcctgtcacagaaggcaggaaaactgggaactttaccaaagtagcactcagcctgagaggcctgtataatcatgcttttcaaactaaattcacttaaaaattaaaaagcagaattgaatattttaagcagcctcagtacctttggccaatgctgttttcatggtggattatgaacattatataatctttgggaaaagtgaaagtagtacaatttttagaataatgacaactgcctcactgcatctctccactcacacagcaaccgtgtagccccctaagctgcagtaccatgactaaccatgatgtcaatttcatatgctgatcctcacaacagcagtgcacaaacatgccccaaatattttaacagaatttagctcttccttaagctgtcttttcatagtaaaaacaaaacaaaaacacccaatgttaaaaccacataataaacttacaaacttgaaaaattagacacttcagatagataggcaataaaacttcatattatgaaagcaatatattccaagtttcaaagatttgacaagttctgtagagtatctttcatcagtacatgaaaacttccaaactgcatgatcttctgccaggcaggactgggtgctattcgctggtttgaggtcgaatccatttcaaggcatgtcgtggtgggacattaatggtgggatggtagaatgtgcagtccggtcttgtacattgagtgttaaacctacaatgttttggatgatagaagggacattccatcttcttacaagcagggaagtaacggcagagctgactactggaaggtggtgctggtggtgcaactggttttggagacagtactggaattcttctactcacatgagtgaagggacaatctggtttagtacactttgcatcatatttacaatttgggtgaacaaacaaacatttttcagcaaatttacaattggggaaggctttgcagggtgagatggggtgatggtaggcacactcatccccatttttacaagcaggccagtacttgcagcgctccaaaagtttttctggtttctgtgccacactcagttcactcatctcagcttgatttttttctacagaatctccttttgtttcctcttctttaatggggggacttattctgggggtcctactttgtccctggaccacttctgctagcaattcttcttgagaagttcgagttctgggagcaactggaagtgtctgtttctgtggaactgtagagtagttagttgtttttgttacggattcttgagcttcagatatagccttcaaaatcagattcttgttagcttgtttagaaggtggaagagaaggtctcctttcaggctttgcaggcacagacacactgctggagatgcttcctgttcgagacccgtaatcatcatcttcttcctcctcttctccatcatgattgaatttttttactttaacaactgaacttaccacaggcaactttctcttccgaaagttttcatcctccatactcattttctccgagttgtttctaaagaacggactatacgtttcttctaagctgttaagcacctctggttcacacaaacgtcctgtttcatatacccaactactctgcatatcaagctgcttggcagcatgaatactattctgctgctgttgaaattgcaacctgtttaaatgaacaccactatctgcatttctacttgcaggtggtcgataaatttcaatagaagggcgagaagaaccatatgtaagtgtcactgtaggttttttctgagataagggattctcctgcacaaagttgaggtcttcgtcaatgagatcatctggttctggcttaatatcaatcacatcttcagagggtgctggctccctcaaaggtttcactgttgacattagtcgggttgcagctccatcatcgtaagtctgtctgacatttgtggtttttgactcctgcgaacttgtagaaactctggaatctcttttttcaggtctcgcgctaggaatggcaagtggtggcactgcagcttcatgcctcctctcatctccccgactgaaattgctcttgtttgaaggcacgttactatcaaagatgttggtatcagaagacttcagactagagggttcagttgtaacagagcgaagtttatctaatacaccatgaagccatacggtgaatcgaattgtgttgttccctagaaacagggacagatcctctgtcatttggtcctgacttttcttgttggccaccatcaccataatgtaatcaggaagttcttcatctatttaaaaggaaaggtagatcaaaactttgtttcctcaaaactttcttcttaaagttgatgtgcttgaaaatatagatgtagctctaagctttagagtcgcagagctctactggaattacattggacaagatggcttagctttaatttttttctcttcattccacaggtatttcaaatacaacataagctcctaattcttgtaatttccccttaatggcactccggatcttgcggctgatctcggtgccgatctccatggctctgcggcgtgcgggaactcagcactgcgcggcgcttggcttacccggaggctgccgcggactcctaccccgcagccgggacaccaccgcctcc

SEQ ID NO: 9895 - RNA, 410 nt, Homo sapiens
  source 1..410: mol_type = other RNA
caaagtttaagatccttgaagtaaggagctaggtcttccttggtttttgtgcattcactctgaagtattggcttgaacccaggcatcttccactctggaaaagaagagcaggaacccgagacccccagcccttggttaaaatcagccctgctggaaacagctttgttgagtccatgagaaggtggagctgagacaagtggctgcgtgagcccagctgctgtggaggaatccgctcagaggagatggggctgagatcatgcatgccaccaagtgccagcgctgctggagggcagatgtgggtcagtctcacctcctgagcaacatagccacctcctctgctgtcttctcctctttatttattcattcattcaaatcagagatggggtctctctctgatgcccagactagcc

SEQ ID NO: 9896 - RNA, 7480 nt, Homo sapiens
  source 1..7480: mol_type = other RNA
caaatgagcttaatttccttttaattccttccaattactatgcactgttctttgtgccaagtgccagtccagttatccagttggtgcattttgtgagaactgtaggatcatggagatcatgtttcttttcttttcttttcttttctttttttgagacagcgtcttgctctgtcaccaggctggagtgcagtggcacaatcttggcttaccgcaacctctgcttcctgggttcaagtgattcttctgcctcagcctcccaagtagctgggattacaggcacgcaccaccatgcctggctaattttttgtagttttagtagagatggggtttcgccatgttggccaggctggtcgcgaactcccgacctcaggtgatccgcctgcctcagatcacccaaagtgctgggattacaggcatgagccactgtgcctggccaggatcatgtttctttaaaccacacatgatacccagaaggcatcataatagagttggcttcatcatcttccttatcctaggttatgcttgatttcaaaagaaatttgttcctcgacaatacacagaaaatgcacttaacaatagcccctgaagttttccccagccaatgactggttagcagtctaataaggatcatattggacaagtatctttaacacaaaacagcacagggaatcatgggccactctcatcgttaggctctcttcacaggtatagcctatgttagaaggcttctgaaccacagatgctaaagaaaaattagttaaactgaagactgatgaagtattccctacaaatgaaaaggcaatcttatatgacaaaggacactatcaggaggttgaaaaacaacctatagaatgggagaaaatatttgtaaatcatatgtctatgattaatatccagaatatataaagaactcctgtaagtcaacaaccatcaccacacccagttcacaaatgggcagaggaatcttatggacatttctccagcggagatatatgcacagccaaggagcacgtgaaaagatactcagcatcattagttgctagagaaatgcaaagcaaaccccaagaaggtaccacttcctagccagcaggatgtagctattaaaacaacaacagaaaatcagtgttggcaagggtgtggaggaattgcagtccgtgtgcgttgctggtgggaatgtaaaatggcatagtcattgtggaaaggagtgtggcagttcctccaagagtcgcatatagaattgtcacatggtccagcaattccattcctaggttacccaaaagaatggaaagcaggggagctggaggccattatgctaagtgaagtaactcaggaagggaaagccacattcctatgttctcaggtataagtgggagctaagctgagggtccacaaaggcagagtggaggaatggacattggagactccgaaggggaaaggagatggaggattaaaacgctacattttgggtacaacatatactacttcggtgacaggtgcaccacaatctcagacctcaccactatacagttcatccacgtaaccaaaaaccacttggacccctaaagctattaaataaaataaataaatataaacattcagtaacattatctttagaagaacactttttaataaacctgggcatgaagaaaaaaggctgaataatattccatcgtatgcgtgtgtatatccatatatatatatatatatatatatatatatatatatgcacacacacacacaatgtatatgtctagtgttaccaacttagtttcctttccttcaatattaaacgtctcatatttcccccagactttttgagagatagttgagaaataaagctgtgtaagtttagagtgtagtatgtgatgatttgatatatattgtgaaattattaacacaagttaggtgacacacctgtcacctgtcctagttatcatttttttttgtattgtagtgaaataaatgtctcatttaaaaaaaaaagaattgaaagcaggaaatgaaacagatacttgtataccaatgctcatagtagcattaagcataatagccaagaggtaggaacaacccaattgttcatccacaaatgaggagagaaaatgtggtatgtaaatataatggaatatacgtttcatggaaaagaatgtatctttcaatttttaatttttgtgggtacatagtaggtgaatatatctatgggatccatgagatgttgggatacagacatgcaatgtgaaataagcacgtcatggagaatggggtatccatcccctcaagcatttatcctttgagttacaaacaattcaattacactcttttaggtacttaaaaacgtacaattaagttgttatagtcaccctgttgtactttcaaatactagatcttattctttcaaaaattggttgaacctattaaccatccccacatcccccatactctcccaatacctttcccagcctctggtaaccatccttctactctctatgcccatgagttcaattgctttgatttttaggtctcacaaacaagtgagaacatgtgatgtttgtctttctgttcctggcttatttcacaaaatgatctccatttccatccatgatgttgcaaacaacaggatctcattcttttccatggctgaatagtactccattgtgtatatataccacattttctttatccattcacctgttgatggacatttaggttgcttccaaatctaatggaatatattattcactcataaaaagtgtgaaattctgatacatgctgttaatataacacggatgtaccttgcaagcatgttgagtaacataagccacaccccaaaggacaaatattgtatgattccacttatacaaggtacctggcacaggcaaattcatagagacacaaagtagaatggtggttaccgggggccgggggagtagggagtggggagttgttacttaatgggtagagtttgtttgtttgggaaggttctggagataaaggatgtgatggttgcacaacaatgtgaacgggcgcaatgccactaaactgtgcgcttagttgcaaggttacaataggacattttatgtatatttcaccacaataaaaataggaaaaggcaggtgatttctaaggacacaagtcccttggggttgctagttctgtcagacttttccccttgtttttctgaatgacaaggattagtagtggatgataatgagtggattcatggatttgagcaggacatgaaacaatttccatagacagagatgaaagggcatttctgacttgaaacctgggatgagcaccgatgcaggagaggcacgaaagctcacagcgtgttcagggcgtagtgaatagaggggtgcgtgccccgagcctgcagagcgggcagggatgtgtaggaaggcaccttcatcctcctcactcagcctcccagctccaggtccaaagccgccaaatcatctttcttgtcaccatcacatgataagggggagtccttccagactgccagtcaatgaagtaacacacacagccacggtcatgccagtctgagcccatcgggcgagccctgaggggaataacagtcttggtggcattgggcaagccccgaggactccatctcggggaataacagtcttggtggcatcggcgcttcaccaggcctcctggaaccatattcgggatccccaactgagtgctggaaagaccactggtcaggagcagggagcaggggtggaaggaggtggctcgtcctgaccttgacaatgagaatcctgttttaagcttcacgctgctgactaaacagaaaggccacggcacagggacagacgtgcgcatgaaatcacaggaagaaagacatttcacgaacaaatgcatcctcccaaaccagtctgaatccctccggacagggtgatgttaccacgcaactggcctggcctaatgagctggtttctgtcatccctcctggaaggttaccctgtaacacaaggcgtgcccactgacatgcagcctgatggagcaaggttacacctgtctgccttttgtgtgcacaagatcagaacacagtcaagtgaatacaaatgcaacagctgcttggggctcaaacttgcatagtctattttatttggatagagagcataaaattggctctaccaaagtctggaggctggaagtaatcataattgtaatctagtataattaccaagcctagacctttacctagtcctatttaacctccctttcacctttccaaggaatgtggagggataagagagtcactgaataagttggttggtaatactgtattgtatctctcaaatccattgtttttttttaaagaatgagatcaataaatataaattccaatattttcttccccaaagcaccatcttgtaccgctttggagaacattagagggactcacctgggtttccagagctggaaaacataagccccataatgcacccagtccccacggcgcgctgccatcttaggcccagtccccactgcacgctgtcatcttaggcccagtccccgctgggcgctgccatcttaggcccagtccccgctgcgcgctgccatcttaggcccagtccccgctgcgcgctgccatattaggcccagtccccgctgcgcgctgccatcttaggcccagtccccgctgcgcgctgccatcttgggcccagtccccgaggcccagtccccgctgggcgctgccatcttaggcccagtccccgctgggcgctgccatcttaggcccagtccccgctgcgcgctgccatcttaggcccagtccccgctgcgcgctgccatcttaggcccagtccccgctgcgcgctgccatcttaggcccagtccccgctgcgcgctgccatcttaggcccagtccccgctgcgcgctgccatcttagggttttgcttagggggcagatagaaaatagtaaatgaaaccctttcagatatttcctggccttatttagtaaacacgtctttttgaaagaactctgaatacacctgcagatttttcaaagcccagattctacacacttctaatgtcaaccttgaagggagatcgtagattgaattacagaaaggggtgctgtcaaaatgccacatcaaatataaacttcacatatgtttcttacctgaaacactcactcacactcatggaaaagcacaggaatgttctaaaaatgcaagtttatcacgaaggagacacaggaggttcagagacgatgaagcggcaagccgggaggaaagatctgagagaagccaccaggctggggcaggatttcattatatccagaattccacttgggctctgcagtttctttcttcctgagaattatttaaaagtcccctccactgcgcatattgaagacagagcccaagacgcatccaggtgcaacgtctctgctaagaatgtgtgccaggaatggggcctggcttcctcgtcgagtgcggctgtccgtgggtttcccacagtcttccctccctgaggccagaagcaggtcacgtgtaaaatggtctgctctctgctgacagtggcctgagtctcccatagtgtctgctgagctggatagtccctctccagggagctttgcaggggatgggtgatgagacatggacatggggacgaattcctctcatctggaatcgcagacacagcatggagatatgagcacgcggcatgggaaataggcttcctcagcccttcaggatcagggaacgtgccagagatgcaatgacatttggcagcagttgagagtatgagtgctcagcagcagcatctgcagactcgtgtggggacttctgtctggactcagggatgttaagagtagaaggcccaatgtcagcttctcacgtgggctgtcagcaccgcagatgataccggaagatggactgtgatgggccagcgacccctctgactgcacgcagctgtcagccaggcctggaacaggaggggcgagggggtgggctcagcctctgttagtgggagaggtcctggttggaagtttcactgaagtatcagtgttgactttctcaggtcaaatctgggccatttcatgcggtaaatccatgtcggcaggtatcagcccaagtgttttgaacatgctgcacttgtacatgcctggaccaaatgccaggctgatgagcagggaggggttgaaaagcagaagggagcccaacccaccggcgtcagcaggaggctggccctggctgtggctccccgatcagacaggcggcgtccaatggggcaccacacgactcccgccagggtggggcttcccctgtacctttcttagagctgatggtcccctgaccccactcgcagcctggaaggaggggatccctggcagagaccgggcttggcagaaaactgggcatctgcttgagaggtggaaatgctggagcatgcagaaaatctaagaacccttatttatatggggccccagaccaggaccctcgggtcagtctttctttgcccagggatggcatagcagtaacatcgcttcctgtgccctttccagtaatgtgagggcaccatctccgcccctgaactcccttcaggccacttcactccatttcctcagcctgaccacattacccctgccccagtacttggcttccctcaccatcacctaagtgaagctcacatgcacctctggagggagacaggcgcggggagagggagcctcagctggaggtgcaggaactgagtatcaatccattcacgggattgaggttctggtacccaaattcagaattttacgaaaatccaagacacttgttcattcgtgtgcaggaaaaaggtattcctagcccccaaaccacacctaacctgacagtgggcactcacttcaccttgagagggatcgatgtggtgaggaagttcaaggttgctagatggcatggaaaggaggcaatgggaaggaagtagatacccgccaggatatttctgtgaagctgttgtagcccagtgaaatgtcactctccaggtgtttttaccttctctactcccagctcacacggtgccctggcacgggtattggcaggactctccaggtgtttttaccttctctactcccagctcacacggtgccctggcacgggtattggcaggactctccaggcgtttttaccttctctactcccagctcacacggtgccctggcacgggtattggcaggactctccaggtgtttttctctactcccatctcacacggtgccctggcacgggtattggcaggagatggagggtggctcttatccaagacattttcccatctgatcatatcccatccgcggtagccaggctccaagatggcccccatggtctctgcctcctggtgttcacacccttgtgtagtcccctcccgtatttaccagagttggtctaggtgctcctgtggtgtgggctgggtgtgagcagaagggccctttctcctctctgtctgtgtgctaggaggccatgtgcttcaatgcaa

SEQ ID NO: 9897 - RNA, 730 nt, Homo sapiens
  source 1..730: mol_type = other RNA
caaatgagcttaatttccttttcagcttggagttttcttgaatggcgcagatttcattagtgcttaaaggctttctgcaatcgctgcgggcaatttctacatcaataaggtattccagaagatttgtgacctgaagctgggcttgcagtgtcttgaccaccaggaagacatacttgtcctcgctctctttgttgtattcttgcatggcaaaccacagacactgcttcacgttggcatttgaggcattgacgggttttaatttcctcagcacccctgtctcattcttttttgggtctttcctggccaccagggccaggggaatggtgaggaggatcagggagagccaccggcacctgggcatggtcccttgggcaagaggcaaagtcgactctcctcctcgtcgtctcagggctggagctgtgggcaggatggggtggccgcagctgctgctgtgggttcaagaatcttcgagccacacactgcctcctgttagcgtcagcccagccctgtgagcgtcactcttgttatctgcttctcagtcctgtatgatgtgatcatgaaaactgtggctgccccagaggccttgtggcctcagcccttggtggactttcagcctgctgtgcctgcagctccttcttactccctgtggagctgggagctgacctgaccagtggttctcctaggtcttcagcactcttagttcatgcctgtggcccagtcaagggtctct

SEQ ID NO: 9898 - RNA, 770 nt, Homo sapiens
  source 1..770: mol_type = other RNA
caaatgagcttaatttccttttcagcttggagttttcttgaatggcgcagatttcattagtgcttaaaggctttctgcaatcgctgcgggcaatttctacatcaataaggtattccagaagatttgtgacctgaagctgggcttgcagtgtcttgaccaccaggaagacatacttgtcctcgctctctttgttgtattcttgcatggcaaaccacagacactgcttcacgttggcatttgaggcattgacgggttttaatttcctcagcacccctgtctcattcttttttgggtctttcctggccaccagggccaggggaatggtgaggaggatcagggagagccaccggcacctgggcatggtcccttgggcaagaggcaaagtcgactctcctcctcgtcgtctcagggctggagctgtgggcaggatggggtggccgcagctgctgctgtgggttcaagaatcttcgagccacacactgcctcctgttagcgtcagcccagccctgtgagcgtcactcttgttatctgcttctcagtcctgtatgatgtgatcatgaaaactgtggctgccccagaggccttgtggcctcagcccttggtggactttcagcctgctgtgcctgcagctccttcttactccctgtggagctgggagctgacctgaccagtggttctcctaggtcttcagcactcttagttcatgcctgtggcccagtcaagggtctctgtgggtcctggtctgcggtctctcttgcccctctgagtcc

SEQ ID NO: 9899 - RNA, 837 nt, Homo sapiens
  source 1..837: mol_type = other RNA
caaatgagcttaatttccttttcagcttggagttttcttgaatggcgcagatttcattagtgcttaaaggctttctgcaatcgctgcgggcaatttctacatcaataaggtattccagaagatttgtgacctgaagctgggcttgcagtgtcttgaccaccaggaagacatacttgtcctcgctctctttgttgtattcttgcatggcaaaccacagacactgcttcacgttggcatttgaggcattgacgggttttaatttcctcagcacccctgtctcattcttttttgggtctttcctggccaccagggccaggggaatggtgaggaggatcagggagagccaccggcacctgggcatggtcccttgggcaagaggcaaagtcgactctcctcctcgtcgtctcagggctggagctgtgggcaggatggggtggccgcagctgctgctgtgggttcaagaatcttcgagccacacactgcctcctgttagcgtcagcccagcctgagagcaatctgtgtgtctagggagagttcctctccccttcggccccagtgtgtctatgcctacccctgtgagcgtcactcttgttatctgcttctcagtcctgtatgatgtgatcatgaaaactgtggctgccccagaggccttgtggcctcagcccttggtggactttcagcctgctgtgcctgcagctccttcttactccctgtggagctgggagctgacctgaccagtggttctcctaggtcttcagcactcttagttcatgcctgtggcccagtcaagggtctctgtgggtcctggtctgcggtctctcttgcccctctgagtcc

SEQ ID NO: 9900 - RNA, 571 nt, Homo sapiens
  source 1..571: mol_type = other RNA
caaatgagcttaatttccttttcagcttggagttttcttgaatggcgcagatttcattagtgcttaaaggctttctgcaatcgctgcgggcaatttctacatcaataaggtattccagaagatttgtgacctgaagctgggcttgcagtgtcttgaccaccaggaagacatacttgtcctcgctctctttgttgtattcttgcatggcaaaccacagacactgcttcacgttggcatttgaggcattgacgggttttaatttcctcagcacccctgtctcattcttttttgggtctttcctggccaccagggccaggggaatggtgaggaggatcagggagagccaccggcacctgggcatggtcccttgggcaagaggcaaagtcgactctcctcctcgtcgtctcagggctggagctgtgggcaggatggggtggccgcagctgctgctgtgggttcaagaatcttcgagccacacactgcctcctgttagcgtcagcccagctgaccagtggttctcctaggtcttcagcactcttagttcatgcctgtggcccagtcaagggtctct

SEQ ID NO: 9901 - RNA, 607 nt, Homo sapiens
  source 1..607: mol_type = other RNA
caaatgagcttaatttccttttcagcttggagttttcttgaatggcgcagatttcattagtgcttaaaggctttctgcaatcgctgcgggcaatttctacatcaataaggtattccagaagatttgtgacctgaagctgggcttgcagtgtcttgaccaccaggaagacatacttgtcctcgctctctttgttgtattcttgcatggcaaaccacagacactgcttcacgttggcatttgaggcattgacgggttttaatttcctcagcacccctgtctcattcttttttgggtctttcctggccaccagggccaggggaatggtgaggaggatcagggagagccaccggcacctgggcatggtcccttgggcaagaggcaaagtcgactctcctcctcgtcgtctcagggctggagctgtgggcaggatggggtggccgcagctgctgctgtgggttcaagaatcttcgagccacacactgcctcctgttagcgtcagcccagctgaccagtggttctcctaggtcttcagcactcttagttcatgcctgtggcccagtcaagggtctctgtgggtcctggtctgcggtctctcttgcccctctga

SEQ ID NO: 9902 - RNA, 29 nt, Homo sapiens
  source 1..29: mol_type = other RNA
caacaaatcccagtctacctaatggtgcc

SEQ ID NO: 9903 - RNA, 4666 nt, Homo sapiens
  source 1..4666: mol_type = other RNA
caaccaccactgtctctccccagaaggccttcaaggttaacacacaacaatgccctgccccttgattactggcctgggcttacaaaggcgaatactcagacagaatcaggaggcactcagcttaatgaaggggcagggatctgcagccagcagattgcctggcctatattcctctccctcggactctttctgaattgtctttagggtgtggtttgctgcccagtgacaacatacattcctttatatcctggaatgttacatagtctctcttagtgtctggcatacagttctacagtagttctagcatttacatcacttcagaacttactaataacataaggacaggagaagcagcaacgtaacaggatgtgcccaatctctcagaagcttctctacaagcactacatccagaccagctttccgtaagttccgaaacctggcctggcaagacctgcctgatgttccgccaggtaaggagcctcctcagtgcagaggacagtggctctcaactgtaatcccagcgctttgggaggcagaggcaggaggattgcttgacgccagggattggagagcagcctgggcagcacagtgggaacccatctcatgtccctgcacaagatgctcacccactccaccttcccatcctggagctgcacaaattgtccctttcttgaagttgatgcaatgtgtctctgtgttagatatgagctcccaactgggcccaaggacttggggtgatggaggctgcaggctcttgccaaagccaggtttaaatccctgtttctattttaccagcagggaagaaatgagagtcgagttgagaaaatgctcagttaagacagtcagtcacgggacagctgtatcctcaggaccagcctgtcatcgataagtccaagccctggctactgctgctggagaggcaaaggaacaatcttgcctttcagcgccgtcggaaagctcgagatattctccaggcattgggttcctcatagcggttgtacaagggttcaagacgctgttgcttcttctgtttgcttagcttagttgggtctgagaccttgaagaaggctggggcaaactccacaagccaccgagggtcgatggtggtaacttcacgcatgtattccttggtggtgagcaccagctcatggtacaccacccattctggctgtctgttgaagagggcactggaaggatggatatagaccacctgctggtcgatcagtgtccggtaaccctcctgcgggtctttcttggcagcattacggaagaacccactgcagatggccttctgcactcggactgtggacttgccacaggaaacaacatccagcttgtgtctgtccattatgcctaacatctgcttgcgaatgtcctgggcccggcgcagggaacgagcctggataaagttctcatagcaccatgggttggagaacttgttgttcttccaggagttgtacacagctagcagggtgaggtggtccccttcagtctggtggaatttggccttcttctgatctgcaagggcttgtttatccttgggcctatagaagacgttctgcacagacagcatggatacaatggtcagcatttcctcactgcagcccagatgcacagacatgatgagcattttgcatagcattggctccagagggaactctgccatccggcggcccaagcgagtgagcaggccctcgtcatccagggcccccagtgtgtacagctgctccatggctgtgatcaaagtttccataggtggggcatccatgaaatcaaaggacagcagatcattgatacccatggccttgagtgacagcactgtgcttgctaagttggttctctggatttccggcacgttggtggtcagcatttcatctcggtaggcacgttctgtgtacaacctgtaacacttccctgggcctgttctcccagctctgccagctcgttgctttgcctgagcctgagaaataggcgtcaccacgagctggtcaatccctgtcttggaattgtaaactttctgtttcacgaatcctgggtccaccacatagtagataccatcaatagtcagcgatgtctctgcgatattggtggcaatcacaacctttctgctgcctggtggagctgggtcaaagattcgggtctgcatctcactgggaagagcagagtacactgggaggataattaactctggaacatcaggtcccagggatttcattctttcatacaggatctcacaagcagtatcaatttcttcctgaccagtcaggaagaccaggatatcacctggtggttctgttaaatgaatctgcataacagtaatcaggctggcatccagataatctgtctcaggttcctttgtgtacagtatttccactggatatgttcgacctgggatggtgaaaatgggagcttcatagaagtattgagaaaacttcactgcatccaaggtggctgaggtgacaatcagcttcatgtcctgccgtttctgaactgtctttttcaacaatccaaagagcacatcagtgtgaattgtcctctcatgtgcctcgtccaacatgatgatcgcgtactgagtgaggtcagggtcaatcaagcactctctaagcaacatcccatctgtcatgtacttgatgactgtttcagggctagtgcagtcctcaaatcgaatggtgtagcccacctcttggcctaagcaacaaccaaactcctctgacactcttttggccaccgacatagctgccactcttctgggctgggtacacccaatcttgcccctggaagtgtagcctgcctccgccaggtactgggtgatctgtgttgtctttccagatcctgtctcaccaatgacaatcaggatctgattgtcatggacggcctggaccaattgctccttcagtttgtagatgggcaggctctccctctgctcaaggattgacatctgggtcttttttccgtaagaggctttgttgcccccaaaggcatgcttcttccactcaggaatatcattgggcatcatcccaatacccctcatgttggcagcaatctgtctgccttccgcatcaggcagagggtcaacccagtgtttgttgagtcccatgggaatagaatccatctcagcttcccgctgggcctgtttgagttcccgcctttctttggccaaggcactctgcatcattgctgcttgggagagggagccgtctgggttcttgacaattttaatggggctcatgtccatgctttgcttagtgtgccctctcaggaatggaggctcttcctcaaccaattcaatctcaaggtcctcatcttcttcatcatccaccttagggagaatgccagtctcttcatcaaagtctggaaattcttctttggaaaggacattggcagcaatcatctgtttgatctcccacttctctgggtcagagattcgggtgaggcgcttgcgttccagtgagtcgtcctctacttcaggagcactgacaagggacaagtgagtgggtctatcaggattccgcattgaggtctcctcattggtctccccgacaagatttcgccgtctatttgggtttagatcttctccagtctcttgatccacatccttcatgctcaggctggtcttggtcccagtgaaggacagcactttgactttgaccctctggcctttgctcacgacatcagctacattggccacacgaccctcccgccggagctcagagatgtgcaccaggccttcccaccgcttccttagtccttccagctgcacaaagcaaccaaactgcatgatgctggtaactttgccattataaatgtcaccaatggtgggctcttctggaggagggcggtccacatgcttatcccgccatctatccagattccgctctccatatttgtcccggtccttccggtctttggggggactctgactcctgctcctggaccgatatctagacttcactttattcctctcccgggtcctggaacgtgatcgagagcgggatcggtgtctccgcttgtggtctctatctcggtttcgttccctatctctgtctcgatctcggtttcgatctcggcttcgactccgcttcttcttctttgtcctgtcccggtgttcagcatctctttgcttctcctggcctgctgcgctgggcattaaagcttccagttctttcaggacatccacagcaactttcacatcatcttcatccaacatggtccgaacagaagggttgtccggttggcaaaggactgggaagagttccttcagcttttctttttctgttttaggtttaacaactggatctttgctagtggaaggcttcgctggaggccgcatggtttgtatgagacgcagcaagttactaataagagaatccgtaaattctgcaccatttttgacgagagaagccttaaaagtatcaaaggtggtatttttctcagcaagactgatcacaaattcagcaaggtccttgtcgttgatccccaagtgattgtccagctcagtgcaaacctttgacaccaaagacaggtactcgagtttggcaagttcttccgcggggcctggctccgacccgattaaggctcccgccatggctacagccacagccatggctatagcttgcccagaacctccttcctcacagccggcgctcagagctactccggccgggtt

SEQ ID NO: 9904 - RNA, 5709 nt, Homo sapiens
  source 1..5709: mol_type = other RNA
caaccaccactgtctctccccagaaggccttcaaggttaacacacaacaatgccctgccccttgattactggcctgggcttacaaaggcgaatactcagacagaatcaggaggcactcagcttaatgaaggggcagggatctgcagccagcagattgcctggcctatattcctctccctcggactctttctgaattgtctttagggtgtggtttgctgcccagtgacaacatacattcctttatatcctggaatgttacatagtctctcttagtgtctggcatacagttctacagtagttctagcatttacatcacttcagaacttactaataacataaggacaggagaagcagcaacgtaacaggatgtgcccaatctctcagaagcttctctacaagcactacatccagaccagctttccgtaagttccgaaacctggcctggcaagacctgcctgatgttccgccaggtaaggagcctcctcagtgcagaggacagtggctctcaactgtaatcccagcgctttgggaggcagaggcaggaggattgcttgacgccagggattggagagcagcctgggcagcacagtgggaacccatctctatgggaagaaaaaaaaaaaaccctcctcaggagctgtgaggagggcacaaggaggtggctattctccaagcaagtgctaggaaaaaaccactaagaacaagccctgcagcacagatactggcagcacaaaccagctgagaggagaggtgttatgtttgttttctgtttggagtggggaaagggaggttttgaccataaaatccctttgttaaagtccatccaggacctcaggggaaaaaaataaaaacaaaataaaataaaagctgtgttgttacttagtatgtttcaaaaggaaatgggacatgctgcacattgcgaatgtgggaggtggagggagcaaggggaaaccttctgtatttaatatgtgccatctgtagccactcaggcctccagactgaagtgctctgtggagaggacatggttgatcatcgggtgatcccccagcacggcccggctagtgctgatgctgaaagacaaggctggaagtctgggttgtacgtcgtttccgagcgcaaagaggccctgcgttctggtttcaggggattcaggggattctcatcatgtgtgccagagcacagatactaaatctccctcaccctgagcccaggccaatatcctaacctttcggctaaaagaaaacagtcacagaaaaccatttttgtttccttaagaaaataaatatttccacgaggtcaagccaaagtacaggggctggagacggggtgggaagtggggcaaacactttagatgagcacagtagctcctgctagctggggcatcagggcactcaccatgtccctgcacaagatgctcacccactccaccttcccatcctggagctgcacaaattgtccctttcttgaagttgatgcaatgtgtctctgtgttagatatgagctcccaactgggcccaaggacttggggtgatggaggctgcaggctcttgccaaagccaggtttaaatccctgtttctattttaccagcagggaagaaatgagagtcgagttgagaaaatgctcagttaagacagtcagtcacgggacagctgtatcctcaggaccagcctgtcatcgataagtccaagccctggctactgctgctggagaggcaaaggaacaatcttgcctttcagcgccgtcggaaagctcgagatattctccaggcattgggttcctcatagcggttgtacaagggttcaagacgctgttgcttcttctgtttgcttagcttagttgggtctgagaccttgaagaaggctggggcaaactccacaagccaccgagggtcgatggtggtaacttcacgcatgtattccttggtggtgagcaccagctcatggtacaccacccattctggctgtctgttgaagagggcactggaaggatggatatagaccacctgctggtcgatcagtgtccggtaaccctcctgcgggtctttcttggcagcattacggaagaacccactgcagatggccttctgcactcggactgtggacttgccacaggaaacaacatccagcttgtgtctgtccattatgcctaacatctgcttgcgaatgtcctgggcccggcgcagggaacgagcctggataaagttctcatagcaccatgggttggagaacttgttgttcttccaggagttgtacacagctagcagggtgaggtggtccccttcagtctggtggaatttggccttcttctgatctgcaagggcttgtttatccttgggcctatagaagacgttctgcacagacagcatggatacaatggtcagcatttcctcactgcagcccagatgcacagacatgatgagcattttgcatagcattggctccagagggaactctgccatccggcggcccaagcgagtgagcaggccctcgtcatccagggcccccagtgtgtacagctgctccatggctgtgatcaaagtttccataggtggggcatccatgaaatcaaaggacagcagatcattgatacccatggcccaaagtcgcagtttggagctgaagtccaagccacagatgcctctctgttggcacttcagagactggagtaggtttcttttttctttccaaagctctgttttagcctctttgacagggaataaataataaatgacaacagagcactctgcaccagaaagtaccagggctccagggtagcatcagtgtcgggggaaacgccatcagctgggaaattactcatacagctcctccttgagtgacagcactgtgcttgctaagttggttctctggatttccggcacgttggtggtcagcatttcatctcggtaggcacgttctgtgtacaacctgtaacacttccctgggcctgttctcccagctctgccagctcgttgctttgcctgagcctgagaaataggcgtcaccacgagctggtcaatccctgtcttggaattgtaaactttctgtttcacgaatcctgggtccaccacatagtagataccatcaatagtcagcgatgtctctgcgatattggtggcaatcacaacctttctgctgcctggtggagctgggtcaaagattcgggtctgcatctcactgggaagagcagagtacactgggaggataattaactctggaacatcaggtcccagggatttcattctttcatacaggatctcacaagcagtatcaatttcttcctgaccagtcaggaagaccaggatatcacctggtggttctgttaaatgaatctgcataacagtaatcaggctggcatccagataatctgtctcaggttcctttgtgtacagtatttccactggatatgttcgacctgggatggtgaaaatgggagcttcatagaagtattgagaaaacttcactgcatccaaggtggctgaggtgacaatcagcttcatgtcctgccgtttctgaactgtctttttcaacaatccaaagagcacatcagtgtgaattgtcctctcatgtgcctcgtccaacatgatgatcgcgtactgagtgaggtcagggtcaatcaagcactctctaagcaacatcccatctgtcatgtacttgatgactgtttcagggctagtgcagtcctcaaatcgaatggtgtagcccacctcttggcctaagcaacaaccaaactcctctgacactcttttggccaccgacatagctgccactcttctgggctgggtacacccaatcttgcccctggaagtgtagcctgcctccgccaggtactgggtgatctgtgttgtctttccagatcctgtctcaccaatgacaatcaggatctgattgtcatggacggcctggaccaattgctccttcagtttgtagatgggcaggctctccctctgctcaaggattgacatctgggtcttttttccgtaagaggctttgttgcccccaaaggcatgcttcttccactcaggaatatcattgggcatcatcccaatacccctcatgttggcagcaatctgtctgccttccgcatcaggcagagggtcaacccagtgtttgttgagtcccatgggaatagaatccatctcagcttcccgctgggcctgtttgagttcccgcctttctttggccaaggcactctgcatcattgctgcttgggagagggagccgtctgggttcttgacaattttaatggggctcatgtccatgctttgcttagtgtgccctctcaggaatggaggctcttcctcaaccaattcaatctcaaggtcctcatcttcttcatcatccaccttagggagaatgccagtctcttcatcaaagtctggaaattcttctttggaaaggacattggcagcaatcatctgtttgatctcccacttctctgggtcagagattcgggtgaggcgcttgcgttccagtgagtcgtcctctacttcaggagcactgacaagggacaagtgagtgggtctatcaggattccgcattgaggtctcctcattggtctccccgacaagatttcgccgtctatttgggtttagatcttctccagtctcttgatccacatccttcatgctcaggctggtcttggtcccagtgaaggacagcactttgactttgaccctctggcctttgctcacgacatcagctacattggccacacgaccctcccgccggagctcagagatgtgcaccaggccttcccaccgcttccttagtccttccagctgcacaaagcaaccaaactgcatgatgctggtaactttgccattataaatgtcaccaatggtgggctcttctggaggagggcggtccacatgcttatcccgccatctatccagattccgctctccatatttgtcccggtccttccggtctttggggggactctgactcctgctcctggaccgatatctagacttcactttattcctctcccgggtcctggaacgtgatcgagagcgggatcggtgtctccgcttgtggtctctatctcggtttcgttccctatctctgtctcgatctcggtttcgatctcggcttcgactccgcttcttcttctttgtcctgtccctaacaaatcaataagcaccggtgttcagcatctctttgcttctcctggcctgctgcgctgggcattaaagcttccagttctttcaggacatccacagcaactttcacatcatcttcatccaacatggtccgaacagaagggttgtccggttggcaaaggactgggaagagttccttcagcttttctttttctgttttaggtttaacaactggatctttgctagtggaaggcttcgctggaggccgcatggtttgtatgagacgcagcaagttactaataagagaatccgtaaattctgcaccatttttgacgagagaagccttaaaagtatcaaaggtggtatttttctcagcaagactgatcacaaattcagcaaggtccttgtcgttgatccccaagtgattgtccagctcagtgcaaacctttgacaccaaagacaggtactcgagtttggcaagttcttccgcggggcctggctccgacccgattaaggctcccgccatggctacagccacagccatggctatagcttgcccagaacctccttcctcacagccggcgctcagagctactccggccgggtt

SEQ ID NO: 9905 - RNA, 5277 nt, Homo sapiens
  source 1..5277: mol_type = other RNA
caaccaccactgtctctccccagaaggccttcaaggttaacacacaacaatgccctgccccttgattactggcctgggcttacaaaggcgaatactcagacagaatcaggaggcactcagcttaatgaaggggcagggatctgcagccagcagattgcctggcctatattcctctccctcggactctttctgaattgtctttagggtgtggtttgctgcccagtgacaacatacattcctttatatcctggaatgttacatagtctctcttagtgtctggcatacagttctacagtagttctagcatttacatcacttcagaacttactaataacataaggacaggagaagcagcaacgtaacaggatgtgcccaatctctcagaagcttctctacaagcactacatccagaccagctttccgtaagttccgaaacctggcctggcaagacctgcctgatgttccgccaggtaaggagcctcctcagtgcagaggacagtggctctcaactgtaatcccagcgctttgggaggcagaggcaggaggattgcttgacgccagggattggagagcagcctgggcagcacagtgggaacccatctctatgggaagaaaaaaaaaaaaccctcctcaggagctgtgaggagggcacaaggaggtggctattctccaagcaagtgctaggaaaaaaccactaagaacaagccctgcagcacagatactggcagcacaaaccagctgagaggagaggtgttatgtttgttttctgtttggagtggggaaagggaggttttgaccataaaatccctttgttaaagtccatccaggacctcaggggaaaaaaataaaaacaaaataaaataaaagctgtgttgttacttagtatgtttcaaaaggaaatgggacatgctgcacattgcgaatgtgggaggtggagggagcaaggggaaaccttctgtatttaatatgtgccatctgtagccactcaggcctccagactgaagtgctctgtggagaggacatggttgatcatcgggtgatcccccagcacggcccggctagtgctgatgctgaaagacaaggctggaagtctgggttgtacgtcgtttccgagcgcaaagaggccctgcgttctggtttcaggggattcaggggattctcatcatgtgtgccagagcacagatactaaatctccctcaccctgagcccaggccaatatcctaacctttcggctaaaagaaaacagtcacagaaaaccatttttgtttccttaagaaaataaatatttccacgaggtcaagccaaagtacaggggctggagacggggtgggaagtggggcaaacactttagatgagcacagtagctcctgctagctggggcatcagggcactcaccatgtccctgcacaagatgctcacccactccaccttcccatcctggagctgcacaaattgtccctttcttgaagttgatgcaatgtgtctctgtgttagatatgagctcccaactgggcccaaggacttggggtgatggaggctgcaggctcttgccaaagccaggtttaaatccctgtttctattttaccagcagggaagaaatgagagtcgagttgagaaaatgctcagttaagacagtcagtcacgggacagctgtatcctcaggaccagcctgtcatcgataagtccaagccctggctactgctgctggagaggcaaaggaacaatcttgcctttcagcgccgtcggaaagctcgagatattctccaggcattgggttcctcatagcggttgtacaagggttcaagacgctgttgcttcttctgtttgcttagcttagttgggtctgagaccttgaagaaggctggggcaaactccacaagccaccgagggtcgatggtggtaacttcacgcatgtattccttggtggtgagcaccagctcatggtacaccacccattctggctgtctgttgaagagggcactggaaggatggatatagaccacctgctggtcgatcagtgtccggtaaccctcctgcgggtctttcttggcagcattacggaagaacccactgcagatggccttctgcactcggactgtggacttgccacaggaaacaacatccagcttgtgtctgtccattatgcctaacatctgcttgcgaatgtcctgggcccggcgcagggaacgagcctggataaagttctcatagcaccatgggttggagaacttgttgttcttccaggagttgtacacagctagcagggtgaggtggtccccttcagtctggtggaatttggccttcttctgatctgcaagggcttgtttatccttgggcctatagaagacgttctgcacagacagcatggatacaatggtcagcatttcctcactgcagcccagatgcacagacatgatgagcattttgcatagcattggctccagagggaactctgccatccggcggcccaagcgagtgagcaggccctcgtcatccagggcccccagtgtgtacagctgctccatggctgtgatcaaagtttccataggtggggcatccatgaaatcaaaggacagcagatcattgatacccatggccttgagtgacagcactgtgcttgctaagttggttctctggatttccggcacgttggtggtcagcatttcatctcggtaggcacgttctgtgtacaacctgtaacacttccctgggcctgttctcccagctctgccagctcgttgctttgcctgagcctgagaaataggcgtcaccacgagctggtcaatccctgtcttggaattgtaaactttctgtttcacgaatcctgggtccaccacatagtagataccatcaatagtcagcgatgtctctgcgatattggtggcaatcacaacctggtggttctgttaaatgaatctgcataacagtaatcaggctggcatccagataatctgtctcaggttcctttgtgtacagtatttccactggatatgttcgacctgggatggtgaaaatgggagcttcatagaagtattgagaaaacttcactgcatccaaggtggctgaggtgacaatcagcttcatgtcctgccgtttctgaactgtctttttcaacaatccaaagagcacatcagtgtgaattgtcctctcatgtgcctcgtccaacatgatgatcgcgtactgagtgaggtcagggtcaatcaagcactctctaagcaacatcccatctgtcatgtacttgatgactgtttcagggctagtgcagtcctcaaatcgaatggtgtagcccacctcttggcctaagcaacaaccaaactcctctgacactcttttggccaccgacatagctgccactcttctgggctgggtacacccaatcttgcccctggaagtgtagcctgcctccgccaggtactgggtgatctgtgttgtctttccagatcctgtctcaccaatgacaatcaggatctgattgtcatggacggcctggaccaattgctccttcagtttgtagatgggcaggctctccctctgctcaaggattgacatctgggtcttttttccgtaagaggctttgttgcccccaaaggcatgcttcttccactcaggaatatcattgggcatcatcccaatacccctcatgttggcagcaatctgtctgccttccgcatcaggcagagggtcaacccagtgtttgttgagtcccatgggaatagaatccatctcagcttcccgctgggcctgtttgagttcccgcctttctttggccaaggcactctgcatcattgctgcttgggagagggagccgtctgggttcttgacaattttaatggggctcatgtccatgctttgcttagtgtgccctctcaggaatggaggctcttcctcaaccaattcaatctcaaggtcctcatcttcttcatcatccaccttagggagaatgccagtctcttcatcaaagtctggaaattcttctttggaaaggacattggcagcaatcatctgtttgatctcccacttctctgggtcagagattcgggtgaggcgcttgcgttccagtgagtcgtcctctacttcaggagcactgacaagggacaagtgagtgggtctatcaggattccgcattgaggtctcctcattggtctccccgacaagatttcgccgtctatttgggtttagatcttctccagtctcttgatccacatccttcatgctcaggctggtcttggtcccagtgaaggacagcactttgactttgaccctctggcctttgctcacgacatcagctacattggccacacgaccctcccgccggagctcagagatgtgcaccaggccttcccaccgcttccttagtccttccagctgcacaaagcaaccaaactgcatgatgctggtaactttgccattataaatgtcaccaatggtgggctcttctggaggagggcggtccacatgcttatcccgccatctatccagattccgctctccatatttgtcccggtccttccggtctttggggggactctgactcctgctcctggaccgatatctagacttcactttattcctctcccgggtcctggaacgtgatcgagagcgggatcggtgtctccgcttgtggtctctatctcggtttcgttccctatctctgtctcgatctcggtttcgatctcggcttcgactccgcttcttcttctttgtcctgtcccggtgttcagcatctctttgcttctcctggcctgctgcgctgggcattaaagcttccagttctttcaggacatccacagcaactttcacatcatcttcatccaacatggtccgaacagaagggttgtccggttggcaaaggactgggaagagttccttcagcttttctttttctgttttaggtttaacaactggatctttgctagtggaaggcttcgctggaggccgcatggtttgtatgagacgcagcaagttactaataagagaatccgtaaattctgcaccatttttgacgagagaagccttaaaagtatcaaaggtggtatttttctcagcaagactgatcacaaattcagcaaggtccttgtcgttgatccccaagtgattgtccagctcagtgcaaacctttgacaccaaagacaggtactcgagtttggcaagttcttccgcggggcctggctccgacccgattaaggctcccgccatggctacagccacagccatggctatagcttgcccagaacctccttcctcacagccggcgctcagagctactccggccgggtt

SEQ ID NO: 9906 - RNA, 5453 nt, Homo sapiens
  source 1..5453: mol_type = other RNA
caaccaccactgtctctccccagaaggccttcaaggttaacacacaacaatgccctgccccttgattactggcctgggcttacaaaggcgaatactcagacagaatcaggaggcactcagcttaatgaaggggcagggatctgcagccagcagattgcctggcctatattcctctccctcggactctttctgaattgtctttagggtgtggtttgctgcccagtgacaacatacattcctttatatcctggaatgttacatagtctctcttagtgtctggcatacagttctacagtagttctagcatttacatcacttcagaacttactaataacataaggacaggagaagcagcaacgtaacaggatgtgcccaatctctcagaagcttctctacaagcactacatccagaccagctttccgtaagttccgaaacctggcctggcaagacctgcctgatgttccgccaggtaaggagcctcctcagtgcagaggacagtggctctcaactgtaatcccagcgctttgggaggcagaggcaggaggattgcttgacgccagggattggagagcagcctgggcagcacagtgggaacccatctctatgggaagaaaaaaaaaaaaccctcctcaggagctgtgaggagggcacaaggaggtggctattctccaagcaagtgctaggaaaaaaccactaagaacaagccctgcagcacagatactggcagcacaaaccagctgagaggagaggtgttatgtttgttttctgtttggagtggggaaagggaggttttgaccataaaatccctttgttaaagtccatccaggacctcaggggaaaaaaataaaaacaaaataaaataaaagctgtgttgttacttagtatgtttcaaaaggaaatgggacatgctgcacattgcgaatgtgggaggtggagggagcaaggggaaaccttctgtatttaatatgtgccatctgtagccactcaggcctccagactgaagtgctctgtggagaggacatggttgatcatcgggtgatcccccagcacggcccggctagtgctgatgctgaaagacaaggctggaagtctgggttgtacgtcgtttccgagcgcaaagaggccctgcgttctggtttcaggggattcaggggattctcatcatgtgtgccagagcacagatactaaatctccctcaccctgagcccaggccaatatcctaacctttcggctaaaagaaaacagtcacagaaaaccatttttgtttccttaagaaaataaatatttccacgaggtcaagccaaagtacaggggctggagacggggtgggaagtggggcaaacactttagatgagcacagtagctcctgctagctggggcatcagggcactcaccatgtccctgcacaagatgctcacccactccaccttcccatcctggagctgcacaaattgtccctttcttgaagttgatgcaatgtgtctctgtgttagatatgagctcccaactgggcccaaggacttggggtgatggaggctgcaggctcttgccaaagccaggtttaaatccctgtttctattttaccagcagggaagaaatgagagtcgagttgagaaaatgctcagttaagacagtcagtcacgggacagctgtatcctcaggaccagcctgtcatcgataagtccaagccctggctactgctgctggagaggcaaaggaacaatcttgcctttcagcgccgtcggaaagctcgagatattctccaggcattgggttcctcatagcggttgtacaagggttcaagacgctgttgcttcttctgtttgcttagcttagttgggtctgagaccttgaagaaggctggggcaaactccacaagccaccgagggtcgatggtggtaacttcacgcatgtattccttggtggtgagcaccagctcatggtacaccacccattctggctgtctgttgaagagggcactggaaggatggatatagaccacctgctggtcgatcagtgtccggtaaccctcctgcgggtctttcttggcagcattacggaagaacccactgcagatggccttctgcactcggactgtggacttgccacaggaaacaacatccagcttgtgtctgtccattatgcctaacatctgcttgcgaatgtcctgggcccggcgcagggaacgagcctggataaagttctcatagcaccatgggttggagaacttgttgttcttccaggagttgtacacagctagcagggtgaggtggtccccttcagtctggtggaatttggccttcttctgatctgcaagggcttgtttatccttgggcctatagaagacgttctgcacagacagcatggatacaatggtcagcatttcctcactgcagcccagatgcacagacatgatgagcattttgcatagcattggctccagagggaactctgccatccggcggcccaagcgagtgagcaggccctcgtcatccagggcccccagtgtgtacagctgctccatggctgtgatcaaagtttccataggtggggcatccatgaaatcaaaggacagcagatcattgatacccatggccttgagtgacagcactgtgcttgctaagttggttctctggatttccggcacgttggtggtcagcatttcatctcggtaggcacgttctgtgtacaacctgtaacacttccctgggcctgttctcccagctctgccagctcgttgctttgcctgagcctgagaaataggcgtcaccacgagctggtcaatccctgtcttggaattgtaaactttctgtttcacgaatcctgggtccaccacatagtagataccatcaatagtcagcgatgtctctgcgatattggtggcaatcacaacctttctgctgcctggtggagctgggtcaaagattcgggtctgcatctcactgggaagagcagagtacactgggaggataattaactctggaacatcaggtcccagggatttcattctttcatacaggatctcacaagcagtatcaatttcttcctgaccagtcaggaagaccaggatatcacctggtggttctgttaaatgaatctgcataacagtaatcaggctggcatccagataatctgtctcaggttcctttgtgtacagtatttccactggatatgttcgacctgggatggtgaaaatgggagcttcatagaagtattgagaaaacttcactgcatccaaggtggctgaggtgacaatcagcttcatgtcctgccgtttctgaactgtctttttcaacaatccaaagagcacatcagtgtgaattgtcctctcatgtgcctcgtccaacatgatgatcgcgtactgagtgaggtcagggtcaatcaagcactctctaagcaacatcccatctgtcatgtacttgatgactgtttcagggctagtgcagtcctcaaatcgaatggtgtagcccacctcttggcctaagcaacaaccaaactcctctgacactcttttggccaccgacatagctgccactcttctgggctgggtacacccaatcttgcccctggaagtgtagcctgcctccgccaggtactgggtgatctgtgttgtctttccagatcctgtctcaccaatgacaatcaggatctgattgtcatggacggcctggaccaattgctccttcagtttgtagatgggcaggctctccctctgctcaaggattgacatctgggtcttttttccgtaagaggctttgttgcccccaaaggcatgcttcttccactcaggaatatcattgggcatcatcccaatacccctcatgttggcagcaatctgtctgccttccgcatcaggcagagggtcaacccagtgtttgttgagtcccatgggaatagaatccatctcagcttcccgctgggcctgtttgagttcccgcctttctttggccaaggcactctgcatcattgctgcttgggagagggagccgtctgggttcttgacaattttaatggggctcatgtccatgctttgcttagtgtgccctctcaggaatggaggctcttcctcaaccaattcaatctcaaggtcctcatcttcttcatcatccaccttagggagaatgccagtctcttcatcaaagtctggaaattcttctttggaaaggacattggcagcaatcatctgtttgatctcccacttctctgggtcagagattcgggtgaggcgcttgcgttccagtgagtcgtcctctacttcaggagcactgacaagggacaagtgagtgggtctatcaggattccgcattgaggtctcctcattggtctccccgacaagatttcgccgtctatttgggtttagatcttctccagtctcttgatccacatccttcatgctcaggctggtcttggtcccagtgaaggacagcactttgactttgaccctctggcctttgctcacgacatcagctacattggccacacgaccctcccgccggagctcagagatgtgcaccaggccttcccaccgcttccttagtccttccagctgcacaaagcaaccaaactgcatgatgctggtaactttgccattataaatgtcaccaatggtgggctcttctggaggagggcggtccacatgcttatcccgccatctatccagattccgctctccatatttgtcccggtccttccggtctttggggggactctgactcctgctcctggaccgatatctagacttcactttattcctctcccgggtcctggaacgtgatcgagagcgggatcggtgtctccgcttgtggtctctatctcggtttcgttccctatctctgtctcgatctcggtttcgatctcggcttcgactccgcttcttcttctttgtccggtgttcagcatctctttgcttctcctggcctgctgcgctgggcattaaagcttccagttctttcaggacatccacagcaactttcacatcatcttcatccaacatggtccgaacagaagggttgtccggttggcaaaggactgggaagagttccttcagcttttctttttctgttttaggtttaacaactggatctttgctagtggaaggcttcgctggaggccgcatggtttgtatgagacgcagcaagttactaataagagaatccgtaaattctgcaccatttttgacgagagaagccttaaaagtatcaaaggtggtatttttctcagcaagactgatcacaaattcagcaaggtccttgtcgttgatccccaagtgattgtccagctcagtgcaaacctttgacaccaaagacaggtactcgagtttggcaagttcttccgcggggcctggctccgacccgattaaggctcccgccatggctacagccacagccatggctatagcttgcccagaacctccttcctcacagccggcgctcagagctactccggccgggtt

SEQ ID NO: 9907 - RNA, 5541 nt, Homo sapiens
  source 1..5541: mol_type = other RNA
caaccaccactgtctctccccagaaggccttcaaggttaacacacaacaatgccctgccccttgattactggcctgggcttacaaaggcgaatactcagacagaatcaggaggcactcagcttaatgaaggggcagggatctgcagccagcagattgcctggcctatattcctctccctcggactctttctgaattgtctttagggtgtggtttgctgcccagtgacaacatacattcctttatatcctggaatgttacatagtctctcttagtgtctggcatacagttctacagtagttctagcatttacatcacttcagaacttactaataacataaggacaggagaagcagcaacgtaacaggatgtgcccaatctctcagaagcttctctacaagcactacatccagaccagctttccgtaagttccgaaacctggcctggcaagacctgcctgatgttccgccaggtaaggagcctcctcagtgcagaggacagtggctctcaactgtaatcccagcgctttgggaggcagaggcaggaggattgcttgacgccagggattggagagcagcctgggcagcacagtgggaacccatctctatgggaagaaaaaaaaaaaaccctcctcaggagctgtgaggagggcacaaggaggtggctattctccaagcaagtgctaggaaaaaaccactaagaacaagccctgcagcacagatactggcagcacaaaccagctgagaggagaggtgttatgtttgttttctgtttggagtggggaaagggaggttttgaccataaaatccctttgttaaagtccatccaggacctcaggggaaaaaaataaaaacaaaataaaataaaagctgtgttgttacttagtatgtttcaaaaggaaatgggacatgctgcacattgcgaatgtgggaggtggagggagcaaggggaaaccttctgtatttaatatgtgccatctgtagccactcaggcctccagactgaagtgctctgtggagaggacatggttgatcatcgggtgatcccccagcacggcccggctagtgctgatgctgaaagacaaggctggaagtctgggttgtacgtcgtttccgagcgcaaagaggccctgcgttctggtttcaggggattcaggggattctcatcatgtgtgccagagcacagatactaaatctccctcaccctgagcccaggccaatatcctaacctttcggctaaaagaaaacagtcacagaaaaccatttttgtttccttaagaaaataaatatttccacgaggtcaagccaaagtacaggggctggagacggggtgggaagtggggcaaacactttagatgagcacagtagctcctgctagctggggcatcagggcactcaccatgtccctgcacaagatgctcacccactccaccttcccatcctggagctgcacaaattgtccctttcttgaagttgatgcaatgtgtctctgtgttagatatgagctcccaactgggcccaaggacttggggtgatggaggctgcaggctcttgccaaagccaggtttaaatccctgtttctattttaccagcagggaagaaatgagagtcgagttgagaaaatgctcagttaagacagtcagtcacgggacagctgtatcctcaggaccagcctgtcatcgataagtccaagccctggctactgctgctggagaggcaaaggaacaatcttgcctttcagcgccgtcggaaagctcgagatattctccaggcattgggttcctcatagcggttgtacaagggttcaagacgctgttgcttcttctgtttgcttagcttagttgggtctgagaccttgaagaaggctggggcaaactccacaagccaccgagggtcgatggtggtaacttcacgcatgtattccttggtggtgagcaccagctcatggtacaccacccattctggctgtctgttgaagagggcactggaaggatggatatagaccacctgctggtcgatcagtgtccggtaaccctcctgcgggtctttcttggcagcattacggaagaacccactgcagatggccttctgcactcggactgtggacttgccacaggaaacaacatccagcttgtgtctgtccattatgcctaacatctgcttgcgaatgtcctgggcccggcgcagggaacgagcctggataaagttctcatagcaccatgggttggagaacttgttgttcttccaggagttgtacacagctagcagggtgaggtggtccccttcagtctggtggaatttggccttcttctgatctgcaagggcttgtttatccttgggcctatagaagacgttctgcacagacagcatggatacaatggtcagcatttcctcactgcagcccagatgcacagacatgatgagcattttgcatagcattggctccagagggaactctgccatccggcggcccaagcgagtgagcaggccctcgtcatccagggcccccagtgtgtacagctgctccatggctgtgatcaaagtttccataggtggggcatccatgaaatcaaaggacagcagatcattgatacccatggccttgagtgacagcactgtgcttgctaagttggttctctggatttccggcacgttggtggtcagcatttcatctcggtaggcacgttctgtgtacaacctgtaacacttccctgggcctgttctcccagctctgccagctcgttgctttgcctgagcctgagaaataggcgtcaccacgagctggtcaatccctgtcttggaattgtaaactttctgtttcacgaatcctgggtccaccacatagtagataccatcaatagtcagcgatgtctctgcgatattggtggcaatcacaacctttctgctgcctggtggagctgggtcaaagattcgggtctgcatctcactgggaagagcagagtacactgggaggataattaactctggaacatcaggtcccagggatttcattctttcatacaggatctcacaagcagtatcaatttcttcctgaccagtcaggaagaccaggatatcacctggtggttctgttaaatgaatctgcataacagtaatcaggctggcatccagataatctgtctcaggttcctttgtgtacagtatttccactggatatgttcgacctgggatggtgaaaatgggagcttcatagaagtattgagaaaacttcactgcatccaaggtggctgaggtgacaatcagcttcatgtcctgccgtttctgaactgtctttttcaacaatccaaagagcacatcagtgtgaattgtcctctcatgtgcctcgtccaacatgatgatcgcgtactgagtgaggtcagggtcaatcaagcactctctaagcaacatcccatctgtcatgtacttgatgactgtttcagggctagtgcagtcctcaaatcgaatggtgtagcccacctcttggcctaagcaacaaccaaactcctctgacactcttttggccaccgacatagctgccactcttctgggctgggtacacccaatcttgcccctggaagtgtagcctgcctccgccaggtactgggtgatctgtgttgtctttccagatcctgtctcaccaatgacaatcaggatctgattgtcatggacggcctggaccaattgctccttcagtttgtagatgggcaggctctccctctgctcaaggattgacatctgggtcttttttccgtaagaggctttgttgcccccaaaggcatgcttcttccactcaggaatatcattgggcatcatcccaatacccctcatgttggcagcaatctgtctgccttccgcatcaggcagagggtcaacccagtgtttgttgagtcccatgggaatagaatccatctcagcttcccgctgggcctgtttgagttcccgcctttctttggccaaggcactctgcatcattgctgcttgggagagggagccgtctgggttcttgacaattttaatggggctcatgtccatgctttgcttagtgtgccctctcaggaatggaggctcttcctcaaccaattcaatctcaaggtcctcatcttcttcatcatccaccttagggagaatgccagtctcttcatcaaagtctggaaattcttctttggaaaggacattggcagcaatcatctgtttgatctcccacttctctgggtcagagattcgggtgaggcgcttgcgttccagtgagtcgtcctctacttcaggagcactgacaagggacaagtgagtgggtctatcaggattccgcattgaggtctcctcattggtctccccgacaagatttcgccgtctatttgggtttagatcttctccagtctcttgatccacatccttcatgctcaggctggtcttggtcccagtgaaggacagcactttgactttgaccctctggcctttgctcacgacatcagctacattggccacacgaccctcccgccggagctcagagatgtgcaccaggccttcccaccgcttccttagtccttccagctgcacaaagcaaccaaactgcatgatgctggtaactttgccattataaatgtcaccaatggtgggctcttctggaggagggcggtccacatgcttatcccgccatctatccagattccgctctccatatttgtcccggtccttccggtctttggggggactctgactcctgctcctggaccgatatctagacttcactttattcctctcccgggtcctggaacgtgatcgagagcgggatcggtgtctccgcttgtggtctctatctcggtttcgttccctatctctgtctcgatctcggtttcgatctcggcttcgactccgcttcttcttctttgtcctgtccccaaaattttgcttggctggtccataatattcaactgtcacagtaccctaaacttccaaaggacaggacactaaggacaaaccggtgttcagcatctctttgcttctcctggcctgctgcgctgggcattaaagcttccagttctttcaggacatccacagcaactttcacatcatcttcatccaacatggtccgaacagaagggttgtccggttggcaaaggactgggaagagttccttcagcttttctttttctgttttaggtttaacaactggatctttgctagtggaaggcttcgctggaggccgcatggtttgtatgagacgcagcaagttactaataagagaatccgtaaattctgcaccatttttgacgagagaagccttaaaagtatcaaaggtggtatttttctcagcaagactgatcacaaattcagcaaggtccttgtcgttgatccccaagtgattgtccagctcagtgcaaacctttgacaccaaagacaggtactcgagtttggcaagttcttccgcggggcctggctccgacccgattaaggctcccgccatggctacagccacagccatggctatagcttgcccagaacctccttcctcacagccggcgctcagagctactccggccgggtt

SEQ ID NO: 9908 - RNA, 5373 nt, Homo sapiens
  source 1..5373: mol_type = other RNA
caaccaccactgtctctccccagaaggccttcaaggttaacacacaacaatgccctgccccttgattactggcctgggcttacaaaggcgaatactcagacagaatcaggaggcactcagcttaatgaaggggcagggatctgcagccagcagattgcctggcctatattcctctccctcggactctttctgaattgtctttagggtgtggtttgctgcccagtgacaacatacattcctttatatcctggaatgttacatagtctctcttagtgtctggcatacagttctacagtagttctagcatttacatcacttcagaacttactaataacataaggacaggagaagcagcaacgtaacaggatgtgcccaatctctcagaagcttctctacaagcactacatccagaccagctttccgtaagttccgaaacctggcctggcaagacctgcctgatgttccgccaggtaaggagcctcctcagtgcagaggacagtggctctcaactgtaatcccagcgctttgggaggcagaggcaggaggattgcttgacgccagggattggagagcagcctgggcagcacagtgggaacccatctctatgggaagaaaaaaaaaaaaccctcctcaggagctgtgaggagggcacaaggaggtggctattctccaagcaagtgctaggaaaaaaccactaagaacaagccctgcagcacagatactggcagcacaaaccagctgagaggagaggtgttatgtttgttttctgtttggagtggggaaagggaggttttgaccataaaatccctttgttaaagtccatccaggacctcaggggaaaaaaataaaaacaaaataaaataaaagctgtgttgttacttagtatgtttcaaaaggaaatgggacatgctgcacattgcgaatgtgggaggtggagggagcaaggggaaaccttctgtatttaatatgtgccatctgtagccactcaggcctccagactgaagtgctctgtggagaggacatggttgatcatcgggtgatcccccagcacggcccggctagtgctgatgctgaaagacaaggctggaagtctgggttgtacgtcgtttccgagcgcaaagaggccctgcgttctggtttcaggggattcaggggattctcatcatgtgtgccagagcacagatactaaatctccctcaccctgagcccaggccaatatcctaacctttcggctaaaagaaaacagtcacagaaaaccatttttgtttccttaagaaaataaatatttccacgaggtcaagccaaagtacaggggctggagacggggtgggaagtggggcaaacactttagatgagcacagtagctcctgctagctggggcatcagggcactcaccatgtccctgcacaagatgctcacccactccaccttcccatcctggagctgcacaaattgtccctttcttgaagttgatgcaatgtgtctctgtgttagatatgagctcccaactgggcccaaggacttggggtgatggaggctgcaggctcttgccaaagccaggtttaaatccctgtttctattttaccagcagggaagaaatgagagtcgagttgagaaaatgctcagttaagacagtcagtcacgggacagctgtatcctcaggaccagcctgtcatcgataagtccaagccctggctactgctgctggagaggcaaaggaacaatcttgcctttcagcgccgtcggaaagctcgagatattctccaggcattgggttcctcatagcggttgtacaagggttcaagacgctgttgcttcttctgtttgcttagcttagttgggtctgagaccttgaagaaggctggggcaaactccacaagccaccgagggtcgatggtggtaacttcacgcatgtattccttggtggtgagcaccagctcatggtacaccacccattctggctgtctgttgaagagggcactggaaggatggatatagaccacctgctggtcgatcagtgtccggtaaccctcctgcgggtctttcttggcagcattacggaagaacccactgcagatggccttctgcactcggactgtggacttgccacaggaaacaacatccagcttgtgtctgtccattatgcctaacatctgcttgcgaatgtcctgggcccggcgcagggaacgagcctggataaagttctcatagcaccatgggttggagaacttgttgttcttccaggagttgtacacagctagcagggtgaggtggtccccttcagtctggtggaatttggccttcttctgatctgcaagggcttgtttatccttgggcctatagaagacgttctgcacagacagcatggatacaatggtcagcatttcctcactgcagcccagatgcacagacatgatgagcattttgcatagcattggctccagagggaactctgccatccggcggcccaagcgagtgagcaggccctcgtcatccagggcccccagtgtgtacagctgctccatggctgtgatcaaagtttccataggtggggcatccatgaaatcaaaggacagcagatcattgatacccatggccttgagtgacagcactgtgcttgctaagttggttctctggatttccggcacgttggtggtcagcatttcatctcggtaggcacgttctgtgtacaacctgtaacacttccctgggcctgttctcccagctctgccagctcgttgctttgcctgagcctgagaaataggcgtcaccacgagctggtcaatccctgtcttggaattgtaaactttctgtttcacgaatcctgggtccaccacatagtagataccatcaatagtcagcgatgtctctgcgatattggtggcaatcacaacctttctgctgcctggtggagctgggtcaaagattcgggtctgcatctcactgggaagagcagagtacactgggaggataattaactctggaacatcaggtcccagggatttcattctttcatacaggatctcacaagcagtatcaatttcttcctgaccagtcaggaagaccaggatatcacctggtggttctgttaaatgaatctgcataacagtaatcaggctggcatccagataatctgtctcaggttcctttgtgtacagtatttccactggatatgttcgacctgggatggtgaaaatgggagcttcatagaagtattgagaaaacttcactgcatccaaggtggctgaggtgacaatcagcttcatgtcctgccgtttctgaactgtctttttcaacaatccaaagagcacatcagtgtgaattgtcctctcatgtgcctcgtccaacatgatgatcgcgtactgagtgaggtcagggtcaatcaagcactctctaagcaacatcccatctgtcatgtacttgatgactgtttcagggctagtgcagtcctcaaatcgaatggtgtagcccacctcttggcctaagcaacaaccaaactcctctgacactcttttggccaccgacatagctgccactcttctgggctgggtacacccaatcttgcccctggaagtgtagcctgcctccgccaggtactgggtgatctgtgttgtctttccagatcctgtctcaccaatgacaatcaggatctgattgtcatggacggcctggaccaattgctccttcagtttgtagatgggcaggctctccctctgctcaaggattgacatctgggtcttttttccgtaagaggctttgttgcccccaaaggcatgcttcttccactcaggaatatcattgggcatcatcccaatacccctcatgttggcagcaatctgtctgccttccgcatcaggcagagggtcaacccagtgtttgttgagtcccatgggaatagaatccatctcagcttcccgctgggcctgtttgagttcccgcctttctttggccaaggcactctgcatcattgctgcttgggagagggagccgtctgggttcttgacaattttaatggggctcatgtccatgctttgcttagtgtgccctctcaggaatggaggctcttcctcaaccaattcaatctcaaggtcctcatcttcttcatcatccaccttagggagaatgccagtctcttcatcaaagtctggaaattcttctttggaaaggacattggcagcaatcatctgtttgatctcccacttctctgggtcagagattcgggtgaggcgcttgcgttccagtgagtcgtcctctacttcaggagcactgacaagggacaagtgagtgggtctatcaggattccgcattgaggtctcctcattggtctccccgacaagatttcgccgtctatttgggtttagatcttctccagtctcttgatccacatccttcatgctcaggctggtcttggtcccagtgaaggacagcactttgactttgaccctctggcctttgctcacgacatcagctacattggccacacgaccctcccgccggagctcagagatgtgcaccaggccttcccaccgcttccttagtccttccagctgcacaaagcaaccaaactgcatgatgctggtaactttgccattataaatgtcaccaatggtgggctcttctggaggagggcggtccacatgcttatcccgccatctatccagattccgctctccatatttgtcccggtccttccggtctttggggggactctgactcctgctcctggaccgatatctagacttcactttattcctctcccgggtcctggaacgtgatcgagagcgggatcggtgtctccgcttgtggtctctatctcggtttcgttccctatctctgtctcgatctcggtttcgatctcggcttcgactccgcttcttcttctttgtcctgtcccggtgttcagcatctctttgcttctcctggcctgctgcgctgggcattaaagcttccagttctttcaggacatccacagcaactttcacatcatcttcatccaacatggtccgaacagaagggttgtccggttggcaaaggactgggaagagttccttcagcttttctttttctgttttaggtttaacaactggatctttgctagtggaaggcttcgctggaggccgcatggtttgtatgagacgcagcaagttactaataagagaatccaaggtccttgtcgttgatccccaagtgattgtccagctcagtgcaaacctttgacaccaaagacaggtactcgagtttggcaagttcttccgcggggcctggctccgacccgattaaggctcccgccatggctacagccacagccatggctatagcttgcccagaacctccttcctcacagccggcgctcagagctactccggccgggtt

SEQ ID NO: 9909 - RNA, 5459 nt, Homo sapiens
  source 1..5459: mol_type = other RNA
caaccaccactgtctctccccagaaggccttcaaggttaacacacaacaatgccctgccccttgattactggcctgggcttacaaaggcgaatactcagacagaatcaggaggcactcagcttaatgaaggggcagggatctgcagccagcagattgcctggcctatattcctctccctcggactctttctgaattgtctttagggtgtggtttgctgcccagtgacaacatacattcctttatatcctggaatgttacatagtctctcttagtgtctggcatacagttctacagtagttctagcatttacatcacttcagaacttactaataacataaggacaggagaagcagcaacgtaacaggatgtgcccaatctctcagaagcttctctacaagcactacatccagaccagctttccgtaagttccgaaacctggcctggcaagacctgcctgatgttccgccaggtaaggagcctcctcagtgcagaggacagtggctctcaactgtaatcccagcgctttgggaggcagaggcaggaggattgcttgacgccagggattggagagcagcctgggcagcacagtgggaacccatctctatgggaagaaaaaaaaaaaaccctcctcaggagctgtgaggagggcacaaggaggtggctattctccaagcaagtgctaggaaaaaaccactaagaacaagccctgcagcacagatactggcagcacaaaccagctgagaggagaggtgttatgtttgttttctgtttggagtggggaaagggaggttttgaccataaaatccctttgttaaagtccatccaggacctcaggggaaaaaaataaaaacaaaataaaataaaagctgtgttgttacttagtatgtttcaaaaggaaatgggacatgctgcacattgcgaatgtgggaggtggagggagcaaggggaaaccttctgtatttaatatgtgccatctgtagccactcaggcctccagactgaagtgctctgtggagaggacatggttgatcatcgggtgatcccccagcacggcccggctagtgctgatgctgaaagacaaggctggaagtctgggttgtacgtcgtttccgagcgcaaagaggccctgcgttctggtttcaggggattcaggggattctcatcatgtgtgccagagcacagatactaaatctccctcaccctgagcccaggccaatatcctaacctttcggctaaaagaaaacagtcacagaaaaccatttttgtttccttaagaaaataaatatttccacgaggtcaagccaaagtacaggggctggagacggggtgggaagtggggcaaacactttagatgagcacagtagctcctgctagctggggcatcagggcactcaccatgtccctgcacaagatgctcacccactccaccttcccatcctggagctgcacaaattgtccctttcttgaagttgatgcaatgtgtctctgtgttagatatgagctcccaactgggcccaaggacttggggtgatggaggctgcaggctcttgccaaagccaggtttaaatccctgtttctattttaccagcagggaagaaatgagagtcgagttgagaaaatgctcagttaagacagtcagtcacgggacagctgtatcctcaggaccagcctgtcatcgataagtccaagccctggctactgctgctggagaggcaaaggaacaatcttgcctttcagcgccgtcggaaagctcgagatattctccaggcattgggttcctcatagcggttgtacaagggttcaagacgctgttgcttcttctgtttgcttagcttagttgggtctgagaccttgaagaaggctggggcaaactccacaagccaccgagggtcgatggtggtaacttcacgcatgtattccttggtggtgagcaccagctcatggtacaccacccattctggctgtctgttgaagagggcactggaaggatggatatagaccacctgctggtcgatcagtgtccggtaaccctcctgcgggtctttcttggcagcattacggaagaacccactgcagatggccttctgcactcggactgtggacttgccacaggaaacaacatccagcttgtgtctgtccattatgcctaacatctgcttgcgaatgtcctgggcccggcgcagggaacgagcctggataaagttctcatagcaccatgggttggagaacttgttgttcttccaggagttgtacacagctagcagggtgaggtggtccccttcagtctggtggaatttggccttcttctgatctgcaagggcttgtttatccttgggcctatagaagacgttctgcacagacagcatggatacaatggtcagcatttcctcactgcagcccagatgcacagacatgatgagcattttgcatagcattggctccagagggaactctgccatccggcggcccaagcgagtgagcaggccctcgtcatccagggcccccagtgtgtacagctgctccatggctgtgatcaaagtttccataggtggggcatccatgaaatcaaaggacagcagatcattgatacccatggccttgagtgacagcactgtgcttgctaagttggttctctggatttccggcacgttggtggtcagcatttcatctcggtaggcacgttctgtgtacaacctgtaacacttccctgggcctgttctcccagctctgccagctcgttgctttgcctgagcctgagaaataggcgtcaccacgagctggtcaatccctgtcttggaattgtaaactttctgtttcacgaatcctgggtccaccacatagtagataccatcaatagtcagcgatgtctctgcgatattggtggcaatcacaacctttctgctgcctggtggagctgggtcaaagattcgggtctgcatctcactgggaagagcagagtacactgggaggataattaactctggaacatcaggtcccagggatttcattctttcatacaggatctcacaagcagtatcaatttcttcctgaccagtcaggaagaccaggatatcacctggtggttctgttaaatgaatctgcataacagtaatcaggctggcatccagataatctgtctcaggttcctttgtgtacagtatttccactggatatgttcgacctgggatggtgaaaatgggagcttcatagaagtattgagaaaacttcactgcatccaaggtggctgaggtgacaatcagcttcatgtcctgccgtttctgaactgtctttttcaacaatccaaagagcacatcagtgtgaattgtcctctcatgtgcctcgtccaacatgatgatcgcgtactgagtgaggtcagggtcaatcaagcactctctaagcaacatcccatctgtcatgtacttgatgactgtttcagggctagtgcagtcctcaaatcgaatggtgtagcccacctcttggcctaagcaacaaccaaactcctctgacactcttttggccaccgacatagctgccactcttctgggctgggtacacccaatcttgcccctggaagtgtagcctgcctccgccaggtactgggtgatctgtgttgtctttccagatcctgtctcaccaatgacaatcaggatctgattgtcatggacggcctggaccaattgctccttcagtttgtagatgggcaggctctccctctgctcaaggattgacatctgggtcttttttccgtaagaggctttgttgcccccaaaggcatgcttcttccactcaggaatatcattgggcatcatcccaatacccctcatgttggcagcaatctgtctgccttccgcatcaggcagagggtcaacccagtgtttgttgagtcccatgggaatagaatccatctcagcttcccgctgggcctgtttgagttcccgcctttctttggccaaggcactctgcatcattgctgcttgggagagggagccgtctgggttcttgacaattttaatggggctcatgtccatgctttgcttagtgtgccctctcaggaatggaggctcttcctcaaccaattcaatctcaaggtcctcatcttcttcatcatccaccttagggagaatgccagtctcttcatcaaagtctggaaattcttctttggaaaggacattggcagcaatcatctgtttgatctcccacttctctgggtcagagattcgggtgaggcgcttgcgttccagtgagtcgtcctctacttcaggagcactgacaagggacaagtgagtgggtctatcaggattccgcattgaggtctcctcattggtctccccgacaagatttcgccgtctatttgggtttagatcttctccagtctcttgatccacatccttcatgctcaggctggtcttggtcccagtgaaggacagcactttgactttgaccctctggcctttgctcacgacatcagctacattggccacacgaccctcccgccggagctcagagatgtgcaccaggccttcccaccgcttccttagtccttccagctgcacaaagcaaccaaactgcatgatgctggtaactttgccattataaatgtcaccaatggtgggctcttctggaggagggcggtccacatgcttatcccgccatctatccagattccgctctccatatttgtcccggtccttccggtctttggggggactctgactcctgctcctggaccgatatctagacttcactttattcctctcccgggtcctggaacgtgatcgagagcgggatcggtgtctccgcttgtggtctctatctcggtttcgttccctatctctgtctcgatctcggtttcgatctcggcttcgactccgcttcttcttctttgtcctgtcccggtgttcagcatctctttgcttctcctggcctgctgcgctgggcattaaagcttccagttctttcaggacatccacagcaactttcacatcatcttcatccaacatggtccgaacagaagggttgtccggttggcaaaggactgggaagagttccttcagcttttctttttctgttttaggtttaacaactggatctttgctagtggaaggcttcgctggaggccgcatggtttgtatgagacgcagcaagttactaataagagaatccgtaaattctgcaccatttttgacgagagaagccttaaaagtatcaaaggtggtatttttctcagcaagactgatcacaaattcagcaaggtccttgtcgttgatccccaagtgattgtccagctcagtgcaaacctttgacaccaaagacaggtactcgagtttggcaagttcttccgcggggcctggctccgacccgattaaggctcccgccatggctacagccacagccatggctatagcttgcccagaacctccttcctcacagccggcgctcagagctactccggccgggtt

SEQ ID NO: 9910 - RNA, 5455 nt, Homo sapiens
  source 1..5455: mol_type = other RNA
caaccaccactgtctctccccagaaggccttcaaggttaacacacaacaatgccctgccccttgattactggcctgggcttacaaaggcgaatactcagacagaatcaggaggcactcagcttaatgaaggggcagggatctgcagccagcagattgcctggcctatattcctctccctcggactctttctgaattgtctttagggtgtggtttgctgcccagtgacaacatacattcctttatatcctggaatgttacatagtctctcttagtgtctggcatacagttctacagtagttctagcatttacatcacttcagaacttactaataacataaggacaggagaagcagcaacgtaacaggatgtgcccaatctctcagaagcttctctacaagcactacatccagaccagctttccgtaagttccgaaacctggcctggcaagacctgcctgatgttccgccaggtaaggagcctcctcagtgcagaggacagtggctctcaactgtaatcccagcgctttgggaggcagaggcaggaggattgcttgacgccagggattggagagcagcctgggcagcacagtgggaacccatctctatgggaagaaaaaaaaaaaaccctcctcaggagctgtgaggagggcacaaggaggtggctattctccaagcaagtgctaggaaaaaaccactaagaacaagccctgcagcacagatactggcagcacaaaccagctgagaggagaggtgttatgtttgttttctgtttggagtggggaaagggaggttttgaccataaaatccctttgttaaagtccatccaggacctcaggggaaaaaaataaaaacaaaataaaataaaagctgtgttgttacttagtatgtttcaaaaggaaatgggacatgctgcacattgcgaatgtgggaggtggagggagcaaggggaaaccttctgtatttaatatgtgccatctgtagccactcaggcctccagactgaagtgctctgtggagaggacatggttgatcatcgggtgatcccccagcacggcccggctagtgctgatgctgaaagacaaggctggaagtctgggttgtacgtcgtttccgagcgcaaagaggccctgcgttctggtttcaggggattcaggggattctcatcatgtgtgccagagcacagatactaaatctccctcaccctgagcccaggccaatatcctaacctttcggctaaaagaaaacagtcacagaaaaccatttttgtttccttaagaaaataaatatttccacgaggtcaagccaaagtacaggggctggagacggggtgggaagtggggcaaacactttagatgagcacagtagctcctgctagctggggcatcagggcactcaccatgtccctgcacaagatgctcacccactccaccttcccatcctggagctgcacaaattgtccctttcttgaagttgatgcaatgtgtctctgtgttagatatgagctcccaactgggcccaaggacttggggtgatggaggctgcaggctcttgccaaagccaggtttaaatccctgtttctattttaccagcagggaagaaatgagagtcgagttgagaaaatgctcagttaagacagtcagtcacgggacagctgtatcctcaggaccagcctgtcatcgataagtccaagccctggctactgctgctggagaggcaaaggaacaatcttgcctttcagcgccgtcggaaagctcgagatattctccaggcattgggttcctcatagcggttgtacaagggttcaagacgctgttgcttcttctgtttgcttagcttagttgggtctgagaccttgaagaaggctggggcaaactccacaagccaccgagggtcgatggtggtaacttcacgcatgtattccttggtggtgagcaccagctcatggtacaccacccattctggctgtctgttgaagagggcactggaaggatggatatagaccacctgctggtcgatcagtgtccggtaaccctcctgcgggtctttcttggcagcattacggaagaacccactgcagatggccttctgcactcggactgtggacttgccacaggaaacaacatccagcttgtgtctgtccattatgcctaacatctgcttgcgaatgtcctgggcccggcgcagggaacgagcctggataaagttctcatagcaccatgggttggagaacttgttgttcttccaggagttgtacacagctagcagggtgaggtggtccccttcagtctggtggaatttggccttcttctgatctgcaagggcttgtttatccttgggcctatagaagacgttctgcacagacagcatggatacaatggtcagcatttcctcactgcagcccagatgcacagacatgatgagcattttgcatagcattggctccagagggaactctgccatccggcggcccaagcgagtgagcaggccctcgtcatccagggcccccagtgtgtacagctgctccatggctgtgatcaaagtttccataggtggggcatccatgaaatcaaaggacagcagatcattgatacccatggccttgagtgacagcactgtgcttgctaagttggttctctggatttccggcacgttggtggtcagcatttcatctcggtaggcacgttctgtgtacaacctgtaacacttccctgggcctgttctcccagctctgccagctcgttgctttgcctgagcctgagaaataggcgtcaccacgagctggtcaatccctgtcttggaattgtaaactttctgtttcacgaatcctgggtccaccacatagtagataccatcaatagtcagcgatgtctctgcgatattggtggcaatcacaacctttctgctgcctggtggagctgggtcaaagattcgggtctgcatctcactgggaagagcagagtacactgggaggataattaactctggaacatcaggtcccagggatttcattctttcatacaggatctcacaagcagtatcaatttcttcctgaccagtcaggaagaccaggatatcacctggtggttctgttaaatgaatctgcataacagtaatcaggctggcatccagataatctgtctcaggttcctttgtgtacagtatttccactggatatgttcgacctgggatggtgaaaatgggagcttcatagaagtattgagaaaacttcactgcatccaaggtggctgaggtgacaatcagcttcatgtcctgccgtttctgaactttttcaacaatccaaagagcacatcagtgtgaattgtcctctcatgtgcctcgtccaacatgatgatcgcgtactgagtgaggtcagggtcaatcaagcactctctaagcaacatcccatctgtcatgtacttgatgactgtttcagggctagtgcagtcctcaaatcgaatggtgtagcccacctcttggcctaagcaacaaccaaactcctctgacactcttttggccaccgacatagctgccactcttctgggctgggtacacccaatcttgcccctggaagtgtagcctgcctccgccaggtactgggtgatctgtgttgtctttccagatcctgtctcaccaatgacaatcaggatctgattgtcatggacggcctggaccaattgctccttcagtttgtagatgggcaggctctccctctgctcaaggattgacatctgggtcttttttccgtaagaggctttgttgcccccaaaggcatgcttcttccactcaggaatatcattgggcatcatcccaatacccctcatgttggcagcaatctgtctgccttccgcatcaggcagagggtcaacccagtgtttgttgagtcccatgggaatagaatccatctcagcttcccgctgggcctgtttgagttcccgcctttctttggccaaggcactctgcatcattgctgcttgggagagggagccgtctgggttcttgacaattttaatggggctcatgtccatgctttgcttagtgtgccctctcaggaatggaggctcttcctcaaccaattcaatctcaaggtcctcatcttcttcatcatccaccttagggagaatgccagtctcttcatcaaagtctggaaattcttctttggaaaggacattggcagcaatcatctgtttgatctcccacttctctgggtcagagattcgggtgaggcgcttgcgttccagtgagtcgtcctctacttcaggagcactgacaagggacaagtgagtgggtctatcaggattccgcattgaggtctcctcattggtctccccgacaagatttcgccgtctatttgggtttagatcttctccagtctcttgatccacatccttcatgctcaggctggtcttggtcccagtgaaggacagcactttgactttgaccctctggcctttgctcacgacatcagctacattggccacacgaccctcccgccggagctcagagatgtgcaccaggccttcccaccgcttccttagtccttccagctgcacaaagcaaccaaactgcatgatgctggtaactttgccattataaatgtcaccaatggtgggctcttctggaggagggcggtccacatgcttatcccgccatctatccagattccgctctccatatttgtcccggtccttccggtctttggggggactctgactcctgctcctggaccgatatctagacttcactttattcctctcccgggtcctggaacgtgatcgagagcgggatcggtgtctccgcttgtggtctctatctcggtttcgttccctatctctgtctcgatctcggtttcgatctcggcttcgactccgcttcttcttctttgtcctgtcccggtgttcagcatctctttgcttctcctggcctgctgcgctgggcattaaagcttccagttctttcaggacatccacagcaactttcacatcatcttcatccaacatggtccgaacagaagggttgtccggttggcaaaggactgggaagagttccttcagcttttctttttctgttttaggtttaacaactggatctttgctagtggaaggcttcgctggaggccgcatggtttgtatgagacgcagcaagttactaataagagaatccgtaaattctgcaccatttttgacgagagaagccttaaaagtatcaaaggtggtatttttctcagcaagactgatcacaaattcagcaaggtccttgtcgttgatccccaagtgattgtccagctcagtgcaaacctttgacaccaaagacaggtactcgagtttggcaagttcttccgcggggcctggctccgacccgattaaggctcccgccatggctacagccacagccatggctatagcttgcccagaacctccttcctcacagccggcgctcagagctactccggccgggtt

SEQ ID NO: 9911 - RNA, 489 nt, Homo sapiens
  source 1..489: mol_type = other RNA
caaccctaggagagggtgccattcaacatgtggtgggatccagactgaaaccaggaggggttctgagggactgctttggaggaggagggctgaggtcgaagatgggcaggcagggagcaggacatttcagtcctacatggactttttcttcttgctgtggtggtcaatacacagaatattctggaatctcaggctgaatttatacaatctcctactgctgactgataccggtagttctgcagaagatgcaaattcttcacatgatcattttttgtatcaattctctgtagtaccagttacttgggaggctgaggcaagagaactgcttgaacccgggaggcagaggttgcagtgaaccgagattgtgccactgcactccagcctgggcgacagagcgaaactaggcagctgtttgtctaggaaacagcttattgttttcatttgtcatcaccgcggctcactaggtatcaggaagctcggctccagccg

SEQ ID NO: 9912 - RNA, 555 nt, Homo sapiens
  source 1..555: mol_type = other RNA
caaccctaggagagggtgccattcaacatgtggtgggatccagactgaaaccaggaggggttctgagggactgctttggaggaggagggctgaggtcgaagatgggcaggcagggagcaggaccttaaggacaggaactgtgtcaatatcttgatatgctcccaacactgggaaagggctcagcatatgatttcagtcctacatggactttttcttcttgctgtggtggtcaatacacagaatattctggaatctcaggctgaatttatacaatctcctactgctgactgataccggtagttctgcagaagatgcaaattcttcacatgatcattttttgtatcaattctctgtagtaccagttacttgggaggctgaggcaagagaactgcttgaacccgggaggcagaggttgcagtgaaccgagattgtgccactgcactccagcctgggcgacagagcgaaactaggcagctgtttgtctaggaaacagcttattgttttcatttgtcatcaccgcggctcactaggtatcaggaagctcggctccagccg

SEQ ID NO: 9913 - RNA, 72 nt, Homo sapiens
  source 1..72: mol_type = other RNA
caacctcgacgatctcctcagcacctgaacgccaaggctggggagatcctcgaggttggcctgctttccctc

SEQ ID NO: 9914 - RNA, 258 nt, Homo sapiens
  source 1..258: mol_type = other RNA
caacctcgacgatctcctcagcacctgaacgccaaggctggggagatcctcgaggttggcctgctttccctccttttcttacaacttctggagaagcgtcagccctctgcagggaggcggccaagctggcaggcgagtcggcgagggtgtcattgcttatatggctgcggggaccgaagctaggaatagacgcgctgagggctaggagggctccgaccggacggaaggatgccgcatcgcgggtcgctgcccggagct

SEQ ID NO: 9915 - RNA, 132 nt, Homo sapiens
  source 1..132: mol_type = other RNA
caacctcgacgatctcctcagctggtcaggtggcctgaaaacagagctccagccatccacgacagcgccacgggcccgagggacgaggacctgcctctctggcccacccgggcctcgcgcccggagggcgga

SEQ ID NO: 9916 - RNA, 138 nt, Homo sapiens
  source 1..138: mol_type = other RNA
caacctcgacgatctcctcagctggtcaggtggcctgaaaacagagctccagcccctggttcgtgtctccctctgcatagcccagggcccaggcaagcggaacccctacatccacgacagcgccacgggcccgaggga

SEQ ID NO: 9917 - RNA, 209 nt, Homo sapiens
  source 1..209: mol_type = other RNA
caacctcgacgatctcctcagctggtcaggtggcctgaaaacagagctccagcccctggttcgtgtctccctctgcatagcccagggcccaggcaagcggaacccctacatccacgacagcgccacgggcccgagggacgaggacctgcctctctggcccacccgggcctcgcgcccggagggcggagccacagccgcgccgggaaact

SEQ ID NO: 9918 - RNA, 885 nt, Homo sapiens
  source 1..885: mol_type = other RNA
caacctcgacgatctcctcagctggtcaggtggcctgaaaacagagctccagccctggggcagacaaacctgggtgatgactcagctccccctcctagctgtgtgacctcgggcaagtttacctctctgagccttggtgtccctgggccagataaacatgaggaggccaggaccatcggggccgactggtggaatgcccgatgggggcactccccactggccacccatcagtaaagctgtgtgccctttcccaggcaccctgggacccaggacaacagcatgaccaggaggagcgcaggcccagggtggctctcatcaccctgctatcactcccagcagcaaaggagtaaccccaatgcagaaacccagggtacaggccctgcttccccagccactccccaccctttcccctgcctccagaagctggcttttctccccaaccattctgtgggccttccatatcttgactcctctaatccttccaacaatgctctgacgtaggcacacgtgttacctcgtctgtccattttacagacgagatagatgaggcacatactgaccaagagccaagcccctggccaccatcctgcactcgcccacgttccagcccagggtcaggagagggtgtgaaaataggcacattcagtcagcgcttacaaagcacggcgcgcttcatgtatttaaaaaataaaatgtgtgcctgtcaaaaagggagacaggacagtaaacatgattcctggcgtccgctatgtaggctctgagtggcaagtcacagatctaactgttcaagcgcagagatcaatttcaacaaaggaagacgcgagcgcctcctgctgggcagagcccccgcgcccgggaacccgggacgctccccgctccccggtc

SEQ ID NO: 9919 - RNA, 886 nt, Homo sapiens
  source 1..886: mol_type = other RNA
caacctcgacgatctcctcagctggtcaggtggcctgaaaacagagctccagccctggggcagacaaacctgggtgatgactcagctccccctcctagctgtgtgacctcgggcaagtttacctctctgagccttggtgtccctgggccagataaacatgaggaggccaggaccatcggggccgactggtggaatgcccgatgggggcactccccactggccacccatcagtaaagctgtgtgccctttcccaggcaccctgggacccaggacaacagcatgaccaggaggagcgcaggcccagggtggctctcatcaccctgctatcactcccagcagcaaaggagtaaccccaatgcagaaacccagggtacaggccctgcttccccagccactccccaccctttcccctgcctccagaagctggcttttctccccaaccattctgtgggccttccatatcttgactcctctaatccttccaacaatgctctgacgtaggcacacgtgttacctcgtctgtccattttacagacgagatagatgaggcacatactgaccaagagccaagcccctggccaccatcctgcactcgcccacgttccagcccagggtcaggagagggtgtgaaaataggcacattcagtcagcgcttacaaagcacggcgcgcttcatgtatttaaaaaataaaatgtgtgcctgtcaaaaagggagacaggacagtaaacatgattcctggcgtccgctatgtaggctctgagtggcaagtcacagatctaactgttcaagcgcagagatcaatttcaacaaaggaagacgcgagcgcctcctgctgggcagagcccccgcgcccgggaacccgggacgctccccgctccccggtcc

SEQ ID NO: 9920 - RNA, 887 nt, Homo sapiens
  source 1..887: mol_type = other RNA
caacctcgacgatctcctcagctggtcaggtggcctgaaaacagagctccagccctggggcagacaaacctgggtgatgactcagctccccctcctagctgtgtgacctcgggcaagtttacctctctgagccttggtgtccctgggccagataaacatgaggaggccaggaccatcggggccgactggtggaatgcccgatgggggcactccccactggccacccatcagtaaagctgtgtgccctttcccaggcaccctgggacccaggacaacagcatgaccaggaggagcgcaggcccagggtggctctcatcaccctgctatcactcccagcagcaaaggagtaaccccaatgcagaaacccagggtacaggccctgcttccccagccactccccaccctttcccctgcctccagaagctggcttttctccccaaccattctgtgggccttccatatcttgactcctctaatccttccaacaatgctctgacgtaggcacacgtgttacctcgtctgtccattttacagacgagatagatgaggcacatactgaccaagagccaagcccctggccaccatcctgcactcgcccacgttccagcccagggtcaggagagggtgtgaaaataggcacattcagtcagcgcttacaaagcacggcgcgcttcatgtatttaaaaaataaaatgtgtgcctgtcaaaaagggagacaggacagtaaacatgattcctggcgtccgctatgtaggctctgagtggcaagtcacagatctaactgttcaagcgcagagatcaatttcaacaaaggaagacgcgagcgcctcctgctgggcagagcccccgcgcccgggaacccgggacgctccccgctccccggtccc

SEQ ID NO: 9921 - RNA, 888 nt, Homo sapiens
  source 1..888: mol_type = other RNA
caacctcgacgatctcctcagctggtcaggtggcctgaaaacagagctccagccctggggcagacaaacctgggtgatgactcagctccccctcctagctgtgtgacctcgggcaagtttacctctctgagccttggtgtccctgggccagataaacatgaggaggccaggaccatcggggccgactggtggaatgcccgatgggggcactccccactggccacccatcagtaaagctgtgtgccctttcccaggcaccctgggacccaggacaacagcatgaccaggaggagcgcaggcccagggtggctctcatcaccctgctatcactcccagcagcaaaggagtaaccccaatgcagaaacccagggtacaggccctgcttccccagccactccccaccctttcccctgcctccagaagctggcttttctccccaaccattctgtgggccttccatatcttgactcctctaatccttccaacaatgctctgacgtaggcacacgtgttacctcgtctgtccattttacagacgagatagatgaggcacatactgaccaagagccaagcccctggccaccatcctgcactcgcccacgttccagcccagggtcaggagagggtgtgaaaataggcacattcagtcagcgcttacaaagcacggcgcgcttcatgtatttaaaaaataaaatgtgtgcctgtcaaaaagggagacaggacagtaaacatgattcctggcgtccgctatgtaggctctgagtggcaagtcacagatctaactgttcaagcgcagagatcaatttcaacaaaggaagacgcgagcgcctcctgctgggcagagcccccgcgcccgggaacccgggacgctccccgctccccggtcccc

SEQ ID NO: 9922 - RNA, 69 nt, Homo sapiens
  source 1..69: mol_type = other RNA
caacctcgaggatctccccagccttggcgttcaggtgctgaggagatcgtcgaggttggcctgcttccc

SEQ ID NO: 9923 - RNA, 3316 nt, Homo sapiens
  source 1..3316: mol_type = other RNA
caacctggaggactccatgctggcctgagtggctgctctgccaagactccacatagctctgtgtattagactgaagactgaaagccctggtggagtgggttcacaaggagatctcctgacttgagggttgcaaagacctaatgctcaccccttctgttcctttccatgacagccacacacactagctgcttctggtcagccatcttgcccactcctccacttctcctctagttttcttaaggtttgaattggcattcttttttcaatttttttctgattcacagctttgttactttattgtatttcttttcaaaagattgttacttctgattttagctttggctacatctcataaatattgctttattttattcatatgtaccttgtatattaataagcaatttggcaccttatacattaaggggtattgaagaagggaggaggctttgatatctgcaatgttagtttggattcccaccccttcacttactagctgtgtttctgaatttctctggcctaagtttattcatctgtgaagttggtataacagtaaaacttagctcaactgaaaccatttaaattctttgaacatagaaagcacttaataaataataatacatgattcacgtatagcgtttattatatgctggggtccctattctgagttttgaataagtatcagctcaataatcctaaacaactccaaaatagatatataatatctcaattttacaaatgagaaaactgaggcacaaaagattgtgtggcttgcccagcatcacacaccttgggggtggcagagcctgaattttacgccaggcagtttggacaaggagaaaatttttaattttaaattatgaagtatattggttaactactgctgtataacaaactgcaaaatccagtgctgactgcaacattcatttattatcactcacatatcctcagatcatctggagatcagctgggactggctgatgtagagtaggcttaaatgcatgacttctctgaacatgactgcaggttagcttgtctaggttgagcttgactgaaatatatttgacccatgtttctttcatcctctcctggattcaatagttacccagtcaaacaagagtaaattttctaaatttaatgggggagaaaaagaaagtttgagtcccacagtatcagatgttgctattggctgtgaactttgaatatcatctccattataatttcccactagactctagatacaagaaatcaaatcatcagactcataagtaaatatgattgcaggaaccatatccttgtttctatcccacttcatgattaaaatcacctccttctttcttatgctacagctggtgtaggcaaggaaattgccaaaaatgtattagatgattagctgagagaggtcttaggcaaactgcagctatctcatgttgctctttcttaaagacacaaccaggccaatatattgcttttttttccctttccaatggcagaacccctctgtctgtttattctttcccatccagaaacacagaataaacaatggttaccaccatgtctttattatgctgtatcagcatatatgggagatgatgtttctgaactcctgggggtctgtgccaggcctcatttctgtagtggcaaagtcctaacattgagccatctttgatctgagaagccacaggaaacaaaagatttctaaatcttgttgtttcacaaataattttggacaaattcataaatgatgaggccacattatttatcctgatgtaggataaaaataatgaacctccaggacctaaagatcctgatgtctgtggcattgagtcatctgttggtccatattggcatattttgtgcatcaaatcaagccttctttgtccaaaggcagtaggcagcatgaattttgttatagtccattcattatcatattttgtgggttagggagattctgatgggccatatctggcagaaatctcagaatctgtaaactcagcagcactttctcttttgcaacctctttaaggcatctttaatttctttgttcctcaaactgtaaatcaagggatttaacatgggaatgaccacagtgtagaaaacagatgcaaatctgtcaaagcttgaagaacctccagagctggaactcaaatagacaaagattcctgatgtatagaagagggaaacagctgttagatgagaagcacaggtgttgaatgccttggacctgcctttagctgaagtgatcttcatgatggagatgccaatatagccataggatatcatgataactagggcacttgctatcccaaagaacatggttaatatagcagtcatgacctgtacaaagaaagtgtcagtacaggacaagattaacagttggggcatgtcacagaagaaatgtctgatgacattagacccacagaagtggagttgaagcaaagcaccaatttggaataaagaagcagtgaggccagtcatgtaggctcccagtaccatccaaacacagagggtgggtgacatgatggatgaatagagcagggggttacaaatggcagcataacgatcataagccatggctgtcatgagacaagactcactcagtcccatcgttgaaaagataaagtactgaataatacaaccaacaaaagtgatagtttgctgttcctgtaagaggttggagagcatcttggggactgtggagctgatatagcagacatctatgaaggacaggttactgaggaagaaatacatgggtgtatggaggtgggaatccatccttattaaaacaatgagggagaggttccaggccagagatgtaatgtagatcaccaggaatatagtgaagagcacttttatgatcctgggaaaatctgagaatcccagcaggatgaaataggtgatttctgtaatatttcctcccccagtcattggctcagtgctcctgaaattttatgtttgaggtttttctttttacagaaggttgagtaaggagtaagagaatccaacgaagagctttaggtacagaatgtggaagtgaggaagtgggaagagttgaagaatgagagagactgaggaccataaactctgttccatgtgtatccttactggaagaattacatggatattgagacggtacagaatccactgttctaagtcttgtcctgtgacctttacccaggtcctccaagaagacagggttcttgccaaaggttgaaattgcttatttcttttccaatggaatttttcaggtgggcgtatcacactccaagatgggcatgtttgaccacaaaattggctgtccactcacagcaagagagat

SEQ ID NO: 9924 - RNA, 2967 nt, Homo sapiens
  source 1..2967: mol_type = other RNA
caacggaatcccaaaagcagctgatattggacaaactcaagaacataaaaagttttcaaactcctccataagaaggtgtccccaaaaatattatgtttgagcagttaaatgtaagaaaaaatccttcaaaactagtatttgtttttatgaaaaaccttgaaaacaaataaaaacagagaggaggaggcaagagataacaaggttaggatattaaatgatgtaagaccttgacctaaagcagaattatctataattacaagttggttaaaaaattagcagaataggaattttttaaaggcttaagcagttgtctacagcaaacttgtttttgggattaaataatcccaatgtgaaggatctatctatagagtgaagcatgttttccaaaatgtaagaattttaaaaagactgaatatttgtgtcttgagaatttcctaaaagcagccagttttgtcagtttacaaagcttaatactccttggggtgacgttgcacaaatttctgtgtttgtgtgacaaaaagaaagagcaagaaatagaaaagttcagtatcgaaatggcctgttgtctacattgactttaatttaatacattgctaaattatgtccacaaaggagccatcatctttcaataggtctatgaaaatgtggaaaaatagtgtagcggcatggaactgggtaagtacaaggttactgggcctagttttaatacatatttatatacacacacattcacgcccctacgcatatacacttcagtaacttaatattcttctcattaatttagtttcactcattcccttttggacattgagattttttgcaattataacatttgaaagataaaagaattatactgctggggccacagattataataggtgcattcagtgaactcttatcttctgaaaagtggccttgcttgttggtacagataggacttcagctattaacaccaagtctcacaagatggcctggaaggaggtgcagagttcaaagacagtccaagcaattctcagaagaggcgtgctcagaattcttaggataactggttcttaaaatatcttcttccaagaaccacaaaggtcagagttatgatatagatgtttatagtttatgaaagtgaccattttttaaaagcagcagcaatttgtttagggaaaggacaggataccatgttgggagtgcaccatagctagaggcattgtggcccacggagaatcactgggagatgagatggtagaaggttcctctcagtgtttttcaagatgtgactcacagatgggtgtaccctttggtatcgctcctactccaaccagcttagctggatgaaatcatctgcatgttaccagtgcatacctgtccgtgatcgttttctctgttttttacaaaggcaatagataggaaatacaaataaacacttgtttcaggcagtatagcatatcacttaacaacacaggctgtggagccaaatgttgggtttgattcctggttctaccacttatgaggttccagtaagtcttaatttcctcaacgattacaaccgctatggcccctagtgccaatcccaaaaccataattagaggtgcaatgaataattttccagcacagactgaccctcgcactaatctccttaaatgaggtctctctgggaggtagcgatatttgcatccaaatatactgaggtttgatgtgtggtctccaaaaaatcggagctggcggtatctctcaccacatcggtaacaaaaattagtgttacattgtgagcaggtcatatggtcacatccttcagttcgctggatgtggatcttgcactttggacacttctgggcattcctctgcccatgctcaatttcgctggcccagtgacgcaacaatttgtctccttttttgtactccttgcagttaacaccttcatgccaaggagagtggcacttaaaacaccagacgaattggcaggtagggcactggatctgggcgctcaggtagactttgaggcactcctcgcacacggccttcttgcagcaaggcaggggcttgatgggcttgtcttccaggcacacccggcacatcagcaccatgaggggcacatagggatcccctacaccgcccaggccagagtagggtggagctcccaacaggctgggcatggagaacggctcgggcgccaggtagaactccagctcgatgctgccgccgtcgggggagagggaatccgttgggagggacagtcgggggctggggaaggaagagcgggtgctgggagggttcaacactggcggagccccaggtggcgacgcgggcggcgagagctgctccgaggcgggggcctcgggcaggtcgctctccacgcagtacacggagcagaagacttgtctcttggcgagggacgggcgccgctgacccagcacgtccaggaccagtccgtcggcggcccccacgcgggtcctgggctccagctcttcgccggggggcgcctcctgctgttcatcccctccctcttttcgatccccagcttcctcctcttcctcctccagctccaactgcagtggcaaggtctggggattgagaggcccggtgagtgccagtcccgcaggctgcgccggtgctcggctcttactccagcccgggggccccaggctcctcgcgggctctggggcgctggtgtccgcgcagccccagtcgcttccgcagccaccgccgctcggctccgcggaggcggcgcgcagcgggggcgcccgggcgctgtccccctgaggcctcgggggctcagggtggcccgcagtgccactggccagggtctgcgactcctggggcccgccgccgccgctcaccgtgctctgctcctcgcccatcgccgcccgcggcccgcgccgccgctgcccatccagccgccgggacccccacccggcgcccgcgggcagcgggggcagtggctcggctcgactcgcggctccgcttctgcttccg

SEQ ID NO: 9925 - RNA, 3193 nt, Homo sapiens
  source 1..3193: mol_type = other RNA
caacggaatcccaaaagcagctgatattggacaaactcaagaacataaaaagttttcaaactcctccataagaaggtgtccccaaaaatattatgtttgagcagttaaatgtaagaaaaaatccttcaaaactagtatttgtttttatgaaaaaccttgaaaacaaataaaaacagagaggaggaggcaagagataacaaggttaggatattaaatgatgtaagaccttgacctaaagcagaattatctataattacaagttggttaaaaaattagcagaataggaattttttaaaggcttaagcagttgtctacagcaaacttgtttttgggattaaataatcccaatgtgaaggatctatctatagagtgaagcatgttttccaaaatgtaagaattttaaaaagactgaatatttgtgtcttgagaatttcctaaaagcagccagttttgtcagtttacaaagcttaatactccttggggtgacgttgcacaaatttctgtgtttgtgtgacaaaaagaaagagcaagaaatagaaaagttcagtatcgaaatggcctgttgtctacattgactttaatttaatacattgctaaattatgtccacaaaggagccatcatctttcaataggtctatgaaaatgtggaaaaatagtgtagcggcatggaactgggtaagtacaaggttactgggcctagttttaatacatatttatatacacacacattcacgcccctacgcatatacacttcagtaacttaatattcttctcattaatttagtttcactcattcccttttggacattgagattttttgcaattataacatttgaaagataaaagaattatactgctggggccacagattataataggtgcattcagtgaactcttatcttctgaaaagtggccttgcttgttggtacagataggacttcagctattaacaccaagtctcacaagatggcctggaaggaggtgcagagttcaaagacagtccaagcaattctcagaagaggcgtgctcagaattcttaggataactggttcttaaaatatcttcttccaagaaccacaaaggtcagagttatgatatagatgtttatagtttatgaaagtgaccattttttaaaagcagcagcaatttgtttagggaaaggacaggataccatgttgggagtgcaccatagctagaggcattgtggcccacggagaatcactgggagatgagatggtagaaggttcctctcagtgtttttcaagatgtgactcacagatgggtgtaccctttggtatcgctcctactccaaccagcttagctggatgaaatcatctgcatgttaccagtgcatacctgtccgtgatcgttttctctgttttttacaaaggcaatagataggaaatacaaataaacacttgtttcaggcagtatagcatatcacttaacaacacaggctgtggagccaaatgttgggtttgattcctggttctaccacttatgaggttccagtaagtcttaatttcctcaacgattacaaccgctatggcccctagtgccaatcccaaaaccataattagaggtgcaatgaataattttccagcacagactgaccctcgcactaatctccttaaatgaggtctctctgggaggtagcgatatttgcatccaaatatactgaggtttgatgtgtggtctccaaaaaatcggagctggcggtatctctcaccacatcggtaacaaaaattagtgttacattgtgagcaggtcatatggtcacatccttcagttcgctggatgtggatcttgcactttggacacttctgggcattcctctgcccatgctcaatttcgctggcccagtgacgcaacaatttgtctccttttttgtactccttgcagttaacaccttcatgccaaggagagtggcacttaaaacaccagacgaattggcaggtagggcactggattttgtatttgctttctgatctggaaggggtgggaatatgtccttttttcttgaaggttgtaaagtgcttgcactgaggacatggcttggtgctggaatcaatacggccaagttccaagaagtacttatacttgatggagtcttcatgcgttaagttatagacaacagttgtttcttccaagaattcaaaacactctgtgatggggcatttgatttctacttggccaagttgtacctgggcgctcaggtagactttgaggcactcctcgcacacggccttcttgcagcaaggcaggggcttgatgggcttgtcttccaggcacacccggcacatcagcaccatgaggggcacatagggatcccctacaccgcccaggccagagtagggtggagctcccaacaggctgggcatggagaacggctcgggcgccaggtagaactccagctcgatgctgccgccgtcgggggagagggaatccgttgggagggacagtcgggggctggggaaggaagagcgggtgctgggagggttcaacactggcggagccccaggtggcgacgcgggcggcgagagctgctccgaggcgggggcctcgggcaggtcgctctccacgcagtacacggagcagaagacttgtctcttggcgagggacgggcgccgctgacccagcacgtccaggaccagtccgtcggcggcccccacgcgggtcctgggctccagctcttcgccggggggcgcctcctgctgttcatcccctccctcttttcgatccccagcttcctcctcttcctcctccagctccaactgcagtggcaaggtctggggattgagaggcccggtgagtgccagtcccgcaggctgcgccggtgctcggctcttactccagcccgggggccccaggctcctcgcgggctctggggcgctggtgtccgcgcagccccagtcgcttccgcagccaccgccgctcggctccgcggaggcggcgcgcagcgggggcgcccgggcgctgtccccctgaggcctcgggggctcagggtggcccgcagtgccactggccagggtctgcgactcctggggcccgccgccgccgctcaccgtgctctgctcctcgcccatcgccgcccgcggcccgcgccgccgctgcccatccagccgccgggacccccacccggcgcccgcgggcagcgggggcagtggctcggctcgactcgcggctccgcttc

SEQ ID NO: 9926 - RNA, 2548 nt, Homo sapiens
  source 1..2548: mol_type = other RNA
caacggaatcccaaaagcagctgatattggacaaactcaagaacataaaaagttttcaaactcctccataagaaggtgtccccaaaaatattatgtttgagcagttaaatgtaagaaaaaatccttcaaaactagtatttgtttttatgaaaaaccttgaaaacaaataaaaacagagaggaggaggcaagagataacaaggttaggatattaaatgatgtaagaccttgacctaaagcagaattatctataattacaagttggttaaaaaattagcagaataggaattttttaaaggcttaagcagttgtctacagcaaacttgtttttgggattaaataatcccaatgtgaaggatctatctatagagtgaagcatgttttccaaaatgtaagaattttaaaaagactgaatatttgtgtcttgagaatttcctaaaagcagccagttttgtcagtttacaaagcttaatactccttggggtgacgttgcacaaatttctgtgtttgtgtgacaaaaagaaagagcaagaaatagaaaagttcagtatcgaaatggcctgttgtctacattgactttaatttaatacattgctaaattatgtccacaaaggagccatcatctttcaataggtctatgaaaatgtggaaaaatagtgtagcggcatggaactgggtaagtacaaggttactgggcctagttttaatacatatttatatacacacacattcacgcccctacgcatatacacttcagtaacttaatattcttctcattaatttagtttcactcattcccttttggacattgagattttttgcaattataacatttgaaagataaaagaattatactgctggggccacagattataataggtgcattcagtgaactcttatcttctgaaaagtggccttgcttgttggtacagataggacttcagctattaacaccaagtctcacaagatggcctggaaggaggtgcagagttcaaagacagtccaagcaattctcagaagaggcgtgctcagaattcttaggataactggttcttaaaatatcttcttccaagaaccacaaaggtcagagttatgatatagatgtttatagtttatgaaagtgaccattttttaaaagcagcagcaatttgtttagggaaaggacaggataccatgttgggagtgcaccatagctagaggcattgtggcccacggagaatcactgggagatgagatggtagaaggttcctctcagtgtttttcaagatgtgactcacagatgggtgtaccctttggtatcgctcctactccaaccagcttagctggatgaaatcatctgcatgttaccagtgcatacctgtccgtgatcgttttctctgttttttacaaaggcaatagataggaaatacaaataaacacttgtttcaggcagtatagcatatcacttaacaacacaggctgtggagccaaatgttgggtttgattcctggttctaccacttatgaggttccagtaagtcttaatttcctcaacgattacaaccgctatggcccctagtgccaatcccaaaaccataattagaggtgcaatgaataattttccagcacagactgaccctcgcactaatctccttaaatgaggtctctctgggaggtagcgatatttgcatccaaatatactgaggtttgatgtgtggtctccaaaaaatcggagctggcggtatctctcaccacatcggtaacaaaaattagtgttacattgtgagcaggtcatatggtcacatccttcagttcgctggatgtggatcttgcactttggacacttctgggcattcctctgcccatgctcaatttcgctggcccagtgacgcaacaatttgtctccttttttgtactccttgcagttaacaccttcatgccaaggagagtggcacttaaaacaccagacgaattggcaggtagggcactggattttgtatttgctttctgatctggaaggggtgggaatatgtccttttttcttgaaggttgtaaagtgcttgcactgaggacatggcttggtgctggaatcaatacggccaagttccaagaagtacttatacttgatggagtcttcatgcgttaagttatagacaacagttgtttcttccaagaattcaaaacactctgtgatggggcatttgatttctacttggccaagttgtaccttcatccctttcttgaactggtttatgggtgtggatgagaagagaactaattatacaacagctttgattctcctactctttatctttactcaagtgctggcaatggacactgtatatgcttcaggttacacaaaacttgactcttcccctcattatgaagtttgccttcaagagccaatgtcaacagagctttaattatataacctgtaaggtccttttcattagtgacaagtgaggacataaatccactaaaccatcactcaggctctaaattcacatttgtcctgaccatatttcactctctaccttaatcttctcatgtttgtgtcctcctctgtatact

SEQ ID NO: 9927 - RNA, 2321 nt, Homo sapiens
  source 1..2321: mol_type = other RNA
caacggaatcccaaaagcagctgatattggacaaactcaagaacataaaaagttttcaaactcctccataagaaggtgtccccaaaaatattatgtttgagcagttaaatgtaagaaaaaatccttcaaaactagtatttgtttttatgaaaaaccttgaaaacaaataaaaacagagaggaggaggcaagagataacaaggttaggatattaaatgatgtaagaccttgacctaaagcagaattatctataattacaagttggttaaaaaattagcagaataggaattttttaaaggcttaagcagttgtctacagcaaacttgtttttgggattaaataatcccaatgtgaaggatctatctatagagtgaagcatgttttccaaaatgtaagaattttaaaaagactgaatatttgtgtcttgagaatttcctaaaagcagccagttttgtcagtttacaaagcttaatactccttggggtgacgttgcacaaatttctgtgtttgtgtgacaaaaagaaagagcaagaaatagaaaagttcagtatcgaaatggcctgttgtctacattgactttaatttaatacattgctaaattatgtccacaaaggagccatcatctttcaataggtctatgaaaatgtggaaaaatagtgtagcggcatggaactgggtaagtacaaggttactgggcctagttttaatacatatttatatacacacacattcacgcccctacgcatatacacttcagtaacttaatattcttctcattaatttagtttcactcattcccttttggacattgagattttttgcaattataacatttgaaagataaaagaattatactgctggggccacagattataataggtgcattcagtgaactcttatcttctgaaaagtggccttgcttgttggtacagataggacttcagctattaacaccaagtctcacaagatggcctggaaggaggtgcagagttcaaagacagtccaagcaattctcagaagaggcgtgctcagaattcttaggataactggttcttaaaatatcttcttccaagaaccacaaaggtcagagttatgatatagatgtttatagtttatgaaagtgaccattttttaaaagcagcagcaatttgtttagggaaaggacaggataccatgttgggagtgcaccatagctagaggcattgtggcccacggagaatcactgggagatgagatggtagaaggttcctctcagtgtttttcaagatgtgactcacagatgggtgtaccctttggtatcgctcctactccaaccagcttagctggatgaaatcatctgcatgttaccagtgcatacctgtccgtgatcgttttctctgttttttacaaaggcaatagataggaaatacaaataaacacttgtttcaggcagtatagcatatcacttaacaacacaggctgtggagccaaatgttgggtttgattcctggttctaccacttatgaggttccagtaagtcttaatttcctcaacgattacaaccgctatggcccctagtgccaatcccaaaaccataattagaggtgcaatgaataattttccagcacagactgaccctcgcactaatctccttaaatgaggtctctctgggaggtagcgatatttgcatccaaatatactgaggtttgatgtgtggtctccaaaaaatcggagctggcggtatctctcaccacatcggtaacaaaaattagtgttacattgtgagcaggtcatatggtcacatccttcagttcgctggatgtggatcttgcactttggacacttctgggcattcctctgcccatgctcaatttcgctggcccagtgacgcaacaatttgtctccttttttgtactccttgcagttaacaccttcatgccaaggagagtggcacttaaaacaccagacgaattggcaggtagggcactggattttgtatttgctttctgatctggaaggggtgggaatatgtccttttttcttgaaggttgtaaagtgcttgcactgaggacatggcttggtgctggaatcaatacggccaagttccaagaagtacttatacttgatggagtcttcatgcgttaagttatagacaacagttgtttcttccaagaattcaaaacactctgtgatggggcatttgatttctacttggccaagttgtaccttgtattgttcttttgtacacatctgctctcacagtgacttccctggaggcgggcttatattttggaaatgtctgaatcccatcgcagggcagcgaaatctgttttgaggatgatg

SEQ ID NO: 9928 - RNA, 3145 nt, Homo sapiens
  source 1..3145: mol_type = other RNA
caacggaatcccaaaagcagctgatattggacaaactcaagaacataaaaagttttcaaactcctccataagaaggtgtccccaaaaatattatgtttgagcagttaaatgtaagaaaaaatccttcaaaactagtatttgtttttatgaaaaaccttgaaaacaaataaaaacagagaggaggaggcaagagataacaaggttaggatattaaatgatgtaagaccttgacctaaagcagaattatctataattacaagttggttaaaaaattagcagaataggaattttttaaaggcttaagcagttgtctacagcaaacttgtttttgggattaaataatcccaatgtgaaggatctatctatagagtgaagcatgttttccaaaatgtaagaattttaaaaagactgaatatttgtgtcttgagaatttcctaaaagcagccagttttgtcagtttacaaagcttaatactccttggggtgacgttgcacaaatttctgtgtttgtgtgacaaaaagaaagagcaagaaatagaaaagttcagtatcgaaatggcctgttgtctacattgactttaatttaatacattgctaaattatgtccacaaaggagccatcatctttcaataggtctatgaaaatgtggaaaaatagtgtagcggcatggaactgggtaagtacaaggttactgggcctagttttaatacatatttatatacacacacattcacgcccctacgcatatacacttcagtaacttaatattcttctcattaatttagtttcactcattcccttttggacattgagattttttgcaattataacatttgaaagataaaagaattatactgctggggccacagattataataggtgcattcagtgaactcttatcttctgaaaagtggccttgcttgttggtacagataggacttcagctattaacaccaagtctcacaagatggcctggaaggaggtgcagagttcaaagacagtccaagcaattctcagaagaggcgtgctcagaattcttaggataactggttcttaaaatatcttcttccaagaaccacaaaggtcagagttatgatatagatgtttatagtttatgaaagtgaccattttttaaaagcagcagcaatttgtttagggaaaggacaggataccatgttgggagtgcaccatagctagaggcattgtggcccacggagaatcactgggagatgagatggtagaaggttcctctcagtgtttttcaagatgtgactcacagatgggtgtaccctttggtatcgctcctactccaaccagcttagctggatgaaatcatctgcatgttaccagtgcatacctgtccgtgatcgttttctctgttttttacaaaggcaatagataggaaatacaaataaaccgattacaaccgctatggcccctagtgccaatcccaaaaccataattagaggtgcaatgaataattttccagcacagactgaccctcgcactaatctccttaaatgaggtctctctgggaggtagcgatatttgcatccaaatatactgaggtttgatgtgtggtctccaaaaaatcggagctggcggtatctctcaccacatcggtaacaaaaattagtgttacattgtgagcaggtcatatggtcacatccttcagttcgctggatgtggatcttgcactttggacacttctgggcattcctctgcccatgctcaatttcgctggcccagtgacgcaacaatttgtctccttttttgtactccttgcagttaacaccttcatgccaaggagagtggcacttaaaacaccagacgaattggcaggtagggcactggatcttaaatggagatgactccaaacagcctttgaaaccacttcatcctgccattttgtttgtatttgctttctgatctggaaggggtgggaatatgtccttttttcttgaaggttgtaaagtgcttgcactgaggacatggcttggtgctggaatcaatacggccaagttccaagaagtacttatacttgatggagtcttcatgcgttaagttatagacaacagttgtttcttccaagaattcaaaacactctgtgatggggcatttgatttctacttggccaagttgtacctgggcgctcaggtagactttgaggcactcctcgcacacggccttcttgcagcaaggcaggggcttgatgggcttgtcttccaggcacacccggcacatcagcaccatgaggggcacatagggatcccctacaccgcccaggccagagtagggtggagctcccaacaggctgggcatggagaacggctcgggcgccaggtagaactccagctcgatgctgccgccgtcgggggagagggaatccgttgggagggacagtcgggggctggggaaggaagagcgggtgctgggagggttcaacactggcggagccccaggtggcgacgcgggcggcgagagctgctccgaggcgggggcctcgggcaggtcgctctccacgcagtacacggagcagaagacttgtctcttggcgagggacgggcgccgctgacccagcacgtccaggaccagtccgtcggcggcccccacgcgggtcctgggctccagctcttcgccggggggcgcctcctgctgttcatcccctccctcttttcgatccccagcttcctcctcttcctcctccagctccaactgcagtggcaaggtctggggattgagaggcccggtgagtgccagtcccgcaggctgcgccggtgctcggctcttactccagcccgggggccccaggctcctcgcgggctctggggcgctggtgtccgcgcagccccagtcgcttccgcagccaccgccgctcggctccgcggaggcggcgcgcagcgggggcgcccgggcgctgtccccctgaggcctcgggggctcagggtggcccgcagtgccactggccagggtctgcgactcctggggcccgccgccgccgctcaccgtgctctgctcctcgcccatcgccgcccgcggcccgcgccgccgctgcccatccagccgccgggacccccacccggcgcccgcgggcagcgggggcagtggctcggctcgactcgcggctccgcttctgcttccgggtc

SEQ ID NO: 9929 - RNA, 2324 nt, Homo sapiens
  source 1..2324: mol_type = other RNA
caacggaatcccaaaagcagctgatattggacaaactcaagaacataaaaagttttcaaactcctccataagaaggtgtccccaaaaatattatgtttgagcagttaaatgtaagaaaaaatccttcaaaactagtatttgtttttatgaaaaaccttgaaaacaaataaaaacagagaggaggaggcaagagataacaaggttaggatattaaatgatgtaagaccttgacctaaagcagaattatctataattacaagttggttaaaaaattagcagaataggaattttttaaaggcttaagcagttgtctacagcaaacttgtttttgggattaaataatcccaatgtgaaggatctatctatagagtgaagcatgttttccaaaatgtaagaattttaaaaagactgaatatttgtgtcttgagaatttcctaaaagcagccagttttgtcagtttacaaagcttaatactccttggggtgacgttgcacaaatttctgtgtttgtgtgacaaaaagaaagagcaagaaatagaaaagttcagtatcgaaatggcctgttgtctacattgactttaatttaatacattgctaaattatgtccacaaaggagccatcatctttcaataggtctatgaaaatgtggaaaaatagtgtagcggcatggaactgggtaagtacaaggttactgggcctagttttaatacatatttatatacacacacattcacgcccctacgcatatacacttcagtaacttaatattcttctcattaatttagtttcactcattcccttttggacattgagattttttgcaattataacatttgaaagataaaagaattatactgctggggccacagattataataggtgcattcagtgaactcttatcttctgaaaagtggccttgcttgttggtacagataggacttcagctattaacaccaagtctcacaagatggcctggaaggaggtgcagagttcaaagacagtccaagcaattctcagaagaggcgtgctcagaattcttaggataactggttcttaaaatatcttcttccaagaaccacaaaggtcagagttatgatatagatgtttatagtttatgaaagtgaccattttttaaaagcagcagcaatttgtttagggaaaggacaggataccatgttgggagtgcaccatagctagaggcattgtggcccacggagaatcactgggagatgagatggtagaaggttcctctcagtgtttttcaagatgtgactcacagatgggtgtaccctttggtatcgctcctactccaaccagcttagctggatgaaatcatctgcatgttaccagtgcatacctgtccgtgatcgttttctctgttttttacaaaggcaatagataggaaatacaaataaaccgattacaaccgctatggcccctagtgccaatcccaaaaccataattagaggtgcaatgaataattttccagcacagactgaccctcgcactaatctccttaaatgaggtctctctgggaggtagcgatatttgcatccaaatatactgaggtttgatgtgtggtctccaaaaaatcggagctggcggtatctctcaccacatcggtaacaaaaattagtgttacattgtgagcaggtcatatggtcacatccttcagttcgctggatgtggatcttgcactttggacacttctgggcattcctctgcccatgctcaatttcgctggcccagtgacgcaacaatttgtctccttttttgtactccttgcagttaacaccttcatgccaaggagagtggcacttaaaacaccagacgaattggcaggtagggcactggattttgtatttgctttctgatctggaaggggtgggaatatgtccttttttcttgaaggttgtaaagtgcttgcactgaggacatggcttggtgctggaatcaatacggccaagttccaagaagtacttatacttgatggagtcttcatgcgttaagttatagacaacagttgtttcttccaagaattcaaaacactctgtgatggggcatttgatttctacttggccaagttgtacactgtatatgcttcaggttacacaaaacttgactcttcccctcattatgaagtttgccttcaagagccaatgtcaacagagctttaattatataacctgtaaggtccttttcattagtgacaagtgaggacataaatccactaaaccatcactcaggctctaaattcacatttgtcctgaccatatttcactctctaccttaatcttctcatgtttgtgtcctcctctgtatact

SEQ ID NO: 9930 - RNA, 3079 nt, Homo sapiens
  source 1..3079: mol_type = other RNA
caacggaatcccaaaagcagctgatattggacaaactcaagaacataaaaagttttcaaactcctccataagaaggtgtccccaaaaatattatgtttgagcagttaaatgtaagaaaaaatccttcaaaactagtatttgtttttatgaaaaaccttgaaaacaaataaaaacagagaggaggaggcaagagataacaaggttaggatattaaatgatgtaagaccttgacctaaagcagaattatctataattacaagttggttaaaaaattagcagaataggaattttttaaaggcttaagcagttgtctacagcaaacttgtttttgggattaaataatcccaatgtgaaggatctatctatagagtgaagcatgttttccaaaatgtaagaattttaaaaagactgaatatttgtgtcttgagaatttcctaaaagcagccagttttgtcagtttacaaagcttaatactccttggggtgacgttgcacaaatttctgtgtttgtgtgacaaaaagaaagagcaagaaatagaaaagttcagtatcgaaatggcctgttgtctacattgactttaatttaatacattgctaaattatgtccacaaaggagccatcatctttcaataggtctatgaaaatgtggaaaaatagtgtagcggcatggaactgggtaagtacaaggttactgggcctagttttaatacatatttatatacacacacattcacgcccctacgcatatacacttcagtaacttaatattcttctcattaatttagtttcactcattcccttttggacattgagattttttgcaattataacatttgaaagataaaagaattatactgctggggccacagattataataggtgcattcagtgaactcttatcttctgaaaagtggccttgcttgttggtacagataggacttcagctattaacaccaagtctcacaagatggcctggaaggaggtgcagagttcaaagacagtccaagcaattctcagaagaggcgtgctcagaattcttaggataactggttcttaaaatatcttcttccaagaaccacaaaggtcagagttatgatatagatgtttatagtttatgaaagtgaccattttttaaaagcagcagcaatttgtttagggaaaggacaggataccatgttgggagtgcaccatagctagaggcattgtggcccacggagaatcactgggagatgagatggtagaaggttcctctcagtgtttttcaagatgtgactcacagatgggtgtaccctttggtatcgctcctactccaaccagcttagctggatgaaatcatctgcatgttaccagtgcatacctgtccgtgatcgttttctctgttttttacaaaggcaatagataggaaatacaaataaaccgattacaaccgctatggcccctagtgccaatcccaaaaccataattagaggtgcaatgaataattttccagcacagactgaccctcgcactaatctccttaaatgaggtctctctgggaggtagcgatatttgcatccaaatatactgaggtttgatgtgtggtctccaaaaaatcggagctggcggtatctctcaccacatcggtaacaaaaattagtgttacattgtgagcaggtcatatggtcacatccttcagttcgctggatgtggatcttgcactttggacacttctgggcattcctctgcccatgctcaatttcgctggcccagtgacgcaacaatttgtctccttttttgtactccttgcagttaacaccttcatgccaaggagagtggcacttaaaacaccagacgaattggcaggtagggcactggattttgtatttgctttctgatctggaaggggtgggaatatgtccttttttcttgaaggttgtaaagtgcttgcactgaggacatggcttggtgctggaatcaatacggccaagttccaagaagtacttatacttgatggagtcttcatgcgttaagttatagacaacagttgtttcttccaagaattcaaaacactctgtgatggggcatttgatttctacttggccaagttgtacctgggcgctcaggtagactttgaggcactcctcgcacacggccttcttgcagcaaggcaggggcttgatgggcttgtcttccaggcacacccggcacatcagcaccatgaggggcacatagggatcccctacaccgcccaggccagagtagggtggagctcccaacaggctgggcatggagaacggctcgggcgccaggtagaactccagctcgatgctgccgccgtcgggggagagggaatccgttgggagggacagtcgggggctggggaaggaagagcgggtgctgggagggttcaacactggcggagccccaggtggcgacgcgggcggcgagagctgctccgaggcgggggcctcgggcaggtcgctctccacgcagtacacggagcagaagacttgtctcttggcgagggacgggcgccgctgacccagcacgtccaggaccagtccgtcggcggcccccacgcgggtcctgggctccagctcttcgccggggggcgcctcctgctgttcatcccctccctcttttcgatccccagcttcctcctcttcctcctccagctccaactgcagtggcaaggtctggggattgagaggcccggtgagtgccagtcccgcaggctgcgccggtgctcggctcttactccagcccgggggccccaggctcctcgcgggctctggggcgctggtgtccgcgcagccccagtcgcttccgcagccaccgccgctcggctccgcggaggcggcgcgcagcgggggcgcccgggcgctgtccccctgaggcctcgggggctcagggtggcccgcagtgccactggccagggtctgcgactcctggggcccgccgccgccgctcaccgtgctctgctcctcgcccatcgccgcccgcggcccgcgccgccgctgcccatccagccgccgggacccccacccggcgcccgcgggcagcgggggcagtggctcggctcgactcgcggctccgcttct

SEQ ID NO: 9931 - RNA, 3092 nt, Homo sapiens
  source 1..3092: mol_type = other RNA
caacggaatcccaaaagcagctgatattggacaaactcaagaacataaaaagttttcaaactcctccataagaaggtgtccccaaaaatattatgtttgagcagttaaatgtaagaaaaaatccttcaaaactagtatttgtttttatgaaaaaccttgaaaacaaataaaaacagagaggaggaggcaagagataacaaggttaggatattaaatgatgtaagaccttgacctaaagcagaattatctataattacaagttggttaaaaaattagcagaataggaattttttaaaggcttaagcagttgtctacagcaaacttgtttttgggattaaataatcccaatgtgaaggatctatctatagagtgaagcatgttttccaaaatgtaagaattttaaaaagactgaatatttgtgtcttgagaatttcctaaaagcagccagttttgtcagtttacaaagcttaatactccttggggtgacgttgcacaaatttctgtgtttgtgtgacaaaaagaaagagcaagaaatagaaaagttcagtatcgaaatggcctgttgtctacattgactttaatttaatacattgctaaattatgtccacaaaggagccatcatctttcaataggtctatgaaaatgtggaaaaatagtgtagcggcatggaactgggtaagtacaaggttactgggcctagttttaatacatatttatatacacacacattcacgcccctacgcatatacacttcagtaacttaatattcttctcattaatttagtttcactcattcccttttggacattgagattttttgcaattataacatttgaaagataaaagaattatactgctggggccacagattataataggtgcattcagtgaactcttatcttctgaaaagtggccttgcttgttggtacagataggacttcagctattaacaccaagtctcacaagatggcctggaaggaggtgcagagttcaaagacagtccaagcaattctcagaagaggcgtgctcagaattcttaggataactggttcttaaaatatcttcttccaagaaccacaaaggtcagagttatgatatagatgtttatagtttatgaaagtgaccattttttaaaagcagcagcaatttgtttagggaaaggacaggataccatgttgggagtgcaccatagctagaggcattgtggcccacggagaatcactgggagatgagatggtagaaggttcctctcagtgtttttcaagatgtgactcacagatgggtgtaccctttggtatcgctcctactccaaccagcttagctggatgaaatcatctgcatgttaccagtgcatacctgtccgtgatcgttttctctgttttttacaaaggcaatagataggaaatacaaataaaccgattacaaccgctatggcccctagtgccaatcccaaaaccataattagaggtgcaatgaataattttccagcacagactgaccctcgcactaatctccttaaatgaggtctctctgggaggtagcgatatttgcatccaaatatactgaggtttgatgtgtggtctccaaaaaatcggagctggcggtatctctcaccacatcggtaacaaaaattagtgttacattgtgagcaggtcatatggtcacatccttcagttcgctggatgtggatcttgcactttggacacttctgggcattcctctgcccatgctcaatttcgctggcccagtgacgcaacaatttgtctccttttttgtactccttgcagttaacaccttcatgccaaggagagtggcacttaaaacaccagacgaattggcaggtagggcactggattttgtatttgctttctgatctggaaggggtgggaatatgtccttttttcttgaaggttgtaaagtgcttgcactgaggacatggcttggtgctggaatcaatacggccaagttccaagaagtacttatacttgatggagtcttcatgcgttaagttatagacaacagttgtttcttccaagaattcaaaacactctgtgatggggcatttgatttctacttggccaagttgtacctgtagtcccaactactcggaaggctgaggcaggagaatcgcttgaacctgggatgtggaggtttccgtgagccgagatcatgccactgcactccagcctggtgacagagtgagactccgtctgggcgctcaggtagactttgaggcactcctcgcacacggccttcttgcagcaaggcaggggcttgatgggcttgtcttccaggcacacccggcacatcagcaccatgaggggcacatagggatcccctacaccgcccaggccagagtagggtggagctcccaacaggctgggcatggagaacggctcgggcgccaggtagaactccagctcgatgctgccgccgtcgggggagagggaatccgttgggagggacagtcgggggctggggaaggaagagcgggtgctgggagggttcaacactggcggagccccaggtggcgacgcgggcggcgagagctgctccgaggcgggggcctcgggcaggtcgctctccacgcagtacacggagcagaagacttgtctcttggcgagggacgggcgccgctgacccagcacgtccaggaccagtccgtcggcggcccccacgcgggtcctgggctccagctcttcgccggggggcgcctcctgctgttcatcccctccctcttttcgatccccagcttcctcctcttcctcctccagctccaactgcagtggcaaggtctggggattgagaggcccggtgagtgccagtcccgcaggctgcgccggtgctcggctcttactccagcccgggggccccaggctcctcgcgggctctggggcgctggtgtccgcgcagccccagtcgcttccgcagccaccgccgctcggctccgcggaggcggcgcgcagcgggggcgcccgggcgctgtccccctgaggcctcgggggctcagggtggcccgcagtgccactggccagggtctgcgactcctggggcccgccgccgccgctcaccgtgctctgctcctcgcccat

SEQ ID NO: 9932 - RNA, 3275 nt, Homo sapiens
  source 1..3275: mol_type = other RNA
caacggaatcccaaaagcagctgatattggacaaactcaagaacataaaaagttttcaaactcctccataagaaggtgtccccaaaaatattatgtttgagcagttaaatgtaagaaaaaatccttcaaaactagtatttgtttttatgaaaaaccttgaaaacaaataaaaacagagaggaggaggcaagagataacaaggttaggatattaaatgatgtaagaccttgacctaaagcagaattatctataattacaagttggttaaaaaattagcagaataggaattttttaaaggcttaagcagttgtctacagcaaacttgtttttgggattaaataatcccaatgtgaaggatctatctatagagtgaagcatgttttccaaaatgtaagaattttaaaaagactgaatatttgtgtcttgagaatttcctaaaagcagccagttttgtcagtttacaaagcttaatactccttggggtgacgttgcacaaatttctgtgtttgtgtgacaaaaagaaagagcaagaaatagaaaagttcagtatcgaaatggcctgttgtctacattgactttaatttaatacattgctaaattatgtccacaaaggagccatcatctttcaataggtctatgaaaatgtggaaaaatagtgtagcggcatggaactgggtaagtacaaggttactgggcctagttttaatacatatttatatacacacacattcacgcccctacgcatatacacttcagtaacttaatattcttctcattaatttagtttcactcattcccttttggacattgagattttttgcaattataacatttgaaagataaaagaattatactgctggggccacagattataataggtgcattcagtgaactcttatcttctgaaaagtggccttgcttgttggtacagataggacttcagctattaacaccaagtctcacaagatggcctggaaggaggtgcagagttcaaagacagtccaagcaattctcagaagaggcgtgctcagaattcttaggataactggttcttaaaatatcttcttccaagaaccacaaaggtcagagttatgatatagatgtttatagtttatgaaagtgaccattttttaaaagcagcagcaatttgtttagggaaaggacaggataccatgttgggagtgcaccatagctagaggcattgtggcccacggagaatcactgggagatgagatggtagaaggttcctctcagtgtttttcaagatgtgactcacagatgggtgtaccctttggtatcgctcctactccaaccagcttagctggatgaaatcatctgcatgttaccagtgcatacctgtccgtgatcgttttctctgttttttacaaaggcaatagataggaaatacaaataaaccgattacaaccgctatggcccctagtgccaatcccaaaaccataattagaggtgcaatgaataattttccagcacagactgaccctcgcactaatctccttaaatgaggtctctctgggaggtagcgatatttgcatccaaatatactgaggtttgatgtgtggtctccaaaaaatcggagctggcggtatctctcaccacatcggtaacaaaaattagtgttacattgtgagcaggtcatatggtcacatccttcagttcgctggatgtggatcttgcactttggacacttctgggcattcctctgcccatgctcaatttcgctggcccagtgacgcaacaatttgtctccttttttgtactccttgcagttaacaccttcatgccaaggagagtggcacttaaaacaccagacgaattggcaggtagggcactggattttgtatttgctttctgatctggaaggggtgggaatatgtccttttttcttgaaggttgtaaagtgcttgcactgaggacatggcttggtgctggaatcaatacggccaagttccaagaagtacttatacttgatggagtcttcatgcgttaagttatagacaacagttgtttcttccaagaattcaaaacactctgtgatggggcatttgatttctacttggccaagttgtaccttgtattgttcttttgtacacatctgctctcacagtgacttccctggaggcgggcttatattttggaaatgtctgaatcccatcgcagggcagcgaaatctgttttgaggatgatgatacagaaactaccacaaccagcagcagacattcctcctgttttaagaatctctgggcgctcaggtagactttgaggcactcctcgcacacggccttcttgcagcaaggcaggggcttgatgggcttgtcttccaggcacacccggcacatcagcaccatgaggggcacatagggatcccctacaccgcccaggccagagtagggtggagctcccaacaggctgggcatggagaacggctcgggcgccaggtagaactccagctcgatgctgccgccgtcgggggagagggaatccgttgggagggacagtcgggggctggggaaggaagagcgggtgctgggagggttcaacactggcggagccccaggtggcgacgcgggcggcgagagctgctccgaggcgggggcctcgggcaggtcgctctccacgcagtacacggagcagaagacttgtctcttggcgagggacgggcgccgctgacccagcacgtccaggaccagtccgtcggcggcccccacgcgggtcctgggctccagctcttcgccggggggcgcctcctgctgttcatcccctccctcttttcgatccccagcttcctcctcttcctcctccagctccaactgcagtggcaaggtctggggattgagaggcccggtgagtgccagtcccgcaggctgcgccggtgctcggctcttactccagcccgggggccccaggctcctcgcgggctctggggcgctggtgtccgcgcagccccagtcgcttccgcagccaccgccgctcggctccgcggaggcggcgcgcagcgggggcgcccgggcgctgtccccctgaggcctcgggggctcagggtggcccgcagtgccactggccagggtctgcgactcctggggcccgccgccgccgctcaccgtgctctgctcctcgcccatcgccgcccgcggcccgcgccgccgctgcccatccagccgccgggacccccacccggcgcccgcgggcagcgggggcagtggctcggctcgactcgcggctccgcttctgcttccgggtccttcctcctgggctgg

SEQ ID NO: 9933 - RNA, 2979 nt, Homo sapiens
  source 1..2979: mol_type = other RNA
caactagactgtgagcttctaggagctgctgggctccttgaccctgccagcctgagcgccagaatccaatcccaattcttttctgagtactcacggagaactgggtagaggcagtaaatggagcctgcaggagtgagcaggtcctctctctccttgccatcatccatgtggcaagagactcaggctgagcattcgcctgattcaggagggacaggcttagaccagctggaagttggctgtgcagggcaacagcaaagcccactggtggtgaccggccaggagtgaggacttgttctgtcatcctgtaccttctcctaccccctagacttccccttcctcctctgcagaggacaagagtctcatcaccatcaatacttgctgatctattgcctcctctcgccagacccagtaactaccagatctcagaggcccacccagagtctatgcttgtcacacttctgccaggttctgctttggggccctggtgctaaaagacagggtttggaccccagcatcaagggaagaatctgagactcgaactcgggtcctacctctgcctgtttctctgtttggctttggctggttacttgacatctctgggcctcagttttctcatctgtaaaataaggctaagaattgctccacacaaagatgtgagaataccctggggagatggcaagggctggctgtctttcctggttccctaggggtaaccccaggcaccaaagaccctgctgcaagctgactttccatagctataggcccccaagggtctctcaggccatgttacagggccagaaaccatattcccacctcaccctcaccctatctgtcctcccacaccccttcaccctgtaacctcttcatccagattctggctctcagtctctctcttctccatggtcaccctgacactccccaagtgtttggctcagcccctcaaatccctcaccacccttaaaagattgaagttggtattccttcttctgccttgggacagccccaggcttgggcagaagtttggccttgggcctctgctctgagacattccctaccccttgggcagctctgggacccctgagactgactgagggccatgggggctactgagatccccttcctgggatgcactgtggaagcacctcagtttgctgattactaggtgagtgacccggggtcagcccctcagtccttctgagcctcattttaccagtctgtaccataggatgttgttttttaatcttgactgggtcttggacccctgtgaaaatctaatgaagtcagtggacctctcctccctagaaaagtgcatatacaaacacagacacaacattttgcccataattgggtgtgtgtttggggtgggggtccttcgggttccagatgaaaagcccctggcccagaagcctgcaagactgcttccagctgtcagtctgaacccagttctctgccctccccatcctctccgcagtgacttttgggtgtgggggaagaggggacagttagggaggtgggttgctggtctatccacaccttttctccctcctgcctcagtgggcccctcccccagcatttcctgtggctggtgccagcttgtctgcagctcagaccagcatttcaatccctcttggaacccactgaactggcttcacctgcctttcaaggtatttaaaggttctttgaccaaatgctttttgatcctccgctgatgggaaccaagcagaagctctttcgccaactgtcccccctccccccacatgattagtctctaagagctcttttgatattgcagaaaccttctgtggtttgttcaaagccctgggcctttcagccacctcccccggggactcaggccagtcagctccagcctccaccacccatacccaggggtggcctagttaatgggggcctcccagcgctgaacgactctggcctgagttggaaccccagacccgagcccagctggtagagcggtcaagccccgctcctctcagggagcccaggccgagtctggtagtgtggggtgggggacctgttccccagccttcagcgggccgttactcttcttcccgcccagctgaggctgcacagacaggcatgcaggcccacgatgatagcaattgacctgtttccaggtctgaggctgaggctgagaaggggaaactgaggctctgagaagtccagggttcaggccttggtgtgtgagagggcaggagccagaatccaccaacccaagacctgctccagcagccccaccccagccagcaccactcgccgcccgcgctcctggtcctccagggccgcgcagaaggcgcgcctgggctgagtcccagctgcagaattcctggggggcgggggacgaggcgtctccgctcttaatagctgagcgcccgcaaacgcccggcctgggctcgaggcctgcccctccagcgacgggcgcccccaacattgaagtctttctctgcaacttggacggacccaccccgagcgccccgagtatccggcccggggcagagatgcgcgtgcgcggagggggtgccgcggagcccgcgtgagcagacaaattaccgcggacctgagaggacccgtccacgccggcccagagggaggagggggacggtacacagatgggggggcgggggacatgactctctgagggatccccaaccccaggattgaggccccaccctctgccctaactggagttgaagaccttagtgggggtggggcctatccctcgcaggtggaagggtgatctgcaccgggagagctgtgactgtcccggttccgcgatccctggctctgggctcaggaggatgacgggaggggccccagcactccgagagctgggcgagttcaggtggccaggccctctccctcaccaaggcctctgggggagctgctgggctccttggttctgccagcctgagcgccagaatccaatcctgctctataataatcatcagagcagccggcagc

SEQ ID NO: 9934 - RNA, 3078 nt, Homo sapiens
  source 1..3078: mol_type = other RNA
caactagactgtgagcttctaggagctgctgggctccttgaccctgccagcctgagcgccagaatccaatcccaattcttttctgagtactcacggagaactgggtagaggcagtaaatggagcctgcaggagtgagcaggtcctctctctccttgccatcatccatgtggcaagagactcaggctgagcattcgcctgattcaggagggacaggcttagaccagctggaagttggctgtgcagggcaacagcaaagcccactggtggtgaccggccaggagtgaggacttgttctgtcatcctgtaccttctcctaccccctagacttccccttcctcctctgcagaggacaagagtctggagaagataaaagtataaagttaacagatatctccaccccagaaaggacatgagagcaaactactaggaggcagctgcagccatctctatacccacctcatcaccatcaatacttgctgatctattgcctcctctcgccagacccagtaactaccagatctcagaggcccacccagagtctatgcttgtcacacttctgccaggttctgctttggggccctggtgctaaaagacagggtttggaccccagcatcaagggaagaatctgagactcgaactcgggtcctacctctgcctgtttctctgtttggctttggctggttacttgacatctctgggcctcagttttctcatctgtaaaataaggctaagaattgctccacacaaagatgtgagaataccctggggagatggcaagggctggctgtctttcctggttccctaggggtaaccccaggcaccaaagaccctgctgcaagctgactttccatagctataggcccccaagggtctctcaggccatgttacagggccagaaaccatattcccacctcaccctcaccctatctgtcctcccacaccccttcaccctgtaacctcttcatccagattctggctctcagtctctctcttctccatggtcaccctgacactccccaagtgtttggctcagcccctcaaatccctcaccacccttaaaagattgaagttggtattccttcttctgccttgggacagccccaggcttgggcagaagtttggccttgggcctctgctctgagacattccctaccccttgggcagctctgggacccctgagactgactgagggccatgggggctactgagatccccttcctgggatgcactgtggaagcacctcagtttgctgattactaggtgagtgacccggggtcagcccctcagtccttctgagcctcattttaccagtctgtaccataggatgttgttttttaatcttgactgggtcttggacccctgtgaaaatctaatgaagtcagtggacctctcctccctagaaaagtgcatatacaaacacagacacaacattttgcccataattgggtgtgtgtttggggtgggggtccttcgggttccagatgaaaagcccctggcccagaagcctgcaagactgcttccagctgtcagtctgaacccagttctctgccctccccatcctctccgcagtgacttttgggtgtgggggaagaggggacagttagggaggtgggttgctggtctatccacaccttttctccctcctgcctcagtgggcccctcccccagcatttcctgtggctggtgccagcttgtctgcagctcagaccagcatttcaatccctcttggaacccactgaactggcttcacctgcctttcaaggtatttaaaggttctttgaccaaatgctttttgatcctccgctgatgggaaccaagcagaagctctttcgccaactgtcccccctccccccacatgattagtctctaagagctcttttgatattgcagaaaccttctgtggtttgttcaaagccctgggcctttcagccacctcccccggggactcaggccagtcagctccagcctccaccacccatacccaggggtggcctagttaatgggggcctcccagcgctgaacgactctggcctgagttggaaccccagacccgagcccagctggtagagcggtcaagccccgctcctctcagggagcccaggccgagtctggtagtgtggggtgggggacctgttccccagccttcagcgggccgttactcttcttcccgcccagctgaggctgcacagacaggcatgcaggcccacgatgatagcaattgacctgtttccaggtctgaggctgaggctgagaaggggaaactgaggctctgagaagtccagggttcaggccttggtgtgtgagagggcaggagccagaatccaccaacccaagacctgctccagcagccccaccccagccagcaccactcgccgcccgcgctcctggtcctccagggccgcgcagaaggcgcgcctgggctgagtcccagctgcagaattcctggggggcgggggacgaggcgtctccgctcttaatagctgagcgcccgcaaacgcccggcctgggctcgaggcctgcccctccagcgacgggcgcccccaacattgaagtctttctctgcaacttggacggacccaccccgagcgccccgagtatccggcccggggcagagatgcgcgtgcgcggagggggtgccgcggagcccgcgtgagcagacaaattaccgcggacctgagaggacccgtccacgccggcccagagggaggagggggacggtacacagatgggggggcgggggacatgactctctgagggatccccaaccccaggattgaggccccaccctctgccctaactggagttgaagaccttagtgggggtggggcctatccctcgcaggtggaagggtgatctgcaccgggagagctgtgactgtcccggttccgcgatccctggctctgggctcaggaggatgacgggaggggccccagcactccgagagctgggcgagttcaggtggccaggccctctccctcaccaaggcctctgggggagctgctgggctccttggttctgccagcctgagcgccagaatccaatcctgctctataataatcatcagagcagccggcagc

SEQ ID NO: 9935 - RNA, 254 nt, Homo sapiens
  source 1..254: mol_type = other RNA
caagcctctcctgcccttccagccagaatcctcctgtctcctgggtgaaaactggagcccgggttctagctctgctgtgtctctcagactctggtgagtgtcagaatcttctggaggccttgttaaaactccgatggcgaggcccaccctaaggttccaattcaggaggtctcagcagagcctgaaagctggctttcccagcagggccccggggtgctgatgctcctccccctagaacgacccctgagagccct

SEQ ID NO: 9936 - RNA, 801 nt, Homo sapiens
  source 1..801: mol_type = other RNA
caagctcgtgtctgtgggtccgtgtcgggggctcaccatcgcggctggggcctccccggccctccccctcatccctggtcctcctggtccctgtctgtctgtctgtcgggtctgtccacctgccgcgccccccgggctgaggtaggaggttgtatagttgaggaggacacccaaggagatcactatacggcctcctagctttccccaggctgcgccctgcacgggacggggcccggcggggacccccagccccactcagggacccttagccccactgggctgccccagggaccctgggaggaagagccgggctcttttctgtccttgtccctgcatcccctccttcccctgaaatctgttttccttccctgtctgtctccatctctgctgtgtctctgtggcttctgtgtctctttcacagtggatcctctgactccctcttattctggctttctaggtctctgcccctcccgatatctctctgtgtctctatttctgtcgtttttggtctttctgtctctggctctcagaatgtctctgtgcctatctccatctctgacccccaccccagggtctaccgggccaccgcacaccatgttgccagtctctaggtccctgagaccctttaacctgtgaggacatccagggtcacaggtgaggttcttgggagcctggcgtctggcccaaccacacacctggggaattgctggcctgacttctgacccctgactcctcatacccttcctccagagcatgacatttgaccaccaactgaaacctgacctctgaccccagaccact

SEQ ID NO: 9937 - RNA, 2116 nt, Homo sapiens
  source 1..2116: mol_type = other RNA
caagtcttatttgagcacctgttgtgttttatttctcagctgattcagaaagcaggaaggaagaaggaggttatttattgggtccctcaaaccccaacaaaagccaactggaatcctctcaggaagtcttcagaacagcagttcgatggccacacaccatccctagctaagtgggagggtcacgggtgttgtggtgactctggagagcaggatggccatggtttggtgcagccaagcacaggtcttctccatccatgactccttcctggcttggtcaggtttgcagagtaattcaaccaaggcccaattccttacacaagacagataacactttcttgacctgtgtatgaaggggtggtggcacccccagagcaccttcagtccctgtagcaggtttcccaacagacgcaagaaagctcctctccctctgcactgtcagcctcttctgctcttcttgtcttaccctccaaaccaaaagtatctctctgctgcactgatgctgaatgaaatacagaactacttagaatgagcaaaaatacacagggaaatagcccctgaagctgtccttgcaaggtgatatgattcctgacaggttcatccttcaggcatacaactcccaactcttcacaaaggcttaatggatgtttcaaatgtgcaggaccacatgtgccatagaatggcagctttgatcaaaccacagaacttacttccaagatttataaagtgcgagtgactgatgacccccgtcttccctgagtgcatgatgaccactttcagtgatctccacaagctcaggtgctggcccagggtccaagctacagctttctgaatgttaataaaacaacttggaatcttctgtgattcactcattttctcatgaaattgtggatcaccaagtctggctgcaacgcctctcatgactctcttctttcaatttcctttactcctattctttttcaggtccttcccgtttcttgtctgaataccagaaattactaactggccctcctgccctggttctccatcctcaggcaccgctgacatggtgatcaccgtgaaacacctacccgactacctgattccctttaaacgctcaacaaagggagaagagcatgggcataccttgagccaggtaacccaaggttcaagtcctgactccactatttacaaagcacaagtcctttaaccacttcagcttgtactttcctcatcccacactagaaagaacaatagcgcccatctaatagagtttgggagaactgagtgggataatgcacttaaagctcttagcacaatgttttggcatctagtaagtaaatgctcaataagtgtatattattatcctatgttctgagcgttagaggccctgcaaattcagggcatagaaaacctttccattcccatctcctatcaattcaaacagtgggtgcaactccttcatccagggattctcaccctgtgctccccggaacactgctctgccacaaacccctccacaaaaatatcgaactttatttctacctctagtacatttgtctccaaaatagcaaaagagtagtgagaatttcatgtatcttcaacaaggcttttcattaggagacaatactctaaaattacccacatagatggcctgttgctttctgaaagtagtacaatgttttgatgtctaatcatctttatctctaagactaagcgtcatattttcccagctgaaataagctgccaccttgaatgccctcacatatactcttcccagactcaccagtagggggcgcgcctgcataaaggagggagctagaacaatttcctcacaccgggacagttgtctgttccagaatgcataatccaatgatgcaattttctttatacttaccagaggcctagaacatggaagcatctcagttcttgcagtttttcatcaacacttgtcataacactgcccatgcttgctattaccaaaatgatttttttttctgtagtttgcacagtatctaaattctagctacagactagactacttgaattacctaaattccaagttggcaatgatccctacacacacttcatttgattcccagcagcccatgtagagtgtaaccatcacacagggcataaa

SEQ ID NO: 9938 - RNA, 1549 nt, Homo sapiens
  source 1..1549: mol_type = other RNA
caatggcacaaactcattcttgattgacacacatctcgactcctcactcatttcttctccacatattattattttctcattacttacctaaaatttaaccttatagataatgaaaagggttctgaacattaagaaataatagaatagttataaatggaggaaaaagtttgaataaaaaagtttcttaaaaggatagtgtcacttgcaaaaatagctctttgaaatacaggttcctataaacattttacacgcattaagatattactcttacacatactggtaacacagacactatacatatttgtctccattttaggaagaaatgaagcaaggctatttttaataataaacttagaaacaattcataacccctagtatttgcattaacctgcaaatactaggcagcacaccacagcagagtgtaactaaaacctaaaatagtgtttcactttcttccacacctacctctgtgcgctcatgcaagtgtttttattttgctttgcattagatgcttctgtaatacaggcatctgattcaccccacataaagctgttgtaagtaatcaatgtgagaaagtctacttattgttaagcatatttgtatattttttactagttatttcatacttgccctgaaagaatacacattcaaaaagcttgaaattaggcaatgtcagtctcatcaaacaaaaccagcattggaagcgaatattaacaaatatcagaatgaaattacaaaatatacatctccagcctcataaaacatgaattttataagcactttcataaacataagaaaaatagctttgacaataactatttgaaaacattattattaataatcttgtatactgtacatgtgcacttaaatgtaatagcaccaacattcattatattatgaaggggatactttataagaattataaattatttttacatgattaaataattttggcagagtaagtccgcaggacttaaataaccagtcagccttagtatctacatctggaccaggaagcctttgtgttacagacacagattccctgtgaagttctccagggtgtaaagaaggccccagggaggtgccgacgggatgtgagggctgcctttcagctcaggcgagcctgcaagcaacagggcagtttgggaagggtcacaggcacaggaagggagcagtgggcaaccattgattacatcaaaccaggatggtttcttctttttaaagaaacttttgttgagtgtttacccacccccatccacacaaatatgctctctaggaaatgtgaaagtataagcttcagaaaaatgtttttctcatcctttaatttctggttttatgatcaaatgttccgaagacactgcttctttttgctcaaaatagttgacattgtcattgcttctagtttttcagctcctactatgcttactatgtccatgggtgccattgacgtctttggctatttatcatctctgggtggcgcaggccaaggacgcccatggacagcgcgacctcctcccattccacacacgcgcccacgaccaaagtgcgc

SEQ ID NO: 9939 - RNA, 4058 nt, Homo sapiens
  source 1..4058: mol_type = other RNA
caattctcaaaggagcctccctagactacagctcccacagccccgatttccccttgttgtcctgttagtaaacacccacaaagtgtttacttgtgccaggctctgttctagacacttcaaatatgttagctcatttaatttgcacaacagcttgaagaggtaggtataatgattatccggatttaatggatgaggaaacaggcacagaaaggtcaagtaactcgcccaaggtcacaagtggagaaggtggaatctgaacccaggctcacgacaatagatgccctctctggatgctccagcatcccacctcaagtgcctaccacagtgcttggcacatagtaggggcacagtgaactatatcagtgaatagatggatgcacagctggatggttgagtaatgaggatgtgtgacacatggaaggaggatggatggaagtctgatacaaggaaggatgacaagcaatcaatagaagatggatagatggatggatgaatggatggataattgatggatgatggatagatgaaggaatggatggatgatagataggtgtaaggataatggatggatagatgatgaatagatgaagaaatggataaagaataaatggataatgcagaaatggataatggatggatggatggttgatggataatgggcagatggagggatgaatggatgtgtggatgacggataatggatggatggatggttgatggataatgggcagatggagggatgaatggatgagtggatgatggataatggatagatggagggatgatggctgatgaatgatggataaaggatggatggatgatggatagatggatgaatggatagatagtggatggaaagatgatggatgatggatggaaggataaataatggataaatgaagaaatgcataatggttgaatggataagggatgaatggatgatggatagatggaggaatggataatggataaatagctaacgaatgggtggatggatgatgaatggatggatgaaagcatagacaatgaatggatagatgatggatggatggatggatggatggatgatggatggatggatgatggatagatagctgatgaataggtgggtggatgatgaatggatggatgaatggatagataatggatggacagatgatggatggatggatgggtggatggatggatgaaggatggatggatggatgatgaaggatggatggttgatggactatagatggataatagatgatgagtgggtggataatggattaatgatgatggagggatgaatgaaaaatggatgaatggacaatggacaatagctggatgagtgatagatgctggatggatggatggatggatagatgatggatagctgatgaatgagtggatggatggcaaatggatggatgaatggatagatgatggatggatggaaggatggatgaatgaatgaatgatggatggatgagtggaaagatgaattatgaatgatggatggatgatgaatgatggatggataatagatgatgaatgggtggataatagatggacgaatgatgaatggatggatggataatggataatggctggatgagtgatggatgatggatggaaggatggaaggataaaggagaagaatatattctacgtggggaaaagctctagaaattcttctgggaaggaataaggcctcttgggaaatgactgaacttggagtcaggagtcctgattcaaaccccatctctgccatttgctagctctgtaatcacaggcaagttacttcattcatctctgtgaccctaattttcctcctctttataataagaatctgtttctccaggcatctaagccctgggattttctgtaaaggtggtgctaggcacagggtaaagcctcctcagggtcagggtggtgtgatgttgctgagctctgaagagaaatgtggcttcttcaccctccctgcttagggcttgggtttgggggcccacttcttgctcgccccacatctcttgcttgcctggcccctgccttgcccactctctggaatacaaggcagccctgccagcctgtgtccagcctgggctctgtgctccctccctgccaccctgcagtgtctggccctggcctctgcacagtctctgctgtcaccttcagcctccttgaggagtaatggggtggggcaatgacagggcagccacagcccacagagcaactggcctccatacaccgcaagaaaacaagttcaacaagcatttattgagcccctgctgtgtgcctgctgtgtgacacccctgcagtgcctgcgccactgccccctccttcaggaagccactctctgccccccaaagggctctgcccctctgggcacctgactggcttgtgggtgccagccattcagtggccagtggccatgtgtctcctggcatcgcagctgtgcccagcagggctcatgtgatgatggcaagagtccggggctgctgtcccaaagtcactctgtgcagccctgtgcattcccttgggcctgccctggccccatttccaaggccatgggacccaggcagcgatgggcaggacaggcctggcatctcccacgcaggctgactgagttcacggcacacaggccagggttctgggggcaccactctggtggtcttgcagcaggggctggtgccagcgatggcctgaggtccgcgggccaggttgaggtcttggtcacacccagtgccccaagacccagcactgtcggttcagctctggtgcttcctgtgcggagctccggggccaggaatccgccatgtgtggctggtgtcgggcagggtatctctcgtggcggcagtctaagtgaaagtcctcctcgctcccgtccctcttctccatccagctgtgtgacctggggcaagtcgccctccctctctgtgcctcgatttgccacctctcccggaagtacttgatggcctcagggtctatgaaggtcggctcttcccggtagccctgctcaaagaccttgcgcttgtgccggaactcaatgaccgtcttggtgtaggagttgagcgtggtgacagaggctgccatgcagcaggtaaaggagccccacgccaggcagaaggaccacccgtagtcccaggaatggggtctccagtcctcaggaccgaggctcacggtgacctggaacacctgcgtgtacatcatgtgggcgaccattcccaggaggcctgagagcaccgtgaagacagccgcgaaggcattgagcttgagcccgtcgatgacattgctggagtggaagagctcgagacacatgaggctgaagccaaccaccagcagcagaatgtacagcacctcggagaccacagacagccacaggacccctttctccgatgccggggccaggtcaatgaagctgcgacatttttcaccaagcccgctgagctcctcctcgcacgagtaccagatgccggtgtggaaattcctgaagaggaagcggtcgtcgccggtctcccagctgtagagcgcgccgccaggggggccgttccccgaggcggtggcggcggcggcggcggcggcgggggcggcggtgccgttggccgtggcgttggcgcccgagttggggcagttggcgcgcccgccctggccgcagcccggcttggggacccgctgcgtgccctggcaccagtgcgtggtgaggaaagcggtggtggcgaacagcagcgccagcaggttcagggccacggccaggagcgctcggccgcggcggctagtcttcatgccgcccgcgccgccgggacgggactgcaccgccggggagctccgcgcgcgaagttggcagctggcgccccgcgtcagcggccgctgcccgccgcgccccggggctcgggtgcctgagatcggcggcggcggacgcggcgcgggcccatgccccccccaaccccggggtgggggcgcggcgcggggggcgtgcggggcgggctggcggggcgggcggcggtggaggagcggctacggcgcgcccggagcccggagcgcgagtgcacctcggctaggagccgctggcgcct

SEQ ID NO: 9940 - RNA, 3415 nt, Homo sapiens
  source 1..3415: mol_type = other RNA
caattctcaaaggagcctccctagactacagctcccacagccccgatttccccttgttgtcctgttagtaaacacccacaaagtgtttacttgtgccaggctctgttctagacacttcaaatatgttagctcatttaatttgcacaacagcttgaagaggtaggtataatgattatccggatttaatggatgaggaaacaggcacagaaaggtcaagtaactcgcccaaggtcacaagtggagaaggtggaatctgaacccaggctcacgacaatagatgccctctctggatgctccagcatcccacctcaagtgcctaccacagtgcttggcacatagtaggggcacagtgaactatatcagtgaatagatggatgcacagctggatggttgagtaatgaggatgtgtgacacatggaaggaggatggatggaagtctgatacaaggaaggatgacaagcaatcaatagaagatggatagatggatggatgaatggatggataattgatggatgatggatagatgaaggaatggatggatgatagataggtgtaaggataatggatggatagatgatgaatagatgaagaaatggataaagaataaatggataatgcagaaatggataatggatggatggatggttgatggataatgggcagatggagggatgaatggatgtgtggatgacggataatggatggatggatggttgatggataatgggcagatggagggatgaatggatgagtggatgatggataatggatagatggagggatgatggctgatgaatgatggataaaggatggatggatgatggatagatggatgaatggatagatagtggatggaaagatgatggatgatggatggaaggataaataatggataaatgaagaaatgcataatggttgaatggataagggatgaatggatgatggatagatggaggaatggataatggataaatagctaacgaatgggtggatggatgatgaatggatggatgaaagcatagacaatgaatggatagatgatggatggatggatggatggatggatgatggatggatggatgatggatagatagctgatgaataggtgggtggatgatgaatggatggatgaatggatagataatggatggacagatgatggatggatggatgggtggatggatggatgaaggatggatggatggatgatgaaggatggatggttgatggactatagatggataatagatgatgagtgggtggataatggattaatgatgatggagggatgaatgaaaaatggatgaatggacaatggacaatagctggatgagtgatagatgctggatggatggatggatggatagatgatggatagctgatgaatgagtggatggatggcaaatggatggatgaatggatagatgatggatggatggaaggatggatgaatgaatgaatgatggatggatgagtggaaagatgaattatgaatgatggatggatgatgaatgatggatggataatagatgatgaatgggtggataatagatggacgaatgatgaatggatggatggataatggataatggctggatgagtgatggatgatggatggaaggatggaaggataaaggagaagaatatattctacgtggggaaaagctctagaaattcttctgggaaggaataaggcctcttgggaaatgactgaacttggagtcaggagtcctgattcaaaccccatctctgccatttgctagctctgtaatcacaggcaagttacttcattcatctctgtgaccctaattttcctcctctttataataagaatctgtttctccaggcatctaagccctgggattttctgtaaaggtggtgctaggcacagggtaaagcctcctcagggtcagggtggtgtgatgttgctgagctctgaagagaaatgtggcttcttcaccctccctgcttagggcttgggtttgggggcccacttcttgctcgccccacatctcttgcttgcctggcccctgccttgcccactctctggaatacaaggcagccctgccagcctgtgtccagcctgggctctgtgctccctccctgccaccctgcagtgtctggccctggcctctgcacagtctctgctgtcaccttcagcctccttgaggagtaatggggtggggcaatgacagggcagccacagcccacagagcaactggcctccatacaccgcaagaaaacaagttcaacaagcatttattgagcccctgctgtgtgcctgctgtgtgacacccctgcagtgcctgcgccactgccccctccttcaggaagccactctctgccccccaaagggctctgcccctctgggcacctgactggcttgtgggtgccagccattcagtggccagtggccatgtgtctcctggcatcgcagctgtgcccagcagggctcatgtgatgatggcaagagtccggggctgctgtcccaaagtcactctgtgcagccctgtgcattcccttgggcctgccctggccccatttccaaggccatgggacccaggcagcgatgggcaggacaggcctggcatctcccacgcaggctgactgagttcacggcacacaggccagggttctgggggcaccactctggtggtcttgcagcaggggctggtgccagcgatggcctgaggtccgcgggccaggttgaggtcttggtcacacccagtgccccaagacccagcactgtcggttcagctctggtgcttcctgtgcggagctccggggccaggaatccgccatgtgtggctggtgtcgggcagggtatctctcgtggcggcagtctaagtgaaagtcctcctcgctcccgtccctcttctccatcctctcccggaagtacttgatggcctcagggtctatgaaggtcggctcttcccggtagccctgctcaaagaccttgcgcttgtgccggaactcaatgaccgtcttggtgtaggagttgagcgtggtgacagaggctgccatgcagcaggtaaaggagccccacgccaggcagaaggaccacccgtagtcccaggaatggggtctccagtcctcaggaccgaggctcacggtgacctggaacacctgcgtgtacatcatgtgggcgaccattcccaggaggcctgagagcaccgtgaagacagccgcgaaggcattgagcttgagcccgtcgatgacattgctggagtggaagagctcgagacacatgaggctgaagccaaccaccagcagcagaatgtacagcacctcggagaccacagacagccacaggacccctcggagatgctgatgctcctatcgctgggtttccagcccctgttggtgctggcagggactgcccctcatcatggcgctgctcactgactcagctgcc

SEQ ID NO: 9941 - RNA, 4004 nt, Homo sapiens
  source 1..4004: mol_type = other RNA
caattctcaaaggagcctccctagactacagctcccacagccccgatttccccttgttgtcctgttagtaaacacccacaaagtgtttacttgtgccaggctctgttctagacacttcaaatatgttagctcatttaatttgcacaacagcttgaagaggtaggtataatgattatccggatttaatggatgaggaaacaggcacagaaaggtcaagtaactcgcccaaggtcacaagtggagaaggtggaatctgaacccaggctcacgacaatagatgccctctctggatgctccagcatcccacctcaagtgcctaccacagtgcttggcacatagtaggggcacagtgaactatatcagtgaatagatggatgcacagctggatggttgagtaatgaggatgtgtgacacatggaaggaggatggatggaagtctgatacaaggaaggatgacaagcaatcaatagaagatggatagatggatggatgaatggatggataattgatggatgatggatagatgaaggaatggatggatgatagataggtgtaaggataatggatggatagatgatgaatagatgaagaaatggataaagaataaatggataatgcagaaatggataatggatggatggatggttgatggataatgggcagatggagggatgaatggatgtgtggatgacggataatggatggatggatggttgatggataatgggcagatggagggatgaatggatgagtggatgatggataatggatagatggagggatgatggctgatgaatgatggataaaggatggatggatgatggatagatggatgaatggatagatagtggatggaaagatgatggatgatggatggaaggataaataatggataaatgaagaaatgcataatggttgaatggataagggatgaatggatgatggatagatggaggaatggataatggataaatagctaacgaatgggtggatggatgatgaatggatggatgaaagcatagacaatgaatggatagatgatggatggatggatggatggatggatgatggatggatggatgatggatagatagctgatgaataggtgggtggatgatgaatggatggatgaatggatagataatggatggacagatgatggatggatggatgggtggatggatggatgaaggatggatggatggatgatgaaggatggatggttgatggactatagatggataatagatgatgagtgggtggataatggattaatgatgatggagggatgaatgaaaaatggatgaatggacaatggacaatagctggatgagtgatagatgctggatggatggatggatggatagatgatggatagctgatgaatgagtggatggatggcaaatggatggatgaatggatagatgatggatggatggaaggatggatgaatgaatgaatgatggatggatgagtggaaagatgaattatgaatgatggatggatgatgaatgatggatggataatagatgatgaatgggtggataatagatggacgaatgatgaatggatggatggataatggataatggctggatgagtgatggatgatggatggaaggatggaaggataaaggagaagaatatattctacgtggggaaaagctctagaaattcttctgggaaggaataaggcctcttgggaaatgactgaacttggagtcaggagtcctgattcaaaccccatctctgccatttgctagctctgtaatcacaggcaagttacttcattcatctctgtgaccctaattttcctcctctttataataagaatctgtttctccaggcatctaagccctgggattttctgtaaaggtggtgctaggcacagggtaaagcctcctcagggtcagggtggtgtgatgttgctgagctctgaagagaaatgtggcttcttcaccctccctgcttagggcttgggtttgggggcccacttcttgctcgccccacatctcttgcttgcctggcccctgccttgcccactctctggaatacaaggcagccctgccagcctgtgtccagcctgggctctgtgctccctccctgccaccctgcagtgtctggccctggcctctgcacagtctctgctgtcaccttcagcctccttgaggagtaatggggtggggcaatgacagggcagccacagcccacagagcaactggcctccatacaccgcaagaaaacaagttcaacaagcatttattgagcccctgctgtgtgcctgctgtgtgacacccctgcagtgcctgcgccactgccccctccttcaggaagccactctctgccccccaaagggctctgcccctctgggcacctgactggcttgtgggtgccagccattcagtggccagtggccatgtgtctcctggcatcgcagctgtgcccagcagggctcatgtgatgatggcaagagtccggggctgctgtcccaaagtcactctgtgcagccctgtgcattcccttgggcctgccctggccccatttccaaggccatgggacccaggcagcgatgggcaggacaggcctggcatctcccacgcaggctgactgagttcacggcacacaggccagggttctgggggcaccactctggtggtcttgcagcaggggctggtgccagcgatggcctgaggtccgcgggccaggttgaggtcttggtcacacccagtgccccaagacccagcactgtcggttcagctctggtgcttcctgtgcggagctccggggccaggaatccgccatgtgtggctggtgtcgggcagggtatctctcgtggcggcagtctaagtgaaagtcctcctcgctcccgtccctcttctccatcctctcccggaagtacttgatggcctcagggtctatgaaggtcggctcttcccggtagccctgctcaaagaccttgcgcttgtgccggaactcaatgaccgtcttggtgtaggagttgagcgtggtgacagaggctgccatgcagcaggtaaaggagccccacgccaggcagaaggaccacccgtagtcccaggaatggggtctccagtcctcaggaccgaggctcacggtgacctggaacacctgcgtgtacatcatgtgggcgaccattcccaggaggcctgagagcaccgtgaagacagccgcgaaggcattgagcttgagcccgtcgatgacattgctggagtggaagagctcgagacacatgaggctgaagccaaccaccagcagcagaatgtacagcacctcggagaccacagacagccacaggacccctttctccgatgccggggccaggtcaatgaagctgcgacatttttcaccaagcccgctgagctcctcctcgcacgagtaccagatgccggtgtggaaattcctgaagaggaagcggtcgtcgccggtctcccagctgtagagcgcgccgccaggggggccgttccccgaggcggtggcggcggcggcggcggcggcgggggcggcggtgccgttggccgtggcgttggcgcccgagttggggcagttggcgcgcccgccctggccgcagcccggcttggggacccgctgcgtgccctggcaccagtgcgtggtgaggaaagcggtggtggcgaacagcagcgccagcaggttcagggccacggccaggagcgctcggccgcggcggctagtcttcatgccgcccgcgccgccgggacgggactgcaccgccggggagctccgcgcgcgaagttggcagctggcgccccgcgtcagcggccgctgcccgccgcgccccggggctcgggtgcctgagatcggcggcggcggacgcggcgcgggcccatgccccccccaaccccggggtgggggcgcggcgcggggggcgtgcggggcgggctggcggggcgggcggcggtggaggagcggctacggcgcgcccggagcccggagcgcgagtgcacctcggctaggagccgctggcgcct

SEQ ID NO: 9942 - RNA, 3851 nt, Homo sapiens
  source 1..3851: mol_type = other RNA
caattctcaaaggagcctccctagactacagctcccacagccccgatttccccttgttgtcctgttagtaaacacccacaaagtgtttacttgtgccaggctctgttctagacacttcaaatatgttagctcatttaatttgcacaacagcttgaagaggtaggtataatgattatccggatttaatggatgaggaaacaggcacagaaaggtcaagtaactcgcccaaggtcacaagtggagaaggtggaatctgaacccaggctcacgacaatagatgccctctctggatgctccagcatcccacctcaagtgcctaccacagtgcttggcacatagtaggggcacagtgaactatatcagtgaatagatggatgcacagctggatggttgagtaatgaggatgtgtgacacatggaaggaggatggatggaagtctgatacaaggaaggatgacaagcaatcaatagaagatggatagatggatggatgaatggatggataattgatggatgatggatagatgaaggaatggatggatgatagataggtgtaaggataatggatggatagatgatgaatagatgaagaaatggataaagaataaatggataatgcagaaatggataatggatggatggatggttgatggataatgggcagatggagggatgaatggatgtgtggatgacggataatggatggatggatggttgatggataatgggcagatggagggatgaatggatgagtggatgatggataatggatagatggagggatgatggctgatgaatgatggataaaggatggatggatgatggatagatggatgaatggatagatagtggatggaaagatgatggatgatggatggaaggataaataatggataaatgaagaaatgcataatggttgaatggataagggatgaatggatgatggatagatggaggaatggataatggataaatagctaacgaatgggtggatggatgatgaatggatggatgaaagcatagacaatgaatggatagatgatggatggatggatggatggatggatgatggatggatggatgatggatagatagctgatgaataggtgggtggatgatgaatggatggatgaatggatagataatggatggacagatgatggatggatggatgggtggatggatggatgaaggatggatggatggatgatgaaggatggatggttgatggactatagatggataatagatgatgagtgggtggataatggattaatgatgatggagggatgaatgaaaaatggatgaatggacaatggacaatagctggatgagtgatagatgctggatggatggatggatggatagatgatggatagctgatgaatgagtggatggatggcaaatggatggatgaatggatagatgatggatggatggaaggatggatgaatgaatgaatgatggatggatgagtggaaagatgaattatgaatgatggatggatgatgaatgatggatggataatagatgatgaatgggtggataatagatggacgaatgatgaatggatggatggataatggataatggctggatgagtgatggatgatggatggaaggatggaaggataaaggagaagaatatattctacgtggggaaaagctctagaaattcttctgggaaggaataaggcctcttgggaaatgactgaacttggagtcaggagtcctgattcaaaccccatctctgccatttgctagctctgtaatcacaggcaagttacttcattcatctctgtgaccctaattttcctcctctttataataagaatctgtttctccaggcatctaagccctgggattttctgtaaaggtggtgctaggcacagggtaaagcctcctcagggtcagggtggtgtgatgttgctgagctctgaagagaaatgtggcttcttcaccctccctgcttagggcttgggtttgggggcccacttcttgctcgccccacatctcttgcttgcctggcccctgccttgcccactctctggaatacaaggcagccctgccagcctgtgtccagcctgggctctgtgctccctccctgccaccctgcagtgtctggccctggcctctgcacagtctctgctgtcaccttcagcctccttgaggagtaatggggtggggcaatgacagggcagccacagcccacagagcaactggcctccatacaccgcaagaaaacaagttcaacaagcatttattgagcccctgctgtgtgcctgctgtgtgacacccctgcagtgcctgcgccactgccccctccttcaggaagccactctctgccccccaaagggctctgcccctctgggcacctgactggcttgtgggtgccagccattcagtggccagtggccatgtgtctcctggcatcgcagctgtgcccagcagggctcatgtgatgatggcaagagtccggggctgctgtcccaaagtcactctgtgcagccctgtgcattcccttgggcctgccctggccccatttccaaggccatgggacccaggcagcgatgggcaggacaggcctggcatctcccacgcaggctgactgagttcacggcacacaggccagggttctgggggcaccactctggtggtcttgcagcaggggctggtgccagcgatggcctgaggtccgcgggccaggttgaggtcttggtcacacccagtgccccaagacccagcactgtcggttcagctctggtgcttcctgtgcggagctccggggccaggaatccgccatgtgtggctggtgtcgggcagggtatctctcgtggcggcagtctaagtgaaagtcctcctcgctcccgtccctcttctccatcctctcccggaagtacttgatggcctcagggtctatgaaggtcggctcttcccggtagccctgctcaaagaccttgcgcttgtgccggaactcaatgaccgtcttggtgtaggagttgagcgtggtgacagaggctgccatgcagcaggtaaaggagccccacgccaggcagaaggaccacccgtagtcccaggaatggggtctccagtcctcaggaccgaggctcacggtgacctggaacacctgcgtgtacatcatgtgggcgaccattcccaggaggcctttctccgatgccggggccaggtcaatgaagctgcgacatttttcaccaagcccgctgagctcctcctcgcacgagtaccagatgccggtgtggaaattcctgaagaggaagcggtcgtcgccggtctcccagctgtagagcgcgccgccaggggggccgttccccgaggcggtggcggcggcggcggcggcggcgggggcggcggtgccgttggccgtggcgttggcgcccgagttggggcagttggcgcgcccgccctggccgcagcccggcttggggacccgctgcgtgccctggcaccagtgcgtggtgaggaaagcggtggtggcgaacagcagcgccagcaggttcagggccacggccaggagcgctcggccgcggcggctagtcttcatgccgcccgcgccgccgggacgggactgcaccgccggggagctccgcgcgcgaagttggcagctggcgccccgcgtcagcggccgctgcccgccgcgccccggggctcgggtgcctgagatcggcggcggcggacgcggcgcgggcccatgccccccccaaccccggggtgggggcgcggcgcggggggcgtgcggggcgggctggcggggcgggcggcggtggaggagcggctacggcgcgcccggagcccggagcgcgagtgcacctcggctaggagccgctggcgcct

SEQ ID NO: 9943 - RNA, 1734 nt, Homo sapiens
  source 1..1734: mol_type = other RNA
cacacacacacacacacgtatacacaaaaccccacaagagtatagtactatctatgaaggaaagagataccacgttaaatttaaccaagtatttaggaatgacagggagctaggaaggcgaaaacacatgtaattttatttttgtttaaccttaagcttgccaacttctttccctgaacagcatttgtcttgttttgatacccacctacacttatattagaaacgtactgcaaactatttagtgactccacttttaatttatggtcgtatgactaagatgttttgaatataagcctatccgtatgccagatataaatttcaggaactcttaatgtctcttcttttacagaaactctacctctatcctgatgtaattaggttgattaagaaaattaaaggccacgggccagaaaactaacttccacaaatgcaacaaaaggaaaatttctccaataacctgtatgcaatgggaaatctttcttttaagtaccaagtcaatttctttaactgtacaatgtattctaatttgaaggttttcaaatataatacagtaacaacaaaatataataaaattaagactataagaaaacagagtaaatggtataattcaataatgactaaaataaaatgacactatggattttgtaatcaacctataattatctatttaaatttcactttacatacataagatcacagctgaggttaaccataatttcaaattttatcaccagccacttgtgctattttatcacatttgaaaatattcactcgtattatttacttcaaacagtaatctataaatttgtttagactataataattaaggacctttccttcttcaggataacttaaaaaattaaatgatgtattgaacatactactaaagaaagtttactttttgattatggtctctgcattgaaaatctgtaggaatttttctttaataattttcaaatcttcccatggcctctctgttcacagaaatatcatctttgaaacaacttgtgtgagtactttataaatcaaaaattgattcacatgaccatattaccataatcaccaattttaacagtctcctacatattttctatatcacttttcttgattacaaaatgtcagtaataagaacacgctcttaatataacagaatatttaattacatcagtttcccatgaacacaccaaagtcacttaataattatattggccatttccactgatcggcaggaggctcttccactaatggctcccatagtttccattccctcatttttcttgccagatttagttcatgttcagcctgaagaatcacctcttctaattgaccgccttgaagttggtcttctaattttttaacatctggttcattttgcttttcaacacaagacgtgatatgttactgcctcagggtatcttgctggatggcccagggtatctgcatcacttgtttcttcaccacttttcaaatctttgctcaaataacaccttcttattgattaactactgataatttgcattatgataggcgctttaaccatagccagcttctcatttgtaatctgttctgtatactttctatatgctgcatttttagggatttcctcaagaacatcaagaatctttgtgtacaatattcttagcctctcgtgaggagtattgcacacagccaatcccacaaggccagtggtcttcttcagcacacccgccatgacagcgccaacgactcggtgac

SEQ ID NO: 9944 - RNA, 1814 nt, Homo sapiens
  source 1..1814: mol_type = other RNA
cacacacacacacacacgtatacacaaaaccccacaagagtatagtactatctatgaaggaaagagataccacgttaaatttaaccaagtatttaggaatgacagggagctaggaaggcgaaaacacatgtaattttatttttgtttaaccttaagcttgccaacttctttccctgaacagcatttgtcttgttttgatacccacctacacttatattagaaacgtactgcaaactatttagtgactccacttttaatttatggtcgtatgactaagatgttttgaatataagcctatccgtatgccagatataaatttcaggaactcttaatgtctcttcttttacagaaactctacctctatcctgatgtaattaggttgattaagaaaattaaaggccacgggccagaaaactaacttccacaaatgcaacaaaaggaaaatttctccaataacctgtatgcaatgggaaatctttcttttaagtaccaagtcaatttctttaactgtacaatgtattctaatttgaaggttttcaaatataatacagtaacaacaaaatataataaaattaagactataagaaaacagagtaaatggtataattcaataatgactaaaataaaatgacactatggattttgtaatcaacctataattatctatttaaatttcactttacatacataagatcacagctgaggttaaccataatttcaaattttatcaccagccacttgtgctattttatcacatttgaaaatattcactcgtattatttacttcaaacagtaatctataaatttgtttagactataataattaaggacctttccttcttcaggataacttaaaaaattaaatgatgtattgaacatactactaaagaaagtttactttttgattatggtctctgcattgaaaatctgtaggaatttttctttaataattttcaaatcttcccatggcctctctgttcacagaaatatcatctttgaaacaacttgtgtgagtactttataaatcaaaaattgattcacatgaccatattaccataatcaccaattttaacagtctcctacatattttctatatcacttttcttgattacaaaatgtcagtaataagaacacgctcttaatataacagaatatttaattacatcagtttcccatgaacacaccaaagtcacttaataattatattggccatttccactgatcggcaggaggctcttccactaatggctcccatagtttccattccctcatttttcttgccagatttagttcatgttcagcctgaagaatcacctcttctaattgaccgccttgaagttggtcttctaattttttaacatctggttccgctttaaccatagccagcttctcatttgtaatctgttctgtatactttctatatgctgcatttttagggatttcctcaagaacatcaagaatctttgtgtacaatattcttagcctcagctgtacggcctgggtgagtcctttaactcctctggaactatgccaatatttccatctgcaccagccatgaattctggggcagaaattgtgtactgttgctccatttccatttgtgaatagagaacatcttttattaatagatgaaaatctccatctatattgtaatggtaaaatatctgtgatcccaacactttgaagggtgggtagattgctcgaactcaggagtttgaaaccagcctggacaacaaggtcaaaccccatctctttaaattgtgcgttaattccaagtggtttggttttgttccatcagtagcaacactccctgc

SEQ ID NO: 9945 - RNA, 1572 nt, Homo sapiens
  source 1..1572: mol_type = other RNA
cacacacacacacacacgtatacacaaaaccccacaagagtatagtactatctatgaaggaaagagataccacgttaaatttaaccaagtatttaggaatgacagggagctaggaaggcgaaaacacatgtaattttatttttgtttaaccttaagcttgccaacttctttccctgaacagcatttgtcttgttttgatacccacctacacttatattagaaacgtactgcaaactatttagtgactccacttttaatttatggtcgtatgactaagatgttttgaatataagcctatccgtatgccagatataaatttcaggaactcttaatgtctcttcttttacagaaactctacctctatcctgatgtaattaggttgattaagaaaattaaaggccacgggccagaaaactaacttccacaaatgcaacaaaaggaaaatttctccaataacctgtatgcaatgggaaatctttcttttaagtaccaagtcaatttctttaactgtacaatgtattctaatttgaaggttttcaaatataatacagtaacaacaaaatataataaaattaagactataagaaaacagagtaaatggtataattcaataatgactaaaataaaatgacactatggattttgtaatcaacctataattatctatttaaatttcactttacatacataagatcacagctgaggttaaccataatttcaaattttatcaccagccacttgtgctattttatcacatttgaaaatattcactcgtattatttacttcaaacagtaatctataaatttgtttagactataataattaaggacctttccttcttcaggataacttaaaaaattaaatgatgtattgaacatactactaaagaaagtttactttttgattatggtctctgcattgaaaatctgtaggaatttttctttaataattttcaaatcttcccatggcctctctgttcacagaaatatcatctttgaaacaacttgtgtgagtactttataaatcaaaaattgattcacatgaccatattaccataatcaccaattttaacagtctcctacatattttctatatcacttttcttgattacaaaatgtcagtaataagaacacgctcttaatataacagaatatttaattacatcagtttcccatgaacacaccaaagtcacttaataattatattggccatttccactgatcggcaggaggctcttccactaatggctcccatagtttccattccctcatttttcttgccagatttagttcatgttcagcctgaagaatcacctcttctaattgaccgccttgaagttggtcttctaattttttaacatctggttccgctttaaccatagccagcttctcatttgtaatctgttctgtatactttctatatgctgcatttttagggatttcctcaagaacatcaagaatctttgtgtacaatattcttagcctcgtgaggagtattgcacacagccaatcccacaaggccagtggtcttcttcagcacacccgccatgacagcgccaacgactcggtgac

SEQ ID NO: 9946 - RNA, 1818 nt, Homo sapiens
  source 1..1818: mol_type = other RNA
cacacacacacacacacgtatacacaaaaccccacaagagtatagtactatctatgaaggaaagagataccacgttaaatttaaccaagtatttaggaatgacagggagctaggaaggcgaaaacacatgtaattttatttttgtttaaccttaagcttgccaacttctttccctgaacagcatttgtcttgttttgatacccacctacacttatattagaaacgtactgcaaactatttagtgactccacttttaatttatggtcgtatgactaagatgttttgaatataagcctatccgtatgccagatataaatttcaggaactcttaatgtctcttcttttacagaaactctacctctatcctgatgtaattaggttgattaagaaaattaaaggccacgggccagaaaactaacttccacaaatgcaacaaaaggaaaatttctccaataacctgtatgcaatgggaaatctttcttttaagtaccaagtcaatttctttaactgtacaatgtattctaatttgaaggttttcaaatataatacagtaacaacaaaatataataaaattaagactataagaaaacagagtaaatggtataattcaataatgactaaaataaaatgacactatggattttgtaatcaacctataattatctatttaaatttcactttacatacataagatcacagctgaggttaaccataatttcaaattttatcaccagccacttgtgctattttatcacatttgaaaatattcactcgtattatttacttcaaacagtaatctataaatttgtttagactataataattaaggacctttccttcttcaggataacttaaaaaattaaatgatgtattgaacatactactaaagaaagtttactttttgattatggtctctgcattgaaaatctgtaggaatttttctttaataattttcaaatcttcccatggcctctctgttcacagaaatatcatctttgaaacaacttgtgtgagtactttataaatcaaaaattgattcacatgaccatattaccataatcaccaattttaacagtctcctacatattttctatatcacttttcttgattacaaaatgtcagtaataagaacacgctcttaatataacagaatatttaattacatcagtttcccatgaacacaccaaagtcacttaataattatattggccatttccactgatcggcaggaggctcttccactaatggctcccatagtttccattccctcatttttcttgccagatttagttcatgttcagcctgaagaatcacctcttctaattgaccgccttgaagttggtcttctaattttttaacatctggttccgctttaaccatagccagcttctcatttgtaatctgttctgtatactttctatatgctgcatttttagggatttcctcaagaacatcaagaatctttgtgtacaatattcttagcctctcgtgaggagtattgcacacagccaatcccacaaggccagtggtcagctgtacggcctgggtgagtcctttaactcctctggaactatgccaatatttccatagtcacaattccattttgactagatgattctaagagtcacctgtgatcccaacactttgaagggtgggtagattgctcgaactcaggagtttgaaaccagcctggacaacaaggtcaaaccccatctctttaaattgtgcgttaattccaagtggtttggttttgttccatcagtagcaacactccctgcagctgaattggcaggtcctttgttttcataagagttcttt

SEQ ID NO: 9947 - RNA, 1715 nt, Homo sapiens
  source 1..1715: mol_type = other RNA
cacacacacacacacacgtatacacaaaaccccacaagagtatagtactatctatgaaggaaagagataccacgttaaatttaaccaagtatttaggaatgacagggagctaggaaggcgaaaacacatgtaattttatttttgtttaaccttaagcttgccaacttctttccctgaacagcatttgtcttgttttgatacccacctacacttatattagaaacgtactgcaaactatttagtgactccacttttaatttatggtcgtatgactaagatgttttgaatataagcctatccgtatgccagatataaatttcaggaactcttaatgtctcttcttttacagaaactctacctctatcctgatgtaattaggttgattaagaaaattaaaggccacgggccagaaaactaacttccacaaatgcaacaaaaggaaaatttctccaataacctgtatgcaatgggaaatctttcttttaagtaccaagtcaatttctttaactgtacaatgtattctaatttgaaggttttcaaatataatacagtaacaacaaaatataataaaattaagactataagaaaacagagtaaatggtataattcaataatgactaaaataaaatgacactatggattttgtaatcaacctataattatctatttaaatttcactttacatacataagatcacagctgaggttaaccataatttcaaattttatcaccagccacttgtgctattttatcacatttgaaaatattcactcgtattatttacttcaaacagtaatctataaatttgtttagactataataattaaggacctttccttcttcaggataacttaaaaaattaaatgatgtattgaacatactactaaagaaagtttactttttgattatggtctctgcattgaaaatctgtaggaatttttctttaataattttcaaatcttcccatggcctctctgttcacagaaatatcatctttgaaacaacttgtgtgagtactttataaatcaaaaattgattcacatgaccatattaccataatcaccaattttaacagtctcctacatattttctatatcacttttcttgattacaaaatgtcagtaataagaacacgctcttaatataacagaatatttaattacatcagtttcccatgaacacaccaaagtcacttaataattatattggccatttccactgatcggcaggaggctcttccactaatggctcccatagtttccattccctcatttttcttgccagatttagttcatgttcagcctgaagaatcacctcttctaattgaccgccttgaagttggtcttctaattttttaacatctggttccgctttaaccatagccagcttctcatttgtaatctgttctgtatactttctatatgctgcatttttagggatttcctcaagaacatcaagaatctttgtgtacaatattcttagcctctcgtgaggagtattgcacacagccaatcccacaaggccagtggtccggtaaggcatgcagaacgagtccccgaaaagcaccgccgagcccgcgacagtaggggtcaacacccgcgggaagtagggctatcggactgagtctacccccacagtctaaattccaacagtgacctccattcgtctcaccttcttcagcacacccgccatgacagcgccaacgactcggtgac

SEQ ID NO: 9948 - RNA, 1724 nt, Homo sapiens
  source 1..1724: mol_type = other RNA
cacacacacacacacacgtatacacaaaaccccacaagagtatagtactatctatgaaggaaagagataccacgttaaatttaaccaagtatttaggaatgacagggagctaggaaggcgaaaacacatgtaattttatttttgtttaaccttaagcttgccaacttctttccctgaacagcatttgtcttgttttgatacccacctacacttatattagaaacgtactgcaaactatttagtgactccacttttaatttatggtcgtatgactaagatgttttgaatataagcctatccgtatgccagatataaatttcaggaactcttaatgtctcttcttttacagaaactctacctctatcctgatgtaattaggttgattaagaaaattaaaggccacgggccagaaaactaacttccacaaatgcaacaaaaggaaaatttctccaataacctgtatgcaatgggaaatctttcttttaagtaccaagtcaatttctttaactgtacaatgtattctaatttgaaggttttcaaatataatacagtaacaacaaaatataataaaattaagactataagaaaacagagtaaatggtataattcaataatgactaaaataaaatgacactatggattttgtaatcaacctataattatctatttaaatttcactttacatacataagatcacagctgaggttaaccataatttcaaattttatcaccagccacttgtgctattttatcacatttgaaaatattcactcgtattatttacttcaaacagtaatctataaatttgtttagactataataattaaggacctttccttcttcaggataacttaaaaaattaaatgatgtattgaacatactactaaagaaagtttactttttgattatggtctctgcattgaaaatctgtaggaatttttctttaataattttcaaatcttcccatggcctctctgttcacagaaatatcatctttgaaacaacttgtgtgagtactttataaatcaaaaattgattcacatgaccatattaccataatcaccaattttaacagtctcctacatattttctatatcacttttcttgattacaaaatgtcagtaataagaacacgctcttaatataacagaatatttaattacatcagtttcccatgaacacaccaaagtcacttaataattatattggccatttccactgatcggcaggaggctcttccactaatggctcccatagtttccattccctcatttttcttgccagatttagttcatgttcagcctgaagaatcacctcttctaattgaccgccttgaagttggtcttctaattttttaacatctggttccgctttaaccatagccagcttctcatttgtaatctgttctgtatactttctatatgctgcatttttagggatttcctcaagaacatcaagaatctttgtgtacaatattcttagcctctcgtgaggagtattgcacacagccaatcccacaaggccagtggtctgccctacccggtaaggcatgcagaacgagtccccgaaaagcaccgccgagcccgcgacagtaggggtcaacacccgcgggaagtagggctatcggactgagtctacccccacagtctaaattccaacagtgacctccattcgtctcaccttcttcagcacacccgccatgacagcgccaacgactcggtgac

SEQ ID NO: 9949 - RNA, 1574 nt, Homo sapiens
  source 1..1574: mol_type = other RNA
cacacacacacacacacgtatacacaaaaccccacaagagtatagtactatctatgaaggaaagagataccacgttaaatttaaccaagtatttaggaatgacagggagctaggaaggcgaaaacacatgtaattttatttttgtttaaccttaagcttgccaacttctttccctgaacagcatttgtcttgttttgatacccacctacacttatattagaaacgtactgcaaactatttagtgactccacttttaatttatggtcgtatgactaagatgttttgaatataagcctatccgtatgccagatataaatttcaggaactcttaatgtctcttcttttacagaaactctacctctatcctgatgtaattaggttgattaagaaaattaaaggccacgggccagaaaactaacttccacaaatgcaacaaaaggaaaatttctccaataacctgtatgcaatgggaaatctttcttttaagtaccaagtcaatttctttaactgtacaatgtattctaatttgaaggttttcaaatataatacagtaacaacaaaatataataaaattaagactataagaaaacagagtaaatggtataattcaataatgactaaaataaaatgacactatggattttgtaatcaacctataattatctatttaaatttcactttacatacataagatcacagctgaggttaaccataatttcaaattttatcaccagccacttgtgctattttatcacatttgaaaatattcactcgtattatttacttcaaacagtaatctataaatttgtttagactataataattaaggacctttccttcttcaggataacttaaaaaattaaatgatgtattgaacatactactaaagaaagtttactttttgattatggtctctgcattgaaaatctgtaggaatttttctttaataattttcaaatcttcccatggcctctctgttcacagaaatatcatctttgaaacaacttgtgtgagtactttataaatcaaaaattgattcacatgaccatattaccataatcaccaattttaacagtctcctacatattttctatatcacttttcttgattacaaaatgtcagtaataagaacacgctcttaatataacagaatatttaattacatcagtttcccatgaacacaccaaagtcacttaataattatattggccatttccactgatcggcaggaggctcttccactaatggctcccatagtttccattccctcatttttcttgccagatttagttcatgttcagcctgaagaatcacctcttctaattgaccgccttgaagttggtcttctaattttttaacatctggttccgctttaaccatagccagcttctcatttgtaatctgttctgtatactttctatatgctgcatttttagggatttcctcaagaacatcaagaatctttgtgtacaatattcttagcctctcgtgaggagtattgcacacagccaatcccacaaggccagtggtcttcttcagcacacccgccatgacagcgccaacgactcggtgac

SEQ ID NO: 9950 - RNA, 1783 nt, Homo sapiens
  source 1..1783: mol_type = other RNA
cacacacacacacacacgtatacacaaaaccccacaagagtatagtactatctatgaaggaaagagataccacgttaaatttaaccaagtatttaggaatgacagggagctaggaaggcgaaaacacatgtaattttatttttgtttaaccttaagcttgccaacttctttccctgaacagcatttgtcttgttttgatacccacctacacttatattagaaacgtactgcaaactatttagtgactccacttttaatttatggtcgtatgactaagatgttttgaatataagcctatccgtatgccagatataaatttcaggaactcttaatgtctcttcttttacagaaactctacctctatcctgatgtaattaggttgattaagaaaattaaaggccacgggccagaaaactaacttccacaaatgcaacaaaaggaaaatttctccaataacctgtatgcaatgggaaatctttcttttaagtaccaagtcaatttctttaactgtacaatgtattctaatttgaaggttttcaaatataatacagtaacaacaaaatataataaaattaagactataagaaaacagagtaaatggtataattcaataatgactaaaataaaatgacactatggattttgtaatcaacctataattatctatttaaatttcactttacatacataagatcacagctgaggttaaccataatttcaaattttatcaccagccacttgtgctattttatcacatttgaaaatattcactcgtattatttacttcaaacagtaatctataaatttgtttagactataataattaaggacctttccttcttcaggataacttaaaaaattaaatgatgtattgaacatactactaaagaaagtttactttttgattatggtctctgcattgaaaatctgtaggaatttttctttaataattttcaaatcttcccatggcctctctgttcacagaaatatcatctttgaaacaacttgtgtgagtactttataaatcaaaaattgattcacatgaccatattaccataatcaccaattttaacagtctcctacatattttctatatcacttttcttgattacaaaatgtcagtaataagaacacgctcttaatataacagaatatttaattacatcagtttcccatgaacacaccaaagtcacttaataattatattggccatttccactgatcggcaggaggctcttccactaatggctcccatagtttccattccctcatttttcttgccagatttagttcatgttcagcctgaagaatcacctcttctaattgaccgccttgaagttggtcttctaattttttaacatctggttccgctttaaccatagccagcttctcatttgtaatctgttctgtatactttctatatgctgcatttttagggatttcctcaagaacatcaagaatctttgtgtacaatattcttagcctctggctattttttctatttttagtagagacagggttttgccatgttggccaggatggtctcaaactcctgacttcaggtgatccgcccacctcagcctcccaaagtgctgggattacaggcgtgagcccacccagcctgaatcagtatttttcaaagtgaggtccgaagcactgcaaatttttttttttaatttttcttatttgaatttctcgtgaggagtattgcacacagccaatcccacaaggccagtggtcttcttcagcacacccgccatgacagcgccaacgactcggtgac

SEQ ID NO: 9951 - RNA, 1529 nt, Homo sapiens
  source 1..1529: mol_type = other RNA
cacacacacacacacacgtatacacaaaaccccacaagagtatagtactatctatgaaggaaagagataccacgttaaatttaaccaagtatttaggaatgacagggagctaggaaggcgaaaacacatgtaattttatttttgtttaaccttaagcttgccaacttctttccctgaacagcatttgtcttgttttgatacccacctacacttatattagaaacgtactgcaaactatttagtgactccacttttaatttatggtcgtatgactaagatgttttgaatataagcctatccgtatgccagatataaatttcaggaactcttaatgtctcttcttttacagaaactctacctctatcctgatgtaattaggttgattaagaaaattaaaggccacgggccagaaaactaacttccacaaatgcaacaaaaggaaaatttctccaataacctgtatgcaatgggaaatctttcttttaagtaccaagtcaatttctttaactgtacaatgtattctaatttgaaggttttcaaatataatacagtaacaacaaaatataataaaattaagactataagaaaacagagtaaatggtataattcaataatgactaaaataaaatgacactatggattttgtaatcaacctataattatctatttaaatttcactttacatacataagatcacagctgaggttaaccataatttcaaattttatcaccagccacttgtgctattttatcacatttgaaaatattcactcgtattatttacttcaaacagtaatctataaatttgtttagactataataattaaggacctttccttcttcaggataacttaaaaaattaaatgatgtattgaacatactactaaagaaagtttactttttgattatggtctctgcattgaaaatctgtaggaatttttctttaataattttcaaatcttcccatggcctctctgttcacagaaatatcatctttgaaacaacttgtgtgagtactttataaatcaaaaattgattcacatgaccatattaccataatcaccaattttaacagtctcctacatattttctatatcacttttcttgattacaaaatgtcagtaataagaacacgctcttaatataacagaatatttaattacatcagtttcccatgaacacaccaaagtcacttaataattatattggccatttccactgatcggcaggaggctcttccactaatggctcccatagtttccattccctcatttttcttgccagatttagttcatgttcagcctgaagaatcacctcttctaattgaccgccttgaagttggtcttctaattttttaacatctggttccgctttaaccatagccagcttctcatttgtaatctgttctgtatactttctatatgctgcatttttagggatttcctcaagaacatcaagaatctttgtgtacaatattcttagcctcttcttcagcacacccgccatgacagcgccaacgactcggtgac

SEQ ID NO: 9952 - RNA, 1457 nt, Homo sapiens
  source 1..1457: mol_type = other RNA
cacacacacacacacacgtatacacaaaaccccacaagagtatagtactatctatgaaggaaagagataccacgttaaatttaaccaagtatttaggaatgacagggagctaggaaggcgaaaacacatgtaattttatttttgtttaaccttaagcttgccaacttctttccctgaacagcatttgtcttgttttgatacccacctacacttatattagaaacgtactgcaaactatttagtgactccacttttaatttatggtcgtatgactaagatgttttgaatataagcctatccgtatgccagatataaatttcaggaactcttaatgtctcttcttttacagaaactctacctctatcctgatgtaattaggttgattaagaaaattaaaggccacgggccagaaaactaacttccacaaatgcaacaaaaggaaaatttctccaataacctgtatgcaatgggaaatctttcttttaagtaccaagtcaatttctttaactgtacaatgtattctaatttgaaggttttcaaatataatacagtaacaacaaaatataataaaattaagactataagaaaacagagtaaatggtataattcaataatgactaaaataaaatgacactatggattttgtaatcaacctataattatctatttaaatttcactttacatacataagatcacagctgaggttaaccataatttcaaattttatcaccagccacttgtgctattttatcacatttgaaaatattcactcgtattatttacttcaaacagtaatctataaatttgtttagactataataattaaggacctttccttcttcaggataacttaaaaaattaaatgatgtattgaacatactactaaagaaagtttactttttgattatggtctctgcattgaaaatctgtaggaatttttctttaataattttcaaatcttcccatggcctctctgttcacagaaatatcatctttgaaacaacttgtgtgagtactttataaatcaaaaattgattcacatgaccatattaccataatcaccaattttaacagtctcctacatattttctatatcacttttcttgattacaaaatgtcagtaataagaacacgctcttaatataacagaatatttaattacatcagtttcccatgaacacaccaaagtcacttaataattatattggccatttccactgatcggcaggaggctcttccactaatggctcccatagtttccattccctcatttttcttgccagatttagttcatgttcagcctgaagaatcacctcttctaattgaccgccttgaagttggtcttctaattttttaacatctggttcctcgtgaggagtattgcacacagccaatcccacaaggccagtggtcttcttcagcacacccgccatgacagcgccaacgactcggtgac

SEQ ID NO: 9953 - RNA, 10078 nt, Homo sapiens
  source 1..10078: mol_type = other RNA
cacacacacacacacacgtatacatacatacaacttgggttccggagggtaaactactgaaaaccttacatattgagccatctagctcatttatcactgacgtctcaatgacaattttaatgaagatgttcattatttttttcattcttactcaaatacctatcattaattaagagaagagtttgagatgtataaggctaataaaggaagtgagagtgtggtgaattaagtgatgagtattatgtacaattgcctttacaaaaaacgtatttttactgtggaagaaattcatgcagagatgcctgtggaaaagtatcaataagaaaacaaaacacctttaacactatgacatactgattataatatactatgatatgtattattacagcattacttacacattctactttaggcaatgtaatctacttctgaatgaccttgttaatttttaaggcatcagtgcatcaagggcaaagctccataaaataaatataaaaacaagaaagcattagctaatttgtggcatagagaatgatcactgtatattatatctgttggccacttccatataggtaataaattgtacatcttattgtaaaaatgttatagcataaatttcacatcatttttcaacacttcatttaaagggctaaactgatctggcagtattctcattttcattgttccatcagctccacaggagaaaatgtgatttgcaggccctgtctcaatttgcatcactccagttccaatatttctaaaaatggactgccgagcatgttcactgacaaaagtatggagaagaccaaaggtagagagactccaaatctttatattgccttcggcagatcctgtaacaaagtactcttcagttggatcaacagcaacggctttaacaggagaatcatggctctggaaaagctgcctctgttgtcgttgacaaaggtcaaatacatatgtaaaaccttttctgccacctgatattagtagctgatgttttggagcatatgctaaaactgtggctccactgtcatggcaggtaaatgcatggactaaactattggcaggtgctacaagagtatcccacaaacatacgtttcaggtatggcttaggcatgcttccagtaactggacaacatttccagtttgtttgatacaaacttaaatatccatcagcatcaactattccaaacttatttccctgatagttaaatctcattcttgtaactcttgaattgccaccagatcgaaaacaggttatttgttgagaatggccccattcaaacattctgacacttccatcttgagctcctgtcagatagtaaggaagagttggatgagaagtcattcttctaacattattaatggctttcttaatcatcacagatgctcctctgccagtctgtgtactaccaagccatggcatgttgattggagtgccaggattgctatgtgtatatggagttgtaccttgaacagctgttaaatcatcacgagcatgtataaccaagaaatcttctgatcctttggtttccacttctatatcatcatctacccaagtgtagacctgtgtggccagaattccagaaacatccagttcttgaacatcatgactggaagcgattgctatgcagtttctatttgccttattaacagcaaacgcagtaatgatatcagattccttatgaataattcttgctttacctccaggatatcccaaatctgcttctatctcatttagacaccgtttctttgtgaatatatttttgataaaggtttcctgaatttcttcctgcttcaccaaatactgccaaagcctcttcacagacagtgccagatggtgtttggatttgaaaggagtgtttgtaggttccagtaaagctttgtggcgaagaattgcaggacctgcagacaaactctcttcggcggtatgacttgcgatataattttgaggtggcccaccatggatttcaagtcgtcggagaagaacttgttcccaacattgaagagtttttagaaccgcatgacaaagaggtgaactaactggaagctctgcaagatcatgacctgcgaagggataaaaagtcttcaaattgttgagcaccaattgcaccatcgccaaccgcatcaaggaccaactatatgaatttgaattagaatgttcctggagatggaaatctgatgctaaaacatcatcatcatcatcattgtcatcatcatcacttcccagactctcctctgaatcatattcggctctactttgagaagagggtagaaaaggcttagctatgaaatagtcccagatactgagctcaggtgggatgaacttttctttaaccgccagtgactcctggcttactggtgccgaggaaggggtcagtggggcagattctctgcaagacatttttgacggcctaaaacgtttgttctgtttttctccttcttcaactagtgaagaaacaggtaaagtttttgaatgtgtctgttctttgctaggaacatgtgcacctccaccaaacacagcagaccacattttctcatttagaggatgggccacaatccgaaatagctcattacttgaatgtgtggccaggccatggatgaagagactaagatacactgctgtgagaatctcacagagcaagactgtaagccctgactgggcttcctcgccagaagaattcaaaagtcgaattagacaagttattcctggccattgagctggtgacgtattgggagttaatgcttcatctaagcttcctgttttcaaagaaggtcgatgaggaagcagtactgtctgatataccattccagtaaactgattcgtctgaaatgaactgtagttatgactaccacaaaggcactgataaatacaagcagaaagtgaagctgctaaagtatgcattacatacactttattgctttggatatcagggtggggtggtgaatcaaagtttattatggcatggagaatatcatgtgtcagattactaaggtgcaataatggattggcaactactgttttggcattggctgtacaagcaaagaggagaggcactgaggtttgctctgacagagggctagaaaatagtggttctgatgtttcctgctgagattcttgcaaaagcaaaatcaattccattcttacagatgcaagacccccaccatgggatccatgaagtatgcagtaactaagaaacattctcaaaagtgactgatacttcaagagccactgtcttttttcctgaaaattttctctcagttgtttcacttttgtttggtgaggcaaatcttcagcatcctcatttaatccaaattcatcttcatttctgccaaatgcagactgtagttcttcagcatctgagcaaaagtcacaagtcctctgaagagctatcacctctttttcaagccagtggtatagttggtaacgcaattttccaccatctatttcatagccagtagataaagtacgaagttctactgtgagaatctttaaacatgctctaaattttaactgaactgcaattatatcttctgatggatttaaaaggtcattttcatctagtgtgctgaaagattctgtgtagttagaacttatgtcatccaactttttatctgtttttctctgtaaaggttttagttctttcattgaaatagggacatcctcattttcttcatcattatcactgtcccattttaactctaaagagtcatcctgaaacacaacacttggttggctccagtcaaaagaaagagtggagtttgattgcttctctgaggaaccctctgaagaagatccaaaaccatttatcagtgactgtgaccaatcaacagcagaagacttatcttcccttgcatccaactttaatggagaagaaggagaacagtctttactagtatccagaaaactagaagccctataaaaaggtcttgttttcttgatgactttaggcatctttgataatacttccaaagccaacattgggcagccagcttttaaatgagcactggcagtggtaaaaaataaacgtctttcacttaaattaattgttcctgccagtccactttttcctgttaggctcatatgtgtggaaaatgtatcagatgatccaaaatgacgtctcagcaaaagaggatgtgttcttagataattgtagaaattaaaaactgtaggattactggctgataaaacttgatcatcattctctctgataggttgctttattaatgtttccagagcaccactataatcttccaaaatccaatatgccatgctccgaagaaaaggatcatgatgcatatttatgttcaatgaacacagttcactgacaggagaatcgattcccaaaacttttttacgtaaaatagatttatatgctgcagatgtatcaaattcagactcatagagtcttgctattacaagagccaactgaatgtcattcaatttctcaagacatacctcaattgcatctctgaggcaaccagctaaaagaaaaaatgctgcagaatgttcaaatctttgtttgcctagcaaagaaaaagcattctttaaagctgctttacgccacctctcatcctcaaaattgtgtccaaaaaactgtgtcatcctggtgtttttttcagctctatataatccccaaatcacagctttctttttcattgcaaggtaaaaaatggcagcatctaaaggatcattctttctataaaaggctgctttagctactttttctatgcatttgcgtaagatgcgggtattccggacccaccaccccacacccatagctcttagttcagaccaagtgggatcatctttctgcatggctggcaacatgttcagcagttcttcttctgctactgagtgaaatgcccaagcaaaatgacttgtagacaggccttggtgaaggagttgagctcgataggctggaagggaagttgtaagaaaggtatggagtcgaacagccaaaagaaattttaacccacattcatcaagagtttctccaccttggcttctgtctcggctttctccaatatcagtgcttgtagttgcaattgtatctgctaaggccatcaaagacatctgctccatccggctgagtcctggtaaactagaatgaagtaagtggccagaaagaacctgagcatgctcaggtccaaagtaagtcggactgtactgtgaaaggtcaataactctaggctttgtattttcttcatctgtctctaacatatgagtatcagtcattagaagttgagtctgaaaaagctcatcataactttctttagataattggtttgatttacttaacgtactctcattactagatttctccaaagatgagtaacagctatcatcatctgctgcaagtaaggcatataaaggaagtggaggaacagaatctatttctgtgtaatctgtattttcagccttgttgaatgcctgggggtctctggtagtgcttccactagcactgattgtgagagacctaaggcggcgttcatgattagattcagcttcattcagagccacaacttccccagcaatgcacttaacaagatgggacaagatggccttggctctccgaactttaccaagatccatgagttccaaaagctgcaagggatgatactgaggtagagtcggggaaagtacatgagctgcttcaaaaagacctgaatcttccatatccactgaaggatcgaatgcagttttctttccacagattttctgtgcaagactggtcatggatcgagtcagagttttctttggaggatgtaacccagaactggagttactctgttttattaaacttgttatagatggagtgctcccactgtacgaatctgttataacaggttcttgtttagaagatggttgccattggcaatacacatgcatttcacagtccattcctaccacaaggatgccatcccggacccacgataaagaaacaggaaaaggtggggagccatctacagaagaaactaggtccacacttcgtaatagtacaaatttagaaaggggcacaactttggtactctcccagagaggaaatgccagggtttccttaccagtttggtcttgtaccttgccagccaggggtccatacataaaaagttttgatccaattcctacagtcaggatatgagaaccgtcttctctagacatccaatctaagtgaactaaatgctttgtgtttgatgtgatattctctttactagataaatacatgtcttgtttattataggccactaaattgctatcaacactaatgccagaatccaatactgtgcttaactcatctaaatgaattgtctgctcaaggacccaacatgaacctcctgttgactcacattcaaaaatacttacatgcatcacaaagtcctgggaagatctactattagatgcaggctgcttataagctactgctaaacgatttgtatgtgcacagctaacttctacaggcctaccaggtacagttatactactattgctctgaagtccatcttcaataagtaatggccattcttcccaaatgtatgcaagatcaatttttccattctttgacgtggcagattctccatctgttactctgcatctccagaatcttactttctcatctgaacatgaagttgccaataaataaggagcactgcatgcaggatatatagaagatgaactcagatgtcctgctgatggcttaatacttattatctcaactccttctggtaaatgcaattcttggctataaaccatttctgaaaacagagtcaacctgctggtactctggagatttgctctgcaagcctgatacttttgtgaaaaaggagataggatcttctctggagaagaagaataatgttcttctggctgccaaaccgcttcggataattttgtatctactttttcatctaatgagacaggaattgactttagatgtaaattccacatgtgtaacagtgaacggttgtcttgagtgcattctattacaattaggtagaacttctcagaaaatccattaggtgagctgcctgcattagataaaatgctgtctttgccaaggcttttcttctcaaggttattcaaaatgaagtcttcttcaaaaacatgaagcagttgggtttttctgccatgaagtttggtaatgggatctaatgcaataatgcatcctggcctggctgttgattgttgactgacgatgttaaagacttcaccaacatatttagaaatttcagggttagaaagctcagataaaagtttcttagcatcaataactgcttcatataatctcagatattgtccatcactggctacaaagcatgcactaggagagttgcagtatgcacccagacaataactgggtataagagtgggcagccatgccacattggaaaaggcagaaacatgaagagaattaatccgggcaagctcagaaactcctccagaaaaagacaatggcccaactgggtcaaccctccacagaataagctcactgtaaactgcactgggatcctgaaatgccacgtcaacagtgcttttattttgttgtgtcaaagagcattcttcaatatttagagcatcaaaaggttgctctgggttatcaacatctggtgtccttaatgcattatggtgtgatgttgtcagcaataatggtaatactgagtggcaagctaaatcattaagatgaaaacgatgaccacaatatctggatttgtgggaaatactgagaacagtagaaaaagcagattcctcggcaaaactgaccagccactgattcagagaaccatcagcatgttttgatatcatcataacattaggcgtaaaaatacttaattttaaactattagatgatttattgtgaccagaagaaataagcattgatgtggaacgggtgaggccagaaggtttttgtttcccctgctgaatagccaagtcaacattcttggtacaggcatacatcattatgcttttacagagagagtttgcatcacctgtggggaaagctactggaattctggaaacaaaggacacctgtacttgacgaaacataccaggctggtattcatccagccaatccacatgccaaactagcaaagaaccatccatgggatgaatactaaatagcatatctgcatttttactccattcagacagaagtacttcaatctgatgatcaatggcagctgacgataatgatgtaaaacttgagtttggtaccattttatcacagcctaattccttcttttcgggatttattttcagatcatcaacaccatcatcagtttcttcatcagattttacatctgcctgattagaatcttctacactggcctcagaagatggttgttcaaaactttttctaagttgctgtaaaaaaacttccatggacaaagtaaaatgcagttctttattgtttagccagtgtacaacaaaaggtccggtcttctcttcattttcatttagactcagagatgtaatagatggaagaagtggaatgtctgtggctgggttgatgctggctgcaatatgaaagtggcaaagtgcattggcatgcagtggagtgttcctgtgaacatgatgaggatcctgctgatgtggtagatatcccgtatgtgctacaagagcaagtgatctcctccgacctctacgaaaatgtctcagatttacttctaaagcattttgaactcgttctttactggaagcatttctcttgaagttatttgttaaattaattgattcagtccaatggctgcagtcacctccgtatagcaaacaatcatttggtaaaaatgtctctacccaaagacgacacacattatctttgcagcaagtcaacagtacattacatacagaagccctaggcatatatttgcttgttttacgccaggaaaatccatttactgctcgaggatgggccagatacacaaaagaaaagtcaatttctccttgggattgtttttctgaacttccatctggagaagtaacagctgtccgccagttttctacattataccaaaccttcaaaagacagtcatccttcccagcagtggcaaaaaattctccatctggtgaaaatttcattaaatgaacttgggaagcagttttgcaatgccaaatgcatttccaatctccaaagttaagatctgttttatttaaattttcatcttcagttggcttctccaagttagtattggaccagagttgcaaatagctggaaccagttaaaagacgactgcctgtgggatcccaggttatattgtgtgctattgattccagaaaaaattggccacttttctgccactgactatataattccaaatttttcttttgttttggtaggttaactggttcaaaaatggagataacatttccataagacgctgcaatcttgccttgttgcattgaacagtctacacatcccacttgaatatttccatgtttagctcctgggattatctgtaatctttcaaaatcgcttcccagtattacaatgtcacatccagatgcataagccgtgaagcgctggtcgccaatgctgcccacggagaagcagtggtcgccagggttcacagccccggtcagcacctggtgcaggttcatgtcggcgccctagtcctgcaacggacaccgcatccagctcatgccacgggtcagcggctgcttccctccctccttccctcaggggcggcggccgctcttcggtggcgacggcagaagcagcgacaggcgcctggagccggagccgctcagctggggcccgcgactcatcccgagccccggagggcgaggcccggagggggcgggtcggcgagagggcggagcgccgcgctccttcgcgcacctgtcactccccgcgctagcccaggtgaagctcagggtcccctcaccggccacgacccggggccgactcaccggccaggaaggccgcgctgtccacacacttcctctggacctcgggcagccgctcctgacccagcccgagtggcgcaagcagtacgcgctcgcactccccgcctgacctgtcccttcccggctccggtgcccgccacccccacagtcctccgccactcactacgcgcctct

SEQ ID NO: 9954 - RNA, 10235 nt, Homo sapiens
  source 1..10235: mol_type = other RNA
cacacacacacacacacgtatacatacatacaacttgggttccggagggtaaactactgaaaaccttacatattgagccatctagctcatttatcactgacgtctcaatgacaattttaatgaagatgttcattatttttttcattcttactcaaatacctatcattaattaagagaagagtttgagatgtataaggctaataaaggaagtgagagtgtggtgaattaagtgatgagtattatgtacaattgcctttacaaaaaacgtatttttactgtggaagaaattcatgcagagatgcctgtggaaaagtatcaataagaaaacaaaacacctttaacactatgacatactgattataatatactatgatatgtattattacagcattacttacacattctactttaggcaatgtaatctacttctgaatgaccttgttaatttttaaggcatcagtgcatcaagggcaaagctccataaaataaatataaaaacaagaaagcattagctaatttgtggcatagagaatgatcactgtatattatatctgttggccacttccatataggtaataaattgtacatcttattgtaaaaatgttatagcataaatttcacatcatttttcaacacttcatttaaagggctaaactgatctggcagtattctcattttcattgttccatcagctccacaggagaaaatgtgatttgcaggccctgtctcaatttgcatcactccagttccaatatttctaaaaatggactgccgagcatgttcactgacaaaagtatggagaagaccaaaggtagagagactccaaatctttatattgccttcggcagatcctgtaacaaagtactcttcagttggatcaacagcaacggctttaacaggagaatcatggctctggaaaagctgcctctgttgtcgttgacaaaggtcaaatacatatgtaaaaccttttctgccacctgatattagtagctgatgttttggagcatatgctaaaactgtggctccactgtcatggcaggtaaatgcatggactaaactattggcaggtgctacaagagtatcccacaaacatacgtttcaggtatggcttaggcatgcttccagtaactggacaacatttccagtttgtttgatacaaacttaaatatccatcagcatcaactattccaaacttatttccctgatagttaaatctcattcttgtaactcttgaattgccaccagatcgaaaacaggttatttgttgagaatggccccattcaaacattctgacacttccatcttgagctcctgtcagatagtaaggaagagttggatgagaagtcattcttctaacattattaatggctttcttaatcatcacagatgctcctctgccagtctgtgtactaccaagccatggcatgttgattggagtgccaggattgctatgtgtatatggagttgtaccttgaacagctgttaaatcatcacgagcatgtataaccaagaaatcttctgatcctttggtttccacttctatatcatcatctacccaagtgtagacctgtgtggccagaattccagaaacatccagttcttgaacatcatgactggaagcgattgctatgcagtttctatttgccttattaacagcaaacgcagtaatgatatcagattccttatgaataattcttgctttacctccaggatatcccaaatctgcttctatctcatttagacaccgtttctttgtgaatatatttttgataaaggtttcctgaatttcttcctgcttcaccaaatactgccaaagcctcttcacagacagtgccagatggtgtttggatttgaaaggagtgtttgtaggttccagtaaagctttgtggcgaagaattgcaggacctgcagacaaactctcttcggcggtatgacttgcgatataattttgaggtggcccaccatggatttcaagtcgtcggagaagaacttgttcccaacattgaagagtttttagaaccgcatgacaaagaggtgaactaactggaagctctgcaagatcatgacctgcgaagggataaaaagtcttcaaattgttgagcaccaattgcaccatcgccaaccgcatcaaggaccaactatatgaatttgaattagaatgttcctggagatggaaatctgatgctaaaacatcatcatcatcatcattgtcatcatcatcacttcccagactctcctctgaatcatattcggctctactttgagaagagggtagaaaaggcttagctatgaaatagtcccagatactgagctcaggtgggatgaacttttctttaaccgccagtgactcctggcttactggtgccgaggaaggggtcagtggggcagattctctgcaagacatttttgacggcctaaaacgtttgttctgtttttctccttcttcaactagtgaagaaactgcaagactgggagggctatgagaactgatggctgaaagagctttggaaaagcccacacattccatggagaataccactacctggtgggggctaggcatagcaaagtgccttccaggtaaagtttttgaatgtgtctgttctttgctaggaacatgtgcacctccaccaaacacagcagaccacattttctcatttagaggatgggccacaatccgaaatagctcattacttgaatgtgtggccaggccatggatgaagagactaagatacactgctgtgagaatctcacagagcaagactgtaagccctgactgggcttcctcgccagaagaattcaaaagtcgaattagacaagttattcctggccattgagctggtgacgtattgggagttaatgcttcatctaagcttcctgttttcaaagaaggtcgatgaggaagcagtactgtctgatataccattccagtaaactgattcgtctgaaatgaactgtagttatgactaccacaaaggcactgataaatacaagcagaaagtgaagctgctaaagtatgcattacatacactttattgctttggatatcagggtggggtggtgaatcaaagtttattatggcatggagaatatcatgtgtcagattactaaggtgcaataatggattggcaactactgttttggcattggctgtacaagcaaagaggagaggcactgaggtttgctctgacagagggctagaaaatagtggttctgatgtttcctgctgagattcttgcaaaagcaaaatcaattccattcttacagatgcaagacccccaccatgggatccatgaagtatgcagtaactaagaaacattctcaaaagtgactgatacttcaagagccactgtcttttttcctgaaaattttctctcagttgtttcacttttgtttggtgaggcaaatcttcagcatcctcatttaatccaaattcatcttcatttctgccaaatgcagactgtagttcttcagcatctgagcaaaagtcacaagtcctctgaagagctatcacctctttttcaagccagtggtatagttggtaacgcaattttccaccatctatttcatagccagtagataaagtacgaagttctactgtgagaatctttaaacatgctctaaattttaactgaactgcaattatatcttctgatggatttaaaaggtcattttcatctagtgtgctgaaagattctgtgtagttagaacttatgtcatccaactttttatctgtttttctctgtaaaggttttagttctttcattgaaatagggacatcctcattttcttcatcattatcactgtcccattttaactctaaagagtcatcctgaaacacaacacttggttggctccagtcaaaagaaagagtggagtttgattgcttctctgaggaaccctctgaagaagatccaaaaccatttatcagtgactgtgaccaatcaacagcagaagacttatcttcccttgcatccaactttaatggagaagaaggagaacagtctttactagtatccagaaaactagaagccctataaaaaggtcttgttttcttgatgactttaggcatctttgataatacttccaaagccaacattgggcagccagcttttaaatgagcactggcagtggtaaaaaataaacgtctttcacttaaattaattgttcctgccagtccactttttcctgttaggctcatatgtgtggaaaatgtatcagatgatccaaaatgacgtctcagcaaaagaggatgtgttcttagataattgtagaaattaaaaactgtaggattactggctgataaaacttgatcatcattctctctgataggttgctttattaatgtttccagagcaccactataatcttccaaaatccaatatgccatgctccgaagaaaaggatcatgatgcatatttatgttcaatgaacacagttcactgacaggagaatcgattcccaaaacttttttacgtaaaatagatttatatgctgcagatgtatcaaattcagactcatagagtcttgctattacaagagccaactgaatgtcattcaatttctcaagacatacctcaattgcatctctgaggcaaccagctaaaagaaaaaatgctgcagaatgttcaaatctttgtttgcctagcaaagaaaaagcattctttaaagctgctttacgccacctctcatcctcaaaattgtgtccaaaaaactgtgtcatcctggtgtttttttcagctctatataatccccaaatcacagctttctttttcattgcaaggtaaaaaatggcagcatctaaaggatcattctttctataaaaggctgctttagctactttttctatgcatttgcgtaagatgcgggtattccggacccaccaccccacacccatagctcttagttcagaccaagtgggatcatctttctgcatggctggcaacatgttcagcagttcttcttctgctactgagtgaaatgcccaagcaaaatgacttgtagacaggccttggtgaaggagttgagctcgataggctggaagggaagttgtaagaaaggtatggagtcgaacagccaaaagaaattttaacccacattcatcaagagtttctccaccttggcttctgtctcggctttctccaatatcagtgcttgtagttgcaattgtatctgctaaggccatcaaagacatctgctccatccggctgagtcctggtaaactagaatgaagtaagtggccagaaagaacctgagcatgctcaggtccaaagtaagtcggactgtactgtgaaaggtcaataactctaggctttgtattttcttcatctgtctctaacatatgagtatcagtcattagaagttgagtctgaaaaagctcatcataactttctttagataattggtttgatttacttaacgtactctcattactagatttctccaaagatgagtaacagctatcatcatctgctgcaagtaaggcatataaaggaagtggaggaacagaatctatttctgtgtaatctgtattttcagccttgttgaatgcctgggggtctctggtagtgcttccactagcactgattgtgagagacctaaggcggcgttcatgattagattcagcttcattcagagccacaacttccccagcaatgcacttaacaagatgggacaagatggccttggctctccgaactttaccaagatccatgagttccaaaagctgcaagggatgatactgaggtagagtcggggaaagtacatgagctgcttcaaaaagacctgaatcttccatatccactgaaggatcgaatgcagttttctttccacagattttctgtgcaagactggtcatggatcgagtcagagttttctttggaggatgtaacccagaactggagttactctgttttattaaacttgttatagatggagtgctcccactgtacgaatctgttataacaggttcttgtttagaagatggttgccattggcaatacacatgcatttcacagtccattcctaccacaaggatgccatcccggacccacgataaagaaacaggaaaaggtggggagccatctacagaagaaactaggtccacacttcgtaatagtacaaatttagaaaggggcacaactttggtactctcccagagaggaaatgccagggtttccttaccagtttggtcttgtaccttgccagccaggggtccatacataaaaagttttgatccaattcctacagtcaggatatgagaaccgtcttctctagacatccaatctaagtgaactaaatgctttgtgtttgatgtgatattctctttactagataaatacatgtcttgtttattataggccactaaattgctatcaacactaatgccagaatccaatactgtgcttaactcatctaaatgaattgtctgctcaaggacccaacatgaacctcctgttgactcacattcaaaaatacttacatgcatcacaaagtcctgggaagatctactattagatgcaggctgcttataagctactgctaaacgatttgtatgtgcacagctaacttctacaggcctaccaggtacagttatactactattgctctgaagtccatcttcaataagtaatggccattcttcccaaatgtatgcaagatcaatttttccattctttgacgtggcagattctccatctgttactctgcatctccagaatcttactttctcatctgaacatgaagttgccaataaataaggagcactgcatgcaggatatatagaagatgaactcagatgtcctgctgatggcttaatacttattatctcaactccttctggtaaatgcaattcttggctataaaccatttctgaaaacagagtcaacctgctggtactctggagatttgctctgcaagcctgatacttttgtgaaaaaggagataggatcttctctggagaagaagaataatgttcttctggctgccaaaccgcttcggataattttgtatctactttttcatctaatgagacaggaattgactttagatgtaaattccacatgtgtaacagtgaacggttgtcttgagtgcattctattacaattaggtagaacttctcagaaaatccattaggtgagctgcctgcattagataaaatgctgtctttgccaaggcttttcttctcaaggttattcaaaatgaagtcttcttcaaaaacatgaagcagttgggtttttctgccatgaagtttggtaatgggatctaatgcaataatgcatcctggcctggctgttgattgttgactgacgatgttaaagacttcaccaacatatttagaaatttcagggttagaaagctcagataaaagtttcttagcatcaataactgcttcatataatctcagatattgtccatcactggctacaaagcatgcactaggagagttgcagtatgcacccagacaataactgggtataagagtgggcagccatgccacattggaaaaggcagaaacatgaagagaattaatccgggcaagctcagaaactcctccagaaaaagacaatggcccaactgggtcaaccctccacagaataagctcactgtaaactgcactgggatcctgaaatgccacgtcaacagtgcttttattttgttgtgtcaaagagcattcttcaatatttagagcatcaaaaggttgctctgggttatcaacatctggtgtccttaatgcattatggtgtgatgttgtcagcaataatggtaatactgagtggcaagctaaatcattaagatgaaaacgatgaccacaatatctggatttgtgggaaatactgagaacagtagaaaaagcagattcctcggcaaaactgaccagccactgattcagagaaccatcagcatgttttgatatcatcataacattaggcgtaaaaatacttaattttaaactattagatgatttattgtgaccagaagaaataagcattgatgtggaacgggtgaggccagaaggtttttgtttcccctgctgaatagccaagtcaacattcttggtacaggcatacatcattatgcttttacagagagagtttgcatcacctgtggggaaagctactggaattctggaaacaaaggacacctgtacttgacgaaacataccaggctggtattcatccagccaatccacatgccaaactagcaaagaaccatccatgggatgaatactaaatagcatatctgcatttttactccattcagacagaagtacttcaatctgatgatcaatggcagctgacgataatgatgtaaaacttgagtttggtaccattttatcacagcctaattccttcttttcgggatttattttcagatcatcaacaccatcatcagtttcttcatcagattttacatctgcctgattagaatcttctacactggcctcagaagatggttgttcaaaactttttctaagttgctgtaaaaaaacttccatggacaaagtaaaatgcagttctttattgtttagccagtgtacaacaaaaggtccggtcttctcttcattttcatttagactcagagatgtaatagatggaagaagtggaatgtctgtggctgggttgatgctggctgcaatatgaaagtggcaaagtgcattggcatgcagtggagtgttcctgtgaacatgatgaggatcctgctgatgtggtagatatcccgtatgtgctacaagagcaagtgatctcctccgacctctacgaaaatgtctcagatttacttctaaagcattttgaactcgttctttactggaagcatttctcttgaagttatttgttaaattaattgattcagtccaatggctgcagtcacctccgtatagcaaacaatcatttggtaaaaatgtctctacccaaagacgacacacattatctttgcagcaagtcaacagtacattacatacagaagccctaggcatatatttgcttgttttacgccaggaaaatccatttactgctcgaggatgggccagatacacaaaagaaaagtcaatttctccttgggattgtttttctgaacttccatctggagaagtaacagctgtccgccagttttctacattataccaaaccttcaaaagacagtcatccttcccagcagtggcaaaaaattctccatctggtgaaaatttcattaaatgaacttgggaagcagttttgcaatgccaaatgcatttccaatctccaaagttaagatctgttttatttaaattttcatcttcagttggcttctccaagttagtattggaccagagttgcaaatagctggaaccagttaaaagacgactgcctgtgggatcccaggttatattgtgtgctattgattccagaaaaaattggccacttttctgccactgactatataattccaaatttttcttttgttttggtaggttaactggttcaaaaatggagataacatttccataagacgctgcaatcttgccttgttgcattgaacagtctacacatcccacttgaatatttccatgtttagctcctgggattatctgtaatctttcaaaatcgcttcccagtattacaatgtcacatccagatgcataagccgtgaagcgctggtcgccaatgctgcccacggagaagcagtggtcgccagggttcacagccccggtcagcacctggtgcaggttcatgtcggcgccctagtcctgcaacggacaccgcatccagctcatgccacgggtcagcggctgcttccctccctccttccctcaggggcggcggccgctcttcggtggcgacggcagaagcagcgacaggcgcctggagccggagccgctcagctggggcccgcgactcatcccgagccccggagggcgaggcccggagggggcgggtcggcgagagggcggagcgccgcgctccttcgcgcacctgtcactccccgcgctagcccaggtgaagctcagggtcccctcaccggccacgacccggggccgactcaccggccaggaaggccgcgctgtccacacacttcctctggacctcgggcagccgctcctgacccagcccgagtggcgcaagcagtacgcgctcgcactccccgcctgacctgtcccttcccggctccggtgcccgccacccccacagtcctccgccactcactacgcgcctctggatccctgcggccgaaatatcgcgagacttcgctcggggcag

SEQ ID NO: 9955 - RNA, 10298 nt, Homo sapiens
  source 1..10298: mol_type = other RNA
cacacacacacacacacgtatacatacatacaacttgggttccggagggtaaactactgaaaaccttacatattgagccatctagctcatttatcactgacgtctcaatgacaattttaatgaagatgttcattatttttttcattcttactcaaatacctatcattaattaagagaagagtttgagatgtataaggctaataaaggaagtgagagtgtggtgaattaagtgatgagtattatgtacaattgcctttacaaaaaacgtatttttactgtggaagaaattcatgcagagatgcctgtggaaaagtatcaataagaaaacaaaacacctttaacactatgacatactgattataatatactatgatatgtattattacagcattacttacacattctactttaggcaatgtaatctacttctgaatgaccttgttaatttttaaggcatcagtgcatcaagggcaaagctccataaaataaatataaaaacaagaaagcattagctaatttgtggcatagagaatgatcactgtatattatatctgttggccacttccatataggtaataaattgtacatcttattgtaaaaatgttatagcataaatttcacatcatttttcaacacttcatttaaagggctaaactgatctggcagtattctcattttcattgttccatcagctccacaggagaaaatgtgatttgcaggccctgtctcaatttgcatcactccagttccaatatttctaaaaatggactgccgagcatgttcactgacaaaagtatggagaagaccaaaggtagagagactccaaatctttatattgccttcggcagatcctgtaacaaagtactcttcagttggatcaacagcaacggctttaacaggagaatcatggctctggaaaagctgcctctgttgtcgttgacaaaggtcaaatacatatgtaaaaccttttctgccacctgatattagtagctgatgttttggagcatatgctaaaactgtggctccactgtcatggcaggtaaatgcatggactaaactattggcaggtgctacaagagtatcccacaaacatacgtttcaggtatggcttaggcatgcttccagtaactggacaacatttccagtttgtttgatacaaacttaaatatccatcagcatcaactattccaaacttatttccctgatagttaaatctcattcttgtaactcttgaattgccaccagatcgaaaacaggttatttgttgagaatggccccattcaaacattctgacacttccatcttgagctcctgtcagatagtaaggaagagttggatgagaagtcattcttctaacattattaatggctttcttaatcatcacagatgctcctctgccagtctgtgtactaccaagccatggcatgttgattggagtgccaggattgctatgtgtatatggagttgtaccttgaacagctgttaaatcatcacgagcatgtataaccaagaaatcttctgatcctttggtttccacttctatatcatcatctacccaagtgtagacctgtgtggccagaattccagaaacatccagttcttgaacatcatgactggaagcgattgctatgcagtttctatttgccttattaacagcaaacgcagtaatgatatcagattccttatgaataattcttgctttacctccaggatatcccaaatctgcttctatcttattgatgtttggctcctccatcatagaatttttgatggtttcactgttgtcctctaatgactcatttagacaccgtttctttgtgaatatatttttgataaaggtttcctgaatttcttcctgcttcaccaaatactgccaaagcctcttcacagacagtgccagatggtgtttggatttgaaaggagtgtttgtaggttccagtaaagctttgtggcgaagaattgcaggacctgcagacaaactctcttcggcggtatgacttgcgatataattttgaggtggcccaccatggatttcaagtcgtcggagaagaacttgttcccaacattgaagagtttttagaaccgcatgacaaagaggtgaactaactggaagctctgcaagatcatgacctgcgaagggataaaaagtcttcaaattgttgagcaccaattgcaccatcgccaaccgcatcaaggaccaactatatgaatttgaattagaatgttcctggagatggaaatctgatgctaaaacatcatcatcatcatcattgtcatcatcatcacttcccagactctcctctgaatcatattcggctctactttgagaagagggtagaaaaggcttagctatgaaatagtcccagatactgagctcaggtgggatgaacttttctttaaccgccagtgactcctggcttactggtgccgaggaaggggtcagtggggcagattctctgcaagacatttttgacggcctaaaacgtttgttctgtttttctccttcttcaactagtgaagaaactgcaagactgggagggctatgagaactgatggctgaaagagctttggaaaagcccacacattccatggagaataccactacctggtgggggctaggcatagcaaagtgccttccaggtaaagtttttgaatgtgtctgttctttgctaggaacatgtgcacctccaccaaacacagcagaccacattttctcatttagaggatgggccacaatccgaaatagctcattacttgaatgtgtggccaggccatggatgaagagactaagatacactgctgtgagaatctcacagagcaagactgtaagccctgactgggcttcctcgccagaagaattcaaaagtcgaattagacaagttattcctggccattgagctggtgacgtattgggagttaatgcttcatctaagcttcctgttttcaaagaaggtcgatgaggaagcagtactgtctgatataccattccagtaaactgattcgtctgaaatgaactgtagttatgactaccacaaaggcactgataaatacaagcagaaagtgaagctgctaaagtatgcattacatacactttattgctttggatatcagggtggggtggtgaatcaaagtttattatggcatggagaatatcatgtgtcagattactaaggtgcaataatggattggcaactactgttttggcattggctgtacaagcaaagaggagaggcactgaggtttgctctgacagagggctagaaaatagtggttctgatgtttcctgctgagattcttgcaaaagcaaaatcaattccattcttacagatgcaagacccccaccatgggatccatgaagtatgcagtaactaagaaacattctcaaaagtgactgatacttcaagagccactgtcttttttcctgaaaattttctctcagttgtttcacttttgtttggtgaggcaaatcttcagcatcctcatttaatccaaattcatcttcatttctgccaaatgcagactgtagttcttcagcatctgagcaaaagtcacaagtcctctgaagagctatcacctctttttcaagccagtggtatagttggtaacgcaattttccaccatctatttcatagccagtagataaagtacgaagttctactgtgagaatctttaaacatgctctaaattttaactgaactgcaattatatcttctgatggatttaaaaggtcattttcatctagtgtgctgaaagattctgtgtagttagaacttatgtcatccaactttttatctgtttttctctgtaaaggttttagttctttcattgaaatagggacatcctcattttcttcatcattatcactgtcccattttaactctaaagagtcatcctgaaacacaacacttggttggctccagtcaaaagaaagagtggagtttgattgcttctctgaggaaccctctgaagaagatccaaaaccatttatcagtgactgtgaccaatcaacagcagaagacttatcttcccttgcatccaactttaatggagaagaaggagaacagtctttactagtatccagaaaactagaagccctataaaaaggtcttgttttcttgatgactttaggcatctttgataatacttccaaagccaacattgggcagccagcttttaaatgagcactggcagtggtaaaaaataaacgtctttcacttaaattaattgttcctgccagtccactttttcctgttaggctcatatgtgtggaaaatgtatcagatgatccaaaatgacgtctcagcaaaagaggatgtgttcttagataattgtagaaattaaaaactgtaggattactggctgataaaacttgatcatcattctctctgataggttgctttattaatgtttccagagcaccactataatcttccaaaatccaatatgccatgctccgaagaaaaggatcatgatgcatatttatgttcaatgaacacagttcactgacaggagaatcgattcccaaaacttttttacgtaaaatagatttatatgctgcagatgtatcaaattcagactcatagagtcttgctattacaagagccaactgaatgtcattcaatttctcaagacatacctcaattgcatctctgaggcaaccagctaaaagaaaaaatgctgcagaatgttcaaatctttgtttgcctagcaaagaaaaagcattctttaaagctgctttacgccacctctcatcctcaaaattgtgtccaaaaaactgtgtcatcctggtgtttttttcagctctatataatccccaaatcacagctttctttttcattgcaaggtaaaaaatggcagcatctaaaggatcattctttctataaaaggctgctttagctactttttctatgcatttgcgtaagatgcgggtattccggacccaccaccccacacccatagctcttagttcagaccaagtgggatcatctttctgcatggctggcaacatgttcagcagttcttcttctgctactgagtgaaatgcccaagcaaaatgacttgtagacaggccttggtgaaggagttgagctcgataggctggaagggaagttgtaagaaaggtatggagtcgaacagccaaaagaaattttaacccacattcatcaagagtttctccaccttggcttctgtctcggctttctccaatatcagtgcttgtagttgcaattgtatctgctaaggccatcaaagacatctgctccatccggctgagtcctggtaaactagaatgaagtaagtggccagaaagaacctgagcatgctcaggtccaaagtaagtcggactgtactgtgaaaggtcaataactctaggctttgtattttcttcatctgtctctaacatatgagtatcagtcattagaagttgagtctgaaaaagctcatcataactttctttagataattggtttgatttacttaacgtactctcattactagatttctccaaagatgagtaacagctatcatcatctgctgcaagtaaggcatataaaggaagtggaggaacagaatctatttctgtgtaatctgtattttcagccttgttgaatgcctgggggtctctggtagtgcttccactagcactgattgtgagagacctaaggcggcgttcatgattagattcagcttcattcagagccacaacttccccagcaatgcacttaacaagatgggacaagatggccttggctctccgaactttaccaagatccatgagttccaaaagctgcaagggatgatactgaggtagagtcggggaaagtacatgagctgcttcaaaaagacctgaatcttccatatccactgaaggatcgaatgcagttttctttccacagattttctgtgcaagactggtcatggatcgagtcagagttttctttggaggatgtaacccagaactggagttactctgttttattaaacttgttatagatggagtgctcccactgtacgaatctgttataacaggttcttgtttagaagatggttgccattggcaatacacatgcatttcacagtccattcctaccacaaggatgccatcccggacccacgataaagaaacaggaaaaggtggggagccatctacagaagaaactaggtccacacttcgtaatagtacaaatttagaaaggggcacaactttggtactctcccagagaggaaatgccagggtttccttaccagtttggtcttgtaccttgccagccaggggtccatacataaaaagttttgatccaattcctacagtcaggatatgagaaccgtcttctctagacatccaatctaagtgaactaaatgctttgtgtttgatgtgatattctctttactagataaatacatgtcttgtttattataggccactaaattgctatcaacactaatgccagaatccaatactgtgcttaactcatctaaatgaattgtctgctcaaggacccaacatgaacctcctgttgactcacattcaaaaatacttacatgcatcacaaagtcctgggaagatctactattagatgcaggctgcttataagctactgctaaacgatttgtatgtgcacagctaacttctacaggcctaccaggtacagttatactactattgctctgaagtccatcttcaataagtaatggccattcttcccaaatgtatgcaagatcaatttttccattctttgacgtggcagattctccatctgttactctgcatctccagaatcttactttctcatctgaacatgaagttgccaataaataaggagcactgcatgcaggatatatagaagatgaactcagatgtcctgctgatggcttaatacttattatctcaactccttctggtaaatgcaattcttggctataaaccatttctgaaaacagagtcaacctgctggtactctggagatttgctctgcaagcctgatacttttgtgaaaaaggagataggatcttctctggagaagaagaataatgttcttctggctgccaaaccgcttcggataattttgtatctactttttcatctaatgagacaggaattgactttagatgtaaattccacatgtgtaacagtgaacggttgtcttgagtgcattctattacaattaggtagaacttctcagaaaatccattaggtgagctgcctgcattagataaaatgctgtctttgccaaggcttttcttctcaaggttattcaaaatgaagtcttcttcaaaaacatgaagcagttgggtttttctgccatgaagtttggtaatgggatctaatgcaataatgcatcctggcctggctgttgattgttgactgacgatgttaaagacttcaccaacatatttagaaatttcagggttagaaagctcagataaaagtttcttagcatcaataactgcttcatataatctcagatattgtccatcactggctacaaagcatgcactaggagagttgcagtatgcacccagacaataactgggtataagagtgggcagccatgccacattggaaaaggcagaaacatgaagagaattaatccgggcaagctcagaaactcctccagaaaaagacaatggcccaactgggtcaaccctccacagaataagctcactgtaaactgcactgggatcctgaaatgccacgtcaacagtgcttttattttgttgtgtcaaagagcattcttcaatatttagagcatcaaaaggttgctctgggttatcaacatctggtgtccttaatgcattatggtgtgatgttgtcagcaataatggtaatactgagtggcaagctaaatcattaagatgaaaacgatgaccacaatatctggatttgtgggaaatactgagaacagtagaaaaagcagattcctcggcaaaactgaccagccactgattcagagaaccatcagcatgttttgatatcatcataacattaggcgtaaaaatacttaattttaaactattagatgatttattgtgaccagaagaaataagcattgatgtggaacgggtgaggccagaaggtttttgtttcccctgctgaatagccaagtcaacattcttggtacaggcatacatcattatgcttttacagagagagtttgcatcacctgtggggaaagctactggaattctggaaacaaaggacacctgtacttgacgaaacataccaggctggtattcatccagccaatccacatgccaaactagcaaagaaccatccatgggatgaatactaaatagcatatctgcatttttactccattcagacagaagtacttcaatctgatgatcaatggcagctgacgataatgatgtaaaacttgagtttggtaccattttatcacagcctaattccttcttttcgggatttattttcagatcatcaacaccatcatcagtttcttcatcagattttacatctgcctgattagaatcttctacactggcctcagaagatggttgttcaaaactttttctaagttgctgtaaaaaaacttccatggacaaagtaaaatgcagttctttattgtttagccagtgtacaacaaaaggtccggtcttctcttcattttcatttagactcagagatgtaatagatggaagaagtggaatgtctgtggctgggttgatgctggctgcaatatgaaagtggcaaagtgcattggcatgcagtggagtgttcctgtgaacatgatgaggatcctgctgatgtggtagatatcccgtatgtgctacaagagcaagtgatctcctccgacctctacgaaaatgtctcagatttacttctaaagcattttgaactcgttctttactggaagcatttctcttgaagttatttgttaaattaattgattcagtccaatggctgcagtcacctccgtatagcaaacaatcatttggtaaaaatgtctctacccaaagacgacacacattatctttgcagcaagtcaacagtacattacatacagaagccctaggcatatatttgcttgttttacgccaggaaaatccatttactgctcgaggatgggccagatacacaaaagaaaagtcaatttctccttgggattgtttttctgaacttccatctggagaagtaacagctgtccgccagttttctacattataccaaaccttcaaaagacagtcatccttcccagcagtggcaaaaaattctccatctggtgaaaatttcattaaatgaacttgggaagcagttttgcaatgccaaatgcatttccaatctccaaagttaagatctgttttatttaaattttcatcttcagttggcttctccaagttagtattggaccagagttgcaaatagctggaaccagttaaaagacgactgcctgtgggatcccaggttatattgtgtgctattgattccagaaaaaattggccacttttctgccactgactatataattccaaatttttcttttgttttggtaggttaactggttcaaaaatggagataacatttccataagacgctgcaatcttgccttgttgcattgaacagtctacacatcccacttgaatatttccatgtttagctcctgggattatctgtaatctttcaaaatcgcttcccagtattacaatgtcacatccagatgcataagccgtgaagcgctggtcgccaatgctgcccacggagaagcagtggtcgccagggttcacagccccggtcagcacctggtgcaggttcatgtcggcgccctagtcctgcaacggacaccgcatccagctcatgccacgggtcagcggctgcttccctccctccttccctcaggggcggcggccgctcttcggtggcgacggcagaagcagcgacaggcgcctggagccggagccgctcagctggggcccgcgactcatcccgagccccggagggcgaggcccggagggggcgggtcggcgagagggcggagcgccgcgctccttcgcgcacctgtcactccccgcgctagcccaggtgaagctcagggtcccctcaccggccacgacccggggccgactcaccggccaggaaggccgcgctgtccacacacttcctctggacctcgggcagccgctcctgacccagcccgagtggcgcaagcagtacgcgctcgcactccccgcctgacctgtcccttcccggctccggtgcccgccacccccacagtcctccgccactcactacgcgcctctggatccctgcggccgaaatatcgcgagacttcgctcggggcag

SEQ ID NO: 9956 - RNA, 9681 nt, Homo sapiens
  source 1..9681: mol_type = other RNA
cacacacacacacacacgtatacatacatacaacttgggttccggagggtaaactactgaaaaccttacatattgagccatctagctcatttatcactgacgtctcaatgacaattttaatgaagatgttcattatttttttcattcttactcaaatacctatcattaattaagagaagagtttgagatgtataaggctaataaaggaagtgagagtgtggtgaattaagtgatgagtattatgtacaattgcctttacaaaaaacgtatttttactgtggaagaaattcatgcagagatgcctgtggaaaagtatcaataagaaaacaaaacacctttaacactatgacatactgattataatatactatgatatgtattattacagcattacttacacattctactttaggcaatgtaatctacttctgaatgaccttgttaatttttaaggcatcagtgcatcaagggcaaagctccataaaataaatataaaaacaagaaagcattagctaatttgtggcatagagaatgatcactgtatattatatctgttggccacttccatataggtaataaattgtacatcttattgtaaaaatgttatagcataaatttcacatcatttttcaacacttcatttaaagggctaaactgatctggcagtattctcattttcattgttccatcagctccacaggagaaaatgtgatttgcaggccctgtctcaatttgcatcactccagttccaatatttctaaaaatggactgccgagcatgttcactgacaaaagtatggagaagaccaaaggtagagagactccaaatctttatattgccttcggcagatcctgtaacaaagtactcttcagttggatcaacagcaacggctttaacaggagaatcatggctctggaaaagctgcctctgttgtcgttgacaaaggtcaaatacatatgtaaaaccttttctgccacctgatattagtagctgatgttttggagcatatgctaaaactgtggctccactgtcatggcaggtaaatgcatggactaaactattggcaggtgctacaagagtatcccacaaacatacgtttctattgtcagttgaaagaccagctgtagctatcagagaggaggaactaacgaagacaaaatcattggctgttttgttatgacactgccaagtcaggtatggcttaggcatgcttccagtaactggacaacatttccagtttgtttgatacaaacttaaatatccatcagcatcaactattccaaacttatttccctgatagttaaatctcattcttgtaactcttgaattgccaccagatcgaaaacaggttatttgttgagaatggccccattcaaacattctgacacttccatcttgagctcctgtcagatagtaaggaagagttggatgagaagtcattcttctaacattattaatggctttcttaatcatcacagatgctcctctgccagtctgtgtactaccaagccatggcatgttgattggagtgccaggattgctatgtgtatatggagttgtaccttgaacagctgttaaatcatcacgagcatgtataaccaagaaatcttctgatcctttggtttccacttctatatcatcatctacccaagtgtagacctgtgtggccagaattccagaaacatccagttcttgaacatcatgactggaagcgattgctatgcagtttctatttgccttattaacagcaaacgcagtaatgatatcagattccttatgaataattcttgctttacctccaggatatcccaaatctgcttctatctcatttagacaccgtttctttgtgaatatatttttgataaaggtttcctgaatttcttcctgcttcaccaaatactgccaaagcctcttcacagacagtgccagatggtgtttggatttgaaaggagtgtttgtaggttccagtaaagctttgtggcgaagaattgcaggacctgcagacaaactctcttcggcggtatgacttgcgatataattttgaggtggcccaccatggatttcaagtcgtcggagaagaacttgttcccaacattgaagagtttttagaaccgcatgacaaagaggtgaactaactggaagctctgcaagatcatgacctgcgaagggataaaaagtcttcaaattgttgagcaccaattgcaccatcgccaaccgcatcaaggaccaactatatgaatttgaattagaatgttcctggagatggaaatctgatgctaaaacatcatcatcatcatcattgtcatcatcatcacttcccagactctcctctgaatcatattcggctctactttgagaagagggtagaaaaggcttagctatgaaatagtcccagatactgagctcaggtgggatgaacttttctttaaccgccagtgactcctggcttactggtgccgaggaaggggtcagtggggcagattctctgcaagacatttttgacggcctaaaacgtttgttctgtttttctccttcttcaactagtgaagaaacaggtaaagtttttgaatgtgtctgttctttgctaggaacatgtgcacctccaccaaacacagcagaccacattttctcatttagaggatgggccacaatccgaaatagctcattacttgaatgtgtggccaggccatggatgaagagactaagatacactgctgtgagaatctcacagagcaagactgtaagccctgactgggcttcctcgccagaagaattcaaaagtcgaattagacaagttattcctggccattgagctggtgacgtattgggagttaatgcttcatctaagcttcctgttttcaaagaaggtcgatgaggaagcagtactgtctgatataccattccagtaaactgattcgtctgaaatgaactgtagttatgactaccacaaaggcactgataaatacaagcagaaagtgaagctgctaaagtatgcattacatacacctgctgagattcttgcaaaagcaaaatcaattccattcttacagatgcaagacccccaccatgggatccatgaagtatgcagtaactaagaaacattctcaaaagtgactgatacttcaagagccactgtcttttttcctgaaaattttctctcagttgtttcacttttgtttggtgaggcaaatcttcagcatcctcatttaatccaaattcatcttcatttctgccaaatgcagactgtagttcttcagcatctgagcaaaagtcacaagtcctctgaagagctatcacctctttttcaagccagtggtatagttggtaacgcaattttccaccatctatttcatagccagtagataaagtacgaagttctactgtgagaatctttaaacatgctctaaattttaactgaactgcaattatatcttctgatggatttaaaaggtcattttcatctagtgtgctgaaagattctgtgtagttagaacttatgtcatccaactttttatctgtttttctctgtaaaggttttagttctttcattgaaatagggacatcctcattttcttcatcattatcactgtcccattttaactctaaagagtcatcctgaaacacaacacttggttggctccagtcaaaagaaagagtggagtttgattgcttctctgaggaaccctctgaagaagatccaaaaccatttatcagtgactgtgaccaatcaacagcagaagacttatcttcccttgcatccaactttaatggagaagaaggagaacagtctttactagtatccagaaaactagaagccctataaaaaggtcttgttttcttgatgactttaggcatctttgataatacttccaaagccaacattgggcagccagcttttaaatgagcactggcagtggtaaaaaataaacgtctttcacttaaattaattgttcctgccagtccactttttcctgttaggctcatatgtgtggaaaatgtatcagatgatccaaaatgacgtctcagcaaaagaggatgtgttcttagataattgtagaaattaaaaactgtaggattactggctgataaaacttgatcatcattctctctgataggttgctttattaatgtttccagagcaccactataatcttccaaaatccaatatgccatgctccgaagaaaaggatcatgatgcatatttatgttcaatgaacacagttcactgacaggagaatcgattcccaaaacttttttacgtaaaatagatttatatgctgcagatgtatcaaattcagactcatagagtcttgctattacaagagccaactgaatgtcattcaatttctcaagacatacctcaattgcatctctgaggcaaccagctaaaagaaaaaatgctgcagaatgttcaaatctttgtttgcctagcaaagaaaaagcattctttaaagctgctttacgccacctctcatcctcaaaattgtgtccaaaaaactgtgtcatcctggtgtttttttcagctctatataatccccaaatcacagctttctttttcattgcaaggtaaaaaatggcagcatctaaaggatcattctttctataaaaggctgctttagctactttttctatgcatttgcgtaagatgcgggtattccggacccaccaccccacacccatagctcttagttcagaccaagtgggatcatctttctgcatggctggcaacatgttcagcagttcttcttctgctactgagtgaaatgcccaagcaaaatgacttgtagacaggccttggtgaaggagttgagctcgataggctggaagggaagttgtaagaaaggtatggagtcgaacagccaaaagaaattttaacccacattcatcaagagtttctccaccttggcttctgtctcggctttctccaatatcagtgcttgtagttgcaattgtatctgctaaggccatcaaagacatctgctccatccggctgagtcctggtaaactagaatgaagtaagtggccagaaagaacctgagcatgctcaggtccaaagtaagtcggactgtactgtgaaaggtcaataactctaggctttgtattttcttcatctgtctctaacatatgagtatcagtcattagaagttgagtctgaaaaagctcatcataactttctttagataattggtttgatttacttaacgtactctcattactagatttctccaaagatgagtaacagctatcatcatctgctgcaagtaaggcatataaaggaagtggaggaacagaatctatttctgtgtaatctgtattttcagccttgttgaatgcctgggggtctctggtagtgcttccactagcactgattgtgagagacctaaggcggcgttcatgattagattcagcttcattcagagccacaacttccccagcaatgcacttaacaagatgggacaagatggccttggctctccgaactttaccaagatccatgagttccaaaagctgcaagggatgatactgaggtagagtcggggaaagtacatgagctgcttcaaaaagacctgaatcttccatatccactgaaggatcgaatgcagttttctttccacagattttctgtgcaagactggtcatggatcgagtcagagttttctttggaggatgtaacccagaactggagttactctgttttattaaacttgttatagatggagtgctcccactgtacgaatctgttataacaggttcttgtttagaagatggttgccattggcaatacacatgcatttcacagtccattcctaccacaaggatgccatcccggacccacgataaagaaacaggaaaaggtggggagccatctacagaagaaactaggtccacacttcgtaatagtacaaatttagaaaggggcacaactttggtactctcccagagaggaaatgccagggtttccttaccagtttggtcttgtaccttgccagccaggggtccatacataaaaagttttgatccaattcctacagtcaggatatgagaaccgtcttctctagacatccaatctaagtgaactaaatgctttgtgtttgatgtgatattctctttactagataaatacatgtcttgtttattataggccactaaattgctatcaacactaatgccagaatccaatactgtgcttaactcatctaaatgaattgtctgctcaaggacccaacatgaacctcctgttgactcacattcaaaaatacttacatgcatcacaaagtcctgggaagatctactattagatgcaggctgcttataagctactgctaaacgatttgtatgtgcacagctaacttctacaggcctaccaggtacagttatactactattgctctgaagtccatcttcaataagtaatggccattcttcccaaatgtatgcaagatcaatttttccattctttgacgtggcagattctccatctgttactctgcatctccagaatcttactttctcatctgaacatgaagttgccaataaataaggagcactgcatgcaggatatatagaagatgaactcagatgtcctgctgatggcttaatacttattatctcaactccttctggtaaatgcaattcttggctataaaccatttctgaaaacagagtcaacctgctggtactctggagatttgctctgcaagcctgatacttttgtgaaaaaggagataggatcttctctggagaagaagaataatgttcttctggctgccaaaccgcttcggataattttgtatctactttttcatctaatgagacaggaattgactttagatgtaaattccacatgtgtaacagtgaacggttgtcttgagtgcattctattacaattaggtagaacttctcagaaaatccattaggtgagctgcctgcattagataaaatgctgtctttgccaaggcttttcttctcaaggttattcaaaatgaagtcttcttcaaaaacatgaagcagttgggtttttctgccatgaagtttggtaatgggatctaatgcaataatgcatcctggcctggctgttgattgttgactgacgatgttaaagacttcaccaacatatttagaaatttcagggttagaaagctcagataaaagtttcttagcatcaataactgcttcatataatctcagatattgtccatcactggctacaaagcatgcactaggagagttgcagtatgcacccagacaataactgggtataagagtgggcagccatgccacattggaaaaggcagaaacatgaagagaattaatccgggcaagctcagaaactcctccagaaaaagacaatggcccaactgggtcaaccctccacagaataagctcactgtaaactgcactgggatcctgaaatgccacgtcaacagtgcttttattttgttgtgtcaaagagcattcttcaatatttagagcatcaaaaggttgctctgggttatcaacatctggtgtccttaatgcattatggtgtgatgttgtcagcaataatggtaatactgagtggcaagctaaatcattaagatgaaaacgatgaccacaatatctggatttgtgggaaatactgagaacagtagaaaaagcagattcctcggcaaaactgaccagccactgattcagagaaccatcagcatgttttgatatcatcataacattaggcgtaaaaatacttaattttaaactattagatgatttattgtgaccagaagaaataagcattgatgtggaacgggtgaggccagaaggtttttgtttcccctgctgaatagccaagtcaacattcttggtacaggcatacatcattatgcttttacagagagagtttgcatcacctgtggggaaagctactggaattctggaaacaaaggacacctgtacttgacgaaacataccaggctggtattcatccagccaatccacatgccaaactagcaaagaaccatccatgggatgaatactaaatagcatatctgcatttttactccattcagacagaagtacttcaatctgatgatcaatggcagctgacgataatgatgtaaaacttgagtttggtaccattttatcacagcctaattccttcttttcgggatttattttcagatcatcaacaccatcatcagtttcttcatcagattttacatctgcctgattagaatcttctacactggcctcagaagatggttgttcaaaactttttctaagttgctgtaaaaaaacttccatggacaaagtaaaatgcagttctttattgtttagccagtgtacaacaaaaggtccggtcttctcttcattttcatttagactcagagatgtaatagatggaagaagtggaatgtctgtggctgggttgatgctggctgcaatatgaaagtggcaaagtgcattggcatgcagtggagtgttcctgtgaacatgatgaggatcctgctgatgtggtagatatcccgtatgtgctacaagagcaagtgatctcctccgacctctacgaaaatgtctcagatttacttctaaagcattttgaactcgttctttactggaagcatttctcttgaagttatttgttaaattaattgattcagtccaatggctgcagtcacctccgtatagcaaacaatcatttggtaaaaatgtctctacccaaagacgacacacattatctttgcagcaagtcaacagtacattacatacagaagccctaggcatatatttgcttgttttacgccaggaaaatccatttactgctcgaggatgggccagatacacaaaagaaaagtcaatttctccttgggattgtttttctgaacttccatctggagaagtaacagctgtccgccagttttctacattataccaaaccttcaaaagacagtcatccttcccagcagtggcaaaaaattctccatctggtgaaaatttcattaaatgaacttgggaagcagttttgcaatgccaaatgcatttccaatctccaaagttaagatctgttttatttaaattttcatcttcagttggcttctccaagttagtattggaccagagttgcaaatagctggaaccagttaaaagacgactgcctgtgggatcccaggttatattgtgtgctattgattccagaaaaaattggccacttttctgccactgactatataattccaaatttttcttttgttttggtaggttaactggttcaaaaatggagataacatttccataagacgctgcaatcttgccttgttgcattgaacagtctacacatcccacttgaatatttccatgtttagctcctgggattatctgtaatctttcaaaatcgcttcccagtattacaatgtcacatccagatgcataagccgtgaagcgctggtcgccaatgctgcccacggagaagcagtggtcgccagggttcacagccccggtcagcacctggtgcaggttcatgtcggcgccctagtccggccaggaaggccgcgctgtccacacacttcctctggacctcgggcagccgctcctgacccagcccgagtggcgcaagcagtacgcgctcgcactccccgcctgacctgtcccttcccggctccggtgcccgccacccccacagtcctccgccactcactacgcgcctct

SEQ ID NO: 9957 - RNA, 9465 nt, Homo sapiens
  source 1..9465: mol_type = other RNA
cacacacacacacacacgtatacatacatacaacttgggttccggagggtaaactactgaaaaccttacatattgagccatctagctcatttatcactgacgtctcaatgacaattttaatgaagatgttcattatttttttcattcttactcaaatacctatcattaattaagagaagagtttgagatgtataaggctaataaaggaagtgagagtgtggtgaattaagtgatgagtattatgtacaattgcctttacaaaaaacgtatttttactgtggaagaaattcatgcagagatgcctgtggaaaagtatcaataagaaaacaaaacacctttaacactatgacatactgattataatatactatgatatgtattattacagcattacttacacattctactttaggcaatgtaatctacttctgaatgaccttgttaatttttaaggcatcagtgcatcaagggcaaagctccataaaataaatataaaaacaagaaagcattagctaatttgtggcatagagaatgatcactgtatattatatctgttggccacttccatataggtaataaattgtacatcttattgtaaaaatgttatagcataaatttcacatcatttttcaacacttcatttaaagggctaaactgatctggcagtattctcattttcattgttccatcagctccacaggagaaaatgtgatttgcaggccctgtctcaatttgcatcactccagttccaatatttctaaaaatggactgccgagcatgttcactgacaaaagtatggagaagaccaaaggtagagagactccaaatctttatattgccttcggcagatcctgtaacaaagtactcttcagttggatcaacagcaacggctttaacaggagaatcatggctctggaaaagctgcctctgttgtcgttgacaaaggtcaaatacatatgtaaaaccttttctgccacctgatattagtagctgatgttttggagcatatgctaaaactgtggctccactgtcatggcaggtaaatgcatggactaaactattggcaggtgctacaagagtatcccacaaacatacgtttctattgtcagttgaaagaccagctgtagctatcagagaggaggaactaacgaagacaaaatcattggctgttttgttatgacactgccaagtcaggtatggcttaggcatgcttccagtaactggacaacatttccagtttgtttgatacaaacttaaatatccatcagcatcaactattccaaacttatttccctgatagttaaatctcattcttgtaactcttgaattgccaccagatcgaaaacaggttatttgttgagaatggccccattcaaacattctgacacttccatcttgagctcctgtcagatagtaaggaagagttggatgagaagtcattcttctaacattattaatggctttcttaatcatcacagatgctcctctgccagtctgtgtactaccaagccatggcatgttgattggagtgccaggattgctatgtgtatatggagttgtaccttgaacagctgttaaatcatcacgagcatgtataaccaagaaatcttctgatcctttggtttccacttctatatcatcatctacccaagtgtagacctgtgtggccagaattccagaaacatccagttcttgaacatcatgactggaagcgattgctatgcagtttctatttgccttattaacagcaaacgcagtaatgatatcagattccttatgaataattcttgctttacctccaggatatcccaaatctgcttctatctcatttagacaccgtttctttgtgaatatatttttgataaaggtttcctgaatttcttcctgcttcaccaaatactgccaaagcctcttcacagacagtgccagatggtgtttggatttgaaaggagtgtttgtaggttccagtaaagctttgtggcgaagaattgcaggacctgcagacaaactctcttcggcggtatgacttgcgatataattttgaggtggcccaccatggatttcaagtcgtcggagaagaacttgttcccaacattgaagagtttttagaaccgcatgacaaagaggtgaactaactggaagctctgcaagatcatgacctgcgaagggataaaaagtcttcaaattgttgagcaccaattgcaccatcgccaaccgcatcaaggaccaactatatgaatttgaattagaatgttcctggagatggaaatctgatgctaaaacatcatcatcatcatcattgtcatcatcatcacttcccagactctcctctgaatcatattcggctctactttgagaagagggtagaaaaggcttagctatgaaatagtcccagatactgagctcaggtgggatgaacttttctttaaccgccagtgactcctggcttactggtgccgaggaaggggtcagtggggcagattctctgcaagacatttttgacggcctaaaacgtttgttctgtttttctccttcttcaactagtgaagaaacaggtaaagtttttgaatgtgtctgttctttgctaggaacatgtgcacctccaccaaacacagcagaccacattttctcatttagaggatgggccacaatccgaaatagctcattacttgaatgtgtggccaggccatggatgaagagactaagatacactgctgtgagaatctcacagagcaagactgtaagccctgactgggcttcctcgccagaagaattcaaaagtcgaattagacaagttattcctggccattgagctggtgacgtattgggagttaatgcttcatctaagcttcctgttttcaaagaaggtcgatgaggaagcagtactgtctgatataccattccagtaaactgattcgtctgaaatgaactgtagttatgactaccacaaaggcactgataaatacaagcagaaagtgaagctgctaaagtatgcattacatacactttattgctttggatatcagggtggggtggtgaatcaaagtttattatggcatggagaatatcatgtgtcagattactaaggtgcaataatggattggcaactactgttttggcattggctgtacaagcaaagaggagaggcactgaggtttgctctgacagagggctagaaaatagtggttctgatgtttcctgctgagattcttgcaaaagcaaaatcaattccattcttacagatgcaagacccccaccatgggatccatgaagtatgcagtaactaagaaacattctcaaaagtgactgatacttcaagagccactgtcttttttcctgaaaattttctctcagttgtttcacttttgtttggtgaggcaaatcttcagcatcctcatttaatccaaattcatcttcatttctgccaaatgcagactgtagttcttcagcatctgagcaaaagtcacaagtcctctgaagagctatcacctctttttcaagccagtggtatagttggtaacgcaattttccaccatctatttcatagccagtagataaagtacgaagttctactgtgagaatctttaaacatgctctaaattttaactgaactgcaattatatcttctgatggatttaaaaggtcattttcatctagtgtgctgaaagattctgtgtagttagaacttatgtcatccaactttttatctgtttttctctgtaaaggttttagttctttcattgaaatagggacatcctcattttcttcatcattatcactgtcccattttaactctaaagagtcatcctgaaacacaacacttggttggctccagtcaaaagaaagagtggagtttgattgcttctctgaggaaccctctgaagaagatccaaaaccatttatcagtgactgtgaccaatcaacagcagaagacttatcttcccttgcatccaactttaatggagaagaaggagaacagtctttactagtatccagaaaactagaagccctataaaaaggtcttgttttcttgatgactttaggcatctttgataatacttccaaagccaacattgggcagccagcttttaaatgagcactggcagtggtaaaaaataaacgtctttcacttaaattaattgttcctgccagtccactttttcctgttaggctcatatgtgtggaaaatgtatcagatgatccaaaatgacgtctcagcaaaagaggatgtgttcttagataattgtagaaattaaaaactgtaggattactggctgataaaacttgatcatcattctctctgataggttgctttattaatgtttccagagcaccactataatcttccaaaatccaatatgccatgctccgaagaaaaggatcatgatgcatatttatgttcaatgaacacagttcactgacaggagaatcgattcccaaaacttttttacgtaaaatagatttatatgctgcagatgtatcaaattcagactcatagagtcttgctattacaagagccaactgaatgtcattcaatttctcaagacatacctcaattgcatctctgaggcaaccagctaaaagaaaaaatgctgcagaatgttcaaatctttgtttgcctagcaaagaaaaagcattctttaaagctgctttacgccacctctcatcctcaaaattgtgtccaaaaaactgtgtcatcctggtgtttttttcagctctatataatccccaaatcacagctttctttttcattgcaaggtaaaaaatggcagcatctaaaggatcattctttctataaaaggctgctttagctactttttctatgcatttgcgtaagatgcgggtattccggacccaccaccccacacccatagctcttagttcagaccaagtgggatcatctttctgcatggctggcaacatgttcagcagttcttcttctgctactgagtgaaatgcccaagcaaaatgacttgtagacaggccttggtgaaggagttgagctcgataggctggaagggaagttgtaagaaaggtatggagtcgaacagccaaaagaaattttaacccacattcatcaagagtttctccaccttggcttctgtctcggctttctccaatatcagtgcttgtagttgcaattgtatctgctaaggccatcaaagacatctgctccatccggctgagtcctggtaaactagaatgaagtaagtggccagaaagaacctgagcatgctcaggtccaaagtaagtcggactgtactgtgaaaggtcaataactctaggctttgtattttcttcatctgtctctaacatatgagtatcagtcattagaagttgagtctgaaaaagctcatcataactttctttagataattggtttgatttacttaacgtactctcattactagatttctccaaagatgagtaacagctatcatcatctgctgcaagtaaggcatataaaggaagtggaggaacagaatctatttctgtgtaatctgtattttcagccttgttgaatgcctgggggtctctggtagtgcttccactagcactgattgtgagagacctaaggcggcgttcatgattagattcagcttcattcagagccacaacttccccagcaatgcacttaacaagatgggacaagatggccttggctctccgaactttaccaagatccatgagttccaaaagctgcaagggatgatactgaggtagagtcggggaaagtacatgagctgcttcaaaaagacctgaatcttccatatccactgaaggatcgaatgcagttttctttccacagattttctgtgcaagactggtcatggatcgagtcagagttttctttggaggatgtaacccagaactggagttactctgttttattaaacttgttatagatggagtgctcccactgtacgaatctgttataacaggttcttgtttagaagatggttgccattggcaatacacatgcatttcacagtccattcctaccacaaggatgccatcccggacccacgataaagaaacaggaaaaggtggggagccatctacagaagaaactaggtccacacttcgtaatagtacaaatttagaaaggggcacaactttggtactctcccagagaggaaatgccagggtttccttaccagtttggtcttgtaccttgccagccaggggtccatacataaaaagttttgatccaattcctacagtcaggatatgagaaccgtcttctctagacatccaatctaagtgaactaaatgctttgtgtttgatgtgatattctctttactagataaatacatgtcttgtttattataggccactaaattgctatcaacactaatgccagaatccaatactgtgcttaactcatctaaatgaattgtctgctcaaggacccaacatgaacctcctgttgactcacattcaaaaatacttacatgcatcacaaagtcctgggaagatctactattagatgcaggctgcttataagctactgctaaacgatttgtatgtgcacagctaacttctacaggcctaccaggtacagttatactactattgctctgaagtccatcttcaataagtaatggccattcttcccaaatgtatgcaagatcaatttttccattctttgacgtggcagattctccatctgttactctgcatctccagaatcttactttctcatctgaacatgaagttgccaataaataaggagcactgcatgcaggatatatagaagatgaactcagatgtcctgctgatggcttaatacttattatctcaactccttctggtaaatgcaattcttggctataaaccatttctgaaaacagagtcaacctgctggtactctggagatttgctctgcaagcctgatacttttgtgaaaaaggagataggatcttctctggagaagaagaataatgttcttctggctgccaaaccgcttcggataattttgtatctactttttcatctaatgagacaggaattgactttagatgtaaattccacatgtgtaacagtgaacggttgtcttgagtgcattctattacaattaggtagaacttctcagaaaatccattaggtgagctgcctgcattagataaaatgctgtctttgccaaggcttttcttctcaaggttattcaaaatgaagtcttcttcaaaaacatgaagcagttgggtttttctgccatgaagtttggtaatgggatctaatgcaataatgcatcctggcctggctgttgattgttgactgacgatgttaaagacttcaccaacatatttagaaatttcagggttagaaagctcagataaaagtttcttagcatcaataactgcttcatataatctcagatattgtccatcactggctacaaagcatgcactaggagagttgcagtatgcaccaggctggtattcatccagccaatccacatgccaaactagcaaagaaccatccatgggatgaatactaaatagcatatctgcatttttactccattcagacagaagtacttcaatctgatgatcaatggcagctgacgataatgatgtaaaacttgagtttggtaccattttatcacagcctaattccttcttttcgggatttattttcagatcatcaacaccatcatcagtttcttcatcagattttacatctgcctgattagaatcttctacactggcctcagaagatggttgttcaaaactttttctaagttgctgtaaaaaaacttccatggacaaagtaaaatgcagttctttattgtttagccagtgtacaacaaaaggtccggtcttctcttcattttcatttagactcagagatgtaatagatggaagaagtggaatgtctgtggctgggttgatgctggctgcaatatgaaagtggcaaagtgcattggcatgcagtggagtgttcctgtgaacatgatgaggatcctgctgatgtggtagatatcccgtatgtgctacaagagcaagtgatctcctccgacctctacgaaaatgtctcagatttacttctaaagcattttgaactcgttctttactggaagcatttctcttgaagttatttgttaaattaattgattcagtccaatggctgcagtcacctccgtatagcaaacaatcatttggtaaaaatgtctctacccaaagacgacacacattatctttgcagcaagtcaacagtacattacatacagaagccctaggcatatatttgcttgttttacgccaggaaaatccatttactgctcgaggatgggccagatacacaaaagaaaagtcaatttctccttgggattgtttttctgaacttccatctggagaagtaacagctgtccgccagttttctacattataccaaaccttcaaaagacagtcatccttcccagcagtggcaaaaaattctccatctggtgaaaatttcattaaatgaacttgggaagcagttttgcaatgccaaatgcatttccaatctccaaagttaagatctgttttatttaaattttcatcttcagttggcttctccaagttagtattggaccagagttgcaaatagctggaaccagttaaaagacgactgcctgtgggatcccaggttatattgtgtgctattgattccagaaaaaattggccacttttctgccactgactatataattccaaatttttcttttgttttggtaggttaactggttcaaaaatggagataacatttccataagacgctgcaatcttgccttgttgcattgaacagtctacacatcccacttgaatatttccatgtttagctcctgggattatctgtaatctttcaaaatcgcttcccagtattacaatgtcacatccagatgcataagccgtgaagcgctggtcgccaatgctgcccacggagaagcagtggtcgccagggttcacagccccggtcagcacctggtgcaggttcatgtcggcgccctagtcctgcaacggacaccgcatccagctcatgccacgggtcagcggctgcttccctccctccttccctcaggggcggcggccgctcttcggtggcgacggcagaagcagcgacaggcgcctggagccggagccgctcagctggggcccgcgactcatcccgagccccggagggcgaggcccggagggggcgggtcggcgagagggcggagcgccgcgctccttcgcgcacctgtcactccccgcgctagcccaggtgaagctcagggtcccctcaccggccacgacccggggccgactcaccggccaggaaggccgcgctgtccacacacttcctctggacctcgggcagccgctcctgacccagcccgagtggcgcaagcagtacgcgctcgcactccccgcctgacctgtcccttcccggctccggtgcccgccacccccacagtcctccgccactcactacgcgcctct

SEQ ID NO: 9958 - RNA, 9873 nt, Homo sapiens
  source 1..9873: mol_type = other RNA
cacacacacacacacacgtatacatacatacaacttgggttccggagggtaaactactgaaaaccttacatattgagccatctagctcatttatcactgacgtctcaatgacaattttaatgaagatgttcattatttttttcattcttactcaaatacctatcattaattaagagaagagtttgagatgtataaggctaataaaggaagtgagagtgtggtgaattaagtgatgagtattatgtacaattgcctttacaaaaaacgtatttttactgtggaagaaattcatgcagagatgcctgtggaaaagtatcaataagaaaacaaaacacctttaacactatgacatactgattataatatactatgatatgtattattacagcattacttacacattctactttaggcaatgtaatctacttctgaatgaccttgttaatttttaaggcatcagtgcatcaagggcaaagctccataaaataaatataaaaacaagaaagcattagctaatttgtggcatagagaatgatcactgtatattatatctgttggccacttccatataggtaataaattgtacatcttattgtaaaaatgttatagcataaatttcacatcatttttcaacacttcatttaaagggctaaactgatctggcagtattctcattttcattgttccatcagctccacaggagaaaatgtgatttgcaggccctgtctcaatttgcatcactccagttccaatatttctaaaaatggactgccgagcatgttcactgacaaaagtatggagaagaccaaaggtagagagactccaaatctttatattgccttcggcagatcctgtaacaaagtactcttcagttggatcaacagcaacggctttaacaggagaatcatggctctggaaaagctgcctctgttgtcgttgacaaaggtcaaatacatatgtaaaaccttttctgccacctgatattagtagctgatgttttggagcatatgctaaaactgtggctccactgtcatggcaggtaaatgcatggactaaactattggcaggtgctacaagagtatcccacaaacatacgtttctattgtcagttgaaagaccagctgtagctatcagagaggaggaactaacgaagacaaaatcattggctgttttgttatgacactgccaagtcaggtatggcttaggcatgcttccagtaactggacaacatttccagtttgtttgatacaaacttaaatatccatcagcatcaactattccaaacttatttccctgatagttaaatctcattcttgtaactcttgaattgccaccagatcgaaaacaggttatttgttgagaatggccccattcaaacattctgacacttccatcttgagctcctgtcagatagtaaggaagagttggatgagaagtcattcttctaacattattaatggctttcttaatcatcacagatgctcctctgccagtctgtgtactaccaagccatggcatgttgattggagtgccaggattgctatgtgtatatggagttgtaccttgaacagctgttaaatcatcacgagcatgtataaccaagaaatcttctgatcctttggtttccacttctatatcatcatctacccaagtgtagacctgtgtggccagaattccagaaacatccagttcttgaacatcatgactggaagcgattgctatgcagtttctatttgccttattaacagcaaacgcagtaatgatatcagattccttatgaataattcttgctttacctccaggatatcccaaatctgcttctatctcatttagacaccgtttctttgtgaatatatttttgataaaggtttcctgaatttcttcctgcttcaccaaatactgccaaagcctcttcacagacagtgccagatggtgtttggatttgaaaggagtgtttgtaggttccagtaaagctttgtggcgaagaattgcaggacctgcagacaaactctcttcggcggtatgacttgcgatataattttgaggtggcccaccatggatttcaagtcgtcggagaagaacttgttcccaacattgaagagtttttagaaccgcatgacaaagaggtgaactaactggaagctctgcaagatcatgacctgcgaagggataaaaagtcttcaaattgttgagcaccaattgcaccatcgccaaccgcatcaaggaccaactatatgaatttgaattagaatgttcctggagatggaaatctgatgctaaaacatcatcatcatcatcattgtcatcatcatcacttcccagactctcctctgaatcatattcggctctactttgagaagagggtagaaaaggcttagctatgaaatagtcccagatactgagctcaggtgggatgaacttttctttaaccgccagtgactcctggcttactggtgccgaggaaggggtcagtggggcagattctctgcaagacatttttgacggcctaaaacgtttgttctgtttttctccttcttcaactagtgaagaaacaggtaaagtttttgaatgtgtctgttctttgctaggaacatgtgcacctccaccaaacacagcagaccacattttctcatttagaggatgggccacaatccgaaatagctcattacttgaatgtgtggccaggccatggatgaagagactaagatacactgctgtgagaatctcacagagcaagactgtaagccctgactgggcttcctcgccagaagaattcaaaagtcgaattagacaagttattcctggccattgagctggtgacgtattgggagttaatgcttcatctaagcttcctgttttcaaagaaggtcgatgaggaagcagtactgtctgatataccattccagtaaactgattcgtctgaaatgaactgtagttatgactaccacaaaggcactgataaatacaagcagaaagtgaagctgctaaagtatgcattacatacactttattgctttggatatcagggtggggtggtgaatcaaagtttattatggcatggagaatatcatgtgtcagattactaaggtgcaataatggattggcaactactgttttggcattggctgtacaagcaaagaggagaggcactgaggtttgctctgacagagggctagaaaatagtggttctgatgtttcctgctgagattcttgcaaaagcaaaatcaattccattcttacagatgcaagacccccaccatgggatccatgaagtatgcagtaactaagaaacattctcaaaagtgactgatacttcaagagccactgtcttttttcctgaaaattttctctcagttgtttcacttttgtttggtgaggcaaatcttcagcatcctcatttaatccaaattcatcttcatttctgccaaatgcagactgtagttcttcagcatctgagcaaaagtcacaagtcctctgaagagctatcacctctttttcaagccagtggtatagttggtaacgcaattttccaccatctatttcatagccagtagataaagtacgaagttctactgtgagaatctttaaacatgctctaaattttaactgaactgcaattatatcttctgatggatttaaaaggtcattttcatctagtgtgctgaaagattctgtgtagttagaacttatgtcatccaactttttatctgtttttctctgtaaaggttttagttctttcattgaaatagggacatcctcattttcttcatcattatcactgtcccattttaactctaaagagtcatcctgaaacacaacacttggttggctccagtcaaaagaaagagtggagtttgattgcttctctgaggaaccctctgaagaagatccaaaaccatttatcagtgactgtgaccaatcaacagcagaagacttatcttcccttgcatccaactttaatggagaagaaggagaacagtctttactagtatccagaaaactagaagccctataaaaaggtcttgttttcttgatgactttaggcatctttgataatacttccaaagccaacattgggcagccagcttttaaatgagcactggcagtggtaaaaaataaacgtctttcacttaaattaattgttcctgccagtccactttttcctgttaggctcatatgtgtggaaaatgtatcagatgatccaaaatgacgtctcagcaaaagaggatgtgttcttagataattgtagaaattaaaaactgtaggattactggctgataaaacttgatcatcattctctctgataggttgctttattaatgtttccagagcaccactataatcttccaaaatccaatatgccatgctccgaagaaaaggatcatgatgcatatttatgttcaatgaacacagttcactgacaggagaatcgattcccaaaacttttttacgtaaaatagatttatatgctgcagatgtatcaaattcagactcatagagtcttgctattacaagagccaactgaatgtcattcaatttctcaagacatacctcaattgcatctctgaggcaaccagctaaaagaaaaaatgctgcagaatgttcaaatctttgtttgcctagcaaagaaaaagcattctttaaagctgctttacgccacctctcatcctcaaaattgtgtccaaaaaactgtgtcatcctggtgtttttttcagctctatataatccccaaatcacagctttctttttcattgcaaggtaaaaaatggcagcatctaaaggatcattctttctataaaaggctgctttagctactttttctatgcatttgcgtaagatgcgggtattccggacccaccaccccacacccatagctcttagttcagaccaagtgggatcatctttctgcatggctggcaacatgttcagcagttcttcttctgctactgagtgaaatgcccaagcaaaatgacttgtagacaggccttggtgaaggagttgagctcgataggctggaagggaagttgtaagaaaggtatggagtcgaacagccaaaagaaattttaacccacattcatcaagagtttctccaccttggcttctgtctcggctttctccaatatcagtgcttgtagttgcaattgtatctgctaaggccatcaaagacatctgctccatccggctgagtcctggtaaactagaatgaagtaagtggccagaaagaacctgagcatgctcaggtccaaagtaagtcggactgtactgtgaaaggtcaataactctaggctttgtattttcttcatctgtctctaacatatgagtatcagtcattagaagttgagtctgaaaaagctcatcataactttctttagataattggtttgatttacttaacgtactctcattactagatttctccaaagatgagtaacagctatcatcatctgctgcaagtaaggcatataaaggaagtggaggaacagaatctatttctgtgtaatctgtattttcagccttgttgaatgcctgggggtctctggtagtgcttccactagcactgattgtgagagacctaaggcggcgttcatgattagattcagcttcattcagagccacaacttccccagcaatgcacttaacaagatgggacaagatggccttggctctccgaactttaccaagatccatgagttccaaaagctgcaagggatgatactgaggtagagtcggggaaagtacatgagctgcttcaaaaagacctgaatcttccatatccactgaaggatcgaatgcagttttctttccacagattttctgtgcaagactggtcatggatcgagtcagagttttctttggaggatgtaacccagaactggagttactctgttttattaaacttgttatagatggagtgctcccactgtacgaatctgttataacaggttcttgtttagaagatggttgccattggcaatacacatgcatttcacagtccattcctaccacaaggatgccatcccggacccacgataaagaaacaggaaaaggtggggagccatctacagaagaaactaggtccacacttcgtaatagtacaaatttagaaaggggcacaactttggtactctcccagagaggaaatgccagggtttccttaccagtttggtcttgtaccttgccagccaggggtccatacataaaaagttttgatccaattcctacagtcaggatatgagaaccgtcttctctagacatccaatctaagtgaactaaatgctttgtgtttgatgtgatattctctttactagataaatacatgtcttgtttattataggccactaaattgctatcaacactaatgccagaatccaatactgtgcttaactcatctaaatgaattgtctgctcaaggacccaacatgaacctcctgttgactcacattcaaaaatacttacatgcatcacaaagtcctgggaagatctactattagatgcaggctgcttataagctactgctaaacgatttgtatgtgcacagctaacttctacaggcctaccaggtacagttatactactattgctctgaagtccatcttcaataagtaatggccattcttcccaaatgtatgcaagatcaatttttccattctttgacgtggcagattctccatctgttactctgcatctccagaatcttactttctcatctgaacatgaagttgccaataaataaggagcactgcatgcaggatatatagaagatgaactcagatgtcctgctgatggcttaatacttattatctcaactccttctggtaaatgcaattcttggctataaaccatttctgaaaacagagtcaacctgctggtactctggagatttgctctgcaagcctgatacttttgtgaaaaaggagataggatcttctctggagaagaagaataatgttcttctggctgccaaaccgcttcggataattttgtatctactttttcatctaatgagacaggaattgactttagatgtaaattccacatgtgtaacagtgaacggttgtcttgagtgcattctattacaattaggtagaacttctcagaaaatccattaggtgagctgcctgcattagataaaatgctgtctttgccaaggcttttcttctcaaggttattcaaaatgaagtcttcttcaaaaacatgaagcagttgggtttttctgccatgaagtttggtaatgggatctaatgcaataatgcatcctggcctggctgttgattgttgactgacgatgttaaagacttcaccaacatatttagaaatttcagggttagaaagctcagataaaagtttcttagcatcaataactgcttcatataatctcagatattgtccatcactggctacaaagcatgcactaggagagttgcagtatgcacccagacaataactgggtataagagtgggcagccatgccacattggaaaaggcagaaacatgaagagaattaatccgggcaagctcagaaactcctccagaaaaagacaatggcccaactgggtcaaccctccacagaataagctcactgtaaactgcactgggatcctgaaatgccacgtcaacagtgcttttattttgttgtgtcaaagagcattcttcaatatttagagcatcaaaaggttgctctgggttatcaacatctggtgtccttaatgcattatggtgtgatgttgtcagcaataatggtaatactgagtggcaagctaaatcattaagatgaaaacgatgaccacaatatctggatttgtgggaaatactgagaacagtagaaaaagcagattcctcggcaaaactgaccagccactgattcagagaaccatcagcatgttttgatatcatcataacattaggcgtaaaaatacttaattttaaactattagatgatttattgtgaccagaagaaataagcattgatgtggaacgggtgaggccagaaggtttttgtttcccctgctgaatagccaagtcaacattcttggtacaggcatacatcattatgcttttacagagagagtttgcatcacctgtggggaaagctactggaattctggaaacaaaggacacctgtacttgacgaaacataccaggctggtattcatccagccaatccacatgccaaactagcaaagaaccatccatgggatgaatactaaatagcatatctgcatttttactccattcagacagaagtacttcaatctgatgatcaatggcagctgacgataatgatgtaaaacttgagtttggtaccattttatcacagcctaattccttcttttcgggatttattttcagatcatcaacaccatcatcagtttcttcatcagattttacatctgcctgattagaatcttctacactggcctcagaagatggttgttcaaaactttttctaagttgctgtaaaaaaacttccatggacaaagtaaaatgcagttctttattgtttagccagtgtacaacaaaaggtccggtcttctcttcattttcatttagactcagagatgtaatagatggaagaagtggaatgtctgtggctgggttgatgctggctgcaatatgaaagtggcaaagtgcattggcatgcagtggagtgttcctgtgaacatgatgaggatcctgctgatgtggtagatatcccgtatgtgctacaagagcaagtgatctcctccgacctctacgaaaatgtctcagatttacttctaaagcattttgaactcgttctttactggaagcatttctcttgaagttatttgttaaattaattgattcagtccaatggctgcagtcacctccgtatagcaaacaatcatttggtaaaaatgtctctacccaaagacgacacacattatctttgcagcaagtcaacagtacattacatacagaagccctaggcatatatttgcttgttttacgccaggaaaatccatttactgctcgaggatgggccagatacacaaaagaaaagtcaatttctccttgggattgtttttctgaacttccatctggagaagtaacagctgtccgccagttttctacattataccaaaccttcaaaagacagtcatccttcccagcagtggcaaaaaattctccatctggtgaaaatttcattaaatgaacttgggaagcagttttgcaatgccaaatgcatttccaatctccaaagttaagatctgttttatttaaattttcatcttcagttggcttctccaagttagtattggaccagagttgcaaatagctggaaccagttaaaagacgactgcctgtgggatcccaggttatattgtgtgctattgattccagaaaaaattggccacttttctgccactgactatataattccaaatttttcttttgttttggtaggttaactggttcaaaaatggagataacatttccataagacgctgcaatcttgccttgttgcattgaacagtctacacatcccacttgaatatttccatgtttagctcctgggattatctgtaatctttcaaaatcgcttcccagtattacaatgtcacatccagatgcataagccgtgaagcgctggtcgccaatgctgcccacggagaagcagtggtcgccagggttcacagccccggtcagcacctggtgcaggttcatgtcggcgccctagtccggccaggaaggccgcgctgtccacacacttcctctggacctcgggcagccgctcctgacccagcccgagtggcgcaagcagtacgcgctcgcactccccgcctgacctgtcccttcccggctccggtgcccgccacccccacagtcctccgccactcactacgcgcctct

SEQ ID NO: 9959 - RNA, 10170 nt, Homo sapiens
  source 1..10170: mol_type = other RNA
cacacacacacacacacgtatacatacatacaacttgggttccggagggtaaactactgaaaaccttacatattgagccatctagctcatttatcactgacgtctcaatgacaattttaatgaagatgttcattatttttttcattcttactcaaatacctatcattaattaagagaagagtttgagatgtataaggctaataaaggaagtgagagtgtggtgaattaagtgatgagtattatgtacaattgcctttacaaaaaacgtatttttactgtggaagaaattcatgcagagatgcctgtggaaaagtatcaataagaaaacaaaacacctttaacactatgacatactgattataatatactatgatatgtattattacagcattacttacacattctactttaggcaatgtaatctacttctgaatgaccttgttaatttttaaggcatcagtgcatcaagggcaaagctccataaaataaatataaaaacaagaaagcattagctaatttgtggcatagagaatgatcactgtatattatatctgttggccacttccatataggtaataaattgtacatcttattgtaaaaatgttatagcataaatttcacatcatttttcaacacttcatttaaagggctaaactgatctggcagtattctcattttcattgttccatcagctccacaggagaaaatgtgatttgcaggccctgtctcaatttgcatcactccagttccaatatttctaaaaatggactgccgagcatgttcactgacaaaagtatggagaagaccaaaggtagagagactccaaatctttatattgccttcggcagatcctgtaacaaagtactcttcagttggatcaacagcaacggctttaacaggagaatcatggctctggaaaagctgcctctgttgtcgttgacaaaggtcaaatacatatgtaaaaccttttctgccacctgatattagtagctgatgttttggagcatatgctaaaactgtggctccactgtcatggcaggtaaatgcatggactaaactattggcaggtgctacaagagtatcccacaaacatacgtttctattgtcagttgaaagaccagctgtagctatcagagaggaggaactaacgaagacaaaatcattggctgttttgttatgacactgccaagtcaggtatggcttaggcatgcttccagtaactggacaacatttccagtttgtttgatacaaacttaaatatccatcagcatcaactattccaaacttatttccctgatagttaaatctcattcttgtaactcttgaattgccaccagatcgaaaacaggttatttgttgagaatggccccattcaaacattctgacacttccatcttgagctcctgtcagatagtaaggaagagttggatgagaagtcattcttctaacattattaatggctttcttaatcatcacagatgctcctctgccagtctgtgtactaccaagccatggcatgttgattggagtgccaggattgctatgtgtatatggagttgtaccttgaacagctgttaaatcatcacgagcatgtataaccaagaaatcttctgatcctttggtttccacttctatatcatcatctacccaagtgtagacctgtgtggccagaattccagaaacatccagttcttgaacatcatgactggaagcgattgctatgcagtttctatttgccttattaacagcaaacgcagtaatgatatcagattccttatgaataattcttgctttacctccaggatatcccaaatctgcttctatctcatttagacaccgtttctttgtgaatatatttttgataaaggtttcctgaatttcttcctgcttcaccaaatactgccaaagcctcttcacagacagtgccagatggtgtttggatttgaaaggagtgtttgtaggttccagtaaagctttgtggcgaagaattgcaggacctgcagacaaactctcttcggcggtatgacttgcgatataattttgaggtggcccaccatggatttcaagtcgtcggagaagaacttgttcccaacattgaagagtttttagaaccgcatgacaaagaggtgaactaactggaagctctgcaagatcatgacctgcgaagggataaaaagtcttcaaattgttgagcaccaattgcaccatcgccaaccgcatcaaggaccaactatatgaatttgaattagaatgttcctggagatggaaatctgatgctaaaacatcatcatcatcatcattgtcatcatcatcacttcccagactctcctctgaatcatattcggctctactttgagaagagggtagaaaaggcttagctatgaaatagtcccagatactgagctcaggtgggatgaacttttctttaaccgccagtgactcctggcttactggtgccgaggaaggggtcagtggggcagattctctgcaagacatttttgacggcctaaaacgtttgttctgtttttctccttcttcaactagtgaagaaacaggtaaagtttttgaatgtgtctgttctttgctaggaacatgtgcacctccaccaaacacagcagaccacattttctcatttagaggatgggccacaatccgaaatagctcattacttgaatgtgtggccaggccatggatgaagagactaagatacactgctgtgagaatctcacagagcaagactgtaagccctgactgggcttcctcgccagaagaattcaaaagtcgaattagacaagttattcctggccattgagctggtgacgtattgggagttaatgcttcatctaagcttcctgttttcaaagaaggtcgatgaggaagcagtactgtctgatataccattccagtaaactgattcgtctgaaatgaactgtagttatgactaccacaaaggcactgataaatacaagcagaaagtgaagctgctaaagtatgcattacatacactttattgctttggatatcagggtggggtggtgaatcaaagtttattatggcatggagaatatcatgtgtcagattactaaggtgcaataatggattggcaactactgttttggcattggctgtacaagcaaagaggagaggcactgaggtttgctctgacagagggctagaaaatagtggttctgatgtttcctgctgagattcttgcaaaagcaaaatcaattccattcttacagatgcaagacccccaccatgggatccatgaagtatgcagtaactaagaaacattctcaaaagtgactgatacttcaagagccactgtcttttttcctgaaaattttctctcagttgtttcacttttgtttggtgaggcaaatcttcagcatcctcatttaatccaaattcatcttcatttctgccaaatgcagactgtagttcttcagcatctgagcaaaagtcacaagtcctctgaagagctatcacctctttttcaagccagtggtatagttggtaacgcaattttccaccatctatttcatagccagtagataaagtacgaagttctactgtgagaatctttaaacatgctctaaattttaactgaactgcaattatatcttctgatggatttaaaaggtcattttcatctagtgtgctgaaagattctgtgtagttagaacttatgtcatccaactttttatctgtttttctctgtaaaggttttagttctttcattgaaatagggacatcctcattttcttcatcattatcactgtcccattttaactctaaagagtcatcctgaaacacaacacttggttggctccagtcaaaagaaagagtggagtttgattgcttctctgaggaaccctctgaagaagatccaaaaccatttatcagtgactgtgaccaatcaacagcagaagacttatcttcccttgcatccaactttaatggagaagaaggagaacagtctttactagtatccagaaaactagaagccctataaaaaggtcttgttttcttgatgactttaggcatctttgataatacttccaaagccaacattgggcagccagcttttaaatgagcactggcagtggtaaaaaataaacgtctttcacttaaattaattgttcctgccagtccactttttcctgttaggctcatatgtgtggaaaatgtatcagatgatccaaaatgacgtctcagcaaaagaggatgtgttcttagataattgtagaaattaaaaactgtaggattactggctgataaaacttgatcatcattctctctgataggttgctttattaatgtttccagagcaccactataatcttccaaaatccaatatgccatgctccgaagaaaaggatcatgatgcatatttatgttcaatgaacacagttcactgacaggagaatcgattcccaaaacttttttacgtaaaatagatttatatgctgcagatgtatcaaattcagactcatagagtcttgctattacaagagccaactgaatgtcattcaatttctcaagacatacctcaattgcatctctgaggcaaccagctaaaagaaaaaatgctgcagaatgttcaaatctttgtttgcctagcaaagaaaaagcattctttaaagctgctttacgccacctctcatcctcaaaattgtgtccaaaaaactgtgtcatcctggtgtttttttcagctctatataatccccaaatcacagctttctttttcattgcaaggtaaaaaatggcagcatctaaaggatcattctttctataaaaggctgctttagctactttttctatgcatttgcgtaagatgcgggtattccggacccaccaccccacacccatagctcttagttcagaccaagtgggatcatctttctgcatggctggcaacatgttcagcagttcttcttctgctactgagtgaaatgcccaagcaaaatgacttgtagacaggccttggtgaaggagttgagctcgataggctggaagggaagttgtaagaaaggtatggagtcgaacagccaaaagaaattttaacccacattcatcaagagtttctccaccttggcttctgtctcggctttctccaatatcagtgcttgtagttgcaattgtatctgctaaggccatcaaagacatctgctccatccggctgagtcctggtaaactagaatgaagtaagtggccagaaagaacctgagcatgctcaggtccaaagtaagtcggactgtactgtgaaaggtcaataactctaggctttgtattttcttcatctgtctctaacatatgagtatcagtcattagaagttgagtctgaaaaagctcatcataactttctttagataattggtttgatttacttaacgtactctcattactagatttctccaaagatgagtaacagctatcatcatctgctgcaagtaaggcatataaaggaagtggaggaacagaatctatttctgtgtaatctgtattttcagccttgttgaatgcctgggggtctctggtagtgcttccactagcactgattgtgagagacctaaggcggcgttcatgattagattcagcttcattcagagccacaacttccccagcaatgcacttaacaagatgggacaagatggccttggctctccgaactttaccaagatccatgagttccaaaagctgcaagggatgatactgaggtagagtcggggaaagtacatgagctgcttcaaaaagacctgaatcttccatatccactgaaggatcgaatgcagttttctttccacagattttctgtgcaagactggtcatggatcgagtcagagttttctttggaggatgtaacccagaactggagttactctgttttattaaacttgttatagatggagtgctcccactgtacgaatctgttataacaggttcttgtttagaagatggttgccattggcaatacacatgcatttcacagtccattcctaccacaaggatgccatcccggacccacgataaagaaacaggaaaaggtggggagccatctacagaagaaactaggtccacacttcgtaatagtacaaatttagaaaggggcacaactttggtactctcccagagaggaaatgccagggtttccttaccagtttggtcttgtaccttgccagccaggggtccatacataaaaagttttgatccaattcctacagtcaggatatgagaaccgtcttctctagacatccaatctaagtgaactaaatgctttgtgtttgatgtgatattctctttactagataaatacatgtcttgtttattataggccactaaattgctatcaacactaatgccagaatccaatactgtgcttaactcatctaaatgaattgtctgctcaaggacccaacatgaacctcctgttgactcacattcaaaaatacttacatgcatcacaaagtcctgggaagatctactattagatgcaggctgcttataagctactgctaaacgatttgtatgtgcacagctaacttctacaggcctaccaggtacagttatactactattgctctgaagtccatcttcaataagtaatggccattcttcccaaatgtatgcaagatcaatttttccattctttgacgtggcagattctccatctgttactctgcatctccagaatcttactttctcatctgaacatgaagttgccaataaataaggagcactgcatgcaggatatatagaagatgaactcagatgtcctgctgatggcttaatacttattatctcaactccttctggtaaatgcaattcttggctataaaccatttctgaaaacagagtcaacctgctggtactctggagatttgctctgcaagcctgatacttttgtgaaaaaggagataggatcttctctggagaagaagaataatgttcttctggctgccaaaccgcttcggataattttgtatctactttttcatctaatgagacaggaattgactttagatgtaaattccacatgtgtaacagtgaacggttgtcttgagtgcattctattacaattaggtagaacttctcagaaaatccattaggtgagctgcctgcattagataaaatgctgtctttgccaaggcttttcttctcaaggttattcaaaatgaagtcttcttcaaaaacatgaagcagttgggtttttctgccatgaagtttggtaatgggatctaatgcaataatgcatcctggcctggctgttgattgttgactgacgatgttaaagacttcaccaacatatttagaaatttcagggttagaaagctcagataaaagtttcttagcatcaataactgcttcatataatctcagatattgtccatcactggctacaaagcatgcactaggagagttgcagtatgcacccagacaataactgggtataagagtgggcagccatgccacattggaaaaggcagaaacatgaagagaattaatccgggcaagctcagaaactcctccagaaaaagacaatggcccaactgggtcaaccctccacagaataagctcactgtaaactgcactgggatcctgaaatgccacgtcaacagtgcttttattttgttgtgtcaaagagcattcttcaatatttagagcatcaaaaggttgctctgggttatcaacatctggtgtccttaatgcattatggtgtgatgttgtcagcaataatggtaatactgagtggcaagctaaatcattaagatgaaaacgatgaccacaatatctggatttgtgggaaatactgagaacagtagaaaaagcagattcctcggcaaaactgaccagccactgattcagagaaccatcagcatgttttgatatcatcataacattaggcgtaaaaatacttaattttaaactattagatgatttattgtgaccagaagaaataagcattgatgtggaacgggtgaggccagaaggtttttgtttcccctgctgaatagccaagtcaacattcttggtacaggcatacatcattatgcttttacagagagagtttgcatcacctgtggggaaagctactggaattctggaaacaaaggacacctgtacttgacgaaacataccaggctggtattcatccagccaatccacatgccaaactagcaaagaaccatccatgggatgaatactaaatagcatatctgcatttttactccattcagacagaagtacttcaatctgatgatcaatggcagctgacgataatgatgtaaaacttgagtttggtaccattttatcacagcctaattccttcttttcgggatttattttcagatcatcaacaccatcatcagtttcttcatcagattttacatctgcctgattagaatcttctacactggcctcagaagatggttgttcaaaactttttctaagttgctgtaaaaaaacttccatggacaaagtaaaatgcagttctttattgtttagccagtgtacaacaaaaggtccggtcttctcttcattttcatttagactcagagatgtaatagatggaagaagtggaatgtctgtggctgggttgatgctggctgcaatatgaaagtggcaaagtgcattggcatgcagtggagtgttcctgtgaacatgatgaggatcctgctgatgtggtagatatcccgtatgtgctacaagagcaagtgatctcctccgacctctacgaaaatgtctcagatttacttctaaagcattttgaactcgttctttactggaagcatttctcttgaagttatttgttaaattaattgattcagtccaatggctgcagtcacctccgtatagcaaacaatcatttggtaaaaatgtctctacccaaagacgacacacattatctttgcagcaagtcaacagtacattacatacagaagccctaggcatatatttgcttgttttacgccaggaaaatccatttactgctcgaggatgggccagatacacaaaagaaaagtcaatttctccttgggattgtttttctgaacttccatctggagaagtaacagctgtccgccagttttctacattataccaaaccttcaaaagacagtcatccttcccagcagtggcaaaaaattctccatctggtgaaaatttcattaaatgaacttgggaagcagttttgcaatgccaaatgcatttccaatctccaaagttaagatctgttttatttaaattttcatcttcagttggcttctccaagttagtattggaccagagttgcaaatagctggaaccagttaaaagacgactgcctgtgggatcccaggttatattgtgtgctattgattccagaaaaaattggccacttttctgccactgactatataattccaaatttttcttttgttttggtaggttaactggttcaaaaatggagataacatttccataagacgctgcaatcttgccttgttgcattgaacagtctacacatcccacttgaatatttccatgtttagctcctgggattatctgtaatctttcaaaatcgcttcccagtattacaatgtcacatccagatgcataagccgtgaagcgctggtcgccaatgctgcccacggagaagcagtggtcgccagggttcacagccccggtcagcacctggtgcaggttcatgtcggcgccctagtcctgcaacggacaccgcatccagctcatgccacgggtcagcggctgcttccctccctccttccctcaggggcggcggccgctcttcggtggcgacggcagaagcagcgacaggcgcctggagccggagccgctcagctggggcccgcgactcatcccgagccccggagggcgaggcccggagggggcgggtcggcgagagggcggagcgccgcgctccttcgcgcacctgtcactccccgcgctagcccaggtgaagctcagggtcccctcaccggccacgacccggggccgactcaccggccaggaaggccgcgctgtccacacacttcctctggacctcgggcagccgctcctgacccagcccgagtggcgcaagcagtacgcgctcgcactccccgcctgacctgtcccttcccggctccggtgcccgccacccccacagtcctccgccactcactacgcgcctct

SEQ ID NO: 9960 - RNA, 9773 nt, Homo sapiens
  source 1..9773: mol_type = other RNA
cacacacacacacacacgtatacatacatacaacttgggttccggagggtaaactactgaaaaccttacatattgagccatctagctcatttatcactgacgtctcaatgacaattttaatgaagatgttcattatttttttcattcttactcaaatacctatcattaattaagagaagagtttgagatgtataaggctaataaaggaagtgagagtgtggtgaattaagtgatgagtattatgtacaattgcctttacaaaaaacgtatttttactgtggaagaaattcatgcagagatgcctgtggaaaagtatcaataagaaaacaaaacacctttaacactatgacatactgattataatatactatgatatgtattattacagcattacttacacattctactttaggcaatgtaatctacttctgaatgaccttgttaatttttaaggcatcagtgcatcaagggcaaagctccataaaataaatataaaaacaagaaagcattagctaatttgtggcatagagaatgatcactgtatattatatctgttggccacttccatataggtaataaattgtacatcttattgtaaaaatgttatagcataaatttcacatcatttttcaacacttcatttaaagggctaaactgatctggcagtattctcattttcattgttccatcagctccacaggagaaaatgtgatttgcaggccctgtctcaatttgcatcactccagttccaatatttctaaaaatggactgccgagcatgttcactgacaaaagtatggagaagaccaaaggtagagagactccaaatctttatattgccttcggcagatcctgtaacaaagtactcttcagttggatcaacagcaacggctttaacaggagaatcatggctctggaaaagctgcctctgttgtcgttgacaaaggtcaaatacatatgtaaaaccttttctgccacctgatattagtagctgatgttttggagcatatgctaaaactgtggctccactgtcatggcaggtaaatgcatggactaaactattggcaggtgctacaagagtatcccacaaacatacgtttctattgtcagttgaaagaccagctgtagctatcagagaggaggaactaacgaagacaaaatcattggctgttttgttatgacactgccaagtcaggtatggcttaggcatgcttccagtaactggacaacatttccagtttgtttgatacaaacttaaatatccatcagcatcaactattccaaacttatttccctgatagttaaatctcattcttgtaactcttgaattgccaccagatcgaaaacaggttatttgttgagaatggccccattcaaacattctgacacttccatcttgagctcctgtcagatagtaaggaagagttggatgagaagtcattcttctaacattattaatggctttcttaatcatcacagatgctcctctgccagtctgtgtactaccaagccatggcatgttgattggagtgccaggattgctatgtgtatatggagttgtaccttgaacagctgttaaatcatcacgagcatgtataaccaagaaatcttctgatcctttggtttccacttctatatcatcatctacccaagtgtagacctgtgtggccagaattccagaaacatccagttcttgaacatcatgactggaagcgattgctatgcagtttctatttgccttattaacagcaaacgcagtaatgatatcagattccttatgaataattcttgctttacctccaggatatcccaaatctgcttctatctcatttagacaccgtttctttgtgaatatatttttgataaaggtttcctgaatttcttcctgcttcaccaaatactgccaaagcctcttcacagacagtgccagatggtgtttggatttgaaaggagtgtttgtaggttccagtaaagctttgtggcgaagaattgcaggacctgcagacaaactctcttcggcggtatgacttgcgatataattttgaggtggcccaccatggatttcaagtcgtcggagaagaacttgttcccaacattgaagagtttttagaaccgcatgacaaagaggtgaactaactggaagctctgcaagatcatgacctgcgaagggataaaaagtcttcaaattgttgagcaccaattgcaccatcgccaaccgcatcaaggaccaactatatgaatttgaattagaatgttcctggagatggaaatctgatgctaaaacatcatcatcatcatcattgtcatcatcatcacttcccagactctcctctgaatcatattcggctctactttgagaagagggtagaaaaggcttagctatgaaatagtcccagatactgagctcaggtgggatgaacttttctttaaccgccagtgactcctggcttactggtgccgaggaaggggtcagtggggcagattctctgcaagacatttttgacggcctaaaacgtttgttctgtttttctccttcttcaactagtgaagaaacaggtaaagtttttgaatgtgtctgttctttgctaggaacatgtgcacctccaccaaacacagcagaccacattttctcatttagaggatgggccacaatccgaaatagctcattacttgaatgtgtggccaggccatggatgaagagactaagatacactgctgtgagaatctcacagagcaagactgtaagccctgactgggcttcctcgccagaagaattcaaaagtcgaattagacaagttattcctggccattgagctggtgacgtattgggagttaatgcttcatctaagcttcctgttttcaaagaaggtcgatgaggaagcagtactgtctgatataccattccagtaaactgattcgtctgaaatgaactgtagttatgactaccacaaaggcactgataaatacaagcagaaagtgaagctgctaaagtatgcattacatacactttattgctttggatatcagggtggggtggtgaatcaaagtttattatggcatggagaatatcatgtgtcagattactaaggtgcaataatggattggcaactactgttttggcattggctgtacaagcaaagaggagaggcactgaggtttgctctgacagagggctagaaaatagtggttctgatgtttcctgctgagattcttgcaaaagcaaaatcaattccattcttacagatgcaagacccccaccatgggatccatgaagtatgcagtaactaagaaacattctcaaaagtgactgatacttcaagagccactgtcttttttcctgaaaattttctctcagttgtttcacttttgtttggtgaggcaaatcttcagcatcctcatttaatccaaattcatcttcatttctgccaaatgcagactgtagttcttcagcatctgagcaaaagtcacaagtcctctgaagagctatcacctctttttcaagccagtggtatagttggtaacgcaattttccaccatctatttcatagccagtagataaagtacgaagttctactgtgagaatctttaaacatgctctaaattttaactgaactgcaattatatcttctgatggatttaaaaggtcattttcatctagtgtgctgaaagattctgtgtagttagaacttatgtcatccaactttttatctgtttttctctgtaaaggttttagttctttcattgaaatagggacatcctcattttcttcatcattatcactgtcccattttaactctaaagagtcatcctgaaacacaacacttggttggctccagtcaaaagaaagagtggagtttgattgcttctctgaggaaccctctgaagaagatccaaaaccatttatcagtgactgtgaccaatcaacagcagaagacttatcttcccttgcatccaactttaatggagaagaaggagaacagtctttactagtatccagaaaactagaagccctataaaaaggtcttgttttcttgatgactttaggcatctttgataatacttccaaagccaacattgggcagccagcttttaaatgagcactggcagtggtaaaaaataaacgtctttcacttaaattaattgttcctgccagtccactttttcctgttaggctcatatgtgtggaaaatgtatcagatgatccaaaatgacgtctcagcaaaagaggatgtgttcttagataattgtagaaattaaaaactgtaggattactggctgataaaacttgatcatcattctctctgataggttgctttattaatgtttccagagcaccactataatcttccaaaatccaatatgccatgctccgaagaaaaggatcatgatgcatatttatgttcaatgaacacagttcactgacaggagaatcgattcccaaaacttttttacgtaaaatagatttatatgctgcagatgtatcaaattcagactcatagagtcttgctattacaagagccaactgaatgtcattcaatttctcaagacatacctcaattgcatctctgaggcaaccagctaaaagaaaaaatgctgcagaatgttcaaatctttgtttgcctagcaaagaaaaagcattctttaaagctgctttacgccacctctcatcctcaaaattgtgtccaaaaaactgtgtcatcctggtgtttttttcagctctatataatccccaaatcacagctttctttttcattgcaaggtaaaaaatggcagcatctaaaggatcattctttctataaaaggctgctttagctactttttctatgcatttgcgtaagatgcgggtattccggacccaccaccccacacccatagctcttagttcagaccaagtgggatcatctttctgcatggctggcaacatgttcagcagttcttcttctgctactgagtgaaatgcccaagcaaaatgacttgtagacaggccttggtgaaggagttgagctcgataggctggaagggaagttgtaagaaaggtatggagtcgaacagccaaaagaaattttaacccacattcatcaagagtttctccaccttggcttctgtctcggctttctccaatatcagtgcttgtagttgcaattgtatctgctaaggccatcaaagacatctgctccatccggctgagtcctggtaaactagaatgaagtaagtggccagaaagaacctgagcatgctcaggtccaaagtaagtcggactgtactgtgaaaggtcaataactctaggctttgtattttcttcatctgtctctaacatatgagtatcagtcattagaagttgagtctgaaaaagctcatcataactttctttagataattggtttgatttacttaacgtactctcattactagatttctccaaagatgagtaacagctatcatcatctgctgcaagtaaggcatataaaggaagtggaggaacagaatctatttctgtgtaatctgtattttcagccttgttgaatgcctgggggtctctggtagtgcttccactagcactgattgtgagagacctaaggcggcgttcatgattagattcagcttcattcagagccacaacttccccagcaatgcacttaacaagatgggacaagatggccttggctctccgaactttaccaagatccatgagttccaaaagctgcaagggatgatactgaggtagagtcggggaaagtacatgagctgcttcaaaaagacctgaatcttccatatccactgaaggatcgaatgcagttttctttccacagattttctgtgcaagactggtcatggatcgagtcagagttttctttggaggatgtaacccagaactggagttactctgttttattaaacttgttatagatggagtgctcccactgtacgaatctgttataacaggttcttgtttagaagatggttgccattggcaatacacatgcatttcacagtccattcctaccacaaggatgccatcccggacccacgataaagaaacaggaaaaggtggggagccatctacagaagaaactaggtccacacttcgtaatagtacaaatttagaaaggggcacaactttggtactctcccagagaggaaatgccagggtttccttaccagtttggtcttgtaccttgccagccaggggtccatacataaaaagttttgatccaattcctacagtcaggatatgagaaccgtcttctctagacatccaatctaagtgaactaaatgctttgtgtttgatgtgatattctctttactagataaatacatgtcttgtttattataggccactaaattgctatcaacactaatgccagaatccaatactgtgcttaactcatctaaatgaattgtctgctcaaggacccaacatgaacctcctgttgactcacattcaaaaatacttacatgcatcacaaagtcctgggaagatctactattagatgcaggctgcttataagctactgctaaacgatttgtatgtgcacagctaacttctacaggcctaccaggtacagttatactactattgctctgaagtccatcttcaataagtaatggccattcttcccaaatgtatgcaagatcaatttttccattctttgacgtggcagattctccatctgttactctgcatctccagaatcttactttctcatctgaacatgaagttgccaataaataaggagcactgcatgcaggatatatagaagatgaactcagatgtcctgctgatggcttaatacttattatctcaactccttctggtaaatgcaattcttggctataaaccatttctgaaaacagagtcaacctgctggtactctggagatttgctctgcaagcctgatacttttgtgaaaaaggagataggatcttctctggagaagaagaataatgttcttctggctgccaaaccgcttcggataattttgtatctactttttcatctaatgagacaggaattgactttagatgtaaattccacatgtgtaacagtgaacggttgtcttgagtgcattctattacaattaggtagaacttctcagaaaatccattaggtgagctgcctgcattagataaaatgctgtctttgccaaggcttttcttctcaaggttattcaaaatgaagtcttcttcaaaaacatgaagcagttgggtttttctgccatgaagtttggtaatgggatctaatgcaataatgcatcctggcctggctgttgattgttgactgacgatgttaaagacttcaccaacatatttagaaatttcagggttagaaagctcagataaaagtttcttagcatcaataactgcttcatataatctcagatattgtccatcactggctacaaagcatgcactaggagagttgcagtatgcacccagacaataactgggtataagagtgggcagccatgccacattggaaaaggcagaaacatgaagagaattaatccgggcaagctcagaaactcctccagaaaaagacaatggcccaactgggtcaaccctccacagaataagctcactgtaaactgcactgggatcctgaaatgccacgtcaacagtgcttttattttgttgtgtcaaagagcattcttcaatatttagagcatcaaaaggttgctctgggttatcaacatctggtgtccttaatgcattatggtgtgatgttgtcagcaataatggtaatactgagtggcaagctaaatcattaagatgaaaacgatgaccacaatatctggatttgtgggaaatactgagaacagtagaaaaagcagattcctcggcaaaactgaccagccactgattcagagaaccatcagcatgttttgatatcatcataacattaggcgtaaaaatacttaattttaaactattagatgatttattgtgaccagaagaaataagcattgatgtggaacgggtgaggccagaaggtttttgtttcccctgctgaatagccaagtcaacattcttggtacaggcatacatcattatgcttttacagagagagtttgcatcacctgtggggaaagctactggaattctggaaacaaaggacacctgtacttgacgaaacataccaggctggtattcatccagccaatccacatgccaaactagcaaagaaccatccatgggatgaatactaaatagcatatctgcatttttactccattcagacagaagtacttcaatctgatgatcaatggcagctgacgataatgatgtaaaacttgagtttggtaccattttatcacagcctaattccttcttttcgggatttattttcagatcatcaacaccatcatcagtttcttcatcagattttacatctgcctgattagaatcttctacactggcctcagaagatggttgttcaaaactttttctaagttgctgtaaaaaaacttccatggacaaagtaaaatgcagttctttattgtttagccagtgtacaacaaaaggtccggtcttctcttcattttcatttagactcagagatgtaatagatggaagaagtggaatgtctgtggctgggttgatgctggctgcaatatgaaagtggcaaagtgcattggcatgcagtggagtgttcctgtgaacatgatgaggatcctgctgatgtggtagatatcccgtatgtgctacaagagcaagtgatctcctccgacctctacgaaaatgtctcagatttacttctaaagcattttgaactcgttctttactggaagcatttctcttgaagttatttgttaaattaattgattcagtccaatggctgcagtcacctccgtatagcaaacaatcatttggtaaaaatgtctctacccaaagacgacacacattatctttgcagcaagtcaacagtacattacatacagaagccctaggcatatatttgcttgttttacgccaggaaaatccatttactgctcgaggatgggccagatacacaaaagaaaagtcaatttctccttgggattgtttttctgaacttccatctggagaagtaacagctgtccgccagttttctacattataccaaaccttcaaaagacagtcatccttcccagcagtggcaaaaaattctccatctggtgaaaatttcattaaatgaacttgggaagcagttttgcaatgccaaatgcatttccaatctccaaagttaagatctgttttatttaaattttcatcttcagttggcttctccaagttagtattggaccagagttgcaaatagctggaaccagttaaaagacgactgcctgtgggatcccaggttatattgtgtgctattgattccagaaaaaattggccacttttctgccactgactatataattccaaatttttcttttgttttggtaggttaactggttcaaaaatggagataacatttccataagacgctgcaatcttgccttgttgcattgaacagtctacacatcccacttgaatatttccatgtttagctcctgggattatctgtaatctttcaaaatcgcttcccagtattacaatgtcacatccagatgcataagccgtgaagcgctggtcgccaatgctgcccacggagaagcagtggtcgccagggttcacagccccggtcagcacctggtgcaggttcatgtcggcgccctagtctacgcgcctctggatccctgcggccgaaatatcgcgagacttcgctcggggcagctgctactgtggtaaag

SEQ ID NO: 9961 - RNA, 11478 nt, Homo sapiens
  source 1..11478: mol_type = other RNA
cacacacacacacacacgtatacatacatacaacttgggttccggagggtaaactactgaaaaccttacatattgagccatctagctcatttatcactgacgtctcaatgacaattttaatgaagatgttcattatttttttcattcttactcaaatacctatcattaattaagagaagagtttgagatgtataaggctaataaaggaagtgagagtgtggtgaattaagtgatgagtattatgtacaattgcctttacaaaaaacgtatttttactgtggaagaaattcatgcagagatgcctgtggaaaagtatcaataagaaaacaaaacacctttaacactatgacatactgattataatatactatgatatgtattattacagcattacttacacattctactttaggcaatgtaatctacttctgaatgaccttgttaatttttaaggcatcagtgcatcaagggcaaagctccataaaataaatataaaaacaagaaagcattagctaatttgtggcatagagaatgatcactgtatattatatctgttggccacttccatataggtaataaattgtacatcttattgtaaaaatgttatagcataaatttcacatcatttttcaacacttcatttaaagggctaaactgatctggcagtattctcattttcattgttccatcagctccacaggagaaaatgtgatttgcaggccctgtctcaatttgcatcactccagttccaatatttctaaaaatggactgccgagcatgttcactgacaaaagtatggagaagaccaaaggtagagagactccaaatctttatattgccttcggcagatcctgtaacaaagtactcttcagttggatcaacagcaacggctttaacaggagaatcatggctctggaaaagctgcctctgttgtcgttgacaaaggtcaaatacatatgtaaaaccttttctgccacctgatattagtagctgatgttttggagcatatgctaaaactgtggctccactgtcatggcaggtaaatgcatggactaaactattggcaggtgctacaagagtatcccacaaacatacgtttctattgtcagttgaaagaccagctgtagctatcagagaggaggaactaacgaagacaaaatcattggctgttttgttatgacactgccaagtcaggtatggcttaggcatgcttccagtaactggacaacatttccagtttgtttgatacaaacttaaatatccatcagcatcaactattccaaacttatttccctgatagttaaatctcattcttgtaactcttgaattgccaccagatcgaaaacaggttatttgttgagaatggccccattcaaacattctgacacttccatcttgagctcctgtcagatagtaaggaagagttggatgagaagtcattcttctaacattattaatggctttcttaatcatcacagatgctcctctgccagtctgtgtactaccaagccatggcatgttgattggagtgccaggattgctatgtgtatatggagttgtaccttgaacagctgttaaatcatcacgagcatgtataaccaagaaatcttctgatcctttggtttccacttctatatcatcatctacccaagtgtagacctgtgtggccagaattccagaaacatccagttcttgaacatcatgactggaagcgattgctatgcagtttctatttgccttattaacagcaaacgcagtaatgatatcagattccttatgaataattcttgctttacctccaggatatcccaaatctgcttctatctcatttagacaccgtttctttgtgaatatatttttgataaaggtttcctgaatttcttcctgcttcaccaaatactgccaaagcctcttcacagacagtgccagatggtgtttggatttgaaaggagtgtttgtaggttccagtaaagctttgtggcgaagaattgcaggacctgcagacaaactctcttcggcggtatgacttgcgatataattttgaggtggcccaccatggatttcaagtcgtcggagaagaacttgttcccaacattgaagagtttttagaaccgcatgacaaagaggtgaactaactggaagctctgcaagatcatgacctgcgaagggataaaaagtcttcaaattgttgagcaccaattgcaccatcgccaaccgcatcaaggaccaactatatgaatttgaattagaatgttcctggagatggaaatctgatgctaaaacatcatcatcatcatcattgtcatcatcatcacttcccagactctcctctgaatcatattcggctctactttgagaagagggtagaaaaggcttagctatgaaatagtcccagatactgagctcaggtgggatgaacttttctttaaccgccagtgactcctggcttactggtgccgaggaaggggtcagtggggcagattctctgcaagacatttttgacggcctaaaacgtttgttctgtttttctccttcttcaactagtgaagaaacaggtaaagtttttgaatgtgtctgttctttgctaggaacatgtgcacctccaccaaacacagcagaccacattttctcatttagaggatgggccacaatccgaaatagctcattacttgaatgtgtggccaggccatggatgaagagactaagatacactgctgtgagaatctcacagagcaagactgtaagccctgactgggcttcctcgccagaagaattcaaaagtcgaattagacaagttattcctggccattgagctggtgacgtattgggagttaatgcttcatctaagcttcctgttttcaaagaaggtcgatgaggaagcagtactgtctgatataccattccagtaaactgattcgtctgaaatgaactgtagttatgactaccacaaaggcactgataaatacaagcagaaagtgaagctgctaaagtatgcattacatacactttattgctttggatatcagggtggggtggtgaatcaaagtttattatggcatggagaatatcatgtgtcagattactaaggtgcaataatggattggcaactactgttttggcattggctgtacaagcaaagaggagaggcactgaggtttgctctgacagagggctagaaaatagtggttctgatgtttcctgctgagattcttgcaaaagcaaaatcaattccattcttacagatgcaagacccccaccatgggatccatgaagtatgcagtaactaagaaacattctcaaaagtgactgatacttcaagagccactgtcttttttcctgaaaattttctctcagttgtttcacttttgtttggtgaggcaaatcttcagcatcctcatttaatccaaattcatcttcatttctgccaaatgcagactgtagttcttcagcatctgagcaaaagtcacaagtcctctgaagagctatcacctctttttcaagccagtggtatagttggtaacgcaattttccaccatctatttcatagccagtagataaagtacgaagttctactgtgagaatctttaaacatgctctaaattttaactgaactgcaattatatcttctgatggatttaaaaggtcattttcatctagtgtgctgaaagattctgtgtagttagaacttatgtcatccaactttttatctgtttttctctgtaaaggttttagttctttcattgaaatagggacatcctcattttcttcatcattatcactgtcccattttaactctaaagagtcatcctgaaacacaacacttggttggctccagtcaaaagaaagagtggagtttgattgcttctctgaggaaccctctgaagaagatccaaaaccatttatcagtgactgtgaccaatcaacagcagaagacttatcttcccttgcatccaactttaatggagaagaaggagaacagtctttactagtatccagaaaactagaagccctataaaaaggtcttgttttcttgatgactttaggcatctttgataatacttccaaagccaacattgggcagccagcttttaaatgagcactggcagtggtaaaaaataaacgtctttcacttaaattaattgttcctgccagtccactttttcctgttaggctcatatgtgtggaaaatgtatcagatgatccaaaatgacgtctcagcaaaagaggatgtgttcttagataattgtagaaattaaaaactgtaggattactggctgataaaacttgatcatcattctctctgataggttgctttattaatgtttccagagcaccactataatcttccaaaatccaatatgccatgctccgaagaaaaggatcatgatgcatatttatgttcaatgaacacagttcactgacaggagaatcgattcccaaaacttttttacgtaaaatagatttatatgctgcagatgtatcaaattcagactcatagagtcttgctattacaagagccaactgaatgtcattcaatttctcaagacatacctcaattgcatctctgaggcaaccagctaaaagaaaaaatgctgcagaatgttcaaatctttgtttgcctagcaaagaaaaagcattctttaaagctgctttacgccacctctcatcctcaaaattgtgtccaaaaaactgtgtcatcctggtgtttttttcagctctatataatccccaaatcacagctttctttttcattgcaaggtaaaaaatggcagcatctaaaggatcattctttctataaaaggctgctttagctactttttctatgcatttgcgtaagatgcgggtattccggacccaccaccccacacccatagctcttagttcagaccaagtgggatcatctttctgcatggctggcaacatgttcagcagttcttcttctgctactgagtgaaatgcccaagcaaaatgacttgtagacaggccttggtgaaggagttgagctcgataggctggaagggaagttgtaagaaaggtatggagtcgaacagccaaaagaaattttaacccacattcatcaagagtttctccaccttggcttctgtctcggctttctccaatatcagtgcttgtagttgcaattgtatctgctaaggccatcaaagacatctgctccatccggctgagtcctggtaaactagaatgaagtaagtggccagaaagaacctgagcatgctcaggtccaaagtaagtcggactgtactgtgaaaggtcaataactctaggctttgtattttcttcatctgtctctaacatatgagtatcagtcattagaagttgagtctgaaaaagctcatcataactttctttagataattggtttgatttacttaacgtactctcattactagatttctccaaagatgagtaacagctatcatcatctgctgcaagtaaggcatataaaggaagtggaggaacagaatctatttctgtgtaatctgtattttcagccttgttgaatgcctgggggtctctggtagtgcttccactagcactgattgtgagagacctaaggcggcgttcatgattagattcagcttcattcagagccacaacttccccagcaatgcacttaacaagatgggacaagatggccttggctctccgaactttaccaagatccatgagttccaaaagctgcaagggatgatactgaggtagagtcggggaaagtacatgagctgcttcaaaaagacctgaatcttccatatccactgaaggatcgaatgcagttttctttccacagattttctgtgcaagactggtcatggatcgagtcagagttttctttggaggatgtaacccagaactggagttactctgttttattaaacttgttatagatggagtgctcccactgtacgaatctgttataacaggttcttgtttagaagatggttgccattggcaatacacatgcatttcacagtccattcctaccacaaggatgccatcccggacccacgataaagaaacaggaaaaggtggggagccatctacagaagaaactaggtccacacttcgtaatagtacaaatttagaaaggggcacaactttggtactctcccagagaggaaatgccagggtttccttaccagtttggtcttgtaccttgccagccaggggtccatacataaaaagttttgatccaattcctacagtcaggatatgagaaccgtcttctctagacatccaatctaagtgaactaaatgctttgtgtttgatgtgatattctctttactagataaatacatgtcttgtttattataggccactaaattgctatcaacactaatgccagaatccaatactgtgcttaactcatctaaatgaattgtctgctcaaggacccaacatgaacctcctgttgactcacattcaaaaatacttacatgcatcacaaagtcctgggaagatctactattagatgcaggctgcttataagctactgctaaacgatttgtatgtgcacagctaacttctacaggcctaccaggtacagttatactactattgctctgaagtccatcttcaataagtaatggccattcttcccaaatgtatgcaagatcaatttttccattctttgacgtggcagattctccatctgttactctgcatctccagaatcttactttctcatctgaacatgaagttgccaataaataaggagcactgcatgcaggatatatagaagatgaactcagatgtcctgctgatggcttaatacttattatctcaactccttctggtaaatgcaattcttggctataaaccatttctgaaaacagagtcaacctgctggtactctggagatttgctctgcaagcctgatacttttgtgaaaaaggagataggatcttctctggagaagaagaataatgttcttctggctgccaaaccgcttcggataattttgtatctactttttcatctaatgagacaggaattgactttagatgtaaattccacatgtgtaacagtgaacggttgtcttgagtgcattctattacaattaggtagaacttctcagaaaatccattaggtgagctgcctgcattagataaaatgctgtctttgccaaggcttttcttctcaaggttattcaaaatgaagtcttcttcaaaaacatgaagcagttgggtttttctgccatgaagtttggtaatgggatctaatgcaataatgcatcctggcctggctgttgattgttgactgacgatgttaaagacttcaccaacatatttagaaatttcagggttagaaagctcagataaaagtttcttagcatcaataactgcttcatataatctcagatattgtccatcactggctacaaagcatgcactaggagagttgcagtatgcacccagacaataactgggtataagagtgggcagccatgccacattggaaaaggcagaaacatgaagagaattaatccgggcaagctcagaaactcctccagaaaaagacaatggcccaactgggtcaaccctccacagaataagctcactgtaaactgcactgggatcctgaaatgccacgtcaacagtgcttttattttgttgtgtcaaagagcattcttcaatatttagagcatcaaaaggttgctctgggttatcaacatctggtgtccttaatgcattatggtgtgatgttgtcagcaataatggtaatactgagtggcaagctaaatcattaagatgaaaacgatgaccacaatatctggatttgtgggaaatactgagaacagtagaaaaagcagattcctcggcaaaactgaccagccactgattcagagaaccatcagcatgttttgatatcatcataacattaggcgtaaaaatacttaattttaaactattagatgatttattgtgaccagaagaaataagcattgatgtggaacgggtgaggccagaaggtttttgtttcccctgctgaatagccaagtcaacattcttggtacaggcatacatcattatgcttttacagagagagtttgcatcacctgtggggaaagctactggaattctggaaacaaaggacacctgtacttgacgaaacataccaggctggtattcatccagccaatccacatgccaaactagcaaagaaccatccatgggatgaatactaaatagcatatctgcatttttactccattcagacagaagtacttcaatctgatgatcaatggcagctgacgataatgatgtaaaacttgagtttggtaccattttatcacagcctaattccttcttttcgggatttattttcagatcatcaacaccatcatcagtttcttcatcagattttacatctgcctgattagaatcttctacactggcctcagaagatggttgttcaaaactttttctaagttgctgtaaaaaaacttccatggacaaagtaaaatgcagttctttattgtttagccagtgtacaacaaaaggtccggtcttctcttcattttcatttagactcagagatgtaatagatggaagaagtggaatgtctgtggctgggttgatgctggctgcaatatgaaagtggcaaagtgcattggcatgcagtggagtgttcctgtgaacatgatgaggatcctgctgatgtggtagatatcccgtatgtgctacaagagcaagtgatctcctccgacctctacgaaaatgtctcagatttacttctaaagcattttgaactcgttctttactggaagcatttctcttgaagttatttgttaaattaattgattcagtccaatggctgcagtcacctccgtatagcaaacaatcatttggtaaaaatgtctctacccaaagacgacacacattatctttgcagcaagtcaacagtacattacatacagaagccctaggcatatatttgcttgttttacgccaggaaaatccatttactgctcgaggatgggccagatacacaaaagaaaagtcaatttctccttgggattgtttttctgaacttccatctggagaagtaacagctgtccgccagttttctacattataccaaaccttcaaaagacagtcatccttcccagcagtggcaaaaaattctccatctggtgaaaatttcattaaatgaacttgggaagcagttttgcaatgccaaatgcatttccaatctccaaagttaagatctgttttatttaaattttcatcttcagttggcttctccaagttagtattggaccagagttgcaaatagctggaaccagttaaaagacgactgtgggatcccaggttatattgtgtgctattgattccagaaaaaattggccacttttctgccactgactatataattccaaatttttcttttgttttggtaggttaactggttcaaaaatggagataacatttccataagacgctgcaatcaacatgatgaaaccccgtttctactaaaaatacaaaaattagccgggtatgatggcgagcacctgtaattccagctatttgggaggctgaggcaggagaattgcttgaacccggaagccagaggctgcagtgagctgagattgcaccactgcactccagcctgggcaacaaagcgagactccatctgaaaaacaaaaaacaaaacaaacaaacaaaaacaaacaaaaaacaaaaaaaaaacccaaagatttccagcattccataataaagatcatttttgttgtacagcgagaagtcataagaggcctcaacaaaagatagaggacacctgtaactatattaaagggaaggaataccatgtaacaaaaagaacagtagtccaacaaatatgtaaagattcagaaaacagaaactcgttttataattaatatctttaagtcccagatggcaacttttaatcctagaaagtttacctcaaatgaagattagatttaaaaacaaatgattgggtccatggactcttaatatgaccattttgattccttacacaaaatgttctagtggaatcatatgagtgtatttgcgaagttcagtccagtctagctacaactatatataggccttaccacctatgcctatatggagttattttaagctatatattatgctgccttgcctagtagtatgactttctcattctggtactacaggaactgtatttaacctgatctagaagaattttatactttgttacttttgtttatgttgttgctattttactttcaaggttacctttctacttttcatatgcaaatagaagtccagataaagtttttcacttttcttatgggcttagaatattataaactctcaaagagtttttcatttccacaaaaagttacacagcccttgttacatagaagttacaaggagataactacctgttcacagacaaaaaaaaaaaaatattctaaatcatttcctttagtttatttgtaaatattgaagattcattgttactcctttcccccagtccaatcaccttttaaatacgtaagctttagactcattctatatcagtaagtattgtatttctttctcagagaagatgatgctataatttaaaattatataagaagagaatttctggcactctatagaatgcatcttagacagccaaaaattcttctagctacactatctttgaaacaaagccaagtctctaattcaataggaaatacacacttcagagattatcctgacaaaaaccatattccaaacaaatttgtatattagaagaagattacaaaccttgccttgttgcattgaacagtctacacatcccacttgaatatttccatgtttagctcctgggattatctgtaatctttcaaaatcgcttcccagtattacaatgtcacatccagatgcataagccgtgaagcgctggtcgccaatgctgcccacggagaagcagtggtcgccagggttcacagccccggtcagcacctggtgcaggttcatgtcggcgccctagtcctgcaacggacaccgcatccagctcatgccacgggtcagcggctgcttccctccctccttccctcaggggcggcggccgctcttcggtggcgacggcagaagcagcgacaggcgcctggagccggagccgctcagctggggcccgcgactcatcccgagccccggagggcgaggcccggagggggcgggtcggcgagagggcggagcgccgcgctccttcgcgcacctgtcactccccgcgctagcccaggtgaagctcagggtcccctcaccggccacgacccggggccgactcaccggccaggaaggccgcgctgtccacacacttcctctggacctcgggcagccgctcctgacccagcccgagtggcgcaagcagtacgcgctcgcactccccgcctgacctgtcccttcccggctccggtgcccgccacccccacagtcctccgccactcactacgcgcctct

SEQ ID NO: 9962 - RNA, 10327 nt, Homo sapiens
  source 1..10327: mol_type = other RNA
cacacacacacacacacgtatacatacatacaacttgggttccggagggtaaactactgaaaaccttacatattgagccatctagctcatttatcactgacgtctcaatgacaattttaatgaagatgttcattatttttttcattcttactcaaatacctatcattaattaagagaagagtttgagatgtataaggctaataaaggaagtgagagtgtggtgaattaagtgatgagtattatgtacaattgcctttacaaaaaacgtatttttactgtggaagaaattcatgcagagatgcctgtggaaaagtatcaataagaaaacaaaacacctttaacactatgacatactgattataatatactatgatatgtattattacagcattacttacacattctactttaggcaatgtaatctacttctgaatgaccttgttaatttttaaggcatcagtgcatcaagggcaaagctccataaaataaatataaaaacaagaaagcattagctaatttgtggcatagagaatgatcactgtatattatatctgttggccacttccatataggtaataaattgtacatcttattgtaaaaatgttatagcataaatttcacatcatttttcaacacttcatttaaagggctaaactgatctggcagtattctcattttcattgttccatcagctccacaggagaaaatgtgatttgcaggccctgtctcaatttgcatcactccagttccaatatttctaaaaatggactgccgagcatgttcactgacaaaagtatggagaagaccaaaggtagagagactccaaatctttatattgccttcggcagatcctgtaacaaagtactcttcagttggatcaacagcaacggctttaacaggagaatcatggctctggaaaagctgcctctgttgtcgttgacaaaggtcaaatacatatgtaaaaccttttctgccacctgatattagtagctgatgttttggagcatatgctaaaactgtggctccactgtcatggcaggtaaatgcatggactaaactattggcaggtgctacaagagtatcccacaaacatacgtttctattgtcagttgaaagaccagctgtagctatcagagaggaggaactaacgaagacaaaatcattggctgttttgttatgacactgccaagtcaggtatggcttaggcatgcttccagtaactggacaacatttccagtttgtttgatacaaacttaaatatccatcagcatcaactattccaaacttatttccctgatagttaaatctcattcttgtaactcttgaattgccaccagatcgaaaacaggttatttgttgagaatggccccattcaaacattctgacacttccatcttgagctcctgtcagatagtaaggaagagttggatgagaagtcattcttctaacattattaatggctttcttaatcatcacagatgctcctctgccagtctgtgtactaccaagccatggcatgttgattggagtgccaggattgctatgtgtatatggagttgtaccttgaacagctgttaaatcatcacgagcatgtataaccaagaaatcttctgatcctttggtttccacttctatatcatcatctacccaagtgtagacctgtgtggccagaattccagaaacatccagttcttgaacatcatgactggaagcgattgctatgcagtttctatttgccttattaacagcaaacgcagtaatgatatcagattccttatgaataattcttgctttacctccaggatatcccaaatctgcttctatctcatttagacaccgtttctttgtgaatatatttttgataaaggtttcctgaatttcttcctgcttcaccaaatactgccaaagcctcttcacagacagtgccagatggtgtttggatttgaaaggagtgtttgtaggttccagtaaagctttgtggcgaagaattgcaggacctgcagacaaactctcttcggcggtatgacttgcgatataattttgaggtggcccaccatggatttcaagtcgtcggagaagaacttgttcccaacattgaagagtttttagaaccgcatgacaaagaggtgaactaactggaagctctgcaagatcatgacctgcgaagggataaaaagtcttcaaattgttgagcaccaattgcaccatcgccaaccgcatcaaggaccaactatatgaatttgaattagaatgttcctggagatggaaatctgatgctaaaacatcatcatcatcatcattgtcatcatcatcacttcccagactctcctctgaatcatattcggctctactttgagaagagggtagaaaaggcttagctatgaaatagtcccagatactgagctcaggtgggatgaacttttctttaaccgccagtgactcctggcttactggtgccgaggaaggggtcagtggggcagattctctgcaagacatttttgacggcctaaaacgtttgttctgtttttctccttcttcaactagtgaagaaactgcaagactgggagggctatgagaactgatggctgaaagagctttggaaaagcccacacattccatggagaataccactacctggtgggggctaggcatagcaaagtgccttccaggtaaagtttttgaatgtgtctgttctttgctaggaacatgtgcacctccaccaaacacagcagaccacattttctcatttagaggatgggccacaatccgaaatagctcattacttgaatgtgtggccaggccatggatgaagagactaagatacactgctgtgagaatctcacagagcaagactgtaagccctgactgggcttcctcgccagaagaattcaaaagtcgaattagacaagttattcctggccattgagctggtgacgtattgggagttaatgcttcatctaagcttcctgttttcaaagaaggtcgatgaggaagcagtactgtctgatataccattccagtaaactgattcgtctgaaatgaactgtagttatgactaccacaaaggcactgataaatacaagcagaaagtgaagctgctaaagtatgcattacatacactttattgctttggatatcagggtggggtggtgaatcaaagtttattatggcatggagaatatcatgtgtcagattactaaggtgcaataatggattggcaactactgttttggcattggctgtacaagcaaagaggagaggcactgaggtttgctctgacagagggctagaaaatagtggttctgatgtttcctgctgagattcttgcaaaagcaaaatcaattccattcttacagatgcaagacccccaccatgggatccatgaagtatgcagtaactaagaaacattctcaaaagtgactgatacttcaagagccactgtcttttttcctgaaaattttctctcagttgtttcacttttgtttggtgaggcaaatcttcagcatcctcatttaatccaaattcatcttcatttctgccaaatgcagactgtagttcttcagcatctgagcaaaagtcacaagtcctctgaagagctatcacctctttttcaagccagtggtatagttggtaacgcaattttccaccatctatttcatagccagtagataaagtacgaagttctactgtgagaatctttaaacatgctctaaattttaactgaactgcaattatatcttctgatggatttaaaaggtcattttcatctagtgtgctgaaagattctgtgtagttagaacttatgtcatccaactttttatctgtttttctctgtaaaggttttagttctttcattgaaatagggacatcctcattttcttcatcattatcactgtcccattttaactctaaagagtcatcctgaaacacaacacttggttggctccagtcaaaagaaagagtggagtttgattgcttctctgaggaaccctctgaagaagatccaaaaccatttatcagtgactgtgaccaatcaacagcagaagacttatcttcccttgcatccaactttaatggagaagaaggagaacagtctttactagtatccagaaaactagaagccctataaaaaggtcttgttttcttgatgactttaggcatctttgataatacttccaaagccaacattgggcagccagcttttaaatgagcactggcagtggtaaaaaataaacgtctttcacttaaattaattgttcctgccagtccactttttcctgttaggctcatatgtgtggaaaatgtatcagatgatccaaaatgacgtctcagcaaaagaggatgtgttcttagataattgtagaaattaaaaactgtaggattactggctgataaaacttgatcatcattctctctgataggttgctttattaatgtttccagagcaccactataatcttccaaaatccaatatgccatgctccgaagaaaaggatcatgatgcatatttatgttcaatgaacacagttcactgacaggagaatcgattcccaaaacttttttacgtaaaatagatttatatgctgcagatgtatcaaattcagactcatagagtcttgctattacaagagccaactgaatgtcattcaatttctcaagacatacctcaattgcatctctgaggcaaccagctaaaagaaaaaatgctgcagaatgttcaaatctttgtttgcctagcaaagaaaaagcattctttaaagctgctttacgccacctctcatcctcaaaattgtgtccaaaaaactgtgtcatcctggtgtttttttcagctctatataatccccaaatcacagctttctttttcattgcaaggtaaaaaatggcagcatctaaaggatcattctttctataaaaggctgctttagctactttttctatgcatttgcgtaagatgcgggtattccggacccaccaccccacacccatagctcttagttcagaccaagtgggatcatctttctgcatggctggcaacatgttcagcagttcttcttctgctactgagtgaaatgcccaagcaaaatgacttgtagacaggccttggtgaaggagttgagctcgataggctggaagggaagttgtaagaaaggtatggagtcgaacagccaaaagaaattttaacccacattcatcaagagtttctccaccttggcttctgtctcggctttctccaatatcagtgcttgtagttgcaattgtatctgctaaggccatcaaagacatctgctccatccggctgagtcctggtaaactagaatgaagtaagtggccagaaagaacctgagcatgctcaggtccaaagtaagtcggactgtactgtgaaaggtcaataactctaggctttgtattttcttcatctgtctctaacatatgagtatcagtcattagaagttgagtctgaaaaagctcatcataactttctttagataattggtttgatttacttaacgtactctcattactagatttctccaaagatgagtaacagctatcatcatctgctgcaagtaaggcatataaaggaagtggaggaacagaatctatttctgtgtaatctgtattttcagccttgttgaatgcctgggggtctctggtagtgcttccactagcactgattgtgagagacctaaggcggcgttcatgattagattcagcttcattcagagccacaacttccccagcaatgcacttaacaagatgggacaagatggccttggctctccgaactttaccaagatccatgagttccaaaagctgcaagggatgatactgaggtagagtcggggaaagtacatgagctgcttcaaaaagacctgaatcttccatatccactgaaggatcgaatgcagttttctttccacagattttctgtgcaagactggtcatggatcgagtcagagttttctttggaggatgtaacccagaactggagttactctgttttattaaacttgttatagatggagtgctcccactgtacgaatctgttataacaggttcttgtttagaagatggttgccattggcaatacacatgcatttcacagtccattcctaccacaaggatgccatcccggacccacgataaagaaacaggaaaaggtggggagccatctacagaagaaactaggtccacacttcgtaatagtacaaatttagaaaggggcacaactttggtactctcccagagaggaaatgccagggtttccttaccagtttggtcttgtaccttgccagccaggggtccatacataaaaagttttgatccaattcctacagtcaggatatgagaaccgtcttctctagacatccaatctaagtgaactaaatgctttgtgtttgatgtgatattctctttactagataaatacatgtcttgtttattataggccactaaattgctatcaacactaatgccagaatccaatactgtgcttaactcatctaaatgaattgtctgctcaaggacccaacatgaacctcctgttgactcacattcaaaaatacttacatgcatcacaaagtcctgggaagatctactattagatgcaggctgcttataagctactgctaaacgatttgtatgtgcacagctaacttctacaggcctaccaggtacagttatactactattgctctgaagtccatcttcaataagtaatggccattcttcccaaatgtatgcaagatcaatttttccattctttgacgtggcagattctccatctgttactctgcatctccagaatcttactttctcatctgaacatgaagttgccaataaataaggagcactgcatgcaggatatatagaagatgaactcagatgtcctgctgatggcttaatacttattatctcaactccttctggtaaatgcaattcttggctataaaccatttctgaaaacagagtcaacctgctggtactctggagatttgctctgcaagcctgatacttttgtgaaaaaggagataggatcttctctggagaagaagaataatgttcttctggctgccaaaccgcttcggataattttgtatctactttttcatctaatgagacaggaattgactttagatgtaaattccacatgtgtaacagtgaacggttgtcttgagtgcattctattacaattaggtagaacttctcagaaaatccattaggtgagctgcctgcattagataaaatgctgtctttgccaaggcttttcttctcaaggttattcaaaatgaagtcttcttcaaaaacatgaagcagttgggtttttctgccatgaagtttggtaatgggatctaatgcaataatgcatcctggcctggctgttgattgttgactgacgatgttaaagacttcaccaacatatttagaaatttcagggttagaaagctcagataaaagtttcttagcatcaataactgcttcatataatctcagatattgtccatcactggctacaaagcatgcactaggagagttgcagtatgcacccagacaataactgggtataagagtgggcagccatgccacattggaaaaggcagaaacatgaagagaattaatccgggcaagctcagaaactcctccagaaaaagacaatggcccaactgggtcaaccctccacagaataagctcactgtaaactgcactgggatcctgaaatgccacgtcaacagtgcttttattttgttgtgtcaaagagcattcttcaatatttagagcatcaaaaggttgctctgggttatcaacatctggtgtccttaatgcattatggtgtgatgttgtcagcaataatggtaatactgagtggcaagctaaatcattaagatgaaaacgatgaccacaatatctggatttgtgggaaatactgagaacagtagaaaaagcagattcctcggcaaaactgaccagccactgattcagagaaccatcagcatgttttgatatcatcataacattaggcgtaaaaatacttaattttaaactattagatgatttattgtgaccagaagaaataagcattgatgtggaacgggtgaggccagaaggtttttgtttcccctgctgaatagccaagtcaacattcttggtacaggcatacatcattatgcttttacagagagagtttgcatcacctgtggggaaagctactggaattctggaaacaaaggacacctgtacttgacgaaacataccaggctggtattcatccagccaatccacatgccaaactagcaaagaaccatccatgggatgaatactaaatagcatatctgcatttttactccattcagacagaagtacttcaatctgatgatcaatggcagctgacgataatgatgtaaaacttgagtttggtaccattttatcacagcctaattccttcttttcgggatttattttcagatcatcaacaccatcatcagtttcttcatcagattttacatctgcctgattagaatcttctacactggcctcagaagatggttgttcaaaactttttctaagttgctgtaaaaaaacttccatggacaaagtaaaatgcagttctttattgtttagccagtgtacaacaaaaggtccggtcttctcttcattttcatttagactcagagatgtaatagatggaagaagtggaatgtctgtggctgggttgatgctggctgcaatatgaaagtggcaaagtgcattggcatgcagtggagtgttcctgtgaacatgatgaggatcctgctgatgtggtagatatcccgtatgtgctacaagagcaagtgatctcctccgacctctacgaaaatgtctcagatttacttctaaagcattttgaactcgttctttactggaagcatttctcttgaagttatttgttaaattaattgattcagtccaatggctgcagtcacctccgtatagcaaacaatcatttggtaaaaatgtctctacccaaagacgacacacattatctttgcagcaagtcaacagtacattacatacagaagccctaggcatatatttgcttgttttacgccaggaaaatccatttactgctcgaggatgggccagatacacaaaagaaaagtcaatttctccttgggattgtttttctgaacttccatctggagaagtaacagctgtccgccagttttctacattataccaaaccttcaaaagacagtcatccttcccagcagtggcaaaaaattctccatctggtgaaaatttcattaaatgaacttgggaagcagttttgcaatgccaaatgcatttccaatctccaaagttaagatctgttttatttaaattttcatcttcagttggcttctccaagttagtattggaccagagttgcaaatagctggaaccagttaaaagacgactgcctgtgggatcccaggttatattgtgtgctattgattccagaaaaaattggccacttttctgccactgactatataattccaaatttttcttttgttttggtaggttaactggttcaaaaatggagataacatttccataagacgctgcaatcttgccttgttgcattgaacagtctacacatcccacttgaatatttccatgtttagctcctgggattatctgtaatctttcaaaatcgcttcccagtattacaatgtcacatccagatgcataagccgtgaagcgctggtcgccaatgctgcccacggagaagcagtggtcgccagggttcacagccccggtcagcacctggtgcaggttcatgtcggcgccctagtcctgcaacggacaccgcatccagctcatgccacgggtcagcggctgcttccctccctccttccctcaggggcggcggccgctcttcggtggcgacggcagaagcagcgacaggcgcctggagccggagccgctcagctggggcccgcgactcatcccgagccccggagggcgaggcccggagggggcgggtcggcgagagggcggagcgccgcgctccttcgcgcacctgtcactccccgcgctagcccaggtgaagctcagggtcccctcaccggccacgacccggggccgactcaccggccaggaaggccgcgctgtccacacacttcctctggacctcgggcagccgctcctgacccagcccgagtggcgcaagcagtacgcgctcgcactccccgcctgacctgtcccttcccggctccggtgcccgccacccccacagtcctccgccactcactacgcgcctctggatccctgcggccgaaatatcgcgagacttcgctcggggcag

SEQ ID NO: 9963 - RNA, 9246 nt, Homo sapiens
  source 1..9246: mol_type = other RNA
cacacacacacacacacgtatacatacatacaacttgggttccggagggtaaactactgaaaaccttacatattgagccatctagctcatttatcactgacgtctcaatgacaattttaatgaagatgttcattatttttttcattcttactcaaatacctatcattaattaagagaagagtttgagatgtataaggctaataaaggaagtgagagtgtggtgaattaagtgatgagtattatgtacaattgcctttacaaaaaacgtatttttactgtggaagaaattcatgcagagatgcctgtggaaaagtatcaataagaaaacaaaacacctttaacactatgacatactgattataatatactatgatatgtattattacagcattacttacacattctactttaggcaatgtaatctacttctgaatgaccttgttaatttttaaggcatcagtgcatcaagggcaaagctccataaaataaatataaaaacaagaaagcattagctaatttgtggcatagagaatgatcactgtatattatatctgttggccacttccatataggtaataaattgtacatcttattgtaaaaatgttatagcataaatttcacatcatttttcaacacttcatttaaagggctaaactgatctggcagtattctcattttcattgttccatcagctccacaggagaaaatgtgatttgcaggccctgtctcaatttgcatcactccagttccaatatttctaaaaatggactgccgagcatgttcactgacaaaagtatggagaagaccaaaggtagagagactccaaatctttatattgccttcggcagatcctgtaacaaagtactcttcagttggatcaacagcaacggctttaacaggagaatcatggctctggaaaagctgcctctgttgtcgttgacaaaggtcaaatacatatgtaaaaccttttctgccacctgatattagtagctgatgttttggagcatatgctaaaactgtggctccactgtcatggcaggtaaatgcatggactaaactattggcaggtgctacaagagtatcccacaaacatacgtttctattgtcagttgaaagaccagctgtagctatcagagaggaggaactaacgaagacaaaatcattggctgttttgttatgacactgccaagtcaggtatggcttaggcatgcttccagtaactggacaacatttccagtttgtttgatacaaacttaaatatccatcagcatcaactattccaaacttatttccctgatagttaaatctcattcttgtaactcttgaattgccaccagatcgaaaacaggttatttgttgagaatggccccattcaaacattctgacacttccatcttgagctcctgtcagatagtaaggaagagttggatgagaagtcattcttctaacattattaatggctttcttaatcatcacagatgctcctctgccagtctgtgtactaccaagccatggcatgttgattggagtgccaggattgctatgtgtatatggagttgtaccttgaacagctgttaaatcatcacgagcatgtataaccaagaaatcttctgatcctttggtttccacttctatatcatcatctacccaagtgtagacctgtgtggccagaattccagaaacatccagttcttgaacatcatgactggaagcgattgctatgcagtttctatttgccttattaacagcaaacgcagtaatgatatcagattccttatgaataattcttgctttacctccaggatatcccaaatctgcttctatcttattgatgtttggctcctccatcatagaatttttgatggtttcactgttgtcctctaatgactcatttagacaccgtttctttgtgaatatatttttgataaaggtttcctgaatttcttcctgcttcaccaaatactgccaaagcctcttcacagacagtgccagatggtgtttggatttgaaaggagtgtttgtaggttccagtaaagctttgtggcgaagaattgcaggacctgcagacaaactctcttcggcggtatgacttgcgatataattttgaggtggcccaccatggatttcaagtcgtcggagaagaacttgttcccaacattgaagagtttttagaaccgcatgacaaagaggtgaactaactggaagctctgcaagatcatgacctgcgaagggataaaaagtcttcaaattgttgagcaccaattgcaccatcgccaaccgcatcaaggaccaactatatgaatttgaattagaatgttcctggagatggaaatctgatgctaaaacatcatcatcatcatcattgtcatcatcatcacttcccagactctcctctgaatcatattcggctctactttgagaagagggtagaaaaggcttagctatgaaatagtcccagatactgagctcaggtgggatgaacttttctttaaccgccagtgactcctggcttactggtgccgaggaaggggtcagtggggcagattctctgcaagacatttttgacggcctaaaacgtttgttctgtttttctccttcttcaactagtgaagaaacaggtaaagtttttgaatgtgtctgttctttgctaggaacatgtgcacctccaccaaacacagcagaccacattttctcatttagaggatgggccacaatccgaaatagctcattacttgaatgtgtggccaggccatggatgaagagactaagatacactgctgtgagaatctcacagagcaagactgtaagccctgactgggcttcctcgccagaagaattcaaaagtcgaattagacaagttattcctggccattgagctggtgacgtattgggagttaatgcttcatctaagcttcctgttttcaaagaaggtcgatgaggaagcagtactgtctgatataccattccagtaaactgattcgtctgaaatgaactgtagttatgactaccacaaaggcactgataaatacaagcagaaagtgaagctgctaaagtatgcattacatacactttattgctttggatatcagggtggggtggtgaatcaaagtttattatggcatggagaatatcatgtgtcagattactaaggtgcaataatggattggcaactactgttttggcattggctgtacaagcaaagaggagaggcactgaggtttgctctgacagagggctagaaaatagtggttctgatgtttcctgctgagattcttgcaaaagcaaaatcaattccattcttacagatgcaagacccccaccatgggatccatgaagtatgcagtaactaagaaacattctcaaaagtgactgatacttcaagagccactgtcttttttcctgaaaattttctctcagttgtttcacttttgtttggtgaggcaaatcttcagcatcctcatttaatccaaattcatcttcatttctgccaaatgcagactgtagttcttcagcatctgagcaaaagtcacaagtcctctgaagagctatcacctctttttcaagccagtggtatagttggtaacgcaattttccaccatctatttcatagccagtagataaagtacgaagttctactgtgagaatctttaaacatgctctaaattttaactgaactgcaattatatcttctgatggatttaaaaggtcattttcatctagtgtgctgaaagattctgtgtagttagaacttatgtcatccaactttttatctgtttttctctgtaaaggttttagttctttcattgaaatagggacatcctcattttcttcatcattatcactgtcccattttaactctaaagagtcatcctgaaacacaacacttggttggctccagtcaaaagaaagagtggagtttgattgcttctctgaggaaccctctgaagaagatccaaaaccatttatcagtgactgtgaccaatcaacagcagaagacttatcttcccttgcatccaactttaatggagaagaaggagaacagtctttactagtatccagaaaactagaagccctataaaaaggtcttgttttcttgatgactttaggcatctttgataatacttccaaagccaacattgggcagccagcttttaaatgagcactggcagtggtaaaaaataaacgtctttcacttaaattaattgttcctgccagtccactttttcctgttaggctcatatgtgtggaaaatgtatcagatgatccaaaatgacgtctcagcaaaagaggatgtgttcttagataattgtagaaattaaaaactgtaggattactggctgataaaacttgatcatcattctctctgataggttgctttattaatgtttccagagcaccactataatcttccaaaatccaatatgccatgctccgaagaaaaggatcatgatgcatatttatgttcaatgaacacagttcactgacaggagaatcgattcccaaaacttttttacgtaaaatagatttatatgctgcagatgtatcaaattcagactcatagagtcttgctattacaagagccaactgaatgtcattcaatttctcaagacatacctcaattgcatctctgaggcaaccagctaaaagaaaaaatgctgcagaatgttcaaatctttgtttgcctagcaaagaaaaagcattctttaaagctgctttacgccacctctcatcctcaaaattgtgtccaaaaaactgtgtcatcctggtgtttttttcagctctatataatccccaaatcacagctttctttttcattgcaaggtaaaaaatggcagcatctaaaggatcattctttctataaaaggctgctttagctactttttctatgcatttgcgtaagatgcgggtattccggacccaccaccccacacccatagctcttagttcagaccaagtgggatcatctttctgcatggctggcaacatgttcagcagttcttcttctgctactgagtgaaatgcccaagcaaaatgacttgtagacaggccttggtgaaggagttgagctcgataggctggaagggaagttgtaagaaaggtatggagtcgaacagccaaaagaaattttaacccacattcatcaagagtttctccaccttggcttctgtctcggctttctccaatatcagtgcttgtagttgcaattgtatctgctaaggccatcaaagacatctgctccatccggctgagtcctggtaaactagaatgaagtaagtggccagaaagaacctgagcatgctcaggtccaaagtaagtcggactgtactgtgaaaggtcaataactctaggctttgtattttcttcatctgtctctaacatatgagtatcagtcattagaagttgagtctgaaaaagctcatcataactttctttagataattggtttgatttacttaacgtactctcattactagatttctccaaagatgagtaacagctatcatcatctgctgcaagtaaggcatataaaggaagtggaggaacagaatctatttctgtgtaatctgtattttcagccttgttgaatgcctgggggtctctggtagtgcttccactagcactgattgtgagagacctaaggcggcgttcatgattagattcagcttcattcagagccacaacttccccagcaatgcacttaacaagatgggacaagatggccttggctctccgaactttaccaagatccatgagttccaaaagctgcaagggatgatactgaggtagagtcggggaaagtacatgagctgcttcaaaaagacctgaatcttccatatccactgaaggatcgaatgcagttttctttccacagattttctgtgcaagactggtcatggatcgagtcagagttttctttggaggatgtaacccagaactggagttactctgttttattaaacttgttatagatggagtgctcccactgtacgaatctgttataacaggttcttgtttagaagatggttgccattggcaatacacatgcatttcacagtccattcctaccacaaggatgccatcccggacccacgataaagaaacaggaaaaggtggggagccatctacagaagaaactaggtccacacttcgtaatagtacaaatttagaaaggggcacaactttggtactctcccagagaggaaatgccagggtttccttaccagtttggtcttgtaccttgccagccaggggtccatacataaaaagttttgatccaattcctacagtcaggatatgagaaccgtcttctctagacatccaatctaagtgaactaaatgctttgtgtttgatgtgatattctctttactagataaatacatgtcttgtttattataggccactaaattgctatcaacactaatgccagaatccaatactgtgcttaactcatctaaatgaattgtctgctcaaggacccaacatgaacctcctgttgactcacattcaaaaatacttacatgcatcacaaagtcctgggaagatctactattagatgcaggctgcttataagctactgctaaacgatttgtatgtgcacagctaacttctacaggcctaccaggtacagttatactactattgctctgaagtccatcttcaataagtaatggccattcttcccaaatgtatgcaagatcaatttttccattctttgacgtggcagattctccatctgttactctgcatctccagaatcttactttctcatctgaacatgaagttgccaataaataaggagcactgcatgcaggatatatagaagatgaactcagatgtcctgcattagataaaatgctgtctttgccaaggcttttcttctcaaggttattcaaaatgaagtcttcttcaaaaacatgaagcagttgggtttttctgccatgaagtttggtaatgggatctaatgcaataatgcatcctggcctggctgttgattgttgactgacgatgttaaagacttcaccaacatatttagaaatttcagggttagaaagctcagataaaagtttcttagcatcaataactgcttcatataatctcagatattgtccatcactggctacaaagcatgcactaggagagttgcagtatgcacctgtggggaaagctactggaattctggaaacaaaggacacctgtacttgacgaaacataccaggctggtattcatccagccaatccacatgccaaactagcaaagaaccatccatgggatgaatactaaatagcatatctgcatttttactccattcagacagaagtacttcaatctgatgatcaatggcagctgacgataatgatgtaaaacttgagtttggtaccattttatcacagcctaattccttcttttcgggatttattttcagatcatcaacaccatcatcagtttcttcatcagattttacatctgcctgattagaatcttctacactggcctcagaagatggttgttcaaaactttttctaagttgctgtaaaaaaacttccatggacaaagtaaaatgcagttctttattgtttagccagtgtacaacaaaaggtccggtcttctcttcattttcatttagactcagagatgtaatagatggaagaagtggaatgtctgtggctgggttgatgctggctgcaatatgaaagtggcaaagtgcattggcatgcagtggagtgttcctgtgaacatgatgaggatcctgctgatgtggtagatatcccgtatgtgctacaagagcaagtgatctcctccgacctctacgaaaatgtctcagatttacttctaaagcattttgaactcgttctttactggaagcatttctcttgaagttatttgttaaattaattgattcagtccaatggctgcagtcacctccgtatagcaaacaatcatttggtaaaaatgtctctacccaaagacgacacacattatctttgcagcaagtcaacagtacattacatacagaagccctaggcatatatttgcttgttttacgccaggaaaatccatttactgctcgaggatgggccagatacacaaaagaaaagtcaatttctccttgggattgtttttctgaacttccatctggagaagtaacagctgtccgccagttttctacattataccaaaccttcaaaagacagtcatccttcccagcagtggcaaaaaattctccatctggtgaaaatttcattaaatgaacttgggaagcagttttgcaatgccaaatgcatttccaatctccaaagttaagatctgttttatttaaattttcatcttcagttggcttctccaagttagtattggaccagagttgcaaatagctggaaccagttaaaagacgactgcctgtgggatcccaggttatattgtgtgctattgattccagaaaaaattggccacttttctgccactgactatataattccaaatttttcttttgttttggtaggttaactggttcaaaaatggagataacatttccataagacgctgcaatcttgccttgttgcattgaacagtctacacatcccacttgaatatttccatgtttagctcctgggattatctgtaatctttcaaaatcgcttcccagtattacaatgtcacatccagatgcataagccgtgaagcgctggtcgccaatgctgcccacggagaagcagtggtcgccagggttcacagccccggtcagcacctggtgcaggttcatgtcggcgccctagtcctgcaacggacaccgcatccagctcatgccacgggtcagcggctgcttccctccctccttccctcaggggcggcggccgctcttcggtggcgacggcagaagcagcgacaggcgcctggagccggagccgctcagctggggcccgcgactcatcccgagccccggagggcgaggcccggagggggcgggtcggcgagagggcggagcgccgcgctccttcgcgcacctgtcactccccgcgctagcccaggtgaagctcagggtcccctcaccggccacgacccggggccgactcaccggccaggaaggccgcgctgtccacacacttcctctggacctcgggcagccgctcctgacccagcccgagtggcgcaagcagtacgcgctcgcactccccgcctgacctgtcccttcccggctccggtgcccgccacccccacagtcctccgccactcactacgcgcctct

SEQ ID NO: 9964 - RNA, 9936 nt, Homo sapiens
  source 1..9936: mol_type = other RNA
cacacacacacacacacgtatacatacatacaacttgggttccggagggtaaactactgaaaaccttacatattgagccatctagctcatttatcactgacgtctcaatgacaattttaatgaagatgttcattatttttttcattcttactcaaatacctatcattaattaagagaagagtttgagatgtataaggctaataaaggaagtgagagtgtggtgaattaagtgatgagtattatgtacaattgcctttacaaaaaacgtatttttactgtggaagaaattcatgcagagatgcctgtggaaaagtatcaataagaaaacaaaacacctttaacactatgacatactgattataatatactatgatatgtattattacagcattacttacacattctactttaggcaatgtaatctacttctgaatgaccttgttaatttttaaggcatcagtgcatcaagggcaaagctccataaaataaatataaaaacaagaaagcattagctaatttgtggcatagagaatgatcactgtatattatatctgttggccacttccatataggtaataaattgtacatcttattgtaaaaatgttatagcataaatttcacatcatttttcaacacttcatttaaagggctaaactgatctggcagtattctcattttcattgttccatcagctccacaggagaaaatgtgatttgcaggccctgtctcaatttgcatcactccagttccaatatttctaaaaatggactgccgagcatgttcactgacaaaagtatggagaagaccaaaggtagagagactccaaatctttatattgccttcggcagatcctgtaacaaagtactcttcagttggatcaacagcaacggctttaacaggagaatcatggctctggaaaagctgcctctgttgtcgttgacaaaggtcaaatacatatgtaaaaccttttctgccacctgatattagtagctgatgttttggagcatatgctaaaactgtggctccactgtcatggcaggtaaatgcatggactaaactattggcaggtgctacaagagtatcccacaaacatacgtttctattgtcagttgaaagaccagctgtagctatcagagaggaggaactaacgaagacaaaatcattggctgttttgttatgacactgccaagtcaggtatggcttaggcatgcttccagtaactggacaacatttccagtttgtttgatacaaacttaaatatccatcagcatcaactattccaaacttatttccctgatagttaaatctcattcttgtaactcttgaattgccaccagatcgaaaacaggttatttgttgagaatggccccattcaaacattctgacacttccatcttgagctcctgtcagatagtaaggaagagttggatgagaagtcattcttctaacattattaatggctttcttaatcatcacagatgctcctctgccagtctgtgtactaccaagccatggcatgttgattggagtgccaggattgctatgtgtatatggagttgtaccttgaacagctgttaaatcatcacgagcatgtataaccaagaaatcttctgatcctttggtttccacttctatatcatcatctacccaagtgtagacctgtgtggccagaattccagaaacatccagttcttgaacatcatgactggaagcgattgctatgcagtttctatttgccttattaacagcaaacgcagtaatgatatcagattccttatgaataattcttgctttacctccaggatatcccaaatctgcttctatcttattgatgtttggctcctccatcatagaatttttgatggtttcactgttgtcctctaatgactcatttagacaccgtttctttgtgaatatatttttgataaaggtttcctgaatttcttcctgcttcaccaaatactgccaaagcctcttcacagacagtgccagatggtgtttggatttgaaaggagtgtttgtaggttccagtaaagctttgtggcgaagaattgcaggacctgcagacaaactctcttcggcggtatgacttgcgatataattttgaggtggcccaccatggatttcaagtcgtcggagaagaacttgttcccaacattgaagagtttttagaaccgcatgacaaagaggtgaactaactggaagctctgcaagatcatgacctgcgaagggataaaaagtcttcaaattgttgagcaccaattgcaccatcgccaaccgcatcaaggaccaactatatgaatttgaattagaatgttcctggagatggaaatctgatgctaaaacatcatcatcatcatcattgtcatcatcatcacttcccagactctcctctgaatcatattcggctctactttgagaagagggtagaaaaggcttagctatgaaatagtcccagatactgagctcaggtgggatgaacttttctttaaccgccagtgactcctggcttactggtgccgaggaaggggtcagtggggcagattctctgcaagacatttttgacggcctaaaacgtttgttctgtttttctccttcttcaactagtgaagaaacaggtaaagtttttgaatgtgtctgttctttgctaggaacatgtgcacctccaccaaacacagcagaccacattttctcatttagaggatgggccacaatccgaaatagctcattacttgaatgtgtggccaggccatggatgaagagactaagatacactgctgtgagaatctcacagagcaagactgtaagccctgactgggcttcctcgccagaagaattcaaaagtcgaattagacaagttattcctggccattgagctggtgacgtattgggagttaatgcttcatctaagcttcctgttttcaaagaaggtcgatgaggaagcagtactgtctgatataccattccagtaaactgattcgtctgaaatgaactgtagttatgactaccacaaaggcactgataaatacaagcagaaagtgaagctgctaaagtatgcattacatacactttattgctttggatatcagggtggggtggtgaatcaaagtttattatggcatggagaatatcatgtgtcagattactaaggtgcaataatggattggcaactactgttttggcattggctgtacaagcaaagaggagaggcactgaggtttgctctgacagagggctagaaaatagtggttctgatgtttcctgctgagattcttgcaaaagcaaaatcaattccattcttacagatgcaagacccccaccatgggatccatgaagtatgcagtaactaagaaacattctcaaaagtgactgatacttcaagagccactgtcttttttcctgaaaattttctctcagttgtttcacttttgtttggtgaggcaaatcttcagcatcctcatttaatccaaattcatcttcatttctgccaaatgcagactgtagttcttcagcatctgagcaaaagtcacaagtcctctgaagagctatcacctctttttcaagccagtggtatagttggtaacgcaattttccaccatctatttcatagccagtagataaagtacgaagttctactgtgagaatctttaaacatgctctaaattttaactgaactgcaattatatcttctgatggatttaaaaggtcattttcatctagtgtgctgaaagattctgtgtagttagaacttatgtcatccaactttttatctgtttttctctgtaaaggttttagttctttcattgaaatagggacatcctcattttcttcatcattatcactgtcccattttaactctaaagagtcatcctgaaacacaacacttggttggctccagtcaaaagaaagagtggagtttgattgcttctctgaggaaccctctgaagaagatccaaaaccatttatcagtgactgtgaccaatcaacagcagaagacttatcttcccttgcatccaactttaatggagaagaaggagaacagtctttactagtatccagaaaactagaagccctataaaaaggtcttgttttcttgatgactttaggcatctttgataatacttccaaagccaacattgggcagccagcttttaaatgagcactggcagtggtaaaaaataaacgtctttcacttaaattaattgttcctgccagtccactttttcctgttaggctcatatgtgtggaaaatgtatcagatgatccaaaatgacgtctcagcaaaagaggatgtgttcttagataattgtagaaattaaaaactgtaggattactggctgataaaacttgatcatcattctctctgataggttgctttattaatgtttccagagcaccactataatcttccaaaatccaatatgccatgctccgaagaaaaggatcatgatgcatatttatgttcaatgaacacagttcactgacaggagaatcgattcccaaaacttttttacgtaaaatagatttatatgctgcagatgtatcaaattcagactcatagagtcttgctattacaagagccaactgaatgtcattcaatttctcaagacatacctcaattgcatctctgaggcaaccagctaaaagaaaaaatgctgcagaatgttcaaatctttgtttgcctagcaaagaaaaagcattctttaaagctgctttacgccacctctcatcctcaaaattgtgtccaaaaaactgtgtcatcctggtgtttttttcagctctatataatccccaaatcacagctttctttttcattgcaaggtaaaaaatggcagcatctaaaggatcattctttctataaaaggctgctttagctactttttctatgcatttgcgtaagatgcgggtattccggacccaccaccccacacccatagctcttagttcagaccaagtgggatcatctttctgcatggctggcaacatgttcagcagttcttcttctgctactgagtgaaatgcccaagcaaaatgacttgtagacaggccttggtgaaggagttgagctcgataggctggaagggaagttgtaagaaaggtatggagtcgaacagccaaaagaaattttaacccacattcatcaagagtttctccaccttggcttctgtctcggctttctccaatatcagtgcttgtagttgcaattgtatctgctaaggccatcaaagacatctgctccatccggctgagtcctggtaaactagaatgaagtaagtggccagaaagaacctgagcatgctcaggtccaaagtaagtcggactgtactgtgaaaggtcaataactctaggctttgtattttcttcatctgtctctaacatatgagtatcagtcattagaagttgagtctgaaaaagctcatcataactttctttagataattggtttgatttacttaacgtactctcattactagatttctccaaagatgagtaacagctatcatcatctgctgcaagtaaggcatataaaggaagtggaggaacagaatctatttctgtgtaatctgtattttcagccttgttgaatgcctgggggtctctggtagtgcttccactagcactgattgtgagagacctaaggcggcgttcatgattagattcagcttcattcagagccacaacttccccagcaatgcacttaacaagatgggacaagatggccttggctctccgaactttaccaagatccatgagttccaaaagctgcaagggatgatactgaggtagagtcggggaaagtacatgagctgcttcaaaaagacctgaatcttccatatccactgaaggatcgaatgcagttttctttccacagattttctgtgcaagactggtcatggatcgagtcagagttttctttggaggatgtaacccagaactggagttactctgttttattaaacttgttatagatggagtgctcccactgtacgaatctgttataacaggttcttgtttagaagatggttgccattggcaatacacatgcatttcacagtccattcctaccacaaggatgccatcccggacccacgataaagaaacaggaaaaggtggggagccatctacagaagaaactaggtccacacttcgtaatagtacaaatttagaaaggggcacaactttggtactctcccagagaggaaatgccagggtttccttaccagtttggtcttgtaccttgccagccaggggtccatacataaaaagttttgatccaattcctacagtcaggatatgagaaccgtcttctctagacatccaatctaagtgaactaaatgctttgtgtttgatgtgatattctctttactagataaatacatgtcttgtttattataggccactaaattgctatcaacactaatgccagaatccaatactgtgcttaactcatctaaatgaattgtctgctcaaggacccaacatgaacctcctgttgactcacattcaaaaatacttacatgcatcacaaagtcctgggaagatctactattagatgcaggctgcttataagctactgctaaacgatttgtatgtgcacagctaacttctacaggcctaccaggtacagttatactactattgctctgaagtccatcttcaataagtaatggccattcttcccaaatgtatgcaagatcaatttttccattctttgacgtggcagattctccatctgttactctgcatctccagaatcttactttctcatctgaacatgaagttgccaataaataaggagcactgcatgcaggatatatagaagatgaactcagatgtcctgctgatggcttaatacttattatctcaactccttctggtaaatgcaattcttggctataaaccatttctgaaaacagagtcaacctgctggtactctggagatttgctctgcaagcctgatacttttgtgaaaaaggagataggatcttctctggagaagaagaataatgttcttctggctgccaaaccgcttcggataattttgtatctactttttcatctaatgagacaggaattgactttagatgtaaattccacatgtgtaacagtgaacggttgtcttgagtgcattctattacaattaggtagaacttctcagaaaatccattaggtgagctgcctgcattagataaaatgctgtctttgccaaggcttttcttctcaaggttattcaaaatgaagtcttcttcaaaaacatgaagcagttgggtttttctgccatgaagtttggtaatgggatctaatgcaataatgcatcctggcctggctgttgattgttgactgacgatgttaaagacttcaccaacatatttagaaatttcagggttagaaagctcagataaaagtttcttagcatcaataactgcttcatataatctcagatattgtccatcactggctacaaagcatgcactaggagagttgcagtatgcacccagacaataactgggtataagagtgggcagccatgccacattggaaaaggcagaaacatgaagagaattaatccgggcaagctcagaaactcctccagaaaaagacaatggcccaactgggtcaaccctccacagaataagctcactgtaaactgcactgggatcctgaaatgccacgtcaacagtgcttttattttgttgtgtcaaagagcattcttcaatatttagagcatcaaaaggttgctctgggttatcaacatctggtgtccttaatgcattatggtgtgatgttgtcagcaataatggtaatactgagtggcaagctaaatcattaagatgaaaacgatgaccacaatatctggatttgtgggaaatactgagaacagtagaaaaagcagattcctcggcaaaactgaccagccactgattcagagaaccatcagcatgttttgatatcatcataacattaggcgtaaaaatacttaattttaaactattagatgatttattgtgaccagaagaaataagcattgatgtggaacgggtgaggccagaaggtttttgtttcccctgctgaatagccaagtcaacattcttggtacaggcatacatcattatgcttttacagagagagtttgcatcacctgtggggaaagctactggaattctggaaacaaaggacacctgtacttgacgaaacataccaggctggtattcatccagccaatccacatgccaaactagcaaagaaccatccatgggatgaatactaaatagcatatctgcatttttactccattcagacagaagtacttcaatctgatgatcaatggcagctgacgataatgatgtaaaacttgagtttggtaccattttatcacagcctaattccttcttttcgggatttattttcagatcatcaacaccatcatcagtttcttcatcagattttacatctgcctgattagaatcttctacactggcctcagaagatggttgttcaaaactttttctaagttgctgtaaaaaaacttccatggacaaagtaaaatgcagttctttattgtttagccagtgtacaacaaaaggtccggtcttctcttcattttcatttagactcagagatgtaatagatggaagaagtggaatgtctgtggctgggttgatgctggctgcaatatgaaagtggcaaagtgcattggcatgcagtggagtgttcctgtgaacatgatgaggatcctgctgatgtggtagatatcccgtatgtgctacaagagcaagtgatctcctccgacctctacgaaaatgtctcagatttacttctaaagcattttgaactcgttctttactggaagcatttctcttgaagttatttgttaaattaattgattcagtccaatggctgcagtcacctccgtatagcaaacaatcatttggtaaaaatgtctctacccaaagacgacacacattatctttgcagcaagtcaacagtacattacatacagaagccctaggcatatatttgcttgttttacgccaggaaaatccatttactgctcgaggatgggccagatacacaaaagaaaagtcaatttctccttgggattgtttttctgaacttccatctggagaagtaacagctgtccgccagttttctacattataccaaaccttcaaaagacagtcatccttcccagcagtggcaaaaaattctccatctggtgaaaatttcattaaatgaacttgggaagcagttttgcaatgccaaatgcatttccaatctccaaagttaagatctgttttatttaaattttcatcttcagttggcttctccaagttagtattggaccagagttgcaaatagctggaaccagttaaaagacgactgcctgtgggatcccaggttatattgtgtgctattgattccagaaaaaattggccacttttctgccactgactatataattccaaatttttcttttgttttggtaggttaactggttcaaaaatggagataacatttccataagacgctgcaatcttgccttgttgcattgaacagtctacacatcccacttgaatatttccatgtttagctcctgggattatctgtaatctttcaaaatcgcttcccagtattacaatgtcacatccagatgcataagccgtgaagcgctggtcgccaatgctgcccacggagaagcagtggtcgccagggttcacagccccggtcagcacctggtgcaggttcatgtcggcgccctagtccggccaggaaggccgcgctgtccacacacttcctctggacctcgggcagccgctcctgacccagcccgagtggcgcaagcagtacgcgctcgcactccccgcctgacctgtcccttcccggctccggtgcccgccacccccacagtcctccgccactcactacgcgcctct

SEQ ID NO: 9965 - RNA, 10233 nt, Homo sapiens
  source 1..10233: mol_type = other RNA
cacacacacacacacacgtatacatacatacaacttgggttccggagggtaaactactgaaaaccttacatattgagccatctagctcatttatcactgacgtctcaatgacaattttaatgaagatgttcattatttttttcattcttactcaaatacctatcattaattaagagaagagtttgagatgtataaggctaataaaggaagtgagagtgtggtgaattaagtgatgagtattatgtacaattgcctttacaaaaaacgtatttttactgtggaagaaattcatgcagagatgcctgtggaaaagtatcaataagaaaacaaaacacctttaacactatgacatactgattataatatactatgatatgtattattacagcattacttacacattctactttaggcaatgtaatctacttctgaatgaccttgttaatttttaaggcatcagtgcatcaagggcaaagctccataaaataaatataaaaacaagaaagcattagctaatttgtggcatagagaatgatcactgtatattatatctgttggccacttccatataggtaataaattgtacatcttattgtaaaaatgttatagcataaatttcacatcatttttcaacacttcatttaaagggctaaactgatctggcagtattctcattttcattgttccatcagctccacaggagaaaatgtgatttgcaggccctgtctcaatttgcatcactccagttccaatatttctaaaaatggactgccgagcatgttcactgacaaaagtatggagaagaccaaaggtagagagactccaaatctttatattgccttcggcagatcctgtaacaaagtactcttcagttggatcaacagcaacggctttaacaggagaatcatggctctggaaaagctgcctctgttgtcgttgacaaaggtcaaatacatatgtaaaaccttttctgccacctgatattagtagctgatgttttggagcatatgctaaaactgtggctccactgtcatggcaggtaaatgcatggactaaactattggcaggtgctacaagagtatcccacaaacatacgtttctattgtcagttgaaagaccagctgtagctatcagagaggaggaactaacgaagacaaaatcattggctgttttgttatgacactgccaagtcaggtatggcttaggcatgcttccagtaactggacaacatttccagtttgtttgatacaaacttaaatatccatcagcatcaactattccaaacttatttccctgatagttaaatctcattcttgtaactcttgaattgccaccagatcgaaaacaggttatttgttgagaatggccccattcaaacattctgacacttccatcttgagctcctgtcagatagtaaggaagagttggatgagaagtcattcttctaacattattaatggctttcttaatcatcacagatgctcctctgccagtctgtgtactaccaagccatggcatgttgattggagtgccaggattgctatgtgtatatggagttgtaccttgaacagctgttaaatcatcacgagcatgtataaccaagaaatcttctgatcctttggtttccacttctatatcatcatctacccaagtgtagacctgtgtggccagaattccagaaacatccagttcttgaacatcatgactggaagcgattgctatgcagtttctatttgccttattaacagcaaacgcagtaatgatatcagattccttatgaataattcttgctttacctccaggatatcccaaatctgcttctatcttattgatgtttggctcctccatcatagaatttttgatggtttcactgttgtcctctaatgactcatttagacaccgtttctttgtgaatatatttttgataaaggtttcctgaatttcttcctgcttcaccaaatactgccaaagcctcttcacagacagtgccagatggtgtttggatttgaaaggagtgtttgtaggttccagtaaagctttgtggcgaagaattgcaggacctgcagacaaactctcttcggcggtatgacttgcgatataattttgaggtggcccaccatggatttcaagtcgtcggagaagaacttgttcccaacattgaagagtttttagaaccgcatgacaaagaggtgaactaactggaagctctgcaagatcatgacctgcgaagggataaaaagtcttcaaattgttgagcaccaattgcaccatcgccaaccgcatcaaggaccaactatatgaatttgaattagaatgttcctggagatggaaatctgatgctaaaacatcatcatcatcatcattgtcatcatcatcacttcccagactctcctctgaatcatattcggctctactttgagaagagggtagaaaaggcttagctatgaaatagtcccagatactgagctcaggtgggatgaacttttctttaaccgccagtgactcctggcttactggtgccgaggaaggggtcagtggggcagattctctgcaagacatttttgacggcctaaaacgtttgttctgtttttctccttcttcaactagtgaagaaacaggtaaagtttttgaatgtgtctgttctttgctaggaacatgtgcacctccaccaaacacagcagaccacattttctcatttagaggatgggccacaatccgaaatagctcattacttgaatgtgtggccaggccatggatgaagagactaagatacactgctgtgagaatctcacagagcaagactgtaagccctgactgggcttcctcgccagaagaattcaaaagtcgaattagacaagttattcctggccattgagctggtgacgtattgggagttaatgcttcatctaagcttcctgttttcaaagaaggtcgatgaggaagcagtactgtctgatataccattccagtaaactgattcgtctgaaatgaactgtagttatgactaccacaaaggcactgataaatacaagcagaaagtgaagctgctaaagtatgcattacatacactttattgctttggatatcagggtggggtggtgaatcaaagtttattatggcatggagaatatcatgtgtcagattactaaggtgcaataatggattggcaactactgttttggcattggctgtacaagcaaagaggagaggcactgaggtttgctctgacagagggctagaaaatagtggttctgatgtttcctgctgagattcttgcaaaagcaaaatcaattccattcttacagatgcaagacccccaccatgggatccatgaagtatgcagtaactaagaaacattctcaaaagtgactgatacttcaagagccactgtcttttttcctgaaaattttctctcagttgtttcacttttgtttggtgaggcaaatcttcagcatcctcatttaatccaaattcatcttcatttctgccaaatgcagactgtagttcttcagcatctgagcaaaagtcacaagtcctctgaagagctatcacctctttttcaagccagtggtatagttggtaacgcaattttccaccatctatttcatagccagtagataaagtacgaagttctactgtgagaatctttaaacatgctctaaattttaactgaactgcaattatatcttctgatggatttaaaaggtcattttcatctagtgtgctgaaagattctgtgtagttagaacttatgtcatccaactttttatctgtttttctctgtaaaggttttagttctttcattgaaatagggacatcctcattttcttcatcattatcactgtcccattttaactctaaagagtcatcctgaaacacaacacttggttggctccagtcaaaagaaagagtggagtttgattgcttctctgaggaaccctctgaagaagatccaaaaccatttatcagtgactgtgaccaatcaacagcagaagacttatcttcccttgcatccaactttaatggagaagaaggagaacagtctttactagtatccagaaaactagaagccctataaaaaggtcttgttttcttgatgactttaggcatctttgataatacttccaaagccaacattgggcagccagcttttaaatgagcactggcagtggtaaaaaataaacgtctttcacttaaattaattgttcctgccagtccactttttcctgttaggctcatatgtgtggaaaatgtatcagatgatccaaaatgacgtctcagcaaaagaggatgtgttcttagataattgtagaaattaaaaactgtaggattactggctgataaaacttgatcatcattctctctgataggttgctttattaatgtttccagagcaccactataatcttccaaaatccaatatgccatgctccgaagaaaaggatcatgatgcatatttatgttcaatgaacacagttcactgacaggagaatcgattcccaaaacttttttacgtaaaatagatttatatgctgcagatgtatcaaattcagactcatagagtcttgctattacaagagccaactgaatgtcattcaatttctcaagacatacctcaattgcatctctgaggcaaccagctaaaagaaaaaatgctgcagaatgttcaaatctttgtttgcctagcaaagaaaaagcattctttaaagctgctttacgccacctctcatcctcaaaattgtgtccaaaaaactgtgtcatcctggtgtttttttcagctctatataatccccaaatcacagctttctttttcattgcaaggtaaaaaatggcagcatctaaaggatcattctttctataaaaggctgctttagctactttttctatgcatttgcgtaagatgcgggtattccggacccaccaccccacacccatagctcttagttcagaccaagtgggatcatctttctgcatggctggcaacatgttcagcagttcttcttctgctactgagtgaaatgcccaagcaaaatgacttgtagacaggccttggtgaaggagttgagctcgataggctggaagggaagttgtaagaaaggtatggagtcgaacagccaaaagaaattttaacccacattcatcaagagtttctccaccttggcttctgtctcggctttctccaatatcagtgcttgtagttgcaattgtatctgctaaggccatcaaagacatctgctccatccggctgagtcctggtaaactagaatgaagtaagtggccagaaagaacctgagcatgctcaggtccaaagtaagtcggactgtactgtgaaaggtcaataactctaggctttgtattttcttcatctgtctctaacatatgagtatcagtcattagaagttgagtctgaaaaagctcatcataactttctttagataattggtttgatttacttaacgtactctcattactagatttctccaaagatgagtaacagctatcatcatctgctgcaagtaaggcatataaaggaagtggaggaacagaatctatttctgtgtaatctgtattttcagccttgttgaatgcctgggggtctctggtagtgcttccactagcactgattgtgagagacctaaggcggcgttcatgattagattcagcttcattcagagccacaacttccccagcaatgcacttaacaagatgggacaagatggccttggctctccgaactttaccaagatccatgagttccaaaagctgcaagggatgatactgaggtagagtcggggaaagtacatgagctgcttcaaaaagacctgaatcttccatatccactgaaggatcgaatgcagttttctttccacagattttctgtgcaagactggtcatggatcgagtcagagttttctttggaggatgtaacccagaactggagttactctgttttattaaacttgttatagatggagtgctcccactgtacgaatctgttataacaggttcttgtttagaagatggttgccattggcaatacacatgcatttcacagtccattcctaccacaaggatgccatcccggacccacgataaagaaacaggaaaaggtggggagccatctacagaagaaactaggtccacacttcgtaatagtacaaatttagaaaggggcacaactttggtactctcccagagaggaaatgccagggtttccttaccagtttggtcttgtaccttgccagccaggggtccatacataaaaagttttgatccaattcctacagtcaggatatgagaaccgtcttctctagacatccaatctaagtgaactaaatgctttgtgtttgatgtgatattctctttactagataaatacatgtcttgtttattataggccactaaattgctatcaacactaatgccagaatccaatactgtgcttaactcatctaaatgaattgtctgctcaaggacccaacatgaacctcctgttgactcacattcaaaaatacttacatgcatcacaaagtcctgggaagatctactattagatgcaggctgcttataagctactgctaaacgatttgtatgtgcacagctaacttctacaggcctaccaggtacagttatactactattgctctgaagtccatcttcaataagtaatggccattcttcccaaatgtatgcaagatcaatttttccattctttgacgtggcagattctccatctgttactctgcatctccagaatcttactttctcatctgaacatgaagttgccaataaataaggagcactgcatgcaggatatatagaagatgaactcagatgtcctgctgatggcttaatacttattatctcaactccttctggtaaatgcaattcttggctataaaccatttctgaaaacagagtcaacctgctggtactctggagatttgctctgcaagcctgatacttttgtgaaaaaggagataggatcttctctggagaagaagaataatgttcttctggctgccaaaccgcttcggataattttgtatctactttttcatctaatgagacaggaattgactttagatgtaaattccacatgtgtaacagtgaacggttgtcttgagtgcattctattacaattaggtagaacttctcagaaaatccattaggtgagctgcctgcattagataaaatgctgtctttgccaaggcttttcttctcaaggttattcaaaatgaagtcttcttcaaaaacatgaagcagttgggtttttctgccatgaagtttggtaatgggatctaatgcaataatgcatcctggcctggctgttgattgttgactgacgatgttaaagacttcaccaacatatttagaaatttcagggttagaaagctcagataaaagtttcttagcatcaataactgcttcatataatctcagatattgtccatcactggctacaaagcatgcactaggagagttgcagtatgcacccagacaataactgggtataagagtgggcagccatgccacattggaaaaggcagaaacatgaagagaattaatccgggcaagctcagaaactcctccagaaaaagacaatggcccaactgggtcaaccctccacagaataagctcactgtaaactgcactgggatcctgaaatgccacgtcaacagtgcttttattttgttgtgtcaaagagcattcttcaatatttagagcatcaaaaggttgctctgggttatcaacatctggtgtccttaatgcattatggtgtgatgttgtcagcaataatggtaatactgagtggcaagctaaatcattaagatgaaaacgatgaccacaatatctggatttgtgggaaatactgagaacagtagaaaaagcagattcctcggcaaaactgaccagccactgattcagagaaccatcagcatgttttgatatcatcataacattaggcgtaaaaatacttaattttaaactattagatgatttattgtgaccagaagaaataagcattgatgtggaacgggtgaggccagaaggtttttgtttcccctgctgaatagccaagtcaacattcttggtacaggcatacatcattatgcttttacagagagagtttgcatcacctgtggggaaagctactggaattctggaaacaaaggacacctgtacttgacgaaacataccaggctggtattcatccagccaatccacatgccaaactagcaaagaaccatccatgggatgaatactaaatagcatatctgcatttttactccattcagacagaagtacttcaatctgatgatcaatggcagctgacgataatgatgtaaaacttgagtttggtaccattttatcacagcctaattccttcttttcgggatttattttcagatcatcaacaccatcatcagtttcttcatcagattttacatctgcctgattagaatcttctacactggcctcagaagatggttgttcaaaactttttctaagttgctgtaaaaaaacttccatggacaaagtaaaatgcagttctttattgtttagccagtgtacaacaaaaggtccggtcttctcttcattttcatttagactcagagatgtaatagatggaagaagtggaatgtctgtggctgggttgatgctggctgcaatatgaaagtggcaaagtgcattggcatgcagtggagtgttcctgtgaacatgatgaggatcctgctgatgtggtagatatcccgtatgtgctacaagagcaagtgatctcctccgacctctacgaaaatgtctcagatttacttctaaagcattttgaactcgttctttactggaagcatttctcttgaagttatttgttaaattaattgattcagtccaatggctgcagtcacctccgtatagcaaacaatcatttggtaaaaatgtctctacccaaagacgacacacattatctttgcagcaagtcaacagtacattacatacagaagccctaggcatatatttgcttgttttacgccaggaaaatccatttactgctcgaggatgggccagatacacaaaagaaaagtcaatttctccttgggattgtttttctgaacttccatctggagaagtaacagctgtccgccagttttctacattataccaaaccttcaaaagacagtcatccttcccagcagtggcaaaaaattctccatctggtgaaaatttcattaaatgaacttgggaagcagttttgcaatgccaaatgcatttccaatctccaaagttaagatctgttttatttaaattttcatcttcagttggcttctccaagttagtattggaccagagttgcaaatagctggaaccagttaaaagacgactgcctgtgggatcccaggttatattgtgtgctattgattccagaaaaaattggccacttttctgccactgactatataattccaaatttttcttttgttttggtaggttaactggttcaaaaatggagataacatttccataagacgctgcaatcttgccttgttgcattgaacagtctacacatcccacttgaatatttccatgtttagctcctgggattatctgtaatctttcaaaatcgcttcccagtattacaatgtcacatccagatgcataagccgtgaagcgctggtcgccaatgctgcccacggagaagcagtggtcgccagggttcacagccccggtcagcacctggtgcaggttcatgtcggcgccctagtcctgcaacggacaccgcatccagctcatgccacgggtcagcggctgcttccctccctccttccctcaggggcggcggccgctcttcggtggcgacggcagaagcagcgacaggcgcctggagccggagccgctcagctggggcccgcgactcatcccgagccccggagggcgaggcccggagggggcgggtcggcgagagggcggagcgccgcgctccttcgcgcacctgtcactccccgcgctagcccaggtgaagctcagggtcccctcaccggccacgacccggggccgactcaccggccaggaaggccgcgctgtccacacacttcctctggacctcgggcagccgctcctgacccagcccgagtggcgcaagcagtacgcgctcgcactccccgcctgacctgtcccttcccggctccggtgcccgccacccccacagtcctccgccactcactacgcgcctct

SEQ ID NO: 9966 - RNA, 9392 nt, Homo sapiens
  source 1..9392: mol_type = other RNA
cacacacacacacacacgtatacatacatacaacttgggttccggagggtaaactactgaaaaccttacatattgagccatctagctcatttatcactgacgtctcaatgacaattttaatgaagatgttcattatttttttcattcttactcaaatacctatcattaattaagagaagagtttgagatgtataaggctaataaaggaagtgagagtgtggtgaattaagtgatgagtattatgtacaattgcctttacaaaaaacgtatttttactgtggaagaaattcatgcagagatgcctgtggaaaagtatcaataagaaaacaaaacacctttaacactatgacatactgattataatatactatgatatgtattattacagcattacttacacattctactttaggcaatgtaatctacttctgaatgaccttgttaatttttaaggcatcagtgcatcaagggcaaagctccataaaataaatataaaaacaagaaagcattagctaatttgtggcatagagaatgatcactgtatattatatctgttggccacttccatataggtaataaattgtacatcttattgtaaaaatgttatagcataaatttcacatcatttttcaacacttcatttaaagggctaaactgatctggcagtattctcattttcattgttccatcagctccacaggagaaaatgtgatttgcaggccctgtctcaatttgcatcactccagttccaatatttctaaaaatggactgccgagcatgttcactgacaaaagtatggagaagaccaaaggtagagagactccaaatctttatattgccttcggcagatcctgtaacaaagtactcttcagttggatcaacagcaacggctttaacaggagaatcatggctctggaaaagctgcctctgttgtcgttgacaaaggtcaaatacatatgtaaaaccttttctgccacctgatattagtagctgatgttttggagcatatgctaaaactgtggctccactgtcatggcaggtaaatgcatggactaaactattggcaggtgctacaagagtatcccacaaacatacgtttctattgtcagttgaaagaccagctgtagctatcagagaggaggaactaacgaagacaaaatcattggctgttttgttatgacactgccaagtcaggtatggcttaggcatgcttccagtaactggacaacatttccagtttgtttgatacaaacttaaatatccatcagcatcaactattccaaacttatttccctgatagttaaatctcattcttgtaactcttgaattgccaccagatcgaaaacaggttatttgttgagaatggccccattcaaacattctgacacttccatcttgagctcctgtcagatagtaaggaagagttggatgagaagtcattcttctaacattattaatggctttcttaatcatcacagatgctcctctgccagtctgtgtactaccaagccatggcatgttgattggagtgccaggattgctatgtgtatatggagttgtaccttgaacagctgttaaatcatcacgagcatgtataaccaagaaatcttctgatcctttggtttccacttctatatcatcatctacccaagtgtagacctgtgtggccagaattccagaaacatccagttcttgaacatcatgactggaagcgattgctatgcagtttctatttgccttattaacagcaaacgcagtaatgatatcagattccttatgaataattcttgctttacctccaggatatcccaaatctgcttctatcttattgatgtttggctcctccatcatagaatttttgatggtttcactgttgtcctctaatgactcatttagacaccgtttctttgtgaatatatttttgataaaggtttcctgaatttcttcctgcttcaccaaatactgccaaagcctcttcacagacagtgccagatggtgtttggatttgaaaggagtgtttgtaggttccagtaaagctttgtggcgaagaattgcaggacctgcagacaaactctcttcggcggtatgacttgcgatataattttgaggtggcccaccatggatttcaagtcgtcggagaagaacttgttcccaacattgaagagtttttagaaccgcatgacaaagaggtgaactaactggaagctctgcaagatcatgacctgcgaagggataaaaagtcttcaaattgttgagcaccaattgcaccatcgccaaccgcatcaaggaccaactatatgaatttgaattagaatgttcctggagatggaaatctgatgctaaaacatcatcatcatcatcattgtcatcatcatcacttcccagactctcctctgaatcatattcggctctactttgagaagagggtagaaaaggcttagctatgaaatagtcccagatactgagctcaggtgggatgaacttttctttaaccgccagtgactcctggcttactggtgccgaggaaggggtcagtggggcagattctctgcaagacatttttgacggcctaaaacgtttgttctgtttttctccttcttcaactagtgaagaaactgcaagactgggagggctatgagaactgatggctgaaagagctttggaaaagcccacacattccatggagaataccactacctggtgggggctaggcatagcaaagtgccttccaggtaaagtttttgaatgtgtctgttctttgctaggaacatgtgcacctccaccaaacacagcagaccacattttctcatttagaggatgggccacaatccgaaatagctcattacttgaatgtgtggccaggccatggatgaagagactaagatacactgctgtgagaatctcacagagcaagactgtaagccctgactgggcttcctcgccagaagaattcaaaagtcgaattagacaagttattcctggccattgagctggtgacgtattgggagttaatgcttcatctaagcttcctgttttcaaagaaggtcgatgaggaagcagtactgtctgatataccattccagtaaactgattcgtctgaaatgaactgtagttatgactaccacaaaggcactgataaatacaagcagaaagtgaagctgctaaagtatgcattacatacactttattgctttggatatcagggtggggtggtgaatcaaagtttattatggcatggagaatatcatgtgtcagattactaaggtgcaataatggattggcaactactgttttggcattggctgtacaagcaaagaggagaggcactgaggtttgctctgacagagggctagaaaatagtggttctgatgtttcctgctgagattcttgcaaaagcaaaatcaattccattcttacagatgcaagacccccaccatgggatccatgaagtatgcagtaactaagaaacattctcaaaagtgactgatacttcaagagccactgtcttttttcctgaaaattttctctcagttgtttcacttttgtttggtgaggcaaatcttcagcatcctcatttaatccaaattcatcttcatttctgccaaatgcagactgtagttcttcagcatctgagcaaaagtcacaagtcctctgaagagctatcacctctttttcaagccagtggtatagttggtaacgcaattttccaccatctatttcatagccagtagataaagtacgaagttctactgtgagaatctttaaacatgctctaaattttaactgaactgcaattatatcttctgatggatttaaaaggtcattttcatctagtgtgctgaaagattctgtgtagttagaacttatgtcatccaactttttatctgtttttctctgtaaaggttttagttctttcattgaaatagggacatcctcattttcttcatcattatcactgtcccattttaactctaaagagtcatcctgaaacacaacacttggttggctccagtcaaaagaaagagtggagtttgattgcttctctgaggaaccctctgaagaagatccaaaaccatttatcagtgactgtgaccaatcaacagcagaagacttatcttcccttgcatccaactttaatggagaagaaggagaacagtctttactagtatccagaaaactagaagccctataaaaaggtcttgttttcttgatgactttaggcatctttgataatacttccaaagccaacattgggcagccagcttttaaatgagcactggcagtggtaaaaaataaacgtctttcacttaaattaattgttcctgccagtccactttttcctgttaggctcatatgtgtggaaaatgtatcagatgatccaaaatgacgtctcagcaaaagaggatgtgttcttagataattgtagaaattaaaaactgtaggattactggctgataaaacttgatcatcattctctctgataggttgctttattaatgtttccagagcaccactataatcttccaaaatccaatatgccatgctccgaagaaaaggatcatgatgcatatttatgttcaatgaacacagttcactgacaggagaatcgattcccaaaacttttttacgtaaaatagatttatatgctgcagatgtatcaaattcagactcatagagtcttgctattacaagagccaactgaatgtcattcaatttctcaagacatacctcaattgcatctctgaggcaaccagctaaaagaaaaaatgctgcagaatgttcaaatctttgtttgcctagcaaagaaaaagcattctttaaagctgctttacgccacctctcatcctcaaaattgtgtccaaaaaactgtgtcatcctggtgtttttttcagctctatataatccccaaatcacagctttctttttcattgcaaggtaaaaaatggcagcatctaaaggatcattctttctataaaaggctgctttagctactttttctatgcatttgcgtaagatgcgggtattccggacccaccaccccacacccatagctcttagttcagaccaagtgggatcatctttctgcatggctggcaacatgttcagcagttcttcttctgctactgagtgaaatgcccaagcaaaatgacttgtagacaggccttggtgaaggagttgagctcgataggctggaagggaagttgtaagaaaggtatggagtcgaacagccaaaagaaattttaacccacattcatcaagagtttctccaccttggcttctgtctcggctttctccaatatcagtgcttgtagttgcaattgtatctgctaaggccatcaaagacatctgctccatccggctgagtcctggtaaactagaatgaagtaagtggccagaaagaacctgagcatgctcaggtccaaagtaagtcggactgtactgtgaaaggtcaataactctaggctttgtattttcttcatctgtctctaacatatgagtatcagtcattagaagttgagtctgaaaaagctcatcataactttctttagataattggtttgatttacttaacgtactctcattactagatttctccaaagatgagtaacagctatcatcatctgctgcaagtaaggcatataaaggaagtggaggaacagaatctatttctgtgtaatctgtattttcagccttgttgaatgcctgggggtctctggtagtgcttccactagcactgattgtgagagacctaaggcggcgttcatgattagattcagcttcattcagagccacaacttccccagcaatgcacttaacaagatgggacaagatggccttggctctccgaactttaccaagatccatgagttccaaaagctgcaagggatgatactgaggtagagtcggggaaagtacatgagctgcttcaaaaagacctgaatcttccatatccactgaaggatcgaatgcagttttctttccacagattttctgtgcaagactggtcatggatcgagtcagagttttctttggaggatgtaacccagaactggagttactctgttttattaaacttgttatagatggagtgctcccactgtacgaatctgttataacaggttcttgtttagaagatggttgccattggcaatacacatgcatttcacagtccattcctaccacaaggatgccatcccggacccacgataaagaaacaggaaaaggtggggagccatctacagaagaaactaggtccacacttcgtaatagtacaaatttagaaaggggcacaactttggtactctcccagagaggaaatgccagggtttccttaccagtttggtcttgtaccttgccagccaggggtccatacataaaaagttttgatccaattcctacagtcaggatatgagaaccgtcttctctagacatccaatctaagtgaactaaatgctttgtgtttgatgtgatattctctttactagataaatacatgtcttgtttattataggccactaaattgctatcaacactaatgccagaatccaatactgtgcttaactcatctaaatgaattgtctgctcaaggacccaacatgaacctcctgttgactcacattcaaaaatacttacatgcatcacaaagtcctgggaagatctactattagatgcaggctgcttataagctactgctaaacgatttgtatgtgcacagctaacttctacaggcctaccaggtacagttatactactattgctctgaagtccatcttcaataagtaatggccattcttcccaaatgtatgcaagatcaatttttccattctttgacgtggcagattctccatctgttactctgcatctccagaatcttactttctcatctgaacatgaagttgccaataaataaggagcactgcatgcaggatatatagaagatgaactcagatgtcctgctgatggcttaatacttattatctcaactccttctggtaaatgcaattcttggctataaaccatttctgaaaacagagtcaacctgctggtactctggagatttgctctgcaagcctgatacttttgtgaaaaaggagataggatcttctctggagaagaagaataatgttcttctggctgccaaaccgcttcggataattttgtatctactttttcatctaatgagacaggaattgactttagatgtaaattccacatgtgtaacagtgaacggttgtcttgagtgcattctattacaattaggtagaacttctcagaaaatccattaggtgagctgcctgcattagataaaatgctgtctttgccaaggcttttcttctcaaggttattcaaaatgaagtcttcttcaaaaacatgaagcagttgggtttttctgccatgaagtttggtaatgggatctaatgcaataatgcatcctggcctggctgttgattgttgactgacgatgttaaagacttcaccaacatatttagaaatttcagggttagaaagctcagataaaagtttcttagcatcaataactgcttcatataatctcagatattgtccatcactggctacaaagcatgcactaggagagttgcagtatgcacccagacaataactgggtataagagtgggcagccatgccacattggaaaaggcagaaacatgaagagaattaatccgggcaagctcagaaactcctccagaaaaagacaatggcccaactgggtcaaccctccacagaataagctcactgtaaactgcactgggatcctgaaatgccacgtcaacagtgcttttattttgttgtgtcaaagagcattcttcaatatttagagcatcaaaaggttgctctgggttatcaacatctggtgtccttaatgcattatggtgtgatgttgtcagcaataatggtaatactgagtggcaagctaaatcattaagatgaaaacgatgaccacaatatctggatttgtgggaaatactgagaacagtagaaaaagcagattcctcggcaaaactgaccagccactgattcagagaaccatcagcatgttttgatatcatcataacattaggcgtaaaaatacttaattttaaactattagatgatttattgtgaccagaagaaataagcattgatgtggaacgggtgaggccagaaggtttttgtttcccctgctgaatagccaagtcaacattcttggtacaggcatacatcattatgcttttacagagagagtttgcatcacctgtggggaaagctactggaattctggaaacaaaggacacctgtacttgacgaaacataccaggctggtattcatccagccaatccacatgccaaactagcaaagaaccatccatgggatgaatactaaatagcatatctgcatttttactccattcagacagaagtacttcaatctgatgatcaatggcagctgacgataatgatgtaaaacttgagtttggtaccattttatcacagcctaattccttcttttcgggatttattttcagatcatcaacaccatcatcagtttcttcatcagattttacatctgcctgattagaatcttctacactggcctcagaagatggttgttcaaaactttttctaagttgctgtaaaaaaacttccatggacaaagtaaaatgcagttctttattgtttagccagtgtacaacaaaaggtccggtcttctcttcattttcatttagactcagagatgtaatagatggaagaagtggaatgtctgtggctgggttgatgctggctgcaatatgaaagtggcaaagtgcattggcatgcagtggagtgttcctgtgaacatgatgaggatcctgctgatgtggtagatatcccgtatgtgctacaagagcaagtgatctcctccgacctctacgaaaatgtctcagatttacttctaaagcattttgaactcgttctttactggaagcatttctcttgaagttatttgttaaattaattgattcagtccaatggctgcagtcacctccgtatagcaaacaatcatttggtaaaaatgtctctacccaaagacgacacacattatctttgcagcaagtcaacagtacattacatacagaagccctaggcatatatttgcttgttttacgccaggaaaatccatttactgctcgaggatgggccagatacacaaaagaaaagtcaatttctccttgggattgtttttctgaacttccatctggagaagtaacagctgtccgccagttttctacattataccaaaccttcaaaagacagtcatccttcccagcagtggcaaaaaattctccatctggtgaaaatttcattaaatgaacttgggaagcagttcaaatttttcttttgttttggtagg

SEQ ID NO: 9967 - RNA, 10193 nt, Homo sapiens
  source 1..10193: mol_type = other RNA
cacacacacacacacacgtatacatacatacaacttgggttccggagggtaaactactgaaaaccttacatattgagccatctagctcatttatcactgacgtctcaatgacaattttaatgaagatgttcattatttttttcattcttactcaaatacctatcattaattaagagaagagtttgagatgtataaggctaataaaggaagtgagagtgtggtgaattaagtgatgagtattatgtacaattgcctttacaaaaaacgtatttttactgtggaagaaattcatgcagagatgcctgtggaaaagtatcaataagaaaacaaaacacctttaacactatgacatactgattataatatactatgatatgtattattacagcattacttacacattctactttaggcaatgtaatctacttctgaatgaccttgttaatttttaaggcatcagtgcatcaagggcaaagctccataaaataaatataaaaacaagaaagcattagctaatttgtggcatagagaatgatcactgtatattatatctgttggccacttccatataggtaataaattgtacatcttattgtaaaaatgttatagcataaatttcacatcatttttcaacacttcatttaaagggctaaactgatctggcagtattctcattttcattgttccatcagctccacaggagaaaatgtgatttgcaggccctgtctcaatttgcatcactccagttccaatatttctaaaaatggactgccgagcatgttcactgacaaaagtatggagaagaccaaaggtagagagactccaaatctttatattgccttcggcagatcctgtaacaaagtactcttcagttggatcaacagcaacggctttaacaggagaatcatggctctggaaaagctgcctctgttgtcgttgacaaaggtcaaatacatatgtaaaaccttttctgccacctgatattagtagctgatgttttggagcatatgctaaaactgtggctccactgtcatggcaggtaaatgcatggactaaactattggcaggtgctacaagagtatcccacaaacatacgtttctattgtcagttgaaagaccagctgtagctatcagagaggaggaactaacgaagacaaaatcattggctgttttgttatgacactgccaagtcaggtatggcttaggcatgcttccagtaactggacaacatttccagtttgtttgatacaaacttaaatatccatcagcatcaactattccaaacttatttccctgatagttaaatctcattcttgtaactcttgaattgccaccagatcgaaaacaggttatttgttgagaatggccccattcaaacattctgacacttccatcttgagctcctgtcagatagtaaggaagagttggatgagaagtcattcttctaacattattaatggctttcttaatcatcacagatgctcctctgccagtctgtgtactaccaagccatggcatgttgattggagtgccaggattgctatgtgtatatggagttgtaccttgaacagctgttaaatcatcacgagcatgtataaccaagaaatcttctgatcctttggtttccacttctatatcatcatctacccaagtgtagacctgtgtggccagaattccagaaacatccagttcttgaacatcatgactggaagcgattgctatgcagtttctatttgccttattaacagcaaacgcagtaatgatatcagattccttatgaataattcttgctttacctccaggatatcccaaatctgcttctatcttattgatgtttggctcctccatcatagaatttttgatggtttcactgttgtcctctaatgactcatttagacaccgtttctttgtgaatatatttttgataaaggtttcctgaatttcttcctgcttcaccaaatactgccaaagcctcttcacagacagtgccagatggtgtttggatttgaaaggagtgtttgtaggttccagtaaagctttgtggcgaagaattgcaggacctgcagacaaactctcttcggcggtatgacttgcgatataattttgaggtggcccaccatggatttcaagtcgtcggagaagaacttgttcccaacattgaagagtttttagaaccgcatgacaaagaggtgaactaactggaagctctgcaagatcatgacctgcgaagggataaaaagtcttcaaattgttgagcaccaattgcaccatcgccaaccgcatcaaggaccaactatatgaatttgaattagaatgttcctggagatggaaatctgatgctaaaacatcatcatcatcatcattgtcatcatcatcacttcccagactctcctctgaatcatattcggctctactttgagaagagggtagaaaaggcttagctatgaaatagtcccagatactgagctcaggtgggatgaacttttctttaaccgccagtgactcctggcttactggtgccgaggaaggggtcagtggggcagattctctgcaagacatttttgacggcctaaaacgtttgttctgtttttctccttcttcaactagtgaagaaactgcaagactgggagggctatgagaactgatggctgaaagagctttggaaaagcccacacattccatggagaataccactacctggtgggggctaggcatagcaaagtgccttccaggtaaagtttttgaatgtgtctgttctttgctaggaacatgtgcacctccaccaaacacagcagaccacattttctcatttagaggatgggccacaatccgaaatagctcattacttgaatgtgtggccaggccatggatgaagagactaagatacactgctgtgagaatctcacagagcaagactgtaagccctgactgggcttcctcgccagaagaattcaaaagtcgaattagacaagttattcctggccattgagctggtgacgtattgggagttaatgcttcatctaagcttcctgttttcaaagaaggtcgatgaggaagcagtactgtctgatataccattccagtaaactgattcgtctgaaatgaactgtagttatgactaccacaaaggcactgataaatacaagcagaaagtgaagctgctaaagtatgcattacatacactttattgctttggatatcagggtggggtggtgaatcaaagtttattatggcatggagaatatcatgtgtcagattactaaggtgcaataatggattggcaactactgttttggcattggctgtacaagcaaagaggagaggcactgaggtttgctctgacagagggctagaaaatagtggttctgatgtttcctgctgagattcttgcaaaagcaaaatcaattccattcttacagatgcaagacccccaccatgggatccatgaagtatgcagtaactaagaaacattctcaaaagtgactgatacttcaagagccactgtcttttttcctgaaaattttctctcagttgtttcacttttgtttggtgaggcaaatcttcagcatcctcatttaatccaaattcatcttcatttctgccaaatgcagactgtagttcttcagcatctgagcaaaagtcacaagtcctctgaagagctatcacctctttttcaagccagtggtatagttggtaacgcaattttccaccatctatttcatagccagtagataaagtacgaagttctactgtgagaatctttaaacatgctctaaattttaactgaactgcaattatatcttctgatggatttaaaaggtcattttcatctagtgtgctgaaagattctgtgtagttagaacttatgtcatccaactttttatctgtttttctctgtaaaggttttagttctttcattgaaatagggacatcctcattttcttcatcattatcactgtcccattttaactctaaagagtcatcctgaaacacaacacttggttggctccagtcaaaagaaagagtggagtttgattgcttctctgaggaaccctctgaagaagatccaaaaccatttatcagtgactgtgaccaatcaacagcagaagacttatcttcccttgcatccaactttaatggagaagaaggagaacagtctttactagtatccagaaaactagaagccctataaaaaggtcttgttttcttgatgactttaggcatctttgataatacttccaaagccaacattgggcagccagcttttaaatgagcactggcagtggtaaaaaataaacgtctttcacttaaattaattgttcctgccagtccactttttcctgttaggctcatatgtgtggaaaatgtatcagatgatccaaaatgacgtctcagcaaaagaggatgtgttcttagataattgtagaaattaaaaactgtaggattactggctgataaaacttgatcatcattctctctgataggttgctttattaatgtttccagagcaccactataatcttccaaaatccaatatgccatgctccgaagaaaaggatcatgatgcatatttatgttcaatgaacacagttcactgacaggagaatcgattcccaaaacttttttacgtaaaatagatttatatgctgcagatgtatcaaattcagactcatagagtcttgctattacaagagccaactgaatgtcattcaatttctcaagacatacctcaattgcatctctgaggcaaccagctaaaagaaaaaatgctgcagaatgttcaaatctttgtttgcctagcaaagaaaaagcattctttaaagctgctttacgccacctctcatcctcaaaattgtgtccaaaaaactgtgtcatcctggtgtttttttcagctctatataatccccaaatcacagctttctttttcattgcaaggtaaaaaatggcagcatctaaaggatcattctttctataaaaggctgctttagctactttttctatgcatttgcgtaagatgcgggtattccggacccaccaccccacacccatagctcttagttcagaccaagtgggatcatctttctgcatggctggcaacatgttcagcagttcttcttctgctactgagtgaaatgcccaagcaaaatgacttgtagacaggccttggtgaaggagttgagctcgataggctggaagggaagttgtaagaaaggtatggagtcgaacagccaaaagaaattttaacccacattcatcaagagtttctccaccttggcttctgtctcggctttctccaatatcagtgcttgtagttgcaattgtatctgctaaggccatcaaagacatctgctccatccggctgagtcctggtaaactagaatgaagtaagtggccagaaagaacctgagcatgctcaggtccaaagtaagtcggactgtactgtgaaaggtcaataactctaggctttgtattttcttcatctgtctctaacatatgagtatcagtcattagaagttgagtctgaaaaagctcatcataactttctttagataattggtttgatttacttaacgtactctcattactagatttctccaaagatgagtaacagctatcatcatctgctgcaagtaaggcatataaaggaagtggaggaacagaatctatttctgtgtaatctgtattttcagccttgttgaatgcctgggggtctctggtagtgcttccactagcactgattgtgagagacctaaggcggcgttcatgattagattcagcttcattcagagccacaacttccccagcaatgcacttaacaagatgggacaagatggccttggctctccgaactttaccaagatccatgagttccaaaagctgcaagggatgatactgaggtagagtcggggaaagtacatgagctgcttcaaaaagacctgaatcttccatatccactgaaggatcgaatgcagttttctttccacagattttctgtgcaagactggtcatggatcgagtcagagttttctttggaggatgtaacccagaactggagttactctgttttattaaacttgttatagatggagtgctcccactgtacgaatctgttataacaggttcttgtttagaagatggttgccattggcaatacacatgcatttcacagtccattcctaccacaaggatgccatcccggacccacgataaagaaacaggaaaaggtggggagccatctacagaagaaactaggtccacacttcgtaatagtacaaatttagaaaggggcacaactttggtactctcccagagaggaaatgccagggtttccttaccagtttggtcttgtaccttgccagccaggggtccatacataaaaagttttgatccaattcctacagtcaggatatgagaaccgtcttctctagacatccaatctaagtgaactaaatgctttgtgtttgatgtgatattctctttactagataaatacatgtcttgtttattataggccactaaattgctatcaacactaatgccagaatccaatactgtgcttaactcatctaaatgaattgtctgctcaaggacccaacatgaacctcctgttgactcacattcaaaaatacttacatgcatcacaaagtcctgggaagatctactattagatgcaggctgcttataagctactgctaaacgatttgtatgtgcacagctaacttctacaggcctaccaggtacagttatactactattgctctgaagtccatcttcaataagtaatggccattcttcccaaatgtatgcaagatcaatttttccattctttgacgtggcagattctccatctgttactctgcatctccagaatcttactttctcatctgaacatgaagttgccaataaataaggagcactgcatgcaggatatatagaagatgaactcagatgtcctgctgatggcttaatacttattatctcaactccttctggtaaatgcaattcttggctataaaccatttctgaaaacagagtcaacctgctggtactctggagatttgctctgcaagcctgatacttttgtgaaaaaggagataggatcttctctggagaagaagaataatgttcttctggctgccaaaccgcttcggataattttgtatctactttttcatctaatgagacaggaattgactttagatgtaaattccacatgtgtaacagtgaacggttgtcttgagtgcattctattacaattaggtagaacttctcagaaaatccattaggtgagctgcctgcattagataaaatgctgtctttgccaaggcttttcttctcaaggttattcaaaatgaagtcttcttcaaaaacatgaagcagttgggtttttctgccatgaagtttggtaatgggatctaatgcaataatgcatcctggcctggctgttgattgttgactgacgatgttaaagacttcaccaacatatttagaaatttcagggttagaaagctcagataaaagtttcttagcatcaataactgcttcatataatctcagatattgtccatcactggctacaaagcatgcactaggagagttgcagtatgcacccagacaataactgggtataagagtgggcagccatgccacattggaaaaggcagaaacatgaagagaattaatccgggcaagctcagaaactcctccagaaaaagacaatggcccaactgggtcaaccctccacagaataagctcactgtaaactgcactgggatcctgaaatgccacgtcaacagtgcttttattttgttgtgtcaaagagcattcttcaatatttagagcatcaaaaggttgctctgggttatcaacatctggtgtccttaatgcattatggtgtgatgttgtcagcaataatggtaatactgagtggcaagctaaatcattaagatgaaaacgatgaccacaatatctggatttgtgggaaatactgagaacagtagaaaaagcagattcctcggcaaaactgaccagccactgattcagagaaccatcagcatgttttgatatcatcataacattaggcgtaaaaatacttaattttaaactattagatgatttattgtgaccagaagaaataagcattgatgtggaacgggtgaggccagaaggtttttgtttcccctgctgaatagccaagtcaacattcttggtacaggcatacatcattatgcttttacagagagagtttgcatcacctgtggggaaagctactggaattctggaaacaaaggacacctgtacttgacgaaacataccaggctggtattcatccagccaatccacatgccaaactagcaaagaaccatccatgggatgaatactaaatagcatatctgcatttttactccattcagacagaagtacttcaatctgatgatcaatggcagctgacgataatgatgtaaaacttgagtttggtaccattttatcacagcctaattccttcttttcgggatttattttcagatcatcaacaccatcatcagtttcttcatcagattttacatctgcctgattagaatcttctacactggcctcagaagatggttgttcaaaactttttctaagttgctgtaaaaaaacttccatggacaaagtaaaatgcagttctttattgtttagccagtgtacaacaaaaggtccggtcttctcttcattttcatttagactcagagatgtaatagatggaagaagtggaatgtctgtggctgggttgatgctggctgcaatatgaaagtggcaaagtgcattggcatgcagtggagtgttcctgtgaacatgatgaggatcctgctgatgtggtagatatcccgtatgtgctacaagagcaagtgatctcctccgacctctacgaaaatgtctcagatttacttctaaagcattttgaactcgttctttactggaagcatttctcttgaagttatttgttaaattaattgattcagtccaatggctgcagtcacctccgtatagcaaacaatcatttggtaaaaatgtctctacccaaagacgacacacattatctttgcagcaagtcaacagtacattacatacagaagccctaggcatatatttgcttgttttacgccaggaaaatccatttactgctcgaggatgggccagatacacaaaagaaaagtcaatttctccttgggattgtttttctgaacttccatctggagaagtaacagctgtccgccagttttctacattataccaaaccttcaaaagacagtcatccttcccagcagtggcaaaaaattctccatctggtgaaaatttcattaaatgaacttgggaagcagttctgtgggatcccaggttatattgtgtgctattgattccagaaaaaattggccacttttctgccactgactatataattccaaatttttcttttgttttggtaggttaactggttcaaaaatggagataacatttccataagacgctgcaatcttgccttgttgcattgaacagtctacacatcccacttgaatatttccatgtttagctcctgggattatctgtaatctttcaaaatcgcttcccagtattacaatgtcacatccagatgcataagccgtgaagcgctggtcgccaatgctgcccacggagaagcagtggtcgccagggttcacagccccggtcagcacctggtgcaggttcatgtcggcgccctagtcctgcaacggacaccgcatccagctcatgccacgggtcagcggctgcttccctccctccttccctcaggggcggcggccgctcttcggtggcgacggcagaagcagcgacaggcgcctggagccggagccgctcagctggggcccgcgactcatcccgagccccggagggcgaggcccggagggggcgggtcggcgagagggcggagcgccgcgctccttcgcgcacctgtcactccccgcgctagcccaggtgaagctcagggtcccctcaccggccacgacccggggccgactcaccggccaggaaggccgcgctgtccacacacttcctctggacctcgggcagccgctcctgacccagcccgagtggcgcaagcagtacgcgctcgcactccccgcctgacctgtcccttcccggctccggtgcccgccacccccacagtcctc

SEQ ID NO: 9968 - RNA, 9556 nt, Homo sapiens
  source 1..9556: mol_type = other RNA
cacacacacacacacacgtatacatacatacaacttgggttccggagggtaaactactgaaaaccttacatattgagccatctagctcatttatcactgacgtctcaatgacaattttaatgaagatgttcattatttttttcattcttactcaaatacctatcattaattaagagaagagtttgagatgtataaggctaataaaggaagtgagagtgtggtgaattaagtgatgagtattatgtacaattgcctttacaaaaaacgtatttttactgtggaagaaattcatgcagagatgcctgtggaaaagtatcaataagaaaacaaaacacctttaacactatgacatactgattataatatactatgatatgtattattacagcattacttacacattctactttaggcaatgtaatctacttctgaatgaccttgttaatttttaaggcatcagtgcatcaagggcaaagctccataaaataaatataaaaacaagaaagcattagctaatttgtggcatagagaatgatcactgtatattatatctgttggccacttccatataggtaataaattgtacatcttattgtaaaaatgttatagcataaatttcacatcatttttcaacacttcatttaaagggctaaactgatctggcagtattctcattttcattgttccatcagctccacaggagaaaatgtgatttgcaggccctgtctcaatttgcatcactccagttccaatatttctaaaaatggactgccgagcatgttcactgacaaaagtatggagaagaccaaaggtagagagactccaaatctttatattgccttcggcagatcctgtaacaaagtactcttcagttggatcaacagcaacggctttaacaggagaatcatggctctggaaaagctgcctctgttgtcgttgacaaaggtcaaatacatatgtaaaaccttttctgccacctgatattagtagctgatgttttggagcatatgctaaaactgtggctccactgtcatggcaggtaaatgcatggactaaactattggcaggtgctacaagagtatcccacaaacatacgtttctattgtcagttgaaagaccagctgtagctatcagagaggaggaactaacgaagacaaaatcattggctgttttgttatgacactgccaagtcaggtatggcttaggcatgcttccagtaactggacaacatttccagtttgtttgatacaaacttaaatatccatcagcatcaactattccaaacttatttccctgatagttaaatctcattcttgtaactcttgaattgccaccagatcgaaaacaggttatttgttgagaatggccccattcaaacattctgacacttccatcttgagctcctgtcagatagtaaggaagagttggatgagaagtcattcttctaacattattaatggctttcttaatcatcacagatgctcctctgccagtctgtgtactaccaagccatggcatgttgattggagtgccaggattgctatgtgtatatggagttgtaccttgaacagctgttaaatcatcacgagcatgtataaccaagaaatcttctgatcctttggtttccacttctatatcatcatctacccaagtgtagacctgtgtggccagaattccagaaacatccagttcttgaacatcatgactggaagcgattgctatgcagtttctatttgccttattaacagcaaacgcagtaatgatatcagattccttatgaataattcttgctttacctccaggatatcccaaatctgcttctatcttattgatgtttggctcctccatcatagaatttttgatggtttcactgttgtcctctaatgactcatttagacaccgtttctttgtgaatatatttttgataaaggtttcctgaatttcttcctgcttcaccaaatactgccaaagcctcttcacagacagtgccagatggtgtttggatttgaaaggagtgtttgtaggttccagtaaagctttgtggcgaagaattgcaggacctgcagacaaactctcttcggcggtatgacttgcgatataattttgaggtggcccaccatggatttcaagtcgtcggagaagaacttgttcccaacattgaagagtttttagaaccgcatgacaaagaggtgaactaactggaagctctgcaagatcatgacctgcgaagggataaaaagtcttcaaattgttgagcaccaattgcaccatcgccaaccgcatcaaggaccaactatatgaatttgaattagaatgttcctggagatggaaatctgatgctaaaacatcatcatcatcatcattgtcatcatcatcacttcccagactctcctctgaatcatattcggctctactttgagaagagggtagaaaaggcttagctatgaaatagtcccagatactgagctcaggtgggatgaacttttctttaaccgccagtgactcctggcttactggtgccgaggaaggggtcagtggggcagattctctgcaagacatttttgacggcctaaaacgtttgttctgtttttctccttcttcaactagtgaagaaactgcaagactgggagggctatgagaactgatggctgaaagagctttggaaaagcccacacattccatggagaataccactacctggtgggggctaggcatagcaaagtgccttccaggtaaagtttttgaatgtgtctgttctttgctaggaacatgtgcacctccaccaaacacagcagaccacattttctcatttagaggatgggccacaatccgaaatagctcattacttgaatgtgtggccaggccatggatgaagagactaagatacactgctgtgagaatctcacagagcaagactgtaagccctgactgggcttcctcgccagaagaattcaaaagtcgaattagacaagttattcctggccattgagctggtgacgtattgggagttaatgcttcatctaagcttcctgttttcaaagaaggtcgatgaggaagcagtactgtctgatataccattccagtaaactgattcgtctgaaatgaactgtagttatgactaccacaaaggcactgataaatacaagcagaaagtgaagctgctaaagtatgcattacatacactttattgctttggatatcagggtggggtggtgaatcaaagtttattatggcatggagaatatcatgtgtcagattactaaggtgcaataatggattggcaactactgttttggcattggctgtacaagcaaagaggagaggcactgaggtttgctctgacagagggctagaaaatagtggttctgatgtttcctgctgagattcttgcaaaagcaaaatcaattccattcttacagatgcaagacccccaccatgggatccatgaagtatgcagtaactaagaaacattctcaaaagtgactgatacttcaagagccactgtcttttttcctgaaaattttctctcagttgtttcacttttgtttggtgaggcaaatcttcagcatcctcatttaatccaaattcatcttcatttctgccaaatgcagactgtagttcttcagcatctgagcaaaagtcacaagtcctctgaagagctatcacctctttttcaagccagtggtatagttggtaacgcaattttccaccatctatttcatagccagtagataaagtacgaagttctactgtgagaatctttaaacatgctctaaattttaactgaactgcaattatatcttctgatggatttaaaaggtcattttcatctagtgtgctgaaagattctgtgtagttagaacttatgtcatccaactttttatctgtttttctctgtaaaggttttagttctttcattgaaatagggacatcctcattttcttcatcattatcactgtcccattttaactctaaagagtcatcctgaaacacaacacttggttggctccagtcaaaagaaagagtggagtttgattgcttctctgaggaaccctctgaagaagatccaaaaccatttatcagtgactgtgaccaatcaacagcagaagacttatcttcccttgcatccaactttaatggagaagaaggagaacagtctttactagtatccagaaaactagaagccctataaaaaggtcttgttttcttgatgactttaggcatctttgataatacttccaaagccaacattgggcagccagcttttaaatgagcactggcagtggtaaaaaataaacgtctttcacttaaattaattgttcctgccagtccactttttcctgttaggctcatatgtgtggaaaatgtatcagatgatccaaaatgacgtctcagcaaaagaggatgtgttcttagataattgtagaaattaaaaactgtaggattactggctgataaaacttgatcatcattctctctgataggttgctttattaatgtttccagagcaccactataatcttccaaaatccaatatgccatgctccgaagaaaaggatcatgatgcatatttatgttcaatgaacacagttcactgacaggagaatcgattcccaaaacttttttacgtaaaatagatttatatgctgcagatgtatcaaattcagactcatagagtcttgctattacaagagccaactgaatgtcattcaatttctcaagacatacctcaattgcatctctgaggcaaccagctaaaagaaaaaatgctgcagaatgttcaaatctttgtttgcctagcaaagaaaaagcattctttaaagctgctttacgccacctctcatcctcaaaattgtgtccaaaaaactgtgtcatcctggtgtttttttcagctctatataatccccaaatcacagctttctttttcattgcaaggtaaaaaatggcagcatctaaaggatcattctttctataaaaggctgctttagctactttttctatgcatttgcgtaagatgcgggtattccggacccaccaccccacacccatagctcttagttcagaccaagtgggatcatctttctgcatggctggcaacatgttcagcagttcttcttctgctactgagtgaaatgcccaagcaaaatgacttgtagacaggccttggtgaaggagttgagctcgataggctggaagggaagttgtaagaaaggtatggagtcgaacagccaaaagaaattttaacccacattcatcaagagtttctccaccttggcttctgtctcggctttctccaatatcagtgcttgtagttgcaattgtatctgctaaggccatcaaagacatctgctccatccggctgagtcctggtaaactagaatgaagtaagtggccagaaagaacctgagcatgctcaggtccaaagtaagtcggactgtactgtgaaaggtcaataactctaggctttgtattttcttcatctgtctctaacatatgagtatcagtcattagaagttgagtctgaaaaagctcatcataactttctttagataattggtttgatttacttaacgtactctcattactagatttctccaaagatgagtaacagctatcatcatctgctgcaagtaaggcatataaaggaagtggaggaacagaatctatttctgtgtaatctgtattttcagccttgttgaatgcctgggggtctctggtagtgcttccactagcactgattgtgagagacctaaggcggcgttcatgattagattcagcttcattcagagccacaacttccccagcaatgcacttaacaagatgggacaagatggccttggctctccgaactttaccaagatccatgagttccaaaagctgcaagggatgatactgaggtagagtcggggaaagtacatgagctgcttcaaaaagacctgaatcttccatatccactgaaggatcgaatgcagttttctttccacagattttctgtgcaagactggtcatggatcgagtcagagttttctttggaggatgtaacccagaactggagttactctgttttattaaacttgttatagatggagtgctcccactgtacgaatctgttataacaggttcttgtttagaagatggttgccattggcaatacacatgcatttcacagtccattcctaccacaaggatgccatcccggacccacgataaagaaacaggaaaaggtggggagccatctacagaagaaactaggtccacacttcgtaatagtacaaatttagaaaggggcacaactttggtactctcccagagaggaaatgccagggtttccttaccagtttggtcttgtaccttgccagccaggggtccatacataaaaagttttgatccaattcctacagtcaggatatgagaaccgtcttctctagacatccaatctaagtgaactaaatgctttgtgtttgatgtgatattctctttactagataaatacatgtcttgtttattataggccactaaattgctatcaacactaatgccagaatccaatactgtgcttaactcatctaaatgaattgtctgctcaaggacccaacatgaacctcctgttgactcacattcaaaaatacttacatgcatcacaaagtcctgggaagatctactattagatgcaggctgcttataagctactgctaaacgatttgtatgtgcacagctaacttctacaggcctaccaggtacagttatactactattgctctgaagtccatcttcaataagtaatggccattcttcccaaatgtatgcaagatcaatttttccattctttgacgtggcagattctccatctgttactctgcatctccagaatcttactttctcatctgaacatgaagttgccaataaataaggagcactgcatgcaggatatatagaagatgaactcagatgtcctgctgatggcttaatacttattatctcaactccttctggtaaatgcaattcttggctataaaccatttctgaaaacagagtcaacctgctggtactctggagatttgctctgcaagcctgatacttttgtgaaaaaggagataggatcttctctggagaagaagaataatgttcttctggctgccaaaccgcttcggataattttgtatctactttttcatctaatgagacaggaattgactttagatgtaaattccacatgtgtaacagtgaacggttgtcttgagtgcattctattacaattaggtagaacttctcagaaaatccattaggtgagctgcctgcattagataaaatgctgtctttgccaaggcttttcttctcaaggttattcaaaatgaagtcttcttcaaaaacatgaagcagttgggtttttctgccatgaagtttggtaatgggatctaatgcaataatgcatcctggcctggctgttgattgttgactgacgatgttaaagacttcaccaacatatttagaaatttcagggttagaaagctcagataaaagtttcttagcatcaataactgcttcatataatctcagatattgtccatcactggctacaaagcatgcactaggagagttgcagtatgcacccagacaataactgggtataagagtgggcagccatgccacattggaaaaggcagaaacatgaagagaattaatccgggcaagctcagaaactcctccagaaaaagacaatggcccaactgggtcaaccctccacagaataagctcactgtaaactgcactgggatcctgaaatgccacgtcaacagtgcttttattttgttgtgtcaaagagcattcttcaatatttagagcatcaaaaggttgctctgggttatcaacatctggtgtccttaatgcattatggtgtgatgttgtcagcaataatggtaatactgagtggcaagctaaatcattaagatgaaaacgatgaccacaatatctggatttgtgggaaatactgagaacagtagaaaaagcagattcctcggcaaaactgaccagccactgattcagagaaccatcagcatgttttgatatcatcataacattaggcgtaaaaatacttaattttaaactattagatgatttattgtgaccagaagaaataagcattgatgtggaacgggtgaggccagaaggtttttgtttcccctgctgaatagccaagtcaacattcttggtacaggcatacatcattatgcttttacagagagagtttgcatcacctgtggggaaagctactggaattctggaaacaaaggacacctgtacttgacgaaacataccaggctggtattcatccagccaatccacatgccaaactagcaaagaaccatccatgggatgaatactaaatagcatatctgcatttttactccattcagacagaagtacttcaatctgatgatcaatggcagctgacgataatgatgtaaaacttgagtttggtaccattttatcacagcctaattccttcttttcgggatttattttcagatcatcaacaccatcatcagtttcttcatcagattttacatctgcctgattagaatcttctacactggcctcagaagatggttgttcaaaactttttctaagttgctgtaaaaaaacttccatggacaaagtaaaatgcagttctttattgtttagccagtgtacaacaaaaggtccggtcttctcttcattttcatttagactcagagatgtaatagatggaagaagtggaatgtctgtggctgggttgatgctggctgcaatatgaaagtggcaaagtgcattggcatgcagtggagtgttcctgtgaacatgatgaggatcctgctgatgtggtagatatcccgtatgtgctacaagagcaagtgatctcctccgacctctacgaaaatgtctcagatttacttctaaagcattttgaactcgttctttactggaagcatttctcttgaagttatttgttaaattaattgattcagtccaatggctgcagtcacctccgtatagcaaacaatcatttggtaaaaatgtctctacccaaagacgacacacattatctttgcagcaagtcaacagtacattacatacagaagccctaggcatatatttgcttgttttacgccaggaaaatccatttactgctcgaggatgggccagatacacaaaagaaaagtcaatttctccttgggattgtttttctgaacttccatctggagaagtaacagctgtccgccagttttctacattataccaaaccttcaaaagacagtcatccttcccagcagtggcaaaaaattctccatctggtgaaaatttcattaaatgaacttgggaagcagttttgcaatgccaaatgcatttccaatctccaaagttaagatctgttttatttaaattttcatcttcagttggcttctccaagttagtattggaccagagttgcaaatagctggaaccagttaaaagacgactgccaaatttttcttttgttttggtaggttaactggttcaaaaatggagataacatttc

SEQ ID NO: 9969 - RNA, 11239 nt, Homo sapiens
  source 1..11239: mol_type = other RNA
cacacacacacacacacgtatacatacatacaacttgggttccggagggtaaactactgaaaaccttacatattgagccatctagctcatttatcactgacgtctcaatgacaattttaatgaagatgttcattatttttttcattcttactcaaatacctatcattaattaagagaagagtttgagatgtataaggctaataaaggaagtgagagtgtggtgaattaagtgatgagtattatgtacaattgcctttacaaaaaacgtatttttactgtggaagaaattcatgcagagatgcctgtggaaaagtatcaataagaaaacaaaacacctttaacactatgacatactgattataatatactatgatatgtattattacagcattacttacacattctactttaggcaatgtaatctacttctgaatgaccttgttaatttttaaggcatcagtgcatcaagggcaaagctccataaaataaatataaaaacaagaaagcattagctaatttgtggcatagagaatgatcactgtatattatatctgttggccacttccatataggtaataaattgtacatcttattgtaaaaatgttatagcataaatttcacatcatttttcaacacttcatttaaagggctaaactgatctggcagtattctcattttcattgttccatcagctccacaggagaaaatgtgatttgcaggccctgtctcaatttgcatcactccagttccaatatttctaaaaatggactgccgagcatgttcactgacaaaagtatggagaagaccaaaggtagagagactccaaatctttatattgccttcggcagatcctgtaacaaagtactcttcagttggatcaacagcaacggctttaacaggagaatcatggctctggaaaagctgcctctgttgtcgttgacaaaggtcaaatacatatgtaaaaccttttctgccacctgatattagtagctgatgttttggagcatatgctaaaactgtggctccactgtcatggcaggtaaatgcatggactaaactattggcaggtgctacaagagtatcccacaaacatacgtttctattgtcagttgaaagaccagctgtagctatcagagaggaggaactaacgaagacaaaatcattggctgttttgttatgacactgccaagtcaggtatggcttaggcatgcttccagtaactggacaacatttccagtttgtttgatacaaacttaaatatccatcagcatcaactattccaaacttatttccctgatagttaaatctcattcttgtaactcttgaattgccaccagatcgaaaacaggttatttgttgagaatggccccattcaaacattctgacacttccatcttgagctcctgtcagatagtaaggaagagttggatgagaagtcattcttctaacattattaatggctttcttaatcatcacagatgctcctctgccagtctgtgtactaccaagccatggcatgttgattggagtgccaggattgctatgtgtatatggagttgtaccttgaacagctgttaaatcatcacgagcatgtataaccaagaaatcttctgatcctttggtttccacttctatatcatcatctacccaagtgtagacctgtgtggccagaattccagaaacatccagttcttgaacatcatgactggaagcgattgctatgcagtttctatttgccttattaacagcaaacgcagtaatgatatcagattccttatgaataattcttgctttacctccaggatatcccaaatctgcttctatcttattgatgtttggctcctccatcatagaatttttgatggtttcactgttgtcctctaatgactcatttagacaccgtttctttgtgaatatatttttgataaaggtttcctgaatttcttcctgcttcaccaaatactgccaaagcctcttcacagacagtgccagatggtgtttggatttgaaaggagtgtttgtaggttccagtaaagctttgtggcgaagaattgcaggacctgcagacaaactctcttcggcggtatgacttgcgatataattttgaggtggcccaccatggatttcaagtcgtcggagaagaacttgttcccaacattgaagagtttttagaaccgcatgacaaagaggtgaactaactggaagctctgcaagatcatgacctgcgaagggataaaaagtcttcaaattgttgagcaccaattgcaccatcgccaaccgcatcaaggaccaactatatgaatttgaattagaatgttcctggagatggaaatctgatgctaaaacatcatcatcatcatcattgtcatcatcatcacttcccagactctcctctgaatcatattcggctctactttgagaagagggtagaaaaggcttagctatgaaatagtcccagatactgagctcaggtgggatgaacttttctttaaccgccagtgactcctggcttactggtgccgaggaaggggtcagtggggcagattctctgcaagacatttttgacggcctaaaacgtttgttctgtttttctccttcttcaactagtgaagaaactgcaagactgggagggctatgagaactgatggctgaaagagctttggaaaagcccacacattccatggagaataccactacctggtgggggctaggcatagcaaagtgccttccaggtaaagtttttgaatgtgtctgttctttgctaggaacatgtgcacctccaccaaacacagcagaccacattttctcatttagaggatgggccacaatccgaaatagctcattacttgaatgtgtggccaggccatggatgaagagactaagatacactgctgtgagaatctcacagagcaagactgtaagccctgactgggcttcctcgccagaagaattcaaaagtcgaattagacaagttattcctggccattgagctggtgacgtattgggagttaatgcttcatctaagcttcctgttttcaaagaaggtcgatgaggaagcagtactgtctgatataccattccagtaaactgattcgtctgaaatgaactgtagttatgactaccacaaaggcactgataaatacaagcagaaagtgaagctgctaaagtatgcattacatacactttattgctttggatatcagggtggggtggtgaatcaaagtttattatggcatggagaatatcatgtgtcagattactaaggtgcaataatggattggcaactactgttttggcattggctgtacaagcaaagaggagaggcactgaggtttgctctgacagagggctagaaaatagtggttctgatgtttcctgctgagattcttgcaaaagcaaaatcaattccattcttacagatgcaagacccccaccatgggatccatgaagtatgcagtaactaagaaacattctcaaaagtgactgatacttcaagagccactgtcttttttcctgaaaattttctctcagttgtttcacttttgtttggtgaggcaaatcttcagcatcctcatttaatccaaattcatcttcatttctgccaaatgcagactgtagttcttcagcatctgagcaaaagtcacaagtcctctgaagagctatcacctctttttcaagccagtggtatagttggtaacgcaattttccaccatctatttcatagccagtagataaagtacgaagttctactgtgagaatctttaaacatgctctaaattttaactgaactgcaattatatcttctgatggatttaaaaggtcattttcatctagtgtgctgaaagattctgtgtagttagaacttatgtcatccaactttttatctgtttttctctgtaaaggttttagttctttcattgaaatagggacatcctcattttcttcatcattatcactgtcccattttaactctaaagagtcatcctgaaacacaacacttggttggctccagtcaaaagaaagagtggagtttgattgcttctctgaggaaccctctgaagaagatccaaaaccatttatcagtgactgtgaccaatcaacagcagaagacttatcttcccttgcatccaactttaatggagaagaaggagaacagtctttactagtatccagaaaactagaagccctataaaaaggtcttgttttcttgatgactttaggcatctttgataatacttccaaagccaacattgggcagccagcttttaaatgagcactggcagtggtaaaaaataaacgtctttcacttaaattaattgttcctgccagtccactttttcctgttaggctcatatgtgtggaaaatgtatcagatgatccaaaatgacgtctcagcaaaagaggatgtgttcttagataattgtagaaattaaaaactgtaggattactggctgataaaacttgatcatcattctctctgataggttgctttattaatgtttccagagcaccactataatcttccaaaatccaatatgccatgctccgaagaaaaggatcatgatgcatatttatgttcaatgaacacagttcactgacaggagaatcgattcccaaaacttttttacgtaaaatagatttatatgctgcagatgtatcaaattcagactcatagagtcttgctattacaagagccaactgaatgtcattcaatttctcaagacatacctcaattgcatctctgaggcaaccagctaaaagaaaaaatgctgcagaatgttcaaatctttgtttgcctagcaaagaaaaagcattctttaaagctgctttacgccacctctcatcctcaaaattgtgtccaaaaaactgtgtcatcctggtgtttttttcagctctatataatccccaaatcacagctttctttttcattgcaaggtaaaaaatggcagcatctaaaggatcattctttctataaaaggctgctttagctactttttctatgcatttgcgtaagatgcgggtattccggacccaccaccccacacccatagctcttagttcagaccaagtgggatcatctttctgcatggctggcaacatgttcagcagttcttcttctgctactgagtgaaatgcccaagcaaaatgacttgtagacaggccttggtgaaggagttgagctcgataggctggaagggaagttgtaagaaaggtatggagtcgaacagccaaaagaaattttaacccacattcatcaagagtttctccaccttggcttctgtctcggctttctccaatatcagtgcttgtagttgcaattgtatctgctaaggccatcaaagacatctgctccatccggctgagtcctggtaaactagaatgaagtaagtggccagaaagaacctgagcatgctcaggtccaaagtaagtcggactgtactgtgaaaggtcaataactctaggctttgtattttcttcatctgtctctaacatatgagtatcagtcattagaagttgagtctgaaaaagctcatcataactttctttagataattggtttgatttacttaacgtactctcattactagatttctccaaagatgagtaacagctatcatcatctgctgcaagtaaggcatataaaggaagtggaggaacagaatctatttctgtgtaatctgtattttcagccttgttgaatgcctgggggtctctggtagtgcttccactagcactgattgtgagagacctaaggcggcgttcatgattagattcagcttcattcagagccacaacttccccagcaatgcacttaacaagatgggacaagatggccttggctctccgaactttaccaagatccatgagttccaaaagctgcaagggatgatactgaggtagagtcggggaaagtacatgagctgcttcaaaaagacctgaatcttccatatccactgaaggatcgaatgcagttttctttccacagattttctgtgcaagactggtcatggatcgagtcagagttttctttggaggatgtaacccagaactggagttactctgttttattaaacttgttatagatggagtgctcccactgtacgaatctgttataacaggttcttgtttagaagatggttgccattggcaatacacatgcatttcacagtccattcctaccacaaggatgccatcccggacccacgataaagaaacaggaaaaggtggggagccatctacagaagaaactaggtccacacttcgtaatagtacaaatttagaaaggggcacaactttggtactctcccagagaggaaatgccagggtttccttaccagtttggtcttgtaccttgccagccaggggtccatacataaaaagttttgatccaattcctacagtcaggatatgagaaccgtcttctctagacatccaatctaagtgaactaaatgctttgtgtttgatgtgatattctctttactagataaatacatgtcttgtttattataggccactaaattgctatcaacactaatgccagaatccaatactgtgcttaactcatctaaatgaattgtctgctcaaggacccaacatgaacctcctgttgactcacattcaaaaatacttacatgcatcacaaagtcctgggaagatctactattagatgcaggctgcttataagctactgctaaacgatttgtatgtgcacagctaacttctacaggcctaccaggtacagttatactactattgctctgaagtccatcttcaataagtaatggccattcttcccaaatgtatgcaagatcaatttttccattctttgacgtggcagattctccatctgttactctgcatctccagaatcttactttctcatctgaacatgaagttgccaataaataaggagcactgcatgcaggatatatagaagatgaactcagatgtcctgctgatggcttaatacttattatctcaactccttctggtaaatgcaattcttggctataaaccatttctgaaaacagagtcaacctgctggtactctggagatttgctctgcaagcctgatacttttgtgaaaaaggagataggatcttctctggagaagaagaataatgttcttctggctgccaaaccgcttcggataattttgtatctactttttcatctaatgagacaggaattgactttagatgtaaattccacatgtgtaacagtgaacggttgtcttgagtgcattctattacaattaggtagaacttctcagaaaatccattaggtgagctgcctgcattagataaaatgctgtctttgccaaggcttttcttctcaaggttattcaaaatgaagtcttcttcaaaaacatgaagcagttgggtttttctgccatgaagtttggtaatgggatctaatgcaataatgcatcctggcctggctgttgattgttgactgacgatgttaaagacttcaccaacatatttagaaatttcagggttagaaagctcagataaaagtttcttagcatcaataactgcttcatataatctcagatattgtccatcactggctacaaagcatgcactaggagagttgcagtatgcacccagacaataactgggtataagagtgggcagccatgccacattggaaaaggcagaaacatgaagagaattaatccgggcaagctcagaaactcctccagaaaaagacaatggcccaactgggtcaaccctccacagaataagctcactgtaaactgcactgggatcctgaaatgccacgtcaacagtgcttttattttgttgtgtcaaagagcattcttcaatatttagagcatcaaaaggttgctctgggttatcaacatctggtgtccttaatgcattatggtgtgatgttgtcagcaataatggtaatactgagtggcaagctaaatcattaagatgaaaacgatgaccacaatatctggatttgtgggaaatactgagaacagtagaaaaagcagattcctcggcaaaactgaccagccactgattcagagaaccatcagcatgttttgatatcatcataacattaggcgtaaaaatacttaattttaaactattagatgatttattgtgaccagaagaaataagcattgatgtggaacgggtgaggccagaaggtttttgtttcccctgctgaatagccaagtcaacattcttggtacaggcatacatcattatgcttttacagagagagtttgcatcacctgtggggaaagctactggaattctggaaacaaaggacacctgtacttgacgaaacataccaggctggtattcatccagccaatccacatgccaaactagcaaagaaccatccatgggatgaatactaaatagcatatctgcatttttactccattcagacagaagtacttcaatctgatgatcaatggcagctgacgataatgatgtaaaacttgagtttggtaccattttatcacagcctaattccttcttttcgggatttattttcagatcatcaacaccatcatcagtttcttcatcagattttacatctgcctgattagaatcttctacactggcctcagaagatggttgttcaaaactttttctaagttgctgtaaaaaaacttccatggacaaagtaaaatgcagttctttattgtttagccagtgtacaacaaaaggtccggtcttctcttcattttcatttagactcagagatgtaatagatggaagaagtggaatgtctgtggctgggttgatgctggctgcaatatgaaagtggcaaagtgcattggcatgcagtggagtgttcctgtgaacatgatgaggatcctgctgatgtggtagatatcccgtatgtgctacaagagcaagtgatctcctccgacctctacgaaaatgtctcagatttacttctaaagcattttgaactcgttctttactggaagcatttctcttgaagttatttgttaaattaattgattcagtccaatggctgcagtcacctccgtatagcaaacaatcatttggtaaaaatgtctctacccaaagacgacacacattatctttgcagcaagtcaacagtacattacatacagaagccctaggcatatatttgcttgttttacgccaggaaaatccatttactgctcgaggatgggccagatacacaaaagaaaagtcaatttctccttgggattgtttttctgaacttccatctggagaagtaacagctgtccgccagttttctacattataccaaaccttcaaaagacagtcatccttcccagcagtggcaaaaaattctccatctggtgaaaatttcattaaatgaacttgggaagcagttttgcaatgccaaatgcatttccaatctccaaagttaagatctgttttatttaaattttcatcttcagttggcttctccaagttagtattggaccagagttgcaaatagctggaaccagttaaaagacgactgcctgtgggatcccaggttatattgtgtgctattgattccagaaaaaattggccacttttctgccactgactatataattccaaatttttcttttgttttggtaggttaactggttcaaaaatggagataacatttccataagacgctgcaatcaacatgatgaaaccccgtttctactaaaaatacaaaaattagccgggtatgatggcgagcacctgtaattccagctatttgggaggctgaggcaggagaattgcttgaacccggaagccagaggctgcagtgagctgagattgcaccactgcactccagcctgggcaacaaagcgagactccatctgaaaaacaaaaaacaaaacaaacaaacaaaaacaaacaaaaaacaaaaaaaaaacccaaagatttccagcattccataataaagatcatttttgttgtacagcgagaagtcataagaggcctcaacaaaagatagaggacacctgtaactatattaaagggaaggaataccatgtaacaaaaagaacagtagtccaacaaatatgtaaagattcagaaaacagaaactcgttttataattaatatctttaagtcccagatggcaacttttaatcctagaaagtttacctcaaatgaagattagatttaaaaacaaatgattgggtccatggactcttaatatgaccattttgattccttacacaaaatgttctagtggaatcatatgagtgtatttgcgaagttcagtccagtctagctacaactatatataggccttaccacctatgcctatatggagttattttaagctatatattatgctgccttgcctagtagtatgactttctcattctggtactacaggaactgtatttaacctgatctagaagaattttatactttgttacttttgtttatgttgttgctattttactttcaaggttacctttctacttttcatatgcaaatagaagtccagataaagtttttcacttttcttatgggcttagaatattataaactctcaaagagtttttcatttccacaaaaagttacacagcccttgttacatagaagttacaaggagataactacctgttcacagacaaaaaaaaaaaaatattctaaatcatttcctttagtttatttgtaaatattgaagattcattgttactcctttcccccagtccaatcaccttttaaatacgtaagctttagactcattctatatcagtaagtattgtatttctttctcagagaagatgatgctataatttaaaattatataagaagagaatttctggcactctatagaatgcatcttagacagccaaaaattcttctagctacactatctttgaaacaaagccaagtctctaattcaataggaaatacacacttcagagattatcctgacaaaaaccatattccaaacaaatttgtatattagaagaagattacaaaccttgccttgttgcattgaacagtctacacatcccacttgaatatttccatgtttagctcctgggattatctgtaatctttcaaaatcgcttcccagtattacaatgtcacatccagatgcataagccggccaggaaggccgcgctgtccacacacttcctctggacctcgggcagccgctcctgacccagcccgagtggcgcaagcagtacgcgctcgcactccccgcctgacctgtcccttcccggctccggtgcccgccacccccacagtcctc

SEQ ID NO: 9970 - RNA, 9927 nt, Homo sapiens
  source 1..9927: mol_type = other RNA
cacacacacacacacacgtatacatacatacaacttgggttccggagggtaaactactgaaaaccttacatattgagccatctagctcatttatcactgacgtctcaatgacaattttaatgaagatgttcattatttttttcattcttactcaaatacctatcattaattaagagaagagtttgagatgtataaggctaataaaggaagtgagagtgtggtgaattaagtgatgagtattatgtacaattgcctttacaaaaaacgtatttttactgtggaagaaattcatgcagagatgcctgtggaaaagtatcaataagaaaacaaaacacctttaacactatgacatactgattataatatactatgatatgtattattacagcattacttacacattctactttaggcaatgtaatctacttctgaatgaccttgttaatttttaaggcatcagtgcatcaagggcaaagctccataaaataaatataaaaacaagaaagcattagctaatttgtggcatagagaatgatcactgtatattatatctgttggccacttccatataggtaataaattgtacatcttattgtaaaaatgttatagcataaatttcacatcatttttcaacacttcatttaaagggctaaactgatctggcagtattctcattttcattgttccatcagctccacaggagaaaatgtgatttgcaggccctgtctcaatttgcatcactccagttccaatatttctaaaaatggactgccgagcatgttcactgacaaaagtatggagaagaccaaaggtagagagactccaaatctttatattgccttcggcagatcctgtaacaaagtactcttcagttggatcaacagcaacggctttaacaggagaatcatggctctggaaaagctgcctctgttgtcgttgacaaaggtcaaatacatatgtaaaaccttttctgccacctgatattagtagctgatgttttggagcatatgctaaaactgtggctccactgtcatggcaggtaaatgcatggactaaactattggcaggtgctacaagagtatcccacaaacatacgtttctattgtcagttgaaagaccagctgtagctatcagagaggaggaactaacgaagacaaaatcattggctgttttgttatgacactgccaagtcaggtatggcttaggcatgcttccagtaactggacaacatttccagtttgtttgatacaaacttaaatatccatcagcatcaactattccaaacttatttccctgatagttaaatctcattcttgtaactcttgaattgccaccagatcgaaaacaggttatttgttgagaatggccccattcaaacattctgacacttccatcttgagctcctgtcagatagtaaggaagagttggatgagaagtcattcttctaacattattaatggctttcttaatcatcacagatgctcctctgccagtctgtgtactaccaagccatggcatgttgattggagtgccaggattgctatgtgtatatggagttgtaccttgaacagctgttaaatcatcacgagcatgtataaccaagaaatcttctgatcctttggtttccacttctatatcatcatctacccaagtgtagacctgtgtggccagaattccagaaacatccagttcttgaacatcatgactggaagcgattgctatgcagtttctatttgccttattaacagcaaacgcagtaatgatatcagattccttatgaataattcttgctttacctccaggatatcccaaatctgcttctatcttattgatgtttggctcctccatcatagaatttttgatggtttcactgttgtcctctaatgactcatttagacaccgtttctttgtgaatatatttttgataaaggtttcctgaatttcttcctgcttcaccaaatactgccaaagcctcttcacagacagtgccagatggtgtttggatttgaaaggagtgtttgtaggttccagtaaagctttgtggcgaagaattgcaggacctgcagacaaactctcttcggcggtatgacttgcgatataattttgaggtggcccaccatggatttcaagtcgtcggagaagaacttgttcccaacattgaagagtttttagaaccgcatgacaaagaggtgaactaactggaagctctgcaagatcatgacctgcgaagggataaaaagtcttcaaattgttgagcaccaattgcaccatcgccaaccgcatcaaggaccaactatatgaatttgaattagaatgttcctggagatggaaatctgatgctaaaacatcatcatcatcatcattgtcatcatcatcacttcccagactctcctctgaatcatattcggctctactttgagaagagggtagaaaaggcttagctatgaaatagtcccagatactgagctcaggtgggatgaacttttctttaaccgccagtgactcctggcttactggtgccgaggaaggggtcagtggggcagattctctgcaagacatttttgacggcctaaaacgtttgttctgtttttctccttcttcaactagtgaagaaactgcaagactgggagggctatgagaactgatggctgaaagagctttggaaaagcccacacattccatggagaataccactacctggtgggggctaggcatagcaaagtgccttccaggtaaagtttttgaatgtgtctgttctttgctaggaacatgtgcacctccaccaaacacagcagaccacattttctcatttagaggatgggccacaatccgaaatagctcattacttgaatgtgtggccaggccatggatgaagagactaagatacactgctgtgagaatctcacagagcaagactgtaagccctgactgggcttcctcgccagaagaattcaaaagtcgaattagacaagttattcctggccattgagctggtgacgtattgggagttaatgcttcatctaagcttcctgttttcaaagaaggtcgatgaggaagcagtactgtctgatataccattccagtaaactgattcgtctgaaatgaactgtagttatgactaccacaaaggcactgataaatacaagcagaaagtgaagctgctaaagtatgcattacatacactttattgctttggatatcagggtggggtggtgaatcaaagtttattatggcatggagaatatcatgtgtcagattactaaggtgcaataatggattggcaactactgttttggcattggctgtacaagcaaagaggagaggcactgaggtttgctctgacagagggctagaaaatagtggttctgatgtttcctgctgagattcttgcaaaagcaaaatcaattccattcttacagatgcaagacccccaccatgggatccatgaagtatgcagtaactaagaaacattctcaaaagtgactgatacttcaagagccactgtcttttttcctgaaaattttctctcagttgtttcacttttgtttggtgaggcaaatcttcagcatcctcatttaatccaaattcatcttcatttctgccaaatgcagactgtagttcttcagcatctgagcaaaagtcacaagtcctctgaagagctatcacctctttttcaagccagtggtatagttggtaacgcaattttccaccatctatttcatagccagtagataaagtacgaagttctactgtgagaatctttaaacatgctctaaattttaactgaactgcaattatatcttctgatggatttaaaaggtcattttcatctagtgtgctgaaagattctgtgtagttagaacttatgtcatccaactttttatctgtttttctctgtaaaggttttagttctttcattgaaatagggacatcctcattttcttcatcattatcactgtcccattttaactctaaagagtcatcctgaaacacaacacttggttggctccagtcaaaagaaagagtggagtttgattgcttctctgaggaaccctctgaagaagatccaaaaccatttatcagtgactgtgaccaatcaacagcagaagacttatcttcccttgcatccaactttaatggagaagaaggagaacagtctttactagtatccagaaaactagaagccctataaaaaggtcttgttttcttgatgactttaggcatctttgataatacttccaaagccaacattgggcagccagcttttaaatgagcactggcagtggtaaaaaataaacgtctttcacttaaattaattgttcctgccagtccactttttcctgttaggctcatatgtgtggaaaatgtatcagatgatccaaaatgacgtctcagcaaaagaggatgtgttcttagataattgtagaaattaaaaactgtaggattactggctgataaaacttgatcatcattctctctgataggttgctttattaatgtttccagagcaccactataatcttccaaaatccaatatgccatgctccgaagaaaaggatcatgatgcatatttatgttcaatgaacacagttcactgacaggagaatcgattcccaaaacttttttacgtaaaatagatttatatgctgcagatgtatcaaattcagactcatagagtcttgctattacaagagccaactgaatgtcattcaatttctcaagacatacctcaattgcatctctgaggcaaccagctaaaagaaaaaatgctgcagaatgttcaaatctttgtttgcctagcaaagaaaaagcattctttaaagctgctttacgccacctctcatcctcaaaattgtgtccaaaaaactgtgtcatcctggtgtttttttcagctctatataatccccaaatcacagctttctttttcattgcaaggtaaaaaatggcagcatctaaaggatcattctttctataaaaggctgctttagctactttttctatgcatttgcgtaagatgcgggtattccggacccaccaccccacacccatagctcttagttcagaccaagtgggatcatctttctgcatggctggcaacatgttcagcagttcttcttctgctactgagtgaaatgcccaagcaaaatgacttgtagacaggccttggtgaaggagttgagctcgataggctggaagggaagttgtaagaaaggtatggagtcgaacagccaaaagaaattttaacccacattcatcaagagtttctccaccttggcttctgtctcggctttctccaatatcagtgcttgtagttgcaattgtatctgctaaggccatcaaagacatctgctccatccggctgagtcctggtaaactagaatgaagtaagtggccagaaagaacctgagcatgctcaggtccaaagtaagtcggactgtactgtgaaaggtcaataactctaggctttgtattttcttcatctgtctctaacatatgagtatcagtcattagaagttgagtctgaaaaagctcatcataactttctttagataattggtttgatttacttaacgtactctcattactagatttctccaaagatgagtaacagctatcatcatctgctgcaagtaaggcatataaaggaagtggaggaacagaatctatttctgtgtaatctgtattttcagccttgttgaatgcctgggggtctctggtagtgcttccactagcactgattgtgagagacctaaggcggcgttcatgattagattcagcttcattcagagccacaacttccccagcaatgcacttaacaagatgggacaagatggccttggctctccgaactttaccaagatccatgagttccaaaagctgcaagggatgatactgaggtagagtcggggaaagtacatgagctgcttcaaaaagacctgaatcttccatatccactgaaggatcgaatgcagttttctttccacagattttctgtgcaagactggtcatggatcgagtcagagttttctttggaggatgtaacccagaactggagttactctgttttattaaacttgttatagatggagtgctcccactgtacgaatctgttataacaggttcttgtttagaagatggttgccattggcaatacacatgcatttcacagtccattcctaccacaaggatgccatcccggacccacgataaagaaacaggaaaaggtggggagccatctacagaagaaactaggtccacacttcgtaatagtacaaatttagaaaggggcacaactttggtactctcccagagaggaaatgccagggtttccttaccagtttggtcttgtaccttgccagccaggggtccatacataaaaagttttgatccaattcctacagtcaggatatgagaaccgtcttctctagacatccaatctaagtgaactaaatgctttgtgtttgatgtgatattctctttactagataaatacatgtcttgtttattataggccactaaattgctatcaacactaatgccagaatccaatactgtgcttaactcatctaaatgaattgtctgctcaaggacccaacatgaacctcctgttgactcacattcaaaaatacttacatgcatcacaaagtcctgggaagatctactattagatgcaggctgcttataagctactgctaaacgatttgtatgtgcacagctaacttctacaggcctaccaggtacagttatactactattgctctgaagtccatcttcaataagtaatggccattcttcccaaatgtatgcaagatcaatttttccattctttgacgtggcagattctccatctgttactctgcatctccagaatcttactttctcatctgaacatgaagttgccaataaataaggagcactgcatgcaggatatatagaagatgaactcagatgtcctgctgatggcttaatacttattatctcaactccttctggtaaatgcaattcttggctataaaccatttctgaaaacagagtcaacctgctggtactctggagatttgctctgcaagcctgatacttttgtgaaaaaggagataggatcttctctggagaagaagaataatgttcttctggctgccaaaccgcttcggataattttgtatctactttttcatctaatgagacaggaattgactttagatgtaaattccacatgtgtaacagtgaacggttgtcttgagtgcattctattacaattaggtagaacttctcagaaaatccattaggtgagctgcctgcattagataaaatgctgtctttgccaaggcttttcttctcaaggttattcaaaatgaagtcttcttcaaaaacatgaagcagttgggtttttctgccatgaagtttggtaatgggatctaatgcaataatgcatcctggcctggctgttgattgttgactgacgatgttaaagacttcaccaacatatttagaaatttcagggttagaaagctcagataaaagtttcttagcatcaataactgcttcatataatctcagatattgtccatcactggctacaaagcatgcactaggagagttgcagtatgcacccagacaataactgggtataagagtgggcagccatgccacattggaaaaggcagaaacatgaagagaattaatccgggcaagctcagaaactcctccagaaaaagacaatggcccaactgggtcaaccctccacagaataagctcactgtaaactgcactgggatcctgaaatgccacgtcaacagtgcttttattttgttgtgtcaaagagcattcttcaatatttagagcatcaaaaggttgctctgggttatcaacatctggtgtccttaatgcattatggtgtgatgttgtcagcaataatggtaatactgagtggcaagctaaatcattaagatgaaaacgatgaccacaatatctggatttgtgggaaatactgagaacagtagaaaaagcagattcctcggcaaaactgaccagccactgattcagagaaccatcagcatgttttgatatcatcataacattaggcgtaaaaatacttaattttaaactattagatgatttattgtgaccagaagaaataagcattgatgtggaacgggtgaggccagaaggtttttgtttcccctgctgaatagccaagtcaacattcttggtacaggcatacatcattatgcttttacagagagagtttgcatcacctgtggggaaagctactggaattctggaaacaaaggacacctgtacttgacgaaacataccaggctggtattcatccagccaatccacatgccaaactagcaaagaaccatccatgggatgaatactaaatagcatatctgcatttttactccattcagacagaagtacttcaatctgatgatcaatggcagctgacgataatgatgtaaaacttgagtttggtaccattttatcacagcctaattccttcttttcgggatttattttcagatcatcaacaccatcatcagtttcttcatcagattttacatctgcctgattagaatcttctacactggcctcagaagatggttgttcaaaactttttctaagttgctgtaaaaaaacttccatggacaaagtaaaatgcagttctttattgtttagccagtgtacaacaaaaggtccggtcttctcttcattttcatttagactcagagatgtaatagatggaagaagtggaatgtctgtggctgggttgatgctggctgcaatatgaaagtggcaaagtgcattggcatgcagtggagtgttcctgtgaacatgatgaggatcctgctgatgtggtagatatcccgtatgtgctacaagagcaagtgatctcctccgacctctacgaaaatgtctcagatttacttctaaagcattttgaactcgttctttactggaagcatttctcttgaagttatttgttaaattaattgattcagtccaatggctgcagtcacctccgtatagcaaacaatcatttggtaaaaatgtctctacccaaagacgacacacattatctttgcagcaagtcaacagtacattacatacagaagccctaggcatatatttgcttgttttacgccaggaaaatccatttactgctcgaggatgggccagatacacaaaagaaaagtcaatttctccttgggattgtttttctgaacttccatctggagaagtaacagctgtccgccagttttctacattataccaaaccttcaaaagacagtcatccttcccagcagtggcaaaaaattctccatctggtgaaaatttcattaaatgaacttgggaagcagttttgcaatgccaaatgcatttccaatctccaaagttaagatctgttttatttaaattttcatcttcagttggcttctccaagttagtattggaccagagttgcaaatagctggaaccagttaaaagacgactgcctgtgggatcccaggttatattgtgtgctattgattccagaaaaaattggccacttttctgccactgactatataattccaaatttttcttttgttttggtaggttaactggttcaaaaatggagataacatttccataagacgctgcaatcttgccttgttgcattgaacagtctacacatcccacttgaatatttccatgtttagctcctgggattatctgtaatctttcaaaatcgcttcccagtattacaatgtcacatccagatgcataagccggccaggaaggccgcgctgtccacacacttcctctggacctcgggcagccgctcctgacccagcccgagtggcgcaagcagtacgcgctcgcactccccgcctgacctgtcccttcccggctccggtgcccgccacccccacagtcctc

SEQ ID NO: 9971 - RNA, 10045 nt, Homo sapiens
  source 1..10045: mol_type = other RNA
cacacacacacacacacgtatacatacatacaacttgggttccggagggtaaactactgaaaaccttacatattgagccatctagctcatttatcactgacgtctcaatgacaattttaatgaagatgttcattatttttttcattcttactcaaatacctatcattaattaagagaagagtttgagatgtataaggctaataaaggaagtgagagtgtggtgaattaagtgatgagtattatgtacaattgcctttacaaaaaacgtatttttactgtggaagaaattcatgcagagatgcctgtggaaaagtatcaataagaaaacaaaacacctttaacactatgacatactgattataatatactatgatatgtattattacagcattacttacacattctactttaggcaatgtaatctacttctgaatgaccttgttaatttttaaggcatcagtgcatcaagggcaaagctccataaaataaatataaaaacaagaaagcattagctaatttgtggcatagagaatgatcactgtatattatatctgttggccacttccatataggtaataaattgtacatcttattgtaaaaatgttatagcataaatttcacatcatttttcaacacttcatttaaagggctaaactgatctggcagtattctcattttcattgttccatcagctccacaggagaaaatgtgatttgcaggccctgtctcaatttgcatcactccagttccaatatttctaaaaatggactgccgagcatgttcactgacaaaagtatggagaagaccaaaggtagagagactccaaatctttatattgccttcggcagatcctgtaacaaagtactcttcagttggatcaacagcaacggctttaacaggagaatcatggctctggaaaagctgcctctgttgtcgttgacaaaggtcaaatacatatgtaaaaccttttctgccacctgatattagtagctgatgttttggagcatatgctaaaactgtggctccactgtcatggcaggtaaatgcatggactaaactattggcaggtgctacaagagtatcccacaaacatacgtttctattgtcagttgaaagaccagctgtagctatcagagaggaggaactaacgaagacaaaatcattggctgttttgttatgacactgccaagtcaggtatggcttaggcatgcttccagtaactggacaacatttccagtttgtttgatacaaacttaaatatccatcagcatcaactattccaaacttatttccctgatagttaaatctcattcttgtaactcttgaattgccaccagatcgaaaacaggttatttgttgagaatggccccattcaaacattctgacacttccatcttgagctcctgtcagatagtaaggaagagttggatgagaagtcattcttctaacattattaatggctttcttaatcatcacagatgctcctctgccagtctgtgtactaccaagccatggcatgttgattggagtgccaggattgctatgtgtatatggagttgtaccttgaacagctgttaaatcatcacgagcatgtataaccaagaaatcttctgatcctttggtttccacttctatatcatcatctacccaagtgtagacctgtgtggccagaattccagaaacatccagttcttgaacatcatgactggaagcgattgctatgcagtttctatttgccttattaacagcaaacgcagtaatgatatcagattccttatgaataattcttgctttacctccaggatatcccaaatctgcttctatcttattgatgtttggctcctccatcatagaatttttgatggtttcactgttgtcctctaatgactcatttagacaccgtttctttgtgaatatatttttgataaaggtttcctgaatttcttcctgcttcaccaaatactgccaaagcctcttcacagacagtgccagatggtgtttggatttgaaaggagtgtttgtaggttccagtaaagctttgtggcgaagaattgcaggacctgcagacaaactctcttcggcggtatgacttgcgatataattttgaggtggcccaccatggatttcaagtcgtcggagaagaacttgttcccaacattgaagagtttttagaaccgcatgacaaagaggtgaactaactggaagctctgcaagatcatgacctgcgaagggataaaaagtcttcaaattgttgagcaccaattgcaccatcgccaaccgcatcaaggaccaactatatgaatttgaattagaatgttcctggagatggaaatctgatgctaaaacatcatcatcatcatcattgtcatcatcatcacttcccagactctcctctgaatcatattcggctctactttgagaagagggtagaaaaggcttagctatgaaatagtcccagatactgagctcaggtgggatgaacttttctttaaccgccagtgactcctggcttactggtgccgaggaaggggtcagtggggcagattctctgcaagacatttttgacggcctaaaacgtttgttctgtttttctccttcttcaactagtgaagaaactgcaagactgggagggctatgagaactgatggctgaaagagctttggaaaagcccacacattccatggagaataccactacctggtgggggctaggcatagcaaagtgccttccaggtaaagtttttgaatgtgtctgttctttgctaggaacatgtgcacctccaccaaacacagcagaccacattttctcatttagaggatgggccacaatccgaaatagctcattacttgaatgtgtggccaggccatggatgaagagactaagatacactgctgtgagaatctcacagagcaagactgtaagccctgactgggcttcctcgccagaagaattcaaaagtcgaattagacaagttattcctggccattgagctggtgacgtattgggagttaatgcttcatctaagcttcctgttttcaaagaaggtcgatgaggaagcagtactgtctgatataccattccagtaaactgattcgtctgaaatgaactgtagttatgactaccacaaaggcactgataaatacaagcagaaagtgaagctgctaaagtatgcattacatacactttattgctttggatatcagggtggggtggtgaatcaaagtttattatggcatggagaatatcatgtgtcagattactaaggtgcaataatggattggcaactactgttttggcattggctgtacaagcaaagaggagaggcactgaggtttgctctgacagagggctagaaaatagtggttctgatgtttcctgctgagattcttgcaaaagcaaaatcaattccattcttacagatgcaagacccccaccatgggatccatgaagtatgcagtaactaagaaacattctcaaaagtgactgatacttcaagagccactgtcttttttcctgaaaattttctctcagttgtttcacttttgtttggtgaggcaaatcttcagcatcctcatttaatccaaattcatcttcatttctgccaaatgcagactgtagttcttcagcatctgagcaaaagtcacaagtcctctgaagagctatcacctctttttcaagccagtggtatagttggtaacgcaattttccaccatctatttcatagccagtagataaagtacgaagttctactgtgagaatctttaaacatgctctaaattttaactgaactgcaattatatcttctgatggatttaaaaggtcattttcatctagtgtgctgaaagattctgtgtagttagaacttatgtcatccaactttttatctgtttttctctgtaaaggttttagttctttcattgaaatagggacatcctcattttcttcatcattatcactgtcccattttaactctaaagagtcatcctgaaacacaacacttggttggctccagtcaaaagaaagagtggagtttgattgcttctctgaggaaccctctgaagaagatccaaaaccatttatcagtgactgtgaccaatcaacagcagaagacttatcttcccttgcatccaactttaatggagaagaaggagaacagtctttactagtatccagaaaactagaagccctataaaaaggtcttgttttcttgatgactttaggcatctttgataatacttccaaagccaacattgggcagccagcttttaaatgagcactggcagtggtaaaaaataaacgtctttcacttaaattaattgttcctgccagtccactttttcctgttaggctcatatgtgtggaaaatgtatcagatgatccaaaatgacgtctcagcaaaagaggatgtgttcttagataattgtagaaattaaaaactgtaggattactggctgataaaacttgatcatcattctctctgataggttgctttattaatgtttccagagcaccactataatcttccaaaatccaatatgccatgctccgaagaaaaggatcatgatgcatatttatgttcaatgaacacagttcactgacaggagaatcgattcccaaaacttttttacgtaaaatagatttatatgctgcagatgtatcaaattcagactcatagagtcttgctattacaagagccaactgaatgtcattcaatttctcaagacatacctcaattgcatctctgaggcaaccagctaaaagaaaaaatgctgcagaatgttcaaatctttgtttgcctagcaaagaaaaagcattctttaaagctgctttacgccacctctcatcctcaaaattgtgtccaaaaaactgtgtcatcctggtgtttttttcagctctatataatccccaaatcacagctttctttttcattgcaaggtaaaaaatggcagcatctaaaggatcattctttctataaaaggctgctttagctactttttctatgcatttgcgtaagatgcgggtattccggacccaccaccccacacccatagctcttagttcagaccaagtgggatcatctttctgcatggctggcaacatgttcagcagttcttcttctgctactgagtgaaatgcccaagcaaaatgacttgtagacaggccttggtgaaggagttgagctcgataggctggaagggaagttgtaagaaaggtatggagtcgaacagccaaaagaaattttaacccacattcatcaagagtttctccaccttggcttctgtctcggctttctccaatatcagtgcttgtagttgcaattgtatctgctaaggccatcaaagacatctgctccatccggctgagtcctggtaaactagaatgaagtaagtggccagaaagaacctgagcatgctcaggtccaaagtaagtcggactgtactgtgaaaggtcaataactctaggctttgtattttcttcatctgtctctaacatatgagtatcagtcattagaagttgagtctgaaaaagctcatcataactttctttagataattggtttgatttacttaacgtactctcattactagatttctccaaagatgagtaacagctatcatcatctgctgcaagtaaggcatataaaggaagtggaggaacagaatctatttctgtgtaatctgtattttcagccttgttgaatgcctgggggtctctggtagtgcttccactagcactgattgtgagagacctaaggcggcgttcatgattagattcagcttcattcagagccacaacttccccagcaatgcacttaacaagatgggacaagatggccttggctctccgaactttaccaagatccatgagttccaaaagctgcaagggatgatactgaggtagagtcggggaaagtacatgagctgcttcaaaaagacctgaatcttccatatccactgaaggatcgaatgcagttttctttccacagattttctgtgcaagactggtcatggatcgagtcagagttttctttggaggatgtaacccagaactggagttactctgttttattaaacttgttatagatggagtgctcccactgtacgaatctgttataacaggttcttgtttagaagatggttgccattggcaatacacatgcatttcacagtccattcctaccacaaggatgccatcccggacccacgataaagaaacaggaaaaggtggggagccatctacagaagaaactaggtccacacttcgtaatagtacaaatttagaaaggggcacaactttggtactctcccagagaggaaatgccagggtttccttaccagtttggtcttgtaccttgccagccaggggtccatacataaaaagttttgatccaattcctacagtcaggatatgagaaccgtcttctctagacatccaatctaagtgaactaaatgctttgtgtttgatgtgatattctctttactagataaatacatgtcttgtttattataggccactaaattgctatcaacactaatgccagaatccaatactgtgcttaactcatctaaatgaattgtctgctcaaggacccaacatgaacctcctgttgactcacattcaaaaatacttacatgcatcacaaagtcctgggaagatctactattagatgcaggctgcttataagctactgctaaacgatttgtatgtgcacagctaacttctacaggcctaccaggtacagttatactactattgctctgaagtccatcttcaataagtaatggccattcttcccaaatgtatgcaagatcaatttttccattctttgacgtggcagattctccatctgttactctgcatctccagaatcttactttctcatctgaacatgaagttgccaataaataaggagcactgcatgcaggatatatagaagatgaactcagatgtcctgctgatggcttaatacttattatctcaactccttctggtaaatgcaattcttggctataaaccatttctgaaaacagagtcaacctgctggtactctggagatttgctctgcaagcctgatacttttgtgaaaaaggagataggatcttctctggagaagaagaataatgttcttctggctgccaaaccgcttcggataattttgtatctactttttcatctaatgagacaggaattgactttagatgtaaattccacatgtgtaacagtgaacggttgtcttgagtgcattctattacaattaggtagaacttctcagaaaatccattaggtgagctgcctgcattagataaaatgctgtctttgccaaggcttttcttctcaaggttattcaaaatgaagtcttcttcaaaaacatgaagcagttgggtttttctgccatgaagtttggtaatgggatctaatgcaataatgcatcctggcctggctgttgattgttgactgacgatgttaaagacttcaccaacatatttagaaatttcagggttagaaagctcagataaaagtttcttagcatcaataactgcttcatataatctcagatattgtccatcactggctacaaagcatgcactaggagagttgcagtatgcacccagacaataactgggtataagagtgggcagccatgccacattggaaaaggcagaaacatgaagagaattaatccgggcaagctcagaaactcctccagaaaaagacaatggcccaactgggtcaaccctccacagaataagctcactgtaaactgcactgggatcctgaaatgccacgtcaacagtgcttttattttgttgtgtcaaagagcattcttcaatatttagagcatcaaaaggttgctctgggttatcaacatctggtgtccttaatgcattatggtgtgatgttgtcagcaataatggtaatactgagtggcaagctaaatcattaagatgaaaacgatgaccacaatatctggatttgtgggaaatactgagaacagtagaaaaagcagattcctcggcaaaactgaccagccactgattcagagaaccatcagcatgttttgatatcatcataacattaggcgtaaaaatacttaattttaaactattagatgatttattgtgaccagaagaaataagcattgatgtggaacgggtgaggccagaaggtttttgtttcccctgctgaatagccaagtcaacattcttggtacaggcatacatcattatgcttttacagagagagtttgcatcacctgtggggaaagctactggaattctggaaacaaaggacacctgtacttgacgaaacataccaggctggtattcatccagccaatccacatgccaaactagcaaagaaccatccatgggatgaatactaaatagcatatctgcatttttactccattcagacagaagtacttcaatctgatgatcaatggcagctgacgataatgatgtaaaacttgagtttggtaccattttatcacagcctaattccttcttttcgggatttattttcagatcatcaacaccatcatcagtttcttcatcagattttacatctgcctgattagaatcttctacactggcctcagaagatggttgttcaaaactttttctaagttgctgtaaaaaaacttccatggacaaagtaaaatgcagttctttattgtttagccagtgtacaacaaaaggtccggtcttctcttcattttcatttagactcagagatgtaatagatggaagaagtggaatgtctgtggctgggttgatgctggctgcaatatgaaagtggcaaagtgcattggcatgcagtggagtgttcctgtgaacatgatgaggatcctgctgatgtggtagatatcccgtatgtgctacaagagcaagtgatctcctccgacctctacgaaaatgtctcagatttacttctaaagcattttgaactcgttctttactggaagcatttctcttgaagttatttgttaaattaattgattcagtccaatggctgcagtcacctccgtatagcaaacaatcatttggtaaaaatgtctctacccaaagacgacacacattatctttgcagcaagtcaacagtacattacatacagaagccctaggcatatatttgcttgttttacgccaggaaaatccatttactgctcgaggatgggccagatacacaaaagaaaagtcaatttctccttgggattgtttttctgaacttccatctggagaagtaacagctgtccgccagttttctacattataccaaaccttcaaaagacagtcatccttcccagcagtggcaaaaaattctccatctggtgaaaatttcattaaatgaacttgggaagcagttttgcaatgccaaatgcatttccaatctccaaagttaagatctgttttatttaaattttcatcttcagttggcttctccaagttagtattggaccagagttgcaaatagctggaaccagttaaaagacgactgcctgtgggatcccaggttatattgtgtgctattgattccagaaaaaattggccacttttctgccactgactatataattccaaatttttcttttgttttggtaggttaactggttcaaaaatggagataacatttccataagacgctgcaatcttgccttgttgcattgaacagtctacacatcccacttgaatatttccatgtttagctcctgggattatctgtaatctttcaaaatcgcttcccagtattacaatgtcacatccagatgcataagccgtgaagcgctggtcgccaatgctgcccacggagaagcagtggtcgccagggttcacagccccggtcagcacctggtgcaggttcatgtcggcgccctagtccggccaggaaggccgcgctgtccacacacttcctctggacctcgggcagccgctcctgacccagcccgagtggcgcaagcagtacgcgctcgcactccccgcctgacctgtcccttcccggctccggtgcccgccacccccacagtcctccgccactcactacgcg

SEQ ID NO: 9972 - RNA, 10390 nt, Homo sapiens
  source 1..10390: mol_type = other RNA
cacacacacacacacacgtatacatacatacaacttgggttccggagggtaaactactgaaaaccttacatattgagccatctagctcatttatcactgacgtctcaatgacaattttaatgaagatgttcattatttttttcattcttactcaaatacctatcattaattaagagaagagtttgagatgtataaggctaataaaggaagtgagagtgtggtgaattaagtgatgagtattatgtacaattgcctttacaaaaaacgtatttttactgtggaagaaattcatgcagagatgcctgtggaaaagtatcaataagaaaacaaaacacctttaacactatgacatactgattataatatactatgatatgtattattacagcattacttacacattctactttaggcaatgtaatctacttctgaatgaccttgttaatttttaaggcatcagtgcatcaagggcaaagctccataaaataaatataaaaacaagaaagcattagctaatttgtggcatagagaatgatcactgtatattatatctgttggccacttccatataggtaataaattgtacatcttattgtaaaaatgttatagcataaatttcacatcatttttcaacacttcatttaaagggctaaactgatctggcagtattctcattttcattgttccatcagctccacaggagaaaatgtgatttgcaggccctgtctcaatttgcatcactccagttccaatatttctaaaaatggactgccgagcatgttcactgacaaaagtatggagaagaccaaaggtagagagactccaaatctttatattgccttcggcagatcctgtaacaaagtactcttcagttggatcaacagcaacggctttaacaggagaatcatggctctggaaaagctgcctctgttgtcgttgacaaaggtcaaatacatatgtaaaaccttttctgccacctgatattagtagctgatgttttggagcatatgctaaaactgtggctccactgtcatggcaggtaaatgcatggactaaactattggcaggtgctacaagagtatcccacaaacatacgtttctattgtcagttgaaagaccagctgtagctatcagagaggaggaactaacgaagacaaaatcattggctgttttgttatgacactgccaagtcaggtatggcttaggcatgcttccagtaactggacaacatttccagtttgtttgatacaaacttaaatatccatcagcatcaactattccaaacttatttccctgatagttaaatctcattcttgtaactcttgaattgccaccagatcgaaaacaggttatttgttgagaatggccccattcaaacattctgacacttccatcttgagctcctgtcagatagtaaggaagagttggatgagaagtcattcttctaacattattaatggctttcttaatcatcacagatgctcctctgccagtctgtgtactaccaagccatggcatgttgattggagtgccaggattgctatgtgtatatggagttgtaccttgaacagctgttaaatcatcacgagcatgtataaccaagaaatcttctgatcctttggtttccacttctatatcatcatctacccaagtgtagacctgtgtggccagaattccagaaacatccagttcttgaacatcatgactggaagcgattgctatgcagtttctatttgccttattaacagcaaacgcagtaatgatatcagattccttatgaataattcttgctttacctccaggatatcccaaatctgcttctatcttattgatgtttggctcctccatcatagaatttttgatggtttcactgttgtcctctaatgactcatttagacaccgtttctttgtgaatatatttttgataaaggtttcctgaatttcttcctgcttcaccaaatactgccaaagcctcttcacagacagtgccagatggtgtttggatttgaaaggagtgtttgtaggttccagtaaagctttgtggcgaagaattgcaggacctgcagacaaactctcttcggcggtatgacttgcgatataattttgaggtggcccaccatggatttcaagtcgtcggagaagaacttgttcccaacattgaagagtttttagaaccgcatgacaaagaggtgaactaactggaagctctgcaagatcatgacctgcgaagggataaaaagtcttcaaattgttgagcaccaattgcaccatcgccaaccgcatcaaggaccaactatatgaatttgaattagaatgttcctggagatggaaatctgatgctaaaacatcatcatcatcatcattgtcatcatcatcacttcccagactctcctctgaatcatattcggctctactttgagaagagggtagaaaaggcttagctatgaaatagtcccagatactgagctcaggtgggatgaacttttctttaaccgccagtgactcctggcttactggtgccgaggaaggggtcagtggggcagattctctgcaagacatttttgacggcctaaaacgtttgttctgtttttctccttcttcaactagtgaagaaactgcaagactgggagggctatgagaactgatggctgaaagagctttggaaaagcccacacattccatggagaataccactacctggtgggggctaggcatagcaaagtgccttccaggtaaagtttttgaatgtgtctgttctttgctaggaacatgtgcacctccaccaaacacagcagaccacattttctcatttagaggatgggccacaatccgaaatagctcattacttgaatgtgtggccaggccatggatgaagagactaagatacactgctgtgagaatctcacagagcaagactgtaagccctgactgggcttcctcgccagaagaattcaaaagtcgaattagacaagttattcctggccattgagctggtgacgtattgggagttaatgcttcatctaagcttcctgttttcaaagaaggtcgatgaggaagcagtactgtctgatataccattccagtaaactgattcgtctgaaatgaactgtagttatgactaccacaaaggcactgataaatacaagcagaaagtgaagctgctaaagtatgcattacatacactttattgctttggatatcagggtggggtggtgaatcaaagtttattatggcatggagaatatcatgtgtcagattactaaggtgcaataatggattggcaactactgttttggcattggctgtacaagcaaagaggagaggcactgaggtttgctctgacagagggctagaaaatagtggttctgatgtttcctgctgagattcttgcaaaagcaaaatcaattccattcttacagatgcaagacccccaccatgggatccatgaagtatgcagtaactaagaaacattctcaaaagtgactgatacttcaagagccactgtcttttttcctgaaaattttctctcagttgtttcacttttgtttggtgaggcaaatcttcagcatcctcatttaatccaaattcatcttcatttctgccaaatgcagactgtagttcttcagcatctgagcaaaagtcacaagtcctctgaagagctatcacctctttttcaagccagtggtatagttggtaacgcaattttccaccatctatttcatagccagtagataaagtacgaagttctactgtgagaatctttaaacatgctctaaattttaactgaactgcaattatatcttctgatggatttaaaaggtcattttcatctagtgtgctgaaagattctgtgtagttagaacttatgtcatccaactttttatctgtttttctctgtaaaggttttagttctttcattgaaatagggacatcctcattttcttcatcattatcactgtcccattttaactctaaagagtcatcctgaaacacaacacttggttggctccagtcaaaagaaagagtggagtttgattgcttctctgaggaaccctctgaagaagatccaaaaccatttatcagtgactgtgaccaatcaacagcagaagacttatcttcccttgcatccaactttaatggagaagaaggagaacagtctttactagtatccagaaaactagaagccctataaaaaggtcttgttttcttgatgactttaggcatctttgataatacttccaaagccaacattgggcagccagcttttaaatgagcactggcagtggtaaaaaataaacgtctttcacttaaattaattgttcctgccagtccactttttcctgttaggctcatatgtgtggaaaatgtatcagatgatccaaaatgacgtctcagcaaaagaggatgtgttcttagataattgtagaaattaaaaactgtaggattactggctgataaaacttgatcatcattctctctgataggttgctttattaatgtttccagagcaccactataatcttccaaaatccaatatgccatgctccgaagaaaaggatcatgatgcatatttatgttcaatgaacacagttcactgacaggagaatcgattcccaaaacttttttacgtaaaatagatttatatgctgcagatgtatcaaattcagactcatagagtcttgctattacaagagccaactgaatgtcattcaatttctcaagacatacctcaattgcatctctgaggcaaccagctaaaagaaaaaatgctgcagaatgttcaaatctttgtttgcctagcaaagaaaaagcattctttaaagctgctttacgccacctctcatcctcaaaattgtgtccaaaaaactgtgtcatcctggtgtttttttcagctctatataatccccaaatcacagctttctttttcattgcaaggtaaaaaatggcagcatctaaaggatcattctttctataaaaggctgctttagctactttttctatgcatttgcgtaagatgcgggtattccggacccaccaccccacacccatagctcttagttcagaccaagtgggatcatctttctgcatggctggcaacatgttcagcagttcttcttctgctactgagtgaaatgcccaagcaaaatgacttgtagacaggccttggtgaaggagttgagctcgataggctggaagggaagttgtaagaaaggtatggagtcgaacagccaaaagaaattttaacccacattcatcaagagtttctccaccttggcttctgtctcggctttctccaatatcagtgcttgtagttgcaattgtatctgctaaggccatcaaagacatctgctccatccggctgagtcctggtaaactagaatgaagtaagtggccagaaagaacctgagcatgctcaggtccaaagtaagtcggactgtactgtgaaaggtcaataactctaggctttgtattttcttcatctgtctctaacatatgagtatcagtcattagaagttgagtctgaaaaagctcatcataactttctttagataattggtttgatttacttaacgtactctcattactagatttctccaaagatgagtaacagctatcatcatctgctgcaagtaaggcatataaaggaagtggaggaacagaatctatttctgtgtaatctgtattttcagccttgttgaatgcctgggggtctctggtagtgcttccactagcactgattgtgagagacctaaggcggcgttcatgattagattcagcttcattcagagccacaacttccccagcaatgcacttaacaagatgggacaagatggccttggctctccgaactttaccaagatccatgagttccaaaagctgcaagggatgatactgaggtagagtcggggaaagtacatgagctgcttcaaaaagacctgaatcttccatatccactgaaggatcgaatgcagttttctttccacagattttctgtgcaagactggtcatggatcgagtcagagttttctttggaggatgtaacccagaactggagttactctgttttattaaacttgttatagatggagtgctcccactgtacgaatctgttataacaggttcttgtttagaagatggttgccattggcaatacacatgcatttcacagtccattcctaccacaaggatgccatcccggacccacgataaagaaacaggaaaaggtggggagccatctacagaagaaactaggtccacacttcgtaatagtacaaatttagaaaggggcacaactttggtactctcccagagaggaaatgccagggtttccttaccagtttggtcttgtaccttgccagccaggggtccatacataaaaagttttgatccaattcctacagtcaggatatgagaaccgtcttctctagacatccaatctaagtgaactaaatgctttgtgtttgatgtgatattctctttactagataaatacatgtcttgtttattataggccactaaattgctatcaacactaatgccagaatccaatactgtgcttaactcatctaaatgaattgtctgctcaaggacccaacatgaacctcctgttgactcacattcaaaaatacttacatgcatcacaaagtcctgggaagatctactattagatgcaggctgcttataagctactgctaaacgatttgtatgtgcacagctaacttctacaggcctaccaggtacagttatactactattgctctgaagtccatcttcaataagtaatggccattcttcccaaatgtatgcaagatcaatttttccattctttgacgtggcagattctccatctgttactctgcatctccagaatcttactttctcatctgaacatgaagttgccaataaataaggagcactgcatgcaggatatatagaagatgaactcagatgtcctgctgatggcttaatacttattatctcaactccttctggtaaatgcaattcttggctataaaccatttctgaaaacagagtcaacctgctggtactctggagatttgctctgcaagcctgatacttttgtgaaaaaggagataggatcttctctggagaagaagaataatgttcttctggctgccaaaccgcttcggataattttgtatctactttttcatctaatgagacaggaattgactttagatgtaaattccacatgtgtaacagtgaacggttgtcttgagtgcattctattacaattaggtagaacttctcagaaaatccattaggtgagctgcctgcattagataaaatgctgtctttgccaaggcttttcttctcaaggttattcaaaatgaagtcttcttcaaaaacatgaagcagttgggtttttctgccatgaagtttggtaatgggatctaatgcaataatgcatcctggcctggctgttgattgttgactgacgatgttaaagacttcaccaacatatttagaaatttcagggttagaaagctcagataaaagtttcttagcatcaataactgcttcatataatctcagatattgtccatcactggctacaaagcatgcactaggagagttgcagtatgcacccagacaataactgggtataagagtgggcagccatgccacattggaaaaggcagaaacatgaagagaattaatccgggcaagctcagaaactcctccagaaaaagacaatggcccaactgggtcaaccctccacagaataagctcactgtaaactgcactgggatcctgaaatgccacgtcaacagtgcttttattttgttgtgtcaaagagcattcttcaatatttagagcatcaaaaggttgctctgggttatcaacatctggtgtccttaatgcattatggtgtgatgttgtcagcaataatggtaatactgagtggcaagctaaatcattaagatgaaaacgatgaccacaatatctggatttgtgggaaatactgagaacagtagaaaaagcagattcctcggcaaaactgaccagccactgattcagagaaccatcagcatgttttgatatcatcataacattaggcgtaaaaatacttaattttaaactattagatgatttattgtgaccagaagaaataagcattgatgtggaacgggtgaggccagaaggtttttgtttcccctgctgaatagccaagtcaacattcttggtacaggcatacatcattatgcttttacagagagagtttgcatcacctgtggggaaagctactggaattctggaaacaaaggacacctgtacttgacgaaacataccaggctggtattcatccagccaatccacatgccaaactagcaaagaaccatccatgggatgaatactaaatagcatatctgcatttttactccattcagacagaagtacttcaatctgatgatcaatggcagctgacgataatgatgtaaaacttgagtttggtaccattttatcacagcctaattccttcttttcgggatttattttcagatcatcaacaccatcatcagtttcttcatcagattttacatctgcctgattagaatcttctacactggcctcagaagatggttgttcaaaactttttctaagttgctgtaaaaaaacttccatggacaaagtaaaatgcagttctttattgtttagccagtgtacaacaaaaggtccggtcttctcttcattttcatttagactcagagatgtaatagatggaagaagtggaatgtctgtggctgggttgatgctggctgcaatatgaaagtggcaaagtgcattggcatgcagtggagtgttcctgtgaacatgatgaggatcctgctgatgtggtagatatcccgtatgtgctacaagagcaagtgatctcctccgacctctacgaaaatgtctcagatttacttctaaagcattttgaactcgttctttactggaagcatttctcttgaagttatttgttaaattaattgattcagtccaatggctgcagtcacctccgtatagcaaacaatcatttggtaaaaatgtctctacccaaagacgacacacattatctttgcagcaagtcaacagtacattacatacagaagccctaggcatatatttgcttgttttacgccaggaaaatccatttactgctcgaggatgggccagatacacaaaagaaaagtcaatttctccttgggattgtttttctgaacttccatctggagaagtaacagctgtccgccagttttctacattataccaaaccttcaaaagacagtcatccttcccagcagtggcaaaaaattctccatctggtgaaaatttcattaaatgaacttgggaagcagttttgcaatgccaaatgcatttccaatctccaaagttaagatctgttttatttaaattttcatcttcagttggcttctccaagttagtattggaccagagttgcaaatagctggaaccagttaaaagacgactgcctgtgggatcccaggttatattgtgtgctattgattccagaaaaaattggccacttttctgccactgactatataattccaaatttttcttttgttttggtaggttaactggttcaaaaatggagataacatttccataagacgctgcaatcttgccttgttgcattgaacagtctacacatcccacttgaatatttccatgtttagctcctgggattatctgtaatctttcaaaatcgcttcccagtattacaatgtcacatccagatgcataagccgtgaagcgctggtcgccaatgctgcccacggagaagcagtggtcgccagggttcacagccccggtcagcacctggtgcaggttcatgtcggcgccctagtcctgcaacggacaccgcatccagctcatgccacgggtcagcggctgcttccctccctccttccctcaggggcggcggccgctcttcggtggcgacggcagaagcagcgacaggcgcctggagccggagccgctcagctggggcccgcgactcatcccgagccccggagggcgaggcccggagggggcgggtcggcgagagggcggagcgccgcgctccttcgcgcacctgtcactccccgcgctagcccaggtgaagctcagggtcccctcaccggccacgacccggggccgactcaccggccaggaaggccgcgctgtccacacacttcctctggacctcgggcagccgctcctgacccagcccgagtggcgcaagcagtacgcgctcgcactccccgcctgacctgtcccttcccggctccggtgcccgccacccccacagtcctccgccactcactacgcgcctctggatccctgcggccgaaatatcgcgagacttcgctcggggcag

SEQ ID NO: 9973 - RNA, 9975 nt, Homo sapiens
  source 1..9975: mol_type = other RNA
cacacacacacacacacgtatacatacatacaacttgggttccggagggtaaactactgaaaaccttacatattgagccatctagctcatttatcactgacgtctcaatgacaattttaatgaagatgttcattatttttttcattcttactcaaatacctatcattaattaagagaagagtttgagatgtataaggctaataaaggaagtgagagtgtggtgaattaagtgatgagtattatgtacaattgcctttacaaaaaacgtatttttactgtggaagaaattcatgcagagatgcctgtggaaaagtatcaataagaaaacaaaacacctttaacactatgacatactgattataatatactatgatatgtattattacagcattacttacacattctactttaggcaatgtaatctacttctgaatgaccttgttaatttttaaggcatcagtgcatcaagggcaaagctccataaaataaatataaaaacaagaaagcattagctaatttgtggcatagagaatgatcactgtatattatatctgttggccacttccatataggtaataaattgtacatcttattgtaaaaatgttatagcataaatttcacatcatttttcaacacttcatttaaagggctaaactgatctggcagtattctcattttcattgttccatcagctccacaggagaaaatgtgatttgcaggccctgtctcaatttgcatcactccagttccaatatttctaaaaatggactgccgagcatgttcactgacaaaagtatggagaagaccaaaggtagagagactccaaatctttatattgccttcggcagatcctgtaacaaagtactcttcagttggatcaacagcaacggctttaacaggagaatcatggctctggaaaagctgcctctgttgtcgttgacaaaggtcaaatacatatgtaaaaccttttctgccacctgatattagtagctgatgttttggagcatatgctaaaactgtggctccactgtcatggcaggtaaatgcatggactaaactattggcaggtgctacaagagtatcccacaaacatacgtttctattgtcagttgaaagaccagctgtagctatcagagaggaggaactaacgaagacaaaatcattggctgttttgttatgacactgccaagtcaggtatggcttaggcatgcttccagtaactggacaacatttccagtttgtttgatacaaacttaaatatccatcagcatcaactattccaaacttatttccctgatagttaaatctcattcttgtaactcttgaattgccaccagatcgaaaacaggttatttgttgagaatggccccattcaaacattctgacacttccatcttgagctcctgtcagatagtaaggaagagttggatgagaagtcattcttctaacattattaatggctttcttaatcatcacagatgctcctctgccagtctgtgtactaccaagccatggcatgttgattggagtgccaggattgctatgtgtatatggagttgtaccttgaacagctgttaaatcatcacgagcatgtataaccaagaaatcttctgatcctttggtttccacttctatatcatcatctacccaagtgtagacctgtgtggccagaattccagaaacatccagttcttgaacatcatgactggaagcgattgctatgcagtttctatttgccttattaacagcaaacgcagtaatgatatcagattccttatgaataattcttgctttacctccaggatatcccaaatctgcttctatcttattgatgtttggctcctccatcatagaatttttgatggtttcactgttgtcctctaatgactcatttagacaccgtttctttgtgaatatatttttgataaaggtttcctgaatttcttcctgcttcaccaaatactgccaaagcctcttcacagacagtgccagatggtgtttggatttgaaaggagtgtttgtaggttccagtaaagctttgtggcgaagaattgcaggacctgcagacaaactctcttcggcggtatgacttgcgatataattttgaggtggcccaccatggatttcaagtcgtcggagaagaacttgttcccaacattgaagagtttttagaaccgcatgacaaagaggtgaactaactggaagctctgcaagatcatgacctgcgaagggataaaaagtcttcaaattgttgagcaccaattgcaccatcgccaaccgcatcaaggaccaactatatgaatttgaattagaatgttcctggagatggaaatctgatgctaaaacatcatcatcatcatcattgtcatcatcatcacttcccagactctcctctgaatcatattcggctctactttgagaagagggtagaaaaggcttagctatgaaatagtcccagatactgagctcaggtgggatgaacttttctttaaccgccagtgactcctggcttactggtgccgaggaaggggtcagtggggcagattctctgcaagacatttttgacggcctaaaacgtttgttctgtttttctccttcttcaactagtgaagaaactgcaagactgggagggctatgagaactgatggctgaaagagctttggaaaagcccacacattccatggagaataccactacctggtgggggctaggcatagcaaagtgccttccaggtaaagtttttgaatgtgtctgttctttgctaggaacatgtgcacctccaccaaacacagcagaccacattttctcatttagaggatgggccacaatccgaaatagctcattacttgaatgtgtggccaggccatggatgaagagactaagatacactgctgtgagaatctcacagagcaagactgtaagccctgactgggcttcctcgccagaagaattcaaaagtcgaattagacaagttattcctggccattgagctggtgacgtattgggagttaatgcttcatctaagcttcctgttttcaaagaaggtcgatgaggaagcagtactgtctgatataccattccagtaaactgattcgtctgaaatgaactgtagttatgactaccacaaaggcactgataaatacaagcagaaagtgaagctgctaaagtatgcattacatacactttattgctttggatatcagggtggggtggtgaatcaaagtttattatggcatggagaatatcatgtgtcagattactaaggtgcaataatggattggcaactactgttttggcattggctgtacaagcaaagaggagaggcactgaggtttgctctgacagagggctagaaaatagtggttctgatgtttcctgctgagattcttgcaaaagcaaaatcaattccattcttacagatgcaagacccccaccatgggatccatgaagtatgcagtaactaagaaacattctcaaaagtgactgatacttcaagagccactgtcttttttcctgaaaattttctctcagttgtttcacttttgtttggtgaggcaaatcttcagcatcctcatttaatccaaattcatcttcatttctgccaaatgcagactgtagttcttcagcatctgagcaaaagtcacaagtcctctgaagagctatcacctctttttcaagccagtggtatagttggtaacgcaattttccaccatctatttcatagccagtagataaagtacgaagttctactgtgagaatctttaaacatgctctaaattttaactgaactgcaattatatcttctgatggatttaaaaggtcattttcatctagtgtgctgaaagattctgtgtagttagaacttatgtcatccaactttttatctgtttttctctgtaaaggttttagttctttcattgaaatagggacatcctcattttcttcatcattatcactgtcccattttaactctaaagagtcatcctgaaacacaacacttggttggctccagtcaaaagaaagagtggagtttgattgcttctctgaggaaccctctgaagaagatccaaaaccatttatcagtgactgtgaccaatcaacagcagaagacttatcttcccttgcatccaactttaatggagaagaaggagaacagtctttactagtatccagaaaactagaagccctataaaaaggtcttgttttcttgatgactttaggcatctttgataatacttccaaagccaacattgggcagccagcttttaaatgagcactggcagtggtaaaaaataaacgtctttcacttaaattaattgttcctgccagtccactttttcctgttaggctcatatgtgtggaaaatgtatcagatgatccaaaatgacgtctcagcaaaagaggatgtgttcttagataattgtagaaattaaaaactgtaggattactggctgataaaacttgatcatcattctctctgataggttgctttattaatgtttccagagcaccactataatcttccaaaatccaatatgccatgctccgaagaaaaggatcatgatgcatatttatgttcaatgaacacagttcactgacaggagaatcgattcccaaaacttttttacgtaaaatagatttatatgctgcagatgtatcaaattcagactcatagagtcttgctattacaagagccaactgaatgtcattcaatttctcaagacatacctcaattgcatctctgaggcaaccagctaaaagaaaaaatgctgcagaatgttcaaatctttgtttgcctagcaaagaaaaagcattctttaaagctgctttacgccacctctcatcctcaaaattgtgtccaaaaaactgtgtcatcctggtgtttttttcagctctatataatccccaaatcacagctttctttttcattgcaaggtaaaaaatggcagcatctaaaggatcattctttctataaaaggctgctttagctactttttctatgcatttgcgtaagatgcgggtattccggacccaccaccccacacccatagctcttagttcagaccaagtgggatcatctttctgcatggctggcaacatgttcagcagttcttcttctgctactgagtgaaatgcccaagcaaaatgacttgtagacaggccttggtgaaggagttgagctcgataggctggaagggaagttgtaagaaaggtatggagtcgaacagccaaaagaaattttaacccacattcatcaagagtttctccaccttggcttctgtctcggctttctccaatatcagtgcttgtagttgcaattgtatctgctaaggccatcaaagacatctgctccatccggctgagtcctggtaaactagaatgaagtaagtggccagaaagaacctgagcatgctcaggtccaaagtaagtcggactgtactgtgaaaggtcaataactctaggctttgtattttcttcatctgtctctaacatatgagtatcagtcattagaagttgagtctgaaaaagctcatcataactttctttagataattggtttgatttacttaacgtactctcattactagatttctccaaagatgagtaacagctatcatcatctgctgcaagtaaggcatataaaggaagtggaggaacagaatctatttctgtgtaatctgtattttcagccttgttgaatgcctgggggtctctggtagtgcttccactagcactgattgtgagagacctaaggcggcgttcatgattagattcagcttcattcagagccacaacttccccagcaatgcacttaacaagatgggacaagatggccttggctctccgaactttaccaagatccatgagttccaaaagctgcaagggatgatactgaggtagagtcggggaaagtacatgagctgcttcaaaaagacctgaatcttccatatccactgaaggatcgaatgcagttttctttccacagattttctgtgcaagactggtcatggatcgagtcagagttttctttggaggatgtaacccagaactggagttactctgttttattaaacttgttatagatggagtgctcccactgtacgaatctgttataacaggttcttgtttagaagatggttgccattggcaatacacatgcatttcacagtccattcctaccacaaggatgccatcccggacccacgataaagaaacaggaaaaggtggggagccatctacagaagaaactaggtccacacttcgtaatagtacaaatttagaaaggggcacaactttggtactctcccagagaggaaatgccagggtttccttaccagtttggtcttgtaccttgccagccaggggtccatacataaaaagttttgatccaattcctacagtcaggatatgagaaccgtcttctctagacatccaatctaagtgaactaaatgctttgtgtttgatgtgatattctctttactagataaatacatgtcttgtttattataggccactaaattgctatcaacactaatgccagaatccaatactgtgcttaactcatctaaatgaattgtctgctcaaggacccaacatgaacctcctgttgactcacattcaaaaatacttacatgcatcacaaagtcctgggaagatctactattagatgcaggctgcttataagctactgctaaacgatttgtatgtgcacagctaacttctacaggcctaccaggtacagttatactactattgctctgaagtccatcttcaataagtaatggccattcttcccaaatgtatgcaagatcaatttttccattctttgacgtggcagattctccatctgttactctgcatctccagaatcttactttctcatctgaacatgaagttgccaataaataaggagcactgcatgcaggatatatagaagatgaactcagatgtcctgctgatggcttaatacttattatctcaactccttctggtaaatgcaattcttggctataaaccatttctgaaaacagagtcaacctgctggtactctggagatttgctctgcaagcctgatacttttgtgaaaaaggagataggatcttctctggagaagaagaataatgttcttctggctgccaaaccgcttcggataattttgtatctactttttcatctaatgagacaggaattgactttagatgtaaattccacatgtgtaacagtgaacggttgtcttgagtgcattctattacaattaggtagaacttctcagaaaatccattaggtgagctgcctgcattagataaaatgctgtctttgccaaggcttttcttctcaaggttattcaaaatgaagtcttcttcaaaaacatgaagcagttgggtttttctgccatgaagtttggtaatgggatctaatgcaataatgcatcctggcctggctgttgattgttgactgacgatgttaaagacttcaccaacatatttagaaatttcagggttagaaagctcagataaaagtttcttagcatcaataactgcttcatataatctcagatattgtccatcactggctacaaagcatgcactaggagagttgcagtatgcacccagacaataactgggtataagagtgggcagccatgccacattggaaaaggcagaaacatgaagagaattaatccgggcaagctcagaaactcctccagaaaaagacaatggcccaactgggtcaaccctccacagaataagctcactgtaaactgcactgggatcctgaaatgccacgtcaacagtgcttttattttgttgtgtcaaagagcattcttcaatatttagagcatcaaaaggttgctctgggttatcaacatctggtgtccttaatgcattatggtgtgatgttgtcagcaataatggtaatactgagtggcaagctaaatcattaagatgaaaacgatgaccacaatatctggatttgtgggaaatactgagaacagtagaaaaagcagattcctcggcaaaactgaccagccactgattcagagaaccatcagcatgttttgatatcatcataacattaggcgtaaaaatacttaattttaaactattagatgatttattgtgaccagaagaaataagcattgatgtggaacgggtgaggccagaaggtttttgtttcccctgctgaatagccaagtcaacattcttggtacaggcatacatcattatgcttttacagagagagtttgcatcacctgtggggaaagctactggaattctggaaacaaaggacacctgtacttgacgaaacataccaggctggtattcatccagccaatccacatgccaaactagcaaagaaccatccatgggatgaatactaaatagcatatctgcatttttactccattcagacagaagtacttcaatctgatgatcaatggcagctgacgataatgatgtaaaacttgagtttggtaccattttatcacagcctaattccttcttttcgggatttattttcagatcatcaacaccatcatcagtttcttcatcagattttacatctgcctgattagaatcttctacactggcctcagaagatggttgttcaaaactttttctaagttgctgtaaaaaaacttccatggacaaagtaaaatgcagttctttattgtttagccagtgtacaacaaaaggtccggtcttctcttcattttcatttagactcagagatgtaatagatggaagaagtggaatgtctgtggctgggttgatgctggctgcaatatgaaagtggcaaagtgcattggcatgcagtggagtgttcctgtgaacatgatgaggatcctgctgatgtggtagatatcccgtatgtgctacaagagcaagtgatctcctccgacctctacgaaaatgtctcagatttacttctaaagcattttgaactcgttctttactggaagcatttctcttgaagttatttgttaaattaattgattcagtccaatggctgcagtcacctccgtatagcaaacaatcatttggtaaaaatgtctctacccaaagacgacacacattatctttgcagcaagtcaacagtacattacatacagaagccctaggcatatatttgcttgttttacgccaggaaaatccatttactgctcgaggatgggccagatacacaaaagaaaagtcaatttctccttgggattgtttttctgaacttccatctggagaagtaacagctgtccgccagttttctacattataccaaaccttcaaaagacagtcatccttcccagcagtggcaaaaaattctccatctggtgaaaatttcattaaatgaacttgggaagcagttttgcaatgccaaatgcatttccaatctccaaagttaagatctgttttatttaaattttcatcttcagttggcttctccaagttagtattggaccagagttgcaaatagctggaaccagttaaaagacgactgcctgtgggatcccaggttatattgtgtgctattgattccagaaaaaattggccacttttctgccactgactatataattccaaatttttcttttgttttggtaggttaactggttcaaaaatggagataacatttccataagacgctgcaatcttgccttgttgcattgaacagtctacacatcccacttgaatatttccatgtttagctcctgggattatctgtaatctttcaaaatcgcttcccagtattacaatgtcacatccagatgcataagccgtgaagcgctggtcgccaatgctgcccacggagaagcagtggtcgccagggttcacagccccggtcagcacctggtgcaggttcatgtcggcgccctagtctacgcgcctctggatccctgcggccgaaatatcgcgagacttcgctcggggcagctgctactgtggtaaagaattcacttttttaccacagcgtgc

SEQ ID NO: 9974 - RNA, 10029 nt, Homo sapiens
  source 1..10029: mol_type = other RNA
cacacacacacacacacgtatacatacatacaacttgggttccggagggtaaactactgaaaaccttacatattgagccatctagctcatttatcactgacgtctcaatgacaattttaatgaagatgttcattatttttttcattcttactcaaatacctatcattaattaagagaagagtttgagatgtataaggctaataaaggaagtgagagtgtggtgaattaagtgatgagtattatgtacaattgcctttacaaaaaacgtatttttactgtggaagaaattcatgcagagatgcctgtggaaaagtatcaataagaaaacaaaacacctttaacactatgacatactgattataatatactatgatatgtattattacagcattacttacacattctactttaggcaatgtaatctacttctgaatgaccttgttaatttttaaggcatcagtgcatcaagggcaaagctccataaaataaatataaaaacaagaaagcattagctaatttgtggcatagagaatgatcactgtatattatatctgttggccacttccatataggtaataaattgtacatcttattgtaaaaatgttatagcataaatttcacatcatttttcaacacttcatttaaagggctaaactgatctggcagtattctcattttcattgttccatcagctccacaggagaaaatgtgatttgcaggccctgtctcaatttgcatcactccagttccaatatttctaaaaatggactgccgagcatgttcactgacaaaagtatggagaagaccaaaggtagagagactccaaatctttatattgccttcggcagatcctgtaacaaagtactcttcagttggatcaacagcaacggctttaacaggagaatcatggctctggaaaagctgcctctgttgtcgttgacaaaggtcaaatacatatgtaaaaccttttctgccacctgatattagtagctgatgttttggagcatatgctaaaactgtggctccactgtcatggcaggtaaatgcatggactaaactattggcaggtgctacaagagtatcccacaaacatacgtttctattgtcagttgaaagaccagctgtagctatcagagaggaggaactaacgaagacaaaatcattggctgttttgttatgacactgccaagtcaggtatggcttaggcatgcttccagtaactggacaacatttccagtttgtttgatacaaacttaaatatccatcagcatcaactattccaaacttatttccctgatagttaaatctcattcttgtaactcttgaattgccaccagatcgaaaacaggttatttgttgagaatggccccattcaaacattctgacacttccatcttgagctcctgtcagatagtaaggaagagttggatgagaagtcattcttctaacattattaatggctttcttaatcatcacagatgctcctctgccagtctgtgtactaccaagccatggcatgttgattggagtgccaggattgctatgtgtatatggagttgtaccttgaacagctgttaaatcatcacgagcatgtataaccaagaaatcttctgatcctttggtttccacttctatatcatcatctacccaagtgtagacctgtgtggccagaattccagaaacatccagttcttgaacatcatgactggaagcgattgctatgcagtttctatttgccttattaacagcaaacgcagtaatgatatcagattccttatgaataattcttgctttacctccaggatatcccaaatctgcttctatcttattgatgtttggctcctccatcatagaatttttgatggtttcactgttgtcctctaatgactcatttagacaccgtttctttgtgaatatatttttgataaaggtttcctgaatttcttcctgcttcaccaaatactgccaaagcctcttcacagacagtgccagatggtgtttggatttgaaaggagtgtttgtaggttccagtaaagctttgtggcgaagaattgcaggacctgcagacaaactctcttcggcggtatgacttgcgatataattttgaggtggcccaccatggatttcaagtcgtcggagaagaacttgttcccaacattgaagagtttttagaaccgcatgacaaagaggtgaactaactggaagctctgcaagatcatgacctgcgaagggataaaaagtcttcaaattgttgagcaccaattgcaccatcgccaaccgcatcaaggaccaactatatgaatttgaattagaatgttcctggagatggaaatctgatgctaaaacatcatcatcatcatcattgtcatcatcatcacttcccagactctcctctgaatcatattcggctctactttgagaagagggtagaaaaggcttagctatgaaatagtcccagatactgagctcaggtgggatgaacttttctttaaccgccagtgactcctggcttactggtgccgaggaaggggtcagtggggcagattctctgcaagacatttttgacggcctaaaacgtttgttctgtttttctccttcttcaactagtgaagaaactgcaagactgggagggctatgagaactgatggctgaaagagctttggaaaagcccacacattccatggagaataccactacctggtgggggctaggcatagcaaagtgccttccaggtaaagtttttgaatgtgtctgttctttgctaggaacatgtgcacctccaccaaacacagcagaccacattttctcatttagaggatgggccacaatccgaaatagctcattacttgaatgtgtggccaggccatggatgaagagactaagatacactgctgtgagaatctcacagagcaagactgtaagccctgactgggcttcctcgccagaagaattcaaaagtcgaattagacaagttattcctggccattgagctggtgacgtattgggagttaatgcttcatctaagcttcctgttttcaaagaaggtcgatgaggaagcagtactgtctgatataccattccagtaaactgattcgtctgaaatgaactgtagttatgactaccacaaaggcactgataaatacaagcagaaagtgaagctgctaaagtatgcattacatacactttattgctttggatatcagggtggggtggtgaatcaaagtttattatggcatggagaatatcatgtgtcagattactaaggtgcaataatggattggcaactactgttttggcattggctgtacaagcaaagaggagaggcactgaggtttgctctgacagagggctagaaaatagtggttctgatgtttcctgctgagattcttgcaaaagcaaaatcaattccattcttacagatgcaagacccccaccatgggatccatgaagtatgcagtaactaagaaacattctcaaaagtgactgatacttcaagagccactgtcttttttcctgaaaattttctctcagttgtttcacttttgtttggtgaggcaaatcttcagcatcctcatttaatccaaattcatcttcatttctgccaaatgcagactgtagttcttcagcatctgagcaaaagtcacaagtcctctgaagagctatcacctctttttcaagccagtggtatagttggtaacgcaattttccaccatctatttcatagccagtagataaagtacgaagttctactgtgagaatctttaaacatgctctaaattttaactgaactgcaattatatcttctgatggatttaaaaggtcattttcatctagtgtgctgaaagattctgtgtagttagaacttatgtcatccaactttttatctgtttttctctgtaaaggttttagttctttcattgaaatagggacatcctcattttcttcatcattatcactgtcccattttaactctaaagagtcatcctgaaacacaacacttggttggctccagtcaaaagaaagagtggagtttgattgcttctctgaggaaccctctgaagaagatccaaaaccatttatcagtgactgtgaccaatcaacagcagaagacttatcttcccttgcatccaactttaatggagaagaaggagaacagtctttactagtatccagaaaactagaagccctataaaaaggtcttgttttcttgatgactttaggcatctttgataatacttccaaagccaacattgggcagccagcttttaaatgagcactggcagtggtaaaaaataaacgtctttcacttaaattaattgttcctgccagtccactttttcctgttaggctcatatgtgtggaaaatgtatcagatgatccaaaatgacgtctcagcaaaagaggatgtgttcttagataattgtagaaattaaaaactgtaggattactggctgataaaacttgatcatcattctctctgataggttgctttattaatgtttccagagcaccactataatcttccaaaatccaatatgccatgctccgaagaaaaggatcatgatgcatatttatgttcaatgaacacagttcactgacaggagaatcgattcccaaaacttttttacgtaaaatagatttatatgctgcagatgtatcaaattcagactcatagagtcttgctattacaagagccaactgaatgtcattcaatttctcaagacatacctcaattgcatctctgaggcaaccagctaaaagaaaaaatgctgcagaatgttcaaatctttgtttgcctagcaaagaaaaagcattctttaaagctgctttacgccacctctcatcctcaaaattgtgtccaaaaaactgtgtcatcctggtgtttttttcagctctatataatccccaaatcacagctttctttttcattgcaaggtaaaaaatggcagcatctaaaggatcattctttctataaaaggctgctttagctactttttctatgcatttgcgtaagatgcgggtattccggacccaccaccccacacccatagctcttagttcagaccaagtgggatcatctttctgcatggctggcaacatgttcagcagttcttcttctgctactgagtgaaatgcccaagcaaaatgacttgtagacaggccttggtgaaggagttgagctcgataggctggaagggaagttgtaagaaaggtatggagtcgaacagccaaaagaaattttaacccacattcatcaagagtttctccaccttggcttctgtctcggctttctccaatatcagtgcttgtagttgcaattgtatctgctaaggccatcaaagacatctgctccatccggctgagtcctggtaaactagaatgaagtaagtggccagaaagaacctgagcatgctcaggtccaaagtaagtcggactgtactgtgaaaggtcaataactctaggctttgtattttcttcatctgtctctaacatatgagtatcagtcattagaagttgagtctgaaaaagctcatcataactttctttagataattggtttgatttacttaacgtactctcattactagatttctccaaagatgagtaacagctatcatcatctgctgcaagtaaggcatataaaggaagtggaggaacagaatctatttctgtgtaatctgtattttcagccttgttgaatgcctgggggtctctggtagtgcttccactagcactgattgtgagagacctaaggcggcgttcatgattagattcagcttcattcagagccacaacttccccagcaatgcacttaacaagatgggacaagatggccttggctctccgaactttaccaagatccatgagttccaaaagctgcaagggatgatactgaggtagagtcggggaaagtacatgagctgcttcaaaaagacctgaatcttccatatccactgaaggatcgaatgcagttttctttccacagattttctgtgcaagactggtcatggatcgagtcagagttttctttggaggatgtaacccagaactggagttactctgttttattaaacttgttatagatggagtgctcccactgtacgaatctgttataacaggttcttgtttagaagatggttgccattggcaatacacatgcatttcacagtccattcctaccacaaggatgccatcccggacccacgataaagaaacaggaaaaggtggggagccatctacagaagaaactaggtccacacttcgtaatagtacaaatttagaaaggggcacaactttggtactctcccagagaggaaatgccagggtttccttaccagtttggtcttgtaccttgccagccaggggtccatacataaaaagttttgatccaattcctacagtcaggatatgagaaccgtcttctctagacatccaatctaagtgaactaaatgctttgtgtttgatgtgatattctctttactagataaatacatgtcttgtttattataggccactaaattgctatcaacactaatgccagaatccaatactgtgcttaactcatctaaatgaattgtctgctcaaggacccaacatgaacctcctgttgactcacattcaaaaatacttacatgcatcacaaagtcctgggaagatctactattagatgcaggctgcttataagctactgctaaacgatttgtatgtgcacagctaacttctacaggcctaccaggtacagttatactactattgctctgaagtccatcttcaataagtaatggccattcttcccaaatgtatgcaagatcaatttttccattctttgacgtggcagattctccatctgttactctgcatctccagaatcttactttctcatctgaacatgaagttgccaataaataaggagcactgcatgcaggatatatagaagatgaactcagatgtcctgctgatggcttaatacttattatctcaactccttctggtaaatgcaattcttggctataaaccatttctgaaaacagagtcaacctgctggtactctggagatttgctctgcaagcctgatacttttgtgaaaaaggagataggatcttctctggagaagaagaataatgttcttctggctgccaaaccgcttcggataattttgtatctactttttcatctaatgagacaggaattgactttagatgtaaattccacatgtgtaacagtgaacggttgtcttgagtgcattctattacaattaggtagaacttctcagaaaatccattaggtgagctgcctgcattagataaaatgctgtctttgccaaggcttttcttctcaaggttattcaaaatgaagtcttcttcaaaaacatgaagcagttgggtttttctgccatgaagtttggtaatgggatctaatgcaataatgcatcctggcctggctgttgattgttgactgacgatgttaaagacttcaccaacatatttagaaatttcagggttagaaagctcagataaaagtttcttagcatcaataactgcttcatataatctcagatattgtccatcactggctacaaagcatgcactaggagagttgcagtatgcacccagacaataactgggtataagagtgggcagccatgccacattggaaaaggcagaaacatgaagagaattaatccgggcaagctcagaaactcctccagaaaaagacaatggcccaactgggtcaaccctccacagaataagctcactgtaaactgcactgggatcctgaaatgccacgtcaacagtgcttttattttgttgtgtcaaagagcattcttcaatatttagagcatcaaaaggttgctctgggttatcaacatctggtgtccttaatgcattatggtgtgatgttgtcagcaataatggtaatactgagtggcaagctaaatcattaagatgaaaacgatgaccacaatatctggatttgtgggaaatactgagaacagtagaaaaagcagattcctcggcaaaactgaccagccactgattcagagaaccatcagcatgttttgatatcatcataacattaggcgtaaaaatacttaattttaaactattagatgatttattgtgaccagaagaaataagcattgatgtggaacgggtgaggccagaaggtttttgtttcccctgctgaatagccaagtcaacattcttggtacaggcatacatcattatgcttttacagagagagtttgcatcacctgtggggaaagctactggaattctggaaacaaaggacacctgtacttgacgaaacataccaggctggtattcatccagccaatccacatgccaaactagcaaagaaccatccatgggatgaatactaaatagcatatctgcatttttactccattcagacagaagtacttcaatctgatgatcaatggcagctgacgataatgatgtaaaacttgagtttggtaccattttatcacagcctaattccttcttttcgggatttattttcagatcatcaacaccatcatcagtttcttcatcagattttacatctgcctgattagaatcttctacactggcctcagaagatggttgttcaaaactttttctaagttgctgtaaaaaaacttccatggacaaagtaaaatgcagttctttattgtttagccagtgtacaacaaaaggtccggtcttctcttcattttcatttagactcagagatgtaatagatggaagaagtggaatgtctgtggctgggttgatgctggctgcaatatgaaagtggcaaagtgcattggcatgcagtggagtgttcctgtgaacatgatgaggatcctgctgatgtggtagatatcccgtatgtgctacaagagcaagtgatctcctccgacctctacgaaaatgtctcagatttacttctaaagcattttgaactcgttctttactggaagcatttctcttgaagttatttgttaaattaattgattcagtccaatggctgcagtcacctccgtatagcaaacaatcatttggtaaaaatgtctctacccaaagacgacacacattatctttgcagcaagtcaacagtacattacatacagaagccctaggcatatatttgcttgttttacgccaggaaaatccatttactgctcgaggatgggccagatacacaaaagaaaagtcaatttctccttgggattgtttttctgaacttccatctggagaagtaacagctgtccgccagttttctacattataccaaaccttcaaaagacagtcatccttcccagcagtggcaaaaaattctccatctggtgaaaatttcattaaatgaacttgggaagcagttttgcaatgccaaatgcatttccaatctccaaagttaagatctgttttatttaaattttcatcttcagttggcttctccaagttagtattggaccagagttgcaaatagctggaaccagttaaaagacgactgcctgtgggatcccaggttatattgtgtgctattgattccagaaaaaattggccacttttctgccactgactatataattccaaatttttcttttgttttggtaggttaactggttcaaaaatggagataacatttccataagacgctgcaatcttgccttgttgcattgaacagtctacacatcccacttgaatatttccatgtttagctcctgggattatctgtaatctttcaaaatcgcttcccagtattacaatgtcacatccagatgcataagcctctggttaaaattggtaaagtctaagttggtcttcaatctttgtttctgcggctctatatcttcttcacattaacttctcatctacacttcttgcatccaacacttaggagttcttattcctccgtgaagcgctggtcgccaatgctgcccacggagaagcagtggtcgccagggttcacagccccggtcagcacctggtgcaggttcatgtcggcgccctagtcctgcaacggacaccgcatccagctca

SEQ ID NO: 9975 - RNA, 10224 nt, Homo sapiens
  source 1..10224: mol_type = other RNA
cacacacacacacacacgtatacatacatacaacttgggttccggagggtaaactactgaaaaccttacatattgagccatctagctcatttatcactgacgtctcaatgacaattttaatgaagatgttcattatttttttcattcttactcaaatacctatcattaattaagagaagagtttgagatgtataaggctaataaaggaagtgagagtgtggtgaattaagtgatgagtattatgtacaattgcctttacaaaaaacgtatttttactgtggaagaaattcatgcagagatgcctgtggaaaagtatcaataagaaaacaaaacacctttaacactatgacatactgattataatatactatgatatgtattattacagcattacttacacattctactttaggcaatgtaatctacttctgaatgaccttgttaatttttaaggcatcagtgcatcaagggcaaagctccataaaataaatataaaaacaagaaagcattagctaatttgtggcatagagaatgatcactgtatattatatctgttggccacttccatataggtaataaattgtacatcttattgtaaaaatgttatagcataaatttcacatcatttttcaacacttcatttaaagggctaaactgatctggcagtattctcattttcattgttccatcagctccacaggagaaaatgtgatttgcaggccctgtctcaatttgcatcactccagttccaatatttctaaaaatggactgccgagcatgttcactgacaaaagtatggagaagaccaaaggtagagagactccaaatctttatattgccttcggcagatcctgtaacaaagtactcttcagttggatcaacagcaacggctttaacaggagaatcatggctctggaaaagctgcctctgttgtcgttgacaaaggtcaaatacatatgtaaaaccttttctgccacctgatattagtagctgatgttttggagcatatgctaaaactgtggctccactgtcatggcaggtaaatgcatggactaaactattggcaggtgctacaagagtatcccacaaacatacgtttctattgtcagttgaaagaccagctgtagctatcagagaggaggaactaacgaagacaaaatcattggctgttttgttatgacactgccaagtcaggtatggcttaggcatgcttccagtaactggacaacatttccagtttgtttgatacaaacttaaatatccatcagcatcaactattccaaacttatttccctgatagttaaatctcattcttgtaactcttgaattgccaccagatcgaaaacaggttatttgttgagaatggccccattcaaacattctgacacttccatcttgagctcctgtcagatagtaaggaagagttggatgagaagtcattcttctaacattattaatggctttcttaatcatcacagatgctcctctgccagtctgtgtactaccaagccatggcatgttgattggagtgccaggattgctatgtgtatatggagttgtaccttgaacagctgttaaatcatcacgagcatgtataaccaagaaatcttctgatcctttggtttccacttctatatcatcatctacccaagtgtagacctgtgtggccagaattccagaaacatccagttcttgaacatcatgactggaagcgattgctatgcagtttctatttgccttattaacagcaaacgcagtaatgatatcagattccttatgaataattcttgctttacctccaggatatcccaaatctgcttctatcttattgatgtttggctcctccatcatagaatttttgatggtttcactgttgtcctctaatgactcatttagacaccgtttctttgtgaatatatttttgataaaggtttcctgaatttcttcctgcttcaccaaatactgccaaagcctcttcacagacagtgccagatggtgtttggatttgaaaggagtgtttgtaggttccagtaaagctttgtggcgaagaattgcaggacctgcagacaaactctcttcggcggtatgacttgcgatataattttgaggtggcccaccatggatttcaagtcgtcggagaagaacttgttcccaacattgaagagtttttagaaccgcatgacaaagaggtgaactaactggaagctctgcaagatcatgacctgcgaagggataaaaagtcttcaaattgttgagcaccaattgcaccatcgccaaccgcatcaaggaccaactatatgaatttgaattagaatgttcctggagatggaaatctgatgctaaaacatcatcatcatcatcattgtcatcatcatcacttcccagactctcctctgaatcatattcggctctactttgagaagagggtagaaaaggcttagctatgaaatagtcccagatactgagctcaggtgggatgaacttttctttaaccgccagtgactcctggcttactggtgccgaggaaggggtcagtggggcagattctctgcaagacatttttgacggcctaaaacgtttgttctgtttttctccttcttcaactagtgaagaaactgcaagactgggagggctatgagaactgatggctgaaagagctttggaaaagcccacacattccatggagaataccactacctggtgggggctaggcatagcaaagtgccttccaggtaaagtttttgaatgtgtctgttctttgctaggaacatgtgcacctccaccaaacacagcagaccacattttctcatttagaggatgggccacaatccgaaatagctcattacttgaatgtgtggccaggccatggatgaagagactaagatacactgctgtgagaatctcacagagcaagactgtaagccctgactgggcttcctcgccagaagaattcaaaagtcgaattagacaagttattcctggccattgagctggtgacgtattgggagttaatgcttcatctaagcttcctgttttcaaagaaggtcgatgaggaagcagtactgtctgatataccattccagtaaactgattcgtctgaaatgaactgtagttatgactaccacaaaggcactgataaatacaagcagaaagtgaagctgctaaagtatgcattacatacactttattgctttggatatcagggtggggtggtgaatcaaagtttattatggcatggagaatatcatgtgtcagattactaaggtgcaataatggattggcaactactgttttggcattggctgtacaagcaaagaggagaggcactgaggtttgctctgacagagggctagaaaatagtggttctgatgtttcctgctgagattcttgcaaaagcaaaatcaattccattcttacagatgcaagacccccaccatgggatccatgaagtatgcagtaactaagaaacattctcaaaagtgactgatacttcaagagccactgtcttttttcctgaaaattttctctcagttgtttcacttttgtttggtgaggcaaatcttcagcatcctcatttaatccaaattcatcttcatttctgccaaatgcagactgtagttcttcagcatctgagcaaaagtcacaagtcctctgaagagctatcacctctttttcaagccagtggtatagttggtaacgcaattttccaccatctatttcatagccagtagataaagtacgaagttctactgtgagaatctttaaacatgctctaaattttaactgaactgcaattatatcttctgatggatttaaaaggtcattttcatctagtgtgctgaaagattctgtgtagttagaacttatgtcatccaactttttatctgtttttctctgtaaaggttttagttctttcattgaaatagggacatcctcattttcttcatcattatcactgtcccattttaactctaaagagtcatcctgaaacacaacacttggttggctccagtcaaaagaaagagtggagtttgattgcttctctgaggaaccctctgaagaagatccaaaaccatttatcagtgactgtgaccaatcaacagcagaagacttatcttcccttgcatccaactttaatggagaagaaggagaacagtctttactagtatccagaaaactagaagccctataaaaaggtcttgttttcttgatgactttaggcatctttgataatacttccaaagccaacattgggcagccagcttttaaatgagcactggcagtggtaaaaaataaacgtctttcacttaaattaattgttcctgccagtccactttttcctgttaggctcatatgtgtggaaaatgtatcagatgatccaaaatgacgtctcagcaaaagaggatgtgttcttagataattgtagaaattaaaaactgtaggattactggctgataaaacttgatcatcattctctctgataggttgctttattaatgtttccagagcaccactataatcttccaaaatccaatatgccatgctccgaagaaaaggatcatgatgcatatttatgttcaatgaacacagttcactgacaggagaatcgattcccaaaacttttttacgtaaaatagatttatatgctgcagatgtatcaaattcagactcatagagtcttgctattacaagagccaactgaatgtcattcaatttctcaagacatacctcaattgcatctctgaggcaaccagctaaaagaaaaaatgctgcagaatgttcaaatctttgtttgcctagcaaagaaaaagcattctttaaagctgctttacgccacctctcatcctcaaaattgtgtccaaaaaactgtgtcatcctggtgtttttttcagctctatataatccccaaatcacagctttctttttcattgcaaggtaaaaaatggcagcatctaaaggatcattctttctataaaaggctgctttagctactttttctatgcatttgcgtaagatgcgggtattccggacccaccaccccacacccatagctcttagttcagaccaagtgggatcatctttctgcatggctggcaacatgttcagcagttcttcttctgctactgagtgaaatgcccaagcaaaatgacttgtagacaggccttggtgaaggagttgagctcgataggctggaagggaagttgtaagaaaggtatggagtcgaacagccaaaagaaattttaacccacattcatcaagagtttctccaccttggcttctgtctcggctttctccaatatcagtgcttgtagttgcaattgtatctgctaaggccatcaaagacatctgctccatccggctgagtcctggtaaactagaatgaagtaagtggccagaaagaacctgagcatgctcaggtccaaagtaagtcggactgtactgtgaaaggtcaataactctaggctttgtattttcttcatctgtctctaacatatgagtatcagtcattagaagttgagtctgaaaaagctcatcataactttctttagataattggtttgatttacttaacgtactctcattactagatttctccaaagatgagtaacagctatcatcatctgctgcaagtaaggcatataaaggaagtggaggaacagaatctatttctgtgtaatctgtattttcagccttgttgaatgcctgggggtctctggtagtgcttccactagcactgattgtgagagacctaaggcggcgttcatgattagattcagcttcattcagagccacaacttccccagcaatgcacttaacaagatgggacaagatggccttggctctccgaactttaccaagatccatgagttccaaaagctgcaagggatgatactgaggtagagtcggggaaagtacatgagctgcttcaaaaagacctgaatcttccatatccactgaaggatcgaatgcagttttctttccacagattttctgtgcaagactggtcatggatcgagtcagagttttctttggaggatgtaacccagaactggagttactctgttttattaaacttgttatagatggagtgctcccactgtacgaatctgttataacaggttcttgtttagaagatggttgccattggcaatacacatgcatttcacagtccattcctaccacaaggatgccatcccggacccacgataaagaaacaggaaaaggtggggagccatctacagaagaaactaggtccacacttcgtaatagtacaaatttagaaaggggcacaactttggtactctcccagagaggaaatgccagggtttccttaccagtttggtcttgtaccttgccagccaggggtccatacataaaaagttttgatccaattcctacagtcaggatatgagaaccgtcttctctagacatccaatctaagtgaactaaatgctttgtgtttgatgtgatattctctttactagataaatacatgtcttgtttattataggccactaaattgctatcaacactaatgccagaatccaatactgtgcttaactcatctaaatgaattgtctgctcaaggacccaacatgaacctcctgttgactcacattcaaaaatacttacatgcatcacaaagtcctgggaagatctactattagatgcaggctgcttataagctactgctaaacgatttgtatgtgcacagctaacttctacaggcctaccaggtacagttatactactattgctctgaagtccatcttcaataagtaatggccattcttcccaaatgtatgcaagatcaatttttccattctttgacgtggcagattctccatctgttactctgcatctccagaatcttactttctcatctgaacatgaagttgccaataaataaggagcactgcatgcaggatatatagaagatgaactcagatgtcctgctgatggcttaatacttattatctcaactccttctggtaaatgcaattcttggctataaaccatttctgaaaacagagtcaacctgctggtactctggagatttgctctgcaagcctgatacttttgtgaaaaaggagataggatcttctctggagaagaagaataatgttcttctggctgccaaaccgcttcggataattttgtatctactttttcatctaatgagacaggaattgactttagatgtaaattccacatgtgtaacagtgaacggttgtcttgagtgcattctattacaattaggtagaacttctcagaaaatccattaggtgagctgcctgcattagataaaatgctgtctttgccaaggcttttcttctcaaggttattcaaaatgaagtcttcttcaaaaacatgaagcagttgggtttttctgccatgaagtttggtaatgggatctaatgcaataatgcatcctggcctggctgttgattgttgactgacgatgttaaagacttcaccaacatatttagaaatttcagggttagaaagctcagataaaagtttcttagcatcaataactgcttcatataatctcagatattgtccatcactggctacaaagcatgcactaggagagttgcagtatgcacccagacaataactgggtataagagtgggcagccatgccacattggaaaaggcagaaacatgaagagaattaatccgggcaagctcagaaactcctccagaaaaagacaatggcccaactgggtcaaccctccacagaataagctcactgtaaactgcactgggatcctgaaatgccacgtcaacagtgcttttattttgttgtgtcaaagagcattcttcaatatttagagcatcaaaaggttgctctgggttatcaacatctggtgtccttaatgcattatggtgtgatgttgtcagcaataatggtaatactgagtggcaagctaaatcattaagatgaaaacgatgaccacaatatctggatttgtgggaaatactgagaacagtagaaaaagcagattcctcggcaaaactgaccagccactgattcagagaaccatcagcatgttttgatatcatcataacattaggcgtaaaaatacttaattttaaactattagatgatttattgtgaccagaagaaataagcattgatgtggaacgggtgaggccagaaggtttttgtttcccctgctgaatagccaagtcaacattcttggtacaggcatacatcattatgcttttacagagagagtttgcatcacctgtggggaaagctactggaattctggaaacaaaggacacctgtacttgacgaaacataccaggctggtattcatccagccaatccacatgccaaactagcaaagaaccatccatgggatgaatactaaatagcatatctgcatttttactccattcagacagaagtacttcaatctgatgatcaatggcagctgacgataatgatgtaaaacttgagtttggtaccattttatcacagcctaattccttcttttcgggatttattttcagatcatcaacaccatcatcagtttcttcatcagattttacatctgcctgattagaatcttctacactggcctcagaagatggttgttcaaaactttttctaagttgctgtaaaaaaacttccatggacaaagtaaaatgcagttctttattgtttagccagtgtacaacaaaaggtccggtcttctcttcattttcatttagactcagagatgtaatagatggaagaagtggaatgtctgtggctgggttgatgctggctgcaatatgaaagtggcaaagtgcattggcatgcagtggagtgttcctgtgaacatgatgaggatcctgctgatgtggtagatatcccgtatgtgctacaagagcaagtgatctcctccgacctctacgaaaatgtctcagatttacttctaaagcattttgaactcgttctttactggaagcatttctcttgaagttatttgttaaattaattgattcagtccaatggctgcagtcacctccgtatagcaaacaatcatttggtaaaaatgtctctacccaaagacgacacacattatctttgcagcaagtcaacagtacattacatacagaagccctaggcatatatttgcttgttttacgccaggaaaatccatttactgctcgaggatgggccagatacacaaaagaaaagtcaatttctccttgggattgtttttctgaacttccatctggagaagtaacagctgtccgccagttttctacattataccaaaccttcaaaagacagtcatccttcccagcagtggcaaaaaattctccatctggtgaaaatttcattaaatgaacttgggaagcagttttgcaatgccaaatgcatttccaatctccaaagttaagatctgttttatttaaattttcatcttcagttggcttctccaagttagtattggaccagagttgcaaatagctggaaccagttaaaagacgactgcctgtgggatcccaggttatattgtgtgctattgattccagaaaaaattggccacttttctgccactgactatataattccaaatttttcttttgttttggtaggttaactggttcaaaaatggagataacatttccataagacgctgcaatcttgccttgttgcattgaacagtctacacatcccacttgaatatttccatgtttagctcctgggattatctgtaatctttcaaaatcgcttcccagtattacaatgtcacatccagatgcataagcctctggttaaaattggtaaagtctaagttggtcttcaatctttgtttctgcggctctatatcttcttcacattaacttctcatctacacttcttgcatccaacacttaggagttcttattcctccgtgaagcgctggtcgccaatgctgcccacggagaagcagtggtcgccagggttcacagccccggtcagcacctggtgcaggttcatgtcggcgccctagtcctgtcactccccgcgctagcccaggtgaagctcagggtcccctcaccggccacgacccggggccgactcaccggccaggaaggccgcgctgtccacacacttcctctggacctcgggcagccgctcctgacccagcccgagtggcgcaagcagtacgcgctcgcactccccgcctgacctgtcccttcccggctccggtgcccgccacccccacagtcctc

SEQ ID NO: 9976 - RNA, 9797 nt, Homo sapiens
  source 1..9797: mol_type = other RNA
cacacacacacacacacgtatacatacatacaacttgggttccggagggtaaactactgaaaaccttacatattgagccatctagctcatttatcactgacgtctcaatgacaattttaatgaagatgttcattatttttttcattcttactcaaatacctatcattaattaagagaagagtttgagatgtataaggctaataaaggaagtgagagtgtggtgaattaagtgatgagtattatgtacaattgcctttacaaaaaacgtatttttactgtggaagaaattcatgcagagatgcctgtggaaaagtatcaataagaaaacaaaacacctttaacactatgacatactgattataatatactatgatatgtattattacagcattacttacacattctactttaggcaatgtaatctacttctgaatgaccttgttaatttttaaggcatcagtgcatcaagggcaaagctccataaaataaatataaaaacaagaaagcattagctaatttgtggcatagagaatgatcactgtatattatatctgttggccacttccatataggtaataaattgtacatcttattgtaaaaatgttatagcataaatttcacatcatttttcaacacttcatttaaagggctaaactgatctggcagtattctcattttcattgttccatcagctccacaggagaaaatgtgatttgcaggccctgtctcaatttgcatcactccagttccaatatttctaaaaatggactgccgagcatgttcactgacaaaagtatggagaagaccaaaggtagagagactccaaatctttatattgccttcggcagatcctgtaacaaagtactcttcagttggatcaacagcaacggctttaacaggagaatcatggctctggaaaagctgcctctgttgtcgttgacaaaggtcaaatacatatgtaaaaccttttctgccacctgatattagtagctgatgttttggagcatatgctaaaactgtggctccactgtcatggcaggtaaatgcatggactaaactattggcaggtgctacaagagtatcccacaaacatacgtttctattgtcagttgaaagaccagctgtagctatcagagaggaggaactaacgaagacaaaatcattggctgttttgttatgacactgccaagtcaggtatggcttaggcatgcttccagtaactggacaacatttccagtttgtttgatacaaacttaaatatccatcagcatcaactattccaaacttatttccctgatagttaaatctcattcttgtaactcttgaattgccaccagatcgaaaacaggttatttgttgagaatggccccattcaaacattctgacacttccatcttgagctcctgtcagatagtaaggaagagttggatgagaagtcattcttctaacattattaatggctttcttaatcatcacagatgctcctctgccagtctgtgtactaccaagccatggcatgttgattggagtgccaggattgctatgtgtatatggagttgtaccttgaacagctgttaaatcatcacgagcatgtataaccaagaaatcttctgatcctttggtttccacttctatatcatcatctacccaagtgtagacctgtgtggccagaattccagaaacatccagttcttgaacatcatgactggaagcgattgctatgcagtttctatttgccttattaacagcaaacgcagtaatgatatcagattccttatgaataattcttgctttacctccaggatatcccaaatctgcttctatcttattgatgtttggctcctccatcatagaatttttgatggtttcactgttgtcctctaatgactcatttagacaccgtttctttgtgaatatatttttgataaaggtttcctgaatttcttcctgcttcaccaaatactgccaaagcctcttcacagacagtgccagatggtgtttggatttgaaaggagtgtttgtaggttccagtaaagctttgtggcgaagaattgcaggacctgcagacaaactctcttcggcggtatgacttgcgatataattttgaggtggcccaccatggatttcaagtcgtcggagaagaacttgttcccaacattgaagagtttttagaaccgcatgacaaagaggtgaactaactggaagctctgcaagatcatgacctgcgaagggataaaaagtcttcaaattgttgagcaccaattgcaccatcgccaaccgcatcaaggaccaactatatgaatttgaattagaatgttcctggagatggaaatctgatgctaaaacatcatcatcatcatcattgtcatcatcatcacttcccagactctcctctgaatcatattcggctctactttgagaagagggtagaaaaggcttagctatgaaatagtcccagatactgagctcaggtgggatgaacttttctttaaccgccagtgactcctggcttactggtgccgaggaaggggtcagtggggcagattctctgcaagacatttttgacggcctaaaacgtttgttctgtttttctccttcttcaactagtgaagaaactgcaagactgggagggctatgagaactgatggctgaaagagctttggaaaagcccacacattccatggagaataccactacctggtgggggctaggcatagcaaagtgccttccaggtaaagtttttgaatgtgtctgttctttgctaggaacatgtgcacctccaccaaacacagcagaccacattttctcatttagaggatgggccacaatccgaaatagctcattacttgaatgtgtggccaggccatggatgaagagactaagatacactgctgtgagaatctcacagagcaagactgtaagccctgactgggcttcctcgccagaagaattcaaaagtcgaattagacaagttattcctggccattgagctggtgacgtattgggagttaatgcttcatctaagcttcctgttttcaaagaaggtcgatgaggaagcagtactgtctgatataccattccagtaaactgattcgtctgaaatgaactgtagttatgactaccacaaaggcactgataaatacaagcagaaagtgaagctgctaaagtatgcattacatacactttattgctttggatatcagggtggggtggtgaatcaaagtttattatggcatggagaatatcatgtgtcagattactaaggtgcaataatggattggcaactactgttttggcattggctgtacaagcaaagaggagaggcactgaggtttgctctgacagagggctagaaaatagtggttctgatgtttcctgctgagattcttgcaaaagcaaaatcaattccattcttacagatgcaagacccccaccatgggatccatgaagtatgcagtaactaagaaacattctcaaaagtgactgatacttcaagagccactgtcttttttcctgaaaattttctctcagttgtttcacttttgtttggtgaggcaaatcttcagcatcctcatttaatccaaattcatcttcatttctgccaaatgcagactgtagttcttcagcatctgagcaaaagtcacaagtcctctgaagagctatcacctctttttcaagccagtggtatagttggtaacgcaattttccaccatctatttcatagccagtagataaagtacgaagttctactgtgagaatctttaaacatgctctaaattttaactgaactgcaattatatcttctgatggatttaaaaggtcattttcatctagtgtgctgaaagattctgtgtagttagaacttatgtcatccaactttttatctgtttttctctgtaaaggttttagttctttcattgaaatagggacatcctcattttcttcatcattatcactgtcccattttaactctaaagagtcatcctgaaacacaacacttggttggctccagtcaaaagaaagagtggagtttgattgcttctctgaggaaccctctgaagaagatccaaaaccatttatcagtgactgtgaccaatcaacagcagaagacttatcttcccttgcatccaactttaatggagaagaaggagaacagtctttactagtatccagaaaactagaagccctataaaaaggtcttgttttcttgatgactttaggcatctttgataatacttccaaagccaacattgggcagccagcttttaaatgagcactggcagtggtaaaaaataaacgtctttcacttaaattaattgttcctgccagtccactttttcctgttaggctcatatgtgtggaaaatgtatcagatgatccaaaatgacgtctcagcaaaagaggatgtgttcttagataattgtagaaattaaaaactgtaggattactggctgataaaacttgatcatcattctctctgataggttgctttattaatgtttccagagcaccactataatcttccaaaatccaatatgccatgctccgaagaaaaggatcatgatgcatatttatgttcaatgaacacagttcactgacaggagaatcgattcccaaaacttttttacgtaaaatagatttatatgctgcagatgtatcaaattcagactcatagagtcttgctattacaagagccaactgaatgtcattcaatttctcaagacatacctcaattgcatctctgaggcaaccagctaaaagaaaaaatgctgcagaatgttcaaatctttgtttgcctagcaaagaaaaagcattctttaaagctgctttacgccacctctcatcctcaaaattgtgtccaaaaaactgtgtcatcctggtgtttttttcagctctatataatccccaaatcacagctttctttttcattgcaaggtaaaaaatggcagcatctaaaggatcattctttctataaaaggctgctttagctactttttctatgcatttgcgtaagatgcgggtattccggacccaccaccccacacccatagctcttagttcagaccaagtgggatcatctttctgcatggctggcaacatgttcagcagttcttcttctgctactgagtgaaatgcccaagcaaaatgacttgtagacaggccttggtgaaggagttgagctcgataggctggaagggaagttgtaagaaaggtatggagtcgaacagccaaaagaaattttaacccacattcatcaagagtttctccaccttggcttctgtctcggctttctccaatatcagtgcttgtagttgcaattgtatctgctaaggccatcaaagacatctgctccatccggctgagtcctggtaaactagaatgaagtaagtggccagaaagaacctgagcatgctcaggtccaaagtaagtcggactgtactgtgaaaggtcaataactctaggctttgtattttcttcatctgtctctaacatatgagtatcagtcattagaagttgagtctgaaaaagctcatcataactttctttagataattggtttgatttacttaacgtactctcattactagatttctccaaagatgagtaacagctatcatcatctgctgcaagtaaggcatataaaggaagtggaggaacagaatctatttctgtgtaatctgtattttcagccttgttgaatgcctgggggtctctggtagtgcttccactagcactgattgtgagagacctaaggcggcgttcatgattagattcagcttcattcagagccacaacttccccagcaatgcacttaacaagatgggacaagatggccttggctctccgaactttaccaagatccatgagttccaaaagctgcaagggatgatactgaggtagagtcggggaaagtacatgagctgcttcaaaaagacctgaatcttccatatccactgaaggatcgaatgcagttttctttccacagattttctgtgcaagactggtcatggatcgagtcagagttttctttggaggatgtaacccagaactggagttactctgttttattaaacttgttatagatggagtgctcccactgtacgaatctgttataacaggttcttgtttagaagatggttgccattggcaatacacatgcatttcacagtccattcctaccacaaggatgccatcccggacccacgataaagaaacaggaaaaggtggggagccatctacagaagaaactaggtccacacttcgtaatagtacaaatttagaaaggggcacaactttggtactctcccagagaggaaatgccagggtttccttaccagtttggtcttgtaccttgccagccaggggtccatacataaaaagttttgatccaattcctacagtcaggatatgagaaccgtcttctctagacatccaatctaagtgaactaaatgctttgtgtttgatgtgatattctctttactagataaatacatgtcttgtttattataggccactaaattgctatcaacactaatgccagaatccaatactgtgcttaactcatctaaatgaattgtctgctcaaggacccaacatgaacctcctgttgactcacattcaaaaatacttacatgcatcacaaagtcctgggaagatctactattagatgcaggctgcttataagctactgctaaacgatttgtatgtgcacagctaacttctacaggcctaccaggtacagttatactactattgctctgaagtccatcttcaataagtaatggccattcttcccaaatgtatgcaagatcaatttttccattctttgacgtggcagattctccatctgttactctgcatctccagaatcttactttctcatctgaacatgaagttgccaataaataaggagcactgcatgcaggatatatagaagatgaactcagatgtcctgctgatggcttaatacttattatctcaactccttctggtaaatgcaattcttggctataaaccatttctgaaaacagagtcaacctgctggtactctggagatttgctctgcaagcctgatacttttgtgaaaaaggagataggatcttctctggagaagaagaataatgttcttctggctgccaaaccgcttcggataattttgtatctactttttcatctaatgagacaggaattgactttagatgtaaattccacatgtgtaacagtgaacggttgtcttgagtgcattctattacaattaggtagaacttctcagaaaatccattaggtgagctgcctgcattagataaaatgctgtctttgccaaggcttttcttctcaaggttattcaaaatgaagtcttcttcaaaaacatgaagcagttgggtttttctgccatgaagtttggtaatgggatctaatgcaataatgcatcctggcctggctgttgattgttgactgacgatgttaaagacttcaccaacatatttagaaatttcagggttagaaagctcagataaaagtttcttagcatcaataactgcttcatataatctcagatattgtccatcactggctacaaagcatgcactaggagagttgcagtatgcacccagacaataactgggtataagagtgggcagccatgccacattggaaaaggcagaaacatgaagagaattaatccgggcaagctcagaaactcctccagaaaaagacaatggcccaactgggtcaaccctccacagaataagctcactgtaaactgcactgggatcctgaaatgccacgtcaacagtgcttttattttgttgtgtcaaagagcattcttcaatatttagagcatcaaaaggttgctctgggttatcaacatctggtgtccttaatgcattatggtgtgatgttgtcagcaataatggtaatactgagtggcaagctaaatcattaagatgaaaacgatgaccacaatatctggatttgtgggaaatactgagaacagtagaaaaagcagattcctcggcaaaactgaccagccactgattcagagaaccatcagcatgttttgatatcatcataacattaggcgtaaaaatacttaattttaaactattagatgatttattgtgaccagaagaaataagcattgatgtggaacgggtgaggccagaaggtttttgtttcccctgctgaatagccaagtcaacattcttggtacaggcatacatcattatgcttttacagagagagtttgcatcacctgtggggaaagctactggaattctggaaacaaaggacacctgtacttgacgaaacataccaggctggtattcatccagccaatccacatgccaaactagcaaagaaccatccatgggatgaatactaaatagcatatctgcatttttactccattcagacagaagtacttcaatctgatgatcaatggcagctgacgataatgatgtaaaacttgagtttggtaccattttatcacagcctaattccttcttttcgggatttattttcagatcatcaacaccatcatcagtttcttcatcagattttacatctgcctgattagaatcttctacactggcctcagaagatggttgttcaaaactttttctaagttgctgtaaaaaaacttccatggacaaagtaaaatgcagttctttattgtttagccagtgtacaacaaaaggtccggtcttctcttcattttcatttagactcagagatgtaatagatggaagaagtggaatgtctgtggctgggttgatgctggctgcaatatgaaagtggcaaagtgcattggcatgcagtggagtgttcctgtgaacatgatgaggatcctgctgatgtggtagatatcccgtatgtgctacaagagcaagtgatctcctccgacctctacgaaaatgtctcagatttacttctaaagcattttgaactcgttctttactggaagcatttctcttgaagttatttgttaaattaattgattcagtccaatggctgcagtcacctccgtatagcaaacaatcatttggtaaaaatgtctctacccaaagacgacacacattatctttgcagcaagtcaacagtacattacatacagaagccctaggcatatatttgcttgttttacgccaggaaaatccatttactgctcgaggatgggccagatacacaaaagaaaagtcaatttctccttgggattgtttttctgaacttccatctggagaagtaacagctgtccgccagttttctacattataccaaaccttcaaaagacagtcatccttcccagcagtggcaaaaaattctccatctggtgaaaatttcattaaatgaacttgggaagcagttttgcaatgccaaatgcatttccaatctccaaagttaagatctgttttatttaaattttcatcttcagttggcttctccaagttagtattggaccagagttgcaaatagctggaaccagttaaaagacgactgcctgtgggatcccaggttatattgtgtgctattgattccagaaaaaattggccacttttctgccactgactatataattccaaatttttcttttgttttggtaggttaactggttcaaaaatggagataacatttccataagacgctgcaatcttgccttgttgcattgaacagtctacacatcccacttgaatatttccatgtttagctcctgggattatctgtaatctttcaaaatcgcttcccagtattacaatgtcacatccagatgcataagctacgcgcctctggatccctg

SEQ ID NO: 9977 - RNA, 10204 nt, Homo sapiens
  source 1..10204: mol_type = other RNA
cacacacacacacacacgtatacatacatacaacttgggttccggagggtaaactactgaaaaccttacatattgagccatctagctcatttatcactgacgtctcaatgacaattttaatgaagatgttcattatttttttcattcttactcaaatacctatcattaattaagagaagagtttgagatgtataaggctaataaaggaagtgagagtgtggtgaattaagtgatgagtattatgtacaattgcctttacaaaaaacgtatttttactgtggaagaaattcatgcagagatgcctgtggaaaagtatcaataagaaaacaaaacacctttaacactatgacatactgattataatatactatgatatgtattattacagcattacttacacattctactttaggcaatgtaatctacttctgaatgaccttgttaatttttaaggcatcagtgcatcaagggcaaagctccataaaataaatataaaaacaagaaagcattagctaatttgtggcatagagaatgatcactgtatattatatctgttggccacttccatataggtaataaattgtacatcttattgtaaaaatgttatagcataaatttcacatcatttttcaacacttcatttaaagggctaaactgatctggcagtattctcattttcattgttccatcagctccacaggagaaaatgtgatttgcaggccctgtctcaatttgcatcactccagttccaatatttctaaaaatggactgccgagcatgttcactgacaaaagtatggagaagaccaaaggtagagagactccaaatctttatattgccttcggcagatcctgtaacaaagtactcttcagttggatcaacagcaacggctttaacaggagaatcatggctctggaaaagctgcctctgttgtcgttgacaaaggtcaaatacatatgtaaaaccttttctgccacctgatattagtagctgatgttttggagcatatgctaaaactgtggctccactgtcatggcaggtaaatgcatggactaaactattggcaggtgctacaagagtatcccacaaacatacgtttctattgtcagttgaaagaccagctgtagctatcagagaggaggaactaacgaagacaaaatcattggctgttttgttatgacactgccaagtctggaatggttacaaacaatacgtgttactcctctcactaaaaatgtcataaccaggtaaatgtattcttcgaaaagtgatcatgtagtttctggctttcttaaatcctctgtatcgtttttttcctttgaacaggtatggcttaggcatgcttccagtaactggacaacatttccagtttgtttgatacaaacttaaatatccatcagcatcaactattccaaacttatttccctgatagttaaatctcattcttgtaactcttgaattgccaccagatcgaaaacaggttatttgttgagaatggccccattcaaacattctgacacttccatcttgagctcctgtcagatagtaaggaagagttggatgagaagtcattcttctaacattattaatggctttcttaatcatcacagatgctcctctgccagtctgtgtactaccaagccatggcatgttgattggagtgccaggattgctatgtgtatatggagttgtaccttgaacagctgttaaatcatcacgagcatgtataaccaagaaatcttctgatcctttggtttccacttctatatcatcatctacccaagtgtagacctgtgtggccagaattccagaaacatccagttcttgaacatcatgactggaagcgattgctatgcagtttctatttgccttattaacagcaaacgcagtaatgatatcagattccttatgaataattcttgctttacctccaggatatcccaaatctgcttctatctcatttagacaccgtttctttgtgaatatatttttgataaaggtttcctgaatttcttcctgcttcaccaaatactgccaaagcctcttcacagacagtgccagatggtgtttggatttgaaaggagtgtttgtaggttccagtaaagctttgtggcgaagaattgcaggacctgcagacaaactctcttcggcggtatgacttgcgatataattttgaggtggcccaccatggatttcaagtcgtcggagaagaacttgttcccaacattgaagagtttttagaaccgcatgacaaagaggtgaactaactggaagctctgcaagatcatgacctgcgaagggataaaaagtcttcaaattgttgagcaccaattgcaccatcgccaaccgcatcaaggaccaactatatgaatttgaattagaatgttcctggagatggaaatctgatgctaaaacatcatcatcatcatcattgtcatcatcatcacttcccagactctcctctgaatcatattcggctctactttgagaagagggtagaaaaggcttagctatgaaatagtcccagatactgagctcaggtgggatgaacttttctttaaccgccagtgactcctggcttactggtgccgaggaaggggtcagtggggcagattctctgcaagacatttttgacggcctaaaacgtttgttctgtttttctccttcttcaactagtgaagaaacaggtaaagtttttgaatgtgtctgttctttgctaggaacatgtgcacctccaccaaacacagcagaccacattttctcatttagaggatgggccacaatccgaaatagctcattacttgaatgtgtggccaggccatggatgaagagactaagatacactgctgtgagaatctcacagagcaagactgtaagccctgactgggcttcctcgccagaagaattcaaaagtcgaattagacaagttattcctggccattgagctggtgacgtattgggagttaatgcttcatctaagcttcctgttttcaaagaaggtcgatgaggaagcagtactgtctgatataccattccagtaaactgattcgtctgaaatgaactgtagttatgactaccacaaaggcactgataaatacaagcagaaagtgaagctgctaaagtatgcattacatacactttattgctttggatatcagggtggggtggtgaatcaaagtttattatggcatggagaatatcatgtgtcagattactaaggtgcaataatggattggcaactactgttttggcattggctgtacaagcaaagaggagaggcactgaggtttgctctgacagagggctagaaaatagtggttctgatgtttcctgctgagattcttgcaaaagcaaaatcaattccattcttacagatgcaagacccccaccatgggatccatgaagtatgcagtaactaagaaacattctcaaaagtgactgatacttcaagagccactgtcttttttcctgaaaattttctctcagttgtttcacttttgtttggtgaggcaaatcttcagcatcctcatttaatccaaattcatcttcatttctgccaaatgcagactgtagttcttcagcatctgagcaaaagtcacaagtcctctgaagagctatcacctctttttcaagccagtggtatagttggtaacgcaattttccaccatctatttcatagccagtagataaagtacgaagttctactgtgagaatctttaaacatgctctaaattttaactgaactgcaattatatcttctgatggatttaaaaggtcattttcatctagtgtgctgaaagattctgtgtagttagaacttatgtcatccaactttttatctgtttttctctgtaaaggttttagttctttcattgaaatagggacatcctcattttcttcatcattatcactgtcccattttaactctaaagagtcatcctgaaacacaacacttggttggctccagtcaaaagaaagagtggagtttgattgcttctctgaggaaccctctgaagaagatccaaaaccatttatcagtgactgtgaccaatcaacagcagaagacttatcttcccttgcatccaactttaatggagaagaaggagaacagtctttactagtatccagaaaactagaagccctataaaaaggtcttgttttcttgatgactttaggcatctttgataatacttccaaagccaacattgggcagccagcttttaaatgagcactggcagtggtaaaaaataaacgtctttcacttaaattaattgttcctgccagtccactttttcctgttaggctcatatgtgtggaaaatgtatcagatgatccaaaatgacgtctcagcaaaagaggatgtgttcttagataattgtagaaattaaaaactgtaggattactggctgataaaacttgatcatcattctctctgataggttgctttattaatgtttccagagcaccactataatcttccaaaatccaatatgccatgctccgaagaaaaggatcatgatgcatatttatgttcaatgaacacagttcactgacaggagaatcgattcccaaaacttttttacgtaaaatagatttatatgctgcagatgtatcaaattcagactcatagagtcttgctattacaagagccaactgaatgtcattcaatttctcaagacatacctcaattgcatctctgaggcaaccagctaaaagaaaaaatgctgcagaatgttcaaatctttgtttgcctagcaaagaaaaagcattctttaaagctgctttacgccacctctcatcctcaaaattgtgtccaaaaaactgtgtcatcctggtgtttttttcagcttttttctatgcatttgcgtaagatgcgggtattccggacccaccaccccacacccatagctcttagttcagaccaagtgggatcatctttctgcatggctggcaacatgttcagcagttcttcttctgctactgagtgaaatgcccaagcaaaatgacttgtagacaggccttggtgaaggagttgagctcgataggctggaagggaagttgtaagaaaggtatggagtcgaacagccaaaagaaattttaacccacattcatcaagagtttctccaccttggcttctgtctcggctttctccaatatcagtgcttgtagttgcaattgtatctgctaaggccatcaaagacatctgctccatccggctgagtcctggtaaactagaatgaagtaagtggccagaaagaacctgagcatgctcaggtccaaagtaagtcggactgtactgtgaaaggtcaataactctaggctttgtattttcttcatctgtctctaacatatgagtatcagtcattagaagttgagtctgaaaaagctcatcataactttctttagataattggtttgatttacttaacgtactctcattactagatttctccaaagatgagtaacagctatcatcatctgctgcaagtaaggcatataaaggaagtggaggaacagaatctatttctgtgtaatctgtattttcagccttgttgaatgcctgggggtctctggtagtgcttccactagcactgattgtgagagacctaaggcggcgttcatgattagattcagcttcattcagagccacaacttccccagcaatgcacttaacaagatgggacaagatggccttggctctccgaactttaccaagatccatgagttccaaaagctgcaagggatgatactgaggtagagtcggggaaagtacatgagctgcttcaaaaagacctgaatcttccatatccactgaaggatcgaatgcagttttctttccacagattttctgtgcaagactggtcatggatcgagtcagagttttctttggaggatgtaacccagaactggagttactctgttttattaaacttgttatagatggagtgctcccactgtacgaatctgttataacaggttcttgtttagaagatggttgccattggcaatacacatgcatttcacagtccattcctaccacaaggatgccatcccggacccacgataaagaaacaggaaaaggtggggagccatctacagaagaaactaggtccacacttcgtaatagtacaaatttagaaaggggcacaactttggtactctcccagagaggaaatgccagggtttccttaccagtttggtcttgtaccttgccagccaggggtccatacataaaaagttttgatccaattcctacagtcaggatatgagaaccgtcttctctagacatccaatctaagtgaactaaatgctttgtgtttgatgtgatattctctttactagataaatacatgtcttgtttattataggccactaaattgctatcaacactaatgccagaatccaatactgtgcttaactcatctaaatgaattgtctgctcaaggacccaacatgaacctcctgttgactcacattcaaaaatacttacatgcatcacaaagtcctgggaagatctactattagatgcaggctgcttataagctactgctaaacgatttgtatgtgcacagctaacttctacaggcctaccaggtacagttatactactattgctctgaagtccatcttcaataagtaatggccattcttcccaaatgtatgcaagatcaatttttccattctttgacgtggcagattctccatctgttactctgcatctccagaatcttactttctcatctgaacatgaagttgccaataaataaggagcactgcatgcaggatatatagaagatgaactcagatgtcctgctgatggcttaatacttattatctcaactccttctggtaaatgcaattcttggctataaaccatttctgaaaacagagtcaacctgctggtactctggagatttgctctgcaagcctgatacttttgtgaaaaaggagataggatcttctctggagaagaagaataatgttcttctggctgccaaaccgcttcggataattttgtatctactttttcatctaatgagacaggaattgactttagatgtaaattccacatgtgtaacagtgaacggttgtcttgagtgcattctattacaattaggtagaacttctcagaaaatccattaggtgagctgcctgcattagataaaatgctgtctttgccaaggcttttcttctcaaggttattcaaaatgaagtcttcttcaaaaacatgaagcagttgggtttttctgccatgaagtttggtaatgggatctaatgcaataatgcatcctggcctggctgttgattgttgactgacgatgttaaagacttcaccaacatatttagaaatttcagggttagaaagctcagataaaagtttcttagcatcaataactgcttcatataatctcagatattgtccatcactggctacaaagcatgcactaggagagttgcagtatgcacccagacaataactgggtataagagtgggcagccatgccacattggaaaaggcagaaacatgaagagaattaatccgggcaagctcagaaactcctccagaaaaagacaatggcccaactgggtcaaccctccacagaataagctcactgtaaactgcactgggatcctgaaatgccacgtcaacagtgcttttattttgttgtgtcaaagagcattcttcaatatttagagcatcaaaaggttgctctgggttatcaacatctggtgtccttaatgcattatggtgtgatgttgtcagcaataatggtaatactgagtggcaagctaaatcattaagatgaaaacgatgaccacaatatctggatttgtgggaaatactgagaacagtagaaaaagcagattcctcggcaaaactgaccagccactgattcagagaaccatcagcatgttttgatatcatcataacattaggcgtaaaaatacttaattttaaactattagatgatttattgtgaccagaagaaataagcattgatgtggaacgggtgaggccagaaggtttttgtttcccctgctgaatagccaagtcaacattcttggtacaggcatacatcattatgcttttacagagagagtttgcatcacctgtggggaaagctactggaattctggaaacaaaggacacctgtacttgacgaaacataccaggctggtattcatccagccaatccacatgccaaactagcaaagaaccatccatgggatgaatactaaatagcatatctgcatttttactccattcagacagaagtacttcaatctgatgatcaatggcagctgacgataatgatgtaaaacttgagtttggtaccattttatcacagcctaattccttcttttcgggatttattttcagatcatcaacaccatcatcagtttcttcatcagattttacatctgcctgattagaatcttctacactggcctcagaagatggttgttcaaaactttttctaagttgctgtaaaaaaacttccatggacaaagtaaaatgcagttctttattgtttagccagtgtacaacaaaaggtccggtcttctcttcattttcatttagactcagagatgtaatagatggaagaagtggaatgtctgtggctgggttgatgctggctgcaatatgaaagtggcaaagtgcattggcatgcagtggagtgttcctgtgaacatgatgaggatcctgctgatgtggtagatatcccgtatgtgctacaagagcaagtgatctcctccgacctctacgaaaatgtctcagatttacttctaaagcattttgaactcgttctttactggaagcatttctcttgaagttatttgttaaattaattgattcagtccaatggctgcagtcacctccgtatagcaaacaatcatttggtaaaaatgtctctacccaaagacgacacacattatctttgcagcaagtcaacagtacattacatacagaagccctaggcatatatttgcttgttttacgccaggaaaatccatttactgctcgaggatgggccagatacacaaaagaaaagtcaatttctccttgggattgtttttctgaacttccatctggagaagtaacagctgtccgccagttttctacattataccaaaccttcaaaagacagtcatccttcccagcagtggcaaaaaattctccatctggtgaaaatttcattaaatgaacttgggaagcagttttgcaatgccaaatgcatttccaatctccaaagttaagatctgttttatttaaattttcatcttcagttggcttctccaagttagtattggaccagagttgcaaatagctggaaccagttaaaagacgactgcctgtgggatcccaggttatattgtgtgctattgattccagaaaaaattggccacttttctgccactgactatataattccaaatttttcttttgttttggtaggttaactggttcaaaaatggagataacatttccataagacgctgcaatcttgccttgttgcattgaacagtctacacatcccacttgaatatttccatgtttagctcctgggattatctgtaatctttcaaaatcgcttcccagtattacaatgtcacatccagatgcataagccgtgaagcgctggtcgccaatgctgcccacggagaagcagtggtcgccagggttcacagccccggtcagcacctggtgcaggttcatgtcggcgccctagtcctgcaacggacaccgcatccagctcatgccacgggtcagcggctgcttccctccctccttccctcaggggcggcggccgctcttcggtggcgacggcagaagcagcgacaggcgcctggagccggagccgctcagctggggcccgcgactcatcccgagccccggagggcgaggcccggagggggcgggtcggcgagagggcggagcgccgcgctccttcgcgcacctgtcactccccgcgctagcccaggtgaagctcagggtcccctcaccggccacgacccggggccgactcaccggccaggaaggccgcgctgtccacacacttcctctggacctcgggcagccgctcctgacccagcccgagtggcgcaagcagtacgcgctcgcactccccgcctgacctgtcccttcccggctccggtgcccgccacccccacagtcctccgccactcactacgcgcctct

SEQ ID NO: 9978 - RNA, 5177 nt, Homo sapiens
  source 1..5177: mol_type = other RNA
cacacacacacacacacgtatacgtgtgtgtgtgtgtgtgtgtgtgtgtagtttattactggttaagtaaatgctctaattagcaaaaatcatgagaaatatatacagtgatataatgcggttaaattttagttctctgtgttaactacttactgttaatttagtactcaattagaattaactctgggattttgagggcagataaatcagtaattagcctttatcccagaaagaatagtggtagcttcaaaagcttcaacagacctaatgatgtaatttattcaggacagaaaaaaaaatatgtagccaacattcttgcaagaattactttcttatggaatttaagatttcctcaaatattttcttttctatatagcgttttgttcttgtgtagttatctgcctaggatacagacaggatattgagactatttcagaaagtagacacactaaaaacatttgacaaattaaaaaaattttgcataaaacaggttaccctttcctgctgactatacttaagaaataccaaagtagcatacaaaatgcttctaaactttcaaaatatctgaataaaaacaaagatcctacttttaactgagatagatttataattcttacttacaagataaaaaaatttcctaaaatttatttttaaatttcacataacctgctataattcgctgtaaaaaatggatgtcaaaatagaattttaaatatacaaattgtttttgataactacctttcatacattttatttaaactgtagcattagctcaagatgaaactttttaaaagaaaccataggcttttgtccaactcaaagattcaagcccagattctgaacaaagtaaatgtgatgaaatttatgaaaaactatactgtacagtcaaaacagtgatggtgcctcagtaaataacttcagtaaaatatccagtgctccaaatagctgagccatctttctaaggttcactctgcttctctcccccagccctcatggcctgtgctaccatctattcttttagcgtttatgctggagggccttatagttcctttaaaagtacactgaaaatactttatatcacagcttattctaaccactggttctcaaattaaaaggtatatttcagtgcatatttcatagccacattgcagaactaatatttgaaaactcttgggggaaattttggtaacaaaattgcaaaatgacatgattatttatgagctttctataaaaagttttttttttttttttttttttactttagagatcatacctactttcctgcctttttgataagtaaggcatgaaatgaaacaaaagttttgagctgtaaggtgcctataaaggatgtcactacagcattcacaatgctaggtgtgtaagatgacatggctgttaccatgtactaaagaaccccatcatgtgagagatcgctcaaagtcattaacacaaagcagtgaaaatcatccagcaaagcagtgcttatgagagactagaattcagagaaatgcaaggtacgaacttctctctaatccaagggtattctgctgtgatcttctaatcagtgatgattgtgcttatgcacacgacatcttcatgggagagaccaggctgattgcaaaataatgacaaccaaccagtttacctcaacatagctcactctgcaatgtcagacatgcagtgtagagcagtcacaaagtcaagccatgaatacagggatggaaaaacattccagtgagctggtctctacaatttttaagacacttcatcctcccaattatattctttgtcataaagaggaaaaacagcaagattattaaatccaaaaagtcacagatgtcacaaggggatgaaataatttcctcattttttttctttatcagtgtaggaaaagctgtctttccatagcccacactcataatagcacttcaactaggctcctttgaaaatgaaaagtgaacaagtttcctaatgctggccttataagatctaaagagatgattaaattcaaaccaggctgagctcttactctgagctatttcagccactgatgtttgtaaaatataggaagaagattccaataggcaatttgcattggcaagcactggactacagaattcatcactgttttctgaaaaaatataattaaaccttaatggaattatgacacttttatgaggtttataattcacagccacctctcatcatattttgttcttctttccatttttaccatttcaaatattgcaatattgcccaccataaaccactgaaaatgattatttatgtatattccatttatttctctagggggtctaggtaatttgaatcaggagctccaagtaccatttaaaaaggtgagtctttaaaaaccatcagtgttttaaacacttgattagaaaaaagataacagctccttgtagtgatctagcttatgtgctttatggtatcttttcaaaaggagagtataaatcattgtacataaaatcaaaatagctaatatacatttttttctggcacttttgagaaattaggcattgaacataaaacatcttataaacttacataacaaaaataaatgtttacattttaatcttagattaccttagggtagcagttaacttatgagatgccacactgttggtgtgggcagcggagaccatgggaaatacacattcatgtccacagcccttcagcgatggatgcatggctgccgtccaaatatgtggtctgtgtcccaacataaagattaaggctctctgttttgaaggaatgagttctgggcttaaacaagtctagaagtaccacaatactcatggaaaatactgaaaagattcggacgagttttcaaacactgggggaaacacgtttttgactagaaaaataaaataaagcatctaaaactgacttcaagtactttggggagaggctgctgatatcgaatgccaaaataagaaggaacaaagacagaagagactccagggacgtccctccccatcccttcacccgcagggtccagatccccaggtgctgatgcgcaactctttggggaggactggcgagctgggcagaaagcagcagccatggtttgtcaccatcctaaaacacctatattgagggcaaaggccaagctttgtgtgaaaatttccttgggatgaaccacaggaatctggacatttcaagggggaaaaagccttaaagtcagtagcagacagagaaaaggaaagagaggaagaaaaacctgcttttctgaatggcagtactttaggccgggggcattgtggtccttggtgagtgcagcttttccatacagcttggctttcctcactaatgagatgagaccactgacagctgggatcttttgtgggtggtgagggtgcagcagggagatgtgcttgggtgtacctgtccatctggcaggcaggggcacactcaggtgcagcctagtccgtacctctctgtctcagaaactgaacaactgggagaacagtcgacagggcctctccaaccatcttcaggtgactaaagcagcatatgaagtataggtttgtgtcacttcttctcttccacagaagaaacgtctccagacactgatcacaggctacccagggttgtcttctgggttgctagagcctggtaatatctctgccttgctgcaagtcacttatgctctcgtagtcgttctcctttgggacgagaccgtggtggccattggtccccagggtggccttttcttcctctctgttgagagtctgtatcgcttcataatcaggctctggctcctcgctgggcctccctgctggtggaagtgtgctgtttggagttttttcgaagtctttaacagtagcatagagatcattacaggaggagggtgacctctgtgggtccccttgaatggaggtgtaggtggactccggaactgtaagcgactgccccgatttattcactaactgtccaggtttatttactgatgagtacatagctgagatctcttcttctgtgagagtggggtcttcttcccgagacttgtatgacaatgagctaaatctcttgttagtttcactggtcgtgtctgtggcactctcttccgcctctcccccttccttctcctgaaggttttcattctcgtccagaagcttaacagggacaggtggtggggcctcctcttctggatcacatgaatttccaaggatactctctacattaacactttgacgacattttttgtttctgtccaccgaggcatattcagcaaactcagctttgccttcagtctggggccctgggagctctttcgaggcagaagtagattttgccttgccactgtggcctttctccaggtgtgcagctgcagccacctccttgatctctttcacagtttcatacaagcagtcctccaccatgttttcttgggaggagctgtccttgagcacttcatagggcccttccatccccagcccctggtccccgtccacacttctcgccgtgagcatggtatccactgcgctctcgggagggattctgggcagctcccgactctgatgacattttggtttccctgtgctgtcctgggaatccagcagatccgaggccgatgtctggacttcctcgtaatgctgcatgcaggtcagagtactgtcctctgaaagaatgtccccattggtgagtgccccattctgctcactgctggcaggagcatctgttgccaggctagtaactgaacggctgaacatctccttgtctgaaggcacgttcatcaggttctcatggtccccactatgctgtcgcggcttcttttccctgtcacaactagagcacaggaagatgaggaaggtgatgacgaagaaaatggcgacagcagccagacttccccacagggtgatctgcatctgtccgctgcccagcaggctccccgcgggccccatggcaggagcaggcactggcaccagccgagggaatcagtcagtccttcaaaggtggtgacatggaggcagagagctgtgtcattttcgtttgcttcagtgataaagctgtgactgttttcagccatccctgagcacagacatcaagacggcaggggtggcttcgcagcaaaccagggtgcctcaatgtatgcagagagagttctgagagatgaagttgttttcctcaatctttgaatcaacatgaacgtcttc

SEQ ID NO: 9979 - RNA, 5188 nt, Homo sapiens
  source 1..5188: mol_type = other RNA
cacacacacacacacacgtatacgtgtgtgtgtgtgtgtgtgtgtgtgtagtttattactggttaagtaaatgctctaattagcaaaaatcatgagaaatatatacagtgatataatgcggttaaattttagttctctgtgttaactacttactgttaatttagtactcaattagaattaactctgggattttgagggcagataaatcagtaattagcctttatcccagaaagaatagtggtagcttcaaaagcttcaacagacctaatgatgtaatttattcaggacagaaaaaaaaatatgtagccaacattcttgcaagaattactttcttatggaatttaagatttcctcaaatattttcttttctatatagcgttttgttcttgtgtagttatctgcctaggatacagacaggatattgagactatttcagaaagtagacacactaaaaacatttgacaaattaaaaaaattttgcataaaacaggttaccctttcctgctgactatacttaagaaataccaaagtagcatacaaaatgcttctaaactttcaaaatatctgaataaaaacaaagatcctacttttaactgagatagatttataattcttacttacaagataaaaaaatttcctaaaatttatttttaaatttcacataacctgctataattcgctgtaaaaaatggatgtcaaaatagaattttaaatatacaaattgtttttgataactacctttcatacattttatttaaactgtagcattagctcaagatgaaactttttaaaagaaaccataggcttttgtccaactcaaagattcaagcccagattctgaacaaagtaaatgtgatgaaatttatgaaaaactatactgtacagtcaaaacagtgatggtgcctcagtaaataacttcagtaaaatatccagtgctccaaatagctgagccatctttctaaggttcactctgcttctctcccccagccctcatggcctgtgctaccatctattcttttagcgtttatgctggagggccttatagttcctttaaaagtacactgaaaatactttatatcacagcttattctaaccactggttctcaaattaaaaggtatatttcagtgcatatttcatagccacattgcagaactaatatttgaaaactcttgggggaaattttggtaacaaaattgcaaaatgacatgattatttatgagctttctataaaaagttttttttttttttttttttttactttagagatcatacctactttcctgcctttttgataagtaaggcatgaaatgaaacaaaagttttgagctgtaaggtgcctataaaggatgtcactacagcattcacaatgctaggtgtgtaagatgacatggctgttaccatgtactaaagaaccccatcatgtgagagatcgctcaaagtcattaacacaaagcagtgaaaatcatccagcaaagcagtgcttatgagagactagaattcagagaaatgcaaggtacgaacttctctctaatccaagggtattctgctgtgatcttctaatcagtgatgattgtgcttatgcacacgacatcttcatgggagagaccaggctgattgcaaaataatgacaaccaaccagtttacctcaacatagctcactctgcaatgtcagacatgcagtgtagagcagtcacaaagtcaagccatgaatacagggatggaaaaacattccagtgagctggtctctacaatttttaagacacttcatcctcccaattatattctttgtcataaagaggaaaaacagcaagattattaaatccaaaaagtcacagatgtcacaaggggatgaaataatttcctcattttttttctttatcagtgtaggaaaagctgtctttccatagcccacactcataatagcacttcaactaggctcctttgaaaatgaaaagtgaacaagtttcctaatgctggccttataagatctaaagagatgattaaattcaaaccaggctgagctcttactctgagctatttcagccactgatgtttgtaaaatataggaagaagattccaataggcaatttgcattggcaagcactggactacagaattcatcactgttttctgaaaaaatataattaaaccttaatggaattatgacacttttatgaggtttataattcacagccacctctcatcatattttgttcttctttccatttttaccatttcaaatattgcaatattgcccaccataaaccactgaaaatgattatttatgtatattccatttatttctctagggggtctaggtaatttgaatcaggagctccaagtaccatttaaaaaggtgagtctttaaaaaccatcagtgttttaaacacttgattagaaaaaagataacagctccttgtagtgatctagcttatgtgctttatggtatcttttcaaaaggagagtataaatcattgtacataaaatcaaaatagctaatatacatttttttctggcacttttgagaaattaggcattgaacataaaacatcttataaacttacataacaaaaataaatgtttacattttaatcttagattaccttagggtagcagttaacttatgagatgccacactgttggtgtgggcagcggagaccatgggaaatacacattcatgtccacagcccttcagcgatggatgcatggctgccgtccaaatatgtggtctgtgtcccaacataaagattaaggctctctgttttgaaggaatgagttctgggcttaaacaagtctagaagtaccacaatactcatggaaaatactgaaaagattcggacgagttttcaaacactgggggaaacacgtttttgactagaaaaataaaataaagcatctaaaactgacttcaagtactttggggagaggctgctgatatcgaatgccaaaataagaaggaacaaagacagaagagactccagggacgtccctccccatcccttcacccgcagggtccagatccccaggtgctgatgcgcaactctttggggaggactggcgagctgggcagaaagcagcagccatggtttgtcaccatcctaaaacacctatattgagggcaaaggccaagctttgtgtgaaaatttccttgggatgaaccacaggaatctggacatttcaagggggaaaaagccttaaagtcagtagcagacagagaaaaggaaagagaggaagaaaaacctgcttttctgaatggcagtactttaggccgggggcattgtggtccttggtgagtgcagcttttccatacagcttggctttcctcactaatgagatgagaccactgacagctgggatcttttgtgggtggtgagggtgcagcagggagatgtgcttgggtgtacctgtccatctggcaggcaggggcacactcaggtgcagcctagtccgtacctctctgtctcagaaactgaacaactgggagaacagtcgacagggcctctccaaccatcttcaggtgactaaagcagcatatgaagtataggtttgtgtcacttcttctcttccacagaagaaacgtctccagacactgatcacaggctacccagggttgtcttctgggttgctagagcctggtaatatctctgccttgctgcaagtcacttatgctctcgtagtcgttctcctttgggacgagaccgtggtggccattggtccccagggtggccttttcttcctctctgttgagagtctgtatcgcttcataatcaggctctggctcctcgctgggcctccctgctggtggaagtgtgctgtttggagttttttcgaagtctttaacagtagcatagagatcattacaggaggagggtgacctctgtgggtccccttgaatggaggtgtaggtggactccggaactgtaagcgactgccccgatttattcactaactgtccaggtttatttactgatgagtacatagctgagatctcttcttctgtgagagtggggtcttcttcccgagacttgtatgacaatgagctaaatctcttgttagtttcactggtcgtgtctgtggcactctcttccgcctctcccccttccttctcctgaaggttttcattctcgtccagaagcttaacagggacaggtggtggggcctcctcttctggatcacatgaatttccaaggatactctctacattaacactttgacgacattttttgtttctgtccaccgaggcatattcagcaaactcagctttgccttcagtctggggccctgggagctctttcgaggcagaagtagattttgccttgccactgtggcctttctccaggtgtgcagctgcagccacctccttgatctctttcacagtttcatacaagcagtcctccaccatgttttcttgggaggagctgtccttgagcacttcatagggcccttccatccccagcccctggtccccgtccacacttctcgccgtgagcatggtatccactgcgctctcgggagggattctgggcagctcccgactctgatgacattttggtttccctgtgctgtcctgggaatccagcagatccgaggccgatgtctggacttcctcgtaatgctgcatgcaggtcagagtactgtcctctgaaagaatgtccccattggtgagtgccccattctgctcactgctggcaggagcatctgttgccaggctagtaactgaacggctgaacatctccttgtctgaaggcacgttcatcaggttctcatggtccccactatgctgtcgcggcttcttttccctgtcacaactagagcacaggaagatgaggaaggtgatgacgaagaaaatggcgacagcagccagacttccccacagggtgatctgcatctgtccgctgcccagcaggctccccgcgggccccatggcaggagcaggcactggcaccagccgagggaatcagtcagtccttcaaaggtggtgacatggaggcagagagctgtgtcattttcgtttgcttcagtgataaagctgtgactgttttcagccatccctgagcacagacatcaagacggcaggggtggcttcgcagcaaaccagggtgcctcctacaatgtatgcagagagagttctgagagatgaagttgttttcctcaatctttgaatcaacatgaacgtcttctaaggct

SEQ ID NO: 9980 - RNA, 5156 nt, Homo sapiens
  source 1..5156: mol_type = other RNA
cacacacacacacacacgtatacgtgtgtgtgtgtgtgtgtgtgtgtgtagtttattactggttaagtaaatgctctaattagcaaaaatcatgagaaatatatacagtgatataatgcggttaaattttagttctctgtgttaactacttactgttaatttagtactcaattagaattaactctgggattttgagggcagataaatcagtaattagcctttatcccagaaagaatagtggtagcttcaaaagcttcaacagacctaatgatgtaatttattcaggacagaaaaaaaaatatgtagccaacattcttgcaagaattactttcttatggaatttaagatttcctcaaatattttcttttctatatagcgttttgttcttgtgtagttatctgcctaggatacagacaggatattgagactatttcagaaagtagacacactaaaaacatttgacaaattaaaaaaattttgcataaaacaggttaccctttcctgctgactatacttaagaaataccaaagtagcatacaaaatgcttctaaactttcaaaatatctgaataaaaacaaagatcctacttttaactgagatagatttataattcttacttacaagataaaaaaatttcctaaaatttatttttaaatttcacataacctgctataattcgctgtaaaaaatggatgtcaaaatagaattttaaatatacaaattgtttttgataactacctttcatacattttatttaaactgtagcattagctcaagatgaaactttttaaaagaaaccataggcttttgtccaactcaaagattcaagcccagattctgaacaaagtaaatgtgatgaaatttatgaaaaactatactgtacagtcaaaacagtgatggtgcctcagtaaataacttcagtaaaatatccagtgctccaaatagctgagccatctttctaaggttcactctgcttctctcccccagccctcatggcctgtgctaccatctattcttttagcgtttatgctggagggccttatagttcctttaaaagtacactgaaaatactttatatcacagcttattctaaccactggttctcaaattaaaaggtatatttcagtgcatatttcatagccacattgcagaactaatatttgaaaactcttgggggaaattttggtaacaaaattgcaaaatgacatgattatttatgagctttctataaaaagttttttttttttttttttttttactttagagatcatacctactttcctgcctttttgataagtaaggcatgaaatgaaacaaaagttttgagctgtaaggtgcctataaaggatgtcactacagcattcacaatgctaggtgtgtaagatgacatggctgttaccatgtactaaagaaccccatcatgtgagagatcgctcaaagtcattaacacaaagcagtgaaaatcatccagcaaagcagtgcttatgagagactagaattcagagaaatgcaaggtacgaacttctctctaatccaagggtattctgctgtgatcttctaatcagtgatgattgtgcttatgcacacgacatcttcatgggagagaccaggctgattgcaaaataatgacaaccaaccagtttacctcaacatagctcactctgcaatgtcagacatgcagtgtagagcagtcacaaagtcaagccatgaatacagggatggaaaaacattccagtgagctggtctctacaatttttaagacacttcatcctcccaattatattctttgtcataaagaggaaaaacagcaagattattaaatccaaaaagtcacagatgtcacaaggggatgaaataatttcctcattttttttctttatcagtgtaggaaaagctgtctttccatagcccacactcataatagcacttcaactaggctcctttgaaaatgaaaagtgaacaagtttcctaatgctggccttataagatctaaagagatgattaaattcaaaccaggctgagctcttactctgagctatttcagccactgatgtttgtaaaatataggaagaagattccaataggcaatttgcattggcaagcactggactacagaattcatcactgttttctgaaaaaatataattaaaccttaatggaattatgacacttttatgaggtttataattcacagccacctctcatcatattttgttcttctttccatttttaccatttcaaatattgcaatattgcccaccataaaccactgaaaatgattatttatgtatattccatttatttctctagggggtctaggtaatttgaatcaggagctccaagtaccatttaaaaaggtgagtctttaaaaaccatcagtgttttaaacacttgattagaaaaaagataacagctccttgtagtgatctagcttatgtgctttatggtatcttttcaaaaggagagtataaatcattgtacataaaatcaaaatagctaatatacatttttttctggcacttttgagaaattaggcattgaacataaaacatcttataaacttacataacaaaaataaatgtttacattttaatcttagattaccttagggtagcagttaacttatgagatgccacactgttggtgtgggcagcggagaccatgggaaatacacattcatgtccacagcccttcagcgatggatgcatggctgccgtccaaatatgtggtctgtgtcccaacataaagattaaggctctctgttttgaaggaatgagttctgggcttaaacaagtctagaagtaccacaatactcatggaaaatactgaaaagattcggacgagttttcaaacactgggggaaacacgtttttgactagaaaaataaaataaagcatctaaaactgacttcaagtactttggggagaggctgctgatatcgaatgccaaaataagaaggaacaaagacagaagagactccagggacgtccctccccatcccttcacccgcagggtccagatccccaggtgctgatgcgcaactctttggggaggactggcgagctgggcagaaagcagcagccatggtttgtcaccatcctaaaacacctatattgagggcaaaggccaagctttgtgtgaaaatttccttgggatgaaccacaggaatctggacatttcaagggggaaaaagccttaaagtcagtagcagacagagaaaaggaaagagaggaagaaaaacctgcttttctgaatggcagtactttaggccgggggcattgtggtccttggtgagtgcagcttttccatacagcttggctttcctcactaatgagatgagaccactgacagctgggatcttttgtgggtggtgagggtgcagcagggagatgtgcttgggtgtacctgtccatctggcaggcaggggcacactcaggtgcagcctagtccgtacctctctgtctcagaaactgaacaactgggagaacagtcgacagggcctctccaaccatcttcaggtgactaaagcagcatatgaagtataggtttgtgtcacttcttctcttccacagaagaaacgtctccagacactgatcacaggctacccagggttgtcttctgggttgctagagcctggtaatatctctgccttgctgcaagtcacttatgctctcgtagtcgttctcctttgggacgagaccgtggtggccattggtccccagggtggccttttcttcctctctgttgagagtctgtatcgcttcataatcaggctctggctcctcgctgggcctccctgctggtggaagtgtgctgtttggagttttttcgaagtctttaacagtagcatagagatcattacaggaggagggtgacctctgtgggtccccttgaatggaggtgtaggtggactccggaactgtaagcgactgccccgatttattcactaactgtccaggtttatttactgatgagtacatagctgagatctcttcttctgtgagagtggggtcttcttcccgagacttgtatgacaatgagctaaatctcttgttagtttcactggtcgtgtctgtggcactctcttccgcctctcccccttccttctcctgaaggttttcattctcgtccagaagcttaacagggacaggtggtggggcctcctcttctggatcacatgaatttccaaggatactctctacattaacactttgacgacattttttgtttctgtccaccgaggcatattcagcaaactcagctttgccttcagtctggggccctgggagctctttcgaggcagaagtagattttgccttgccactgtggcctttctccaggtgtgcagctgcagccacctccttgatctctttcacagtttcatacaagcagtcctccaccatgttttcttgggaggagctgtccttgagcacttcatagggcccttccatccccagcccctggtccccgtccacacttctcgccgtgagcatggtatccactgcgctctcgggagggattctgggcagctcccgactctgatgacattttggtttccctgtgctgtcctgggaatccagcagatccgaggccgatgtctggacttcctcgtaatgctgcatgcaggtcagagtactgtcctctgaaagaatgtccccattggtgagtgccccattctgctcactgctggcaggagcatctgttgccaggctagtaactgaacggctgaacatctccttgtctgaaggcacgttcatcaggttctcatggtccccactatgctgtcgcggcttcttttccctgtcacaactagagcacaggaagatgaggaaggtgatgacgaagaaaatggcgacagcagccagacttccccacagggtgatctgcatctgtccgctgcccagcaggctccccgcgggccccatggcaggagcaggcactggcaccagccgagggaatcagtcagtccttcaaaggtggtgacatggaggcagagagctgtgtcattttcgtttgcttcagtgataaagctgtgactgttttcagccatccctgagcacagacatcaagacggcaggggtggcttcgcagcaaaccagggtgcctccttggaggaaatgtttgtccagtagagtattccaagttctggcaatgta

SEQ ID NO: 9981 - RNA, 5636 nt, Homo sapiens
  source 1..5636: mol_type = other RNA
cacacacacacacacacgtatacgtgtgtgtgtgtgtgtgtgtgtgtgtagtttattactggttaagtaaatgctctaattagcaaaaatcatgagaaatatatacagtgatataatgcggttaaattttagttctctgtgttaactacttactgttaatttagtactcaattagaattaactctgggattttgagggcagataaatcagtaattagcctttatcccagaaagaatagtggtagcttcaaaagcttcaacagacctaatgatgtaatttattcaggacagaaaaaaaaatatgtagccaacattcttgcaagaattactttcttatggaatttaagatttcctcaaatattttcttttctatatagcgttttgttcttgtgtagttatctgcctaggatacagacaggatattgagactatttcagaaagtagacacactaaaaacatttgacaaattaaaaaaattttgcataaaacaggttaccctttcctgctgactatacttaagaaataccaaagtagcatacaaaatgcttctaaactttcaaaatatctgaataaaaacaaagatcctacttttaactgagatagatttataattcttacttacaagataaaaaaatttcctaaaatttatttttaaatttcacataacctgctataattcgctgtaaaaaatggatgtcaaaatagaattttaaatatacaaattgtttttgataactacctttcatacattttatttaaactgtagcattagctcaagatgaaactttttaaaagaaaccataggcttttgtccaactcaaagattcaagcccagattctgaacaaagtaaatgtgatgaaatttatgaaaaactatactgtacagtcaaaacagtgatggtgcctcagtaaataacttcagtaaaatatccagtgctccaaatagctgagccatctttctaaggttcactctgcttctctcccccagccctcatggcctgtgctaccatctattcttttagcgtttatgctggagggccttatagttcctttaaaagtacactgaaaatactttatatcacagcttattctaaccactggttctcaaattaaaaggtatatttcagtgcatatttcatagccacattgcagaactaatatttgaaaactcttgggggaaattttggtaacaaaattgcaaaatgacatgattatttatgagctttctataaaaagttttttttttttttttttttttactttagagatcatacctactttcctgcctttttgataagtaaggcatgaaatgaaacaaaagttttgagctgtaaggtgcctataaaggatgtcactacagcattcacaatgctaggtgtgtaagatgacatggctgttaccatgtactaaagaaccccatcatgtgagagatcgctcaaagtcattaacacaaagcagtgaaaatcatccagcaaagcagtgcttatgagagactagaattcagagaaatgcaaggtacgaacttctctctaatccaagggtattctgctgtgatcttctaatcagtgatgattgtgcttatgcacacgacatcttcatgggagagaccaggctgattgcaaaataatgacaaccaaccagtttacctcaacatagctcactctgcaatgtcagacatgcagtgtagagcagtcacaaagtcaagccatgaatacagggatggaaaaacattccagtgagctggtctctacaatttttaagacacttcatcctcccaattatattctttgtcataaagaggaaaaacagcaagattattaaatccaaaaagtcacagatgtcacaaggggatgaaataatttcctcattttttttctttatcagtgtaggaaaagctgtctttccatagcccacactcataatagcacttcaactaggctcctttgaaaatgaaaagtgaacaagtttcctaatgctggccttataagatctaaagagatgattaaattcaaaccaggctgagctcttactctgagctatttcagccactgatgtttgtaaaatataggaagaagattccaataggcaatttgcattggcaagcactggactacagaattcatcactgttttctgaaaaaatataattaaaccttaatggaattatgacacttttatgaggtttataattcacagccacctctcatcatattttgttcttctttccatttttaccatttcaaatattgcaatattgcccaccataaaccactgaaaatgattatttatgtatattccatttatttctctagggggtctaggtaatttgaatcaggagctccaagtaccatttaaaaaggtgagtctttaaaaaccatcagtgttttaaacacttgattagaaaaaagataacagctccttgtagtgatctagcttatgtgctttatggtatcttttcaaaaggagagtataaatcattgtacataaaatcaaaatagctaatatacatttttttctggcacttttgagaaattaggcattgaacataaaacatcttataaacttacataacaaaaataaatgtttacattttaatcttagattaccttagggtagcagttaacttatgagatgccacactgttggtgtgggcagcggagaccatgggaaatacacattcatgtccacagcccttcagcgatggatgcatggctgccgtccaaatatgtggtctgtgtcccaacataaagattaaggctctctgttttgaaggaatgagttctgggcttaaacaagtctagaagtaccacaatactcatggaaaatactgaaaagattcggacgagttttcaaacactgggggaaacacgtttttgactagaaaaataaaataaagcatctaaaactgacttcaagtactttggggagaggctgctgatatcgaatgccaaaataagaaggaacaaagacagaagagactccagggacgtccctccccatcccttcacccgcagggtccagatccccaggtgctgatgcgcaactctttggggaggactggcgagctgggcagaaagcagcagccatggtttgtcaccatcctaaaacacctatattgagggcaaaggccaagctttgtgtgaaaatttccttgggatgaaccacaggaatctggacatttcaagggggaaaaagccttaaagtcagtagcagacagagaaaaggaaagagaggaagaaaaacctgcttttctgaatggcagtactttaggccgggggcattgtggtccttggtgagtgcagcttttccatacagcttggctttcctcactaatgagatgagaccactgacagctgggatcttttgtgggtggtgagggtgcagcagggagatgtgcttgggtgtacctgtccatctggcaggcaggggcacactcaggtgcagcctagtccgtacctctctgtctcagaaactgaacaactgggagaacagtcgacagggcctctccaaccatcttcaggtgactaaagcagcatatgaagtataggtttgtgtcacttcttctcttccacagaagaaacgtctccagacactgatcacaggctacccagggttgtcttctgggttgctagagcctggtaatatctctgccttgctgcaagtcacttatgctctcgtagtcgttctcctttgggacgagaccgtggtggccattggtccccagggtggccttttcttcctctctgttgagagtctgtatcgcttcataatcaggctctggctcctcgctgggcctccctgctggtggaagtgtgctgtttggagttttttcgaagtctttaacagtagcatagagatcattacaggaggagggtgacctctgtgggtccccttgaatggaggtgtaggtggactccggaactgtaagcgactgccccgatttattcactaactgtccaggtttatttactgatgagtacatagctgagatctcttcttctgtgagagtggggtcttcttcccgagacttgtatgacaatgagctaaatctcttgttagtttcactggtcgtgtctgtggcactctcttccgcctctcccccttccttctcctgaaggttttcattctcgtccagaagcttaacagggacaggtggtggggcctcctcttctggatcacatgaatttccaaggatactctctacattaacactttgacgacattttttgtttctgtccaccgaggcatattcagcaaactcagctttgccttcagtctggggccctgggagctctttcgaggcagaagtagattttgccttgccactgtggcctttctccaggtgtgcagctgcagccacctccttgatctctttcacagtttcatacaagcagtcctccaccatgttttcttgggaggagctgtccttgagcacttcatagggcccttccatccccagcccctggtccccgtccacacttctcgccgtgagcatggtatccactgcgctctcgggagggattctgggcagctcccgactctgatgacattttggtttccctgtgctgtcctgggaatccagcagatccgaggccgatgtctggacttcctcgtaatgctgcatgcaggtcagagtactgtcctctgaaagaatgtccccattggtgagtgccccattctgctcactgctggcaggagcatctgttgccaggctagtaactgaacggctgaacatctccttgtctgaaggcacgttcatcaggttctcatggtccccactatgctgtcgcggcttcttttccctgtcacaactagagcacaggaagatgaggaaggtgatgacgaagaaaatggcgacagcagccagacttccccacagggtgatctgcatctgtccgctgcccagcaggctccccgcgggccccatggcaggagcaggcactggcaccagccgagggaatcagtcagtccttcaaaggtggtgacatggaggcagagagctgtgtccttggaggaaatgtttgtccagtagagtattccaagttctggcaatgtattccctttgaaatgttgtggtgagagttctctcttctttcttggccttttcccagcaatgaagttgtggccaactgctgaaataggagaaaaatctcgtgtttttgggactcaggaggcagggagtcttcctggcggacggcgctcggaggcagcctctgcaaactccggcgcgcagcgccgccgccccggcacagcccggcagcagcggcaagtgcaggaccaggcgccgccgctctgcaccagtcgccttggctcagctgtgccgggcgccgggcattcgccagggcacacgactcagcgaggcggcggctgggactgaggctactgcacccggccgcgcggacccgagcgctgcagctgcctccagccccggagcgcggcgctccgagcccctggtgggtgtctctggctccaagggaatcacggctcaattagggacctgccaggagaaaaaccgatgcgctgccgcaggcagagccgccagcccgcccccagtcggctggtcacatcgcgggcgcgcagacggacaagcgagcgggagggtaccgcagccagcactcgccgccgcgccgcggagaat

SEQ ID NO: 9982 - RNA, 5570 nt, Homo sapiens
  source 1..5570: mol_type = other RNA
cacacacacacacacacgtatacgtgtgtgtgtgtgtgtgtgtgtgtgtagtttattactggttaagtaaatgctctaattagcaaaaatcatgagaaatatatacagtgatataatgcggttaaattttagttctctgtgttaactacttactgttaatttagtactcaattagaattaactctgggattttgagggcagataaatcagtaattagcctttatcccagaaagaatagtggtagcttcaaaagcttcaacagacctaatgatgtaatttattcaggacagaaaaaaaaatatgtagccaacattcttgcaagaattactttcttatggaatttaagatttcctcaaatattttcttttctatatagcgttttgttcttgtgtagttatctgcctaggatacagacaggatattgagactatttcagaaagtagacacactaaaaacatttgacaaattaaaaaaattttgcataaaacaggttaccctttcctgctgactatacttaagaaataccaaagtagcatacaaaatgcttctaaactttcaaaatatctgaataaaaacaaagatcctacttttaactgagatagatttataattcttacttacaagataaaaaaatttcctaaaatttatttttaaatttcacataacctgctataattcgctgtaaaaaatggatgtcaaaatagaattttaaatatacaaattgtttttgataactacctttcatacattttatttaaactgtagcattagctcaagatgaaactttttaaaagaaaccataggcttttgtccaactcaaagattcaagcccagattctgaacaaagtaaatgtgatgaaatttatgaaaaactatactgtacagtcaaaacagtgatggtgcctcagtaaataacttcagtaaaatatccagtgctccaaatagctgagccatctttctaaggttcactctgcttctctcccccagccctcatggcctgtgctaccatctattcttttagcgtttatgctggagggccttatagttcctttaaaagtacactgaaaatactttatatcacagcttattctaaccactggttctcaaattaaaaggtatatttcagtgcatatttcatagccacattgcagaactaatatttgaaaactcttgggggaaattttggtaacaaaattgcaaaatgacatgattatttatgagctttctataaaaagttttttttttttttttttttttactttagagatcatacctactttcctgcctttttgataagtaaggcatgaaatgaaacaaaagttttgagctgtaaggtgcctataaaggatgtcactacagcattcacaatgctaggtgtgtaagatgacatggctgttaccatgtactaaagaaccccatcatgtgagagatcgctcaaagtcattaacacaaagcagtgaaaatcatccagcaaagcagtgcttatgagagactagaattcagagaaatgcaaggtacgaacttctctctaatccaagggtattctgctgtgatcttctaatcagtgatgattgtgcttatgcacacgacatcttcatgggagagaccaggctgattgcaaaataatgacaaccaaccagtttacctcaacatagctcactctgcaatgtcagacatgcagtgtagagcagtcacaaagtcaagccatgaatacagggatggaaaaacattccagtgagctggtctctacaatttttaagacacttcatcctcccaattatattctttgtcataaagaggaaaaacagcaagattattaaatccaaaaagtcacagatgtcacaaggggatgaaataatttcctcattttttttctttatcagtgtaggaaaagctgtctttccatagcccacactcataatagcacttcaactaggctcctttgaaaatgaaaagtgaacaagtttcctaatgctggccttataagatctaaagagatgattaaattcaaaccaggctgagctcttactctgagctatttcagccactgatgtttgtaaaatataggaagaagattccaataggcaatttgcattggcaagcactggactacagaattcatcactgttttctgaaaaaatataattaaaccttaatggaattatgacacttttatgaggtttataattcacagccacctctcatcatattttgttcttctttccatttttaccatttcaaatattgcaatattgcccaccataaaccactgaaaatgattatttatgtatattccatttatttctctagggggtctaggtaatttgaatcaggagctccaagtaccatttaaaaaggtgagtctttaaaaaccatcagtgttttaaacacttgattagaaaaaagataacagctccttgtagtgatctagcttatgtgctttatggtatcttttcaaaaggagagtataaatcattgtacataaaatcaaaatagctaatatacatttttttctggcacttttgagaaattaggcattgaacataaaacatcttataaacttacataacaaaaataaatgtttacattttaatcttagattaccttagggtagcagttaacttatgagatgccacactgttggtgtgggcagcggagaccatgggaaatacacattcatgtccacagcccttcagcgatggatgcatggctgccgtccaaatatgtggtctgtgtcccaacataaagattaaggctctctgttttgaaggaatgagttctgggcttaaacaagtctagaagtaccacaatactcatggaaaatactgaaaagattcggacgagttttcaaacactgggggaaacacgtttttgactagaaaaataaaataaagcatctaaaactgacttcaagtactttggggagaggctgctgatatcgaatgccaaaataagaaggaacaaagacagaagagactccagggacgtccctccccatcccttcacccgcagggtccagatccccaggtgctgatgcgcaactctttggggaggactggcgagctgggcagaaagcagcagccatggtttgtcaccatcctaaaacacctatattgagggcaaaggccaagctttgtgtgaaaatttccttgggatgaaccacaggaatctggacatttcaagggggaaaaagccttaaagtcagtagcagacagagaaaaggaaagagaggaagaaaaacctgcttttctgaatggcagtactttaggccgggggcattgtggtccttggtgagtgcagcttttccatacagcttggctttcctcactaatgagatgagaccactgacagctgggatcttttgtgggtggtgagggtgcagcagggagatgtgcttgggtgtacctgtccatctggcaggcaggggcacactcaggtgcagcctagtccgtacctctctgtctcagaaactgaacaactgggagaacagtcgacagggcctctccaaccatcttcaggtgactaaagcagcatatgaagtataggtttgtgtcacttcttctcttccacagaagaaacgtctccagacactgatcacaggctacccagggttgtcttctgggttgctagagcctggtaatatctctgccttgctgcaagtcacttatgctctcgtagtcgttctcctttgggacgagaccgtggtggccattggtccccagggtggccttttcttcctctctgttgagagtctgtatcgcttcataatcaggctctggctcctcgctgggcctccctgctggtggaagtgtgctgtttggagttttttcgaagtctttaacagtagcatagagatcattacaggaggagggtgacctctgtgggtccccttgaatggaggtgtaggtggactccggaactgtaagcgactgccccgatttattcactaactgtccaggtttatttactgatgagtacatagctgagatctcttcttctgtgagagtggggtcttcttcccgagacttgtatgacaatgagctaaatctcttgttagtttcactggtcgtgtctgtggcactctcttccgcctctcccccttccttctcctgaaggttttcattctcgtccagaagcttaacagggacaggtggtggggcctcctcttctggatcacatgaatttccaaggatactctctacattaacactttgacgacattttttgtttctgtccaccgaggcatattcagcaaactcagctttgccttcagtctggggccctgggagctctttcgaggcagaagtagattttgccttgccactgtggcctttctccaggtgtgcagctgcagccacctccttgatctctttcacagtttcatacaagcagtcctccaccatgttttcttgggaggagctgtccttgagcacttcatagggcccttccatccccagcccctggtccccgtccacacttctcgccgtgagcatggtatccactgcgctctcgggagggattctgggcagctcccgactctgatgacattttggtttccctgtgctgtcctgggaatccagcagatccgaggccgatgtctggacttcctcgtaatgctgcatgcaggtcagagtactgtcctctgaaagaatgtccccattggtgagtgccccattctgctcactgctggcaggagcatctgttgccaggctagtaactgaacggctgaacatctccttgtctgaaggcacgttcatcaggttctcatggtccccactatgctgtcgcggcttcttttccctgtcacaactagagcacaggaagatgaggaaggtgatgacgaagaaaatggcgacagcagccagacttccccacagggtgatctgcatctgtccgctgcccagcaggctccccgcgggccccatggcaggagcaggcactggcaccagccgagggaatcagtcagtccttcaaaggtggtgacatggaggcagagagctgtgtccttggaggaaatgtttgtccagtagagtattccaagttctggcaatgtattccctttgaaatgttgtggtgagagttctctcttctttcttggctgggactcaggaggcagggagtcttcctggcggacggcgctcggaggcagcctctgcaaactccggcgcgcagcgccgccgccccggcacagcccggcagcagcggcaagtgcaggaccaggcgccgccgctctgcaccagtcgccttggctcagctgtgccgggcgccgggcattcgccagggcacacgactcagcgaggcggcggctgggactgaggctactgcacccggccgcgcggacccgagcgctgcagctgcctccagccccggagcgcggcgctccgagcccctggtgggtgtctctggctccaagggaatcacggctcaattagggacctgccaggagaaaaaccgatgcgctgccgcaggcagagccgccagcccgcccccagtcggctggtcacatcgcgggcgcgcagacggacaagcgagcgggagggtaccgcagccagcactcgccgccgcgccgc

SEQ ID NO: 9983 - RNA, 4448 nt, Homo sapiens
  source 1..4448: mol_type = other RNA
cacacacacacacacacgtatagatcacgtatctgtattactaacccagtcatacacatgaagagccgagtgtgcatgtgtgcaccacacatgtatgcatgcaggctcacacaggcacacgcctccacacacacactccccaggggccaagtcttcctcgctcctggctcatcccatccgccctcccgcttcaagtgcactaaagagggagactattttggtctttagcacaagcaataaataaataaataaatacgagggaaggaagaaagagggcaggagaatcaagcatctgccgcctttggggagatgaggcgctggggctgctctcccgcagggtgggggctgggaggtaagagcacagacctccaagagggccaggaggtgggcctggggtcctcggactcagctctgggtcgggggagtagaaggctgtctcactggccctggaagggcacaggcccctacaccagcaccaagtgaccagggtcaccactgtccctcagcatggccatcagggaggcgaagtgtcaagctctcccctgccaacttcaccccagtacccagggctaaggctgagaaggcccctaaggcttcggggctaggcctgggagcaggaaccagctgaggcacccctggcagaccccgagaggaaagagctgcctcggcggaatcttctatgccagaaatgagtgtggggctgaagctgggacaggatgctgagtcgggcctaccccaggatgtaggggtcgggtgtcttgacttccattgccccagacctcagggctgagtcttcagctgctaaggaggggaggaggtggagggaagaggcagacacccccaccccacgcccccagcccctctctgtctcctgcaccccacccactcactgcatgaccccctctgctctctgcctcagcttccccacttgggccagagtcctcggtgccttctggctctgagctgtctcggggtgccttctggctctgagctgtctcggggtgccttctggctctgagctgtctcgggggcagagttggagcaggagacacatcctttctgattactggcttctggagaagcccgactagaagagagcaggttttctccgcagccctgggaagggcctggctctaccatggacctgacccaaccagctgccatgaacaagatggggtggcagagccagcagtgacaacaaggggaccccaaacctcttcctgatgagggtgccatagtgcctcaacctgggggagggtggtggaggagcggccctggaagactcggcaggaattctgttccacggctggtttctgattcagctttgaatgagcgtggccctccccagtcatcccagttggcaggagggggtggcgattcctctcctttcctaagatctttcctctgccattcagcgctgaccagggcctggctgtgccctgcctgaactctgctgtgctgctccaggtgagggagggacaggatgtggtcctatgtcaggcagacctggcccctgccaccttcacaaggcagacagaggggctggaggaacttcagcagtggaggtatgggaggggtggggtgggacagggttggggggagatgagcaagcccagaaagaacaggacaacccggagtctctaaggcacgactcacactgtgggcccagtggggacggggctgccagcttcctcctagcctgggatcccgacttcccttcccaaggagccatcccggcctatagctcctaaccacccctcactgtggaattgggcggaggcctggacagaaatggagagagaagcaaaacaggaaaatcgagggtgcggggaggaaccctcgatggcaggtcccatgcctggccctgagacacatctctaaggtacaaaggcaaactctaaaagctcaaaccagtttcttcccagccccacccaccaccccaacgacagtagaaagcttttattacgatcattaacatggtcttgatttttctatcacaaacagagcctagctggctcgtgagctcgatgaagtgcggtcccagagcaccctgcttgcccagggactgtggtgcccacacacacggggagaggccagtcccacctcggggaaccctctggagccttcagccagctgctgcatcctggcagacccatggaattctaattgttctttttgccccctgtgaattaaaaaaaaattttttcaattgcatggtaattttttttttttgtaaacagtctcacccaagctaaggtcaagaaagctgaaacccggtgtttctccccaagttaaaaaccagcaaggagcaccgcagctagccagccttggacagcagaggctgggcccaccatcgagctgagctgcttccccgcaggctgcagctccatcttcaggcagaagccctggccctcgtggcctggccccccaggaggccacttctttgccctgagcctgtgatagcctctgaggccgggggctgccgctctggctgccccctctccggccaaacttctgaggccgttgcaaagaaacataaaacgactaaaacgctactgagtctgcaacccagggcactgggcccgttctgctcaaacccggggcccctgagcgaccgcggggcctctccccagccgggggtggatgctgcatgtcggccaaggttggctcagatctctgactcccgtctgtagggccgctgctccaggaccccgccgccagcctggagtctgtcaaagtcatgcctggcctgggggctgaggccgtcccggcttcggccgtcctggtctccgtccgcctcatcctcctcgtcacggctcaggaaggccagctcgttctcgtagcagaaggagttggcgctgggcagcaggaacttgttctctaccagatccttcgcactgcagcggggcgtagagggcacctcataggtcttgtggaagtgcgagtagtcaatcttgtactggttcttctcctcgaagagcacgggctcaaagcggtgaccccacaggatctcattggccaggtaggagctgcgggcctgggtggtcatggctgtggcctccaccatgccttccaggatgaccacgatctcaaagtcgtccgtctccaggtcctgccggctgatgccgaagagcgggctggcctcgtcaatctcatgcaagatggtgatgggcgacaccagaaagatgcggtccaggcccttgtcgaagcccacatcgatgtcgatctggtccagcgggatgtactcgccctcctcggtgacccgcggcttgatgagctgcgcgcgcacatgggcctccacaatgtggctcttgcgcaggttacccacacgccacatgaggcagagcttgccgtcacgcagggccaccacggcgttgtggctgaacagcagcgtctgtgcccgcttcttgggccttgccatcttggccatgatggcaccaatcatgaaggagtcgatgatgcagcccacgatggactgggccaccaccatgaagacggccaccgggcactcctccgtcacacagcgcagcccgtagccgatggtggtctgcgtctcgatggagaagaggaaggccgccatgaagccgtgcacctgcatcacacagggtgtgcggccccggccctcagccggctccaggtcaccgtgtgccaccgcgatgacccagaagatgatgccgaacagcagccaggaggcaaggaaggccagcgagaagatgagcagcatgtaccgccagcggatgtccacacaggtggtgaacatgtcagccaggtagcgctgtgacttctcgtccatgttggcgaactcaatgttgcactggccattcttcttgacgaagcggttgcggcacctgcgccgcgtgtgcaccttgccgttgccgaagccgttggcgcccgacatggtgaccaggtgcagcccgtcctcctccgatgacacgatgctgtaggggttggcccggctggccgcggtcatcccgggggttgggggaccctggctcgcccccaggctagctccaggcagggcggctcctcttgagttctatcttctatgtaatggtgctgagtgggcacggtactgtcttcaaggctgaattagtagtggctgccatttcccaggcaccaactggaaaggatccagtcactagaacatcctccgcacctcccagccagggagttcatggggcctgccctttccaaggttacagccaaggctggtttgtcacactggtttttctggctggaattaaggcaaatgttggtaagtcacccccacctcattagcctcctgggacaggtgacagtggtttagaggcacacagacctagattcaaatcccagctctgcccctcataagctgtgtgaccttgagtgagtcacttcccctctctcagcttgttctgaaatgggatggcctgcctggtctctagtggcccttcagtccctcttcaccc

SEQ ID NO: 9984 - RNA, 4469 nt, Homo sapiens
  source 1..4469: mol_type = other RNA
cacacacacacacacacgtatagatcacgtatctgtattactaacccagtcatacacatgaagagccgagtgtgcatgtgtgcaccacacatgtatgcatgcaggctcacacaggcacacgcctccacacacacactccccaggggccaagtcttcctcgctcctggctcatcccatccgccctcccgcttcaagtgcactaaagagggagactattttggtctttagcacaagcaataaataaataaataaatacgagggaaggaagaaagagggcaggagaatcaagcatctgccgcctttggggagatgaggcgctggggctgctctcccgcagggtgggggctgggaggtaagagcacagacctccaagagggccaggaggtgggcctggggtcctcggactcagctctgggtcgggggagtagaaggctgtctcactggccctggaagggcacaggcccctacaccagcaccaagtgaccagggtcaccactgtccctcagcatggccatcagggaggcgaagtgtcaagctctcccctgccaacttcaccccagtacccagggctaaggctgagaaggcccctaaggcttcggggctaggcctgggagcaggaaccagctgaggcacccctggcagaccccgagaggaaagagctgcctcggcggaatcttctatgccagaaatgagtgtggggctgaagctgggacaggatgctgagtcgggcctaccccaggatgtaggggtcgggtgtcttgacttccattgccccagacctcagggctgagtcttcagctgctaaggaggggaggaggtggagggaagaggcagacacccccaccccacgcccccagcccctctctgtctcctgcaccccacccactcactgcatgaccccctctgctctctgcctcagcttccccacttgggccagagtcctcggtgccttctggctctgagctgtctcggggtgccttctggctctgagctgtctcggggtgccttctggctctgagctgtctcgggggcagagttggagcaggagacacatcctttctgattactggcttctggagaagcccgactagaagagagcaggttttctccgcagccctgggaagggcctggctctaccatggacctgacccaaccagctgccatgaacaagatggggtggcagagccagcagtgacaacaaggggaccccaaacctcttcctgatgagggtgccatagtgcctcaacctgggggagggtggtggaggagcggccctggaagactcggcaggaattctgttccacggctggtttctgattcagctttgaatgagcgtggccctccccagtcatcccagttggcaggagggggtggcgattcctctcctttcctaagatctttcctctgccattcagcgctgaccagggcctggctgtgccctgcctgaactctgctgtgctgctccaggtgagggagggacaggatgtggtcctatgtcaggcagacctggcccctgccaccttcacaaggcagacagaggggctggaggaacttcagcagtggaggtatgggaggggtggggtgggacagggttggggggagatgagcaagcccagaaagaacaggacaacccggagtctctaaggcacgactcacactgtgggcccagtggggacggggctgccagcttcctcctagcctgggatcccgacttcccttcccaaggagccatcccggcctatagctcctaaccacccctcactgtggaattgggcggaggcctggacagaaatggagagagaagcaaaacaggaaaatcgagggtgcggggaggaaccctcgatggcaggtcccatgcctggccctgagacacatctctaaggtacaaaggcaaactctaaaagctcaaaccagtttcttcccagccccacccaccaccccaacgacagtagaaagcttttattacgatcattaacatggtcttgatttttctatcacaaacagagcctagctggctcgtgagctcgatgaagtgcggtcccagagcaccctgcttgcccagggactgtggtgcccacacacacggggagaggccagtcccacctcggggaaccctctggagccttcagccagctgctgcatcctggcagacccatggaattctaattgttctttttgccccctgtgaattaaaaaaaaattttttcaattgcatggtaattttttttttttgtaaacagtctcacccaagctaaggtcaagaaagctgaaacccggtgtttctccccaagttaaaaaccagcaaggagcaccgcagctagccagccttggacagcagaggctgggcccaccatcgagctgagctgcttccccgcaggctgcagctccatcttcaggcagaagccctggccctcgtggcctggccccccaggaggccacttctttgccctgagcctgtgatagcctctgaggccgggggctgccgctctggctgccccctctccggccaaacttctgaggccgttgcaaagaaacataaaacgactaaaacgctactgagtctgcaacccagggcactgggcccgttctgctcaaacccggggcccctgagcgaccgcggggcctctccccagccgggggtggatgctgcatgtcggccaaggttggctcagatctctgactcccgtctgtagggccgctgctccaggaccccgccgccagcctggagtctgtcaaagtcatgcctggcctgggggctgaggccgtcccggcttcggccgtcctggtctccgtccgcctcatcctcctcgtcacggctcaggaaggccagctcgttctcgtagcagaaggagttggcgctgggcagcaggaacttgttctctaccagatccttcgcactgcagcggggcgtagagggcacctcataggtcttgtggaagtgcgagtagtcaatcttgtactggttcttctcctcgaagagcacgggctcaaagcggtgaccccacaggatctcattggccaggtaggagctgcgggcctgggtggtcatggctgtggcctccaccatgccttccaggatgaccacgatctcaaagtcgtccgtctccaggtcctgccggctgatgccgaagagcgggctggcctcgtcaatctcatgcaagatggtgatgggcgacaccagaaagatgcggtccaggcccttgtcgaagcccacatcgatgtcgatctggtccagcgggatgtactcgccctcctcggtgacccgcggcttgatgagctgcgcgcgcacatgggcctccacaatgtggctcttgcgcaggttacccacacgccacatgaggcagagcttgccgtcacgcagggccaccacggcgttgtggctgaacagcagcgtctgtgcccgcttcttgggccttgccatcttggccatgatggcaccaatcatgaaggagtcgatgatgcagcccacgatggactgggccaccaccatgaagacggccaccgggcactcctccgtcacacagcgcagcccgtagccgatggtggtctgcgtctcgatggagaagaggaaggccgccatgaagccgtgcacctgcatcacacagggtgtgcggccccggccctcagccggctccaggtcaccgtgtgccaccgcgatgacccagaagatgatgccgaacagcagccaggaggcaaggaaggccagcgagaagatgagcagcatgtaccgccagcggatgtccacacaggtggtgaacatgtcagccaggtagcgctgtgacttctcgtccatgttggcgaactcaatgttgcactggccattcttcttgacgaagcggttgcggcacctgcgccgcgtgtgcaccttgccgttgccgaagccgttggcgcccgacatggtgaccaggtgcagcccgtcctcctccgatgacacgatgctgtaggggttggcccggctggccgcggtcatcccgggggttgggggaccctggctcgcccccaggctagctccaggcagggcggctcctcttgagttctatcttctatgtaatggtgctgagtgggcacggtactgtcttcaaggctgaattagtagtggctgccatttcccaggcaccaactggaaaggatccagtcactagaacatcctcgatcgcggggtctccgggaaggtcacgcgtaggacccgtgccgcgcgccagagtgcttccgcacgctccctcccgagccccctagtgcaaaccagtcagaggggggccgagggctcctcaaagtttcccggagcgccccccaggacgaaggttagccaggagcaaagttccttgtggtggtagccggagacatggcaggaaaagaaaagctcgcagtcagcatttcctccgatgtctcaccaagggagggaaaaaaataaaacgagaggaagaaaacaccctcccgctccaccttccctgttgctgcacaacctcgtg

SEQ ID NO: 9985 - RNA, 4705 nt, Homo sapiens
  source 1..4705: mol_type = other RNA
cacacacacacacacacgtatagatcacgtatctgtattactaacccagtcatacacatgaagagccgagtgtgcatgtgtgcaccacacatgtatgcatgcaggctcacacaggcacacgcctccacacacacactccccaggggccaagtcttcctcgctcctggctcatcccatccgccctcccgcttcaagtgcactaaagagggagactattttggtctttagcacaagcaataaataaataaataaatacgagggaaggaagaaagagggcaggagaatcaagcatctgccgcctttggggagatgaggcgctggggctgctctcccgcagggtgggggctgggaggtaagagcacagacctccaagagggccaggaggtgggcctggggtcctcggactcagctctgggtcgggggagtagaaggctgtctcactggccctggaagggcacaggcccctacaccagcaccaagtgaccagggtcaccactgtccctcagcatggccatcagggaggcgaagtgtcaagctctcccctgccaacttcaccccagtacccagggctaaggctgagaaggcccctaaggcttcggggctaggcctgggagcaggaaccagctgaggcacccctggcagaccccgagaggaaagagctgcctcggcggaatcttctatgccagaaatgagtgtggggctgaagctgggacaggatgctgagtcgggcctaccccaggatgtaggggtcgggtgtcttgacttccattgccccagacctcagggctgagtcttcagctgctaaggaggggaggaggtggagggaagaggcagacacccccaccccacgcccccagcccctctctgtctcctgcaccccacccactcactgcatgaccccctctgctctctgcctcagcttccccacttgggccagagtcctcggtgccttctggctctgagctgtctcggggtgccttctggctctgagctgtctcggggtgccttctggctctgagctgtctcgggggcagagttggagcaggagacacatcctttctgattactggcttctggagaagcccgactagaagagagcaggttttctccgcagccctgggaagggcctggctctaccatggacctgacccaaccagctgccatgaacaagatggggtggcagagccagcagtgacaacaaggggaccccaaacctcttcctgatgagggtgccatagtgcctcaacctgggggagggtggtggaggagcggccctggaagactcggcaggaattctgttccacggctggtttctgattcagctttgaatgagcgtggccctccccagtcatcccagttggcaggagggggtggcgattcctctcctttcctaagatctttcctctgccattcagcgctgaccagggcctggctgtgccctgcctgaactctgctgtgctgctccaggtgagggagggacaggatgtggtcctatgtcaggcagacctggcccctgccaccttcacaaggcagacagaggggctggaggaacttcagcagtggaggtatgggaggggtggggtgggacagggttggggggagatgagcaagcccagaaagaacaggacaacccggagtctctaaggcacgactcacactgtgggcccagtggggacggggctgccagcttcctcctagcctgggatcccgacttcccttcccaaggagccatcccggcctatagctcctaaccacccctcactgtggaattgggcggaggcctggacagaaatggagagagaagcaaaacaggaaaatcgagggtgcggggaggaaccctcgatggcaggtcccatgcctggccctgagacacatctctaaggtacaaaggcaaactctaaaagctcaaaccagtttcttcccagccccacccaccaccccaacgacagtagaaagcttttattacgatcattaacatggtcttgatttttctatcacaaacagagcctagctggctcgtgagctcgatgaagtgcggtcccagagcaccctgcttgcccagggactgtggtgcccacacacacggggagaggccagtcccacctcggggaaccctctggagccttcagccagctgctgcatcctggcagacccatggaattctaattgttctttttgccccctgtgaattaaaaaaaaattttttcaattgcatggtaattttttttttttgtaaacagtctcacccaagctaaggtcaagaaagctgaaacccggtgtttctccccaagttaaaaaccagcaaggagcaccgcagctagccagccttggacagcagaggctgggcccaccatcgagctgagctgcttccccgcaggctgcagctccatcttcaggcagaagccctggccctcgtggcctggccccccaggaggccacttctttgccctgagcctgtgatagcctctgaggccgggggctgccgctctggctgccccctctccggccaaacttctgaggccgttgcaaagaaacataaaacgactaaaacgctactgagtctgcaacccagggcactgggcccgttctgctcaaacccggggcccctgagcgaccgcggggcctctccccagccgggggtggatgctgcatgtcggccaaggttggctcagatctctgactcccgtctgtagggccgctgctccaggaccccgccgccagcctggagtctgtcaaagtcatgcctggcctgggggctgaggccgtcccggcttcggccgtcctggtctccgtccgcctcatcctcctcgtcacggctcaggaaggccagctcgttctcgtagcagaaggagttggcgctgggcagcaggaacttgttctctaccagatccttcgcactgcagcggggcgtagagggcacctcataggtcttgtggaagtgcgagtagtcaatcttgtactggttcttctcctcgaagagcacgggctcaaagcggtgaccccacaggatctcattggccaggtaggagctgcgggcctgggtggtcatggctgtggcctccaccatgccttccaggatgaccacgatctcaaagtcgtccgtctccaggtcctgccggctgatgccgaagagcgggctggcctcgtcaatctcatgcaagatggtgatgggcgacaccagaaagatgcggtccaggcccttgtcgaagcccacatcgatgtcgatctggtccagcgggatgtactcgccctcctcggtgacccgcggcttgatgagctgcgcgcgcacatgggcctccacaatgtggctcttgcgcaggttacccacacgccacatgaggcagagcttgccgtcacgcagggccaccacggcgttgtggctgaacagcagcgtctgtgcccgcttcttgggccttgccatcttggccatgatggcaccaatcatgaaggagtcgatgatgcagcccacgatggactgggccaccaccatgaagacggccaccgggcactcctccgtcacacagcgcagcccgtagccgatggtggtctgcgtctcgatggagaagaggaaggccgccatgaagccgtgcacctgcatcacacagggtgtgcggccccggccctcagccggctccaggtcaccgtgtgccaccgcgatgacccagaagatgatgccgaacagcagccaggaggcaaggaaggccagcgagaagatgagcagcatgtaccgccagcggatgtccacacaggtggtgaacatgtcagccaggtagcgctgtgacttctcgtccatgttggcgaactcaatgttgcactggccattcttcttgacgaagcggttgcggcacctgcgccgcgtgtgcaccttgccgttgccgaagccgttggcgcccgacatggtgaccaggtgcagcccgtcctcctccgatgacacgatgctgtaggggttggcccggctggccgcggtcatcccgggggttgggggaccctggctcgcccccaggctagctccaggcagggcggctcctcttgagttctatcttctatgtaatggtgctgagtgggcacggtactgtcttcaaggctgaattagtagtggctgccatttcccaggcaccaactggaaaggatccagtcactagaacatcctcggtcagtggcccgggcgcggcgcgctcggcgtcctccaagctccgggcggccgttcctggccccggcagctgccgcgctggctgcatcgccgccgctgccgccaccgcctcagggcagctcccgggggcgctccatgccgaggggcgcgtcttctctgcaaagcggatcgccctggtccagccacgggtcgggggcgcgcgcctggacggcgcccccggccgctgggcgctcgcttgggccggggcggctggcgtcggtccctcggtccggctgtgagcacggccggcccaccccctcccccgccggctgttatctgatctcgggcagggcccggcgcgctcccctacgccccggcgccccgcacctcctcgcaggctctgaccgcgccagtccccctcccccggctactgttcccagggaggcggcagcagtggcggtgtggccgggagaagacggggagcgaggaatggagggcgaggaggcggcgggaggcagaggctcggcgcgcacccagctccgcgcctcgctccaccggagctcagctcggcaactc

SEQ ID NO: 9986 - RNA, 2159 nt, Homo sapiens
  source 1..2159: mol_type = other RNA
cacacacacacacacacgtatatatatgtatatatacagtattaggtacaaatggcaattaacagtccctacaaaaattcaatttcagttgaggctatggctcctatgccttgggatggtttcgaacttcaaaactgaaaaatactgctaaaatctcacttccttaacacaaaatttgattatatgttcagtttaagctctcagtctaaaaatggctataaggtaagtattaaaaagccagccaactgagtgcaacttctctctccaatctggccacgctattttgtagaaattattcctaactagactagaaaatctgtggtgacttccaatggtcttgcctaccttactgcccatgttcacgtttcaaactgtgtcaacaaagcccgcacttcgggggtcagctgcttggcagccttagctgcctctgtgatagccttgcgatacaggccctttctcttcttattaaagcgtgactggaagttttctaaaaagggggagagttgtgaaagagcaaggaaagatgttgttggagacccaaaccatgaaatacgggcctcctgtcggactaaaaggccgttatctttccggctcacagttatagtaagaatacgggctggccaccaagggaagccatatatcttggcccaaacaatgtcccctacacatatggtcctgccatctggtgtgacgcatttagagacgtttttggaaaagactttcattttcaaggaattactgagctttttctcttcctttgaagaggaggaagtggaggaggtggaaggtgcatgcatactgcctggaggaaaatcaaagctttcagaagaactacactcagagttggaagatttcaaatcatctgtgctatcaatgctacacactgaagcactggaagagtcagatttcttttgatttagggtcatataaacagagatattgtttttgctgccctttttgcccaatgtctgtggttcatcctgatcaccaggcacatgcacttcatttgtgtcctgaacctcactgctggcctcttcagggccttttgagggactctgattttctgaaggggcctcacctgctgagcgggtagaggtgcagcgagactggggcttgggtgccatcttgccactccgcattttctcaagtcctgtcttcagagaagagtcattttcttcattcctgtacctctgtggttttaaacgaacccggggtggaagggaacctgagctaggattctgatatcgacgtgtgaaatggacttttgaatgtgcatttttggaagtagaggtttcattttgcttcttttgtgccttttctttggcaatttttaacacttcccgagctttcgcatgatccatgttcttactctggagaacttttttagtacttaactgagcttttgatgtatttgcctgagcagaaacttttactactctgcctctgctgtgagcaatatttgaaaccttaaccacagcatttcttttctggctttcattttggtttttcccatccactttatggtcagttttcagttttttgttcacagtagttacactttcatttctccgttttttatcttcatatttagaagagtcagttgcactactaccttttctaatttcctttttttcagcaacaacactgtttttacatttatcacacagaacttgcctgggtcgtagtttaatagcattcattattgaagtgggttcttccctgtacatttttcgtttgggtcgcttaattttccgaggaggtggctgaggtattgattggttatatgtgtccctgataaacaaagggggaggataaggtgctccttcatggaagagaggtggtggtttggaagtccacaggctttcagccaagctcagctcgggatgcgggacaggagaagggtcatcgggaacagcaccatttgcttcacacttgacttctgtcccttcttggaatgtattactttggagcggcatggcttctggtttatccttatattcccttttgggaaatactgtcacagggataccatggggcccaaacctactaaaagactataacaatttcctcataagccatcagccccaggtgctaatgagagaaagagaaaaagattaagaaagaggttacagtgagccaagatcgcaccactgcactcc

SEQ ID NO: 9987 - RNA, 2358 nt, Homo sapiens
  source 1..2358: mol_type = other RNA
cacacacacacacacacgtatatatatgtatatatacagtattaggtacaaatggcaattaacagtccctacaaaaattcaatttcagttgaggctatggctcctatgccttgggatggtttcgaacttcaaaactgaaaaatactgctaaaatctcacttccttaacacaaaatttgattatatgttcagtttaagctctcagtctaaaaatggctataaggtaagtattaaaaagccagccaactgagtgcaacttctctctccaatctggccacgctattttgtagaaattattcctaactagactagaaaatctgtggtgacttccaatggtcttgcctaccttactgcccatgttcacgtttcaaactgtgtcaacaaagcccgcacttcgggggtcagctgcttggcagccttagctgcctctgtgatagccttgcgatacaggccctttctcttcttattaaagcgtgactggaagttttctaaaaagggggagagttgtgaaagagcaaggaaagatgttgttggagacccaaaccatgaaatacgggcctcctgtcggactaaaaggccgttatctttccggctcacagttatagtaagaatacgggctggccaccaagggaagccatatatcttggcccaaacaatgtcccctacacatatggtcctgccatctggtgtgacgcatttagagacgtttttggaaaagactttcattttcaaggaattactgagctttttctcttcctttgaagaggaggaagtggaggaggtggaaggtgcatgcatactgcctggaggaaaatcaaagctttcagaagaactacactcagagttggaagatttcaaatcatctgtgctatcaatgctacacactgaagcactggaagagtcagatttcttttgatttagggtcatataaacagagatattgtttttgctgccctttttgcccaatgtctgtggttcatcctgatcaccaggcacatgcacttcatttgtgtcctgaacctcactgctggcctcttcagggccttttgagggactctgattttctgaaggggcctcacctgctgagcgggtagaggtgcagcgagactggggcttgggtgccatcttgccactccgcattttctcaagtcctgtcttcagagaagagtcattttcttcattcctgtacctctgtggttttaaacgaacccggggtggaagggaacctgagctaggattctgatatcgacgtgtgaaatggacttttgaatgtgcatttttggaagtagaggtttcattttgcttcttttgtgccttttctttggcaatttttaacacttcccgagctttcgcatgatccatgttcttactctggagaacttttttagtacttaactgagcttttgatgtatttgcctgagcagaaacttttactactctgcctctgctgtgagcaatatttgaaaccttaaccacagcatttcttttctggctttcattttggtttttcccatccactttatggtcagttttcagttttttgttcacagtagttacactttcatttctccgttttttatcttcatatttagaagagtcagttgcactactaccttttctaatttcctttttttcagcaacaacactgtttttacatttatcacacagaacttgcctgggtcgtagtttaatagcattcattattgaagtgggttcttccctgtacatttttcgtttgggtcgcttaattttccgaggaggtggctgaggtattgattggttatatgtgtccctgataaacaaagggggaggataaggtgctccttcatggaagagaggtggtggtttggaagtccacaggctttcagccaagctcagctcgggatgcgggacaggagaagggtcatcgggaacagcaccatttgcttcacacttgacttctgtcccttcttggaatgtattactttggagcggcatggcttctggtttatccttatattcccttttgggaaatactgtcacagggataccatggggcccaaacctactaaaagactataacaatttcctcataagccatcagccccaggtgtgcttcaccagaatggctgtatatttttcccaccaaaagtagggctattgcaccatacgtttcatggtctcttctgcaccttccttttgcagatttgaaatccagattctcacacaatcactggccatctcttctgtttcattcaacagcatacacaccagagtgtctcttactattatatacatcagtagaggccgggcgaggtggctcatgcctgtaatctcagcactttgggaggccaaggtgggtggatcacctgaggtcagg

SEQ ID NO: 9988 - RNA, 3876 nt, Homo sapiens
  source 1..3876: mol_type = other RNA
cacacacacacacacacgtatatatatgtatatatacagtattaggtacaaatggcaattaacagtccctacaaaaattcaatttcagttgaggctatggctcctatgccttgggatggtttcgaacttcaaaactgaaaaatactgctaaaatctcacttccttaacacaaaatttgattatatgttcagtttaagctctcagtctaaaaatggctataaggtaagtattaaaaagccagccaactgagtgcaacttctctctccaatctggccacgctattttgtagaaattattcctaactagactagaaaatctgtggtgacttccaatggtcttgcctaccttactgcccatgttcacgtttcaaactgtgtcaacaaagcccgcacttcgggggtcagctgcttggcagccttagctgcctctgtgatagccttgcgatacaggccctttctcttcttattaaagcgtgactggaagttttctaaaaagggggagagttgtgaaagagcaaggaaagatgttgttggagacccaaaccatgaaatacgggcctcctgtcggactaaaaggccgttatctttccggctcacagttatagtaagaatacgggctggccaccaagggaagccatatatcttggcccaaacaatgtcccctacacatatggtcctgccatctggtgtgacgcatttagagacgtttttggaaaagactttcattttcaaggaattactgagctttttctcttcctttgaagaggaggaagtggaggaggtggaaggtgcatgcatactgcctggaggaaaatcaaagctttcagaagaactacactcagagttggaagatttcaaatcatctgtgctatcaatgctacacactgaagcactggaagagtcagatttcttttgatttagggtcatataaacagagatattgtttttgctgccctttttgcccaatgtctgtggttcatcctgatcaccaggcacatgcacttcatttgtgtcctgaacctcactgctggcctcttcagggccttttgagggactctgattttctgaaggggcctcacctgctgagcgggtagaggtgcagcgagactggggcttgggtgccatcttgccactccgcattttctcaagtcctgtcttcagagaagagtcattttcttcattcctgtacctctgtggttttaaacgaacccggggtggaagggaacctgagctaggattctgatatcgacgtgtgaaatggacttttgaatgtgcatttttggaagtagaggtttcattttgcttcttttgtgccttttctttggcaatttttaacacttcccgagctttcgcatgatccatgttcttactctggagaacttttttagtacttaactgagcttttgatgtatttgcctgagcagaaacttttactactctgcctctgctgtgagcaatatttgaaaccttaaccacagcatttcttttctggctttcattttggtttttcccatccactttatggtcagttttcagttttttgttcacagtagttacactttcatttctccgttttttatcttcatatttagaagagtcagttgcactactaccttttctaatttcctttttttcagcaacaacactgtttttacatttatcacacagaacttgcctgggtcgtagtttaatagcattcattattgaagtgggttcttccctgtacatttttcgtttgggtcgcttaattttccgaggaggtggctgaggtattgattggttatatgtgtccctgataaacaaagggggaggataaggtgctccttcatggaagagaggtggtggtttggaagtccacaggctttcagccaagctcagctcgggatgcgggacaggagaagggtcatcgggaacagcaccatttgcttcacacttgacttctgtcccttcttggaatgtattactttggagcggcatggcttctggtttatccttatattcccttttgggaaatactgtcacagggataccatggggcccaaaccttctgcaccttccttttgcagatttgaaatccagattctcacacaatcactggccatctcttctgtttcattcaacagcatacacaccagagtgtctcttactattatatacatcagtagaggccgggcgaggtggctcatgcctgtaatctcagcactttgggaggccaaggtgggtggatcacctgaggtcaggagtttgagaccaacctgaccaacatggtgaaaccccatctctactaaaaatacaaaattagccaggcgtggtggcacatgcctgtaatcccagctacttgggaggctgaggtaggagaatcacttgaaccagggaggtggagggtgcagtgagcagagattgtaccactgcagcctggacaacaagagcgaaactctgtctcaaaaataaataaataaataaataaataaaatacatcaatagaaagcacactcaccttattctgctttctaattatgaaaacaggagtgcaggccgggcacagtggctcacgcctgtaatttcagcactttggaaggccaaggcagtaggatcgcttgagcccaggagtctgagaccagcctaggcagcacagcaagaccctgtctctattaaataagtaaacaaacaaacataaacagaagtgcaaatgccctaatccaaaattatttttaaaaaagatacttgaggccgggcacggcggctcatgcctgtaatcccagccctttgggaggctgaggcgggtggataacctgaggtcaggatttcaagaccagcctggccaacatggtgaaatcccggctctagttaaaaaatacaaaaattagaccagcatggtggcgcacgcctgtagtcccagctacttgggaggctgaggcgggagaatcgcttgaacccaggaggcggaggttgcagtgagacgatatggcgccactgcactccagcctgggtgacagagtgagactccgtctcaaaaaaaaaaaaaaagatatttgagattaaataatacagaataactgctctcatctttcccctcaaacaccatacttcaatatgaaattttaaatggcttttttccccaaatgggaaagaaggattcctgggtcttgatgggagagcaagcaagtttaagagtaaaacatactaataagccattgcaaacaggtgagatacgatcagagcgtgtgctgttgcaggaaacagaatggaaagccgtgaatgggagtctctgcacttcatatcttttggacagatccatgaggaccccggagaagagcttctccccgaagcggaacgacacgacaagcgcgtcctcaatgatgtggtccagcgtgacccgcacctccgagcccgggatcagttgcgacaccgtggagtccccgcccgccggcggcacgagcgccggggctacgggctgaggcagcggcggctcctcgcgctcctcgggagccgggggctgctccggcggcgatgcaggagaaggtggaagttccggccctccctgaggcgcggctgccgccgactccgccacccgaacggacagtttctcctcagcctccagctccggccccaccgcctctgggctgcgggcgagctcccccggcggcggcggtggcggcgggagcggcggctcgtcggcctgaggagcggattgctgcccgtcagtctcgccatccggcacagacgcttcagtggccgtgaccgggagggggtcagtgccggcctcactgccggggatgggctccatctccggctcggcctcgccggcgcccccctccccgggggacgctgcagtcgctgccgcctctgcagccacggccgccattttcttcctagc

SEQ ID NO: 9989 - RNA, 2689 nt, Homo sapiens
  source 1..2689: mol_type = other RNA
cacacacacacacacacgtatatatatgtatatatacagtattaggtacaaatggcaattaacagtccctacaaaaattcaatttcagttgaggctatggctcctatgccttgggatggtttcgaacttcaaaactgaaaaatactgctaaaatctcacttccttaacacaaaatttgattatatgttcagtttaagctctcagtctaaaaatggctataaggtaagtattaaaaagccagccaactgagtgcaacttctctctccaatctggccacgctattttgtagaaattattcctaactagactagaaaatctgtggtgacttccaatggtcttgcctaccttactgcccatgttcacgtttcaaactgtgtcaacaaagcccgcacttcgggggtcagctgcttggcagccttagctgcctctgtgatagccttgcgatacaggccctttctcttcttattaaagcgtgactggaagttttctaaaaagggggagagttgtgaaagagcaaggaaagatgttgttggagacccaaaccatgaaatacgggcctcctgtcggactaaaaggccgttatctttccggctcacagttatagtaagaatacgggctggccaccaagggaagccatatatcttggcccaaacaatgtcccctacacatatggtcctgccatctggtgtgacgcatttagagacgtttttggaaaagactttcattttcaaggaattactgagctttttctcttcctttgaagaggaggaagtggaggaggtggaaggtgcatgcatactgcctggaggaaaatcaaagctttcagaagaactacactcagagttggaagatttcaaatcatctgtgctatcaatgctacacactgaagcactggaagagtcagatttcttttgatttagggtcatataaacagagatattgtttttgctgccctttttgcccaatgtctgtggttcatcctgatcaccaggcacatgcacttcatttgtgtcctgaacctcactgctggcctcttcagggccttttgagggactctgattttctgaaggggcctcacctgctgagcgggtagaggtgcagcgagactggggcttgggtgccatcttgccactccgcattttctcaagtcctgtcttcagagaagagtcattttcttcattcctgtacctctgtggttttaaacgaacccggggtggaagggaacctgagctaggattctgatatcgacgtgtgaaatggacttttgaatgtgcatttttggaagtagaggtttcattttgcttcttttgtgccttttctttggcaatttttaacacttcccgagctttcgcatgatccatgttcttactctggagaacttttttagtacttaactgagcttttgatgtatttgcctgagcagaaacttttactactctgcctctgctgtgagcaatatttgaaaccttaaccacagcatttcttttctggctttcattttggtttttcccatccactttatggtcagttttcagttttttgttcacagtagttacactttcatttctccgttttttatcttcatatttagaagagtcagttgcactactaccttttctaatttcctttttttcagcaacaacactgtttttacatttatcacacagaacttgcctgggtcgtagtttaatagcattcattattgaagtgggttcttccctgtacatttttcgtttgggtcgcttaattttccgaggaggtggctgaggtattgattggttatatgtgtccctgataaacaaagggggaggataaggtgctccttcatggaagagaggtggtggtttggaagtccacaggctttcagccaagctcagctcgggatgcgggacaggagaagggtcatcgggaacagcaccatttgcttcacacttgacttctgtcccttcttggaatgtattactttggagcggcatggcttctggtttatccttatattcccttttgggaaatactgtcacagggataccatggggcccaaaccttttggacagatccatgaggaccccggagaagagcttctccccgaagcggaacgacacgacaagcgcgtcctcaatgatgtggtccagcgtgacccgcacctccgagcccgggatcagttgcgacaccgtggagtccccgcccgccggcggcacgagcgccggggctacgggctgaggcagcggcggctcctcgcgctcctcgggagccgggggctgctccggcggcgatgcaggagaaggtggaagttccggccctccctgaggcgcggctgccgccgactccgccacccgaacggacagtttctcctcagcctccagctccggccccaccgcctctgggctgcgggcgagctcccccggcggcggcggtggcggcgggagcggcggctcgtcggcctgaggagcggattgctgcccgtcagtctcgccatccggcacagacgcttcagtggccgtgaccgggagggggtcagtgccggcctcactgccggggatgggctccatctccggctcggcctcgccggcgcccccctccccgggggacgctgcagtcgctgccgcctctgcagccacggccgccattttcttcctagcttctccctcctccaactccggctgcagcggcggcggcgacagcgctgctt

SEQ ID NO: 9990 - RNA, 3996 nt, Homo sapiens
  source 1..3996: mol_type = other RNA
cacacacacacacacacgtatatatatgtatatatacagtattaggtacaaatggcaattaacagtccctacaaaaattcaatttcagttgaggctatggctcctatgccttgggatggtttcgaacttcaaaactgaaaaatactgctaaaatctcacttccttaacacaaaatttgattatatgttcagtttaagctctcagtctaaaaatggctataaggtaagtattaaaaagccagccaactgagtgcaacttctctctccaatctggccacgctattttgtagaaattattcctaactagactagaaaatctgtggtgacttccaatggtcttgcctaccttactgcccatgttcacgtttcaaactgtgtcaacaaagcccgcacttcgggggtcagctgcttggcagccttagctgcctctgtgatagccttgcgatacaggccctttctcttcttattaaagcgtgactggaagttttctaaaaagggggagagttgtgaaagagcaaggaaagatgttgttggagacccaaaccatgaaatacgggcctcctgtcggactaaaaggccgttatctttccggctcacagttatagtaagaatacgggctggccaccaagggaagccatatatcttggcccaaacaatgtcccctacacatatggtcctgccatctggtgtgacgcatttagagacgtttttggaaaagactttcattttcaaggaattactgagctttttctcttcctttgaagaggaggaagtggaggaggtggaaggtgcatgcatactgcctggaggaaaatcaaagctttcagaagaactacactcagagttggaagatttcaaatcatctgtgctatcaatgctacacactgaagcactggaagagtcagatttcttttgatttagggtcatataaacagagatattgtttttgctgccctttttgcccaatgtctgtggttcatcctgatcaccaggcacatgcacttcatttgtgtcctgaacctcactgctggcctcttcagggccttttgagggactctgattttctgaaggggcctcacctgctgagcgggtagaggtgcagcgagactggggcttgggtgccatcttgccactccgcattttctcaagtcctgtcttcagagaagagtcattttcttcattcctgtacctctgtggttttaaacgaacccggggtggaagggaacctgagctaggattctgatatcgacgtgtgaaatggacttttgaatgtgcatttttggaagtagaggtttcattttgcttcttttgtgccttttctttggcaatttttaacacttcccgagctttcgcatgatccatgttcttactctggagaacttttttagtacttaactgagcttttgatgtatttgcctgagcagaaacttttactactctgcctctgctgtgagcaatatttgaaaccttaaccacagcatttcttttctggctttcattttggtttttcccatccactttatggtcagttttcagttttttgttcacagtagttacactttcatttctccgttttttatcttcatatttagaagagtcagttgcactactaccttttctaatttcctttttttcagcaacaacactgtttttacatttatcacacagaacttgcctgggtcgtagtttaatagcattcattattgaagtgggttcttccctgtacatttttcgtttgggtcgcttaattttccgaggaggtggctgaggtattgattggttatatgtgtccctgataaacaaagggggaggataaggtgctccttcatggaagagaggtggtggtttggaagtccacaggctttcagccaagctcagctcgggatgcgggacaggagaagggtcatcgggaacagcaccatttgcttcacacttgacttctgtcccttcttggaatgtattactttggagcggcatggcttctggtttatccttatattcccttttgggaaatactgtcacagggataccatggggcccaaactgcttcaccagaatggctgtatatttttcccaccaaaagtagggctattgcaccatacgtttcatggtctcttctgcaccttccttttgcagatttgaaatccagattctcacacaatcactggccatctcttctgtttcattcaacagcatacacaccagagtgtctcttactattatatacatcagtagaggccgggcgaggtggctcatgcctgtaatctcagcactttgggaggccaaggtgggtggatcacctgaggtcaggagtttgagaccaacctgaccaacatggtgaaaccccatctctactaaaaatacaaaattagccaggcgtggtggcacatgcctgtaatcccagctacttgggaggctgaggtaggagaatcacttgaaccagggaggtggagggtgcagtgagcagagattgtaccactgcagcctggacaacaagagcgaaactctgtctcaaaaataaataaataaataaataaataaaatacatcaatagaaagcacactcaccttattctgctttctaattatgaaaacaggagtgcaggccgggcacagtggctcacgcctgtaatttcagcactttggaaggccaaggcagtaggatcgcttgagcccaggagtctgagaccagcctaggcagcacagcaagaccctgtctctattaaataagtaaacaaacaaacataaacagaagtgcaaatgccctaatccaaaattatttttaaaaaagatacttgaggccgggcacggcggctcatgcctgtaatcccagccctttgggaggctgaggcgggtggataacctgaggtcaggatttcaagaccagcctggccaacatggtgaaatcccggctctagttaaaaaatacaaaaattagaccagcatggtggcgcacgcctgtagtcccagctacttgggaggctgaggcgggagaatcgcttgaacccaggaggcggaggttgcagtgagacgatatggcgccactgcactccagcctgggtgacagagtgagactccgtctcaaaaaaaaaaaaaaagatatttgagattaaataatacagaataactgctctcatctttcccctcaaacaccatacttcaatatgaaattttaaatggcttttttccccaaatgggaaagaaggattcctgggtcttgatgggagagcaagcaagtttaagagtaaaacatactaataagccattgcaaacaggtgagatacgatcagagcgtgtgctgttgcaggaaacagaatggaaagccgtgaatgggagtctctgcacttcatatcttttggacagatccatgaggaccccggagaagagcttctccccgaagcggaacgacacgacaagcgcgtcctcaatgatgtggtccagcgtgacccgcacctccgagcccgggatcagttgcgacaccgtggagtccccgcccgccggcggcacgagcgccggggctacgggctgaggcagcggcggctcctcgcgctcctcgggagccgggggctgctccggcggcgatgcaggagaaggtggaagttccggccctccctgaggcgcggctgccgccgactccgccacccgaacggacagtttctcctcagcctccagctccggccccaccgcctctgggctgcgggcgagctcccccggcggcggcggtggcggcgggagcggcggctcgtcggcctgaggagcggattgctgcccgtcagtctcgccatccggcacagacgcttcagtggccgtgaccgggagggggtcagtgccggcctcactgccggggatgggctccatctccggctcggcctcgccggcgcccccctccccgggggacgctgcagtcgctgccgcctctgcagccacggccgccattttcttcctagcttctccctcctccaactccggctgcagcggcggcggcgacagcgctgctt

SEQ ID NO: 9991 - RNA, 2780 nt, Homo sapiens
  source 1..2780: mol_type = other RNA
cacacacacacacacacgtatatatatgtatatatacagtattaggtacaaatggcaattaacagtccctacaaaaattcaatttcagttgaggctatggctcctatgccttgggatggtttcgaacttcaaaactgaaaaatactgctaaaatctcacttccttaacacaaaatttgattatatgttcagtttaagctctcagtctaaaaatggctataaggtaagtattaaaaagccagccaactgagtgcaacttctctctccaatctggccacgctattttgtagaaattattcctaactagactagaaaatctgtggtgacttccaatggtcttgcctaccttactgcccatgttcacgtttcaaactgtgtcaacaaagcccgcacttcgggggtcagctgcttggcagccttagctgcctctgtgatagccttgcgatacaggccctttctcttcttattaaagcgtgactggaagttttctaaaaagggggagagttgtgaaagagcaaggaaagatgttgttggagacccaaaccatgaaatacgggcctcctgtcggactaaaaggccgttatctttccggctcacagttatagtaagaatacgggctggccaccaagggaagccatatatcttggcccaaacaatgtcccctacacatatggtcctgccatctggtgtgacgcatttagagacgtttttggaaaagactttcattttcaaggaattactgagctttttctcttcctttgaagaggaggaagtggaggaggtggaaggtgcatgcatactgcctggaggaaaatcaaagctttcagaagaactacactcagagttggaagatttcaaatcatctgtgctatcaatgctacacactgaagcactggaagagtcagatttcttttgatttagggtcatataaacagagatattgtttttgctgccctttttgcccaatgtctgtggttcatcctgatcaccaggcacatgcacttcatttgtgtcctgaacctcactgctggcctcttcagggccttttgagggactctgattttctgaaggggcctcacctgctgagcgggtagaggtgcagcgagactggggcttgggtgccatcttgccactccgcattttctcaagtcctgtcttcagagaagagtcattttcttcattcctgtacctctgtggttttaaacgaacccggggtggaagggaacctgagctaggattctgatatcgacgtgtgaaatggacttttgaatgtgcatttttggaagtagaggtttcattttgcttcttttgtgccttttctttggcaatttttaacacttcccgagctttcgcatgatccatgttcttactctggagaacttttttagtacttaactgagcttttgatgtatttgcctgagcagaaacttttactactctgcctctgctgtgagcaatatttgaaaccttaaccacagcatttcttttctggctttcattttggtttttcccatccactttatggtcagttttcagttttttgttcacagtagttacactttcatttctccgttttttatcttcatatttagaagagtcagttgcactactaccttttctaatttcctttttttcagcaacaacactgtttttacatttatcacacagaacttgcctgggtcgtagtttaatagcattcattattgaagtgggttcttccctgtacatttttcgtttgggtcgcttaattttccgaggaggtggctgaggtattgattggttatatgtgtccctgataaacaaagggggaggataaggtgctccttcatggaagagaggtggtggtttggaagtccacaggctttcagccaagctcagctcgggatgcgggacaggagaagggtcatcgggaacagcaccatttgcttcacacttgacttctgtcccttcttggaatgtattactttggagcggcatggcttctggtttatccttatattcccttttgggaaatactgtcacagggataccatggggcccaaactgcttcaccagaatggctgtatatttttcccaccaaaagtagggctattgcaccatacgtttcatggtctcttttggacagatccatgaggaccccggagaagagcttctccccgaagcggaacgacacgacaagcgcgtcctcaatgatgtggtccagcgtgacccgcacctccgagcccgggatcagttgcgacaccgtggagtccccgcccgccggcggcacgagcgccggggctacgggctgaggcagcggcggctcctcgcgctcctcgggagccgggggctgctccggcggcgatgcaggagaaggtggaagttccggccctccctgaggcgcggctgccgccgactccgccacccgaacggacagtttctcctcagcctccagctccggccccaccgcctctgggctgcgggcgagctcccccggcggcggcggtggcggcgggagcggcggctcgtcggcctgaggagcggattgctgcccgtcagtctcgccatccggcacagacgcttcagtggccgtgaccgggagggggtcagtgccggcctcactgccggggatgggctccatctccggctcggcctcgccggcgcccccctccccgggggacgctgcagtcgctgccgcctctgcagccacggccgccattttcttcctagcttctccctcctccaactccggctgcagcggcggcggcgacagcgctgcttggttccctgggccttcccctc

SEQ ID NO: 9992 - RNA, 29 nt, Homo sapiens
  source 1..29: mol_type = other RNA
cacacacacacacacacgtatatcacaga

SEQ ID NO: 9993 - RNA, 3324 nt, Homo sapiens
  source 1..3324: mol_type = other RNA
cacacacacacacacacgtatcccaggatgctatcctcgtggagctaacatttgatattctaagtattaaagtttgaggcaccaacaggctgtcttaaaaggctcattcagcctgtctgccttggagctattttatttataattcttcttgtcacgtcaaagaactctgtgtttcttgcagactgtgttcgggtggttgagtgtttggtttttggctacagccggttactttttccgaatctgtaggtccaggtgtgcgttgacaaggtttttcccaactcgagaagtttctcagggagccttggagtccttctataaatttctggcattctacgtgtgagagacttccagttttggagaagtcgggagagtgagggaaggagcgtgcggttctgagtccgctgcctcctctcagacagaaagtcaacgggcagcatcttgcagtatatttagaatgcagacttgaaaaactgacggataagatattattagcaaaggtacaaacctttgatgatattcaaaaacccctgcctctgtgcatcattgaaaaccaagcgaaaaaggagtgaaaatagtgaaaatacctatccacgtctctgattactttgaaatcgattttaaaaatatgtttatcatgtaaatattatgtagactttcattttcaaggtcagtgtcccttcttgtctggttgcttacagtaccacttttttggggagttaaaaaaatgaacttcatgttcttttgaaattaggaattataccaaaagttgcctataaaatagcaagaaacaaaaaagcatcggttttcttctttagcattttttggacagcaactaaatattgtcttgtagtgataagttcagttcaaacacttcttgtatttctgtagaaagggtgcctatgaaaaatctgaccttaaccttgaagttaaccaggtctaaaagctaggatactgggacatagtcaggaaaatgaaactggttttatatataaattagtcacctgtgttgtgtgaagtcacatttgattttttaaaaataaaatgggagtctctcaataaataagaccagtgtggtcaaatgccaaacaacttgtaattgacaatcccccaaaaccaaatcccaatttcagtatgagttccatttgtgggcagcttaagtttgttgtagtaattttaaagaagtaatctgtgaaatcttgattttagtaaaaagttcctgcagtcccttgcaacttaacaacaaaccatttgagttcaaaatcagttttttctcctttcttttttttatttattctagaggaatttacctagcccgctgaagacctgtacaataaaatattataagtagcacataaactttttagaaaaatgttaatttccccatttctgattattccatttaagaaattgtagaagtgattgactaaaattaattcagcacccacttctggaatggtaatttttgttttttaaaaatttagtttggtgccctttctcattcctcatttaaagtcagaaatctagctttggcatttgatagatgcatatataaccagagatattggcccgtcatccttaatacatattttcagatttgtgttgttactactttggaatggaaaacattaatcgtaattcctcattcctaaggggaaatttttcatactagcatgttgtttattaatattatgtacaatatattcatatatgattgaacacacgcctgtcgtagacttctagttgttttatgcgctccttttgattgaaaagtaataattaaccccttaagaatgctttcggggttgttagacttctttttgagatacatacgcaggcaccgcaacatgaaacatgaatgtgtagacttccaaagcatgttaaaggtgacaaagcgctgcttacacaggtttagaaccagacatgtgattgcacgcgtgtggagctggcaccatgaaagcacgatgtgcatcactcatagaggcaggcacacttaagtatgttctttacattgaaacagaaaggaaagaagataggaaaaatggtgccagcacgctgggctttttttgtttgctgttttgggtggggtgtgctagtgcagtgtccggtgtacgcttttgtcctcaaacaggcttgttccccggtcagagtttcattattgttgctggtaaacaaatgccaagtttgacaaaaaacagtgaaataaagcaaaagattttgaaaaatgcttcatcatgtcagaaggaaagaacccttttcacgggtgcctgcccacatttccttgcccagcctgagaccctattgactttgaattatcttttgctgttttatttctatgaaaattataaacgcgtatgttcgtccaaggtggattgatgcttagaggttgcgtataaataactgagagtgaaaataaacccatcatgcggtaggagcgtatgttgtcatgaaacaggcctatgaaaatggactctcaaacctgcaaactactttgaaacaaaggcaaaagaaaaaaaatcataagcctggtttgcctttatccagagtccccaaagctgctgagcagctcctcaaaaggcacattgtctaggatgatcgaagtggcatcttatccaggagccactgaaaacttgcaatctcaagtttattgggctggctttaaaaacatcattattcttggatgtgcaactgaatgttcagaacccaagtgaaaatgtaatttttcactcactcgccgtccttgctttaattagattaaatgcatctgtttcctaagtcctcataatgccttggatactgagaaatttaaaatgtcgacccgttgagaaaaaagaaacgaaaccgaagcacccccctcagccttctgaggctggactgtgggccaggggctggcggagaaagcaaggcagcaggaaattgccggctccattcccattaggcggatatctcccggcactgtgcgctgacccctgcctccgccggccggctcccgtgtgccgagtccggactcccacccctctgggcaccccttgctccgcggggccggcggtgtcctggaagccgccgcggggttgcccgtgcgcgcgctccgccctgggggaagcccgctgccaccgtcggccccgagcgctgtcccggggccgcgtcgagagctccgcagcgcacactgttccccgcggggacgagcctggagagcctgaccgctgtccgcggcgcgctcggggctgcgggcaccaggttgcggggactgcagggaccgtcggtcagccaggggtcccagagccgggcccgagcgtgcgcgcgcgtcccgctgcccgcaatcatggc

SEQ ID NO: 9994 - RNA, 4214 nt, Homo sapiens
  source 1..4214: mol_type = other RNA
cacacacacacacacacgtatctgtacacatactctgaactaaaaccagtatttacttctagatggtaggatgatgagtgcttttttttcttattatttacattttctgtttttttcgtacaaaaagtttggataatttataaaatgttctaatataaattttaaattttcactcaagatcacacacataacattaagtgcttctctttggatagtcaggttttgggaaattctgggttttttttttaattttttgaaaactttcaaattttctgtaatgattataatccctttaaaggaaaacatataccttcatttttctaatacataaaactgactctttcagggaaaagaaaatttaaaagggaagggactggttcttagaggtaataactgaacttctggtaaaggataagatcctttcagagagaataagtattggtaggctggctggtagaagagaaaggggtgggagaagagaagaatgaatcagaggctaaataaatgaactgggaaggaagaggaagattgcttatgaagagcatacaaaagacagatgacaggagtggttgcacactgtcacctgcattctagaggtaaactaggtttgctatggttagcttcaaagtgaggttcttgaattgtattcctcctaaacaggctttacccgctcagccagcaaatgaaagccacaagtaaaaatacctgaagtgacagatgtggtctttaaagggatagtcatggtttctacttcaaagaataaaaggataggattagtgtcagtcattgtatcttgagagaggtagtacagatagaagtgaaaaaagaatataaaagaaagtacagtcaagagtgaattcaataaagcctacctcttctgctgattacagctaaaaactctggacaaaatacaaaaaacaactacctaaggactctgaaaggtaaagaaatgcagtcagattatgaagagaagtcaaaaactgaaacagcaatttgcacaggattaagtttctcattttatttcctctttcttttcacaggctttggctgaaagcaatcacacaaatgagctgcgatgggggtgctgcagacagctaatactttcagataaatcccttctgtctagaaagaaggctgggatcctttaagctgaagaacatagaaaggaatccttgcattctcattccctcccccattttcacagcttgcctagcagagccagggtgaaaagtagcatggtcggctaaaatcccaatagaaattctgtttttctagttaaacaaacagaaaagggctcctgtggtccagagagtactggagtaagtcagtaggtaaattttctctctcttttttccatctccacatagcacccaaaatggtcctggtcacaggacctggtagcaacacaggcagccaaaactccaaaagaaccccggtctattgagccagaggatgaggaatagaaaacatataggtaggtgactatggggagtcccggagataagagattagagaaatggatctcctaactctgtgtatgacctagcacaggcccaggcttaaccctgagctgtgcatgcatggaacatactcaaagctgccaagtagaggttccgaaaactgagataacattggaagtatcactcataaagtacagatagtctgaacaaaaccagtgtgattacctactcaaataagcaaacaatcttccaaatctcttgaggattttaatgaaaaacatccaaattaaatactcagaatgtccaggatacaatctaaaatcactcagcgtacaaagaaccaataaaagtttactaatttgcatgaaaagtacagtcaataaatgctaccactgagaagaccaagatggtagaataatcaggcacagattttaaggcaactatcgtaactatgctccacaaagtaaagataaacactcttgaacaaagggaaaaaaacagaaattattggcagaataatagaaactataaaaaaaaagaaccatcttacaaaattaagcatatttttaacatacaatccagcaatcacatcccttggcatttattcaaatgagttaaaaacatatgtccacacaaaaacctgcacatggatgtacatagtgactttattcataactgccaaaaccttgaagcagccaagactgtccttcagtaagtgaatgaataaataaactgtgtgtaatggttaatactgagtgtcaacttgattgaattgaaggatgcaaagtattgttcctgggtgtgtctgtgagggtgttgccaaagaagattaacattcgagtcagtggactgggagaggcagaccccccctcaatctgggtgggcaccatctaatcagctgccagtacagctataaaggcatgcaggagaagatggaaaagtagacttgctcggtcttctggccttcatctttctcccctgctggatgcttcatgccctcaaacaataaattccaagttcttcagcttttggactcttggacttacaccagtgttttgccaagggctctcagaccttcagctgcagacaaggctgcactgttggcttccctacttttgaggttttgggacttggactggcttccttgctcctcagcttgtagatagcttattgagtgactttgccttgtgataatgtgagtcaatactccctaataaactccccttcatatatacatctatcctattagttctgtccctccacggagccctgactaatacactgtggtatatccatacaatggaacattattcagttctaaaaggaatgagctatcaaggcatgaaaatacaaggaagaaacttaaatacatgttattaagttaaagaagccaatctgaaaggattatatattgtatgattcctactatgcgatattctggaaaaggcaaaagtatagaaacagtaaaaaagtcagtgattgccagagtttagcagggaaggagagatgaatatgcagaatatagacaatttttacagcagtgaaactattctgtatgatactataatggtggctatatgtcattatagatttgttcaaacccacagaatctgcaacaccaagaataaaccccttatgtaaattatggactttgggtgatagtgaggtttcagtataggttcatcacccgtaacaaaggtaccactctggtaccagatgttgacagtgtgggaggttgtgcatgtgtaggggtagagggcatatgggaactctctgtacttttcactcaatttgtctgtgaacccacaactgctctaaaaatagtctttttaaagatttttttaaagaatgaaatggaaattttagaagtgaaaaaaatacactgtgtgaagttaagaaatcaattgatgggttcgacagcaaaatacagaaaaaagaaaaaaagagtcagcaaacatagtgagacatcaatagaaagggaaaacagaggaattaaagacagaggagacaactagaaaatcaataataaaataaattcaaacatatcaataattacattaaatataaattatctaagcacaccaattaaaacatcgagtttgtcaaatttgattaaaaataaataagacctaactatctacaagaaacctactttaaaaataaagacatagatgggaatagaagtaataagatgaaagaagagataccatacaaacactaatcgaaagaaaaaatgtagtggctatattaatatcaaagtagatttcaaagcaagaaatactactaaagataaacagagatattgcataatgggataaggttcaattaatcaagaaaacataacaatcttaaatgtacacacctattaagagaagttccaaaaacttaaaacagaaacagaaatgagaactagataaatccacaaccatagttggagactttgactttcctctcacagtaattgatagaagtagacagaaaatcagtaccaacagatgagacccaaacaacgttatgtccagttgacataatttacctttataaaacactctacccaacaaaggtagaaaactttttttttcaaacacacatggaatattcaccatgctaaaccatattctggaccataaaacaaactttcacaaatttggaataactgaagtcatacaaagaatctttttcatgcgcgtccatgtgaagagaccaccaaataggctttgtgtgagcaataaagcttttaaccacctgggtgca

SEQ ID NO: 9995 - RNA, 2199 nt, Homo sapiens
  source 1..2199: mol_type = other RNA
cacacacacacacacacgtatgaataatctttatcccttccattgtctagcataggagacactcaaaaatacttgctgaatgatggtcaggtgcactggatcatgcctgcaatcccagcacgttgggaggctgaggaggcaggattgcttgagcccaggagttccggaccagcctgggcaaaatagtgagacctcgtctctacaaaacacacacatacacaaaaactagccaggcatggtggcacatccctgtagtcccagctacttgagaggctgaggtaggaggatcccctgagcccaggaaggggaggttgcagtgagcaagaatgcgccactgcactacaatgcgggtgacagagtgagactctatctcaaaaaaaaaaaaaaaaaaaaaaatggccaggtgtgatagctcacacctgtaatcccagcactttgggagactgaggtggaaggattgctcgaggccaggagttcaagaccaccctggccaacacagtgagagcccatctctacaataaataaataaataactagacctggcacagtggctcacgcctgtaatcccagcactttgggaggccgaggcgggaggatcacaaggtcaggagttcgagaccagcctgaccaacatagtaaaaccccgtctctactaaaaatataaaaattagccaggcatggtggtgcgcacctgtagtcccagctactcaggaggctgaggcagaagaatcgcttgaacctgggaggcagaggttgcagtgagccaagatcacgccactgcactccagcttgggcaacagagcgagacttcatctcaataaataaataaataaataaataggaaaaatacacatttgctgaatgaaatttactatggagatctactaactgaaaaatccttataatgagttattttataatgcaaatacttcccaatttggtctgagtttctgcacacctgattttctttaaactatgtacaacttgacttatatacagtatatgttatgtgctacatatatgactcatattgcttcacgacttaagcaacctataaatgtataaggtagcatttagcttctactttgtttacttacaactaaagttgtgataaaagatatataacaaaactttacaattagaatcaagaggaagaaacaacccgactatagcaacagtgctgtgcaaacacagagtgcaactgattcagtgaatgagtcattcattagattttttccattgttttcctataatttaataacattatttatactgagccaataagaaaagcaagtgattttgtgcagcagtaatctaaagtagatgagatttataaggcacgaactcagttgctaagagacaactccatggctttatttttcttcaatatttccctcctctatggagaagttctcttggcttggaagagcagaaagcatgaaaagaggcacagtggtcctttgttaacctcaataagtgatatgtgtgtatagtgctttctggtttataaaagcctttcacatatatttcttcctttgacggaagaaacagaattaaacaacaaataaaaatgaagagtacctagtctataatgagtttgatgcttacagtcaaggctattagcaaatattcaggaaaagtaaagcctaaagaagaaaagagggaatgaatagtttgtctagagataataaaaggaaggtgaatttttaaaaagacaaaaataaggctagaaaagactgagtggagaaagcctacagaatttcagaaagctaaagaaattggaaattagattgaatatagatagaaatgggaggacaatgcagccaatgaaagactgtggggactaataaagggagagccctgtggtttggaaagtgtcccttaatcagcctgcagtgctgcaaaacagaaacccagagagggtgcttgagaatatacaagaaccctgcggtggtgactgaacaaaacgcagccagggatttcatcagaagcataatccattcatggcacagtctggcagtgctggggagctggtaagatacacacaggcaccagtgtccagtcttgatttgatatgctggtatcttgggttctgtggtatccttttcatcagatactcagggttcccaatgtgcctccggagggacatattttctccaaccgaccacgttcggggttctagcctcacgggttgcctct

SEQ ID NO: 9996 - RNA, 3317 nt, Homo sapiens
  source 1..3317: mol_type = other RNA
cacacacacacacacacgtatgagtgtgtatgtgtaacaccagaaaaggagcaaaatagtatttaatgaccaatctcatgaatgttatctagacatcaaatgttaaaattgatggcttcttcactttaggacttattttattttttgctttcttctacattttaaaattcactatgtactttttgcagtagttatttgtctagtctctaaggctggcttatgtgaaaaagtgccaaagagtagatgctgtaacattaaatctttcctattaatgaatatctaaaaattagtagagtttgtttttttctaattttactactatcaggaggtgttgtggaggcttcccataaagtattcaatgaaatatacgtaaatttagcagtgtgcctctcattaaccgtaacagatgctgtgtagctacctctccttacataaggcctaatttcacttccaatattaacttatgtattaatttatatgttacttattttatcatggggcaaaactttatatacttgagataaagacaaaaatgtactgttcttcctattaccttctgtttaatgaacttattgctttaaggttgcttaataatccttcaggtactgttgtttatgcatatagtagctatggaaacatacaaattagcccagtgctcttctacaaagatggattcagttttcctatcaccttgcacataaataaatgccaatacataatcttttgtgtgttttctttgcccgtgctcagaatattacatgccattaataaaagaataacaaattgcatattcagcaaatgttatagctcagaacatgaaagaaggggttaatcatcacactaagaaaaatcagctggttaattcattgcaccattcaagggagtgactgaagttattctcatagcttcgtgctataatgaaactagactcatcagtgcattagcaaacaaagtttgtatcaaaactgtccaatttcctttttcttaggctttttcacatctacttccttttatcataacaaatataaaaactctatttggccctttgttctctaagtggaactttacttattttttatacctagcaaaactatctagcatcaaaatcaatactactatggatgagaaacaaagttgttgctttcataggtgcttccttctagcttggcttgtatttgtgcaattgcactttatatgaatttttactctcctgaacattgtttatatttttaatatatttttgtatgctgcataccatctctccagaactaccctattacagtgttctgtttgcaaaagcagtattttatttagatggggtcactgtaaattatcttcagtcccagacccttctggactggaatcaacatcaaggaaggcctctttattggtgaaagttgagctgagggtcatgctctgtcgtggcttcacaagtgcaagttcatctaatttaatattttcatttttgacaagaattgtcttatccatgttttcttcactgtgtcttgcaacaacagcatcaaatacatctaatttaggtggcaaggttccactttcaaatagatacttggctagataggagatgcaaatgttggttaagaatgatgtaaccatggcaagtgttttaaatggaaatttctgattatatataccattatcatcagggtaatagccagggtagaagatcaagggctgaagatacagatatggctcccctccagttattctcaggaagaggccagaaacataacctgccacggccccataggtgttggttcccttaacaaagagtacacaaagcagctgggggaagataacgatgtaaacaaggtcagaactgaggtaccagagcccatacacagttttcgtcagcaaggccatggctgttgcagatgctccaaacacaaacactgtgattcgcataacccaaacgatttctttgtccgaagcattttgtctgaaggaaagctggtagatgttccgtgcaaacatggaacttgctgacaagatggaagaatctgctgatgacataacagcagcagaaactgcaccaagaccaaagaaagaaatatacacagggcagagatactgcagaacaattggtaaaatcatgtctgcctcttctgtagtcttgggatctggaagcccatatgcagtctggttccagtctgttgatgctccaatggccccaatgagtatggctgggatggccatcaccaggcacccgaaagctgccaggaaggacagcacttgagcataggtggctgaggaagaagagagaaccctctgaaagtatgcttgccatgggattccacccagcatcaacaacagaaaactatcaagccaagagtagacttcagatgagtcaacagttcccagccacggcttttggtatttggcatgcacagcagtgaacccgatgtctgcgacagccctacaaaaatgcaaaagagctgaacgacatcagtgtaggccacagaatagagccctcccaccagtgtgtacagagtggcaatgagtgcagagatgatgacagaaatgtgcatatccacatcgatgatcacgctgatggtggctcccaaagcagagaaaattgctgcagcccagaacatttctcccatcagtgcaggaataaacaggagtccgcccatgcgttttccatagatttgctgaaacgggtctaacatggtcacatacccctttgaacgcataggttttgcaaagaacaggccacctaaaatcagactaagagaatatccaattggtgcctgagcccaagctaggccataacctggtacataaactgcttcagctgtgccattgatataccctcctccgacccaggtagctgtcatggtaaatccaccaaccaataaaccaatatctcggccaccaactatgatggcttcgctgcgctcttctgcgctgccactgtttttggttctccaggcagcccatattccaaccagcaaaattagaaggtagaacacgatgatagctatcagtccttccacatggaaagccatttttatctaatgatccagattcttctgcagctggctacttcattaagtcttctggagtggtggctgcacgcgaaagcgctccgcccggggccgccgccccctggaaccgcgaggggtgtgggtgcgagggtgcagaaagggagggtgcggggtgggtcggggtgcagtgcggagcggggccgggcggtcagggcggctcctcactcggcgtctccaagaacctgggagcgcgcagagttgacaggtgttggcgccggcggagggcgcgcggcgcagggcgaggtgggaatc

SEQ ID NO: 9997 - RNA, 2915 nt, Homo sapiens
  source 1..2915: mol_type = other RNA
cacacacacacacacacgtatgagtgtgtatgtgtaacaccagaaaaggagcaaaatagtatttaatgaccaatctcatgaatgttatctagacatcaaatgttaaaattgatggcttcttcactttaggacttattttattttttgctttcttctacattttaaaattcactatgtactttttgcagtagttatttgtctagtctctaaggctggcttatgtgaaaaagtgccaaagagtagatgctgtaacattaaatctttcctattaatgaatatctaaaaattagtagagtttgtttttttctaattttactactatcaggaggtgttgtggaggcttcccataaagtattcaatgaaatatacgtaaatttagcagtgtgcctctcattaaccgtaacagatgctgtgtagctacctctccttacataaggcctaatttcacttccaatattaacttatgtattaatttatatgttacttattttatcatggggcaaaactttatatacttgagataaagacaaaaatgtactgttcttcctattaccttctgtttaatgaacttattgctttaaggttgcttaataatccttcaggtactgttgtttatgcatatagtagctatggaaacatacaaattagcccagtgctcttctacaaagatggattcagttttcctatcaccttgcacataaataaatgccaatacataatcttttgtgtgttttctttgcccgtgctcagaatattacatgccattaataaaagaataacaaattgcatattcagcaaatgttatagctcagaacatgaaagaaggggttaatcatcacactaagaaaaatcagctggttaattcattgcaccattcaagggagtgactgaagttattctcatagcttcgtgctataatgaaactagactcatcagtgcattagcaaacaaagtttgtatcaaaactgtccaatttcctttttcttaggctttttcacatctacttccttttatcataacaaatataaaaactctatttggccctttgttctctaagtggaactttacttattttttatacctagcaaaactatctagcatcaaaatcaatactactatggatgagaaacaaagttgttgctttcataggtgcttccttctagcttggcttgtatttgtgcaattgcactttatatgaatttttactctcctgaacattgtttatatttttaatatatttttgtatgctgcataccatctctccagaactaccctattacagtgttctgtttgcaaaagcagtattttatttagatggggtcactgtaaattatcttcagtcccagacccttctggactggaatcaacatcaaggaaggcctctttattggtgaaagttgagctgagggtcatgctctgtcgtggcttcacaagtgcaagttcatctaatttaatattttcatttttgacaagaattgtcttatccatgttttcttcactgtgtcttgcaacaacagcatcaaatacatctaatttaggtggcaaggttccactttcaaatagatacttggctagataggagatgcaaatgttggttaagaatgatgtaaccatggcaagtgttttaaatggaaatttctgattatatataccattatcatcagggtaatagccagggtagaagatcaagggctgaagatacagatatggctcccctccagttattctcaggaagaggccagaaacataacctgccacggccccataggtgttggttcccttaacaaagagtacacaaagcagctgggggaagataacgatgtaaacaaggtcagaactgaggtaccagagcccatacacagttttcgtcagcaaggccatggctgttgcagatgctccaaacacaaacactgtgattcgcataacccaaacgatttctttgtccgaagcattttgtctgaaggaaagctggtagatgttccgtgcaaacatggaacttgctgacaagatggaagaatctgctgatgacataacagcagcagaaactgcaccaagaccaaagaaagaaatatacacagggcagagatactgcagaacaattggtaaaatcatgtctgcctcttctgtagtcttgggatctggaagcccatatgcagtctggttccagtctgttgatgctccaatggccccaatgagtatggctgggatggccatcaccaggcacccgaaagctgccaggaaggacagcacttgagcataggtggctgaggaagaagagagaaccctctgaaagtatgcttgccatgggattccacccagcatcaacaacagaaaactatcaagccaagagtagacttcagatgagtcaacagttcccagccacggcttttggtatttggcatgcacagcagtgaacccgatgtctgcgactgcaggatgtgacaatgcaaaggggacgctgatccacagccctacaaaaatgcaaaagagctgaacgacatcagtgtaggccacagaatagagccctcccaccagtgtgtacagagtggcaatgagtgcagagatgatgacagaaatgtgcatatccacatcgatgatcacgctgatggtggctcccaaagcagagaaaattgctgcagcccagaacatttctcccatcagtgcaggaataaacaggagtccgcccatgcgttttccatagatttgctgaaacgggtctaacatggtcacatacccctttgaacgcataggttttgcaaagaacaggccaccagtttctggtaatgactccttaaagatctctggggacatttttttacaatggttattcagagtgtttgacttgttattccacttgttatttatactcttgttctgtatactttactgagtgagtcactgagatttgcactttc

SEQ ID NO: 9998 - RNA, 6644 nt, Homo sapiens
  source 1..6644: mol_type = other RNA
cacacacacacacacacgtatgagtgtgtatgtgtaacaccagaaaaggagcaaaatagtatttaatgaccaatctcatgaatgttatctagacatcaaatgttaaaattgatggcttcttcactttaggacttattttattttttgctttcttctacattttaaaattcactatgtactttttgcagtagttatttgtctagtctctaaggctggcttatgtgaaaaagtgccaaagagtagatgctgtaacattaaatctttcctattaatgaatatctaaaaattagtagagtttgtttttttctaattttactactatcaggaggtgttgtggaggcttcccataaagtattcaatgaaatatacgtaaatttagcagtgtgcctctcattaaccgtaacagatgctgtgtagctacctctccttacataaggcctaatttcacttccaatattaacttatgtattaatttatatgttacttattttatcatggggcaaaactttatatacttgagataaagacaaaaatgtactgttcttcctattaccttctgtttaatgaacttattgctttaaggttgcttaataatccttcaggtactgttgtttatgcatatagtagctatggaaacatacaaattagcccagtgctcttctacaaagatggattcagttttcctatcaccttgcacataaataaatgccaatacataatcttttgtgtgttttctttgcccgtgctcagaatattacatgccattaataaaagaataacaaattgcatattcagcaaatgttatagctcagaacatgaaagaaggggttaatcatcacactaagaaaaatcagctggttaattcattgcaccattcaagggagtgactgaagttattctcatagcttcgtgctataatgaaactagactcatcagtgcattagcaaacaaagtttgtatcaaaactgtccaatttcctttttcttaggctttttcacatctacttccttttatcataacaaatataaaaactctatttggccctttgttctctaagtggaactttacttattttttatacctagcaaaactatctagcatcaaaatcaatactactatggatgagaaacaaagttgttgctttcataggtgcttccttctagcttggcttgtatttgtgcaattgcactttatatgaatttttactctcctgaacattgtttatatttttaatatatttttgtatgctgcataccatctctccagaactaccctattacagtgttctgtttgcaaaagcagtattttatttagatggggtcactgtaaattatcttcagtcccagacccttctggactggaatcaacatcaaggaaggcctctttattggtgaaagttgagctgagggtcatgctctgtcgtggcttcacaagtgcaagttcatctaatttaatattttcatttttgacaagaattgtcttatccatgttttcttcactgtgtcttgcaacaacagcatcaaatacatctaatttaggtggcaaggttccactttcaaatagatacttggctagataggagatgcaaatgttggttaagaatgatgtaaccatggcaagtgttttaaatggaaatttctgattatatataccattatcatcagggtaatagccagggtagaagatcaagggctgaagatacagatatggctcccctccagttattctcaggaagaggccagaaacataacctgccacggccccataggtgttggttcccttaacaaagagtacacaaagcagctgggggaagataacgatgtaaacaaggtcagaactgaggtaccagagcccatacacagttttcgtcagcaaggccatggctgttgcagatgctccaaacacaaacactgtgattcgcataacccaaacgatttctttgtccgaagcattttgtctgaaggaaagctggtagatgttccgtgcaaacatggaacttgctgacaagatggaagaatctgctgatgacataacagcagcagaaactgcaccaagaccaaagaaagaaatatacacagggcagagatactgcagaacaattggtaaaatcatgtctgcctcttctgtagtcttgggatctggaagcccatatgcagtctggttccagtctgttgatgctccaatggccccaatgagtatggctgggatggccatcaccaggcacccgaaagctgccaggaaggacagcacttgagcataggtggctgaggaagaagagagaaccctctgaaagtatgcttgccatgggattccacccagcatcaacaacagaaaactatcaagccaagagtagacttcagatgagtcaacagttcccagccacggcttttggtatttggcatgcacagcagtgaacccgatgtctgcgactgcaggatgtgacaatgcaaaggggacgctgatccacagccctacaaaaatgcaaaagagctgaacgacatcagtgtaggccacagaatagagccctcccaccagtgtgtacagagtggcaatgagtgcagagatgatgacagaaatgtgcatatccacatcgatgatcacgctgatggtggctcccaaagcagagaaaattgctgcagcccagaacatttctcccatcagtgcaggaataaacaggagtccgcccatgcgttttccatagatttgctgaaacgggtctaacatggtcacatacccctttgaacgcataggttttgcaaagaacaggccacctaaaaattaagcaactaaaatcagactaagagaatatccaattggtgcctgagcccaagctaggccataacctggtacataaactgcttcagctgtgccattgatataccctcctccgacccaggtagctgaaacagaatgaaaagtgagggagtgatactgtcttacctgttatacctacatctgcctgccaaaccagtggctactagaagttactgagcacctgaaatgtgacgagcctagattgagttgttttaggaatataaaataaacaccagatttcaaatgttttttctttcattaatcacatgttgaaatgaaaacatgttgaatgaattgagttacataagttatactattaacattaatttacctatttctttttgtttttagaggtttgtagaaaatgtaacattatgtttgtggctcatattatatttctattggatagtgctgccctagatgttttctaaatgcattgagtcagcagcattttcatgatattatatgtaatatagtctgaggtcaaggggtaaattttctttatttcaaggcccttccattttacttgtattgatgtttttatactgtcctcacggagtggtgtgcatgtgtacgtacatgtgtgtacacatgcatctatgtaggtgagtgtatgtttgtagaaatgtacttttcactaatagagtcttttcttgaacactctggggatatcagagcttgcaaatcttatctccatcaccactaagttgtacttactaccttaagttattaggagtgaagagaggatcgagatgacacttctactacaaggtgtccaaagtgagtttaaatgttaccttaaggcctagactacctagcactcagaagaaggtaaaatgtgaactgcatacatacttgcaattctatattttaatatggatcttttagtaagatatttactatttgacaagaagtaatgaaaaatgtcttattcagataaataaaatttatgtagcacaatagctgaggcaaggaggtcaaagaaccaaagaaaatgagttttgacttaacaggtttgagccaagaatgatctacagattaatatttttctctgaatagacaatgtaatgctagcaccattttctctgaggaaacagtataatattgaatccttgctgaaaaactaatgttgaagaggacactaaatctttgcagtttacaccttgttgaggttacagtacagtcaaaatattctaagcaatccttatacagaatttgtgtaaagttatgatggtcacaggttggtaataaaaatttatcagatatgaggctgaattctggattgcatcatcccattaggaataaaatttaactctgatgaattttccaaaatctcacagttagaatgtaagtaaatgaaataatatctatacaaaactacctaggatgtgtttctattgtgtttatggcaaaatttatctggcttttaatctaatacaaagcaaagaagagggagtcttagggttgacataaaaagattttcctacataggaattttgagtacatttaaatgaaaagtttatatacaaaatcctggagacaaatacgtatttagcaatcactcccacctttgctgtagcttttaccctcagtgttaacaaataacaaaaataacaaatggcattatttgttttcttattctaagccctgctgaaatttttaaaatggcttttttttttcactgtgtgtgtaaccatgagctgaagaaatgaattcttacaggcagaaaacttgagactttatctttctaccaggcaactggaattgctaacacgtcaatgttttactgcataaagtaaatggtctgatggtcttacaagcacaaagctcattagtgatcattcgtcattgtgtaagtctactgtcccttgtccaaaaagaaaattggtgactgaatcattgcaactattgtgatatagaagtgagggcttggctacttactaagatttaaaagtcccctttataattgaatttagtctcttctataacagtatttgctctccttgtttgtatattttgtgtcagatccatgagtgagaacacaacctcttaaaatatattcatttttaaaagaatcaacattttttatctctattctttataaaatatatccaagtcaatcaatctgacaaggttaggtagtatggttcagattttaaatgaattatgatattgaccaaggttattttgagttctgagaaagaaaaaaaagttttacgaactgaggaagatcatggccctttataaaaaatagcatgattcaaatattttccgtaccttttaatagcttgttaggttgaaaaaaaccattctaaatggtaaaaacaaaatataaaatattatttttatgaccatattaaacagaatattaaatgagaatagtagagggctataattattttcaataaacaacatattttgatatgcagcagctttcttattctttctgcagtgtttacaaactgtgcaccttttgaaagaaataaagtgaaactagttacagggctgcatgtggcacagcatggggcggtcaccagcatgacgcagtacttgcattttggaactaagttaccggagacctgtgtttggttctggctccagccctggtccttgttaaccttgtaacccgggatctccacttaaccccagatgctcatcataatgccgttataaagaccaaatgagtccacgtacagtagatgaagagttaaacaaagataaaatgtcaatgtctgaaagataaaactgatggctcacatagaacactgtaagtttcagattgccaaagtcaaggggttcagaacatgaatggcctctccccagactggtttggtaaactatctgatatacacggtgaatcattttaaaattgcccttcgggactgaaattgggcatcacttgatatcatttcccatgggatatttttccaatgaacgctcacagttcttgctatgttgcaaatgtttaaaaactctactaagactgtataatgaaatatgtgttgttagtgcaactgtattaaatattaaacatataattctaagttgatgtttttcagaattattttcaacgaccaagaagaatataaaaaagaaacaaatcaccctttaaacagaaccactttagtgcaaagtaagaaagaatatcagctcctgctaacacaaagaaggtttgaatgagagatgactgcagatggtggcctggggattcctatgaggacacaccctagcttttcccttttataacaaggttcatgaaatctctttattagtgctgtggactcataacatgtgattgtcttcctgtgaggaattagttattaaatgaaagaattaggtttcaaaacagggaatcactcaattgggaatatcatcacccccaaatttatttatgcagattaaaaaccatcactagatggtattcattggcacttatttaaatctcaaagtcacaactttatgcatgtattaccggacacgttgagatgctgcctatcacattaattagcagatacatagcttgtaatactaggacagcttcccattcccccacctctttgtttttactctgtttccacccactcaatagcccagggagccaagatttgtttcatgactgttcagtccagtgatttattataaaatcatttttgttcaagtactactgagttgaaaccaatttatttttaggttttaaatcaatagaaaattattttaaaatatatataactagtgaacataaagaatccccaaaggacaaagaccaacatttgctttgtcactctgaagccacacgctgcacactcacagatgccaaggaagggaggact

SEQ ID NO: 9999 - RNA, 3125 nt, Homo sapiens
  source 1..3125: mol_type = other RNA
cacacacacacacacacgtatgagtgtgtatgtgtaacaccagaaaaggagcaaaatagtatttaatgaccaatctcatgaatgttatctagacatcaaatgttaaaattgatggcttcttcactttaggacttattttattttttgctttcttctacattttaaaattcactatgtactttttgcagtagttatttgtctagtctctaaggctggcttatgtgaaaaagtgccaaagagtagatgctgtaacattaaatctttcctattaatgaatatctaaaaattagtagagtttgtttttttctaattttactactatcaggaggtgttgtggaggcttcccataaagtattcaatgaaatatacgtaaatttagcagtgtgcctctcattaaccgtaacagatgctgtgtagctacctctccttacataaggcctaatttcacttccaatattaacttatgtattaatttatatgttacttattttatcatggggcaaaactttatatacttgagataaagacaaaaatgtactgttcttcctattaccttctgtttaatgaacttattgctttaaggttgcttaataatccttcaggtactgttgtttatgcatatagtagctatggaaacatacaaattagcccagtgctcttctacaaagatggattcagttttcctatcaccttgcacataaataaatgccaatacataatcttttgtgtgttttctttgcccgtgctcagaatattacatgccattaataaaagaataacaaattgcatattcagcaaatgttatagctcagaacatgaaagaaggggttaatcatcacactaagaaaaatcagctggttaattcattgcaccattcaagggagtgactgaagttattctcatagcttcgtgctataatgaaactagactcatcagtgcattagcaaacaaagtttgtatcaaaactgtccaatttcctttttcttaggctttttcacatctacttccttttatcataacaaatataaaaactctatttggccctttgttctctaagtggaactttacttattttttatacctagcaaaactatctagcatcaaaatcaatactactatggatgagaaacaaagttgttgctttcataggtgcttccttctagcttggcttgtatttgtgcaattgcactttatatgaatttttactctcctgaacattgtttatatttttaatatatttttgtatgctgcataccatctctccagaactaccctattacagtgttctgtttgcaaaagcagtattttatttagatggggtcactgtaaattatcttcagtcccagacccttctggactggaatcaacatcaaggaaggcctctttattggtgaaagttgagctgagggtcatgctctgtcgtggcttcacaagtgcaagttcatctaatttaatattttcatttttgacaagaattgtcttatccatgttttcttcactgtgtcttgcaacaacagcatcaaatacatctaatttaggtggcaaggttccactttcaaatagatacttggctagataggagatgcaaatgttggttaagaatgatgtaaccatggcaagtgttttaaatggaaatttctgattatatataccattatcatcagggtaatagccagggtagaagatcaagggctgaagatacagatatggctcccctccagttattctcaggaagaggccagaaacataacctgccacggccccataggtgttggttcccttaacaaagagtacacaaagcagctgggggaagataacgatgtaaacaaggtcagaactgaggtaccagagcccatacacagttttcgtcagcaaggccatggctgttgcagatgctccaaacacaaacactgtgattcgcataacccaaacgatttctttgtccgaagcattttgtctgaaggaaagctggtagatgttccgtgcaaacatggaacttgctgacaagatggaagaatctgctgatgacataacagcagcagaaactgcaccaagaccaaagaaagaaatatacacagggcagagatactgcagaacaattggtaaaatcatgtctgcctcttctgtagtcttgggatctggaagcccatatgcagtctggttccagtctgttgatgctccaatggccccaatgagtatggctgggatggccatcaccaggcacccgaaagctgccaggaaggacagcacttgagcataggtggctgaggaagaagagagaaccctctgaaagtatgcttgccatgggattccacccagcatcaacaacagaaaactatcaagccaagagtagacttcagatgagtcaacagttcccagccacggcttttggtatttggcatgcacagcagtgaacccgatgtctgcgactgcaggatgtgacaatgcaaaggggacgctgatccacagccctacaaaaatgcaaaagagctgaacgacatcagtgtaggccacagaatagagccctcccaccagtgtgtacagagtggcaatgagtgcagagatgatgacagaaatgtgcatatccacatcgatgatcacgctgatggtggctcccaaagcagagaaaattgctgcagcccagaacatttctcccatcagtgcaggaataaacaggagtccgcccatgcgttttccatagatttgctgaaacgggtctaacatggtcacatacccctttgaacgcataggttttgcaaagaacaggccacctaaaatcagactaagagaatatccaattggtgcctgagcccaagctaggccataacctggtacataaactgcttcagctgtgccattgatataccctcctccgacccaggtagctggagtggtggctgcacgcgaaagcgctccgcccggggccgccgccccctggaaccgcgaggggtgtgggtgcgagggtgcagaaagggagggtgcggggtgggtcggggtgcagtgcggagcggggccgggcggtcagggcggctcctcactcggcgtctccaagaacctgggagcgcgcagagttgacaggtgttggcgccggcggagggcgcgcggcgcagggcgaggtgggaatc

SEQ ID NO: 10000 - RNA, 3351 nt, Homo sapiens
  source 1..3351: mol_type = other RNA
cacacacacacacacacgtatgagtgtgtatgtgtaacaccagaaaaggagcaaaatagtatttaatgaccaatctcatgaatgttatctagacatcaaatgttaaaattgatggcttcttcactttaggacttattttattttttgctttcttctacattttaaaattcactatgtactttttgcagtagttatttgtctagtctctaaggctggcttatgtgaaaaagtgccaaagagtagatgctgtaacattaaatctttcctattaatgaatatctaaaaattagtagagtttgtttttttctaattttactactatcaggaggtgttgtggaggcttcccataaagtattcaatgaaatatacgtaaatttagcagtgtgcctctcattaaccgtaacagatgctgtgtagctacctctccttacataaggcctaatttcacttccaatattaacttatgtattaatttatatgttacttattttatcatggggcaaaactttatatacttgagataaagacaaaaatgtactgttcttcctattaccttctgtttaatgaacttattgctttaaggttgcttaataatccttcaggtactgttgtttatgcatatagtagctatggaaacatacaaattagcccagtgctcttctacaaagatggattcagttttcctatcaccttgcacataaataaatgccaatacataatcttttgtgtgttttctttgcccgtgctcagaatattacatgccattaataaaagaataacaaattgcatattcagcaaatgttatagctcagaacatgaaagaaggggttaatcatcacactaagaaaaatcagctggttaattcattgcaccattcaagggagtgactgaagttattctcatagcttcgtgctataatgaaactagactcatcagtgcattagcaaacaaagtttgtatcaaaactgtccaatttcctttttcttaggctttttcacatctacttccttttatcataacaaatataaaaactctatttggccctttgttctctaagtggaactttacttattttttatacctagcaaaactatctagcatcaaaatcaatactactatggatgagaaacaaagttgttgctttcataggtgcttccttctagcttggcttgtatttgtgcaattgcactttatatgaatttttactctcctgaacattgtttatatttttaatatatttttgtatgctgcataccatctctccagaactaccctattacagtgttctgtttgcaaaagcagtattttatttagatggggtcactgtaaattatcttcagtcccagacccttctggactggaatcaacatcaaggaaggcctctttattggtgaaagttgagctgagggtcatgctctgtcgtggcttcacaagtgcaagttcatctaatttaatattttcatttttgacaagaattgtcttatccatgttttcttcactgtgtcttgcaacaacagcatcaaatacatctaatttaggtggcaaggttccactttcaaatagatacttggctagataggagatgcaaatgttggttaagaatgatgtaaccatggcaagtgttttaaatggaaatttctgattatatataccattatcatcagggtaatagccagggtagaagatcaagggctgaagatacagatatggctcccctccagttattctcaggaagaggccagaaacataacctgccacggccccataggtgttggttcccttaacaaagagtacacaaagcagctgggggaagataacgatgtaaacaaggtcagaactgaggtaccagagcccatacacagttttcgtcagcaaggccatggctgttgcagatgctccaaacacaaacactgtgattcgcataacccaaacgatttctttgtccgaagcattttgtctgaaggaaagctggtagatgttccgtgcaaacatggaacttgctgacaagatggaagaatctgctgatgacataacagcagcagaaactgcaccaagaccaaagaaagaaatatacacagggcagagatactgcagaacaattggtaaaatcatgtctgcctcttctgtagtcttgggatctggaagcccatatgcagtctggttccagtctgttgatgctccaatggccccaatgagtatggctgggatggccatcaccaggcacccgaaagctgccaggaaggacagcacttgagcataggtggctgaggaagaagagagaaccctctgaaagtatgcttgccatgggattccacccagcatcaacaacagaaaactatcaagccaagagtagacttcagatgagtcaacagttcccagccacggcttttggtatttggcatgcacagcagtgaacccgatgtctgcgactgcaggatgtgacaatgcaaaggggacgctgatccacagccctacaaaaatgcaaaagagctgaacgacatcagtgtaggccacagaatagagccctcccaccagtgtgtacagagtggcaatgagtgcagagatgatgacagaaatgtgcatatccacatcgatgatcacgctgatggtggctcccaaagcagagaaaattgctgcagcccagaacatttctcccatcagtgcaggaataaacaggagtccgcccatgcgttttccatagatttgctgaaacgggtctaacatggtcacatacccctttgaacgcataggttttgcaaagaacaggccacctaaaatcagactaagagaatatccaattggtgcctgagcccaagctaggccataacctggtacataaactgcttcagctgtgccattgatataccctcctccgacccaggtagctgtcatggtaaatccaccaaccaataaaccaatatctcggccaccaactatgatggcttcgctgcgctcttctgcgctgccactgtttttggttctccaggcagcccatattccaaccagcaaaattagaaggtagaacacgatgatagctatcagtccttccacatggaaagccatttttatctaatgatccagattcttctgcagctggctacttcattaagtctggagtggtggctgcacgcgaaagcgctccgcccggggccgccgccccctggaaccgcgaggggtgtgggtgcgagggtgcagaaagggagggtgcggggtgggtcggggtgcagtgcggagcggggccgggcggtcagggcggctcctcactcggcgtctccaagaacctgggagcgcgcagagttgacaggtgttggcgccggcggagggcgcgcggcgcagggcgaggtgggaatc

SEQ ID NO: 10001 - RNA, 3354 nt, Homo sapiens
  source 1..3354: mol_type = other RNA
cacacacacacacacacgtatgagtgtgtatgtgtaacaccagaaaaggagcaaaatagtatttaatgaccaatctcatgaatgttatctagacatcaaatgttaaaattgatggcttcttcactttaggacttattttattttttgctttcttctacattttaaaattcactatgtactttttgcagtagttatttgtctagtctctaaggctggcttatgtgaaaaagtgccaaagagtagatgctgtaacattaaatctttcctattaatgaatatctaaaaattagtagagtttgtttttttctaattttactactatcaggaggtgttgtggaggcttcccataaagtattcaatgaaatatacgtaaatttagcagtgtgcctctcattaaccgtaacagatgctgtgtagctacctctccttacataaggcctaatttcacttccaatattaacttatgtattaatttatatgttacttattttatcatggggcaaaactttatatacttgagataaagacaaaaatgtactgttcttcctattaccttctgtttaatgaacttattgctttaaggttgcttaataatccttcaggtactgttgtttatgcatatagtagctatggaaacatacaaattagcccagtgctcttctacaaagatggattcagttttcctatcaccttgcacataaataaatgccaatacataatcttttgtgtgttttctttgcccgtgctcagaatattacatgccattaataaaagaataacaaattgcatattcagcaaatgttatagctcagaacatgaaagaaggggttaatcatcacactaagaaaaatcagctggttaattcattgcaccattcaagggagtgactgaagttattctcatagcttcgtgctataatgaaactagactcatcagtgcattagcaaacaaagtttgtatcaaaactgtccaatttcctttttcttaggctttttcacatctacttccttttatcataacaaatataaaaactctatttggccctttgttctctaagtggaactttacttattttttatacctagcaaaactatctagcatcaaaatcaatactactatggatgagaaacaaagttgttgctttcataggtgcttccttctagcttggcttgtatttgtgcaattgcactttatatgaatttttactctcctgaacattgtttatatttttaatatatttttgtatgctgcataccatctctccagaactaccctattacagtgttctgtttgcaaaagcagtattttatttagatggggtcactgtaaattatcttcagtcccagacccttctggactggaatcaacatcaaggaaggcctctttattggtgaaagttgagctgagggtcatgctctgtcgtggcttcacaagtgcaagttcatctaatttaatattttcatttttgacaagaattgtcttatccatgttttcttcactgtgtcttgcaacaacagcatcaaatacatctaatttaggtggcaaggttccactttcaaatagatacttggctagataggagatgcaaatgttggttaagaatgatgtaaccatggcaagtgttttaaatggaaatttctgattatatataccattatcatcagggtaatagccagggtagaagatcaagggctgaagatacagatatggctcccctccagttattctcaggaagaggccagaaacataacctgccacggccccataggtgttggttcccttaacaaagagtacacaaagcagctgggggaagataacgatgtaaacaaggtcagaactgaggtaccagagcccatacacagttttcgtcagcaaggccatggctgttgcagatgctccaaacacaaacactgtgattcgcataacccaaacgatttctttgtccgaagcattttgtctgaaggaaagctggtagatgttccgtgcaaacatggaacttgctgacaagatggaagaatctgctgatgacataacagcagcagaaactgcaccaagaccaaagaaagaaatatacacagggcagagatactgcagaacaattggtaaaatcatgtctgcctcttctgtagtcttgggatctggaagcccatatgcagtctggttccagtctgttgatgctccaatggccccaatgagtatggctgggatggccatcaccaggcacccgaaagctgccaggaaggacagcacttgagcataggtggctgaggaagaagagagaaccctctgaaagtatgcttgccatgggattccacccagcatcaacaacagaaaactatcaagccaagagtagacttcagatgagtcaacagttcccagccacggcttttggtatttggcatgcacagcagtgaacccgatgtctgcgactgcaggatgtgacaatgcaaaggggacgctgatccacagccctacaaaaatgcaaaagagctgaacgacatcagtgtaggccacagaatagagccctcccaccagtgtgtacagagtggcaatgagtgcagagatgatgacagaaatgtgcatatccacatcgatgatcacgctgatggtggctcccaaagcagagaaaattgctgcagcccagaacatttctcccatcagtgcaggaataaacaggagtccgcccatgcgttttccatagatttgctgaaacgggtctaacatggtcacatacccctttgaacgcataggttttgcaaagaacaggccacctaaaatcagactaagagaatatccaattggtgcctgagcccaagctaggccataacctggtacataaactgcttcagctgtgccattgatataccctcctccgacccaggtagctgtcatggtaaatccaccaaccaataaaccaatatctcggccaccaactatgatggcttcgctgcgctcttctgcgctgccactgtttttggttctccaggcagcccatattccaaccagcaaaattagaaggtagaacacgatgatagctatcagtccttccacatggaaagccatttttatctaatgatccagattcttctgcagctggctacttcattaagtcttctggagtggtggctgcacgcgaaagcgctccgcccggggccgccgccccctggaaccgcgaggggtgtgggtgcgagggtgcagaaagggagggtgcggggtgggtcggggtgcagtgcggagcggggccgggcggtcagggcggctcctcactcggcgtctccaagaacctgggagcgcgcagagttgacaggtgttggcgccggcggagggcgcgcggcgcagggcgaggtgggaatc

SEQ ID NO: 10002 - RNA, 4135 nt, Homo sapiens
  source 1..4135: mol_type = other RNA
cacacacacacacacacgtatgagtgtgtatgtgtaacaccagaaaaggagcaaaatagtatttaatgaccaatctcatgaatgttatctagacatcaaatgttaaaattgatggcttcttcactttaggacttattttattttttgctttcttctacattttaaaattcactatgtactttttgcagtagttatttgtctagtctctaaggctggcttatgtgaaaaagtgccaaagagtagatgctgtaacattaaatctttcctattaatgaatatctaaaaattagtagagtttgtttttttctaattttactactatcaggaggtgttgtggaggcttcccataaagtattcaatgaaatatacgtaaatttagcagtgtgcctctcattaaccgtaacagatgctgtgtagctacctctccttacataaggcctaatttcacttccaatattaacttatgtattaatttatatgttacttattttatcatggggcaaaactttatatacttgagataaagacaaaaatgtactgttcttcctattaccttctgtttaatgaacttattgctttaaggttgcttaataatccttcaggtactgttgtttatgcatatagtagctatggaaacatacaaattagcccagtgctcttctacaaagatggattcagttttcctatcaccttgcacataaataaatgccaatacataatcttttgtgtgttttctttgcccgtgctcagaatattacatgccattaataaaagaataacaaattgcatattcagcaaatgttatagctcagaacatgaaagaaggggttaatcatcacactaagaaaaatcagctggttaattcattgcaccattcaagggagtgactgaagttattctcatagcttcgtgctataatgaaactagactcatcagtgcattagcaaacaaagtttgtatcaaaactgtccaatttcctttttcttaggctttttcacatctacttccttttatcataacaaatataaaaactctatttggccctttgttctctaagtggaactttacttattttttatacctagcaaaactatctagcatcaaaatcaatactactatggatgagaaacaaagttgttgctttcataggtgcttccttctagcttggcttgtatttgtgcaattgcactttatatgaatttttactctcctgaacattgtttatatttttaatatatttttgtatgctgcataccatctctccagaactaccctattacagtgttctgtttgcaaaagcagtattttatttagatggggtcactgtaaattatcttcagtcccagacccttctggactggaatcaacatcaaggaaggcctctttattggtgaaagttgagctgagggtcatgctctgtcgtggcttcacaagtgcaagttcatctaatttaatattttcatttttgacaagaattgtcttatccatgttttcttcactgtgtcttgcaacaacagcatcaaatacatctaatttaggtggcaaggttccactttcaaatagatacttggctagataggagatgcaaatgttggttaagaatgatgtaaccatggcaagtgttttaaatggaaatttctgattatatataccattatcatcagggtaatagccagggtagaagatcaagggctgaagatacagatatggctcccctccagttattctcaggaagaggccagaaacataacctgccacggccccataggtgttggttcccttaacaaagagtacacaaagcagctgggggaagataacgatgtaaacaaggtcagaactgaggtaccagagcccatacacagttttcgtcagcaaggccatggctgttgcagatgctccaaacacaaacactgtgattcgcataacccaaacgatttctttgtccgaagcattttgtctgaaggaaagctggtagatgttccgtgcaaacatggaacttgctgacaagatggaagaatctgctgatgacataacagcagcagaaactgcaccaagaccaaagaaagaaatatacacagggcagagatactgcagaacaattggtaaaatcatgtctgcctcttctgtagtcttgggatctggaagcccatatgcagtctggttccagtctgttgatgctccaatggccccaatgagtatggctgggatggccatcaccaggcacccgaaagctgccaggaaggacagcacttgagcataggtggctgaggaagaagagagaaccctctgaaagtatgcttgccatgggattccacccagcatcaacaacagaaaactatcaagccaagagtagacttcagatgagtcaacagttcccagccacggcttttggtatttggcatgcacagcagtgaacccgatgtctgcgactgcaggatgtgacaatgcaaaggggacgctgatccacagccctacaaaaatgcaaaagagctgaacgacatcagtgtaggccacagaatagagccctcccaccagtgtgtacagagtggcaatgagtgcagagatgatgacagaaatgtgcatatccacatcgatgatcacgctgatggtggctcccaaagcagagaaaattgctgcagcccagaacatttctcccatcagtgcaggaataaacaggagtccgcccatgcgttttccatagatttgctgaaacgggtctaacatggtcacatacccctttgaacgcataggttttgcaaagaacaggccacctgtcatggtaaatccaccaaccaataaaccaatatctcggccaccaactatgatggcttcgctgcgctcttctgcgctgccactgtttttggttctccaggcagcccatattccaaccagcaaaattagaaggtagaacacgatgatagctatcagtccttccacatggaaagccatttttatctaatgatccagattcttctgcagctggctacttcattaagtcttctgaagaaaatacagggatgcattataaaccagtcaagcactatgcacatgtaggcagccaggaataaaccagctggctcatgcgagatcctgtgccactcacagaaagagtacaaccctgaaaccacacgtgaaacgggcagttaacaataagtgtccactacattatcctacttctatttaacaatttaacattattttgagtttgcaagaaacagaaaaaaaaacggaaatgtagtttaacaaatggaatcataatccttgtgtgtttcatacatgctttaaatttaaaattaaccttgtcgtgtatatcttaactcagtaactgtcaaatcatttacaaagagtagcgctgtatctgcgttttggaactaagttactcttctagaattatttattctagaagtgttaagtgtttcataaatgaccattctgaaaattttaaaatattcattaatttattcattcttttatctgtcctttcaaacaacttcagagaatggcttcagtagtaatctgatataaaaatatctgaaaaaaatctttagaaaaatccatttcaaaaacacatcaaactccacattttcaacaagcttctgtagttcaagttactatagcaactaagtatgttttttgttgttgaaaggatccattctcttgatcttcttcgcccaatatccttcattcaattcatcaccccccattaatggtacatacaggaaaaggttttgttgttgttgttgctgttgttttaaacacaattgcctaaaagcacatcagaagcctcaaagatattaaaatcaagactcttagaagacagatgtcaagttcgaaagcattcaccttctgaaattcttgtccccttttatttttatttttatttattttttacctttgtgaccacagctgttccatgaacccaaactctcacatacaagtttctgggggaaactctgacatttgtgcgtgcaggtgggtgaagagacgttgggggaaagaatcagcctctctggaatttaaaggaggcaaaagaagcgcccgcgggctgtgtcttctctgcctttgtgagcaaccaagcaggcaagttcctctccgcagcagcccgatgctctcccggccccctgcggcctttcct

SEQ ID NO: 10003 - RNA, 3627 nt, Homo sapiens
  source 1..3627: mol_type = other RNA
cacacacacacacacacgtatgcacatgcgatgcacgtgtcatgcaaatacatttatgttatgttaggttaattacacaagcctccatgacctccctgtgctgtgttaattacgccagcctcctgacatactgactgcatttttataagtacattttcttatcccaacaaacccccccaaagcttgacagtatttataaagtatagcaaagctacattaaatatttagaaaaagttactttttagctcatctctcaattaagaaaatttaaaaaaacaatatttttaaaaatctctggcttgtcaggctaaaaacatttctatattaaatagctttatttttgccttccagaataatgccatcatgcattccagggagaaccccatttctagaactcaagggtcaagatttgggagaaattcccagttcctccctttacagctgtgtgaggtgcgtgttttcttcatttaaatctcctgttggagattgaaatgcccagaatggggggtaagcggcgctgagaggaggtctgacgccaggtctcatcctgacagtggcccgggctgtgtggctgagctctttgctgccctagaagactgcctggcagtgaatggctgaagcgtgaggccacagtgcatgtaaagtcagcacctgtcagtgatttgtcatcctgtctaaaagctagggacccaggtctacgagaaaagagatgtctgggtgtaatttccaggggcagcaccccgtcatttagttataaaccctcaggtttgacagcttgctagtttctgtcctgaggacgggtcagccccctgggtgggtggtgtggccccctcctgcgggcccaggaaggaaggaagtgccacgcccagggccatccctgcttcccgctgtcctggctcatcccaggcctcggacccagagtgaggagggaaggtgaagatggctgtgtcctgatcttcatggcgcaccccctccaggaactcagaggaaacagtgcactctcccccgagaagtcccagacacacagccctctccatgacttgtgtagggcttagaccagctaagacccaggacggaccctcgtaggggaaggagggggcccgcgtgaaaaagctcagggagggatcatggcctccttggacccttctggatcctctctgagtagagggtataggacaagggcagggctgttatgagagtgatcggggacccaaacagccgtacaagggtcagcactggccgatgctggggtgcggagcctctaaaagcctggtcaggctgagctggctggggaccggggacaggggaccggtcctcaggaggacccggacgtggtgagaggagagggccaggtgccatcctcagcagacacaagctcctgcactaatacacttttctctcttgcaggcagcttgcctgagagaagcgggtggaaggggctttggctttctgattcaatctgcactgggctaggctgcagggcagctttgggatggacactcatggccaagaggagtgttcttccctcctcaggagtgctcgggtccctcacacctgcctcatgtaaccactctctccgttttgatgagggagtcacaggcacactgccactcttgcttcggcttgtgaggaagtagcgagcagatcccacgaatacccaggacagcaggcggcaggaagcctgggtgacgggggagagtgagcagagctgcggctacgaggctgggggccttggacaggcaacggcatctctgagtgcaagagaaacttcctctccaatgtgccttctgacttccctgccatccagctcacagagaagcccagatggtcgagccccaggaaggcgtttagcctgcccagggacctgagcagggctgcactctgagcccatcgcagcttcaaagtcttgtatttgtccttaaggaaggttcctgctggcatggtcaggaacacattcttactcattgtcaaggaaagacagaggtttgaggtgagttaatgtcacaaatctgaaagggttgattgcggaaacagagctggatttgaacctcttccgcacagcaagacaaacccaatttagaatcacgacatgtgtttcttttacaaaccgtagggccaagctcccaaccctaccccccaaccaactatgtgtggaggcgtcctgaccctgaggccggcctgggctaggcaggtcgcaccttcatctctgacaccttgtagctataattgtatcctttccccgacttccagttgatgccatttgcaaagctgccatgagtccccctgaggtagcgaccattcaggtttgacacatggcagtttttgtaccaccaagctccctgaaacatcacagcacaatttccggtgttaagatcattgtcctggtctttggtggagaaggactggttgttgtggaacgtcagggaatctcccgcactgccctccacgaaggcccccaggaccagattgtacttctccgcctcgtcggccaccttgaatgatctgtacttagcaaactggtagttgtcctcaaagtccaccaggtctacacggagctcgctggttccctgggcggtcagggcgtggatgttgtcattccccagccagaactcccccagccgactgccgaagccctgcttgtacgtggcccagtcccggtagaagtccacagagccatccaccctccgctggaaaacggtccagccccctccgtccgtgtccatgtcacagagcacagtcaggggccggcagtcgggcaggtagatggtgtgccagccgctcaggaagtgccctcggtctagcaggtccttgcaggtacgcgggcctgtcaggcacggctggggctccccaggtgctccgttgggcccaggtggtcctgccttcccaggaggtccaggggggccacgttctcctctctttccattggtgcctgcctctcccttgggcccaggggccccaggcagccccggacagcctcggagaatggtgagcttgtcagagccctccaggcccaccatcttcacctctggacaggtgtcttcagtcaaggccatggtccacaggaaggagagggccaggagagcaggtcccatggctacggcagctcggctcagccctggggctctggtctttgccactgaaggaactccgtggttcttacagggctgcagccacccactgtaacctctctctccatttcccaaccccagtggggatggccactccctcccgaaggcttggtggcaccaactggcggtggagacagcctcagggccgctgtcttccgcaggccccacaggcttcccacttaacgagcctggcttcccctggcagggacgctctgcccagcagaaggctccctgaggcccgtgtgggaagggcctgcctgtttgtgtctttagggaaagcttggcgggaacactgcctgaggcccgcagcaggacagaagggcttgtggaatccagcccttgaggaaatctcttgcagagaatctgccgtgagtccacagaagtttaggaacgtccactgcggtctgagtggttcccaggggagggagagggaagcaggatgattaccaggaacctccctgggccagcatgcagggagttggttgcaaccctagaggac

SEQ ID NO: 10004 - RNA, 3513 nt, Homo sapiens
  source 1..3513: mol_type = other RNA
cacacacacacacacacgtatgcacatgcgatgcacgtgtcatgcaaatacatttatgttatgttaggttaattacacaagcctccatgacctccctgtgctgtgttaattacgccagcctcctgacatactgactgcatttttataagtacattttcttatcccaacaaacccccccaaagcttgacagtatttataaagtatagcaaagctacattaaatatttagaaaaagttactttttagctcatctctcaattaagaaaatttaaaaaaacaatatttttaaaaatctctggcttgtcaggctaaaaacatttctatattaaatagctttatttttgccttccagaataatgccatcatgcattccagggagaaccccatttctagaactcaagggtcaagatttgggagaaattcccagttcctccctttacagctgtgtgaggtgcgtgttttcttcatttaaatctcctgttggagattgaaatgcccagaatggggggtaagcggcgctgagaggaggtctgacgccaggtctcatcctgacagtggcccgggctgtgtggctgagctctttgctgccctagaagactgcctggcagtgaatggctgaagcgtgaggccacagtgcatgtaaagtcagcacctgtcagtgatttgtcatcctgtctaaaagctagggacccaggtctacgagaaaagagatgtctgggtgtaatttccaggggcagcaccccgtcatttagttataaaccctcaggtttgacagcttgctagtttctgtcctgaggacgggtcagccccctgggtgggtggtgtggccccctcctgcgggcccaggaaggaaggaagtgccacgcccagggccatccctgcttcccgctgtcctggctcatcccaggcctcggacccagagtgaggagggaaggtgaagatggctgtgtcctgatcttcatggcgcaccccctccaggaactcagaggaaacagtgcactctcccccgagaagtcccagacacacagccctctccatgacttgtgtagggcttagaccagctaagacccaggacggaccctcgtaggggaaggagggggcccgcgtgaaaaagctcagggagggatcatggcctccttggacccttctggatcctctctgagtagagggtataggacaagggcagggctgttatgagagtgatcggggacccaaacagccgtacaagggtcagcactggccgatgctggggtgcggagcctctaaaagcctggtcaggctgagctggctggggaccggggacaggggaccggtcctcaggaggacccggacgtggtgagaggagagggccaggtgccatcctcagcagacacaagctcctgcactaatacacttttctctcttgcaggcagcttgcctgagagaagcgggtggaaggggctttggctttctgattcaatctgcactgggctaggctgcagggcagctttgggatggacactcatggccaagaggagtgttcttccctcctcaggagtgctcgggtccctcacacctgcctcatgtaaccactctctccgttttgatgagggagtcacaggcacactgccactcttgcttcggcttgtgaggaagtagcgagcagatcccacgaatacccaggacagcaggcggcaggaagcctgggtgacgggggagagtgagcagagctgcggctacgaggctgggggccttggacaggcaacggcatctctgagtgcaagagaaacttcctctccaatgtgccttctgacttccctgccatccagctcacagagaagcccagatggtcgagccccaggaaggcgtttagcctgcccagggacctgagcagggctgcactctgagcccatcgcagcttcaaagtcttgtatttgtccttaaggaaggttcctgctggcatggtcaggaacacattcttactcattgtcaaggaaagacagaggtttgaggtgagttaatgtcacaaatctgaaagggttgattgcggaaacagagctggatttgaacctcttccgcacagcaagacaaacccaatttagaatcacgacatgtgtttcttttacaaaccgtagggccaagctcccaaccctaccccccaaccaactatgtgtggaggcgtcctgaccctgaggccggcctgggctaggcaggtcgcaccttcatctctgacaccttgtagctataattgtatcctttccccgacttccagttgatgccatttgcaaagctgccatgagtccccctgaggtagcgaccattcaggtttgacacatggcagtttttgtaccaccaagctccctgaaacatcacagcacaatttccggtgttaagatcattgtcctggtctttggtggagaaggactggttgttgtggaacgtcagggaatctcccgcactgccctccacgaaggcccccaggaccagattgtacttctccgcctcgtcggccaccttgaatgatctgtacttagcaaactggtagttgtcctcaaagtccaccaggtctacacggagctcgctggttccctgggcggtcagggcgtggatgttgtcattccccagccagaactcccccagccgactgccgaagccctgcttgtacgtggcccagtcccggtagaagtccacagagccatccaccctccgctggaaaacggtccagccccctccgtccgtgtccatgtcacagagcacagtcaggggccggcagtcgggcaggtagatggtgtgccagccgctcaggaagtgccctcggtctagcaggtccttgcaggtacgcgggcctgtcaggcacggctggggctccccaggtgctccgttgggcccaggtggtcctgccttcccaggaggtccaggggggccacgttctcctggacaggtgtcttcagtcaaggccatggtccacaggaaggagagggccaggagagcaggtcccatggctacggcagctcggctcagccctggggctctggtctttgccactgaaggaactccgtggttcttacagggctgcagccacccactgtaacctctctctccatttcccaaccccagtggggatggccactccctcccgaaggcttggtggcaccaactggcggtggagacagcctcagggccgctgtcttccgcaggccccacaggcttcccacttaacgagcctggcttcccctggcagggacgctctgcccagcagaaggctccctgaggcccgtgtgggaagggcctgcctgtttgtgtctttagggaaagcttggcgggaacactgcctgaggcccgcagcaggacagaagggcttgtggaatccagcccttgaggaaatctcttgcagagaatctgccgtgagtccacagaagtttaggaacgtccactgcggtctgagtggttcccaggggagggagagggaagcaggatgattaccaggaacctccctgggccagcatgcagggagttggttgcaaccctagaggac

SEQ ID NO: 10005 - RNA, 4425 nt, Homo sapiens
  source 1..4425: mol_type = other RNA
cacacacacacacacacgtatgtgggaagaaacttccttctgcctttgaacaggtgttatctggagctgttgcagccacctcgttatcatgagaaagcagctgacacagcaggaagagcaggaagatggaaacctagaaccttgacaactttcttgaatgtatagccctggaatgccttactttcgaagttcctgttatacaacataattcatttccctaccgcttaagtttctgttaagtgtggcttgaagctgagaggaccatgactgatgcagggttatctagtgaagtaggggacagaatgccacaaccttaaactttgatcctaaaaaagacaaaagacagctgtaagtaattgcagaaagcccctttaatgtctgtggaacagaagaaccatgttggatggggaaagcaggggcaggacacacgtgtcgcgtatctatggggtgttatcagggttatatctgtgacaggatcaactaacttactggctctcatttcacctgataacataagaccctccccgctgactacacacagtttaggttatcactccttatgactcctgctccctgccctgcaccctagattctctgggactcactgcagttttcctgactctgatggaatgtgctggagtctattacgagccctgcttttcagaaggtgctcaacaggccctgaagatgtgcatctggccgatggtgggtcaaaaccagagttctgcaggctgagatttttccttttattattattaaacttggctgtgttttccttcggtggctctggcatcctatgcagtagtgctggacatttgcaggcagttaaggcccagtacagcaggaagaatgatttctgtgactgctggtctgtgcaagccctccagctgcgggagcaacctcccttgaggagaagttgtgggggtgggcctggtggggagggcgataggctgggacagaaggaaggatggaatactggacctggtggccaggggtcaatgggatgtccttctcaccagaagcaacagaacgccgactccagcatgctcccatttcaactaaagtagtgggagacccacccaatgtgcatcaaaggcctgggtccttctgggctgcactttgaggaggagcagcatagtaagggatggggcgcccattctgctagcagagtgattcctggagatgcaatctgggagggatgtatccacgtggctgacccctcgtgtccagatgtcacatcttagtgtcatgagcctggtataaacattgaatttttaggatgcattttcactgagaggctaccactctgggagcctctctttttcctgcaaggagcgcctctcaaaggagtgattctggttctcagaggcattctgagctttgggatctagtctcaggctttccagggaaggaaaaagctatggctggatgacttttagttttctgcagtgccggatgccaactagaaaagctcatttttatctgaaaggaaagaaccagctagaattgagcatgccctcctttcccatccctgtatcatgtccttggttccacatccccccttgccatgctgttgtgaagttgttttgttttcctctctctttcccataaaaggtcatgagctctgtttctgtctttaagattcccgtacttggtggcacaaatgaggcagcctcaacattctgttgaaggagtgaagggtttggaagttccaggtggtgcaggaaactagactggctcccagcaggtagatctttcccaaacctgaaatggccatacaatcctgtatgtgagacaggctgaatgcagagaatgagcatttccaggtggtagctctcatctcatctcacaaaaaaaaccagaccaccactgggagtcctgttccccggcttttatgctcacccctcccagtcacttcagatcagttaattctccagatttacaagctagaaaactccagctctggcactcagcacacaggcctcaaccggggctgtggatttcaacccagaagcccaaacttctcagccggcttaaggccccttccaactgccagtctgtaccacgacagcagtgctgtgggcacaatgccaagcacacccatgccaggcagtcctcctgggccctgacttgatggggtgcagccatgggtcctctggacacgttttgctcaattataccttcctctccagctgcctaaccttgaccaagatggggacctgattaaaaaccccatcagtttctagctcttcccataattttgattgacaacattaaatgctaatacaaaaacatcttatctctgataaaacaaaagctgacagaaagacggatgctgaaaaccagccatatggtggacacgattcctgggcctggccctgttcacagtagcactctctggcagaaaagagatgacactgagaagcttgaggacctacatttaataaatcaaactgtactggcatcatcagaatattcacagtttgcaacaggatcagtgcgttttctcacttgcagactcggaggtatttcaggagaaggcgacgtgagcgcaccattccgatgcttcattcttgaccctctctggggctttcaatgtgtcattgtgtcagatccctctccccttcaggttttcacggtgctcctcatgcctccgccctctgggatccctttgccgtcttccggtgtggaagctttggctgctggccggctggcctcgaaggagtccaggtgagatttagggagctccccctggatggccaggcctggcggggctggccccgtctcactcctctgaccttctatgggactctctcttctgacctcttccagttctgcagctgcctgttcctttgtcagtttaattatttccctcccaaggctgtttacttcttcctcagaaggtaactggggtaatgaaggatgaaagagcttgcattggttcccgcggctctgatttgctggggagttgacagcgggcctcccagcatcctcaggcgctgtcaacgcctcagcagcggcacaactttcatcttcttcttgcttctgagcctccccatccttgggatctgctttgttctcagtgggctgctcgacaaacttcagcagtggggatctcgacctctgtccactaggaagagtggggtcgctgaacagtatggtgtccttgccccctggaagactccacaaaccagaaacttccagagttcttaattttttttccagctcagccacccgattccctaggattttgttggtttgcctctggtgctgaatgaccatgtttttctcgtggattgtttccaacagggctgttgccagagatttcaggtcagaaatggactgcggagtagctgggaggctgcatccatgatcctcagatagcagatcctgaacttgctttgcagacaggactcctgtcagagcactgctgctggatttaccctggcccttcgagtttttccgtctctccagagcattcttgtatttggcaatgtttgatttcaagaggttgacctcttcatggagttgctttaatctctcttgaaggtacctgttctccatacacagggcgtccacgtcaatgatgcggttctcgtgcccactcaggatatggttcagctcctggttgagcctctccactttgtcctggtaggaagaccgttcttctttaacatcctgaagctcgtccacagaagcctgcaggtcgtgctccagagactcaatctgttccttagctcgctctagctgctgcaccaagtcttcacgctcatgggctgcaaagtgtcgcacgccgattgcttcgtctccgagcctttgtttggcaatcgtcatcctcaagagcttgttgtcgccctggacttctccaagcctttgctgaagttctttaatttcttctcccagatgtttatttcggtcctgagaatctctcaatagttgtgcaagattagcctgtttccttttttcaggaggaagtgatggatctccatcaatcagctctcggtacttcttcttcagtgactggtggcgctcccggagctgattggccatgagtttgtactggtccctttcctgttgacaggtgtccagctccttggagaggatcagcagggcttccttcttactctccagcttcctcttacacaccaggtactcagaatcccaagtggccgctctggcgatgatgatgatgatgacgacgacgatgacgaccatgatggtgatgatgatgagttaatgacgtggcaactatccactacttatgaataagtagtgctgacagatgtgaggctctgtgcaagttccttagcctgtctgagccactgtttccttatctcgctcaccagcccctgccagtcgctctcagtccggtcgccgttcatggcctcctcctccatgcgctggccggcctcctggacccccgcc

SEQ ID NO: 10006 - RNA, 4331 nt, Homo sapiens
  source 1..4331: mol_type = other RNA
cacacacacacacacacgtatgtgggaagaaacttccttctgcctttgaacaggtgttatctggagctgttgcagccacctcgttatcatgagaaagcagctgacacagcaggaagagcaggaagatggaaacctagaaccttgacaactttcttgaatgtatagccctggaatgccttactttcgaagttcctgttatacaacataattcatttccctaccgcttaagtttctgttaagtgtggcttgaagctgagaggaccatgactgatgcagggttatctagtgaagtaggggacagaatgccacaaccttaaactttgatcctaaaaaagacaaaagacagctgtaagtaattgcagaaagcccctttaatgtctgtggaacagaagaaccatgttggatggggaaagcaggggcaggacacacgtgtcgcgtatctatggggtgttatcagggttatatctgtgacaggatcaactaacttactggctctcatttcacctgataacataagaccctccccgctgactacacacagtttaggttatcactccttatgactcctgctccctgccctgcaccctagattctctgggactcactgcagttttcctgactctgatggaatgtgctggagtctattacgagccctgcttttcagaaggtgctcaacaggccctgaagatgtgcatctggccgatggtgggtcaaaaccagagttctgcaggctgagatttttccttttattattattaaacttggctgtgttttccttcggtggctctggcatcctatgcagtagtgctggacatttgcaggcagttaaggcccagtacagcaggaagaatgatttctgtgactgctggtctgtgcaagccctccagctgcgggagcaacctcccttgaggagaagttgtgggggtgggcctggtggggagggcgataggctgggacagaaggaaggatggaatactggacctggtggccaggggtcaatgggatgtccttctcaccagaagcaacagaacgccgactccagcatgctcccatttcaactaaagtagtgggagacccacccaatgtgcatcaaaggcctgggtccttctgggctgcactttgaggaggagcagcatagtaagggatggggcgcccattctgctagcagagtgattcctggagatgcaatctgggagggatgtatccacgtggctgacccctcgtgtccagatgtcacatcttagtgtcatgagcctggtataaacattgaatttttaggatgcattttcactgagaggctaccactctgggagcctctctttttcctgcaaggagcgcctctcaaaggagtgattctggttctcagaggcattctgagctttgggatctagtctcaggctttccagggaaggaaaaagctatggctggatgacttttagttttctgcagtgccggatgccaactagaaaagctcatttttatctgaaaggaaagaaccagctagaattgagcatgccctcctttcccatccctgtatcatgtccttggttccacatccccccttgccatgctgttgtgaagttgttttgttttcctctctctttcccataaaaggtcatgagctctgtttctgtctttaagattcccgtacttggtggcacaaatgaggcagcctcaacattctgttgaaggagtgaagggtttggaagttccaggtggtgcaggaaactagactggctcccagcaggtagatctttcccaaacctgaaatggccatacaatcctgtatgtgagacaggctgaatgcagagaatgagcatttccaggtggtagctctcatctcatctcacaaaaaaaaccagaccaccactgggagtcctgttccccggcttttatgctcacccctcccagtcacttcagatcagttaattctccagatttacaagctagaaaactccagctctggcactcagcacacaggcctcaaccggggctgtggatttcaacccagaagcccaaacttctcagccggcttaaggccccttccaactgccagtctgtaccacgacagcagtgctgtgggcacaatgccaagcacacccatgccaggcagtcctcctgggccctgacttgatggggtgcagccatgggtcctctggacacgttttgctcaattataccttcctctccagctgcctaaccttgaccaagatggggacctgattaaaaaccccatcagtttctagctcttcccataattttgattgacaacattaaatgctaatacaaaaacatcttatctctgataaaacaaaagctgacagaaagacggatgctgaaaaccagccatatggtggacacgattcctgggcctggccctgttcacagtagcactctctggcagaaaagagatgacactgagaagcttgaggacctacatttaataaatcaaactgtactggcatcatcagaatattcacagtttgcaacaggatcagtgcgttttctcacttgcagactcggaggtatttcaggagaaggcgacgtgagcgcaccattccgatgcttcattcttgaccctctctggggctttcaatgtgtcattgtgtcagatccctctccccttcaggttttcacggtgctcctcatgcctccgccctctgggatccctttgccgtcttccggtgtggaagctttggctgctggccggctggcctcgaaggagtccaggtgagatttagggagctccccctggatggccaggcctggcggggctggccccgtctcactcctctgaccttctatgggactctctcttctgacctcttccagttctgcagctgcctgttcctttgtcagtttaattatttccctcccaaggctgtttacttcttcctcagaaggtaactggggtaatgaaggatgaaagagcttgcattggttcccgcggctctgatttgctggggagttgacagcgggcctcccagcatcctcaggcgctgtcaacgcctcagcagcggcacaactttcatcttcttcttgcttctgagcctccccatccttgggatctgctttgttctcagtgggctgctcgacaaacttcagcagtggggatctcgacctctgtccactaggaagagtggggtcgctgaacagtatggtgtccttgcccctcccaaatcctactgaaacattgtagctcaggcctggaagactccacaaaccagaaacttccagagttcttaattttttttccagctcagccacccgattccctaggattttgttggtttgcctctggtgctgaatgaccatgtttttctcgtggattgtttccaacagggctgttgccagagatttcaggtcagaaatggactgcggagtagctgggaggctgcatccatgatcctcagatagcagatcctgaacttgctttgcagacaggactcctgtcagagcactgctgctggatttaccctggcccttcgagtttttccgtctctccagagcattcttgtatttggcaatgtttgatttcaagaggttgacctcttcatggagttgctttaatctctcttgaaggtacctgttctccatacacagggcgtccacgtcaatgatgcggttctcgtgcccactcaggatatggttcagctcctggttgagcctctccactttgtcctggtaggaagaccgttcttctttaacatcctgaagctcgtccacagaagcctgcaggtcgtgctccagagactcaatctgttccttagctcgctctagctgctgcaccaagtcttcacgctcatgggctgcaaagtgtcgcacgccgattgcttcgtctccgagcctttgtttggcaatcgtcatcctcaagagcttgttgtcgccctggacttctccaagcctttgctgaagttctttaatttcttctcccagatgtttatttcggtcctgagaatctctcaatagttgtgcaagattagcctgtttccttttttcaggaggaagtgatggatctccatcaatcagctctcggtacttcttcttcagtgactggtggcgctcccggagctgattggccatgagtttgtactggtccctttcctgttgacaggtgtccagctccttggagaggatcagcagggcttccttcttactctccagcttcctcttacacaccaggtacagatgtgaggctctgtgcaagttccttagcctgtctgagccactgtttccttatctcgctcaccagcccctgccagtcgctctcagtccggtcgccgttcatggcctcctcctccatgcgctggccggcctcctggacccccgcc

SEQ ID NO: 10007 - RNA, 4458 nt, Homo sapiens
  source 1..4458: mol_type = other RNA
cacacacacacacacacgtatgtgggaagaaacttccttctgcctttgaacaggtgttatctggagctgttgcagccacctcgttatcatgagaaagcagctgacacagcaggaagagcaggaagatggaaacctagaaccttgacaactttcttgaatgtatagccctggaatgccttactttcgaagttcctgttatacaacataattcatttccctaccgcttaagtttctgttaagtgtggcttgaagctgagaggaccatgactgatgcagggttatctagtgaagtaggggacagaatgccacaaccttaaactttgatcctaaaaaagacaaaagacagctgtaagtaattgcagaaagcccctttaatgtctgtggaacagaagaaccatgttggatggggaaagcaggggcaggacacacgtgtcgcgtatctatggggtgttatcagggttatatctgtgacaggatcaactaacttactggctctcatttcacctgataacataagaccctccccgctgactacacacagtttaggttatcactccttatgactcctgctccctgccctgcaccctagattctctgggactcactgcagttttcctgactctgatggaatgtgctggagtctattacgagccctgcttttcagaaggtgctcaacaggccctgaagatgtgcatctggccgatggtgggtcaaaaccagagttctgcaggctgagatttttccttttattattattaaacttggctgtgttttccttcggtggctctggcatcctatgcagtagtgctggacatttgcaggcagttaaggcccagtacagcaggaagaatgatttctgtgactgctggtctgtgcaagccctccagctgcgggagcaacctcccttgaggagaagttgtgggggtgggcctggtggggagggcgataggctgggacagaaggaaggatggaatactggacctggtggccaggggtcaatgggatgtccttctcaccagaagcaacagaacgccgactccagcatgctcccatttcaactaaagtagtgggagacccacccaatgtgcatcaaaggcctgggtccttctgggctgcactttgaggaggagcagcatagtaagggatggggcgcccattctgctagcagagtgattcctggagatgcaatctgggagggatgtatccacgtggctgacccctcgtgtccagatgtcacatcttagtgtcatgagcctggtataaacattgaatttttaggatgcattttcactgagaggctaccactctgggagcctctctttttcctgcaaggagcgcctctcaaaggagtgattctggttctcagaggcattctgagctttgggatctagtctcaggctttccagggaaggaaaaagctatggctggatgacttttagttttctgcagtgccggatgccaactagaaaagctcatttttatctgaaaggaaagaaccagctagaattgagcatgccctcctttcccatccctgtatcatgtccttggttccacatccccccttgccatgctgttgtgaagttgttttgttttcctctctctttcccataaaaggtcatgagctctgtttctgtctttaagattcccgtacttggtggcacaaatgaggcagcctcaacattctgttgaaggagtgaagggtttggaagttccaggtggtgcaggaaactagactggctcccagcaggtagatctttcccaaacctgaaatggccatacaatcctgtatgtgagacaggctgaatgcagagaatgagcatttccaggtggtagctctcatctcatctcacaaaaaaaaccagaccaccactgggagtcctgttccccggcttttatgctcacccctcccagtcacttcagatcagttaattctccagatttacaagctagaaaactccagctctggcactcagcacacaggcctcaaccggggctgtggatttcaacccagaagcccaaacttctcagccggcttaaggccccttccaactgccagtctgtaccacgacagcagtgctgtgggcacaatgccaagcacacccatgccaggcagtcctcctgggccctgacttgatggggtgcagccatgggtcctctggacacgttttgctcaattataccttcctctccagctgcctaaccttgaccaagatggggacctgattaaaaaccccatcagtttctagctcttcccataattttgattgacaacattaaatgctaatacaaaaacatcttatctctgataaaacaaaagctgacagaaagacggatgctgaaaaccagccatatggtggacacgattcctgggcctggccctgttcacagtagcactctctggcagaaaagagatgacactgagaagcttgaggacctacatttaataaatcaaactgtactggcatcatcagaatattcacagtttgcaacaggatcagtgcgttttctcacttgcagactcggaggtatttcaggagaaggcgacgtgagcgcaccattccgatgcttcattcttgaccctctctggggctttcaatgtgtcattgtgtcagatccctctccccttcaggttttcacggtgctcctcatgcctccgccctctgggatccctttgccgtcttccggtgtggaagctttggctgctggccggctggcctcgaaggagtccaggtgagatttagggagctccccctggatggccaggcctggcggggctggccccgtctcactcctctgaccttctatgggactctctcttctgacctcttccagttctgcagctgcctgttcctttgtcagtttaattatttccctcccaaggctgtttacttcttcctcagaaggtaactggggtaatgaaggatgaaagagcttgcattggttcccgcggctctgatttgctggggagttgacagcgggcctcccagcatcctcaggcgctgtcaacgcctcagcagcggcacaactttcatcttcttcttgcttctgagcctccccatccttgggatctgctttgttctcagtgggctgctcgacaaacttcagcagtggggatctcgacctctgtccactaggaagagtggggtcgctgaacagtatggtgtccttgcccctcccaaatcctactgaaacattgtagctcaggcctggaagactccacaaaccagaaacttccagagttcttaattttttttccagctcagccacccgattccctaggattttgttggtttgcctctggtgctgaatgaccatgtttttctcgtggattgtttccaacagggctgttgccagagatttcaggtcagaaatggactgcggagtagctgggaggctgcatccatgatcctcagatagcagatcctgaacttgctttgcagacaggactcctgtcagagcactgctgctggatttaccctggcccttcgagtttttccgtctctccagagcattcttgtatttggcaatgtttgatttcaagaggttgacctcttcatggagttgctttaatctctcttgaaggtacctgttctccatacacagggcgtccacgtcaatgatgcggttctcgtgcccactcaggatatggttcagctcctggttgagcctctccactttgtcctggtaggaagaccgttcttctttaacatcctgaagctcgtccacagaagcctgcaggtcgtgctccagagactcaatctgttccttagctcgctctagctgctgcaccaagtcttcacgctcatgggctgcaaagtgtcgcacgccgattgcttcgtctccgagcctttgtttggcaatcgtcatcctcaagagcttgttgtcgccctggacttctccaagcctttgctgaagttctttaatttcttctcccagatgtttatttcggtcctgagaatctctcaatagttgtgcaagattagcctgtttccttttttcaggaggaagtgatggatctccatcaatcagctctcggtacttcttcttcagtgactggtggcgctcccggagctgattggccatgagtttgtactggtccctttcctgttgacaggtgtccagctccttggagaggatcagcagggcttccttcttactctccagcttcctcttacacaccaggtactcagaatcccaagtggccgctctggcgatgatgatgatgatgacgacgacgatgacgaccatgatggtgatgatgatgagttaatgacgtggcaactatccactacttatgaataagtagtgctgacagatgtgaggctctgtgcaagttccttagcctgtctgagccactgtttccttatctcgctcaccagcccctgccagtcgctctcagtccggtcgccgttcatggcctcctcctccatgcgctggccggcctcctggacccccgcc

SEQ ID NO: 10008 - RNA, 4253 nt, Homo sapiens
  source 1..4253: mol_type = other RNA
cacacacacacacacacgtatgtgggaagaaacttccttctgcctttgaacaggtgttatctggagctgttgcagccacctcgttatcatgagaaagcagctgacacagcaggaagagcaggaagatggaaacctagaaccttgacaactttcttgaatgtatagccctggaatgccttactttcgaagttcctgttatacaacataattcatttccctaccgcttaagtttctgttaagtgtggcttgaagctgagaggaccatgactgatgcagggttatctagtgaagtaggggacagaatgccacaaccttaaactttgatcctaaaaaagacaaaagacagctgtaagtaattgcagaaagcccctttaatgtctgtggaacagaagaaccatgttggatggggaaagcaggggcaggacacacgtgtcgcgtatctatggggtgttatcagggttatatctgtgacaggatcaactaacttactggctctcatttcacctgataacataagaccctccccgctgactacacacagtttaggttatcactccttatgactcctgctccctgccctgcaccctagattctctgggactcactgcagttttcctgactctgatggaatgtgctggagtctattacgagccctgcttttcagaaggtgctcaacaggccctgaagatgtgcatctggccgatggtgggtcaaaaccagagttctgcaggctgagatttttccttttattattattaaacttggctgtgttttccttcggtggctctggcatcctatgcagtagtgctggacatttgcaggcagttaaggcccagtacagcaggaagaatgatttctgtgactgctggtctgtgcaagccctccagctgcgggagcaacctcccttgaggagaagttgtgggggtgggcctggtggggagggcgataggctgggacagaaggaaggatggaatactggacctggtggccaggggtcaatgggatgtccttctcaccagaagcaacagaacgccgactccagcatgctcccatttcaactaaagtagtgggagacccacccaatgtgcatcaaaggcctgggtccttctgggctgcactttgaggaggagcagcatagtaagggatggggcgcccattctgctagcagagtgattcctggagatgcaatctgggagggatgtatccacgtggctgacccctcgtgtccagatgtcacatcttagtgtcatgagcctggtataaacattgaatttttaggatgcattttcactgagaggctaccactctgggagcctctctttttcctgcaaggagcgcctctcaaaggagtgattctggttctcagaggcattctgagctttgggatctagtctcaggctttccagggaaggaaaaagctatggctggatgacttttagttttctgcagtgccggatgccaactagaaaagctcatttttatctgaaaggaaagaaccagctagaattgagcatgccctcctttcccatccctgtatcatgtccttggttccacatccccccttgccatgctgttgtgaagttgttttgttttcctctctctttcccataaaaggtcatgagctctgtttctgtctttaagattcccgtacttggtggcacaaatgaggcagcctcaacattctgttgaaggagtgaagggtttggaagttccaggtggtgcaggaaactagactggctcccagcaggtagatctttcccaaacctgaaatggccatacaatcctgtatgtgagacaggctgaatgcagagaatgagcatttccaggtggtagctctcatctcatctcacaaaaaaaaccagaccaccactgggagtcctgttccccggcttttatgctcacccctcccagtcacttcagatcagttaattctccagatttacaagctagaaaactccagctctggcactcagcacacaggcctcaaccggggctgtggatttcaacccagaagcccaaacttctcagccggcttaaggccccttccaactgccagtctgtaccacgacagcagtgctgtgggcacaatgccaagcacacccatgccaggcagtcctcctgggccctgacttgatggggtgcagccatgggtcctctggacacgttttgctcaattataccttcctctccagctgcctaaccttgaccaagatggggacctgattaaaaaccccatcagtttctagctcttcccataattttgattgacaacattaaatgctaatacaaaaacatcttatctctgataaaacaaaagctgacagaaagacggatgctgaaaaccagccatatggtggacacgattcctgggcctggccctgttcacagtagcactctctggcagaaaagagatgacactgagaagcttgaggacctacatttaataaatcaaactgtactggcatcatcagaatattcacagtttgcaacaggatcagtgcgttttctcacttgcagactcggaggtatttcaggagaaggcgacgtgagcgcaccattccgatgcttcattcttgaccctctctggggctttcaatgtgtcattgtgtcagatccctctccccttcaggttttcacggtgctcctcatgcctccgccctctgggatccctttgccgtcttccggtgtggaagctttggctgctggccggctggcctcgaaggagtccaggtgagatttagggagctccccctggatggccaggcctggcggggctggccccgtctcactcctctgaccttctatgggactctctcttctgacctcttccagttctgcagctgcctgttcctttgtcagtttaattatttccctcccaaggctgtttacttcttcctcagaaggtaactggggtaatgaaggatgaaagagcttgcattggttcccgcggctctgatttgctggggagttgacagcgggcctcccagcatcctcaggcgctgtcaacgcctcagcagcggcacaactttcatcttcttcttgcttctgagcctccccatccttgggatctgctttgttctcagtgggctgctcgacaaacttcagcagtggggatctcgacctctgtccactaggaagagtggggtcgctgaacagtatggtgtccttgcccctcccaaatcctactgaaacattgtagctcaggcctggaagactccacaaaccagaaacttccagagttcttaattttttttccagctcagccacccgattccctaggattttgttggtttgcctctggtgctgaatgaccatgtttttctcgtggattgtttccaacagggctgttgccagagatttcaggtcagaaatggactgcggagtagctgggaggctgcatccatgatcctcagatagcagatcctgaacttgctttgcagacaggactcctgtcagagcactgctgctggatttaccctggcccttcgagtttttccgtctctccagagcattcttgtatttggcaatgtttgatttcaagaggttgacctcttcatggagttgctttaatctctcttgaaggtacctgttctccatacacagggcgtccacgtcaatgatgcggttctcgtgcccactcaggatatggttcagctcctggttgagcctctccactttgtcctggtaggaagaccgttcttctttaacatcctgaagctcgtccacagaagcctgcaggtcgtgctccagagactcaatctgttccttagctcgctctagctgctgcaccaagtcttcacgctcatgggctgcaaagtgtcgcacgccgattgcttcgtctccgagcctttgtttggcaatcgtcatcctcaagagcttgttgtcgccctggacttctccaagcctttgctgaagttctttaatttcttctcccagatgtttatttcggtcctgagaatctctcaatagttgtgcaagattagcctgtttccttttttcaggaggaagtgatggatctccatcaatcagctctcggtacttcttcttcagtgactggtggcgctcccggagctgattggccatgagtttgtactggtccctttcctgttgacaggtgtccagctccttggagaggatcagcagggcttccttcttactctccagcttcctcttacacaccaggtactgacgttcacatcgcttcacaaggtttagtggattcagaaggacatctggactccaggaaaatttaa

SEQ ID NO: 10009 - RNA, 15512 nt, Homo sapiens
  source 1..15512: mol_type = other RNA
cacacacacacacacacgtatgtttattgcggcactattcacaatagcaaagacttggaaccaacccaaatgtccaacaatgatagactggattaagaaaatgtggcacatatacacatatgcagccataaaaaatgatgagttcatgtcctttgtagggacacggatgaaattgaaaatcatcattctcagtaaactatcgcaagaacaaaaaaccaaacaccgcatattctcactcataggtgggaattgaacaatgagaacacatggacacaggaaggggaacatcacactctggggactattgaggggtggggggaggggggagggatagcattgggagatatacctaatgctagatgacgagttagtgggtgcagcgaccagcatgtcacatgtatacatatgtaactaacctgcacagtgtgcacatgtaccctaaaacttaaataataaaaaaaaaagacaatacgcgcacagttgaacatagacccttatcagtagttctgttttgccttttgtcttgtttcctcagaagcatgtgatctttgttctgcttttgccctttgaagcatgtgatctttgtacctactccctgttttacaccccctccccttttgaaacccttaataaaaaacttgctggtttgaggctcaggtgggcatcacagtcctactgatatgcgacgtcacccccggcagcccagctgttaaaattcctctctttgtactatttctctttatttctcagtcggccgacacttatggaaaatagaaagaacctatgttgaaatattgggggtgggttcccccaatacttctgtatttttcagattctctttactgagcatatattatttttacaatcagaaaaaaatgaacggatttattttcaaatgccccccattgctcttctttaaatatacagaatatattctttacatataaaacactgctccttcagagccaagcaaaggatcactcattttccccttaactgagaacaagggctgcacatgaacaaaacgcctgctttaaaatgtacccatggctggatgctgtggctcacacttataatcccagcactttgagaggctaaggtgggtggatcacttgagctcaggagtttgagaccagcctgggcaacatagcgaaactctgtctctataacaaatacaccaaaaattagctaggcatggtggtgtgtgcctgtagtctcagctatttgcaaggctgacgtgggaggatcactagagcccaggaggtcgaggctgcagtgacctgtgattacaccactgcactccagcctgggagacagagtgagaccctctctctcaaaaaaaaaaaaaaatgtacccatatttgttttcatcaggtatggtaagatgacagacacagagaaaactatctctgcaagaagagtttgttatgcagttcccaggaggagaggtgtgtcacgccttgcagggccacacaggaagaacttgggtcagccaagaagcagagggggtgagggaaaagcacgatccagcgcctttaatgtagtttccagcagaaaggcaaggcaaggcagggaagcaggcttaggattggctaatctgtataactttggcaggccctggctatagggattgtccctagttgtcccatgcctggccctggagtgatttagggcagggggaatattggcttgctgtgtcagagtttgataaaggaggtgactgggggtgtgggctctggattgactggtttgcatacgaaaggcacgctcgaccaagttgtttactctctccccaaagtagctagccctgggaggggcagtctctccaggataatgcattataaaaacaacaacagcacctgattagtataatgacatatgtttctcttcacagcagtttgtaatagcaaaggttggaaaccgttgaatgggatttccatcacataaagaactggttatgtaaattatgttacactgatacaatccaatgagcctcccttcagagagaggcaccctcatggcctaattacttctttaaggaccccatctcaatactatcacattggcaataacctgaattttggaagggacacattcaaaccatagcagagatgtaatcaaattaagatgaaatcattgggctgggcctaagccaatatgactggtgtctttataagaagagggaaatttggacatagacctatagacacagggagaagatggccatgtgacaacgaggcagagactgcagtgatgcatctatatgccaggcaacgccaagaaattcctcatgaaggaaccaaccttgccaacactttgattttagacttctagcctccagaaccgtaaggtgataaatttctgttgtttaagccacccagcctgtggtactctcttacagtagccctcctgactaatataggccctttctcaactttccctagaagcccaggtttccttgctacaaccctggcagaggctttggcacatttcacccctcctctctttgtgattggttttcacaaagaagctcaaagtggaggaatgatctctggacatgaagcctgaggaccatgcaagctccttcctgccagaggctctgttctgggttctacctgacctggactctgagggctctgagcagggaagggttagaacccagcgtggatcaaacatttgagatgaatcagcactgatagctggaatgtgagctcccaagtggcttgagctcactctgctcaggaccctctgcagctcctgggggaacactggcacagacgggtgcacagttaatattcagttaacaccggctggctgaatgaagggcgagctatcttgagcctgacttttctgatccttcaatgagcatgctaacatcatccaacccctgaccttgtggtgaggatcaaagacgttaatgcccactaaacgctttctacgatgcctggaaacaactgttatcaatactgtgctatgttttagtaaagagggctgttccctgagagcaaaattggcaagtgggtctcacctcccatgctgactccaattgttgggtgcggttgcatggattgatgtcaaaagcctcccaaggcccagtctgggccagatgcagggactgtcatgatcccttagcagtgtttgctctggaaaaggaggaacagggacctgggtgccatctcttcacagcgctccacccctagggcctgcttaaatggcacagccagctcctcagagagacaggacacactctccttctgcctgcagttgtgaggaaagaaggggcactgaggaggatgggtcaccccgggagcagagcctggctcatatcctggtatccctgcagaggctggaggtggggccagcaccacctgaggacatgtagccttcccaggattctggcgtgtgttcccatccctagcaggaaagaagtggaaattagccaatcaccctggaagtgggcaaccagtctttctcccctttcctgtgaattcactcaggacactggggacaaaagacatcacagaccctatctcccgtgctcttttacagtggctatttcatttagtactagggggctttttgcctgtattttataaatgagcaaagaggactggagggtctgagtgatttgtccagggtcatcctctgtcctttggcttttacctgtgtcaccacagcctcctggggagatggctgtgaaagtgggcaaagggtgagtctcagcttcacagggctgcagcatcagcagcctctcttgcctgtccgtcagcactgacaggggcaacacctggcctggcacaaggctctccgcttcttgccctcaggacttggagtctcttggaaggagcctcagcccttctcttggttcctgcttttgtctctagccttcctagagtagctcagatcagttcacacccctctacccacgactacccaggaaaggacatgatccctcattaagacccagctattgcctaagggtcactgagggcctcaaaccccagaggctctgtggcaggcacctgggagcccacttggcgggccttgccctggcccagacatcacagaccactctcactgcactggctattaagtgcctgctctctactagggattcctagggggtggccaagagaaggaaagacacccccacaggaaggatgggcccagaaactgactttccatggctccgacgaggggtcctgaggcactctatcgaagtgcaagtccctgaatctgtgtcccaagctctgaaaatgcaagaggtgcttggagcaaacagggagtgtcctgtcactgaaggtctgcaagcagaggggtaagggactgtttgcctcctacagatttcccttctttctcttcttctgggcctctgggccagagacaggcattttacttgatgcgatcatcctcagcacatgcctgacacatagtaggtgctcagtaattgttagctgttgttattaaccattatgtgagtttagagtgcccgtcctattgcagagagggagagagcagagacaaatggtgattctaagaacctgtccccttccctgggactcactccagtggctggtcgccagttgcacccacacgcggctggctgcgggcaggagagctgggctcattcgttctggcagctgtccctgcagatgaggatcgagggtatgtgactgcctgagcagctacttcaatcctaatgtccctttaatagctctcgtcaaattgccacagctctccccagagattttcatggctatggaaaataaatagccattatctgacctccaggggaatgaagatgtctgcagaattcggggaaaagcagttataaaactgagtagagccagcgcaccctttccctattagcaacctctaagggagtcctagctactgcctaggaaatcacaaaataaatgtattcactcctcagactctcttttttcacctattagtatgtatatgagtacatttggcttgtggtagatcaggagagagaaagaaagaaaaaacaactacaaaaatatgtaatgattagttagtccaggggtagcaggaaaagaagctggtcaagtaaagggtttaatccttttttatttttattatttttttagacagggtatcacgctgttgcccaggttggagtacagtggtacaaccatagctcactgcagcctcaaactcctgggctcaagcaatcctcctgccccagcctcccgagcagctgggactacagtgcacaccaccacacaaggctaattttcaaattttgggcagttttactatgttgcccaggctggtcctgaactcctggcctcaagggatcctcccatctcagcctcccatagtgctggggttacaggtatgagccaccaagcccagctggaagtttttaaaacgtttcaacattcaaagaatgtgagaatgaaaatgcccttccttttcttaccacctaatttggaaaagagaaactatttttttaatcccaaaaacatttggtatagctggcaaaaagtgttctgttcttatatatgagacagttcctgaaataggccctagagacagcactcacggccaagtgggaccttgctctggtactagctcaggtggccaaggggtttcaggagagggtctggacttccccacatcctgctttcatcagctctaagactaggtggtgacatctgcttctcaataaccttcaccaggcttgctgtgaaggtcacctgagataagagacgtgaaaggatgctgaagatgcaaaagcctaagccaggcagccctgcttggcctggcctcctggaaaggggcaatgccccagcccagcacacaaccagggcctcatgatgacaattctgcaaaactggtccttggctcgtcctcccttgccaggatgagactgtgcaaagccccacccacaggcagctgctccaggtgtcgtttaagggctccaaattccttccaactaaaagtatctttccatccctgttggtatagtggttaggggaaaaaaaattaaaagaaaatgaacaatgtattttccacgtcaagatgcctgaacttcccataacagctgtcactttaagaagccataagagaaagggccaggtctccataggtcattattcttcccaggcggggtcaacttcctctattaacacccatgcacgtatcagaagctacccatgaaaggccaagggcctacagcaaagctcccatgactggaaagtatttaagcataaggaacagaatagtttcgagggaaggataagaaagagagtcgggaaggctgggcagaacactacttggacaactaaaaaagcaagtggggacatctcaaagagtgggctggccactcccagaacctgtgtaagcaggaaacaaaaagcatttattgctggtaaatgcttaacaactggctctctgggataaaaatgtatatatgtacagaaatttattataaatttcattgataaaaatgatgtgcagcacataatttataaataaaatatacaatgccatttattgtaattctagaaaagttttttacagaatgcttttgttgatttttgctgactcttctatccaacctgtttgcaattcaaccatgatatgacacaaccagactacaaataaatgtttgttactatctgattcaacaaagcagtcactcatttcatggaatggatatgggctgttactcagtgaaaagacacatgagatggttcagtgctaactcacccttctgacagaaaatgccagaaagtttccaccccattgacaggcttggagtcttgagtaccatctgggtgggtggagctggcactggcacgaaacctctccactgctatcctgacagagatggggcatgtacttcccagggccacttgccaacccagggaggttttccatcttgctggtttggtgagggaggctgctttcagatttcaagtggacactgctggcctggatagggctgaggggctctgcctccaagaggtgttcttcgctttgtggcattacctctctgaagtactttagagtactttacaggcctgctttactcctcagaatcctgctgcagagctgagggctggataatttcatgttctctggcaactgatggccactgtggtaccagaggagggatgtatgtctgggcactttcaaaagtatgttattagaaagttgcgcatcacggccgggcacggtggttcatgcctgtaatcccagcactttgggaggccgaggtgggtggatcacctgaggtcaggagttcgagaccagcctggccaacactggtgaaaccccgtctctaccaaaaatacaaaaattagtggggcgtggtggcgcacgcctgtaatcccagctactccggaggctgaggaagaactgcttgaacctggggggtggaggttgcagtgagctgagatcatgccactgcactccagccctgggcaacaagaatgaaactctgtctcaaaaaaaaaaaaaaaaaaagaaagttctgcatcaatcctgttgtctcactgtaaatagcataagaacaatgttctggcccctccctccacttgagttgccaggttctacgacagggtcttccccaccatggaccagaatacaagatagcattttttctgcagtagtatccaaagcaaaaatttcatcagaaggatggcattggagtctctttcagttgaaaagtgcatgcagacaattgagtgtcagatccaggggagaggaaaaggcggcagagaactagggagacaggtcgagagtaaggagatgaagggacatttgagactctgaattttttctttttttgtagaggtgggatcttgctatgttgcccaggctagtcctgaactcctgggctcaagtgattctcccactttgacctctcaaagtgctgggaatataggcatgagccaccatgccaagccgagggaagctgtttcttacagctgggtttcttgcacatccagacttcacatcccgccttgtgcatacagactgggagtcccttgggtagcgggggacaggaatgggattggctttggccatgaggcagattaagcaacacctaaggggagttgctagtggaccaaggcccagaccacaatgcaggggagagggagaaaaggggtggaagagtgacaggaactgatatttttttagcagttactatgagaggaataaaactggacaggaaagaaagagaaaatacataaaacaaggacaggttgttcggcatctcttcaggagatgactgtctggtacatcctttaccaccattatcctcaatcaccaatcactaagcattgccatgtaccaggcccaggggctgggactatgggagctagttcttatagtggctcatgatctacttgggaaggcaagacctaaagaaatgacaagtaagccacaatggcatatgctttgtcgaatgagagggtaccaatcagcgagtgtgccggggacttagaggaaggggtcacaatgccctgggatggctgaggtccccacggagatgttgggccttgagccagaacttgagtgctggataacacttgagtggaaaggaggggcacagagactgtccagattggaatggacaaggcatagcagaaagtacggtggtacactcaaggcactgtgaacagcagtttattattattttttccttcatgctgtcttttggggtccttaggaaatgactctgttgtccttcacaagcccagctaggccctggaacaaatggcctttagagagttcaacagtatgaaactcctactacgagtaaatcaatgttaggtgttgtggggtatgtggaaaagtgaaaaaataatagtccctgccttaaaggacaagaaatgattttccctttatcaaatgtccagggaaggaaactgtgggatgacactgtggcagtgaagtctcacatctgataaaaggcagtgggctctgggcagcatggacaagtttaagaaacactggatttgccatctatcaagatgctccatttaggggtggtccaaaaggtctttcagtaactcagcagttctcttctcagaattagttcccagtctgtgccttccaatcttcccagtatattcctttaccagcacaaaaactcatgtacagccaatgaccagttcagaatagatgccaaagtaatcagactataccagtagctcaccccatgtctggtcaccaagtaagccatcacagactctgcaaataatcctggaaaggaagaggtaccaggacaagaaggaaagaactaaaacaaggatgtgaataacttctaaactggtcagccttggacaaaaggaaatctggaaatctcgacttggcctgagagaaacctcatcctggcccttaaagtgccaattaaggctgagttgaaaaggagctgggcatcatcaaactgcaaacaaacttagcttaggcacccacagtgtgatgatgtgtttatttccatgaaggagcagtctatggagaagtgcaggaactttcaaagttgcatgggcagagctgcttcttatatgacagaattggcagctgcctgtcacttcacagtgggtcacatgaatatgaagcagagaactggctgtgtgcgtcagcaggggagcttaagactgcagattctggggaatcagcactcactgtgacacatgtgatcctctgtctcctcagacaactgaaggatgatgagaaggggatctctggagccttgaccttctgggccccgaatttctagctagaaaacctcttttcaagacaaaaacataccaaagtacattttgaagtatttcgaagaatgaatcacatgccctaactttataatagaggaaggcacagatctcatttttgtgacaggtgaaacataatccttgccacaggttaactccagaagaaggaactgtacagctgaacagagcagattcttagaaactacaaactaaccaacaaacaaacaaataaggcaaagaacagctgcacatcatcttaagattccttatttaaaggttgtatctctaagccaggctattatataatcaagcaggaaaatactactaaaacttgatagttttgactggtggccttgtcttggatgttaagaaaaaatttgctgttgtttttcaaaataatagagatgggggtctcactatgttggccaggtcggtctcaaactcctgacctcaagcaatcctcccacctcccgaagtgctgcaatcataggtatgagactctgtgccccacctgttgttttttaaccaagcaatctgcaactcaactttcatgttaattcagaaaactccatttcctgacacatcaggccctgaagtgaaggagaagtgagcacaactctcactgcactaaaattcccaaggcaaggagtcaatggagctgaccaaatagcccatggtaaggtgttccaaaggaagacaccatatatagaatttgactattaagaaagggaagattcaacctcatataaagaactctttaaagaactgtacaacagctctccaagcaagtgaatgaggttttaacatactgttaagttgttaaaagaaatatttggatctaagagaatctgacaatgttatctgaatgaacaccaattttgatctatcctaagtgttaagatatatttttgaatgttaaagatattcgtgtactagggaaaaaagagtggtgagcagacggagagatggccaaggaaaaacagatcacctgactggcaggttatagctattgtgacactcttaataaagtcccttacttcctccacactgtacagaccaggctgagaaagacatgttgccaggctaccgtaagaacatttgacagcccaagtcatgtctcgaggtgaacttggagataaatcacctgtcctttcgatctctccaaaaggtctaaatatttccatggcctctccttcatccatttctaaaccaaaggcatttcagagcattcatgggttccccaagatattgcgatgaaataaccatgtctcaaccaggctcatgcctgtaatcccagcacttcaggaggctgaggtgggcagatcacaaggtcaggagtttgagatcagcctggccaacatggtgaaaacccgtctctactaaaaatacaaaaattagccgggcgtggtggcagcacctgtaatccccgctactcgggaggctgaggcaggagaatcgcttgaacccaggaggcggaggttgcagtgagccaagatcatgccattgcactccagcctgggcaacagagcaagactgtctcaaaaaaaaaaaaaaaaaagaaataaccatatctctagctcagcaatggttctgtcaaagcattatttgtaacactcaactagactaagcaatcaagaattttgggccacgttctcaactttttctcttgcctactgaatactgtttcttcctttcctaccttatttttttcattcaacaaatatttattcaatacttactacgtgcctgggtcagtactaggtgctgtgtctacaggagtgaacaagagggataaagtccctctcacaaagcatacattctaactggagagacaaacaatttcagatagagattagtgctagaaagagacaaatgatttcagatagagattagtgctagaaagaaacagggaagcaggccaggcgtggtggctcacgcctgtaataccaggactttgggaggtcgaggtgggcggatcacctgaggtcaggagttcaagaccagcctagtcaacatggtgaaaccccatctctactaaaaatacaaaatttagccaagaatggtggcgtgcacctgtagtcccagctacttgggagggtgaggcgggaaagtcgcttgaacccgggaggtggaggttgcaatgagctgagacagcgccattgcactccagcctgggcgacagagtgagactccatctcaaaaaaaaaaaaaaaagaagaagaaacagggaagcagatttcagtaagggggcaagatagaggggaggggaagaaaagccctactttagatagtctgggaagagctccaggaggaggcgacaactagtggagatctgagtgacaagtaaaagatgcaagggaaaaactctccaggcaaagggaacggatacaaaggctctgaggtggtcaagagtcaagagatggaaggaaggcctgtgtagccaaaagtgaatgaagaagagagtggataaagacaagcagaggtgatagggctgaagagcccagggaatcaaatgttataggaagacaagatttcaatcaaagtgagatgtcaaacccctggagtttttcagtaggtgtgaagccatcttaaggggcagacttaatgaggatcaagtgtcctcattaaggaggacttagagagctagtggatacgatgaaaagggaggtgctctatgagagaaatgcaggtcatcgctaaccaggctagtgtctttaggccactgcaggccaattcaactggaaatcccctcatctgacaaacacataagtgctgctctctgtcaggccccacctccccccattcttttccaagtgtctccgcctgcagcgattaggttagaaagcatttctctctgctctcgcttagacagttcctgcagtgtgtaagactacagagctgaattaggaatgtcaaagaatgttcatacataataaaggagtcacacatattagaaatgacgttgttactaaaaagccacacaatatctcatttagagaatatgcttaacaaaatatacatcttaaaaattcagcactccagaatgctttttcaggtgtttccatttgagaaataaagaataaaaattggtaataattatagacacaacttcatacaataatctggataatatgcaagaagcatcatgttgactttcagatatttctctttgtggctaacgaaccacacatcaaaggatggaccaaagttcagatgtacacagtccagggcacctccgagcacagtggcagtgcccttggggattttctttccctcagtgagagacacgggggatggggaggagcccaggagtgtcaccagaaagtacacaacccagcttcttacccagcctgctgccatcatcaactatcaaaccatttgctcctctttgcaagaggtgctcctttagaaggtcccaataatttctgcttatattgttcgaccagctggttgaagcgggtttccgtcttatttcccttagcttttttcctagatacctgctcggacgataattgctgcttctcctgcttccactggtttatctgtggctttggctttttgggatggacgggcttcactttgcctttgtcccgcaacctgattttggggcctcggtgtgaggggagcgccaggacctttcttctcttctttccatcaggcagctccacctgctccacttcagccttggtctggaacccggtccatgaggtagagcccgcctttctcttctgctctgggggcaccttgctttgttcctctgtgtggtgttgagctgccttctgttgctggtcttttgcaggctctggttgccccttctgaggctcaccagttgcaggcttggatctcattttttgcaagctgcgctggatccttaattccttcattttaagttttcttcgatcttctaaagagaactccactattggtctcttcagaggcccaaagatttctggattgttgttgatgaggcggagggctttcagggcatgctcgtgctcttggaactccgcaaaggcgtagcccagggactgacccttcatgttcccatgaactcctttgaggtctcgcatcactctacactccttgatgcgcacccctttctctccactagtagcactcagcagcagctttctgagctgtttgtcatctacagcctttgggagattgtgcaggcagagcctggttcgggagacaaagatattctggtccttgagtttctgatgcttcagcagctcaaaccgttctcttttggccatatcagcagcactcacaccctctgcagccttcgtcccagcacgaatcaagccttctcgggccagatagagattccgggtgccagtcggcttcttcaccttcgtcgtctgaagctttgcagcctcatcacgggtcaccgccaagtcaaccttgagctgccggccatccagtttaagcccaccagcctcattctctggagaagcagctagaaggcatttctgagctgcttcttgagtcatgaactgggcaaatgcacaacctttagaatgctctgtgtctggatgcaagacaatgcggacatatttgagttctccaaactgttggagaagctccccaagttcttcttcttctgagtcaaaggacagatttctgataaaaacagttttcccttcattcacatcagagggtaatttcctcttctttttgtttgagacttgcacagctttatcctcttgctcctcagtgctggtatcactctgagccagttcctctccatcatcaatactatcgctttcctctaggtcactgtcctcctcagaatgatcactgctttttgcaggggctggtctcttgactgctctcttctgaatttgcacaggcttggtcacctttgattctatattctcttcctcttcatcttcatcatcaaaaaccccatcttcttcatcatcatcatcgtcatcatcatcgttttcttcctcttccatatcctcttcctctctgcccttctttttaactgattcctgatgtttagattcatggctcttttcctcacctatagcagaaacagactgtgtatctttatatttatcctttgccacggcccaatccacagccactgtccggccttttatctctttcatgttcatgcctttgagagctttacctgcttctaggaggtttttgaactgaacaaaaccaaaaccgcgcatcttcccatctggtttcctagggatatttacttccaggacagctccaaattgagcaaatactgtcttcaagtcatcttctgaacacttaaagctcaggttccgaataattaatctggctttcttatctgccactttggcttttttagccttcggctccttctttgggcactctgagttttcatttttccccttttcctttgtcttgttcctcagttttttcttggcaacagtcacgttgatcttgcaaccttcaaaggtggtaatctccttgagggccctctgaacatcttccagcattgaaaaagtgacatagccaaagcctcgacatgccttactccctttttcagtcaccacgaagcactgcttcaccggccccacctgactgaacagttcctccagctgctcactgcgggccgagggcgggaggcggcccacaaataaggtcaggccggccatgagaccgggaaacccaaagcgcgtgaggacgcgagcaaactaggccggcgcacgcgagccgaaacgctggctttggtaggacaaccaagctcacacgccgagagattccggaagt

SEQ ID NO: 10010 - RNA, 15089 nt, Homo sapiens
  source 1..15089: mol_type = other RNA
cacacacacacacacacgtatgtttattgcggcactattcacaatagcaaagacttggaaccaacccaaatgtccaacaatgatagactggattaagaaaatgtggcacatatacacatatgcagccataaaaaatgatgagttcatgtcctttgtagggacacggatgaaattgaaaatcatcattctcagtaaactatcgcaagaacaaaaaaccaaacaccgcatattctcactcataggtgggaattgaacaatgagaacacatggacacaggaaggggaacatcacactctggggactattgaggggtggggggaggggggagggatagcattgggagatatacctaatgctagatgacgagttagtgggtgcagcgaccagcatgtcacatgtatacatatgtaactaacctgcacagtgtgcacatgtaccctaaaacttaaataataaaaaaaaaagacaatacgcgcacagttgaacatagacccttatcagtagttctgttttgccttttgtcttgtttcctcagaagcatgtgatctttgttctgcttttgccctttgaagcatgtgatctttgtacctactccctgttttacaccccctccccttttgaaacccttaataaaaaacttgctggtttgaggctcaggtgggcatcacagtcctactgatatgcgacgtcacccccggcagcccagctgttaaaattcctctctttgtactatttctctttatttctcagtcggccgacacttatggaaaatagaaagaacctatgttgaaatattgggggtgggttcccccaatacttctgtatttttcagattctctttactgagcatatattatttttacaatcagaaaaaaatgaacggatttattttcaaatgccccccattgctcttctttaaatatacagaatatattctttacatataaaacactgctccttcagagccaagcaaaggatcactcattttccccttaactgagaacaagggctgcacatgaacaaaacgcctgctttaaaatgtacccatggctggatgctgtggctcacacttataatcccagcactttgagaggctaaggtgggtggatcacttgagctcaggagtttgagaccagcctgggcaacatagcgaaactctgtctctataacaaatacaccaaaaattagctaggcatggtggtgtgtgcctgtagtctcagctatttgcaaggctgacgtgggaggatcactagagcccaggaggtcgaggctgcagtgacctgtgattacaccactgcactccagcctgggagacagagtgagaccctctctctcaaaaaaaaaaaaaaatgtacccatatttgttttcatcaggtatggtaagatgacagacacagagaaaactatctctgcaagaagagtttgttatgcagttcccaggaggagaggtgtgtcacgccttgcagggccacacaggaagaacttgggtcagccaagaagcagagggggtgagggaaaagcacgatccagcgcctttaatgtagtttccagcagaaaggcaaggcaaggcagggaagcaggcttaggattggctaatctgtataactttggcaggccctggctatagggattgtccctagttgtcccatgcctggccctggagtgatttagggcagggggaatattggcttgctgtgtcagagtttgataaaggaggtgactgggggtgtgggctctggattgactggtttgcatacgaaaggcacgctcgaccaagttgtttactctctccccaaagtagctagccctgggaggggcagtctctccaggataatgcattataaaaacaacaacagcacctgattagtataatgacatatgtttctcttcacagcagtttgtaatagcaaaggttggaaaccgttgaatgggatttccatcacataaagaactggttatgtaaattatgttacactgatacaatccaatgagcctcccttcagagagaggcaccctcatggcctaattacttctttaaggaccccatctcaatactatcacattggcaataacctgaattttggaagggacacattcaaaccatagcagagatgtaatcaaattaagatgaaatcattgggctgggcctaagccaatatgactggtgtctttataagaagagggaaatttggacatagacctatagacacagggagaagatggccatgtgacaacgaggcagagactgcagtgatgcatctatatgccaggcaacgccaagaaattcctcatgaaggaaccaaccttgccaacactttgattttagacttctagcctccagaaccgtaaggtgataaatttctgttgtttaagccacccagcctgtggtactctcttacagtagccctcctgactaatataggccctttctcaactttccctagaagcccaggtttccttgctacaaccctggcagaggctttggcacatttcacccctcctctctttgtgattggttttcacaaagaagctcaaagtggaggaatgatctctggacatgaagcctgaggaccatgcaagctccttcctgccagaggctctgttctgggttctacctgacctggactctgagggctctgagcagggaagggttagaacccagcgtggatcaaacatttgagatgaatcagcactgatagctggaatgtgagctcccaagtggcttgagctcactctgctcaggaccctctgcagctcctgggggaacactggcacagacgggtgcacagttaatattcagttaacaccggctggctgaatgaagggcgagctatcttgagcctgacttttctgatccttcaatgagcatgctaacatcatccaacccctgaccttgtggtgaggatcaaagacgttaatgcccactaaacgctttctacgatgcctggaaacaactgttatcaatactgtgctatgttttagtaaagagggctgttccctgagagcaaaattggcaagtgggtctcacctcccatgctgactccaattgttgggtgcggttgcatggattgatgtcaaaagcctcccaaggcccagtctgggccagatgcagggactgtcatgatcccttagcagtgtttgctctggaaaaggaggaacagggacctgggtgccatctcttcacagcgctccacccctagggcctgcttaaatggcacagccagctcctcagagagacaggacacactctccttctgcctgcagttgtgaggaaagaaggggcactgaggaggatgggtcaccccgggagcagagcctggctcatatcctggtatccctgcagaggctggaggtggggccagcaccacctgaggacatgtagccttcccaggattctggcgtgtgttcccatccctagcaggaaagaagtggaaattagccaatcaccctggaagtgggcaaccagtctttctcccctttcctgtgaattcactcaggacactggggacaaaagacatcacagaccctatctcccgtgctcttttacagtggctatttcatttagtactagggggctttttgcctgtattttataaatgagcaaagaggactggagggtctgagtgatttgtccagggtcatcctctgtcctttggcttttacctgtgtcaccacagcctcctggggagatggctgtgaaagtgggcaaagggtgagtctcagcttcacagggctgcagcatcagcagcctctcttgcctgtccgtcagcactgacaggggcaacacctggcctggcacaaggctctccgcttcttgccctcaggacttggagtctcttggaaggagcctcagcccttctcttggttcctgcttttgtctctagccttcctagagtagctcagatcagttcacacccctctacccacgactacccaggaaaggacatgatccctcattaagacccagctattgcctaagggtcactgagggcctcaaaccccagaggctctgtggcaggcacctgggagcccacttggcgggccttgccctggcccagacatcacagaccactctcactgcactggctattaagtgcctgctctctactagggattcctagggggtggccaagagaaggaaagacacccccacaggaaggatgggcccagaaactgactttccatggctccgacgaggggtcctgaggcactctatcgaagtgcaagtccctgaatctgtgtcccaagctctgaaaatgcaagaggtgcttggagcaaacagggagtgtcctgtcactgaaggtctgcaagcagaggggtaagggactgtttgcctcctacagatttcccttctttctcttcttctgggcctctgggccagagacaggcattttacttgatgcgatcatcctcagcacatgcctgacacatagtaggtgctcagtaattgttagctgttgttattaaccattatgtgagtttagagtgcccgtcctattgcagagagggagagagcagagacaaatggtgattctaagaacctgtccccttccctgggactcactccagtggctggtcgccagttgcacccacacgcggctggctgcgggcaggagagctgggctcattcgttctggcagctgtccctgcagatgaggatcgagggtatgtgactgcctgagcagctacttcaatcctaatgtccctttaatagctctcgtcaaattgccacagctctccccagagattttcatggctatggaaaataaatagccattatctgacctccaggggaatgaagatgtctgcagaattcggggaaaagcagttataaaactgagtagagccagcgcaccctttccctattagcaacctctaagggagtcctagctactgcctaggaaatcacaaaataaatgtattcactcctcagactctcttttttcacctattagtatgtatatgagtacatttggcttgtggtagatcaggagagagaaagaaagaaaaaacaactacaaaaatatgtaatgattagttagtccaggggtagcaggaaaagaagctggtcaagtaaagggtttaatccttttttatttttattatttttttagacagggtatcacgctgttgcccaggttggagtacagtggtacaaccatagctcactgcagcctcaaactcctgggctcaagcaatcctcctgccccagcctcccgagcagctgggactacagtgcacaccaccacacaaggctaattttcaaattttgggcagttttactatgttgcccaggctggtcctgaactcctggcctcaagggatcctcccatctcagcctcccatagtgctggggttacaggtatgagccaccaagcccagctggaagtttttaaaacgtttcaacattcaaagaatgtgagaatgaaaatgcccttccttttcttaccacctaatttggaaaagagaaactatttttttaatcccaaaaacatttggtatagctggcaaaaagtgttctgttcttatatatgagacagttcctgaaataggccctagagacagcactcacggccaagtgggaccttgctctggtactagctcaggtggccaaggggtttcaggagagggtctggacttccccacatcctgctttcatcagctctaagactaggtggtgacatctgcttctcaataaccttcaccaggcttgctgtgaaggtcacctgagataagagacgtgaaaggatgctgaagatgcaaaagcctaagccaggcagccctgcttggcctggcctcctggaaaggggcaatgccccagcccagcacacaaccagggcctcatgatgacaattctgcaaaactggtccttggctcgtcctcccttgccaggatgagactgtgcaaagccccacccacaggcagctgctccaggtgtcgtttaagggctccaaattccttccaactaaaagtatctttccatccctgttggtatagtggttaggggaaaaaaaattaaaagaaaatgaacaatgtattttccacgtcaagatgcctgaacttcccataacagctgtcactttaagaagccataagagaaagggccaggtctccataggtcattattcttcccaggcggggtcaacttcctctattaacacccatgcacgtatcagaagctacccatgaaaggccaagggcctacagcaaagctcccatgactggaaagtatttaagcataaggaacagaatagtttcgagggaaggataagaaagagagtcgggaaggctgggcagaacactacttggacaactaaaaaagcaagtggggacatctcaaagagtgggctggccactcccagaacctgtgtaagcaggaaacaaaaagcatttattgctggtaaatgcttaacaactggctctctgggataaaaatgtatatatgtacagaaatttattataaatttcattgataaaaatgatgtgcagcacataatttataaataaaatatacaatgccatttattgtaattctagaaaagttttttacagaatgcttttgttgatttttgctgactcttctatccaacctgtttgcaattcaaccatgatatgacacaaccagactacaaataaatgtttgttactatctgattcaacaaagcagtcactcatttcatggaatggatatgggctgttactcagtgaaaagacacatgagatggttcagtgctaactcacccttctgacagaaaatgccagaaagtttccaccccattgacaggcttggagtcttgagtaccatctgggtgggtggagctggcactggcacgaaacctctccactgctatcctgacagagatggggcatgtacttcccagggccacttgccaacccagggaggttttccatcttgctggtttggtgagggaggctgctttcagatttcaagtggacactgctggcctggatagggctgaggggctctgcctccaagaggtgttcttcgctttgtggcattacctctctgaagtactttagagtactttacaggcctgctttactcctcagaatcctgctgcagagctgagggctggataatttcatgttctctggcaactgatggccactgtggtaccagaggagggatgtatgtctgggcactttcaaaagtatgttattagaaagttgcgcatcacggccgggcacggtggttcatgcctgtaatcccagcactttgggaggccgaggtgggtggatcacctgaggtcaggagttcgagaccagcctggccaacactggtgaaaccccgtctctaccaaaaatacaaaaattagtggggcgtggtggcgcacgcctgtaatcccagctactccggaggctgaggaagaactgcttgaacctggggggtggaggttgcagtgagctgagatcatgccactgcactccagccctgggcaacaagaatgaaactctgtctcaaaaaaaaaaaaaaaaaaagaaagttctgcatcaatcctgttgtctcactgtaaatagcataagaacaatgttctggcccctccctccacttgagttgccaggttctacgacagggtcttccccaccatggaccagaatacaagatagcattttttctgcagtagtatccaaagcaaaaatttcatcagaaggatggcattggagtctctttcagttgaaaagtgcatgcagacaattgagtgtcagatccaggggagaggaaaaggcggcagagaactagggagacaggtcgagagtaaggagatgaagggacatttgagactctgaattttttctttttttgtagaggtgggatcttgctatgttgcccaggctagtcctgaactcctgggctcaagtgattctcccactttgacctctcaaagtgctgggaatataggcatgagccaccatgccaagccgagggaagctgtttcttacagctgggtttcttgcacatccagacttcacatcccgccttgtgcatacagactgggagtcccttgggtagcgggggacaggaatgggattggctttggccatgaggcagattaagcaacacctaaggggagttgctagtggaccaaggcccagaccacaatgcaggggagagggagaaaaggggtggaagagtgacaggaactgatatttttttagcagttactatgagaggaataaaactggacaggaaagaaagagaaaatacataaaacaaggacaggttgttcggcatctcttcaggagatgactgtctggtacatcctttaccaccattatcctcaatcaccaatcactaagcattgccatgtaccaggcccaggggctgggactatgggagctagttcttatagtggctcatgatctacttgggaaggcaagacctaaagaaatgacaagtaagccacaatggcatatgctttgtcgaatgagagggtaccaatcagcgagtgtgccggggacttagaggaaggggtcacaatgccctgggatggctgaggtccccacggagatgttgggccttgagccagaacttgagtgctggataacacttgagtggaaaggaggggcacagagactgtccagattggaatggacaaggcatagcagaaagtacggtggtacactcaaggcactgtgaacagcagtttattattattttttccttcatgctgtcttttggggtccttaggaaatgactctgttgtccttcacaagcccagctaggccctggaacaaatggcctttagagagttcaacagtatgaaactcctactacgagtaaatcaatgttaggtgttgtggggtatgtggaaaagtgaaaaaataatagtccctgccttaaaggacaagaaatgattttccctttatcaaatgtccagggaaggaaactgtgggatgacactgtggcagtgaagtctcacatctgataaaaggcagtgggctctgggcagcatggacaagtttaagaaacactggatttgccatctatcaagatgctccatttaggggtggtccaaaaggtctttcagtaactcagcagttctcttctcagaattagttcccagtctgtgccttccaatcttcccagtatattcctttaccagcacaaaaactcatgtacagccaatgaccagttcagaatagatgccaaagtaatcagactataccagtagctcaccccatgtctggtcaccaagtaagccatcacagactctgcaaataatcctggaaaggaagaggtaccaggacaagaaggaaagaactaaaacaaggatgtgaataacttctaaactggtcagccttggacaaaaggaaatctggaaatctcgacttggcctgagagaaacctcatcctggcccttaaagtgccaattaaggctgagttgaaaaggagctgggcatcatcaaactgcaaacaaacttagcttaggcacccacagtgtgatgatgtgtttatttccatgaaggagcagtctatggagaagtgcaggaactttcaaagttgcatgggcagagctgcttcttatatgacagaattggcagctgcctgtcacttcacagtgggtcacatgaatatgaagcagagaactggctgtgtgcgtcagcaggggagcttaagactgcagattctggggaatcagcactcactgtgacacatgtgatcctctgtctcctcagacaactgaaggatgatgagaaggggatctctggagccttgaccttctgggccccgaatttctagctagaaaacctcttttcaagacaaaaacataccaaagtacattttgaagtatttcgaagaatgaatcacatgccctaactttataatagaggaaggcacagatctcatttttgtgacaggtgaaacataatccttgccacaggttaactccagaagaaggaactgtacagctgaacagagcagattcttagaaactacaaactaaccaacaaacaaacaaataaggcaaagaacagctgcacatcatcttaagattccttatttaaaggttgtatctctaagccaggctattatataatcaagcaggaaaatactactaaaacttgatagttttgactggtggccttgtcttggatgttaagaaaaaatttgctgttgtttttcaaaataatagagatgggggtctcactatgttggccaggtcggtctcaaactcctgacctcaagcaatcctcccacctcccgaagtgctgcaatcataggtatgagactctgtgccccacctgttgttttttaaccaagcaatctgcaactcaactttcatgttaattcagaaaactccatttcctgacacatcaggccctgaagtgaaggagaagtgagcacaactctcactgcactaaaattcccaaggcaaggagtcaatggagctgaccaaatagcccatggtaaggtgttccaaaggaagacaccatatatagaatttgactattaagaaagggaagattcaacctcatataaagaactctttaaagaactgtacaacagctctccaagcaagtgaatgaggttttaacatactgttaagttgttaaaagaaatatttggatctaagagaatctgacaatgttatctgaatgaacaccaattttgatctatcctaagtgttaagatatatttttgaatgttaaagatattcgtgtactagggaaaaaagagtggtgagcagacggagagatggccaaggaaaaacagatcacctgactggcaggttatagctattgtgacactcttaataaagtcccttacttcctccacactgtacagaccaggctgagaaagacatgttgccaggctaccgtaagaacatttgacagcccaagtcatgtctcgaggtgaacttggagataaatcacctgtcctttcgatctctccaaaaggtctaaatatttccatggcctctccttcatccatttctaaaccaaaggcatttcagagcattcatgggttccccaagatattgcgatgaaataaccatgtctcaaccaggctcatgcctgtaatcccagcacttcaggaggctgaggtgggcagatcacaaggtcaggagtttgagatcagcctggccaacatggtgaaaacccgtctctactaaaaatacaaaaattagccgggcgtggtggcagcacctgtaatccccgctactcgggaggctgaggcaggagaatcgcttgaacccaggaggcggaggttgcagtgagccaagatcatgccattgcactccagcctgggcaacagagcaagactgtctcaaaaaaaaaaaaaaaaaagaaataaccatatctctagctcagcaatggttctgtcaaagcattatttgtaacactcaactagactaagcaatcaagaattttgggccacgttctcaactttttctcttgcctactgaatactgtttcttcctttcctaccttatttttttcattcaacaaatatttattcaatacttactacgtgcctgggtcagtactaggtgctgtgtctacaggagtgaacaagagggataaagtccctctcacaaagcatacattctaactggagagacaaacaatttcagatagagattagtgctagaaagagacaaatgatttcagatagagattagtgctagaaagaaacagggaagcaggccaggcgtggtggctcacgcctgtaataccaggactttgggaggtcgaggtgggcggatcacctgaggtcaggagttcaagaccagcctagtcaacatggtgaaaccccatctctactaaaaatacaaaatttagccaagaatggtggcgtgcacctgtagtcccagctacttgggagggtgaggcgggaaagtcgcttgaacccgggaggtggaggttgcaatgagctgagacagcgccattgcactccagcctgggcgacagagtgagactccatctcaaaaaaaaaaaaaaaagaagaagaaacagggaagcagatttcagtaagggggcaagatagaggggaggggaagaaaagccctactttagatagtctgggaagagctccaggaggaggcgacaactagtggagatctgagtgacaagtaaaagatgcaagggaaaaactctccaggcaaagggaacggatacaaaggctctgaggtggtcaagagtcaagagatggaaggaaggcctgtgtagccaaaagtgaatgaagaagagagtggataaagacaagcagaggtgatagggctgaagagcccagggaatcaaatgttataggaagacaagatttcaatcaaagtgagatgtcaaacccctggagtttttcagtaggtgtgaagccatcttaaggggcagacttaatgaggatcaagtgtcctcattaaggaggacttagagagctagtggatacgatgaaaagggaggtgctctatgagagaaatgcaggtcatcgctaaccaggctagtgtctttaggccactgcaggccaattcaactggaaatcccctcatctgacaaacacataagtgctgctctctgtcaggccccacctccccccattcttttccaagtgtctccgcctgcagcgattaggttagaaagcatttctctctgctctcgcttagacagttcctgcagtgtgtaagactacagagctgaattaggaatgtcaaagaatgttcatacataataaaggagtcacacatattagaaatgacgttgttactaaaaagccacacaatatctcatttagagaatatgcttaacaaaatatacatcttaaaaattcagcactccagaatgctttttcaggtgtttccatttgagaaataaagaataaaaattggtaataattatagacacaacttcatacaataatctggataatatgcaagaagcatcatgttgactttcagatatttctctttgtggctaacgaaccacacatcaaaggatggaccaaagttcagatgtacacagtccagggcacctccgagcacagtggcagtgcccttggggattttctttccctcagtgagagacacgggggatggggaggagcccaggagtgtcaccagaaagtacacaacccagcttcttacccagcctgctgccatcatcaactatcaaaccatttgctcctctttgcaagaggtgctcctttagaaggtcccaataatttctgcttatattgttcgaccagctggttgaagcgggtttccgtcttatttcccttagcttttttcctagatacctgctcggacgataattgctgcttctcctgcttccactggtttatctgtggctttggctttttgggatggacgggcttcactttgcctttgtcccgcaacctgattttggggcctcggtgtgaggggagcgccaggacctttcttctcttctttccatcaggcagctccacctgctccacttcagccttggtctggaacccggtccatgaggtagagcccgcctttctcttctgctctgggggcaccttgctttgttcctctgtgtggtgttgagctgccttctgttgctggtcttttgcaggctctggttgccccttctgaggctcaccagttgcaggcttggatctcattttttgcaagctgcgctggatccttaattccttcattttaagttttcttcgatcttctaaagagaactccactattggtctcttcagaggcccaaagatttctggattgttgttgatgaggcggagggctttcagggcatgctcgtgctcttggaactccgcaaaggcgtagcccagggactgacccttcatgttcccatgaactcctttgaggtctcgcatcactctacactccttgatgcgcacccctttctctccactagtagcactcagcagcagctttctgagctgtttgtcatctacagcctttgggagattgtgcaggcagagcctggttcgggagacaaagatattctggtccttgagtttctgatgcttcagcagctcaaaccgttctcttttggccatatcagcagcactcacaccctctgcagccttcgtcccagcacgaatcaagccttctcgggccagatagagattccgggtgccagtcggcttcttcaccttcgtcgtctgaagctttgcagcctcatcacgggtcaccgccaagtcaaccttgagctgccggccatccagtttaagcccaccagcctcattctctggagaagcagctagaaggcatttctgagctgcttcttgagtcatgaactgggcaaatgcacaacctttagaatgctctgtgtctggatgcaagacaatgcggacatatttgagttctccaaactgttggagaagctccccaagttcttcttcttctgagtcaaaggacagatttctgataaaaacagttttcccttcattcacatcagagggtaatttcctcttctttttgtttgagacttgcacagctttatcctcttgctcctcagtgctggtatcactctgagccagttcctctccatcatcaatactatcgctttcctctaggtcactgtcctcctcagaatgatcactgctttttgcaggggctggtctcttgactgctctcttctgaatttgcacaggcttggtcacctttgattctatattctcttcctcttcatcttcatcatcaaaaaccccatcttcttcatcatcatcatcgtcatcatcatcgttttcttcctcttccatatcctcttcctctctgcccttctttttaactgattcctgatgtttagattcatggctcttttcctcacctatagcagaaacagactgtgtatctttatatttatcctttgccacggcccaatccacagccactgtccggcctttttcagtcaccacgaagcactgcttcaccggccccacctgactgaacagttcctccagctgctcactgcgggccgagggcgggaggcggcccacaaataaggtcaggccggccatgagaccgggaaacccaaagcgcgtgaggacgcgagcaaactaggccggcgcacgcgagccgaaacgctggctttggtaggacaaccaagctcacacgccgagagattccggaagt

SEQ ID NO: 10011 - RNA, 3278 nt, Homo sapiens
  source 1..3278: mol_type = other RNA
cacacacacacacacacgtattccctaagctacccagatctatcacctggttacctcaggccattaccatgacctctatcttaatttcttttaatcctcacaacctctataaagcacttttatttcatttattttacaggtgtggaaattgaggcacagaaaggttaatgattatacccagggccagacactaggtgctagatccaaaatttaagacagggaacattcccaagggtagcagattataccttggcgaaggcttaggcagtgtttcctcaaagatggtccctcaaccactttcatcaaaatcatatagtaattgctaaaatatatattccagcaccttcccagtgctactaaatcaaaatttctgggataacgtctgggaattggcatgttagtaaaattccatcagatgacttttatgcacactgaattgtgagaatctattagaggaatgaaattgtgaaggcccccttttctggaaaggaaggagagagagcagccctctgaaagcacagcaggatggaatccaggctcaggaaccatcctatagtctttttaataggtactccgtgtgcattggagactttcttcctgattaccaacaggcctcaggtggcctcatcccgcccacctgcctccagacatacacctgttcgttggaagagactctaactcactcaagtcactgtggggagcttccagcacattcagatgcctagaataacccagaccaatcaaaccagtgtcttttggtatgaggcccagataattgctattaaaaatatttttcccctgtgattctcatgtggagccggagttgactactactgttcttgagcaacaattcccaaatggaattttaaacaattacttcagaggtaattagcatgctgatattttgcaaaatgtgctttgagaaatggtctaaaagatatgaatgtacaactgggaaaagaatgccaatgaagttaaaaaagttggactatgacccctctaggcaacattaaactaaggctggttttgtggctctggagactgggcagctttggaccataaagagggtgagggatctgtcaaggagccgtcaagttcagccatagtctctctgctcatgcctgatccacctggccagagggccatattttgcaaaagatgagacccagctggctatgtgggcatgctggacacatgcccaccagaacaattgtacattaggtgtacctattgtgtctgaggaaacattgcttacctattgcagcctctgaggcttcattttgagccccattcctgggtcccccaacacacagattcatatctgcagacctctatcgtcacacttttcttatttaattgtcacccttcacttctgtatggaggctcagaagagatgaccccatgtggcttaatcatcagtattttcagagtttggtacagctcctggagtcccttctaaaggacttcctatccttccttcatcactgtaaaaaatagtgggataattcttcaaaatgaaacccctttgtgcctgcttagcagaaaacctgaagtacctatgagagccagagtagatgactgtggctggggagtgacctcacatctctttatcctgttccatacacttgcactgcattccttattctctgtgtttccaaggggtggtgtccctgagggaggcatttcagggcgtggaaatggtactgacctggatgggccctcaaggggtctttctgtactacttcctcattttatggaaataaatatattacttcttaagtttacttcaagtttcatgtcttgtattttatagcagaaacccaggcctagaaaagcctttgtagagccaacacttatgaatgaggccaagagttcatatgagcctacagattacccttcgtatatcaaatgaggcccgactagcccactgactaggtgtccttcctgccatacttgtccctttgctgattggcatcctagaaggagtactgtggcaagggctgtcactacagcctcattactctttgggcctcagctttatttacattttgtagaggactcaaggaattcctatttaggttttatgaatctcagggaggatactactccattaggtacagaagcattataacctcagttgaaattagaagctggactctcataagatgggatagttggcctttattgtatcagcaaaagaatgaaatatttattgaattgtctagaactgctttttgaagcaaaattaacattattagtttatatatttacccgatgcctttaaaatatttctgtctggagcaaataaacttctctatatcattttccagctcagctgtgtactacctagcaagatttagctggtcacactaatttactttaattaaaattcccttggaacaattactcagaagtatgctctctttctaaaacccagttagtcatcactaggatgttctctccctacctgcctgaatctcccttcggctgtcatttatacagacccggtagactgtgaaactttcacaaaatgaaggagcaatctaactaatggagaacatctaaagacctatgtcttctcatctctattaagtcaaattgatactgtaaactgatataatccattgaaagaaatagcaaatttgaattgagtaagaggacatttttagaaatatacatacaaatacgtgtttatcgtagatacaaattgtctcagatgtgtactgcagttattaattgcagcttgagaatttccttttcatcccagcaataatatacagccagtcaacaattagggatgagtaaactctcatagctacatagcaagagtcatgattatttaaaactactaatgattatattgcaattgaaccaaaactgctcaaatttatttacctaaaaatctgtttagttataccttgtgttcctcatactttggaaatgtggcaatccactcttcttatctaaatggggcacagcatttgcctgtaattagtttcctaattggttactcatggggctaggtgtgtggctgactccttattcatcaagtgtcatgttgcttttcatcgaaagtagccacaagggccatttcctctgctaaatggaaattccacctaggcctgtacctgtgcatctaggaaaaaaccaacaattcttttattaaactaaagtataaaaataaataaaaccaatgtgaacattgtttaaatgctacattatccttctttaacactgatttccaactacacgatatggtttggctctgtgtccccacc

SEQ ID NO: 10012 - RNA, 43 nt, Homo sapiens
  source 1..43: mol_type = other RNA
cacacactgcaattacttttgcaccaaaccaacagcatcaatc

SEQ ID NO: 10013 - RNA, 218 nt, Homo sapiens
  source 1..218: mol_type = other RNA
cacacactgcaattacttttgcaccaacctaaaatataataaaaaagtgtcttctctttataacttttctgttgttttgcttaagttatcattgctattcctctgcaacctaaaaagaaatcattgaatatacatttaattttagaataatcactacacaaatgccctaaaagtgtatgtataacatccctgatgtctgcatttgtcctttgactggt

SEQ ID NO: 10014 - RNA, 38 nt, Homo sapiens
  source 1..38: mol_type = other RNA
cacacactgcaattacttttgcaccaacctaatacctt

SEQ ID NO: 10015 - RNA, 1506 nt, Homo sapiens
  source 1..1506: mol_type = other RNA
cacacactgcaattacttttgcaccaacttaaatatataacctctctgagctcccattttctcatctaaaaaatgaaataataccaacctcacagcactgttggaagggttggggtaaagcaccaagtacgtgggtagcttatatcctacagaataattttcaccaacatgacccatgaccatgaagtttatggtttgactatctgtaggaagggtacaaaaatacatcatgcaacaaggtcattcatttggaaatgtaatgctttctgaaaaacttgagcattcacttttcttcacttgcctgttctaataagagaggtttggtgtggtgatttttcaatagaaaggatgttaccaatatataaataacataaaaggatcacatgagaattaaagtgaagtaacttaacatacaattttcattctaatcttatacaataatttttcttgactattgatagatcacaataaaggtatgctgatgatataagttattttaagactttggggaaaaaggcttccgtctctggcattgaccttattgtggaggaccctccaaaatcttcagctctgcaccagcaggtatgctgagtcatgtatgatgacataaaccacaaggagtcaaggagctaaaacaaccacagcgactggctcagatctcagatgtgcaagatgaatcctcaggatttttcacacactgaagaaacttgtcaggtctgtagatattcttgcaggaaaattgaatattccttttgcttataatcgattccagctcttttatggtgggatcctggcataagtctctggaatcttctcttccaccatgtatcacccaggcctctagtgtctgaaccttctctggttgcaaattatggacttccacactcccaaaagtgctgtttttgtcaaagattttactgcgggatccattgagcatcacatggaccacatcacaggcagcttctgcaaacctgcgggaaaccgttttccagaatactgaaacagggttgttgctgcagtcctttctccagtctgggcaagattgatagtttatttcttgttgcaaggtacggtctgagttcccaacttcattagtggctgatagtcttcttcagtaatgttgcaaggatgttttgaaataaatgcacccttgaaagcatcccatacactttggcagtctacatgtctcatctcaggatgaatttcagtgtacttgacgcatcgcgccaggacggtctcgggaaagcgcttggtggtgcccggaccgctccactgctggcgccacctcgggacgaccaccgcgagcaccacgacgaggatcaggaccaggatactgacgccaagacagagttgggctctcctagagagccggcagcagggtttgtccccggacaccgggctgaactcgcagttggccatagggctccaggcggggttggctgggcgaagatgaggccggcaggaggctaggcagcaagagagaggctggctgggttctgaaactgc

SEQ ID NO: 10016 - RNA, 1642 nt, Homo sapiens
  source 1..1642: mol_type = other RNA
cacacactgcaattacttttgcaccaacttaaatatataacctctctgagctcccattttctcatctaaaaaatgaaataataccaacctcacagcactgttggaagggttggggtaaagcaccaagtacgtgggtagcttatatcctacagaataattttcaccaacatgacccatgaccatgaagtttatggtttgactatctgtaggaagggtacaaaaatacatcatgcaacaaggtcattcatttggaaatgtaatgctttctgaaaaacttgagcattcacttttcttcacttgcctgttctaataagagaggtttggtgtggtgatttttcaatagaaaggatgttaccaatatataaataacataaaaggatcacatgagaattaaagtgaagtaacttaacatacaattttcattctaatcttatacaataatttttcttgactattgatagatcacaataaaggtatgctgatgatataagttattttaagactttggggaaaaaggcttccgtctctggcattgaccttattgtggaggaccctccaaaatcttcagctctgcaccagcaggtatgctgagtcatgtatgatgacataaaccacaaggagtcaaggagctaaaacaaccacagcgactggctcagatctcagatgtgcaagatgaatcctcaggatttttcacacactgaagaaacttgtcaggtctgtagatattcttgcaggaaaattgaatattccttttgcttataatcgattccagctcttttatggtgggatcctggcataagtctctggaatcttctcttccaccatgtatcacccaggcctctagtgtctgaaccttctctggttgcaaattatggacttccacactcccaaaagtgctgtttttgtcaaagattttactgcgggatccattgagcatcacatggaccacatcacaggcagcttctgcaaacctgcgggaaaccgttttccagaatactgaaacagggttgttgctgcagtcctttctccagtctgggcaagattgatagtttattttggaagtgttgaattcaccacaccatgtgaggtcatcagcaaggtagcctagcagcgtgtcctccagggtgaacatgtcccgctggacctgtgtgaactgatgggccagatcttttattctgctccaaagaagaatcttgttgcaaggtacggtctgagttcccaacttcattagtggctgatagtcttcttcagtaatgttgcaaggatgttttgaaataaatgcacccttgaaagcatcccatacactttggcagtctacatgtctcatctcaggatgaatttcagtgtacttgacgcatcgcgccaggacggtctcgggaaagcgcttggtggtgcccggaccgctccactgctggcgccacctcgggacgaccaccgcgagcaccacgacgaggatcaggaccaggatactgacgccaagacagagttgggctctcctagagagccggcagcagggtttgtccccggacaccgggctgaactcgcagttggccatagggctccaggcggggttggctgggcgaagatgaggccggcaggaggctaggcagcaagagagaggctggctgggttctgaaactgc

SEQ ID NO: 10017 - RNA, 30 nt, Homo sapiens
  source 1..30: mol_type = other RNA
cacacactgcaattacttttgcactaacct

SEQ ID NO: 10018 - RNA, 37 nt, Homo sapiens
  source 1..37: mol_type = other RNA
cacacactgcaattacttttgcactaatctaataact

SEQ ID NO: 10019 - RNA, 2612 nt, Homo sapiens
  source 1..2612: mol_type = other RNA
cacacactgcaattacttttgcatcaacctaatattattgacattatggtataattatcattttacagaagatgaaagtgaggctcagggtgaagtcacttaagtcccttgactggtacacgccacagccaacatctgaactaatgttctggttctctttcaaccttaccgctctcgtacctccagcgaggcatccttctgcctccaacagataaagtctgtgcaccttaaaatcgccacggcatgtcttcacactttattctttctctgttcttcatgtcaagagaggcagcatggtgcaatgaaaagggtgtcagaacacctagttccgtggtctggggcaaactcctctctctgggcctcagtttcctgttggcctccacgtggtgcagcctgaaggcttctcctgtgctctcattcaccacatcaaattggtgtcgataagccacacagatgagattgtcactctcttcagctggcccatccactaaggtcatcaccatgggagagtcagacagacagatctccctgatgtactggaattcttcaacaggtgactcagacaggggagataacaatgaggtgctggtgaccccgcttggcttgttgtgttttcttgtgatcagaagcagtttattccgaattgcaaccacaatcctcagctctctgctgtggtgagtgttaatagcatacaggtggcagccttttgttttctccaacttgttttctctgcagtcagacctgctcttcccagcctgcttcccctcaaggcccttttgcagagcacttagcctgaagacaaagaggcgagcatcttttcctttgtctgctctgagaaccagaaggtccagggtctcaagcacatgcatttgcttcactggcagagttctgtcaaacacgggcactgatggaaggtcatcatccactagcaagacgccagcatcagtggaaaccagcaaggcctggccccagggatctgcacacacggcttcatgagggaaattactgcagaaacactggggctcccacggctcttttttacagatccctgaagctgccaagcttgatggagcatcccctctcacaatggatttcagttttagtgcctgccctattctaacaaactccgcctggcgggcctcctctttcttccgcgctgacttgggtgactctggtaagacatcactaaaagatcgtctattaagcatgttcttatgcaaatctggcatcaaatcctggtgtaaagatctaatcaacatatccagggtacgccgacgtttctgggcaaatgttggggtttccaaagtggctttttcaccattaattaatttcactagcaaaaagtccctgaattcctggtggtctgtaaacactggtggagttggcaagggagggccaaagagtggtacgctctcttctgaaaatattttcagcctgtaattgtcattttgttgattgtatctcactaaggcaaaaatatgtgtaaagtgggagcggatcatggaaggcttaaaggcaggagaagattcctctccttcttggaacacaatggtgacgatatcgtttccaatgtggcgtttcctttccacctgctgtttgttctctttggaatatggcaacatggtggaaacatgaaacatgatctcatgcccttggtacacagtataaactgaatgtatccctgtggtatcatttttggtatccagaccgccacggtagcccgtccagccctttagagtgattgtgtcacccagaagatttaaaaatttttgaaaaggctcgcttccaatttcattgctgaacatctcatcatcagtgagctgcccatctttggcaaaaagaaccccaaacttgaaattcacagagccctcttgttcttcaagaaccagcaagtccttttgtatttcaggatgaaaaatttccctggggcctttctcaaatttgtccagattcatggcacttaagatggacttcacagaaagagtttttgtgggactgtagggaaggcatattttctgggtacctgtttttctccaaagaattgcacggtattgagggacacgttgattgttttggtcagaaagggtcacggacaagaagaaagggctcttctcggcatcgtttccaatgtagttctgatggacttgtcctaaaaaatatttgaaataccatctggtgtggtattctgggttctctaagtgcacgtctgttcttcgccaagtaccaggcagggcagttgcattctcatctgaagagccattttccactctgaatcttccagccctttggatggctccatcagcatcactggaaataagcagctccacagatccataatgtttcctactgaaatccccacgtctacagcctaggtcttccgagacagagttacaggttgacctgggactctagttcagggtctttcgttggccatgtctgaaggggctggatgccgaaggagagagacgactttgctttccatagaatggtttgtgctatctgactcccacaaggcaccttcgttaacgggtccatcagtgggcctggaggctgggcagctgtccttgggctctcgaagctgcaccccctgcgccgcagcgccgccctcttct

SEQ ID NO: 10020 - RNA, 4025 nt, Homo sapiens
  source 1..4025: mol_type = other RNA
cacacactgcaattacttttgcatcaacttaatagaacatctgtattcccaagatctactgcctgttctttttttgtgaaaaatgctttattgtcctacacagtttttaaagtaatagtttaagtatcaggaatatcaagatattaataatataaagcaacagtttaaaatcaataacaagaaaacatttcttcttctgtgtagctcaaattcatttcatggtggaaaacaactgacagccccagcagtctctatccttgagcctgcagtggccttcaatgaatggtaggtcataacttcacagaatccaagtaggaggctttgtgtattttgttcttagggatgtttgttttcttgtttgtttaaaagaatgaaaacatggcagcgtatctctcaaactgatccctaagtattataatcactgtggaatataacaggctgcaatcactgctgaaggatgtttagtaataaagacagcaaaactgcgagtaaaacctcaagattctagtggtctagcttcccacatactccaaagctcagcaaacttttgcccaagggccaagattggccaaatatttttgttgaataaaagccacgcccatttgttaaagtatcttctatggccgctctctaagatagcagagttgagtggttggaacagagatcacacggcttgcaaagccaaaaatatgtactatatagccccaaactacaaagccctttaaatctctaaaattgtgtaaagactgttggcttattttcagagctctgtcaactctctgtaaacgataataaagttaaaaagagttgctgcataacttcaatgggctaagatatttggagaggggtttgctgggaaaaggagacatctggacatctgcattacagcagctaaggtcatagctgacacctccgctaggtaactcggaggaaggacattgaacttgtggcaactctggaatttagtttaactctttcgtttaaaaatacagaaggggttagcctggatgacctttaagcttttgaaaattcatgatcgtttaaaatgacgtaactaaaaccgtaagcaaattcagaactacatgactgcgcaacatcatcataaacgtcccatagcacctgcctaaggagcaggaaagtaatatatttaagaaaaatgggaactgaactggttacacaagtgtatgtggaagtttcttgtactattgaaacttttcagtaaatctgaaataaagaaaacggtatgaaatagttaaaacaatttaaatgttagcacttaaaaggggaaacttcagtgaaccttcttcaacaagcgaagttaacacagcagcagccataagggatctgtaaaacataaaccacgtcgtgtgctcgctgaatggagcatgcctgaggctgcagacctccctcattccctctcatagtgcatcctaaagttccccgtacaaatgttacctttgagtttatcttacttgacggaaaccaacctaatatctaaagagagcaaagagagttaaaacacaaaagaagccaggagtggagagagggacaggagggacaggggagagggaaaaggagtggtaagagaaggaaaggatggagggggaggaatacaaatagaagagcctcgttaatcaacaaacgagataaacgtggtccaaatgattagaagtataactgtcttttgtgatcttttctttggcagaataggaagctgacttaaccaaaaatacttgactctcacacaatatatgtacatcccatatattttacatatacacatattccaaaaagagaggttatttttataaaatacaaacactaagcaaaaattatgctaactgaaaaagtgcctagagagccacatacatccacgttgttaaatatagaaactaactgtaatgagaatcattatctccagtttccaaggataccaggataagcactactcctaaattgcagttcattcagcaaagggcacagaataatttatattcagggtcatccctagctgagagcagatgtggaaggaggaccagggtaaatcaccttgtttcttctattccatttgctacctgatccagttcccagccctcgacccccacactctggtcccaaccttggccaatgttttatggaagaaatttggaaaatctgcttgtaaatggcaacttccaagagaaaaagaatcttcaaagggcagggcagtctgagatgtgattaatactgggggtagggtgggggctggtatttccatttgctttgtctgtgaaaaggaaaggagtctgggagtctggttttgtgtgtcagtcacactagtcgccatctttcccagtgcctataaggaaatttcaacttcccactcgaccaaggctatgcaaagcttgccactcataaactgccatggtctctagaatcaaattcagcttcaacttgttcttccttcttagactctagaatctagatctttcataacaattactttttgtttctacagcaataaaaatataaaagctactttctgaaaacctaggagatagtgcctctgaatcatttatttgtttattcaagaccacttactgttgttttcaatgtggcaggcattgcgccaggccaggcagacaggcattacgccaggcagacaggcattgcgccaggcaggcagggacaagaagtgatagataaggtatcaataacaggccacgccacttaggcagtttaaaaagaggcattcttcctcttagtcaaatcgtcacttactaaaatactgatgcggattttatggatactctagatttgtcttaaacttacagaaagtacatataaacatacgattcagatataataccaattttccatttagttccttccccatcacctgtctacccaatacaataataagatctgccatatagcacctcagctaggagcagacatccttctaacgggcagaagagctctctctgccttcaaatgcttcctcttaatggacaggagacactgtaccaagataagcgtcttagcttaatgtgataatacaggagaataggctattttgataatgaaggccttctaggatgtcccttctttgcaggttatattaatcgatactggtcactgtttttaagaggacgaaggaatgaaacacaacaaaggttcccaacagttacgtaacatatacagtctatctcaataaggcaagctattttaagattaacagttaatacaaaatttactacacgtcctttcctatatattttagatgacttgacgactgcatacctaaatgcatcctcatgataatgcctgtacagcctcatcttttcccaacaacagactcaaggttttttttttggactattaagcttgtttctaaatcccttcaagtaataacagcaaattttaaaactatatgaaataaaagtctcggttctcttacaacttacatcagtgattattttgatgtattattatgacactttctcacaaggcgcaacattttgaggtaagatggcttcagacaagattttatgtctgaatcttgaggctttgaaaatgctgagcttgtgaaggctcaatataataggccactatttcatcttttccctcgtcccacccaaagctagcacttggtagggcaaaaacagacactttgttaggtggagcaccaaacacagaaagcattcacaagtcactggcagaaaggtcattttctgttttaacatctttttctgataacccagatcagttttcataaaacccctgaaggtagaaaccagcttacattaagcgacatcattgtactccctacttgtgcataataatcaactttttaaaaaattttaatcttcagcattaaaagtatcctacccaccaattcaggaacctcgaactcggactggagccacttcgctctctggatgtaaaaacctcagacgatcacctctttttttctctccctactgttcaaacacctaaattatggtttagtgtgttgcacatgtcctcaaaaatactttctagta

SEQ ID NO: 10021 - RNA, 50 nt, Homo sapiens
  source 1..50: mol_type = other RNA
cacagcaagtgtagacaggcagacacatgacaactctgtccagccaggcc

SEQ ID NO: 10022 - RNA, 2072 nt, Homo sapiens
  source 1..2072: mol_type = other RNA
cacagcaagtgtagacaggcagacacatgacaactctgtccagccaggcccttggttccttcaggtttcctttgctcatagacagatacaatcagcctgttttccagatttggtgattttggagagtaaggggaaagggagaaaaatacacaatataattaaacattaaaacattatggaactaaaaacaagttagacttttgactttattcagaaagtacatttatacatttgttccaaatgtgctaacatggataatttgcgtaacagaaaactcacattaaaattttaaggaaaaaaagagattaaacacaaggtttattcttaagtccaattcatattattactggcccacatgtagtcagagttcagcgtaattgaaccagatgtttttcctctttgcaaaaaactgcatattttaatactgaagttaaagataaaaactatgtttatgcatgtttcttttagtagataagtaccataaccttgtccatgaaaaagaaaattatcatttacatggaaacagcagcccttttcaaaataattaatgagcctaatttatttggcaacccaagttgctgactttggtatttgatgctctgataataggatcctacaagggaatatgtttttaccaattatatgtgaaacaacaggaacctatttaaatgtctcattttccttttaaatgcaaagtttataactgtggatgtgaaatcaaattaaaggcagttgtgagcttaagttatccacctcttaattaactatagggccatgctgtgaatcaaaagggtacaaactggaaggctgttactcacagtgatgctcagaatgtgttttggatatagttagtgcaatatagttacaaaatagtacttaagaaaaggcagaaaaggcaaattcatttcatatccaaaaaattaaaaccagatcctttgaaaatttttcttataatttatatgagctaatagtgttaaatatgcagatataaaatttaattctggtgagttgagagtaattctattttaatatcaattatcaattcacatctttagaagtattaagcaaattcccctccccttttaaaaacaaaaatatccaaatagtcaaaattccagtaagtaggacttcttaaaaaacacagcaccaaaaaaacacagtattgtccaaggattgtataattagacattttctcaaagaactttaagaaaaacaaacagtttgtgatttatctttaattgtaaaattctgagaaaatagcaaatagaaacttaatggaaagcaaaatagttttagatactgagaaaattacaattttctacaaatctggacttttatgcagtgattaggtaaggtaatgttttaacaaaagctaataagtgccattttctgtgtatttatgtaatttcaagaaaacaaatttccgattctgtttcggccatcactttcgagtaaaggaactttttttttttcttgacagaatcaaaaacatgagtaaacttggctgttatttaaataattacaaggttagagtatgccaaaaaccagtgccttaaaatactattgtgttattgttgctgcattcagtgcaacagaaagtaattatagagtgattcacttacaaagagtatattggtggaaattaaaaattactataattctttataacttttcctctctctcccataaataatttgatccagttaactctgctcaattaaaggaatgatgcatgcaacacttattacatccaggggtagttttagttgaagatgctcactgttggttagtttcctctggaatagattccatgatccccgctggtcttcccttcggcagtcttttctcagcagtgtccccgagggcttcttggtccctagtgtgcaaaacttaaaatcctctcccggtcctcaggaaaagcctcccttcctgcaccaggggttgcattcagctttcccccctgaattctgctgcgctgactgagacacactcaagggctgtgatttccagtcttgacgtggcacatttgctgcagactggggaactggcaatgaatttaggaccaggaaaag

SEQ ID NO: 10023 - RNA, 5978 nt, Homo sapiens
  source 1..5978: mol_type = other RNA
cacagcaagtgtagacaggcagacacatgacaactctgtccagccaggcccttggttccttcaggtttcctttgctcatagacagatacaatcagcctgttttccagatttggtgattttggagagtaaggggaaagggagaaaaatacacaatataattaaacattaaaacattatggaactaaaaacaagttagacttttgactttattcagaaagtacatttatacatttgttccaaatgtgctaacatggataatttgcgtaacagaaaactcacattaaaattttaaggaaaaaaagagattaaacacaaggtttattcttaagtccaattcatattattactggcccacatgtagtcagagttcagcgtaattgaaccagatgtttttcctctttgcaaaaaactgcatattttaatactgaagttaaagataaaaactatgtttatgcatgtttcttttagtagataagtaccataaccttgtccatgaaaaagaaaattatcatttacatggaaacagcagcccttttcaaaataattaatgagcctaatttatttggcaacccaagttgctgactttggtatttgatgctctgataataggatcctacaagggaatatgtttttaccaattatatgtgaaacaacaggaacctatttaaatgtctcattttccttttaaatgcaaagtttataactgtggatgtgaaatcaaattaaaggcagttgtgagcttaagttatccacctcttaattaactatagggccatgctgtgaatcaaaagggtacaaactggaaggctgttactcacagtgatgctcagaatgtgttttggatatagttagtgcaatatagttacaaaatagtacttaagaaaaggcagaaaaggcaaattcatttcatatccaaaaaattaaaaccagatcctttgaaaatttttcttataatttatatgagctaatagtgttaaatatgcagatataaaatttaattctggtgagttgagagtaattctattttaatatcaattatcaattcacatctttagaagtattaagcaaattcccctccccttttaaaaacaaaaatatccaaatagtcaaaattccagtaagtaggacttcttaaaaaacacagcaccaaaaaaacacagtattgtccaaggattgtataattagacattttctcaaagaactttaagaaaaacaaacagtttgtgatttatctttaattgtaaaattctgagaaaatagcaaatagaaacttaatggaaagcaaaatagttttagatactgagaaaattacaattttctacaaatctggacttttatgcagtgattaggtaaggtaatgttttaacaaaagctaataagtgccattttctgtgtatttatgtaatttcaagaaaacaaatttccgattctgtttcggccatcactttcgagtaaaggaactttttttttttcttgacagaatcaaaaacatgagtaaacttggctgttatttaaataattacaaggttagagtatgccaaaaaccagtgccttaaaatactattgtgttattgttgctgcattcagtgcaacagaaagtaattatagagtgattcacttacaaagagtatattggtggaaattaaaaattactataattctttataacttttcctctctctcccataaataatttgatccagttaactctgctcaattaaaggaatgatgcatgcaacctgaaaaaataaaaagaaatatttgtgagtttgtatgttatgctttaatataaaacagttttattaaggcaagatataaaaattttttgagccagaaaaaccacaacagtttttcaggggaaaaaaaaaatcttgctgaaaacaattgttctattcataaggcttttggacaatttatgtttctgatagatttttaaaacacacttacagtaactatgtgacatatgcacacttcattgttatgttgaacctgcccctaaacttgttaaaaagatgaaagactgaaaaccatattgacctttttttaatctcccaaattataggttgaatattagtttattattacttaaaatactagctaaaacataaaagagctatttgtattattatcataccatgtaatttttagtgtggttattacaccttgttttctttttgtcttttatttcttaaggaaaaaaatgtaagaaaagaattgtcttctaagtcttctgtagtgaaattaaaccaaagcaactccaggaaactggctgtcacgctaagtcaaaaaattcaaaatgaagatttaattatttttcctaatttacttcgttatctctaactattaaaactgataaaaattatttgtaagagacctttgaaaatgagtaaatatttatttctacttaatttacagaacatgaaagtaagaagggatttgaagtaagaaagtttctatcttaactcaggaatttcctgtctcaggttaaagcctgaccttctagttattttaagccaggatttctgagtgatggtctcttagttattattttgacgttattgtgatgggtgggctattctccttagagcagagtaaagtgcattgtttataaagagcagatcccttacagagtaagtgaaagctttggcgtctctttaccgagcatggatgcttgtggatgagtgaattttttcacattaccaagttgtactttttatatcttataacagcttaagacttcaaccaaaaaagtggggagaattctttcgttaggatttttatgcctaaactgtttcccacagagtgaaatacatgggtggtctgtaggcgagaggtgggggtagatagtatattttggtcttttacaaacataaacatattatctgggccgaaagcccgaatgccaagcaggaaggatattaagcctattgactaactacaggaaagtgatcagtgtgaaactttgtcctatagtaaacagtctttctttgattttgagatctgtggcctaaaagaaaaatgagtttgaaaatttaagtccaccgttttagattgatccttttccagttaagaaattgtggtgttgaagctaaggctctgaacttcctttctcttagatggtggaaaagtccttttaacccagtacctagtccaatttatcaatcattcacatgctaaaatgaaaaataattatgaaatttctatgaagtgtagtttggacagaccctgaaacaattttctcttcatgaccacatataatgtttaattttaatacttacacttattacatccaggggtagttttagttgaagatgctcactgttggttagtttcctctggaatagattccatgatccctaaaatatttgtatatctccttataaagtaatatgaaaataaaattaaacatttttctaatttacctggatatagatatggctataatgtatataaatgtgggcgtgtgtaccagcgcataaactacaatcctgccttcattcagcagagctttataaaatgagcttttacctttgatctttaatttagcccatataattgaaaaataagtactattcgttttcatttgttaaaactttgcctcgaaaataagtcgctagagccacatcaagcatgtgcaggaactccttggttatccttttacaaagtaattcttatatttctactcctgtacttatgccagaggcacccttatgtcccttctatctccagactaaaagtcatcctgagggagaaaataggtgagggacccatagggattcatttctttgaaacaaaaagaccgtttaacatgaagaaagaaattgaaattaaatatacattaaatgaaagcaaattttgaaatgtaatcatttctagagtaaaaaaaaaaaaaaaacccagaaaatttgagaaaaacattaccaaagtaccttgttagctatttttcctcttcagtaattgtatcaattagaaaaaatatatttcttgaaaaaatgagctcctctaagttactttttttagttttcttatgtaaaagaaactatatagatttttaacatctcatttgttctactaaaaataattaatatggaactctccaagtcacaatagaaaatgaaaggataactttactatatcatctaagtgaaagtagctaaatttctccttgctgtttatattttaactaataatcatgaatatatgagaatacttaatgttttctttatacacattttggggtgatcagaagggtaatttttaaagtaagttgttttgacaaaagaaaacttagggaatcttttataataaaatattttgctaaagagaacttgagtcaatttttgaattgttgcaaaatgtataacttagaaaagaatttgttcaggaaccactgtaactttaaaggaggacaaaagagattatgtttatttttcacaaaccctgtagaagagatgttttcattatatagaattgtttcggaatagaaattaatgggggttaagaaaattagggatgaggcaataacatttttccagaactttctttaaggggccgacctctaaagttcagcacagatcacattgcaatccagacttgctctattattttctctattaggatttcattcagcttgagggttttcttccctcccaccttcctccccctctcccaccctctttcacctccaggacagctggaaactgaccaaagaaaacttctgccttcgtttacaaattccttttttatcagtgggtttctagacaaagtgccttattttaaatgctcagagaagtggaagcattgtaagctataggcaagagggctcagctgagcagcaattattaaccactctttgatttaaaaaaaatgtaaaacagatatttacaggggtatctaaagatagaggtttttattccctgatttactcagttgctgactcaataagttgtgggtcggtgctcttctctgggcaaatcccatctgcattgtctggtaggcaagacttggcaggttcttcttttattgttaggtactattattcctgttgtttatattacagaaggaaatcttcagaaaagcactatccatatagcatttaaaaaccagcaagtattctttactttggggaaaaatgacttcagtcctgggatgttaaaagttatacatacagccttcatccatataagtttttaaatctttgaattattattaaacaattcaaaagtagcctcattaaactattcttaagtgtctggaatgagttttttcatatttcattttgaagtgggaaaacctttaagaaaacacttgaattatcaatcttcagaaataaaaaaaaaaaaaacagtaaatcgctatataccacacacttttgctcttttaaaattaaatacatctctacccatcacacatgtacctctgtttcccttgcatgttaacacaaatcatgggctccccacctaggttcccttggtcacagaccaggtgagcagtcaagaaggccttacccgctggtcttcccttcggcagtcttttctcagcagtgtccccgagggcttcttggtccctagtgtgcaaaacctgtgaagaaaaacactggatatgagattcaaaaaaggagcaaacaaatgtcttctccttggaaacagcccattttgtccccagcggtccatggcgttgctctcccttgcccagtctaaccaatgtgcagactactgtacaacggcattgtcctgaacaggtagtctgaacactggggcgacggagcaggatctccagaagcttccttctatgtacttaaaatcctctcccggtcctcaggaaaagcctcccttcctgcaccaggggttgcattcagctttcccccctgaattctgctgcgctgactgagacacactcaagggctgtgatttccagtcttgacgtggcacatttgctgcagactggggaactggcaatgaatttaggaccaggaaaag

SEQ ID NO: 10024 - RNA, 2658 nt, Homo sapiens
  source 1..2658: mol_type = other RNA
cacaggactgactcctcaccccagtgcctgtctggagctcacccaaggtcaccaaacaacttggttgtgaaccaactgccttaaccttctgggggagggggattagctagactaggagaccagaagtgaatgggaaagggtgaggacttcacaatgttggcctgtcagagcttgattagaagccaagacagtggcagcaaaggaagacttggcccaggaaaaacctgtgggttgtgctaatttctgtccagaaaatagggtggacagaagcttgtggggtacatggaggaattgggacctggttatgttgttattctcggactgtgaattttggtgatgtaaaacagaatattctgtaaacctaatgtctgtataaataatgagcgttaacacagtaaaatattcaataagaagtcaaactactagggttacttttttttcctcaatcagagtctcattttatccatttggagtagagtggctaaaacaatactgaggcttctggaggctttcggtaagcaaggcatctggttggacagtgggtgagcaccaggctttaaatctgcatacatgagccttaaggaaatggactagaggctgagccaaaccaaagcagaatggccttagagcaacagcaggttcctaggtggtttttatattgtatttgaaaacagccctgggcagggatatcataatttcaaggccaaactaaacatcatcttccctacaatctgcatcccccaaaggaattgcaagatgagggggaacagactgtttctgcataatatacatagtttcatttacgaacattggaatacagactttctatacacacattacctatataataaaaatgtacatggcatgagtatatgtcactgtataaatatagagttttagaaatcttgaacccgcgcttcctgttcacatcagtttctcttcttcttcctccccagtcaggtccgtcatttaagagttggacaaaagggacaagtgtcatttgtgttggtctgggcccagaatttgatacactccttgtgcaatacatgggtacacgccattggatgcagctcactgggctggacgagtttctggcacattagacatagcttacaggtggctggagcatgtgaagaccttccaggatatgaaacttgggcagaaggcaagaacattggggtactgatttgggccagtggagcagggaacaaggcccggatgcgaccaagtggctgagtacttgctgccacccgctcatgttctgccagtcgtgcagcaaccaactggataagttcctccatggtcaggcctgccatggtggtacgtgctgtcttgatctgctgaagaatgttggtcatctgggccttattgcactgtgggaaccgggtcagcagcttctccaggatcttctccagtttgtctactggttggggccggggagtttcagcagaagccttaacaccgcccaagcctgggggaggtgggatggaggcggcagggggcatgtgtggaccgtgggggctgacaagggaacccaagccagggctatttctgccatgggagccaggaaggggtgaggaaggctggctgggctgggaaagggcagggttcaggattgggaaagacaaggagcggggatctgcactgggcataaccatgggcattgtgacctgcccaatggagaagggcatccgaggagccagagagggactgggttgaaacacctgaagcatgaagtctgtctctgatgggggtggaggtaaagtgggagtagggatttgaggaaggctgctcagcttggctccgttcctcactaactggatatgactattaaattggtcacgaacattctttttcattatccgaactccattcagtctcgtctcccactcctgtttggaacgaactgtctccagtgttgggggagttgacttgaggtaagtaaggtgcaattctgcctctttttctgcttcttctagtttcagtaccagtaactctttccggctctctagtgataagatctctgccttccaggcccgttcagtctcttccataatgttcctatttatttcgccatcctgattcttgagtctatccagttccatttcccacacctctcttctgcccttctcacaaagcttctcaatttcagctttcagatcctgctccttctgcaaaaactccttcttctctttctctatcttcttctttgtttcttcccgctttattgtcacatcctgaatagcctttaatatctcctggtgattcttcatttcctcttctctcctttgctgaagctgctttaattgcacttggagctgattctccacttgcctctgtttgtccaggacctcctggtaacgctctttcaacagggttctctctgtcatcattttatccaaattcttttcaatatcttgatctgtgtttacctctgaatcagctgtcttaaagtcagtactcaacagaggcgagttcttctgcttctgtgcagagtctttggtgcttagaccatctgggagaccttcgtctgatttggaagcacataaactagaagattccggaggactgggggcattggccacaacaccagcaacctcagacgctgccattatgctctcccgcgccgcgcccccgggaggaaagtgggggagggac

SEQ ID NO: 10025 - RNA, 3123 nt, Homo sapiens
  source 1..3123: mol_type = other RNA
cacaggactgactcctcaccccagtgcctgtctggagctcacccaaggtcaccaaacaacttggttgtgaaccaactgccttaaccttctgggggagggggattagctagactaggagaccagaagtgaatgggaaagggtgaggacttcacaatgttggcctgtcagagcttgattagaagccaagacagtggcagcaaaggaagacttggcccaggaaaaacctgtgggttgtgctaatttctgtccagaaaatagggtggacagaagcttgtggggtacatggaggaattgggacctggttatgttgttattctcggactgtgaattttggtgatgtaaaacagaatattctgtaaacctaatgtctgtataaataatgagcgttaacacagtaaaatattcaataagaagtcaaactactagggttacttttttttcctcaatcagagtctcattttatccatttggagtagagtggctaaaacaatactgaggcttctggaggctttcggtaagcaaggcatctggttggacagtgggtgagcaccaggctttaaatctgcatacatgagccttaaggaaatggactagaggctgagccaaaccaaagcagaatggccttagagcaacagcaggttcctaggtggtttttatattgtatttgaaaacagccctgggcagggatatcataatttcaaggccaaactaaacatcatcttccctacaatctgcatcccccaaaggaattgcaagatgagggggaacagactgtttctgcataatatacatagtttcatttacgaacattggaatacagactttctatacacacattacctatataataaaaatgtacatggcatgagtatatgtcactgtataaatatagagttttagaaatcttgaacccgcgcttcctgttcacatcagtttctcttcttcttcctccccagtcaggtccgtcatttaagagttggacaaaagggacaagtgtcatttgtgttggtctgggcccagaatttgatacactccttgtgcaatacatgggtacacgccattggatgcagctcactgggctggacgagtttctggcacattagacatagcttacaggtggctggagcatgtgaagaccttccaggatatgaaacttgggcagaaggcaagaacattggggtactgatttgggccagtggagcagggaacaaggcccggatgcgaccaagtggctgagtacttgctgccacccgctcatgttctgccagtcgtgcagcaaccaactggataagttcctccatggtcaggcctgccatggtggtacgtgctgtcttgatctgctgaagaatgttggtcatctgggccttattgcactgtgggaaccgggtcagcagcttctccaggatcttctccagtttgtctactggttggggccggggagtttcagcagaagccttaacaccgcccaagcctgggggaggtgggatggaggcggcagggggcatgtgtggaccgtgggggctgacaagggaacccaagccagggctatttctgccatgggagccaggaaggggtgaggaaggctggctgggctgggaaagggcagggttcaggattgggaaagacaaggagcggggatctgcactgggcataaccatgggcattgtgacctgcccaatggagaagggcatccgaggagccagagagggactgggttgaaacacctgaagcatgaagtctgtctctgatgggggtggaggtaaagtgggagtagggatttgaggaaggctgctcagcttggctccgttcctcactaactggatatgactattaaattggtcacgaacattctttttcattatccgaactccattcagtctcgtctcccactcctgtttggaacgaactgtctccagtgttgggggagttgacttgaggtaagtaaggtgcaattctgcctctttttctgcttcttctagtttcagtaccagtaactctttccggctctctagtgataagatctctgccttccaggcccgttcagtctcttccataatgttcctatttatttcgccatcctgattcttgagtctatccagttccatttcccacacctctcttctgcccttctcacaaagcttctcaatttcagctttcagatcctgctccttctgcaaaaactccttcttctctttctctatcttcttctttgtttcttcccgctttattgtcacatcctgaatagcctttaatatctcctggtgattcttcatttcctcttctctcctttgctgaagctgctttaattgcacttggagctgattctccacttgcctctgtttgtccaggacctcctggtaacgctctttcaacagggttctctctgtcatcattttatccaaattcttttcaatatcttgatctgtgtttacctctgaatcagctgtcttaaagtcagtctgtacagcaatgttctgagaaagcttcagggaagagctatcttgatcatcatcctgatccactcggactccttcaaccccatttgctggagacactacaggtcggaaatccaagcttgtgtccctgttaccttcctttaggatggaggtttgtggggatttctcttcagagcaattcctggaggcaagctgcttagtatggcaccctgccttaagagaccgagtgactggatggaggctctcccgaaggcttgtgtccccctcctctcctgctgtgctggccacatccttcaaatcagactgagacccactgccagaaagacaaagggctgtggctatcaagttttctcctaaaaccacctggtgcgctgctgaggtgtcacctgctgatgaaccaggattctgctctgagtgctccaaatggacatttctgttattctccttggttattgtttggctacttacactcaacagaggcgagttcttctgcttctgtgcagagtctttggtgcttagaccatctgggagaccttcgtctgatttggaagcacataaactagaagattccggaggactgggggcattggccacaacaccagcaacctcagacgctgccattatgctctcccgcgccgcgcccccgggaggaaagtgggggagggac

SEQ ID NO: 10026 - RNA, 3139 nt, Homo sapiens
  source 1..3139: mol_type = other RNA
cacaggactgactcctcaccccagtgcctgtctggagctcacccaaggtcaccaaacaacttggttgtgaaccaactgccttaaccttctgggggagggggattagctagactaggagaccagaagtgaatgggaaagggtgaggacttcacaatgttggcctgtcagagcttgattagaagccaagacagtggcagcaaaggaagacttggcccaggaaaaacctgtgggttgtgctaatttctgtccagaaaatagggtggacagaagcttgtggggtacatggaggaattgggacctggttatgttgttattctcggactgtgaattttggtgatgtaaaacagaatattctgtaaacctaatgtctgtataaataatgagcgttaacacagtaaaatattcaataagaagtcaaactactagggttacttttttttcctcaatcagagtctcattttatccatttggagtagagtggctaaaacaatactgaggcttctggaggctttcggtaagcaaggcatctggttggacagtgggtgagcaccaggctttaaatctgcatacatgagccttaaggaaatggactagaggctgagccaaaccaaagcagaatggccttagagcaacagcaggttcctaggtggtttttatattgtatttgaaaacagccctgggcagggatatcataatttcaaggccaaactaaacatcatcttccctacaatctgcatcccccaaaggaattgcaagatgagggggaacagactgtttctgcataatatacatagtttcatttacgaacattggaatacagactttctatacacacattacctatataataaaaatgtacatggcatgagtatatgtcactgtataaatatagagttttagaaatcttgaacccgcgcttcctgttcacatcagtttctcttcttcttcctccccagtcaggtccgtcatttaagagttggacaaaagggacaagtgtcatttgtgttggtctgggcccagaatttgatacactccttgtgcaatacatgggtacacgccattggatgcagctcactgggctggacgagtttctggcacattagacatagcttacaggtggctggagcatgtgaagaccttccaggatatgaaacttgggcagaaggcaagaacattggggtactgatttgggccagtggagcagggaacaaggcccggatgcgaccaagtggctgagtacttgctgccacccgctcatgttctgccagtcgtgcagcaaccaactggataagttcctccatggtcaggcctgccatggtggtacgtgctgtcttgatctgctgaagaatgttggtcatctgggccttattgcactgtgggaaccgggtcagcagcttctccaggatcttctccagtttgtctactggttggggccggggagtttcagcagaagccttaacaccgcccaagcctgggggaggtgggatggaggcggcagggggcatgtgtggaccgtgggggctgacaagggaacccaagccagggctatttctgccatgggagccaggaaggggtgaggaaggctggctgggctgggaaagggcagggttcaggattgggaaagacaaggagcggggatctgcactgggcataaccatgggcattgtgacctgcccaatggagaagggcatccgaggagccagagagggactgggttgaaacacctgaagcatgaagtctgtctctgatgggggtggaggtaaagtgggagtagggatttgaggaaggctgctcagcttggctccgttcctcactaactggatatgactattaaattggtcacgaacattctttttcattatccgaactccattcagtctcgtctcccactcctgtttggaacgaactgtctccagtgttgggggagttgacttgaggtaagtaaggtgcaattctgcctctttttctgcttcttctagtttcagtaccagtaactctttccggctctctagtgataagatctctgccttccaggcccgttcagtctcttccataatgttcctatttatttcgccatcctgattcttgagtctatccagttccatttcccacacctctcttctgcccttctcacaaagcttctcaatttcagctttcagatcctgctccttctgcaaaaactccttcttctctttctctatcttcttctttgtttcttcccgctttattgtcacatcctgaatagcctttaatatctcctggtgattcttcatttcctcttctctcctttgctgaagctgctttaattgcacttggagctgattctccacttgcctctgtttgtccaggacctcctggtaacgctctttcaacagggttctctctgtcatcattttatccaaattcttttcaatatcttgatctgtgtttacctctgaatcagctgtcttaaagtcagtctgtacagcaatgttctgagaaagcttcagggaagagctatcttgatcatcatcctgatccactcggactccttcaaccccatttgctggagacactacaggtcggaaatccaagcttgtgtccctgttaccttcctttaggatggaggtttgtggggatttctcttcagagcaattcctggaggcaagctgcttagtatggcaccctgccttaagagaccgagtgactggatggaggctctcccgaaggcttgtgtccccctcctctcctgctgtgctggccacatccttcaaatcagactgagacccactgccagaaagacaaagggctgtggctatcaagttttctcctaaaaccacctggtgcgctgctgaggtgtcacctgctgatgaaccaggattctgctctgagtgctccaaatggacatttctgttattctccttggttattgtttggctacttacactcaacagaggcgagttcttctgcttctgtgcagagtctttggtgcttagaccatctgggagaccttcgtctgatttggaagcacataaactagaagattccggaggactgggggcattggccacaacaccagcaacctcagacgctgccattatgctctgagcgggcggagcggggggagggggcggccgagccacggggggaggggtcgagc

SEQ ID NO: 10027 - RNA, 3655 nt, Homo sapiens
  source 1..3655: mol_type = other RNA
cacaggactgactcctcaccccagtgtcttctcccattcccagtcgcttgctgcgcccctcccctcactctctcctaactctgctctccccctccaacgctgggcttggtttgcatctttgaggaactccctcctaccccaactccctcccacggggctcccgcatcctcccgcatttaactcggaccctctgtcccgcagcgcccctaccccaggccgactggactgtccgggaaggcgccggcggggaaggggagcccagcgctgggaccagagcactgcggggaggctttgcccgggaggagtaagtggaggagtgaagtcgggacttggtaagttccaggtggcaggaacccactaggtcccaacatctgattccggctagggtccagagtggggagacaggcaggggacttctagggtctttcttggaaaccctaactctcaggtccaagtcctgtggaaatgaacacaaggttggcaaacacatggcgctcaagcgaccctctcccctccgccgaggcccgaggcggcttcccctggcatcctgcagggcaccgccccttccctgcaggtccaggccgccaggagggggcgctggacgaagccggtctgcaccagcaactagtgctgagggagctgtccaggccccagggcagggaggctccccgggagagatggctctgccgccagacccacaggggaatgacgggtgttcaaaaaataccaggagtctccctcacctgctccctgccaaggggaagggagacgcccccacagtgggtggaggggggagaaacttctcacctgtcccccaacacacacacacacacacacgctcacacgcgcacacacacgcacacacatttcacccacatacacatacactcatgcctcggctccaagcactgcccataggtgcagaccctgggcatatcgcaaggcgagaggtgggccaggaggaggaagaggctgggacagggtaacaaggcttaggaagggggacaggggtaccctgttcagagatgacctgcaagttcaagttatgcagaaaagtatcaaagagacaagacagtctctgcccttggtagacgcctggggtatggagggcatgaaaaggggcagaaggggtaatgcatcccccaactccccacctctggggtcccctccacacccccaaccctgacaacagggccaagaagtctgtgctgtacaaaacaggccagggtcaagggtccagtcattggtgagacatcccagcagagaggaggcctgggcaaaagaggccaaggtcaagggctcagtcatcagtgagatgttccagcagagaggaagaggaggccaggccagcccgggctgagcagcttctaagctccaactgccgaggccacgtaccccctcccgctacctccagagcctgaaagtcttttctgactctgggctgatcagggccccggtctgcagctgacagcagggccctgtgcatccctcggtgcagctctccctcagggtgagctgggagcaggccggaatggagcagaggaggtcccaggggagactggtggcacctggagctttgtggcagatgtggtggaaccaacatcagccaaaaaagaaaaaaaaaaaaagtaggaaagagtccagcccaccctggagcagtatctagaataaatttcttgaagaggcagggaccagaagaggtgcggatacagccaggcggcagccctccagactgagggggcctggggagctggaactacagctccgctctccctggggatctgcagggacctccaggccagtctagagaggagaggagaagcccaagggcctacgcagatgcaggctcccttaggtcaaattgagggaggagcaagaattagaccctcccaaggtttggagggcctctcctctcccccaggccacatccaggctttcctctcctcaaagcctggagcttgcagggtagtcggtgagaagtaagtctgagatcagggtcttccctcagagcttgaatggagtgacgagagggcagaaggcaggacaagctgaggtcaggccaattactgggctgtgatcctggcctttcagggtccctgtgagtgagccacggggcagggaaggactccccatccagagacatcacccccgggccgcaacacggagcttactgtagagcccacaaaatctttgttctccggcttgagctcctcctgcagcaggtctgtttgccggttgcccagcacgaaggcgaggaaggagaggatgagggcgttgaggatgccgatgatggccaggatgtatgcccagcgcactgaacagtcccccagggagtacttccccgtcttggccccacacatgtcccggatggtctcggcatcccagccatcaggaaagatcatgcagcccaggacgaggcacagagctgccaagagctgcatccaggcgcagatcttgtagaccgtagccgtgttgcagaagaagaaaagcgaaaagcaggtgatgcagccgaggatcagcaccatggagagcagcacgaagaaggcggccgccttgaaggcgctggacgggatggtgctgaagtcggtgaaggagccccggcaggtgagctcgcggcccgccagcccgctgcccacgcagtagtggaagaggccgaagtagccaggcttgggggtgctcacgctgtcgcccacccagtagggctggatgaagaccaccacgttgatgatggcgaagcagatggtgaagatggcccacagcacgccgatggcccgcgagttccgcatgtagtgctcgtggtagagcttggaggcctcctgcgagggcagcatggtgcccggaggcggggccggcggcggcggcggctggcgggggccgccggcccgggacggagcgccgggctgccgggcgggagctggggacgcacgcgagaagcggccctgagtcaaggaacccgcgagggcggggcctggggcagagctgggggcgtctgggagctgctaagggagagaggaaggggtcatgagagtgttgaggccgtgtctagggggactggcaaaggtctcctactggggggcctaggagggggccatgagaaagttggggggcgcctaggatggggatatgagacctggaagtgcggggggaggtgcttgaaagtggccatgggggagttggggagggggtttgagagctggtattacgggagtaggaggggacaaggggaggtggaatggaggctggagactggtgttggaggactagcagaggggctgaatttagggagctcagaagggaatttggggactggtattaaggggtagaaggaggtctggtattgggtgtctagcaagggactatgaggcggtggtgggcgcttctaggatgggggaagagggaatttaagaggctgggactgggtggttgggaaggtaatatgggggctgggacggggaatgggggctggtatgagggtctaagagggcaaagtggcagaattaggatacagctagagcgggatcgggggctgggactgctggacacggggcgaggaagggggggctgtcctcagaagccagggctggaggtaggctggagggagcctaggattggcgggccagggttggagagagggggtttccaggccaaaggaacg

SEQ ID NO: 10028 - RNA, 3137 nt, Homo sapiens
  source 1..3137: mol_type = other RNA
cacaggactgactcctcaccccagtgtcttctcccattcccagtcgcttgctgcgcccctcccctcactctctcctaactctgctctccccctccaacgctgggcttggtttgcatctttgaggaactccctcctaccccaactccctcccacggggctcccgcatcctcccgcatttaactcggaccctctgtcccgcagcgcccctaccccaggccgactggactgtccgggaaggcgccggcggggaaggggagcccagcgctgggaccagagcactgcggggaggctttgcccgggaggagtaagtggaggagtgaagtcgggacttggtaagttccaggtggcaggaacccactaggtcccaacatctgattccggctagggtccagagtggggagacaggcaggggacttctagggtctttcttggaaaccctaactctcaggtccaagtcctgtggaaatgaacacaaggttggcaaacacatggcgctcaagcgaccctctcccctccgccgaggcccgaggcggcttcccctggcatcctgcagggcaccgccccttccctgcaggtccaggccgccaggagggggcgctggacgaagccggtctgcaccagcaactagtgctgagggagctgtccaggccccagggcagggaggctccccgggagagatggctctgccgccagacccacaggggaatgacgggtgttcaaaaaataccaggagtctccctcacctgctccctgccaaggggaagggagacgcccccacagtgggtggaggggggagaaacttctcacctgtcccccaacacacacacacacacacacgctcacacgcgcacacacacgcacacacatttcacccacatacacatacactcatgcctcggctccaagcactgcccataggtgcagaccctgggcatatcgcaaggcgagaggtgggccaggaggaggaagaggctgggacagggtaacaaggcttaggaagggggacaggggtaccctgttcagagatgacctgcaagttcaagttatgcagaaaagtatcaaagagacaagacagtctctgcccttggtagacgcctggggtatggagggcatgaaaaggggcagaaggggtaatgcatcccccaactccccacctctggggtcccctccacacccccaaccctgacaacagggccaagaagtctgtgctgtacaaaacaggccagggtcaagggtccagtcattggtgagacatcccagcagagaggaggcctgggcaaaagaggccaaggtcaagggctcagtcatcagtgagatgttccagcagagaggaagaggaggccaggccagcccgggctgagcagcttctaagctccaactgccgaggccacgtaccccctcccgctacctccagagcctgaaagtcttttctgactctgggctgatcagggccccggtctgcagctgacagcagggccctgtgcatccctcggtgcagctctccctcagggtgagctgggagcaggccggaatggagcagaggaggtcccaggggagactggtggcacctggagctttgtggcagatgtggtggaaccaacatcagccaaaaaagaaaaaaaaaaaaagtaggaaagagtccagcccaccctggagcagtatctagaataaatttcttgaagaggcagggaccagaagaggtgcggatacagccaggcggcagccctccagactgagggggcctggggagctggaactacagctccgctctccctggggatctgcagggacctccaggccagtctagagaggagaggagaagcccaagggcctacgcagatgcaggctcccttaggtcaaattgagggaggagcaagaattagaccctcccaaggtttggagggcctctcctctcccccaggccacatccaggctttcctctcctcaaagcctggagcttgcagggtagtcggtgagaagtaagtctgagatcagggtcttccctcagagcttgaatggagtgacgagagggcagaaggcaggacaagctgaggtcaggccaattactgggctgtgatcctggcctttcagggtccctgtgagtgagccacggggcagggaaggactccccatccagagacatcacccccgggccgcaacacggagcttactgtagagcccacaaaatctttgttctccggcttgagctcctcctgcagcaggtctgtttgccggttgcccagcacgaaggcgaggaaggagaggatgagggcgttgaggatgccgatgatggccaggatgtatgcccagcgcactgaacagtcccccagggagtacttccccgtcttggccccacacatgtcccggatggtctcggcatcccagccatcaggaaagatcatgcagcccaggacgaggcacagagctgccaagagctgcatccaggcgcagatcttgtagaccgtagccgtgttgcagaagaagaaaagcgaaaagcaggtgatgcagccgaggatcagcaccatggagagcagcacgaagaaggcggccgccttgaaggcgctggacgggatggtgctgaagtcggtgaaggagccccggcaggtgagctcgcggcccgccagcccgctgcccacgcagtagtggaagaggccgaagtagccaggcttgggggtgctcacgctgtcgcccacccagtagggctggatgaagaccaccacgttgatgatggcgaagcagatggtgaagatggcccacagcacgccgatggcccgcgagttccgcatgtagtgctcgtggtagagcttggaggcctcctgcgagggcagcatggtgcccggaggcggggccggcggcggcggcggctggcgggggccgccggcccgggacggagcgccgggctgccgggcgggagctggggacgcacgcgagaagcggccctgagtcaaggaacccgcgagggcggggcctggggcagagctgggggcgtctgggagctgctgggcacggccggaggcagcggatccgggactggcacggcctaggcgccgcggctcggcgctcccagcagcggctgcctcggcccaggcggcggcctctgcgcggcctccatcttgctcgggttctccccggggcgc

SEQ ID NO: 10029 - RNA, 1270 nt, Homo sapiens
  source 1..1270: mol_type = other RNA
cacaggactgactcctcaccccagtgtggtcatggtgacaatggtgtaccaaaacgaggcagggatgcttgtgaacttgctggccgaggagcccttctcggcataaaacatcacagtggcaaagatgatgatggccatggtgagggagaagagaagaaagcccagttcggaggcacagctcttcagtgtgtagcccaggatccgcaggccctgggagtggcgggaaaacttgaagatcctgaagacgcggaagacccggagcgtgacgaaggcgccggacacgtcctcgttgttggtcatgaccagaccgatgtagtagggcatgatggccaccacgtcgatgatgctcatgacgctgcggatgaagcggtagcggctgggagccgcgaagagccgcaggaggtactccacggtgaagatcatgacgcacgccgtgtccaggcagaagaaggccaccgagtagcgctccccgcacggcagctccttgctgcccgggaccgtgccgcacggcaccgtctccaccacgttggtgatgaccgagacagcgatgaagaagccagtcacgtagtagaagaccagggccagcgtgctggtgtgggggttctcgaaggcccgccacatggtctggcggaagctgagcgagggcatggactcctggttgttctccgagtcgttgtcgtccatgagccgctcggcgttctccctcttgcggtccttgtactcctcgtagcagcagtccccgatgatctccgggaggatgccgtagaaggccagctcgtcgtcgtaggcagagatgcactcgtagcgcgggtagtgcagcttccccgtgcggtagaagttgagcacgcagcggaacacctcggggtcccggtcgaagaagtactccttggtgtcctcgttgaagaagaactccttctccgtgctgcccagcagggtgtccgggtagcgctccagcgtggtcctccaggtctggaacctccgcccactcacgttgaggacaatcagctcatcctgccgcttgttcttgtcggccggggccaggggcatggggcagttggccaccggcatccacccgatggccgcagcccgggcaaaaggcagccaggccgcaactccggccgccatggtgactccagctcttgggccggcagccgcgcggacgctaggcacaccagcttggagttagttcagcaaacccttccgcgaagccagcccgggccccgcgcccggcgccccgcgcgcgcgaggaagctgcggccgggagccgggg

SEQ ID NO: 10030 - RNA, 38 nt, Homo sapiens
  source 1..38: mol_type = other RNA
cacaggcttagaaaagacagtccttaagtttacactta

SEQ ID NO: 10031 - RNA, 86 nt, Homo sapiens
  source 1..86: mol_type = other RNA
caccagggcagagcagggctgagtggctgtaaacactcagctccctcagaaaacagcctcccacagggaacttcagccccaaatgc

SEQ ID NO: 10032 - RNA, 68 nt, Homo sapiens
  source 1..68: mol_type = other RNA
cacccagatctgcggcctaatcacaggccacatttctgaataggccacggatctgggcaaaatgtcct

SEQ ID NO: 10033 - RNA, 1266 nt, Homo sapiens
  source 1..1266: mol_type = other RNA
cacccggctgtgtgcacatgtgcaaaaactgaaaaccatgttgcccagcccagagtatttgcactttatatgcaggtgtataaaaaatatattgggcacctaccagatgctcacgtcctatagattagcagttgttcccccaaatccaatgtaattcaagaattctcattttcaggagaaacattaatttgggtaaaccaaggatttttacagtaaagatctataacgactttcaactgaattatcccttaagtacatttgtgtacatgcatatgtagaaatacatttaccttacaataggacatagtatttttattttttaaaatgcagttttttttaaaagaaaatttgcagaatttactacactaaacccttcacttttttcatgccactgtacaatttttcctacagctgtgcctggaccaaagagagctcaaagaaaggctaagaattcacttctgggacttggaaagcttcaaaagagtgaaccagaactagggggaacattgatcctggatgcagctggctggcagaggtgctggtgtgctgtttcttcagaggtttcaggaaggcccccccatcccaaaatcacccttccttcacctgggaagtcaatgcctgagactccaccattacagatacaatgcaaaccttcctgggagacaaaactcctcatatacaccttaaagtgagtttttatgatcttttcaagagggtcaatgttgagaagaatccaagtggagaaaggatgaggttggttgagggtagcaccaaaagattctctttttcactcagaataggcgctgcaagtctgtcctgctggtgatgcacatacttgatgcctcccagaagtgagatgcttttgttccaagagggcttcctgtaggcagatgtgggagcaggagtcactggtgacactggagcattctcctgggtgcgggccggcgggcacctgtcactgatgggaagagctcctgtttccttgccttgtgccaagagggcccaaggcagacctgccagcagccacgagatggcgctgcgatccaggcgactccgggccctgcagccaccctccccgaggctgccccgcggaggacccaagcggtcgtggaggacgctctcccactccccagcttccctcttccctccctcctccttcctcgccccctggccctgcgaagagtggaggccgcatcagggagccctaggcccaagggcgggctaggactccccagtgactcccaggcagcccggggacagctgctt

SEQ ID NO: 10034 - RNA, 624 nt, Homo sapiens
  source 1..624: mol_type = other RNA
cacccggctgtgtgcacatgtgcaaaacgtaggtggagaaacgcatgagacttgtgacgtacatgaggaattccttgtgtggttattatagaaagtccttgagacagttcttatctcaaacatcagccgtcctttgtgcattcctggcttggtgtgcttgggtctgagtagagttgtctcatcctggtagctgggaaggctgaagagtgcaatttcagcagaatgtcaggggaggagcaggattgtactaggtggagaatattctagactgaaggaacaccacagaaaagacaagaaagcgtggaagggcgtggcttgaggaaaaaggtcgggaaactgggggttgaagaatgaacaggtgagatgggtaaggacttccagagaagaatgactactgggctgggggggggtgacatctgggccagtcacaattctcctcacgtgtcgccttccacaatgccaggcacgcgcctggggttgaatacatatttctgggctgaataaccgaatgtacaaaaggcaggccctaaatttcctctccgccccttagcgtgccccgcagcgacatcgtcacaagcgcgcggcttttggtccccgccctgggcctcagggcctcggggccgc

SEQ ID NO: 10035 - RNA, 373 nt, Homo sapiens
  source 1..373: mol_type = other RNA
cacccggctgtgtgcacatgtgcaaaacgtaggtggagaaacgcatgagacttgtgacgtacatgaggaattccttgtgtggttattatagaaagtccttgagacagttcttatctcaaacatcagccgtcctttgtgcattcctggcttggtgtgcttgggtctgagtagagttgtctcatcctggtaggtgtcgccttccacaatgccaggcacgcgcctggggttgaatacatatttctgggctgaataaccgaatgtacaaaaggcaggccctaaatttcctctccgccccttagcgtgccccgcagcgacatcgtcacaagcgcgcggcttttggtccccgccctgggcctcagggcctcggggccgc

SEQ ID NO: 10036 - RNA, 2787 nt, Homo sapiens
  source 1..2787: mol_type = other RNA
cacccggctgtgtgcacatgtgcacagcaggtgcaagtgtgtgttaagtatgtgtgcacgtgtgtttgtgtgtgatatgcacgtgtttgtgtgtgtgcgtgtgtgtgatatgcacgtgtttgggtgtgtgtgcgtgtgtgtgatatgcacgtttgtgtgcatgtgtgtgatatgcacgtgtttgtgtgtgtgcatgtgtgtgatatgcacgtgtttgggtgtgtgcgcgtgtgtgatatgcacatgtgtttgtgtgtgtgcatgtgtgtgatatgcacatgtgtttgtgtgtgtgtgtgtgggtgcacatgtgtcacagacaaggaggaagagggagggagggaaagctgtgcacagtttcacacccatgaccctctggactccctcccacctagggacgggccacttgctttcacagaagtcttgctgtcatccacatctgtcctttgagtcagggcttggtacccagatgttcatggagacgagaaaaagggaaagggattttgtccatgagaatctcccgtctgtcagccccttttctttttggaataaaccttcgtgttgctaagtgcctatactggagtggaatccagtcccagcggtggctggttttggaagtcgagtcttcactaaaggatgtctgggcattttcccaagccttgggcccgtgaaagccccccattggccctctgaggctgacagccatccccaaagtccagagcagcccccagcatctgtggtgctctcagccctgcagggctggggctacgacaaggacagggctgacagggcacactgagtgggcagaggtgtgcaggggccctgtgaagctgcaggggtggctcagacacacgacagcggagggtcccgagggttctgcccagagcgagaatgctggggacagacctgccgccgccacccccggagtagaacgcaagacacacacattgaacactgggaaaggtcagggcagccccctcctgcgatctcggccctgcccggccacaccaggggaagccaggactccgtgggcagcagggcatctcgggcagggccatgctggggtctcagtgggtcctttgatggaatcccctgctctgcctctagggtgccccaggactggagaccacaggacagaaaccggatgaccgtgtgcgggaccagcacgcggaattgggataaggggagtgggcgtggcccggagcgtttccccgctgaggtctttcacaaggaaggggcaggggtgtgatcacaaggaaggggcaggggtgtgatcacaaggaaggggcaggggtgtgatcacaaggaaggggcaggggtgtgaacggcttctgaaaggcggggtcacttcggtacccccagtgacctcatgtggcagatgggccccccactctgctctgaagctcctccaggaacaccgtgtcctctgcccccatctacacagtagtttcgtttttccagggtcccgttcggatgttgccggtcccgtcggtgccaaacggcaggccttctagcaatttacccttgggcagcccgttctggctggggccaccaaagggcagggactgtgtcctccgcagcatctccaagtggccgggcccgagcgctgcctccctgcccggctgcgtggggcagctgtagagggcagggctcccatcactgccctcgggctgggtgaccatggggaaggggtcgccctgggtgcagcaggccagcgtgtgtgtccccgccgggccatccagagagctgggggggctgtctgtgcgcgagctgcgggggctgccatccaggctggatgggatgtggtaggcgtactcgggctcctctgctgggtgccggctaaagtagggcggcttagttctgccctgaaggcacccgtgcaggtgggggtcgtgcccgaaggcgccctcctcctgcaggtgcacgtgcgcctcgtccgccgtcagtggctcgcagtgcatcttggcgcagcacggggtggccggtgacaggcaactggcgtggccctgcgcggcctgcaggttggtcatcttgcaggggcccggtgggtgcgcgaagccccgtggctggcccagtcccggcgagtgcaggcaggcggcgcggcccagcgcggccccgttggcgtcaagtgcggggtgggcgtccttgcggggcgggcagcatgcccaccagcactgccacacgtcctcacgcttggcgcagtggtggatgagcacgaagagtcccagggtcacgcagaaggcgccgtacaggcagctgaagaccatgtccaggaagtggccctgtgacaccgccagcgccccgaaggcccacgtggccgtgaacaggaacagcgtgaaggcggcggcgcgcagctgtgcctggaatgagtgctcgttctgcagcacggaggcgccgggggcatcgtgtgcgggtggggtgcctggccggatcccacggccgccctcgggtgtcgccagccgccgctgctcctcgggctgtgtgcgcagctcgtacctgcgccctgggtggcgccgcagctgcacgtaggtgcccaggaagtacacacaggtgaccagggtgatgatggcggctgggccgtagaaggcgcccaggctgggctcccaggccatccagcagtacgccgtgtcctcgtcctctgtcccgtaattcctgatgttcgtggcagccgtgaccccacagatgataaaggggacccctccgctgacgaggtaaaaccgcctggcacaggatggggtacttggtgcgattgatgccgccggcgaacacagtgaaggtcagggccgc

SEQ ID NO: 10037 - RNA, 3536 nt, Homo sapiens
  source 1..3536: mol_type = other RNA
cacccggctgtgtgcacatgtgcacagcaggtgcaagtgtgtgttaagtatgtgtgcacgtgtgtttgtgtgtgatatgcacgtgtttgtgtgtgtgcgtgtgtgtgatatgcacgtgtttgggtgtgtgtgcgtgtgtgtgatatgcacgtttgtgtgcatgtgtgtgatatgcacgtgtttgtgtgtgtgcatgtgtgtgatatgcacgtgtttgggtgtgtgcgcgtgtgtgatatgcacatgtgtttgtgtgtgtgcatgtgtgtgatatgcacatgtgtttgtgtgtgtgtgtgtgggtgcacatgtgtcacagacaaggaggaagagggagggagggaaagctgtgcacagtttcacacccatgaccctctggactccctcccacctagggacgggccacttgctttcacagaagtcttgctgtcatccacatctgtcctttgagtcagggcttggtacccagatgttcatggagacgagaaaaagggaaagggattttgtccatgagaatctcccgtctgtcagccccttttctttttggaataaaccttcgtgttgctaagtgcctatactggagtggaatccagtcccagcggtggctggttttggaagtcgagtcttcactaaaggatgtctgggcattttcccaagccttgggcccgtgaaagccccccattggccctctgaggctgacagccatccccaaagtccagagcagcccccagcatctgtggtgctctcagccctgcagggctggggctacgacaaggacagggctgacagggcacactgagtgggcagaggtgtgcaggggccctgtgaagctgcaggggtggctcagacacacgacagcggagggtcccgagggttctgcccagagcgagaatgctggggacagacctgccgccgccacccccggagtagaacgcaagacacacacattgaacactgggaaaggtcagggcagccccctcctgcgatctcggccctgcccggccacaccaggggaagccaggactccgtgggcagcagggcatctcgggcagggccatgctggggtctcagtgggtcctttgatggaatcccctgctctgcctctagggtgccccaggactggagaccacaggacagaaaccggatgaccgtgtgcgggaccagcacgcggaattgggataaggggagtgggcgtggcccggagcgtttccccgctgaggtctttcacaaggaaggggcaggggtgtgatcacaaggaaggggcaggggtgtgatcacaaggaaggggcaggggtgtgatcacaaggaaggggcaggggtgtgaacggcttctgaaaggcggggtcacttcggtacccccagtgacctcatgtggcagatgggccccccactctgctctgaagctcctccaggaacaccgtgtcctctgcccccatctacacagtagtttcgtttttccagggtcccgttcggatgttgccggtcccgtcggtgccaaacggcaggccttctagcaatttacccttgggcagcccgttctggctggggccaccaaagggcagggactgtgtcctccgcagcatctccaagtggccgggcccgagcgctgcctccctgcccggctgcgtggggcagctgtagagggcagggctcccatcactgccctcgggctgggtgaccatggggaaggggtcgccctgggtgcagcaggccagcgtgtgtgtccccgccgggccatccagagagctgggggggctgtctgtgcgcgagctgcgggggctgccatccaggctggatgggatgtggtaggcgtactcgggctcctctgctgggtgccggctaaagtagggcggcttagttctgccctgaaggcacccgtgcaggtgggggtcgtgcccgaaggcgccctcctcctgcaggtgcacgtgcgcctcgtccgccgtcagtggctcgcagtgcatcttggcgcagcacggggtggccggtgacaggcaactggcgtggccctgcgcggcctgcaggttggtcatcttgcaggggcccggtgggtgcgcgaagccccgtggctggcccagtcccggcgagtgcaggcaggcggcgcggcccagcgcggccccgttggcgtcaagtgcggggtgggcgtccttgcggggcgggcagcatgcccaccagcactgccacacgtcctcacgcttggcgcagtggtggatgagcacgaagagtcccagggtcacgcagaaggcgccgtacaggcagctgaagaccatgtccaggaagtggccctgtgacaccgccagcgccccgaaggcccacgtggccgtgaacaggaacagcgtgaaggcggcggcgcgcagctgtgcctggaatgagtgctcgttctgcagcacggaggcgccgggggcatcgtgtgcgggtggggtgcctggccggatcccacggccgccctcgggtgtcgccagccgccgctgctcctcgggctgtgtgcgcagctcgtacctgcgccctgggtggcgccgcagctgcacgtaggtgcccaggaagtacacacaggtgaccagggtgatgatggcggctgggccgtagaaggcgcccaggctgggctcccaggccatccagcagtacgccgtgtcctcgtcctctgtcccgtaattcctgatgttcgtggcagccgtgaccccacagatgataaaggggacccctccgctgacgaggtaaaacctgagcaggggctgcctggggtacggtggctggtctgtgtccaggcacagaggggccttcttggtcacctgcttgtagatgttcctggcggtcactcctatccacagcatggtggacagtgtagaatagtgcagcacgatgcccaccgcctggcacaggatggggtacttggtgcgattgatgccgccggcgaacacagtgaaggtcagggccgcgtggaagcagaaattcaggagcgtgtgccggcccttgcggctgatgcggatggcgctctggtgcacgatgtaggtgacgaaggaggccaggaggcagagcagcatgacggccgtgcacgcgtacaccacggggtgcaggaactcccctgggtagcggggcagggagagcactgtcttcagatccatgagcgctgcaaagttgcggaagcgtgagcgccgctggaggaggcgtccagggggaggcgatcaggtggcgccctgctccccgccagcctccatggcctctggaaggtcaaagtcccagacggcggccaggaggtcgcgctcccgggcccctggcctcagggtgaccgcggcggggcgggcgcagtccgggagctgctcccatctgctgtggccgaagcggctgccggggcggccgggccgcgctcccggagacagacgcgctgcgctccccccgccggggacccgctctccattcgcgagggcagcggccgagctgggaccgagttatcaacagattgcggggctgcggcgccggccggtgagtcacagccccgcgcacgagcggcccagcccggccagcagcgccgccgcctctgc

SEQ ID NO: 10038 - RNA, 2957 nt, Homo sapiens
  source 1..2957: mol_type = other RNA
cacccggctgtgtgcacatgtgcacagcaggtgcaagtgtgtgttaagtatgtgtgcacgtgtgtttgtgtgtgatatgcacgtgtttgtgtgtgtgcgtgtgtgtgatatgcacgtgtttgggtgtgtgtgcgtgtgtgtgatatgcacgtttgtgtgcatgtgtgtgatatgcacgtgtttgtgtgtgtgcatgtgtgtgatatgcacgtgtttgggtgtgtgcgcgtgtgtgatatgcacatgtgtttgtgtgtgtgcatgtgtgtgatatgcacatgtgtttgtgtgtgtgtgtgtgggtgcacatgtgtcacagacaaggaggaagagggagggagggaaagctgtgcacagtttcacacccatgaccctctggactccctcccacctagggacgggccacttgctttcacagaagtcttgctgtcatccacatctgtcctttgagtcagggcttggtacccagatgttcatggagacgagaaaaagggaaagggattttgtccatgagaatctcccgtctgtcagccccttttctttttggaataaaccttcgtgttgctaagtgcctatactggagtggaatccagtcccagcggtggctggttttggaagtcgagtcttcactaaaggatgtctgggcattttcccaagccttgggcccgtgaaagccccccattggccctctgaggctgacagccatccccaaagtccagagcagcccccagcatctgtggtgctctcagccctgcagggctggggctacgacaaggacagggctgacagggcacactgagtgggcagaggtgtgcaggggccctgtgaagctgcaggggtggctcagacacacgacagcggagggtcccgagggttctgcccagagcgagaatgctggggacagacctgccgccgccacccccggagtagaacgcaagacacacacattgaacactgggaaaggtcagggcagccccctcctgcgatctcggccctgcccggccacaccaggggaagccaggactccgtgggcagcagggcatctcgggcagggccatgctggggtctcagtgggtcctttgatggaatcccctgctctgcctctagggtgccccaggactggagaccacaggacagaaaccggatgaccgtgtgcgggaccagcacgcggaattgggataaggggagtgggcgtggcccggagcgtttccccgctgaggtctttcacaaggaaggggcaggggtgtgatcacaaggaaggggcaggggtgtgatcacaaggaaggggcaggggtgtgatcacaaggaaggggcaggggtgtgaacggcttctgaaaggcggggtcacttcggtacccccagtgacctcatgtggcagatgggccccccactctgctctgaagctcctccaggaacaccgtgtcctctgcccccatctacacagtagtttcgtttttccagggtcccgttcggatgttgccggtcccgtcggtgccaaacggcaggccttctagcaatttacccttgggcagcccgttctggctggggccaccaaagggcagggactgtgtcctccgcagcatctccaagtggccgggcccgagcgctgcctccctgcccggctgcgtggggcagctgtagagggcagggctcccatcactgccctcgggctgggtgaccatggggaaggggtcgccctgggtgcagcaggccagcgtgtgtgtccccgccgggccatccagagagctgggggggctgtctgtgcgcgagctgcgggggctgccatccaggctggatgggatgtggtaggcgtactcgggctcctctgctgggtgccggctaaagtagggcggcttagttctgccctgaaggcacccgtgcaggtgggggtcgtgcccgaaggcgccctcctcctgcaggtgcacgtgcgcctcgtccgccgtcagtggctcgcagtgcatcttggcgcagcacggggtggccggtgacaggcaactggcgtggccctgcgcggcctgcaggttggtcatcttgcaggggcccggtgggtgcgcgaagccccgtggctggcccagtcccggcgagtgcaggcaggcggcgcggcccagcgcggccccgttggcgtcaagtgcggggtgggcgtccttgcggggcgggcagcatgcccaccagcactgccacacgtcctcacgcttggcgcagtggtggatgagcacgaagagtcccagggtcacgcagaaggcgccgtacaggcagctgaagaccatgtccaggaagtggccctgtgacaccgccagcgccccgaaggcccacgtggccgtgaacaggaacagcgtgaaggcggcggcgcgcagctgtgcctggaatgagtgctcgttctgcagcacggaggcgccgggggcatcgtgtgcgggtggggtgcctggccggatcccacggccgccctcgggtgtcgccagccgccgctgctcctcgggctgtgtgcgcagctcgtacctgcgccctgggtggcgccgcagctgcacgtaggtgcccaggaagtacacacaggtgaccagggtgatgatggcggctgggccgtagaaggcgcccaggctgggctcccaggccatccagcagtacgccgtgtcctcgtcctctgtcccgtaattcctgatgttcgtggcagccgtgaccccacagatgataaaggggacccctccgctgacgaggtaaaacctgagcaggggctgcctggggtacggtggctggtctgtgtccaggcacagaggggccttcttggtcacctgcttgtagatgttcctggcggtcactcctatccacagcatggtggacagtgtagaatagtgcagcacgatgcccacctggataggtgtccaccaagggagaggaggtgaagtcctcagtggggtcacgccaggatgctcttactgtgggtaggatgagccccccacggg

SEQ ID NO: 10039 - RNA, 2123 nt, Homo sapiens
  source 1..2123: mol_type = other RNA
cacccggctgtgtgcacatgtgcacatgtgtgccttgcaggatggcaatctgggggtagtgaacaatactcagggaagatcttattagtgaatatttttaaagtttccaaacagaataaattccccatgaagtttattggagaggtgtgggagagagggtaaggtgggagtgggcaaccctttaaacaaaacacaggatgcaagatctccttcataaactggagggctccagggctctagtcacacccctcatagcccagcaggtcacactggacatcatttcaaactagactctgcctgaagtatggcccttatgatggatttgcttctgctatgtttttatactcattccggcagaaggggagacacctgaacccagcccaccctcaggttgctctccaggtggataatccacctggctttctcagggaatggggtggggccgggctggcacactttcaccctcccagtccccatagatcttcctctctcctcctcccttttgtggccacccagggtctacgaatccgtggaaggcagagagtccctctgccttagaataggtcataggaggccttgtaaaatgaaacaaaaacaacttcttgctaaacatggttgcagataatcagtaccatggctgacatccactaaggtggataactgagaattgatagtaatcatgtttcaaaaggtgtttatgcatgcccttacttcagtaccagagataggagaagagctcttgcttctgcatcacagaaggagacagtgtgggctaagagcactacgagcctgcagggagagacaagggagaaggtgactgacaccaaaggcccactgagaggggctttcttctggggcctggcatttggatgcatgagggagaaaagaaaaagaatttgttttgacccaaaagcccatctccacattgccatagaagacaaaaaggtgggggtagagccagagcaggtatgcgtgctcaggcagacagataccaggagagagcagggccagaagattggcctttgcctctgggagggagacccacaggtttctgtgccctgagttggagacctggactctcattaaacttgactcctcatctcccaagtcaggaccagcatgtgcaggattcctagcttgaggtctggaccctccagctggcccccaaggacctggcagccctggacacgaacctggatgctgcaccagatcctcaggggatggtgccccctctcaggaagtctctgttccctgagcaaaagccagacacagtggcctgagagctgaaacagtgcttgacaccacagctgtggggagacagctctgtgcacccccacaccccttctacatccctgaatatccatctcacacagcattgaggggcaccttcttgaagtgtcccatgaaggaacagtggccagggctcccacaccacccactgtctgggccatgtgtccaccacaggcagcaagggccctgaaggcagggtctccccttcccccacgtggatgcagcgtgagtttctacacggaagaggaaccctgcagctcctatactgtggaggaggaacctccacagggccacggacaaatagtgacctgcccaaggccacacagccaatgcctacagagcaagttcagggccccagggccccagctgcctggccaaaggctccttccttttactctcaggaaaagggaaggttggatcctgaccgcacagcaaatccacccccacctatgtagagcagttcatgttgttggtgacttctctagattgcctgttcgcatgaaaacagaataatcagtagatcctctcacggggctcagaggagaacaacgtcagaggaaaggatacctcaagtctgcttcataattcataattcaatctcagctgggaatcgcatcaactcagagcagctggtccagcctccacctcagccagcttgtcctgggcatctccgatggctaccttgcccttctgctctgcctccaggatggtgtcttgcagggcagcacactgctgagttggggtcccatctgtttcctgaggttggtgatttctgcctgaagtctctgggtggctcagttcagctcatcgacctccatctaaatggctttgag

SEQ ID NO: 10040 - RNA, 2178 nt, Homo sapiens
  source 1..2178: mol_type = other RNA
cacccggctgtgtgcacatgtgcacatgtgtgccttgcaggatggcaatctgggggtagtgaacaatactcagggaagatcttattagtgaatatttttaaagtttccaaacagaataaattccccatgaagtttattggagaggtgtgggagagagggtaaggtgggagtgggcaaccctttaaacaaaacacaggatgcaagatctccttcataaactggagggctccagggctctagtcacacccctcatagcccagcaggtcacactggacatcatttcaaactagactctgcctgaagtatggcccttatgatggatttgcttctgctatgtttttatactcattccggcagaaggggagacacctgaacccagcccaccctcaggttgctctccaggtggataatccacctggctttctcagggaatggggtggggccgggctggcacactttcaccctcccagtccccatagatcttcctctctcctcctcccttttgtggccacccagggtctacgaatccgtggaaggcagagagtccctctgccttagaataggtcataggaggccttgtaaaatgaaacaaaaacaacttcttgctaaacatggttgcagataatcagtaccatggctgacatccactaaggtggataactgagaattgatagtaatcatgtttcaaaaggtgtttatgcatgcccttacttcagtaccagagataggagaagagctcttgcttctgcatcacagaaggagacagtgtgggctaagagcactacgagcctgcagggagagacaagggagaaggtgactgacaccaaaggcccactgagaggggctttcttctggggcctggcatttggatgcatgagggagaaaagaaaaagaatttgttttgacccaaaagcccatctccacattgccatagaagacaaaaaggtgggggtagagccagagcaggtatgcgtgctcaggcagacagataccaggagagagcagggccagaagattggcctttgcctctgggagggagacccacaggtttctgtgccctgagttggagacctggactctcattaaacttgactcctcatctcccaagtcaggaccagcatgtgcaggattcctagcttgaggtctggaccctccagctggcccccaaggacctggcagccctggacacgaacctggatgctgcaccagatcctcaggggatggtgccccctctcaggaagtctctgttccctgagcaaaagccagacacagtggcctgagagctgaaacagtgcttgacaccacagctgtggggagacagctctgtgcacccccacaccccttctacatccctgaatatccatctcacacagcattgaggggcaccttcttgaagtgtcccatgaaggaacagtggccagggctcccacaccacccactgtctgggccatgtgtccaccacaggcagcaagggccctgaaggcagggtctccccttcccccacgtggatgcagcgtgagtttctacacggaagaggaaccctgcagctcctatactgtggaggaggaacctccacagggccacggacaaatagtgacctgcccaaggccacacagccaatgcctacagagcaagttcagggccccagggccccagctgcctggccaaaggctccttccttttactctcaggaaaagggaaggttggatcctgaccgcacagcaaatccacccccacctatgtagagcagttcatgttgttggtgacttctctagattgcctgttcgcatgaaaacagaataatcagtagatcctctcacggggctcagaggagaacaacgtcagaggaaaggatacctcaagtctgcttcataattcataattcaatctcagctgggaatcgcatcaactcctgcacgcctggccctccagggccaccttgatgctcatcagctcctggtactcacagagcagctggtccagcctccacctcagccagcttgtcctgggcatctccgatggctaccttgcccttctgctctgcctccaggatggtgtcttgcagggcagcacactgctgagttggggtcccatctgtttcctgaggttggtgatttctgcctgaagtctctgggtggctcagttcagctcatcgacctccatctaaatggctttgag

SEQ ID NO: 10041 - RNA, 3069 nt, Homo sapiens
  source 1..3069: mol_type = other RNA
cacccggctgtgtgcacatgtgcactgtgtatgcatggtaatgtgcacgcgtgcactgtgtgtatgcatggtaatgtgcacgtgtgcactgtgtgtggtgtgtatgcatggtgtgtgcacgtgtgcactgtgtatgcatggtaatgtgcacgtgtgcactgtgtggtgtgtatgcatggtgtgtgcacgtgtgcactgtgtatgcatagtgtgtgcacgtgtgcactgtgtgtggatgcatggtaatgtgcacgtgtgcactgtgtgtggtgtgtatgcatggtgtgtgcacgtgtgcacggtgtgtggtgtgtatgcatggtgtgtgcacgtgtgcactgtgtatgcatagtgtgtgcacgtgtgcactgtgtgtggatgcatggtaatgtgcacgtgtgcactgtgtgtggtgtgtatgcatggtgtgtgcacgtgtgcacggtgtgtggtgtgtatgcatggtgtgtgcacgtgtgcactgtgtgcatgcgtgtgtggtgtgtgtgcatgtatgcatggtgtgtgcatacgtgtgcagcagcacctggtcccatctccagtgcccagcagcatcacacgcactttggtgctttataaatgcatggtcagtgaggctgacagcaccaagctgtccctttaccataacacctggaatagtcacctgtgataagctatcacataggaaacatttttaaaatttcattctcattattttctgtaatcttgagaggttccaatcaacatttattgccttattctttttatctcattcctttttgaatgtgtttatctcctaagattttatctgtgatggagatgggatgcctgtgaatacaaaagttgcagtggtggcaccagggtgggggggtgcggccggggccaccatggtctcccctgagagggggtgctgtcttaggtgccccaagaggccctcgggcagcaagcgtggggtgctgccaaaatacagctccccctgggtgggcaggacacacgtggcctcctggcagacaggtgcctgggtgagcccgctgctcctgattagtcatgaatggcacctggtctgggcgacagtcacccgcaggaagccctgagctggccaccatcaccctgggcagtggctcccggggtgccaacaagacctgggcccctcgttctttggtgctgagagccccagctgaggctgtggaggaggccctggacctggtctggtgtctgtcagaggcaggtgcccagtcctttgacttgcttctctgaattgtcataattgtgctggaattgtgccagaaactggtagtgataacagctcctggaaggcctgtggctgctgagggctgcctggtccccctcaggacggccgggggagcctctccagaagcaccagctttgtctgcaggtggacgttgaaggggggcagttgggtcaggttcagactcacacctgtggtccccacgacgctggccaggacccggtgtgtgtccctgtagagggccaggagcccaggggccgcctccatgaggatgtgtgtgtatgccagcatgcctgtccccggctgcacatcctccctcttgtcgtacctccaggcgctgttgacttggagaaaccgagacacacctgtctgggcggctgccacgtcaatgtgcagaaggacgtctgtctgggggggcaccagctggtgcagcctctgcattgcgacgccacctgggtagttgaaatgggacacatacagggccgtggctgagtaggcggcattcaccacgaggtgtccgatcacaagcagagaccccgctttgtacagccaagactttttatagttattcagcaggtaggagcagcctctggcagccgtgatgttgagcatggggaaggcatagatgatgaagcgtagctccttgtgtggcaggagggagtagagtgccatgaagcccagtgccagcaccgtcggcgcgtgcgtccttctgtctaccaagcccagggggatgaagagcaggctgcagcccaggccgcggggcagggctgagtagaagtaccacagcagcggggaggtcccccagttggagcttttgttcaggacagtgttgtaccaaagcacctttccttccggccaagtgagctgccgccaaaaataagagtccacagcaaccgtcagtcctaaacagaggatccctgccgggacggcgtggcgaagggctctgactacagaaacctttcggttgcccaaggccagcagcagcaggaggcccaggaacaggcacagctccaccctgaacacgatgatggcgaaggctgacagccagatgaagcgggcccactcgtgccgcagccaggccgcgagggccagcaggactacaggcagggccagcacattgggcagtgtccgcgtgcagtagaacatcaggtggaactgcatggccgtcacccagcagaacatggtggccaccatggccccgaagtgccgtctcacttccttttgtaacgtccagagtccaaaaatcacgccgagtccaagcactcctctaactattagctgagagtaaaacttggacatttctaacagcgaaagcacgtaaaccgcggggctggagaacactgcgatcaccactggcccgaggaacgtcctggggacgactccggggaactcaagatggtcgtactgctccaggtcttgccagtggtagagcaggtcatgtgtggcctgcaggttgaagctctcctccactttggtgtagggacagatgaccaggtggacagtggctacggccaccagcagccccagcagcaggggccgcctgcctgatgacccctttccagccattccaggctttcagcttcacgtaccttcacaggccaacagtgcgagacaccagccgttagcactgccactccacgcatgctccgcagctcccggcggcgtccttcgaagcgcggctgcctgggccagcctcggcaggaagcaggacggcggaaacagaacagagcccgaatctaaagtccttgcccaaatctaaagtggctaccgcagccccggccgctacggccgcagagaccctctgtgccctgagtaaagat

SEQ ID NO: 10042 - RNA, 3166 nt, Homo sapiens
  source 1..3166: mol_type = other RNA
cacccggctgtgtgcacatgtgcactgtgtatgcatggtgtgtgcacgtgtgcactgtgtatgcatggtgtgtgcacgtgtgcactgtgtggtgtgtatgcatggtgtgtgcacatgtgcactgtgtatgcatggtaatgtgcacgcgtgcactgtgtgtatgcatggtaatgtgcacgtgtgcactgtgtgtggtgtgtatgcatggtgtgtgcacgtgtgcactgtgtatgcatggtaatgtgcacgtgtgcactgtgtggtgtgtatgcatggtgtgtgcacgtgtgcactgtgtatgcatagtgtgtgcacgtgtgcactgtgtgtggatgcatggtaatgtgcacgtgtgcactgtgtgtggtgtgtatgcatggtgtgtgcacgtgtgcacggtgtgtggtgtgtatgcatggtgtgtgcacgtgtgcactgtgtatgcatagtgtgtgcacgtgtgcactgtgtgtggatgcatggtaatgtgcacgtgtgcactgtgtgtggtgtgtatgcatggtgtgtgcacgtgtgcacggtgtgtggtgtgtatgcatggtgtgtgcacgtgtgcactgtgtgcatgcgtgtgtggtgtgtgtgcatgtatgcatggtgtgtgcatacgtgtgcagcagcacctggtcccatctccagtgcccagcagcatcacacgcactttggtgctttataaatgcatggtcagtgaggctgacagcaccaagctgtccctttaccataacacctggaatagtcacctgtgataagctatcacataggaaacatttttaaaatttcattctcattattttctgtaatcttgagaggttccaatcaacatttattgccttattctttttatctcattcctttttgaatgtgtttatctcctaagattttatctgtgatggagatgggatgcctgtgaatacaaaagttgcagtggtggcaccagggtgggggggtgcggccggggccaccatggtctcccctgagagggggtgctgtcttaggtgccccaagaggccctcgggcagcaagcgtggggtgctgccaaaatacagctccccctgggtgggcaggacacacgtggcctcctggcagacaggtgcctgggtgagcccgctgctcctgattagtcatgaatggcacctggtctgggcgacagtcacccgcaggaagccctgagctggccaccatcaccctgggcagtggctcccggggtgccaacaagacctgggcccctcgttctttggtgctgagagccccagctgaggctgtggaggaggccctggacctggtctggtgtctgtcagaggcaggtgcccagtcctttgacttgcttctctgaattgtcataattgtgctggaattgtgccagaaactggtagtgataacagctcctggaaggcctgtggctgctgagggctgcctggtccccctcaggacggccgggggagcctctccagaagcaccagctttgtctgcaggtggacgttgaaggggggcagttgggtcaggttcagactcacacctgtggtccccacgacgctggccaggacccggtgtgtgtccctgtagagggccaggagcccaggggccgcctccatgaggatgtgtgtgtatgccagcatgcctgtccccggctgcacatcctccctcttgtcgtacctccaggcgctgttgacttggagaaaccgagacacacctgtctgggcggctgccacgtcaatgtgcagaaggacgtctgtctgggggggcaccagctggtgcagcctctgcattgcgacgccacctgggtagttgaaatgggacacatacagggccgtggctgagtaggcggcattcaccacgaggtgtccgatcacaagcagagaccccgctttgtacagccaagactttttatagttattcagcaggtaggagcagcctctggcagccgtgatgttgagcatggggaaggcatagatgatgaagcgtagctccttgtgtggcaggagggagtagagtgccatgaagcccagtgccagcaccgtcggcgcgtgcgtccttctgtctaccaagcccagggggatgaagagcaggctgcagcccaggccgcggggcagggctgagtagaagtaccacagcagcggggaggtcccccagttggagcttttgttcaggacagtgttgtaccaaagcacctttccttccggccaagtgagctgccgccaaaaataagagtccacagcaaccgtcagtcctaaacagaggatccctgccgggacggcgtggcgaagggctctgactacagaaacctttcggttgcccaaggccagcagcagcaggaggcccaggaacaggcacagctccaccctgaacacgatgatggcgaaggctgacagccagatgaagcgggcccactcgtgccgcagccaggccgcgagggccagcaggactacaggcagggccagcacattgggcagtgtccgcgtgcagtagaacatcaggtggaactgcatggccgtcacccagcagaacatggtggccaccatggccccgaagtgccgtctcacttccttttgtaacgtccagagtccaaaaatcacgccgagtccaagcactcctctaactattagctgagagtaaaacttggacatttctaacagcgaaagcacgtaaaccgcggggctggagaacactgcgatcaccactggcccgaggaacgtcctggggacgactccggggaactcaagatggtcgtactgctccaggtcttgccagtggtagagcaggtcatgtgtggcctgcaggttgaagctctcctccactttggtgtagggacagatgaccaggtggacagtggctacggccaccagcagccccagcagcaggggccgcctgcctgatgacccctttccagccattccaggctttcagcttcacgtaccttcacaggccaacagtgcgagacaccagccgttagcactgccactccacgcatgctccgcagctcccggcggcgtccttcgaagcgcggctgcctgggccagcctcggcaggaagcaggacggcggaaacagaacagagcccgaatctaaagtccttgcccaaatctaaagtggctaccgcagccccggccgctacggccgcagagaccctctgtgccctgagtaaagat

SEQ ID NO: 10043 - RNA, 3372 nt, Homo sapiens
  source 1..3372: mol_type = other RNA
cacccggctgtgtgcacatgtgcactgtgtggtgtgtatgcatggtgtgtgcacgtgtgcactgtgtatgcatggtgtgtgcatgtgtgcactgtatgcatagtgtgcacgtgtgcactgtgtgtggatgcatggtaatgtgcacgtgtgcactgtgtgtggtgtgtatgcatggtgtgtgcacgtgtgcacggtgtgtggtgtgtatgcatggtgtgtgcacatgtgcactgtgtatgcatggtgtgtgcacgtgtgcactgtgtatgcatggtgtgtgcacgtgtgcactgtgtggtgtgtatgcatggtgtgtgcacatgtgcactgtgtatgcatggtaatgtgcacgcgtgcactgtgtgtatgcatggtaatgtgcacgtgtgcactgtgtgtggtgtgtatgcatggtgtgtgcacgtgtgcactgtgtatgcatggtaatgtgcacgtgtgcactgtgtggtgtgtatgcatggtgtgtgcacgtgtgcactgtgtatgcatagtgtgtgcacgtgtgcactgtgtgtggatgcatggtaatgtgcacgtgtgcactgtgtgtggtgtgtatgcatggtgtgtgcacgtgtgcacggtgtgtggtgtgtatgcatggtgtgtgcacgtgtgcactgtgtatgcatagtgtgtgcacgtgtgcactgtgtgtggatgcatggtaatgtgcacgtgtgcactgtgtgtggtgtgtatgcatggtgtgtgcacgtgtgcacggtgtgtggtgtgtatgcatggtgtgtgcacgtgtgcactgtgtgcatgcgtgtgtggtgtgtgtgcatgtatgcatggtgtgtgcatacgtgtgcagcagcacctggtcccatctccagtgcccagcagcatcacacgcactttggtgctttataaatgcatggtcagtgaggctgacagcaccaagctgtccctttaccataacacctggaatagtcacctgtgataagctatcacataggaaacatttttaaaatttcattctcattattttctgtaatcttgagaggttccaatcaacatttattgccttattctttttatctcattcctttttgaatgtgtttatctcctaagattttatctgtgatggagatgggatgcctgtgaatacaaaagttgcagtggtggcaccagggtgggggggtgcggccggggccaccatggtctcccctgagagggggtgctgtcttaggtgccccaagaggccctcgggcagcaagcgtggggtgctgccaaaatacagctccccctgggtgggcaggacacacgtggcctcctggcagacaggtgcctgggtgagcccgctgctcctgattagtcatgaatggcacctggtctgggcgacagtcacccgcaggaagccctgagctggccaccatcaccctgggcagtggctcccggggtgccaacaagacctgggcccctcgttctttggtgctgagagccccagctgaggctgtggaggaggccctggacctggtctggtgtctgtcagaggcaggtgcccagtcctttgacttgcttctctgaattgtcataattgtgctggaattgtgccagaaactggtagtgataacagctcctggaaggcctgtggctgctgagggctgcctggtccccctcaggacggccgggggagcctctccagaagcaccagctttgtctgcaggtggacgttgaaggggggcagttgggtcaggttcagactcacacctgtggtccccacgacgctggccaggacccggtgtgtgtccctgtagagggccaggagcccaggggccgcctccatgaggatgtgtgtgtatgccagcatgcctgtccccggctgcacatcctccctcttgtcgtacctccaggcgctgttgacttggagaaaccgagacacacctgtctgggcggctgccacgtcaatgtgcagaaggacgtctgtctgggggggcaccagctggtgcagcctctgcattgcgacgccacctgggtagttgaaatgggacacatacagggccgtggctgagtaggcggcattcaccacgaggtgtccgatcacaagcagagaccccgctttgtacagccaagactttttatagttattcagcaggtaggagcagcctctggcagccgtgatgttgagcatggggaaggcatagatgatgaagcgtagctccttgtgtggcaggagggagtagagtgccatgaagcccagtgccagcaccgtcggcgcgtgcgtccttctgtctaccaagcccagggggatgaagagcaggctgcagcccaggccgcggggcagggctgagtagaagtaccacagcagcggggaggtcccccagttggagcttttgttcaggacagtgttgtaccaaagcacctttccttccggccaagtgagctgccgccaaaaataagagtccacagcaaccgtcagtcctaaacagaggatccctgccgggacggcgtggcgaagggctctgactacagaaacctttcggttgcccaaggccagcagcagcaggaggcccaggaacaggcacagctccaccctgaacacgatgatggcgaaggctgacagccagatgaagcgggcccactcgtgccgcagccaggccgcgagggccagcaggactacaggcagggccagcacattgggcagtgtccgcgtgcagtagaacatcaggtggaactgcatggccgtcacccagcagaacatggtggccaccatggccccgaagtgccgtctcacttccttttgtaacgtccagagtccaaaaatcacgccgagtccaagcactcctctaactattagctgagagtaaaacttggacatttctaacagcgaaagcacgtaaaccgcggggctggagaacactgcgatcaccactggcccgaggaacgtcctggggacgactccggggaactcaagatggtcgtactgctccaggtcttgccagtggtagagcaggtcatgtgtggcctgcaggttgaagctctcctccactttggtgtagggacagatgaccaggtggacagtggctacggccaccagcagccccagcagcaggggccgcctgcctgatgacccctttccagccattccaggctttcagcttcacgtaccttcacaggccaacagtgcgagacaccagccgttagcactgccactccacgcatgctccgcagctcccggcggcgtccttcgaagcgcggctgcctgggccagcctcggcaggaagcaggacggcggaaacagaacagagcccgaatctaaagtccttgcccaaatctaaagtggctaccgcagccccggccgctacggccgcagagaccctctgtgccctgagtaaagat

SEQ ID NO: 10044 - RNA, 2460 nt, Homo sapiens
  source 1..2460: mol_type = other RNA
cacccggctgtgtgcacatgtgcatgtatatgtgtacataaaggggcaggagatggcaggtagagggggtgcccccgctcctggatggagagcaggcatgagagttgaccctgagctcccaacaaattagccgaaagaaaagggaggccagtagtggatcctagatggattaagggtgtactacacatccagttgtctacacatctatgccctctttatttgcactgtgataggtgaaatgggtctgaaggctgctgagggaagcggctactcagagctgcaggatgacctacccagggtcacacaactgaactgggacatgaagaggacagaaaacctaaagggaggggcccttctctgggtcggtctctgatgggcactgagcacacctcacctcactaactcttcccagcctcctgggaaggaggtctgaccatagtcactttacagatgaggaaaacgaggctcatagaggtggagtgagttgcccaaggtcacacaagccatcgatggcagggctggaatttgagaccttttggggttagcagattggctcctatgcctcacaagcaagccataggtttggccactcttcccccgtgccctgcttctcctcctgtgctgtgatcccaggtctagcacctctcccagcagtcacctcctggtggacatcacagtgagagctatttgcttattcagggtgcctgccctgtactagcgagagatcactccctcagctattgctgggatggtgtctttgggtgggtactggtgccaccagcccccactgggggtatagtgggtgctggggtgctctcatccatgcaggggagcctgggtagacctccagaatggagtgactccactttctgggctgccgtcatcaccagttggctctggccccacaagaggccctagttgtccatcttcctccacctcagggcgtgggatgcctctaggatggcctgcaggagttgagggaccaagaaggtgagggagcactcacagagctcattcctctcggaagaggtgctgggaggtgcggcgtctattctggggctggccagctccagctatgcttctggcttccggtctaagggctgccctggagattggggacctggtgtcgggcagagctggctgagaatggtgacttttctgctctcaggaactgcatccgagaccaggggctgccccctgctgcaccctgaggcggtgaccacctcacccgatgaagggccaggggccagggctgggcctgggagttggtttcccttcaggcttctcaggaaaatgtccttgggaaaccagggcatccagtgtaagacagggtcactgaagcaaggcaggacctcctcactgtccaggcatgtgctgccatggcactgggggccctagaggactggagagccactggggaggctgttgggggctgttgagacctcagatgggctcagagccatgggcagagatctctggccagcagtgccctctgccagggccgtctcggaccccaccccttctgagggaccttgctgtggtcccccggaacctgggcctggctgaaccccctcgaggcagctgcagggcttcaccagccttttctctgagctgtgcctgctgtgggtcctagcgagtttctctgtgcccggctcaagcatccgtgtgcccgcggttctgagaacggcttcacatgagaccctcaccaggaagatcttgaacaccatctgcttgacattctctttgctgatggcctggaccagtgagaactcagactccaaggtggccgtgtagcccagcctgcccaggatggcgtccagtttgtgtctggaaagcatagatcgcacccagtaggtaaagctcccagtgtacatcattgcactccagcgtaggcgactgagtgagacccctggtggagaatctgggtacagctccctgagcaccgtggcatccacgtccccgtcagagctgatgtccaagggtgggggccagtcctctgaggagctgcaggcatagcgcatcctgcggcttgagcggctgtatgtgtgctcgtccgacacgtagccgtgctcgtactctcggtgtcgacgccggcggtggtgatgatggtggtggtggtggcggtggtggcggtggcggtgccgctgaagccgggcctgcctgtccctgcggatgctgcccacaatgatggtgatgcaggagaggatgatgaccacacctatgacggcactcgccaccagcacgggggacacgagcagatggctgtgctccgagctctctgagaatgtggggtagaagtagctggtgcggttgtatcgtgctatcggcttggctgcagcgctccgctccgtgcgccgcagtgccggctccagcttcggctccagctccggttcccgccccggctccggctcccagtccggttcccgctcggaggccactgcgctcgggctcgggcgtcgc

SEQ ID NO: 10045 - RNA, 2464 nt, Homo sapiens
  source 1..2464: mol_type = other RNA
cacccggctgtgtgcacatgtgcatgtatatgtgtacataaaggggcaggagatggcaggtagagggggtgcccccgctcctggatggagagcaggcatgagagttgaccctgagctcccaacaaattagccgaaagaaaagggaggccagtagtggatcctagatggattaagggtgtactacacatccagttgtctacacatctatgccctctttatttgcactgtgataggtgaaatgggtctgaaggctgctgagggaagcggctactcagagctgcaggatgacctacccagggtcacacaactgaactgggacatgaagaggacagaaaacctaaagggaggggcccttctctgggtcggtctctgatgggcactgagcacacctcacctcactaactcttcccagcctcctgggaaggaggtctgaccatagtcactttacagatgaggaaaacgaggctcatagaggtggagtgagttgcccaaggtcacacaagccatcgatggcagggctggaatttgagaccttttggggttagcagattggctcctatgcctcacaagcaagccataggtttggccactcttcccccgtgccctgcttctcctcctgtgctgtgatcccaggtctagcacctctcccagcagtcacctcctggtggacatcacagtgagagctatttgcttattcagggtgcctgccctgtactagcgagagatcactccctcagctattgctgggatggtgtctttgggtgggtactggtgccaccagcccccactgggggtatagtgggtgctggggtgctctcatccatgcaggggagcctgggtagacctccagaatggagtgactccactttctgggctgccgtcatcaccagttggctctggccccacaagaggccctagttgtccatcttcctccacctcagggcgtgggatgcctctaggatggcctgcaggagttgagggaccaagaaggtgagggagcactcacagagctcattcctctcggaagaggtgctgggaggtgcggcgtctattctggggctggccagctccagctatgcttctggcttccggtctaagggctgccctggagattggggacctggtgtcgggcagagctggctgagaatggtgacttttctgctctcaggaactgcatccgagaccaggggctgccccctgctgcaccctgaggcggtgaccacctcacccgatgaagggccaggggccagggctgggcctgggagttggtttcccttcaggcttctcaggaaaatgtccttgggaaaccagggcatccagtgtaagacagggtcactgaagcaaggcaggacctcctcactgtccaggcatgtgctgccatggcactgggggccctagaggactggagagccactggggaggctgttgggggctgttgagacctcagatgggctcagagccatgggcagagatctctggccagcagtgccctctgccagggccgtctcggaccccaccccttctgagggaccttgctgtggtcccccggaacctgggcctggctgaaccccctcgaggcagctgcagggcttcaccagccttttctctgagctgtgcctgctgtgggtcctagcgagtttctctgtgcccggctcaagcatccgtgtgcccgcggttctgagaacggcttcacatgagaccctcaccaggaagatcttgaacaccatctgcttgacattctctttgctgatggcctggaccagtgagaactcagactccaaggtggccgtgtagcccagcctgcccaggatggcgtccagtttgtgtctggaaagcatagatcgcacccagtaggtaaagctcccagtgtacatcattgcactccagcgtaggcgactgagtgagaccctgtcctggtggagaatctgggtacagctccctgagcaccgtggcatccacgtccccgtcagagctgatgtccaagggtgggggccagtcctctgaggagctgcaggcatagcgcatcctgcggcttgagcggctgtatgtgtgctcgtccgacacgtagccgtgctcgtactctcggtgtcgacgccggcggtggtgatgatggtggtggtggtggcggtggtggcggtggcggtgccgctgaagccgggcctgcctgtccctgcggatgctgcccacaatgatggtgatgcaggagaggatgatgaccacacctatgacggcactcgccaccagcacgggggacacgagcagatggctgtgctccgagctctctgagaatgtggggtagaagtagctggtgcggttgtatcgtgctatcggcttggctgcagcgctccgctccgtgcgccgcagtgccggctccagcttcggctccagctccggttcccgccccggctccggctcccagtccggttcccgctcggaggccactgcgctcgggctcgggcgtcgc

SEQ ID NO: 10046 - RNA, 9494 nt, Homo sapiens
  source 1..9494: mol_type = other RNA
cacccggctgtgtgcacatgtgcatgtgttcatgtgtgtatgcgtgtggggtgtgtgcatgtgcactgattgtctcccttcaccagaacctaagtcccatgagatcagggaacctcgtctcttggttcctgctttgccccacgcctatgacagtgcctgacagagtaggtactcgataaatagctgctgaatgcagaacaaaggaggccccatctgggcaaccctgggggaagggggccagtggtctccaagtagacagtgtccaggggcccccaggtggagggaccccaagtccagggcggccctatcaggtgacccagctgctgtggatgagaaccctgggcatgtcagagggacatgctggtgaggttgtcctggctcaacagtcccttccggcccgcaccagtcccatgcccactgcccccagcacccccaccacccccacagtactcgtgcagcctgtgccgcagtgtgacgagggctgaccccaggcaggcgccgttgggtgcatggggcccgccaggcagctggagcagcagtgtggccacgccagccatgccatcttctgtgggctcgagagtgatgggcccagctcgcagcccagcagtggtggcggggatggctggtgggcagcagccccctcccatgggtccccagggcccaccggcccctgtcagcagcaggggtgccaggaagggctcagagcggcggaaggcgggaggtgggagcccagccggcttccaggcggaggccggggcagtagggtcaggtgggaagcagacggtgaccttggcgaaggggcggctggccatcttggtcatctcctgcaagtgccggcgctgctcctgccgctggtccagagcctgcttggccttccagaggagcacacagagtgagaggaagaggaagaagcaggagaagaagacggagaagaagacaaacaggtcaatgtgggcctggtcctgccggaagaagagcaggccctgcgagtcggctgagccgttggcgccgggcccacttgggtctcccacgcccagcagcagcaggtagaagcggctcgacttgagggcatggtgctcgtgtgggtaggtgatgaccagccggtcccgcacgccgcggaccaccagcactgccgacggctccgtcaccgtcacgtaggtaatcaggccccgcggccatacctcccgtacccgtggctctgctggggcgcccggcccactgctggcccctgctcctcctggatccccagccccccggggcccaccatctgcagggggtggtggaggtggtggggctgggggtggctggatgtgtacagtatggacgccagtgtcaggggccacacggaccacgaaggtgtcataggaggtggagacatagaggtccacggccccgaaggtcacgtccagcgtcaggcggatgtccacgttggtgaatttgggctgcacgccaaagaggacagtgcggccggggcctagcgcccggcgtttgggctcatggaagcagttggtctgggacgtggggtccaggcagcactcctgctccaccgagatgaggcggtagcactgctggccgcccagcggactcccgtgaaatgattcccggcacttggcgcactggtacttgtagcagtctcgacggtcactgggggagctgccctggcatgtgcccgtctctgtgttattctgacatggacagcccgtcccatcctgctcgttacatgtgtccgcgtggccattacactggcatttggtgcacttcccgtccaggaggaagtagccctgcaggcagctctcgcatttctccccatagctgttattctggcagttcacgcacacggcctcgtcttcactaggaccctctgtcacccagttttcaatctcctctgggtccagtgagtacttctttggctctcccttggacatttgtaactccttcctggagatgcagatgtggctatttccacgacaaaaggcgtggcagggccggcaggtcccgcctccgacagctgaacccacaaacagcgggaggcactgctcacagtggctgcccttggtgtggttgcggcagagcaagcagtggtcacgcgccccaacaccagcgcattcactgtggcggttgcagcggcattccgtggagcagttgcggcccacaaagccaaagtggcagcggcagtggtcgggctccacacatgagccgttcacgcagccctgggcgcacacagggcggcacagccctgtcatgttgtccatggtatagccggtcttgcagctgcactcatagccgtggggctggtcgtggcaattctgcgtctcgttgcagtcgtggtgcccgtttgcacactcgtcctcaggggggcaggacaggaaggcccaggaggcccccggacgcccacatgtcagcccatcacgggggccgctgagtccaccctccatgcagcggccacccccatcctggcccccccaggcacaccagccgcaatgggggcgccgcaggcacaaggcgcactgagttgcctgagcacagcccagggagcagctctcaggtccccggagcagccgcccacagcctccggccatacatcgcaggggcaggtaggaagggctcagacactgctgcaggctgctgctccaaacacagtgctgccagcccccatctgctcccttagagtccaggcaggaggtacagttgggtaggaggtgacaaggggtggggcagggcagtgggggtgatgattccaccggcatgggggacacattcagcagagagtggctgaagcacgtccagtcataggtgggctgcacggagaggatgcggcgggtctcccctgtcctcttgaactgccgcgtccacatgcacttgccctcccgcgtgcactgctcgcagtcagcagccccgcacgcagcctcggagcagttccctgcccagaagacctctcgctggttgatccgacagtcattctcagaggtgcaggacccattgcgtccaatgcaagcaccttcggggcagttggtacaccacttacagcggggggtggacgcctctccatctccaggttgcagggtccgaggatggcgggccaggcactcactgcaggtccggagacgtcgacattcctccggggagcgaggcattggggagcagggggagcccccgcagcccagcctgtgggcctgatccccggacaagcaggccccatggcaccaggtgcaggccccagactggttacaagcttcaggtgaggacagcaggcggcaggggtcagggggcagggtcagtgccagcaggcggcccagggccactcccccgaaacccccagagatatacaggcggctcccgactgctgccacagcatgggccacagactcctccattgggggccccacagaggccgagcgggtgaggtcgggcagaagccaggcattgcagttgacctggtagagcagaacgtcgctgctgaactcgtcagggtccgagcgccccccaagaaccaccatggtgtcccctaacagggctgaggcgtggaaaagccgggggcggggctccttcaggtgaggtgagatttcctccaggaaacctcctgtaccagcaagagcagcccacagagccatcttcttcctgacttcccggaacccccatgacccaggctgctccccaggaacttggcccagaccccgagatgagccacgcacattcctcatacgatctcgctttgccccctgagaaggggccagcagactccaggtgcggtcaggacagtgcagggagtagagctcgggggatggggccgccagctccacatggaatcggaaccccccaaacacgtagagggagtcggtggcctcgtggtagacagcagagtgaccatagagacctgtggggggtgtcccactctgggctcctgacacccaggtgccggttgccagctggtactccagcagctgctggttgaagccattttccggggagtaaccgcccaccaggagcagagacaggcctcggcgggcagtaagggtgtgaccagcaacggctggcagctccacggtctggggggccttctcctgccgccattgcagggtggtgaggttgaggacccagaaatcacgggtgacgcctccagcggtaagtccccccagcagatacatggcaccacggccagcgggcacatatgcggctgcatggaaggagcggggcgatgggcctgggcccccgtcctcggctcccgccagcatctgtgtccaccgccgctcactcactgagtacctgtacaggtttcccagcagcccctggggcaggcccaggcccccaaacatccacaaggtggcatcgggtccatccaccatggtgtggcccaggcggtgcaggaagcggctggcagtgtcggctgagaggcggctgtccatgagggtctcccagaccagctgcccgccatccagcttggtggcgcagtcggggcccccgaagccctcggcacagatgcacacacccaggctctggttacaagttcctgccccagtgtgggcattgcagttctcaggacacagagccatgcggcagtgtgggccagcccagccctgaggacatcggcagagccccgcacctgcagcaccgtcctggggcacgcattcctgggggacgggacagctcccggggccccctgacccacagcgggcagagcccaccgaagcattgaagccccaggatgaggagccattggcctcccagtgcagcacgagcagcccagacagggcctgaacagtgaggggcctgtcccgtcgctggccgcagaaggcagctatgaggctgcggtccgactggacaacaccagtgtccaggaagcgtgggaatccatcaaacgccaggacgtagctcagcgtgcagggggtgctgctgtcgggggagaaggtgagggtgagtgggggacagagggtcccgggagcacagggctgtagctcctcagtggccgagacaacccacacacagtaggacaggccaggcccggctcttgcagccccgccacctggaggcagcagccccccgacccggcgtgagcccagtgccactgaggacacgttggtgaggagggcgcgacccccacactcccgaaagcaggaaccaccggcccggggatccccataatagcctggggagcagagctggcagtgggcaccctcggtgtggtcctggcagaagcagagcccactgaggttgtcgcagtggccacggcgtgggtccccgtgcccgttgcactggcagggccggcagcccctagagcctgtggcgttgccgaagctgccgggccggcatcgttcgcagtgctccccccatgtccagtcctggcactcgtcgcagaagccagggccccgcttgcggcagtggctgtggaagctgcagccacagtcccgggagcagcggggggctggcggacccggggcgggtgtgggagggggcaggtctgatgtccagcctaggtcacacacgcaggtaaagtccggggggccactgcacacaccatggccacagtcctccaagcacgtgcggttgcagtgtgagatgccatcaccctggtagccccgctggcagtgacactcgtagctgaggggcgtgttcaggcaggtcgcccgcgggtggcaccgggccaggcccaggcgacactcatccacgtcaggacagcgggcgtatgcccagcgggcagggagggccacgggaagccccaggccctcccccacccacagggagcagttacccccaccgaggggccctgagaagtccccctgtaggcaccgtcccagtgtggggttgtcctcattgccacaccagccacactcgtggctctgcagacactcatggcaggtcaggaagccatcgcagctccggcaccgtggctccgagtgtacactgtcgtcccagcctcgacagcccccgtgtgggtaccgggccaagtaggcagcaaacaggaagcaggtgtgggtggactggcaccaggcgcactggctagagttggccaggcagtcctcacaggtcagtcgctggctgcagagcgggggacactcctctggactcttcagggcaccccgaccccggccccgccggctgcatgccgcgtcccctttgcggctggtgctctgatgccactcacagaaggggtcctgggtgcaggcgtggcagtcccgatgctcctcgcagagtgggcagagggtaggcaccagcaccagcagggacccaccagccccgtcatccccgcaatgggctccgccctggcgcaggtggcaggtggcactggtcaggcaccagccacagccctggtctgccaagcagcccaggcaggaagaataggaggtgcaggacgacgagcggtagggctccaggaagaagaaggagatctcgctgcctcctggcacaccagtccgatcccacagcagagttagctcgctgtgcccagggcctgccgagccattgagctggccctggatctctactgcatacttgtggtcccgcccaggcagagggaagaggcgagcagacccagggcgctgcagccgccgcgtctccttctcctgatgagccacccagcgccccacctcctccatgttctccgtgtcagggccacgggccatccgggccaggacgtgtaggcgctgggcccgcgtccacacggccacgtcctcagcccctggtccacctggccctccaggcagcattgggtagatgaagccacggtagaccagggacacatctgtctctgcgctgggtgttagggtgatggtcgtgctgcggacaattgagaccttgtcaggctgggaggtattgggcggctgctgaaaggtgagcaagtgcaggccaggcaggaagctctgggtgacgcaggcctccagggacgtgacgaagacaggcgcaggcccccaccagcccacagtgcctgagatctgctcccctcggcagcgggcctgctcaggcctagggaggcagctctcattgtgcacgcaccagcccagggtgccaggtccccgtggaggggctgtggggctgctgaaggccaggcaggcctggcagtcacccaggaggcggcccaggcccaggcagctggcggctggacaagcccccaagggggtcccaggagggggtgcagcttggcaggctccttggcaccaactgcattccgggtcccgggagcagacgctgtggtctgtgtacatggagcagtagtccaagtggtagtcaggggcaggtgcctggaacacaaaggggggcaccttgtacgccatcaagtccccacggggccggccgctgtaccccccagccaccaacaggacgctgccaccaagcaccgcagctacatgtgagtaccgaccactgggaggcgctgctcggccctcaggggttcctggcggggcaagctcagctcctgacacccattgatggcagccaaggtggtagaagaagatgccatcttcgtagcacttttcctcctggtaatgggtgtgcacattgcccccatagaccaccatgtaattgcccagaacactggctgtgtggaaggctcgctcccttgggccctgaagcccatcccgccccttcagcgtcgtccacacatgccgatccacgtggaaaagctcagtggagttcactcgcacagagaaccgggcagtggagggccggtgtccaccatggaccagcagggcacgggagggggcatggaacaccatggagtggccagtggcagcagggggccgtccgcctgccggaatcacctgctcccaatagcccccgctggtgctgtcaaggcggaaacggaagaggccagaggagaagaggtcgtgcggggtgcggcctccagacacatatagccagacatcatccaccagggcagccgcgtgacctgccaggcctgggggccccgaggagctggaggcaggtggtgccaggagctcccagtggcccctgcccagtggactgaaggcccacacgtcgttggtgagcgagccgtcagccagctcaccacccatcagtaccagggagccggcccaggccacggccacatgggagtgacgggcagccggggcaggactcaggtcccaagactcccaggtgttggcggagaagttgtataggacgaggtcacccagggcattgttgaggtcctggcctccgaaaactgccagcagccctggtggggacaggaaggcgccagctgccccaatacgggcagagaaggcagggtccctggcactcacgttgtgccaccacccagccccctggttctcccacaggtgcaggtcacaggcacgtcccaagaagccaggctcacagcggcatggtcccaggggcgaggcgcaggtgccgtggctgccacagtaggctgagcactcctgcaggccacagtcaggacccccccagcccggctcgcaggcacacacacccggtggctggcactgcccgtggctctggcagccacccgggcacagggagaagcggaatgaggcgttaaagcccagcaggttgtagttggcatcactgaagaggtgcagcagcatcttgcctgaggaagcttcgatgggcggaggtcgggtgctcccacttagactggcaagcagcggccctcgcggggagtcaccgtcatacacgaacaggtagtcatacgtgcactctgtgtccaggaaaaggaagtccagcaggatccggtgctgggggcttggggcctcgatgagccactcgcagttgccattgacgctgtagttgcccgcaccatccgtcacgaagcctggcgcctcccgcagcacctgccgctgccccttgcagtcccccgcccgggccccaggggacagcgaccccagcacggccaaggccaaaaccagtgccatggccagaaccttgcccagggccatcgccgcctcctgcactgacccttagagcggggacaggccgtaaaaacctggagaggaccctctacccggggtgaggccctgcaaatgcgacctctataggcataacatgaccttgtagatcgaagaggtcccggagacccggcagtcccggcgaagggtacggccactgctgacaggctctggaagccgagggctgagccctatagagcgatggaaggccctgtatatggagtcattatggacggggccgaaccctagggaccgtaggagtcccctatagacacagggctccatagggggccgatcccatgaacagtgcccagcattacggactcaggctgctgcaggccaaacggaccttatagacgggtgggtccccagggggcgaagggctctacggcccggcaggagcctccatagaggctgcgggccgggacaggctaggttcggatggtccaggagagactcctccagccgggggcggggcgcgagcgggtgccgggggcggagcccgtcttcaggggttcgggcctggaccccacagacccaatccctttgctcacccaccctcgcctccctccgaagccggatgggccagatcagagagac

SEQ ID NO: 10047 - RNA, 9293 nt, Homo sapiens
  source 1..9293: mol_type = other RNA
cacccggctgtgtgcacatgtgcatgtgttcatgtgtgtatgcgtgtggggtgtgtgcatgtgcactgattgtctcccttcaccagaacctaagtcccatgagatcagggaacctcgtctcttggttcctgctttgccccacgcctatgacagtgcctgacagagtaggtactcgataaatagctgctgaatgcagaacaaaggaggccccatctgggcaaccctgggggaagggggccagtggtctccaagtagacagtgtccaggggcccccaggtggagggaccccaagtccagggcggccctatcaggtgacccagctgctgtggatgagaaccctgggcatgtcagagggacatgctggtgaggttgtcctggctcaacagtcccttccggcccgcaccagtcccatgcccactgcccccagcacccccaccacccccacagtactcgtgcagcctgtgccgcagtgtgacgagggctgaccccaggcaggcgccgttgggtgcatggggcccgccaggcagctggagcagcagtgtggccacgccagccatgccatcttctgtgggctcgagagtgatgggcccagctcgcagcccagcagtggtggcggggatggctggtgggcagcagccccctcccatgggtccccagggcccaccggcccctgtcagcagcaggggtgccaggaagggctcagagcggcggaaggcgggaggtgggagcccagccggcttccaggcggaggccggggcagtagggtcaggtgggaagcagacggtgaccttggcgaaggggcggctggccatcttggtcatctcctgcaagtgccggcgctgctcctgccgctggtccagagcctgcttggccttccagaggagcacacagagtgagaggaagaggaagaagcaggagaagaagacggagaagaagacaaacaggtcaatgtgggcctggtcctgccggaagaagagcaggccctgcgagtcggctgagccgttggcgccgggcccacttgggtctcccacgcccagcagcagcaggtagaagcggctcgacttgagggcatggtgctcgtgtgggtaggtgatgaccagccggtcccgcacgccgcggaccaccagcactgccgacggctccgtcaccgtcacgtaggtaatcaggccccgcggccatacctcccgtacccgtggctctgctggggcgcccggcccactgctggcccctgctcctcctggatccccagccccccggggcccaccatctgcagggggtggtggaggtggtggggctgggggtggctggatgtgtacagtatggacgccagtgtcaggggccacacggaccacgaaggtgtcataggaggtggagacatagaggtccacggccccgaaggtcacgtccagcgtcaggcggatgtccacgttggtgaatttgggctgcacgccaaagaggacagtgcggccggggcctagcgcccggcgtttgggctcatggaagcagttggtctgggacgtggggtccaggcagcactcctgctccaccgagatgaggcggtagcactgctggccgcccagcggactcccgtgaaatgattcccggcacttggcgcactggtacttgtagcagtctcgacggtcactgggggagctgccctggcatgtgcccgtctctgtgttattctgacatggacagcccgtcccatcctgctcgttacatgtgtccgcgtggccattacactggcatttggtgcacttcccgtccaggaggaagtagccctgcaggcagctctcgcatttctccccatagctgttattctggcagttcacgcacacggcctcgtcttcactaggaccctctgtcacccagttttcaatctcctctgggtccagtgagtacttctttggctctcccttggacatttgtaactccttcctggagatgcagatgtggctatttccacgacaaaaggcgtggcagggccggcaggtcccgcctccgacagctgaacccacaaacagcgggaggcactgctcacagtggctgcccttggtgtggttgcggcagagcaagcagtggtcacgcgccccaacaccagcgcattcactgtggcggttgcagcggcattccgtggagcagttgcggcccacaaagccaaagtggcagcggcagtggtcgggctccacacatgagccgttcacgcagccctgggcgcacacagggcggcacagccctgtcatgttgtccatggtatagccggtcttgcagctgcactcatagccgtggggctggtcgtggcaattctgcgtctcgttgcagtcgtggtgcccgtttgcacactcgtcctcaggggggcaggacaggaaggcccaggaggcccccggacgcccacatgtcagcccatcacgggggccgctgagtccaccctccatgcagcggccacccccatcctggcccccccaggcacaccagccgcaatgggggcgccgcaggcacaaggcgcactgagttgcctgagcacagcccagggagcagctctcaggtccccggagcagccgcccacagcctccggccatacatcgcaggggcaggtaggaagggctcagacactgctgcaggctgctgctccaaacacagtgctgccagcccccatctgctcccttagagtccaggcaggaggtacagttgggtaggaggtgacaaggggtggggcagggcagtgggggtgatgattccaccggcatgggggacacattcagcagagagtggctgaagcacgtccagtcataggtgggctgcacggagaggatgcggcgggtctcccctgtcctcttgaactgccgcgtccacatgcacttgccctcccgcgtgcactgctcgcagtcagcagccccgcacgcagcctcggagcagttccctgcccagaagacctctcgctggttgatccgacagtcattctcagaggtgcaggacccattgcgtccaatgcaagcaccttcggggcagttggtacaccacttacagcggggggtggacgcctctccatctccaggttgcagggtccgaggatggcgggccaggcactcactgcaggtccggagacgtcgacattcctccggggagcgaggcattggggagcagggggagcccccgcagcccagcctgtgggcctgatccccggacaagcaggccccatggcaccaggtgcaggccccagactggttacaagcttcaggtgaggacagcaggcggcaggggtcagggggcagggtcagtgccagcaggcggcccagggccactcccccgaaacccccagagatatacaggcggctcccgactgctgccacagcatgggccacagactcctccattgggggccccacagaggccgagcgggtgaggtcgggcagaagccaggcattgcagttgacctggtagagcagaacgtcgctgctgaactcgtcagggtccgagcgccccccaagaaccaccatggtgtcccctaacagggctgaggcgtggaaaagccgggggcggggctccttcaggtgaggtgagatttcctccaggaaacctcctgtaccagcaagagcagcccacagagccatcttcttcctgacttcccggaacccccatgacccaggctgctccccaggaacttggcccagaccccgagatgagccacgcacattcctcatacgatctcgctttgccccctgagaaggggccagcagactccaggtgcggtcaggacagtgcagggagtagagctcgggggatggggccgccagctccacatggaatcggaaccccccaaacacgtagagggagtcggtggcctcgtggtagacagcagagtgaccatagagacctgtggggggtgtcccactctgggctcctgacacccaggtgccggttgccagctggtactccagcagctgctggttgaagccattttccggggagtaaccgcccaccaggagcagagacaggcctcggcgggcagtaagggtgtgaccagcaacggctggcagctccacggtctggggggccttctcctgccgccattgcagggtggtgaggttgaggacccagaaatcacgggtgacgcctccagcggtaagtccccccagcagatacatggcaccacggccagcgggcacatatgcggctgcatggaaggagcggggcgatgggcctgggcccccgtcctcggctcccgccagcatctgtgtccaccgccgctcactcactgagtacctgtacaggtttcccagcagcccctggggcaggcccaggcccccaaacatccacaaggtggcatcgggtccatccaccatggtgtggcccaggcggtgcaggaagcggctggcagtgtcggctgagaggcggctgtccatgagggtctcccagaccagctgcccgccatccagcttggtggcgcagtcggggcccccgaagccctcggcacagatgcacacacccaggctctggttacaagttcctgccccagtgtgggcattgcagttctcaggacacagagccatgcggcagtgtgggccagcccagccctgaggacatcggcagagccccgcacctgcagcaccgtcctggggcacgcattcctgggggacgggacagctcccggggccccctgacccacagcgggcagagcccaccgaagcattgaagccccaggatgaggagccattggcctcccagtgcagcacgagcagcccagacagggcctgaacagtgaggggcctgtcccgtcgctggccgcagaaggcagctatgaggctgcggtccgactggacaacaccagtgtccaggaagcgtgggaatccatcaaacgccaggacgtagctcagcgtgcagggggtgctgctgtcgggggagaaggtgagggtgagtgggggacagagggtcccgggagcacagggctgtagctcctcagtggccgagacaacccacacacagtaggacaggccaggcccggctcttgcagccccgccacctggaggcagcagccccccgacccggcgtgagcccagtgccactgaggacacgttggtgaggagggcgcgacccccacactcccgaaagcaggaaccaccggcccggggatccccataatagcctggggagcagagctggcagtgggcaccctcggtgtggtcctggcagaagcagagcccactgaggttgtcgcagtggccacggcgtgggtccccgtgcccgttgcactggcagggccggcagcccctagagcctgtggcgttgccgaagctgccgggccggcatcgttcgcagtgctccccccatgtccagtcctggcactcgtcgcagaagccagggccccgcttgcggcagtggctgtggaagctgcagccacagtcccgggagcagcggggggctggcggacccggggcgggtgtgggagggggcaggtctgatgtccagcctaggtcacacacgcaggtaaagtccggggggccactgcacacaccatggccacagtcctccaagcacgtgcggttgcagtgtgagatgccatcaccctggtagccccgctggcagtgacactcgtagctgaggggcgtgttcaggcaggtcgcccgcgggtggcaccgggccaggcccaggcgacactcatccacgtcaggacagcgggcgtatgcccagcgggcagggagggccacgggaagccccaggccctcccccacccacagggagcagttacccccaccgaggggccctgagaagtccccctgtaggcaccgtcccagtgtggggttgtcctcattgccacaccagccacactcgtggctctgcagacactcatggcaggtcaggaagccatcgcagctccggcaccgtggctccgagtgtacactgtcgtcccagcctcgacagcccccgtgtgggtaccgggccaagtaggcagcaaacaggaagcaggtgtgggtggactggcaccaggcgcactggctagagttggccaggcagtcctcacaggtcagtcgctggctgcagagcgggggacactcctctggactcttcagggcaccccgaccccggccccgccggctgcatgccgcgtcccctttgcggctggtgctctgatgccactcacagaaggggtcctgggtgcaggcgtggcagtcccgatgctcctcgcagagtgggcagagggtaggcaccagcaccagcagggacccaccagccccgtcatccccgcaatgggctccgccctggcgcaggtggcaggtggcactggtcaggcaccagccacagccctggtctgccaagcagcccaggcaggaagaataggaggtgcaggacgacgagcggtagggctccaggaagaagaaggagatctcgctgcctcctggcacaccagtccgatcccacagcagagttagctcgctgtgcccagggcctgccgagccattgagctggccctggatctctactgcatacttgtggtcccgcccaggcagagggaagaggcgagcagacccagggcgctgcagccgccgcgtctccttctcctgatgagccacccagcgccccacctcctccttgtcaggctgggaggtattgggcggctgctgaaaggtgagcaagtgcaggccaggcaggaagctctgggtgacgcaggcctccagggacgtgacgaagacaggcgcaggcccccaccagcccacagtgcctgagatctgctcccctcggcagcgggcctgctcaggcctagggaggcagctctcattgtgcacgcaccagcccagggtgccaggtccccgtggaggggctgtggggctgctgaaggccaggcaggcctggcagtcacccaggaggcggcccaggcccaggcagctggcggctggacaagcccccaagggggtcccaggagggggtgcagcttggcaggctccttggcaccaactgcattccgggtcccgggagcagacgctgtggtctgtgtacatggagcagtagtccaagtggtagtcaggggcaggtgcctggaacacaaaggggggcaccttgtacgccatcaagtccccacggggccggccgctgtaccccccagccaccaacaggacgctgccaccaagcaccgcagctacatgtgagtaccgaccactgggaggcgctgctcggccctcaggggttcctggcggggcaagctcagctcctgacacccattgatggcagccaaggtggtagaagaagatgccatcttcgtagcacttttcctcctggtaatgggtgtgcacattgcccccatagaccaccatgtaattgcccagaacactggctgtgtggaaggctcgctcccttgggccctgaagcccatcccgccccttcagcgtcgtccacacatgccgatccacgtggaaaagctcagtggagttcactcgcacagagaaccgggcagtggagggccggtgtccaccatggaccagcagggcacgggagggggcatggaacaccatggagtggccagtggcagcagggggccgtccgcctgccggaatcacctgctcccaatagcccccgctggtgctgtcaaggcggaaacggaagaggccagaggagaagaggtcgtgcggggtgcggcctccagacacatatagccagacatcatccaccagggcagccgcgtgacctgccaggcctgggggccccgaggagctggaggcaggtggtgccaggagctcccagtggcccctgcccagtggactgaaggcccacacgtcgttggtgagcgagccgtcagccagctcaccacccatcagtaccagggagccggcccaggccacggccacatgggagtgacgggcagccggggcaggactcaggtcccaagactcccaggtgttggcggagaagttgtataggacgaggtcacccagggcattgttgaggtcctggcctccgaaaactgccagcagccctggtggggacaggaaggcgccagctgccccaatacgggcagagaaggcagggtccctggcactcacgttgtgccaccacccagccccctggttctcccacaggtgcaggtcacaggcacgtcccaagaagccaggctcacagcggcatggtcccaggggcgaggcgcaggtgccgtggctgccacagtaggctgagcactcctgcaggccacagtcaggacccccccagcccggctcgcaggcacacacacccggtggctggcactgcccgtggctctggcagccacccgggcacagggagaagcggaatgaggcgttaaagcccagcaggttgtagttggcatcactgaagaggtgcagcagcatcttgcctgaggaagcttcgatgggcggaggtcgggtgctcccacttagactggcaagcagcggccctcgcggggagtcaccgtcatacacgaacaggtagtcatacgtgcactctgtgtccaggaaaaggaagtccagcaggatccggtgctgggggcttggggcctcgatgagccactcgcagttgccattgacgctgtagttgcccgcaccatccgtcacgaagcctggcgcctcccgcagcacctgccgctgccccttgcagtcccccgcccgggccccaggggacagcgaccccagcacggccaaggccaaaaccagtgccatggccagaaccttgcccagggccatcgccgcctcctgcactgacccttagagcggggacaggccgtaaaaacctggagaggaccctctacccggggtgaggccctgcaaatgcgacctctataggcataacatgaccttgtagatcgaagaggtcccggagacccggcagtcccggcgaagggtacggccactgctgacaggctctggaagccgagggctgagccctatagagcgatggaaggccctgtatatggagtcattatggacggggccgaaccctagggaccgtaggagtcccctatagacacagggctccatagggggccgatcccatgaacagtgcccagcattacggactcaggctgctgcaggccaaacggaccttatagacgggtgggtccccagggggcgaagggctctacggcccggcaggagcctccatagaggctgcgggccgggacaggctaggttcggatggtccaggagagactcctccagccgggggcggggcgcgagcgggtgccgggggcggagcccgtcttcaggggttcgggcctggaccccacagacccaatccctttgctcacccaccctcgcctccctccgaagccggatgggccagatcagagagac

SEQ ID NO: 10048 - RNA, 2045 nt, Homo sapiens
  source 1..2045: mol_type = other RNA
cacccggctgtgtgcacatgtgctgctggtggttggtgttattgttattatcaggagtggcgtattcccagcctctggaagctcacctcgtggttttctttcttcttccacttttcgttttttagatcatgtctgcccttagcctgacatccccgccatgtagggctccaggactgctgtggcctcagcccttccgggctccaggaggccctgattcattgctctcccctccccccttggctggcctaggtgccttgtcctctttcttgggacggtgctcactgacgggccccatgggaggagggagacacggccagctgccatgcgggaacagctgccacagcatcgcctcctccagacattgctcaccacccctggctttcctgagcttctcaccagccctggtggaagtgagcaaacatgattacttattcttgtcttccccatcaggaggccagggtgggggaaaggcagtgtgccactgagttgttggtcctctaacttagtgctggtcgcccgcatgtgctctagggcctcggggcacggtgctgggacagctcagctggcagacctaggacagggctggaaggtggggggcagggctggggtcagaacttttctcccttcttccctccggactcagggaggtcccttgggcaaattccttgtccagacagagatgtgtggggcgagagacactcagtctccttaggagcagtgagcagcggggggcccaagacaacagccccctgtggccgcctccagccccaggacagtggcctgagccctgggtcaccatgctcactccacccagcgcagaattctccagcgcccagccttgcagaggcaacgcggctccgacaggacctgtaacctcttcctgccgcttctttgtcatgcaaccagcccttccctccaaatctttcaaaatcctcttccccaggggtcactgccctgatcttcggagcaggctgtggacatggactcactctgctgagctcttcctcctctgtgtaccgaggccacagcccccactccgatcccccacgcagcctctgcctgcgcttttgtcccttgtccttacctttatcaagctcaagggaccccgtaaccgcacgccctcctcagggccttttcattggaattcccacactctctgcatttctgaaggactggttgaaaccgcagcgttcttctaagtggtgagctccccgagtgaatcaaaatcacacttgattcccccaaaatcccatttgtcaggagtgcggctgctgcagaaagtgtctctggagcttgggaagcaggcgcggggccactctaaactctcctgtgctcatcacgcgccctttctgcatcctgcgggcacgttggtcggacccaggtggtgccaggcctgtagcaggtaccctggatcggatcggctgctctgctccacgaggctcccagcaccatctcagcaggtagctgatgtggagtctctgtcacctccagggcagccagtgcccctcactggaagcctctcgatgtcagagaattccccgctgtgtgttcctggcattgttgtggggacgcacctcctctgtgcttctggatggcagggaggtcccacgtgctccataaattccctggacgaggctcgagtggatcatagcgtcgggtttggagtccaccttgtcttccgtagtcactcacacttacgcagtggcacaggcttctggcaggctatgtgtgtggatcctgtatttctgagaatttattccttctgagaggctggagatgaaggccccaaggtctgggaagaaggaaatccctgggttcttgcagaaacttcctaacaggtgtgtccaggaagcacttcagatgttttctctgctgcttctggttatcttttaaatcagagatgggggagtcaggccccatttaaacgtctcctggagccgagtgggaggacagctcttgggcgttgcctgggctggtggggccagctccctcctgactgccccgctgtctgccaagagcatttttcccatttttccagagtccag

SEQ ID NO: 10049 - RNA, 1613 nt, Homo sapiens
  source 1..1613: mol_type = other RNA
cacccggctgtgtgcacatgtgctgctggtggttggtgttattgttattatcaggagtggcgtattcccagcctctggaagctcacctcgtggttttctttcttcttccacttttcgttttttagatcatgtctgcccttagcctgacatccccgccatgtagggctccaggactgctgtggcctcagcccttccgggctccaggaggccctgattcattgctctcccctccccccttggctggcctaggtgccttgtcctctttcttgggacggtgctcactgacgggccccatgggaggagggagacacggccagctgccatgcgggaacagctgccacagcatcgcctcctccagacattgctcaccacccctggctttcctgagcttctcaccagccctggtggaagtgagcaaacatgattacttattcttgtcttccccatcaggaggccagggtgggggaaaggcagtgtgccactgagttgttggtcctctaacttagtgctggtcgcccgcatgtgctctagggcctcggggcacggtgctgggacagctcagctggcagacctaggacagggctggaaggtggggggcagggctggggtcagaacttttctcccttcttccctccggactcagggaggtcccttgggcaaattccttgtccagacagagatgtgtggggcgagagacactcagtctccttaggagcagtgagcagcggggggcccaagacaacagccccctgtggccgcctccagccccaggacagtggcctgagccctgggtcaccatgctcactccacccagcgcagaattctccagcgcccagccttgcagaggcaacgcggctccgacaggacctgtaacctcttcctgccgcttctttgtcatgcaaccagcccttccctccaaatctttcaaaatcctcttccccaggggtcactgccctgatcttcggagcaggctgtggacatggactcactctgctgagctcttcctcctctgtgtaccgaggccacagcccccactccgatcccccacgcagcctctgcctgcgcttttgtcccttgtccttacctttatcaagctcaagggaccccgtaaccgcacgccctcctcagggccttttcattggaattcccacactctctgcatttctgaaggactggttgaaaccgcagcgttcttctaagtggtgagctccccgagtgaatcaaaatcacacttgattcccccaaaatcccatttgtcaggagtgcggctgctgcagaaagtgtctctggagcttgggaagcaggcgcggggccactctaaactctcctgtgctcatcacgcgccctttctgcatcctgcgggcacgttggtcggaccctgggttcttgcagaaacttcctaacaggtgtgtccaggaagcacttcagatgttttctctgctgcttctggttatcttttaaatcagagatgggggagtcaggccccatttaaacgtctcctggagccgagtgggaggacagctcttgggcgttgcctgggctggtggggccagctccctcctgactgccccgctgtctgccaagagcatttttcccatttttccagagtccag

SEQ ID NO: 10050 - RNA, 6329 nt, Homo sapiens
  source 1..6329: mol_type = other RNA
cacccggctgtgtgcacatgtgcttgtgtgtaggtagacacatatacaccatacacgcacacacacacaccagcccctgtagagcctgagctagtccacaggactgttgcaataggaggagcaggcaagggcagaggacagcccctctccacggagaggtacctgtcacgagtactctgatgcaaggccactgaagggcgttaggcttgggttgccctctcatctcagccacctgtttggtaacagaaggaatcactgaacgaacagccactaagctagtattgcactttatgccttacaaagcatctcagatacattcatacgccatgaacaggaggcagtaaacaaaacagggacttcagcgtccaactgggctggaatcccaactccgctccttcctcgttctggggccctggggacgtcacggagcctctccctgcctccgcgttccacgtctgcaccatgagcacggctaagccaagtggccacgcggttccctcccaccacactggagggcaagcccacgttggagtcccctccccctcacccccagggcctgggacagcaccaggcgagaggggtgggtcagtaagggtttgaggagtgggcaggggacagggggttctgaggacatccagcccagtgcctggaaacagccacgaggaaaggtgctcggtgcaccagagtcgtgccttctcttcccactgcaacaaccaagcccggtttctgccccatgggtgtggtctgtccctgatgtcaggctgggggaatgactttttgtgggtttctaagatgagttttcacctcaaagctccatgtaccatttcctggtcctgaaggcgcctcccccaggtgatgtaatccaattctggcactgactgcataaaactttgcacagttactccccttcctgggcacagcttcccacttcacccacacagggagtttcggagaattcaatctccagtggatattcagccagaggagaagaaagagaggcacaaaatgctttggatgaggacaaaggcaaaaggccccagcagtttccctgaaacctccattttcacctctactaaccactggggcatctgcaaatcttttatccaaggtttaatccttccttctaatggaagaaactcaaccagagatgaaaggaatatcttggtcaatgcattcagaaattactgaaacaaattagatttggggagttggtctgggtttaacgtccaacatgtgaaagatagcacattgccgtgtgtgtcttaaccacagctggttagaaaagtaaaccagtgagttgcttgatattatcttaggccattggaataaggcattttaccaaactaccttaacacaaaaagcagtggggaaatatctgggaatctaaacaatggcatttgagccaatgctgccaaaggttacgaggaaaatgcccagccagggacccttgctgaacctggaagagggaggccggctgcacctaggacagatgcatcctctcctcccttggcggtaggctttcctccagtctacgggggagggctgagcaaagccatcctggggcgtcaactgcagaatcctcacctactccagttcacccttcaaaaaataaacccacatggtctcacatatccattcccttcttgcagcctaacagccctcatggttcccaagctcttcccccttagaattacccccatcaagttcctacgagagtcattccatcagagggcttaggtgctctccgaaaccagatttaaaatctagaggcatctcactgtttcctcctgaaattgatgaggcacagcaagcggtctcagcaaacgagaccaaagctgcttctgaggcagggctgtgggccccatgcagtgcagttcctggcagacacacccctattagggccatgaagccacaacactaatccacaatggggaaggctcacctggagggaatgggcgttttcaacactgacctcactcgatgtagttctgagtcatgagcaaggacttttgcctttttccaattctgcatttcaccaggctattcctaggtaggtcttccctatgtgcaatgtcttacaagaagatctattttgaaattaaatgaggactttttataaaggctaagtttgactctggttaaaaacttaatctggaaggcaatgccatatttgtatagaacaagcacacttaaaattacactttaatatctatctcaattgtgtttactaaaaaagatctagcagtaaaaaaggaatctctaagaattagcaaactaaatccatgtgtaaataaaattcagacccttttcgttctttcgaagtgggaaataagagcttcagggacatcgccaaggaatcccaccacctttgagctggcatggccttgggcatgatgtactgtaactatttacagatgaggaaaaatgtagcttagaaaggttcactgattttcccgcaaaaacacagcctttccatcggaagccctgattctaggagaatgatattctagagggagtaaacaatggcattttcctaaaggtggacttctttggccagaatcaccttctctgcatgtagtcaaactgcttctgagagctgacaaactcacaggcagccttgttgtgaattcaaagaccacttgacctccagataggcacctgtttctgccctagcgggatttgacttatgtgattcagtcataggaaagaagcggtttccaacgtgcaaagtttacacaggcctaacactgaggcggtgatgcagctgtgaggtcgcaaaacccagagatgaaatctcccaccactcgaagtgcgttgtttgatcaagtttcaaatgcctccacatgctgaagtctactgacttcgtcctaagcccttggattctgatgccatctcgttggcctcctcccctcttgcacagttagcccatctttcactgctggccactcctgctgagccaaccctcaaaggtcgtgcctgaatttccctaagccccattcttccaggttcagtggaggcagctgaggtgatacaggaggaaagggaagctgtttgtttgtttgtttaaatcaacctaggcaaaattaaaggtagtcagaaagttaggaagaaacaaacaatatatttcgcttaaaataagaagcacgtggaaaaagaaagactttgaaagagttggccaatgtcttctcacaattttttgtatagcttttaaaaatgtctgcatggctcagtggagatggtgtccacgtcttccctccacctggaacctgcattcaatccttcacaagtgctgtctatgtatgagaccagctgggtgactcggttaaacccctcgcctctctaaacaaagtatgtgatttaccctgaatcattcttcagcaagtactaaaaaggtataatttcttaaaatgaatgcgattgatcgacttttggcttgcaaaaatgacttctcattggaaaagagacacaccttagaaagatgaaaatgtgaaaaacaacagtcataaaatggaatcgctccatgctcggactctctgccaccagacatctgactgtgcagccatcagctgagaggctgcttgcagttccccatccaggacccacggtgcctggtgctaaggagcgactggactgaggaagcctctcatcaccagctgtgttgcagctttaaattctgccccagttgtggtatttaaaattctgtatgttaaaaaaaaaaaaaccaccaatctgcctacatcttcctagttaaagctagaaaggggaatggagagaagatccaacccagctgggcagagtggctgagcacgagacacccacaaacccaacgcggttctaggggttggatcagaagagtctctgtgtcgtcggtcgggcacaggcttgcctcctcgattctagacgtgccctcggccacagtgtctaatcttcctgtttcctggcattcaggtgttttacctctctgcccggattttgtacctgaggacaaaataggcaatgaggcggagggagatgaagaaaatcccgagtacgatgaagtccaggtacagcttggcattttccacgtccagctcccgcaggatggcctccgacttctggaagtggcacgtctcgtcgatgtcacagtgcagatcttcccggtctaagccatagatggagaggatgaccccttcgaacccatacctgacataggagatgtaggacatccactgtaggtacgtggggatggtgtcgaagctgacgaagaaccccgagaacaggagcaccgggatggctgtcactgggcccacgaaagtggccacctgcagggacgtggaggcggctccgatcagcaggcccagggactgtgccaccagggaggtcatggtgcccagcgcggcaaacagcacaaagcgcacggcgtcggacggctgcgacgtcatccagtacacgatgctgcagtaggccactgggaacatgatctgaaagggcacgtctgccatggtcttggccaggtagtaggccttcaggctgtaccagtagttcaggtgttcccgaagaaagactcccatctccaggggaaatgtcagaacagtaggcatgagggccgcgaacatgaggaacagcatggagaagaagaggaagccggagttgctcaagaccttcttggcttcgttcccgatccccaagtacagcaggccaatgaggaggccgatcccaatgtgcgaggtgatgcgcaggtgtgtcaggaccgagtccctcatgatgctgaggaaggtcctcttgaagaggatgcagaactgcgtgaggcagctggcagagaagctgtggcagccttccatggacgaggagtcctttctcaacccctttaatcgttttgtctgctttacctcttcagagggccggtgccaaagaaaagggttcacctcggcatcacccccgaggtctctcttgtggtctgagtcacacatgccctcccgaaccgctctcaccagccgactgttctgatcaccgtactcgccggatgcaacctccatgacaaaatctgctgggttgtggtaggttgggcagttcagacccaaatccctcaaatatggcacaagattgcagacttttccccggtacacacattgtccttgactcaggacgtaaagctggtcgaacagctcgaagagtttggcgctgggctggtggatggtgcaaatgatggagcgacccccttgagcgagccctttcatcagcgagaccacctggaagcaggaggcgctgtccaggccgctggtgggctcatcgaagaacatgactggagggttgttcaccagctccagcgcgatggccaggcgcttgcgctgaccacctgacaggctcccggtccgcgtgttggcgcaagacagcaagcccagcgctgtcagtatctccttgaccatttcccttctgccttcatccttctcctgaagcttcagatgtgccgacaccatcatggcctcctgcacagtgagatgcggcagcagcatgtcatcctgcatgatgtagcaggacaccttccggaagcagcgcaggtcccggggcaggccgttgatgaggacggcccccttcatgcccgtctccctgtatccagccaggatgttcatcagcgtggacttcccggccccggaaggacccataatggccaccaactcaccactattgaacttcccggaaattcctttcaggagggtcttgtatccttcctccatgggatcgccaggaaacccccaaccataggcccttcctgccccatgagctgctgacaagactttgccactgatagcgaccacccccaggtgatggggccctccctggacttggactgaccacgtgcaggatgccgcactggccttgagtggacggttggatgggggcatgatgacaatgcttgagccctgtaggccagacatcggcaccctttttccctgaagagctgaatcacagacattttcgattttgcaggacacgcagtctgtcacaaacactgagctctccagtttagcagaagctaaagctgccacctgtacatgcacggctgtggctgtgcctgtaaaaactgtgagaactgctttctcttcatgggtcagtgtcccagagaatgcagatgggatatttgttgtgacattatttctcatcacccaggcacgcaggtgacctggagccacagccatctgtagccagtacacccagccagggtgtggatactctgcggcctctggatactctgacaggaaggtgtgagtagggaccagacaccacagtctggccaagagaatggcggtacagacagaccaacctctcctgaccatgtcccggagccccag

SEQ ID NO: 10051 - RNA, 6174 nt, Homo sapiens
  source 1..6174: mol_type = other RNA
cacccggctgtgtgcacatgtgcttgtgtgtaggtagacacatatacaccatacacgcacacacacacaccagcccctgtagagcctgagctagtccacaggactgttgcaataggaggagcaggcaagggcagaggacagcccctctccacggagaggtacctgtcacgagtactctgatgcaaggccactgaagggcgttaggcttgggttgccctctcatctcagccacctgtttggtaacagaaggaatcactgaacgaacagccactaagctagtattgcactttatgccttacaaagcatctcagatacattcatacgccatgaacaggaggcagtaaacaaaacagggacttcagcgtccaactgggctggaatcccaactccgctccttcctcgttctggggccctggggacgtcacggagcctctccctgcctccgcgttccacgtctgcaccatgagcacggctaagccaagtggccacgcggttccctcccaccacactggagggcaagcccacgttggagtcccctccccctcacccccagggcctgggacagcaccaggcgagaggggtgggtcagtaagggtttgaggagtgggcaggggacagggggttctgaggacatccagcccagtgcctggaaacagccacgaggaaaggtgctcggtgcaccagagtcgtgccttctcttcccactgcaacaaccaagcccggtttctgccccatgggtgtggtctgtccctgatgtcaggctgggggaatgactttttgtgggtttctaagatgagttttcacctcaaagctccatgtaccatttcctggtcctgaaggcgcctcccccaggtgatgtaatccaattctggcactgactgcataaaactttgcacagttactccccttcctgggcacagcttcccacttcacccacacagggagtttcggagaattcaatctccagtggatattcagccagaggagaagaaagagaggcacaaaatgctttggatgaggacaaaggcaaaaggccccagcagtttccctgaaacctccattttcacctctactaaccactggggcatctgcaaatcttttatccaaggtttaatccttccttctaatggaagaaactcaaccagagatgaaaggaatatcttggtcaatgcattcagaaattactgaaacaaattagatttggggagttggtctgggtttaacgtccaacatgtgaaagatagcacattgccgtgtgtgtcttaaccacagctggttagaaaagtaaaccagtgagttgcttgatattatcttaggccattggaataaggcattttaccaaactaccttaacacaaaaagcagtggggaaatatctgggaatctaaacaatggcatttgagccaatgctgccaaaggttacgaggaaaatgcccagccagggacccttgctgaacctggaagagggaggccggctgcacctaggacagatgcatcctctcctcccttggcggtaggctttcctccagtctacgggggagggctgagcaaagccatcctggggcgtcaactgcagaatcctcacctactccagttcacccttcaaaaaataaacccacatggtctcacatatccattcccttcttgcagcctaacagccctcatggttcccaagctcttcccccttagaattacccccatcaagttcctacgagagtcattccatcagagggcttaggtgctctccgaaaccagatttaaaatctagaggcatctcactgtttcctcctgaaattgatgaggcacagcaagcggtctcagcaaacgagaccaaagctgcttctgaggcagggctgtgggccccatgcagtgcagttcctggcagacacacccctattagggccatgaagccacaacactaatccacaatggggaaggctcacctggagggaatgggcgttttcaacactgacctcactcgatgtagttctgagtcatgagcaaggacttttgcctttttccaattctgcatttcaccaggctattcctaggtaggtcttccctatgtgcaatgtcttacaagaagatctattttgaaattaaatgaggactttttataaaggctaagtttgactctggttaaaaacttaatctggaaggcaatgccatatttgtatagaacaagcacacttaaaattacactttaatatctatctcaattgtgtttactaaaaaagatctagcagtaaaaaaggaatctctaagaattagcaaactaaatccatgtgtaaataaaattcagacccttttcgttctttcgaagtgggaaataagagcttcagggacatcgccaaggaatcccaccacctttgagctggcatggccttgggcatgatgtactgtaactatttacagatgaggaaaaatgtagcttagaaaggttcactgattttcccgcaaaaacacagcctttccatcggaagccctgattctaggagaatgatattctagagggagtaaacaatggcattttcctaaaggtggacttctttggccagaatcaccttctctgcatgtagtcaaactgcttctgagagctgacaaactcacaggcagccttgttgtgaattcaaagaccacttgacctccagataggcacctgtttctgccctagcgggatttgacttatgtgattcagtcataggaaagaagcggtttccaacgtgcaaagtttacacaggcctaacactgaggcggtgatgcagctgtgaggtcgcaaaacccagagatgaaatctcccaccactcgaagtgcgttgtttgatcaagtttcaaatgcctccacatgctgaagtctactgacttcgtcctaagcccttggattctgatgccatctcgttggcctcctcccctcttgcacagttagcccatctttcactgctggccactcctgctgagccaaccctcaaaggtcgtgcctgaatttccctaagccccattcttccaggttcagtggaggcagctgaggtgatacaggaggaaagggaagctgtttgtttgtttgtttaaatcaacctaggcaaaattaaaggtagtcagaaagttaggaagaaacaaacaatatatttcgcttaaaataagaagcacgtggaaaaagaaagactttgaaagagttggccaatgtcttctcacaattttttgtatagcttttaaaaatgtctgcatggctcagtggagatggtgtccacgtcttccctccacctggaacctgcattcaatccttcacaagtgctgtctatgtatgagaccagctgggtgactcggttaaacccctcgcctctctaaacaaagtatgtgatttaccctgaatcattcttcagcaagtactaaaaaggtataatttcttaaaatgaatgcgattgatcgacttttggcttgcaaaaatgacttctcattggaaaagagacacaccttagaaagatgaaaatgtgaaaaacaacagtcataaaatggaatcgctccatgctcggactctctgccaccagacatctgactgtgcagccatcagctgagaggctgcttgcagttccccatccaggacccacggtgcctggtgctaaggagcgactggactgaggaagcctctcatcaccagctgtgttgcagctttaaattctgccccagttgtggtatttaaaattctgtatgttaaaaaaaaaaaaaccaccaatctgcctacatcttcctagttaaagctagaaaggggaatggagagaagatccaacccagctgggcagagtggctgagcacgagacacccacaaacccaacgcggttctaggggttggatcagaagagtctctgtgtcgtcggtcgggcacaggcttgcctcctcgattctagacgtgccctcggccacagtgtctaatcttcctgtttcctggcattcaggtgttttacctctctgcccggattttgtacctgaggacaaaataggcaatgaggcggagggagatgaagaaaatcccgagtacgatgaagtccaggtacagcttggcattttccacgtccagctcccgcaggatggcctccgacttctggaagtggcacgtctcgtcgatgtcacagtgcagatcttcccggtctaagccatagatggagaggatgaccccttcgaacccatacctgacataggagatgtaggacatccactgtaggtacgtggggatggtgtcgaagctgacgaagaaccccgagaacaggagcaccgggatggctgtcactgggcccacgaaagtggccacctgcagggacgtggaggcggctccgatcagcaggcccagggactgtgccaccagggaggtcatggtgcccagcgcggcaaacagcacaaagcgcacggcgtcggacggctgcgacgtcatccagtacacgatgctgcagtaggccactgggaacatgatctgaaagggcacgtctgccatggtcttggccaggtagtaggccttcaggctgtaccagtagttcaggtgttcccgaagaaagactcccatctccaggggaaatgtcagaacagtaggcatgagggccgcgaacatgaggaacagcatggagaagaagaggaagccggagttgctcaagaccttcttggcttcgttcccgatccccaagtacagcaggccaatgaggaggccgatcccaatgtgcgaggtgatgcgcaggtgtgtcaggaccgagtccctcatgatgctgaggaaggtcctcttgaagaggatgcagaactgcgtgaggcagctggcagagaagctgtggcagccttccatggacgaggagtcctttctcaacccctttaatcgttttgtctgctttacctcttcagagggccggtgccaaagaaaagggttcacctcggcatcacccccgaggtctctcttgtggtctgagtcacacatgccctcccgaaccgctctcaccagccgactgttctgatcaccgtactcgccggatgcaacctccatgacaaaatctgctgggttgtggtaggttgggcagttcagacccaaatccctcaaatatggcacaagattgcagacttttccccggtacacacattgtccttgactcaggacgtaaagctggtcgaacagctcgaagagtttggcgctgggctggtggatggtgcaaatgatggagcgacccccttgagcgagccctttcatcagcgagaccacctggaagcaggaggcgctgtccaggccgctggtgggctcatcgaagaacatgactggagggttgttcaccagctccagcgcgatggccaggcgcttgcgctgaccacctgacaggctcccggtccgcgtgttggcgcaagacagcaagcccagcgctgtcagtatctccttgaccatttcccttctgccttcatccttctcctgaagcttcagatgtgccgacaccatcatggcctcctgcacagtgagatgcggcagcagcatgtcatcctgcatgatgtagcaggacaccttccggaagcagcgcaggtcccggggcaggccgttgatgaggacggcccccttcatgcccgtctccctgtatccagccaggatgttcatcagcgtggacttcccggccccggaaggacccataatggccaccaactcaccactattgaacttcccggaaattcctttcaggagggtcttgtatcctttcttcctccaccagggtccttcaggaaccgaataggaaaggtccctgaattcaatgttcacagctgccctccgaggcaaggaggagaagcgctgggcttccgtgaggttattatctacttttttcagatgtccattcagcaggtccgtctcagtggcctccatgttgctggacaccacctcatccaccgagacacacaccgacttgggctccgtcatctctgcagagtaactgctggcattagtaactgtgtccagcagtgaactcgccgacaccccgccatccctctccggagctcggggaagtgaaatgcgcatccctgtccccaccgcgtctctctctccggcgcgcgcagaaaggcggccggcaggaatccgggcttgcccctcgcgggtctccccgggccttcgccgccgcctccccgagtgggtccgggagagggtgtccccgggagtgcagtcgcaggct

SEQ ID NO: 10052 - RNA, 6196 nt, Homo sapiens
  source 1..6196: mol_type = other RNA
cacccggctgtgtgcacatgtgcttgtgtgtaggtagacacatatacaccatacacgcacacacacacaccagcccctgtagagcctgagctagtccacaggactgttgcaataggaggagcaggcaagggcagaggacagcccctctccacggagaggtacctgtcacgagtactctgatgcaaggccactgaagggcgttaggcttgggttgccctctcatctcagccacctgtttggtaacagaaggaatcactgaacgaacagccactaagctagtattgcactttatgccttacaaagcatctcagatacattcatacgccatgaacaggaggcagtaaacaaaacagggacttcagcgtccaactgggctggaatcccaactccgctccttcctcgttctggggccctggggacgtcacggagcctctccctgcctccgcgttccacgtctgcaccatgagcacggctaagccaagtggccacgcggttccctcccaccacactggagggcaagcccacgttggagtcccctccccctcacccccagggcctgggacagcaccaggcgagaggggtgggtcagtaagggtttgaggagtgggcaggggacagggggttctgaggacatccagcccagtgcctggaaacagccacgaggaaaggtgctcggtgcaccagagtcgtgccttctcttcccactgcaacaaccaagcccggtttctgccccatgggtgtggtctgtccctgatgtcaggctgggggaatgactttttgtgggtttctaagatgagttttcacctcaaagctccatgtaccatttcctggtcctgaaggcgcctcccccaggtgatgtaatccaattctggcactgactgcataaaactttgcacagttactccccttcctgggcacagcttcccacttcacccacacagggagtttcggagaattcaatctccagtggatattcagccagaggagaagaaagagaggcacaaaatgctttggatgaggacaaaggcaaaaggccccagcagtttccctgaaacctccattttcacctctactaaccactggggcatctgcaaatcttttatccaaggtttaatccttccttctaatggaagaaactcaaccagagatgaaaggaatatcttggtcaatgcattcagaaattactgaaacaaattagatttggggagttggtctgggtttaacgtccaacatgtgaaagatagcacattgccgtgtgtgtcttaaccacagctggttagaaaagtaaaccagtgagttgcttgatattatcttaggccattggaataaggcattttaccaaactaccttaacacaaaaagcagtggggaaatatctgggaatctaaacaatggcatttgagccaatgctgccaaaggttacgaggaaaatgcccagccagggacccttgctgaacctggaagagggaggccggctgcacctaggacagatgcatcctctcctcccttggcggtaggctttcctccagtctacgggggagggctgagcaaagccatcctggggcgtcaactgcagaatcctcacctactccagttcacccttcaaaaaataaacccacatggtctcacatatccattcccttcttgcagcctaacagccctcatggttcccaagctcttcccccttagaattacccccatcaagttcctacgagagtcattccatcagagggcttaggtgctctccgaaaccagatttaaaatctagaggcatctcactgtttcctcctgaaattgatgaggcacagcaagcggtctcagcaaacgagaccaaagctgcttctgaggcagggctgtgggccccatgcagtgcagttcctggcagacacacccctattagggccatgaagccacaacactaatccacaatggggaaggctcacctggagggaatgggcgttttcaacactgacctcactcgatgtagttctgagtcatgagcaaggacttttgcctttttccaattctgcatttcaccaggctattcctaggtaggtcttccctatgtgcaatgtcttacaagaagatctattttgaaattaaatgaggactttttataaaggctaagtttgactctggttaaaaacttaatctggaaggcaatgccatatttgtatagaacaagcacacttaaaattacactttaatatctatctcaattgtgtttactaaaaaagatctagcagtaaaaaaggaatctctaagaattagcaaactaaatccatgtgtaaataaaattcagacccttttcgttctttcgaagtgggaaataagagcttcagggacatcgccaaggaatcccaccacctttgagctggcatggccttgggcatgatgtactgtaactatttacagatgaggaaaaatgtagcttagaaaggttcactgattttcccgcaaaaacacagcctttccatcggaagccctgattctaggagaatgatattctagagggagtaaacaatggcattttcctaaaggtggacttctttggccagaatcaccttctctgcatgtagtcaaactgcttctgagagctgacaaactcacaggcagccttgttgtgaattcaaagaccacttgacctccagataggcacctgtttctgccctagcgggatttgacttatgtgattcagtcataggaaagaagcggtttccaacgtgcaaagtttacacaggcctaacactgaggcggtgatgcagctgtgaggtcgcaaaacccagagatgaaatctcccaccactcgaagtgcgttgtttgatcaagtttcaaatgcctccacatgctgaagtctactgacttcgtcctaagcccttggattctgatgccatctcgttggcctcctcccctcttgcacagttagcccatctttcactgctggccactcctgctgagccaaccctcaaaggtcgtgcctgaatttccctaagccccattcttccaggttcagtggaggcagctgaggtgatacaggaggaaagggaagctgtttgtttgtttgtttaaatcaacctaggcaaaattaaaggtagtcagaaagttaggaagaaacaaacaatatatttcgcttaaaataagaagcacgtggaaaaagaaagactttgaaagagttggccaatgtcttctcacaattttttgtatagcttttaaaaatgtctgcatggctcagtggagatggtgtccacgtcttccctccacctggaacctgcattcaatccttcacaagtgctgtctatgtatgagaccagctgggtgactcggttaaacccctcgcctctctaaacaaagtatgtgatttaccctgaatcattcttcagcaagtactaaaaaggtataatttcttaaaatgaatgcgattgatcgacttttggcttgcaaaaatgacttctcattggaaaagagacacaccttagaaagatgaaaatgtgaaaaacaacagtcataaaatggaatcgctccatgctcggactctctgccaccagacatctgactgtgcagccatcagctgagaggctgcttgcagttccccatccaggacccacggtgcctggtgctaaggagcgactggactgaggaagcctctcatcaccagctgtgttgcagctttaaattctgccccagttgtggtatttaaaattctgtatgttaaaaaaaaaaaaaccaccaatctgcctacatcttcctagttaaagctagaaaggggaatggagagaagatccaacccagctgggcagagtggctgagcacgagacacccacaaacccaacgcggttctaggggttggatcagaagagtctctgtgtcgtcggtcgggcacaggcttgcctcctcgattctagacgtgccctcggccacagtgtctaatcttcctgtttcctggcattcaggtgttttacctctctgcccggattttgtacctgaggacaaaataggcaatgaggcggagggagatgaagaaaatcccgagtacgatgaagtccaggtacagcttggcattttccacgtccagctcccgcaggatggcctccgacttctggaagtggcacgtctcgtcgatgtcacagtgcagatcttcccggtctaagccatagatggagaggatgaccccttcgaacccatacctgacataggagatgtaggacatccactgtaggtacgtggggatggtgtcgaagctgacgaagaaccccgagaacaggagcaccgggatggctgtcactgggcccacgaaagtggccacttagcgcctcctgggctggcacctgcagggacgtggaggcggctccgatcagcaggcccagggactgtgccaccagggaggtcatggtgcccagcgcggcaaacagcacaaagcgcacggcgtcggacggctgcgacgtcatccagtacacgatgctgcagtaggccactgggaacatgatctgaaagggcacgtctgccatggtcttggccaggtagtaggccttcaggctgtaccagtagttcaggtgttcccgaagaaagactcccatctccaggggaaatgtcagaacagtaggcatgagggccgcgaacatgaggaacagcatggagaagaagaggaagccggagttgctcaagaccttcttggcttcgttcccgatccccaagtacagcaggccaatgaggaggccgatcccaatgtgcgaggtgatgcgcaggtgtgtcaggaccgagtccctcatgatgctgaggaaggtcctcttgaagaggatgcagaactgcgtgaggcagctggcagagaagctgtggcagccttccatggacgaggagtcctttctcaacccctttaatcgttttgtctgctttacctcttcagagggccggtgccaaagaaaagggttcacctcggcatcacccccgaggtctctcttgtggtctgagtcacacatgccctcccgaaccgctctcaccagccgactgttctgatcaccgtactcgccggatgcaacctccatgacaaaatctgctgggttgtggtaggttgggcagttcagacccaaatccctcaaatatggcacaagattgcagacttttccccggtacacacattgtccttgactcaggacgtaaagctggtcgaacagctcgaagagtttggcgctgggctggtggatggtgcaaatgatggagcgacccccttgagcgagccctttcatcagcgagaccacctggaagcaggaggcgctgtccaggccgctggtgggctcatcgaagaacatgactggagggttgttcaccagctccagcgcgatggccaggcgcttgcgctgaccacctgacaggctcccggtccgcgtgttggcgcaagacagcaagcccagcgctgtcagtatctccttgaccatttcccttctgccttcatccttctcctgaagcttcagatgtgccgacaccatcatggcctcctgcacagtgagatgcggcagcagcatgtcatcctgcatgatgtagcaggacaccttccggaagcagcgcaggtcccggggcaggccgttgatgaggacggcccccttcatgcccgtctccctgtatccagccaggatgttcatcagcgtggacttcccggccccggaaggacccataatggccaccaactcaccactattgaacttcccggaaattcctttcaggagggtcttgtatcctttcttcctccaccagggtccttcaggaaccgaataggaaaggtccctgaattcaatgttcacagctgccctccgaggcaaggaggagaagcgctgggcttccgtgaggttattatctacttttttcagatgtccattcagcaggtccgtctcagtggcctccatgttgctggacaccacctcatccaccgagacacacaccgacttgggctccgtcatctctgcagagtaactgctggcattagtaactgtgtccagcagtgaactcgccgacaccccgccatccctctccggagctcggggaagtgaaatgcgcatccctgtccccaccgcgtctctctctccggcgcgcgcagaaaggcggccggcaggaatccgggcttgcccctcgcgggtctccccgggccttcgccgccgcctccccgagtgggtccgggagagggtgtccccgggagtgcagtcgcaggct

SEQ ID NO: 10053 - RNA, 524 nt, Homo sapiens
  source 1..524: mol_type = other RNA
cacccggctgtgtgcacatgtgcttgtgtgtgcatgtgtgtgcaagtgtgcatgtgtgcgagtgtgcatatgtgcattgtgtgcgtgagtgtgcgtgtggtccgtgtacacatctgtccatacatgtgagcttgcatgcacatgtgcgcatgtgagtgtgcatgcatgtgttgtgtgtgtacgtgtctgcacgttggtgtgtgtatgtgtgtgcctgtgagtgtgcagagaggccctggcgctcgaggagggcctacagctcatagtactcacccggcgggcccagttgacgaggtcatccagcttggccaccacatactcgccccggctgctgggtttgggagccacggctctggcctttggcagggcaggctgggtgctgcttgggccatcggtggccacgctctgatggacacctcgtgcctgcacagccgggcccacgctggagcgcagaccaaggatccggaagccgcgcaggccaggagctgacagcaccgccatcttggcctcggccttcagacaac

SEQ ID NO: 10054 - RNA, 1586 nt, Homo sapiens
  source 1..1586: mol_type = other RNA
caccgactctgtctcctgcagattcatgcaaccctcagtacctggctagggcagtttttgtcttcagtgaggtcactgccggttgtctctagaaggcagtagctttgtcttatgtacatcttggtccccactcccggggcctggcactgtgcctgggacaccatagatgttggctgtatgctgttgaactgagacccttgtgctgtctaatcagtgagctctgggagagtgtgggagaggcagagaaaggttagaggtcagggacagatgagtgggtgggcgcatgctcaggtcacctcacgggctggctggggtggtgggccttgctgtgctggctcagcatcacttgggactggtcctgcaaggcctctacgtgctcaggatccttcaggccccgcgtctctggcttgaagaggaccaaggccttcatgcaggcaaactccgtggggtccaccgccaatgcccggaaccgagagatagtttcctgcaggacacgcgtctccatgctggccagcgtgagccggccctgggcaccaccggcagcagaggcctcgggcggtgccagcagaggacagctgtccagaggcagagaccactggatggccccgaggagaaagagttcactccacgcctcttccagcaggatcacctgatcccggaagggcaggctggagaacacaggcaggttcttggcccacttgacggccatgaagagtaggcgagccgaggtctcatggatgctgtccaggccgcagggggaggaagaggagtatggagaggaggggaactcagggtcattgctggtgacatcaatattctcatcagcatcctctggctccagcttagcacaggtttcagctgttataaggctggccatgaagtggtggcccagggctctggctgcagacatgggtgtggggccccgtgggctgcgccctgccggggccgggggagccaccagggactccggccgggactcagtgttggactccatgctgtccaggtggacctgggctgtgcttcgcggctggcgctcgttctgcacggcgtcctggttcatccccgcctgcaggcacttcttcagccggcaggcctggcactggttgcggtgggccttgtccacggggcacatccctgcccccacctggcacctgtagatgagcctccgccgtacgctcctcttgaagaagccgctgcagccgttgcaggcatagatgccatagtgcttcccgctgctgctgtctccgcacacgcggcactggagcgaggggctcacgcctgtgggatcctcccccaggccccatctgcctggagactccttcctggaggcagccccagctgcaggcgcagctgcagccactgtggagctcatcagagctgttggtctggtctccatgggttacagggcagcctctgcctgcctgcgggaggcctgggttgctgagcctggcccagcctttgcctcagtccatgaacctctgtctctctgtgcccctgtctcccttcctgaactctgtctgaactcaggagctgccccaaggtcccgaagcccctcacagcacaggctctggcttgaggagatttct

SEQ ID NO: 10055 - RNA, 1705 nt, Homo sapiens
  source 1..1705: mol_type = other RNA
caccgactctgtctcctgcagcctctccatggcttcctcaggcccaatctgggactccgtgttgggggagaatgacggctccagctccccattatgtgtggtgggtgatgagggtgaaactggagctgggggagatgacacagctggcagggcgcctctgacactcccttcttccgtcttcaggccttccagagcagaggctgacagtccctgagccatcagcagttcccgcagccgggctacttcctcctgcagctctctaatcagccgggcattagggtcctcgttgatgatggcattgcagcggatttgcttggtgcggtcagcatacctgagggtgctgagagtctcctcgtaattgatgtcagcagggctcagggctgcaatcatggctgtgcgtgagttcccccccaaattttccttgagcagccaggtgagcacagagtccctgtaggggataaaatccgactttcgcttctttgattgcatatctgcaagggccgagatcactttccctagtgtagtcagggacttattgatgttggctccttccttcaggcgcatgccccgggcccctgaggagtcggctcgctcactcccagcaaggtccaccaaactgatcttactgaccttctccgagtccagccccgtgagctggtcatggcagcgctgtgtgaagacgatggtaaagacggcatgggaacggctgctggtctcattcatgttggtggcagccacagtccgtgctttatttccacagtccatgaggtcagcaatgtctgcgtaggaggtcacagccaatttggacaggtcctgcacgtacgggcccaggatggggtgctcccggacccgcagagaaccccgactcttggggttcaagaggtctcgtacccgctcacagtagatctccatatagctcacctccacagagtaggatagctgagcactctggttctcactaacgcgagagaagaggtcctcacagagctggggcacgatgccctgctgccctggctcctgtcgccccatcatggtataggatttcccagccccggtctgcccataggcaaagatgcacacgttgtagccttcaaaggcgtggagcagcatctcttctccaatgtcccgatacacttgctgctgagatgcaaactgggggtcctccgtcgaagtgtgtgaccagtaggagtagtcaaaggtgaagcttttgggggcatccttgctctgtttaggattgatgatggaggtggtgttgccctgcatgctgaccacacacttggcatcctggctggtctcacgggcgttaaagggccgaaccctcactgccactttcaccgaggcaccagccatagctccagacactcctgccctcctcagctggcgtcctggccccagaccaggggggctgtatcagttctggctgccaccggccctcgtagggggagccccatcctactcctggggcctggccacaccagctggggctctgggagataccctcggcgcggcggggctcccggagcagctcggcggagagggacaagctttccgggaagcgtgaggcggaagcgggaaggatctggggccggttcggagctgcccccgcccctcgccgggtgcccgggcggcgggcggcggactcgcgccccgggggcggcagcagtagcggcgccagcggccggcgcccgcccgggcagcgcgagct

SEQ ID NO: 10056 - RNA, 1698 nt, Homo sapiens
  source 1..1698: mol_type = other RNA
caccgactctgtctcctgcagcctctccatggcttcctcaggcccaatctgggactccgtgttgggggagaatgacggctccagctccccattatgtgtggtgggtgatgagggtgaaactggagctgggggagatgacacagctggcagggcgcctctgacactcccttcttccgtcttcaggccttccagagcagaggctgacagtccctgagccatcagcagttcccgcagccgggctacttcctcctgcagctctctaatcagccgggcattagggtcctcgttgatgatggcattgcagcggatttgcttggtgcggtcagcatacctgagggtgctgagagtctcctcgtaattgatgtcagcagggctcagggctgcaatcatggctgtgcgtgagttcccccccaaattttccttgagcagccaggtgagcacagagtccctgtaggggataaaatccgactttcgcttctttgattgcatatctgcaagggccgagatcactttccctagtgtagtcagggacttattgatgttggctccttccttcaggcgcatgccccgggcccctgaggagtcggctcgctcactcccagcaaggtccaccaaactgatcttactgaccttctccgagtccagccccgtgagctggtcatggcagcgctgtgtgaagacgatggtaaagacggcatgggaacggctgctggtctcattcatgttggtggcagccacagtccgtgctttatttccacagtccatgaggtcagcaatgtctgcgtaggaggtcacagccaatttggacaggtcctgcacgtacgggcccaggatggggtgctcccggacccgcagagaaccccgactcttggggttcaagaggtctcgtacccgctcacagtagatctccatatagctcacctccacagagtaggatagctgagcactctggttctcactaacgcgagagaagaggtcctcacagagctggggcacgatgccctgctgccctggctcctgtcgccccatcatggtataggatttcccagccccggtctgcccataggcaaagatgcacacgttgtagccttcaaaggcgtggagcagcatctcttctccaatgtcccgatacacttgctgctgagatgcaaactgggggtcctccgtcgaagtgtgtgaccagtaggagtagtcaaaggtgaagcttttgggggcatccttgctctgtttaggattgatgatggaggtggtgttgccctgcatgctgaccacacacttggcatcctggctggtctcacgggcgttaaagggccgaaccctcactgccactttcaccgaggcaccagccatagctccagacactcctgccctcctcagctggcgtcctggccccagaccaggggggctgtatcagttctggctgccaccggccctcgtagggggagccccatcctactcctggggcctggccacaccagctggggctctgggagataccctgtgtttgagggtagagggtccctggggcctccctcggcgcggcggggctcccggagcagctcggcggagagggacaagctttccgggaagcgtgaggcggaagcgggaaggatctggggccggttcggagctgcccccgcccctcgccgggtgcccgggcggcgggcggcggactcgcgccccgggggcggcagcagt

SEQ ID NO: 10057 - RNA, 2636 nt, Homo sapiens
  source 1..2636: mol_type = other RNA
caccgactctgtctcctgcagcttaaatactttttggtggcagcgggtgcttagctgcttcttgttttctttcagacattcgataatctgagcgttgccatattgcacagcggaacagaagtttttgatgtcactcttgcaggcttcgtatagatctggctccaagcggatgtcctccgtcatctccagctcctccacacggagctgcctgcggcacttcagggacaccctgtgctccttggcttcctgcagagtgtcattgcgcacggtcgtgctcaggcagatcaccacgtccaccttcttttttatgtttgggcaaagcttcaacacgtcctccttgcaggccattttaaacttgtaagaaaaccgaaaatccttcatctgcaccagctggaagtgggtaactccgatggcacacttctcgttcatgtccttctggtgtttgttctgtatcagacactccatcaggtccccagagtctatctggttatctgccacatcgtggcagaagttctgaattatgggctcacaggctctcatcagcaaggcttctatttgaatatcctctgattctaactcagtgaggttgccaactatatctctacactccaccaccaagtcatccagatggtcctgaaggcactccagctcctgtccagtctctgttttctcactgcaccattttcccagatcaatcaggcacttatcctggagggcaggatccagcttgacatccatggcacgctggtgtaggatcctttggacttcagctcggcactcccgtgagagcctccttccctgttcctcagtgcggtaggcgtgtctgtataaacaagagaacacagctccctgaggcataaattcactggtctcattccaaccgtgggtgtggcaaagacgagaagcgtctccctggcacttgcggtacaggacagggtccagcttccaatcccgggagatgaaatactgcagctctaagagacggtgttcacagtcttctaccatcttctctgtgtataaatgttccatcaggcacgacaagatcattgggtctccagatcttatatgtttgcaggctgtctggattacagattcacaagcttcattcaaagctcgatcaatgcggtaatctgcaccagggtcagtctcctgaatcagtgtttgaagcgcctgctggcagttcattccaaggttccccttctcccctcgaactactttcatcagacagtgtagggtccgcccttttcgatgtaatccggaacaatggtgttcaatctccccccgacagcttaggatgatctcagggctcagagaaaagtcttccatcaacatgcgtcggtaatccagcatctccccctggcactcactgctgacttgtcgccctctgtgtacagctgactccaggcacattaacaagtaggagagcctggcttcacgcgatcgcggaaggttttccacattgcaccggtatttcttcaagtcacttttacaggatttggccaatgaataactgactttataatcctgggcaatcagcttttggcgggttgtaagtgcttctcgacacttttcactcatggattcttcaaatttatggttaaagaggcacttatacactctgccctcaccagcttgtgtattttcacaaaaacgctcccgatcatctcggcaagcaaaatataaatgccggtctaagtgaaagtcatccgatgacagctcagccacccggagaatggctttcttgcagagttcagaaacttgaatcttgggttctctttcttctgcttctttcaccaggcctttctccaagcatgataccacctcaccttgtgaatgtgcatccttttctccaagccgaatactgccacatttcagaatgttgatgtcatttttgcagtcatccatgaagccacagattaaacggtaatcactaaaaatgatggccgtcatcttggtaatgtactggtgacactgatactcagtgatgttgcctcggtgatccaccaagcaggaaaccatgtaaccttttccaaccggttcatcagcacattctttaatctctgttatagtagatttgcaaacctctctggccacagattcaaatttgggatctgtagttaggttcagcttataattccacaacaaatgattgcagtctgaagaaatttcattttcaggctccctcacatcctgcaggcactcgagcaccgccaggttgttgctccaggtgtgcttagggcacacgcgggtcacgtcctccctgcaggactcttcctccgccagcttccagcccccaccagcccccgctcctccccgccgggccggaggcccacccgccgggaaaggcggctgcggcggctgaggctgctgttgctgttgctgctgctgctgttgctgctgaagctgcgatgactgaggcagctggggcagctgctgacccgccgggccgccgcctccggcctgccctacgaaggacacaaagttggccccgggaccctggccctggctgtggacgccctggccggggagtttctcggccccggccgcgaatagcagcagcagatgcagcgccgccgacaagcggaacatcctccgtacacgtccacacgccgccatcttgagtccgcggcgagctc

SEQ ID NO: 10058 - RNA, 2603 nt, Homo sapiens
  source 1..2603: mol_type = other RNA
caccgactctgtctcctgcagcttaaatactttttggtggcagcgggtgcttagctgcttcttgttttctttcagacattcgataatctgagcgttgccatattgcacagcggaacagaagtttttgatgtcactcttgcaggcttcgtatagatctggctccaagcggatgtcctccgtcatctccagctcctccacacggagctgcctgcggcacttcagggacaccctgtgctccttggcttcctgcagagtgtcattgcgcacggtcgtgctcaggcagatcaccacgtccaccttcttttttatgtttgggcaaagcttcaacacgtcctccttgcaggccattttaaacttgtaagaaaaccgaaaatccttcatctgcaccagctggaagtgggtaactccgatggcacacttctcgttcatgtccttctggtgtttgttctgtatcagacactccatcaggtccccagagtctatctggttatctgccacatcgtggcagaagttctgaattatgggctcacaggctctcatcagcaaggcttctatttgaatatcctctgattctaactcagtgaggttgccaactatatctctacactccaccaccaagtcatccagatggtcctgaaggcactccagctcctgtccagtctctgttttctcactgcaccattttcccagatcaatcaggcacttatcctggagggcaggatccagcttgacatccatggcacgctggtgtaggatcctttggacttcagctcggcactcccgtgagagcctccttccctgttcctcagtgcggtaggcgtgtctgtataaacaagagaacacagctccctgaggcataaattcactggtctcattccaaccgtgggtgtggcaaagacgagaagcgtctccctggcacttgcggtacaggacagggtccagcttccaatcccgggagatgaaatactgcagctctaagagacggtgttcacagtcttctaccatcttctctgtgtataaatgttccatcaggcacgacaagatcattgggtctccagatcttatatgtttgcaggctgtctggattacagattcacaagcttcattcaaagctcgatcaatgcggtaatctgcaccagggtcagtctcctgaatcagtgtttgaagcgcctgctggcagttcattccaaggttccccttctcccctcgaactactttcatcagacagtgtagggtccgcccttttcgatgtaatccggaacaatggtgttcaatctccccccgacagcttaggatgatctcagggctcagagaaaagtcttccatcaacatgcgtcggtaatccagcatctccccctggcactcactgctgacttgtcgccctctgtgtacagctgactccaggcacattaacaagtaggagagcctggcttcacgcgatcgcggaaggttttccacattgcaccggtatttcttcaagtcacttttacaggatttggccaatgaataactgactttataatcctgggcaatcagcttttggcgggttgtaagtgcttctcgacacttttcactcatggattcttcaaatttatggttaaagaggcacttatacactctgccctcaccagcttgtgtattttcacaaaaacgctcccgatcatctcggcaagcaaaatataaatgccggtctaagtgaaagtcatccgatgacagctcagccacccggagaatggctttcttgcagagttcagaaacttgaatcttgggttctctttcttctgcttctttcaccaggcctttctccaagcatgataccacctcaccttgtgaatgtgcatccttttctccaagccgaatactgccacatttcagaatgttgatgtcatttttgcagtcatccatgaagccacagattaaacggtaatcactaaaaatgatggccgtcatcttggtaatgtactggtgacactgatactcagtgatgttgcctcggtgatccaccaagcaggaaaccatgtaaccttttccaaccggttcatcagcacattctttaatctctgttatagtagatttgcaaacctctctggccacagattcaaatttgggatctgtagttaggttcagcttataattccacaacaactccctcacatcctgcaggcactcgagcaccgccaggttgttgctccaggtgtgcttagggcacacgcgggtcacgtcctccctgcaggactcttcctccgccagcttccagcccccaccagcccccgctcctccccgccgggccggaggcccacccgccgggaaaggcggctgcggcggctgaggctgctgttgctgttgctgctgctgctgttgctgctgaagctgcgatgactgaggcagctggggcagctgctgacccgccgggccgccgcctccggcctgccctacgaaggacacaaagttggccccgggaccctggccctggctgtggacgccctggccggggagtttctcggccccggccgcgaatagcagcagcagatgcagcgccgccgacaagcggaacatcctccgtacacgtccacacgccgccatcttgagtccgcggcgagctc

SEQ ID NO: 10059 - RNA, 1633 nt, Homo sapiens
  source 1..1633: mol_type = other RNA
caccgactctgtctcctgcagcttaaatactttttggtggcagcgggtgcttagctgcttcttgttttctttcagacattcgataatctgagcgttgccatattgcacagcggaacagaagtttttgatgtcactcttgcaggcttcgtatagatctggctccaagcggatgtcctccgtcatctccagctcctccacacggagctgcctgcggcacttcagggacaccctgtgctccttggcttcctgcagagtgtcattgcgcacggtcgtgctcaggcagatcaccacgtccaccttcttttttatgtttgggcaaagcttcaacacgtcctccttgcaggccattttaaacttgtaagaaaaccgaaaatccttcatctgcaccagctggaagtgggtaactccgatggcacacttctcgttcatgtccttctggtgtttgttctgtatcagacactccatcaggtccccagagtctatctggttatctgccacatcgtggcagaagttctgaattatgggctcacaggctctcatcagcaaggcttctatttgaatatcctctgattctaactcagtgaggttgccaactatatctctacactccaccaccaagtcatccagatggtcctgaaggcactccagctcctgtccagtctctgttttctcactgcaccattttcccagatcaatcaggcacttatcctggagggcaggatccagcttgacatccatggcacgctggtgtaggatcctttggacttcagctcggcactcccgtgagagcctccttccctgttcctcagtgcggtaggcgtgtcttgtgaatgtgcatccttttctccaagccgaatactgccacatttcagaatgttgatgtcatttttgcagtcatccatgaagccacagattaaacggtaatcactaaaaatgatggccgtcatcttggtaatgtactggtgacactgatactcagtgatgttgcctcggtgatccaccaagcaggaaaccatgtaaccttttccaaccggttcatcagcacattctttaatctctgttatagtagatttgcaaacctctctggccacagattcaaatttgggatctgtagttaggttcagcttataattccacaacaaatgattgcagtctgaagaaatttcattttcaggctccctcacatcctgcaggcactcgagcaccgccaggttgttgctccaggtgtgcttagggcacacgcgggtcacgtcctccctgcaggactcttcctccgccagcttccagcccccaccagcccccgctcctccccgccgggccggaggcccacccgccgggaaaggcggctgcggcggctgaggctgctgttgctgttgctgctgctgctgttgctgctgaagctgcgatgactgaggcagctggggcagctgctgacccgccgggccgccgcctccggcctgccctacgaaggacacaaagttggccccgggaccctggccctggctgtggacgccctggccggggagtttctcggccccggccgcgaatagcagcagcagatgcagcgccgccgacaagcggaacatcctccgtacacgtccacacgccgccatcttgagtccgcggcgagctc

SEQ ID NO: 10060 - RNA, 2745 nt, Homo sapiens
  source 1..2745: mol_type = other RNA
caccgactctgtctcctgcagcttaaatactttttggtggcagcgggtgcttagctgcttcttgttttctttcagacattcgataatctgagcgttgccatattgcacagcggaacagaagtttttgatgtcactcttgcaggcttcgtatagatctggctccaagcggatgtcctccgtcatctccagctcctccacacggagctgcctgcggcacttcagggacaccctgtgctccttggcttcctgcagagtgtcattgcgcacggtcgtgctcaggcagatcaccacgtccaccttcttttttatgtttgggcaaagcttcaacacgtcctccttgcaggccattttaaacttgtaagaaaaccgaaaatccttcatctgcaccagctggaagtgggtaactccgatggcacacttctcgttcatgtccttctggtgtttgttctgtatcagacactccatcaggtccccagagtctatctggttatctgccacatcgtggcagaagttctgaattatgggctcacaggctctcatcagcaaggcttctatttgaatatcttttggaaacgattctagtatttgaagtagatagccccagaataaatatagaactgctcctccgttatactttgaaaggcaaatttttaaagacatattccctttcggcctctgattctaactcagtgaggttgccaactatatctctacactccaccaccaagtcatccagatggtcctgaaggcactccagctcctgtccagtctctgttttctcactgcaccattttcccagatcaatcaggcacttatcctggagggcaggatccagcttgacatccatggcacgctggtgtaggatcctttggacttcagctcggcactcccgtgagagcctccttccctgttcctcagtgcggtaggcgtgtctgtataaacaagagaacacagctccctgaggcataaattcactggtctcattccaaccgtgggtgtggcaaagacgagaagcgtctccctggcacttgcggtacaggacagggtccagcttccaatcccgggagatgaaatactgcagctctaagagacggtgttcacagtcttctaccatcttctctgtgtataaatgttccatcaggcacgacaagatcattgggtctccagatcttatatgtttgcaggctgtctggattacagattcacaagcttcattcaaagctcgatcaatgcggtaatctgcaccagggtcagtctcctgaatcagtgtttgaagcgcctgctggcagttcattccaaggttccccttctcccctcgaactactttcatcagacagtgtagggtccgcccttttcgatgtaatccggaacaatggtgttcaatctccccccgacagcttaggatgatctcagggctcagagaaaagtcttccatcaacatgcgtcggtaatccagcatctccccctggcactcactgctgacttgtcgccctctgtgtacagctgactccaggcacattaacaagtaggagagcctggcttcacgcgatcgcggaaggttttccacattgcaccggtatttcttcaagtcacttttacaggatttggccaatgaataactgactttataatcctgggcaatcagcttttggcgggttgtaagtgcttctcgacacttttcactcatggattcttcaaatttatggttaaagaggcacttatacactctgccctcaccagcttgtgtattttcacaaaaacgctcccgatcatctcggcaagcaaaatataaatgccggtctaagtgaaagtcatccgatgacagctcagccacccggagaatggctttcttgcagagttcagaaacttgaatcttgggttctctttcttctgcttctttcaccaggcctttctccaagcatgataccacctcaccttgtgaatgtgcatccttttctccaagccgaatactgccacatttcagaatgttgatgtcatttttgcagtcatccatgaagccacagattaaacggtaatcactaaaaatgatggccgtcatcttggtaatgtactggtgacactgatactcagtgatgttgcctcggtgatccaccaagcaggaaaccatgtaaccttttccaaccggttcatcagcacattctttaatctctgttatagtagatttgcaaacctctctggccacagattcaaatttgggatctgtagttaggttcagcttataattccacaacaaatgattgcagtctgaagaaatttcattttcaggctccctcacatcctgcaggcactcgagcaccgccaggttgttgctccaggtgtgcttagggcacacgcgggtcacgtcctccctgcaggactcttcctccgccagcttccagcccccaccagcccccgctcctccccgccgggccggaggcccacccgccgggaaaggcggctgcggcggctgaggctgctgttgctgttgctgctgctgctgttgctgctgaagctgcgatgactgaggcagctggggcagctgctgacccgccgggccgccgcctccggcctgccctacgaaggacacaaagttggccccgggaccctggccctggctgtggacgccctggccggggagtttctcggccccggccgcgaatagcagcagcagatgcagcgccgccgacaagcggaacatcctccgtacacgtccacacgccgccatcttgagtccgcggcgagctc

SEQ ID NO: 10061 - RNA, 445 nt, Homo sapiens
  source 1..445: mol_type = other RNA
caccgactctgtctcctgcagcttggcagcaacctgactttttgccatgctcagaccctgaatcagggcctctgacttttggatctggtccctttcaatgtcatcacagcggcgctgccagtccaggcccagctgcacctgatcacgctccaggctccgctccctttccactgccagggacagctgttgcttgtacctttcaatgtcctgctgggatcgggccacctgtgccttgagcttcacctcttcttcctgcagcgtctgaatctgaaggtctctggagaccatctccttagatagttgagcaatttgagcatcccaggcagattttacagttgatgcatcttcacgaagtcaacggcctctggtgctctgggaagcagctttatccctggaccatgagccacctaattatgagggccagccccactcccagcatcaggat

SEQ ID NO: 10062 - RNA, 1888 nt, Homo sapiens
  source 1..1888: mol_type = other RNA
caccgactctgtctcctgcagcttggcagcaacctgactttttgccatgctcagaccctgaatcagggcctctgacttttggatctggtccctttcaatgtcatcacagcggcgctgccagtccaggcccagctgcacctgatcacgctccaggctccgctccctttccactgccagggacagctgttgcttgtacctttcaatgtcctgctgggatcgggccacctgtgccttgagcttcacctcttcttcctgcagcgtctgaatctgaaggtctctggagaccatctccttagatagttgagcaatttgagcatcccaggcagattttacagttgatgcatcttcacgaagtcctctgggtggagccaagcacacgctcactggtcaatggcagcgtccttctccttggcggtgtcagcctgtctccactctgccctgcggagctgcgcctcgagggtctcgcagtgggcctgcagctccagaaccctggtctgcagctcctgcagctgctccacgtgggctcccttcaccgccaccagcactgcatccttctccctggccagacggtcgagctcctcatgcttcctcttaaatgtttcctcttccttcttcctggttagctgcacagagtgaagtttatcctctaaatcctttaccctgaaaagaaacaaatatttatggaaggagcaagtgagatgaaagcaaagaccagcctggaatgagcagaaaaggtagaatcccccagactccagtcctggcctgcgaggctgccacagagcacgcctcgggagatgaaggactcgcgcaccgggcgcggctcatggcctccaggtcctggagctccccggctcggctctggagcttcctctccagctcggcgttggtggcctctgccctctgcagactctctgcagcctttgccccggcttccttcagagcctccagctctttgtgcagtagtttaaccttaagctcccgggacaaggctgtgttgctcatgttgtcagcctgcagacggaattcgtgctccctcttccgcattttcgattcaaactccagcagcagttcctgtctctgcagagcaagctcaccgtcgagctcctcaagttttctctccagtgtccattttagattttcatactgttcccggtggtggtcaatctcaccattcttgtcactgtggacgcgctccagctccaggcgatgctcctggaatgccagctgctgctgctgctgcagctcctccaccttcctggcctctctggctagcgcctgcctcagcttagctgcctctatcttgagctcgctcacctctgcccgcctggcctcttcccactccctggcctgggcgaaggcggcgtcatagcgctccagctcgaggtcccgctcctccagcacctgaaggttgtagacaaagtcctcctgcaggcaccgcagtttcccctgcgcctcctccagctggctccgtgtgtcctgcagagccgcctcctgcagctgggtgcggtgtgcctgcagcgccctccactcctcctccttgcgaagcagcagctcattcagggcgggctctgagcccagtggcagcatggtggccgctctctccaggcaggcggtgttggaactgaaccgaaggacacccgccgagtctgcggcagaactgactgctcatgtgctggtgaaaacctccctctcccaccacatttgatcacagaagtcttcctctgtgctgatgattcttgtggtatcagagtagaggaaaaacagtttgagttttccagaaataccctaacgcccgccagcagcgctggccaggtcccgccgcgttgccacagcgaccgggtcagtcggccgcgtccggctgcgctcggtgcagcgctcgggtcccgcc

SEQ ID NO: 10063 - RNA, 1408 nt, Homo sapiens
  source 1..1408: mol_type = other RNA
caccgactctgtctcctgcagcttggcagcaacctgactttttgccatgctcagaccctgaatcagggcctctgacttttggatctggtccctttcaatgtcatcacagcggcgctgccagtccaggcccagctgcacctgatcacgctccaggctccgctccctttccactgccagggacagctgttgcttgtacctttcaatgtcctgctgggatcgggccacctgtgccttgagcttcacctcttcttcctgcagcgtctgaatctgaaggtctctggagaccatctccttagatagttgagcaatttgagcatcccaggcagattttacagttgatgcatcttcacgaagttggtcaatggcagcgtccttctccttggcggtgtcagcctgtctccactctgccctgcggagctgcgcctcgagggtctcgcagtgggcctgcagctccagaaccctggtctgcagctcctgcagctgctccacgtgggctcccttcaccgccaccagcactgcatccttctccctggccagacggtcgagctcctcatgcccctgtaatcgcagcactttgggaggccgaggtgcgcggaccacttgaggacaagagtttgagaccagcctggccagcatggcaaactccatctttcctcttaaatgtttcctcttccttcttcctggttagctgcacagagtgaagtttatcctctaaatcctttacccgggcgcggctcatggcctccaggtcctggagctccccggctcggctctggagcttcctctccagctcggcgttggtggcctctgccctctgcagactctctgcagcctttgccccggcttccttcagagcctccagctctttgtgcagtagtttaaccttaagctcccgggacaaggctgtgttgctcatgttgtcagcctgcagacggaattcgtgctccctcttccgcattttcgattcaaactccagcagcagttcctgtctctgcagagcaagctcaccgtcgagctcctcaagttttctctccagtgtccattttagattttcatactgttcccggtggtggtcaatctcaccattcttgtcactctgcccgcctggcctcttcccactccctggcctgggcgaaggcggcgtcatagcgctccagctcgaggtcccgctcctccagcacctgaaggttgtagacaaagtcctcctgcaggcaccgcagtttcccctgcgcctcctccagctggctccgtgtgtcctgcagagccgcctcctgcagctgggtgcggtgtgcctgcagcgccctccactcctcctccttgcgaagcagcagctcattcagggcgggctctgagcccagtggcagcatggtggccgcctaacgcccgccagcagcgctggccaggtccc

SEQ ID NO: 10064 - RNA, 2081 nt, Homo sapiens
  source 1..2081: mol_type = other RNA
caccgactctgtctcctgcagcttggcagcaacctgactttttgccatgctcagaccctgaatcagggcctctgacttttggatctggtccctttcaatgtcatcacagcggcgctgccagtccaggcccagctgcacctgatcacgctccaggctccgctccctttccactgccagggacagctgttgcttgtacctttcaatgtcctgctgggatcgggccacctgtgccttgagcttcacctcttcttcctgcagcgtctgaatctgaaggtctctggagaccatctccttagatagttgagcaatttgagcatcccaggcagattttacagttgatgcatcttcacgaagttggtcaatggcagcgtccttctccttggcggtgtcagcctgtctccactctgccctgcggagctgcgcctcgagggtctcgcagtgggcctgcagctccagaaccctggtctgcagctcctgcagctgctccacgtgggctcccttcaccgccaccagcactgcatccttctccctggccagacggtcgagctcctcatgcttcctcttaaatgtttcctcttccttcttcctggttagctgcacagagtgaagtttatcctctaaatcctttacccgggcgcggctcatggcctccaggtcctggagctccccggctcggctctggagcttcctctccagctcggcgttggtggcctctgccctctgcagactctctgcagcctttgccccggcttccttcagagcctccagctctttgtgcagtagtttaaccttaagctcccgggacaaggctgtgttgctcatgttgtcagcctgcagacggaattcgtgctccctcttccgcattttcgattcaaactccagcagcagttcactgtccaggagagaagctggggtcagcgacactggtaacagcactctgggaggccgaggcgggaggatcgcttgagcccaggaattcaagaccagcctgggcaacacagtgaggccctgtcgctacagaaaaaaaaaagaaaagaaaaagaaaaatccttatctccattgagtcaattctacctctgacaataacaaacaccaagatcttccaaaacaagacaagaaatcagagcaaaggaaaccatgaaactgacaagcacgtaagaccctagcttagtaactaaaaggctgagatgccggcagtagaacagagcttcccgacagccagtgccagcatcccagagcccacacaggatcggactacccagaaccacaccggatgtgtgctgcccaagtttcccctagtaaccaaagctgccacgttaaaacgtcacgtttccttctttccagagacaaggatactatctgaacatgataaaaaatccatgttcccaacgtctgagatggctctccctgaacgagccctgctgagtctgagaaattcggcgtggacagcctgggaagtcagccatagtcacggcccagccagaaactctgacaagaatggctgcgccctgccaactacaaccagcctcaaatcgccactgtccccagatgctgccaagagccccccacctgctgggcaggaccacccacagctggatcctcctcaaactccttctttggaagtgactttggagccacttgaggaagcctcactacttagaaaagtcaccactggtctcttactgaccacggattttagacgctggcttcatgcctaaagaactccggctgttctcaaactcatccataatcgacaaagctctttggtttctgagaattccaagagaaagtcctctgcaggccatttcagaagcagcctcagggacctgtgaacaacgggagtgagctcagcacttccggggacaactggacagtccacaggagggcccatcatgacgtgagcgtggcctccttctctgctgacctgactgtggcaaattagtgacacactggcctatcctactatgaccaagctcccaacatccgacaggaccagagaggggaccctgtcacacctgcacaaagcccttcatcactgctgcacctgcacagacgcagccccttatgacacccccatagac

SEQ ID NO: 10065 - RNA, 1699 nt, Homo sapiens
  source 1..1699: mol_type = other RNA
caccgactctgtctcctgcagcttggcagcaacctgactttttgccatgctcagaccctgaatcagggcctctgacttttggatctggtccctttcaatgtcatcacagcggcgctgccagtccaggcccagctgcacctgatcacgctccaggctccgctccctttccactgccagggacagctgttgcttgtacctttcaatgtcctgctgggatcgggccacctgtgccttgagcttcacctcttcttcctgcagcgtctgaatctgaaggtctctggagaccatctccttagatagttgagcaatttgagcatcccaggcagattttacagttgatgcatcttcacgaagttggtcaatggcagcgtccttctccttggcggtgtcagcctgtctccactctgccctgcggagctgcgcctcgagggtctcgcagtgggcctgcagctccagaaccctggtctgcagctcctgcagctgctccacgtgggctcccttcaccgccaccagcactgcatccttctccctggccagacggtcgagctcctcatgcttcctcttaaatgtttcctcttccttcttcctggttagctgcacagagtgaagtttatcctctaaatcctttacccgggcgcggctcatggcctccaggtcctggagctccccggctcggctctggagcttcctctccagctcggcgttggtggcctctgccctctgcagactctctgcagcctttgccccggcttccttcagagcctccagctctttgtgcagtagtttaaccttaagctcccgggacaaggctgtgttgctcatgttgtcagcctgcagacggaattcgtgctccctcttccgcattttcgattcaaactccagcagcagttccgtcgagctcctcaagttttctctccagtgtccattttagattttcatactgttcccggtggtggtcaatctcaccattcttgtcactgtggacgcgctccagctccaggcgatgctcctggaatgccagctgctgctgctgctgcagctcctccaccttcctggcctctctggctagcgcctgcctcagcttagctgcctctatcttgagctcgctcacctctgcccgcctggcctcttcccactccctggcctgggcgaaggcggcgtcatagcgctccagctcgaggtcccgctcctccagcacctgaaggttgtagacaaagtcctcctgcaggcaccgcagtttcccctgcgcctcctccagctggctccgtgtgtcctgcagagccgcctcctgcagctgggtgcggtgtgcctgcagcgccctccactcctcctccttgcgaagcagcagctcattcagggcgggctctgagcccagtggcagcatggtggccgcctgtggtctgacctctctccaggcaggcggtgttggaactgaaccgaaggacacccgccgagtctgcggcagaactgactgctcatgtgctggtgaaaacctccctctcccaccacatttgatcacagaagtcttcctctgtgctgatgattcttgtggtatcagagtagaggaaaaacagtttgagttttccagaaataccctaacgcccgccagcagcgctggccaggtcccgccgcgttgccacagcgaccgggtcagtcggccgcgtccggctgcgctcggtgcagcgctcgggtcccgccg

SEQ ID NO: 10066 - RNA, 1686 nt, Homo sapiens
  source 1..1686: mol_type = other RNA
caccgactctgtctcctgcagcttggcagcaacctgactttttgccatgctcagaccctgaatcagggcctctgacttttggatctggtccctttcaatgtcatcacagcggcgctgccagtccaggcccagctgcacctgatcacgctccaggctccgctccctttccactgccagggacagctgttgcttgtacctttcaatgtcctgctgggatcgggccacctgtgccttgagcttcacctcttcttcctgcagcgtctgaatctgaaggtctctggagaccatctccttagatagttgagcaatttgagcatcccaggcagattttacagttgatgcatcttcacgaagttggtcaatggcagcgtccttctccttggcggtgtcagcctgtctccactctgccctgcggagctgcgcctcgagggtctcgcagtgggcctgcagctccagaaccctggtctgcagctcctgcagctgctccacgtgggctcccttcaccgccaccagcactgcatccttctccctggccagacggtcgagctcctcatgcttcctcttaaatgtttcctcttccttcttcctggttagctgcacagagtgaagtttatcctctaaatcctttacccgggcgcggctcatggcctccaggtcctggagctccccggctcggctctggagcttcctctccagctcggcgttggtggcctctgccctctgcagactctctgcagcctttgccccggcttccttcagagcctccagctctttgtgcagtagtttaaccttaagctcccgggacaaggctgtgttgctcatgttgtcagcctgcagacggaattcgtgctccctcttccgcattttcgattcaaactccagcagcagttccgtcgagctcctcaagttttctctccagtgtccattttagattttcatactgttcccggtggtggtcaatctcaccattcttgtcactgtggacgcgctccagctccaggcgatgctcctggaatgccagctgctgctgctgctgcagctcctccaccttcctggcctctctggctagcgcctgcctcagcttagctgcctctatcttgagctcgctcacctctgcccgcctggcctcttcccactccctggcctgggcgaaggcggcgtcatagcgctccagctcgaggtcccgctcctccagcacctgaaggttgtagacaaagtcctcctgcaggcaccgcagtttcccctgcgcctcctccagctggctccgtgtgtcctgcagagccgcctcctgcagctgggtgcggtgtgcctgcagcgccctccactcctcctccttgcgaagcagcagctcattcagggcgggctctgagcccagtggcagcatggtggccgctctctccaggcaggcggtgttggaactgaaccgaaggacacccgccgagtctgcggcagaactgactgctcatgtgctggtgaaaacctccctctcccaccacatttgatcacagaagtcttcctctgtgctgatgattcttgtggtatcagagtagaggaaaaacagtttgagttttccagaaataccctaacgcccgccagcagcgctggccaggtcccgccgcgttgccacagcgaccgggtcagtcggccgcgtccggctgcgctcggtgcagcgctcgggtcccgccg

SEQ ID NO: 10067 - RNA, 1478 nt, Homo sapiens
  source 1..1478: mol_type = other RNA
caccgactctgtctcctgcagcttggcagcaacctgactttttgccatgctcagaccctgaatcagggcctctgacttttggatctggtccctttcaatgtcatcacagcggcgctgccagtccaggcccagctgcacctgatcacgctccaggctccgctccctttccactgccagggacagctgttgcttgtacctttcaatgtcctgctgggatcgggccacctgtgccttgagcttcacctcttcttcctgcagcgtctgaatctgaaggtctctggagaccatctccttagatagttgagcaatttgagcatcccaggcagattttacagttgatgcatcttcacgaagttggtcaatggcagcgtccttctccttggcggtgtcagcctgtctccactctgccctgcggagctgcgcctcgagggtctcgcagtgggcctgcagctccagaaccctggtctgcagctcctgcagctgctccacgtgggctcccttcaccgccaccagcactgcatccttctccctggccagacggtcgagctcctcatgcttcctcttaaatgtttcctcttccttcttcctggttagctgcacagagtgaagtttatcctctaaatcctttacccgggcgcggctcatggcctccaggtcctggagctccccggctcggctctggagcttcctctccagctcggcgttggtggcctctgccctctgcagactctctgcagcctttgccccggcttccttcagagcctccagctctttgtgcagtagtttaaccttaagctcccgggacaaggctgtgttgctcatgttgtcagcctgcagacggaattcgtgctccctcttccgcattttcgattcaaactccagcagcagttcctgcatagacagagccatttattacacctgcacctgcagagacgcagcccctcatcacacctgcaccttcacagaagaagcccctcaggacacctgcagagacgcagcccctcatgactcctgcacctgcagagacgcagcccctcgtgactcctgcagagacgcagcccctcatgactcctgcacctgcagagacgcagcccctcgtgactcctgcacctgcagagacgcagcccctcgtgactcctgcacctgcagagacgcagcccctcgtgactcctgcagagactcagcccctcgtgactcctgcagacgcagcccctcatgactcctgcagagatgcagcccctcgtgactcctgcagagacgcagcccctcgtgactcctgcacctgtctctgcagagcaagctcaccgtcgagctcctcaagttttctctccagtgtccattttagattttcatactgttcccggtggtggtcaatctcaccattcttgtcactctgcccgcctggcctcttcccactccctggcctgggcgaaggcggcgtcatagcgctccagctcgaggtcccgctcctccagcac

SEQ ID NO: 10068 - RNA, 1081 nt, Homo sapiens
  source 1..1081: mol_type = other RNA
caccgactctgtctcctgcagcttggcagcaacctgactttttgccatgctcagaccctgaatcagggcctctgacttttggatctggtccctttcaatgtcatcacagcggcgctgccagtccaggcccagctgcacctgatcacgctccaggctccgctccctttccactgccagggacagctgttgcttgtacctttcaatgtcctgctgggatcgggccacctgtgccttgagcttcacctcttcttcctgcagcgtctgaatctgaaggtctctggagaccatctccttagatagttgagcaatttgagcatcccaggcagattttacagttgatgcatcttcacgaagttggtcaatggcagcgtccttctccttggcggtgtcagcctgtctccactctgccctgcggagctgcgcctcgagggtctcgcagtgggcctgcagctccagaaccctggtctgcagctcctgcagctgctccacgtgggctcccttcaccgccaccagcactgcatccttctccctggccagacggtcgagctcctcatgcttcctcttaaatgtttcctcttccttcttcctggttagctgcacagagtgaagtttatcctctaaatcctttacccgggcgcggctcatggcctccaggtcctggagctccccggctcggctctggagcttcctctccagctcggcgttggtggcctctgccctctgcagactctctgcagcctttgccccggcttccttcagagcctccagctctttgtgcagtagtttaaccttaagctcccgggacaaggctgtgttgctcatgttgtcagcctgcagacggaattcgtgctccctcttccgcattttcgattcaaactccagcagcagttcctgtctctgcagagcaagctcaccgtcgagctcctcaagttttctctccagtgtccattttagattttcatactgttcccggtggtggtcaatctcaccattcttgtcactctgcccgcctggcctcttcccactccctggcctgggcgaaggcggcgtcatagcgctccagctcgaggtcccgctcctc

SEQ ID NO: 10069 - RNA, 1302 nt, Homo sapiens
  source 1..1302: mol_type = other RNA
caccgactctgtctcctgcagcttggcagcaacctgactttttgccatgctcagaccctgaatcagggcctctgacttttggatctggtccctttcaatgtcatcacagcggcgctgccagtccaggcccagctgcacctgatcacgctccaggctccgctccctttccactgccagggacagctgttgcttgtacctttcaatgtcctgctgggatcgggccacctgtgccttgagcttcacctcttcttcctgcagcgtctgaatctgaaggtctctggagaccatctccttagatagttgagcaatttgagcatcccaggcagattttacagttgatgcatcttcacgaagttggtcaatggcagcgtccttctccttggcggtgtcagcctgtctccactctgccctgcggagctgcgcctcgagggtctcgcagtgggcctgcagctccagaaccctggtctgcagctcctgcagctgctccacgtgggctcccttcaccgccaccagcactgcatccttctccctggccagacggtcgagctcctcatgcttcctcttaaatgtttcctcttccttcttcctggttagctgcacagagtgaagtttatcctctaaatcctttacccgggcgcggctcatggcctccaggtcctggagctccccggctcggctctggagcttcctctccagctcggcgttggtggcctctgccctctgcagactctctgcagcctttgccccggcttccttcagagcctccagctctttgtgcagtagtttaaccttaagctcccgggacaaggctgtgttgctcatgttgtcagcctgcagacggaattcgtgctccctcttccgcattttcgattcaaactccagcagcagttcctgtctctgcagagcaagctcaccgtcgagctcctcaagttttctctccagtgtccattttagattttcatactgttcccggtggtggtcaatctcaccattcttgtcactgaaggttgtagacaaagtcctcctgcaggcaccgcagtttcccctgcgcctcctccagctggctccgtgtgtcctgcagagccgcctcctgcagctgggtgcggtgtgcctgcagcgccctccactcctcctccttgcgaagcagcagctcattcagggcgggctctgagcccagtggcagcatggtggccgcctaacgcccgccagcagcgctggccaggtcccgccgcgttgccacagcgaccgggtcagtcggccgcgtccggctgcgctcggtgcagcgctcgggtcccgccgaca

SEQ ID NO: 10070 - RNA, 1501 nt, Homo sapiens
  source 1..1501: mol_type = other RNA
caccgactctgtctcctgcagcttggcagcaacctgactttttgccatgctcagaccctgaatcagggcctctgacttttggatctggtccctttcaatgtcatcacagcggcgctgccagtccaggcccagctgcacctgatcacgctccaggctccgctccctttccactgccagggacagctgttgcttgtacctttcaatgtcctgctgggatcgggccacctgtgccttgagcttcacctcttcttcctgcagcgtctgaatctgaaggtctctggagaccatctccttagatagttgagcaatttgagcatcccaggcagattttacagttgatgcatcttcacgaagttggtcaatggcagcgtccttctccttggcggtgtcagcctgtctccactctgccctgcggagctgcgcctcgagggtctcgcagtgggcctgcagctccagaaccctggtctgcagctcctgcagctgctccacgtgggctcccttcaccgccaccagcactgcatccttctccctggccagacggtcgagctcctcatgcttcctcttaaatgtttcctcttccttcttcctggttagctgcacagagtgaagtttatcctctaaatcctttacccgggcgcggctcatggcctccaggtcctggagctccccggctcggctctggagcttcctctccagctcggcgttggtggcctctgccctctgcagactctctgcagcctttgccccggcttccttcagagcctccagctctttgtgcagtagtttaaccttaagctcccgggacaaggctgtgttgctcatgttgtcagcctgcagacggaattcgtgctccctcttccgcattttcgattcaaactccagcagcagttcctgtctctgcagagcaagctcaccgtcgagctcctcaagttttctctccagtgtccattttagattttcatactgttcccggtggtggtcaatctcaccattcttgtcactgaaggttgtagacaaagtcctcctgcaggcaccgcagtttcccctgcgcctcctccagctggctccgtgtgtcctgcagagccgcctcctgcagctgggtgcggtgtgcctgcagcgccctccactcctcctccttgcgaagcagcagctcattcagggcgggctctgagcccagtggcagcatggtggccgcctgtggtctgacctctctccaggcaggcggtgttggaactgaaccgaaggacacccgccgagtctgcggcagaactgactgctcatgtgctggtgaaaacctccctctcccaccacatttgatcacagaagtcttcctctgtgctgatgattcttgtggtatcagagtagaggaaaaacagtttgagttttccagaaataccctaacgcccgccagcagcgctggccaggtcccgccgcgttgccacagcgaccgggtcagtcggccgcgtccggctgcgctcggtgcagcgctcgggtcccgccg

SEQ ID NO: 10071 - RNA, 1473 nt, Homo sapiens
  source 1..1473: mol_type = other RNA
caccgactctgtctcctgcagcttggcagcaacctgactttttgccatgctcagaccctgaatcagggcctctgacttttggatctggtccctttcaatgtcatcacagcggcgctgccagtccaggcccagctgcacctgatcacgctccaggctccgctccctttccactgccagggacagctgttgcttgtacctttcaatgtcctgctgggatcgggccacctgtgccttgagcttcacctcttcttcctgcagcgtctgaatctgaaggtctctggagaccatctccttagatagttgagcaatttgagcatcccaggcagattttacagttgatgcatcttcacgaagttggtcaatggcagcgtccttctccttggcggtgtcagcctgtctccactctgccctgcggagctgcgcctcgagggtctcgcagtgggcctgcagctccagaaccctggtctgcagctcctgcagctgctccacgtgggctcccttcaccgccaccagcactgcatccttctccctggccagacggtcgagctcctcatgcttcctcttaaatgtttcctcttccttcttcctggttagctgcacagagtgaagtttatcctctaaatcctttacccgggcgcggctcatggcctccaggtcctggagctccccggctcggctctggagcttcctctccagctcggcgttggtggcctctgccctctgcagactctctgcagcctttgccccggcttccttcagagcctccagctctttgtgcagtagtttaaccttaagctcccgggacaaggctgtgttgctcatgttgtcagcctgcagacggaattcgtgctccctcttccgcattttcgattcaaactccagcagcagttcctgtctctgcagagcaagctcaccgtcgagctcctcaagttttctctccagtgtccattttagattttcatactgttcccggtggtggtcaatctcaccattcttgtcactgtggacgcgctccagctccaggcgatgctcctggaatgccagctgctgctgctgctgcagctcctccaccttcctggcctctctggctagcgcctgcctcagcttagctgcctctatcttgagctcgctcacctctgcccgcctggcctcttcccactccctggcctgggcgaaggcggcgtcatagcgctccagctcgaggtcccgctcctccagcacctgaaggttgtagacaaagtcctcctgcaggcaccgcagtttcccctgcgcctcctccagctggctccgtgtgtcctgcagagccgcctcctgcagctgggtgcggtgtgcctgcagcgccctccactcctcctccttgcgaagcagcagctcattcagggcgggctctgagcccagtggcagcatggtggccgcctaacgcccgccagcagcgctggccaggtcccgccgcgttgccacagcgaccgggtc

SEQ ID NO: 10072 - RNA, 1523 nt, Homo sapiens
  source 1..1523: mol_type = other RNA
caccgactctgtctcctgcagcttggcagcaacctgactttttgccatgctcagaccctgaatcagggcctctgacttttggatctggtccctttcaatgtcatcacagcggcgctgccagtccaggcccagctgcacctgatcacgctccaggctccgctccctttccactgccagggacagctgttgcttgtacctttcaatgtcctgctgggatcgggccacctgtgccttgagcttcacctcttcttcctgcagcgtctgaatctgaaggtctctggagaccatctccttagatagttgagcaatttgagcatcccaggcagattttacagttgatgcatcttcacgaagttggtcaatggcagcgtccttctccttggcggtgtcagcctgtctccactctgccctgcggagctgcgcctcgagggtctcgcagtgggcctgcagctccagaaccctggtctgcagctcctgcagctgctccacgtgggctcccttcaccgccaccagcactgcatccttctccctggccagacggtcgagctcctcatgcttcctcttaaatgtttcctcttccttcttcctggttagctgcacagagtgaagtttatcctctaaatcctttacccgggcgcggctcatggcctccaggtcctggagctccccggctcggctctggagcttcctctccagctcggcgttggtggcctctgccctctgcagactctctgcagcctttgccccggcttccttcagagcctccagctctttgtgcagtagtttaaccttaagctcccgggacaaggctgtgttgctcatgttgtcagcctgcagacggaattcgtgctccctcttccgcattttcgattcaaactccagcagcagttcctgtctctgcagagcaagctcaccgtcgagctcctcaagttttctctccagtgtccattttagattttcatactgttcccggtggtggtcaatctcaccattcttgtcactgtggacgcgctccagctccaggcgatgctcctggaatgccagctgctgctgctgctgcagctcctccaccttcctggcctctctggctagcgcctgcctcagcttagctgcctctatcttgagctcgctcacctctgcccgcctggcctcttcccactccctggcctgggcgaaggcggcgtcatagcgctccagctcgaggtcccgctcctccagcacctgaaggttgtagacaaagtcctcctgcaggcaccgcagtttcccctgcgcctcctccagctggctccgtgtgtcctgcagagccgcctcctgcagctgggtgcggtgtgcctgcagcgccctccactcctcctccttgcgaagcagcagctcattcagggcgggctctgagcccagtggcagcatggtggccgcctaacgcccgccagcagcgctggccaggtcccgccgcgttgccacagcgaccgggtcagtcggccgcgtccggctgcgctcggtgcagcgctcgggtcccgccgaca

SEQ ID NO: 10073 - RNA, 1722 nt, Homo sapiens
  source 1..1722: mol_type = other RNA
caccgactctgtctcctgcagcttggcagcaacctgactttttgccatgctcagaccctgaatcagggcctctgacttttggatctggtccctttcaatgtcatcacagcggcgctgccagtccaggcccagctgcacctgatcacgctccaggctccgctccctttccactgccagggacagctgttgcttgtacctttcaatgtcctgctgggatcgggccacctgtgccttgagcttcacctcttcttcctgcagcgtctgaatctgaaggtctctggagaccatctccttagatagttgagcaatttgagcatcccaggcagattttacagttgatgcatcttcacgaagttggtcaatggcagcgtccttctccttggcggtgtcagcctgtctccactctgccctgcggagctgcgcctcgagggtctcgcagtgggcctgcagctccagaaccctggtctgcagctcctgcagctgctccacgtgggctcccttcaccgccaccagcactgcatccttctccctggccagacggtcgagctcctcatgcttcctcttaaatgtttcctcttccttcttcctggttagctgcacagagtgaagtttatcctctaaatcctttacccgggcgcggctcatggcctccaggtcctggagctccccggctcggctctggagcttcctctccagctcggcgttggtggcctctgccctctgcagactctctgcagcctttgccccggcttccttcagagcctccagctctttgtgcagtagtttaaccttaagctcccgggacaaggctgtgttgctcatgttgtcagcctgcagacggaattcgtgctccctcttccgcattttcgattcaaactccagcagcagttcctgtctctgcagagcaagctcaccgtcgagctcctcaagttttctctccagtgtccattttagattttcatactgttcccggtggtggtcaatctcaccattcttgtcactgtggacgcgctccagctccaggcgatgctcctggaatgccagctgctgctgctgctgcagctcctccaccttcctggcctctctggctagcgcctgcctcagcttagctgcctctatcttgagctcgctcacctctgcccgcctggcctcttcccactccctggcctgggcgaaggcggcgtcatagcgctccagctcgaggtcccgctcctccagcacctgaaggttgtagacaaagtcctcctgcaggcaccgcagtttcccctgcgcctcctccagctggctccgtgtgtcctgcagagccgcctcctgcagctgggtgcggtgtgcctgcagcgccctccactcctcctccttgcgaagcagcagctcattcagggcgggctctgagcccagtggcagcatggtggccgcctgtggtctgacctctctccaggcaggcggtgttggaactgaaccgaaggacacccgccgagtctgcggcagaactgactgctcatgtgctggtgaaaacctccctctcccaccacatttgatcacagaagtcttcctctgtgctgatgattcttgtggtatcagagtagaggaaaaacagtttgagttttccagaaataccctaacgcccgccagcagcgctggccaggtcccgccgcgttgccacagcgaccgggtcagtcggccgcgtccggctgcgctcggtgcagcgctcgggtcccgccg

SEQ ID NO: 10074 - RNA, 1661 nt, Homo sapiens
  source 1..1661: mol_type = other RNA
caccgactctgtctcctgcagcttggcagcaacctgactttttgccatgctcagaccctgaatcagggcctctgacttttggatctggtccctttcaatgtcatcacagcggcgctgccagtccaggcccagctgcacctgatcacgctccaggctccgctccctttccactgccagggacagctgttgcttgtacctttcaatgtcctgctgggatcgggccacctgtgccttgagcttcacctcttcttcctgcagcgtctgaatctgaaggtctctggagaccatctccttagatagttgagcaatttgagcatcccaggcagattttacagttgatgcatcttcacgaagttggtcaatggcagcgtccttctccttggcggtgtcagcctgtctccactctgccctgcggagctgcgcctcgagggtctcgcagtgggcctgcagctccagaaccctggtctgcagctcctgcagctgctccacgtgggctcccttcaccgccaccagcactgcatccttctccctggccagacggtcgagctcctcatgcttcctcttaaatgtttcctcttccttcttcctggttagctgcacagagtgaagtttatcctctaaatcctttacccgggcgcggctcatggcctccaggtcctggagctccccggctcggctctggagcttcctctccagctcggcgttggtggcctctgccctctgcagactctctgcagcctttgccccggcttccttcagagcctccagctctttgtgcagtagtttaaccttaagctcccgggacaaggctgtgttgctcatgttgtcagcctgcagacggaattcgtgctccctcttccgcattttcgattcaaactccagcagcagttcctgtctctgcagagcaagctcaccgtcgagctcctcaagttttctctccagtgtccattttagattttcatactgttcccggtggtggtcaatctcaccattcttgtcactgtggacgcgctccagctccaggcgatgctcctggaatgccagctgctgctgctgctgcagctcctccaccttcctggcctctctggctagcgcctgcctcagcttagctgcctctatcttgagctcgctcacctctgcccgcctggcctcttcccactccctggcctgggcgaaggcggcgtcatagcgctccagctcgaggtcccgctcctccagcacctgaaggttgtagacaaagtcctcctgcaggcaccgcagtttcccctgcgcctcctccagctggctccgtgtgtcctgcagagccgcctcctgcagctgggtgcggtgtgcctgcagcgccctccactcctcctccttgcgaagcagcagctcattcagggcgggctctgagcccagtggcagcatggtggccgcctgtggtctgacctctctccaggcaggcggtgttggaactgaaccgaaggacacccgccgagtctgcggcagaactgactgctcatgtgctggtgaaaacctccctctcccaccacatttgatcacagaagtcttcctctgtgctgatgattcttgtggtatcagagtagaggaaaaacagtttgagttttccagaaatacctgtgaccccgtgttttttttcacttcctccactgactgccgaa

SEQ ID NO: 10075 - RNA, 1668 nt, Homo sapiens
  source 1..1668: mol_type = other RNA
caccgactctgtctcctgcagcttggcagcaacctgactttttgccatgctcagaccctgaatcagggcctctgacttttggatctggtccctttcaatgtcatcacagcggcgctgccagtccaggcccagctgcacctgatcacgctccaggctccgctccctttccactgccagggacagctgttgcttgtacctttcaatgtcctgctgggatcgggccacctgtgccttgagcttcacctcttcttcctgcagcgtctgaatctgaaggtctctggagaccatctccttagatagttgagcaatttgagcatcccaggcagattttacagttgatgcatcttcacgaagttggtcaatggcagcgtccttctccttggcggtgtcagcctgtctccactctgccctgcggagctgcgcctcgagggtctcgcagtgggcctgcagctccagaaccctggtctgcagctcctgcagctgctccacgtgggctcccttcaccgccaccagcactgcatccttctccctggccagacggtcgagctcctcatgcttcctcttaaatgtttcctcttccttcttcctggttagctgcacagagtgaagtttatcctctaaatcctttacccgggcgcggctcatggcctccaggtcctggagctccccggctcggctctggagcttcctctccagctcggcgttggtggcctctgccctctgcagactctctgcagcctttgccccggcttccttcagagcctccagctctttgtgcagtagtttaaccttaagctcccgggacaaggctgtgttgctcatgttgtcagcctgcagacggaattcgtgctccctcttccgcattttcgattcaaactccagcagcagttcctgtctctgcagagcaagctcaccgtcgagctcctcaagttttctctccagtgtccattttagattttcatactgttcccggtggtggtcaatctcaccattcttgtcactgtggacgcgctccagctccaggcgatgctcctggaatgccagctgctgctgctgctgcagctcctccaccttcctggcctctctggctagcgcctgcctcagcttagctgcctctatcttgagctcgctcacctctgcccgcctggcctcttcccactccctggcctgggcgaaggcggcgtcatagcgctccagctcgaggtcccgctcctccagcacctgaaggttgtagacaaagtcctcctgcaggcaccgcagtttcccctgcgcctcctccagctggctccgtgtgtcctgcagagccgcctcctgcagctgggtgcggtgtgcctgcagcgccctccactcctcctccttgcgaagcagcagctcattcagggcgggctctgagcccagtggcagcatggtggccgcctgtggtctgacctctctccaggcaggcggtgttggaactgaaccgaaggacacccgccgagtctgcggcagaactgactgctcatgtgctggtgaaaacctccctctcccaccacatttgatcacagaagtcttcctctgtgctgatgattcttgtggtatcagagtagaggaaaaacagtttgagttttccagaaatacctgtgaccccgtgttttttttcacttcctccactgactgccgaagagtagc

SEQ ID NO: 10076 - RNA, 1670 nt, Homo sapiens
  source 1..1670: mol_type = other RNA
caccgactctgtctcctgcagcttggcagcaacctgactttttgccatgctcagaccctgaatcagggcctctgacttttggatctggtccctttcaatgtcatcacagcggcgctgccagtccaggcccagctgcacctgatcacgctccaggctccgctccctttccactgccagggacagctgttgcttgtacctttcaatgtcctgctgggatcgggccacctgtgccttgagcttcacctcttcttcctgcagcgtctgaatctgaaggtctctggagaccatctccttagatagttgagcaatttgagcatcccaggcagattttacagttgatgcatcttcacgaagttggtcaatggcagcgtccttctccttggcggtgtcagcctgtctccactctgccctgcggagctgcgcctcgagggtctcgcagtgggcctgcagctccagaaccctggtctgcagctcctgcagctgctccacgtgggctcccttcaccgccaccagcactgcatccttctccctggccagacggtcgagctcctcatgcttcctcttaaatgtttcctcttccttcttcctggttagctgcacagagtgaagtttatcctctaaatcctttacccgggcgcggctcatggcctccaggtcctggagctccccggctcggctctggagcttcctctccagctcggcgttggtggcctctgccctctgcagactctctgcagcctttgccccggcttccttcagagcctccagctctttgtgcagtagtttaaccttaagctcccgggacaaggctgtgttgctcatgttgtcagcctgcagacggaattcgtgctccctcttccgcattttcgattcaaactccagcagcagttcctgtctctgcagagcaagctcaccgtcgagctcctcaagttttctctccagtgtccattttagattttcatactgttcccggtggtggtcaatctcaccattcttgtcactgtggacgcgctccagctccaggcgatgctcctggaatgccagctgctgctgctgctgcagctcctccaccttcctggcctctctggctagcgcctgcctcagcttagctgcctctatcttgagctcgctcacctctgcccgcctggcctcttcccactccctggcctgggcgaaggcggcgtcatagcgctccagctcgaggtcccgctcctccagcacctgaaggttgtagacaaagtcctcctgcaggcaccgcagtttcccctgcgcctcctccagctggctccgtgtgtcctgcagagccgcctcctgcagctgggtgcggtgtgcctgcagcgccctccactcctcctccttgcgaagcagcagctcattcagggcgggctctgagcccagtggcagcatggtggccgcctgtggtctgacctctctccaggcaggcggtgttggaactgaaccgaaggacacccgccgagtctgcggcagaactgactgctcatgtgctggtgaaaacctccctctcccaccacatttgatcacagaagtcttcctctgtgctgatgattcttgtggtatcagagtagaggaaaaacagtttgagttttccagaaatacctgtgaccccgtgttttttttcacttcctccactgactgccgaagagtagcca

SEQ ID NO: 10077 - RNA, 1671 nt, Homo sapiens
  source 1..1671: mol_type = other RNA
caccgactctgtctcctgcagcttggcagcaacctgactttttgccatgctcagaccctgaatcagggcctctgacttttggatctggtccctttcaatgtcatcacagcggcgctgccagtccaggcccagctgcacctgatcacgctccaggctccgctccctttccactgccagggacagctgttgcttgtacctttcaatgtcctgctgggatcgggccacctgtgccttgagcttcacctcttcttcctgcagcgtctgaatctgaaggtctctggagaccatctccttagatagttgagcaatttgagcatcccaggcagattttacagttgatgcatcttcacgaagttggtcaatggcagcgtccttctccttggcggtgtcagcctgtctccactctgccctgcggagctgcgcctcgagggtctcgcagtgggcctgcagctccagaaccctggtctgcagctcctgcagctgctccacgtgggctcccttcaccgccaccagcactgcatccttctccctggccagacggtcgagctcctcatgcttcctcttaaatgtttcctcttccttcttcctggttagctgcacagagtgaagtttatcctctaaatcctttacccgggcgcggctcatggcctccaggtcctggagctccccggctcggctctggagcttcctctccagctcggcgttggtggcctctgccctctgcagactctctgcagcctttgccccggcttccttcagagcctccagctctttgtgcagtagtttaaccttaagctcccgggacaaggctgtgttgctcatgttgtcagcctgcagacggaattcgtgctccctcttccgcattttcgattcaaactccagcagcagttcctgtctctgcagagcaagctcaccgtcgagctcctcaagttttctctccagtgtccattttagattttcatactgttcccggtggtggtcaatctcaccattcttgtcactgtggacgcgctccagctccaggcgatgctcctggaatgccagctgctgctgctgctgcagctcctccaccttcctggcctctctggctagcgcctgcctcagcttagctgcctctatcttgagctcgctcacctctgcccgcctggcctcttcccactccctggcctgggcgaaggcggcgtcatagcgctccagctcgaggtcccgctcctccagcacctgaaggttgtagacaaagtcctcctgcaggcaccgcagtttcccctgcgcctcctccagctggctccgtgtgtcctgcagagccgcctcctgcagctgggtgcggtgtgcctgcagcgccctccactcctcctccttgcgaagcagcagctcattcagggcgggctctgagcccagtggcagcatggtggccgcctgtggtctgacctctctccaggcaggcggtgttggaactgaaccgaaggacacccgccgagtctgcggcagaactgactgctcatgtgctggtgaaaacctccctctcccaccacatttgatcacagaagtcttcctctgtgctgatgattcttgtggtatcagagtagaggaaaaacagtttgagttttccagaaatacctgtgaccccgtgttttttttcacttcctccactgactgccgaagagtagccac

SEQ ID NO: 10078 - RNA, 1672 nt, Homo sapiens
  source 1..1672: mol_type = other RNA
caccgactctgtctcctgcagcttggcagcaacctgactttttgccatgctcagaccctgaatcagggcctctgacttttggatctggtccctttcaatgtcatcacagcggcgctgccagtccaggcccagctgcacctgatcacgctccaggctccgctccctttccactgccagggacagctgttgcttgtacctttcaatgtcctgctgggatcgggccacctgtgccttgagcttcacctcttcttcctgcagcgtctgaatctgaaggtctctggagaccatctccttagatagttgagcaatttgagcatcccaggcagattttacagttgatgcatcttcacgaagttggtcaatggcagcgtccttctccttggcggtgtcagcctgtctccactctgccctgcggagctgcgcctcgagggtctcgcagtgggcctgcagctccagaaccctggtctgcagctcctgcagctgctccacgtgggctcccttcaccgccaccagcactgcatccttctccctggccagacggtcgagctcctcatgcttcctcttaaatgtttcctcttccttcttcctggttagctgcacagagtgaagtttatcctctaaatcctttacccgggcgcggctcatggcctccaggtcctggagctccccggctcggctctggagcttcctctccagctcggcgttggtggcctctgccctctgcagactctctgcagcctttgccccggcttccttcagagcctccagctctttgtgcagtagtttaaccttaagctcccgggacaaggctgtgttgctcatgttgtcagcctgcagacggaattcgtgctccctcttccgcattttcgattcaaactccagcagcagttcctgtctctgcagagcaagctcaccgtcgagctcctcaagttttctctccagtgtccattttagattttcatactgttcccggtggtggtcaatctcaccattcttgtcactgtggacgcgctccagctccaggcgatgctcctggaatgccagctgctgctgctgctgcagctcctccaccttcctggcctctctggctagcgcctgcctcagcttagctgcctctatcttgagctcgctcacctctgcccgcctggcctcttcccactccctggcctgggcgaaggcggcgtcatagcgctccagctcgaggtcccgctcctccagcacctgaaggttgtagacaaagtcctcctgcaggcaccgcagtttcccctgcgcctcctccagctggctccgtgtgtcctgcagagccgcctcctgcagctgggtgcggtgtgcctgcagcgccctccactcctcctccttgcgaagcagcagctcattcagggcgggctctgagcccagtggcagcatggtggccgcctgtggtctgacctctctccaggcaggcggtgttggaactgaaccgaaggacacccgccgagtctgcggcagaactgactgctcatgtgctggtgaaaacctccctctcccaccacatttgatcacagaagtcttcctctgtgctgatgattcttgtggtatcagagtagaggaaaaacagtttgagttttccagaaatacctgtgaccccgtgttttttttcacttcctccactgactgccgaagagtagccaca

SEQ ID NO: 10079 - RNA, 1673 nt, Homo sapiens
  source 1..1673: mol_type = other RNA
caccgactctgtctcctgcagcttggcagcaacctgactttttgccatgctcagaccctgaatcagggcctctgacttttggatctggtccctttcaatgtcatcacagcggcgctgccagtccaggcccagctgcacctgatcacgctccaggctccgctccctttccactgccagggacagctgttgcttgtacctttcaatgtcctgctgggatcgggccacctgtgccttgagcttcacctcttcttcctgcagcgtctgaatctgaaggtctctggagaccatctccttagatagttgagcaatttgagcatcccaggcagattttacagttgatgcatcttcacgaagttggtcaatggcagcgtccttctccttggcggtgtcagcctgtctccactctgccctgcggagctgcgcctcgagggtctcgcagtgggcctgcagctccagaaccctggtctgcagctcctgcagctgctccacgtgggctcccttcaccgccaccagcactgcatccttctccctggccagacggtcgagctcctcatgcttcctcttaaatgtttcctcttccttcttcctggttagctgcacagagtgaagtttatcctctaaatcctttacccgggcgcggctcatggcctccaggtcctggagctccccggctcggctctggagcttcctctccagctcggcgttggtggcctctgccctctgcagactctctgcagcctttgccccggcttccttcagagcctccagctctttgtgcagtagtttaaccttaagctcccgggacaaggctgtgttgctcatgttgtcagcctgcagacggaattcgtgctccctcttccgcattttcgattcaaactccagcagcagttcctgtctctgcagagcaagctcaccgtcgagctcctcaagttttctctccagtgtccattttagattttcatactgttcccggtggtggtcaatctcaccattcttgtcactgtggacgcgctccagctccaggcgatgctcctggaatgccagctgctgctgctgctgcagctcctccaccttcctggcctctctggctagcgcctgcctcagcttagctgcctctatcttgagctcgctcacctctgcccgcctggcctcttcccactccctggcctgggcgaaggcggcgtcatagcgctccagctcgaggtcccgctcctccagcacctgaaggttgtagacaaagtcctcctgcaggcaccgcagtttcccctgcgcctcctccagctggctccgtgtgtcctgcagagccgcctcctgcagctgggtgcggtgtgcctgcagcgccctccactcctcctccttgcgaagcagcagctcattcagggcgggctctgagcccagtggcagcatggtggccgcctgtggtctgacctctctccaggcaggcggtgttggaactgaaccgaaggacacccgccgagtctgcggcagaactgactgctcatgtgctggtgaaaacctccctctcccaccacatttgatcacagaagtcttcctctgtgctgatgattcttgtggtatcagagtagaggaaaaacagtttgagttttccagaaatacctgtgaccccgtgttttttttcacttcctccactgactgccgaagagtagccacag

SEQ ID NO: 10080 - RNA, 1676 nt, Homo sapiens
  source 1..1676: mol_type = other RNA
caccgactctgtctcctgcagcttggcagcaacctgactttttgccatgctcagaccctgaatcagggcctctgacttttggatctggtccctttcaatgtcatcacagcggcgctgccagtccaggcccagctgcacctgatcacgctccaggctccgctccctttccactgccagggacagctgttgcttgtacctttcaatgtcctgctgggatcgggccacctgtgccttgagcttcacctcttcttcctgcagcgtctgaatctgaaggtctctggagaccatctccttagatagttgagcaatttgagcatcccaggcagattttacagttgatgcatcttcacgaagttggtcaatggcagcgtccttctccttggcggtgtcagcctgtctccactctgccctgcggagctgcgcctcgagggtctcgcagtgggcctgcagctccagaaccctggtctgcagctcctgcagctgctccacgtgggctcccttcaccgccaccagcactgcatccttctccctggccagacggtcgagctcctcatgcttcctcttaaatgtttcctcttccttcttcctggttagctgcacagagtgaagtttatcctctaaatcctttacccgggcgcggctcatggcctccaggtcctggagctccccggctcggctctggagcttcctctccagctcggcgttggtggcctctgccctctgcagactctctgcagcctttgccccggcttccttcagagcctccagctctttgtgcagtagtttaaccttaagctcccgggacaaggctgtgttgctcatgttgtcagcctgcagacggaattcgtgctccctcttccgcattttcgattcaaactccagcagcagttcctgtctctgcagagcaagctcaccgtcgagctcctcaagttttctctccagtgtccattttagattttcatactgttcccggtggtggtcaatctcaccattcttgtcactgtggacgcgctccagctccaggcgatgctcctggaatgccagctgctgctgctgctgcagctcctccaccttcctggcctctctggctagcgcctgcctcagcttagctgcctctatcttgagctcgctcacctctgcccgcctggcctcttcccactccctggcctgggcgaaggcggcgtcatagcgctccagctcgaggtcccgctcctccagcacctgaaggttgtagacaaagtcctcctgcaggcaccgcagtttcccctgcgcctcctccagctggctccgtgtgtcctgcagagccgcctcctgcagctgggtgcggtgtgcctgcagcgccctccactcctcctccttgcgaagcagcagctcattcagggcgggctctgagcccagtggcagcatggtggccgcctgtggtctgacctctctccaggcaggcggtgttggaactgaaccgaaggacacccgccgagtctgcggcagaactgactgctcatgtgctggtgaaaacctccctctcccaccacatttgatcacagaagtcttcctctgtgctgatgattcttgtggtatcagagtagaggaaaaacagtttgagttttccagaaatacctgtgaccccgtgttttttttcacttcctccactgactgccgaagagtagccacagcca

SEQ ID NO: 10081 - RNA, 1680 nt, Homo sapiens
  source 1..1680: mol_type = other RNA
caccgactctgtctcctgcagcttggcagcaacctgactttttgccatgctcagaccctgaatcagggcctctgacttttggatctggtccctttcaatgtcatcacagcggcgctgccagtccaggcccagctgcacctgatcacgctccaggctccgctccctttccactgccagggacagctgttgcttgtacctttcaatgtcctgctgggatcgggccacctgtgccttgagcttcacctcttcttcctgcagcgtctgaatctgaaggtctctggagaccatctccttagatagttgagcaatttgagcatcccaggcagattttacagttgatgcatcttcacgaagttggtcaatggcagcgtccttctccttggcggtgtcagcctgtctccactctgccctgcggagctgcgcctcgagggtctcgcagtgggcctgcagctccagaaccctggtctgcagctcctgcagctgctccacgtgggctcccttcaccgccaccagcactgcatccttctccctggccagacggtcgagctcctcatgcttcctcttaaatgtttcctcttccttcttcctggttagctgcacagagtgaagtttatcctctaaatcctttacccgggcgcggctcatggcctccaggtcctggagctccccggctcggctctggagcttcctctccagctcggcgttggtggcctctgccctctgcagactctctgcagcctttgccccggcttccttcagagcctccagctctttgtgcagtagtttaaccttaagctcccgggacaaggctgtgttgctcatgttgtcagcctgcagacggaattcgtgctccctcttccgcattttcgattcaaactccagcagcagttcctgtctctgcagagcaagctcaccgtcgagctcctcaagttttctctccagtgtccattttagattttcatactgttcccggtggtggtcaatctcaccattcttgtcactgtggacgcgctccagctccaggcgatgctcctggaatgccagctgctgctgctgctgcagctcctccaccttcctggcctctctggctagcgcctgcctcagcttagctgcctctatcttgagctcgctcacctctgcccgcctggcctcttcccactccctggcctgggcgaaggcggcgtcatagcgctccagctcgaggtcccgctcctccagcacctgaaggttgtagacaaagtcctcctgcaggcaccgcagtttcccctgcgcctcctccagctggctccgtgtgtcctgcagagccgcctcctgcagctgggtgcggtgtgcctgcagcgccctccactcctcctccttgcgaagcagcagctcattcagggcgggctctgagcccagtggcagcatggtggccgcctgtggtctgacctctctccaggcaggcggtgttggaactgaaccgaaggacacccgccgagtctgcggcagaactgactgctcatgtgctggtgaaaacctccctctcccaccacatttgatcacagaagtcttcctctgtgctgatgattcttgtggtatcagagtagaggaaaaacagtttgagttttccagaaatacctgtgaccccgtgttttttttcacttcctccactgactgccgaagagtagccacagccatttc

SEQ ID NO: 10082 - RNA, 1681 nt, Homo sapiens
  source 1..1681: mol_type = other RNA
caccgactctgtctcctgcagcttggcagcaacctgactttttgccatgctcagaccctgaatcagggcctctgacttttggatctggtccctttcaatgtcatcacagcggcgctgccagtccaggcccagctgcacctgatcacgctccaggctccgctccctttccactgccagggacagctgttgcttgtacctttcaatgtcctgctgggatcgggccacctgtgccttgagcttcacctcttcttcctgcagcgtctgaatctgaaggtctctggagaccatctccttagatagttgagcaatttgagcatcccaggcagattttacagttgatgcatcttcacgaagttggtcaatggcagcgtccttctccttggcggtgtcagcctgtctccactctgccctgcggagctgcgcctcgagggtctcgcagtgggcctgcagctccagaaccctggtctgcagctcctgcagctgctccacgtgggctcccttcaccgccaccagcactgcatccttctccctggccagacggtcgagctcctcatgcttcctcttaaatgtttcctcttccttcttcctggttagctgcacagagtgaagtttatcctctaaatcctttacccgggcgcggctcatggcctccaggtcctggagctccccggctcggctctggagcttcctctccagctcggcgttggtggcctctgccctctgcagactctctgcagcctttgccccggcttccttcagagcctccagctctttgtgcagtagtttaaccttaagctcccgggacaaggctgtgttgctcatgttgtcagcctgcagacggaattcgtgctccctcttccgcattttcgattcaaactccagcagcagttcctgtctctgcagagcaagctcaccgtcgagctcctcaagttttctctccagtgtccattttagattttcatactgttcccggtggtggtcaatctcaccattcttgtcactgtggacgcgctccagctccaggcgatgctcctggaatgccagctgctgctgctgctgcagctcctccaccttcctggcctctctggctagcgcctgcctcagcttagctgcctctatcttgagctcgctcacctctgcccgcctggcctcttcccactccctggcctgggcgaaggcggcgtcatagcgctccagctcgaggtcccgctcctccagcacctgaaggttgtagacaaagtcctcctgcaggcaccgcagtttcccctgcgcctcctccagctggctccgtgtgtcctgcagagccgcctcctgcagctgggtgcggtgtgcctgcagcgccctccactcctcctccttgcgaagcagcagctcattcagggcgggctctgagcccagtggcagcatggtggccgcctgtggtctgacctctctccaggcaggcggtgttggaactgaaccgaaggacacccgccgagtctgcggcagaactgactgctcatgtgctggtgaaaacctccctctcccaccacatttgatcacagaagtcttcctctgtgctgatgattcttgtggtatcagagtagaggaaaaacagtttgagttttccagaaatacctgtgaccccgtgttttttttcacttcctccactgactgccgaagagtagccacagccatttct

SEQ ID NO: 10083 - RNA, 1682 nt, Homo sapiens
  source 1..1682: mol_type = other RNA
caccgactctgtctcctgcagcttggcagcaacctgactttttgccatgctcagaccctgaatcagggcctctgacttttggatctggtccctttcaatgtcatcacagcggcgctgccagtccaggcccagctgcacctgatcacgctccaggctccgctccctttccactgccagggacagctgttgcttgtacctttcaatgtcctgctgggatcgggccacctgtgccttgagcttcacctcttcttcctgcagcgtctgaatctgaaggtctctggagaccatctccttagatagttgagcaatttgagcatcccaggcagattttacagttgatgcatcttcacgaagttggtcaatggcagcgtccttctccttggcggtgtcagcctgtctccactctgccctgcggagctgcgcctcgagggtctcgcagtgggcctgcagctccagaaccctggtctgcagctcctgcagctgctccacgtgggctcccttcaccgccaccagcactgcatccttctccctggccagacggtcgagctcctcatgcttcctcttaaatgtttcctcttccttcttcctggttagctgcacagagtgaagtttatcctctaaatcctttacccgggcgcggctcatggcctccaggtcctggagctccccggctcggctctggagcttcctctccagctcggcgttggtggcctctgccctctgcagactctctgcagcctttgccccggcttccttcagagcctccagctctttgtgcagtagtttaaccttaagctcccgggacaaggctgtgttgctcatgttgtcagcctgcagacggaattcgtgctccctcttccgcattttcgattcaaactccagcagcagttcctgtctctgcagagcaagctcaccgtcgagctcctcaagttttctctccagtgtccattttagattttcatactgttcccggtggtggtcaatctcaccattcttgtcactgtggacgcgctccagctccaggcgatgctcctggaatgccagctgctgctgctgctgcagctcctccaccttcctggcctctctggctagcgcctgcctcagcttagctgcctctatcttgagctcgctcacctctgcccgcctggcctcttcccactccctggcctgggcgaaggcggcgtcatagcgctccagctcgaggtcccgctcctccagcacctgaaggttgtagacaaagtcctcctgcaggcaccgcagtttcccctgcgcctcctccagctggctccgtgtgtcctgcagagccgcctcctgcagctgggtgcggtgtgcctgcagcgccctccactcctcctccttgcgaagcagcagctcattcagggcgggctctgagcccagtggcagcatggtggccgcctgtggtctgacctctctccaggcaggcggtgttggaactgaaccgaaggacacccgccgagtctgcggcagaactgactgctcatgtgctggtgaaaacctccctctcccaccacatttgatcacagaagtcttcctctgtgctgatgattcttgtggtatcagagtagaggaaaaacagtttgagttttccagaaatacctgtgaccccgtgttttttttcacttcctccactgactgccgaagagtagccacagccatttcta

SEQ ID NO: 10084 - RNA, 1684 nt, Homo sapiens
  source 1..1684: mol_type = other RNA
caccgactctgtctcctgcagcttggcagcaacctgactttttgccatgctcagaccctgaatcagggcctctgacttttggatctggtccctttcaatgtcatcacagcggcgctgccagtccaggcccagctgcacctgatcacgctccaggctccgctccctttccactgccagggacagctgttgcttgtacctttcaatgtcctgctgggatcgggccacctgtgccttgagcttcacctcttcttcctgcagcgtctgaatctgaaggtctctggagaccatctccttagatagttgagcaatttgagcatcccaggcagattttacagttgatgcatcttcacgaagttggtcaatggcagcgtccttctccttggcggtgtcagcctgtctccactctgccctgcggagctgcgcctcgagggtctcgcagtgggcctgcagctccagaaccctggtctgcagctcctgcagctgctccacgtgggctcccttcaccgccaccagcactgcatccttctccctggccagacggtcgagctcctcatgcttcctcttaaatgtttcctcttccttcttcctggttagctgcacagagtgaagtttatcctctaaatcctttacccgggcgcggctcatggcctccaggtcctggagctccccggctcggctctggagcttcctctccagctcggcgttggtggcctctgccctctgcagactctctgcagcctttgccccggcttccttcagagcctccagctctttgtgcagtagtttaaccttaagctcccgggacaaggctgtgttgctcatgttgtcagcctgcagacggaattcgtgctccctcttccgcattttcgattcaaactccagcagcagttcctgtctctgcagagcaagctcaccgtcgagctcctcaagttttctctccagtgtccattttagattttcatactgttcccggtggtggtcaatctcaccattcttgtcactgtggacgcgctccagctccaggcgatgctcctggaatgccagctgctgctgctgctgcagctcctccaccttcctggcctctctggctagcgcctgcctcagcttagctgcctctatcttgagctcgctcacctctgcccgcctggcctcttcccactccctggcctgggcgaaggcggcgtcatagcgctccagctcgaggtcccgctcctccagcacctgaaggttgtagacaaagtcctcctgcaggcaccgcagtttcccctgcgcctcctccagctggctccgtgtgtcctgcagagccgcctcctgcagctgggtgcggtgtgcctgcagcgccctccactcctcctccttgcgaagcagcagctcattcagggcgggctctgagcccagtggcagcatggtggccgcctgtggtctgacctctctccaggcaggcggtgttggaactgaaccgaaggacacccgccgagtctgcggcagaactgactgctcatgtgctggtgaaaacctccctctcccaccacatttgatcacagaagtcttcctctgtgctgatgattcttgtggtatcagagtagaggaaaaacagtttgagttttccagaaatacctgtgaccccgtgttttttttcacttcctccactgactgccgaagagtagccacagccatttctaaa

SEQ ID NO: 10085 - RNA, 1709 nt, Homo sapiens
  source 1..1709: mol_type = other RNA
caccgactctgtctcctgcagcttggcagcaacctgactttttgccatgctcagaccctgaatcagggcctctgacttttggatctggtccctttcaatgtcatcacagcggcgctgccagtccaggcccagctgcacctgatcacgctccaggctccgctccctttccactgccagggacagctgttgcttgtacctttcaatgtcctgctgggatcgggccacctgtgccttgagcttcacctcttcttcctgcagcgtctgaatctgaaggtctctggagaccatctccttagatagttgagcaatttgagcatcccaggcagattttacagttgatgcatcttcacgaagttggtcaatggcagcgtccttctccttggcggtgtcagcctgtctccactctgccctgcggagctgcgcctcgagggtctcgcagtgggcctgcagctccagaaccctggtctgcagctcctgcagctgctccacgtgggctcccttcaccgccaccagcactgcatccttctccctggccagacggtcgagctcctcatgcttcctcttaaatgtttcctcttccttcttcctggttagctgcacagagtgaagtttatcctctaaatcctttacccgggcgcggctcatggcctccaggtcctggagctccccggctcggctctggagcttcctctccagctcggcgttggtggcctctgccctctgcagactctctgcagcctttgccccggcttccttcagagcctccagctctttgtgcagtagtttaaccttaagctcccgggacaaggctgtgttgctcatgttgtcagcctgcagacggaattcgtgctccctcttccgcattttcgattcaaactccagcagcagttcctgtctctgcagagcaagctcaccgtcgagctcctcaagttttctctccagtgtccattttagattttcatactgttcccggtggtggtcaatctcaccattcttgtcactgtggacgcgctccagctccaggcgatgctcctggaatgccagctgctgctgctgctgcagctcctccaccttcctggcctctctggctagcgcctgcctcagcttagctgcctctatcttgagctcgctcacctctgcccgcctggcctcttcccactccctggcctgggcgaaggcggcgtcatagcgctccagctcgaggtcccgctcctccagcacctgaaggttgtagacaaagtcctcctgcaggcaccgcagtttcccctgcgcctcctccagctggctccgtgtgtcctgcagagccgcctcctgcagctgggtgcggtgtgcctgcagcgccctccactcctcctccttgcgaagcagcagctcattcagggcgggctctgagcccagtggcagcatggtggccgctctctccaggcaggcggtgttggaactgaaccgaaggacacccgccgagtctgcggcagaactgactgctcatgtgctggtgaaaacctccctctcccaccacatttgatcacagaagtcttcctctgtgctgatgattcttgtggtatcagagtagaggaaaaacagtttgagttttccagaaataccctaacgcccgccagcagcgctggccaggtcccgccgcgttgccacagcgaccgggtcagtcggccgcgtccggctgcgctcggtgcagcgctcgggtcccgccg

SEQ ID NO: 10086 - RNA, 2013 nt, Homo sapiens
  source 1..2013: mol_type = other RNA
caccgactctgtctcctgcagcttggcagcaacctgactttttgccatgctcagaccctgaatcagggcctctgacttttggatctggtccctttcaatgtcatcacagcggcgctgccagtccaggcccagctgcacctgatcacgctccaggctccgctccctttccactgccagggacagctgttgcttgtacctttcaatgtcctgctgggatcgggccacctgtgccttgagcttcacctcttcttcctgcagcgtctgaatctgaaggtctctggagaccatctccttagatagttgagcaatttgagcatcccaggcagattttacagttgatgcatcttcacgaagttggtcaatggcagcgtccttctccttggcggtgtcagcctgtctccactctgccctgcggagctgcgcctcgagggtctcgcagtgggcctgcagctccagaaccctggtctgcagctcctgcagctgctccacgtgggctcccttcaccgccaccagcactgcatccttctccctggccagacggtcgagctcctcatgcttcctcttaaatgtttcctcttccttcttcctggttagctgcacagagtgaagtttatcctctaaatcctttacccgggcgcggctcatggcctccaggtcctggagctccccggctcggctctggagcttcctctccagctcggcgttggtggcctctgccctctgcagactctctgcagcctttgccccggcttccttcagagcctccagctctttgtgcagtagtttaaccttaagctcccgggacaaggctgtgttgctcatgttgtcagcctgcagacggaattcgtgctccctcttccgcattttcgattcaaactccagcagcagttcctgtctctgcagagcaagctcaccgtcgagctcctcaagttttctctccagtgtccattttagattttcatactgttcccggtggtggtcaatctcaccattcttgtcactgtggacgcgctccagctccaggcgatgctcctggaatgccagctgctgctgctgctgcagctcctccaccttcctggcctctctggctagcgcctgcctcagcttagctgcctctatcttgagctcgctcacctctgcccgcctggcctcttcccactccctggcctgggcgaaggcggcgtcatagcgctccagctcgaggtcccgctcctccagcacctgaaggttgtagacaaagtcctcctgcaggcaccgcagtttcccctgcgcctcctccagctggctccgtgtgtcctgcagagccgcctcctgcagctgggtgcggtgtgcctgcagcgccctccactcctcctccttgcgaagcagcagctcattcagggcgggctctgagcccagtggcagcatggtggccgctgttgtggtacaatgacacatcatggttttcttgcacagttcctggctcataactctcacacgtcacagtcttttgttgcaatgttgggcgtgtcaggcctcaggaaacagaatccttccaggtctccactctcacctgactttccattgtaggtcataagatcctccccagagctcccaccctctaccctgggggaaggaatgctgacttcaggaagcctccctaaacacccaagaggacagggtgtggagaggttcctggggagtggtgggtggggtgtgggggggtcctccaggaagcctcttcccccatatctccccttacgcatctcctcatctgtatcctctgtaataccctttataataaactgttacacgtatgtgtttccctgggttctgtgagtcaccccagcaaatcaatcgaacccaaagagggggctgtgggaaccccaacttgaagccagtggtcagtcagaagttccggaggccaggactcgcgactggtgtcagaagcgggcagtctttgaaccaccattgcaaaattataactcagacagtgaaagagatctgacctaaccaattccatcgtgcttctaa

SEQ ID NO: 10087 - RNA, 1791 nt, Homo sapiens
  source 1..1791: mol_type = other RNA
caccgactctgtctcctgcagcttggcagcaacctgactttttgccatgctcagaccctgaatcagggcctctgacttttggatctggtccctttcaatgtcatcacagcggcgctgccagtccaggcccagctgcacctgatcacgctccaggctccgctccctttccactgccagggacagctgttgcttgtacctttcaatgtcctgctgggatcgggccacctgtgccttgagcttcacctcttcttcctgcagcgtctgaatctgaaggtctctggagaccatctccttagatagttgagcaatttgagcatcccaggcagattttacagttgatgcatcttcacgaagttggtcaatggcagcgtccttctccttggcggtgtcagcctgtctccactctgccctgcggagctgcgcctcgagggtctcgcagtgggcctgcagctccagaaccctggtctgcagctcctgcagctgctccacgtgggctcccttcaccgccaccagcactgcatccttctccctggccagacggtcgagctcctcatgcttcctcttaaatgtttcctcttccttcttcctggttagctgcacagagtgaagtttatcctctaaatcctttacccgggcgcggctcatggcctccaggtcctggagctccccggctcggctctggagcttcctctccagctcggcgttggtggcctctgccctctgcagactctctgcagcctttgccccggcttccttcagagcctccagctctttgtgcagtagtttaaccttaagctcccgggacaaggctgtgttgctcatgttgtcagcctgcagacggaattcgtgctccctcttccgcattttcgattcaaactccagcagcagttcctgtctctgcagagcaagctcaccgtcgagctcctcaagttttctctccagtgtccattttagattttcatactgttcccggtggtggtcaatctcaccattcttgtcactgtggacgcgctccagctccaggcgatgctcctggaatgccagctgctgctgctgctgcagctcctccaccttcctggcctctctggctagcgcctgcctcagcttagctgcctctatcttgagctcgctcacctctgcccgcctggcctcttcccactccctggcctgggcgaaggcggcgtcatagcgctccagctcgaggtcccgctcctccagcacctgaaggttgtagacaaagtcctcctgcaggcaccgcagtttcccctgcgcctcctccagctggctccgtgtgtcctgcagagccgcctcctgcagctgggtgcggtgtgcctgcagcgccctccactcctcctccttgcgaagcagcagctcattcagggcgggctctgagcccagtggcagcatggtggccgtctttctctatcctaattcccgtcttggtgaatcggctctgcctgggcagcaggcggggtggacctgttgggtgtttatgtcttgggtgtttatgtcttggggactgagccctcaccctgtggtctgacctctctccaggcaggcggtgttggaactgaaccgaaggacacccgccgagtctgcggcagaactgactgctcatgtgctggtgaaaacctccctctcccaccacatttgatcacagaagtcttcctctgtgctgatgattcttgtggtatcagagtagaggaaaaacagtttgagttttccagaaataccctaacgcccgccagcagcgctggccaggtcccgccgcgttgccacagcgaccgggtc

SEQ ID NO: 10088 - RNA, 1837 nt, Homo sapiens
  source 1..1837: mol_type = other RNA
caccgactctgtctcctgcagcttggcagcaacctgactttttgccatgctcagaccctgaatcagggcctctgacttttggatctggtccctttcaatgtcatcacagcggcgctgccagtccaggcccagctgcacctgatcacgctccaggctccgctccctttccactgccagggacagctgttgcttgtacctttcaatgtcctgctgggatcgggccacctgtgccttgagcttcacctcttcttcctgcagcgtctgaatctgaaggtctctggagaccatctccttagatagttgagcaatttgagcatcccaggcagattttacagttgatgcatcttcacgaagttggtcaatggcagcgtccttctccttggcggtgtcagcctgtctccactctgccctgcggagctgcgcctcgagggtctcgcagtgggcctgcagctccagaaccctggtctgcagctcctgcagctgctccacgtgggctcccttcaccgccaccagcactgcatccttctccctggccagacggtcgagctcctcatgcttcctcttaaatgtttcctcttccttcttcctggttagctgcacagagtgaagtttatcctctaaatcctttacccgggcgcggctcatggcctccaggtcctggagctccccggctcggctctggagcttcctctccagctcggcgttggtggcctctgccctctgcagactctctgcagcctttgccccggcttccttcagagcctccagctctttgtgcagtagtttaaccttaagctcccgggacaaggctgtgttgctcatgttgtcagcctgcagacggaattcgtgctccctcttccgcattttcgattcaaactccagcagcagttcctgtctctgcagagcaagctcaccgtcgagctcctcaagttttctctccagtgtccattttagattttcatactgttcccggtggtggtcaatctcaccattcttgtcactgtggacgcgctccagctccaggcgatgctcctggaatgccagctgctgctgctgctgcagctcctccaccttcctggcctctctggctagcgcctgcctcagcttagctgcctctatcttgagctcgctcacctctgcccgcctggcctcttcccactccctggcctgggcgaaggcggcgtcatagcgctccagctcgaggtcccgctcctccagcacctgaaggttgtagacaaagtcctcctgcaggcaccgcagtttcccctgcgcctcctccagctggctccgtgtgtcctgcagagccgcctcctgcagctgggtgcggtgtgcctgcagcgccctccactcctcctccttgcgaagcagcagctcattcagggcgggctctgagcccagtggcagcatggtggccgtctttctctatcctaattcccgtcttggtgaatcggctctgcctgggcagcaggcggggtggacctgttgggtgtttatgtcttgggtgtttatgtcttggggactgagccctcaccctgtggtctgacctctctccaggcaggcggtgttggaactgaaccgaaggacacccgccgagtctgcggcagaactgactgctcatgtgctggtgaaaacctccctctcccaccacatttgatcacagaagtcttcctctgtgctgatgattcttgtggtatcagagtagaggaaaaacagtttgagttttccagaaataccctaacgcccgccagcagcgctggccaggtcccgccgcgttgccacagcgaccgggtcagtcggccgcgtccggctgcgctcggtgcagcgctcgggtcccgcc

SEQ ID NO: 10089 - RNA, 1838 nt, Homo sapiens
  source 1..1838: mol_type = other RNA
caccgactctgtctcctgcagcttggcagcaacctgactttttgccatgctcagaccctgaatcagggcctctgacttttggatctggtccctttcaatgtcatcacagcggcgctgccagtccaggcccagctgcacctgatcacgctccaggctccgctccctttccactgccagggacagctgttgcttgtacctttcaatgtcctgctgggatcgggccacctgtgccttgagcttcacctcttcttcctgcagcgtctgaatctgaaggtctctggagaccatctccttagatagttgagcaatttgagcatcccaggcagattttacagttgatgcatcttcacgaagttggtcaatggcagcgtccttctccttggcggtgtcagcctgtctccactctgccctgcggagctgcgcctcgagggtctcgcagtgggcctgcagctccagaaccctggtctgcagctcctgcagctgctccacgtgggctcccttcaccgccaccagcactgcatccttctccctggccagacggtcgagctcctcatgcttcctcttaaatgtttcctcttccttcttcctggttagctgcacagagtgaagtttatcctctaaatcctttacccgggcgcggctcatggcctccaggtcctggagctccccggctcggctctggagcttcctctccagctcggcgttggtggcctctgccctctgcagactctctgcagcctttgccccggcttccttcagagcctccagctctttgtgcagtagtttaaccttaagctcccgggacaaggctgtgttgctcatgttgtcagcctgcagacggaattcgtgctccctcttccgcattttcgattcaaactccagcagcagttcctgtctctgcagagcaagctcaccgtcgagctcctcaagttttctctccagtgtccattttagattttcatactgttcccggtggtggtcaatctcaccattcttgtcactgtggacgcgctccagctccaggcgatgctcctggaatgccagctgctgctgctgctgcagctcctccaccttcctggcctctctggctagcgcctgcctcagcttagctgcctctatcttgagctcgctcacctctgcccgcctggcctcttcccactccctggcctgggcgaaggcggcgtcatagcgctccagctcgaggtcccgctcctccagcacctgaaggttgtagacaaagtcctcctgcaggcaccgcagtttcccctgcgcctcctccagctggctccgtgtgtcctgcagagccgcctcctgcagctgggtgcggtgtgcctgcagcgccctccactcctcctccttgcgaagcagcagctcattcagggcgggctctgagcccagtggcagcatggtggccgtctttctctatcctaattcccgtcttggtgaatcggctctgcctgggcagcaggcggggtggacctgttgggtgtttatgtcttgggtgtttatgtcttggggactgagccctcaccctgtggtctgacctctctccaggcaggcggtgttggaactgaaccgaaggacacccgccgagtctgcggcagaactgactgctcatgtgctggtgaaaacctccctctcccaccacatttgatcacagaagtcttcctctgtgctgatgattcttgtggtatcagagtagaggaaaaacagtttgagttttccagaaataccctaacgcccgccagcagcgctggccaggtcccgccgcgttgccacagcgaccgggtcagtcggccgcgtccggctgcgctcggtgcagcgctcgggtcccgccg

SEQ ID NO: 10090 - RNA, 1752 nt, Homo sapiens
  source 1..1752: mol_type = other RNA
caccgactctgtctcctgcagcttggcagcaacctgactttttgccatgctcagaccctgaatcagggcctctgacttttggatctggtccctttcaatgtcatcacagcggcgctgccagtccaggcccagctgcacctgatcacgctccaggctccgctccctttccactgccagggacagctgttgcttgtacctttcaatgtcctgctgggatcgggccacctgtgccttgagcttcacctcttcttcctgcagcgtctgaatctgaaggtctctggagaccatctccttagatagttgagcaatttgagcatcccaggcagattttacagttgatgcatcttcacgaagttggtcaatggcagcgtccttctccttggcggtgtcagcctgtctccactctgccctgcggagctgcgcctcgagggtctcgcagtgggcctgcagctccagaaccctggtctgcagctcctgcagctgctccacgtgggctcccttcaccgccaccagcactgcatccttctccctggccagacggtcgagctcctcatgcttcctcttaaatgtttcctcttccttcttcctggttagctgcacagagtgaagtttatcctctaaatcctttaccctgaaaagaaacaaatatttatggaaggagcaagtgagatgaaagcaaagaccagcctggaatgagcagaaaaggtagaatcccccagactccagtcctggcctgcgaggctgccacagagcacgcctcgggagatgaaggactcgcgcaccgggcgcggctcatggcctccaggtcctggagctccccggctcggctctggagcttcctctccagctcggcgttggtggcctctgccctctgcagactctctgcagcctttgccccggcttccttcagagcctccagctctttgtgcagtagtttaaccttaagctcccgggacaaggctgtgttgctcatgttgtcagcctgcagacggaattcgtgctccctcttccgcattttcgattcaaactccagcagcagttcactgtccaggagagaagctggggtcagcgacactggtaacagcactctgggaggccgaggcgggaggatcgcttgagcccaggaattcaagaccagcctgggcaacacagtgaggccctgtcgctgcatagacagagccatttattacacctgcacctgcagagacgcagcccctcatcacacctgcaccttcacagaagaagcccctcaggacacctgcagagacgcagcccctcatgactcctgcacctgcagagacgcagcccctcgtgactcctgcagagacgcagcccctcatgactcctgcacctgcagagacgcagcccctcgtgactcctgcacctgcagagacgcagcccctcgtgactcctgcacctgcagagacgcagcccctcgtgactcctgcagagactcagcccctcgtgactcctgcagacgcagcccctcatgactcctgcagagatgcagcccctcgtgactcctgcagagacgcagcccctcgtgactcctgcacctgtctctgcagagcaagctcaccgtcgagctcctcaagttttctctccagtgtccattttagattttcatactgttcccggtggtggtcaatctcaccattcttgtcactctgcccgcctggcctcttcccactccctggcctgggcgaaggcggcgtcatagcgctccagctcgaggtcccgctcctccagcac

SEQ ID NO: 10091 - RNA, 1215 nt, Homo sapiens
  source 1..1215: mol_type = other RNA
caccgactctgtctcctgcagcttggcagcaacctgactttttgccatgctcagaccctgaatcagggcctctgacttttggatctggtccctttcaatgtcatcacagcggcgctgccagtccaggcccagctgcacctgatcacgctccaggctccgctccctttccactgccagggacagctgttgcttgtacctttcaatgtcctgctgggatcgggccacctgtgccttgagcttcacctcttcttcctgcagcgtctgaatctgaaggtctctggagaccatctccttagatagttgagcaatttgagcatcccaggcagattttacagttgatgcatcttcacgaagttggtcaatggcagcgtccttctccttggcggtgtcagcctgtctccactctgccctgcggagctgcgcctcgagggtctcgcagtgggcctgcagctccagaaccctggtctgcagctcctgcagctgctccacgtgggctcccttcaccgccaccagcactgcatccttctccctggccagacggtcgagctcctcatgcttcctcttaaatgtttcctcttccttcttcctggttagctgcacagagtgaagtttatcctctaaatcctttaccctgaaaagaaacaaatatttatggaaggagcaagtgagatgaaagcaaagaccagcctggaatgagcagaaaaggtagaatcccccagactccagtcctggcctgcgaggctgccacagagcacgcctcgggagatgaaggactcgcgcaccgggcgcggctcatggcctccaggtcctggagctccccggctcggctctggagcttcctctccagctcggcgttggtggcctctgccctctgcagactctctgcagcctttgccccggcttccttcagagcctccagctctttgtgcagtagtttaaccttaagctcccgggacaaggctgtgttgctcatgttgtcagcctgcagacggaattcgtgctccctcttccgcattttcgattcaaactccagcagcagttccgtcgagctcctcaagttttctctccagtgtccattttagattttcatactgttcccggtggtggtcaatctcaccattcttgtcactctgcccgcctggcctcttcccactccctggcctgggcgaaggcggcgtcatagcgctccagctcgaggtcccgctcctccagcac

SEQ ID NO: 10092 - RNA, 1584 nt, Homo sapiens
  source 1..1584: mol_type = other RNA
caccgactctgtctcctgcagcttggcagcaacctgactttttgccatgctcagaccctgaatcagggcctctgacttttggatctggtccctttcaatgtcatcacagcggcgctgccagtccaggcccagctgcacctgatcacgctccaggctccgctccctttccactgccagggacagctgttgcttgtacctttcaatgtcctgctgggatcgggccacctgtgccttgagcttcacctcttcttcctgcagcgtctgaatctgaaggtctctggagaccatctccttagatagttgagcaatttgagcatcccaggcagattttacagttgatgcatcttcacgaagttggtcaatggcagcgtccttctccttggcggtgtcagcctgtctccactctgccctgcggagctgcgcctcgagggtctcgcagtgggcctgcagctccagaaccctggtctgcagctcctgcagctgctccacgtgggctcccttcaccgccaccagcactgcatccttctccctggccagacggtcgagctcctcatgcttcctcttaaatgtttcctcttccttcttcctggttagctgcacagagtgaagtttatcctctaaatcctttaccctgaaaagaaacaaatatttatggaaggagcaagtgagatgaaagcaaagaccagcctggaatgagcagaaaaggtagaatcccccagactccagtcctggcctgcgaggctgccacagagcacgcctcgggagatgaaggactcgcgcaccgggcgcggctcatggcctccaggtcctggagctccccggctcggctctggagcttcctctccagctcggcgttggtggcctctgccctctgcagactctctgcagcctttgccccggcttccttcagagcctccagctctttgtgcagtagtttaaccttaagctcccgggacaaggctgtgttgctcatgttgtcagcctgcagacggaattcgtgctccctcttccgcattttcgattcaaactccagcagcagttccgtcgagctcctcaagttttctctccagtgtccattttagattttcatactgttcccggtggtggtcaatctcaccattcttgtcactgtggacgcgctccagctccaggcgatgctcctggaatgccagctgctgctgctgctgcagctcctccaccttcctggcctctctggctagcgcctgcctcagcttagctgcctctatcttgagctcgctcacctctgcccgcctggcctcttcccactccctggcctgggcgaaggcggcgtcatagcgctccagctcgaggtcccgctcctccagcacctgaaggttgtagacaaagtcctcctgcaggcaccgcagtttcccctgcgcctcctccagctggctccgtgtgtcctgcagagccgcctcctgcagctgggtgcggtgtgcctgcagcgccctccactcctcctccttgcgaagcagcagctcattcagggcgggctctgagcccagtggcagcatggtggccgcctaacgcccgccagcagcgctggccaggtcccgccgcgtt

SEQ ID NO: 10093 - RNA, 1883 nt, Homo sapiens
  source 1..1883: mol_type = other RNA
caccgactctgtctcctgcagcttggcagcaacctttcaatgtcctgctgggatcgggccacctgtgccttgagcttcacctcttcttcctgcagcgtctgaatctgaaggtctctggagaccatctccttagatagttgagcaatttgagcatcccaggcagattttacagttgatgcatcttcacgaagtcaacggcctctggtgctctgggaagcagctttatccctggaccatgagccacctaattatgagggccagccccactcccagcatcaggatggtgatgtgactctgcctggggcctcctggacagtctcccctgatgcacagtctcaggtgtagatcaatgggcacggctgctgagccctcactgcagggacagaggacaccacggccacgagcgggagtgcactgctcaccacaagagcgtaaatgctttttgtgagaagccaaggtggaaggatcacctgagcccaggaggtcgaggctccagtgagccatgatcgcactgctgctttccagtcttctctttctttggtcaatggcagcgtccttctccttggcggtgtcagcctgtctccactctgccctgcggagctgcgcctcgagggtctcgcagtgggcctgcagctccagaaccctggtctgcagctcctgcagctgctccacgtgggctcccttcaccgccaccagcactgcatccttctccctggccagacggtcgagctcctcatgcttcctcttaaatgtttcctcttccttcttcctggttagctgcacagagtgaagtttatcctctaaatcctttacccgggcgcggctcatggcctccaggtcctggagctccccggctcggctctggagcttcctctccagctcggcgttggtggcctctgccctctgcagactctctgcagcctttgccccggcttccttcagagcctccagctctttgtgcagtagtttaaccttaagctcccgggacaaggctgtgttgctcatgttgtcagcctgcagacggaattcgtgctccctcttccgcattttcgattcaaactccagcagcagttcctgtctctgcagagcaagctcaccgtcgagctcctcaagttttctctccagtgtccattttagattttcatactgttcccggtggtggtcaatctcaccattcttgtcactgtggacgcgctccagctccaggcgatgctcctggaatgccagctgctgctgctgctgcagctcctccaccttcctggcctctctggctagcgcctgcctcagcttagctgcctctatcttgagctcgctcacctctgcccgcctggcctcttcccactccctggcctgggcgaaggcggcgtcatagcgctccagctcgaggtcccgctcctccagcacctgaaggttgtagacaaagtcctcctgcaggcaccgcagtttcccctgcgcctcctccagctggctccgtgtgtcctgcagagccgcctcctgcagctgggtgcggtgtgcctgcagcgccctccactcctcctccttgcgaagcagcagctcattcagggcgggctctgagcccagtggcagcatggtggccgcctgtggtctgacctctctccaggcaggcggtgttggaactgaaccgaaggacacccgccgagtctgcggcagaactgactgctcatgtgctggtgaaaacctccctctcccaccacatttgatcacagaagtcttcctctgtgctgatgattcttgtggtatcagagtagaggaaaaacagtttgagttttccagaaatacctgtgaccccgtgttttttttcacttcctccactgactgccgaagagtagccacagccatttctaaaacctaacgcccgccag

SEQ ID NO: 10094 - RNA, 1519 nt, Homo sapiens
  source 1..1519: mol_type = other RNA
caccgactctgtctcctgcagcttggcagcaacctttcaatgtcctgctgggatcgggccacctgtgccttgagcttcacctcttcttcctgcagcgtctgaatctgaaggtctctggagaccatctccttagatagttgagcaatttgagcatcccaggcagattttacagttgatgcatcttcacgaagttggtcaatggcagcgtccttctccttggcggtgtcagcctgtctccactctgccctgcggagctgcgcctcgagggtctcgcagtgggcctgcagctccagaaccctggtctgcagctcctgcagctgctccacgtgggctcccttcaccgccaccagcactgcatccttctccctggccagacggtcgagctcctcatgcttcctcttaaatgtttcctcttccttcttcctggttagctgcacagagtgaagtttatcctctaaatcctttacccgggcgcggctcatggcctccaggtcctggagctccccggctcggctctggagcttcctctccagctcggcgttggtggcctctgccctctgcagactctctgcagcctttgccccggcttccttcagagcctccagctctttgtgcagtagtttaaccttaagctcccgggacaaggctgtgttgctcatgttgtcagcctgcagacggaattcgtgctccctcttccgcattttcgattcaaactccagcagcagttcctgtctctgcagagcaagctcaccgtcgagctcctcaagttttctctccagtgtccattttagattttcatactgttcccggtggtggtcaatctcaccattcttgtcactgtggacgcgctccagctccaggcgatgctcctggaatgccagctgctgctgctgctgcagctcctccaccttcctggcctctctggctagcgcctgcctcagcttagctgcctctatcttgagctcgctcacctctgcccgcctggcctcttcccactccctggcctgggcgaaggcggcgtcatagcgctccagctcgaggtcccgctcctccagcacctgaaggttgtagacaaagtcctcctgcaggcaccgcagtttcccctgcgcctcctccagctggctccgtgtgtcctgcagagccgcctcctgcagctgggtgcggtgtgcctgcagcgccctccactcctcctccttgcgaagcagcagctcattcagggcgggctctgagcccagtggcagcatggtggccgcctgtggtctgacctctctccaggcaggcggtgttggaactgaaccgaaggacacccgccgagtctgcggcagaactgactgctcatgtgctggtgaaaacctccctctcccaccacatttgatcacagaagtcttcctctgtgctgatgattcttgtggtatcagagtagaggaaaaacagtttgagttttccagaaatacctgtgaccccgtgttttttttcacttcctccactgactgccgaagagtagccacagccatttcta

SEQ ID NO: 10095 - RNA, 1521 nt, Homo sapiens
  source 1..1521: mol_type = other RNA
caccgactctgtctcctgcagcttggcagcaacctttcaatgtcctgctgggatcgggccacctgtgccttgagcttcacctcttcttcctgcagcgtctgaatctgaaggtctctggagaccatctccttagatagttgagcaatttgagcatcccaggcagattttacagttgatgcatcttcacgaagttggtcaatggcagcgtccttctccttggcggtgtcagcctgtctccactctgccctgcggagctgcgcctcgagggtctcgcagtgggcctgcagctccagaaccctggtctgcagctcctgcagctgctccacgtgggctcccttcaccgccaccagcactgcatccttctccctggccagacggtcgagctcctcatgcttcctcttaaatgtttcctcttccttcttcctggttagctgcacagagtgaagtttatcctctaaatcctttacccgggcgcggctcatggcctccaggtcctggagctccccggctcggctctggagcttcctctccagctcggcgttggtggcctctgccctctgcagactctctgcagcctttgccccggcttccttcagagcctccagctctttgtgcagtagtttaaccttaagctcccgggacaaggctgtgttgctcatgttgtcagcctgcagacggaattcgtgctccctcttccgcattttcgattcaaactccagcagcagttcctgtctctgcagagcaagctcaccgtcgagctcctcaagttttctctccagtgtccattttagattttcatactgttcccggtggtggtcaatctcaccattcttgtcactgtggacgcgctccagctccaggcgatgctcctggaatgccagctgctgctgctgctgcagctcctccaccttcctggcctctctggctagcgcctgcctcagcttagctgcctctatcttgagctcgctcacctctgcccgcctggcctcttcccactccctggcctgggcgaaggcggcgtcatagcgctccagctcgaggtcccgctcctccagcacctgaaggttgtagacaaagtcctcctgcaggcaccgcagtttcccctgcgcctcctccagctggctccgtgtgtcctgcagagccgcctcctgcagctgggtgcggtgtgcctgcagcgccctccactcctcctccttgcgaagcagcagctcattcagggcgggctctgagcccagtggcagcatggtggccgcctgtggtctgacctctctccaggcaggcggtgttggaactgaaccgaaggacacccgccgagtctgcggcagaactgactgctcatgtgctggtgaaaacctccctctcccaccacatttgatcacagaagtcttcctctgtgctgatgattcttgtggtatcagagtagaggaaaaacagtttgagttttccagaaatacctgtgaccccgtgttttttttcacttcctccactgactgccgaagagtagccacagccatttctaaa

SEQ ID NO: 10096 - RNA, 1327 nt, Homo sapiens
  source 1..1327: mol_type = other RNA
caccgactctgtctcctgcagcttggcagcaacctttcaatgtcctgctgggatcgggccacctgtgccttgagcttcacctcttcttcctgcagcgtctgaatctgaaggtctctggagaccatctccttagatagttgagcaatttgagcatcccaggcagattttacagttgatgcatcttcacgaagttggtcaatggcagcgtccttctccttggcggtgtcagcctgtctccactctgccctgcggagctgcgcctcgagggtctcgcagtgggcctgcagctccagaaccctggtctgcagctcctgcagctgctccacgtgggctcccttcaccgccaccagcactgcatccttctccctggccagacggtcgagctcctcatgcttcctcttaaatgtttcctcttccttcttcctggttagctgcacagagtgaagtttatcctctaaatcctttaccctgaaaagaaacaaatatttatggaaggagcaagtgagatgaaagcaaagaccagcctggaatgagcagaaaaggtagaatcccccagactccagtcctggcctgcgaggctgccacagagcacgcctcgggagatgaaggactcgcgcaccgggcgcggctcatggcctccaggtcctggagctccccggctcggctctggagcttcctctccagctcggcgttggtggcctctgccctctgcagactctctgcagcctttgccccggcttccttcagagcctccagctctttgtgcagtagtttaaccttaagctcccgggacaaggctgtgttgctcatgttgtcagcctgcagacggaattcgtgctccctcttccgcattttcgattcaaactccagcagcagttcctgtctctgcagagcaagctcaccgtcgagctcctcaagttttctctccagtgtccattttagattttcatactgttcccggtggtggtcaatctcaccattcttgtcactctgcccgcctggcctcttcccactccctggcctgggcgaaggcggcgtcatagcgctccagctcgaggtcccgctcctccagcacctgaaggttgtagacaaagtcctcctgcaggcaccgcagtttcccctgcgcctcctccagctggctccgtgtgtcctgcagagccgcctcctgcagctgggtgcggtgtgcctgcagcgccctccactcctcctccttgcgaagcagcagctcattcagggcgggctctgagcccagtggcagcatggtggccgcctaacgcccgccagcagcgctggccaggtcccgccgcgttgccacagcgaccgggtc

SEQ ID NO: 10097 - RNA, 2960 nt, Homo sapiens
  source 1..2960: mol_type = other RNA
caccgactctgtctcctgcaggagtggccttggagggtgacccacaaccacctgcccccattcagcttcccaggtctagatcattccagagaggggcatttgtgaacctgttttggccaagagtgcaagccatattctccatctacatttcacttttgaaggtgaaatttggttccctgtccaagtccagagtctatttcccaataagttctatttctctaagagaaaaagcatgtgagtaacttgcaccctcaagcacaaaggtttccactggccatcactttgtctaaagcaaggtgtctaaagcgaggtgcctgggaatgggaagtggacccgccatttcatcctcagcatgcctgctgcatctgtcataaagcctctgcccatagctccctggcttgccccagagtttttatttggtgtcctcaggctcctctaactgtgctctacctactgtgcctcccatacccggtcctcttagcactccttcccactcacatcctttctctccttccttcaccccgtgtcccctgggccatcagaaaaagatctgaggctcaatcacattgagttacagttttagagctgaaggaggccctgtgctcatctaaaccacatcctcattttgacaggaggaaactaaagctcagagaggctaaatggcctccccaaggtcacacagctggagaggattggagccagggctcgactcctggtcccagggttctagaccaaagctttctcacccttccttctttgtttccctttctggggtccaataggtaacgacgccttcagcagaaggaatgactttctcacggtgggctttcagacaccagcccacagtagagggtcattgtcttgcacagaggaccctccaccccccatggagatccaggtttaggaagttccctgaataactccacggtagcctgcatgggagcccagacacagaaatagcccctgagacctctcgcatgtgggtgttcaatgttctctgatcccccaaactctgagctggactggagcctagtggcagtaagagagctccctctcagccctctggaatggaacctgcaatgcagagagggctgcagcctgccacgctaggaggccgctccagggccctgtagatgagctgcacgtctcccctggcctcctctaaggagaacagggaaggggccagcaggaagacctattccttgtagcaaaactgtgccgggaacaaaccatgtggccacgcggccagcagcgctgtgattccaggtggtaagcagcagtcagggctggttgttgcccgggtgaccccagtgcttagcatcatttctggcgcagaaagcatcatcaataatacttgttgaaataataactaagtgaataaatgaatgaacaaatgacagcaaattcacagcagagcaaaattcagcaaatggtgtaagaatccatctctggaagcttagatgctcgttatcaggctgtaatttcacctccaagttattcattcccacagtagaccccaagaaaaacactccagaggcttctgtgtatttccctgcctaagccttccatctctgggagatggaagccagaccccattctgttccgggaatgataggctctgtttgcagcttctgtttattctcatacagatggtagaaatgagacactaacaaatgatcccaaaatataatgcattttctgctactgtggaaccccctgaaggagcggccaccccctgggagcacgggccccataaattttgccatttctgctcgcctgtgaatccatcccaatgacaagcctcacccaggagacaaggcactagtctttcctttgtagaagcaaaagtccccctgtctttcctccccctgcaaaagagcccctaactgctcagatataaaccacaaagccctcagccatgccattcctaggagacaaccacaacagctgatattcaccagccagaagtcatcctaaacatttctgggggtgggggatagaagatggaggagctgagcagctgcctttcataattggatcctcattaactgcaaagagctggctgacgatctaaggcagaaaggcaactttagtgatttgaaaaataaaacaatttgatgtgatttagggatctataaaaaagggggagtggggggcagtggaggtggcagcaccaaggaaccagtaacagccagaaggaacttacccacttcaaggaagacttaggaaagatgacaagaggtgaaatcatctcccacactggttgttccatacggaaacaatttagtaggaaaagaagaactacgcactaaaagcttcagaagaacccagagttttttcccttcagggcccaggaggtctgaaaggcagataaacatcctcagtgtctccatgagtaactagggggcataaataaggattaagttctatccattggcagaacaccaacattgggaaaaggggcttatgcctcaaaatataggcctggaatccaagaagactggcaatgcgggacactgaccaggaataagttggaagccagccaatgaaggaaagctgggtgaagcacacatccaagatggcgactgactagcaaggcatgaatcagacagacgaggttcagaaggtcaccgtggaccctaagctgttgttgatcctaagattatgatgcagctccctgaaagccaacttgaagaaaatggggaccagatggatccaagaggaaagaacttgaaaaaaaaaaaaaaaaaggtctgagagctgtactccctactcttcctcagtgacctgtgggcacacagttaggacactgcattgtacaagcagaagaaaagccacaaaacatgtcaagtctagaaaatagaccctcctgggagatactaacatgaagtgtcatttcagagaaaagaaaagctaaaggtaacttattaagctttttcctctggttttcctctctcatt

SEQ ID NO: 10098 - RNA, 2997 nt, Homo sapiens
  source 1..2997: mol_type = other RNA
caccgactctgtctcctgcaggagtggccttggagggtgacccacaaccacctgcccccattcagcttcccaggtctagatcattccagagaggggcatttgtgaacctgttttggccaagagtgcaagccatattctccatctacatttcacttttgaaggtgaaatttggttccctgtccaagtccagagtctatttcccaataagttctatttctctaagagaaaaagcatgtgagtaacttgcaccctcaagcacaaaggtttccactggccatcactttgtctaaagcaaggtgtctaaagcgaggtgcctgggaatgggaagtggacccgccatttcatcctcagcatgcctgctgcatctgtcataaagcctctgcccatagctccctggcttgccccagagtttttatttggtgtcctcaggctcctctaactgtgctctacctactgtgcctcccatacccggtcctcttagcactccttcccactcacatcctttctctccttccttcaccccgtgtcccctgggccatcagaaaaagatctgaggctcaatcacattgagttacagttttagagctgaaggaggccctgtgctcatctaaaccacatcctcattttgacaggaggaaactaaagctcagagaggctaaatggcctccccaaggtcacacagctggagaggattggagccagggctcgactcctggtcccagggttctagaccaaagctttctcacccttccttctttgtttccctttctggggtccaataggtaacgacgccttcagcagaaggaatgactttctcacggtgggctttcagacaccagcccacagtagagggtcattgtcttgcacagaggaccctccaccccccatggagatccaggtttaggaagttccctgaataactccacggtagcctgcatgggagcccagacacagaaatagcccctgagacctctcgcatgtgggtgttcaatgttctctgatcccccaaactctgagctggactggagcctagtggcagtaagagagctccctctcagccctctggaatggaacctgcaatgcagagagggctgcagcctgccacgctaggaggccgctccagggccctgtagatgagctgcacgtctcccctggcctcctctaaggagaacagggaaggggccagcaggaagacctattccttgtagcaaaactgtgccgggaacaaaccatgtggccacgcggccagcagcgctgtgattccaggtggtaagcagcagtcagggctggttgttgcccgggtgaccccagtgcttagcatcatttctggcgcagaaagcatcatcaataatacttgttgaaataataactaagtgaataaatgaatgaacaaatgacagcaaattcacagcagagcaaaattcagcaaatggtgtaagaatccatctctggaagcttagatgctcgttatcaggctgtaatttcacctccaagttattcattcccacagtagaccccaagaaaaacactccagaggcttctgtgtatttccctgcctaagccttccatctctgggagatggaagccagaccccattctgttccgggaatgataggctctgtttgcagcttctgtttattctcatacagatggtagaaatgagacactaacaaatgatcccaaaatataatgcattttctgctactgtggaaccccctgaaggagcggccaccccctgggagcacgggccccataaattttgccatttctgctcgcctgtgaatccatcccaatgacaagcctcacccaggagacaaggcactagtctttcctttgtagaagcaaaagtccccctgtctttcctccccctgcaaaagagcccctaactgctcagatataaaccacaaagccctcagccatgccattcctaggagacaaccacaacagctgatattcaccagccagaagtcatcctaaacatttctgggggtgggggatagaagatggaggagctgagcagctgcctttcataattggatcctcattaactgcaaagagctggctgacgatctaaggcagaaaggcaactttagtgatttgaaaaataaaacaatttgatgtgatttagggatctataaaaaagggggagtggggggcagtggaggtggcagcaccaaggaaccagtaacagccagaaggaacttacccacttcaaggaagacttaggaaagatgacaagaggtgaaatcatctcccacactggttgttccatacggaaacaatttagtaggaaaagaagaactacgcactaaaagcttcagaagaacccagagttttttcccttcagggcccaggaggtctgaaaggcagataaacatcctcagtgtctccatgagtaactagggggcataaataaggattaagttctatccattggcagaacaccaacattgggaaaaggggcttatgcctcaaaatataggcctggaatccaagaagactggcaatgcgggacactgaccaggaataagttggaagccagccaatgaaggaaagctgggtgaagcacacatccaagatggcgactgactagcaaggcatgaatcagacagacgaggttcagaaggtcaccgtggaccctaagctgttgttgatcctaagattatgatgcagctccctgaaagccaacttgaagaaaatggggaccagatggatccaagaggaaagaacttgaaaaaaaaaaaaaaaaaggtctgagagctgtactccctactcttcctcagtgacctgtgggcacacagttaggacactgcattgtacaagcagaagaaaagccacaaaacatgtcaagtctagaaaatagaccctcctgggagatactaacatgaagtgtcatttcagagaaaagaaaagctaaaggtaacttattaagctttttcctctggttttcctctctcattttttgtgtgtaaatctgtaaaatattaggttggtgca

SEQ ID NO: 10099 - RNA, 2589 nt, Homo sapiens
  source 1..2589: mol_type = other RNA
caccgactctgtctcctgcagggcagacaaggtgtccccaggcatagcaaagcttgccagctgctcctcccctgggcccgagagccactgcaacacctgctggagtcgccgcaggcactgccgctgctcttgctgctgcacgtgcaggttggagaggcgcacaagctggtgaatggcctcgtccacttcctgatacagtgtagctgggccttggccctccagcttgctgctgggagtggagcgcagcctcatcaggatggcccccccatccctctgcagtgccgtcagccggggatctgccagcaccttctgcagtggcttgggcattcccactgcctcctcttcctctggctctgctgctccctccagctcctcaatggcctgccgtaccgagcccagcacaccttggcacaggcgacatagccttaccacttcctggtgtatctctacccagtgactgggagaggggtccctgtgacctcctaactcccactgcagctcctctggcttggccactcttttcagatcattctctgacagcacctcagcaccctgaaatccacagagttcagttggaaggtcatcatgaatgagaatcagcagccgctgaacaaggggaggatctcctgagtcctaagggcagaaaagaataaccctaaactgaagttggctcaaggcaggaatgagtgctggaggcagtggaggtgcctgacgaaggtccagcaggacggacagccccagtgtctgtagatcaggcctgagcagtgagtggaggtaatgaagagttgtgttcagcgtgtctcgggagggtgggggctcctcaggagggcacggtggggtaatggtcagcagagctcgcccactctggtccacccctcccgtcaggatgaggaatccagatgccatcaagtcccaagctacatcagggtgatcagagacggagactgcaagggcctcttctggaatgttgtccccttttccttcctgcacagtctccagcggaggtgttggagtgtcagacagggggccttctgggcctgtgtgtcctgccatacacagcaggcctggcccctccagctctctctctccggccccctcttctgtaggcccacaggcttcagagagctgaggctctttctcgcctgctgttttgagctcttttggctcagattctggcttccctgagccttcatattcctccttaaccaggtggcattctggaagcttgtgctcacttggtgagggcagattgccaagggcttcttggtggctggcatcttccttgtccccagggctcagtggggcactgtcccctcctcggctaagagcccctcgacctgcagctcgcttctttcttctgtttcctttgcctgttctccgaggggtaccaggtggtccttcagccccctggcctcctcctcctcctcctctaagctcccctggcctcagggggcaagatccggaggcttctcccacagcctctgctgggggctcagacacctccaagactgctgcctctgggacagcctcagctcctgggggagactcaggggaggctccggtgctgctcccctcgccgggtgggcgtgctccatcctggccccgaggccccaggcccttctggtgcatccacgcccggtgtctccggtggcggcccttccctccagcgcccttgcgggtgggtaccgtccggactctggagaggcctggggagccttcagcatctgttgggctccccctcacgggcagcgtcacctctaacagctccacatactcgccctcaggtccttccacaggggcattgtgcccatccccaggactccgggtacccagcgcctcctcaggaagtggagggctgggaagccctggaggtccagagggcagttctgggggcagtgtacttggctgatgtccaaccatgaggccctctttgtgcacaaatcgtggacagatgagctcagcccagggcagccgctgaatcccagagggcgcagacagtaggcaggtactgaggcgacctgttggccggtccttgttgatgccttgtagccactcaggtgtgaataggtaggcacaagcctcattgggcacaggaacctcctgcacccgcccacccccaggggccagacacttgagtgctagtcggggtgcttgggcagctgagggcaccacctgcagatagaagtctcctgggcgcagcagttgccagggtagggctgctagctgcaccaccacctgttcatgcaggcagagcggccacccctcatggaagaagaggaatccactgtattgggcacaggcttcctgctggaccttggcaagcaggtgcttggctggtaccaggaagtccagcgtgtacctcagtgcgtcctcccgataagtcctctccaccacctggaacacctggcccaacagggtgggggctgttgcctcaaagggtggatacagggcggcgagagtgctctgcacacagtcctccactggctcaggctccatggctcggcgccgggccgcgtccgacgcttggtcgggcgggcggggccgggcgcgccaccgcctccctcccgccgctcgtgtctcgccgggtct

SEQ ID NO: 10100 - RNA, 899 nt, Homo sapiens
  source 1..899: mol_type = other RNA
caccgactctgtctcctgcagggcagacaaggtgtccccaggcatagcaaagcttgccagctgctcctcccctgggcccgagagccactgcaacacctgctggagtcgccgcaggcactgccgctgctcttgctgctgcacgtgcaggttggagaggcgcacaagctggtgaatggcctcgtccacttcctgatacagtgtagctgggccttggccctccagcttgctgctgggagtggagcgcagcctcatcaggatggcccccccatccctctgcagtgccgtcagccggggatctgccagcaccttctgcagtggcttgggcattcccactgcctcctcttcctctggctctgctgctccctccagctcctcaatggcctgccgtaccgagcccagcacaccttggcacaggcgacatagccttaccacttcctggtgtatctctacccagtgactgggagaggggtccctgtgacctcctaactcccactgcagctcctctggcttggccactcttttcagatcattctctgacagcacctcagcaccctgaaatccacagagttcagttggaaggtcatcatgaatgagaatcagcagccgctgaacaaggggaggatctcctgagtcctgaagttggctcaaggcaggaatgagtgctggaggcagtggaggtgcctgacgaaggtccagcaggacggacagccccagtgtctgtagatcaggcccgtcaggatgaggaatccagatgccatcaagtcccaagctacatcagggtgatcagagacggagactgcaagggcctcttctggaatgttgtccccttttccttcctgcacagtctccagcggaggtgttggagtgtcagacagggggccttctgggcctgtgtgtcc

SEQ ID NO: 10101 - RNA, 2562 nt, Homo sapiens
  source 1..2562: mol_type = other RNA
caccgactctgtctcctgcagggcagacaaggtgtccccaggcatagcaaagcttgccagctgctcctcccctgggcccgagagccactgcaacacctgctggagtcgccgcaggcactgccgctgctcttgctgctgcacgtgcaggttggagaggcgcacaagctggtgaatggcctcgtccacttcctgatacagtgtagctgggccttggccctccagcttgctgctgggagtggagcgcagcctcatcaggatggcccccccatccctctgcagtgccgtcagccggggatctgccagcaccttctgcagtggcttgggcattcccactgcctcctcttcctctggctctgctgctccctccagctcctcaatggcctgccgtaccgagcccagcacaccttggcacaggcgacatagccttaccacttcctggtgtatctctacccagtgactgggagaggggtccctgtgacctcctaactcccactgcagctcctctggcttggccactcttttcagatcattctctgacagcacctcagcaccctgaaatccacagagttcagttggaaggtcatcatgaatgagaatcagcagccgctgaacaaggggaggatctcctgagtcctgaagttggctcaaggcaggaatgagtgctggaggcagtggaggtgcctgacgaaggtccagcaggacggacagccccagtgtctgtagatcaggcctgagcagtgagtggaggtaatgaagagttgtgttcagcgtgtctcgggagggtgggggctcctcaggagggcacggtggggtaatggtcagcagagctcgcccactctggtccacccctcccgtcaggatgaggaatccagatgccatcaagtcccaagctacatcagggtgatcagagacggagactgcaagggcctcttctggaatgttgtccccttttccttcctgcacagtctccagcggaggtgttggagtgtcagacagggggccttctgggcctgtgtgtcctgccatacacagcaggcctggcccctccagctctctctctccggccccctcttctgtaggcccacaggcttcagagagctgaggctctttctcgcctgctgttttgagctcttttggctcagattctggcttccctgagccttcatattcctccttaaccaggtggcattctggaagcttgtgctcacttggtgagggcagattgccaagggcttcttggtggctggcatcttccttgtccccagggctcagtggggcactgtcccctcctcggctaagagcccctcgacctgcagctcgcttctttcttctgtttcctttgcctgttctccgaggggtaccaggtggtccttcagccccctggcctcctcctcctcctcctctaagctcccctggcctcagggggcaagatccggaggcttctcccacagcctctgctgggggctcagacacctccaagactgctgcctctgggacagcctcagctcctgggggagactcaggggaggctccggtgctgctcccctcgccgggtgggcgtgctccatcctggccccgaggccccaggcccttctggtgcatccacgcccggtgtctccggtggcggcccttccctccagcgcccttgcgggtgggtaccgtccggactctggagaggcctggggagccttcagcatctgttgggctccccctcacgggcagcgtcacctctaacagctccacatactcgccctcaggtccttccacaggggcattgtgcccatccccaggactccgggtacccagcgcctcctcaggaagtggagggctgggaagccctggaggtccagagggcagttctgggggcagtgtacttggctgatgtccaaccatgaggccctctttgtgcacaaatcgtggacagatgagctcagcccagggcagccgctgaatcccagagggcgcagacagtaggcaggtactgaggcgacctgttggccggtccttgttgatgccttgtagccactcaggtgtgaataggtaggcacaagcctcattgggcacaggaacctcctgcacccgcccacccccaggggccagacacttgagtgctagtcggggtgcttgggcagctgagggcaccacctgcagatagaagtctcctgggcgcagcagttgccagggtagggctgctagctgcaccaccacctgttcatgcaggcagagcggccacccctcatggaagaagaggaatccactgtattgggcacaggcttcctgctggaccttggcaagcaggtgcttggctggtaccaggaagtccagcgtgtacctcagtgcgtcctcccgataagtcctctccaccacctggaacacctggcccaacagggtgggggctgttgcctcaaagggtggatacagggcggcgagagtgctctgcacacagtcctccactggctcaggctccatggctcggcgccgggccgcgtccgacgcttggtcgggcgggcggggccgggcgcgccaccgcctccctcccgccgctcgtgtctcgccgggtct

SEQ ID NO: 10102 - RNA, 2642 nt, Homo sapiens
  source 1..2642: mol_type = other RNA
caccgactctgtctcctgcagggcagacaaggtgtccccaggcatagcaaagcttgccagctgctcctcccctgggcccgagagccactgcaacacctgctggagtcgccgcaggcactgccgctgctcttgctgctgcacgtgcaggttggagaggcgcacaagctggtgaatggcctcgtccacttcctgatacagtgtagctgggccttggccctccagcttgctgctgggagtggagcgcagcctcatcaggatggcccccccatccctctgcagtgccgtcagccggggatctgccagcaccttctgcagtggcttgggcattcccactgcctcctcttcctctggctctgctgctccctccagctcctcaatggcctgccgtaccgagcccagcacaccttggcacaggcgacatagccttaccacttcctggtgtatctctacccagtgactgggagaggggtccctgtgacctcctaactcccactgcagctcctctggcttggccactcttttcagatcattctctgacagcacctcagcaccctgaaatccacagagttcagttggaaggtcatcatgaatgagaatcagcagccgctgaacaaggggaggatctcctgagtcctgaagttggctcaaggcaggaatgagtgctggaggcagtggaggtgcctgacgaaggtccagcaggacggacagccccagtgtctgtagatcaggcctgagcagtgagtggaggtaatgaagagttgtgttcagcgtgtctcgggagggtgggggctcctcaggagggcacggtggggtaatggtcagcagagctcgcccactctggtccacccctcccgtcaggatgaggaatccagatgccatcaagtcccaagctacatcagggtgatcagagacggagactgcaagggcctcttctggaatgttgtccccttttccttcctgcacagtctccagcggaggtgttggagtgtcagacagggggccttctgggcctgtgtgtcctgccatacacagcaggcctggcccctccagctctctctctccggccccctcttctgtaggcccacaggcttcagagagctgaggctctttctcgcctgctgttttgagctcttttggctcagattctggcttccctgagccttcatattcctccttaaccaggtggcattctggaagcttgtgctcacttggtgagggcagattgccaagggcttcttggtggctggcatcttccttgtccccagggctcagtggggcactgtcccctcctcggctaagagcccctcgacctgcagctcgcttctttcttctgtttcctttgcctgttctccgaggggtaccaggtggtccttcagccccctggcctcctcctcctcctcctctaagctcccctggcctcagggggcaagatccggaggcttctcccacagcctctgctgggggctcagacacctccaagactgctgcctctgggacagcctcagctcctgggggagactcaggggaggctccggtgctgctcccctcgccgggtgggcgtgctccatcctggccccgaggccccaggcccttctggtgcatccacgcccggtgtctccggtggcggcccttccctccagcgcccttgcgggtgggtaccgtccggactctggagaggcctggggagccttcagcatctgttgggctccccctcacgggcagcgtcacctctaacagctccacatactcgccctcaggtccttccacaggggcattgtgcccatccccaggactccgggtacccagcgcctcctcaggaagtggagggctgggaagccctggaggtccagagggcagttctgggggcagtgtacttggctgatgtccaaccatgaggccctctttgtgcacaaatcgtggacagatgagctcagcccagggcagccgctgaatcccagagggcgcagacagtaggcaggtactgaggcgacctgttggccggtccttgttgatgccttgtagccactcaggtgtgaataggtaggcacaagcctcattgggcacaggaacctcctgcacccgcccacccccaggggccagacacttgagtgctagtcggggtgcttgggcagctgagggcaccacctgcagatagaagtctcctgggcgcagcagttgccagggtagggctgctagctgcaccaccacctgttcatgcaggcagagcggccacccctcatggaagaagaggaatccactgtattgggcacaggcttcctgctggaccttggcaagcaggtgcttggctggtaccaggaagtccagcgtgtacctcagtgcgtcctcccgataagtcctctccaccacctggaacacctggcccaacagggtgggggctgttgcctcaaagggtggatacagggcggcgagagtgctctgcacacagtcctccactggctcaggctccatggctcggcgccgggccgcgtccgacgcttggtcgggcgggcggggccgggcgcgccaccgcctccctcccgccgctcgtgtctcgccgggtctggctaagggacagctccggccgcggtggcggctcggcccgctccggcttccaggccgcggggccccgccagggagggccg

SEQ ID NO: 10103 - RNA, 2643 nt, Homo sapiens
  source 1..2643: mol_type = other RNA
caccgactctgtctcctgcagggcagacaaggtgtccccaggcatagcaaagcttgccagctgctcctcccctgggcccgagagccactgcaacacctgctggagtcgccgcaggcactgccgctgctcttgctgctgcacgtgcaggttggagaggcgcacaagctggtgaatggcctcgtccacttcctgatacagtgtagctgggccttggccctccagcttgctgctgggagtggagcgcagcctcatcaggatggcccccccatccctctgcagtgccgtcagccggggatctgccagcaccttctgcagtggcttgggcattcccactgcctcctcttcctctggctctgctgctccctccagctcctcaatggcctgccgtaccgagcccagcacaccttggcacaggcgacatagccttaccacttcctggtgtatctctacccagtgactgggagaggggtccctgtgacctcctaactcccactgcagctcctctggcttggccactcttttcagatcattctctgacagcacctcagcaccctgaaatccacagagttcagttggaaggtcatcatgaatgagaatcagcagccgctgaacaaggggaggatctcctgagtcctgaagttggctcaaggcaggaatgagtgctggaggcagtggaggtgcctgacgaaggtccagcaggacggacagccccagtgtctgtagatcaggcctgagcagtgagtggaggtaatgaagagttgtgttcagcgtgtctcgggagggtgggggctcctcaggagggcacggtggggtaatggtcagcagagctcgcccactctggtccacccctcccgtcaggatgaggaatccagatgccatcaagtcccaagctacatcagggtgatcagagacggagactgcaagggcctcttctggaatgttgtccccttttccttcctgcacagtctccagcggaggtgttggagtgtcagacagggggccttctgggcctgtgtgtcctgccatacacagcaggcctggcccctccagctctctctctccggccccctcttctgtaggcccacaggcttcagagagctgaggctctttctcgcctgctgttttgagctcttttggctcagattctggcttccctgagccttcatattcctccttaaccaggtggcattctggaagcttgtgctcacttggtgagggcagattgccaagggcttcttggtggctggcatcttccttgtccccagggctcagtggggcactgtcccctcctcggctaagagcccctcgacctgcagctcgcttctttcttctgtttcctttgcctgttctccgaggggtaccaggtggtccttcagccccctggcctcctcctcctcctcctctaagctcccctggcctcagggggcaagatccggaggcttctcccacagcctctgctgggggctcagacacctccaagactgctgcctctgggacagcctcagctcctgggggagactcaggggaggctccggtgctgctcccctcgccgggtgggcgtgctccatcctggccccgaggccccaggcccttctggtgcatccacgcccggtgtctccggtggcggcccttccctccagcgcccttgcgggtgggtaccgtccggactctggagaggcctggggagccttcagcatctgttgggctccccctcacgggcagcgtcacctctaacagctccacatactcgccctcaggtccttccacaggggcattgtgcccatccccaggactccgggtacccagcgcctcctcaggaagtggagggctgggaagccctggaggtccagagggcagttctgggggcagtgtacttggctgatgtccaaccatgaggccctctttgtgcacaaatcgtggacagatgagctcagcccagggcagccgctgaatcccagagggcgcagacagtaggcaggtactgaggcgacctgttggccggtccttgttgatgccttgtagccactcaggtgtgaataggtaggcacaagcctcattgggcacaggaacctcctgcacccgcccacccccaggggccagacacttgagtgctagtcggggtgcttgggcagctgagggcaccacctgcagatagaagtctcctgggcgcagcagttgccagggtagggctgctagctgcaccaccacctgttcatgcaggcagagcggccacccctcatggaagaagaggaatccactgtattgggcacaggcttcctgctggaccttggcaagcaggtgcttggctggtaccaggaagtccagcgtgtacctcagtgcgtcctcccgataagtcctctccaccacctggaacacctggcccaacagggtgggggctgttgcctcaaagggtggatacagggcggcgagagtgctctgcacacagtcctccactggctcaggctccatggctcggcgccgggccgcgtccgacgcttggtcgggcgggcggggccgggcgcgccaccgcctccctcccgccgctcgtgtctcgccgggtctggctaagggacagctccggccgcggtggcggctcggcccgctccggcttccaggccgcggggccccgccagggagggccga

SEQ ID NO: 10104 - RNA, 2645 nt, Homo sapiens
  source 1..2645: mol_type = other RNA
caccgactctgtctcctgcagggcagacaaggtgtccccaggcatagcaaagcttgccagctgctcctcccctgggcccgagagccactgcaacacctgctggagtcgccgcaggcactgccgctgctcttgctgctgcacgtgcaggttggagaggcgcacaagctggtgaatggcctcgtccacttcctgatacagtgtagctgggccttggccctccagcttgctgctgggagtggagcgcagcctcatcaggatggcccccccatccctctgcagtgccgtcagccggggatctgccagcaccttctgcagtggcttgggcattcccactgcctcctcttcctctggctctgctgctccctccagctcctcaatggcctgccgtaccgagcccagcacaccttggcacaggcgacatagccttaccacttcctggtgtatctctacccagtgactgggagaggggtccctgtgacctcctaactcccactgcagctcctctggcttggccactcttttcagatcattctctgacagcacctcagcaccctgaaatccacagagttcagttggaaggtcatcatgaatgagaatcagcagccgctgaacaaggggaggatctcctgagtcctgaagttggctcaaggcaggaatgagtgctggaggcagtggaggtgcctgacgaaggtccagcaggacggacagccccagtgtctgtagatcaggcctgagcagtgagtggaggtaatgaagagttgtgttcagcgtgtctcgggagggtgggggctcctcaggagggcacggtggggtaatggtcagcagagctcgcccactctggtccacccctcccgtcaggatgaggaatccagatgccatcaagtcccaagctacatcagggtgatcagagacggagactgcaagggcctcttctggaatgttgtccccttttccttcctgcacagtctccagcggaggtgttggagtgtcagacagggggccttctgggcctgtgtgtcctgccatacacagcaggcctggcccctccagctctctctctccggccccctcttctgtaggcccacaggcttcagagagctgaggctctttctcgcctgctgttttgagctcttttggctcagattctggcttccctgagccttcatattcctccttaaccaggtggcattctggaagcttgtgctcacttggtgagggcagattgccaagggcttcttggtggctggcatcttccttgtccccagggctcagtggggcactgtcccctcctcggctaagagcccctcgacctgcagctcgcttctttcttctgtttcctttgcctgttctccgaggggtaccaggtggtccttcagccccctggcctcctcctcctcctcctctaagctcccctggcctcagggggcaagatccggaggcttctcccacagcctctgctgggggctcagacacctccaagactgctgcctctgggacagcctcagctcctgggggagactcaggggaggctccggtgctgctcccctcgccgggtgggcgtgctccatcctggccccgaggccccaggcccttctggtgcatccacgcccggtgtctccggtggcggcccttccctccagcgcccttgcgggtgggtaccgtccggactctggagaggcctggggagccttcagcatctgttgggctccccctcacgggcagcgtcacctctaacagctccacatactcgccctcaggtccttccacaggggcattgtgcccatccccaggactccgggtacccagcgcctcctcaggaagtggagggctgggaagccctggaggtccagagggcagttctgggggcagtgtacttggctgatgtccaaccatgaggccctctttgtgcacaaatcgtggacagatgagctcagcccagggcagccgctgaatcccagagggcgcagacagtaggcaggtactgaggcgacctgttggccggtccttgttgatgccttgtagccactcaggtgtgaataggtaggcacaagcctcattgggcacaggaacctcctgcacccgcccacccccaggggccagacacttgagtgctagtcggggtgcttgggcagctgagggcaccacctgcagatagaagtctcctgggcgcagcagttgccagggtagggctgctagctgcaccaccacctgttcatgcaggcagagcggccacccctcatggaagaagaggaatccactgtattgggcacaggcttcctgctggaccttggcaagcaggtgcttggctggtaccaggaagtccagcgtgtacctcagtgcgtcctcccgataagtcctctccaccacctggaacacctggcccaacagggtgggggctgttgcctcaaagggtggatacagggcggcgagagtgctctgcacacagtcctccactggctcaggctccatggctcggcgccgggccgcgtccgacgcttggtcgggcgggcggggccgggcgcgccaccgcctccctcccgccgctcgtgtctcgccgggtctggctaagggacagctccggccgcggtggcggctcggcccgctccggcttccaggccgcggggccccgccagggagggccgaga

SEQ ID NO: 10105 - RNA, 2899 nt, Homo sapiens
  source 1..2899: mol_type = other RNA
caccgactctgtctcctgcagggcagacaaggtgtccccaggcatagcaaagcttgccagctgctcctcccctgggcccgagagccactgcaacacctgctggagtcgccgcaggcactgccgctgctcttgctgctgcacgtgcaggttggagaggcgcacaagctggtgaatggcctcgtccacttcctgatacagtgtagctgggccttggccctccagcttgctgctgggagtggagcgcagcctcatcaggatggcccccccatccctctgcagtgccgtcagccggggatctgccagcaccttctgcagtggcttgggcattcccactgcctcctcttcctctggctctgctgctccctccagctcctcaatggcctgccgtaccgagcccagcacaccttggcacaggcgacatagccttaccacttcctggtgtatctctacccagtgactgggagaggggtccctgtgacctcctaactcccactgcagctcctctggcttggccactcttttcagatcattctctgacagcacctcagcaccctgaaatccacagagttcagttggaaggtcatcatgaatgagaatcagcagccgctgaacaaggggaggatctcctgagtcctgaagttggctcaaggcaggaatgagtgctggaggcagtggaggtgcctgacgaaggtccagcaggacggacagccccagtgtctgtagatcaggcctgagcagtgagtggaggtaatgaagagttgtgttcagcgtgtctcgggagggtgggggctcctcaggagggcacggtggggtaatggtcagcagagctcgcccactctggtccacccctcccgtcaggatgaggaatccagatgccatcaagtcccaagctacatcagggtgatcagagacggagactgcaagggcctcttctggaatgttgtccccttttccttcctgcacagtctccagcggaggtgttggagtgtcagacagggggccttctgggcctgtgtgtcctgccatacacagcaggcctggcccctccagctctctctctccggccccctcttctgtaggcccacaggcttcagagagctgaggctctttctcgcctgctgttttgagctcttttggctcagattctggcttccctgagccttcatattcctccttaaccaggtggcattctggaagcttgtgctcacttggtgagggcagattgccaagggcttcttggtggctggcatcttccttgtccccagggctcagtggggcactgtcccctcctcggctaagagcccctcgacctgcagctcgcttctttcttctgtttcctttgcctgttctccgaggggtaccaggtggtccttcagccccctggcctcctcctcctcctcctctaagctcccctggcctcagggggcaagatccggaggcttctcccacagcctctgctgggggctcagacacctccaagactgctgcctctgggacagcctcagctcctgggggagactcaggggaggctccggtgctgctcccctcgccgggtgggcgtgctccatcctggccccgaggccccaggcccttctggtgcatccacgcccggtgtctccggtggcggcccttccctccagcgcccttgcgggtgggtaccgtccggactctggagaggcctggggagccttcagcatctgttgggctccccctcacgggcagcgtcacctctaacagctccacatactcgccctcaggtccttccacaggggcattgtgcccatccccaggactccgggtacccagcgcctcctcaggaagtggagggctgggaagccctggaggtccagagggcagttctgggggcagtgtacttggctgatgtccaaccatgaggccctctttgtgcacaaatcgtggacagatgagctcagcccagggcagccgctgaatcccagagggcgcagacagtaggcaggtactgaggcgacctgttggccggtccttgttgatgccttgtagccactcaggtgtgaataggtaggcacaagcctcattgggcacaggaacctcctgcacccgcccacccccaggggccagacacttgagtgctagtcggggtgcttgggcagctgagggcaccacctgcagatagaagtctcctgggcgcagcagttgccagggtagggctgctagctgcaccaccacctgttcatgcaggcagagcggccacccctcatggaagaagaggaatccactgtattgggcacaggcttcctgctggaccttggcaagcaggtgcttggctggtaccaggaagtccagcgtgtacctcagtgcgtcctcccgataagtcctctccaccacctggaacacctggcccaacagggtgggggctgttgcctcaaagggtggatacagggcggcgagagtgctctgcacacagtcctccactggctcaggctcctcctctggacgctaacctccacctttttctccgctccgctgagcccactggaaaatatttatgtcctcccaaatggctgaggagccccttctcaagtgattttttggaaacacgttctcaggggcccagagaacacacccagtagagattcggtcccaaggctattgggcagctcttctgtggtcccagcttcaccactgagccctgttttatgggtgctgtgtcattaccctcagagtgggccagttttacagcccatgacccctagattccagttacacgccatctaattcttcagcctacacaaggaagtcagaaactcctacccaggttgctacccccacttgtttggatataattagtctccttaacgattcattctactctgaatgcttttcacactcttcccagcttccggggccacaactctta

SEQ ID NO: 10106 - RNA, 2395 nt, Homo sapiens
  source 1..2395: mol_type = other RNA
caccgactctgtctcctgcagggcagacaaggtgtccccaggcatagcaaagcttgccagctgctcctcccctgggcccgagagccactgcaacacctgctggagtcgccgcaggcactgccgctgctcttgctgctgcacgtgcaggttggagaggcgcacaagctggtgaatggcctcgtccacttcctgatacagtgtagctgggccttggccctccagcttgctgctgggagtggagcgcagcctcatcaggatggcccccccatccctctgcagtgccgtcagccggggatctgccagcaccttctgcagtggcttgggcattcccactgcctcctcttcctctggctctgctgctccctccagctcctcaatggcctgccgtaccgagcccagcacaccttggcacaggcgacatagccttaccacttcctggtgtatctctacccagtgactgggagaggggtccctgtgacctcctaactcccactgcagctcctctggcttggccactcttttcagatcattctctgacagcacctcagcaccctgaaatccacagagttcagttggaaggtcatcatgaatgagaatcagcagccgctgaacaaggggaggatctcctgagtcctgaagttggctcaaggcaggaatgagtgctggaggcagtggaggtgcctgacgaaggtccagcaggacggacagccccagtgtctgtagatcaggcctgagcagtgagtggaggtaatgaagagttgtgttcagcgtgtctcgggagggtgggggctcctcaggagggcacggtggggtaatggtcagcagagctcgcccactctggtccacccctcctgaagacacaaaatggccaggccgtcaggatgaggaatccagatgccatcaagtcccaagctacatcagggtgatcagagacggagactgcaagggcctcttctggaatgttgtccccttttccttcctgcacagtctccagcggaggtgttggagtgtcagacagggggccttctgggcctgtgtgtcttggtgagggcagattgccaagggcttcttggtggctggcatcttccttgtccccagggctcagtggggcactgtcccctcctcggctaagagcccctcgacctgcagctcgcttctttcttctgtttcctttgcctgttctccgaggggtaccaggtggtccttcagccccctggcctcctcctcctcctcctctaagctcccctggcctcagggggcaagatccggaggcttctcccacagcctctgctgggggctcagacacctccaagactgctgcctctgggacagcctcagctcctgggggagactcaggggaggctccggtgctgctcccctcgccgggtgggcgtgctccatcctggccccgaggccccaggcccttctggtgcatccacgcccggtgtctccggtggcggcccttccctccagcgcccttgcgggtgggtaccgtccggactctggagaggcctggggagccttcagcatctgttgggctccccctcacgggcagcgtcacctctaacagctccacatactcgccctcaggtccttccacaggggcattgtgcccatccccaggactccgggtacccagcgcctcctcaggaagtggagggctgggaagccctggaggtccagagggcagttctgggggcagtgtacttggctgatgtccaaccatgaggccctctttgtgcacaaatcgtggacagatgagctcagcccagggcagccgctgaatcccagagggcgcagacagtaggcaggtactgaggcgacctgttggccggtccttgttgatgccttgtagccactcaggtgtgaataggtaggcacaagcctcattgggcacaggaacctcctgcacccgcccacccccaggggccagacacttgagtgctagtcggggtgcttgggcagctgagggcaccacctgcagatagaagtctcctgggcgcagcagttgccagggtagggctgctagctgcaccaccacctgttcatgcaggcagagcggccacccctcatggaagaagaggaatccactgtattgggcacaggcttcctgctggaccttggcaagcaggtgcttggctggtaccaggaagtccagcgtgtacctcagtgcgtcctcccgataagtcctctccaccacctggaacacctggcccaacagggtgggggctgttgcctcaaagggtggatacagggcggcgagagtgctctgcacacagtcctccactggctcaggctccatggctcggcgccgggccgcgtccgacgcttggtcgggcgggcggggccgggcgcgccaccgcctccctcccgccgctcgtgtctcgccgggtct

SEQ ID NO: 10107 - RNA, 3118 nt, Homo sapiens
  source 1..3118: mol_type = other RNA
caccgactctgtctcctgcagggcagacaaggtgtccccaggcatagcaaagcttgccagctgctcctcccctgggcccgagagccactgcaacacctgctggagtcgccgcaggcactgccgctgctcttgctgctgcacgtgcaggttggagaggcgcacaagctggtgaatggcctcgtccacttcctgatacagtgtagctgggccttggccctccagcttgctgctgggagtggagcgcagcctcatcaggatggcccccccatccctctgcagtgccgtcagccggggatctgccagcaccttctgcagtggcttgggcattcccactgcctcctcttcctctggctctgctgctccctccagctcctcaatggcctgccgtaccgagcccagcacaccttggcacaggcgacatagccttaccacttcctggtgtatctctacccagtgactgggagaggggtccctgtgacctcctaactcccactgcagctcctctggcttggccactcttttcagatcattctctgacagcacctcagcaccctgaaatccacagagttcagttggaaggtcatcatgaatgagaatcagcagccgctgaacaaggggaggatctcctgagtcctgaagttggctcaaggcaggaatgagtgctggaggcagtggaggtgcctgacgaaggtccagcaggacggacagccccagtgtctgtagatcaggcctgcgggagcaggaagagccaaggaggctgctgtgtgtgtgttttgggggatagcagataaggcaaggcagacatacggggtctgtttttagttaatagtcctgaggagaaattagttgccggtacatttgggaagaaatgggcaaagggccaaattctggggtgtgtgtacaagaggaagtcacctagcagtcaggggtctatattcatatggctactaggtcaagggattaaggtctggaaaattaagaattctgttctgaaatggcgtgcattcaatatcagcctgtagtatggtgcctaataggtactcagtgctcaataaatgtttgttgaatcagtgaaccaatgtcctgatgatcttggtagggttggaagagagtgaaagtcaacagtgttgcttttgaagatcagtgaagatatgaagctggaggtcagggtaagtaaggccaaaggtcaatggcttgaagtctgaaggttgaagaagtaggtgtccttagaggtcagaaggtcagtgtcctgagaagaaggaggtgagggtcctcatgaatcaggaggttagtgtccagggtgccaggactgggcctcggttacccgtcaggatgaggaatccagatgccatcaagtcccaagctacatcagggtgatcagagacggagactgcaagggcctcttctggaatgttgtccccttttccttcctgcacagtctccagcggaggtgttggagtgtcagacagggggccttctgggcctgtgtgtcctgccatacacagcaggcctggcccctccagctctctctctccggccccctcttctgtaggcccacaggcttcagagagctgaggctctttctcgcctgctgttttgagctcttttggctcagattctggcttccctgagccttcatattcctccttaaccaggtggcattctggaagcttgtgctcacttggtgagggcagattgccaagggcttcttggtggctggcatcttccttgtccccagggctcagtggggcactgtcccctcctcggctaagagcccctcgacctgcagctcgcttctttcttctgtttcctttgcctgttctccgaggggtaccaggtggtccttcagccccctggcctcctcctcctcctcctctaagctcccctggcctcagggggcaagatccggaggcttctcccacagcctctgctgggggctcagacacctccaagactgctgcctctgggacagcctcagctcctgggggagactcaggggaggctccggtgctgctcccctcgccgggtgggcgtgctccatcctggccccgaggccccaggcccttctggtgcatccacgcccggtgtctccggtggcggcccttccctccagcgcccttgcgggtgggtaccgtccggactctggagaggcctggggagccttcagcatctgttgggctccccctcacgggcagcgtcacctctaacagctccacatactcgccctcaggtccttccacaggggcattgtgcccatccccaggactccgggtacccagcgcctcctcaggaagtggagggctgggaagccctggaggtccagagggcagttctgggggcagtgtacttggctgatgtccaaccatgaggccctctttgtgcacaaatcgtggacagatgagctcagcccagggcagccgctgaatcccagagggcgcagacagtaggcaggtactgaggcgacctgttggccggtccttgttgatgccttgtagccactcaggtgtgaataggtaggcacaagcctcattgggcacaggaacctcctgcacccgcccacccccaggggccagacacttgagtgctagtcggggtgcttgggcagctgagggcaccacctgcagatagaagtctcctgggcgcagcagttgccagggtagggctgctagctgcaccaccacctgttcatgcaggcagagcggccacccctcatggaagaagaggaatccactgtattgggcacaggcttcctgctggaccttggcaagcaggtgcttggctggtaccaggaagtccagcgtgtacctcagtgcgtcctcccgataagtcctctccaccacctggaacacctggcccaacagggtgggggctgttgcctcaaagggtggatacagggcggcgagagtgctctgcacacagtcctccactggctcaggctccatggctcggcgccgggccgcgtccgacgcttggtcgggcgggcggggccgggcgcgccaccgcctccctcccgccgctcgtgtctcgccgggtctggctaagggacagctccggccgcggtggcggctcggcccgctccggcttccaggccgcggggccccgccagggagggccgaga

SEQ ID NO: 10108 - RNA, 365 nt, Homo sapiens
  source 1..365: mol_type = other RNA
caccgactctgtctcctgcagtgaagtctgtttgaaggatgtatttggctgtcttctggacaggccattatttgtttctgtttcactccatgacaaagtctataggacacccctggcaagaagggcgacttttctagaaaaacttagcggcaagttaacgggaagcgcggcgacacagttcctacgattgtggggggcactctgccgccaggcagtctcatcctttgtcctttgagaggcctccttgaagccgaaggctcttaagtgtccctgggcaacccttgactcgatctccattacgggccctcactgacagcagccatgacagttgcttccggatatattgaatcgccgcggccagagtc

SEQ ID NO: 10109 - RNA, 951 nt, Homo sapiens
  source 1..951: mol_type = other RNA
caccgactctgtctcctgcagtttactgagccccacactacgctttagctccagaggaacctgatttagcttcatcgtgtggagcgcatcatggcttggtttggtctcatagtcaatgtcaaactgtttcaagatgaactcttcatcgatgtccgaaattccaaaagtagtaacccacttgcagaagtcactaactgctttgcatacattttcatgaagaccaggacgaggaccattttcatggagcaaatccattttatgtggcttttcttcataaagccattggcctgcgtttgacacagacgtcttcttggaaggtcccaggtagacttgggtagaatgtttttttaaaagcttcgtgggttccttcattcctttcctggtgtcctgacaataagcccatgtgtcctccagcttccggtcaggatcaagcacttccagcacctttgataagagctgagattgggtagtgaaaagaggtttatttggctcatggttctgcaggctggacaagacgcacggcacagacatctgcattggatgagggcctcaggctgcttccactccgtttccttctccgtgaaatgcctcctcctcccttttttgcacatcttccattcttgcacatgccccttacgtgacaaacttatgcatcccccaggccccagttcaatgtggggccctaggtcatccaggcagaacatgcttgctggcatgatctcagcaggcacctggtagaagcacttgctacattgtgttgtaattgcggtaacggtgtccccgctaacttgcgagcgcctctagagcaggggaatgtcccagccaccttgaatccccagcgcgtggcccatgggaggccctcagacctatctgcggaatgagtaaatgagtgtgtgaaccaggttcggcaatttcggtggggcgagcgctgggcctgcggtgcagggcgct

SEQ ID NO: 10110 - RNA, 857 nt, Homo sapiens
  source 1..857: mol_type = other RNA
caccgactctgtctcctgcagtttactgagccccacactacgctttagctccagaggaacctgatttagcttcatcgtgtggagcgcatcatggcttggtttggtctcatagtcaatgtcaaactgtttcaagatgaactcttcatcgatgtccgaaattccattttcatgaagaccaggacgaggaccattttcatggagcaaatccattttatgtggcttttcttcataaagccattggcctgcgtttgacacagacgtcttcttggaaggtcccaggtagacttgggtagaatgtttttttaaaagcttcgtgggttccttcattcctttcctggtgtcctgacaataagcccatgtgtcctccagcttccggtcaggatcaagcacttccagcacctttgataagagctctatgggcatagcttcttccagattcaggtagagcgctaagggatgtggggtcaggtgggcctccacgtcctccaggaatgccttccgagcctgctgggctggcgagagcttggaaagcacgtctgcttccttgagcagcttgatctgcctcttctttggggccagttggggagctctgtgataaatctggggcagaaagccctccacagggacctgagtcaccagaccagtgcaaggcgggcagcccttcctgaagtcgtccagcccctttcttggaaataccaactgccggctgtgcagagaggtggggaacttcagcccgttcttgtgctttgtgaaacatctggacctgcagttcacgccctcgcgcaccggggccaacgtccccggccggagccgccgcctgcggtccgccatggtggccctagcttcgcggccaccgt

SEQ ID NO: 10111 - RNA, 2710 nt, Homo sapiens
  source 1..2710: mol_type = other RNA
cacctttgtgtccccatcctgcacatgaaggcagtactctggcaggcctctcgctaggctaggagggagacaggattcaggaaccatgcctgggaggccctgagtgggataggccttcagatggacatggccctcagatggcctcttgttggctgtagaagtggtgcttagtttttgcagtttgaaggtctttaggtgcaaaaagccctctctgtttgcccatagtccccacacatccctcttggtcaacacctttgcccatccacatttccatcacctgcctggcctctgaaggcatttgtttttgagcacctggctttagcaatttcaagttcaaacagccccctttccgccaggatgaggctcattcattcattcaacaaatgtgtacagagcacctcatctttgtcagaccctgttccaggtgctgggatggatcaatgaaccaagcaatcgaaagccctgtcttcctggcacttccattcatgtggtcctggatagtgagaggaagttacaaagagcatggggcctggggcctgcatggtcagttcctggggccagcgggctcccaggagcctgactacaagctcagtccttgcctcgtgtccttcccccatcagctcaacctaaggcccaagttcatgggtccagtgggagtcaaaggaggaaacagccagcaactccctcctcgagcagcagcccggtccatcaggcaccctggtgtcagcagggtgcatcatcagctcctggaaggttaatgccagcccagatgctaggctctaggactgggagggggaatgagtcgagcagcttagaatagccatccaatagccagaggaaagggcaccattattatccttactctacagttagaggaactgaggctcaggcaggcaaagtcacacagctaggaaaggatatgtagggacccacgtctgcctgaccccaaagccaggagtcaggtccagactctcaagggagtggtttcctattattcaagagacttcaccttctttctcctttctcctttcctgcctgatcttcgggcccaccgctgtaaagcagatgctgctgtttgtccttagtgaagctcccattccattgctattggcaccccagacccggcgtctttgttatgctgacgggtggtcctatgtagggggagctggtttcttaatcctaggatgccccttctccaaggagttgtgtcagaggctgacccaaagctgggtgcaatcatatgtgctcaataactgtctgtggataacttttgtggactaatttacttgaccagaagccagcattcgagaggagcctggcatagtgagcaaatctctgaaatcagctacatgtggcctcaccacttaacggcgatgggaccttggacctgtgagccaattctttatccataaaatggggatgctccttcctcccctgcagatggctatgaggatgcatccagtagaagccccgtaagtgcctgtgtggggcttcttctaccacagacatggaattagcatgagtagccaagagggggagaagtcaggaaggcctgacataggagaaggatccatttgtgaaacttgatcctgaacaggaggctgagaacagggccttgaaacagccctgtggaccaaatggggcaggtgaaccctctttgcttggctcaggtggagagggtgatttgttttgagatcttatcttattggacaagtcagtcatacgcctgccctaaacagccatgggccatggggatgtgatgtgctgactggcacagtcatgtgttcctcctggtgcagtccagatcctgttgcctgaagtggggatgggggacccctggtcaactatgggggactactgcctcttggcagagaggcaccatgacaacccaccaaagtgggctaatcaggcctctgctctgatttatttggagtcatccttcctcctcttgcaacttctattcatccttaaaaacccagcttaaacactgctgctggaagcatccctgtgcaacttcaaccttctctgagcctctgtggtgcgggcagcctctgccacataatgtatcaacctccagatcatcactgctccagcatagctgaaatattgcctatggtttgccaagtgtgggcacgttatcctcataacaactgagaaaggggaaagccctctgacagcctgggctggcctggcattcacagccaggccatggtgttctgttggacatgaacagttctacagcccagaaacatcagacaagaccgctcggtaaccatgaaggatcaaaacaaagacgagaccattctgtagtcctgcctgaacgcagacgaaaacgtgaacatcgtccaaatgacaaaactgcccaaatgttccccttcctggctcaaatgtttcttaactaattgcagttgtagctttgctcagttcctcctgccgtctagaagagaatcattgacatacccaatcacagaattacccttgcttcctgacagcatccagcctagagaaacagcctgcaaaatcacttaatgcgagcccaaatcccatgatcagtcctactaacatcccctccccgagacatccaggggtgcgcattcccctccagtgcagtgactcaaaaagccaactttgttcaaccgaaaggtgtgttcctggtagcctttggccggagggcattgcatgatcctgcaaaagagatgttattgttctt

SEQ ID NO: 10112 - RNA, 881 nt, Homo sapiens
  source 1..881: mol_type = other RNA
cacgctcatgcacacacccacacacatacacaaatgaatgcacacacgtgcacacgtgtgcacacacacaaatgcacacaaggatccatgcagatgcccccacacagatgcacacaaataagtgcacacacaaatgtacacactcaaacacgcccatgcacgtgtacacactcacaaacacacacaagaatgcatgcaaattcccacatgcacacacacacatgcacatacacaaacacacacaagcatgcatgcaaattcccacatgcacacacacacatgcacatacacaaacacacaaggatacacacatgcctgcatgcaatccccccatgcacatgcacgcacatgtgtgcacacatacaaatgcacacacaagcacacctatgcacgcacccacaaatgcagccaaggatacatgcgcgtgccccacacacaaatatgcaaacaaatcacacacccagacacacccatgtacatgtgtacatctatacacacacacacacgagcacgcttgtacatgaacaaacacagagaaatgcacacacaacactcagagtccatcacaaaggtctgagcaacgcgagtgcctggggggagctagggctgtttggggaaaagaaggggaaacccagagtctggggggcagctcagggttcacgcgcctctgggggacttctgaggggcagattgcttcagtgctctgtgtcttagtcgcttcatcctgtctggctctggatgtggggtttgagggactctgaggatgcatgggaggagtgggtctcagggatcaggagacacatccagcagctgcagcctaactgcttcatcatcagtcccggtttcccctcctgtgcaatggggcaagtcccttcttgctt

SEQ ID NO: 10113 - RNA, 5737 nt, Homo sapiens
  source 1..5737: mol_type = other RNA
cacgctcatgcacacacccacacagagcttaaccacacatggatttcctttaataataaatctaccacatactattatattacaatttataatagcgtttttgaagacacaatggggaaagctttgtcattcatttataaaccgtccataaattacaaaagaaaggcagtctgaaaagtatgtataaagagtaaaaacaatttacaagtggacaagaattacaaaagagtaaccatcaaatacatctgccagcaactttgtaagtaagtcttttgttcaaatgccaatgatgaagatgggtatggactcatttggagcagatttaaattgagtctggttttggtgtggcttatgcattatgtggattacttgtgtgccattcattgctgtgtatttgggtatggcattttgacaacgaaagtaacagaaaaccatatgccacagaatagaacattaaaagcaatgaagataatcggctttctggaaggttggagtactggtgctttaccaaacaaagttactttctctccttttctcttttttgaatgattgagtaaacattttctgtgtgtagcctggctggctttgaaagactgaaactagtatcttaaaatgcacagcctgtacaacttgatctcaaaccactgtgtcaggatgaagaccactgaatgcacgacacatacaaagtatacactgtttttattagacagtacaaatcattgtgcatttataaggcagaacatcaaggcgaattaaactaggaatttcaagaccagagtcaaagtgaaagttatgcattatgaggcaagcattttgagaagggagaaaggttgaaaatcattcctttaagggcagatgacaaatgcacaaagactggaattacaggtagggagggagctacaggtgatagctatgcgcccccgtttgttaataagacgtcccctcccacctcccaaatcagagcttggacaatgagagcagactgccagcggtgacagagagcaaccgctcctctttgttctcgtggttggtttaaagtggttggtagtgcaaaagtgcatttctctactggtgtcaggggagaagattgggtttttttaggaagtacttgagtcatgaaagcccctttttgcctttgagcgcattggcgtatcttgagagtagtgggatggagcatcagaaagatagacttctacgtcatcaggcacttcttccaagaagtttgagggcacaaggcctttctgcccattcagctccccataataaaatccatcttcatcaatttcaccaaaaactgtaataatatctcctgtgcaaaatgtaagttcggcctcgacatcgacgttgggcgagctttctctggggtcgtagtcatacagggccaccattctccgcgtcgataccgaatgacgcctgccacttctcctgcttctctctattttctccacaggtgtattcagagggagaaagccctgtctaagaagctgatccatcatctcctcatcatctgcttgtatctcagagaccatgttacaaggaataaggccaagccgggcacaggtttccccacggtagaatccatcagcgtctttatcaccataaaccttgatgatctggccttctttaaagggaagctcctcctctgcagcatctgggtttggggacatggtgagcgggtcgtagtcaaagagagccacaaagatccgggccgggagctcttcggcaccagggtcagtttctgactcttcatagaagtctggagaaaggcggtctcgcccgtaatcgtcgatggatgggactgtcacgggccgggacctctgaggaccagcgctgccacggggaaacctccggcccatgtgatccacccgtcctgcagaggctgggttccctaaaatcagggggccttgtgcgactctgggaggtggctttgcgtggggggcagctgccctactgtcgggcatggttatgcttttcttccagacaccccgaaaatcttggtgctcggtgggctcgccccagccgtgcttcctggggggcggcctctccgggccgggctgggggtcgtcgttcctgaggaggccaccagggcccacctgctccccaaagtcctcctccacgctgctctgccgggtcagcgtccgccgccgggccagcagcggcctcgggcccctcctgcagggacagtgaccagggcctgggctgcacgcggccacggtgtttccgaagccaaaccgcgactcgtcctcttcactcccacagtccaggccgctgtccgggctccgggtggccgagcggctgaaccgacagcccctgtcttccagaaggaagtcctccacgtgggggacggcccccgagcccctgtgcttcaccgggaaccaggagccccgaggggcctcgtcgcccctgtagggcctgccgggcctgggctctctggccagccccgtcctggccctgggggacggccctgcaccctgcttgtgtagcagcccacagcactctccgtcctcttccgctacttcggggatactgaaaagtctcttcctgtggggctggtggggaaactcgggctgctcccagaaagtgccttccgaggtcctatggtcagtgcagtccttgagggcattgtgggacgtgccgctgggccgcctccttcccccatcttccagctgcatttcagaatacagctcctcctcgtcctcctccatgatgtctgagaggtcagacccccggctgctctctgtgtggtactcgtctccatggcaacagtgcggctgcttgccaagttcagagcctttcaggaagtcgtccaccgaggcgcccctcctcttgaagtctggagagtcataggcgtcctcctcgtctgaggcggcgtactgccccgcgctgcttctctctaggaagacgctccttttctctaacctgctgctctcggccaccctctgcgcggcctcccgggccatggccttggcgacggtggtggacaccggggtgccctgtggctgtggcaggatgcggctgggtgagggcgaccgccttccggggcccacgggcggctccagcatgtgcccatgcacagggccaggtgcacggctctgctcccaggcctcatccatcctggcgtggggacccaggtgctcgtctttggtttcggggactccagaacttgctaatggctttgattggggtgcaggtctcgggtggggggtaggaggcaccaggagctcggggggaacggcagcaactgcagagtccacggactcgccctgggcggagagggtccgcacggtcacgcccttggcctccaggctccgcagccgcacaagctccacggccgtgctgtctgccgtggggaagatgacttcagccaccctctgccctttggcatacacgccgtagccggtaacgtttgcgccattggacagcccggtgggcgtcagcacaggtggtctccaggagacccggatggtggcgggggtcaccccagcctggacggtaacatcttgtgggggtgctgggggtcctgcaggcaacgtggagaactccacaaaggcctccttcttctccctttgctccagcgggagctgccacggcatctggtggggtttggccagaaccttcaccttataggccatgttgggcctgagattgaagaactggtacttgtacctggcggccttgacgatgtcgaactcctcctcgttgaggaagatgacgtggctgtagttgctgttggtgggtagccaggagagctgggcggagatctgcgtgatgttgtccacccgcaggtgggagggggccaccaccacgtccttgcccaccagcagcgtgcactgcagctcatccgagctgcccctgctggtgacgcactgcacggagatgcggtaggtgcaggctgccatgttgagcttctcgatgagggctttagttctgctccccagcgtgaggttcatgcgtgtctccttgtccaccaggacgttgtagctgctcaccgttccccatcctggtggcaccgccgggggctcccagcccacaataacacttttggcgagttgtttgatgagggtgatttttctagggtaaggcacgatgtcttctccgatgtcgtcgatgttcacgtccagggtcccggcactgttgtcggtgatgcccgcatctatgtgggttggggagtggaggtccaggatgtgctctccctccaggccgatgccggaatggttgatgaagttctgatcctgctcgttccccagcgtgcttgccaaccgcgactcgttgtcctgcacaaagtccacgaagttggagggcaccagacccctctggccatcgaggagctctccttcatagaacccatcctcatccatgtctccatagacgtagaggtattttcccgccgtgaggggcagctcagcttcggggttctcgttcggtccatcgaaggggttgtaactatagcgggcaacacagaggtggaccttccccgagtatctctgcttggaggtattggaattccgttcattctccatgtctgactcagatctgcatcttgcgctaccggatctcgacaggaaggtgggcttggcggacagaggctccggcctgtcaccaggctgcggaaggggccggatatattcaccgatcgcagagctgcctccaatagcgctctcctgacctttgccgagggaggtggctaggccattcatgaactgtgggaaaggcttgctgggggccgtggagatgtccaggggggccaccgcgctgccacccagcaggtcaatcttgccagcgtgctgccggaacttctccaggtcccgggacagcaggttgaactgctcactttgagtccggcatttctcttccagctctcgaaccttggactctagcagccgcactgcgccttcatgctccttcttagcctcaacctgagccttctgcagaaggtcaatttcctgctgcttggcactgagaacagccagggcctggtcatgctccaactgcagctgctgccgccgttcagccgcctctcgcatatgcttcaggacctgttctaggttctccagcttggcttggagctggtgtttctccttcacggccaaatcgcgctctctggtcacgagggtgagcggatggttgagatgcacatactctgccttcaccttgtcatgctgccgggcccttgtgggaaggcctgcatgatgggatctcaggagatactctccctgggtggcatccttcagttcattttccacaaagtttctctgctgagttcctggtctcaggagaggaagtgggaaatttccccagcggtctcccaaagcttgggtctgatcgaatgtggcctcagcacctgcaggcttcaggtgtggcgggtcatttccaagctctgtccccattagactgtcactccaggaggggagggaccctgcttatcgtattctaagcacccaggagagcatccggccaaaggagctactgaaacacttgttgagatgccaaatgaatgaagtcttcaacctctctgttgccttcccatatgtagcagtgaggataggctggactctgctgtggttacaaataattctgattacagtggcttaagatcacctgggtgcattggtggcacctgccctgtgtctgcagctctgctccaaatcatccccacctgggacccaagctgacagaatggccaccacccaggtcactgcacatcagcaggaaggagaagctcgaggggatactgctg

SEQ ID NO: 10114 - RNA, 5020 nt, Homo sapiens
  source 1..5020: mol_type = other RNA
cacgctcatgcacacacccacacagagcttaaccacacatggatttcctttaataataaatctaccacatactattatattacaatttataatagcgtttttgaagacacaatggggaaagctttgtcattcatttataaaccgtccataaattacaaaagaaaggcagtctgaaaagtatgtataaagagtaaaaacaatttacaagtggacaagaattacaaaagagtaaccatcaaatacatctgccagcaactttgtaagtaagtcttttgttcaaatgccaatgatgaagatgggtatggactcatttggagcagatttaaattgagtctggttttggtgtggcttatgcattatgtggattacttgtgtgccattcattgctgtgtatttgggtatggcattttgacaacgaaagtaacagaaaaccatatgccacagaatagaacattaaaagcaatgaagataatcggctttctggaaggttggagtactggtgctttaccaaacaaagttactttctctccttttctcttttttgaatgattgagtaaacattttctgtgtgtagcctggctggctttgaaagactgaaactagtatcttaaaatgcacagcctgtacaacttgatctcaaaccactgtgtcaggatgaagaccactgaatgcacgacacatacaaagtatacactgtttttattagacagtacaaatcattgtgcatttataaggcagaacatcaaggcgaattaaactaggaatttcaagaccagagtcaaagtgaaagttatgcattatgaggcaagcattttgagaagggagaaaggttgaaaatcattcctttaagggcagatgacaaatgcacaaagactggaattacaggtagggagggagctacaggtgatagctatgcgcccccgtttgttaataagacgtcccctcccacctcccaaatcagagcttggacaatgagagcagactgccagcggtgacagagagcaaccgctcctctttgttctcgtggttggtttaaagtggttggtagtgcaaaagtgcatttctctactggtgtcaggggagaagattgggtttttttaggaagtacttgagtcatgaaagcccctttttgcctttgagcgcattggcgtatcttgagagtagtgggatggagcatcagaaagatagacttctacgtcatcaggcacttcttccaagaagtttgagggcacaaggcctttctgcccattcagctccccataataaaatccatcttcatcaatttcaccaaaaactgtaataatatctcctgtgcaaaatgtaagttcggcctcgacatcgacgttgggcgagctttctctggggtcgtagtcatacagggccaccattctccgcgtcgataccgaatgacgcctgccacttctcctgcttctctctattttctccacaggtgtattcagagggagaaagccctgtctaagaagctgatccatcatctcctcatcatctgcttgtatctcagagaccatgttacaaggaataaggccaagccgggcacaggtttccccacggtagaatccatcagcgtctttatcaccataaaccttgatgatctggccttctttaaagggaagctcctcctctgcagcatctgggtttggggacatggtgagcgggtcgtagtcaaagagagccacaaagatccgggccgggagctcttcggcaccagggtcagtttctgactcttcatagaagtctggagaaaggcggtctcgcccgtaatcgtcgatggatgggactgtcacgggccgggacctctgaggaccagcgctgccacggggaaacctccggcccatgtgatccacccgtcctgcagaggctgggttccctaaaatcttgagggcattgtgggacgtgccgctgggccgcctccttcccccatcttccagctgcatttcagaatacagctcctcctcgtcctcctccatgatgtctgagaggtcagacccccggctgctctctgtgtggtactcgtctccatggcaacagtgcggctgcttgccaagttcagagcctttcaggaagtcgtccaccgaggcgcccctcctcttgaagtctggagagtcataggcgtcctcctcgtctgaggcggcgtactgccccgcgctgcttctctctaggaagacgctccttttctctaacctgctgctctcggccaccctctgcgcggcctcccgggccatggccttggcgacggtggtggacaccggggtgccctgtggctgtggcaggatgcggctgggtgagggcgaccgccttccggggcccacgggcggctccagcatgtgcccatgcacagggccaggtgcacggctctgctcccaggcctcatccatcctggcgtggggacccaggtgctcgtctttggtttcggggactccagaacttgctaatggctttgattggggtgcaggtctcgggtggggggtaggaggcaccaggagctcggggggaacggcagcaactgcagagtccacggactcgccctgggcggagagggtccgcacggtcacgcccttggcctccaggctccgcagccgcacaagctccacggccgtgctgtctgccgtggggaagatgacttcagccaccctctgccctttggcatacacgccgtagccggtaacgtttgcgccattggacagcccggtgggcgtcagcacaggtggtctccaggagacccggatggtggcgggggtcaccccagcctggacggtaacatcttgtgggggtgctgggggtcctgcaggcaacgtggagaactccacaaaggcctccttcttctccctttgctccagcgggagctgccacggcatctggtggggtttggccagaaccttcaccttataggccatgttgggcctgagattgaagaactggtacttgtacctggcggccttgacgatgtcgaactcctcctcgttgaggaagatgacgtggctgtagttgctgttggtgggtagccaggagagctgggcggagatctgcgtgatgttgtccacccgcaggtgggagggggccaccaccacgtccttgcccaccagcagcgtgcactgcagctcatccgagctgcccctgctggtgacgcactgcacggagatgcggtaggtgcaggctgccatgttgagcttctcgatgagggctttagttctgctccccagcgtgaggttcatgcgtgtctccttgtccaccaggacgttgtagctgctcaccgttccccatcctggtggcaccgccgggggctcccagcccacaataacacttttggcgagttgtttgatgagggtgatttttctagggtaaggcacgatgtcttctccgatgtcgtcgatgttcacgtccagggtcccggcactgttgtcggtgatgcccgcatctatgtgggttggggagtggaggtccaggatgtgctctccctccaggccgatgccggaatggttgatgaagttctgatcctgctcgttccccagcgtgcttgccaaccgcgactcgttgtcctgcacaaagtccacgaagttggagggcaccagacccctctggccatcgaggagctctccttcatagaacccatcctcatccatgtctccatagacgtagaggtattttcccgccgtgaggggcagctcagcttcggggttctcgttcggtccatcgaaggggttgtaactatagcgggcaacacagaggtggaccttccccgagtatctctgcttggaggtattggaattccgttcattctccatgtctgactcagatctgcatcttgcgctaccggatctcgacaggaaggtgggcttggcggacagaggctccggcctgtcaccaggctgcggaaggggccggatatattcaccgatcgcagagctgcctccaatagcgctctcctgacctttgccgagggaggtggctaggccattcatgaactgtgggaaaggcttgctgggggccgtggagatgtccaggggggccaccgcgctgccacccagcaggtcaatcttgccagcgtgctgccggaacttctccaggtcccgggacagcaggttgaactgctcactttgagtccggcatttctcttccagctctcgaaccttggactctagcagccgcactgcgccttcatgctccttcttagcctcaacctgagccttctgcagaaggtcaatttcctgctgcttggcactgagaacagccagggcctggtcatgctccaactgcagctgctgccgccgttcagccgcctctcgcatatgcttcaggacctgttctaggttctccagcttggcttggagctggtgtttctccttcacggccaaatcgcgctctctggtcacgagggtgagcggatggttgagatgcacatactctgccttcaccttgtcatgctgccgggcccttgtgggaaggcctgcatgatgggatctcaggagatactctccctgggtggcatccttcagttcattttccacaaagtttctctgctgagttcctggtctcaggagaggaagtgggaaatttccccagcggtctcccaaagcttgggtctgatcgaatgtggcctcagcacctgcaggcttcaggtgtggcgggtcatttccaagctctgtccccattagactgtcactccaggaggggagggaccctgcttatcgtattctaagcacccaggagagcatccggccaaaggagctactgaaacacttgttgagatgccaaatgaatgaagtcttcaacctctctgttgccttcccatatgtagcagtgaggataggctggactctgctgtggttacaaataattctgattacagtggcttaagatcacctgggtgcattggtggcacctgccctgtgtctgcagctctgctccaaatcatccccacctgggacccaagctgacagaatggccaccacccaggtcactgcacatcagcaggaaggagaagctcgaggggatactgctg

SEQ ID NO: 10115 - RNA, 4736 nt, Homo sapiens
  source 1..4736: mol_type = other RNA
cacgctcatgcacacacccacacagagcttaaccacacatggatttcctttaataataaatctaccacatactattatattacaatttataatagcgtttttgaagacacaatggggaaagctttgtcattcatttataaaccgtccataaattacaaaagaaaggcagtctgaaaagtatgtataaagagtaaaaacaatttacaagtggacaagaattacaaaagagtaaccatcaaatacatctgccagcaactttgtaagtaagtcttttgttcaaatgccaatgatgaagatgggtatggactcatttggagcagatttaaattgagtctggttttggtgtggcttatgcattatgtggattacttgtgtgccattcattgctgtgtatttgggtatggcattttgacaacgaaagtaacagaaaaccatatgccacagaatagaacattaaaagcaatgaagataatcggctttctggaaggttggagtactggtgctttaccaaacaaagttactttctctccttttctcttttttgaatgattgagtaaacattttctgtgtgtagcctggctggctttgaaagactgaaactagtatcttaaaatgcacagcctgtacaacttgatctcaaaccactgtgtcaggatgaagaccactgaatgcacgacacatacaaagtatacactgtttttattagacagtacaaatcattgtgcatttataaggcagaacatcaaggcgaattaaactaggaatttcaagaccagagtcaaagtgaaagttatgcattatgaggcaagcattttgagaagggagaaaggttgaaaatcattcctttaagggcagatgacaaatgcacaaagactggaattacaggtagggagggagctacaggtgatagctatgcgcccccgtttgttaataagacgtcccctcccacctcccaaatcagagcttggacaatgagagcagactgccagcggtgacagagagcaaccgctcctctttgttctcgtggttggtttaaagtggttggtagtgcaaaagtgcatttctctactggtgtcaggggagaagattgggtttttttaggaagtacttgagtcatgaaagcccctttttgcctttgagcgcattggcgtatcttgagagtagtgggatggagcatcagaaagatagacttctacgtcatcaggcacttcttccaagaagtttgagggcacaaggcctttctgcccattcagctccccataataaaatccatcttcatcaatttcaccaaaaactgtaataatatctcctgtgcaaaatgtaagttcggcctcgacatcgacgttgggcgagctttctctggggtcgtagtcatacagggccaccattctccgcgtcgataccgaatgacgcctgccacttctcctgcttctctctattttctccacaggtgtattcagagggagaaagccctgtctaagaagctgatccatcatctcctcatcatctgcttgtatctcagagaccatgttacaaggaataaggccaagccgggcacaggtttccccacggtagaatccatcagcgtctttatcaccataaaccttgatgatctggccttctttaaagggaagctcctcctctgcagcatctgggtttggggacatggtgagcgggtcgtagtcaaagagagccacaaagatccgggccgggagctcttcggcaccagggtcagtttctgactcttcatagaagtctggagaaaggcggtctcgcccgtaatcgtcgatggatgggactgtcacgggccgggacctctgaggaccagcgctgccacggggaaacctccggcccatgtgatccacccgtcctgcagaggctgggttccctaaaatcttgagggcattgtgggacgtgccgctgggccgcctccttcccccatcttccagctgcatttcagaatacagctcctcctcgtcctcctccatgatgtctgagaggtcagacccccggctgctctctgtgtggtactcgtctccatggcaacagtgcggctgcttgccaagttcagagcctttcaggaagtcgtccaccgaggcgcccctcctcttgaagtctggagagtcataggcgtcctcctcgtctgaggcggcgtactgccccgcgctgcttctctctaggaagacgctccttttctctaacctgctgctctcggccaccctctgcgcggcctcccgggccatggccttggcgacggtggtggacaccggggtgccctgtggctgtggcaggatgcggctgggtgagggcgaccgccttccggggcccacgggcggctccagcatgtgcccatgcacagggccaggtgcacggctctgctcccaggcctcatccatcctggcgtggggacccaggtgctcgtctttggtttcggggactccagaacttgctaatggctttgattggggtgcaggtctcgggtggggggtaggaggcaccaggagctcggggggaacggcagcaactgcagagtccacggactcgccctgggcggagagggtccgcacggtcacgcccttggcctccaggctccgcagccgcacaagctccacggccgtgctgtctgccgtggggaagatgacttcagccaccctctgccctttggcatacacgccgtagccggtaacgtttgcgccattggacagcccggtgggcgtcagcacaggtggtctccaggagacccggatggtggcgggggtcaccccagcctggacggtaacatcttgtgggggtgctgggggtcctgcaggcaacgtggagaactccacaaaggcctccttcttctccctttgctccagcgggagctgccacggcatctggtggggtttggccagaaccttcaccttataggccatgttgggcctgagattgaagaactggtacttgtacctggcggccttgacgatgtcgaactcctcctcgttgaggaagatgacgtggctgtagttgctgttggtgggtagccaggagagctgggcggagatctgcgtgatgttgtccacccgcaggtgggagggggccaccaccacgtccttgcccaccagcagcgtgcactgcagctcatccgagctgcccctgctggtgacgcactgcacggagatgcggtaggtgcaggctgccatgttgagcttctcgatgagggctttagttctgctccccagcgtgaggttcatgcgtgtctccttgtccaccaggacgttgtagctgctcaccgttccccatcctggtggcaccgccgggggctcccagcccacaataacacttttggcgagttgtttgatgagggtgatttttctagggtaaggcacgatgtcttctccgatgtcgtcgatgttcacgtccagggtcccggcactgttgtcggtgatgcccgcatctatgtgggttggggagtggaggtccaggatgtgctctccctccaggccgatgccggaatggttgatgaagttctgatcctgctcgttccccagcgtgcttgccaaccgcgactcgttgtcctgcacaaagtccacgaagttggagggcaccagacccctctggccatcgaggagctctccttcatagaacccatcctcatccatgtctccatagacgtagaggtattttcccgccgtgaggggcagctcagcttcggggttctcgttcggtccatcgaaggggttgtaactatagcgggcaacacagaggtggaccttccccgagtatctctgcttggaggtattggaattccgttcattctccatgtctgactcagatctgcatcttgcgctaccggatctcgacaggaaggtgggcttggcggacagaggctccggcctgtcaccaggctgcggaaggggccggatatattcaccgatcgcagagctgcctccaatagcgctctcctgacctttgccgagggaggtggctaggccattcatgaactgtgggaaaggcttgctgggggccgtggagatgtccaggggggccaccgcgctgccacccagcaggtcaatcttgccagcgtgctgccggaacttctccaggtcccgggacagcaggttgaactgctcactttgagtccggcatttctcttccagctctcgaaccttggactctagcagccgcactgcgccttcatgctccttcttagcctcaacctgagccttctgcagaaggtcaatttcctgctgcttggcactgagaacagccagggcctggtcatgctccaactgcagctgctgccgccgttcagccgcctctcgcatatgcttcaggacctgttctaggttctccagcttggcttggagctggtgtttctccttcacggccaaatcgcgctctctggtcacgagggtgagcggatggttgagatgcacatactctgccttcaccttgtcatgctgccgggcccttgtgggaaggcctgcatgatgggatctcaggagatactctccctgggtggcatccttcagttcattttccacaaagtttctctgctgagttcctggtctcaggagaggaagtgggaaatttccccagcggtctcccaaagcttgggtctgatcgaatgtggcctcagcacctgcaggcttcaggtgtggcgggtcatttccaagctttagaagcgagctgtgccaaggctccggaggttcacctcggagacaactgcagtgtactgtgtcagattacaaact

SEQ ID NO: 10116 - RNA, 5484 nt, Homo sapiens
  source 1..5484: mol_type = other RNA
cacgctcatgcacacacccacacagagcttaaccacacatggatttcctttaataataaatctaccacatactattatattacaatttataatagcgtttttgaagacacaatggggaaagctttgtcattcatttataaaccgtccataaattacaaaagaaaggcagtctgaaaagtatgtataaagagtaaaaacaatttacaagtggacaagaattacaaaagagtaaccatcaaatacatctgccagcaactttgtaagtaagtcttttgttcaaatgccaatgatgaagatgggtatggactcatttggagcagatttaaattgagtctggttttggtgtggcttatgcattatgtggattacttgtgtgccattcattgctgtgtatttgggtatggcattttgacaacgaaagtaacagaaaaccatatgccacagaatagaacattaaaagcaatgaagataatcggctttctggaaggttggagtactggtgctttaccaaacaaagttactttctctccttttctcttttttgaatgattgagtaaacattttctgtgtgtagcctggctggctttgaaagactgaaactagtatcttaaaatgcacagcctgtacaacttgatctcaaaccactgtgtcaggatgaagaccactgaatgcacgacacatacaaagtatacactgtttttattagacagtacaaatcattgtgcatttataaggcagaacatcaaggcgaattaaactaggaatttcaagaccagagtcaaagtgaaagttatgcattatgaggcaagcattttgagaagggagaaaggttgaaaatcattcctttaagggcagatgacaaatgcacaaagactggaattacaggtagggagggagctacaggtgatagctatgcgcccccgtttgttaataagacgtcccctcccacctcccaaatcagagcttggacaatgagagcagactgccagcggtgacagagagcaaccgctcctctttgttctcgtggttggtttaaagtggttggtagtgcaaaagtgcatttctctactggtgtcaggggagaagattgggtttttttaggaagtacttgagtcatgaaagccctagtttggaattaaagaaaattacatagatttggcagttgtccggaagcacatgaatcatttcactgcacccagctttttcagcagtttcttgcctttggaaagcagcccctttttctttttcgaggacatttccctgcctctcccaggactaccagaacccatagatgacgtaggtgaccccgaatggagatggactgtgggggatggagctctccttgctgtacctgaaccctcaggaggaaccctttttgcctttgagcgcattggcgtatcttgagagtagtgggatggagcatcagaaagatagacttctacgtcatcaggcacttcttccaagaagtttgagggcacaaggcctttctgcccattcagctccccataataaaatccatcttcatcaatttcaccaaaaactgtaataatatctcctgtgcaaaatgtaagttcggcctcgacatcgacgttgggcgagctttctctggggtcgtagtcatacagggccaccattctccgcgtcgataccgaatgacgcctgccacttctcctgcttctctctattttctccacaggtgtattcagagggagaaagccctgtctaagaagctgatccatcatctcctcatcatctgcttgtatctcagagaccatgttacaaggaataaggccaagccgggcacaggtttccccacggtagaatccatcagcgtctttatcaccataaaccttgatgatctggccttctttaaagggaagctcctcctctgcagcatctgggtttggggacatggtgagcgggtcgtagtcaaagagagccacaaagatccgggccgggagctcttcggcaccagggtcagtttctgactcttcatagaagtctggagaaaggcggtctcgcccgtaatcgtcgatggatgggactgtcacgggccgggacctctgaggaccagcgctgccacggggaaacctccggcccatgtgatccacccgtcctgcagaggctgggttccctaaaatcagggggccttgtgcgactctgggaggtggctttgcgtggggggcagctgccctactgtcgggcatggttatgcttttcttccagacaccccgaaaatcttggtgctcggtgggctcgccccagccgtgcttcctggggggcggcctctccgggccgggctgggggtcgtcgttcctgaggaggccaccagggcccacctgctccccaaagtcctcctccacgctgctctgccgggtcagcgtccgccgccgggccagcagcggcctcgggcccctcctgcagggacagtgaccagggcctgggctgcacgcggccacggtgtttccgaagccaaaccgcgactcgtcctcttcactcccacagtccaggccgctgtccgggctccgggtggccgagcggctgaaccgacagcccctgtcttccagaaggaagtcctccacgtgggggacggcccccgagcccctgtgcttcaccgggaaccaggagccccgaggggcctcgtcgcccctgtagggcctgccgggcctgggctctctggccagccccgtcctggccctgggggacggccctgcaccctgcttgtgtagcagcccacagcactctccgtcctcttccgctacttcggggatactgaaaagtctcttcctgtggggctggtggggaaactcgggctgctcccagaaagtgccttccgaggtcctatggtcagtgcagtccttgagggcattgtgggacgtgccgctgggccgcctccttcccccatcttccagctgcatttcagaatacagctcctcctcgtcctcctccatgatgtctgagaggtcagacccccggctgctctctgtgtggtactcgtctccatggcaacagtgcggctgcttgccaagttcagagcctttcaggaagtcgtccaccgaggcgcccctcctcttgaagtctggagagtcataggcgtcctcctcgtctgaggcggcgtactgccccgcgctgcttctctctaggaagacgctccttttctctaacctgctgctctcggccaccctctgcgcggcctcccgggccatggccttggcgacggtggtggacaccggggtgccctgtggctgtggcaggatgcggctgggtgagggcgaccgccttccggggcccacgggcggctccagcatgtgcccatgcacagggccaggtgcacggctctgctcccaggcctcatccatcctggcgtggggacccaggtgctcgtctttggtttcggggactccagaacttgctaatggctttgattggggtgcaggtctcgggtggggggtaggaggcaccaggagctcggggggaacggcagcaactgcagagtccacggactcgccctgggcggagagggtccgcacggtcacgcccttggcctccaggctccgcagccgcacaagctccacggccgtgctgtctgccgtggggaagatgacttcagccaccctctgccctttggcatacacgccgtagccggtaacgtttgcgccattggacagcccggtgggcgtcagcacaggtggtctccaggagacccggatggtggcgggggtcaccccagcctggacggtaacatcttgtgggggtgctgggggtcctgcaggcaacgtggagaactccacaaaggcctccttcttctccctttgctccagcgggagctgccacggcatctggtggggtttggccagaaccttcaccttataggccatgttgggcctgagattgaagaactggtacttgtacctggcggccttgacgatgtcgaactcctcctcgttgaggaagatgacgtggctgtagttgctgttggtgggtagccaggagagctgggcggagatctgcgtgatgttgtccacccgcaggtgggagggggccaccaccacgtccttgcccaccagcagcgtgcactgcagctcatccgagctgcccctgctggtgacgcactgcacggagatgcggtaggtgcaggctgccatgttgagcttctcgatgagggctttagttctgctccccagcgtgaggttcatgcgtgtctccttgtccaccaggacgttgtagctgctcaccgttccccatcctggtggcaccgccgggggctcccagcccacaataacacttttggcgagttgtttgatgagggtgatttttctagggtaaggcacgatgtcttctccgatgtcgtcgatgttcacgtccagggtcccggcactgttgtcggtgatgcccgcatctatgtgggttggggagtggaggtccaggatgtgctctccctccaggccgatgccggaatggttgatgaagttctgatcctgctcgttccccagcgtgcttgccaaccgcgactcgttgtcctgcacaaagtccacgaagttggagggcaccagacccctctggccatcgaggagctctccttcatagaacccatcctcatccatgtctccatagacgtagaggtattttcccgccgtgaggggcagctcagcttcggggttctcgttcggtccatcgaaggggttgtaactatagcgggcaacacagaggtggaccttccccgagtatctctgcttggaggtattggaattccgttcattctccatgtctgactcagatctgcatcttgcgctaccggatctcgacaggaaggtgggcttggcggacagaggctccggcctgtcaccaggctgcggaaggggccggatatattcaccgatcgcagagctgcctccaatagcgctctcctgacctttgccgagggaggtggctaggccattcatgaactgtgggaaaggcttgctgggggccgtggagatgtccaggggggccaccgcgctgccacccagcaggtcaatcttgccagcgtgctgccggaacttctccaggtcccgggacagcaggttgaactgctcactttgagtccggcatttctcttccagctctcgaaccttggactctagcagccgcactgcgccttcatgctccttcttagcctcaacctgagccttctgcagaaggtcaatttcctgctgcttggcactgagaacagccagggcctggtcatgctccaactgcagctgctgccgccgttcagccgcctctcgcatatgcttcaggacctgttctaggttctccagcttggcttggagctggtgtttctccttcacggccaaatcgcgctctctggtcacgagggtgagcggatggttgagatgcacatactctgccttcaccacaaagtttctctgctgagttcctggtctcaggagaggaagtgggaaatttccccagcggtctcccaaagcttgggtctgatcgaat

SEQ ID NO: 10117 - RNA, 5959 nt, Homo sapiens
  source 1..5959: mol_type = other RNA
cacgctcatgcacacacccacacagagcttaaccacacatggatttcctttaataataaatctaccacatactattatattacaatttataatagcgtttttgaagacacaatggggaaagctttgtcattcatttataaaccgtccataaattacaaaagaaaggcagtctgaaaagtatgtataaagagtaaaaacaatttacaagtggacaagaattacaaaagagtaaccatcaaatacatctgccagcaactttgtaagtaagtcttttgttcaaatgccaatgatgaagatgggtatggactcatttggagcagatttaaattgagtctggttttggtgtggcttatgcattatgtggattacttgtgtgccattcattgctgtgtatttgggtatggcattttgacaacgaaagtaacagaaaaccatatgccacagaatagaacattaaaagcaatgaagataatcggctttctggaaggttggagtactggtgctttaccaaacaaagttactttctctccttttctcttttttgaatgattgagtaaacattttctgtgtgtagcctggctggctttgaaagactgaaactagtatcttaaaatgcacagcctgtacaacttgatctcaaaccactgtgtcaggatgaagaccactgaatgcacgacacatacaaagtatacactgtttttattagacagtacaaatcattgtgcatttataaggcagaacatcaaggcgaattaaactaggaatttcaagaccagagtcaaagtgaaagttatgcattatgaggcaagcattttgagaagggagaaaggttgaaaatcattcctttaagggcagatgacaaatgcacaaagactggaattacaggtagggagggagctacaggtgatagctatgcgcccccgtttgttaataagacgtcccctcccacctcccaaatcagagcttggacaatgagagcagactgccagcggtgacagagagcaaccgctcctctttgttctcgtggttggtttaaagtggttggtagtgcaaaagtgcatttctctactggtgtcaggggagaagattgggtttttttaggaagtacttgagtcatgaaagccctagtttggaattaaagaaaattacatagatttggcagttgtccggaagcacatgaatcatttcactgcacccagctttttcagcagtttcttgcctttggaaagcagcccctttttctttttcgaggacatttccctgcctctcccaggactaccagaacccatagatgacgtaggtgaccccgaatggagatggactgtgggggatggagctctccttgctgtacctgaaccctcaggaggaaccctttttgcctttgagcgcattggcgtatcttgagagtagtgggatggagcatcagaaagatagacttctacgtcatcaggcacttcttccaagaagtttgagggcacaaggcctttctgcccattcagctccccataataaaatccatcttcatcaatttcaccaaaaactgtaataatatctcctgtgcaaaatgtaagttcggcctcgacatcgacgttgggcgagctttctctggggtcgtagtcatacagggccaccattctccgcgtcgataccgaatgacgcctgccacttctcctgcttctctctattttctccacaggtgtattcagagggagaaagccctgtctaagaagctgatccatcatctcctcatcatctgcttgtatctcagagaccatgttacaaggaataaggccaagccgggcacaggtttccccacggtagaatccatcagcgtctttatcaccataaaccttgatgatctggccttctttaaagggaagctcctcctctgcagcatctgggtttggggacatggtgagcgggtcgtagtcaaagagagccacaaagatccgggccgggagctcttcggcaccagggtcagtttctgactcttcatagaagtctggagaaaggcggtctcgcccgtaatcgtcgatggatgggactgtcacgggccgggacctctgaggaccagcgctgccacggggaaacctccggcccatgtgatccacccgtcctgcagaggctgggttccctaaaatcagggggccttgtgcgactctgggaggtggctttgcgtggggggcagctgccctactgtcgggcatggttatgcttttcttccagacaccccgaaaatcttggtgctcggtgggctcgccccagccgtgcttcctggggggcggcctctccgggccgggctgggggtcgtcgttcctgaggaggccaccagggcccacctgctccccaaagtcctcctccacgctgctctgccgggtcagcgtccgccgccgggccagcagcggcctcgggcccctcctgcagggacagtgaccagggcctgggctgcacgcggccacggtgtttccgaagccaaaccgcgactcgtcctcttcactcccacagtccaggccgctgtccgggctccgggtggccgagcggctgaaccgacagcccctgtcttccagaaggaagtcctccacgtgggggacggcccccgagcccctgtgcttcaccgggaaccaggagccccgaggggcctcgtcgcccctgtagggcctgccgggcctgggctctctggccagccccgtcctggccctgggggacggccctgcaccctgcttgtgtagcagcccacagcactctccgtcctcttccgctacttcggggatactgaaaagtctcttcctgtggggctggtggggaaactcgggctgctcccagaaagtgccttccgaggtcctatggtcagtgcagtccttgagggcattgtgggacgtgccgctgggccgcctccttcccccatcttccagctgcatttcagaatacagctcctcctcgtcctcctccatgatgtctgagaggtcagacccccggctgctctctgtgtggtactcgtctccatggcaacagtgcggctgcttgccaagttcagagcctttcaggaagtcgtccaccgaggcgcccctcctcttgaagtctggagagtcataggcgtcctcctcgtctgaggcggcgtactgccccgcgctgcttctctctaggaagacgctccttttctctaacctgctgctctcggccaccctctgcgcggcctcccgggccatggccttggcgacggtggtggacaccggggtgccctgtggctgtggcaggatgcggctgggtgagggcgaccgccttccggggcccacgggcggctccagcatgtgcccatgcacagggccaggtgcacggctctgctcccaggcctcatccatcctggcgtggggacccaggtgctcgtctttggtttcggggactccagaacttgctaatggctttgattggggtgcaggtctcgggtggggggtaggaggcaccaggagctcggggggaacggcagcaactgcagagtccacggactcgccctgggcggagagggtccgcacggtcacgcccttggcctccaggctccgcagccgcacaagctccacggccgtgctgtctgccgtggggaagatgacttcagccaccctctgccctttggcatacacgccgtagccggtaacgtttgcgccattggacagcccggtgggcgtcagcacaggtggtctccaggagacccggatggtggcgggggtcaccccagcctggacggtaacatcttgtgggggtgctgggggtcctgcaggcaacgtggagaactccacaaaggcctccttcttctccctttgctccagcgggagctgccacggcatctggtggggtttggccagaaccttcaccttataggccatgttgggcctgagattgaagaactggtacttgtacctggcggccttgacgatgtcgaactcctcctcgttgaggaagatgacgtggctgtagttgctgttggtgggtagccaggagagctgggcggagatctgcgtgatgttgtccacccgcaggtgggagggggccaccaccacgtccttgcccaccagcagcgtgcactgcagctcatccgagctgcccctgctggtgacgcactgcacggagatgcggtaggtgcaggctgccatgttgagcttctcgatgagggctttagttctgctccccagcgtgaggttcatgcgtgtctccttgtccaccaggacgttgtagctgctcaccgttccccatcctggtggcaccgccgggggctcccagcccacaataacacttttggcgagttgtttgatgagggtgatttttctagggtaaggcacgatgtcttctccgatgtcgtcgatgttcacgtccagggtcccggcactgttgtcggtgatgcccgcatctatgtgggttggggagtggaggtccaggatgtgctctccctccaggccgatgccggaatggttgatgaagttctgatcctgctcgttccccagcgtgcttgccaaccgcgactcgttgtcctgcacaaagtccacgaagttggagggcaccagacccctctggccatcgaggagctctccttcatagaacccatcctcatccatgtctccatagacgtagaggtattttcccgccgtgaggggcagctcagcttcggggttctcgttcggtccatcgaaggggttgtaactatagcgggcaacacagaggtggaccttccccgagtatctctgcttggaggtattggaattccgttcattctccatgtctgactcagatctgcatcttgcgctaccggatctcgacaggaaggtgggcttggcggacagaggctccggcctgtcaccaggctgcggaaggggccggatatattcaccgatcgcagagctgcctccaatagcgctctcctgacctttgccgagggaggtggctaggccattcatgaactgtgggaaaggcttgctgggggccgtggagatgtccaggggggccaccgcgctgccacccagcaggtcaatcttgccagcgtgctgccggaacttctccaggtcccgggacagcaggttgaactgctcactttgagtccggcatttctcttccagctctcgaaccttggactctagcagccgcactgcgccttcatgctccttcttagcctcaacctgagccttctgcagaaggtcaatttcctgctgcttggcactgagaacagccagggcctggtcatgctccaactgcagctgctgccgccgttcagccgcctctcgcatatgcttcaggacctgttctaggttctccagcttggcttggagctggtgtttctccttcacggccaaatcgcgctctctggtcacgagggtgagcggatggttgagatgcacatactctgccttcaccttgtcatgctgccgggcccttgtgggaaggcctgcatgatgggatctcaggagatactctccctgggtggcatccttcagttcattttccacaaagtttctctgctgagttcctggtctcaggagaggaagtgggaaatttccccagcggtctcccaaagcttgggtctgatcgaatgtggcctcagcacctgcaggcttcaggtgtggcgggtcatttccaagaaggcaccggagattagtggtctagtggaccagacagactggtccaggcctccccgccggccccccttccggtccccgtggacgccagcctctctgagcctcggatgtttgtgctcggcaccaggctggaaggctatttacttattcatgggctgcccaagccggccaggaactgctttgtgtcagctgaataggatggtaattcaatctgcgaatgggagccgttggcacacagcacgcctgtcataatgagtcacaggggggacaagcacccagcgttcagagccactgggaacctgtccttcgacaacgagctgtgtcacaagacaccaccttcc

SEQ ID NO: 10118 - RNA, 5761 nt, Homo sapiens
  source 1..5761: mol_type = other RNA
cacgctcatgcacacacccacacagagcttaaccacacatggatttcctttaataataaatctaccacatactattatattacaatttataatagcgtttttgaagacacaatggggaaagctttgtcattcatttataaaccgtccataaattacaaaagaaaggcagtctgaaaagtatgtataaagagtaaaaacaatttacaagtggacaagaattacaaaagagtaaccatcaaatacatctgccagcaactttgtaagtaagtcttttgttcaaatgccaatgatgaagatgggtatggactcatttggagcagatttaaattgagtctggttttggtgtggcttatgcattatgtggattacttgtgtgccattcattgctgtgtatttgggtatggcattttgacaacgaaagtaacagaaaaccatatgccacagaatagaacattaaaagcaatgaagataatcggctttctggaaggttggagtactggtgctttaccaaacaaagttactttctctccttttctcttttttgaatgattgagtaaacattttctgtgtgtagcctggctggctttgaaagactgaaactagtatcttaaaatgcacagcctgtacaacttgatctcaaaccactgtgtcaggatgaagaccactgaatgcacgacacatacaaagtatacactgtttttattagacagtacaaatcattgtgcatttataaggcagaacatcaaggcgaattaaactaggaatttcaagaccagagtcaaagtgaaagttatgcattatgaggcaagcattttgagaagggagaaaggttgaaaatcattcctttaagggcagatgacaaatgcacaaagactggaattacaggtagggagggagctacaggtgatagctatgcgcccccgtttgttaataagacgtcccctcccacctcccaaatcagagcttggacaatgagagcagactgccagcggtgacagagagcaaccgctcctctttgttctcgtggttggtttaaagtggttggtagtgcaaaagtgcatttctctactggtgtcaggggagaagattgggtttttttaggaagtacttgagtcatgaaagccctagtttggaattaaagaaaattacatagatttggcagttgtccggaagcacatgaatcatttcactgcacccagctttttcagcagtttcttgcctttggaaagcagcccctttttctttttcgaggacatttccctgcctctcccaggactaccagaacccatagatgacgtaggtgaccccgaatggagatggactgtgggggatggagctctccttgctgtacctgaaccctcaggaggaaccctttttgcctttgagcgcattggcgtatcttgagagtagtgggatggagcatcagaaagatagacttctacgtcatcaggcacttcttccaagaagtttgagggcacaaggcctttctgcccattcagctccccataataaaatccatcttcatcaatttcaccaaaaactgtaataatatctcctgtgcaaaatgtaagttcggcctcgacatcgacgttgggcgagctttctctggggtcgtagtcatacagggccaccattctccgcgtcgataccgaatgacgcctgccacttctcctgcttctctctattttctccacaggtgtattcagagggagaaagccctgtctaagaagctgatccatcatctcctcatcatctgcttgtatctcagagaccatgttacaaggaataaggccaagccgggcacaggtttccccacggtagaatccatcagcgtctttatcaccataaaccttgatgatctggccttctttaaagggaagctcctcctctgcagcatctgggtttggggacatggtgagcgggtcgtagtcaaagagagccacaaagatccgggccgggagctcttcggcaccagggtcagtttctgactcttcatagaagtctggagaaaggcggtctcgcccgtaatcgtcgatggatgggactgtcacgggccgggacctctgaggaccagcgctgccacggggaaacctccggcccatgtgatccacccgtcctgcagaggctgggttccctaaaatcagggggccttgtgcgactctgggaggtggctttgcgtggggggcagctgccctactgtcgggcatggttatgcttttcttccagacaccccgaaaatcttggtgctcggtgggctcgccccagccgtgcttcctggggggcggcctctccgggccgggctgggggtcgtcgttcctgaggaggccaccagggcccacctgctccccaaagtcctcctccacgctgctctgccgggtcagcgtccgccgccgggccagcagcggcctcgggcccctcctgcagggacagtgaccagggcctgggctgcacgcggccacggtgtttccgaagccaaaccgcgactcgtcctcttcactcccacagtccaggccgctgtccgggctccgggtggccgagcggctgaaccgacagcccctgtcttccagaaggaagtcctccacgtgggggacggcccccgagcccctgtgcttcaccgggaaccaggagccccgaggggcctcgtcgcccctgtagggcctgccgggcctgggctctctggccagccccgtcctggccctgggggacggccctgcaccctgcttgtgtagcagcccacagcactctccgtcctcttccgctacttcggggatactgaaaagtctcttcctgtggggctggtggggaaactcgggctgctcccagaaagtgccttccgaggtcctatggtcagtgcagtccttgagggcattgtgggacgtgccgctgggccgcctccttcccccatcttccagctgcatttcagaatacagctcctcctcgtcctcctccatgatgtctgagaggtcagacccccggctgctctctgtgtggtactcgtctccatggcaacagtgcggctgcttgccaagttcagagcctttcaggaagtcgtccaccgaggcgcccctcctcttgaagtctggagagtcataggcgtcctcctcgtctgaggcggcgtactgccccgcgctgcttctctctaggaagacgctccttttctctaacctgctgctctcggccaccctctgcgcggcctcccgggccatggccttggcgacggtggtggacaccggggtgccctgtggctgtggcaggatgcggctgggtgagggcgaccgccttccggggcccacgggcggctccagcatgtgcccatgcacagggccaggtgcacggctctgctcccaggcctcatccatcctggcgtggggacccaggtgctcgtctttggtttcggggactccagaacttgctaatggctttgattggggtgcaggtctcgggtggggggtaggaggcaccaggagctcggggggaacggcagcaactgcagagtccacggactcgccctgggcggagagggtccgcacggtcacgcccttggcctccaggctccgcagccgcacaagctccacggccgtgctgtctgccgtggggaagatgacttcagccaccctctgccctttggcatacacgccgtagccggtaacgtttgcgccattggacagcccggtgggcgtcagcacaggtggtctccaggagacccggatggtggcgggggtcaccccagcctggacggtaacatcttgtgggggtgctgggggtcctgcaggcaacgtggagaactccacaaaggcctccttcttctccctttgctccagcgggagctgccacggcatctggtggggtttggccagaaccttcaccttataggccatgttgggcctgagattgaagaactggtacttgtacctggcggccttgacgatgtcgaactcctcctcgttgaggaagatgacgtggctgtagttgctgttggtgggtagccaggagagctgggcggagatctgcgtgatgttgtccacccgcaggtgggagggggccaccaccacgtccttgcccaccagcagcgtgcactgcagctcatccgagctgcccctgctggtgacgcactgcacggagatgcggtaggtgcaggctgccatgttgagcttctcgatgagggctttagttctgctccccagcgtgaggttcatgcgtgtctccttgtccaccaggacgttgtagctgctcaccgttccccatcctggtggcaccgccgggggctcccagcccacaataacacttttggcgagttgtttgatgagggtgatttttctagggtaaggcacgatgtcttctccgatgtcgtcgatgttcacgtccagggtcccggcactgttgtcggtgatgcccgcatctatgtgggttggggagtggaggtccaggatgtgctctccctccaggccgatgccggaatggttgatgaagttctgatcctgctcgttccccagcgtgcttgccaaccgcgactcgttgtcctgcacaaagtccacgaagttggagggcaccagacccctctggccatcgaggagctctccttcatagaacccatcctcatccatgtctccatagacgtagaggtattttcccgccgtgaggggcagctcagcttcggggttctcgttcggtccatcgaaggggttgtaactatagcgggcaacacagaggtggaccttccccgagtatctctgcttggaggtattggaattccgttcattctccatgtctgactcagatctgcatcttgcgctaccggatctcgacaggaaggtgggcttggcggacagaggctccggcctgtcaccaggctgcggaaggggccggatatattcaccgatcgcagagctgcctccaatagcgctctcctgacctttgccgagggaggtggctaggccattcatgaactgtgggaaaggcttgctgggggccgtggagatgtccaggggggccaccgcgctgccacccagcaggtcaatcttgccagcgtgctgccggaacttctccaggtcccgggacagcaggttgaactgctcactttgagtccggcatttctcttccagctctcgaaccttggactctagcagccgcactgcgccttcatgctccttcttagcctcaacctgagccttctgcagaaggtcaatttcctgctgcttggcactgagaacagccagggcctggtcatgctccaactgcagctgctgccgccgttcagccgcctctcgcatatgcttcaggacctgttctaggttctccagcttggcttggagctggtgtttctccttcacggccaaatcgcgctctctggtcacgagggtgagcggatggttgagatgcacatactctgccttcaccttgtcatgctgccgggcccttgtgggaaggcctgcatgatgggatctcaggagatactctccctgggtggcatccttcagttcattttccacaaagtttctctgctgagttcctggtctcaggagaggaagtgggaaatttccccagcggtctcccaaagcttgggtctgatcgaatgtggcctcagcacctgcaggcttcaggtgtggcgggtcatttccaagctttagaagcgagctgtgccaaggctccggaggttcacctcggagacaactgcagtgtactgtgtcagattacaaactgggggcgagacggagggagggaggagggggagagggagagaaggagggagggaggaggggga

SEQ ID NO: 10119 - RNA, 5107 nt, Homo sapiens
  source 1..5107: mol_type = other RNA
cacgctcatgcacacacccacacagagcttaaccacacatggatttcctttaataataaatctaccacatactattatattacaatttataatagcgtttttgaagacacaatggggaaagctttgtcattcatttataaaccgtccataaattacaaaagaaaggcagtctgaaaagtatgtataaagagtaaaaacaatttacaagtggacaagaattacaaaagagtaaccatcaaatacatctgccagcaactttgtaagtaagtcttttgttcaaatgccaatgatgaagatgggtatggactcatttggagcagatttaaattgagtctggttttggtgtggcttatgcattatgtggattacttgtgtgccattcattgctgtgtatttgggtatggcattttgacaacgaaagtaacagaaaaccatatgccacagaatagaacattaaaagcaatgaagataatcggctttctggaaggttggagtactggtgctttaccaaacaaagttactttctctccttttctcttttttgaatgattgagtaaacattttctgtgtgtagcctggctggctttgaaagactgaaactagtatcttaaaatgcacagcctgtacaacttgatctcaaaccactgtgtcaggatgaagaccactgaatgcacgacacatacaaagtatacactgtttttattagacagtacaaatcattgtgcatttataaggcagaacatcaaggcgaattaaactaggaatttcaagaccagagtcaaagtgaaagttatgcattatgaggcaagcattttgagaagggagaaaggttgaaaatcattcctttaagggcagatgacaaatgcacaaagactggaattacaggtagggagggagctacaggtgatagctatgcgcccccgtttgttaataagacgtcccctcccacctcccaaatcagagcttggacaatgagagcagactgccagcggtgacagagagcaaccgctcctctttgttctcgtggttggtttaaagtggttggtagtgcaaaagtgcatttctctactggtgtcaggggagaagattgggtttttttaggaagtacttgagtcatgaaagccctagtttggaattaaagaaaattacatagatttggcagttgtccggaagcacatgaatcatttcactgcacccagctttttcagcagtttcttgcctttggaaagcagcccctttttctttttcgaggacatttccctgcctctcccaggactaccagaacccatagatgacgtaggtgaccccgaatggagatggactgtgggggatggagctctccttgctgtacctgaaccctcaggaggaaccctttttgcctttgagcgcattggcgtatcttgagagtagtgggatggagcatcagaaagatagacttctacgtcatcaggcacttcttccaagaagtttgagggcacaaggcctttctgcccattcagctccccataataaaatccatcttcatcaatttcaccaaaaactgtaataatatctcctgtgcaaaatgtaagttcggcctcgacatcgacgttgggcgagctttctctggggtcgtagtcatacagggccaccattctccgcgtcgataccgaatgacgcctgccacttctcctgcttctctctattttctccacaggtgtattcagagggagaaagccctgtctaagaagctgatccatcatctcctcatcatctgcttgtatctcagagaccatgttacaaggaataaggccaagccgggcacaggtttccccacggtagaatccatcagcgtctttatcaccataaaccttgatgatctggccttctttaaagggaagctcctcctctgcagcatctgggtttggggacatggtgagcgggtcgtagtcaaagagagccacaaagatccgggccgggagctcttcggcaccagggtcagtttctgactcttcatagaagtctggagaaaggcggtctcgcccgtaatcgtcgatggatgggactgtcacgggccgggacctctgaggaccagcgctgccacggggaaacctccggcccatgtgatccacccgtcctgcagaggctgggttccctaaaatctgcttgccaagttcagagcctttcaggaagtcgtccaccgaggcgcccctcctcttgaagtctggagagtcataggcgtcctcctcgtctgaggcggcgtactgccccgcgctgcttctctctaggaagacgctccttttctctaacctgctgctctcggccaccctctgcgcggcctcccgggccatggccttggcgacggtggtggacaccggggtgccctgtggctgtggcaggatgcggctgggtgagggcgaccgccttccggggcccacgggcggctccagcatgtgcccatgcacagggccaggtgcacggctctgctcccaggcctcatccatcctggcgtggggacccaggtgctcgtctttggtttcggggactccagaacttgctaatggctttgattggggtgcaggtctcgggtggggggtaggaggcaccaggagctcggggggaacggcagcaactgcagagtccacggactcgccctgggcggagagggtccgcacggtcacgcccttggcctccaggctccgcagccgcacaagctccacggccgtgctgtctgccgtggggaagatgacttcagccaccctctgccctttggcatacacgccgtagccggtaacgtttgcgccattggacagcccggtgggcgtcagcacaggtggtctccaggagacccggatggtggcgggggtcaccccagcctggacggtaacatcttgtgggggtgctgggggtcctgcaggcaacgtggagaactccacaaaggcctccttcttctccctttgctccagcgggagctgccacggcatctggtggggtttggccagaaccttcaccttataggccatgttgggcctgagattgaagaactggtacttgtacctggcggccttgacgatgtcgaactcctcctcgttgaggaagatgacgtggctgtagttgctgttggtgggtagccaggagagctgggcggagatctgcgtgatgttgtccacccgcaggtgggagggggccaccaccacgtccttgcccaccagcagcgtgcactgcagctcatccgagctgcccctgctggtgacgcactgcacggagatgcggtaggtgcaggctgccatgttgagcttctcgatgagggctttagttctgctccccagcgtgaggttcatgcgtgtctccttgtccaccaggacgttgtagctgctcaccgttccccatcctggtggcaccgccgggggctcccagcccacaataacacttttggcgagttgtttgatgagggtgatttttctagggtaaggcacgatgtcttctccgatgtcgtcgatgttcacgtccagggtcccggcactgttgtcggtgatgcccgcatctatgtgggttggggagtggaggtccaggatgtgctctccctccaggccgatgccggaatggttgatgaagttctgatcctgctcgttccccagcgtgcttgccaaccgcgactcgttgtcctgcacaaagtccacgaagttggagggcaccagacccctctggccatcgaggagctctccttcatagaacccatcctcatccatgtctccatagacgtagaggtattttcccgccgtgaggggcagctcagcttcggggttctcgttcggtccatcgaaggggttgtaactatagcgggcaacacagaggtggaccttccccgagtatctctgcttggaggtattggaattccgttcattctccatgtctgactcagatctgcatcttgcgctaccggatctcgacaggaaggtgggcttggcggacagaggctccggcctgtcaccaggctgcggaaggggccggatatattcaccgatcgcagagctgcctccaatagcgctctcctgacctttgccgagggaggtggctaggccattcatgaactgtgggaaaggcttgctgggggccgtggagatgtccaggggggccaccgcgctgccacccagcaggtcaatcttgccagcgtgctgccggaacttctccaggtcccgggacagcaggttgaactgctcactttgagtccggcatttctcttccagctctcgaaccttggactctagcagccgcactgcgccttcatgctccttcttagcctcaacctgagccttctgcagaaggtcaatttcctgctgcttggcactgagaacagccagggcctggtcatgctccaactgcagctgctgccgccgttcagccgcctctcgcatatgcttcaggacctgttctaggttctccagcttggcttggagctggtgtttctccttcacggccaaatcgcgctctctggtcacgagggtgagcggatggttgagatgcacatactctgccttcaccttgtcatgctgccgggcccttgtgggaaggcctgcatgatgggatctcaggagatactctccctgggtggcatccttcagttcattttccacaaagtttctctgctgagttcctggtctcaggagaggaagtgggaaatttccccagcggtctcccaaagcttgggtctgatcgaatgtggcctcagcacctgcaggcttcaggtgtggcgggtcatttccaagctctgtccccattagactgtcactccaggaggggagggaccctgcttatcgtattctaagcacccaggagagcatccggccaaaggagctactgaaacacttgttgagatgccaaatgaatgaagtcttcaacctctctgttgccttcccatatgtagcagtgaggataggctggactctgctgtggttacaaataattctgattacagtggcttaagatcacctgggtgcattggtggcacctgccctgtgtctgcagctctgctccaaatcatccccacctgggacccaagctgacagaatggccaccacccaggtcactgcacatcagcaggaaggagaagctcgaggggatactgctg

SEQ ID NO: 10120 - RNA, 4892 nt, Homo sapiens
  source 1..4892: mol_type = other RNA
cacgctcatgcacacacccacacagagcttaaccacacatggatttcctttaataataaatctaccacatactattatattacaatttataatagcgtttttgaagacacaatggggaaagctttgtcattcatttataaaccgtccataaattacaaaagaaaggcagtctgaaaagtatgtataaagagtaaaaacaatttacaagtggacaagaattacaaaagagtaaccatcaaatacatctgccagcaactttgtaagtaagtcttttgttcaaatgccaatgatgaagatgggtatggactcatttggagcagatttaaattgagtctggttttggtgtggcttatgcattatgtggattacttgtgtgccattcattgctgtgtatttgggtatggcattttgacaacgaaagtaacagaaaaccatatgccacagaatagaacattaaaagcaatgaagataatcggctttctggaaggttggagtactggtgctttaccaaacaaagttactttctctccttttctcttttttgaatgattgagtaaacattttctgtgtgtagcctggctggctttgaaagactgaaactagtatcttaaaatgcacagcctgtacaacttgatctcaaaccactgtgtcaggatgaagaccactgaatgcacgacacatacaaagtatacactgtttttattagacagtacaaatcattgtgcatttataaggcagaacatcaaggcgaattaaactaggaatttcaagaccagagtcaaagtgaaagttatgcattatgaggcaagcattttgagaagggagaaaggttgaaaatcattcctttaagggcagatgacaaatgcacaaagactggaattacaggtagggagggagctacaggtgatagctatgcgcccccgtttgttaataagacgtcccctcccacctcccaaatcagagcttggacaatgagagcagactgccagcggtgacagagagcaaccgctcctctttgttctcgtggttggtttaaagtggttggtagtgcaaaagtgcatttctctactggtgtcaggggagaagattgggtttttttaggaagtacttgagtcatgaaagccctagtttggaattaaagaaaattacatagatttggcagttgtccggaagcacatgaatcatttcactgcacccagctttttcagcagtttcttgcctttggaaagcagcccctttttctttttcgaggacatttccctgcctctcccaggactaccagaacccatagatgacgtaggtgaccccgaatggagatggactgtgggggatggagctctccttgctgtacctgaaccctcaggaggaaccctttttgcctttgagcgcattggcgtatcttgagagtagtgggatggagcatcagaaagatagacttctacgtcatcaggcacttcttccaagaagtttgagggcacaaggcctttctgcccattcagctccccataataaaatccatcttcatcaatttcaccaaaaactgtaataatatctcctgtgcaaaatgtaagttcggcctcgacatcgacgttgggcgagctttctctggggtcgtagtcatacagggccaccattctccgcgtcgataccgaatgacgcctgccacttctcctgcttctctctattttctccacaggtgtattcagagggagaaagccctgtctaagaagctgatccatcatctcctcatcatctgcttgtatctcagagaccatgttacaaggaataaggccaagccgggcacaggtttccccacggtagaatccatcagcgtctttatcaccataaaccttgatgatctggccttctttaaagggaagctcctcctctgcagcatctgggtttggggacatggtgagcgggtcgtagtcaaagagagccacaaagatccgggccgggagctcttcggcaccagggtcagtttctgactcttcatagaagtctggagaaaggcggtctcgcccgtaatcgtcgatggatgggactgtcacgggccgggacctctgaggaccagcgctgccacggggaaacctccggcccatgtgatccacccgtcctgcagaggctgggttccctaaaatcttgagggcattgtgggacgtgccgctgggccgcctccttcccccatcttccagctgcatttcagaatacagctcctcctcgtcctcctccatgatgtctgagaggtcagacccccggctgctctctgtgtggtactcgtctccatggcaacagtgcggctgcttgccaagttcagagcctttcaggaagtcgtccaccgaggcgcccctcctcttgaagtctggagagtcataggcgtcctcctcgtctgaggcggcgtactgccccgcgctgcttctctctaggaagacgctccttttctctaacctgctgctctcggccaccctctgcgcggcctcccgggccatggccttggcgacggtggtggacaccggggtgccctgtggctgtggcaggatgcggctgggtgagggcgaccgccttccggggcccacgggcggctccagcatgtgcccatgcacagggccaggtgcacggctctgctcccaggcctcatccatcctggcgtggggacccaggtgctcgtctttggtttcggggactccagaacttgctaatggctttgattggggtgcaggtctcgggtggggggtaggaggcaccaggagctcggggggaacggcagcaactgcagagtccacggactcgccctgggcggagagggtccgcacggtcacgcccttggcctccaggctccgcagccgcacaagctccacggccgtgctgtctgccgtggggaagatgacttcagccaccctctgccctttggcatacacgccgtagccggtaacgtttgcgccattggacagcccggtgggcgtcagcacaggtggtctccaggagacccggatggtggcgggggtcaccccagcctggacggtaacatcttgtgggggtgctgggggtcctgcaggcaacgtggagaactccacaaaggcctccttcttctccctttgctccagcgggagctgccacggcatctggtggggtttggccagaaccttcaccttataggccatgttgggcctgagattgaagaactggtacttgtacctggcggccttgacgatgtcgaactcctcctcgttgaggaagatgacgtggctgtagttgctgttggtgggtagccaggagagctgggcggagatctgcgtgatgttgtccacccgcaggtgggagggggccaccaccacgtccttgcccaccagcagcgtgcactgcagctcatccgagctgcccctgctggtgacgcactgcacggagatgcggtaggtgcaggctgccatgttgagcttctcgatgagggctttagttctgctccccagcgtgaggttcatgcgtgtctccttgtccaccaggacgttgtagctgctcaccgttccccatcctggtggcaccgccgggggctcccagcccacaataacacttttggcgagttgtttgatgagggtgatttttctagggtaaggcacgatgtcttctccgatgtcgtcgatgttcacgtccagggtcccggcactgttgtcggtgatgcccgcatctatgtgggttggggagtggaggtccaggatgtgctctccctccaggccgatgccggaatggttgatgaagttctgatcctgctcgttccccagcgtgcttgccaaccgcgactcgttgtcctgcacaaagtccacgaagttggagggcaccagacccctctggccatcgaggagctctccttcatagaacccatcctcatccatgtctccatagacgtagaggtattttcccgccgtgaggggcagctcagcttcggggttctcgttcggtccatcgaaggggttgtaactatagcgggcaacacagaggtggaccttccccgagtatctctgcttggaggtattggaattccgttcattctccatgtctgactcagatctgcatcttgcgctaccggatctcgacaggaaggtgggcttggcggacagaggctccggcctgtcaccaggctgcggaaggggccggatatattcaccgatcgcagagctgcctccaatagcgctctcctgacctttgccgagggaggtggctaggccattcatgaactgtgggaaaggcttgctgggggccgtggagatgtccaggggggccaccgcgctgccacccagcaggtcaatcttgccagcgtgctgccggaacttctccaggtcccgggacagcaggttgaactgctcactttgagtccggcatttctcttccagctctcgaaccttggactctagcagccgcactgcgccttcatgctccttcttagcctcaacctgagccttctgcagaaggtcaatttcctgctgcttggcactgagaacagccagggcctggtcatgctccaactgcagctgctgccgccgttcagccgcctctcgcatatgcttcaggacctgttctaggttctccagcttggcttggagctggtgtttctccttcacggccaaatcgcgctctctggtcacgagggtgagcggatggttgagatgcacatactctgccttcaccacaaagtttctctgctgagttcctggtctcaggagaggaagtgggaaatttccccagcggtctcccaaagcttgggtctgatcgaatgtggcctcagcacctgcaggcttcaggtgtggcgggtcatttccaagctttagaagcgagctgtgccaaggctccggaggttcacctcggagacaactgcagtgtactgtgtcagattacaaact

SEQ ID NO: 10121 - RNA, 5020 nt, Homo sapiens
  source 1..5020: mol_type = other RNA
cacgctcatgcacacacccacacagagcttaaccacacatggatttcctttaataataaatctaccacatactattatattacaatttataatagcgtttttgaagacacaatggggaaagctttgtcattcatttataaaccgtccataaattacaaaagaaaggcagtctgaaaagtatgtataaagagtaaaaacaatttacaagtggacaagaattacaaaagagtaaccatcaaatacatctgccagcaactttgtaagtaagtcttttgttcaaatgccaatgatgaagatgggtatggactcatttggagcagatttaaattgagtctggttttggtgtggcttatgcattatgtggattacttgtgtgccattcattgctgtgtatttgggtatggcattttgacaacgaaagtaacagaaaaccatatgccacagaatagaacattaaaagcaatgaagataatcggctttctggaaggttggagtactggtgctttaccaaacaaagttactttctctccttttctcttttttgaatgattgagtaaacattttctgtgtgtagcctggctggctttgaaagactgaaactagtatcttaaaatgcacagcctgtacaacttgatctcaaaccactgtgtcaggatgaagaccactgaatgcacgacacatacaaagtatacactgtttttattagacagtacaaatcattgtgcatttataaggcagaacatcaaggcgaattaaactaggaatttcaagaccagagtcaaagtgaaagttatgcattatgaggcaagcattttgagaagggagaaaggttgaaaatcattcctttaagggcagatgacaaatgcacaaagactggaattacaggtagggagggagctacaggtgatagctatgcgcccccgtttgttaataagacgtcccctcccacctcccaaatcagagcttggacaatgagagcagactgccagcggtgacagagagcaaccgctcctctttgttctcgtggttggtttaaagtggttggtagtgcaaaagtgcatttctctactggtgtcaggggagaagattgggtttttttaggaagtacttgagtcatgaaagccctagtttggaattaaagaaaattacatagatttggcagttgtccggaagcacatgaatcatttcactgcacccagctttttcagcagtttcttgcctttggaaagcagcccctttttctttttcgaggacatttccctgcctctcccaggactaccagaacccatagatgacgtaggtgaccccgaatggagatggactgtgggggatggagctctccttgctgtacctgaaccctcaggaggaaccctttttgcctttgagcgcattggcgtatcttgagagtagtgggatggagcatcagaaagatagacttctacgtcatcaggcacttcttccaagaagtttgagggcacaaggcctttctgcccattcagctccccataataaaatccatcttcatcaatttcaccaaaaactgtaataatatctcctgtgcaaaatgtaagttcggcctcgacatcgacgttgggcgagctttctctggggtcgtagtcatacagggccaccattctccgcgtcgataccgaatgacgcctgccacttctcctgcttctctctattttctccacaggtgtattcagagggagaaagccctgtctaagaagctgatccatcatctcctcatcatctgcttgtatctcagagaccatgttacaaggaataaggccaagccgggcacaggtttccccacggtagaatccatcagcgtctttatcaccataaaccttgatgatctggccttctttaaagggaagctcctcctctgcagcatctgggtttggggacatggtgagcgggtcgtagtcaaagagagccacaaagatccgggccgggagctcttcggcaccagggtcagtttctgactcttcatagaagtctggagaaaggcggtctcgcccgtaatcgtcgatggatgggactgtcacgggccgggacctctgaggaccagcgctgccacggggaaacctccggcccatgtgatccacccgtcctgcagaggctgggttccctaaaatcttgagggcattgtgggacgtgccgctgggccgcctccttcccccatcttccagctgcatttcagaatacagctcctcctcgtcctcctccatgatgtctgagaggtcagacccccggctgctctctgtgtggtactcgtctccatggcaacagtgcggctgcttgccaagttcagagcctttcaggaagtcgtccaccgaggcgcccctcctcttgaagtctggagagtcataggcgtcctcctcgtctgaggcggcgtactgccccgcgctgcttctctctaggaagacgctccttttctctaacctgctgctctcggccaccctctgcgcggcctcccgggccatggccttggcgacggtggtggacaccggggtgccctgtggctgtggcaggatgcggctgggtgagggcgaccgccttccggggcccacgggcggctccagcatgtgcccatgcacagggccaggtgcacggctctgctcccaggcctcatccatcctggcgtggggacccaggtgctcgtctttggtttcggggactccagaacttgctaatggctttgattggggtgcaggtctcgggtggggggtaggaggcaccaggagctcggggggaacggcagcaactgcagagtccacggactcgccctgggcggagagggtccgcacggtcacgcccttggcctccaggctccgcagccgcacaagctccacggccgtgctgtctgccgtggggaagatgacttcagccaccctctgccctttggcatacacgccgtagccggtaacgtttgcgccattggacagcccggtgggcgtcagcacaggtggtctccaggagacccggatggtggcgggggtcaccccagcctggacggtaacatcttgtgggggtgctgggggtcctgcaggcaacgtggagaactccacaaaggcctccttcttctccctttgctccagcgggagctgccacggcatctggtggggtttggccagaaccttcaccttataggccatgttgggcctgagattgaagaactggtacttgtacctggcggccttgacgatgtcgaactcctcctcgttgaggaagatgacgtggctgtagttgctgttggtgggtagccaggagagctgggcggagatctgcgtgatgttgtccacccgcaggtgggagggggccaccaccacgtccttgcccaccagcagcgtgcactgcagctcatccgagctgcccctgctggtgacgcactgcacggagatgcggtaggtgcaggctgccatgttgagcttctcgatgagggctttagttctgctccccagcgtgaggttcatgcgtgtctccttgtccaccaggacgttgtagctgctcaccgttccccatcctggtggcaccgccgggggctcccagcccacaataacacttttggcgagttgtttgatgagggtgatttttctagggtaaggcacgatgtcttctccgatgtcgtcgatgttcacgtccagggtcccggcactgttgtcggtgatgcccgcatctatgtgggttggggagtggaggtccaggatgtgctctccctccaggccgatgccggaatggttgatgaagttctgatcctgctcgttccccagcgtgcttgccaaccgcgactcgttgtcctgcacaaagtccacgaagttggagggcaccagacccctctggccatcgaggagctctccttcatagaacccatcctcatccatgtctccatagacgtagaggtattttcccgccgtgaggggcagctcagcttcggggttctcgttcggtccatcgaaggggttgtaactatagcgggcaacacagaggtggaccttccccgagtatctctgcttggaggtattggaattccgttcattctccatgtctgactcagatctgcatcttgcgctaccggatctcgacaggaaggtgggcttggcggacagaggctccggcctgtcaccaggctgcggaaggggccggatatattcaccgatcgcagagctgcctccaatagcgctctcctgacctttgccgagggaggtggctaggccattcatgaactgtgggaaaggcttgctgggggccgtggagatgtccaggggggccaccgcgctgccacccagcaggtcaatcttgccagcgtgctgccggaacttctccaggtcccgggacagcaggttgaactgctcactttgagtccggcatttctcttccagctctcgaaccttggactctagcagccgcactgcgccttcatgctccttcttagcctcaacctgagccttctgcagaaggtcaatttcctgctgcttggcactgagaacagccagggcctggtcatgctccaactgcagctgctgccgccgttcagccgcctctcgcatatgcttcaggacctgttctaggttctccagcttggcttggagctggtgtttctccttcacggccaaatcgcgctctctggtcacgagggtgagcggatggttgagatgcacatactctgccttcaccttgtcatgctgccgggcccttgtgggaaggcctgcatgatgggatctcaggagatactctccctgggtggcatccttcagttcattttccacaaagtttctctgctgagttcctggtctcaggagaggaagtgggaaatttccccagcggtctcccaaagcttgggtctgatcgaatgtggcctcagcacctgcaggcttcaggtgtggcgggtcatttccaagaaggcaccggagattagtggtctagtggaccagacagactggtccaggcctccccgccggccccccttccggtccccgtggacgccagcctctctgagcctcggatgtttgtgctc

SEQ ID NO: 10122 - RNA, 5266 nt, Homo sapiens
  source 1..5266: mol_type = other RNA
cacgctcatgcacacacccacacagagcttaaccacacatggatttcctttaataataaatctaccacatactattatattacaatttataatagcgtttttgaagacacaatggggaaagctttgtcattcatttataaaccgtccataaattacaaaagaaaggcagtctgaaaagtatgtataaagagtaaaaacaatttacaagtggacaagaattacaaaagagtaaccatcaaatacatctgccagcaactttgtaagtaagtcttttgttcaaatgccaatgatgaagatgggtatggactcatttggagcagatttaaattgagtctggttttggtgtggcttatgcattatgtggattacttgtgtgccattcattgctgtgtatttgggtatggcattttgacaacgaaagtaacagaaaaccatatgccacagaatagaacattaaaagcaatgaagataatcggctttctggaaggttggagtactggtgctttaccaaacaaagttactttctctccttttctcttttttgaatgattgagtaaacattttctgtgtgtagcctggctggctttgaaagactgaaactagtatcttaaaatgcacagcctgtacaacttgatctcaaaccactgtgtcaggatgaagaccactgaatgcacgacacatacaaagtatacactgtttttattagacagtacaaatcattgtgcatttataaggcagaacatcaaggcgaattaaactaggaatttcaagaccagagtcaaagtgaaagttatgcattatgaggcaagcattttgagaagggagaaaggttgaaaatcattcctttaagggcagatgacaaatgcacaaagactggaattacaggtagggagggagctacaggtgatagctatgcgcccccgtttgttaataagacgtcccctcccacctcccaaatcagagcttggacaatgagagcagactgccagcggtgacagagagcaaccgctcctctttgttctcgtggttggtttaaagtggttggtagtgcaaaagtgcatttctctactggtgtcaggggagaagattgggtttttttaggaagtacttgagtcatgaaagccctagtttggaattaaagaaaattacatagatttggcagttgtccggaagcacatgaatcatttcactgcacccagctttttcagcagtttcttgcctttggaaagcagcccctttttctttttcgaggacatttccctgcctctcccaggactaccagaacccatagatgacgtaggtgaccccgaatggagatggactgtgggggatggagctctccttgctgtacctgaaccctcaggaggaaccctttttgcctttgagcgcattggcgtatcttgagagtagtgggatggagcatcagaaagatagacttctacgtcatcaggcacttcttccaagaagtttgagggcacaaggcctttctgcccattcagctccccataataaaatccatcttcatcaatttcaccaaaaactgtaataatatctcctgtgcaaaatgtaagttcggcctcgacatcgacgttgggcgagctttctctggggtcgtagtcatacagggccaccattctccgcgtcgataccgaatgacgcctgccacttctcctgcttctctctattttctccacaggtgtattcagagggagaaagccctgtctaagaagctgatccatcatctcctcatcatctgcttgtatctcagagaccatgttacaaggaataaggccaagccgggcacaggtttccccacggtagaatccatcagcgtctttatcaccataaaccttgatgatctggccttctttaaagggaagctcctcctctgcagcatctgggtttggggacatggtgagcgggtcgtagtcaaagagagccacaaagatccgggccgggagctcttcggcaccagggtcagtttctgactcttcatagaagtctggagaaaggcggtctcgcccgtaatcgtcgatggatgggactgtcacgggccgggacctctgaggaccagcgctgccacggggaaacctccggcccatgtgatccacccgtcctgcagaggctgggttccctaaaatcttgagggcattgtgggacgtgccgctgggccgcctccttcccccatcttccagctgcatttcagaatacagctcctcctcgtcctcctccatgatgtctgagaggtcagacccccggctgctctctgtgtggtactcgtctccatggcaacagtgcggctgcttgccaagttcagagcctttcaggaagtcgtccaccgaggcgcccctcctcttgaagtctggagagtcataggcgtcctcctcgtctgaggcggcgtactgccccgcgctgcttctctctaggaagacgctccttttctctaacctgctgctctcggccaccctctgcgcggcctcccgggccatggccttggcgacggtggtggacaccggggtgccctgtggctgtggcaggatgcggctgggtgagggcgaccgccttccggggcccacgggcggctccagcatgtgcccatgcacagggccaggtgcacggctctgctcccaggcctcatccatcctggcgtggggacccaggtgctcgtctttggtttcggggactccagaacttgctaatggctttgattggggtgcaggtctcgggtggggggtaggaggcaccaggagctcggggggaacggcagcaactgcagagtccacggactcgccctgggcggagagggtccgcacggtcacgcccttggcctccaggctccgcagccgcacaagctccacggccgtgctgtctgccgtggggaagatgacttcagccaccctctgccctttggcatacacgccgtagccggtaacgtttgcgccattggacagcccggtgggcgtcagcacaggtggtctccaggagacccggatggtggcgggggtcaccccagcctggacggtaacatcttgtgggggtgctgggggtcctgcaggcaacgtggagaactccacaaaggcctccttcttctccctttgctccagcgggagctgccacggcatctggtggggtttggccagaaccttcaccttataggccatgttgggcctgagattgaagaactggtacttgtacctggcggccttgacgatgtcgaactcctcctcgttgaggaagatgacgtggctgtagttgctgttggtgggtagccaggagagctgggcggagatctgcgtgatgttgtccacccgcaggtgggagggggccaccaccacgtccttgcccaccagcagcgtgcactgcagctcatccgagctgcccctgctggtgacgcactgcacggagatgcggtaggtgcaggctgccatgttgagcttctcgatgagggctttagttctgctccccagcgtgaggttcatgcgtgtctccttgtccaccaggacgttgtagctgctcaccgttccccatcctggtggcaccgccgggggctcccagcccacaataacacttttggcgagttgtttgatgagggtgatttttctagggtaaggcacgatgtcttctccgatgtcgtcgatgttcacgtccagggtcccggcactgttgtcggtgatgcccgcatctatgtgggttggggagtggaggtccaggatgtgctctccctccaggccgatgccggaatggttgatgaagttctgatcctgctcgttccccagcgtgcttgccaaccgcgactcgttgtcctgcacaaagtccacgaagttggagggcaccagacccctctggccatcgaggagctctccttcatagaacccatcctcatccatgtctccatagacgtagaggtattttcccgccgtgaggggcagctcagcttcggggttctcgttcggtccatcgaaggggttgtaactatagcgggcaacacagaggtggaccttccccgagtatctctgcttggaggtattggaattccgttcattctccatgtctgactcagatctgcatcttgcgctaccggatctcgacaggaaggtgggcttggcggacagaggctccggcctgtcaccaggctgcggaaggggccggatatattcaccgatcgcagagctgcctccaatagcgctctcctgacctttgccgagggaggtggctaggccattcatgaactgtgggaaaggcttgctgggggccgtggagatgtccaggggggccaccgcgctgccacccagcaggtcaatcttgccagcgtgctgccggaacttctccaggtcccgggacagcaggttgaactgctcactttgagtccggcatttctcttccagctctcgaaccttggactctagcagccgcactgcgccttcatgctccttcttagcctcaacctgagccttctgcagaaggtcaatttcctgctgcttggcactgagaacagccagggcctggtcatgctccaactgcagctgctgccgccgttcagccgcctctcgcatatgcttcaggacctgttctaggttctccagcttggcttggagctggtgtttctccttcacggccaaatcgcgctctctggtcacgagggtgagcggatggttgagatgcacatactctgccttcaccttgtcatgctgccgggcccttgtgggaaggcctgcatgatgggatctcaggagatactctccctgggtggcatccttcagttcattttccacaaagtttctctgctgagttcctggtctcaggagaggaagtgggaaatttccccagcggtctcccaaagcttgggtctgatcgaatgtggcctcagcacctgcaggcttcaggtgtggcgggtcatttccaagctctgtccccattagactgtcactccaggaggggagggaccctgcttatcgtattctaagcacccaggagagcatccggccaaaggagctactgaaacacttgttgagatgccaaatgaatgaagtcttcaacctctctgttgccttcccatatgtagcagtgaggataggctggactctgctgtggttacaaataattctgattacagtggcttaagatcacctgggtgcattggtggcacctgccctgtgtctgcagctctgctccaaatcatccccacctgggacccaagctgacagaatggccaccacccaggtcactgcacatcagcaggaaggagaagctcgaggggatactgctg

SEQ ID NO: 10123 - RNA, 4982 nt, Homo sapiens
  source 1..4982: mol_type = other RNA
cacgctcatgcacacacccacacagagcttaaccacacatggatttcctttaataataaatctaccacatactattatattacaatttataatagcgtttttgaagacacaatggggaaagctttgtcattcatttataaaccgtccataaattacaaaagaaaggcagtctgaaaagtatgtataaagagtaaaaacaatttacaagtggacaagaattacaaaagagtaaccatcaaatacatctgccagcaactttgtaagtaagtcttttgttcaaatgccaatgatgaagatgggtatggactcatttggagcagatttaaattgagtctggttttggtgtggcttatgcattatgtggattacttgtgtgccattcattgctgtgtatttgggtatggcattttgacaacgaaagtaacagaaaaccatatgccacagaatagaacattaaaagcaatgaagataatcggctttctggaaggttggagtactggtgctttaccaaacaaagttactttctctccttttctcttttttgaatgattgagtaaacattttctgtgtgtagcctggctggctttgaaagactgaaactagtatcttaaaatgcacagcctgtacaacttgatctcaaaccactgtgtcaggatgaagaccactgaatgcacgacacatacaaagtatacactgtttttattagacagtacaaatcattgtgcatttataaggcagaacatcaaggcgaattaaactaggaatttcaagaccagagtcaaagtgaaagttatgcattatgaggcaagcattttgagaagggagaaaggttgaaaatcattcctttaagggcagatgacaaatgcacaaagactggaattacaggtagggagggagctacaggtgatagctatgcgcccccgtttgttaataagacgtcccctcccacctcccaaatcagagcttggacaatgagagcagactgccagcggtgacagagagcaaccgctcctctttgttctcgtggttggtttaaagtggttggtagtgcaaaagtgcatttctctactggtgtcaggggagaagattgggtttttttaggaagtacttgagtcatgaaagccctagtttggaattaaagaaaattacatagatttggcagttgtccggaagcacatgaatcatttcactgcacccagctttttcagcagtttcttgcctttggaaagcagcccctttttctttttcgaggacatttccctgcctctcccaggactaccagaacccatagatgacgtaggtgaccccgaatggagatggactgtgggggatggagctctccttgctgtacctgaaccctcaggaggaaccctttttgcctttgagcgcattggcgtatcttgagagtagtgggatggagcatcagaaagatagacttctacgtcatcaggcacttcttccaagaagtttgagggcacaaggcctttctgcccattcagctccccataataaaatccatcttcatcaatttcaccaaaaactgtaataatatctcctgtgcaaaatgtaagttcggcctcgacatcgacgttgggcgagctttctctggggtcgtagtcatacagggccaccattctccgcgtcgataccgaatgacgcctgccacttctcctgcttctctctattttctccacaggtgtattcagagggagaaagccctgtctaagaagctgatccatcatctcctcatcatctgcttgtatctcagagaccatgttacaaggaataaggccaagccgggcacaggtttccccacggtagaatccatcagcgtctttatcaccataaaccttgatgatctggccttctttaaagggaagctcctcctctgcagcatctgggtttggggacatggtgagcgggtcgtagtcaaagagagccacaaagatccgggccgggagctcttcggcaccagggtcagtttctgactcttcatagaagtctggagaaaggcggtctcgcccgtaatcgtcgatggatgggactgtcacgggccgggacctctgaggaccagcgctgccacggggaaacctccggcccatgtgatccacccgtcctgcagaggctgggttccctaaaatcttgagggcattgtgggacgtgccgctgggccgcctccttcccccatcttccagctgcatttcagaatacagctcctcctcgtcctcctccatgatgtctgagaggtcagacccccggctgctctctgtgtggtactcgtctccatggcaacagtgcggctgcttgccaagttcagagcctttcaggaagtcgtccaccgaggcgcccctcctcttgaagtctggagagtcataggcgtcctcctcgtctgaggcggcgtactgccccgcgctgcttctctctaggaagacgctccttttctctaacctgctgctctcggccaccctctgcgcggcctcccgggccatggccttggcgacggtggtggacaccggggtgccctgtggctgtggcaggatgcggctgggtgagggcgaccgccttccggggcccacgggcggctccagcatgtgcccatgcacagggccaggtgcacggctctgctcccaggcctcatccatcctggcgtggggacccaggtgctcgtctttggtttcggggactccagaacttgctaatggctttgattggggtgcaggtctcgggtggggggtaggaggcaccaggagctcggggggaacggcagcaactgcagagtccacggactcgccctgggcggagagggtccgcacggtcacgcccttggcctccaggctccgcagccgcacaagctccacggccgtgctgtctgccgtggggaagatgacttcagccaccctctgccctttggcatacacgccgtagccggtaacgtttgcgccattggacagcccggtgggcgtcagcacaggtggtctccaggagacccggatggtggcgggggtcaccccagcctggacggtaacatcttgtgggggtgctgggggtcctgcaggcaacgtggagaactccacaaaggcctccttcttctccctttgctccagcgggagctgccacggcatctggtggggtttggccagaaccttcaccttataggccatgttgggcctgagattgaagaactggtacttgtacctggcggccttgacgatgtcgaactcctcctcgttgaggaagatgacgtggctgtagttgctgttggtgggtagccaggagagctgggcggagatctgcgtgatgttgtccacccgcaggtgggagggggccaccaccacgtccttgcccaccagcagcgtgcactgcagctcatccgagctgcccctgctggtgacgcactgcacggagatgcggtaggtgcaggctgccatgttgagcttctcgatgagggctttagttctgctccccagcgtgaggttcatgcgtgtctccttgtccaccaggacgttgtagctgctcaccgttccccatcctggtggcaccgccgggggctcccagcccacaataacacttttggcgagttgtttgatgagggtgatttttctagggtaaggcacgatgtcttctccgatgtcgtcgatgttcacgtccagggtcccggcactgttgtcggtgatgcccgcatctatgtgggttggggagtggaggtccaggatgtgctctccctccaggccgatgccggaatggttgatgaagttctgatcctgctcgttccccagcgtgcttgccaaccgcgactcgttgtcctgcacaaagtccacgaagttggagggcaccagacccctctggccatcgaggagctctccttcatagaacccatcctcatccatgtctccatagacgtagaggtattttcccgccgtgaggggcagctcagcttcggggttctcgttcggtccatcgaaggggttgtaactatagcgggcaacacagaggtggaccttccccgagtatctctgcttggaggtattggaattccgttcattctccatgtctgactcagatctgcatcttgcgctaccggatctcgacaggaaggtgggcttggcggacagaggctccggcctgtcaccaggctgcggaaggggccggatatattcaccgatcgcagagctgcctccaatagcgctctcctgacctttgccgagggaggtggctaggccattcatgaactgtgggaaaggcttgctgggggccgtggagatgtccaggggggccaccgcgctgccacccagcaggtcaatcttgccagcgtgctgccggaacttctccaggtcccgggacagcaggttgaactgctcactttgagtccggcatttctcttccagctctcgaaccttggactctagcagccgcactgcgccttcatgctccttcttagcctcaacctgagccttctgcagaaggtcaatttcctgctgcttggcactgagaacagccagggcctggtcatgctccaactgcagctgctgccgccgttcagccgcctctcgcatatgcttcaggacctgttctaggttctccagcttggcttggagctggtgtttctccttcacggccaaatcgcgctctctggtcacgagggtgagcggatggttgagatgcacatactctgccttcaccttgtcatgctgccgggcccttgtgggaaggcctgcatgatgggatctcaggagatactctccctgggtggcatccttcagttcattttccacaaagtttctctgctgagttcctggtctcaggagaggaagtgggaaatttccccagcggtctcccaaagcttgggtctgatcgaatgtggcctcagcacctgcaggcttcaggtgtggcgggtcatttccaagctttagaagcgagctgtgccaaggctccggaggttcacctcggagacaactgcagtgtactgtgtcagattacaaact

SEQ ID NO: 10124 - RNA, 6629 nt, Homo sapiens
  source 1..6629: mol_type = other RNA
cacgctcatgcacacacccacacagagcttaaccacacatggatttcctttaataataaatctaccacatactattatattacaatttataatagcgtttttgaagacacaatggggaaagctttgtcattcatttataaaccgtccataaattacaaaagaaaggcagtctgaaaagtatgtataaagagtaaaaacaatttacaagtggacaagaattacaaaagagtaaccatcaaatacatctgccagcaactttgtaagtaagtcttttgttcaaatgccaatgatgaagatgggtatggactcatttggagcagatttaaattgagtctggttttggtgtggcttatgcattatgtggattacttgtgtgccattcattgctgtgtatttgggtatggcattttgacaacgaaagtaacagaaaaccatatgccacagaatagaacattaaaagcaatgaagataatcggctttctggaaggttggagtactggtgctttaccaaacaaagttactttctctccttttctcttttttgaatgattgagtaaacattttctgtgtgtagcctggctggctttgaaagactgaaactagtatcttaaaatgcacagcctgtacaacttgatctcaaaccactgtgtcaggatgaagaccactgaatgcacgacacatacaaagtatacactgtttttattagacagtacaaatcattgtgcatttataaggcagaacatcaaggcgaattaaactaggaatttcaagaccagagtcaaagtgaaagttatgcattatgaggcaagcattttgagaagggagaaaggttgaaaatcattcctttaagggcagatgacaaatgcacaaagactggaattacaggtagggagggagctacaggtgatagctatgcgcccccgtttgttaataagacgtcccctcccacctcccaaatcagagcttggacaatgagagcagactgccagcggtgacagagagcaaccgctcctctttgttctcgtggttggtttaaagtggttggtagtgcaaaagtgcatttctctactggtgtcaggggagaagattgggtttttttaggaagtacttgagtcatgaaagccctagtttggaattaaagaaaattacatagatttggcagttgtccggaagcacatgaatcatttcactgcacccagctttttcagcagtttcttgcctttggaaagcagcccctttttctttttcgaggacatttccctgcctctcccaggactaccagaacccatagatgacgtaggtgaccccgaatggagatggactgtgggggatggagctctccttgctgtacctgaaccctcaggaggaacctagtaggtacagtgttacagtttattgagtgtgtgagcgccaacaacagaattcacttggtaacatcgtactgtccccgtttcccaccaggaaaggtcaggggggttcatttgttctttcagttgttgaagtatgccatgagaagcaaaggtcctctcccacagcacgccagagagaggccccagacataaatgtgtgggttccgtttctctgtctcgagggagtgcggggtggccgttgctttggcaaagctaaggcaggtaataattcacttcataaatgaagactaagggcaggggagacatgatctgaaattaggttgatagtaaagttggccgagtacccatcagtagtcttaaaaagcgaaagttcataaagggaattttgttgtatttgaaactatttggttatataaaatcctgatattgttaaagtgcattcctggggtggttggtatactatagaaatattggagatggcacactggttgaaagaaaaaaaaaaactaaaatgaaccttaattataatcaaagaaagcttaaaggcccttagtggatgcttgcattatttccaaataattgaacatgaatcttcctcagtagatagcacatggtagtatttaaatatacgttaagcgcttaatagtgcttcagaggggtagacttttactctaatacgctgcaggacgacttcacctcgcttccctttacagctaagcatgtgcctgagttggcagtgcagcagcattcctctggccctacctctccagagcaactcttgccatgtgagtgtttagtattcagcaggcaaatgctgtaagccaaggggcttcaagcttgcttggatttaaaatcaaggtctaattctaatggaaaacacctagtaaagcatcccaaagtacacctgaagataccatctattccatctaatgtgatcatttgagctgcgtgcttcatcaacttagtattgcattggtataccaacaacaaacgcgtgttgcagcaacttctgtcacaggatgattgtgctttgaggaggagcatagctctctcgtaaggtagaggcagggttacttaaggaaaacacgttctggccactcgagccagtgtttggagtgttcagagccaacactcgatcacctgtgttcactactcatctgcttgaccttgggttaagtttctaaagtaaagcttcctatagtaaacatgtttgttaggttgtgctttttccaagagtggctaacaatgcaatatgcagctctctctatgtaaacacacagttagcttgttaagaaatatgttcccaatgttggcctttcaaatattcttaatgcaaatagtaggaaatgattattaaagatgatttgcttcactataaattcagttgctttacaactgagaccaagtaatattctaattatttaggtccaatagttttttgagacatatttctttgtatctttttttttttttaaccccacaatgaagccttaagtctaccacactggcccggttaaggtagcttaagttggtatctttatcggtatcttcagttgctcacttacgtgaaggctacattgcctgattaaggtgtgaaatgaacactcttcctttttgcctttgagcgcattggcgtatcttgagagtagtgggatggagcatcagaaagatagacttctacgtcatcaggcacttcttccaagaagtttgagggcacaaggcctttctgcccattcagctccccataataaaatccatcttcatcaatttcaccaaaaactgtaataatatctcctgtgcaaaatgtaagttcggcctcgacatcgacgttgggcgagctttctctggggtcgtagtcatacagggccaccattctccgcgtcgataccgaatgacgcctgccacttctcctgcttctctctattttctccacaggtgtattcagagggagaaagccctgtctaagaagctgatccatcatctcctcatcatctgcttgtatctcagagaccatgttacaaggaataaggccaagccgggcacaggtttccccacggtagaatccatcagcgtctttatcaccataaaccttgatgatctggccttctttaaagggaagctcctcctctgcagcatctgggtttggggacatggtgagcgggtcgtagtcaaagagagccacaaagatccgggccgggagctcttcggcaccagggtcagtttctgactcttcatagaagtctggagaaaggcggtctcgcccgtaatcgtcgatggatgggactgtcacgggccgggacctctgaggaccagcgctgccacggggaaacctccggcccatgtgatccacccgtcctgcagaggctgggttccctaaaatcttgagggcattgtgggacgtgccgctgggccgcctccttcccccatcttccagctgcatttcagaatacagctcctcctcgtcctcctccatgatgtctgagaggtcagacccccggctgctctctgtgtggtactcgtctccatggcaacagtgcggctgcttgccaagttcagagcctttcaggaagtcgtccaccgaggcgcccctcctcttgaagtctggagagtcataggcgtcctcctcgtctgaggcggcgtactgccccgcgctgcttctctctaggaagacgctccttttctctaacctgctgctctcggccaccctctgcgcggcctcccgggccatggccttggcgacggtggtggacaccggggtgccctgtggctgtggcaggatgcggctgggtgagggcgaccgccttccggggcccacgggcggctccagcatgtgcccatgcacagggccaggtgcacggctctgctcccaggcctcatccatcctggcgtggggacccaggtgctcgtctttggtttcggggactccagaacttgctaatggctttgattggggtgcaggtctcgggtggggggtaggaggcaccaggagctcggggggaacggcagcaactgcagagtccacggactcgccctgggcggagagggtccgcacggtcacgcccttggcctccaggctccgcagccgcacaagctccacggccgtgctgtctgccgtggggaagatgacttcagccaccctctgccctttggcatacacgccgtagccggtaacgtttgcgccattggacagcccggtgggcgtcagcacaggtggtctccaggagacccggatggtggcgggggtcaccccagcctggacggtaacatcttgtgggggtgctgggggtcctgcaggcaacgtggagaactccacaaaggcctccttcttctccctttgctccagcgggagctgccacggcatctggtggggtttggccagaaccttcaccttataggccatgttgggcctgagattgaagaactggtacttgtacctggcggccttgacgatgtcgaactcctcctcgttgaggaagatgacgtggctgtagttgctgttggtgggtagccaggagagctgggcggagatctgcgtgatgttgtccacccgcaggtgggagggggccaccaccacgtccttgcccaccagcagcgtgcactgcagctcatccgagctgcccctgctggtgacgcactgcacggagatgcggtaggtgcaggctgccatgttgagcttctcgatgagggctttagttctgctccccagcgtgaggttcatgcgtgtctccttgtccaccaggacgttgtagctgctcaccgttccccatcctggtggcaccgccgggggctcccagcccacaataacacttttggcgagttgtttgatgagggtgatttttctagggtaaggcacgatgtcttctccgatgtcgtcgatgttcacgtccagggtcccggcactgttgtcggtgatgcccgcatctatgtgggttggggagtggaggtccaggatgtgctctccctccaggccgatgccggaatggttgatgaagttctgatcctgctcgttccccagcgtgcttgccaaccgcgactcgttgtcctgcacaaagtccacgaagttggagggcaccagacccctctggccatcgaggagctctccttcatagaacccatcctcatccatgtctccatagacgtagaggtattttcccgccgtgaggggcagctcagcttcggggttctcgttcggtccatcgaaggggttgtaactatagcgggcaacacagaggtggaccttccccgagtatctctgcttggaggtattggaattccgttcattctccatgtctgactcagatctgcatcttgcgctaccggatctcgacaggaaggtgggcttggcggacagaggctccggcctgtcaccaggctgcggaaggggccggatatattcaccgatcgcagagctgcctccaatagcgctctcctgacctttgccgagggaggtggctaggccattcatgaactgtgggaaaggcttgctgggggccgtggagatgtccaggggggccaccgcgctgccacccagcaggtcaatcttgccagcgtgctgccggaacttctccaggtcccgggacagcaggttgaactgctcactttgagtccggcatttctcttccagctctcgaaccttggactctagcagccgcactgcgccttcatgctccttcttagcctcaacctgagccttctgcagaaggtcaatttcctgctgcttggcactgagaacagccagggcctggtcatgctccaactgcagctgctgccgccgttcagccgcctctcgcatatgcttcaggacctgttctaggttctccagcttggcttggagctggtgtttctccttcacggccaaatcgcgctctctggtcacgagggtgagcggatggttgagatgcacatactctgccttcaccttgtcatgctgccgggcccttgtgggaaggcctgcatgatgggatctcaggagatactctccctgggtggcatccttcagttcattttccacaaagtttctctgctgagttcctggtctcaggagaggaagtgggaaatttccccagcggtctcccaaagcttgggtctgatcgaatgtggcctcagcacctgcaggcttcaggtgtggcgggtcatttccaagaaggcaccggagattagtggtctagtggaccagacagactggtccaggcctccccgccggccccccttccggtccccgtggacgccagcctctctgagcctcggatgtttgtgctc

SEQ ID NO: 10125 - RNA, 6594 nt, Homo sapiens
  source 1..6594: mol_type = other RNA
cacgctcatgcacacacccacacagagcttaaccacacatggatttcctttaataataaatctaccacatactattatattacaatttataatagcgtttttgaagacacaatggggaaagctttgtcattcatttataaaccgtccataaattacaaaagaaaggcagtctgaaaagtatgtataaagagtaaaaacaatttacaagtggacaagaattacaaaagagtaaccatcaaatacatctgccagcaactttgtaagtaagtcttttgttcaaatgccaatgatgaagatgggtatggactcatttggagcagatttaaattgagtctggttttggtgtggcttatgcattatgtggattacttgtgtgccattcattgctgtgtatttgggtatggcattttgacaacgaaagtaacagaaaaccatatgccacagaatagaacattaaaagcaatgaagataatcggctttctggaaggttggagtactggtgctttaccaaacaaagttactttctctccttttctcttttttgaatgattgagtaaacattttctgtgtgtagcctggctggctttgaaagactgaaactagtatcttaaaatgcacagcctgtacaacttgatctcaaaccactgtgtcaggatgaagaccactgaatgcacgacacatacaaagtatacactgtttttattagacagtacaaatcattgtgcatttataaggcagaacatcaaggcgaattaaactaggaatttcaagaccagagtcaaagtgaaagttatgcattatgaggcaagcattttgagaagggagaaaggttgaaaatcattcctttaagggcagatgacaaatgcacaaagactggaattacaggtagggagggagctacaggtgatagctatgcgcccccgtttgttaataagacgtcccctcccacctcccaaatcagagcttggacaatgagagcagactgccagcggtgacagagagcaaccgctcctctttgttctcgtggttggtttaaagtggttggtagtgcaaaagtgcatttctctactggtgtcaggggagaagattgggtttttttaggaagtacttgagtcatgaaagccctagtttggaattaaagaaaattacatagatttggcagttgtccggaagcacatgaatcatttcactgcacccagctttttcagcagtttcttgcctttggaaagcagcccctttttctttttcgaggacatttccctgcctctcccaggactaccagaacccatagatgacgtaggtgaccccgaatggagatggactgtgggggatggagctctccttgctgtacctgaaccctcaggaggaacctagtaggtacagtgttacagtttattgagtgtgtgagcgccaacaacagaattcacttggtaacatcgtactgtccccgtttcccaccaggaaaggtcaggggggttcatttgttctttcagttgttgaagtatgccatgagaagcaaaggtcctctcccacagcacgccagagagaggccccagacataaatgtgtgggttccgtttctctgtctcgagggagtgcggggtggccgttgctttggcaaagctaaggcaggtaataattcacttcataaatgaagactaagggcaggggagacatgatctgaaattaggttgatagtaaagttggccgagtacccatcagtagtcttaaaaagcgaaagttcataaagggaattttgttgtatttgaaactatttggttatataaaatcctgatattgttaaagtgcattcctggggtggttggtatactatagaaatattggagatggcacactggttgaaagaaaaaaaaaaactaaaatgaaccttaattataatcaaagaaagcttaaaggcccttagtggatgcttgcattatttccaaataattgaacatgaatcttcctcagtagatagcacatggtagtatttaaatatacgttaagcgcttaatagtgcttcagaggggtagacttttactctaatacgctgcaggacgacttcacctcgcttccctttacagctaagcatgtgcctgagttggcagtgcagcagcattcctctggccctacctctccagagcaactcttgccatgtgagtgtttagtattcagcaggcaaatgctgtaagccaaggggcttcaagcttgcttggatttaaaatcaaggtctaattctaatggaaaacacctagtaaagcatcccaaagtacacctgaagataccatctattccatctaatgtgatcatttgagctgcgtgcttcatcaacttagtattgcattggtataccaacaacaaacgcgtgttgcagcaacttctgtcacaggatgattgtgctttgaggaggagcatagctctctcgtaaggtagaggcagggttacttaaggaaaacacgttctggccactcgagccagtgtttggagtgttcagagccaacactcgatcacctgtgttcactactcatctgcttgaccttgggttaagtttctaaagtaaagcttcctatagtaaacatgtttgttaggttgtgctttttccaagagtggctaacaatgcaatatgcagctctctctatgtaaacacacagttagcttgttaagaaatatgttcccaatgttggcctttcaaatattcttaatgcaaatagtaggaaatgattattaaagatgatttgcttcactataaattcagttgctttacaactgagaccaagtaatattctaattatttaggtccaatagttttttgagacatatttctttgtatctttttttttttttaaccccacaatgaagccttaagtctaccacactggcccggttaaggtagcttaagttggtatctttatcggtatcttcagttgctcacttacgtgaaggctacattgcctgattaaggtgtgaaatgaacactcttcttcctttttgcctttgagcgcattggcgtatcttgagagtagtgggatggagcatcagaaagatagacttctacgtcatcaggcacttcttccaagaagtttgagggcacaaggcctttctgcccattcagctccccataataaaatccatcttcatcaatttcaccaaaaactgtaataatatctcctgtgcaaaatgtaagttcggcctcgacatcgacgttgggcgagctttctctggggtcgtagtcatacagggccaccattctccgcgtcgataccgaatgacgcctgccacttctcctgcttctctctattttctccacaggtgtattcagagggagaaagccctgtctaagaagctgatccatcatctcctcatcatctgcttgtatctcagagaccatgttacaaggaataaggccaagccgggcacaggtttccccacggtagaatccatcagcgtctttatcaccataaaccttgatgatctggccttctttaaagggaagctcctcctctgcagcatctgggtttggggacatggtgagcgggtcgtagtcaaagagagccacaaagatccgggccgggagctcttcggcaccagggtcagtttctgactcttcatagaagtctggagaaaggcggtctcgcccgtaatcgtcgatggatgggactgtcacgggccgggacctctgaggaccagcgctgccacggggaaacctccggcccatgtgatccacccgtcctgcagaggctgggttccctaaaatcttgagggcattgtgggacgtgccgctgggccgcctccttcccccatcttccagctgcatttcagaatacagctcctcctcgtcctcctccatgatgtctgagaggtcagacccccggctgctctctgtgtggtactcgtctccatggcaacagtgcggctgcttgccaagttcagagcctttcaggaagtcgtccaccgaggcgcccctcctcttgaagtctggagagtcataggcgtcctcctcgtctgaggcggcgtactgccccgcgctgcttctctctaggaagacgctccttttctctaacctgctgctctcggccaccctctgcgcggcctcccgggccatggccttggcgacggtggtggacaccggggtgccctgtggctgtggcaggatgcggctgggtgagggcgaccgccttccggggcccacgggcggctccagcatgtgcccatgcacagggccaggtgcacggctctgctcccaggcctcatccatcctggcgtggggacccaggtgctcgtctttggtttcggggactccagaacttgctaatggctttgattggggtgcaggtctcgggtggggggtaggaggcaccaggagctcggggggaacggcagcaactgcagagtccacggactcgccctgggcggagagggtccgcacggtcacgcccttggcctccaggctccgcagccgcacaagctccacggccgtgctgtctgccgtggggaagatgacttcagccaccctctgccctttggcatacacgccgtagccggtaacgtttgcgccattggacagcccggtgggcgtcagcacaggtggtctccaggagacccggatggtggcgggggtcaccccagcctggacggtaacatcttgtgggggtgctgggggtcctgcaggcaacgtggagaactccacaaaggcctccttcttctccctttgctccagcgggagctgccacggcatctggtggggtttggccagaaccttcaccttataggccatgttgggcctgagattgaagaactggtacttgtacctggcggccttgacgatgtcgaactcctcctcgttgaggaagatgacgtggctgtagttgctgttggtgggtagccaggagagctgggcggagatctgcgtgatgttgtccacccgcaggtgggagggggccaccaccacgtccttgcccaccagcagcgtgcactgcagctcatccgagctgcccctgctggtgacgcactgcacggagatgcggtaggtgcaggctgccatgttgagcttctcgatgagggctttagttctgctccccagcgtgaggttcatgcgtgtctccttgtccaccaggacgttgtagctgctcaccgttccccatcctggtggcaccgccgggggctcccagcccacaataacacttttggcgagttgtttgatgagggtgatttttctagggtaaggcacgatgtcttctccgatgtcgtcgatgttcacgtccagggtcccggcactgttgtcggtgatgcccgcatctatgtgggttggggagtggaggtccaggatgtgctctccctccaggccgatgccggaatggttgatgaagttctgatcctgctcgttccccagcgtgcttgccaaccgcgactcgttgtcctgcacaaagtccacgaagttggagggcaccagacccctctggccatcgaggagctctccttcatagaacccatcctcatccatgtctccatagacgtagaggtattttcccgccgtgaggggcagctcagcttcggggttctcgttcggtccatcgaaggggttgtaactatagcgggcaacacagaggtggaccttccccgagtatctctgcttggaggtattggaattccgttcattctccatgtctgactcagatctgcatcttgcgctaccggatctcgacaggaaggtgggcttggcggacagaggctccggcctgtcaccaggctgcggaaggggccggatatattcaccgatcgcagagctgcctccaatagcgctctcctgacctttgccgagggaggtggctaggccattcatgaactgtgggaaaggcttgctgggggccgtggagatgtccaggggggccaccgcgctgccacccagcaggtcaatcttgccagcgtgctgccggaacttctccaggtcccgggacagcaggttgaactgctcactttgagtccggcatttctcttccagctctcgaaccttggactctagcagccgcactgcgccttcatgctccttcttagcctcaacctgagccttctgcagaaggtcaatttcctgctgcttggcactgagaacagccagggcctggtcatgctccaactgcagctgctgccgccgttcagccgcctctcgcatatgcttcaggacctgttctaggttctccagcttggcttggagctggtgtttctccttcacggccaaatcgcgctctctggtcacgagggtgagcggatggttgagatgcacatactctgccttcaccttgtcatgctgccgggcccttgtgggaaggcctgcatgatgggatctcaggagatactctccctgggtggcatccttcagttcattttccacaaagtttctctgctgagttcctggtctcaggagaggaagtgggaaatttccccagcggtctcccaaagcttgggtctgatcgaatgtggcctcagcacctgcaggcttcaggtgtggcgggtcatttccaagctttagaagcgagctgtgccaaggctccggaggttcacctcggagacaactgcagtgtactgtgtcagattacaaact

SEQ ID NO: 10126 - RNA, 6465 nt, Homo sapiens
  source 1..6465: mol_type = other RNA
cacgctcatgcacacacccacacagagcttaaccacacatggatttcctttaataataaatctaccacatactattatattacaatttataatagcgtttttgaagacacaatggggaaagctttgtcattcatttataaaccgtccataaattacaaaagaaaggcagtctgaaaagtatgtataaagagtaaaaacaatttacaagtggacaagaattacaaaagagtaaccatcaaatacatctgccagcaactttgtaagtaagtcttttgttcaaatgccaatgatgaagatgggtatggactcatttggagcagatttaaattgagtctggttttggtgtggcttatgcattatgtggattacttgtgtgccattcattgctgtgtatttgggtatggcattttgacaacgaaagtaacagaaaaccatatgccacagaatagaacattaaaagcaatgaagataatcggctttctggaaggttggagtactggtgctttaccaaacaaagttactttctctccttttctcttttttgaatgattgagtaaacattttctgtgtgtagcctggctggctttgaaagactgaaactagtatcttaaaatgcacagcctgtacaacttgatctcaaaccactgtgtcaggatgaagaccactgaatgcacgacacatacaaagtatacactgtttttattagacagtacaaatcattgtgcatttataaggcagaacatcaaggcgaattaaactaggaatttcaagaccagagtcaaagtgaaagttatgcattatgaggcaagcattttgagaagggagaaaggttgaaaatcattcctttaagggcagatgacaaatgcacaaagactggaattacaggtagggagggagctacaggtgatagctatgcgcccccgtttgttaataagacgtcccctcccacctcccaaatcagagcttggacaatgagagcagactgccagcggtgacagagagcaaccgctcctctttgttctcgtggttggtttaaagtggttggtagtgcaaaagtgcatttctctactggtgtcaggggagaagattgggtttttttaggaagtacttgagtcatgaaagccctagtttggaattaaagaaaattacatagatttggcagttgtccggaagcacatgaatcatttcactgcacccagctttttcagcagtttcttgcctttggaaagcagcccctttttctttttcgaggacatttccctgcctctcccaggactaccagaacccatagatgacgtaggtgaccccgaatggagatggactgtgggggatggagctctccttgctgtacctgaaccctcaggaggaacctagtaggtacagtgttacagtttattgagtgtgtgagcgccaacaacagaattcacttggtaacatcgtactgtccccgtttcccaccaggaaaggtcaggggggttcatttgttctttcagttgttgaagtatgccatgagaagcaaaggtcctctcccacagcacgccagagagaggccccagacataaatgtgtgggttccgtttctctgtctcgagggagtgcggggtggccgttgctttggcaaagctaaggcaggtaataattcacttcataaatgaagactaagggcaggggagacatgatctgaaattaggttgatagtaaagttggccgagtacccatcagtagtcttaaaaagcgaaagttcataaagggaattttgttgtatttgaaactatttggttatataaaatcctgatattgttaaagtgcattcctggggtggttggtatactatagaaatattggagatggcacactggttgaaagaaaaaaaaaaactaaaatgaaccttaattataatcaaagaaagcttaaaggcccttagtggatgcttgcattatttccaaataattgaacatgaatcttcctcagtagatagcacatggtagtatttaaatatacgttaagcgcttaatagtgcttcagaggggtagacttttactctaatacgctgcaggacgacttcacctcgcttccctttacagctaagcatgtgcctgagttggcagtgcagcagcattcctctggccctacctctccagagcaactcttgccatgtgagtgtttagtattcagcaggcaaatgctgtaagccaaggggcttcaagcttgcttggatttaaaatcaaggtctaattctaatggaaaacacctagtaaagcatcccaaagtacacctgaagataccatctattccatctaatgtgatcatttgagctgcgtgcttcatcaacttagtattgcattggtataccaacaacaaacgcgtgttgcagcaacttctgtcacaggatgattgtgctttgaggaggagcatagctctctcgtaaggtagaggcagggttacttaaggaaaacacgttctggccactcgagccagtgtttggagtgttcagagccaacactcgatcacctgtgttcactactcatctgcttgaccttgggttaagtttctaaagtaaagcttcctatagtaaacatgtttgttaggttgtgctttttccaagagtggctaacaatgcaatatgcagctctctctatgtaaacacacagttagcttgttaagaaatatgttcccaatgttggcctttcaaatattcttaatgcaaatagtaggaaatgattattaaagatgatttgcttcactataaattcagttgctttacaactgagaccaagtaatattctaattatttaggtccaatagttttttgagacatatttctttgtatctttttttttttttaaccccacaatgaagccttaagtctaccacactggcccggttaaggtagcttaagttggtatctttatcggtatcttcagttgctcacttacgtgaaggctacattgcctgattaaggtgtgaaatgaacactcttcttcctttttgcctttgagcgcattggcgtatcttgagagtagtgggatggagcatcagaaagatagacttctacgtcatcaggcacttcttccaagaagtttgagggcacaaggcctttctgcccattcagctccccataataaaatccatcttcatcaatttcaccaaaaactgtaataatatctcctgtgcaaaatgtaagttcggcctcgacatcgacgttgggcgagctttctctggggtcgtagtcatacagggccaccattctccgcgtcgataccgaatgacgcctgccacttctcctgcttctctctattttctccacaggtgtattcagagggagaaagccctgtctaagaagctgatccatcatctcctcatcatctgcttgtatctcagagaccatgttacaaggaataaggccaagccgggcacaggtttccccacggtagaatccatcagcgtctttatcaccataaaccttgatgatctggccttctttaaagggaagctcctcctctgcagcatctgggtttggggacatggtgagcgggtcgtagtcaaagagagccacaaagatccgggccgggagctcttcggcaccagggtcagtttctgactcttcatagaagtctggagaaaggcggtctcgcccgtaatcgtcgatggatgggactgtcacgggccgggacctctgaggaccagcgctgccacggggaaacctccggcccatgtgatccacccgtcctgcagaggctgggttccctaaaatcttgagggcattgtgggacgtgccgctgggccgcctccttcccccatcttccagctgcatttcagaatacagctcctcctcgtcctcctccatgatgtctgagaggtcagacccccggctgctctctgtgtggtactcgtctccatggcaacagtgcggctgcttgccaagttcagagcctttcaggaagtcgtccaccgaggcgcccctcctcttgaagtctggagagtcataggcgtcctcctcgtctgaggcggcgtactgccccgcgctgcttctctctaggaagacgctccttttctctaacctgctgctctcggccaccctctgcgcggcctcccgggccatggccttggcgacggtggtggacaccggggtgccctgtggctgtggcaggatgcggctgggtgagggcgaccgccttccggggcccacgggcggctccagcatgtgcccatgcacagggccaggtgcacggctctgctcccaggcctcatccatcctggcgtggggacccaggtgctcgtctttggtttcggggactccagaacttgctaatggctttgattggggtgcaggtctcgggtggggggtaggaggcaccaggagctcggggggaacggcagcaactgcagagtccacggactcgccctgggcggagagggtccgcacggtcacgcccttggcctccaggctccgcagccgcacaagctccacggccgtgctgtctgccgtggggaagatgacttcagccaccctctgccctttggcatacacgccgtagccggtaacgtttgcgccattggacagcccggtgggcgtcagcacaggtggtctccaggagacccggatggtggcgggggtcaccccagcctggacggtaacatcttgtgggggtgctgggggtcctgcaggcaacgtggagaactccacaaaggcctccttcttctccctttgctccagcgggagctgccacggcatctggtggggtttggccagaaccttcaccttataggccatgttgggcctgagattgaagaactggtacttgtacctggcggccttgacgatgtcgaactcctcctcgttgaggaagatgacgtggctgtagttgctgttggtgggtagccaggagagctgggcggagatctgcgtgatgttgtccacccgcaggtgggagggggccaccaccacgtccttgcccaccagcagcgtgcactgcagctcatccgagctgcccctgctggtgacgcactgcacggagatgcggtaggtgcaggctgccatgttgagcttctcgatgagggctttagttctgctccccagcgtgaggttcatgcgtgtctccttgtccaccaggacgttgtagctgctcaccgttccccatcctggtggcaccgccgggggctcccagcccacaataacacttttggcgagttgtttgatgagggtgatttttctagggtaaggcacgatgtcttctccgatgtcgtcgatgttcacgtccagggtcccggcactgttgtcggtgatgcccgcatctatgtgggttggggagtggaggtccaggatgtgctctccctccaggccgatgccggaatggttgatgaagttctgatcctgctcgttccccagcgtgcttgccaaccgcgactcgttgtcctgcacaaagtccacgaagttggagggcaccagacccctctggccatcgaggagctctccttcatagaacccatcctcatccatgtctccatagacgtagaggtattttcccgccgtgaggggcagctcagcttcggggttctcgttcggtccatcgaaggggttgtaactatagcgggcaacacagaggtggaccttccccgagtatctctgcttggaggtattggaattccgttcattctccatgtctgactcagatctgcatcttgcgctaccggatctcgacaggaaggtgggcttggcggacagaggctccggcctgtcaccaggctgcggaaggggccggatatattcaccgatcgcagagctgcctccaatagcgctctcctgacctttgccgagggaggtggctaggccattcatgaactgtgggaaaggcttgctgggggccgtggagatgtccaggggggccaccgcgctgccacccagcaggtcaatcttgccagcgtgctgccggaacttctccaggtcccgggacagcaggttgaactgctcactttgagtccggcatttctcttccagctctcgaaccttggacttctgcagaaggtcaatttcctgctgcttggcactgagaacagccagggcctggtcatgctccaactgcagctgctgccgccgttcagccgcctctcgcatatgcttcaggacctgttctaggttctccagcttggcttggagctggtgtttctccttcacggccaaatcgcgctctctggtcacgagggtgagcggatggttgagatgcacatactctgccttcaccttgtcatgctgccgggcccttgtgggaaggcctgcatgatgggatctcaggagatactctccctgggtggcatccttcagttcattttccacaaagtttctctgctgagttcctggtctcaggagaggaagtgggaaatttccccagcggtctcccaaagcttgggtctgatcgaatgtggcctcagcacctgcaggcttcaggtgtggcgggtcatttccaag

SEQ ID NO: 10127 - RNA, 969 nt, Homo sapiens
  source 1..969: mol_type = other RNA
cacggcaaaagaaacaatccaaattttgacttggcaatcctgaccacatgatgccagtcgaaaaaactgaagaccttgttctccatcagaaactggctgtgaagaaaaatcgcagcaggtaattccaagatcatgtgctttttcactatgcagacacctcattttatcatcccacactgttaaatcaccacatgaggagccagtgacaaagaagcttccattaggagaaaatgcacatgccgccaaggagccatctttaacactaccacatctatataatttgtatgactgtgcattccacaaaaccacagttccatcagctgcccctgatgccaaacacgtggagtctggggaaaactggcaaaccctcacagggctgccactaggctgttccatcactgccagcatctgtccattttcagtattccataggacagtggtaccatctgttgaacacgatgccaaaatatgtcctgaaggggagaaacagcagcagtggacagcataggtatgaaacttcaatggagaatgtggcagttcagtaaagtcacgtaacgagtacaggcgaattgttttgtccaaggagcaagtagccaagagggaaaaggagaaggcacagcagttgacatcgtcaccatgatcagctaatgtgtgaatcagtttcaccatgttctttatttgaagaaaaacagccacgcctcgccgcactcaaggtcccggttgggccctgctgcgcggttagaaccgggaaatggagggctcagacgccccgcgcgagcaggcccagccgcgcttccccacctgccgccaccgccgctgagccggcccgtgggcgcggccgctctcacctgcaggagcgggggcgcgcgggatccgccttcaaggtgcccacgggcggtgcgggtcacgtgccgcgcaggtgaggctggcggggcgggcgccggcggagacccagagcagagggaacag

SEQ ID NO: 10128 - RNA, 1037 nt, Homo sapiens
  source 1..1037: mol_type = other RNA
cacggcaaaagaaacaatccaaattttgacttggcaatcctgaccacatgatgccagtcgaaaaaactgaagaccttgttctccatcagaaactggctgtgaagaaaaatcgcagcaggtaattccaagatcatgtgctttttcactatgcagacacctcattttatcatcccacactgttaaatcaccacatgaggagccagtgacaaagaagcttccattaggagaaaatgcacatgccgccaaggagccatctttaacactaccacatctatataatttgtatgactgtgcattccacaaaaccacagttccatcagctgcccctgatgccaaacacgtggagtctggggaaaactggcaaaccctcacagggctgccactaggctgttccatcactgccagcatctgtccattttcagtattccataggacagtggtaccatctgttgaacacgatgccaaaatatgtcctgaaggggagaaacagcagcagtggacagcataggtatgaaacttcaatggagaatgtggcagttcagtaaagtcacgtaacgagtacaggcgaattgttttgtccaaggagcaagtagccaagagggaaaaggagaaggcacagcagttgacatcgtcaccatgatcagctaatgtgtgaatcagtttcaccatgttctttatttgaagaaaaacagcccgcaaggggcttccttccacccgacgccgacacgcccgccctagccccgggccaagggtgcacgaaccacgcctcgccgcactcaaggtcccggttgggccctgctgcgcggttagaaccgggaaatggagggctcagacgccccgcgcgagcaggcccagccgcgcttccccacctgccgccaccgccgctgagccggcccgtgggcgcggccgctctcacctgcaggagcgggggcgcgcgggatccgccttcaaggtgcccacgggcggtgcgggtcacgtgccgcgcaggtgaggctggcggggcgggcgccggcggagacccagagcagagggaacag

SEQ ID NO: 10129 - RNA, 814 nt, Homo sapiens
  source 1..814: mol_type = other RNA
cacggcaaaagaaacaatccaaattttgacttggcaatcctgaccacatgatgccagtcgaaaaaactgaagaccttgttctccatcagaaactggctgtgaagaaaaatcgcagcaggtaattccaagatcatgtgctttttcactatgcagacacctcattttatcatcccacactgttaaatcaccacatgaggagccagtgacaaagaagcttccattaggagaaaatgcacatgccgccaaggagccatctttaacactaccacatctatataatttgtatgactgtgcattccacaaaaccacagttccatcagctgcccctgatgccaaacacgtggagtctggggaaaactggcaaaccctcacagggctgccactaggctgttccatcactgccagcatctgtccattttcagtattccataggacagtggtaccatctgttgaacacgatgccaaaatatgtcctgaaggggagaaacagcagcagtggacagcataggtatgaaacttcaatggagaatgtggcagttcagtaaagtcacgtaacgagtacaggcgaattgttttgtccaaggagcaagtagccaagagggaaaaggagaaggcacagcagttgacatcgtcaccatgatcagctaatgtgtgaatcagtttcaccatgttctttatttgaagaaaaacagcctgcaggagcgggggcgcgcgggatccgccttcaaggtgcccacgggcggtgcgggtcacgtgccgcgcaggtgaggctggcggggcgggcgccggcggagacccagagcagagggaacag

SEQ ID NO: 10130 - RNA, 904 nt, Homo sapiens
  source 1..904: mol_type = other RNA
cacggcaaaagaaacaatccaaattttgacttggcaatcctgaccacatgatgccagtcgaaaaaactgaagaccttgttctccatcagaaactggctgtgaagaaaaatcgcagcaggtaattccaagatcatgtgctttttcactatgcagacacctcattttatcatcccacactgttaaatcaccacatgaggagccagtgacaaagaagcttccattaggagaaaatgcacatgccgccaaggagccatctttaacactaccacatctatataatttgtatgactgtgcattccacaaaaccacagttccatcagctgcccctgatgccaaacacgtggagtctggggaaaactggcaaaccctcacagggctgccactaggctgttccatcactgccagcatctgtccattttcagtattccataggacagtggtaccatctgttgaacacgatgccaaaatatgtcctgaaggggagaaacagcagcagtggacagcataggtatgaaacttcaatggagaatgtggcagttcagtaaagtcacgtaacgagtacaggcgaattgttttgtccaaggagcaagtagccaagagggaaaaggagaaggcacagcagttgacatcgtcaccatgatcagctaatgtgtgaatcagtttcaccatgttctttatttgaagaaaaacagcctgcaggagcgggggcgcgcgggatccgccttcaaggtgcccacgggcggtgcgggtcacgtgccgcgcaggtgaggctggcggggcgggcgccggcggagacccagagcagagggaacaggccccgcccccgaacgcccgcggggacccagagcggagggaacaggccccgccccccgaacgcccgctgtgacccagagcggagggagta

SEQ ID NO: 10131 - RNA, 861 nt, Homo sapiens
  source 1..861: mol_type = other RNA
cacggcaaaagaaacaatccaaattttgacttggcaatcctgaccacatgatgccagtcgaaaaaactgaagaccttgttctccatcagaaactggctgtgaagaaaaatcgcagcaggtaattccaagatcatgtgctttttcactatgcagacacctcattttatcatcccacactgttaaatcaccacatgaggagccagtgacaaagaagcttccattaggagaaaatgcacatgccgccaaggagccatctttaacactaccacatctatataatttgtatgactgtgcattccacaaaaccacagttccatcagctgcccctgatgccaaacacgtggagtctggggaaaactggcaaaccctcacagggctgccactaggctgttccatcactgccagcatctgtccattttcagtattccataggacagtggtaccatctgttgaacacgatgccaaaatatgtcctgaaggggagaaacagcagcagtggacagcataggtatgaaacttcaatggagaatgtggcagttcagtaaagtcacgtaacgagtacaggcgaattgttttgtccaaggagcaagtagccaagagggaaaaggagaaggcacagcagttgacatcgtcaccatgatcagctaatgtgtgaatcagtttcaccatgttctttatttgaagaaaaacagcctgccgccaccgccgctgagccggcccgtgggcgcggccgctctcacctgcaggagcgggggcgcgcgggatccgccttcaaggtgcccacgggcggtgcgggtcacgtgccgcgcaggtgaggctggcggggcgggcgccggcggagacccagagcagagggaacag

SEQ ID NO: 10132 - RNA, 484 nt, Homo sapiens
  source 1..484: mol_type = other RNA
cacggcaaaagaaacaatccaaattttgacttggcaatcctgaccacatgatgccagtcgaaaaaactgaagaccttgttctccatcagaaactggctgtgaagaaaaatcgcagcaggtaattccaagatcatgtgctttttcactatgcagacacctcattttatcatcccacactgttaaatcaccacatgaggagccagtgacaaagaagcttccattaggagaaaatgcacatgccgccaaggagccatctttaacactaccacatctatataatttgtatgactgtgcattccacaaaaccacagttccatcagctgcccctgatgccaaacacgtggagtctggggaaaactggcaaaccctcacagggctgccactaggctgttccatcactgccagcatctgtccattttcagtattccataggacagtggtaccatctgttgaacacgatgccaaaatatgtcctgcaggagcg

SEQ ID NO: 10133 - RNA, 594 nt, Homo sapiens
  source 1..594: mol_type = other RNA
cacggcaaaagaaacaatccaaattttgacttggcaatcctgaccacatgatgccagtcgaaaaaactgaagaccttgttctccatcagaaactggctgtgaagaaaaatcgcagcaggtaattccaagatcatgtgctttttcactatgcagacacctcattttatcatcccacactgttaaatcaccacatgaggagccagtgacaaagaagcttccattaggagaaaatgcacatgccgccaaggagccatctttaacactaccacatctatataatttgtatgactgtgcattccacaaaaccacagttccatcagctgcccctgatgccaaacacgtggagtctggggaaaactggcaaaccctcacagggctgccactaggctgttccatcactgccagcatctgtccattttcagtattccataggacagtggtaccatctgttgaacacgatgccaaaatatgtcctgcaggagcgggggcgcgcgggatccgccttcaaggtgcccacgggcggtgcgggtcacgtgccgcgcaggtgaggctggcggggcgggcgccggcggagacccagagcagagggaacag

SEQ ID NO: 10134 - RNA, 392 nt, Homo sapiens
  source 1..392: mol_type = other RNA
cacggcaaaagaaacaatccaaattttgacttggcaatcctgaccacatgatgccagtcgaaaaaactgaagaccttgttctccatcagaaactggctgtgaagaaaaatcgcagcaggtaattccaagatcatgtgctttttcactatgcagacacctcattttatcatcccacactgttaaatcaccacatgaggagccagtgacaaagaagcttccattaggagaaaatgcacatgccgccaaggagccatctttaacactaccacatctgcaggagcgggggcgcgcgggatccgccttcaaggtgcccacgggcggtgcgggtcacgtgccgcgcaggtgaggctggcggggcgggcgccggcggagacccagagcagagggaacag

SEQ ID NO: 10135 - RNA, 2024 nt, Homo sapiens
  source 1..2024: mol_type = other RNA
cacggcaaaagaaacaatccaagtacatactactaaattatacaaagttacattatttacgtttagtttattgcagagatgaagacagcatactagaagttggcttctatttcacaccgttcacagcactcactctgttctccatttcatccactcacccatgcaaaaggtctgtacacgcaatgatgtctgatgtttcttggtttccatagtgtaacaggaaacttgacatttcaattaaaaaggtaaaatgaagacatttaccatcagactataaaactcctcttctgtaagagaatactatagtacttgaagatatgatttgaaaaaaaatcatgtaccaaatgaaaggggcaccatttcaagagcactaggactacattaaacttaaatatattcccacattcttaaaaatgtaactcaaaaccaaatctagtcttaaaaaagctccagtaactaaaactacattaacaggcacgatgaacagtgtaaacactgttaatgggcaccaagtttaacagggcagacaatatttgcttctgcattcacacttattcaattacattttttaaaaaaatgatgctgcttaaactattaatgttttaccaaaaaaataataattttaataaatacagcaaatgctagaaatctagctaggttatcatgcaaggtataaccaagacaaactcaaatttataataaaggcaacttgcattcaaaatgaactctacccttatattttattaaaagggcaaacatcatgaattaacccagccgcttacttgaattacaaaagtaacatgattcaatatgaaaataagaaactgtctacaaatctctgacagtaataaattgcaatatacaatgcatacaggagtcatacagagcaacaaactctcgtacaaaacaaaaatattttaatacctttaaaatccaaatttttctttaaaatcattcatgaaaaagattctcaagtcagaattaacacctcaattagtcaagcatcaggaagctacattacagctattaatatacaaagatacatcttttcaccagtctttccttctgatgtctctgttccagaatcatacagactctcatttctctacactccccattccatcatttcttcagatcatgaaaactgaatttgctgaacaccagaaatctgttgatatgatgttgtgtaaaccataacattttgttgttgaccgtctgtggttattaagccagctggtaactggttagtaaatgcctcctctgtaagctcttcacttagtccatctgtagctgtgactgctccaccaattcccttttctcctttcatagcctctctgaatttctgaaggtataatttcagaggttccacataactgtcaaagcctaaagtagacatagcaaagagaatatcttctccattgattgttttccgtttctcttgatggcacctttcacttgcttcagatgttataaaactgatgaactcacttacacattcttgaacacattctttggcatcttttgcaatctttcccgtttgaggtatggcatttttcattatcctagccacgtttgctattggaagatatatatcttgttctctgaaactttcttttgaaccatttgtgtcttcatgatcattcatgctgtcctcagtatcatcatgaggctgtataacataatgacttcctccaatatagtctgcagagattcctagttgagaagcatctgttgtagaactgtcaccatccatcaggttcatgctatgtgctggtcacgtagctgtcaacaacagacaaggtctctgtcctcagcttgcaggacaaatgttacataactgtcatgaaatactgtcagaaccgtgttgtcagtggtgctgaagaacacctatctaaaaaggtgtctaatctttgtgatttcaacctccaatgcagccctggttggctcccgtctccaatcggctgtttggttggacagaaaatggctgcgaaggaaccagtcccagcgcggagctccgcttccag

SEQ ID NO: 10136 - RNA, 2679 nt, Homo sapiens
  source 1..2679: mol_type = other RNA
cacggcaaaagaaacaatccaagtacatactactaaattatacaaagttacattatttacgtttagtttattgcagagatgaagacagcatactagaagttggcttctatttcacaccgttcacagcactcactctgttctccatttcatccactcacccatgcaaaaggtctgtacacgcaatgatgtctgatgtttcttggtttccatagtgtaacaggaaacttgacatttcaattaaaaaggtaaaatgaagacatttaccatcagactataaaactcctcttctgtaagagaatactatagtacttgaagatatgatttgaaaaaaaatcatgtaccaaatgaaaggggcaccatttcaagagcactaggactacattaaacttaaatatattcccacattcttaaaaatgtaactcaaaaccaaatctagtcttaaaaaagctccagtaactaaaactacattaacaggcacgatgaacagtgtaaacactgttaatgggcaccaagtttaacagggcagacaatatttgcttctgcattcacacttattcaattacattttttaaaaaaatgatgctgcttaaactattaatgttttaccaaaaaaataataattttaataaatacagcaaatgctagaaatctagctaggttatcatgcaaggtataaccaagacaaactcaaatttataataaaggcaacttgcattcaaaatgaactctacccttatattttattaaaagggcaaacatcatgaattaacccagccgcttacttgaattacaaaagtaacatgattcaatatgaaaataagaaactgtctacaaatctctgacagtaataaattgcaatatacaatgcatacaggagtcatacagagcaacaaactctcgtacaaaacaaaaatattttaatacctttaaaatccaaatttttctttaaaatcattcatgaaaaagattctcaagtcagaattaacacctcaattagtcaagcatcaggaagctacattacagctattaatatacaaagatacatcttttcaccagtctttccttctgatgtctctgttccagaatcatacagactctcatttctctacactccccattccatcatttcttcagatcatgaaaactgaatttgctgaacaccagaaatctgttgatatgatgttgtgtaaaccataacattttgttgttgaccgtctgtggttattaagccagctggtaactggttagtaaatgcctcctctgtaagctcttcacttagtccatctgtagctgtgactgctccaccaattcccttttctcctttcatagcctctctgaatttctgaaggtataatttcagaggttccacataactgtcaaagcctaaagtagacatagcaaagagaatatcttctccattgattgttttccgtttctcttgatggcacctttcacttgcttcagatgttataaaactgatgaactcacttacacattcttgaacacattctttggcatcttttgcaatctttcccgtttgaggtatggcatttttcattatcctagccacgtttgctattggaagatatatatcttgttctctgaaactttcttttgaaccatttgtgtcttcatgatcattcatgctgtcctcagtatcatcatgaggctgtataacataatgacttcctccaatatagtctgcagagattcctagttgagaagcatctgttgtagaactgtcaccatccatcaggttcatgctatgtgctggtcacgtagctgtcaacaacagacaaggtctctgtcctcagcttgcaggacaaatgttacataactgtcatgaaatactgtcagaaccgtgttgtcagtggtgctgaagaacacctatctaaaaaggtgtctaatctttgtgatttcaaccttagtccaatccgaagggcttccttcccaccttcggggcaagtacagggaccgcaaaccgccagatggctgcattctttacgcgcaaaccaggctgcggggaagctaaagccatgccttcctccccacgcaggtgcctgggtggccccggccccacggcctggtcccggcgacctgtcagccctgcgagtgccaggaggccgcccccagagcgcatcccctgactcgcccggccgccccggccccgcgcccaacgcctgcctcccacccgccgcgcggcccccgggatgtgcgggcagacaaagcgccgggccccgccacagccccgcgggcgggaggagggcgcccccggggactcgcgccgccgccggggctacggggccagggcccgggccgcgtctcccgcccctcggccggctccccgcacaaaatggagccggcccgggacgccgtcgagagcggggccccgacgcagccccgcggcccctcctcggccccgggcccggagctcaacggcggcgagggtgaggtggcctggcccgcgtcccgccgctcctcagcccggcgcacaaagagccgcgccgcggccccgcgcccgctccccggcccggcccgctgcgggagcggcctcgcaggcgcggggcccggcctcggcccgcgcgggagggcgggaggctagtgcccccggccgcggcggcgttggcggcggggacggcgccgggaggagacggacatttcattcgagctaaagtggag

SEQ ID NO: 10137 - RNA, 2007 nt, Homo sapiens
  source 1..2007: mol_type = other RNA
cacggcaaaagaaacaatccaagtacatactactaaattatacaaagttacattatttacgtttagtttattgcagagatgaagacagcatactagaagttggcttctatttcacaccgttcacagcactcactctgttctccatttcatccactcacccatgcaaaaggtctgtacacgcaatgatgtctgatgtttcttggtttccatagtgtaacaggaaacttgacatttcaattaaaaaggtaaaatgaagacatttaccatcagactataaaactcctcttctgtaagagaatactatagtacttgaagatatgatttgaaaaaaaatcatgtaccaaatgaaaggggcaccatttcaagagcactaggactacattaaacttaaatatattcccacattcttaaaaatgtaactcaaaaccaaatctagtcttaaaaaagctccagtaactaaaactacattaacaggcacgatgaacagtgtaaacactgttaatgggcaccaagtttaacagggcagacaatatttgcttctgcattcacacttattcaattacattttttaaaaaaatgatgctgcttaaactattaatgttttaccaaaaaaataataattttaataaatacagcaaatgctagaaatctagctaggttatcatgcaaggtataaccaagacaaactcaaatttataataaaggcaacttgcattcaaaatgaactctacccttatattttattaaaagggcaaacatcatgaattaacccagccgcttacttgaattacaaaagtaacatgattcaatatgaaaataagaaactgtctacaaatctctgacagtaataaattgcaatatacaatgcatacaggagtcatacagagcaacaaactctcgtacaaaacaaaaatattttaatacctttaaaatccaaatttttctttaaaatcattcatgaaaaagattctcaagtcagaattaacacctcaattagtcaagcatcaggaagctacattacagctattaatatacaaagatacatcttttcaccagtctttccttctgatgtctctgttccagaatcatacagactctcatttctctacactccccattccatcatttcttcagatcatgaaaactgaatttgctgaacaccagaaatctgttgatatgatgttgtgtaaaccataacattttgttgttgaccgtctgtggttattaagccagctggtaactggttagtaaatgcctcctctgtaagctcttcacttagtccatctgtagctgtgactgctccaccaattcccttttctcctttcatagcctctctgaatttctgaaggtataatttcagaggttccacataactgtcaaagcctaaagtagacatagcaaagagaatatcttctccattgattgttttccgtttctcttgatggcacctttcacttgcttcagatgttataaaactgatgaactcacttacacattcttgaacacattctttggcatcttttgcaatctttcccgtttgaggtatggcatttttcattatcctagccacgtttgctattggaagatatatatcttgttctctgaaactttcttttgaaccatttgtgtcttcatgatcattcatgctgtcctcagtatcatcatgaggctgtataacataatgacttcctccaatatagtctgcagagattcctagttgagaagcatctgttgtagaactgtcaccatccatcaggttcatgctatgtgctggtcacgtagctgtcaacaacagacaaggtctctgtcctcagcttgcaggacaaatgttacataactgtcatgaaatactgtcagaaccgtgttgtcagtggtgctgaagaacacctatctaaaaaggtgtctaatctttgtgatttcaaccttcggggcaagtacagggaccgcaaaccgccagatggctgcattctttacgcgcaaaccaggctgcggggaagctaaagccat

SEQ ID NO: 10138 - RNA, 1908 nt, Homo sapiens
  source 1..1908: mol_type = other RNA
cacggcaaaagaaacaatccaagtacatactactaaattatacaaagttacattatttacgtttagtttattgcagagatgaagacagcatactagaagttggcttctatttcacaccgttcacagcactcactctgttctccatttcatccactcacccatgcaaaaggtctgtacacgcaatgatgtctgatgtttcttggtttccatagtgtaacaggaaacttgacatttcaattaaaaaggtaaaatgaagacatttaccatcagactataaaactcctcttctgtaagagaatactatagtacttgaagatatgatttgaaaaaaaatcatgtaccaaatgaaaggggcaccatttcaagagcactaggactacattaaacttaaatatattcccacattcttaaaaatgtaactcaaaaccaaatctagtcttaaaaaagctccagtaactaaaactacattaacaggcacgatgaacagtgtaaacactgttaatgggcaccaagtttaacagggcagacaatatttgcttctgcattcacacttattcaattacattttttaaaaaaatgatgctgcttaaactattaatgttttaccaaaaaaataataattttaataaatacagcaaatgctagaaatctagctaggttatcatgcaaggtataaccaagacaaactcaaatttataataaaggcaacttgcattcaaaatgaactctacccttatattttattaaaagggcaaacatcatgaattaacccagccgcttacttgaattacaaaagtaacatgattcaatatgaaaataagaaactgtctacaaatctctgacagtaataaattgcaatatacaatgcatacaggagtcatacagagcaacaaactctcgtacaaaacaaaaatattttaatacctttaaaatccaaatttttctttaaaatcattcatgaaaaagattctcaagtcagaattaacacctcaattagtcaagcatcaggaagctacattacagctattaatatacaaagatacatcttttcaccagtctttccttctgatgtctctgttccagaatcatacagactctcatttctctacactccccattccatcatttcttcagatcatgaaaactgaatttgctgaacaccagaaatctgttgatatgatgttgtgtaaaccataacattttgttgttgaccgtctgtggttattaagccagctggtaactggttagtaaatgcctcctctgtaagctcttcacttagtccatctgtagctgtgactgctccaccaattcccttttctcctttcatagcctctctgaatttctgaaggtataatttcagaggttccacataactgtcaaagcctaaagtagacatagcaaagagaatatcttctccattgattgttttccgtttctcttgatggcacctttcacttgcttcagatgttataaaactgatgaactcacttacacattcttgaacacattctttggcatcttttgcaatctttcccgtttgaggtatggcatttttcattatcctagccacgtttgctattggaagatatatatcttgttctctgaaactttcttttgaaccatttgtgtcttcatgatcattcatgctgtcctcagtatcatcatgaggctgtataacataatgacttcctccaatatagtctgcagagattcctagttgagaagcatctgttgtagaactgtcaccatccattgtcatgaaatactgtcagaaccgtgttgtcagtggtgctgaagaacacctatctaaaaaggtgtctaatctttgtgatttcaacctccaatgcagccctggttggctcccgtctccaatcggctgtttggttggacagaaaatggctgcgaagg

SEQ ID NO: 10139 - RNA, 2506 nt, Homo sapiens
  source 1..2506: mol_type = other RNA
cacggcaaaagaaacaatccaagtacatactactaaattatacaaagttacattatttacgtttagtttattgcagagatgaagacagcatactagaagttggcttctatttcacaccgttcacagcactcactctgttctccatttcatccactcacccatgcaaaaggtctgtacacgcaatgatgtctgatgtttcttggtttccatagtgtaacaggaaacttgacatttcaattaaaaaggtaaaatgaagacatttaccatcagactataaaactcctcttctgtaagagaatactatagtacttgaagatatgatttgaaaaaaaatcatgtaccaaatgaaaggggcaccatttcaagagcactaggactacattaaacttaaatatattcccacattcttaaaaatgtaactcaaaaccaaatctagtcttaaaaaagctccagtaactaaaactacattaacaggcacgatgaacagtgtaaacactgttaatgggcaccaagtttaacagggcagacaatatttgcttctgcattcacacttattcaattacattttttaaaaaaatgatgctgcttaaactattaatgttttaccaaaaaaataataattttaataaatacagcaaatgctagaaatctagctaggttatcatgcaaggtataaccaagacaaactcaaatttataataaaggcaacttgcattcaaaatgaactctacccttatattttattaaaagggcaaacatcatgaattaacccagccgcttacttgaattacaaaagtaacatgattcaatatgaaaataagaaactgtctacaaatctctgacagtaataaattgcaatatacaatgcatacaggagtcatacagagcaacaaactctcgtacaaaacaaaaatattttaatacctttaaaatccaaatttttctttaaaatcattcatgaaaaagattctcaagtcagaattaacacctcaattagtcaagcatcaggaagctacattacagctattaatatacaaagatacatcttttcaccagtctttccttctgatgtctctgttccagaatcatacagactctcatttctctacactccccattccatcatttcttcagatcatgaaaactgaatttgctgaacaccagaaatctgttgatatgatgttgtgtaaaccataacattttgttgttgaccgtctgtggttattaagccagctggtaactggttagtaaatgcctcctctgtaagctcttcacttagtccatctgtagctgtgactgctccaccaattcccttttctcctttcatagcctctctgaatttctgaaggtataatttcagaggttccacataactgtcaaagcctaaagtagacatagcaaagagaatatcttctccattgattgttttccgtttctcttgatggcacctttcacttgcttcagatgttataaaactgatgaactcacttacacattcttgaacacattctttggcatcttttgcaatctttcccgtttgaggtatggcatttttcattatcctagccacgtttgctattggaagatatatatcttgttctctgaaactttcttttgaaccatttgtgtcttcatgatcattcatgctgtcctcagtatcatcatgaggctgtataacataatgacttcctccaatatagtctgcagagattcctagttgagaagcatctgttgtagaactgtcaccatccattgtcatgaaatactgtcagaaccgtgttgtcagtggtgctgaagaacacctatctaaaaaggtgtctaatctttgtgatttcaaccttagtccaatccgaagggcttccttcccaccttcggggcaagtacagggaccgcaaaccgccagatggctgcattctttacgcgcaaaccaggctgcggggaagctaaagccatgccttcctccccacgcaggtgcctgggtggccccggccccacggcctggtcccggcgacctgtcagccctgcgagtgccaggaggccgcccccagagcgcatcccctgactcgcccggccgccccggccccgcgcccaacgcctgcctcccacccgccgcgcggcccccgggatgtgcgggcagacaaagcgccgggccccgccacagccccgcgggcgggaggagggcgcccccggggactcgcgccgccgccggggctacggggccagggcccgggccgcgtctcccgcccctcggccggctccccgcacaaaatggagccggcccgggacgccgtcgagagcggggccccgacgcagccccgcggcccctcctcggccccgggcccggagctcaacggcggcgagggtgaggtggcctggcccgcgtcccgccgctcctcagcccggcgcacaaagagccgcgccgcggccccgcgcccgctccccggcccggcccgctgcgggagcggcctcgcaggcgcggggcccggcctcggcccgcgcgggaggg

SEQ ID NO: 10140 - RNA, 2511 nt, Homo sapiens
  source 1..2511: mol_type = other RNA
cacggcaaaagaaacaatccaagtacatactactaaattatacaaagttacattatttacgtttagtttattgcagagatgaagacagcatactagaagttggcttctatttcacaccgttcacagcactcactctgttctccatttcatccactcacccatgcaaaaggtctgtacacgcaatgatgtctgatgtttcttggtttccatagtgtaacaggaaacttgacatttcaattaaaaaggtaaaatgaagacatttaccatcagactataaaactcctcttctgtaagagaatactatagtacttgaagatatgatttgaaaaaaaatcatgtaccaaatgaaaggggcaccatttcaagagcactaggactacattaaacttaaatatattcccacattcttaaaaatgtaactcaaaaccaaatctagtcttaaaaaagctccagtaactaaaactacattaacaggcacgatgaacagtgtaaacactgttaatgggcaccaagtttaacagggcagacaatatttgcttctgcattcacacttattcaattacattttttaaaaaaatgatgctgcttaaactattaatgttttaccaaaaaaataataattttaataaatacagcaaatgctagaaatctagctaggttatcatgcaaggtataaccaagacaaactcaaatttataataaaggcaacttgcattcaaaatgaactctacccttatattttattaaaagggcaaacatcatgaattaacccagccgcttacttgaattacaaaagtaacatgattcaatatgaaaataagaaactgtctacaaatctctgacagtaataaattgcaatatacaatgcatacaggagtcatacagagcaacaaactctcgtacaaaacaaaaatattttaatacctttaaaatccaaatttttctttaaaatcattcatgaaaaagattctcaagtcagaattaacacctcaattagtcaagcatcaggaagctacattacagctattaatatacaaagatacatcttttcaccagtctttccttctgatgtctctgttccagaatcatacagactctcatttctctacactccccattccatcatttcttcagatcatgaaaactgaatttgctgaacaccagaaatctgttgatatgatgttgtgtaaaccataacattttgttgttgaccgtctgtggttattaagccagctggtaactggttagtaaatgcctcctctgtaagctcttcacttagtccatctgtagctgtgactgctccaccaattcccttttctcctttcatagcctctctgaatttctgaaggtataatttcagaggttccacataactgtcaaagcctaaagtagacatagcaaagagaatatcttctccattgattgttttccgtttctcttgatggcacctttcacttgcttcagatgttataaaactgatgaactcacttacacattcttgaacacattctttggcatcttttgcaatctttcccgtttgaggtatggcatttttcattatcctagccacgtttgctattggaagatatatatcttgttctctgaaactttcttttgaaccatttgtgtcttcatgatcattcatgctgtcctcagtatcatcatgaggctgtataacataatgacttcctccaatatagtctgcagagattcctagttgagaagcatctgttgtagaactgtcaccatccattgtcatgaaatactgtcagaaccgtgttgtcagtggtgctgaagaacacctatctaaaaaggtgtctaatctttgtgatttcaaccttcggggcaagtacagggaccgcaaaccgccagatggctgcattctttacgcgcaaaccaggctgcggggaagctaaagccatgccttcctccccacgcaggtgcctgggtggccccggccccacggcctggtcccggcgacctgtcagccctgcgagtgccaggaggccgcccccagagcgcatcccctgactcgcccggccgccccggccccgcgcccaacgcctgcctcccacccgccgcgcggcccccgggatgtgcgggcagacaaagcgccgggccccgccacagccccgcgggcgggaggagggcgcccccggggactcgcgccgccgccggggctacggggccagggcccgggccgcgtctcccgcccctcggccggctccccgcacaaaatggagccggcccgggacgccgtcgagagcggggccccgacgcagccccgcggcccctcctcggccccgggcccggagctcaacggcggcgagggtgaggtggcctggcccgcgtcccgccgctcctcagcccggcgcacaaagagccgcgccgcggccccgcgcccgctccccggcccggcccgctgcgggagcggcctcgcaggcgcggggcccggcctcggcccgcgcgggagggcgggaggctagtgcccccggccgcggcggcgttggc

SEQ ID NO: 10141 - RNA, 2970 nt, Homo sapiens
  source 1..2970: mol_type = other RNA
cacggcaaaagaaacaatccagcctggcttgccctaatgaaggcagcaagacaaggtccaaaccatctgtaccaaaaacgtcacgaattcagatgtaacttaggtggtcattgcacctttaagtctcttcttttgggtaggtattgtgttttacatgaatttgcagaaagagatcacaatctaataaaagtctcaagtttaatcctgaaaaggaagcagatttatgtgtgaagctttctctgggctctaatttcctaatcacatatatattaatgctgatagaacttgtctttgagaggtacagctcttaccaatcttaggaagtggtaaaagattctgctacttcactctctttttacatttttggttcatatcagtatcctatcagagtttacattgccaatatgaatactggcatttgcaggaattatgacaaatgttagtggtttgggcagcaatgtgctaagaaatgtttaacaaatgactctccagaaaaaaaagtatgcacatatatggatacataagtttagcataaatgttataatacataggacacaagttacaaatagtaacaaaatatgtgatattctttattgtaaattttacacagccaattgatttttgaagactgttcccttgatttttgtcaaactctggtatttattgccaatgtgctggtaataattgatcaactactacagcacattctgacatgaatattggtattttaatttacattcataagacaaaacaataaatatattggaacgtcactaattcaccaatggccaacttctttgctgattcaaataattgttttcaagcactaagataatatttcttaattttgtttgtactattaataatgttacagctactgacatgagtttgaaatttatctatatttttaatattttctccattactttcttaaccctagactaagggtcaccaactacagcccacagggtaaatctggcctaccacctgtctttctaaataaagtttgatggagtactactagcttatttgtttgtgtattgtccgtgtctacttttatgttagaaccacagagttgagtagttgctgcagaaaacatatggtgcacaaagtataaatatttattctctggccctatagaggagatttgtattttcagtcaaaataataaattgagccttgatttgtggtgtttgctggtttccatagtataaacatttccactctgttttcaagttatcaatgcaatatgactaacgataacagctaagtatagagttggggagaaatgctcagtagcacatcattggatggaatttacgccatacccatgcaagggggcggtaagcaagtccaagaacataagagtaaaatgtggtaaattttacttaagttatgaagttgtagattgaattgtctctctcaaaaaagatatgttgaaattctaaaacctttggtacctgtgaatgtggactttatttggaaatagggtctttgcaaacgtaatgaagttaagatgaggtcatactggataatggtgagtcccaatttcagtggagagaaagatttgatgacagagaagagacacacggaaggccctgattgtgttgcctcatcttttgatgtgattcctgtttcagtcaagactggctcaagtagtgcatgggactgaatatcagttgcccaatcttggacttctgctgttgtttggagtctattaccatttaatgttctaggcctgacttctaggcattttcttattgttttcagtcacatagagagagctcagaggaaggaaagcggcaacttgatgaagattatactgatgttctttggcaacataggtcctcctttggcagaagaggccatcttcactatggggtgcagattcttagaaaataatattggaattcctctaggttgaatattaaaatagccatgacacttgaggaaatcactcttagggtccatgcttaaattagattcttgtaaagttgcatgatgtttctaggtatgcatctcagagaaacaaaaatatatgtccacaaaagccttgtacaaggatattcacggcagccttactagtaagagctacaacctagaaacaatcctctctcttgtctaactagaaaaggatagattattgaataaagggtacgtttatttataatggaatactacatgggagtaaaaagggggacaaagatctacattggttaatctcagagatctacattggttatgttgaaggacagaattcaggctcaataggccatgtattctatacttccacttcttcaaagttctagaacctgcaaagcaaatcaatggtgatgaaaatcagaagagttcttgctttgagtgaggggagtgaactgggtgtgaagaagcatgagaaatatttctagaataaaggaaatgccctatatcttaacaggcatgtaggttactggtgtatatatttgttaaaattgattgtgttcttaagatctatgcattcactctgtgtaaattatacctcactataaagtcaccaggtactttggagaaaataatgatttttaagttacttttttatacataataatttgccttcctccaattctcttaattttttcacaatacaatcccatctactatattattttatcctgtggttaataaagcatggatggaaggcttctgacaagaaggcttctgacgagagtagggagcactagaagtctgtctccctacctacacaaaaattgcactggcagaatcagtctgatgtaaatattttgaaactctggagtctgttgaaggcttgcaacttccaagggaaggcttagatggtacatttcagttaatttatgaccatttcacctcatagcacagtaagagctacccatcccttgtccccagcagctcacacacagattgcagggccagggttgatgaaaaataaccctgctttccaaatgtcagaga

SEQ ID NO: 10142 - RNA, 775 nt, Homo sapiens
  source 1..775: mol_type = other RNA
cactgcaggactcagcagggcggggccagggaggaggggctgggggaggccgcaggcgggtgcactggagggcccaagcctgcctccctggccaggtgctgctgggacatgcccagagggcacactcagagagctggaggaagaggtgcatgtgctcccagcccacccacagagccctagcagagtggaggccatgctgtgtagggagcagcagctccagccaagcctcagcccagtctccagctcaatcttgcaggcaaagagcaaaacccaccaaaactcagaattaaaacaatcccccctctgcccccagcaaaaattgagtgccgacatctgtgccccacactgacagggagcagacatcacagattttgtccagacatgttatttaacaaacaaaactccaataactgccctctggaatccagagttgatgtgaagtgtccagtattcaacaaaactcatgagacacaccagggaacaagagtaaccccttttcattcttaggggcaaatacaggatacttggcatgtatgtggggccctctctaaccacaaggacgtgacaactcaggcagactcagacgttctgatgatgcagtgtcatcaacacgcagacaccacatatcctaatacgaactctttcttgatgaacttttgggaaaattaatgtctgcaagttaaatctccctgcttttgcaagccgaggcccaaagaaataaaattaaattcaaatctgagtttgggccaggcgcggtgtctcacacctgtaattt

SEQ ID NO: 10143 - RNA, 781 nt, Homo sapiens
  source 1..781: mol_type = other RNA
cactgcaggactcagcagggcggggccagggaggaggggctgggggaggccgcaggcgggtgcactggagggcccaagcctgcctccctggccaggtgctgctgggacatgcccagagggcacactcagagagctggaggaagaggtgcatgtgctcccagcccacccacagagccctagcagagtggaggccatgctgtgtagggagcagcagctccagccaagcctcagcccagtctccagctcaatcttgcaggcaaagagcaaaacccaccaaaactcagaattaaaacaatcccccctctgcccccagcaaaaattgagtgccgacatctgtgccccacactgacagggagcagacatcacagattttgtccagacatgttatttaacaaacaaaactccaataactgccctctggaatccagagttgatgtgaagtgtccagtattcaacaaaactcatgagacacaccagggaacaagagtaaccccttttcattcttaggggcaaatacaggatacttggcatgtatgtggggccctctctaaccacaaggacgtgacaactcaggcagactcagacgttctgatgatgcagtgtcatcaacacgcagacaccacatatcctaatacgaactctttcttgatgaacttttgggaaaattaatgtctgcaagttaaatctccctgcttttgcaagccgaggcccaaagaaataaaattaaattcaaatctgagtttgggccaggcgcggtgtctcacacctgtaatttcagcac

SEQ ID NO: 10144 - RNA, 1169 nt, Homo sapiens
  source 1..1169: mol_type = other RNA
cactgtaggtgatggtgagagtgggcatagtgggcagagggggtggcagcaccttcaggttctggtcactctggatctcgttggtagagatctggttgatgatgcggttgtaggtgggtggttggtagacccggggcggggcagcggggggtggctgggggacgggcctggccgagggcaccctctggcagtgctcctcaagctgcgcgatgatctctgattggttgtgggccagtgtggccaggtgctggtacttgtgctccaggtccttgtacttgctggccagctgcagcatgtcggctgtctggttcaggatcctgttctccagctgggagagctccaacgcgttgtcccgcttgcggatgatctcgtgcaggagctgcatgtagagctgcgtgacccgcgagttcatgttgcggctctccttgcgcagcagcttcacctcgctcacaatgccgccgtccacctccaccagctgctgcagcgtctcgatctgccgcttctgcttgagcagctcattgttgagcagctctagctcctgcttatgcactcggttctccagaagcacctcaggctccttggagttgacgcagatggcacccgtgacccgctgctggggcacaatgaaggtgtaggtgcacttgtcctgggactcgcccgcccgcttgtacctgtttaggtaaatgaactctcttggcgagccctcctcagtgccctcaaaaccgtcctcctggcctgcaacagctcccatggcagccagcagtccgagccaccagcatgtcacgcacagtggcctcatggtccttgcaaaatggtggttattctttgtgaatagaatctatgaaagcctcttccctcctgcttggctccggggcggctcctcacatgcttcaccctggccgtcagcggggcagcctgtccatggcctctggaggggttcctgagttgcaggccggtggctgccaagcagccctgcctcactgggctccactggctctgcctccacagagggctccggcagaggctggggccagggctggccaggggtcctgcggggctgctcacaaccttctttccctcacagtagcgtcagccgctgcctcagtgccacgctcggcaggtccagggcttggggtccatcctcaggccgtccgcagcagcctcatttg

SEQ ID NO: 10145 - RNA, 1218 nt, Homo sapiens
  source 1..1218: mol_type = other RNA
cactgtaggtgatggtgagagtgggcatagtgggcagagggggtggcagcaccttcaggttctggtcactctggatctcgttggtagagatctggttgatgatgcggttgtaggtgggtggttggtagacccggggcggggcagcggggggtggctgggggacgggcctggccgagggcaccctctggcagtgctcctcaagctgcgcgatgatctctgattggttgtgggccagtgtggccaggtgctggtacttgtgctccaggtccttgtacttgctggccagctgcagcatgtcggctgtctggttcaggatcctgttctccagctgggagagctccaacgcgttgtcccgcttgcggatgatctcgtgcaggagctgcatgtagagctgcgtgacccgcgagttcatgttgcggctctccttgcgcagcagcttcacctcgctcacaatgccgccgtccacctccaccagctgctgcagcgtctcgatctgccgcttctgcttgagcagctcattgttgagcagctctagctcctgcttatgcactcggttctccagaagcacctcaggctccttggagttgacgcagatggcacccgtgacccgctgctggggcacaatgaaggtgtaggtgcacttgtcctgggactcgcccgcccgcttgtacctgtttaggtaaatgaactctcttggcgagccctcctcagtgccctcaaaaccgtcctcctggcctgcaacagctcccatggcagccagcagtccgagccaccagcatgtcacgcacagtggcctcatggtccttgcaaaatggtggttattctttgtgaatagaatctatgaaagcctcttccctcctgcttggctccggggcggctcctcacatgcttcaccctggccgtcagcggggcagcctgtccatggcctctggaggggttcctgagttgcaggccggtggctgccaagcagccctgcctcactgggctccactggctctgcctccacagagggctccggcagaggctggggccagggctggccaggggtcctgcggggctgctcacaaccttctttccctcacagtagcgtcagccgctgcctcagtgccacgctcggcaggtccagggcttggggtccatcctcaggccgtccgcagcagcctcatttgaactcccaactcctttgtggagcctttacatgccgccagaggaaactgt

SEQ ID NO: 10146 - RNA, 29 nt, Homo sapiens
  source 1..29: mol_type = other RNA
cactgtttcaccactggctctttcattca

SEQ ID NO: 10147 - RNA, 32 nt, Homo sapiens
  source 1..32: mol_type = other RNA
cacttagcaggttgtattatatccatccgagt

SEQ ID NO: 10148 - RNA, 31 nt, Homo sapiens
  source 1..31: mol_type = other RNA
cagaacaggagcatagaaaggctggggagca

SEQ ID NO: 10149 - RNA, 539 nt, Homo sapiens
  source 1..539: mol_type = other RNA
cagcaccctgtggctcccacagacttaagtcagatgtgtaattttcaagtttccaaaggcatacagtgaattgatggcagagccggaattgcaggcgagcatccttagaggttgtctattgttcagcacactcagcgcaaggcctctcggcagtgtgttttttcttccaagcatcacattttcttattccttcgctaaacaattcttagaagtaagatttctttctccagctttcaggaataacacttaaatacatatttatctaattttgtggttttgtataaaaagtattcagtcacattcttcctggagaggctacttgtatctcctttctccttattccatggtgttcttcctctgctacgctaagttccaacagggtgatctggaaaacgcgccactggctccctggcgggcttccggactcgccttttcgcgccctcggcggcggctcttttctccaggggggaccacctagcgctcggctttgcacggccaatttatggcgctgtcaggggctcgggcgccgcgcccattgt

SEQ ID NO: 10150 - RNA, 1932 nt, Homo sapiens
  source 1..1932: mol_type = other RNA
cagcaggaggtgaggggagaaagagaactagagaaaggcaatgatgtggttgaagggtgagagaaaaagacctacttacagaccagtagcaactttccaccactgaggactgaaatttcaactactgtgtttttttctccaatgtattcccttttctgaaaataagaataaaaggacattacacataacagacacaacaaaataaccgcagttgtatttttaatgatacaaaattcatgacatattgagttgtgtgttcagaaacatacatttttcactttaaaatctgctttaaggaatgtcagtgttttggacaaaatatgattataagcatggaataaaacgagagagggccaagaatatttctgagaaaagggtgaaaaggaagatagacttaaattaaaaccgatgtttttgaaaagcacacacaatatctagtgtacccagtttgaggttataagtcacagatatgaatttcagcccactcactcattaagtgattaataaattatcttattttagatattcagagatccagtggtccttgttagcaccctttcttcaacaacctctgcattccctgcttaatttcttgggttctcaccccgtaaatgatggggttaagggctgcaggaatgacatggtggagaacattgagcaagactggcacatcaggggagactttcttcttagccacatgtgtgaggacaaaaaccagaaggatggtgctgaagaagaggatgagcatgaagtgggagccacatgtgcttagggcctttgccacggcaccctctgccttgagtctcagcacagctcgcagaatgaaggtgtaggagaggaagataaggatgaggtcagatcctagcagagtccagcctccagcaaattggtaaaggtgattgatggtgacatcatcgcaggagagtctggaaacagacatattggcacagatgcagttctcaatgacatttcttccacaataacggagttgtgctgaaaggatggggatgggcagagtcataagcacatttctggtcaaaataaacatggcagccttgactacaaagtgatcagtgatgattgatggatatctcagtgggtggcagatggctacataacgatcataggccatgaccatgaatgtgcaagactccatggctaggaaacaattcatgatgtacatctggaggaagcaggcagggaagctgatgggcctgaggtcaaaccagaagatggtcaggaccttggggatgacagtgaggcagagcacgatgtccagcagggagaggaggctgagcaggtagtacaggggctggtgcagagaggcctccagccagatggtcatcaggagggtggtgttggcccctacggccaagaggaaaaggaggctgaggggcagggacagccagtgctgccagctgggggatctgacaaaacaattcaagaggaagtctgaagcttcagtggagagggtgtcatttcggtgtgttgtcatattttcccatatattttactgctttctttcagtgattttttggaagaggttcaggtaggctttttgttttcagttgtctttcctattccccaaaagcagttccagtccttgctcaactgggtcctgtcagattctcctcatcagaaagaccctgttagtaactgtggctgctgtcagtggagggaggacgggcattcctccagggatcctctcttcactcctcttgatcctctgattccccatgtagtctgccaggcatggcccttcacctcatatatagaagagatttagatattctcccaattcttttctcctgagacagggtgcagtctttatttatttccttctcagactacttcagcagtattgacgcaggaatggaaaagagcacagatagggactgaagacagagatctctctagtcttctggctaatct

SEQ ID NO: 10151 - RNA, 5014 nt, Homo sapiens
  source 1..5014: mol_type = other RNA
cagcaggaggtgaggggagacattccctgctataagcacttctttctggatccttcaatttctctgggaggcggggactttttcttttactcctcctaccattatgtagttttgagagagaaataacacaggtgccaagtaacccagctcagaaataaggctcttgatttctaggtagaacccaagcaattcttgacctcttgtgcaaaagggcattaatatatatcaaatgctttttatgtgcaaggcttcatatactatttctttaatttctccaaccactttatgaagtaggaaatcttccctttttacagatgaggaaactcaagcctactgtcacgtgacagagttgggctttgaatcaaagtctgactctactgcaccatgtggcctcctgtgagaatggtatgtgtgttatgggtgaagggtcaaaggaagacgtgactcatctcttctaaaatatcttaaataagttcaatttacaaaaagtaggacaatcagaatgctttggatattacctagccaacttagtgactgtactgcttgtgagtgagtgtgtgtgtatgtgagagagagagagacagagaaataggggagaggaataggcaggataagagagaatggggcagtggggagaagtgggggagaggtgggcagagagagaggtacaatatatacaggggtcgggctagcccctttgggtctggctgtgggtcatattctgctgctgtctctcccctactttaggagttgggatttctcaaatcctcatcttcaaaggactacaaaggaggttactgtaaaactttacctaaagaaagcaagactgacttgactattcaaaatgaaatgaaacaaaagctcctcagttgcatataaatgttccttgagtcaggtccaggtggagctctgttcaggaggtagtaggcctccgctgtttgggcctttgacctgctagtatgtcctggcttgccccatttgaagtgttagtgataaagacaacgaagggcattcatctcgcccaaggtgcagtctttgcctttggaaccacagagctagtctgaccagaaatttcccacatgaactcattgtatctgcctctgcccataacttgcctgctgcctctcacagttcccatatttccctggagggaagagggagaagggacctttttgctccaactttgaacatttcctccatgttccattctacccagcaactccctaattttttatattgcattttaaaaatgagatttccactaaaatcccagtggaaggagattctctctgactcactgctcccccaatttgttctgggctcatgatttatgtcccatcactccgctttcaagactgaattttctcaggttgagaccctttcatttccatttccctctttcctcctgagcccactctgagccttgtgtctgggtaggattatagaacatggaaagtttctccttgcttacagctttcagttgtctttaaatggaaagtaggaaaagaagtagcgtcaggatggcataatgtctaagaagaacattgcctctagagccaggctgctggtgttgaaatcctgactctgccacttactagctgtctgatcttaggcaaattacctaatctcactcagcttcaatttcctcatctgtaaaatggggttaataacagtacctacctcatagggttcttgtgaaggcttcggagtcaatcagtagagtgtttagaacagcacctggcacatagtgcttgagcattatgagctctgcctccccacccagcctgcttccttctcccctcaagtcatccactgatgaccccctgagtaaagctgaaggagagaggctgctgagtcttagctatgactctgggttccatgactgtatgaaagaaggctctcagcagcaagggagagaacacttgtctttcagacactggcacaccattgagagggactgcagtcagagcagggatctgtgtgtggctccacctcgaattttaggcctggtaaggcttgattttgtgctgctatagctcccacctgctctgtgctcatctctcaaaaggggacaagtatctgaagaagttaatacatgaggctgagtctgtttttcttttctttccctacgacctgcagtggtggttttgaagtttcctaagtaacaagctggggactcctctgaggaagggagagaatcgtttgccttctgctacagaaacgggaggcctcaggaagaaggggttcttgcccgtgagccagctggagggccccagagaacattctgctctgattggatacatcttaccaagctctctcccactgcagggtttttctaacagtgaagcaatggttcagataacatttgctgcccagtgccctagaaggggaaatgacaaacaagttcaagaatgttttgggctgggcgtggtggctcacgcctgtaatcccagcactttgggaggccgaggcgggtggatcgcgaggtcaggagatagagaccatcctggctaacatggtcaaaacccgtctctactaaaaatacaaaacgttagccgggtgtggtggtgggcgcctgtagtcccagcttctcgggaggctgaggcaggagaatggcatgaacccaggagacggagcttgcggtgagccaagatcgcgccactgcactccagcctgggcgcaaggcaagactccgtctcaaaaaaaaaaaaaaaaggatgttttgtaccctgctacccacccctcatcctgtaaggaaaatccagctacacttgcttaaagtgtaagctggtttctgttgtgctcgtgctgccctctgctgtcacctcagggtagaggaaccagttaaaacagccagttcatcactgaatttaggatttacttttctgaaagactttggagagctgggcaggggcccgggttaggaaaggaagaacttctacccccaacccactgcccaaggcctgtcctcagtccctacctagcttctagggaaactattacacagtcctaaaaggatgcctggaaacaccgcaggatttgtcaaactcacccacctcagagtcctgtccctagaactgtgggaaaacatttcctccttttattaggtcccagtttcagctaactagaggagcttttcccttgactttaaccatgccctggctcaagttcactcgcatatgtccctttgctcccgacgctgggtcaactcctgattgctcagtaggtagtcatcaatgaatgtgaagatttcctcgggggtgacaggttccatgtagcggtctcggtcaataccctgcttgtcaatcaacaccatgttgaagtaggagcgagtgaggcgctgaaattgcctgagctcctcgatgatgttggctgacagctgttgctcccggatgcgccccacctcctgaggtggctgtcccaccagttcaatgatggtcacatgccgcaaatccagtccacaggtggattgctgtagcatagagatctgcattttataatatcggttggaaggatcaggagctgagatgatgaggagtcgctgtttctcatagaattgatccaagagaccagcagctgagttgacgttgacgttaatcttcataggagcacagattggtggtgaacctgaccactggcggctggactgacagacccgggagggtgtcccctggcgatcataaccgccatcacagtggtattcacaggtggcaccatagttgtcccccgctgaggtgcaggtgaggtagccgtgctgcggaggtttcagagttgggcagcgtctcacttgtactttcacaatgaacttgcagctggcccggttgtaggctcggtcataggcagtgtaacgaatcacatgctctccttcgggaaagtgagagccaggctcagggccccgaagtgtcaccctggtgatggtaccatcagcagaatctttcaccaacggtgggtcccagtatactcgagcagtcaatttctctggctctgccatcttctcacgtgagtggggacagcggatcttggggggatctatgtctacacatacaggctcgcctccactccatctcccatcttccatgcagattcggctgcgatcaccttccaggtggtagccactggaacagctgtagtcacagcgagagtcaagaagcactccatttgtgcaggtgtaagtgccactagtgatgaatggtagtgcgtggcatctcatctgcctgcagtaggcagttccagaccaacgacggcttggcaggcattgcaccgacctccttccaatcaatcgaaagccccggtcacaggagagctcacaacgcgtgcccaggctgctgtgataatttcctcccttcggtgagtagcatgtggcttctccatcctggatatttaatgtataacaccatcgggggactcggtagtccagggcaggagcctgtgggacctcctctgcatatacttcattgtagctttcatccggatagtagccagaacctgcataccatgttggtgtcactgccggagttaggaagaacagcagaaagagagctcctctttgagttagctgactggccatccttgaaagggaggattatggagacaagaaaagatgtatatggcctgaagtaccagggcaaaggaaagtgactttcagaagtcagccatcaattaacttctaaaagtgaggggaagcagaaatatgggatctgttttatggtattttgtgccctttttctctctcctcctctttctccttcctctctgctcctctcatcaattggaaaaaaccttctactttaacattcctagaacgagtggctcctggtctgtcccggcctccgggattctgttaacactgcccagatgttacgacgtccacatctgccaaaagtttccttaaagctatattatccctgaagctatagttattcctctctcagagaagggttttagaaagatgggggagaaggaacacagggattagaggaactcagtccgtctgctgcagaagagggggaagtgt

SEQ ID NO: 10152 - RNA, 1232 nt, Homo sapiens
  source 1..1232: mol_type = other RNA
cagcaggaggtgaggggagtctctttgaaagtaaggatggcagtagaactctaacttattcaagatggagaccagcctttttgcggagaaaatgcgggtgaaggtcctgaaagtgcattgacgccgttttcggaagccatacaagtttagctggcggaagaagctctttatcgaagttgtggcaaacactttgtgtgcgacgtcccttttgagaatctccttttcaaagagtttttgattgatcactctacaagccccactgtcatcccaccagatggacgaaaactggttgctgctgaccagtctccacagtttctgtggaaaggggagggagaggagattatcttctccctggggcgggacgtcaccgtcagggtgcggccttctgaacgaagcttcctcggccagaggttggaaagcgatttcttctgtcagcagcctcaagttagggctcccagtggaccccgggtcgtcccaggcaggggaaggatctgctgggtgaaggtaggtctctgactgcaactggggagggaaaggcaccctttccaagccatgatcctgtcccctcgaatttctttcttcacagcgagccatactcaatgatcgcttgtcctccatctggcaaacttgctagtgcagtgtggccagcagcaccccttggcagtcatgtaaccagccccatgacatcataaaggggctctgactgccggggggtggcatctccacccccagcaagttgtgtaataaagggccaaggcagacaagtagctgcccatctgcatgtgcacattctggtcctcacagtcatttcaatgggaaagatgacactagtgcacaagagtgccgaggggccctgccacaccgtagatgcagacctggagcggtccccttgtcctagagctcctgagccaggcacaactacagcaaagccctggctcaggaaggtcagagctcaccgtctgagtcatgggcccacagaccccagcacatgactgacactcggaagcacagaacaaagggtaggacggtgcccatgggtcaggctgtagccacgccaccctttccaccctgtcctagccagaggcagcaatgtgctccatacagatcctcctaacacacccacactgtcggtccccagcacgcagatgcccgacagccccttaggcaaatggcttagctgactgccccaccacacgccgtcgccatgcagtccagtggggagtcggaggcag

SEQ ID NO: 10153 - RNA, 1232 nt, Homo sapiens
  source 1..1232: mol_type = other RNA
cagcaggaggtgaggggagtctctttgaaagtaaggatggcagtagaactctaacttattcaagatggagaccagcctttttgcggagaaaatgcgggtgaaggtcctgaaagtgcattgacgccgttttcggaagccatacaagtttagctggcggaagaagctctttatcgaagttgtggcaaacactttgtgtgcgacgtcccttttgagaatctccttttcaaagagtttttgattgatcactctacaagccccactgtcatcccaccagatggacgaaaactggttgctgctgaccagtctccacagtttctgtggaaaggggagggagaggagattatcttctccctggggcgggacgtcaccgtcagggtgcggccttctgaacgaagcttcctcggccagaggttggaaagcgatttcttctgtcagcagcctcaagttagggctcccagtggaccccgggtcgtcccaggcaggggaaggatctgctgggtgaaggtaggtctctgactgcaactggggagggaaaggcaccctttccaagccatgatcctgtcctctcgaatttctttcttcacagcgagccatactcaatgatcgcttgtcctccatctggcaaacttgctagtgcagtgtggccagcagcaccccttggcagtcatgtaaccagccccatgacatcataaaggggctctgactgccggggggtggcatctccacccccagcaagttgtgtaataaagggccaaggcagacaagtagctgcccatctgcatgtgcacattctggtcctcacagtcatttcaatgggaaagatgacactagtgcacaagagtgccgaggggccctgccacaccgtagatgcagacctggagcggtccccttgtcctagagctcctgagccaggcacaactacagcaaagccctggctcaggaaggtcagagctcaccgtctgagtcatgggcccacagaccccagcacatgactgacactcggaagcacagaacaaagggtaggacggtgcccatgggtcaggctgtagccacgccaccctttccaccctgtcctagccagaggcagcaatgtgctccatacagatcctcctaacacacccacactgtcggtccccagcacgcagatgcccgacagccccttaggcaaatggcttagctgactgccccaccacacgccgtcgccatgcagtccagtggggagtcggaggcag

SEQ ID NO: 10154 - RNA, 323 nt, Homo sapiens
  source 1..323: mol_type = other RNA
cagcaggaggtgaggggagtgatttggctgtgactcactcaaaatctcatcttgaattgtaataatccccacatgtcaagggcgggaccaggtggagataattggatcatgggggcagtttcccccatgctgttcttgtgatagtgagttctcacaagatgtgatggttttataaggggcttcccccttccctcactctcattctctttcctgccgccatgtgaagaaggacgtgtttgcttccctttctgccatgtttgtaagtttcctgaggctttgccagccatgcaaaactgtgagtcaattaaacctcttttctttat

SEQ ID NO: 10155 - RNA, 342 nt, Homo sapiens
  source 1..342: mol_type = other RNA
cagcaggggagagagaggagtcaagaagtcatcttctgggccgggcgcgatggttcatatctgtaatcccagcactttgggaggccgaggtgcgcagatcacgaggtcaggagatcgagaccatcctggctaacacggtgaaaccccgtctctacggcaaatttgccccactccctggcagctggagatatgggcattactggctctcttctgtcataccttgctacaaatcacaggctgggctcttgtatggatgagagtcaagttagccccgaatggcagctccccaggctggaccctgcggttcccataggcagtcagccccatgtgcaggagtgctgc

SEQ ID NO: 10156 - RNA, 918 nt, Homo sapiens
  source 1..918: mol_type = other RNA
cagcaggggagagagaggagtcactgtcagaagggacactgaggggagaggcacagtgggcccaggagtggactccgttagacccagagttcccttccccttctaggaagtgacacccctagcccaggcagtggtcaggatcttcagtctcctgtggcctctctctggagctgttcacttctagcaggcgctgatagtcttgaggccggaaacgctgtagatacacaatcagcttggctggtgctgtctcctgtgcaggcacacagagttgggccacaattgtaggttccgctgtgagttccttatactccgtgtggggtcctaagacacctgctgctccaggacatttgagctcccatccactatcctctcgtcgtcgcagccagtggtcagcctgcatgaggctcagctcaggggtgtcatagtaggtgtctcggaaggtgacccggtactccagggtgccccccaactcctgcagccgctcctctgtgccaggccctggaaggaactttcgctccacctcaatcaagccctgggccatgctacctgcaattggctcaaagcccgagagtctcctcgcgggacccacagagggggaagggagcccacgccatacactcgcgaggaatgccgggagcagttccggatcccggacctcggcccgaccctccgcgcgcccggcaggtcccggcaccagcggccatattacgcccgttgtggcggtgccgagagcaggccagggctcgagacacgcgctatgtaatgggaggccgcgacccccgcggtggccaggggagcgaggccgccccttgcattctgctcctcattgttggccccgcacggctcccgggggctggtacaggtctcatgcctgaggctgagccaggcaccccgaggcgcggatgcatgatgggagat

SEQ ID NO: 10157 - RNA, 1317 nt, Homo sapiens
  source 1..1317: mol_type = other RNA
cagcaggggagagagaggagtcactgtcagaagggacactgaggggagaggcacagtgggcccaggagtggactccgttagacccagagttcccttccccttctaggaagtgacacccctagcccaggcagtggtcaggatcttcagtctcctgtggcctctctctggagctgttcacttctagcaggcgctgatagtcttgaggccggaaacgctgtagatacacaatcagcttggctggtgctgtctcctgtgcaggcacacagagttgggccacaattgtaggttccgctgtgagttccttatactccgtgtggggtcctaagacacctgctgctccaggacatttgagctcccatccactatcctctcgtcgtcgcagccagtggtcagcctgcatgaggctcagctcaggggtgtcatagtaggtgtctcggaaggtgacccggtactccagggtgccccccaactcctgcagccgctcctctgtgccaggccctggaaggaactttcgctccacctcaatcaagccctgggccatgctacctgcaattggctgaacaaacgtttgctgagttcccaaggatgcaaagcctggtgctcagctcctggggcgtcaactcagtacagaacccctccctggaaaaacttatgaggggcacactgtgtcgcaatagtctctagggctactgcccttttctctctacctcggtgacattaaggccccgtcggtgatattttaaggctctgacagtgacaggtctccagtaaaatcccttccactgctgctgatgtcctcaatccaaagagacccctagaaagcaggccgggtagcgggtgtcctttcaacgcccccctctctacaccttgccaccccaggaggctactggctcacgacccgggaggacctgccctttcctgctacactaccggccagcggaacttcaggtctcacctcaaagcccgagagtctcctcgcgggacccacagagggggaagggagcccacgccatacactcgcgaggaatgccgggagcagttccggatcccggacctcggcccgaccctccgcgcgcccggcaggtcccggcaccagcggccatattacgcccgttgtggcggtgccgagagcaggccagggctcgagacacgcgctatgtaatgggaggccgcgacccccgcggtggccaggggagcgaggccgccccttgcattctgctcctcattgttggccccgcacggctcccgggggctggtacaggtctcatgcctgaggctgagccaggcaccccgaggcgcggatgcatgatgggagat

SEQ ID NO: 10158 - RNA, 1188 nt, Homo sapiens
  source 1..1188: mol_type = other RNA
cagcaggggagagagaggagtcactgtcagaagggacactgaggggagaggcacagtgggcccaggagtggactccgttagacccagagttcccttccccttctaggaagtgacacccctagcccaggcagtggtcaggatcttcagtctcctgtggcctctctctggagctgttcacttctagcaggcgctgatagtcttgaggccggaaacgctgtagatacacaatcagcttggctggtgctgtctcctgtgcaggcacaccaagcatgctgctgagcctgtggatcttctctagggcagttggtacttcagcctcctcatgcaccagggcctctacctcacccacagcgtagccaaagtcggctgtatccaagtccaccctgagctgtggctcctcttcatcagctcccaagagcaccagcttccaggcactccgcttagtcacaaaactagctacttcctgcagccccagtgggcccagcacagcagccacatctccagcccccaggccgtcagcccgcagcaccttacagagttgggccacaattgtaggttccgctgtgagttccttatactccgtgtggggtcctaagacacctgctgctccaggacatttgagctcccatccactatcctctcgtcgtcgcagccagtggtcagcctgcatgaggctcagctcaggggtgtcatagtaggtgtctcggaaggtgacccggtactccagggtgccccccaactcctgcagccgctcctctgtgccaggccctggaaggaactttcgctccacctcaatcaagccctgggccatgctacctgcaattggctcaaagcccgagagtctcctcgcgggacccacagagggggaagggagcccacgccatacactcgcgaggaatgccgggagcagttccggatcccggacctcggcccgaccctccgcgcgcccggcaggtcccggcaccagcggccatattacgcccgttgtggcggtgccgagagcaggccagggctcgagacacgcgctatgtaatgggaggccgcgacccccgcggtggccaggggagcgaggccgccccttgcattctgctcctcattgttggccccgcacggctcccgggggctggtacaggtctcatgcctgaggctgagccaggcaccccgaggcgcggatgcatgatgggagat

SEQ ID NO: 10159 - RNA, 1298 nt, Homo sapiens
  source 1..1298: mol_type = other RNA
cagcaggggagagagaggagtcactgtcagaagggacactgaggggagaggcacagtgggcccaggagtggactccgttagacccagagttcccttccccttctaggaagtgacacccctagcccaggcagtggtcaggatcttcagtctcctgtggcctctctctggagctgttcacttctagcaggcgctgatagtcttgaggccggaaacgctgtagatacacaatcagcttggctggtgctgtctcctgtgcaggcacaccaagcatgctgctgagcctgtggatcttctctagggcagttggtacttcagcctcctcatgcaccagggcctctacctcacccacagcgtagccaaagtcggctgtatccaagtccaccctgagctgtggctcctcttcatcagctcccaagagcaccagcttccaggcactccgcttagtcacaaaactagctacttcctgcagccccagtgggcccagcacagcagccacatctccagcccccaggccgtcagcccgcagcaccttacagagttgggccacaattgtaggttccgctgtgagttccttatactccgtgtggggtcctaagacacctgctgctccaggacatttgagctcccatccactatcctctcgtcgtcgcagccagtggtcagcctgcatgaggctcagctcaggggtgtcatagtaggtgtctcggaaggtgacccggtactccagggtgccccccaactcctgcagccgctcctctgtgccaggccctggaaggaactttcgctccacctcaatcaagccctgggccatgctacctgcaattggctgaacaaacgtttgctgagttcccaaggatgcaaagcctggtgctcagctcctggggcgtcaactcagtacagaacccctccctggaaaaacttatgaggggcacactgtgtcgcaatagtctctagggctactgcccttttctctctacctcggtgacattaaggccccgtcggtgatattttaaggctctgacagtgacaggtctccagtaaaatcccttccactgctgctgatgtcctcaatccaaagagacccctagaaagcaggccgggtagcgggtgtcctttcaacgcccccctctctacaccttgccaccccaggaggctactggctcacgacccgggaggacctgccctttcctgctacactaccggccagcggaacttcaggtctcacctcaaagcccgagagtctcctcgcgggacccacagagggggaagggagcccacgccatacactcgcgaggaat

SEQ ID NO: 10160 - RNA, 509 nt, Homo sapiens
  source 1..509: mol_type = other RNA
cagcaggggagagagaggagtcactgtcagaagggacactgaggggagaggcacagtgggcccaggagtggactccgttagacccagagttcccttccccttctaggaagtgacacccctagcccaggcagtggtcaggatcttcagtctcctgtggcctctctctggagctgttcacttctagcaggcgctgatagtcttgaggccggaaacgctgtagatacacaatcagcttggctggtgctgtctcctgtgcaggcacaccagacaaggggatctggccatcttcagcagggaactggctgggggccaggcaggactgccagcgctttccatccttcttccttggggtcttggcaatggtgtgcttcctcctttgtgtcttcatgccactctccgtctgttgctccactccccatgcctaagagggaaggggaaggaggaccacaccataccaccaccaagccatctgtgctctcctcctggctcagtcaccttctttcactcgc

SEQ ID NO: 10161 - RNA, 729 nt, Homo sapiens
  source 1..729: mol_type = other RNA
cagcaggggagagagaggagtcactgtcagaagggacactgaggggagaggcacagtgggcccaggagtggactccgttagacccagagttcccttccccttctaggaagtgacacccctagcccaggcagtggtcaggatcttcagtctcctgtggcctctctctggagctgttcacttctagcaggcgctgatagtcttgaggccggaaacgctgtagatacacaatcagcttggctggtgctgtctcctgtgcaggcacaccagacaaggggatctggccatcttcagcagggaactggctgggggccaggcaggactgccagcgctttccatccttcttccttggggtcttggcaatggtgtgcttcctcctttgtgtcttcatgccactctccgtctgttgctccactccccatgcctaagagggaaggggaaggaggacccgaggaggcagccggattcagcacctgatccagcacccgtttgggattgggtgggtaggcgggcgggcggaggggtgatggaggcagacgatggccctaggttggcagccgatggagcacaccataccaccaccaagccatctgtgctctcctcctggctcagtcaccttctttcactcgcccaaattaagactcagccagttccttgtcttcaagctcatttccccaccccagcctagagaagtatattcctcaggcagctgactccaacagttgcttctcc

SEQ ID NO: 10162 - RNA, 626 nt, Homo sapiens
  source 1..626: mol_type = other RNA
cagcaggggagagagaggagtcactgtcagaagggacactgaggggagaggcacagtgggcccaggagtggactccgttagacccagagttcccttccccttctaggaagtgacacccctagcccaggcagtggtcaggatcttcagtctcctgtggcctctctctggagctgttcacttctagcaggcgctgatagtcttgaggccggaaacgctgtagatacacaatcagcttggctggtgctgtctcctgtgcaggcacacctcaaagcccgagagtctcctcgcgggacccacagagggggaagggagcccacgccatacactcgcgaggaatgccgggagcagttccggatcccggacctcggcccgaccctccgcgcgcccggcaggtcccggcaccagcggccatattacgcccgttgtggcggtgccgagagcaggccagggctcgagacacgcgctatgtaatgggaggccgcgacccccgcggtggccaggggagcgaggccgccccttgcattctgctcctcattgttggccccgcacggctcccgggggctggtacaggtctcatgcctgaggctgagccaggcaccccgaggcgcggatgcatgatgggagat

SEQ ID NO: 10163 - RNA, 923 nt, Homo sapiens
  source 1..923: mol_type = other RNA
cagcaggggagagagaggagtcactgtcagaagggacactgaggggagaggcacagtgggcccaggagtggactccgttagacccagagttcccttccccttctaggaagtgacacccctagcccaggcagtggtcaggatcttcagtctcctgtggcctctctctggagctgttcacttctagcaggcgctgatagtcttgaggccggaaacgctgtagatacacaatcagcttggctggtgctgtctcctgtgcaggcacaccttacagagttgggccacaattgtaggttccgctgtgagttccttatactccgtgtggggtcctaagacacctgctgctccaggacatttgagctcccatccactatcctctcgtcgtcgcagccagtggtcagcctgcatgaggctcagctcaggggtgtcatagtaggtgtctcggaaggtgacccggtactccagggtgccccccaactcctgcagccgctcctctgtgccaggccctggaaggaactttcgctccacctcaatcaagccctgggccatgctacctgcaattggctcaaagcccgagagtctcctcgcgggacccacagagggggaagggagcccacgccatacactcgcgaggaatgccgggagcagttccggatcccggacctcggcccgaccctccgcgcgcccggcaggtcccggcaccagcggccatattacgcccgttgtggcggtgccgagagcaggccagggctcgagacacgcgctatgtaatgggaggccgcgacccccgcggtggccaggggagcgaggccgccccttgcattctgctcctcattgttggccccgcacggctcccgggggctggtacaggtctcatgcctgaggctgagccaggcaccccgaggcgcggatgcatgatgggagat

SEQ ID NO: 10164 - RNA, 1322 nt, Homo sapiens
  source 1..1322: mol_type = other RNA
cagcaggggagagagaggagtcactgtcagaagggacactgaggggagaggcacagtgggcccaggagtggactccgttagacccagagttcccttccccttctaggaagtgacacccctagcccaggcagtggtcaggatcttcagtctcctgtggcctctctctggagctgttcacttctagcaggcgctgatagtcttgaggccggaaacgctgtagatacacaatcagcttggctggtgctgtctcctgtgcaggcacaccttacagagttgggccacaattgtaggttccgctgtgagttccttatactccgtgtggggtcctaagacacctgctgctccaggacatttgagctcccatccactatcctctcgtcgtcgcagccagtggtcagcctgcatgaggctcagctcaggggtgtcatagtaggtgtctcggaaggtgacccggtactccagggtgccccccaactcctgcagccgctcctctgtgccaggccctggaaggaactttcgctccacctcaatcaagccctgggccatgctacctgcaattggctgaacaaacgtttgctgagttcccaaggatgcaaagcctggtgctcagctcctggggcgtcaactcagtacagaacccctccctggaaaaacttatgaggggcacactgtgtcgcaatagtctctagggctactgcccttttctctctacctcggtgacattaaggccccgtcggtgatattttaaggctctgacagtgacaggtctccagtaaaatcccttccactgctgctgatgtcctcaatccaaagagacccctagaaagcaggccgggtagcgggtgtcctttcaacgcccccctctctacaccttgccaccccaggaggctactggctcacgacccgggaggacctgccctttcctgctacactaccggccagcggaacttcaggtctcacctcaaagcccgagagtctcctcgcgggacccacagagggggaagggagcccacgccatacactcgcgaggaatgccgggagcagttccggatcccggacctcggcccgaccctccgcgcgcccggcaggtcccggcaccagcggccatattacgcccgttgtggcggtgccgagagcaggccagggctcgagacacgcgctatgtaatgggaggccgcgacccccgcggtggccaggggagcgaggccgccccttgcattctgctcctcattgttggccccgcacggctcccgggggctggtacaggtctcatgcctgaggctgagccaggcaccccgaggcgcggatgcatgatgggagat

SEQ ID NO: 10165 - RNA, 13209 nt, Homo sapiens
  source 1..13209: mol_type = other RNA
cagccagcccctgctcacccctaaagagcagcacaagtaactcagagccactgtcccctctggccagaggccctggtttgtgtctgcccagtgaccagcctgaagatagaggcaacccaatccaggtccatgcaggtctccgtgatgcggagcatgcccagcttaccatcctgatgcagaggcaaggacaacactgggccctgacttgctaagatgggagcaagagcttagggctaaaactcagcagtcccagctctgggggacaaggacccacaaagtgatgcaagatatcctgagttgggtgtgacaagtacaccttgacacacaaactgcacagggaggggaggaatctgagccagcttcctccacaaagcacagaagtctgccaaaagcccaggctggatagggagcatcacactgttgggaaatgtgcaattttcactcagccagcatcactaccagctccgggcttctctcctctggcctcccaccttgcagctttgagatcccaggcctctcagggctctggctgagggctgtgagccagaggctgaggtagccaggtctgccttgggctgtcactcagggctgagctctgctgaaggatctgggaggtcagtaggcacctgtgtccacccagctgtccatacagatccctgcctgcacaagagctgctgcagcatttcaatagggccatcccaggcaccctaggacttgagaccagcctcctctgtatggtcccttccctggtgcacctaccacagcccactctgatgaccccctgtcaaggaggtgtgactgagaaaggaaggggcagagatcccttctccattcctctcaggcccctgtaaaaattgggacctgtccttgccagccaggtctcagggagctcagggttcagtgttggaatgggtctgggcccagatttcaagccagtaaccagcaaatcatggggagactgagaagaggagccccttagcaggcctaaccacacccctaagccacccagcctggcccccctcctctgccccaactggctccaggccaaactctggttcctgaggagcctcaaaggctggacttggggtgtcccgcggaaatcctggtgggatggaaaatccccagcagttgtgaggctgcacttctcccacccgctgtgggtcagccaggccgctgcttcctgcttccctttgatgtctcctcgtgcgagggaggggtcagcacccctctaggcttgggcaggcacacactccactcagctgcagccatggagttggtgcttctagggcctgggtatgctggagtcaggcaggggacctggtgggggtggggatacaggctgaggtggagagaccccacgcagctccctaggcctctgcagacagctcccaagcaagggggcaggaggggctgcactgagcccaccaaaggttgtagccactcatacagggctgtttgatctgagagggaggcgccatgacctctgtttagacaaggaaaatgaagactctggaaaatctaagcacgtcacacacacagcttccatgggggtcttcctctcgtgtctggggaacttccccgtagaggtttcaataactgccatcctttgctgatcctctgtgtaggcactgggccccagcccctgcctgtgccatcactatttcacaggagaacaccacactgaggctctgcctctggttgccctgctctgggtgatgaggtagaggtcacacagccaggccagtggccctagtgtcaaggttccacaccacagcctcatagcagccagtgctcgctcactgaggccaggcactcatcttgtgctgtgcctgggtgagctctggacctgcctcctaaacatagggctgcctgcttcgttcatttccacacaccacgtgcctaggcccagctggggctggcatacaaattgggtggcccggctctgagctgctgctggttactgtggcagtttccacctataccacacctatatacttgccctcccccacacacagcccacctggcccatcccacaaagagagatggcactccaggtggagagggctgggccagaggtcatgcagcaaggtcaggttggaagctgaggtggggctagggccaccccacacaggcctgtctcacaggctgtcacccactgggcctagggctctgagagtaggggtctgatctggagagcaggggagcctgcaggtccctgggttggaatcctggagccctgggctgcagggttttgaggggcagttacctcctcctccccggtggcacatccggcctggaagttgggtagtctggcccaaggcctgccctggtgtgaaagcctgagaccctaaggagagctacaggtggctcaagggcctgctcctcctccttttctgtgcaaacagctcagcttgctgactttgatgcagtggtttaggccaagctttgaagtcagcccttggaggacgttcctatcagcctttgcacagatatctcccactccaaccctaagactcaatgccacctcaggactgcccctatccgcagagcttgaggcctttaggtcagccttgggaagaggtgcttgagtggggtggaagaagcccactcttgggaaatggggagcataggggaggaggaagacactgccttggaatgacactcccagagacctctgctctgcctacctgcattctgctgaaggttttgggtcaccttgttttatggtccctgtcccagcatgaagcttgcacaggaagaacagaatgaatgatgtggaaatctgttagcagtggtgtcttctagattctcaaggatccgggtattttaggaacaaaacaagccagcaggtgcagaggtcacaagcctcctgagagggccagggcagagtgagtagctgcaggggcagctgtcctttgcacctgggcctagagtgccagagacttagtctcatttgtttacaggagactgatgggttcctgagcagcctaggaggggaggggaagcactgcgttctcagtgtggtgcttggccctcccaggtgcctggttgtggcctgccacttagcacccacccctgcctatccagccccatccctggggaaggttcccacctgctccaacttctggtactcccaggctgcctcacccaacgatgacagtgactagcctcagagcctggctgcttggaagacctttgcccaagcagagaactgttgaggaaggtgagccttccgagggccagccctgcctctcctcccctctcctagcctgcttctgtctgggctgaaggcacagcagggacaatcgctcttccggggttagaactgggggagcagggacaaaaagcgggcagccctccccagcatgacaggatgtggaaggctggtctctccagagactgggctaaactctgctgtgtcaagtgcctggtgacctcaagcaagtcattccatgtggctgagctgctccttgctgcatctgcacatatgtgtagtgtcttcctccctgtaggattgtcacaaggattaaatgatgtcaagtctgaggctgccctgcagctgctgtttccactacttggcatggaacatgtgccagaccaaaagagctatctctctccctgcgaaaggctggggtcctgggagctagagctgggttaagataagagcagagactgggtcctgggaacagccactgggcccagtcgggggggtctcagcacctatcacaaagaaagtgccactgggcctagggaaggacaagaagtaacatgtcaaagatgggacagaacccacctcctggcagggagtggggcacacatatgtgcatgttcatatatgtgtcagaatgcgtatttgtcagtgtatgtgtgtcagtgcacataggtataggggctgtctctcagaattcctgagggctttccatttgatcccagtggttgaagatggagtatgatcccaaatcccttaggtggatgtggcctggcagggggtcagcaggagggaggtccctgtctccttggcttccagcttccaggctctggcactcccactgttaggaacaggtacctttagggacacaggagtgtaagccactgtttccgtctgggttttgtcatgtgtaggtcccagcggctttaagccaacctgaaaggttcatttgggagtcacgggtatgtgtcaacaaaagcccaccagaccatcaatgaagtgggcaaaagctctgggtgaactcttggctcaggtatcaggatatgctgggtgagggaaataatggaggcacctttgttctagatgcctgcagattcctgacaacagtaggggtggaggctgtgcagacctggtgcagagtctgtgctggcctctggcctctcacagccttgggaggggtgctcagagctcagctgtgtttaaaaattagcaagtggaggagttagaggatctgcagttaaccccttgagtctcggaaggctgtttgagccactaatcaggaaggagagctgacaagaaaaaggcgatgtctcacccctgagctacaatccactgcacttacagtgaccacccatcctgacatcttgggctcaggcctctgggtctgggcatagaagcccaggaactgctgtctgtggggagtccactgaagctccctgcccccactgagtctctgatgttgacagcctctttgttttttcatctcagcctattcaaggccatttttcagcttgcttggctttgcattaaagttggggggatttctctatcctgaggttatgaaatacctcagcaaggacgaggcctccctgagggagtcaacctagcttgttccctgcacgtactgtggggaggtcctctttaccgccacagttccaagggtgaaacagagaaccaggtggggaaggggtctctccccatctgtccaggggagaggcagcccacagggagccacacaggcaggggacattccactagggccatttgcaggccagtggccatccactgccagcaatcagagaatcacaagcactggatccaatgtgacctctgccaggaccatgacccctaggtcctcttttccatccctccagttctcctggctttcttgccatctttctggctctatcctcagtctccttggcaggttttcccttctggcatggccactaaatgccagtgcctttctctatgcaaaccatttccctaagctgttccctcagcaccaagggcttccagaccacctgtgaggccctgaccccccaaatgtctctccaacccagccagacccacattccagtcacctgcccccacctcctctccacagcctccatcattttatagcccactctactgaaggcccctgtcctttcagtgtcacccatcctttcagtggcacaagtcagaagttctggggtcatttccgatacacccgcttcctcaccacctgcccatcacctcaagcccatcaccaagccaggcttacttcacccatccatagttctagaggttccctgcttccctccatccctattgccactgtcctgataggccaccatttctctgtactgcaggcatctcctaactggcattctcacatcccctgccccattccaatcaattatctactcagtggacagacatcctttcaaagtttagagacctgtgggtcttgcttaatcctgcagctgcctttctggtagttcagatgcttggcttctttccatcccaggtgctcacaggctccctaccaccagagggcccttggcctgcccctgccactttccccaagggagtttttcagaccccaggctagttccagtgggttcctgctatacacctgctgtgctcccaggcctcagcactcccctcagggtgcaaacggtccttcaacattagttagtctttctcccctttgtccactaaccctgggagggtaggcaggtccctgctcctatcaaatccctccctctgggccagggtctagtacctgctgagtgtttgacaaatatttcttgaatgactgcatccctaacatgaggcaatgatcattcccctgcctgttagacataattcactgcctgggaaggcactgtgctgtgtagatgcagcaagctggctaaaatcaactgtagcatggcctatgtcccaagcaggttgtcctgcccatacgctcaataatgaggcccactgaactctcctggtttccagaagcctcataagcaagcacgctcagtgaaggaacaggaagtcctttctggagcagggggagagaaaggcatccagttagccatagaggggaatggctccttactctttaagagtcatttgccccaagactactttctgtcaatcaccagatagccctcagtctacactctgtgatccactcatgaatatctggtctggctctgcgttccagtcagacccttttctgagaggaccacaagtcatagcccagggctacctgtacagctaccaggcttaacaactcagatgcacaccctccacaactgctcttagcacccacaggcctgggccctctctccctgccctgaagccaaccagaccctgggtgggggccgagtctggccaagcagcagtgtgtggagctgggcctgggcctaagctgggaataagcttgttttgccaggcgctggccccccatcgagtccccattctctaatgctaattgctacaattagcaggagaaaggccttttagatccatttcttctcctggctgaggcccgggctgctagggaggttgagcccaaggcttttcggaggagcagggattcttccataaatgaggccacatttaaattgcaaacaagagcttcgcccagccgtaggaaaggctctgggagaaaggcttttagttccgcagacagagcagccagagactgggtgcgctccagcctcatgggccttcctggctggtgtgactggaaccctgggttatacaggctcctgccagtaacctggacatgctggggccggccagttcagaggagcatggcacaggctgataaaggcaccggaaggaaaggcagtattagaggccaccccttgccctcccatccaggcctgctctgagggaaaccctactcgtcctcctcctggagtgtactgcaaacctggatccggtatccgctgagaaccactcattcatcagtctgcactaactggagaaggtgagcaggcccagcccggcctctctaggccacctccaacttggtcaagccacaggtgcccatgccatagatggctgagggacggcagctgacacgtagttccaactaaacctctgggtggcagcccataggttgtgggactggaagtgcttgccaaacaaattatactgctgaccagggaagagggtactctgattggccaggcctgggccagggtctttctcaccgaggtggtgaggctataggtgttagatgtggcaggatgcaagccagggcctgctgcctttaaagagccacagcagagacaccatcccagtcccaagagctgttctaaggaagtggttgtcatctgcggtgccccccaggggacatatggcaatgtctggagatatttttggctatcatgactatgggagaattactaatatcaactaggtagagaccaggcagggtgctaaacatcttacaatataaatgacagcccctcacaacaaagatacatcctgtcccaagcattaccagtgtggctggctaagaaaccctggttgcaaggggtcagattttgacatgctatttgctttctcactgagttgtgaaaatggaggcacactttcctggcctggcctcttccttcgttcaataaatgaatgaaaccattcaacagaaatctgtgacacacccaccatgtgcggaccctatacggaagacagatatgctctcttggggcctctcttccggtggaagagataggcagccaacaaataagtagatgtctaaggaactagaaaagcgtagcctgtgctttgcagagactcgaaaggtagtcgtcagctagtgagtgactgaaggggatgacagatatggcaggtcagagcaaaatttcctgtgagatttaaataagaagaaggaattgtcaagggaagatcaccagaaaagacaagccaggcagaggtggtgaaggccttggggcaggagggatacttggcagatttaacaaagaagaagaaggctggcagagccaaagctcagtgagggaggacagtggtcagagaggtaagcagggcagatcttgtaaaaacctgatggaatttgaattttatttcctagaaatagaagccactagagggtatctggcaggagagtcatggaggcacattcattcgttggttcttggcttttgggactctgcacagagttgatcacagccctcagcctatgaaacactgtcaccctgtaagggtctgcataaagtcaccgctctcttcctctccatgcttttccacttcatctctagcctctatccttgctctcctccctacacaaacagcttctccagggtaatttatttatatcattgtgtgtgtgtgtgtgcactcacgagcactccctagtactgcgtgtctgggtggtgtgtaattttaatttaaatacacagtcatgtactgaggccctctttctgtttggcatttgtgtcactcagcactgtgtttccacgcgtctctatcttgtgaagtgtacatctagtcccctgctcctaaccacagtgaccagctccaactgcccacccctatgggccatgctgccctgagcatgcacacacacagcctctcgttgttctgggtgagaactgctccagcatgtttacttaggagggaaactgctgggccacaggtataaaatattttatttgaggaagaagtgttggccagctcttcagaacgtctgtgcctgtctccgtccccacctgcagcacacagggaggcttgttccttgccttctgccaacacttggccttatcctactttctaatgcttctcctatgaagaatagctgttgctttcatttacatttctctgataactgattagcttgggcaaattttcatctgtttgttaaccctcctgcaaactggcaatcttcctacctttttcttaatgatttgtggtgctttctggtatattttagctgttgttccctcctcagctttaattgtttcaaatatcttgtaatgagtcatggcaaagttacattcatgagtgtaaaagtgaaaaacgcaaattgtttccttagtattattatgaaaacagtcttgacccttgccatgatggatttatttaacagaaatccttaatccataatcattaatgcattcaagttcatacattttagtcttgaggtttgtgctttctggatcctgtttaagaaccccacggccaccctggccctggagattattcattttttctcctattaaacaaatggcaactaccttttgctttcaaatatttagtccatttggagtctacttttcctaggggctcagttaggaatccatattcctattcctccattttagggctggctttccaacatcatcttctgaacagtccccactgatatgtggtgccacctttatcacatgtccccttcctctagacttggagttacctctgagctctcttctgggcctctgtcaccacaccgctctgattgctgaagttggcgtgtgccctggtatctgccagcagaagtcctctgctctccttttcaaaagttcagttggcatttacaaatatttttcttccacatacattttagaatatgtttgttaaattactcaagccctccaactggaagtttgagtggagtcctgttgaacttaacagatttggaaaatcctgacgtcattctaatgccaagttgccctgttcaagaaaataaaatgtctctgcatatggaaagatctccctctatatcctccaatagagttttaaaattttttccataaaagtcgtcgtctttgttaattcctagactggtataaattttgctgctattctgattgctgtcctaatctctattatgcttttttttagtcagttgctattggcataaagaaatgtggtttgtttttgttttttgttttgagtacactgatcttatatccaaaacctctctgaaatctgaaatctctctttagttgttaagttccttaattttttttttccatgtagcccagtaattttcaaagtgtagtctggggattccagagagccccccagaccctttcaggaaaggtcaaaaacattttcataataatactcgacattatttgccttttctttcattctcacaaagataaagagttttccagaggcagcacaccatgaccccagtggaatatgtgcttgtatagttctgctttaaacatttcttagttttaacttctaagatggtaactatcaacagatagaatctctatcaagaaaagccctttgggggtttcaataacttttaagaatacaacaagtcgtaacaccaaaatgtttgagaatctttatggagaccatcaaccctatgagctacactaagttttatcacttcctacctgatcctcacatccccatttctttttcttgtattagggtatggccaggatgacatccttggcctactccttatcttaaagagaatgatacacttttaatttctctatcaagtttactgaaaagttaagttttggtttataacttgtatcaagttgaagaagttcctctctagtcctggcttgctaagtggtgtactccactaccccaaaatcacacataggcgttaaactttatcacatcatttttttctgcctctattgagggaaccatatggtttttctcctgtagcctcttaatgtgaattacatggataaagtttctgatattggatcatctttgcattcctaagagcaatcccacttgtttaagaattgttgtttaatacatattattggattcagttagctagcattgtacaaggaacttctgcatctacattcataagggaaattctttatagttttcttgtgctttctatctgaatttggacatgctctgattcgcaattttaaaaaatccctctagctggagcataaatcctgaaacagacccacttttctcctcagcatgttaggaaacacattaaaatacacccataatcaagcaactcaatccttaaatttttctcctactgagtatctggaaaacaggtgcagaaatggatcatttgagacaccatagaaatctggttaatcctgcctgcctgctttccttcaagtactgactgagtaaggctgtgtatcaggctcttggctgggtacagagcaggcagcagaaaacaaaacagagttcctcgttgggagcttttggtctagcaaaaggggcaccacagtaaagaaagaactggtaaatgcacatcaaatgtggatattatcaggaaagtttttatactttgtgataatctaagacagaactattctacctggatgaattattctctttcataaccagaacagtgctgtgggaaggcactcttactctcaattttatataaaaggctatttgacctgctcagggaccacagtggggtactgggatctgaacatagtggtggcccttcaagcctactacccagactgagacctgcatctgatcaactctcatctccaatatgaccaagagacttctaccactacctctcacctggcaggtgatcaccacccccaactcagactgcaacctttacttcgccccctaattcctgactcagaatccccacctagaggcagaacttcgacttcaattcctgactcccataccccactgagacctctaaccccaatcccaatctcttaactcagagccccccattcagaacctctacccaaagacagactccagaccctgactccagtcgccaactcggacctcccttggatctcaactcagagccatgatgcagactccagaccgggattcaggtccccaactcagactcccgatcctctgtccctaatgaggccctacctaaaaccaccatgcggactccagacccggactgactgggaccccaactactcagatcccaactcaggcaaactcccagccaggatgtggaccctagacccgaattctgatcccaactaggatacctaactcagaaccacaacggggattcccacctccgatcctaattcgggccctgactcagaaccactaagtggatttccgactccggtcccaattcgggctttgactcaaaaccacaacatggattcccaacttccatcccaatagcgcggactcagaaccacgatgcggattccagactccaatcccaattcagcccactctgaaccaccatgagaactatagacccggaatccgatccttgggacgcggccaggaactcggacctcgaccctggccacgctgtccataaggtgcagatgggagcgcactgcccaggccaggctgcactgctgacgcctgtgatctgggacggccgcggggcacacagctcacctcagcaacgccagtgatcacccgtcccgcgccgtccgcccaggtccgtgctgaccgtgttcaaaccctcccagagagatggggagggccgcgctgaggagagtctgggagaaccgcactgaggagccgccgggagagtgccgcgctgaggagcccccggggagagtgccgcgctgaggagcccccaggagagtgccgcgctgaggaggcccagggaggaccgcgcggaggagaaccatgctgaggagcccccggggagaacagaaccgcggcgagaggcccccggagagaaccgcgccgaagaacccccggggacaaccgcgccgaagaacccccggggagaaccgcgccgaaaagccccgggtgccccgaggagaacggcgccgaggagtccccggggagaactgcgccgaggagcccccagaagagcgccgcgctgaggagccccgaggagaaccgcgccgaggggcgcgccggggagaaccacgatgactgacgcaccgaggaggaccgcgctgaggggcgcaccgggagaatcgtgctgaggagccccggggaggaccacgctgagaggcaccccggcagaatcgcgctgaggggcgccctggcaggatcttgctgaggagctccctggaggtccgtgctgaggcgacgcggcgaccgttctgcct

SEQ ID NO: 10166 - RNA, 1555 nt, Homo sapiens
  source 1..1555: mol_type = other RNA
cagccagcccctgctcacccctaggcaggcaaggaagctaagactgtgggccacccaatggcacacagtggtagcctcggcgaggacaaacccaacccaattcagactcccttcagctgggagggagtgggtctgtgcctgtgactgaaaaggccaggtgcctctgcctcggacaggcatagatcttggggttcagatcacacctccagctgtggtttagcttttctctgccatagcctcactctcagctgcaccagttcagcaactccaacccaaagctagagagggttcctttgccactgattccagccaaagtcccaaggaggcatccattggcccggtctgggtctcaagtgcccgtctctgagccagtcaggtggcaggaagggctgggaggctgtgattggacaggcctaggccacatgcctatcccagcaggtggtggaggcgtaggggagcctatcggaatcacatgggctgaaggcctggcaggcatcctcctctggtgggtgggcaaagggaggggaagtggctgctggagccaaattggtagatgctccccatgctgctgtccatcttcaggtactgctggagtgtcccgagttcagaggacctccagaaagtaccgtgagaagaggcaagctggcaggtgggtggctctgcagaacaggaattggcaatccctgcacagggcgcgagccctgctttggctgaggtgggtgtgcagaggaggatggtcgtgcttctgctgtaggtttctagtgtggtgtttcacccggtatcttgattggcagaggaggccttgcaacatgacgtgtgcgggtgtcctgtgtgcagcaatcgcatggccttgagcagctctctctgctctccttccctgggctggtatttcctcatgggtcagtgaaatggggcccacttgcctgtgtgagtgtacatttgggataaagtcctagaagtgacattcatgctctttttaatcctcacaccaacccctcggactgggatggacctcgttggcaccaacctcttctgcaggggcagctgcaccgtgttcgagtcgtttgtgacctcccagggctgcaggggctcagggtcgggctctgtcagccacgacaacctgtacggaaacttcttggcaaaattctcctgggcctggatcctccacttcttactctggtgagacttcttgcaggcactggagtccatcactgagtgggttaagctgaggcacacctctcagccatggcaggcagctaccttgaattctggcagtgacgatgatcaggtgtgatcagagagtcctggaactgctcctatccagcaagatgctggtgtgagagccgctgtggcccccgaggctggcagggccctggctacagccctctctggaaagacccagtcccaggctatgcccagagcttccagccagaaaggacaagctgcaggaccctgtgggctggcttatgtgacgccaggcagactgaagctggccatggtcccagctgccacattaccacaggaacagcagccccagggtccccggacaggcagt

SEQ ID NO: 10167 - RNA, 2846 nt, Homo sapiens
  source 1..2846: mol_type = other RNA
cagccagcccctgctcacccctaggcaggcaaggaagctaagactgtgggccacccaatggcacacagtggtagcctcggcgaggacaaacccaacccaattcagactcccttcagctgggagggagtgggtctgtgcctgtgactgaaaaggccaggtgcctctgcctcggacaggcatagatcttggggttcagatcacacctccagctgtggtttagcttttctctgccatagcctcactctcagctgcaccagttcagcaactccaacccaaagctagagagggttcctttgccactgattccagccaaagtcccaaggaggcatccattggcccggtctgggtctcaagtgcccgtctctgagccagtcaggtggcaggaagggctgggaggctgtgattggacaggcctaggccacatgcctatcccagcaggtggtggaggcgtaggggagcctatcggaatcacatgggctgaaggcctggcaggcatcctcctctggtgggtgggcaaagggaggggaagtggctgctggagccaaattggtagatgctccccatgctgctgtccatcttcaggtactgctggagtgtcccgagttcagaggacctccagaaagtaccgtgagaagaggcaagctggcaggtgggtggctctgcagaacaggaattggcaatcctattttgcagaaaagaaaagatcaagagagaggaagttacttgctcaagtcaggaagtatggggccaggatttaaatcccagctgaaaccccaaatcctttttctttccattctacagggcaggggcatttgtgttgggctttgaaagctgcataggagtttaacaggtaggaaaaggaggagaggaaactgcaagcagaaggaatggcacagagaaaagcatggaggagtgaaatggcctggggtgtgaatggatgtgctgtgggtggggctctgggtccttgagagagaatggtgggatggaaggcaggaagatactctaagttggggctcagtcatgaatagtcttgaatgggatgctaggggctggggtgctcttcctatggctgtcagagggcatcagtctttaaataaatagtcactggcactgggcaaggttgcaggggttacagaaaagcaaaaagtccccttccatgtagatctgaccttccagagtgatcaacctacacagaactcaaaagatttcagcaataaagagtgccgtggctggagctgagcagtgaaccaggaagggtggtagtgcactggtgggccttggggggaaccagggattgctgcaaggagtgagaagccctgtgggtttagagatcaccaaggtggggcgaggagaaataggagataggtgaggtgtctccttccagtcttggtaattgttccagggagagccctggggcctacccggggctggccatgggcagggaaggtggaagtggggtccggagggttctggaggcacagccgacaggactgtgctcaagggggatctgggcagactggggttccattctagatggcctgtggagttcagcaaatggagtttgaactaaatacacgtggagagatctctagttctctcccctaaacagaattgcttataataatacatgaagggcttgtccaatgtgtccttcccttgggcctgatccccagaaggaatgtccctgactctgagacatgcaggtcaccccagaaagcccctaggggaaggaatggggcaggacagaggccctcggaggccacgtgggaacctatgcctgctggcaggagcttgctggggcctggctgccctgcttatctcctcttgcaacactgtaacctgctggaacttattaaccagaagccgagtgtcatcatctctgcttgctggactagggagtctgcaaacagcatccccctacatgatggctgtgccctcaccctgcacagggcgcgagccctgctttggctgaggtgggtgtgcagaggaggatggtcgtgcttctgctgtaggtttctagtgtggtgtttcacccggtatcttgattggcagaggaggccttgcaacatgacgtgtgcgggtgtcctgtgtgcagcaatcgcatggccttgagcagctctctctgctctccttccctgggctggtatttcctcatgggtcagtgaaatggggcccacttgcctgtgtgagtgtacatttgggataaagtcctagaagtgacattcatgctctttttaatcctcacaccaacccctcggactgggatggacctcgttggcaccaacctcttctgcaggggcagctgcaccgtgttcgagtcgtttgtgacctcccagggctgcaggggctcagggtcgggctctgtcagccacgacaacctgtacggaaacttcttggcaaaattctcctgggcctggatcctccacttcttactctggtgagacttcttgcaggcactggagtccatcactgagtgggttaagctgaggcacacctctcagccatggcaggcagctaccttgaattctggcagtgacgatgatcaggtgtgatcagagagtcctggaactgctcctatccagcaagatgctggtgtgagagccgctgtggcccccgaggctggcagggccctggctacagccctctctggaaagacccagtcccaggctatgcccagagcttccagccagaaaggacaagctgcaggaccctgtgggctggcttatgtgacgccaggcagactgaagctggccatggtcccagctgccacattaccacaggaacagcagccccagggtccccggacaggcagtgccaacaagctcactgcaaggtcagaagccctt

SEQ ID NO: 10168 - RNA, 573 nt, Homo sapiens
  source 1..573: mol_type = other RNA
cagccagcccctgctcacccctcaggacccgaccgctctcggcttccgtcggaacagcagcccccagcccccgacacaagccccctgagggcctgaggcatcctgggtctcactcggcccccaaaaactgataaaagaataaaacacttaaatgaataacaaggaactgagtatatgtatatttcatcaggggaggggctaggactcccacttggaggcctcaggagttctgctgggcgtcgcgaaggagcttctcctcccgccgcttccgtaacctctctttgaattcctctatctcttgaagaaaggggtccgcgtgggatccgcttcactcttccaggagaaggcaataaggaaaccatctactcctctgctctcggttccttactcatggcttctcaggtggccacagctccctcttgcgctgtatgacatcgtcctcaaaccactcggcctgattggaaacccagaacatagccacagggaaagtgaggtagattatcatccgaaatatctccagcttcacccccatctcgtttctcccggtcaacaaagccagttccgcccaaagcc

SEQ ID NO: 10169 - RNA, 483 nt, Homo sapiens
  source 1..483: mol_type = other RNA
cagccagcccctgctcacccctcaggacccgaccgctctcggcttccgtcggaacagcagcccccagcccccgacacaagccccctgagggcctgaggcatcctgggtctcactcggcccccaaaaactgataaaagaataaaacacttaaatgaataacaaggaactgagtatatgtatatttcatcaggggaggggctaggactcccacttggaggcctcaggagttctgctgggcgtcgcgaaggagcttctcctcccgccgcttccgtaacctctctttgaattcctctatctcttgaagcttctcaggtggccacagctccctcttgcgctgtatgacatcgtcctcaaaccactcggcctgattggaaacccagaacatagccacagggaaagtgaggtagattatcatccgaaatatctccagcttcacccccatctcgtttctcccggtcaacaaagccagttccgcccaaagcc

SEQ ID NO: 10170 - RNA, 1378 nt, Homo sapiens
  source 1..1378: mol_type = other RNA
cagccccacagcctcagactccctgggcaccccctaccactgcaggaaatctggccagcttctccggggatctcaaagtatcctgaaggcctgagcagcaaagtcggggttctgggcaagcgtctgcatcatgctgcgcatgtagggtgctgagatcacattctgcatcagctgggggttctcagagatctgctggaggagggcttgcatttctgggctattgaacatccctgaccccaggctagccgcattgatcccaaaggggttcgagactgtcgggtgcacctggctggtccccgatcctccggtgccctccccaccggacccgggggcctgggaggtggggggcgaggggctccaggggttagggaggggctctcgattctcagtccgcagaggctgggaggatgagctgtcggagttcccggccagggaagagaagggattgttgccaaactgttcccgggcagcactgaacatgggctcctggatgtccgtgtacatgcggcggagggcattataccctccagggatgctctcaaggttgctcagggcccggtcctggttccgcatcatctcttgcatcatggctggattccgagcaagctccattgtctgcctcatgagttcagggttattgagcatgtggctgatctcagggttccgctccatcaactgctgcatctgggggttggccataatcatgtgacgcatcagatcagggttagacatcatatcctggaccagggggttctccatgatctgtgacagcatctcaggattggacatcagctgccgctgcatctgctgctgcagctccatgaagttggcagagcccaggcctaggctgcccagccccaggatgcccccaaagccagagagtatggacgcagtagcactgggggatccctccccagcccccggagagggccccccaccactgctcctccggcttccactgccagcatctgaagaggcactgccagaggtggagggctgggcaggggtggcgggtgaagcaggcgtggtggagggtgctgaggcagggtcaggtgtggagggggaagaagcagtggcagcagctggatcttgagccttctgaggggtcttgatgaccagatggacagtgagcccgtccttgattccgtgctggttcagtgtgtccccatccttgaggatcttgcctgcgaagatcaggaccagctgatcctgctgagccttaaacctccgggagatttcctctttgaactccttgaccgaggctcgatcgcagatcacaatttcctccttgtccttgggggtcttgacggtgacccgaatggggggcctcgtctcggccccgctcggctccgccatgccgccgccgccacccggccgc

SEQ ID NO: 10171 - RNA, 1037 nt, Homo sapiens
  source 1..1037: mol_type = other RNA
cagcccggatcccagcccactttgcggtcttctgttcctgggtccatgtcataaaatgttgggattcattatgacttcatctgtggccttattttctcacagcatccaatctttctgtgtgatttggttcaaccccctggcttctgctgccacctgagagctaataactctcttctgggcatgacagaccctcccctaacgctcactgggtccccttcttgggtgtctccaaaacacttcgagtcaagcatgtcaaaacggaacacgtcctcctgctccataaactggctttccatgcattttccctcttatggataacctcaccgccttcccccatttacctaatgcagaagcctcagaggtttctctcttctttcccctcaacatctaaccaagctgcaggtcccatcaattgcttttccctaagtagccatcaaatctactcttccatctccagccgacttctcttggtttaaactgtcatctctcctgtgctgggttatttaagtagcttcctaacagatctttctgatgttttcattcccgtaaacccatcatttacacactgcctcagtaatccttccaagtgcaaacaagtccatattaatccaacccatcacggccttcaataaccgctccatgacatttaagacattttctgagggaaagttctgtcattatctggcctcgtcccagccgtccaatcttgataccttgataagcatgttgaaaatgccccatcaggtccgctcagcagggcaaagccgttttgtggaagccggaatgtttatttttgatatggcagtgctgggttgcagagggtgtgtagcacaggtagactacgcaggttgactgtggggcttccagagcctggagaggaaagaagactctaaagaaaagataaatgtccttttcattactgcttcatttcttgagataaaatcattaaaatcatacatgtgtaatgactaaccgaatactcttggtagacaaggagcaaacatgcatgtcctcttaaacatcacgtgttcattgca

SEQ ID NO: 10172 - RNA, 572 nt, Homo sapiens
  source 1..572: mol_type = other RNA
cagcctctgcccttggcctccatcctgtcgtcaggggaactgtggctgtcgtttgtcccagcgagcggcaagtggggagcgcaagaaaaagtagtaattgttaggagatctcgtctcctaactcggggagttctccaagagagttctccaacttctgtccgaggactggagacgcagagtactcacaagtccggcacttgagtggctgcggctgcgacggcaatttagtgacacgcggctcctttatctcccgactttttctctggcatcaaactcgtgcatgctgtgaagctctcagtccctcgctgagttccactgccccctcactaaaaccctggggctagtcggacctctcggtacagcccattcccaggaagggtcggacttctgctggctccgtactgcgggcgacagtcatctccgaagatctcagatcccagtagtgcgggagcactagccgcctcgggttgtagatttcactcaaatgacaagtgaagctagttctcattgagaatgccacccacacgcacaaatacaacaaggcttaccccgattagtgacagctgtggact

SEQ ID NO: 10173 - RNA, 1422 nt, Homo sapiens
  source 1..1422: mol_type = other RNA
cagcctctgcccttggcctccatcctgtcgtcaggggaactgtggctgtcgtttgtcccagcgagcggcaagtggggagcgcaagaaaaagtagtaattgttaggagatctcgtctcctaactcggggagttctccaagagagttctccaacttctgtccgaggactggagacgcagagtactcacaagtccggcacttgagtggctgcggctgcgacggcaatttagtgacacgcggctcctttatctcccgactttttctctggcatcaaactcgtgcatgctgtgaagctctcagtccctcgctgagttccactgccccctcactaaaaccctggggctagtcggacctctcggtacagcccattcccaggaagggtcggacttctgctggctccgtactgcgggcgacagtcatctccgaagatctcagatcccagtagtgcgggagcactagccgcctcgggttgtagatttcactcaaatgacaagtgaagctagttctcattgagaatgccacccacacgcacaaatacaacaaggcttaccccgattagtgacagctgtggactggccagacagctttctaacaacgcctcctcctctagggaggccccgcccaaagcccctccctaccccaattaccggtaggatctgaaactctggagttggcatttccacccgttattctgaatgctactctcaatagcaggttctttgggatggaacctcataagcatattacgttttgttttgcaaattaagaattatgccctatctaattggaaaaatgaatagattctatcagaagtagaatttttgtcaccattttaagatttcagttttgtaaagatttaacacagaggaagacatttggctacattatcttttaaaataataaatgtatcaaggacgatactaaataagagattctctcccttatgagttccataaaagtgaatgctttcaagtttctcctgctgcgaccaacatgtcctgctcctcttgagtatcctcagcgtgacaaagaaatttgggagtgggagatggtaacacctctgtatctatgatggaagtttggatgttgtgtgccacacttcgatttgtcttaaggaatgtgttccaatttttagtaaatagcactttaaggaaagtttcctttagctccagcttatacagtgtgctacatcataacatcctcagtagagatgttgaacagtactttttaccctaaatattcttagtctgaaaagtaattatctttgagcttataaaatggatccccgctaaattcatgaagtcagtagaaaaagggaagaatattgcaatatatattttagatacacagtcataaactgtatttgacccaagaccattgggtattttaacatcatcttaaatataccttgttcaaaacagagt

SEQ ID NO: 10174 - RNA, 1440 nt, Homo sapiens
  source 1..1440: mol_type = other RNA
cagcctctgcccttggcctccatcctgtcgtcaggggaactgtggctgtcgtttgtcccagcgagcggcaagtggggagcgcaagaaaaagtagtaattgttaggagatctcgtctcctaactcggggagttctccaagagagttctccaacttctgtccgaggactggagacgcagagtactcacaagtccggcacttgagtggctgcggctgcgacggcaatttagtgacacgcggctcctttatctcccgactttttctctggcatcaaactcgtgcatgctgtgaagctctcagtccctcgctgagttccactgccccctcactaaaaccctggggctagtcggacctctcggtacagcccattcccaggaagggtcggacttctgctggctccgtactgcgggcgacagtcatctccgaagatctcagatcccagtagtgcgggagcactagccgcctcgggttgtagatttcactcaaatgacaagtgaagctagttctcattgagaatgccacccacacgcacaaatacaacaaggcttaccccgattagtgacagctgtggactggccagacagctttctaacaacgcctcctcctctagggaggccccgcccaaagcccctccctaccccaattaccggtaggatctgaaactctggagttggcatttccacccgttattctgaatgctactctcaatagcaggttctttgggatggaacctcataagcatattacgttttgttttgcaaattaagaattatgccctatctaattggaaaaatgaatagattctatcagaagtagaatttttgtcaccattttaagatttcagttttgtaaagatttaacacagaggaagacatttggctacattatcttttaaaataataaatgtatcaaggacgatactaaataagagattctctcccttatgagttccataaaagtgaatgctttcaagtttctcctgctgcgaccaacatgtcctgctcctcttgagtatcctcagcgtgacaaagaaatttgggagtgggagatggtaacacctctgtatctatgatggaagtttggatgttgtgtgccacacttcgatttgtcttaaggaatgtgttccaatttttagtaaatagcactttaaggaaagtttcctttagctccagcttatacagtgtgctacatcataacatcctcagtagagatgttgaacagtactttttaccctaaatattcttagtctgaaaagtaattatctttgagcttataaaatggatccccgctaaattcatgaagtcagtagaaaaagggaagaatattgcaatatatattttagatacacagtcataaactgtatttgacccaagaccattgggtattttaacatcatcttaaatataccttgttcaaaacagagtgaatgatttgcaaatttt

SEQ ID NO: 10175 - RNA, 905 nt, Homo sapiens
  source 1..905: mol_type = other RNA
cagcctctgcccttggcctcctgcatgagcagcagcctctcccgccgcagtcgcagcccaatgagcaggtagagcacgctcatgatggccatgggcaggcagaagaagagcagcgcggtggtctgcactaccatgttgtagagggcccgtgggcggaccagcatgcaaacagctgagtctggcactgggccccggcagggcacgtgcagctgccggatgccgtgcaggctggtgttgggcagggagcagagcatggcaagaccccagacggccccaagcactcggcgcacatgggcccgcgtcaccatggacctggcctggagtgggtgcaccacggccacatagcgttccacgctcagggcagtgacgttgagcactgaggccaggcagaccatctcaaacagtagcgtgcggaaatagcagccaccaacgcccagcaggaaggggtagttgtgccacatctcatagagctccaggggcaggcccaccagcagcaccagcaggtccgacacggccaggctgaagaggtagtagttggtaggcgtgcgcatggccttgtggcgcaggatgaccagacaggtcagcccattgcccacagcgcccaccacgaagatcagcaggtatgtggcacagatgggcatgaacagctctgtctgctggggccccaggtacttgagtctcagtgcctcgtcagtcaggttcaagtcctcagggtcaaagtgccccctggccgcactgccattgcaagccatggggttccttgcaccccctgggtacaggtctccagggaggacagagcaattgaggcagagaggagtcatgcggcccgcggcccgcgagaccccggcttccaccctccgagcgacggacacagacgcggcgcgggagccagtggactgactgac

SEQ ID NO: 10176 - RNA, 920 nt, Homo sapiens
  source 1..920: mol_type = other RNA
cagcctctgcccttggcctcctgcatgagcagcagcctctcccgccgcagtcgcagcccaatgagcaggtagagcacgctcatgatggccatgggcaggcagaagaagagcagcgcggtggtctgcactaccatgttgtagagggcccgtgggcggaccagcatgcaaacagctgagtctggcactgggccccggcagggcacgtgcagctgccggatgccgtgcaggctggtgttgggcagggagcagagcatggcaagaccccagacggccccaagcactcggcgcacatgggcccgcgtcaccatggacctggcctggagtgggtgcaccacggccacatagcgttccacgctcagggcagtgacgttgagcactgaggccaggcagaccatctcaaacagtagcgtgcggaaatagcagccaccaacgcccagcaggaaggggtagttgtgccacatctcatagagctccaggggcaggcccaccagcagcaccagcaggtccgacacggccaggctgaagaggtagtagttggtaggcgtgcgcatggccttgtggcgcaggatgaccagacaggtcagcccattgcccacagcgcccaccacgaagatcagcaggtatgtggcacagatgggcatgaacagctctgtctgctggggccccaggtacttgagtctcagtgcctcgtcagtcaggttcaagtcctcagggtcaaagtgccccctggccgcactgccattgcaagccatggggttccttgcaccccctgggtacaggtctccagggaggacagagcaattgaggcagagaggagtctaccatgcggcccgcggcccgcgagaccccggcttccaccctccgagcgacggacacagacgcggcgcgggagccagtggactgactgacagcggccccag

SEQ ID NO: 10177 - RNA, 1495 nt, Homo sapiens
  source 1..1495: mol_type = other RNA
cagcctctgcccttggcctcctgtgccctctaccggtgcacgcctgtgtgggcccagcccccatctgtctggtctggccctgagaggctcgggcaccagctgcatcatttctctttcttctccagccccttcgatgctgatgcctctgttccctctttggattctgtcactgccgctggatccttaggatttgactcctcataaatggcgctgggattctgcgggcgccggcggcgagggccagctagcttctgctgcatggagtcggccaggctggctggggagcccgagactgtggggaagtgggtgagcctcggggtatgaggcaggatttccgccgaggactcgtagctgaacatctctgtcacttctcccttggccagcgccaccaggacaggaaaaccgatgcaggcggggaccaggtataggagggcaggctgagcatgcttgaagatgtgcatgatgaagatggtaaggcccaggccgaagatgtaggctgcaaagctggtgtagaagtaggtgtgggtattcttcttcaagctgatgtcaaagcgcagcagcaaggcaatgaagatccctggaatgacgacatctccaagtcccagcatggcaaagttgtttgcttcgaggcctttctccagcagatcctggggaaacaccaattttattggtgcctcgaaggacttggccactgtcaccatcacattggtgccaaatacccagaagacatcgtagatgaagagtccgcccagcaggatgcagccagtgctgacattgttgaggtgcaggagctctactccattaagggagaaggccaggccaaaaaggttgttggcaatccagtgcttcctcagcaggtaccagacgccaacgatgctgctcaggcccaggcacaccaggtccttggtgtcaaattcataattgatgatctcttccttgttttccccagaaccctgtgtgaagagcagctggtactgtcgatttggaaagctggctggaaaaaacttattcatgaaggggctgatggtgtgggacagggccaggattcccagcacgaagaaatacatggacagcaggaggttgatgtactcctgggagaatattttgaaaaagaggtagagccccaagagtgtgcagctggcgatgatggggaagcgggcggcatcccggctggtgattgtttcaggcatgtctgaagcattcttgccgcgggcgcagcgtacggagcgcagggcgccgaagaagatgggcagcagcgccatgagcaggaggctgccgtaggccagcgcgatgccctcgggcgtggaaggcggccgcgtagtgctgttggtggggccgcctgcctcggcactgccgttatgcggatcgctgagggccgagtccatggcgagggtgcgttcgggatccgactccagctccggttgctgcagcagggacgcaggcggagacaccggctctgcagggaaagccacgttcccctaaggcaacaggaagt

SEQ ID NO: 10178 - RNA, 1348 nt, Homo sapiens
  source 1..1348: mol_type = other RNA
cagcctctgcccttggcctcctgtgccctctaccggtgcacgcctgtgtgggcccagcccccatctgtctggtctggccctgagaggctcgggcaccagctgcatcatttctctttcttctccagccccttcgatgctgatgcctctgttccctctttggattctgtcactgccgctggatccttaggatttgactcctcataactgaacatctctgtcacttctcccttggccagcgccaccaggacaggaaaaccgatgcaggcggggaccaggtataggagggcaggctgagcatgcttgaagatgtgcatgatgaagatggtaaggcccaggccgaagatgtaggctgcaaagctggtgtagaagtaggtgtgggtattcttcttcaagctgatgtcaaagcgcagcagcaaggcaatgaagatccctggaatgacgacatctccaagtcccagcatggcaaagttgtttgcttcgaggcctttctccagcagatcctggggaaacaccaattttattggtgcctcgaaggacttggccactgtcaccatcacattggtgccaaatacccagaagacatcgtagatgaagagtccgcccagcaggatgcagccagtgctgacattgttgaggtgcaggagctctactccattaagggagaaggccaggccaaaaaggttgttggcaatccagtgcttcctcagcaggtaccagacgccaacgatgctgctcaggcccaggcacaccaggtccttggtgtcaaattcataattgatgatctcttccttgttttccccagaaccctgtgtgaagagcagctggtactgtcgatttggaaagctggctggaaaaaacttattcatgaaggggctgatggtgtgggacagggccaggattcccagcacgaagaaatacatggacagcaggaggttgatgtactcctgggagaatattttgaaaaagaggtagagccccaagagtgtgcagctggcgatgatggggaagcgggcggcatcccggctggtgattgtttcaggcatgtctgaagcattcttgccgcgggcgcagcgtacggagcgcagggcgccgaagaagatgggcagcagcgccatgagcaggaggctgccgtaggccagcgcgatgccctcgggcgtggaaggcggccgcgtagtgctgttggtggggccgcctgcctcggcactgccgttatgcggatcgctgagggccgagtccatggcgagggtgcgttcgggatccgactccagctccggttgctgcagcagggacgcaggcggagacaccggctctgcagggaaagccacgttcccctaaggcaacaggaagt

SEQ ID NO: 10179 - RNA, 1551 nt, Homo sapiens
  source 1..1551: mol_type = other RNA
cagcctctgcccttggcctcctgtgccctctaccggtgcacgcctgtgtgggcccagcccccatctgtctggtctggccctgagaggctcgggcaccagctgcatcatttctctttcttctccagccccttcgatgctgatgcctctgttccctctttggattctgtcactgccgctggatccttaggatttgactcctcataacttgggccccggggcagtagggggaagcgggcaggtgggcacccgctgggcattacatggcgctgggattctgcgggcgccggcggcgagggccagctagcttctgctgcatggagtcggccaggctggctggggagcccgagactgtggggaagtgggtgagcctcggggtatgaggcaggatttccgccgaggactcgtagctgaacatctctgtcacttctcccttggccagcgccaccaggacaggaaaaccgatgcaggcggggaccaggtataggagggcaggctgagcatgcttgaagatgtgcatgatgaagatggtaaggcccaggccgaagatgtaggctgcaaagctggtgtagaagtaggtgtgggtattcttcttcaagctgatgtcaaagcgcagcagcaaggcaatgaagatccctggaatgacgacatctccaagtcccagcatggcaaagttgtttgcttcgaggcctttctccagcagatcctggggaaacaccaattttattggtgcctcgaaggacttggccactgtcaccatcacattggtgccaaatacccagaagacatcgtagatgaagagtccgcccagcaggatgcagccagtgctgacattgttgaggtgcaggagctctactccattaagggagaaggccaggccaaaaaggttgttggcaatccagtgcttcctcagcaggtaccagacgccaacgatgctgctcaggcccaggcacaccaggtccttggtgtcaaattcataattgatgatctcttccttgttttccccagaaccctgtgtgaagagcagctggtactgtcgatttggaaagctggctggaaaaaacttattcatgaaggggctgatggtgtgggacagggccaggattcccagcacgaagaaatacatggacagcaggaggttgatgtactcctgggagaatattttgaaaaagaggtagagccccaagagtgtgcagctggcgatgatggggaagcgggcggcatcccggctggtgattgtttcaggcatgtctgaagcattcttgccgcgggcgcagcgtacggagcgcagggcgccgaagaagatgggcagcagcgccatgagcaggaggctgccgtaggccagcgcgatgccctcgggcgtggaaggcggccgcgtagtgctgttggtggggccgcctgcctcggcactgccgttatgcggatcgctgagggccgagtccatggcgagggtgcgttcgggatccgactccagctccggttgctgcagcagggacgcaggcggagacaccggctctgcagggaaagccacgttcccctaaggcaacaggaagt

SEQ ID NO: 10180 - RNA, 1474 nt, Homo sapiens
  source 1..1474: mol_type = other RNA
cagcggagcctggagagaaggcaatgacacctctgtgctatatgctgggagggatgacggcccgcaacccagcctggggggtcagggaaggctccctggtgggagtgatagcattgctgtcattatcagtcaccataatcaatatcataacaacatgtgttgttatgataatgataatgcccaacattatgtgctgggcagggtactaggcaaagtatatgtcataccagttgactcctgacaacctcctagagcaggtatgcttctcatcattttacaaatgtggagactgaggcctgaagttcacccagccgtgaagtggggagatgagatttggctctagagctcatgctcttgatgactgtgctctgcagttccctgctttaaactgacccttgactgagcaataggaattcaccacgtggttctgtgcaagggaacggcattcagcaatcatgggtttcacacctcctatgcaccagctgtaggtgctggagagagggaagtaaggtcagtggcctgctcttgagggctcacagattatctgagaagaaggtaagaagacagagaattccagcagaatggtaagtactggtagacaaatgctggaggttatggaagtcagaaggcacctcgacagcctttaaggtagagacagaggcccatcagggaaggcttcctggaagaggtaaggctagaaataatgctggaagtgatgccagaaaacaccatgggagttagcaaacagtggaaagaagaaccaggtgtagtggctcacacttgtaatcccagcattttgggaggctgaggcagatggatcacctgagctcaggagtttgagaccagcctgaccaacatagtgaaaccctgtctctaccaaaaatacaaaattatccaggtgtggtggcgtgtgactgtaatcccagctacttgggaggctgaggcaggagaattgcttgaacccgggaggcagaggttacagtgagctgagatcacgcgattgcactccagccatgcacttgcggtcatctatgcctgtcagatcctcctcaaactccttcccaacctggaagtccatgatgtagttcctaaaagtgctcagcgtgcggatgatcatatggtcaccgtcctgcacgatctctttgtctggcttcagcaagttggcgattttgcgcaaggccacattgacgtcgagggcgcgcaggtactcctcgaaattctcgttgaccaacatcttccagtacccagtgaagtcgactggcatttcggggagtgactggagccagttggccacaagcgggcgggacggctggagactgccgggacagcggctgccggtgctacgcgggtggtgggcggcccggaaatgagcgccctccggggacagggggctctgcggggcggcgacagctggattcccagcgcgcacaaagcctgcgggaggatccattgtagcggtcgctcctccccgctt

SEQ ID NO: 10181 - RNA, 604 nt, Homo sapiens
  source 1..604: mol_type = other RNA
cagcggagcctggagagaaggctgggaggcaggagctgggtctaaagaggccattgtaacgatggagctgtgcccgtggaggctgttgtgaggcagtagcctcatctgcggaggctgccgtgacgtagggtatgggcctaaataggccattgagagtcatgagcttggtctgtagaggctgactggagaaagttctgggcctggagaggctgccgggaggtaggagcataatgtagaatcagtgggcgtgttaagcttgttttcctgcaactggatggtcccacctgaataacatgttgcccagtcagtctctcttcctggattcacaagtctttcatggtagatccagctccagctctgtggccctgtggttggagaccgctgctcaagtgcatttgaaaggaaccatcccacgccattcttcagagtcatctttactgctgcagtggtcaacttgtagcacccctaagctcgcaggacatatgcttcaactggcatttcacaatcaacagtatgtggcagcttgagtcattgtgagctcacttcctgtaatcccagctactcgggaggctgaggcaggagaattgcttgagcctggcaggtg

SEQ ID NO: 10182 - RNA, 1022 nt, Homo sapiens
  source 1..1022: mol_type = other RNA
cagcggagcctggagagaaggctgggaggcaggagctgggtctaaagaggccattgtaacgatggagctgtgcccgtggaggctgttgtgaggcagtagcctcatctgcggaggctgccgtgacgtagggtatgggcctaaataggccattgagagtcatgagcttggtctgtagaggctgactggagaaagttctgggcctggagaggctgccgggaggtaggagcataatgtagaatcagtgggcgtgttaagcttgttttcctgcaactggatggtcccacctgaataacatgttgcccagtcagtctctcttcctggattcacaagtctttcatggtagatccagctccagctctgtggccctgtggttggagaccgctgctcaagtgcatttgaaaggaaccatcccacgccattcttcagagtcatctttactgctgcagtggtcaacttgtagcacccctaagctcgcaggacatatgcttcaactggcatttcacaatcaacagtatgtggcagcttgagtcattgtgagctcacttcctgtagtcccagctactgggaaggctgacatggtaggattgcttgagcctgggagtttgaggctataatgagccatgataggaccactgaactccatcctagtgacagggcaaggtcctgtttctcatttctgtgctgcttgggaggcctggacagcccaataaccagctcctcgctgatgaagcaatcaggaaatggctcgagttgagctaaggagaatttggatccttcctttggttctcagtaggcagggtaggggccaggcatggtggctcatacctgtaatccttgcacttgtcctgtgcatctctttcattggctgttcctgagatggagccattacattgagccagtaatagaaaataaggtggccagatgcgctggctcatgcccgtaatcccagcactttgggaggcagaggtgggcggaatcacttgagcctaggaatttgagaccaacctgggcaacataagaag

SEQ ID NO: 10183 - RNA, 1073 nt, Homo sapiens
  source 1..1073: mol_type = other RNA
cagcggagcctggagagaaggctgggaggcaggagctgggtctaaagaggccattgtaacgatggagctgtgcccgtggaggctgttgtgaggcagtagcctcatctgcggaggctgccgtgacgtagggtatgggcctaaataggccattgagagtcatgagcttggtctgtagaggctgactggagaaagttctgggcctggagaggctgccgggaggtaggagcataatgtagaatcagtgggcgtgttaagcttgttttcctgcaactggatggtcccacctgaataacatgttgcccagtcagtctctcttcctggattcacaagtctttcatggtagatccagctccagctctgtggccctgtggttggagaccgctgctcaagtgcatttgaaaggaaccatcccacgccattcttcagagtcatctttactgctgcagtggtcaacttgtagcacccctaagctcgcaggacatatgcttcaactggcatttcacaatcaacagtatgtggcagcttgagtcattgtgagctcacttcctgtagtcccagctactgggaaggctgacatggtaggattgcttgagcctgggagtttgaggctataatgagccatgataggaccactgaactccatcctagtgacagggcaaggtcctgtttctcgtgactccatattcaaggccagaagtgcagcatcttcaaatctccctctctgacctcttcttccattaccacatcactttctctaattctgactctcctacctcattctcttataaagatccttgtgattggtgggtatgggggctcccatctgtaatcccaacattttgggaggccaaagaggaaggattgcttgaggccaagagttagagatcagccttgtcctgtgcatctctttcattggctgttcctgagatggagccattacattgagccagtaatagaaaataaggtggccagatgcgctggctcatgcccgtaatcccagcactttgggaggcagaggtgggcggaatcacttgagcctaggaatttgagaccaacctgggcaacataagaag

SEQ ID NO: 10184 - RNA, 718 nt, Homo sapiens
  source 1..718: mol_type = other RNA
cagcggagcctggagagaaggctgggaggcaggagctgggtctaaagaggccattgtaacgatggagctgtgcccgtggaggctgttgtgaggcagtagcctcatctgcggaggctgccgtgacgtagggtatgggcctaaataggccattgagagtcatgagcttggtctgtagaggctgactggagaaagttctgggcctggagaggctgccgggaggtaggagcataatgtagaatcagtgggcgtgttaagcttgttttcctgcaactggatggtcccacctgaataacatgttgcccagtcagtctctcttcctggattcacaagtctttcatggtagatccagctccagctctgtggccctgtggttggagaccgctgctcaagtgcatttgaaaggaaccatcccacgccattcttcagagtcatctttactgctgcagtggtcaacttgtagcacccctaagctcgcaggacatatgcttcaactggcatttcacaatcaacagtatgtggcagcttgagtcattgtgagctcacttcctgtagtcccagctactgggaaggctgacatggtaggattgcttgagcctgggagtttgaggctataatgagccatgataggaccactgaactccatcctagtgacagggcaaggtcctgtttctggacatggtggcacatgtctgtagtcccagctacttgggagactgaa

SEQ ID NO: 10185 - RNA, 852 nt, Homo sapiens
  source 1..852: mol_type = other RNA
cagcggagcctggagagaaggctgggaggcaggagctgggtctaaagaggccattgtaacgatggagctgtgcccgtggaggctgttgtgaggcagtagcctcatctgcggaggctgccgtgacgtagggtatgggcctaaataggccattgagagtcatgagcttggtctgtagaggctgactggagaaagttctgggcctggagaggctgccgggaggtaggagcataatgtagaatcagtgggcgtgttaagcttgttttcctgcaactggatggtcccacctgaataacatgttgcccagtcagtctctcttcctggattcacaagtctttcatggtagatccagctccagctctgtggccctgtggttggagaccgctgctcaagtgcatttgaaaggaaccatcccacgccattcttcagagtcatctttactgctgcagtggtcaacttgtagcacccctaagctcgcaggacatatgcttcaactggcatttcacaatcaacagtatgtggcagcttgagtcattgtgagctcacttcctgtagtcccagctactgggaaggctgacatggtaggattgcttgagcctgggagtttgaggctataatgagccatgataggaccactgaactccatcctagtgacagggcaaggtcctgtttcttgtcctgtgcatctctttcattggctgttcctgagatggagccattacattgagccagtaatagaaaataaggtggccagatgcgctggctcatgcccgtaatcccagcactttgggaggcagaggtgggcggaatcacttgagcctaggaatttgagaccaacctgggcaacataagaag

SEQ ID NO: 10186 - RNA, 392 nt, Homo sapiens
  source 1..392: mol_type = other RNA
cagcggagcctggagagaaggctgggaggcaggagctgggtctaaagaggccattgtaacgatggagctgtgcccgtggaggctgttgtgaggcagtagcctcatctgcggaggctgccgtgacgtagggtatgggcctaaataggccattgagagtcatgagcttggtctgtagaggctgactggagaaagttctgggcctggagaggctgccgggaggtaggagcataatgtagaatcagtgggcgtgttaagcttgttttcctgcaactggatggtcccacctgaataacatgttgcccagtcagtctctcttcctggattcacaagtctttcatggtagatccagctgtaatcccagctactcgggaggctgaggcaggagaattgct

SEQ ID NO: 10187 - RNA, 655 nt, Homo sapiens
  source 1..655: mol_type = other RNA
cagcggagcctggagagaaggctgggaggcaggagctgggtctaaagaggccattgtaacgatggagctgtgcccgtggaggctgttgtgaggcagtagcctcatctgcggaggctgccgtgacgtagggtatgggcctaaataggccattgagagtcatgagcttggtctgtagaggctgactggagaaagttctgggcctggagaggctgccgggaggtaggagcataatgtagaatcagtgggcgtgttaagcttgttttcctgcaactggatggtcccacctgaataacatgttgcccagtcagtctctcttcctggattcacaagtctttcatggtagatccagctgtagtcccagctactgggaaggctgacatggtaggattgcttgagcctgggagtttgaggctataatgagccatgataggaccactgaactccatcctagtgacagggcaaggtcctgtttcttgtcctgtgcatctctttcattggctgttcctgagatggagccattacattgagccagtaatagaaaataaggtggccagatgcgctggctcatgcccgtaatcccagcactttgggaggcagaggtgggcggaatcacttgagcctaggaatttgagaccaacctgggcaacataagaag

SEQ ID NO: 10188 - RNA, 532 nt, Homo sapiens
  source 1..532: mol_type = other RNA
cagcggagcctggagagaaggctgggaggcaggagctgggtctaaagaggccattgtaacgatggagctgtgcccgtggaggctgttgtgaggcagtagcctcatctgcggaggctgccgtgacgtagggtatgggcctaaataggccattgagagtcatgagcttggtctgtagaggctgactggagaaagttctgggcctggagaggctgccgggaggtaggagcataatgtagaatcagtgggcgtgttaagcttgttttcctgcaactggatggtcccacctgaataacatgttgcccagtcagtctctcttcctggattcacaagtctttcatggtagatccagcttgtcctgtgcatctctttcattggctgttcctgagatggagccattacattgagccagtaatagaaaataaggtggccagatgcgctggctcatgcccgtaatcccagcactttgggaggcagaggtgggcggaatcacttgagcctaggaatttgagaccaacctgggcaacataagaag

SEQ ID NO: 10189 - RNA, 909 nt, Homo sapiens
  source 1..909: mol_type = other RNA
cagcggagcctggagagaaggctgggaggcaggagctgggtctaaagaggccattgtaacgatggagctgtgcccgtggaggctgttgtgaggcagtagcctcatctgcggaggctgccgtgacgtagggtatgggcctaaataggccattgagagtcatgagcttggtctgtagaggctgactggagaaagttctgggcctggagaggctgccgggaggtaggagcataatgtagaatcagtgggcgtgttaagcttgttttcctgcaactggatggtcccacctgaataacatgttgcccagtcagtctctcttcctggattcacaagtctttcatggtagatccagtataacgtagactcagtgggatctctgagcttgttttcctgcaactagactgtccacctccagctctgtggccctgtggttggagaccgctgctcaagtgcatttgaaaggaaccatcccacgccattcttcagagtcatctttactgctgcagtggtcaacttgtagcacccctaagctcgcaggacatatgcttcaactggcatttcacaatcaacagtatgtggcagcttgagtcattgtgagctcacttcctgtagtcccagctactgggaaggctgacatggtaggattgcttgagcctgggagtttgaggctataatgagccatgataggaccactgaactccatcctagtgacagggcaaggtcctgtttcttgtcctgtgcatctctttcattggctgttcctgagatggagccattacattgagccagtaatagaaaataaggtggccagatgcgctggctcatgcccgtaatcccagcactttgggaggcagaggtgggcggaatcacttgagcctaggaatttgagaccaacctgggcaacataagaag

SEQ ID NO: 10190 - RNA, 449 nt, Homo sapiens
  source 1..449: mol_type = other RNA
cagcggagcctggagagaaggctgggaggcaggagctgggtctaaagaggccattgtaacgatggagctgtgcccgtggaggctgttgtgaggcagtagcctcatctgcggaggctgccgtgacgtagggtatgggcctaaataggccattgagagtcatgagcttggtctgtagaggctgactggagaaagttctgggcctggagaggctgccgggaggtaggagcataatgtagaatcagtgggcgtgttaagcttgttttcctgcaactggatggtcccacctgaataacatgttgcccagtcagtctctcttcctggattcacaagtctttcatggtagatccagtataacgtagactcagtgggatctctgagcttgttttcctgcaactagactgtccacctgtaatcccagctactcgggaggctgaggcaggagaattgct

SEQ ID NO: 10191 - RNA, 589 nt, Homo sapiens
  source 1..589: mol_type = other RNA
cagcggagcctggagagaaggctgggaggcaggagctgggtctaaagaggccattgtaacgatggagctgtgcccgtggaggctgttgtgaggcagtagcctcatctgcggaggctgccgtgacgtagggtatgggcctaaataggccattgagagtcatgagcttggtctgtagaggctgactggagaaagttctgggcctggagaggctgccgggaggtaggagcataatgtagaatcagtgggcgtgttaagcttgttttcctgcaactggatggtcccacctgaataacatgttgcccagtcagtctctcttcctggattcacaagtctttcatggtagatccagtataacgtagactcagtgggatctctgagcttgttttcctgcaactagactgtccaccttgtcctgtgcatctctttcattggctgttcctgagatggagccattacattgagccagtaatagaaaataaggtggccagatgcgctggctcatgcccgtaatcccagcactttgggaggcagaggtgggcggaatcacttgagcctaggaatttgagaccaacctgggcaacataagaag

SEQ ID NO: 10192 - RNA, 429 nt, Homo sapiens
  source 1..429: mol_type = other RNA
cagcggagcctggagagaaggctgggaggcaggagctgggtctaaagaggccattgtaacgatggagctgtgcccgtggaggctgttgtgaggcagtagcctcatctgcggaggctgccgtgacgtagggtatgggcctaaataggccattgagagtcatgagcttggtctgtagaggctgactggagaaagttctgggcctggagaggctgccgggaggtaggagcataatgtagaatcagtgggcgtgttaagcttgttttcctgcaactggatggtcccacgtttcgctgtcacccctctggaatccacgtatacgaaaattccaaatgttagttgggcatagtggcaagcacctgtagtctcagccacgtgggaggttgaggtgggaggatcgcttcagcctggaaggttgaggctgcagtcagc

SEQ ID NO: 10193 - RNA, 433 nt, Homo sapiens
  source 1..433: mol_type = other RNA
cagcggagcctggagagaaggctgggaggcaggagctgggtctaaagaggccattgtaacgatggagctgtgcccgtggaggctgttgtgaggcagtagcctcatctgcggaggctgccgtgacgtagggtatgggcctaaataggccattgagagtcatgagcttggtctgtagaggctgactggagaaagttctgggcctggagaggctgccgggaggtaggagcataatgtagaatcagtgggcgtgttaagcttgttttcctgcaactggatggtcccactcacgtttcgctgtcacccctctggaatccacgtatacgaaaattccaaatgttagttgggcatagtggcaagcacctgtagtctcagccacgtgggaggttgaggtgggaggatcgcttcagcctggaaggttgaggctgcagtcagc

SEQ ID NO: 10194 - RNA, 852 nt, Homo sapiens
  source 1..852: mol_type = other RNA
cagcggagcctggagagaaggctgggaggcaggagctgggtctaaagaggccattgtaacgatggagctgtgcctgtggaggctgctgtgaggcagtaggctcatctgcggaggctgccgtgacgtagggtatgggcctaaataggccattgtgagtcatgagcttggtctgtagaggctgactggagaaagttctgggcctggagaggctgccgggaggtaggagcataatgtagaatcagggggcgtgttaagcttgttttcctgcaactggatgttcccacctgaataacatgttgcccagtcagtctctcttcctggattcacaagtctttcatggtagatccagctccagctctgtggccctgtggttggagaccgctgctcaagtgcatttgaaaggaaccatcccacgccattcttcagagtcatctttactgctgcagtggtcaacttgtagcacccctaagctcgcaggacatatgcttcaactggcatttcacaatcaacagtatgtggcagcttgagtcattgtgagctcacttcctgtagtcccagctactgggaaggctgacatggtaggattgcttgagcctgggagtttgaggctataatgagccatgataggaccactgaactccatcctagtgacagggcaaggtcctgtttcttgtcctgtgcatctctttcattggctgttcctgagatggagccattacattgagccagtaatagaaaataaggtggccagatgcgctggctcatgcccgtaatcccagcactttgggaggcagaggtgggcggaatcacttgagcctaggaatttgagaccaacctgggcaacataagaag

SEQ ID NO: 10195 - RNA, 655 nt, Homo sapiens
  source 1..655: mol_type = other RNA
cagcggagcctggagagaaggctgggaggcaggagctgggtctaaagaggccattgtaacgatggagctgtgcctgtggaggctgctgtgaggcagtaggctcatctgcggaggctgccgtgacgtagggtatgggcctaaataggccattgtgagtcatgagcttggtctgtagaggctgactggagaaagttctgggcctggagaggctgccgggaggtaggagcataatgtagaatcagggggcgtgttaagcttgttttcctgcaactggatgttcccacctgaataacatgttgcccagtcagtctctcttcctggattcacaagtctttcatggtagatccagctgtagtcccagctactgggaaggctgacatggtaggattgcttgagcctgggagtttgaggctataatgagccatgataggaccactgaactccatcctagtgacagggcaaggtcctgtttcttgtcctgtgcatctctttcattggctgttcctgagatggagccattacattgagccagtaatagaaaataaggtggccagatgcgctggctcatgcccgtaatcccagcactttgggaggcagaggtgggcggaatcacttgagcctaggaatttgagaccaacctgggcaacataagaag

SEQ ID NO: 10196 - RNA, 909 nt, Homo sapiens
  source 1..909: mol_type = other RNA
cagcggagcctggagagaaggctgggaggcaggagctgggtctaaagaggccattgtaacgatggagctgtgcctgtggaggctgctgtgaggcagtaggctcatctgcggaggctgccgtgacgtagggtatgggcctaaataggccattgtgagtcatgagcttggtctgtagaggctgactggagaaagttctgggcctggagaggctgccgggaggtaggagcataatgtagaatcagggggcgtgttaagcttgttttcctgcaactggatgttcccacctgaataacatgttgcccagtcagtctctcttcctggattcacaagtctttcatggtagatccagtataacgtagactcagtgggatctctgagcttgttttcctgcaactagactgtccacctccagctctgtggccctgtggttggagaccgctgctcaagtgcatttgaaaggaaccatcccacgccattcttcagagtcatctttactgctgcagtggtcaacttgtagcacccctaagctcgcaggacatatgcttcaactggcatttcacaatcaacagtatgtggcagcttgagtcattgtgagctcacttcctgtagtcccagctactgggaaggctgacatggtaggattgcttgagcctgggagtttgaggctataatgagccatgataggaccactgaactccatcctagtgacagggcaaggtcctgtttcttgtcctgtgcatctctttcattggctgttcctgagatggagccattacattgagccagtaatagaaaataaggtggccagatgcgctggctcatgcccgtaatcccagcactttgggaggcagaggtgggcggaatcacttgagcctaggaatttgagaccaacctgggcaacataagaag

SEQ ID NO: 10197 - RNA, 417 nt, Homo sapiens
  source 1..417: mol_type = other RNA
cagcggagcctggagagaaggctgggaggcaggagctgggtctaaagaggccattgtaacgatggagctgtgcctgtggaggctgttgtgaggcagtagcctcatctgcggaggctgccgtgacgtagggtatgggcctaaataggccattgagagtcatgagcttggtctgtagaggctgactggagaaagttctgggcctggagaggctgccgggaggtaggagcataatgtagaatcagtgggcgtgttaagcttgttttcctgcaactggatggtcccacctcctgctgtgtggctccttgcggctccatggctcaggggttggggacccctgctcaagtgcatccaaagcgacccttcccacaccagtcttcacagtggtccagggcagcaaccacttagctcccaaggcat

SEQ ID NO: 10198 - RNA, 592 nt, Homo sapiens
  source 1..592: mol_type = other RNA
cagcggagcctggagagaaggctgggaggcaggagctgggtctaaagaggccattgtaacgatggagctgtgcctgtggaggctgttgtgaggcagtagcctcatctgcggaggctgccgtgacgtagggtatgggcctaaataggccattgagagtcatgagcttggtctgtagaggctgactggagaaagttctgggcctggagaggctgccgggaggtaggagcataatgtagaatcagtgggcgtgttaagcttgttttcctgcaactggatggtcccacctcctgctgtgtggctccttgcggctccatggctcaggggttggggacccctgctcaagtgcatccaaagcgacccttcccacaccagtcttcacagtggtccagggcagcaaccacttagctcccaaggcatgtgcctcagctggcatttcgtcacaatcaacagtaagtggtagcttgagtcactgtgaggtcacctactggaaatcaccagcatcccatttcccactggcaaagagctcagcactgccccctgggaaaccaaacctatgcccaaatcccatctgtgtgggtttacctcctgggac

SEQ ID NO: 10199 - RNA, 916 nt, Homo sapiens
  source 1..916: mol_type = other RNA
cagcggagcctggagagaaggctgggaggcaggagctgggtctaaagaggccattgtaacgatggagctgtgcctgtggaggctgttgtgaggcagtaggctcatctgcggaggctgccgtgacgtagggtatgggcctaaataggccattgtgagtcatgagcttggtctgtagaggctgactggagaaagttctgggcctggagaggctgccgggaggtaggagcataatgtagaatcagtgggcgtgttaagcttgttttcccgcaactggatgttcccacctgaataacatgttgcccagtcagtctctcttcctggattcacaagtctttcatggtagatccagtataacgtagactcagtgggatctctgagcttgttttcctgcaactagactgtccaccttgtcctgtgcatctctttcattggctgttcctgagatggagccattacattgagccagtaatagaaaataaggtggccagatgcgctggctcatgcccgtaatcccagcactttgggaggcagaggtgggcggaatcacttgagcctaggaatttgagaccaacctgggcaacataagaagaccccatctgaataacatgttgcccagtcagtttctcttcctggattcagaagtctttcatggtaggtccagttgtccatccattttctatattccagcactgggaaaccagggacagtacttgttctcaagggaatcttcagcttaggtggctcttttaataacaaaaaaatcctttccttctaaagtaacatcctctcaaggccaggaattccattagtagaaagccttcctaaaaaacaaaattcctggccaggcatgggttcacgtctgtaatctcagcactctgggaggccgaggcgggaagatcacttgatatcaggagtc

SEQ ID NO: 10200 - RNA, 6984 nt, Homo sapiens
  source 1..6984: mol_type = other RNA
caggaaggagacaggcagttcactgtgaattctgagtagtttccctaaaacactgtttccacataaatacaataaactctattattggtatgtcacaagtgctagataaactttttttcttaatatgacaaatgtttaagtagtcctttttatttttcttacaataaaaagtacaatttcttaagaataagttcaataagacgcaaacttccccgccctcctctccttcaaggttttgttttacagaaaaatttccatcttttgtatctgcaaatgtcatgagaggggaacagaaaggcatttttcttcttccccaaagctgccgagtttggcgtgcaaaatctgtatacaatataaagtcatgccggtcgtacagtccatgcaacctccaggtgtaggaaacttaaaaaaatatattcatatatatttatatctatatatttatatatgtatcaatgcccataaaacacgtgggcccaaagtctacaaaaagaagaatggaatgagcacgtggctgtgaccagtaaagaaggaatgttctgatcaaaaagaaaaacaacaaagtccattgctagtgctgcaaaaatcaaacttgcttttgtgtcagaccattacgaaatggtccttccccttgcaaacagattttcaaaagaagtaaagaaaaactgaaacaccttgacaaagtggccctccagaaccagagccctgggacgctggggaggggcggccagtcccagcgggccacggcctccgggacagccgcctgctggtggggcgtgggcacgtgggcacgctgcggcacggcgggaagccgcgagggcagggcagacgccaagaggcccagtggcgtcatcagggtttccctcaaagggatataaagtgctcgcttgctgactcccagccagtgcccccaaggcctttgcaaaggaagaaaaaggctaaaggtccaaggacccacagggagaacacatgaaggaaccctccctgacgtggtcccgcctgcagacgccgaggcagatcctctgccatctgccctggacgcttgctgtggagaagagccgagtgtgtcttcaaagaaaaggctacacagtaatgctctcagcacatttgtgaagctggagtgagctgacagatgaaacgtgcctccccctgccaggcctttgcagagggcgtctccatttgaatgagattagaattaagtccccccactgataacctggccactgagcagtccatgttatcccatcatctgcttaaaaaaaaaaagtgagatgatgcattcctccccataagccacggcggggtaagagggcaggtggcaggatccccagagggctatgcagagaatgaggccaaggaggccagaagagcctgctagctgggccctgccactgctctgtgccatgaatggggaatggaccagctcctcttgccaatctgggcttcagagcaaagagtggccaccagggaggggaaagtcaaacaagtcccaagaccgttctgcctgctctcaaaccactgtctcagagctgaccatcagcagcccagtgaccaagtgaatccaagaatctgcactcatttggtcaaaagtttgagttaatttcagaagctaccctgtaaactttaccaaactccgaaactcggctctgggtccctcctgagcacggtgtgtctgaacttctgcccccaagtctgaacccaatatacactttggaatgaaactggtggcttcatgtgctggaaaataagttaccagtaaaacgtgactgtcagttactgttgaagagaaaaagagtaaagactggctgtcctggtcaggcaatcataccctccctgcaggttcaccaggcaacaagggtccctgggttccttgcagccacaggctccaaaatccagggctggccacgtggctgcagtggaaaaacccaagtgggtaaagagccccacgtgtgccccatgcattgctgacatgctcaaaaggtctttggaaaactcaagttagaattctatcctgacgatgtggtcagagaagtttaaacatgagtttcattaatgctgactgcccccggcatctggcaagcctcccagggtggccgggcatcctaagcaaccctccctgcccttgccacggaggggaaaaacacaccacccctcgtaatactactagtgttgaaagttaaaaagagcccctgggcttctttatacagctcctaggacagaccaggaaagacacaatcgttggtgtcactccgaaaagacctacggtccctcctctcactttctgaaaatagaatctgacagcaacaattctgtacgctgcagaaaactcatcgtacaaaaataaaaacaaaaataattaaaaacctttgaaaggtaaaaaaaaatgtacaagcaagaattcagaaaggaaaaagatttagacattattaccattcagaaaattgctaaatggtgaggaaaaatgtaaaattcataaaacaatgcttattcaggatctttttgtgaaaaaattcatacaaaaatcaacagcaaatttatattctttgctataaaaactcattaggtacatatgtgcatgaaggcttggagacgggagcggttctgttagaaaataattaaaatgaaagtacaaacttgtagggtagttgcccagtggcgaatgtgttggcgatctgaaatctagccaatctggagcttgagaaaacatgaatttcaatcaatcaggatccctttccataagcaccttgagagcaaattcacaagccatccatttgcagggaccttcgcaatctgcattcattttatatatatatatatactttttctataaatgcattataaatattttatcaagatttcataagaatcaagtaagtttcttagcttggaatacattggaatatatattatacatatatatatttatttatacctaaaatttaagcaatacttcatgctacttgcttttaataaaaagcattccgatcgtaacactgcaagtgtgcctaccacatgcttcacgaccagatggagatgctcaatcgtatgtgacgtgtgagaacactttggattcgtttaaaatttgttggacttcaaaacctccaacgggatttgccacttttttggaactacctccatttttcttaaacagcaataaagcaaaacagggaccgccgggctgcagcccctggccccggagatgacggctggtgcccgtgcttgaggcgtcaggccagctcgcggtgccagcactgccaggctcggctggccacaggaaactgtcccaccgattcctgctgtttgttttttcttaaggcattgttcctcagacttcagaaaacccagccacaaaaatccaccagagcaataaaaaaaaaggcacaaactcgcatcttccgatggcttttgagaaactcaagccagctcccccagctcacattcctgtttctgtccagttttgttttctttaaaggtccctctgtcccccacccgggtgcagaccccccgccgcacaccgctatggttcacagaggcgggccacagccgtagaaaacgtcctctttaaaaaaaaataagctacaagatgagtcgagtggtttacacagagactgtggagttgtgggtaataaactttaagcaccagttttaatcaagtttgttttgtattattagatctttgatatttgttttctgtgcctcgtgtcaactgaattcggcagctcggccgcctgttgccacaggctcctttcttccacggcgtcccttgcgggacccgccagagtgtgcttggcttccgcgtgtccgtgtgtctgcgcgtcgccggcgtctgtcccgtgttccctgtgaggctgccacgcccaggcgtgcatgtgcgtctcgagacctgtgggcctgggcggcagaaaggcttcccgtggctgttgcacgctgggtgtccctgggtgctccaagagagccccacggtgggacgcaggcgtgacacgggaaagtttcttggctgagcttcaagacagagacagacagacaagagaacagcagcttcgagggagtgctacaggggcggctcctcttccatgggctcctcatctggtctcttttcggcgggcttcacgcccacggacagcgaggccatggcggtgaccgtctcggcttcttcgttctcgcaagtctgagcctcgatcagagaacgccccgctgtggaggttgtgcgctgcaggcagcgccagtacttgctgtggatctccatgactttctccatggaacggacagcgtttgcattgggtctttgctgtaaaaccttttctgggagaggatcaagctcgtttcccagcaaggcagaaacacatgcttccgaggcgtcgcaaatggcggtcaggtcgtggcctccctcgagggccaggacaatccggccgccagccaggcccatcagctgcttcgtcaggtacccgaagcatctggcggagaggttgtagcccccaagaggggtggggtggccctccacggcatcgaagcctgatgacaccagcaccacatccggggcaaactcgctggcgatcggcatgaccaccgttctgaaggccgccaagtactcagcgtctcccatgggggggtccaggccgccggtgaaagccatgttgacgttgaaacccacgccgggccctgtgcccacctcatcaggagccccgctgcctgggaagaagttcccatcgtcgtagcggtggagggacatgtacaggacgctggggtcgctgtagaaagcctgctgggtcccgtttccatggtgcacgtcccagtccacgatgaggatcttgctcacgctcaacctctgctgcagaagcttggctgccacggccacggagttgaagtagcaaaagcccatgggcgtgctctcctccgcatggtgtccaggggggcggaccacagcaaagccattcttcagctcccctgtggccaccttgaagaccagctctaccacgcagcccacagccaggcgggctgcccccgccgagtgcacctcgttccatatggtgtcactgtccaccccaacaccaccgcaagggagccggacgaacacggaggcgagcgagcctagaagtttcttactgtccagtttctgccggttgagggggttcgtgccatacaggagggtgtgggcttccgagtgcaccgtctgtagctcctccagggtggccttgcgtccgcggatgcactcgcatttgccccggaggcccgtctcctgcaggcgggaccagatgctctggatcctcccggcgtgctcggggtggctgctgctactcccgcaggtgcactggtgcttcagcatcagcgtgtcatacacgaggcctgtcgtgaacctcggcttggtggggggctcctgcacagacacggggaaggtggcagacgcgggtgaggactgcgcccgggacagaggcctgtggccgccgaaggacacggggatgccggcggcctccatggacgcctggtagttcctcagctggtggatccgctgctgctccagcaggagggcttgctgtctgaagagcagctcctgctcactgggctggcgctggcccggctccacctcccgtgggggctctgcctcttcctcatcgctctcaatgggctcctgcttcacctgcacgccggcctgtgcgtgcgcctccttctgccccggcagccggtccaggtagggctcgtccagcagagcctggtgctcacggagctcctcctccgtctcctccgggtggctctccggctgccgggctggctcgcttggcttggggatgatcttgttcatctgcagttgctgctgctggaactgctgcttgtgtttctccagaaactgctgatgctgctgctggatgaccaggtgctgcagagcctgggcgttctggggcagcggggccgactgggtccgccccagtgggcggtgctgccgcagcttgtggatggagggggacacccggtctgcaccaaccaaggactgtgcgtggaggggcagtgctcccaggcctgaaagataccagtctgtgacgaggggtgcttgtgccggcggctgctccagtaagaccatgtgctgcagaagagggctgtgcgctgcccctccgtcccgctccaagggcgaggtgctcaggtagggagtgaggtgggtgccggggaaaagggagagcctctgctggagggcgggaagggtgagtctctcggcgtcctgctggcccgccgtgcccgcagaggggccggtggcaggcaggcccagcgtgatgttgggcaaggatggcgatgtgtagaggggaagtggagcggccgagccttctcgtgccacaagtctgtgcgccaaactcgtctccgccgggatgctggggacggcgggcgcgataccgttctccgcgctgacgctcccggagctgttgttgggtgagctgggtccggagcctggggcgctgctgcacgcggagtctgtgacatccaacggacgcttttttagagcagtgaccactggcccgtctttcctgcgtaacagggggctgctccgtctttcggccactttctgctttagcctggaccgtaatttcagattcggttcagaagcgcggactttggttttgttgatggaatttgattaataatagcatcagtccccagaaagggaacctggagggcgatttgtaagaatcagcccacagattctctcctgatactactgggcacatctttctggaaaaaatactgatctctaaatccgttctttctgtcaagctttagggcgctctccaggtgaaatccaggaccattctcagtagaagcatcagtaagaaccacaggctcacacccatgaaacaaagcagcagaagctctaggttcacttttcccaataaaggtttatggcccaaatggaaatgcgcccatgtttgcagggttcttgacttggagaggacatggccgtgctgatatggcccactccagcagggtctccaccagcccgat

SEQ ID NO: 10201 - RNA, 6850 nt, Homo sapiens
  source 1..6850: mol_type = other RNA
caggaaggagacaggcagttcactgtgaattctgagtagtttccctaaaacactgtttccacataaatacaataaactctattattggtatgtcacaagtgctagataaactttttttcttaatatgacaaatgtttaagtagtcctttttatttttcttacaataaaaagtacaatttcttaagaataagttcaataagacgcaaacttccccgccctcctctccttcaaggttttgttttacagaaaaatttccatcttttgtatctgcaaatgtcatgagaggggaacagaaaggcatttttcttcttccccaaagctgccgagtttggcgtgcaaaatctgtatacaatataaagtcatgccggtcgtacagtccatgcaacctccaggtgtaggaaacttaaaaaaatatattcatatatatttatatctatatatttatatatgtatcaatgcccataaaacacgtgggcccaaagtctacaaaaagaagaatggaatgagcacgtggctgtgaccagtaaagaaggaatgttctgatcaaaaagaaaaacaacaaagtccattgctagtgctgcaaaaatcaaacttgcttttgtgtcagaccattacgaaatggtccttccccttgcaaacagattttcaaaagaagtaaagaaaaactgaaacaccttgacaaagtggccctccagaaccagagccctgggacgctggggaggggcggccagtcccagcgggccacggcctccgggacagccgcctgctggtggggcgtgggcacgtgggcacgctgcggcacggcgggaagccgcgagggcagggcagacgccaagaggcccagtggcgtcatcagggtttccctcaaagggatataaagtgctcgcttgctgactcccagccagtgcccccaaggcctttgcaaaggaagaaaaaggctaaaggtccaaggacccacagggagaacacatgaaggaaccctccctgacgtggtcccgcctgcagacgccgaggcagatcctctgccatctgccctggacgcttgctgtggagaagagccgagtgtgtcttcaaagaaaaggctacacagtaatgctctcagcacatttgtgaagctggagtgagctgacagatgaaacgtgcctccccctgccaggcctttgcagagggcgtctccatttgaatgagattagaattaagtccccccactgataacctggccactgagcagtccatgttatcccatcatctgcttaaaaaaaaaaagtgagatgatgcattcctccccataagccacggcggggtaagagggcaggtggcaggatccccagagggctatgcagagaatgaggccaaggaggccagaagagcctgctagctgggccctgccactgctctgtgccatgaatggggaatggaccagctcctcttgccaatctgggcttcagagcaaagagtggccaccagggaggggaaagtcaaacaagtcccaagaccgttctgcctgctctcaaaccactgtctcagagctgaccatcagcagcccagtgaccaagtgaatccaagaatctgcactcatttggtcaaaagtttgagttaatttcagaagctaccctgtaaactttaccaaactccgaaactcggctctgggtccctcctgagcacggtgtgtctgaacttctgcccccaagtctgaacccaatatacactttggaatgaaactggtggcttcatgtgctggaaaataagttaccagtaaaacgtgactgtcagttactgttgaagagaaaaagagtaaagactggctgtcctggtcaggcaatcataccctccctgcaggttcaccaggcaacaagggtccctgggttccttgcagccacaggctccaaaatccagggctggccacgtggctgcagtggaaaaacccaagtgggtaaagagccccacgtgtgccccatgcattgctgacatgctcaaaaggtctttggaaaactcaagttagaattctatcctgacgatgtggtcagagaagtttaaacatgagtttcattaatgctgactgcccccggcatctggcaagcctcccagggtggccgggcatcctaagcaaccctccctgcccttgccacggaggggaaaaacacaccacccctcgtaatactactagtgttgaaagttaaaaagagcccctgggcttctttatacagctcctaggacagaccaggaaagacacaatcgttggtgtcactccgaaaagacctacggtccctcctctcactttctgaaaatagaatctgacagcaacaattctgtacgctgcagaaaactcatcgtacaaaaataaaaacaaaaataattaaaaacctttgaaaggtaaaaaaaaatgtacaagcaagaattcagaaaggaaaaagatttagacattattaccattcagaaaattgctaaatggtgaggaaaaatgtaaaattcataaaacaatgcttattcaggatctttttgtgaaaaaattcatacaaaaatcaacagcaaatttatattctttgctataaaaactcattaggtacatatgtgcatgaaggcttggagacgggagcggttctgttagaaaataattaaaatgaaagtacaaacttgtagggtagttgcccagtggcgaatgtgttggcgatctgaaatctagccaatctggagcttgagaaaacatgaatttcaatcaatcaggatccctttccataagcaccttgagagcaaattcacaagccatccatttgcagggaccttcgcaatctgcattcattttatatatatatatatactttttctataaatgcattataaatattttatcaagatttcataagaatcaagtaagtttcttagcttggaatacattggaatatatattatacatatatatatttatttatacctaaaatttaagcaatacttcatgctacttgcttttaataaaaagcattccgatcgtaacactgcaagtgtgcctaccacatgcttcacgaccagatggagatgctcaatcgtatgtgacgtgtgagaacactttggattcgtttaaaatttgttggacttcaaaacctccaacgggatttgccacttttttggaactacctccatttttcttaaacagcaataaagcaaaacagggaccgccgggctgcagcccctggccccggagatgacggctggtgcccgtgcttgaggcgtcaggccagctcgcggtgccagcactgccaggctcggctggccacaggaaactgtcccaccgattcctgctgtttgttttttcttaaggcattgttcctcagacttcagaaaacccagccacaaaaatccaccagagcaataaaaaaaaaggcacaaactcgcatcttccgatggcttttgagaaactcaagccagctcccccagctcacattcctgtttctgtccagttttgttttctttaaaggtccctctgtcccccacccgggtgcagaccccccgccgcacaccgctatggttcacagaggcgggccacagccgtagaaaacgtcctctttaaaaaaaaataagctacaagatgagtcgagtggtttacacagagactgtggagttgtgggtaataaactttaagcaccagttttaatcaagtttgttttgtattattagatctttgatatttgttttctgtgcctcgtgtcaactgaattcggcagctcggccgcctgttgccacaggctcctttcttccacggcgtcccttgcgggacccgccagagtgtgcttggcttccgcgtgtccgtgtgtctgcgcgtcgccggcgtctgtcccgtgttccctgtgaggctgccacgcccaggcgtgcatgtgcgtctcgagacctgtgggcctgggcggcagaaaggcttcccgtggctgttgcacgctgggtgtccctgggtgctccaagagagccccacggtgggacgcaggcgtgacacgggaaagtttcttggctgagcttcaagacagagacagacagacaagagaacagcagcttcgagggagtgctacaggggcggctcctcttccatgggctcctcatctggtctcttttcggcgggcttcacgcccacggacagcgaggccatggcggtgaccgtctcggcttcttcgttctcgcaagtctgagcctcgatcagagaacgccccgctgtggaggttgtgcgctgcaggcagcgccagtacttgctgtggatctccatgactttctccatggaacggacagcgtttgcattgggtctttgctgtaaaaccttttctgggagaggatcaagctcgtttcccagcaaggcagaaacacatgcttccgaggcgtcgcaaatggcggtcaggtcgtggcctccctcgagggccaggacaatccggccgccagccaggcccatcagctgcttcgtcaggtacccgaagcatctggcggagaggttgtagcccccaagaggggtggggtggccctccacggcatcgaagcctgatgacaccagcaccacatccggggcaaactcgctggcgatcggcatgaccaccgttctgaaggccgccaagtactcagcgtctcccatgggggggtccaggccgccggtgaaagccatgttgacgttgaaacccacgccgggccctgtgcccacctcatcaggagccccgctgcctgggaagaagttcccatcgtcgtagcggtggagggacatgtacaggacgctggggtcgctgtagaaagcctgctgggtcccgtttccatggtgcacgtcccagtccacgatgaggatcttgctcacgctcaacctctgctgcagaagcttggctgccacggccacggagttgaagtagcaaaagcccatgggcgtgctctcctccgcatggtgtccaggggggcggaccacagcaaagccattcttcagctcccctgtggccaccttgaagaccagctctaccacgcagcccacagccaggcgggctgcccccgccgagtgcacctcgttccatatggtgtcactgtccaccccaacaccaccgcaagggagccggacgaacacggaggcgagcgagcctagaagtttcttactgtccagtttctgccggttgagggggttcgtgccatacaggagggtgtgggcttccgagtgcaccgtctgtagctcctccagggtggccttgcgtccgcggatgcactcgcatttgccccggaggcccgtctcctgcaggcgggaccagatgctctggatcctcccggcgtgctcggggtggctgctgctactcccgcaggtgcactggtgcttcagcatcagcgtgtcatacacgaggcctgtcgtgaacctcggcttggtggggggctcctgcacagacacggggaaggtggcagacgcgggtgaggactgcgcccgggacagaggcctgtggccgccgaaggacacggggatgccggcggcctccatggacgcctggtagttcctcagctggtggatccgctgctgctccagcaggagggcttgctgtctgaagagcagctcctgctcactgggctggcgctggcccggctccacctcccgtgggggctctgcctcttcctcatcgctctcaatgggctcctgcttcacctgcacgccggcctgtgcgtgcgcctccttctgccccggcagccggtccaggtagggctcgtccagcagagcctggtgctcacggagctcctcctccgtctcctccgggtggctctccggctgccgggctggctcgcttggcttggggatgatcttgttcatctgcagttgctgctgctggaactgctgcttgtgtttctccagaaactgctgatgctgctgctggatgaccaggtgctgcagagcctgggcgttctggggcagcggggccgactgggtccgccccagtgggcggtgctgccgcagcttgtggatggagggggacacccggtctgcaccaaccaaggactgtgcgtggaggggcagtgctcccaggcctgaaagataccagtctgtgacgaggggtgcttgtgccggcggctgctccagtaagaccatgtgctgcagaagagggctgtgcgctgcccctccgtcccgctccaagggcgaggtgctcaggtagggagtgaggtgggtgccggggaaaagggagagcctctgctggagggcgggaagggtgagtctctcggcgtcctgctggcccgccgtgcccgcagaggggccggtggcaggcaggcccagcgtgatgttgggcaaggatggcgatgtgtagaggggaagtggagcggccgagccttctcgtgccacaagtctgtgcgccaaactcgtctccgccgggatgctggggacggcgggcgcgataccgttctccgcgctgacgctcccggagctgttgttgggtgagctgggtccggagcctggggcgctgctgcacgcggagtctgtgacatccaacggacgcttttttagagcagtgaccactggcccgtctttcctgcgtaacagggggctgctccgtctttcggccactttctgctttagcctggaccgtaatttcagattcggttcagaagctgttttcctaagagggaagtcatctttggcgtcgtacattcccaggaccgggtggttataggaggtcgacactccgctctggggtggagaactctggtcaagggaactgtgctgcgttttcccgtaccagtagcgagggtcgctggaaatgcagtggttcagattccggtgggccagcgccttctttttattgaggacaaattcttgtaacttcatcttcacttctgtgctggccacggcaccttttcctcagtagatgcg

SEQ ID NO: 10202 - RNA, 13073 nt, Homo sapiens
  source 1..13073: mol_type = other RNA
caggaaggagacaggcagttcactgtgaattctgagtagtttccctaaaacactgtttccacataaatacaataaactctattattggtatgtcacaagtgctagataaactttttttcttaatatgacaaatgtttaagtagtcctttttatttttcttacaataaaaagtacaatttcttaagaataagttcaataagacgcaaacttccccgccctcctctccttcaaggttttgttttacagaaaaatttccatcttttgtatctgcaaatgtcatgagaggggaacagaaaggcatttttcttcttccccaaagctgccgagtttggcgtgcaaaatctgtatacaatataaagtcatgccggtcgtacagtccatgcaacctccaggtgtaggaaacttaaaaaaatatattcatatatatttatatctatatatttatatatgtatcaatgcccataaaacacgtgggcccaaagtctacaaaaagaagaatggaatgagcacgtggctgtgaccagtaaagaaggaatgttctgatcaaaaagaaaaacaacaaagtccattgctagtgctgcaaaaatcaaacttgcttttgtgtcagaccattacgaaatggtccttccccttgcaaacagattttcaaaagaagtaaagaaaaactgaaacaccttgacaaagtggccctccagaaccagagccctgggacgctggggaggggcggccagtcccagcgggccacggcctccgggacagccgcctgctggtggggcgtgggcacgtgggcacgctgcggcacggcgggaagccgcgagggcagggcagacgccaagaggcccagtggcgtcatcagggtttccctcaaagggatataaagtgctcgcttgctgactcccagccagtgcccccaaggcctttgcaaaggaagaaaaaggctaaaggtccaaggacccacagggagaacacatgaaggaaccctccctgacgtggtcccgcctgcagacgccgaggcagatcctctgccatctgccctggacgcttgctgtggagaagagccgagtgtgtcttcaaagaaaaggctacacagtaatgctctcagcacatttgtgaagctggagtgagctgacagatgaaacgtgcctccccctgccaggcctttgcagagggcgtctccatttgaatgagattagaattaagtccccccactgataacctggccactgagcagtccatgttatcccatcatctgcttaaaaaaaaaaagtgagatgatgcattcctccccataagccacggcggggtaagagggcaggtggcaggatccccagagggctatgcagagaatgaggccaaggaggccagaagagcctgctagctgggccctgccactgctctgtgccatgaatggggaatggaccagctcctcttgccaatctgggcttcagagcaaagagtggccaccagggaggggaaagtcaaacaagtcccaagaccgttctgcctgctctcaaaccactgtctcagagctgaccatcagcagcccagtgaccaagtgaatccaagaatctgcactcatttggtcaaaagtttgagttaatttcagaagctaccctgtaaactttaccaaactccgaaactcggctctgggtccctcctgagcacggtgtgtctgaacttctgcccccaagtctgaacccaatatacactttggaatgaaactggtggcttcatgtgctggaaaataagttaccagtaaaacgtgactgtcagttactgttgaagagaaaaagagtaaagactggctgtcctggtcaggcaatcataccctccctgcaggttcaccaggcaacaagggtccctgggttccttgcagccacaggctccaaaatccagggctggccacgtggctgcagtggaaaaacccaagtgggtaaagagccccacgtgtgccccatgcattgctgacatgctcaaaaggtctttggaaaactcaagttagaattctatcctgacgatgtggtcagagaagtttaaacatgagtttcattaatgctgactgcccccggcatctggcaagcctcccagggtggccgggcatcctaagcaaccctccctgcccttgccacggaggggaaaaacacaccacccctcgtaatactactagtgttgaaagttaaaaagagcccctgggcttctttatacagctcctaggacagaccaggaaagacacaatcgttggtgtcactccgaaaagacctacggtccctcctctcactttctgaaaatagaatctgacagcaacaattctgtacgctgcagaaaactcatcgtacaaaaataaaaacaaaaataattaaaaacctttgaaaggtaaaaaaaaatgtacaagcaagaattcagaaaggaaaaagatttagacattattaccattcagaaaattgctaaatggtgaggaaaaatgtaaaattcataaaacaatgcttattcaggatctttttgtgaaaaaattcatacaaaaatcaacagcaaatttatattctttgctataaaaactcattaggtacatatgtgcatgaaggcttggagacgggagcggttctgttagaaaataattaaaatgaaagtacaaacttgtagggtagttgcccagtggcgaatgtgttggcgatctgaaatctagccaatctggagcttgagaaaacatgaatttcaatcaatcaggatccctttccataagcaccttgagagcaaattcacaagccatccatttgcagggaccttcgcaatctgcattcattttatatatatatatatactttttctataaatgcattataaatattttatcaagatttcataagaatcaagtaagtttcttagcttggaatacattggaatatatattatacatatatatatttatttatacctaaaatttaagcaatacttcatgctacttgcttttaataaaaagcattccgatcgtaacactgcaagtgtgcctaccacatgcttcacgaccagatggagatgctcaatcgtatgtgacgtgtgagaacactttggattcgtttaaaatttgttggacttcaaaacctccaacgggatttgccacttttttggaactacctccatttttcttaaacagcaataaagcaaaacagggaccgccgggctgcagcccctggccccggagatgacggctggtgcccgtgcttgaggcgtcaggccagctcgcggtgccagcactgccaggctcggctggccacaggaaactgtcccaccgattcctgctgtttgttttttcttaaggcattgttcctcagacttcagaaaacccagccacaaaaatccaccagagcaataaaaaaaaaggcacaaactcgcatcttccgatggcttttgagaaactcaagccagctcccccagctcacattcctgtttctgtccagttttgttttctttaaaggtccctctgtcccccacccgggtgcagaccccccgccgcacaccgctatggttcacagaggcgggccacagccgtagaaaacgtcctctttaaaaaaaaataagctacaagatgagtcgagtggtttacacagagactgtggagttgtgggtaataaactttaagcaccagttttaatcaagtttgttttgtattattagatctttgatatttgttttctgtgcctcgtgtcaactgaattcggcagctcggccgcctgttgccacaggctcctttcttccacggcgtcccttgcgggacccgccagagtgtgcttggcttccgcgtgtccgtgtgtctgcgcgtcgccggcgtctgtcccgtgttccctgtgaggctgccacgcccaggcgtgcatgtgcgtctcgagacctgtgggcctgggcggcagaaaggcttcccgtggctgttgcacgctgggtgtccctgggtgctccaagagagccccacggtgggacgcaggcgtgacacgggaaagtttcttggctgagcttcaagacagagacagacagacaagagaacagcagcttcgagggagtgctacaggggcggctcctcttccatgggctcctcatctggtctcttttcggcgggcttcacgcccacggacagcgaggccatggcggtgaccgtctcggcttcttcgttctcgcaagtctgagcctcgatcagagaacgccccgctgtggaggttgtgcgctgcaggcagcgccagtacttgctgtggatctccatgactttctccatggaacggacagcgtttgcattgggtctttgctgtaaaaccttttctgggagaggatcaagctcgtttcccagcaaggcagaaacacatgcttccgaggcgtcgcaaatggcggtcaggtcgtggcctccctcgagggccaggacaatccggccgccagccaggcccatcagctgcttcgtcaggtacccgaagcatctggcggagaggttgtagcccccaagaggggtggggtggccctccacggcatcgaagcctgatgacaccagcaccacatccggggcaaactcgctggcgatcggcatgaccaccgttctgaaggccgccaagtactcagcgtctcccatgggggggtccaggccgccggtgaaagccatgttgacgttgaaacccacgccgggccctgtgcccacctcatcaggagccccgctgcctgggaagaagttcccatcgtcgtagcggtggagggacatgtacaggacgctggggtcgctgtagaaagcctgctgggtcccgtttccatggtgcacgtcccagtccacgatgaggatcttgctcacgctcaacctctgctgcagaagcttggctgccacggccacggagttgaagtagcaaaagcccatgggcgtgctctcctccgcatggtgtccaggggggcggaccacagcaaagccattcttcagctcccctgtggccaccttgaagaccagctctaccacgcagcccacagccaggcgggctgcccccgccgagtgcacctcgttccatatggtgtcactgtccaccccaacaccaccgcaagggagccggacgaacacggaggcgagcgagcctagaagtttcttactgtccagtttctgccggttgagggggttcgtgccatacaggagggtgtgggcttccgagtgcaccgtctgtagctcctccagggtggccttgcgtccgcggatgcactcgcatttgccccggaggcccgtctcctgcaggcgggaccagatgctctggatcctcccggcgtgctcggggtggctgctgctactcccgcaggtgcactggtgcttcagcatcagcgtgtcatacacgaggcctgtcgtgaacctcggcttggtggggggctcctgcacagacacggggaaggtggcagacgcgggtgaggactgcgcccgggacagaggcctgtggccgccgaaggacacggggatgccggcggcctccatggacgcctggtagttcctcagctggtggatccgctgctgctccagcaggagggcttgctgtctgaagagcagctcctgctcactgggctggcgctggcccggctccacctcccgtgggggctctgcctcttcctcatcgctctcaatgggctcctgcttcacctgcacgccggcctgtgcgtgcgcctccttctgccccggcagccggtccaggtagggctcgtccagcagagcctggtgctcacggagctcctcctccgtctcctccgggtggctctccggctgccgggctggctcgcttggcttggggatgatcttgttcatctgcagttgctgctgctggaactgctgcttgtgtttctccagaaactgctgatgctgctgctggatgaccaggtgctgcagagcctgggcgttctggggcagcggggccgactgggtccgccccagtgggcggtgctgccgcagcttgtggatggagggggacacccggtctgcaccaaccaaggactgtgcgtggaggggcagtgctcccaggcctgaaagataccagtctgtgacgaggggtgcttgtgccggcggctgctccagtaagaccatgtgctgcagaagagggctgtgcgctgcccctccgtcccgctccaagggcgaggtgctcaggtagggagtgaggtgggtgccggggaaaagggagagcctctgctggagggcgggaagggtgagtctctcggcgtcctgctggcccgccgtgcccgcagaggggccggtggcaggcaggcccagcgtgatgttgggcaaggatggcgatgtgtagaggggaagtggagcggccgagccttctcgtgccacaagtctgtgcgccaaactcgtctccgccgggatgctggggacggcgggcgcgataccgttctccgcgctgacgctcccggagctgttgttgggtgagctgggtccggagcctggggcgctgctgcacgcggagtctgtgacatccaacggacgcttttttagagcagtgaccactggcccgtctttcctgcgtaacagggggctgctccgtctttcggccactttctgctttagcctggaccgtaatttcagattcggttcagaagctgttttcctaagagggaagtcatctttggcgtcgtacattcccaggaccgggtggttataggaggtcgacactccgctctggggtggagaactctggtcaagggaactgtgctgcgttttcccgtaccagtagcgagggtcgctggaaatgcagtggttcagattccggtgggccagcgccttctttttattgaggacaaattcttgtaacttcatcttcacttctgtgctggccacggcactctctttgcccttctccttgttcttgagctgctgcagcttctgctcccggtgctgcttctccagctcctgctcctggcggtgcctctccagcttccgctggtgttccagcagctcctgctggtgcttcatggccagcatctcctgttgttgcttgatgtgctcgtggagctgcgcctcgtgctgccgggagagctgctcgtgctgcctctggaactcagcgatgaggatctgcctctggatctgctgcttctgcttgagcgccaggagctcctgctgcagctgctgctcccgcagggccggctctgccacaggcagtgagaactggtggtccaggcgcaggtccatgggcactgccgagggggccacttgcagaggcagcgccgtggccacatccaccacaagagcagatccacgaaggcagaagtcggtctgcgggagagtaaagcatagctggactcccaccacctgcagggtgcccccaccccagggggggatgagaaacacctggatggaggggtggagcctggctgggctcaagagcaggagagggaagccaggaaggcggggaaggcaggtcggcaggggagggcaggcccgcccaggaaggcccacgcagggctgggtgctgtagaactgaaagaagtgccagccccttcctcaggcgcctgactaaaccgccttcaatttcttcccctcgcccgtggccacgtactgctacccaagggacacctccagtcctccctcacctggtcagacacctggctctgatggcccctcggagcccctcattggaaacacagagggcctgagtttggttctgcatcacgtgtgacagtgtgtgcatcttgctgtgaggtccagaaatggaaaccttccttaaaagatgggcaggttcctctggtaggggacatggtgttggtacggcgaaaacatgacattagggtcaaatgtggctgctgagaaggaactccctttcagctgcaccgcgacaccctaacacagacaagggtcggcaaagagccatctccctcgtcctggcggcacaggcttccagatgccactgaggggctccgcaggccctctggatacattttacagtccacagccttaaagcacacaaagctggtaataaaagaaaaaagataaaaagccctttaaccagaaatgatgtcatgatgcaaaaattcattcctggataatacttttggccaccagtgacactccgaatacacaaaccaaaccaaattctcagtggaaaaaaaaaatcctttcttccaaccaatcatcacttagaactgtggaatcctccctgagagatactcagtgagatttctctgtattctgtatcaacacggttgaggggcactgctgggactgccacatagctttctctctccctctaaagtagagaaacaaccagtcaccagctccaccccatccagatttgctgtggatgtgtggacggttttagaagcacccagaggatatttctcagacagcacccccaattctccacgacgccccaaccaataaccgtctgctttcttaccacccatgttccttgctaagggcagacagtaagctcttcagaaatctttgggtcgacagcaacaacaacaatgtaacatgtaatggggggggtgataaatgtagataacccaaacaatctaatgtccacccaggatggagaaactttctatctttctgcctcaggcactgcggacagggaaagaaccagttggaaagtgaggccggcaggctcacgggtggggctggcaggcagcagtgtcctgggccgcgtggggaggcacggtcccacctgccagccacagggtggcatttcagagccacagggcatttctggtcaaaaataacagagtgaacacaatcacgttgtcaggatccctccaagattctgctgaaacagtgtgtggattgtttagaaagacacaccaacacaacacacacacaggagatgagagagcagccacaaaatgctggaagtcagaaaggatctgggtgaataaggtatcagagacagcaaagctgacccatcagccagggtgggccaagggaggggcagaccagtctcggtcacacagccctccggggcacaggggctggtgggaccaggactggaggtgaaggagaatgaaatatctgctcagggaatgcagggccccaaccaccgcttaccccacgtggctggcagagcccagggactactaccctctggagagggagatggaacagcactgaaaactgcggaccagtggaagctggccagctacacgtgaggtgtcctggtcttcctgccccagcatgggggcagggcaggcagcattgggccctcccagtgaggtcacaggggctaagcagcctgctggacaccatgccaagtgggaccgggcagcccccagcggccagcaccctgcatgcccctgcaggtcccgccagcctcagtgccctctgctacagatggcagataccgtgctcaccagaaaggccaggaagactgtcatcacagaaggcagagcctggacagacagacaagcaccttggggaaatgcagacagagagaagggaagacaggccctccaaagacaagcggaaggagcgggaggcagccctggagttccaggacaggagggcatgcctcgggtgcggaggaacatagtctctgcccggtgaaatgagcaagcaagcctcagagggctaacaccattaaaagccagaagggccctctgaaggcaaatgtgactgactcagcagcttcacgagagtcatcgccctgcagatcaggtccagcggactgcaggtccagcagctgccactgcagggtggcccgggccctctgctaggtctcccagctgcttccatccaccaggcatcttctcaagacacattttcaacgcaattcaagccctcctgttgttatgcttcccagcatcagctgggctgggtttcacttgagacagttgctcctagggacattgccacaaagggatgggaaggtggaagggacggtggttgagctgcaggaagggcagagccacgaacctggggccaggcacaccagagggcaccaggaagcaagagtgcaagagaacacagacccctcctgtgtgccagacgctacgccagacacttgcccttgctgcctgcgccctggcccaggaccaagcagccccgggacaccaggtgaggagcagcctgctggaggccatgtggccaaagggagacaggaagactgtgctgcccccatgtctgccaggctcccaggccttggagcaactcagctgagcccaggacctgatccttcactggcctctgtcaatactgagccggaacgggatggcaggagggagctgtcactgtgagagttaggaggaaagtgaatggggtgcaaatacaggctgtgtacgccacgtgaaaggtggtgttcttggccccgcagtgtttccagagaaacctgatgttactgctcatgggagttcacagatctgaggggaaggagagcagaaatcagaagtgacttgtctccaggtggcaaaaagcaaacagcatcagagaaaaacagaacgatctgaaggtttaggggcggatagggatgagatattgggaaggactggagaagggggcatgggtatgaacagaccttgaaaaataacaccttttgaaattcttaagaggtaatatgccttcagccatcgaaggggaattggaacttgaggattactcgacaccacatctagtgaacaaggtagtgaccaagcaggagggcgcagcttctggtccaaaactattctctactataaagtaacaagggctgggcacagtcgttcacacctgtaatcccagcactttgggaggctgaggtaggcagatcacttgaggtcaggagttcgagaccagcctggccaatgtggtgaaacctcgtctctactaaaaatacaaaaactagccgggcgtggtggcgggcgcctgtaatcccagctattcaggaggctgaggcaggagaatcgcttgaacctgggaggcagaggtggcagtgagccgagatcctgccactgcactccagccctgcactccagtcaacacagtgagactctatgtctcaaaaaataaataaaaataaaaataaaatgaataaagtaatggggccaattcgcctaattgccaaaagtgactcttaaagcatttctaaattgctcataattgtacacgacacacacatggcctccaggagtaacgctatattgcagtcagcttctaaagccatgtggggggcagactcctgcgtctggcctttgagtcatggctattcataccggccctcaggttaacttgatggagggcagtcaacaaactctcaacattagtttgaactaagagaatcaaaccatgggaattcttttcagatttttcaaatgttgacgaaaaaggccaaactctgtaaaatagttgaagaggtttattttaagccaaatacgagtgaccatggcccaggacacagcctcaggaagtctgtgcctgaggttgtcacgttacaggttggctttatgcgttttagggagacagaaattacaggcaacacatgtaaggtatatattggtttggcccagaacatcttgaagaagtagggtgaggacctcacagatcctaggcagactgaaaggttttctgactgaagagttgatgtcagcataaaaaaatgtttgagttaagataagcggagattctcgttatgtggatgaggcctccaggaagcaggcttcagagagaatagatggtaaatgtctcctatgggactttaaaaggtgacttgtagttaaatctctcctggatcaggaaaaagagacctggaaagggcatgggattctctccagaatgcaaatttcccccccaagaggcagttttctatagccactcaaaataggtggaaggaatatattctggggtaaaatacttttatttcctgcagggcctgctctctgtcgcctgctgctatcccagagtcagggtggaaccgggaatcttactgctgtgtctgttttatcagtcgtgagatcgctgttttgatgttaacgctggtcagctgggcctgaacgccaaaaggagggggcgtctaaggaggcctgtccaaccccccattcccatcagggcctgaactcatttttcaagtttctttgggaccccttggtcaagaagggggtccattcattgggttgggggacttagaattttatttttggtttacacaaacagttttactttgatgtctttacattctacacttcattttacctctaaaaattaaaacaaagcaagcaagcaaaaaaaaaaaaaaaaaaaaaagcaaagcaggtgacatgttccgtggcggacatgaccgtcctggccaatccttgcccgtggctggcaagctgccgagtccgtgggccggagggcattgattcctcaaagacacttccctgatcggaggaaaataacccaagcagtcacggcaggcgccgccaggacgaggccgccacggcctctcttcttcctgccactcctgcccagtccttccgtgggggccactcgaggaaccaccagagatggccgtgggtccttcactggaccctatccaaaccccagaaatgccagctttatgatgaaaactcacaaaggggcaccacgcaggaatattacaaccaaggactttgttaccacgggctctgtgtatgaaggtaattaacagcttccggtgccaataaagggagactttcgaagcttcccctgaggtcacacgtccttgcagatttgtaccagattccactttcttctcaccaaacgaaacaatgcaacaaccgccacaaaacacatctaggaggcagcatgagctccaggcaccagccaacctcaaatacttcctgttccaaaatgtaagagcagtgtctggaaatacagctcctttgacagtgtgctggtcaaacaccccttagatgtgggaatccaacgctgaagccaaacgtgaattttgcgttattttggagagtttctctacagtttctagttaatcccctttaaggttccagagttttcttttaaaaatggtgcttttgaaacataaccttaaaaagagcctccctaactctgacagatacacgtttcccaggacacaggtacagagggtgatgaaaccgccacccctatgcctcaggaaaccgtggaacgtgcttctctttagtccagcatc

SEQ ID NO: 10203 - RNA, 7989 nt, Homo sapiens
  source 1..7989: mol_type = other RNA
caggaaggagacaggcagttcactgtgaattctgagtagtttccctaaaacactgtttccacataaatacaataaactctattattggtatgtcacaagtgctagataaactttttttcttaatatgacaaatgtttaagtagtcctttttatttttcttacaataaaaagtacaatttcttaagaataagttcaataagacgcaaacttccccgccctcctctccttcaaggttttgttttacagaaaaatttccatcttttgtatctgcaaatgtcatgagaggggaacagaaaggcatttttcttcttccccaaagctgccgagtttggcgtgcaaaatctgtatacaatataaagtcatgccggtcgtacagtccatgcaacctccaggtgtaggaaacttaaaaaaatatattcatatatatttatatctatatatttatatatgtatcaatgcccataaaacacgtgggcccaaagtctacaaaaagaagaatggaatgagcacgtggctgtgaccagtaaagaaggaatgttctgatcaaaaagaaaaacaacaaagtccattgctagtgctgcaaaaatcaaacttgcttttgtgtcagaccattacgaaatggtccttccccttgcaaacagattttcaaaagaagtaaagaaaaactgaaacaccttgacaaagtggccctccagaaccagagccctgggacgctggggaggggcggccagtcccagcgggccacggcctccgggacagccgcctgctggtggggcgtgggcacgtgggcacgctgcggcacggcgggaagccgcgagggcagggcagacgccaagaggcccagtggcgtcatcagggtttccctcaaagggatataaagtgctcgcttgctgactcccagccagtgcccccaaggcctttgcaaaggaagaaaaaggctaaaggtccaaggacccacagggagaacacatgaaggaaccctccctgacgtggtcccgcctgcagacgccgaggcagatcctctgccatctgccctggacgcttgctgtggagaagagccgagtgtgtcttcaaagaaaaggctacacagtaatgctctcagcacatttgtgaagctggagtgagctgacagatgaaacgtgcctccccctgccaggcctttgcagagggcgtctccatttgaatgagattagaattaagtccccccactgataacctggccactgagcagtccatgttatcccatcatctgcttaaaaaaaaaaagtgagatgatgcattcctccccataagccacggcggggtaagagggcaggtggcaggatccccagagggctatgcagagaatgaggccaaggaggccagaagagcctgctagctgggccctgccactgctctgtgccatgaatggggaatggaccagctcctcttgccaatctgggcttcagagcaaagagtggccaccagggaggggaaagtcaaacaagtcccaagaccgttctgcctgctctcaaaccactgtctcagagctgaccatcagcagcccagtgaccaagtgaatccaagaatctgcactcatttggtcaaaagtttgagttaatttcagaagctaccctgtaaactttaccaaactccgaaactcggctctgggtccctcctgagcacggtgtgtctgaacttctgcccccaagtctgaacccaatatacactttggaatgaaactggtggcttcatgtgctggaaaataagttaccagtaaaacgtgactgtcagttactgttgaagagaaaaagagtaaagactggctgtcctggtcaggcaatcataccctccctgcaggttcaccaggcaacaagggtccctgggttccttgcagccacaggctccaaaatccagggctggccacgtggctgcagtggaaaaacccaagtgggtaaagagccccacgtgtgccccatgcattgctgacatgctcaaaaggtctttggaaaactcaagttagaattctatcctgacgatgtggtcagagaagtttaaacatgagtttcattaatgctgactgcccccggcatctggcaagcctcccagggtggccgggcatcctaagcaaccctccctgcccttgccacggaggggaaaaacacaccacccctcgtaatactactagtgttgaaagttaaaaagagcccctgggcttctttatacagctcctaggacagaccaggaaagacacaatcgttggtgtcactccgaaaagacctacggtccctcctctcactttctgaaaatagaatctgacagcaacaattctgtacgctgcagaaaactcatcgtacaaaaataaaaacaaaaataattaaaaacctttgaaaggtaaaaaaaaatgtacaagcaagaattcagaaaggaaaaagatttagacattattaccattcagaaaattgctaaatggtgaggaaaaatgtaaaattcataaaacaatgcttattcaggatctttttgtgaaaaaattcatacaaaaatcaacagcaaatttatattctttgctataaaaactcattaggtacatatgtgcatgaaggcttggagacgggagcggttctgttagaaaataattaaaatgaaagtacaaacttgtagggtagttgcccagtggcgaatgtgttggcgatctgaaatctagccaatctggagcttgagaaaacatgaatttcaatcaatcaggatccctttccataagcaccttgagagcaaattcacaagccatccatttgcagggaccttcgcaatctgcattcattttatatatatatatatactttttctataaatgcattataaatattttatcaagatttcataagaatcaagtaagtttcttagcttggaatacattggaatatatattatacatatatatatttatttatacctaaaatttaagcaatacttcatgctacttgcttttaataaaaagcattccgatcgtaacactgcaagtgtgcctaccacatgcttcacgaccagatggagatgctcaatcgtatgtgacgtgtgagaacactttggattcgtttaaaatttgttggacttcaaaacctccaacgggatttgccacttttttggaactacctccatttttcttaaacagcaataaagcaaaacagggaccgccgggctgcagcccctggccccggagatgacggctggtgcccgtgcttgaggcgtcaggccagctcgcggtgccagcactgccaggctcggctggccacaggaaactgtcccaccgattcctgctgtttgttttttcttaaggcattgttcctcagacttcagaaaacccagccacaaaaatccaccagagcaataaaaaaaaaggcacaaactcgcatcttccgatggcttttgagaaactcaagccagctcccccagctcacattcctgtttctgtccagttttgttttctttaaaggtccctctgtcccccacccgggtgcagaccccccgccgcacaccgctatggttcacagaggcgggccacagccgtagaaaacgtcctctttaaaaaaaaataagctacaagatgagtcgagtggtttacacagagactgtggagttgtgggtaataaactttaagcaccagttttaatcaagtttgttttgtattattagatctttgatatttgttttctgtgcctcgtgtcaactgaattcggcagctcggccgcctgttgccacaggctcctttcttccacggcgtcccttgcgggacccgccagagtgtgcttggcttccgcgtgtccgtgtgtctgcgcgtcgccggcgtctgtcccgtgttccctgtgaggctgccacgcccaggcgtgcatgtgcgtctcgagacctgtgggcctgggcggcagaaaggcttcccgtggctgttgcacgctgggtgtccctgggtgctccaagagagccccacggtgggacgcaggcgtgacacgggaaagtttcttggctgagcttcaagacagagacagacagacaagagaacagcagcttcgagggagtgctacaggggcggctcctcttccatgggctcctcatctggtctcttttcggcgggcttcacgcccacggacagcgaggccatggcggtgaccgtctcggcttcttcgttctcgcaagtctgagcctcgatcagagaacgccccgctgtggaggttgtgcgctgcaggcagcgccagtacttgctgtggatctccatgactttctccatggaacggacagcgtttgcattgggtctttgctgtaaaaccttttctgggagaggatcaagctcgtttcccagcaaggcagaaacacatgcttccgaggcgtcgcaaatggcggtcaggtcgtggcctccctcgagggccaggacaatccggccgccagccaggcccatcagctgcttcgtcaggtacccgaagcatctggcggagaggttgtagcccccaagaggggtggggtggccctccacggcatcgaagcctgatgacaccagcaccacatccggggcaaactcgctggcgatcggcatgaccaccgttctgaaggccgccaagtactcagcgtctcccatgggggggtccaggccgccggtgaaagccatgttgacgttgaaacccacgccgggccctgtgcccacctcatcaggagccccgctgcctgggaagaagttcccatcgtcgtagcggtggagggacatgtacaggacgctggggtcgctgtagaaagcctgctgggtcccgtttccatggtgcacgtcccagtccacgatgaggatcttgctcacgctcaacctctgctgcagaagcttggctgccacggccacggagttgaagtagcaaaagcccatgggcgtgctctcctccgcatggtgtccaggggggcggaccacagcaaagccattcttcagctcccctgtggccaccttgaagaccagctctaccacgcagcccacagccaggcgggctgcccccgccgagtgcacctcgttccatatggtgtcactgtccaccccaacaccaccgcaagggagccggacgaacacggaggcgagcgagcctagaagtttcttactgtccagtttctgccggttgagggggttcgtgccatacaggagggtgtgggcttccgagtgcaccgtctgtagctcctccagggtggccttgcgtccgcggatgcactcgcatttgccccggaggcccgtctcctgcaggcgggaccagatgctctggatcctcccggcgtgctcggggtggctgctgctactcccgcaggtgcactggtgcttcagcatcagcgtgtcatacacgaggcctgtcgtgaacctcggcttggtggggggctcctgcacagacacggggaaggtggcagacgcgggtgaggactgcgcccgggacagaggcctgtggccgccgaaggacacggggatgccggcggcctccatggacgcctggtagttcctcagctggtggatccgctgctgctccagcaggagggcttgctgtctgaagagcagctcctgctcactgggctggcgctggcccggctccacctcccgtgggggctctgcctcttcctcatcgctctcaatgggctcctgcttcacctgcacgccggcctgtgcgtgcgcctccttctgccccggcagccggtccaggtagggctcgtccagcagagcctggtgctcacggagctcctcctccgtctcctccgggtggctctccggctgccgggctggctcgcttggcttggggatgatcttgttcatctgcagttgctgctgctggaactgctgcttgtgtttctccagaaactgctgatgctgctgctggatgaccaggtgctgcagagcctgggcgttctggggcagcggggccgactgggtccgccccagtgggcggtgctgccgcagcttgtggatggagggggacacccggtctgcaccaaccaaggactgtgcgtggaggggcagtgctcccaggcctgaaagataccagtctgtgacgaggggtgcttgtgccggcggctgctccagtaagaccatgtgctgcagaagagggctgtgcgctgcccctccgtcccgctccaagggcgaggtgctcaggtagggagtgaggtgggtgccggggaaaagggagagcctctgctggagggcgggaagggtgagtctctcggcgtcctgctggcccgccgtgcccgcagaggggccggtggcaggcaggcccagcgtgatgttgggcaaggatggcgatgtgtagaggggaagtggagcggccgagccttctcgtgccacaagtctgtgcgccaaactcgtctccgccgggatgctggggacggcgggcgcgataccgttctccgcgctgacgctcccggagctgttgttgggtgagctgggtccggagcctggggcgctgctgcacgcggagtctgtgacatccaacggacgcttttttagagcagtgaccactggcccgtctttcctgcgtaacagggggctgctccgtctttcggccactttctgctttagcctggaccgtaatttcagattcggttcagaagctgttttcctaagagggaagtcatctttggcgtcgtacattcccaggaccgggtggttataggaggtcgacactccgctctggggtggagaactctggtcaagggaactgtgctgcgttttcccgtaccagtagcgagggtcgctggaaatgcagtggttcagattccggtgggccagcgccttctttttattgaggacaaattcttgtaacttcatcttcacttctgtgctggccacggcactctctttgcccttctccttgttcttgagctgctgcagcttctgctcccggtgctgcttctccagctcctgctcctggcggtgcctctccagcttccgctggtgttccagcagctcctgctggtgcttcatggccagcatctcctgttgttgcttgatgtgctcgtggagctgcgcctcgtgctgccgggagagctgctcgtgctgcctctggaactcagcgatgaggatctgcctctggatctgctgcttctgcttgagcgccaggagctcctgctgcagctgctgctcccgcagggccggctctgccacaggcagtgagaactggtggtccaggcgcaggtccatgggcactgccgagggggccacttgcagaggcagcgccgtggccacatccaccgtgctgggcatgtggttcacgcgggcaggattcagcagctccactggctggtctcggccagaaagtccatcaaacatttgctgacagcaagctcagggaacagcagaggcccgtctcggtattccggaagcagccagacctaagatcaaatccaggcttgacgacagactgggctggtgccctggacaagcggtggcttccagaagctgggggagcccctgggcatcacgtggagatgagagaagatgcttccagaacctgacacacagtagggatccggaatcgccagagctcttgcacctcagagggaaacagggtatcctgaagttcaagtgcatgcacaccgtggatactctagggtcccagcaaccccagctattacaatcacactgtcactgggtgaacgctgtgcactctacaggggcctcctcatttagtcatcatagccactggggatgcaggtgcccctgcagcctcattccacccacatccggtgcacagcacacacaggatcagcagtgataggaacagcctgccactctttacagagccgtgagactgtggctaaatcatttatccagcacccaacaacgtggaaatcatgacactccacctacaggggctaggctagaaaggcatttaatcaaacattttagaatgattttcatttaattatctctcggagacttaactgtgtcatatgatgaacaacattatttcctcctaaatgtactgaatccggaagcaacccttcatggcc

SEQ ID NO: 10204 - RNA, 9136 nt, Homo sapiens
  source 1..9136: mol_type = other RNA
caggaaggagacaggcagttcactgtgaattctgagtagtttccctaaaacactgtttccacataaatacaataaactctattattggtatgtcacaagtgctagataaactttttttcttaatatgacaaatgtttaagtagtcctttttatttttcttacaataaaaagtacaatttcttaagaataagttcaataagacgcaaacttccccgccctcctctccttcaaggttttgttttacagaaaaatttccatcttttgtatctgcaaatgtcatgagaggggaacagaaaggcatttttcttcttccccaaagctgccgagtttggcgtgcaaaatctgtatacaatataaagtcatgccggtcgtacagtccatgcaacctccaggtgtaggaaacttaaaaaaatatattcatatatatttatatctatatatttatatatgtatcaatgcccataaaacacgtgggcccaaagtctacaaaaagaagaatggaatgagcacgtggctgtgaccagtaaagaaggaatgttctgatcaaaaagaaaaacaacaaagtccattgctagtgctgcaaaaatcaaacttgcttttgtgtcagaccattacgaaatggtccttccccttgcaaacagattttcaaaagaagtaaagaaaaactgaaacaccttgacaaagtggccctccagaaccagagccctgggacgctggggaggggcggccagtcccagcgggccacggcctccgggacagccgcctgctggtggggcgtgggcacgtgggcacgctgcggcacggcgggaagccgcgagggcagggcagacgccaagaggcccagtggcgtcatcagggtttccctcaaagggatataaagtgctcgcttgctgactcccagccagtgcccccaaggcctttgcaaaggaagaaaaaggctaaaggtccaaggacccacagggagaacacatgaaggaaccctccctgacgtggtcccgcctgcagacgccgaggcagatcctctgccatctgccctggacgcttgctgtggagaagagccgagtgtgtcttcaaagaaaaggctacacagtaatgctctcagcacatttgtgaagctggagtgagctgacagatgaaacgtgcctccccctgccaggcctttgcagagggcgtctccatttgaatgagattagaattaagtccccccactgataacctggccactgagcagtccatgttatcccatcatctgcttaaaaaaaaaaagtgagatgatgcattcctccccataagccacggcggggtaagagggcaggtggcaggatccccagagggctatgcagagaatgaggccaaggaggccagaagagcctgctagctgggccctgccactgctctgtgccatgaatggggaatggaccagctcctcttgccaatctgggcttcagagcaaagagtggccaccagggaggggaaagtcaaacaagtcccaagaccgttctgcctgctctcaaaccactgtctcagagctgaccatcagcagcccagtgaccaagtgaatccaagaatctgcactcatttggtcaaaagtttgagttaatttcagaagctaccctgtaaactttaccaaactccgaaactcggctctgggtccctcctgagcacggtgtgtctgaacttctgcccccaagtctgaacccaatatacactttggaatgaaactggtggcttcatgtgctggaaaataagttaccagtaaaacgtgactgtcagttactgttgaagagaaaaagagtaaagactggctgtcctggtcaggcaatcataccctccctgcaggttcaccaggcaacaagggtccctgggttccttgcagccacaggctccaaaatccagggctggccacgtggctgcagtggaaaaacccaagtgggtaaagagccccacgtgtgccccatgcattgctgacatgctcaaaaggtctttggaaaactcaagttagaattctatcctgacgatgtggtcagagaagtttaaacatgagtttcattaatgctgactgcccccggcatctggcaagcctcccagggtggccgggcatcctaagcaaccctccctgcccttgccacggaggggaaaaacacaccacccctcgtaatactactagtgttgaaagttaaaaagagcccctgggcttctttatacagctcctaggacagaccaggaaagacacaatcgttggtgtcactccgaaaagacctacggtccctcctctcactttctgaaaatagaatctgacagcaacaattctgtacgctgcagaaaactcatcgtacaaaaataaaaacaaaaataattaaaaacctttgaaaggtaaaaaaaaatgtacaagcaagaattcagaaaggaaaaagatttagacattattaccattcagaaaattgctaaatggtgaggaaaaatgtaaaattcataaaacaatgcttattcaggatctttttgtgaaaaaattcatacaaaaatcaacagcaaatttatattctttgctataaaaactcattaggtacatatgtgcatgaaggcttggagacgggagcggttctgttagaaaataattaaaatgaaagtacaaacttgtagggtagttgcccagtggcgaatgtgttggcgatctgaaatctagccaatctggagcttgagaaaacatgaatttcaatcaatcaggatccctttccataagcaccttgagagcaaattcacaagccatccatttgcagggaccttcgcaatctgcattcattttatatatatatatatactttttctataaatgcattataaatattttatcaagatttcataagaatcaagtaagtttcttagcttggaatacattggaatatatattatacatatatatatttatttatacctaaaatttaagcaatacttcatgctacttgcttttaataaaaagcattccgatcgtaacactgcaagtgtgcctaccacatgcttcacgaccagatggagatgctcaatcgtatgtgacgtgtgagaacactttggattcgtttaaaatttgttggacttcaaaacctccaacgggatttgccacttttttggaactacctccatttttcttaaacagcaataaagcaaaacagggaccgccgggctgcagcccctggccccggagatgacggctggtgcccgtgcttgaggcgtcaggccagctcgcggtgccagcactgccaggctcggctggccacaggaaactgtcccaccgattcctgctgtttgttttttcttaaggcattgttcctcagacttcagaaaacccagccacaaaaatccaccagagcaataaaaaaaaaggcacaaactcgcatcttccgatggcttttgagaaactcaagccagctcccccagctcacattcctgtttctgtccagttttgttttctttaaaggtccctctgtcccccacccgggtgcagaccccccgccgcacaccgctatggttcacagaggcgggccacagccgtagaaaacgtcctctttaaaaaaaaataagctacaagatgagtcgagtggtttacacagagactgtggagttgtgggtaataaactttaagcaccagttttaatcaagtttgttttgtattattagatctttgatatttgttttctgtgcctcgtgtcaactgaattcggcagctcggccgcctgttgccacaggctcctttcttccacggcgtcccttgcgggacccgccagagtgtgcttggcttccgcgtgtccgtgtgtctgcgcgtcgccggcgtctgtcccgtgttccctgtgaggctgccacgcccaggcgtgcatgtgcgtctcgagacctgtgggcctgggcggcagaaaggcttcccgtggctgttgcacgctgggtgtccctgggtgctccaagagagccccacggtgggacgcaggcgtgacacgggaaagtttcttggctgagcttcaagacagagacagacagacaagagaacagcagcttcgagggagtgctacaggggcggctcctcttccatgggctcctcatctggtctcttttcggcgggcttcacgcccacggacagcgaggccatggcggtgaccgtctcggcttcttcgttctcgcaagtctgagcctcgatcagagaacgccccgctgtggaggttgtgcgctgcaggcagcgccagtacttgctgtggatctccatgactttctccatggaacggacagcgtttgcattgggtctttgctgtaaaaccttttctgggagaggatcaagctcgtttcccagcaaggcagaaacacatgcttccgaggcgtcgcaaatggcggtcaggtcgtggcctccctcgagggccaggacaatccggccgccagccaggcccatcagctgcttcgtcaggtacccgaagcatctggcggagaggttgtagcccccaagaggggtggggtggccctccacggcatcgaagcctgatgacaccagcaccacatccggggcaaactcgctggcgatcggcatgaccaccgttctgaaggccgccaagtactcagcgtctcccatgggggggtccaggccgccggtgaaagccatgttgacgttgaaacccacgccgggccctgtgcccacctcatcaggagccccgctgcctgggaagaagttcccatcgtcgtagcggtggagggacatgtacaggacgctggggtcgctgtagaaagcctgctgggtcccgtttccatggtgcacgtcccagtccacgatgaggatcttgctcacgctcaacctctgctgcagaagcttggctgccacggccacggagttgaagtagcaaaagcccatgggcgtgctctcctccgcatggtgtccaggggggcggaccacagcaaagccattcttcagctcccctgtggccaccttgaagaccagctctaccacgcagcccacagccaggcgggctgcccccgccgagtgcacctcgttccatatggtgtcactgtccaccccaacaccaccgcaagggagccggacgaacacggaggcgagcgagcctagaagtttcttactgtccagtttctgccggttgagggggttcgtgccatacaggagggtgtgggcttccgagtgcaccgtctgtagctcctccagggtggccttgcgtccgcggatgcactcgcatttgccccggaggcccgtctcctgcaggcgggaccagatgctctggatcctcccggcgtgctcggggtggctgctgctactcccgcaggtgcactggtgcttcagcatcagcgtgtcatacacgaggcctgtcgtgaacctcggcttggtggggggctcctgcacagacacggggaaggtggcagacgcgggtgaggactgcgcccgggacagaggcctgtggccgccgaaggacacggggatgccggcggcctccatggacgcctggtagttcctcagctggtggatccgctgctgctccagcaggagggcttgctgtctgaagagcagctcctgctcactgggctggcgctggcccggctccacctcccgtgggggctctgcctcttcctcatcgctctcaatgggctcctgcttcacctgcacgccggcctgtgcgtgcgcctccttctgccccggcagccggtccaggtagggctcgtccagcagagcctggtgctcacggagctcctcctccgtctcctccgggtggctctccggctgccgggctggctcgcttggcttggggatgatcttgttcatctgcagttgctgctgctggaactgctgcttgtgtttctccagaaactgctgatgctgctgctggatgaccaggtgctgcagagcctgggcgttctggggcagcggggccgactgggtccgccccagtgggcggtgctgccgcagcttgtggatggagggggacacccggtctgcaccaaccaaggactgtgcgtggaggggcagtgctcccaggcctgaaagataccagtctgtgacgaggggtgcttgtgccggcggctgctccagtaagaccatgtgctgcagaagagggctgtgcgctgcccctccgtcccgctccaagggcgaggtgctcaggtagggagtgaggtgggtgccggggaaaagggagagcctctgctggagggcgggaagggtgagtctctcggcgtcctgctggcccgccgtgcccgcagaggggccggtggcaggcaggcccagcgtgatgttgggcaaggatggcgatgtgtagaggggaagtggagcggccgagccttctcgtgccacaagtctgtgcgccaaactcgtctccgccgggatgctggggacggcgggcgcgataccgttctccgcgctgacgctcccggagctgttgttgggtgagctgggtccggagcctggggcgctgctgcacgcggagtctgtgacatccaacggacgcttttttagagcagtgaccactggcccgtctttcctgcgtaacagggggctgctccgtctttcggccactttctgctttagcctggaccgtaatttcagattcggttcagaagctgttttcctaagagggaagtcatctttggcgtcgtacattcccaggaccgggtggttataggaggtcgacactccgctctggggtggagaactctggtcaagggaactgtgctgcgttttcccgtaccagtagcgagggtcgctggaaatgcagtggttcagattccggtgggccagcgccttctttttattgaggacaaattcttgtaacttcatcttcacttctgtgctggccacggcactctctttgcccttctccttgttcttgagctgctgcagcttctgctcccggtgctgcttctccagctcctgctcctggcggtgcctctccagcttccgctggtgttccagcagctcctgctggtgcttcatggccagcatctcctgttgttgcttgatgtgctcgtggagctgcgcctcgtgctgccgggagagctgctcgtgctgcctctggaactcagcgatgaggatctgcctctggatctgctgcttctgcttgagcgccaggagctcctgctgcagctgctgctcccgcagggccggctctgccacaggcagtgagaactggtggtccaggcgcaggtccatgggcactgccgagggggccacttgcagaggcagcgccgtggccacatccaccgtgctgggcatgtggttcacgcgggcaggattcagcagctccactggctggtctcggccagaaagtccatcctcccgaggaagccgatggagtctgaagagcaccagtggccaacagttcccagcggagcaccagggcccatggcaccactcagcagttgcccagggtccccagatacaacggtggacagcaaggactccccaaacccttgaggacgtgctgaaggcagcaaaaatctacaactgttcccggaagggcttggcacagctatagagagttgtacacacaagaaactagccacaaaccggaaacgttaaaccacagctccgtgacacttcctcaccaggaggcggagccctgagccaaggcagacctggagggctccacagaagaggcctgtgccaggggccctgcgcccttctacacggcaatggggactcaaatcacagggacgaggcccctcacgaagagctctgccctggggcaggtcctctgcatcccctcgcaggcttctccctccgtcaaggacagagactgctccagccagctggttagtttccacccaaagccagccgcttgccattgttcccagcttctgagttcttacatggtaattctgcacattccaaacagtctttcaaataccgtctcgtctaagaatgagtgcactttcctaaaaagacaaatatcaagcacttaaaacacacacaccaagctacaggctatacttgaattccaggcataaatctgaatttctctaactgttgtccaaattaggtcaaagagttaccagaataatcagaaaatgttttgagaggggtttaaattcacttggttgtaattttttttatttgctcaattcatcccattctcgctgctgagctttctccttaggaagttggaatgggtgctggaggaagtgaacttggtcctcagcaaactgggaatgccaacagcgctggccactcccagactcgggctggtggccaggacggtggccctggcgggccaggccccactgacagccctaggcaggcctgtcctggaaggagcagggcccattccacactgtgaagagtgacccaagagatcagagattagacttgggtctagatttttctcaggataaagtgtgattttgaaaagacgctgagtaaataagccacatgtcaaggataaagatattcatcatgaaagtaaacaaatttctctctgagttctaacttaccacaaaaaggaatcaacatacttcttccctgctggcttttaccaagcatttccacagtacaatcggtttggtgctcatgaccacctggagggacagaagaacctgccctgtgactagatggcctgcaggccaaggaagacagggtaatcccaggtgaccacccatttcctgtcagggacacagcccctcaggagggctggacagagaaaagggaacaggactccccaggaaaccgcagagatccaggtgtgagaactgaacttctcttagccttttcatcagttgtcaaccaagaacagggtcagacaggcaagcttttgtgcagaagcctaccaggggaccttagggcaccaggtggatggtgccaggctccctacccccacaaaatggaaagaaacaaagaaatggcgacatagaagaatggaattgagctggcttttaaagaaagactaatcgcactggcaagaaatctcaaggacccatcacttccatagctgagcttccagcggcttgattctaggagctaccattggaaacgttcaattagaagaccctcttactgtgcacactaagacctaatttaccagcagatggaagccatccaagcacccccatcattcagacgtacatacattcattatctacatacattcatacatctacacaattcacacaccca

SEQ ID NO: 10205 - RNA, 7798 nt, Homo sapiens
  source 1..7798: mol_type = other RNA
caggaaggagacaggcagttcactgtgaattctgagtagtttccctaaaacactgtttccacataaatacaataaactctattattggtatgtcacaagtgctagataaactttttttcttaatatgacaaatgtttaagtagtcctttttatttttcttacaataaaaagtacaatttcttaagaataagttcaataagacgcaaacttccccgccctcctctccttcaaggttttgttttacagaaaaatttccatcttttgtatctgcaaatgtcatgagaggggaacagaaaggcatttttcttcttccccaaagctgccgagtttggcgtgcaaaatctgtatacaatataaagtcatgccggtcgtacagtccatgcaacctccaggtgtaggaaacttaaaaaaatatattcatatatatttatatctatatatttatatatgtatcaatgcccataaaacacgtgggcccaaagtctacaaaaagaagaatggaatgagcacgtggctgtgaccagtaaagaaggaatgttctgatcaaaaagaaaaacaacaaagtccattgctagtgctgcaaaaatcaaacttgcttttgtgtcagaccattacgaaatggtccttccccttgcaaacagattttcaaaagaagtaaagaaaaactgaaacaccttgacaaagtggccctccagaaccagagccctgggacgctggggaggggcggccagtcccagcgggccacggcctccgggacagccgcctgctggtggggcgtgggcacgtgggcacgctgcggcacggcgggaagccgcgagggcagggcagacgccaagaggcccagtggcgtcatcagggtttccctcaaagggatataaagtgctcgcttgctgactcccagccagtgcccccaaggcctttgcaaaggaagaaaaaggctaaaggtccaaggacccacagggagaacacatgaaggaaccctccctgacgtggtcccgcctgcagacgccgaggcagatcctctgccatctgccctggacgcttgctgtggagaagagccgagtgtgtcttcaaagaaaaggctacacagtaatgctctcagcacatttgtgaagctggagtgagctgacagatgaaacgtgcctccccctgccaggcctttgcagagggcgtctccatttgaatgagattagaattaagtccccccactgataacctggccactgagcagtccatgttatcccatcatctgcttaaaaaaaaaaagtgagatgatgcattcctccccataagccacggcggggtaagagggcaggtggcaggatccccagagggctatgcagagaatgaggccaaggaggccagaagagcctgctagctgggccctgccactgctctgtgccatgaatggggaatggaccagctcctcttgccaatctgggcttcagagcaaagagtggccaccagggaggggaaagtcaaacaagtcccaagaccgttctgcctgctctcaaaccactgtctcagagctgaccatcagcagcccagtgaccaagtgaatccaagaatctgcactcatttggtcaaaagtttgagttaatttcagaagctaccctgtaaactttaccaaactccgaaactcggctctgggtccctcctgagcacggtgtgtctgaacttctgcccccaagtctgaacccaatatacactttggaatgaaactggtggcttcatgtgctggaaaataagttaccagtaaaacgtgactgtcagttactgttgaagagaaaaagagtaaagactggctgtcctggtcaggcaatcataccctccctgcaggttcaccaggcaacaagggtccctgggttccttgcagccacaggctccaaaatccagggctggccacgtggctgcagtggaaaaacccaagtgggtaaagagccccacgtgtgccccatgcattgctgacatgctcaaaaggtctttggaaaactcaagttagaattctatcctgacgatgtggtcagagaagtttaaacatgagtttcattaatgctgactgcccccggcatctggcaagcctcccagggtggccgggcatcctaagcaaccctccctgcccttgccacggaggggaaaaacacaccacccctcgtaatactactagtgttgaaagttaaaaagagcccctgggcttctttatacagctcctaggacagaccaggaaagacacaatcgttggtgtcactccgaaaagacctacggtccctcctctcactttctgaaaatagaatctgacagcaacaattctgtacgctgcagaaaactcatcgtacaaaaataaaaacaaaaataattaaaaacctttgaaaggtaaaaaaaaatgtacaagcaagaattcagaaaggaaaaagatttagacattattaccattcagaaaattgctaaatggtgaggaaaaatgtaaaattcataaaacaatgcttattcaggatctttttgtgaaaaaattcatacaaaaatcaacagcaaatttatattctttgctataaaaactcattaggtacatatgtgcatgaaggcttggagacgggagcggttctgttagaaaataattaaaatgaaagtacaaacttgtagggtagttgcccagtggcgaatgtgttggcgatctgaaatctagccaatctggagcttgagaaaacatgaatttcaatcaatcaggatccctttccataagcaccttgagagcaaattcacaagccatccatttgcagggaccttcgcaatctgcattcattttatatatatatatatactttttctataaatgcattataaatattttatcaagatttcataagaatcaagtaagtttcttagcttggaatacattggaatatatattatacatatatatatttatttatacctaaaatttaagcaatacttcatgctacttgcttttaataaaaagcattccgatcgtaacactgcaagtgtgcctaccacatgcttcacgaccagatggagatgctcaatcgtatgtgacgtgtgagaacactttggattcgtttaaaatttgttggacttcaaaacctccaacgggatttgccacttttttggaactacctccatttttcttaaacagcaataaagcaaaacagggaccgccgggctgcagcccctggccccggagatgacggctggtgcccgtgcttgaggcgtcaggccagctcgcggtgccagcactgccaggctcggctggccacaggaaactgtcccaccgattcctgctgtttgttttttcttaaggcattgttcctcagacttcagaaaacccagccacaaaaatccaccagagcaataaaaaaaaaggcacaaactcgcatcttccgatggcttttgagaaactcaagccagctcccccagctcacattcctgtttctgtccagttttgttttctttaaaggtccctctgtcccccacccgggtgcagaccccccgccgcacaccgctatggttcacagaggcgggccacagccgtagaaaacgtcctctttaaaaaaaaataagctacaagatgagtcgagtggtttacacagagactgtggagttgtgggtaataaactttaagcaccagttttaatcaagtttgttttgtattattagatctttgatatttgttttctgtgcctcgtgtcaactgaattcggcagctcggccgcctgttgccacaggctcctttcttccacggcgtcccttgcgggacccgccagagtgtgcttggcttccgcgtgtccgtgtgtctgcgcgtcgccggcgtctgtcccgtgttccctgtgaggctgccacgcccaggcgtgcatgtgcgtctcgagacctgtgggcctgggcggcagaaaggcttcccgtggctgttgcacgctgggtgtccctgggtgctccaagagagccccacggtgggacgcaggcgtgacacgggaaagtttcttggctgagcttcaagacagagacagacagacaagagaacagcagcttcgagggagtgctacaggggcggctcctcttccatgggctcctcatctggtctcttttcggcgggcttcacgcccacggacagcgaggccatggcggtgaccgtctcggcttcttcgttctcgcaagtctgagcctcgatcagagaacgccccgctgtggaggttgtgcgctgcaggcagcgccagtacttgctgtggatctccatgactttctccatggaacggacagcgtttgcattgggtctttgctgtaaaaccttttctgggagaggatcaagctcgtttcccagcaaggcagaaacacatgcttccgaggcgtcgcaaatggcggtcaggtcgtggcctccctcgagggccaggacaatccggccgccagccaggcccatcagctgcttcgtcaggtacccgaagcatctggcggagaggttgtagcccccaagaggggtggggtggccctccacggcatcgaagcctgatgacaccagcaccacatccggggcaaactcgctggcgatcggcatgaccaccgttctgaaggccgccaagtactcagcgtctcccatgggggggtccaggccgccggtgaaagccatgttgacgttgaaacccacgccgggccctgtgcccacctcatcaggagccccgctgcctgggaagaagttcccatcgtcgtagcggtggagggacatgtacaggacgctggggtcgctgtagaaagcctgctgggtcccgtttccatggtgcacgtcccagtccacgatgaggatcttgctcacgctcaacctctgctgcagaagcttggctgccacggccacggagttgaagtagcaaaagcccatgggcgtgctctcctccgcatggtgtccaggggggcggaccacagcaaagccattcttcagctcccctgtggccaccttgaagaccagctctaccacgcagcccacagccaggcgggctgcccccgccgagtgcacctcgttccatatggtgtcactgtccaccccaacaccaccgcaagggagccggacgaacacggaggcgagcgagcctagaagtttcttactgtccagtttctgccggttgagggggttcgtgccatacaggagggtgtgggcttccgagtgcaccgtctgtagctcctccagggtggccttgcgtccgcggatgcactcgcatttgccccggaggcccgtctcctgcaggcgggaccagatgctctggatcctcccggcgtgctcggggtggctgctgctactcccgcaggtgcactggtgcttcagcatcagcgtgtcatacacgaggcctgtcgtgaacctcggcttggtggggggctcctgcacagacacggggaaggtggcagacgcgggtgaggactgcgcccgggacagaggcctgtggccgccgaaggacacggggatgccggcggcctccatggacgcctggtagttcctcagctggtggatccgctgctgctccagcaggagggcttgctgtctgaagagcagctcctgctcactgggctggcgctggcccggctccacctcccgtgggggctctgcctcttcctcatcgctctcaatgggctcctgcttcacctgcacgccggcctgtgcgtgcgcctccttctgccccggcagccggtccaggtagggctcgtccagcagagcctggtgctcacggagctcctcctccgtctcctccgggtggctctccggctgccgggctggctcgcttggcttggggatgatcttgttcatctgcagttgctgctgctggaactgctgcttgtgtttctccagaaactgctgatgctgctgctggatgaccaggtgctgcagagcctgggcgttctggggcagcggggccgactgggtccgccccagtgggcggtgctgccgcagcttgtggatggagggggacacccggtctgcaccaaccaaggactgtgcgtggaggggcagtgctcccaggcctgaaagataccagtctgtgacgaggggtgcttgtgccggcggctgctccagtaagaccatgtgctgcagaagagggctgtgcgctgcccctccgtcccgctccaagggcgaggtgctcaggtagggagtgaggtgggtgccggggaaaagggagagcctctgctggagggcgggaagggtgagtctctcggcgtcctgctggcccgccgtgcccgcagaggggccggtggcaggcaggcccagcgtgatgttgggcaaggatggcgatgtgtagaggggaagtggagcggccgagccttctcgtgccacaagtctgtgcgccaaactcgtctccgccgggatgctggggacggcgggcgcgataccgttctccgcgctgacgctcccggagctgttgttgggtgagctgggtccggagcctggggcgctgctgcacgcggagtctgtgacatccaacggacgcttttttagagcagtgaccactggcccgtctttcctgcgtaacagggggctgctccgtctttcggccactttctgctttagcctggaccgtaatttcagattcggttcagaagctgttttcctaagagggaagtcatctttggcgtcgtacattcccaggaccgggtggttataggaggtcgacactccgctctggggtggagaactctggtcaagggaactgtgctgcgttttcccgtaccagtagcgagggtcgctggaaatgcagtggttcagattccggtgggccagcgccttctttttattgaggacaaattcttgtaacttcatcttcacttctgtgctggccacggcactctctttgcccttctccttgttcttgagctgctgcagcttctgctcccggtgctgcttctccagctcctgctcctggcggtgcctctccagcttccgctggtgttccagcagctcctgctggtgcttcatggccagcatctcctgttgttgcttgatgtgctcgtggagctgcgcctcgtgctgccgggagagctgctcgtgctgcctctggaactcagcgatgaggatctgcctctggatctgctgcttctgcttgagcgccaggagctcctgctgcagctgctgctcccgcagggccggctctgccacaggcagtgagaactggtggtccaggcgcaggtccatgggcactgccgagggggccacttgcagaggcagcgccgtggccacatccaccgtgctgggcatgtggttcacgcgggcaggattcagcagctccactggctggtctcggccagaaagtccatcctccctgggccccagcttcctcatctgtgagatgggggtggtcagcgtgcaggaagccctccttgacgatgagctatcagcttagggacaagagagctagagacccgggggggagtccactgccttggggacacgagggagccagggtcactttcttcctcatcaagctggccccctggtgacacgggacaagaggataacctgcttggtactcagcaacaggctttcctaataagaattccacacttccatgaggctgtaatcaacttgggagtgaggagttccttagcttcctgttttcagagagtcttcttagcaaagtgaggaatctgcagatctctctgaaagatcagctaccaaaggaaaataacaataatgaagatatcgttggtggaatacataacctccatccacagccagatactgcttccggaaccacacttcgtatccaggtgagctcgttttttgtatttcaaaagcacaaagatctatgttcat

SEQ ID NO: 10206 - RNA, 14059 nt, Homo sapiens
  source 1..14059: mol_type = other RNA
caggaaggagacaggcagttcactgtgaattctgagtagtttccctaaaacactgtttccacataaatacaataaactctattattggtatgtcacaagtgctagataaactttttttcttaatatgacaaatgtttaagtagtcctttttatttttcttacaataaaaagtacaatttcttaagaataagttcaataagacgcaaacttccccgccctcctctccttcaaggttttgttttacagaaaaatttccatcttttgtatctgcaaatgtcatgagaggggaacagaaaggcatttttcttcttccccaaagctgccgagtttggcgtgcaaaatctgtatacaatataaagtcatgccggtcgtacagtccatgcaacctccaggtgtaggaaacttaaaaaaatatattcatatatatttatatctatatatttatatatgtatcaatgcccataaaacacgtgggcccaaagtctacaaaaagaagaatggaatgagcacgtggctgtgaccagtaaagaaggaatgttctgatcaaaaagaaaaacaacaaagtccattgctagtgctgcaaaaatcaaacttgcttttgtgtcagaccattacgaaatggtccttccccttgcaaacagattttcaaaagaagtaaagaaaaactgaaacaccttgacaaagtggccctccagaaccagagccctgggacgctggggaggggcggccagtcccagcgggccacggcctccgggacagccgcctgctggtggggcgtgggcacgtgggcacgctgcggcacggcgggaagccgcgagggcagggcagacgccaagaggcccagtggcgtcatcagggtttccctcaaagggatataaagtgctcgcttgctgactcccagccagtgcccccaaggcctttgcaaaggaagaaaaaggctaaaggtccaaggacccacagggagaacacatgaaggaaccctccctgacgtggtcccgcctgcagacgccgaggcagatcctctgccatctgccctggacgcttgctgtggagaagagccgagtgtgtcttcaaagaaaaggctacacagtaatgctctcagcacatttgtgaagctggagtgagctgacagatgaaacgtgcctccccctgccaggcctttgcagagggcgtctccatttgaatgagattagaattaagtccccccactgataacctggccactgagcagtccatgttatcccatcatctgcttaaaaaaaaaaagtgagatgatgcattcctccccataagccacggcggggtaagagggcaggtggcaggatccccagagggctatgcagagaatgaggccaaggaggccagaagagcctgctagctgggccctgccactgctctgtgccatgaatggggaatggaccagctcctcttgccaatctgggcttcagagcaaagagtggccaccagggaggggaaagtcaaacaagtcccaagaccgttctgcctgctctcaaaccactgtctcagagctgaccatcagcagcccagtgaccaagtgaatccaagaatctgcactcatttggtcaaaagtttgagttaatttcagaagctaccctgtaaactttaccaaactccgaaactcggctctgggtccctcctgagcacggtgtgtctgaacttctgcccccaagtctgaacccaatatacactttggaatgaaactggtggcttcatgtgctggaaaataagttaccagtaaaacgtgactgtcagttactgttgaagagaaaaagagtaaagactggctgtcctggtcaggcaatcataccctccctgcaggttcaccaggcaacaagggtccctgggttccttgcagccacaggctccaaaatccagggctggccacgtggctgcagtggaaaaacccaagtgggtaaagagccccacgtgtgccccatgcattgctgacatgctcaaaaggtctttggaaaactcaagttagaattctatcctgacgatgtggtcagagaagtttaaacatgagtttcattaatgctgactgcccccggcatctggcaagcctcccagggtggccgggcatcctaagcaaccctccctgcccttgccacggaggggaaaaacacaccacccctcgtaatactactagtgttgaaagttaaaaagagcccctgggcttctttatacagctcctaggacagaccaggaaagacacaatcgttggtgtcactccgaaaagacctacggtccctcctctcactttctgaaaatagaatctgacagcaacaattctgtacgctgcagaaaactcatcgtacaaaaataaaaacaaaaataattaaaaacctttgaaaggtaaaaaaaaatgtacaagcaagaattcagaaaggaaaaagatttagacattattaccattcagaaaattgctaaatggtgaggaaaaatgtaaaattcataaaacaatgcttattcaggatctttttgtgaaaaaattcatacaaaaatcaacagcaaatttatattctttgctataaaaactcattaggtacatatgtgcatgaaggcttggagacgggagcggttctgttagaaaataattaaaatgaaagtacaaacttgtagggtagttgcccagtggcgaatgtgttggcgatctgaaatctagccaatctggagcttgagaaaacatgaatttcaatcaatcaggatccctttccataagcaccttgagagcaaattcacaagccatccatttgcagggaccttcgcaatctgcattcattttatatatatatatatactttttctataaatgcattataaatattttatcaagatttcataagaatcaagtaagtttcttagcttggaatacattggaatatatattatacatatatatatttatttatacctaaaatttaagcaatacttcatgctacttgcttttaataaaaagcattccgatcgtaacactgcaagtgtgcctaccacatgcttcacgaccagatggagatgctcaatcgtatgtgacgtgtgagaacactttggattcgtttaaaatttgttggacttcaaaacctccaacgggatttgccacttttttggaactacctccatttttcttaaacagcaataaagcaaaacagggaccgccgggctgcagcccctggccccggagatgacggctggtgcccgtgcttgaggcgtcaggccagctcgcggtgccagcactgccaggctcggctggccacaggaaactgtcccaccgattcctgctgtttgttttttcttaaggcattgttcctcagacttcagaaaacccagccacaaaaatccaccagagcaataaaaaaaaaggcacaaactcgcatcttccgatggcttttgagaaactcaagccagctcccccagctcacattcctgtttctgtccagttttgttttctttaaaggtccctctgtcccccacccgggtgcagaccccccgccgcacaccgctatggttcacagaggcgggccacagccgtagaaaacgtcctctttaaaaaaaaataagctacaagatgagtcgagtggtttacacagagactgtggagttgtgggtaataaactttaagcaccagttttaatcaagtttgttttgtattattagatctttgatatttgttttctgtgcctcgtgtcaactgaattcggcagctcggccgcctgttgccacaggctcctttcttccacggcgtcccttgcgggacccgccagagtgtgcttggcttccgcgtgtccgtgtgtctgcgcgtcgccggcgtctgtcccgtgttccctgtgaggctgccacgcccaggcgtgcatgtgcgtctcgagacctgtgggcctgggcggcagaaaggcttcccgtggctgttgcacgctgggtgtccctgggtgctccaagagagccccacggtgggacgcaggcgtgacacgggaaagtttcttggctgagcttcaagacagagacagacagacaagagaacagcagcttcgagggagtgctacaggggcggctcctcttccatgggctcctcatctggtctcttttcggcgggcttcacgcccacggacagcgaggccatggcggtgaccgtctcggcttcttcgttctcgcaagtctgagcctcgatcagagaacgccccgctgtggaggttgtgcgctgcaggcagcgccagtacttgctgtggatctccatgactttctccatggaacggacagcgtttgcattgggtctttgctgtaaaaccttttctgggagaggatcaagctcgtttcccagcaaggcagaaacacatgcttccgaggcgtcgcaaatggcggtcaggtcgtggcctccctcgagggccaggacaatccggccgccagccaggcccatcagctgcttcgtcaggtacccgaagcatctggcggagaggttgtagcccccaagaggggtggggtggccctccacggcatcgaagcctgatgacaccagcaccacatccggggcaaactcgctggcgatcggcatgaccaccgttctgaaggccgccaagtactcagcgtctcccatgggggggtccaggccgccggtgaaagccatgttgacgttgaaacccacgccgggccctgtgcccacctcatcaggagccccgctgcctgggaagaagttcccatcgtcgtagcggtggagggacatgtacaggacgctggggtcgctgtagaaagcctgctgggtcccgtttccatggtgcacgtcccagtccacgatgaggatcttgctcacgctcaacctctgctgcagaagcttggctgccacggccacggagttgaagtagcaaaagcccatgggcgtgctctcctccgcatggtgtccaggggggcggaccacagcaaagccattcttcagctcccctgtggccaccttgaagaccagctctaccacgcagcccacagccaggcgggctgcccccgccgagtgcacctcgttccatatggtgtcactgtccaccccaacaccaccgcaagggagccggacgaacacggaggcgagcgagcctagaagtttcttactgtccagtttctgccggttgagggggttcgtgccatacaggagggtgtgggcttccgagtgcaccgtctgtagctcctccagggtggccttgcgtccgcggatgcactcgcatttgccccggaggcccgtctcctgcaggcgggaccagatgctctggatcctcccggcgtgctcggggtggctgctgctactcccgcaggtgcactggtgcttcagcatcagcgtgtcatacacgaggcctgtcgtgaacctcggcttggtggggggctcctgcacagacacggggaaggtggcagacgcgggtgaggactgcgcccgggacagaggcctgtggccgccgaaggacacggggatgccggcggcctccatggacgcctggtagttcctcagctggtggatccgctgctgctccagcaggagggcttgctgtctgaagagcagctcctgctcactgggctggcgctggcccggctccacctcccgtgggggctctgcctcttcctcatcgctctcaatgggctcctgcttcacctgcacgccggcctgtgcgtgcgcctccttctgccccggcagccggtccaggtagggctcgtccagcagagcctggtgctcacggagctcctcctccgtctcctccgggtggctctccggctgccgggctggctcgcttggcttggggatgatcttgttcatctgcagttgctgctgctggaactgctgcttgtgtttctccagaaactgctgatgctgctgctggatgaccaggtgctgcagagcctgggcgttctggggcagcggggccgactgggtccgccccagtgggcggtgctgccgcagcttgtggatggagggggacacccggtctgcaccaaccaaggactgtgcgtggaggggcagtgctcccaggcctgaaagataccagtctgtgacgaggggtgcttgtgccggcggctgctccagtaagaccatgtgctgcagaagagggctgtgcgctgcccctccgtcccgctccaagggcgaggtgctcaggtagggagtgaggtgggtgccggggaaaagggagagcctctgctggagggcgggaagggtgagtctctcggcgtcctgctggcccgccgtgcccgcagaggggccggtggcaggcaggcccagcgtgatgttgggcaaggatggcgatgtgtagaggggaagtggagcggccgagccttctcgtgccacaagtctgtgcgccaaactcgtctccgccgggatgctggggacggcgggcgcgataccgttctccgcgctgacgctcccggagctgttgttgggtgagctgggtccggagcctggggcgctgctgcacgcggagtctgtgacatccaacggacgcttttttagagcagtgaccactggcccgtctttcctgcgtaacagggggctgctccgtctttcggccactttctgctttagcctggaccgtaatttcagattcggttcagaagctgttttcctaagagggaagtcatctttggcgtcgtacattcccaggaccgggtggttataggaggtcgacactccgctctggggtggagaactctggtcaagggaactgtgctgcgttttcccgtaccagtagcgagggtcgctggaaatgcagtggttcagattccggtgggccagcgccttctttttattgaggacaaattcttgtaacttcatcttcacttctgtgctggccacggcactctctttgcccttctccttgttcttgagctgctgcagcttctgctcccggtgctgcttctccagctcctgctcctggcggtgcctctccagcttccgctggtgttccagcagctcctgctggtgcttcatggccagcatctcctgttgttgcttgatgtgctcgtggagctgcgcctcgtgctgccgggagagctgctcgtgctgcctctggaactcagcgatgaggatctgcctctggatctgctgcttctgcttgagcgccaggagctcctgctgcagctgctgctcccgcagggccggctctgccacaggcagtgagaactggtggtccaggcgcaggtccatgggcactgccgagggggccacttgcagaggcagcgccgtggccacatccaccgtgctgggcatgtggttcacgcgggcaggattcagcagctccactggctggtctcggccagaaagtccatctccatccacagccagatactgcttccggaaccacacttcgtatccaggtgagctcgttttttgtatttcaaaagcacaaagatctatgttcatggtgtagtccaggcagagtgtggttaacaggcctccgggtgtcccccccttccagcccagtgcaggggttcagccgctgcagaaactccgaatctgctaacgtgaagtgccaagactgctgtccgccagcgccctcactcccccagggcctgtacctgtagcaggaggctcacgttccgagtcctcattgctcccagacccaagggcaaggctgtcacaggcgaaagacgggttccccttcctctacacccaagccctcggaagcacgctgcaggcccctggaggtgccacagtgctcccagctcccccagaggctgagttcaaacattctaaacggattcttgataacaagccgccggctcgctggaagacactgagcagttacataacagcacagaaaatcccttacaagtttcttaaaaaagagttaatcgtactgacttggtgctttaccttcagcccagactttcgcttaatcccggaaactgctccaaaggcgtttttctcagggcgttcggcgccgtaactcaggagaaacccaagtcctgctctcccggcggcctcgctggggaagaattcagccgctccaccctgacatctggtttctatttcatatccatgttgtcacattacataacaagcagatgatacgagagatcaccacagtgtttcggctcgagagtcacaaagaacgcccagaacactgtttatattgggggccatgaacgttcaccaaaccagacttagtgcagaggctgcacccttccaggctgaaacccagcacctacagcaaatgcccaaggaagcaagaagcgggaccccgccttctcagccacctctcactaacactcagctccactcctgcttccttcctctcactccacatccgagttagagggaaatacgatttatctctggcctgcatttacttctcctgcacctggcgggaggctctggccttgcaggcgtgcaggagcccctgccagtgagggccagcgaggggcccagggagaagatggaggtcaagtcatagggcctccaccgcaggcagagctccgccagcaagtatcctgggagctggggggcctcaagggaggcaatccccccacacaccatccccttccccttcgctcatctggggaagctgtgaggactggtgttgataaaacattccaaccacacactcagaccatggatgtggccgtgccagcagggaggccagcagcccctagcagaagggtgttctggaagctgccccctcccatgctgctgcctggtcccatggggcatgaagggagggtggccagggtggcccgagccagcatcaggcacaaggcccaaggagtttctccagagcagcctgtcctcttcggtccagaaaaagtcagattccacagcagggttagccgtccagttagggaacccactaaggggctctgtgcgtagaggtgctcagaatcaaaccactaaaccccaggaccccctgctgggggaatggtccgtggcagtcattcagccttggagtgaaccgttctgcccaagtgcaagtgagaacacaatacttcttattatatacagaattgccaaagccaacgtgattagtagaaaaaccgacatgtcagtgacttgggggtctggtttgccccagatgtgggtggaaaccccaggcgtccctcaagcctggtccagagctccacagacagcagatacacaaactctgagtgacagcattggtgtttagcagattctggattttgctcccccccgaaccaagtatagagaatgtttcacagagtagcttcaacagaaaatggccacagtgtgtctgtgagagagtgtgatgttcccggggggatggctggggccaagggaaggcccctcccatgagccctgcctccatgagactgcgtagggcaggactgccaggcagaaagaacacagcacaggcacaagggcagacccaggctggcagggctaaatggcttcaggagctcccccctctgccccccagggagtaaaggcaatgatgcaaatatgataagcaaacagaggtcccaaaacacagaaagggccaggaccctgatgccaaccaagcagacccaaaactgggtctgggagcacagggcagggtcgctgagtgcagaggggcctcactcaatgtccaacacttccctccaaaacagacatgctggtgagaggcttcaacccttccactggcctgacacctggatctctgctgccctgtgccaggttagccacgtccaacaccaccacggccaccggccatttaagaaaacgaaccctgacgttaacctgcttgagccctaatactaagcaagagcagcgccacaattccaaaactgcagagagcgccttttaaacattctgctgagatctgcgcggtcgcggtctgacaggcaggccttcttggctacctgtggtttcattccagcattaacaggcacctaaaaggcctgtgagcttttgtggggtcaagcagcatcagctccactttacaaccccgcagagtgaggtgttagctctgcagctccagggcagagccttgcagccttagggccagggggacggcctggccccttccgagctctcagcagcctgaactccacgtgtcccctgctgtgtcactggcatgctggtcttgcatggcactgagatgtgtggcacaagcaggcaccaagcccggagacacccgacgctcaccgttagactgggtagcatttgtcaagcgccgagcaaacagtggatgaagtgtcctcagccggcgtcagctgttctgatccgcagaacacataactcctggcactcctttccaagcatccgggaaatgtagaatccaagtgttacaccatccagttgaagatgacagatttacgatataaaacggcacccgcgactgaggactttgtaggaatggaggccgctgtcattatttcatgggtgagggggagagggacactgtgacccatgacaggaaaggacagctcagcccctccaaaaccacacacaggggactccgtttctcacaaaacttcaagtttctgttctacgcaaacattacaacacattttaaactacattctgacacgaagctcccgtgctttttaatggcaggtgttacaatgatcatggaacagtgatggggcggtgcttcctcacggtgacatggcagggagaagtctggaccggagccagcagggtccttgacctaagaggccttgggcagcccacggggcagctctgagcaatctcctgtgaaaggaagagctcagaacgggttcctctaaaggttccttccagagcaggggttctgtggttccctggggccctagactaacatgaggaaggggaaacagagaagaatgcccactaaaagccttacccaaaaattgaaagccaagaaaaatcacaccagatcatctcagtttagacttgaggaacctcggcgctgacatcactgtcaccatcacaaaacactggccaccaaggtgccacctaccacactgcaacctggaaggaggggcgggcaggggcacccctgggcagggcaggacaccaggccagccagccacccacgctacagaggaaatgcagcccctcccaactaagagaaccctggtaccatcaccacagccttggtgccagggctcctagcacctgacagggaagatgagaaggacattggctgccgccaagaggcctgctgcccacccccaactgcacggtggtggtgctgccagcaccaccatccatgctggcccaggagcccacacgcagggcacgcacgcacgtagttccacattaggccctttcttcctcaattgttggaaagaaggccaaagccagatgatggtgaaattcacgaggaaaatgtccccgactgtcctccattctaaagcaaacgctaagaatgggctgctgggcttcagcagaagccaagtcacctttcctctatgcgtccaatgaaacgaaaacatccacacttgtctttataaaaacggaaaactgcatctggaacaaggtctgtggcgtttcttccagcgtgtcccatggacatgaagttggtcttcctatgggtcctccaaggcacacccctcgactgcaccacagcactgagggcagaatgtggtggtggcccagctgccgtggcgccggcagactagcctggtacacggagaggggagcctgctgactgtgggtaggccacgttcccccagtgtcttcatctgcagagggagaccgggagcctctgaagaccgctccagctctgcactgtgggggcggccggccagcaggcaggcaatgctctcaggccccacgctcctctcactggctgccgacgggaggcagacgaggtgccgggggcagcctgcagagcaaggagtcaaggtggccagcctggggcagggtgttcccccagccagggagcttcactcaggcttgggctctgtcccgtgcctccccgggggcgttccgaggtggcggaggaggaagctgcagcccgttatccaccgcccagtctctccctctcaccagcacacagatgttctcagcggcagagcctggcttctgcctgaattcatttcatatttttaaatatgctcttaatggaaagcaacaaaagtacttaacaaaatgcgctgatgtaaatgtccctgcagcagccagggactaattttagaaggggctttgaggagaaacccaagggacactcacttgctggaaacggcctcctccccaaagagtgtgaggatctggattagaaccaagtatccccaggctgcccaggagcccgctcctccaattgggggctggccatcccaccgagcactgataccgcaggctggactcttcctaacctcacgagaggtgatgaccggaatcatcccagttttccatggcacttcgcaaacacagctggtcaggcccttagcacctcctgaccccccgatctcccagactctctgctggaagttaaggacacagagaaagtttcttatgaaaataagcgcctcaaaagaaagccaacgtacagcactggtgacagaaaggaagattcagaaaagccttcacgcctggcaatatggcacacgcacttttagagacgtctaattatactcagggctgagttggctgaagagtgaggaatatactccaaagacaggaattcaaggcagggcaaatagaacatgaaagccagcctggagcccagggcctgtcctggggcagccacctgcactgcctcttaccactgcaccgtccctgtgagtgtgcgtggggaggggctgtagttcccttggcaggggaagccagaagacaggcctgcaagggacacatccgggcctgggcttggtgctggctagaaggggtcaaatcgagagaggactcccctcagaactcataatcccagacccctcgcaatggtttggggagaattcagacaacccatgaggcctgatgagcatccctagcacctgcaaacacaggcatgtcccaggtggcacctcccagcaccaggcagaaaccttctctagaggaacacgctatgaacctcaaaaaaacatccaagaaggacggacataaagtcacaatcaagaaccatgggtagcgggagtaagtcccggaaagacctcagttgtaggaaaatcaggcactgacccaaaacacatacgaaggacactcgacaaaacaagagaggtcatccagggtcaggctggagctagaggcctccagatcctgtcacttagtgactgtacaaacctggtggcttcctcaacctccctgtgccttagcttcccatttgccaaaaagggggattagaagagcccacactctccctggagcaaggctaaggaagaaaggagacagatgtctcagctgttattattaataactatcagaagtgtcacatggatctgaatgatccaaatggaacttgtagaaacaaaactgtcatcattaaaatttaaaactaaatgagtgagttaactaatcaagtattaatagacagagctgaagagagaattagtgaacagtaaaatagcacggaagaaataaaccaggatgcaacacataaaggtaaagagatagaaagctggagacgttagaggactggaaggacagaggaagatatgctaacacacatctgtaaaccaaaaataaaattctaagctcccaaccatctgaatggacccctcctctcaagccaagggcattccaacattaacctgaaaagctagttcaggtcgtgatggggacgggcattcagatgtgcctcatgataccctcctcccttttggaattgctgatagaacagactctttaagtctgatgagaaacatttcagtctattctctctgaagcctgctacccggaggcttcgtcggcatggtaaatccttggtctccacaaacccttatcataatccagacattcctttgtgttgataataactctttcaaccaactgccaatcagaacattttaaaatctacctataatctgaaagcctcacacttcgagttgtcccgcgtttctggactggaccaatgttcatcttccacatactgacagacgcctcatgtctccctaaaaatgtatgaaaccaagctgttccccgaccaccttgggcacatgttgtcagcacctc

SEQ ID NO: 10207 - RNA, 7788 nt, Homo sapiens
  source 1..7788: mol_type = other RNA
caggaaggagacaggcagttcactgtgaattctgagtagtttccctaaaacactgtttccacataaatacaataaactctattattggtatgtcacaagtgctagataaactttttttcttaatatgacaaatgtttaagtagtcctttttatttttcttacaataaaaagtacaatttcttaagaataagttcaataagacgcaaacttccccgccctcctctccttcaaggttttgttttacagaaaaatttccatcttttgtatctgcaaatgtcatgagaggggaacagaaaggcatttttcttcttccccaaagctgccgagtttggcgtgcaaaatctgtatacaatataaagtcatgccggtcgtacagtccatgcaacctccaggtgtaggaaacttaaaaaaatatattcatatatatttatatctatatatttatatatgtatcaatgcccataaaacacgtgggcccaaagtctacaaaaagaagaatggaatgagcacgtggctgtgaccagtaaagaaggaatgttctgatcaaaaagaaaaacaacaaagtccattgctagtgctgcaaaaatcaaacttgcttttgtgtcagaccattacgaaatggtccttccccttgcaaacagattttcaaaagaagtaaagaaaaactgaaacaccttgacaaagtggccctccagaaccagagccctgggacgctggggaggggcggccagtcccagcgggccacggcctccgggacagccgcctgctggtggggcgtgggcacgtgggcacgctgcggcacggcgggaagccgcgagggcagggcagacgccaagaggcccagtggcgtcatcagggtttccctcaaagggatataaagtgctcgcttgctgactcccagccagtgcccccaaggcctttgcaaaggaagaaaaaggctaaaggtccaaggacccacagggagaacacatgaaggaaccctccctgacgtggtcccgcctgcagacgccgaggcagatcctctgccatctgccctggacgcttgctgtggagaagagccgagtgtgtcttcaaagaaaaggctacacagtaatgctctcagcacatttgtgaagctggagtgagctgacagatgaaacgtgcctccccctgccaggcctttgcagagggcgtctccatttgaatgagattagaattaagtccccccactgataacctggccactgagcagtccatgttatcccatcatctgcttaaaaaaaaaaagtgagatgatgcattcctccccataagccacggcggggtaagagggcaggtggcaggatccccagagggctatgcagagaatgaggccaaggaggccagaagagcctgctagctgggccctgccactgctctgtgccatgaatggggaatggaccagctcctcttgccaatctgggcttcagagcaaagagtggccaccagggaggggaaagtcaaacaagtcccaagaccgttctgcctgctctcaaaccactgtctcagagctgaccatcagcagcccagtgaccaagtgaatccaagaatctgcactcatttggtcaaaagtttgagttaatttcagaagctaccctgtaaactttaccaaactccgaaactcggctctgggtccctcctgagcacggtgtgtctgaacttctgcccccaagtctgaacccaatatacactttggaatgaaactggtggcttcatgtgctggaaaataagttaccagtaaaacgtgactgtcagttactgttgaagagaaaaagagtaaagactggctgtcctggtcaggcaatcataccctccctgcaggttcaccaggcaacaagggtccctgggttccttgcagccacaggctccaaaatccagggctggccacgtggctgcagtggaaaaacccaagtgggtaaagagccccacgtgtgccccatgcattgctgacatgctcaaaaggtctttggaaaactcaagttagaattctatcctgacgatgtggtcagagaagtttaaacatgagtttcattaatgctgactgcccccggcatctggcaagcctcccagggtggccgggcatcctaagcaaccctccctgcccttgccacggaggggaaaaacacaccacccctcgtaatactactagtgttgaaagttaaaaagagcccctgggcttctttatacagctcctaggacagaccaggaaagacacaatcgttggtgtcactccgaaaagacctacggtccctcctctcactttctgaaaatagaatctgacagcaacaattctgtacgctgcagaaaactcatcgtacaaaaataaaaacaaaaataattaaaaacctttgaaaggtaaaaaaaaatgtacaagcaagaattcagaaaggaaaaagatttagacattattaccattcagaaaattgctaaatggtgaggaaaaatgtaaaattcataaaacaatgcttattcaggatctttttgtgaaaaaattcatacaaaaatcaacagcaaatttatattctttgctataaaaactcattaggtacatatgtgcatgaaggcttggagacgggagcggttctgttagaaaataattaaaatgaaagtacaaacttgtagggtagttgcccagtggcgaatgtgttggcgatctgaaatctagccaatctggagcttgagaaaacatgaatttcaatcaatcaggatccctttccataagcaccttgagagcaaattcacaagccatccatttgcagggaccttcgcaatctgcattcattttatatatatatatatactttttctataaatgcattataaatattttatcaagatttcataagaatcaagtaagtttcttagcttggaatacattggaatatatattatacatatatatatttatttatacctaaaatttaagcaatacttcatgctacttgcttttaataaaaagcattccgatcgtaacactgcaagtgtgcctaccacatgcttcacgaccagatggagatgctcaatcgtatgtgacgtgtgagaacactttggattcgtttaaaatttgttggacttcaaaacctccaacgggatttgccacttttttggaactacctccatttttcttaaacagcaataaagcaaaacagggaccgccgggctgcagcccctggccccggagatgacggctggtgcccgtgcttgaggcgtcaggccagctcgcggtgccagcactgccaggctcggctggccacaggaaactgtcccaccgattcctgctgtttgttttttcttaaggcattgttcctcagacttcagaaaacccagccacaaaaatccaccagagcaataaaaaaaaaggcacaaactcgcatcttccgatggcttttgagaaactcaagccagctcccccagctcacattcctgtttctgtccagttttgttttctttaaaggtccctctgtcccccacccgggtgcagaccccccgccgcacaccgctatggttcacagaggcgggccacagccgtagaaaacgtcctctttaaaaaaaaataagctacaagatgagtcgagtggtttacacagagactgtggagttgtgggtaataaactttaagcaccagttttaatcaagtttgttttgtattattagatctttgatatttgttttctgtgcctcgtgtcaactgaattcggcagctcggccgcctgttgccacaggctcctttcttccacggcgtcccttgcgggacccgccagagtgtgcttggcttccgcgtgtccgtgtgtctgcgcgtcgccggcgtctgtcccgtgttccctgtgaggctgccacgcccaggcgtgcatgtgcgtctcgagacctgtgggcctgggcggcagaaaggcttcccgtggctgttgcacgctgggtgtccctgggtgctccaagagagccccacggtgggacgcaggcgtgacacgggaaagtttcttggctgagcttcaagacagagacagacagacaagagaacagcagcttcgagggagtgctacaggggcggctcctcttccatgggctcctcatctggtctcttttcggcgggcttcacgcccacggacagcgaggccatggcggtgaccgtctcggcttcttcgttctcgcaagtctgagcctcgatcagagaacgccccgctgtggaggttgtgcgctgcaggcagcgccagtacttgctgtggatctccatgactttctccatggaacggacagcgtttgcattgggtctttgctgtaaaaccttttctgggagaggatcaagctcgtttcccagcaaggcagaaacacatgcttccgaggcgtcgcaaatggcggtcaggtcgtggcctccctcgagggccaggacaatccggccgccagccaggcccatcagctgcttcgtcaggtacccgaagcatctggcggagaggttgtagcccccaagaggggtggggtggccctccacggcatcgaagcctgatgacaccagcaccacatccggggcaaactcgctggcgatcggcatgaccaccgttctgaaggccgccaagtactcagcgtctcccatgggggggtccaggccgccggtgaaagccatgttgacgttgaaacccacgccgggccctgtgcccacctcatcaggagccccgctgcctgggaagaagttcccatcgtcgtagcggtggagggacatgtacaggacgctggggtcgctgtagaaagcctgctgggtcccgtttccatggtgcacgtcccagtccacgatgaggatcttgctcacgctcaacctctgctgcagaagcttggctgccacggccacggagttgaagtagcaaaagcccatgggcgtgctctcctccgcatggtgtccaggggggcggaccacagcaaagccattcttcagctcccctgtggccaccttgaagaccagctctaccacgcagcccacagccaggcgggctgcccccgccgagtgcacctcgttccatatggtgtcactgtccaccccaacaccaccgcaagggagccggacgaacacggaggcgagcgagcctagaagtttcttactgtccagtttctgccggttgagggggttcgtgccatacaggagggtgtgggcttccgagtgcaccgtctgtagctcctccagggtggccttgcgtccgcggatgcactcgcatttgccccggaggcccgtctcctgcaggcgggaccagatgctctggatcctcccggcgtgctcggggtggctgctgctactcccgcaggtgcactggtgcttcagcatcagcgtgtcatacacgaggcctgtcgtgaacctcggcttggtggggggctcctgcacagacacggggaaggtggcagacgcgggtgaggactgcgcccgggacagaggcctgtggccgccgaaggacacggggatgccggcggcctccatggacgcctggtagttcctcagctggtggatccgctgctgctccagcaggagggcttgctgtctgaagagcagctcctgctcactgggctggcgctggcccggctccacctcccgtgggggctctgcctcttcctcatcgctctcaatgggctcctgcttcacctgcacgccggcctgtgcgtgcgcctccttctgccccggcagccggtccaggtagggctcgtccagcagagcctggtgctcacggagctcctcctccgtctcctccgggtggctctccggctgccgggctggctcgcttggcttggggatgatcttgttcatctgcagttgctgctgctggaactgctgcttgtgtttctccagaaactgctgatgctgctgctggatgaccaggtgctgcagagcctgggcgttctggggcagcggggccgactgggtccgccccagtgggcggtgctgccgcagcttgtggatggagggggacacccggtctgcaccaaccaaggactgtgcgtggaggggcagtgctcccaggcctgaaagataccagtctgtgacgaggggtgcttgtgccggcggctgctccagtaagaccatgtgctgcagaagagggctgtgcgctgcccctccgtcccgctccaagggcgaggtgctcaggtagggagtgaggtgggtgccggggaaaagggagagcctctgctggagggcgggaagggtgagtctctcggcgtcctgctggcccgccgtgcccgcagaggggccggtggcaggcaggcccagcgtgatgttgggcaaggatggcgatgtgtagaggggaagtggagcggccgagccttctcgtgccacaagtctgtgcgccaaactcgtctccgccgggatgctggggacggcgggcgcgataccgttctccgcgctgacgctcccggagctgttgttgggtgagctgggtccggagcctggggcgctgctgcacgcggagtctgtgacatccaacggacgcttttttagagcagtgaccactggcccgtctttcctgcgtaacagggggctgctccgtctttcggccactttctgctttagcctggaccgtaatttcagattcggttcagaagctgttttcctaagagggaagtcatctttggcgtcgtacattcccaggaccgggtggttataggaggtcgacactccgctctggggtggagaactctggtcaagggaactgtgctgcgttttcccgtaccagtagcgagggtcgctggaaatgcagtggttcagattccggtgggccagcgccttctttttattgaggacaaattcttgtaacttcatcttcacttctgtgctggccacggcactctctttgcccttctccttgttcttgagctgctgcagcttctgctcccggtgctgcttctccagctcctgctcctggcggtgcctctccagcttccgctggtgttccagcagctcctgctggtgcttcatggccagcatctcctgttgttgcttgatgtgctcgtggagctgcgcctcgtgctgccgggagagctgctcgtgctgcctctggaactcagcgatgaggatctgcctctggatctgctgcttctgcttgagcgccaggagctcctgctgcagctgctgctcccgcagggccggctctgccacaggcagtgagaactggtggtccaggcgcaggtccatgggcactgccgagggggccacttgcagaggcagcgccgtggccacatccaccgtgctgggcatgtggttcacgcgggcaggattcagcagctccactggctggtctcggccagaaagtccatctggatggctttgggagctcattgctagcaatgtccactcctttaagtgattcgaaatggctcaaaatttccacggaaacgatagctccaacgagctccaaactcccaccaacacatacaagtaccgggacggtgagggctgggtcacagacgttcaagcgccgagcctcgccggcaaggtctcatgagccaggtaacccacaagttgaacagaggcgtccgctggcttctgcagatgaaccaaaagacgctccaggcgccagccgctgggtgcttcgcggttgaggaggcgcagggaccgggggccagtagtggccgtaaacacgggccccggccgtgtccggtcgcactcggtagcccgcatggctgcctagcggtcagcaccgcatgtctgcgagcctaattcgcgcttagagggcacacaatggggtgcaggctaacgcggggagccggccaggcctcgccgcggcgtccatcttggatactggc

SEQ ID NO: 10208 - RNA, 7601 nt, Homo sapiens
  source 1..7601: mol_type = other RNA
caggaaggagacaggcagttcactgtgaattctgagtagtttccctaaaacactgtttccacataaatacaataaactctattattggtatgtcacaagtgctagataaactttttttcttaatatgacaaatgtttaagtagtcctttttatttttcttacaataaaaagtacaatttcttaagaataagttcaataagacgcaaacttccccgccctcctctccttcaaggttttgttttacagaaaaatttccatcttttgtatctgcaaatgtcatgagaggggaacagaaaggcatttttcttcttccccaaagctgccgagtttggcgtgcaaaatctgtatacaatataaagtcatgccggtcgtacagtccatgcaacctccaggtgtaggaaacttaaaaaaatatattcatatatatttatatctatatatttatatatgtatcaatgcccataaaacacgtgggcccaaagtctacaaaaagaagaatggaatgagcacgtggctgtgaccagtaaagaaggaatgttctgatcaaaaagaaaaacaacaaagtccattgctagtgctgcaaaaatcaaacttgcttttgtgtcagaccattacgaaatggtccttccccttgcaaacagattttcaaaagaagtaaagaaaaactgaaacaccttgacaaagtggccctccagaaccagagccctgggacgctggggaggggcggccagtcccagcgggccacggcctccgggacagccgcctgctggtggggcgtgggcacgtgggcacgctgcggcacggcgggaagccgcgagggcagggcagacgccaagaggcccagtggcgtcatcagggtttccctcaaagggatataaagtgctcgcttgctgactcccagccagtgcccccaaggcctttgcaaaggaagaaaaaggctaaaggtccaaggacccacagggagaacacatgaaggaaccctccctgacgtggtcccgcctgcagacgccgaggcagatcctctgccatctgccctggacgcttgctgtggagaagagccgagtgtgtcttcaaagaaaaggctacacagtaatgctctcagcacatttgtgaagctggagtgagctgacagatgaaacgtgcctccccctgccaggcctttgcagagggcgtctccatttgaatgagattagaattaagtccccccactgataacctggccactgagcagtccatgttatcccatcatctgcttaaaaaaaaaaagtgagatgatgcattcctccccataagccacggcggggtaagagggcaggtggcaggatccccagagggctatgcagagaatgaggccaaggaggccagaagagcctgctagctgggccctgccactgctctgtgccatgaatggggaatggaccagctcctcttgccaatctgggcttcagagcaaagagtggccaccagggaggggaaagtcaaacaagtcccaagaccgttctgcctgctctcaaaccactgtctcagagctgaccatcagcagcccagtgaccaagtgaatccaagaatctgcactcatttggtcaaaagtttgagttaatttcagaagctaccctgtaaactttaccaaactccgaaactcggctctgggtccctcctgagcacggtgtgtctgaacttctgcccccaagtctgaacccaatatacactttggaatgaaactggtggcttcatgtgctggaaaataagttaccagtaaaacgtgactgtcagttactgttgaagagaaaaagagtaaagactggctgtcctggtcaggcaatcataccctccctgcaggttcaccaggcaacaagggtccctgggttccttgcagccacaggctccaaaatccagggctggccacgtggctgcagtggaaaaacccaagtgggtaaagagccccacgtgtgccccatgcattgctgacatgctcaaaaggtctttggaaaactcaagttagaattctatcctgacgatgtggtcagagaagtttaaacatgagtttcattaatgctgactgcccccggcatctggcaagcctcccagggtggccgggcatcctaagcaaccctccctgcccttgccacggaggggaaaaacacaccacccctcgtaatactactagtgttgaaagttaaaaagagcccctgggcttctttatacagctcctaggacagaccaggaaagacacaatcgttggtgtcactccgaaaagacctacggtccctcctctcactttctgaaaatagaatctgacagcaacaattctgtacgctgcagaaaactcatcgtacaaaaataaaaacaaaaataattaaaaacctttgaaaggtaaaaaaaaatgtacaagcaagaattcagaaaggaaaaagatttagacattattaccattcagaaaattgctaaatggtgaggaaaaatgtaaaattcataaaacaatgcttattcaggatctttttgtgaaaaaattcatacaaaaatcaacagcaaatttatattctttgctataaaaactcattaggtacatatgtgcatgaaggcttggagacgggagcggttctgttagaaaataattaaaatgaaagtacaaacttgtagggtagttgcccagtggcgaatgtgttggcgatctgaaatctagccaatctggagcttgagaaaacatgaatttcaatcaatcaggatccctttccataagcaccttgagagcaaattcacaagccatccatttgcagggaccttcgcaatctgcattcattttatatatatatatatactttttctataaatgcattataaatattttatcaagatttcataagaatcaagtaagtttcttagcttggaatacattggaatatatattatacatatatatatttatttatacctaaaatttaagcaatacttcatgctacttgcttttaataaaaagcattccgatcgtaacactgcaagtgtgcctaccacatgcttcacgaccagatggagatgctcaatcgtatgtgacgtgtgagaacactttggattcgtttaaaatttgttggacttcaaaacctccaacgggatttgccacttttttggaactacctccatttttcttaaacagcaataaagcaaaacagggaccgccgggctgcagcccctggccccggagatgacggctggtgcccgtgcttgaggcgtcaggccagctcgcggtgccagcactgccaggctcggctggccacaggaaactgtcccaccgattcctgctgtttgttttttcttaaggcattgttcctcagacttcagaaaacccagccacaaaaatccaccagagcaataaaaaaaaaggcacaaactcgcatcttccgatggcttttgagaaactcaagccagctcccccagctcacattcctgtttctgtccagttttgttttctttaaaggtccctctgtcccccacccgggtgcagaccccccgccgcacaccgctatggttcacagaggcgggccacagccgtagaaaacgtcctctttaaaaaaaaataagctacaagatgagtcgagtggtttacacagagactgtggagttgtgggtaataaactttaagcaccagttttaatcaagtttgttttgtattattagatctttgatatttgttttctgtgcctcgtgtcaactgaattcggcagctcggccgcctgttgccacaggctcctttcttccacggcgtcccttgcgggacccgccagagtgtgcttggcttccgcgtgtccgtgtgtctgcgcgtcgccggcgtctgtcccgtgttccctgtgaggctgccacgcccaggcgtgcatgtgcgtctcgagacctgtgggcctgggcggcagaaaggcttcccgtggctgttgcacgctgggtgtccctgggtgctccaagagagccccacggtgggacgcaggcgtgacacgggaaagtttcttggctgagcttcaagacagagacagacagacaagagaacagcagcttcgagggagtgctacaggggcggctcctcttccatgggctcctcatctggtctcttttcggcgggcttcacgcccacggacagcgaggccatggcggtgaccgtctcggcttcttcgttctcgcaagtctgagcctcgatcagagaacgccccgctgtggaggttgtgcgctgcaggcagcgccagtacttgctgtggatctccatgactttctccatggaacggacagcgtttgcattgggtctttgctgtaaaaccttttctgggagaggatcaagctcgtttcccagcaaggcagaaacacatgcttccgaggcgtcgcaaatggcggtcaggtcgtggcctccctcgagggccaggacaatccggccgccagccaggcccatcagctgcttcgtcaggtacccgaagcatctggcggagaggttgtagcccccaagaggggtggggtggccctccacggcatcgaagcctgatgacaccagcaccacatccggggcaaactcgctggcgatcggcatgaccaccgttctgaaggccgccaagtactcagcgtctcccatgggggggtccaggccgccggtgaaagccatgttgacgttgaaacccacgccgggccctgtgcccacctcatcaggagccccgctgcctgggaagaagttcccatcgtcgtagcggtggagggacatgtacaggacgctggggtcgctgtagaaagcctgctgggtcccgtttccatggtgcacgtcccagtccacgatgaggatcttgctcacgctcaacctctgctgcagaagcttggctgccacggccacggagttgaagtagcaaaagcccatgggcgtgctctcctccgcatggtgtccaggggggcggaccacagcaaagccattcttcagctcccctgtggccaccttgaagaccagctctaccacgcagcccacagccaggcgggctgcccccgccgagtgcacctcgttccatatggtgtcactgtccaccccaacaccaccgcaagggagccggacgaacacggaggcgagcgagcctagaagtttcttactgtccagtttctgccggttgagggggttcgtgccatacaggagggtgtgggcttccgagtgcaccgtctgtagctcctccagggtggccttgcgtccgcggatgcactcgcatttgccccggaggcccgtctcctgcaggcgggaccagatgctctggatcctcccggcgtgctcggggtggctgctgctactcccgcaggtgcactggtgcttcagcatcagcgtgtcatacacgaggcctgtcgtgaacctcggcttggtggggggctcctgcacagacacggggaaggtggcagacgcgggtgaggactgcgcccgggacagaggcctgtggccgccgaaggacacggggatgccggcggcctccatggacgcctggtagttcctcagctggtggatccgctgctgctccagcaggagggcttgctgtctgaagagcagctcctgctcactgggctggcgctggcccggctccacctcccgtgggggctctgcctcttcctcatcgctctcaatgggctcctgcttcacctgcacgccggcctgtgcgtgcgcctccttctgccccggcagccggtccaggtagggctcgtccagcagagcctggtgctcacggagctcctcctccgtctcctccgggtggctctccggctgccgggctggctcgcttggcttggggatgatcttgttcatctgcagttgctgctgctggaactgctgcttgtgtttctccagaaactgctgatgctgctgctggatgaccaggtgctgcagagcctgggcgttctggggcagcggggccgactgggtccgccccagtgggcggtgctgccgcagcttgtggatggagggggacacccggtctgcaccaaccaaggactgtgcgtggaggggcagtgctcccaggcctgaaagataccagtctgtgacgaggggtgcttgtgccggcggctgctccagtaagaccatgtgctgcagaagagggctgtgcgctgcccctccgtcccgctccaagggcgaggtgctcaggtagggagtgaggtgggtgccggggaaaagggagagcctctgctggagggcgggaagggtgagtctctcggcgtcctgctggcccgccgtgcccgcagaggggccggtggcaggcaggcccagcgtgatgttgggcaaggatggcgatgtgtagaggggaagtggagcggccgagccttctcgtgccacaagtctgtgcgccaaactcgtctccgccgggatgctggggacggcgggcgcgataccgttctccgcgctgacgctcccggagctgttgttgggtgagctgggtccggagcctggggcgctgctgcacgcggagtctgtgacatccaacggacgcttttttagagcagtgaccactggcccgtctttcctgcgtaacagggggctgctccgtctttcggccactttctgctttagcctggaccgtaatttcagattcggttcagaagctgttttcctaagagggaagtcatctttggcgtcgtacattcccaggaccgggtggttataggaggtcgacactccgctctggggtggagaactctggtcaagggaactgtgctgcgttttcccgtaccagtagcgagggtcgctggaaatgcagtggttcagattccggtgggccagcgccttctttttattgaggacaaattcttgtaacttcatcttcacttctgtgctggccacggcactctctttgcccttctccttgttcttgagctgctgcagcttctgctcccggtgctgcttctccagctcctgctcctggcggtgcctctccagcttccgctggtgttccagcagctcctgctggtgcttcatggccagcatctcctgttgttgcttgatgtgctcgtggagctgcgcctcgtgctgccgggagagctgctcgtgctgcctctggaactcagcgatgaggatctgcctctggatctgctgcttctgcttgagcgccaggagctcctgctgcagctgctgctcccgcagggccggctctgccacaggcagtgagaactggtggtccaggcgcaggtccatgggcactgccgagggggccacttgcagaggcagcgccgtggccacatccaccgtgctgggcatgtggttcacgcgggcaggattcagcagctccactggctggtctcggccagaaagtccatctggatggctttgggagctcattgctagcaatgtccactcctttaagtgattcgaaatggctcaaaatttccacggaaacgatagctccaacgagctccaaactcccaccaacacatacaagtaccgggacggtgagggctgggtcacagacgttcaagcgccgagcctcgccggcaaggtctcatgagccaggtaacccacaagttgaacagaggcgtccgctggcttctgcagatgaaccgcggcgggcggcggcggccggctctagccctgctccggcgctccgcgccgcatctcctca

SEQ ID NO: 10209 - RNA, 7582 nt, Homo sapiens
  source 1..7582: mol_type = other RNA
caggaaggagacaggcagttcactgtgaattctgagtagtttccctaaaacactgtttccacataaatacaataaactctattattggtatgtcacaagtgctagataaactttttttcttaatatgacaaatgtttaagtagtcctttttatttttcttacaataaaaagtacaatttcttaagaataagttcaataagacgcaaacttccccgccctcctctccttcaaggttttgttttacagaaaaatttccatcttttgtatctgcaaatgtcatgagaggggaacagaaaggcatttttcttcttccccaaagctgccgagtttggcgtgcaaaatctgtatacaatataaagtcatgccggtcgtacagtccatgcaacctccaggtgtaggaaacttaaaaaaatatattcatatatatttatatctatatatttatatatgtatcaatgcccataaaacacgtgggcccaaagtctacaaaaagaagaatggaatgagcacgtggctgtgaccagtaaagaaggaatgttctgatcaaaaagaaaaacaacaaagtccattgctagtgctgcaaaaatcaaacttgcttttgtgtcagaccattacgaaatggtccttccccttgcaaacagattttcaaaagaagtaaagaaaaactgaaacaccttgacaaagtggccctccagaaccagagccctgggacgctggggaggggcggccagtcccagcgggccacggcctccgggacagccgcctgctggtggggcgtgggcacgtgggcacgctgcggcacggcgggaagccgcgagggcagggcagacgccaagaggcccagtggcgtcatcagggtttccctcaaagggatataaagtgctcgcttgctgactcccagccagtgcccccaaggcctttgcaaaggaagaaaaaggctaaaggtccaaggacccacagggagaacacatgaaggaaccctccctgacgtggtcccgcctgcagacgccgaggcagatcctctgccatctgccctggacgcttgctgtggagaagagccgagtgtgtcttcaaagaaaaggctacacagtaatgctctcagcacatttgtgaagctggagtgagctgacagatgaaacgtgcctccccctgccaggcctttgcagagggcgtctccatttgaatgagattagaattaagtccccccactgataacctggccactgagcagtccatgttatcccatcatctgcttaaaaaaaaaaagtgagatgatgcattcctccccataagccacggcggggtaagagggcaggtggcaggatccccagagggctatgcagagaatgaggccaaggaggccagaagagcctgctagctgggccctgccactgctctgtgccatgaatggggaatggaccagctcctcttgccaatctgggcttcagagcaaagagtggccaccagggaggggaaagtcaaacaagtcccaagaccgttctgcctgctctcaaaccactgtctcagagctgaccatcagcagcccagtgaccaagtgaatccaagaatctgcactcatttggtcaaaagtttgagttaatttcagaagctaccctgtaaactttaccaaactccgaaactcggctctgggtccctcctgagcacggtgtgtctgaacttctgcccccaagtctgaacccaatatacactttggaatgaaactggtggcttcatgtgctggaaaataagttaccagtaaaacgtgactgtcagttactgttgaagagaaaaagagtaaagactggctgtcctggtcaggcaatcataccctccctgcaggttcaccaggcaacaagggtccctgggttccttgcagccacaggctccaaaatccagggctggccacgtggctgcagtggaaaaacccaagtgggtaaagagccccacgtgtgccccatgcattgctgacatgctcaaaaggtctttggaaaactcaagttagaattctatcctgacgatgtggtcagagaagtttaaacatgagtttcattaatgctgactgcccccggcatctggcaagcctcccagggtggccgggcatcctaagcaaccctccctgcccttgccacggaggggaaaaacacaccacccctcgtaatactactagtgttgaaagttaaaaagagcccctgggcttctttatacagctcctaggacagaccaggaaagacacaatcgttggtgtcactccgaaaagacctacggtccctcctctcactttctgaaaatagaatctgacagcaacaattctgtacgctgcagaaaactcatcgtacaaaaataaaaacaaaaataattaaaaacctttgaaaggtaaaaaaaaatgtacaagcaagaattcagaaaggaaaaagatttagacattattaccattcagaaaattgctaaatggtgaggaaaaatgtaaaattcataaaacaatgcttattcaggatctttttgtgaaaaaattcatacaaaaatcaacagcaaatttatattctttgctataaaaactcattaggtacatatgtgcatgaaggcttggagacgggagcggttctgttagaaaataattaaaatgaaagtacaaacttgtagggtagttgcccagtggcgaatgtgttggcgatctgaaatctagccaatctggagcttgagaaaacatgaatttcaatcaatcaggatccctttccataagcaccttgagagcaaattcacaagccatccatttgcagggaccttcgcaatctgcattcattttatatatatatatatactttttctataaatgcattataaatattttatcaagatttcataagaatcaagtaagtttcttagcttggaatacattggaatatatattatacatatatatatttatttatacctaaaatttaagcaatacttcatgctacttgcttttaataaaaagcattccgatcgtaacactgcaagtgtgcctaccacatgcttcacgaccagatggagatgctcaatcgtatgtgacgtgtgagaacactttggattcgtttaaaatttgttggacttcaaaacctccaacgggatttgccacttttttggaactacctccatttttcttaaacagcaataaagcaaaacagggaccgccgggctgcagcccctggccccggagatgacggctggtgcccgtgcttgaggcgtcaggccagctcgcggtgccagcactgccaggctcggctggccacaggaaactgtcccaccgattcctgctgtttgttttttcttaaggcattgttcctcagacttcagaaaacccagccacaaaaatccaccagagcaataaaaaaaaaggcacaaactcgcatcttccgatggcttttgagaaactcaagccagctcccccagctcacattcctgtttctgtccagttttgttttctttaaaggtccctctgtcccccacccgggtgcagaccccccgccgcacaccgctatggttcacagaggcgggccacagccgtagaaaacgtcctctttaaaaaaaaataagctacaagatgagtcgagtggtttacacagagactgtggagttgtgggtaataaactttaagcaccagttttaatcaagtttgttttgtattattagatctttgatatttgttttctgtgcctcgtgtcaactgaattcggcagctcggccgcctgttgccacaggctcctttcttccacggcgtcccttgcgggacccgccagagtgtgcttggcttccgcgtgtccgtgtgtctgcgcgtcgccggcgtctgtcccgtgttccctgtgaggctgccacgcccaggcgtgcatgtgcgtctcgagacctgtgggcctgggcggcagaaaggcttcccgtggctgttgcacgctgggtgtccctgggtgctccaagagagccccacggtgggacgcaggcgtgacacgggaaagtttcttggctgagcttcaagacagagacagacagacaagagaacagcagcttcgagggagtgctacaggggcggctcctcttccatgggctcctcatctggtctcttttcggcgggcttcacgcccacggacagcgaggccatggcggtgaccgtctcggcttcttcgttctcgcaagtctgagcctcgatcagagaacgccccgctgtggaggttgtgcgctgcaggcagcgccagtacttgctgtggatctccatgactttctccatggaacggacagcgtttgcattgggtctttgctgtaaaaccttttctgggagaggatcaagctcgtttcccagcaaggcagaaacacatgcttccgaggcgtcgcaaatggcggtcaggtcgtggcctccctcgagggccaggacaatccggccgccagccaggcccatcagctgcttcgtcaggtacccgaagcatctggcggagaggttgtagcccccaagaggggtggggtggccctccacggcatcgaagcctgatgacaccagcaccacatccggggcaaactcgctggcgatcggcatgaccaccgttctgaaggccgccaagtactcagcgtctcccatgggggggtccaggccgccggtgaaagccatgttgacgttgaaacccacgccgggccctgtgcccacctcatcaggagccccgctgcctgggaagaagttcccatcgtcgtagcggtggagggacatgtacaggacgctggggtcgctgtagaaagcctgctgggtcccgtttccatggtgcacgtcccagtccacgatgaggatcttgctcacgctcaacctctgctgcagaagcttggctgccacggccacggagttgaagtagcaaaagcccatgggcgtgctctcctccgcatggtgtccaggggggcggaccacagcaaagccattcttcagctcccctgtggccaccttgaagaccagctctaccacgcagcccacagccaggcgggctgcccccgccgagtgcacctcgttccatatggtgtcactgtccaccccaacaccaccgcaagggagccggacgaacacggaggcgagcgagcctagaagtttcttactgtccagtttctgccggttgagggggttcgtgccatacaggagggtgtgggcttccgagtgcaccgtctgtagctcctccagggtggccttgcgtccgcggatgcactcgcatttgccccggaggcccgtctcctgcaggcgggaccagatgctctggatcctcccggcgtgctcggggtggctgctgctactcccgcaggtgcactggtgcttcagcatcagcgtgtcatacacgaggcctgtcgtgaacctcggcttggtggggggctcctgcacagacacggggaaggtggcagacgcgggtgaggactgcgcccgggacagaggcctgtggccgccgaaggacacggggatgccggcggcctccatggacgcctggtagttcctcagctggtggatccgctgctgctccagcaggagggcttgctgtctgaagagcagctcctgctcactgggctggcgctggcccggctccacctcccgtgggggctctgcctcttcctcatcgctctcaatgggctcctgcttcacctgcacgccggcctgtgcgtgcgcctccttctgccccggcagccggtccaggtagggctcgtccagcagagcctggtgctcacggagctcctcctccgtctcctccgggtggctctccggctgccgggctggctcgcttggcttggggatgatcttgttcatctgcagttgctgctgctggaactgctgcttgtgtttctccagaaactgctgatgctgctgctggatgaccaggtgctgcagagcctgggcgttctggggcagcggggccgactgggtccgccccagtgggcggtgctgccgcagcttgtggatggagggggacacccggtctgcaccaaccaaggactgtgcgtggaggggcagtgctcccaggcctgaaagataccagtctgtgacgaggggtgcttgtgccggcggctgctccagtaagaccatgtgctgcagaagagggctgtgcgctgcccctccgtcccgctccaagggcgaggtgctcaggtagggagtgaggtgggtgccggggaaaagggagagcctctgctggagggcgggaagggtgagtctctcggcgtcctgctggcccgccgtgcccgcagaggggccggtggcaggcaggcccagcgtgatgttgggcaaggatggcgatgtgtagaggggaagtggagcggccgagccttctcgtgccacaagtctgtgcgccaaactcgtctccgccgggatgctggggacggcgggcgcgataccgttctccgcgctgacgctcccggagctgttgttgggtgagctgggtccggagcctggggcgctgctgcacgcggagtctgtgacatccaacggacgcttttttagagcagtgaccactggcccgtctttcctgcgtaacagggggctgctccgtctttcggccactttctgctttagcctggaccgtaatttcagattcggttcagaagctgttttcctaagagggaagtcatctttggcgtcgtacattcccaggaccgggtggttataggaggtcgacactccgctctggggtggagaactctggtcaagggaactgtgctgcgttttcccgtaccagtagcgagggtcgctggaaatgcagtggttcagattccggtgggccagcgccttctttttattgaggacaaattcttgtaacttcatcttcacttctgtgctggccacggcactctctttgcccttctccttgttcttgagctgctgcagcttctgctcccggtgctgcttctccagctcctgctcctggcggtgcctctccagcttccgctggtgttccagcagctcctgctggtgcttcatggccagcatctcctgttgttgcttgatgtgctcgtggagctgcgcctcgtgctgccgggagagctgctcgtgctgcctctggaactcagcgatgaggatctgcctctggatctgctgcttctgcttgagcgccaggagctcctgctgcagctgctgctcccgcagggccggctctgccacaggcagtgagaactggtggtccaggcgcaggtccatgggcactgccgagggggccacttgcagaggcagcgccgtggccacatccaccgtgctgggcatgtggttcacgcgggcaggattcagcagctccactggctggtctcggccagaaagtccatctggatggctttgggagctcattgctagcaatgtccactcctttaagtgattcgaaatggctcaaaatttccacggaaacgatagctccaacgagctccaaactcccaccaacacatacaagtaccgggacggtgagggctgggtcacagacgttcaagcgccgagcctcgccggcaaggtctcatgagccaggtaacccacaagttgaacagaggcgtccgctggcttctgcagatgaacctgctcggggggcgcgggccccgcaccgggagacggcgccgc

SEQ ID NO: 10210 - RNA, 7583 nt, Homo sapiens
  source 1..7583: mol_type = other RNA
caggaaggagacaggcagttcactgtgaattctgagtagtttccctaaaacactgtttccacataaatacaataaactctattattggtatgtcacaagtgctagataaactttttttcttaatatgacaaatgtttaagtagtcctttttatttttcttacaataaaaagtacaatttcttaagaataagttcaataagacgcaaacttccccgccctcctctccttcaaggttttgttttacagaaaaatttccatcttttgtatctgcaaatgtcatgagaggggaacagaaaggcatttttcttcttccccaaagctgccgagtttggcgtgcaaaatctgtatacaatataaagtcatgccggtcgtacagtccatgcaacctccaggtgtaggaaacttaaaaaaatatattcatatatatttatatctatatatttatatatgtatcaatgcccataaaacacgtgggcccaaagtctacaaaaagaagaatggaatgagcacgtggctgtgaccagtaaagaaggaatgttctgatcaaaaagaaaaacaacaaagtccattgctagtgctgcaaaaatcaaacttgcttttgtgtcagaccattacgaaatggtccttccccttgcaaacagattttcaaaagaagtaaagaaaaactgaaacaccttgacaaagtggccctccagaaccagagccctgggacgctggggaggggcggccagtcccagcgggccacggcctccgggacagccgcctgctggtggggcgtgggcacgtgggcacgctgcggcacggcgggaagccgcgagggcagggcagacgccaagaggcccagtggcgtcatcagggtttccctcaaagggatataaagtgctcgcttgctgactcccagccagtgcccccaaggcctttgcaaaggaagaaaaaggctaaaggtccaaggacccacagggagaacacatgaaggaaccctccctgacgtggtcccgcctgcagacgccgaggcagatcctctgccatctgccctggacgcttgctgtggagaagagccgagtgtgtcttcaaagaaaaggctacacagtaatgctctcagcacatttgtgaagctggagtgagctgacagatgaaacgtgcctccccctgccaggcctttgcagagggcgtctccatttgaatgagattagaattaagtccccccactgataacctggccactgagcagtccatgttatcccatcatctgcttaaaaaaaaaaagtgagatgatgcattcctccccataagccacggcggggtaagagggcaggtggcaggatccccagagggctatgcagagaatgaggccaaggaggccagaagagcctgctagctgggccctgccactgctctgtgccatgaatggggaatggaccagctcctcttgccaatctgggcttcagagcaaagagtggccaccagggaggggaaagtcaaacaagtcccaagaccgttctgcctgctctcaaaccactgtctcagagctgaccatcagcagcccagtgaccaagtgaatccaagaatctgcactcatttggtcaaaagtttgagttaatttcagaagctaccctgtaaactttaccaaactccgaaactcggctctgggtccctcctgagcacggtgtgtctgaacttctgcccccaagtctgaacccaatatacactttggaatgaaactggtggcttcatgtgctggaaaataagttaccagtaaaacgtgactgtcagttactgttgaagagaaaaagagtaaagactggctgtcctggtcaggcaatcataccctccctgcaggttcaccaggcaacaagggtccctgggttccttgcagccacaggctccaaaatccagggctggccacgtggctgcagtggaaaaacccaagtgggtaaagagccccacgtgtgccccatgcattgctgacatgctcaaaaggtctttggaaaactcaagttagaattctatcctgacgatgtggtcagagaagtttaaacatgagtttcattaatgctgactgcccccggcatctggcaagcctcccagggtggccgggcatcctaagcaaccctccctgcccttgccacggaggggaaaaacacaccacccctcgtaatactactagtgttgaaagttaaaaagagcccctgggcttctttatacagctcctaggacagaccaggaaagacacaatcgttggtgtcactccgaaaagacctacggtccctcctctcactttctgaaaatagaatctgacagcaacaattctgtacgctgcagaaaactcatcgtacaaaaataaaaacaaaaataattaaaaacctttgaaaggtaaaaaaaaatgtacaagcaagaattcagaaaggaaaaagatttagacattattaccattcagaaaattgctaaatggtgaggaaaaatgtaaaattcataaaacaatgcttattcaggatctttttgtgaaaaaattcatacaaaaatcaacagcaaatttatattctttgctataaaaactcattaggtacatatgtgcatgaaggcttggagacgggagcggttctgttagaaaataattaaaatgaaagtacaaacttgtagggtagttgcccagtggcgaatgtgttggcgatctgaaatctagccaatctggagcttgagaaaacatgaatttcaatcaatcaggatccctttccataagcaccttgagagcaaattcacaagccatccatttgcagggaccttcgcaatctgcattcattttatatatatatatatactttttctataaatgcattataaatattttatcaagatttcataagaatcaagtaagtttcttagcttggaatacattggaatatatattatacatatatatatttatttatacctaaaatttaagcaatacttcatgctacttgcttttaataaaaagcattccgatcgtaacactgcaagtgtgcctaccacatgcttcacgaccagatggagatgctcaatcgtatgtgacgtgtgagaacactttggattcgtttaaaatttgttggacttcaaaacctccaacgggatttgccacttttttggaactacctccatttttcttaaacagcaataaagcaaaacagggaccgccgggctgcagcccctggccccggagatgacggctggtgcccgtgcttgaggcgtcaggccagctcgcggtgccagcactgccaggctcggctggccacaggaaactgtcccaccgattcctgctgtttgttttttcttaaggcattgttcctcagacttcagaaaacccagccacaaaaatccaccagagcaataaaaaaaaaggcacaaactcgcatcttccgatggcttttgagaaactcaagccagctcccccagctcacattcctgtttctgtccagttttgttttctttaaaggtccctctgtcccccacccgggtgcagaccccccgccgcacaccgctatggttcacagaggcgggccacagccgtagaaaacgtcctctttaaaaaaaaataagctacaagatgagtcgagtggtttacacagagactgtggagttgtgggtaataaactttaagcaccagttttaatcaagtttgttttgtattattagatctttgatatttgttttctgtgcctcgtgtcaactgaattcggcagctcggccgcctgttgccacaggctcctttcttccacggcgtcccttgcgggacccgccagagtgtgcttggcttccgcgtgtccgtgtgtctgcgcgtcgccggcgtctgtcccgtgttccctgtgaggctgccacgcccaggcgtgcatgtgcgtctcgagacctgtgggcctgggcggcagaaaggcttcccgtggctgttgcacgctgggtgtccctgggtgctccaagagagccccacggtgggacgcaggcgtgacacgggaaagtttcttggctgagcttcaagacagagacagacagacaagagaacagcagcttcgagggagtgctacaggggcggctcctcttccatgggctcctcatctggtctcttttcggcgggcttcacgcccacggacagcgaggccatggcggtgaccgtctcggcttcttcgttctcgcaagtctgagcctcgatcagagaacgccccgctgtggaggttgtgcgctgcaggcagcgccagtacttgctgtggatctccatgactttctccatggaacggacagcgtttgcattgggtctttgctgtaaaaccttttctgggagaggatcaagctcgtttcccagcaaggcagaaacacatgcttccgaggcgtcgcaaatggcggtcaggtcgtggcctccctcgagggccaggacaatccggccgccagccaggcccatcagctgcttcgtcaggtacccgaagcatctggcggagaggttgtagcccccaagaggggtggggtggccctccacggcatcgaagcctgatgacaccagcaccacatccggggcaaactcgctggcgatcggcatgaccaccgttctgaaggccgccaagtactcagcgtctcccatgggggggtccaggccgccggtgaaagccatgttgacgttgaaacccacgccgggccctgtgcccacctcatcaggagccccgctgcctgggaagaagttcccatcgtcgtagcggtggagggacatgtacaggacgctggggtcgctgtagaaagcctgctgggtcccgtttccatggtgcacgtcccagtccacgatgaggatcttgctcacgctcaacctctgctgcagaagcttggctgccacggccacggagttgaagtagcaaaagcccatgggcgtgctctcctccgcatggtgtccaggggggcggaccacagcaaagccattcttcagctcccctgtggccaccttgaagaccagctctaccacgcagcccacagccaggcgggctgcccccgccgagtgcacctcgttccatatggtgtcactgtccaccccaacaccaccgcaagggagccggacgaacacggaggcgagcgagcctagaagtttcttactgtccagtttctgccggttgagggggttcgtgccatacaggagggtgtgggcttccgagtgcaccgtctgtagctcctccagggtggccttgcgtccgcggatgcactcgcatttgccccggaggcccgtctcctgcaggcgggaccagatgctctggatcctcccggcgtgctcggggtggctgctgctactcccgcaggtgcactggtgcttcagcatcagcgtgtcatacacgaggcctgtcgtgaacctcggcttggtggggggctcctgcacagacacggggaaggtggcagacgcgggtgaggactgcgcccgggacagaggcctgtggccgccgaaggacacggggatgccggcggcctccatggacgcctggtagttcctcagctggtggatccgctgctgctccagcaggagggcttgctgtctgaagagcagctcctgctcactgggctggcgctggcccggctccacctcccgtgggggctctgcctcttcctcatcgctctcaatgggctcctgcttcacctgcacgccggcctgtgcgtgcgcctccttctgccccggcagccggtccaggtagggctcgtccagcagagcctggtgctcacggagctcctcctccgtctcctccgggtggctctccggctgccgggctggctcgcttggcttggggatgatcttgttcatctgcagttgctgctgctggaactgctgcttgtgtttctccagaaactgctgatgctgctgctggatgaccaggtgctgcagagcctgggcgttctggggcagcggggccgactgggtccgccccagtgggcggtgctgccgcagcttgtggatggagggggacacccggtctgcaccaaccaaggactgtgcgtggaggggcagtgctcccaggcctgaaagataccagtctgtgacgaggggtgcttgtgccggcggctgctccagtaagaccatgtgctgcagaagagggctgtgcgctgcccctccgtcccgctccaagggcgaggtgctcaggtagggagtgaggtgggtgccggggaaaagggagagcctctgctggagggcgggaagggtgagtctctcggcgtcctgctggcccgccgtgcccgcagaggggccggtggcaggcaggcccagcgtgatgttgggcaaggatggcgatgtgtagaggggaagtggagcggccgagccttctcgtgccacaagtctgtgcgccaaactcgtctccgccgggatgctggggacggcgggcgcgataccgttctccgcgctgacgctcccggagctgttgttgggtgagctgggtccggagcctggggcgctgctgcacgcggagtctgtgacatccaacggacgcttttttagagcagtgaccactggcccgtctttcctgcgtaacagggggctgctccgtctttcggccactttctgctttagcctggaccgtaatttcagattcggttcagaagctgttttcctaagagggaagtcatctttggcgtcgtacattcccaggaccgggtggttataggaggtcgacactccgctctggggtggagaactctggtcaagggaactgtgctgcgttttcccgtaccagtagcgagggtcgctggaaatgcagtggttcagattccggtgggccagcgccttctttttattgaggacaaattcttgtaacttcatcttcacttctgtgctggccacggcactctctttgcccttctccttgttcttgagctgctgcagcttctgctcccggtgctgcttctccagctcctgctcctggcggtgcctctccagcttccgctggtgttccagcagctcctgctggtgcttcatggccagcatctcctgttgttgcttgatgtgctcgtggagctgcgcctcgtgctgccgggagagctgctcgtgctgcctctggaactcagcgatgaggatctgcctctggatctgctgcttctgcttgagcgccaggagctcctgctgcagctgctgctcccgcagggccggctctgccacaggcagtgagaactggtggtccaggcgcaggtccatgggcactgccgagggggccacttgcagaggcagcgccgtggccacatccaccgtgctgggcatgtggttcacgcgggcaggattcagcagctccactggctggtctcggccagaaagtccatctggatggctttgggagctcattgctagcaatgtccactcctttaagtgattcgaaatggctcaaaatttccacggaaacgatagctccaacgagctccaaactcccaccaacacatacaagtaccgggacggtgagggctgggtcacagacgttcaagcgccgagcctcgccggcaaggtctcatgagccaggtaacccacaagttgaacagaggcgtccgctggcttctgcagatgaacgttgaaccatgatgcttctccccactccagcgtcgagccaggc

SEQ ID NO: 10211 - RNA, 13511 nt, Homo sapiens
  source 1..13511: mol_type = other RNA
caggaaggagacaggcagttcactgtgaattctgagtagtttccctaaaacactgtttccacataaatacaataaactctattattggtatgtcacaagtgctagataaactttttttcttaatatgacaaatgtttaagtagtcctttttatttttcttacaataaaaagtacaatttcttaagaataagttcaataagacgcaaacttccccgccctcctctccttcaaggttttgttttacagaaaaatttccatcttttgtatctgcaaatgtcatgagaggggaacagaaaggcatttttcttcttccccaaagctgccgagtttggcgtgcaaaatctgtatacaatataaagtcatgccggtcgtacagtccatgcaacctccaggtgtaggaaacttaaaaaaatatattcatatatatttatatctatatatttatatatgtatcaatgcccataaaacacgtgggcccaaagtctacaaaaagaagaatggaatgagcacgtggctgtgaccagtaaagaaggaatgttctgatcaaaaagaaaaacaacaaagtccattgctagtgctgcaaaaatcaaacttgcttttgtgtcagaccattacgaaatggtccttccccttgcaaacagattttcaaaagaagtaaagaaaaactgaaacaccttgacaaagtggccctccagaaccagagccctgggacgctggggaggggcggccagtcccagcgggccacggcctccgggacagccgcctgctggtggggcgtgggcacgtgggcacgctgcggcacggcgggaagccgcgagggcagggcagacgccaagaggcccagtggcgtcatcagggtttccctcaaagggatataaagtgctcgcttgctgactcccagccagtgcccccaaggcctttgcaaaggaagaaaaaggctaaaggtccaaggacccacagggagaacacatgaaggaaccctccctgacgtggtcccgcctgcagacgccgaggcagatcctctgccatctgccctggacgcttgctgtggagaagagccgagtgtgtcttcaaagaaaaggctacacagtaatgctctcagcacatttgtgaagctggagtgagctgacagatgaaacgtgcctccccctgccaggcctttgcagagggcgtctccatttgaatgagattagaattaagtccccccactgataacctggccactgagcagtccatgttatcccatcatctgcttaaaaaaaaaaagtgagatgatgcattcctccccataagccacggcggggtaagagggcaggtggcaggatccccagagggctatgcagagaatgaggccaaggaggccagaagagcctgctagctgggccctgccactgctctgtgccatgaatggggaatggaccagctcctcttgccaatctgggcttcagagcaaagagtggccaccagggaggggaaagtcaaacaagtcccaagaccgttctgcctgctctcaaaccactgtctcagagctgaccatcagcagcccagtgaccaagtgaatccaagaatctgcactcatttggtcaaaagtttgagttaatttcagaagctaccctgtaaactttaccaaactccgaaactcggctctgggtccctcctgagcacggtgtgtctgaacttctgcccccaagtctgaacccaatatacactttggaatgaaactggtggcttcatgtgctggaaaataagttaccagtaaaacgtgactgtcagttactgttgaagagaaaaagagtaaagactggctgtcctggtcaggcaatcataccctccctgcaggttcaccaggcaacaagggtccctgggttccttgcagccacaggctccaaaatccagggctggccacgtggctgcagtggaaaaacccaagtgggtaaagagccccacgtgtgccccatgcattgctgacatgctcaaaaggtctttggaaaactcaagttagaattctatcctgacgatgtggtcagagaagtttaaacatgagtttcattaatgctgactgcccccggcatctggcaagcctcccagggtggccgggcatcctaagcaaccctccctgcccttgccacggaggggaaaaacacaccacccctcgtaatactactagtgttgaaagttaaaaagagcccctgggcttctttatacagctcctaggacagaccaggaaagacacaatcgttggtgtcactccgaaaagacctacggtccctcctctcactttctgaaaatagaatctgacagcaacaattctgtacgctgcagaaaactcatcgtacaaaaataaaaacaaaaataattaaaaacctttgaaaggtaaaaaaaaatgtacaagcaagaattcagaaaggaaaaagatttagacattattaccattcagaaaattgctaaatggtgaggaaaaatgtaaaattcataaaacaatgcttattcaggatctttttgtgaaaaaattcatacaaaaatcaacagcaaatttatattctttgctataaaaactcattaggtacatatgtgcatgaaggcttggagacgggagcggttctgttagaaaataattaaaatgaaagtacaaacttgtagggtagttgcccagtggcgaatgtgttggcgatctgaaatctagccaatctggagcttgagaaaacatgaatttcaatcaatcaggatccctttccataagcaccttgagagcaaattcacaagccatccatttgcagggaccttcgcaatctgcattcattttatatatatatatatactttttctataaatgcattataaatattttatcaagatttcataagaatcaagtaagtttcttagcttggaatacattggaatatatattatacatatatatatttatttatacctaaaatttaagcaatacttcatgctacttgcttttaataaaaagcattccgatcgtaacactgcaagtgtgcctaccacatgcttcacgaccagatggagatgctcaatcgtatgtgacgtgtgagaacactttggattcgtttaaaatttgttggacttcaaaacctccaacgggatttgccacttttttggaactacctccatttttcttaaacagcaataaagcaaaacagggaccgccgggctgcagcccctggccccggagatgacggctggtgcccgtgcttgaggcgtcaggccagctcgcggtgccagcactgccaggctcggctggccacaggaaactgtcccaccgattcctgctgtttgttttttcttaaggcattgttcctcagacttcagaaaacccagccacaaaaatccaccagagcaataaaaaaaaaggcacaaactcgcatcttccgatggcttttgagaaactcaagccagctcccccagctcacattcctgtttctgtccagttttgttttctttaaaggtccctctgtcccccacccgggtgcagaccccccgccgcacaccgctatggttcacagaggcgggccacagccgtagaaaacgtcctctttaaaaaaaaataagctacaagatgagtcgagtggtttacacagagactgtggagttgtgggtaataaactttaagcaccagttttaatcaagtttgttttgtattattagatctttgatatttgttttctgtgcctcgtgtcaactgaattcggcagctcggccgcctgttgccacaggctcctttcttccacggcgtcccttgcgggacccgccagagtgtgcttggcttccgcgtgtccgtgtgtctgcgcgtcgccggcgtctgtcccgtgttccctgtgaggctgccacgcccaggcgtgcatgtgcgtctcgagacctgtgggcctgggcggcagaaaggcttcccgtggctgttgcacgctgggtgtccctgggtgctccaagagagccccacggtgggacgcaggcgtgacacgggaaagtttcttggctgagcttcaagacagagacagacagacaagagaacagcagcttcgagggagtgctacaggggcggctcctcttccatgggctcctcatctggtctcttttcggcgggcttcacgcccacggacagcgaggccatggcggtgaccgtctcggcttcttcgttctcgcaagtctgagcctcgatcagagaacgccccgctgtggaggttgtgcgctgcaggcagcgccagtacttgctgtggatctccatgactttctccatggaacggacagcgtttgcattgggtctttgctgtaaaaccttttctgggagaggatcaagctcgtttcccagcaaggcagaaacacatgcttccgaggcgtcgcaaatggcggtcaggtcgtggcctccctcgagggccaggacaatccggccgccagccaggcccatcagctgcttcgtcaggtacccgaagcatctggcggagaggttgtagcccccaagaggggtggggtggccctccacggcatcgaagcctgatgacaccagcaccacatccggggcaaactcgctggcgatcggcatgaccaccgttctgaaggccgccaagtactcagcgtctcccatgggggggtccaggccgccggtgaaagccatgttgacgttgaaacccacgccgggccctgtgcccacctcatcaggagccccgctgcctgggaagaagttcccatcgtcgtagcggtggagggacatgtacaggacgctggggtcgctgtagaaagcctgctgggtcccgtttccatggtgcacgtcccagtccacgatgaggatcttgctcacgctcaacctctgctgcagaagcttggctgccacggccacggagttgaagtagcaaaagcccatgggcgtgctctcctccgcatggtgtccaggggggcggaccacagcaaagccattcttcagctcccctgtggccaccttgaagaccagctctaccacgcagcccacagccaggcgggctgcccccgccgagtgcacctcgttccatatggtgtcactgtccaccccaacaccaccgcaagggagccggacgaacacggaggcgagcgagcctagaagtttcttactgtccagtttctgccggttgagggggttcgtgccatacaggagggtgtgggcttccgagtgcaccgtctgtagctcctccagggtggccttgcgtccgcggatgcactcgcatttgccccggaggcccgtctcctgcaggcgggaccagatgctctggatcctcccggcgtgctcggggtggctgctgctactcccgcaggtgcactggtgcttcagcatcagcgtgtcatacacgaggcctgtcgtgaacctcggcttggtggggggctcctgcacagacacggggaaggtggcagacgcgggtgaggactgcgcccgggacagaggcctgtggccgccgaaggacacggggatgccggcggcctccatggacgcctggtagttcctcagctggtggatccgctgctgctccagcaggagggcttgctgtctgaagagcagctcctgctcactgggctggcgctggcccggctccacctcccgtgggggctctgcctcttcctcatcgctctcaatgggctcctgcttcacctgcacgccggcctgtgcgtgcgcctccttctgccccggcagccggtccaggtagggctcgtccagcagagcctggtgctcacggagctcctcctccgtctcctccgggtggctctccggctgccgggctggctcgcttggcttggggatgatcttgttcatctgcagttgctgctgctggaactgctgcttgtgtttctccagaaactgctgatgctgctgctggatgaccaggtgctgcagagcctgggcgttctggggcagcggggccgactgggtccgccccagtgggcggtgctgccgcagcttgtggatggagggggacacccggtctgcaccaaccaaggactgtgcgtggaggggcagtgctcccaggcctgaaagataccagtctgtgacgaggggtgcttgtgccggcggctgctccagtaagaccatgtgctgcagaagagggctgtgcgctgcccctccgtcccgctccaagggcgaggtgctcaggtagggagtgaggtgggtgccggggaaaagggagagcctctgctggagggcgggaagggtgagtctctcggcgtcctgctggcccgccgtgcccgcagaggggccggtggcaggcaggcccagcgtgatgttgggcaaggatggcgatgtgtagaggggaagtggagcggccgagccttctcgtgccacaagtctgtgcgccaaactcgtctccgccgggatgctggggacggcgggcgcgataccgttctccgcgctgacgctcccggagctgttgttgggtgagctgggtccggagcctggggcgctgctgcacgcggagtctgtgacatccaacggacgcttttttagagcagtgaccactggcccgtctttcctgcgtaacagggggctgctccgtctttcggccactttctgctttagcctggaccgtaatttcagattcggttcagaagctgttttcctaagagggaagtcatctttggcgtcgtacattcccaggaccgggtggttataggaggtcgacactccgctctggggtggagaactctggtcaagggaactgtgctgcgttttcccgtaccagtagcgagggtcgctggaaatgcagtggttcagattccggtgggccagcgccttctttttattgaggacaaattcttgtaacttcatcttcacttctgtgctggccacggcactctctttgcccttctccttgttcttgagctgctgcagcttctgctcccggtgctgcttctccagctcctgctcctggcggtgcctctccagcttccgctggtgttccagcagctcctgctggtgcttcatggccagcatctcctgttgttgcttgatgtgctcgtggagctgcgcctcgtgctgccgggagagctgctcgtgctgcctctggaactcagcgatgaggatctgcctctggatctgctgcttctgcttgagcgccaggagctcctgctgcagctgctgctcccgcagggccggctctgccacaggcagtgagaactggtggtccaggcgcaggtccatgggcactgccgagggggccacttgcagaggcagcgccgtggccacatccaccgtgctgggcatgtggttcacgcgggcaggattcagcagctccactggctggtctcggccagaaagtccatcttcagcccagactttcgcttaatcccggaaactgctccaaaggcgtttttctcagggcgttcggcgccgtaactcaggagaaacccaagtcctgctctcccggcggcctcgctggggaagaattcagccgctccaccctgacatctggtttctatttcatatccatgttgtcacattacataacaagcagatgatacgagagatcaccacagtgtttcggctcgagagtcacaaagaacgcccagaacactgtttatattgggggccatgaacgttcaccaaaccagacttagtgcagaggctgcacccttccaggctgaaacccagcacctacagcaaatgcccaaggaagcaagaagcgggaccccgccttctcagccacctctcactaacactcagctccactcctgcttccttcctctcactccacatccgagttagagggaaatacgatttatctctggcctgcatttacttctcctgcacctggcgggaggctctggccttgcaggcgtgcaggagcccctgccagtgagggccagcgaggggcccagggagaagatggaggtcaagtcatagggcctccaccgcaggcagagctccgccagcaagtatcctgggagctggggggcctcaagggaggcaatccccccacacaccatccccttccccttcgctcatctggggaagctgtgaggactggtgttgataaaacattccaaccacacactcagaccatggatgtggccgtgccagcagggaggccagcagcccctagcagaagggtgttctggaagctgccccctcccatgctgctgcctggtcccatggggcatgaagggagggtggccagggtggcccgagccagcatcaggcacaaggcccaaggagtttctccagagcagcctgtcctcttcggtccagaaaaagtcagattccacagcagggttagccgtccagttagggaacccactaaggggctctgtgcgtagaggtgctcagaatcaaaccactaaaccccaggaccccctgctgggggaatggtccgtggcagtcattcagccttggagtgaaccgttctgcccaagtgcaagtgagaacacaatacttcttattatatacagaattgccaaagccaacgtgattagtagaaaaaccgacatgtcagtgacttgggggtctggtttgccccagatgtgggtggaaaccccaggcgtccctcaagcctggtccagagctccacagacagcagatacacaaactctgagtgacagcattggtgtttagcagattctggattttgctcccccccgaaccaagtatagagaatgtttcacagagtagcttcaacagaaaatggccacagtgtgtctgtgagagagtgtgatgttcccggggggatggctggggccaagggaaggcccctcccatgagccctgcctccatgagactgcgtagggcaggactgccaggcagaaagaacacagcacaggcacaagggcagacccaggctggcagggctaaatggcttcaggagctcccccctctgccccccagggagtaaaggcaatgatgcaaatatgataagcaaacagaggtcccaaaacacagaaagggccaggaccctgatgccaaccaagcagacccaaaactgggtctgggagcacagggcagggtcgctgagtgcagaggggcctcactcaatgtccaacacttccctccaaaacagacatgctggtgagaggcttcaacccttccactggcctgacacctggatctctgctgccctgtgccaggttagccacgtccaacaccaccacggccaccggccatttaagaaaacgaaccctgacgttaacctgcttgagccctaatactaagcaagagcagcgccacaattccaaaactgcagagagcgccttttaaacattctgctgagatctgcgcggtcgcggtctgacaggcaggccttcttggctacctgtggtttcattccagcattaacaggcacctaaaaggcctgtgagcttttgtggggtcaagcagcatcagctccactttacaaccccgcagagtgaggtgttagctctgcagctccagggcagagccttgcagccttagggccagggggacggcctggccccttccgagctctcagcagcctgaactccacgtgtcccctgctgtgtcactggcatgctggtcttgcatggcactgagatgtgtggcacaagcaggcaccaagcccggagacacccgacgctcaccgttagactgggtagcatttgtcaagcgccgagcaaacagtggatgaagtgtcctcagccggcgtcagctgttctgatccgcagaacacataactcctggcactcctttccaagcatccgggaaatgtagaatccaagtgttacaccatccagttgaagatgacagatttacgatataaaacggcacccgcgactgaggactttgtaggaatggaggccgctgtcattatttcatgggtgagggggagagggacactgtgacccatgacaggaaaggacagctcagcccctccaaaaccacacacaggggactccgtttctcacaaaacttcaagtttctgttctacgcaaacattacaacacattttaaactacattctgacacgaagctcccgtgctttttaatggcaggtgttacaatgatcatggaacagtgatggggcggtgcttcctcacggtgacatggcagggagaagtctggaccggagccagcagggtccttgacctaagaggccttgggcagcccacggggcagctctgagcaatctcctgtgaaaggaagagctcagaacgggttcctctaaaggttccttccagagcaggggttctgtggttccctggggccctagactaacatgaggaaggggaaacagagaagaatgcccactaaaagccttacccaaaaattgaaagccaagaaaaatcacaccagatcatctcagtttagacttgaggaacctcggcgctgacatcactgtcaccatcacaaaacactggccaccaaggtgccacctaccacactgcaacctggaaggaggggcgggcaggggcacccctgggcagggcaggacaccaggccagccagccacccacgctacagaggaaatgcagcccctcccaactaagagaaccctggtaccatcaccacagccttggtgccagggctcctagcacctgacagggaagatgagaaggacattggctgccgccaagaggcctgctgcccacccccaactgcacggtggtggtgctgccagcaccaccatccatgctggcccaggagcccacacgcagggcacgcacgcacgtagttccacattaggccctttcttcctcaattgttggaaagaaggccaaagccagatgatggtgaaattcacgaggaaaatgtccccgactgtcctccattctaaagcaaacgctaagaatgggctgctgggcttcagcagaagccaagtcacctttcctctatgcgtccaatgaaacgaaaacatccacacttgtctttataaaaacggaaaactgcatctggaacaaggtctgtggcgtttcttccagcgtgtcccatggacatgaagttggtcttcctatgggtcctccaaggcacacccctcgactgcaccacagcactgagggcagaatgtggtggtggcccagctgccgtggcgccggcagactagcctggtacacggagaggggagcctgctgactgtgggtaggccacgttcccccagtgtcttcatctgcagagggagaccgggagcctctgaagaccgctccagctctgcactgtgggggcggccggccagcaggcaggcaatgctctcaggccccacgctcctctcactggctgccgacgggaggcagacgaggtgccgggggcagcctgcagagcaaggagtcaaggtggccagcctggggcagggtgttcccccagccagggagcttcactcaggcttgggctctgtcccgtgcctccccgggggcgttccgaggtggcggaggaggaagctgcagcccgttatccaccgcccagtctctccctctcaccagcacacagatgttctcagcggcagagcctggcttctgcctgaattcatttcatatttttaaatatgctcttaatggaaagcaacaaaagtacttaacaaaatgcgctgatgtaaatgtccctgcagcagccagggactaattttagaaggggctttgaggagaaacccaagggacactcacttgctggaaacggcctcctccccaaagagtgtgaggatctggattagaaccaagtatccccaggctgcccaggagcccgctcctccaattgggggctggccatcccaccgagcactgataccgcaggctggactcttcctaacctcacgagaggtgatgaccggaatcatcccagttttccatggcacttcgcaaacacagctggtcaggcccttagcacctcctgaccccccgatctcccagactctctgctggaagttaaggacacagagaaagtttcttatgaaaataagcgcctcaaaagaaagccaacgtacagcactggtgacagaaaggaagattcagaaaagccttcacgcctggcaatatggcacacgcacttttagagacgtctaattatactcagggctgagttggctgaagagtgaggaatatactccaaagacaggaattcaaggcagggcaaatagaacatgaaagccagcctggagcccagggcctgtcctggggcagccacctgcactgcctcttaccactgcaccgtccctgtgagtgtgcgtggggaggggctgtagttcccttggcaggggaagccagaagacaggcctgcaagggacacatccgggcctgggcttggtgctggctagaaggggtcaaatcgagagaggactcccctcagaactcataatcccagacccctcgcaatggtttggggagaattcagacaacccatgaggcctgatgagcatccctagcacctgcaaacacaggcatgtcccaggtggcacctcccagcaccaggcagaaaccttctctagaggaacacgctatgaacctcaaaaaaacatccaagaaggacggacataaagtcacaatcaagaaccatgggtagcgggagtaagtcccggaaagacctcagttgtaggaaaatcaggcactgacccaaaacacatacgaaggacactcgacaaaacaagagaggtcatccagggtcaggctggagctagaggcctccagatcctgtcacttagtgactgtacaaacctggtggcttcctcaacctccctgtgccttagcttcccatttgccaaaaagggggattagaagagcccacactctccctggagcaaggctaaggaagaaaggagacagatgtctcagctgttattattaataactatcagaagtgtcacatggatctgaatgatccaaatggaacttgtagaaacaaaactgtcatcattaaaatttaaaactaaatgagtgagttaactaatcaagtattaatagacagagctgaagagagaattagtgaacagtaaaatagcacggaagaaataaaccaggatgcaacacataaaggtaaagagatagaaagctggagacgttagaggactggaaggacagaggaagatatgctaacacacatctgtaaaccaaaaataaaattctaagctcccaaccatctgaatggacccctcctctcaagccaagggcattccaacattaacctgaaaagctagttcaggtcgtgatggggacgggcattcagatgtgcctcatgataccctcctcccttttggaattgctgatagaacagactctttaagtctgatgagaaacatttcagtctattctctctgaagcctgctacccggaggcttcgtcggcatggtaaatccttggtctccacaaacccttatcataatccagacattcctttgtgttgataataactctttcaaccaactgccaatcagaacattttaaaatctacctataatctgaaagcctcacacttcgagttgtcccgcgtttctggactggaccaatgttcatcttccacatactgacagacgcctcatgtctccctaaaaatgtatgaaaccaagctgttccccgaccaccttgggcacatgttgtcagcacct

SEQ ID NO: 10212 - RNA, 13523 nt, Homo sapiens
  source 1..13523: mol_type = other RNA
caggaaggagacaggcagttcactgtgaattctgagtagtttccctaaaacactgtttccacataaatacaataaactctattattggtatgtcacaagtgctagataaactttttttcttaatatgacaaatgtttaagtagtcctttttatttttcttacaataaaaagtacaatttcttaagaataagttcaataagacgcaaacttccccgccctcctctccttcaaggttttgttttacagaaaaatttccatcttttgtatctgcaaatgtcatgagaggggaacagaaaggcatttttcttcttccccaaagctgccgagtttggcgtgcaaaatctgtatacaatataaagtcatgccggtcgtacagtccatgcaacctccaggtgtaggaaacttaaaaaaatatattcatatatatttatatctatatatttatatatgtatcaatgcccataaaacacgtgggcccaaagtctacaaaaagaagaatggaatgagcacgtggctgtgaccagtaaagaaggaatgttctgatcaaaaagaaaaacaacaaagtccattgctagtgctgcaaaaatcaaacttgcttttgtgtcagaccattacgaaatggtccttccccttgcaaacagattttcaaaagaagtaaagaaaaactgaaacaccttgacaaagtggccctccagaaccagagccctgggacgctggggaggggcggccagtcccagcgggccacggcctccgggacagccgcctgctggtggggcgtgggcacgtgggcacgctgcggcacggcgggaagccgcgagggcagggcagacgccaagaggcccagtggcgtcatcagggtttccctcaaagggatataaagtgctcgcttgctgactcccagccagtgcccccaaggcctttgcaaaggaagaaaaaggctaaaggtccaaggacccacagggagaacacatgaaggaaccctccctgacgtggtcccgcctgcagacgccgaggcagatcctctgccatctgccctggacgcttgctgtggagaagagccgagtgtgtcttcaaagaaaaggctacacagtaatgctctcagcacatttgtgaagctggagtgagctgacagatgaaacgtgcctccccctgccaggcctttgcagagggcgtctccatttgaatgagattagaattaagtccccccactgataacctggccactgagcagtccatgttatcccatcatctgcttaaaaaaaaaaagtgagatgatgcattcctccccataagccacggcggggtaagagggcaggtggcaggatccccagagggctatgcagagaatgaggccaaggaggccagaagagcctgctagctgggccctgccactgctctgtgccatgaatggggaatggaccagctcctcttgccaatctgggcttcagagcaaagagtggccaccagggaggggaaagtcaaacaagtcccaagaccgttctgcctgctctcaaaccactgtctcagagctgaccatcagcagcccagtgaccaagtgaatccaagaatctgcactcatttggtcaaaagtttgagttaatttcagaagctaccctgtaaactttaccaaactccgaaactcggctctgggtccctcctgagcacggtgtgtctgaacttctgcccccaagtctgaacccaatatacactttggaatgaaactggtggcttcatgtgctggaaaataagttaccagtaaaacgtgactgtcagttactgttgaagagaaaaagagtaaagactggctgtcctggtcaggcaatcataccctccctgcaggttcaccaggcaacaagggtccctgggttccttgcagccacaggctccaaaatccagggctggccacgtggctgcagtggaaaaacccaagtgggtaaagagccccacgtgtgccccatgcattgctgacatgctcaaaaggtctttggaaaactcaagttagaattctatcctgacgatgtggtcagagaagtttaaacatgagtttcattaatgctgactgcccccggcatctggcaagcctcccagggtggccgggcatcctaagcaaccctccctgcccttgccacggaggggaaaaacacaccacccctcgtaatactactagtgttgaaagttaaaaagagcccctgggcttctttatacagctcctaggacagaccaggaaagacacaatcgttggtgtcactccgaaaagacctacggtccctcctctcactttctgaaaatagaatctgacagcaacaattctgtacgctgcagaaaactcatcgtacaaaaataaaaacaaaaataattaaaaacctttgaaaggtaaaaaaaaatgtacaagcaagaattcagaaaggaaaaagatttagacattattaccattcagaaaattgctaaatggtgaggaaaaatgtaaaattcataaaacaatgcttattcaggatctttttgtgaaaaaattcatacaaaaatcaacagcaaatttatattctttgctataaaaactcattaggtacatatgtgcatgaaggcttggagacgggagcggttctgttagaaaataattaaaatgaaagtacaaacttgtagggtagttgcccagtggcgaatgtgttggcgatctgaaatctagccaatctggagcttgagaaaacatgaatttcaatcaatcaggatccctttccataagcaccttgagagcaaattcacaagccatccatttgcagggaccttcgcaatctgcattcattttatatatatatatatactttttctataaatgcattataaatattttatcaagatttcataagaatcaagtaagtttcttagcttggaatacattggaatatatattatacatatatatatttatttatacctaaaatttaagcaatacttcatgctacttgcttttaataaaaagcattccgatcgtaacactgcaagtgtgcctaccacatgcttcacgaccagatggagatgctcaatcgtatgtgacgtgtgagaacactttggattcgtttaaaatttgttggacttcaaaacctccaacgggatttgccacttttttggaactacctccatttttcttaaacagcaataaagcaaaacagggaccgccgggctgcagcccctggccccggagatgacggctggtgcccgtgcttgaggcgtcaggccagctcgcggtgccagcactgccaggctcggctggccacaggaaactgtcccaccgattcctgctgtttgttttttcttaaggcattgttcctcagacttcagaaaacccagccacaaaaatccaccagagcaataaaaaaaaaggcacaaactcgcatcttccgatggcttttgagaaactcaagccagctcccccagctcacattcctgtttctgtccagttttgttttctttaaaggtccctctgtcccccacccgggtgcagaccccccgccgcacaccgctatggttcacagaggcgggccacagccgtagaaaacgtcctctttaaaaaaaaataagctacaagatgagtcgagtggtttacacagagactgtggagttgtgggtaataaactttaagcaccagttttaatcaagtttgttttgtattattagatctttgatatttgttttctgtgcctcgtgtcaactgaattcggcagctcggccgcctgttgccacaggctcctttcttccacggcgtcccttgcgggacccgccagagtgtgcttggcttccgcgtgtccgtgtgtctgcgcgtcgccggcgtctgtcccgtgttccctgtgaggctgccacgcccaggcgtgcatgtgcgtctcgagacctgtgggcctgggcggcagaaaggcttcccgtggctgttgcacgctgggtgtccctgggtgctccaagagagccccacggtgggacgcaggcgtgacacgggaaagtttcttggctgagcttcaagacagagacagacagacaagagaacagcagcttcgagggagtgctacaggggcggctcctcttccatgggctcctcatctggtctcttttcggcgggcttcacgcccacggacagcgaggccatggcggtgaccgtctcggcttcttcgttctcgcaagtctgagcctcgatcagagaacgccccgctgtggaggttgtgcgctgcaggcagcgccagtacttgctgtggatctccatgactttctccatggaacggacagcgtttgcattgggtctttgctgtaaaaccttttctgggagaggatcaagctcgtttcccagcaaggcagaaacacatgcttccgaggcgtcgcaaatggcggtcaggtcgtggcctccctcgagggccaggacaatccggccgccagccaggcccatcagctgcttcgtcaggtacccgaagcatctggcggagaggttgtagcccccaagaggggtggggtggccctccacggcatcgaagcctgatgacaccagcaccacatccggggcaaactcgctggcgatcggcatgaccaccgttctgaaggccgccaagtactcagcgtctcccatgggggggtccaggccgccggtgaaagccatgttgacgttgaaacccacgccgggccctgtgcccacctcatcaggagccccgctgcctgggaagaagttcccatcgtcgtagcggtggagggacatgtacaggacgctggggtcgctgtagaaagcctgctgggtcccgtttccatggtgcacgtcccagtccacgatgaggatcttgctcacgctcaacctctgctgcagaagcttggctgccacggccacggagttgaagtagcaaaagcccatgggcgtgctctcctccgcatggtgtccaggggggcggaccacagcaaagccattcttcagctcccctgtggccaccttgaagaccagctctaccacgcagcccacagccaggcgggctgcccccgccgagtgcacctcgttccatatggtgtcactgtccaccccaacaccaccgcaagggagccggacgaacacggaggcgagcgagcctagaagtttcttactgtccagtttctgccggttgagggggttcgtgccatacaggagggtgtgggcttccgagtgcaccgtctgtagctcctccagggtggccttgcgtccgcggatgcactcgcatttgccccggaggcccgtctcctgcaggcgggaccagatgctctggatcctcccggcgtgctcggggtggctgctgctactcccgcaggtgcactggtgcttcagcatcagcgtgtcatacacgaggcctgtcgtgaacctcggcttggtggggggctcctgcacagacacggggaaggtggcagacgcgggtgaggactgcgcccgggacagaggcctgtggccgccgaaggacacggggatgccggcggcctccatggacgcctggtagttcctcagctggtggatccgctgctgctccagcaggagggcttgctgtctgaagagcagctcctgctcactgggctggcgctggcccggctccacctcccgtgggggctctgcctcttcctcatcgctctcaatgggctcctgcttcacctgcacgccggcctgtgcgtgcgcctccttctgccccggcagccggtccaggtagggctcgtccagcagagcctggtgctcacggagctcctcctccgtctcctccgggtggctctccggctgccgggctggctcgcttggcttggggatgatcttgttcatctgcagttgctgctgctggaactgctgcttgtgtttctccagaaactgctgatgctgctgctggatgaccaggtgctgcagagcctgggcgttctggggcagcggggccgactgggtccgccccagtgggcggtgctgccgcagcttgtggatggagggggacacccggtctgcaccaaccaaggactgtgcgtggaggggcagtgctcccaggcctgaaagataccagtctgtgacgaggggtgcttgtgccggcggctgctccagtaagaccatgtgctgcagaagagggctgtgcgctgcccctccgtcccgctccaagggcgaggtgctcaggtagggagtgaggtgggtgccggggaaaagggagagcctctgctggagggcgggaagggtgagtctctcggcgtcctgctggcccgccgtgcccgcagaggggccggtggcaggcaggcccagcgtgatgttgggcaaggatggcgatgtgtagaggggaagtggagcggccgagccttctcgtgccacaagtctgtgcgccaaactcgtctccgccgggatgctggggacggcgggcgcgataccgttctccgcgctgacgctcccggagctgttgttgggtgagctgggtccggagcctggggcgctgctgcacgcggagtctgtgacatccaacggacgcttttttagagcagtgaccactggcccgtctttcctgcgtaacagggggctgctccgtctttcggccactttctgctttagcctggaccgtaatttcagattcggttcagaagctgttttcctaagagggaagtcatctttggcgtcgtacattcccaggaccgggtggttataggaggtcgacactccgctctggggtggagaactctggtcaagggaactgtgctgcgttttcccgtaccagtagcgagggtcgctggaaatgcagtggttcagattccggtgggccagcgccttctttttattgaggacaaattcttgtaacttcatcttcacttctgtgctggccacggcactctctttgcccttctccttgttcttgagctgctgcagcttctgctcccggtgctgcttctccagctcctgctcctggcggtgcctctccagcttccgctggtgttccagcagctcctgctggtgcttcatggccagcatctcctgttgttgcttgatgtgctcgtggagctgcgcctcgtgctgccgggagagctgctcgtgctgcctctggaactcagcgatgaggatctgcctctggatctgctgcttctgcttgagcgccaggagctcctgctgcagctgctgctcccgcagggccggctctgccacaggcagtgagaactggtggtccaggcgcaggtccatgggcactgccgagggggccacttgcagaggcagcgccgtggccacatccaccgtgctgggcatgtggttcacgcgggcaggattcagcagctccactggctggtctcggccagaaagtccatttggtgctttaccttcagcccagactttcgcttaatcccggaaactgctccaaaggcgtttttctcagggcgttcggcgccgtaactcaggagaaacccaagtcctgctctcccggcggcctcgctggggaagaattcagccgctccaccctgacatctggtttctatttcatatccatgttgtcacattacataacaagcagatgatacgagagatcaccacagtgtttcggctcgagagtcacaaagaacgcccagaacactgtttatattgggggccatgaacgttcaccaaaccagacttagtgcagaggctgcacccttccaggctgaaacccagcacctacagcaaatgcccaaggaagcaagaagcgggaccccgccttctcagccacctctcactaacactcagctccactcctgcttccttcctctcactccacatccgagttagagggaaatacgatttatctctggcctgcatttacttctcctgcacctggcgggaggctctggccttgcaggcgtgcaggagcccctgccagtgagggccagcgaggggcccagggagaagatggaggtcaagtcatagggcctccaccgcaggcagagctccgccagcaagtatcctgggagctggggggcctcaagggaggcaatccccccacacaccatccccttccccttcgctcatctggggaagctgtgaggactggtgttgataaaacattccaaccacacactcagaccatggatgtggccgtgccagcagggaggccagcagcccctagcagaagggtgttctggaagctgccccctcccatgctgctgcctggtcccatggggcatgaagggagggtggccagggtggcccgagccagcatcaggcacaaggcccaaggagtttctccagagcagcctgtcctcttcggtccagaaaaagtcagattccacagcagggttagccgtccagttagggaacccactaaggggctctgtgcgtagaggtgctcagaatcaaaccactaaaccccaggaccccctgctgggggaatggtccgtggcagtcattcagccttggagtgaaccgttctgcccaagtgcaagtgagaacacaatacttcttattatatacagaattgccaaagccaacgtgattagtagaaaaaccgacatgtcagtgacttgggggtctggtttgccccagatgtgggtggaaaccccaggcgtccctcaagcctggtccagagctccacagacagcagatacacaaactctgagtgacagcattggtgtttagcagattctggattttgctcccccccgaaccaagtatagagaatgtttcacagagtagcttcaacagaaaatggccacagtgtgtctgtgagagagtgtgatgttcccggggggatggctggggccaagggaaggcccctcccatgagccctgcctccatgagactgcgtagggcaggactgccaggcagaaagaacacagcacaggcacaagggcagacccaggctggcagggctaaatggcttcaggagctcccccctctgccccccagggagtaaaggcaatgatgcaaatatgataagcaaacagaggtcccaaaacacagaaagggccaggaccctgatgccaaccaagcagacccaaaactgggtctgggagcacagggcagggtcgctgagtgcagaggggcctcactcaatgtccaacacttccctccaaaacagacatgctggtgagaggcttcaacccttccactggcctgacacctggatctctgctgccctgtgccaggttagccacgtccaacaccaccacggccaccggccatttaagaaaacgaaccctgacgttaacctgcttgagccctaatactaagcaagagcagcgccacaattccaaaactgcagagagcgccttttaaacattctgctgagatctgcgcggtcgcggtctgacaggcaggccttcttggctacctgtggtttcattccagcattaacaggcacctaaaaggcctgtgagcttttgtggggtcaagcagcatcagctccactttacaaccccgcagagtgaggtgttagctctgcagctccagggcagagccttgcagccttagggccagggggacggcctggccccttccgagctctcagcagcctgaactccacgtgtcccctgctgtgtcactggcatgctggtcttgcatggcactgagatgtgtggcacaagcaggcaccaagcccggagacacccgacgctcaccgttagactgggtagcatttgtcaagcgccgagcaaacagtggatgaagtgtcctcagccggcgtcagctgttctgatccgcagaacacataactcctggcactcctttccaagcatccgggaaatgtagaatccaagtgttacaccatccagttgaagatgacagatttacgatataaaacggcacccgcgactgaggactttgtaggaatggaggccgctgtcattatttcatgggtgagggggagagggacactgtgacccatgacaggaaaggacagctcagcccctccaaaaccacacacaggggactccgtttctcacaaaacttcaagtttctgttctacgcaaacattacaacacattttaaactacattctgacacgaagctcccgtgctttttaatggcaggtgttacaatgatcatggaacagtgatggggcggtgcttcctcacggtgacatggcagggagaagtctggaccggagccagcagggtccttgacctaagaggccttgggcagcccacggggcagctctgagcaatctcctgtgaaaggaagagctcagaacgggttcctctaaaggttccttccagagcaggggttctgtggttccctggggccctagactaacatgaggaaggggaaacagagaagaatgcccactaaaagccttacccaaaaattgaaagccaagaaaaatcacaccagatcatctcagtttagacttgaggaacctcggcgctgacatcactgtcaccatcacaaaacactggccaccaaggtgccacctaccacactgcaacctggaaggaggggcgggcaggggcacccctgggcagggcaggacaccaggccagccagccacccacgctacagaggaaatgcagcccctcccaactaagagaaccctggtaccatcaccacagccttggtgccagggctcctagcacctgacagggaagatgagaaggacattggctgccgccaagaggcctgctgcccacccccaactgcacggtggtggtgctgccagcaccaccatccatgctggcccaggagcccacacgcagggcacgcacgcacgtagttccacattaggccctttcttcctcaattgttggaaagaaggccaaagccagatgatggtgaaattcacgaggaaaatgtccccgactgtcctccattctaaagcaaacgctaagaatgggctgctgggcttcagcagaagccaagtcacctttcctctatgcgtccaatgaaacgaaaacatccacacttgtctttataaaaacggaaaactgcatctggaacaaggtctgtggcgtttcttccagcgtgtcccatggacatgaagttggtcttcctatgggtcctccaaggcacacccctcgactgcaccacagcactgagggcagaatgtggtggtggcccagctgccgtggcgccggcagactagcctggtacacggagaggggagcctgctgactgtgggtaggccacgttcccccagtgtcttcatctgcagagggagaccgggagcctctgaagaccgctccagctctgcactgtgggggcggccggccagcaggcaggcaatgctctcaggccccacgctcctctcactggctgccgacgggaggcagacgaggtgccgggggcagcctgcagagcaaggagtcaaggtggccagcctggggcagggtgttcccccagccagggagcttcactcaggcttgggctctgtcccgtgcctccccgggggcgttccgaggtggcggaggaggaagctgcagcccgttatccaccgcccagtctctccctctcaccagcacacagatgttctcagcggcagagcctggcttctgcctgaattcatttcatatttttaaatatgctcttaatggaaagcaacaaaagtacttaacaaaatgcgctgatgtaaatgtccctgcagcagccagggactaattttagaaggggctttgaggagaaacccaagggacactcacttgctggaaacggcctcctccccaaagagtgtgaggatctggattagaaccaagtatccccaggctgcccaggagcccgctcctccaattgggggctggccatcccaccgagcactgataccgcaggctggactcttcctaacctcacgagaggtgatgaccggaatcatcccagttttccatggcacttcgcaaacacagctggtcaggcccttagcacctcctgaccccccgatctcccagactctctgctggaagttaaggacacagagaaagtttcttatgaaaataagcgcctcaaaagaaagccaacgtacagcactggtgacagaaaggaagattcagaaaagccttcacgcctggcaatatggcacacgcacttttagagacgtctaattatactcagggctgagttggctgaagagtgaggaatatactccaaagacaggaattcaaggcagggcaaatagaacatgaaagccagcctggagcccagggcctgtcctggggcagccacctgcactgcctcttaccactgcaccgtccctgtgagtgtgcgtggggaggggctgtagttcccttggcaggggaagccagaagacaggcctgcaagggacacatccgggcctgggcttggtgctggctagaaggggtcaaatcgagagaggactcccctcagaactcataatcccagacccctcgcaatggtttggggagaattcagacaacccatgaggcctgatgagcatccctagcacctgcaaacacaggcatgtcccaggtggcacctcccagcaccaggcagaaaccttctctagaggaacacgctatgaacctcaaaaaaacatccaagaaggacggacataaagtcacaatcaagaaccatgggtagcgggagtaagtcccggaaagacctcagttgtaggaaaatcaggcactgacccaaaacacatacgaaggacactcgacaaaacaagagaggtcatccagggtcaggctggagctagaggcctccagatcctgtcacttagtgactgtacaaacctggtggcttcctcaacctccctgtgccttagcttcccatttgccaaaaagggggattagaagagcccacactctccctggagcaaggctaaggaagaaaggagacagatgtctcagctgttattattaataactatcagaagtgtcacatggatctgaatgatccaaatggaacttgtagaaacaaaactgtcatcattaaaatttaaaactaaatgagtgagttaactaatcaagtattaatagacagagctgaagagagaattagtgaacagtaaaatagcacggaagaaataaaccaggatgcaacacataaaggtaaagagatagaaagctggagacgttagaggactggaaggacagaggaagatatgctaacacacatctgtaaaccaaaaataaaattctaagctcccaaccatctgaatggacccctcctctcaagccaagggcattccaacattaacctgaaaagctagttcaggtcgtgatggggacgggcattcagatgtgcctcatgataccctcctcccttttggaattgctgatagaacagactctttaagtctgatgagaaacatttcagtctattctctctgaagcctgctacccggaggcttcgtcggcatggtaaatccttggtctccacaaacccttatcataatccagacattcctttgtgttgataataactctttcaaccaactgccaatcagaacattttaaaatctacctataatctgaaagcctcacacttcgagttgtcccgcgtttctggactggaccaatgttcatcttccacatactgacagacgcctcatgtctccctaaaaatgtatgaaaccaagctgttccccgaccaccttgggcacatgttgtcagcacct

SEQ ID NO: 10213 - RNA, 7546 nt, Homo sapiens
  source 1..7546: mol_type = other RNA
caggaaggagacaggcagttcactgtgaattctgagtagtttccctaaaacactgtttccacataaatacaataaactctattattggtatgtcacaagtgctagataaactttttttcttaatatgacaaatgtttaagtagtcctttttatttttcttacaataaaaagtacaatttcttaagaataagttcaataagacgcaaacttccccgccctcctctccttcaaggttttgttttacagaaaaatttccatcttttgtatctgcaaatgtcatgagaggggaacagaaaggcatttttcttcttccccaaagctgccgagtttggcgtgcaaaatctgtatacaatataaagtcatgccggtcgtacagtccatgcaacctccaggtgtaggaaacttaaaaaaatatattcatatatatttatatctatatatttatatatgtatcaatgcccataaaacacgtgggcccaaagtctacaaaaagaagaatggaatgagcacgtggctgtgaccagtaaagaaggaatgttctgatcaaaaagaaaaacaacaaagtccattgctagtgctgcaaaaatcaaacttgcttttgtgtcagaccattacgaaatggtccttccccttgcaaacagattttcaaaagaagtaaagaaaaactgaaacaccttgacaaagtggccctccagaaccagagccctgggacgctggggaggggcggccagtcccagcgggccacggcctccgggacagccgcctgctggtggggcgtgggcacgtgggcacgctgcggcacggcgggaagccgcgagggcagggcagacgccaagaggcccagtggcgtcatcagggtttccctcaaagggatataaagtgctcgcttgctgactcccagccagtgcccccaaggcctttgcaaaggaagaaaaaggctaaaggtccaaggacccacagggagaacacatgaaggaaccctccctgacgtggtcccgcctgcagacgccgaggcagatcctctgccatctgccctggacgcttgctgtggagaagagccgagtgtgtcttcaaagaaaaggctacacagtaatgctctcagcacatttgtgaagctggagtgagctgacagatgaaacgtgcctccccctgccaggcctttgcagagggcgtctccatttgaatgagattagaattaagtccccccactgataacctggccactgagcagtccatgttatcccatcatctgcttaaaaaaaaaaagtgagatgatgcattcctccccataagccacggcggggtaagagggcaggtggcaggatccccagagggctatgcagagaatgaggccaaggaggccagaagagcctgctagctgggccctgccactgctctgtgccatgaatggggaatggaccagctcctcttgccaatctgggcttcagagcaaagagtggccaccagggaggggaaagtcaaacaagtcccaagaccgttctgcctgctctcaaaccactgtctcagagctgaccatcagcagcccagtgaccaagtgaatccaagaatctgcactcatttggtcaaaagtttgagttaatttcagaagctaccctgtaaactttaccaaactccgaaactcggctctgggtccctcctgagcacggtgtgtctgaacttctgcccccaagtctgaacccaatatacactttggaatgaaactggtggcttcatgtgctggaaaataagttaccagtaaaacgtgactgtcagttactgttgaagagaaaaagagtaaagactggctgtcctggtcaggcaatcataccctccctgcaggttcaccaggcaacaagggtccctgggttccttgcagccacaggctccaaaatccagggctggccacgtggctgcagtggaaaaacccaagtgggtaaagagccccacgtgtgccccatgcattgctgacatgctcaaaaggtctttggaaaactcaagttagaattctatcctgacgatgtggtcagagaagtttaaacatgagtttcattaatgctgactgcccccggcatctggcaagcctcccagggtggccgggcatcctaagcaaccctccctgcccttgccacggaggggaaaaacacaccacccctcgtaatactactagtgttgaaagttaaaaagagcccctgggcttctttatacagctcctaggacagaccaggaaagacacaatcgttggtgtcactccgaaaagacctacggtccctcctctcactttctgaaaatagaatctgacagcaacaattctgtacgctgcagaaaactcatcgtacaaaaataaaaacaaaaataattaaaaacctttgaaaggtaaaaaaaaatgtacaagcaagaattcagaaaggaaaaagatttagacattattaccattcagaaaattgctaaatggtgaggaaaaatgtaaaattcataaaacaatgcttattcaggatctttttgtgaaaaaattcatacaaaaatcaacagcaaatttatattctttgctataaaaactcattaggtacatatgtgcatgaaggcttggagacgggagcggttctgttagaaaataattaaaatgaaagtacaaacttgtagggtagttgcccagtggcgaatgtgttggcgatctgaaatctagccaatctggagcttgagaaaacatgaatttcaatcaatcaggatccctttccataagcaccttgagagcaaattcacaagccatccatttgcagggaccttcgcaatctgcattcattttatatatatatatatactttttctataaatgcattataaatattttatcaagatttcataagaatcaagtaagtttcttagcttggaatacattggaatatatattatacatatatatatttatttatacctaaaatttaagcaatacttcatgctacttgcttttaataaaaagcattccgatcgtaacactgcaagtgtgcctaccacatgcttcacgaccagatggagatgctcaatcgtatgtgacgtgtgagaacactttggattcgtttaaaatttgttggacttcaaaacctccaacgggatttgccacttttttggaactacctccatttttcttaaacagcaataaagcaaaacagggaccgccgggctgcagcccctggccccggagatgacggctggtgcccgtgcttgaggcgtcaggccagctcgcggtgccagcactgccaggctcggctggccacaggaaactgtcccaccgattcctgctgtttgttttttcttaaggcattgttcctcagacttcagaaaacccagccacaaaaatccaccagagcaataaaaaaaaaggcacaaactcgcatcttccgatggcttttgagaaactcaagccagctcccccagctcacattcctgtttctgtccagttttgttttctttaaaggtccctctgtcccccacccgggtgcagaccccccgccgcacaccgctatggttcacagaggcgggccacagccgtagaaaacgtcctctttaaaaaaaaataagctacaagatgagtcgagtggtttacacagagactgtggagttgtgggtaataaactttaagcaccagttttaatcaagtttgttttgtattattagatctttgatatttgttttctgtgcctcgtgtcaactgaattcggcagctcggccgcctgttgccacaggctcctttcttccacggcgtcccttgcgggacccgccagagtgtgcttggcttccgcgtgtccgtgtgtctgcgcgtcgccggcgtctgtcccgtgttccctgtgaggctgccacgcccaggcgtgcatgtgcgtctcgagacctgtgggcctgggcggcagaaaggcttcccgtggctgttgcacgctgggtgtccctgggtgctccaagagagccccacggtgggacgcaggcgtgacacgggaaagtttcttggctgagcttcaagacagagacagacagacaagagaacagcagcttcgagggagtgctacaggggcggctcctcttccatgggctcctcatctggtctcttttcggcgggcttcacgcccacggacagcgaggccatggcggtgaccgtctcggcttcttcgttctcgcaagtctgagcctcgatcagagaacgccccgctgtggaggttgtgcgctgcaggcagcgccagtacttgctgtggatctccatgactttctccatggaacggacagcgtttgcattgggtctttgctgtaaaaccttttctgggagaggatcaagctcgtttcccagcaaggcagaaacacatgcttccgaggcgtcgcaaatggcggtcaggtcgtggcctccctcgagggccaggacaatccggccgccagccaggcccatcagctgcttcgtcaggtacccgaagcatctggcggagaggttgtagcccccaagaggggtggggtggccctccacggcatcgaagcctgatgacaccagcaccacatccggggcaaactcgctggcgatcggcatgaccaccgttctgaaggccgccaagtactcagcgtctcccatgggggggtccaggccgccggtgaaagccatgttgacgttgaaacccacgccgggccctgtgcccacctcatcaggagccccgctgcctgggaagaagttcccatcgtcgtagcggtggagggacatgtacaggacgctggggtcgctgtagaaagcctgctgggtcccgtttccatggtgcacgtcccagtccacgatgaggatcttgctcacgctcaacctctgctgcagaagcttggctgccacggccacggagttgaagtagcaaaagcccatgggcgtgctctcctccgcatggtgtccaggggggcggaccacagcaaagccattcttcagctcccctgtggccaccttgaagaccagctctaccacgcagcccacagccaggcgggctgcccccgccgagtgcacctcgttccatatggtgtcactgtccaccccaacaccaccgcaagggagccggacgaacacggaggcgagcgagcctagaagtttcttactgtccagtttctgccggttgagggggttcgtgccatacaggagggtgtgggcttccgagtgcaccgtctgtagctcctccagggtggccttgcgtccgcggatgcactcgcatttgccccggaggcccgtctcctgcaggcgggaccagatgctctggatcctcccggcgtgctcggggtggctgctgctactcccgcaggtgcactggtgcttcagcatcagcgtgtcatacacgaggcctgtcgtgaacctcggcttggtggggggctcctgcacagacacggggaaggtggcagacgcgggtgaggactgcgcccgggacagaggcctgtggccgccgaaggacacggggatgccggcggcctccatggacgcctggtagttcctcagctggtggatccgctgctgctccagcaggagggcttgctgtctgaagagcagctcctgctcactgggctggcgctggcccggctccacctcccgtgggggctctgcctcttcctcatcgctctcaatgggctcctgcttcacctgcacgccggcctgtgcgtgcgcctccttctgccccggcagccggtccaggtagggctcgtccagcagagcctggtgctcacggagctcctcctccgtctcctccgggtggctctccggctgccgggctggctcgcttggcttggggatgatcttgttcatctgcagttgctgctgctggaactgctgcttgtgtttctccagaaactgctgatgctgctgctggatgaccaggtgctgcagagcctgggcgttctggggcagcggggccgactgggtccgccccagtgggcggtgctgccgcagcttgtggatggagggggacacccggtctgcaccaaccaaggactgtgcgtggaggggcagtgctcccaggcctgaaagataccagtctgtgacgaggggtgcttgtgccggcggctgctccagtaagaccatgtgctgcagaagagggctgtgcgctgcccctccgtcccgctccaagggcgaggtgctcaggtagggagtgaggtgggtgccggggaaaagggagagcctctgctggagggcgggaagggtgagtctctcggcgtcctgctggcccgccgtgcccgcagaggggccggtggcaggcaggcccagcgtgatgttgggcaaggatggcgatgtgtagaggggaagtggagcggccgagccttctcgtgccacaagtctgtgcgccaaactcgtctccgccgggatgctggggacggcgggcgcgataccgttctccgcgctgacgctcccggagctgttgttgggtgagctgggtccggagcctggggcgctgctgcacgcggagtctgtgacatccaacggacgcttttttagagcagtgaccactggcccgtctttcctgcgtaacagggggctgctccgtctttcggccactttctgctttagcctggaccgtaatttcagattcggttcagaagctgttttcctaagagggaagtcatctttggcgtcgtacattcccaggaccgggtggttataggaggtcgacactccgctctggggtggagaactctggtcaagggaactgtgctgcgttttcccgtaccagtagcgagggtcgctggaaatgcagtggttcagattccggtgggccagcgccttctttttattgaggacaaattcttgtaacttcatcttcacttctgtgctggccacggcactctctttgcccttctccttgttcttgagctgctgcagcttctgctcccggtgctgcttctccagctcctgctcctggcggtgcctctccagcttccgctggtgttccagcagctcctgctggtgcttcatggccagcatctcctgttgttgcttgatgtgctcgtggagctgcgcctcgtgctgccgggagagctgctcgtgctgcctctggaactcagcgatgaggatctgcctctggatctgctgcttctgcttgagcgccaggagctcctgctgcagctgctgctcccgcagggccggctctgccacaggcagtgagaactggtggtccaggcgcaggtccatgggcactgccgagggggccacttgcagaggcagcgccgtggccacatccactggatggctttgggagctcattgctagcaatgtccactcctttaagtgattcgaaatggctcaaaatttccacggaaacgatagctccaacgagctccaaactcccaccaacacatacaagtaccgggacggtgagggctgggtcacagacgttcaagcgccgagcctcgccggcaaggtctcatgagccaggtaacccacaagttgaacagaggcgtccgctggcttctgcagatgaacgttgaaccatgatgcttctccccactccagcgtcgagccaggcggcgataggccaccccgcacgcccgtcagccggcc

SEQ ID NO: 10214 - RNA, 13928 nt, Homo sapiens
  source 1..13928: mol_type = other RNA
caggaaggagacaggcagttcactgtgaattctgagtagtttccctaaaacactgtttccacataaatacaataaactctattattggtatgtcacaagtgctagataaactttttttcttaatatgacaaatgtttaagtagtcctttttatttttcttacaataaaaagtacaatttcttaagaataagttcaataagacgcaaacttccccgccctcctctccttcaaggttttgttttacagaaaaatttccatcttttgtatctgcaaatgtcatgagaggggaacagaaaggcatttttcttcttccccaaagctgccgagtttggcgtgcaaaatctgtatacaatataaagtcatgccggtcgtacagtccatgcaacctccaggtgtaggaaacttaaaaaaatatattcatatatatttatatctatatatttatatatgtatcaatgcccataaaacacgtgggcccaaagtctacaaaaagaagaatggaatgagcacgtggctgtgaccagtaaagaaggaatgttctgatcaaaaagaaaaacaacaaagtccattgctagtgctgcaaaaatcaaacttgcttttgtgtcagaccattacgaaatggtccttccccttgcaaacagattttcaaaagaagtaaagaaaaactgaaacaccttgacaaagtggccctccagaaccagagccctgggacgctggggaggggcggccagtcccagcgggccacggcctccgggacagccgcctgctggtggggcgtgggcacgtgggcacgctgcggcacggcgggaagccgcgagggcagggcagacgccaagaggcccagtggcgtcatcagggtttccctcaaagggatataaagtgctcgcttgctgactcccagccagtgcccccaaggcctttgcaaaggaagaaaaaggctaaaggtccaaggacccacagggagaacacatgaaggaaccctccctgacgtggtcccgcctgcagacgccgaggcagatcctctgccatctgccctggacgcttgctgtggagaagagccgagtgtgtcttcaaagaaaaggctacacagtaatgctctcagcacatttgtgaagctggagtgagctgacagatgaaacgtgcctccccctgccaggcctttgcagagggcgtctccatttgaatgagattagaattaagtccccccactgataacctggccactgagcagtccatgttatcccatcatctgcttaaaaaaaaaaagtgagatgatgcattcctccccataagccacggcggggtaagagggcaggtggcaggatccccagagggctatgcagagaatgaggccaaggaggccagaagagcctgctagctgggccctgccactgctctgtgccatgaatggggaatggaccagctcctcttgccaatctgggcttcagagcaaagagtggccaccagggaggggaaagtcaaacaagtcccaagaccgttctgcctgctctcaaaccactgtctcagagctgaccatcagcagcccagtgaccaagtgaatccaagaatctgcactcatttggtcaaaagtttgagttaatttcagaagctaccctgtaaactttaccaaactccgaaactcggctctgggtccctcctgagcacggtgtgtctgaacttctgcccccaagtctgaacccaatatacactttggaatgaaactggtggcttcatgtgctggaaaataagttaccagtaaaacgtgactgtcagttactgttgaagagaaaaagagtaaagactggctgtcctggtcaggcaatcataccctccctgcaggttcaccaggcaacaagggtccctgggttccttgcagccacaggctccaaaatccagggctggccacgtggctgcagtggaaaaacccaagtgggtaaagagccccacgtgtgccccatgcattgctgacatgctcaaaaggtctttggaaaactcaagttagaattctatcctgacgatgtggtcagagaagtttaaacatgagtttcattaatgctgactgcccccggcatctggcaagcctcccagggtggccgggcatcctaagcaaccctccctgcccttgccacggaggggaaaaacacaccacccctcgtaatactactagtgttgaaagttaaaaagagcccctgggcttctttatacagctcctaggacagaccaggaaagacacaatcgttggtgtcactccgaaaagacctacggtccctcctctcactttctgaaaatagaatctgacagcaacaattctgtacgctgcagaaaactcatcgtacaaaaataaaaacaaaaataattaaaaacctttgaaaggtaaaaaaaaatgtacaagcaagaattcagaaaggaaaaagatttagacattattaccattcagaaaattgctaaatggtgaggaaaaatgtaaaattcataaaacaatgcttattcaggatctttttgtgaaaaaattcatacaaaaatcaacagcaaatttatattctttgctataaaaactcattaggtacatatgtgcatgaaggcttggagacgggagcggttctgttagaaaataattaaaatgaaagtacaaacttgtagggtagttgcccagtggcgaatgtgttggcgatctgaaatctagccaatctggagcttgagaaaacatgaatttcaatcaatcaggatccctttccataagcaccttgagagcaaattcacaagccatccatttgcagggaccttcgcaatctgcattcattttatatatatatatatactttttctataaatgcattataaatattttatcaagatttcataagaatcaagtaagtttcttagcttggaatacattggaatatatattatacatatatatatttatttatacctaaaatttaagcaatacttcatgctacttgcttttaataaaaagcattccgatcgtaacactgcaagtgtgcctaccacatgcttcacgaccagatggagatgctcaatcgtatgtgacgtgtgagaacactttggattcgtttaaaatttgttggacttcaaaacctccaacgggatttgccacttttttggaactacctccatttttcttaaacagcaataaagcaaaacagggaccgccgggctgcagcccctggccccggagatgacggctggtgcccgtgcttgaggcgtcaggccagctcgcggtgccagcactgccaggctcggctggccacaggaaactgtcccaccgattcctgctgtttgttttttcttaaggcattgttcctcagacttcagaaaacccagccacaaaaatccaccagagcaataaaaaaaaaggcacaaactcgcatcttccgatggcttttgagaaactcaagccagctcccccagctcacattcctgtttctgtccagttttgttttctttaaaggtccctctgtcccccacccgggtgcagaccccccgccgcacaccgctatggttcacagaggcgggccacagccgtagaaaacgtcctctttaaaaaaaaataagctacaagatgagtcgagtggtttacacagagactgtggagttgtgggtaataaactttaagcaccagttttaatcaagtttgttttgtattattagatctttgatatttgttttctgtgcctcgtgtcaactgaattcggcagctcggccgcctgttgccacaggctcctttcttccacggcgtcccttgcgggacccgccagagtgtgcttggcttccgcgtgtccgtgtgtctgcgcgtcgccggcgtctgtcccgtgttccctgtgaggctgccacgcccaggcgtgcatgtgcgtctcgagacctgtgggcctgggcggcagaaaggcttcccgtggctgttgcacgctgggtgtccctgggtgctccaagagagccccacggtgggacgcaggcgtgacacgggaaagtttcttggctgagcttcaagacagagacagacagacaagagaacagcagcttcgagggagtgctacaggggcggctcctcttccatgggctcctcatctggtctcttttcggcgggcttcacgcccacggacagcgaggccatggcggtgaccgtctcggcttcttcgttctcgcaagtctgagcctcgatcagagaacgccccgctgtggaggttgtgcgctgcaggcagcgccagtacttgctgtggatctccatgactttctccatggaacggacagcgtttgcattgggtctttgctgtaaaaccttttctgggagaggatcaagctcgtttcccagcaaggcagaaacacatgcttccgaggcgtcgcaaatggcggtcaggtcgtggcctccctcgagggccaggacaatccggccgccagccaggcccatcagctgcttcgtcaggtacccgaagcatctggcggagaggttgtagcccccaagaggggtggggtggccctccacggcatcgaagcctgatgacaccagcaccacatccggggcaaactcgctggcgatcggcatgaccaccgttctgaaggccgccaagtactcagcgtctcccatgggggggtccaggccgccggtgaaagccatgttgacgttgaaacccacgccgggccctgtgcccacctcatcaggagccccgctgcctgggaagaagttcccatcgtcgtagcggtggagggacatgtacaggacgctggggtcgctgtagaaagcctgctgggtcccgtttccatggtgcacgtcccagtccacgatgaggatcttgctcacgctcaacctctgctgcagaagcttggctgccacggccacggagttgaagtagcaaaagcccatgggcgtgctctcctccgcatggtgtccaggggggcggaccacagcaaagccattcttcagctcccctgtggccaccttgaagaccagctctaccacgcagcccacagccaggcgggctgcccccgccgagtgcacctcgttccatatggtgtcactgtccaccccaacaccaccgcaagggagccggacgaacacggaggcgagcgagcctagaagtttcttactgtccagtttctgccggttgagggggttcgtgccatacaggagggtgtgggcttccgagtgcaccgtctgtagctcctccagggtggccttgcgtccgcggatgcactcgcatttgccccggaggcccgtctcctgcaggcgggaccagatgctctggatcctcccggcgtgctcggggtggctgctgctactcccgcaggtgcactggtgcttcagcatcagcgtgtcatacacgaggcctgtcgtgaacctcggcttggtggggggctcctgcacagacacggggaaggtggcagacgcgggtgaggactgcgcccgggacagaggcctgtggccgccgaaggacacggggatgccggcggcctccatggacgcctggtagttcctcagctggtggatccgctgctgctccagcaggagggcttgctgtctgaagagcagctcctgctcactgggctggcgctggcccggctccacctcccgtgggggctctgcctcttcctcatcgctctcaatgggctcctgcttcacctgcacgccggcctgtgcgtgcgcctccttctgccccggcagccggtccaggtagggctcgtccagcagagcctggtgctcacggagctcctcctccgtctcctccgggtggctctccggctgccgggctggctcgcttggcttggggatgatcttgttcatctgcagttgctgctgctggaactgctgcttgtgtttctccagaaactgctgatgctgctgctggatgaccaggtgctgcagagcctgggcgttctggggcagcggggccgactgggtccgccccagtgggcggtgctgccgcagcttgtggatggagggggacacccggtctgcaccaaccaaggactgtgcgtggaggggcagtgctcccaggcctgaaagataccagtctgtgacgaggggtgcttgtgccggcggctgctccagtaagaccatgtgctgcagaagagggctgtgcgctgcccctccgtcccgctccaagggcgaggtgctcaggtagggagtgaggtgggtgccggggaaaagggagagcctctgctggagggcgggaagggtgagtctctcggcgtcctgctggcccgccgtgcccgcagaggggccggtggcaggcaggcccagcgtgatgttgggcaaggatggcgatgtgtagaggggaagtggagcggccgagccttctcgtgccacaagtctgtgcgccaaactcgtctccgccgggatgctggggacggcgggcgcgataccgttctccgcgctgacgctcccggagctgttgttgggtgagctgggtccggagcctggggcgctgctgcacgcggagtctgttttcctaagagggaagtcatctttggcgtcgtacattcccaggaccgggtggttataggaggtcgacactccgctctggggtggagaactctggtcaagggaactgtgctgcgttttcccgtaccagtagcgagggtcgctggaaatgcagtggttcagattccggtgggccagcgccttctttttattgaggacaaattcttgtaacttcatcttcacttctgtgctggccacggcactctctttgcccttctccttgttcttgagctgctgcagcttctgctcccggtgctgcttctccagctcctgctcctggcggtgcctctccagcttccgctggtgttccagcagctcctgctggtgcttcatggccagcatctcctgttgttgcttgatgtgctcgtggagctgcgcctcgtgctgccgggagagctgctcgtgctgcctctggaactcagcgatgaggatctgcctctggatctgctgcttctgcttgagcgccaggagctcctgctgcagctgctgctcccgcagggccggctctgccacaggcagtgagaactggtggtccaggcgcaggtccatgggcactgccgagggggccacttgcagaggcagcgccgtggccacatccaccgtgctgggcatgtggttcacgcgggcaggattcagcagctccactggctggtctcggccagaaagtccatctccatccacagccagatactgcttccggaaccacacttcgtatccaggtgagctcgttttttgtatttcaaaagcacaaagatctatgttcatggtgtagtccaggcagagtgtggttaacaggcctccgggtgtcccccccttccagcccagtgcaggggttcagccgctgcagaaactccgaatctgctaacgtgaagtgccaagactgctgtccgccagcgccctcactcccccagggcctgtacctgtagcaggaggctcacgttccgagtcctcattgctcccagacccaagggcaaggctgtcacaggcgaaagacgggttccccttcctctacacccaagccctcggaagcacgctgcaggcccctggaggtgccacagtgctcccagctcccccagaggctgagttcaaacattctaaacggattcttgataacaagccgccggctcgctggaagacactgagcagttacataacagcacagaaaatcccttacaagtttcttaaaaaagagttaatcgtactgacttggtgctttaccttcagcccagactttcgcttaatcccggaaactgctccaaaggcgtttttctcagggcgttcggcgccgtaactcaggagaaacccaagtcctgctctcccggcggcctcgctggggaagaattcagccgctccaccctgacatctggtttctatttcatatccatgttgtcacattacataacaagcagatgatacgagagatcaccacagtgtttcggctcgagagtcacaaagaacgcccagaacactgtttatattgggggccatgaacgttcaccaaaccagacttagtgcagaggctgcacccttccaggctgaaacccagcacctacagcaaatgcccaaggaagcaagaagcgggaccccgccttctcagccacctctcactaacactcagctccactcctgcttccttcctctcactccacatccgagttagagggaaatacgatttatctctggcctgcatttacttctcctgcacctggcgggaggctctggccttgcaggcgtgcaggagcccctgccagtgagggccagcgaggggcccagggagaagatggaggtcaagtcatagggcctccaccgcaggcagagctccgccagcaagtatcctgggagctggggggcctcaagggaggcaatccccccacacaccatccccttccccttcgctcatctggggaagctgtgaggactggtgttgataaaacattccaaccacacactcagaccatggatgtggccgtgccagcagggaggccagcagcccctagcagaagggtgttctggaagctgccccctcccatgctgctgcctggtcccatggggcatgaagggagggtggccagggtggcccgagccagcatcaggcacaaggcccaaggagtttctccagagcagcctgtcctcttcggtccagaaaaagtcagattccacagcagggttagccgtccagttagggaacccactaaggggctctgtgcgtagaggtgctcagaatcaaaccactaaaccccaggaccccctgctgggggaatggtccgtggcagtcattcagccttggagtgaaccgttctgcccaagtgcaagtgagaacacaatacttcttattatatacagaattgccaaagccaacgtgattagtagaaaaaccgacatgtcagtgacttgggggtctggtttgccccagatgtgggtggaaaccccaggcgtccctcaagcctggtccagagctccacagacagcagatacacaaactctgagtgacagcattggtgtttagcagattctggattttgctcccccccgaaccaagtatagagaatgtttcacagagtagcttcaacagaaaatggccacagtgtgtctgtgagagagtgtgatgttcccggggggatggctggggccaagggaaggcccctcccatgagccctgcctccatgagactgcgtagggcaggactgccaggcagaaagaacacagcacaggcacaagggcagacccaggctggcagggctaaatggcttcaggagctcccccctctgccccccagggagtaaaggcaatgatgcaaatatgataagcaaacagaggtcccaaaacacagaaagggccaggaccctgatgccaaccaagcagacccaaaactgggtctgggagcacagggcagggtcgctgagtgcagaggggcctcactcaatgtccaacacttccctccaaaacagacatgctggtgagaggcttcaacccttccactggcctgacacctggatctctgctgccctgtgccaggttagccacgtccaacaccaccacggccaccggccatttaagaaaacgaaccctgacgttaacctgcttgagccctaatactaagcaagagcagcgccacaattccaaaactgcagagagcgccttttaaacattctgctgagatctgcgcggtcgcggtctgacaggcaggccttcttggctacctgtggtttcattccagcattaacaggcacctaaaaggcctgtgagcttttgtggggtcaagcagcatcagctccactttacaaccccgcagagtgaggtgttagctctgcagctccagggcagagccttgcagccttagggccagggggacggcctggccccttccgagctctcagcagcctgaactccacgtgtcccctgctgtgtcactggcatgctggtcttgcatggcactgagatgtgtggcacaagcaggcaccaagcccggagacacccgacgctcaccgttagactgggtagcatttgtcaagcgccgagcaaacagtggatgaagtgtcctcagccggcgtcagctgttctgatccgcagaacacataactcctggcactcctttccaagcatccgggaaatgtagaatccaagtgttacaccatccagttgaagatgacagatttacgatataaaacggcacccgcgactgaggactttgtaggaatggaggccgctgtcattatttcatgggtgagggggagagggacactgtgacccatgacaggaaaggacagctcagcccctccaaaaccacacacaggggactccgtttctcacaaaacttcaagtttctgttctacgcaaacattacaacacattttaaactacattctgacacgaagctcccgtgctttttaatggcaggtgttacaatgatcatggaacagtgatggggcggtgcttcctcacggtgacatggcagggagaagtctggaccggagccagcagggtccttgacctaagaggccttgggcagcccacggggcagctctgagcaatctcctgtgaaaggaagagctcagaacgggttcctctaaaggttccttccagagcaggggttctgtggttccctggggccctagactaacatgaggaaggggaaacagagaagaatgcccactaaaagccttacccaaaaattgaaagccaagaaaaatcacaccagatcatctcagtttagacttgaggaacctcggcgctgacatcactgtcaccatcacaaaacactggccaccaaggtgccacctaccacactgcaacctggaaggaggggcgggcaggggcacccctgggcagggcaggacaccaggccagccagccacccacgctacagaggaaatgcagcccctcccaactaagagaaccctggtaccatcaccacagccttggtgccagggctcctagcacctgacagggaagatgagaaggacattggctgccgccaagaggcctgctgcccacccccaactgcacggtggtggtgctgccagcaccaccatccatgctggcccaggagcccacacgcagggcacgcacgcacgtagttccacattaggccctttcttcctcaattgttggaaagaaggccaaagccagatgatggtgaaattcacgaggaaaatgtccccgactgtcctccattctaaagcaaacgctaagaatgggctgctgggcttcagcagaagccaagtcacctttcctctatgcgtccaatgaaacgaaaacatccacacttgtctttataaaaacggaaaactgcatctggaacaaggtctgtggcgtttcttccagcgtgtcccatggacatgaagttggtcttcctatgggtcctccaaggcacacccctcgactgcaccacagcactgagggcagaatgtggtggtggcccagctgccgtggcgccggcagactagcctggtacacggagaggggagcctgctgactgtgggtaggccacgttcccccagtgtcttcatctgcagagggagaccgggagcctctgaagaccgctccagctctgcactgtgggggcggccggccagcaggcaggcaatgctctcaggccccacgctcctctcactggctgccgacgggaggcagacgaggtgccgggggcagcctgcagagcaaggagtcaaggtggccagcctggggcagggtgttcccccagccagggagcttcactcaggcttgggctctgtcccgtgcctccccgggggcgttccgaggtggcggaggaggaagctgcagcccgttatccaccgcccagtctctccctctcaccagcacacagatgttctcagcggcagagcctggcttctgcctgaattcatttcatatttttaaatatgctcttaatggaaagcaacaaaagtacttaacaaaatgcgctgatgtaaatgtccctgcagcagccagggactaattttagaaggggctttgaggagaaacccaagggacactcacttgctggaaacggcctcctccccaaagagtgtgaggatctggattagaaccaagtatccccaggctgcccaggagcccgctcctccaattgggggctggccatcccaccgagcactgataccgcaggctggactcttcctaacctcacgagaggtgatgaccggaatcatcccagttttccatggcacttcgcaaacacagctggtcaggcccttagcacctcctgaccccccgatctcccagactctctgctggaagttaaggacacagagaaagtttcttatgaaaataagcgcctcaaaagaaagccaacgtacagcactggtgacagaaaggaagattcagaaaagccttcacgcctggcaatatggcacacgcacttttagagacgtctaattatactcagggctgagttggctgaagagtgaggaatatactccaaagacaggaattcaaggcagggcaaatagaacatgaaagccagcctggagcccagggcctgtcctggggcagccacctgcactgcctcttaccactgcaccgtccctgtgagtgtgcgtggggaggggctgtagttcccttggcaggggaagccagaagacaggcctgcaagggacacatccgggcctgggcttggtgctggctagaaggggtcaaatcgagagaggactcccctcagaactcataatcccagacccctcgcaatggtttggggagaattcagacaacccatgaggcctgatgagcatccctagcacctgcaaacacaggcatgtcccaggtggcacctcccagcaccaggcagaaaccttctctagaggaacacgctatgaacctcaaaaaaacatccaagaaggacggacataaagtcacaatcaagaaccatgggtagcgggagtaagtcccggaaagacctcagttgtaggaaaatcaggcactgacccaaaacacatacgaaggacactcgacaaaacaagagaggtcatccagggtcaggctggagctagaggcctccagatcctgtcacttagtgactgtacaaacctggtggcttcctcaacctccctgtgccttagcttcccatttgccaaaaagggggattagaagagcccacactctccctggagcaaggctaaggaagaaaggagacagatgtctcagctgttattattaataactatcagaagtgtcacatggatctgaatgatccaaatggaacttgtagaaacaaaactgtcatcattaaaatttaaaactaaatgagtgagttaactaatcaagtattaatagacagagctgaagagagaattagtgaacagtaaaatagcacggaagaaataaaccaggatgcaacacataaaggtaaagagatagaaagctggagacgttagaggactggaaggacagaggaagatatgctaacacacatctgtaaaccaaaaataaaattctaagctcccaaccatctgaatggacccctcctctcaagccaagggcattccaacattaacctgaaaagctagttcaggtcgtgatggggacgggcattcagatgtgcctcatgataccctcctcccttttggaattgctgatagaacagactctttaagtctgatgagaaacatttcagtctattctctctgaagcctgctacccggaggcttcgtcggcatggtaaatccttggtctccacaaacccttatcataatccagacattcctttgtgttgataataactctttcaaccaactgccaatcagaacattttaaaatctacctataatctgaaagcctcacacttcgagttgtcccgcgtttctggactggaccaatgttcatcttccacatactgacagacgcctcatgtctccctaaaaatgtatgaaaccaagctgttccccgaccaccttgggcacatgttgtcagcacctct

SEQ ID NO: 10215 - RNA, 7974 nt, Homo sapiens
  source 1..7974: mol_type = other RNA
caggaaggagacaggcagttcactgtgaattctgagtagtttccctaaaacactgtttccacataaatacaataaactctattattggtatgtcacaagtgctagataaactttttttcttaatatgacaaatgtttaagtagtcctttttatttttcttacaataaaaagtacaatttcttaagaataagttcaataagacgcaaacttccccgccctcctctccttcaaggttttgttttacagaaaaatttccatcttttgtatctgcaaatgtcatgagaggggaacagaaaggcatttttcttcttccccaaagctgccgagtttggcgtgcaaaatctgtatacaatataaagtcatgccggtcgtacagtccatgcaacctccaggtgtaggaaacttaaaaaaatatattcatatatatttatatctatatatttatatatgtatcaatgcccataaaacacgtgggcccaaagtctacaaaaagaagaatggaatgagcacgtggctgtgaccagtaaagaaggaatgttctgatcaaaaagaaaaacaacaaagtccattgctagtgctgcaaaaatcaaacttgcttttgtgtcagaccattacgaaatggtccttccccttgcaaacagattttcaaaagaagtaaagaaaaactgaaacaccttgacaaagtggccctccagaaccagagccctgggacgctggggaggggcggccagtcccagcgggccacggcctccgggacagccgcctgctggtggggcgtgggcacgtgggcacgctgcggcacggcgggaagccgcgagggcagggcagacgccaagaggcccagtggcgtcatcagggtttccctcaaagggatataaagtgctcgcttgctgactcccagccagtgcccccaaggcctttgcaaaggaagaaaaaggctaaaggtccaaggacccacagggagaacacatgaaggaaccctccctgacgtggtcccgcctgcagacgccgaggcagatcctctgccatctgccctggacgcttgctgtggagaagagccgagtgtgtcttcaaagaaaaggctacacagtaatgctctcagcacatttgtgaagctggagtgagctgacagatgaaacgtgcctccccctgccaggcctttgcagagggcgtctccatttgaatgagattagaattaagtccccccactgataacctggccactgagcagtccatgttatcccatcatctgcttaaaaaaaaaaagtgagatgatgcattcctccccataagccacggcggggtaagagggcaggtggcaggatccccagagggctatgcagagaatgaggccaaggaggccagaagagcctgctagctgggccctgccactgctctgtgccatgaatggggaatggaccagctcctcttgccaatctgggcttcagagcaaagagtggccaccagggaggggaaagtcaaacaagtcccaagaccgttctgcctgctctcaaaccactgtctcagagctgaccatcagcagcccagtgaccaagtgaatccaagaatctgcactcatttggtcaaaagtttgagttaatttcagaagctaccctgtaaactttaccaaactccgaaactcggctctgggtccctcctgagcacggtgtgtctgaacttctgcccccaagtctgaacccaatatacactttggaatgaaactggtggcttcatgtgctggaaaataagttaccagtaaaacgtgactgtcagttactgttgaagagaaaaagagtaaagactggctgtcctggtcaggcaatcataccctccctgcaggttcaccaggcaacaagggtccctgggttccttgcagccacaggctccaaaatccagggctggccacgtggctgcagtggaaaaacccaagtgggtaaagagccccacgtgtgccccatgcattgctgacatgctcaaaaggtctttggaaaactcaagttagaattctatcctgacgatgtggtcagagaagtttaaacatgagtttcattaatgctgactgcccccggcatctggcaagcctcccagggtggccgggcatcctaagcaaccctccctgcccttgccacggaggggaaaaacacaccacccctcgtaatactactagtgttgaaagttaaaaagagcccctgggcttctttatacagctcctaggacagaccaggaaagacacaatcgttggtgtcactccgaaaagacctacggtccctcctctcactttctgaaaatagaatctgacagcaacaattctgtacgctgcagaaaactcatcgtacaaaaataaaaacaaaaataattaaaaacctttgaaaggtaaaaaaaaatgtacaagcaagaattcagaaaggaaaaagatttagacattattaccattcagaaaattgctaaatggtgaggaaaaatgtaaaattcataaaacaatgcttattcaggatctttttgtgaaaaaattcatacaaaaatcaacagcaaatttatattctttgctataaaaactcattaggtacatatgtgcatgaaggcttggagacgggagcggttctgttagaaaataattaaaatgaaagtacaaacttgtagggtagttgcccagtggcgaatgtgttggcgatctgaaatctagccaatctggagcttgagaaaacatgaatttcaatcaatcaggatccctttccataagcaccttgagagcaaattcacaagccatccatttgcagggaccttcgcaatctgcattcattttatatatatatatatactttttctataaatgcattataaatattttatcaagatttcataagaatcaagtaagtttcttagcttggaatacattggaatatatattatacatatatatatttatttatacctaaaatttaagcaatacttcatgctacttgcttttaataaaaagcattccgatcgtaacactgcaagtgtgcctaccacatgcttcacgaccagatggagatgctcaatcgtatgtgacgtgtgagaacactttggattcgtttaaaatttgttggacttcaaaacctccaacgggatttgccacttttttggaactacctccatttttcttaaacagcaataaagcaaaacagggaccgccgggctgcagcccctggccccggagatgacggctggtgcccgtgcttgaggcgtcaggccagctcgcggtgccagcactgccaggctcggctggccacaggaaactgtcccaccgattcctgctgtttgttttttcttaaggcattgttcctcagacttcagaaaacccagccacaaaaatccaccagagcaataaaaaaaaaggcacaaactcgcatcttccgatggcttttgagaaactcaagccagctcccccagctcacattcctgtttctgtccagttttgttttctttaaaggtccctctgtcccccacccgggtgcagaccccccgccgcacaccgctatggttcacagaggcgggccacagccgtagaaaacgtcctctttaaaaaaaaataagctacaagatgagtcgagtggtttacacagagactgtggagttgtgggtaataaactttaagcaccagttttaatcaagtttgttttgtattattagatctttgatatttgttttctgtgcctcgtgtcaactgaattcggcagctcggccgcctgttgccacaggctcctttcttccacggcgtcccttgcgggacccgccagagtgtgcttggcttccgcgtgtccgtgtgtctgcgcgtcgccggcgtctgtcccgtgttccctgtgaggctgccacgcccaggcgtgcatgtgcgtctcgagacctgtgggcctgggcggcagaaaggcttcccgtggctgttgcacgctgggtgtccctgggtgctccaagagagccccacggtgggacgcaggcgtgacacgggaaagtttcttggctgagcttcaagacagagacagacagacaagagaacagcagcttcgagggagtgctacaggggcggctcctcttccatgggctcctcatctggtctcttttcggcgggcttcacgcccacggacagcgaggccatggcggtgaccgtctcggcttcttcgttctcgcaagtctgagcctcgatcagagaacgccccgctgtggaggttgtgcgctgcaggcagcgccagtacttgctgtggatctccatgactttctccatggaacggacagcgtttgcattgggtctttgctgtaaaaccttttctgggagaggatcaagctcgtttcccagcaaggcagaaacacatgcttccgaggcgtcgcaaatggcggtcaggtcgtggcctccctcgagggccaggacaatccggccgccagccaggcccatcagctgcttcgtcaggtacccgaagcatctggcggagaggttgtagcccccaagaggggtggggtggccctccacggcatcgaagcctgatgacaccagcaccacatccggggcaaactcgctggcgatcggcatgaccaccgttctgaaggccgccaagtactcagcgtctcccatgggggggtccaggccgccggtgaaagccatgttgacgttgaaacccacgccgggccctgtgcccacctcatcaggagccccgctgcctgggaagaagttcccatcgtcgtagcggtggagggacatgtacaggacgctggggtcgctgtagaaagcctgctgggtcccgtttccatggtgcacgtcccagtccacgatgaggatcttgctcacgctcaacctctgctgcagaagcttggctgccacggccacggagttgaagtagcaaaagcccatgggcgtgctctcctccgcatggtgtccaggggggcggaccacagcaaagccattcttcagctcccctgtggccaccttgaagaccagctctaccacgcagcccacagccaggcgggctgcccccgccgagtgcacctcgttccatatggtgtcactgtccaccccaacaccaccgcaagggagccggacgaacacggaggcgagcgagcctagaagtttcttactgtccagtttctgccggttgagggggttcgtgccatacaggagggtgtgggcttccgagtgcaccgtctgtagctcctccagggtggccttgcgtccgcggatgcactcgcatttgccccggaggcccgtctcctgcaggcgggaccagatgctctggatcctcccggcgtgctcggggtggctgctgctactcccgcaggtgcactggtgcttcagcatcagcgtgtcatacacgaggcctgtcgtgaacctcggcttggtggggggctcctgcacagacacggggaaggtggcagacgcgggtgaggactgcgcccgggacagaggcctgtggccgccgaaggacacggggatgccggcggcctccatggacgcctggtagttcctcagctggtggatccgctgctgctccagcaggagggcttgctgtctgaagagcagctcctgctcactgggctggcgctggcccggctccacctcccgtgggggctctgcctcttcctcatcgctctcaatgggctcctgcttcacctgcacgccggcctgtgcgtgcgcctccttctgccccggcagccggtccaggtagggctcgtccagcagagcctggtgctcacggagctcctcctccgtctcctccgggtggctctccggctgccgggctggctcgcttggcttggggatgatcttgttcatctgcagttgctgctgctggaactgctgcttgtgtttctccagaaactgctgatgctgctgctggatgaccaggtgctgcagagcctgggcgttctggggcagcggggccgactgggtccgccccagtgggcggtgctgccgcagcttgtggatggagggggacacccggtctgcaccaaccaaggactgtgcgtggaggggcagtgctcccaggcctgtgacgaggggtgcttgtgccggcggctgctccagtaagaccatgtgctgcagaagagggctgtgcgctgcccctccgtcccgctccaagggcgaggtgctcaggtagggagtgaggtgggtgccggggaaaagggagagcctctgctggagggcgggaagggtgagtctctcggcgtcctgctggcccgccgtgcccgcagaggggccggtggcaggcaggcccagcgtgatgttgggcaaggatggcgatgtgtagaggggaagtggagcggccgagccttctcgtgccacaagtctgtgcgccaaactcgtctccgccgggatgctggggacggcgggcgcgataccgttctccgcgctgacgctcccggagctgttgttgggtgagctgggtccggagcctggggcgctgctgcacgcggagtctgtgacatccaacggacgcttttttagagcagtgaccactggcccgtctttcctgcgtaacagggggctgctccgtctttcggccactttctgctttagcctggaccgtaatttcagattcggttcagaagctgttttcctaagagggaagtcatctttggcgtcgtacattcccaggaccgggtggttataggaggtcgacactccgctctggggtggagaactctggtcaagggaactgtgctgcgttttcccgtaccagtagcgagggtcgctggaaatgcagtggttcagattccggtgggccagcgccttctttttattgaggacaaattcttgtaacttcatcttcacttctgtgctggccacggcactctctttgcccttctccttgttcttgagctgctgcagcttctgctcccggtgctgcttctccagctcctgctcctggcggtgcctctccagcttccgctggtgttccagcagctcctgctggtgcttcatggccagcatctcctgttgttgcttgatgtgctcgtggagctgcgcctcgtgctgccgggagagctgctcgtgctgcctctggaactcagcgatgaggatctgcctctggatctgctgcttctgcttgagcgccaggagctcctgctgcagctgctgctcccgcagggccggctctgccacaggcagtgagaactggtggtccaggcgcaggtccatgggcactgccgagggggccacttgcagaggcagcgccgtggccacatccaccgtgctgggcatgtggttcacgcgggcaggattcagcagctccactggctggtctcggccagaaagtccatcaaacatttgctgacagcaagctcagggaacagcagaggcccgtctcggtattccggaagcagccagacctaagatcaaatccaggcttgacgacagactgggctggtgccctggacaagcggtggcttccagaagctgggggagcccctgggcatcacgtggagatgagagaagatgcttccagaacctgacacacagtagggatccggaatcgccagagctcttgcacctcagagggaaacagggtatcctgaagttcaagtgcatgcacaccgtggatactctagggtcccagcaaccccagctattacaatcacactgtcactgggtgaacgctgtgcactctacaggggcctcctcatttagtcatcatagccactggggatgcaggtgcccctgcagcctcattccacccacatccggtgcacagcacacacaggatcagcagtgataggaacagcctgccactctttacagagccgtgagactgtggctaaatcatttatccagcacccaacaacgtggaaatcatgacactccacctacaggggctaggctagaaaggcatttaatcaaacattttagaatgattttcatttaattatctctcggagacttaactgtgtcatatgatgaacaacattatttcctcctaaatgtactgaatccggaagcaacccttcatggcc

SEQ ID NO: 10216 - RNA, 14044 nt, Homo sapiens
  source 1..14044: mol_type = other RNA
caggaaggagacaggcagttcactgtgaattctgagtagtttccctaaaacactgtttccacataaatacaataaactctattattggtatgtcacaagtgctagataaactttttttcttaatatgacaaatgtttaagtagtcctttttatttttcttacaataaaaagtacaatttcttaagaataagttcaataagacgcaaacttccccgccctcctctccttcaaggttttgttttacagaaaaatttccatcttttgtatctgcaaatgtcatgagaggggaacagaaaggcatttttcttcttccccaaagctgccgagtttggcgtgcaaaatctgtatacaatataaagtcatgccggtcgtacagtccatgcaacctccaggtgtaggaaacttaaaaaaatatattcatatatatttatatctatatatttatatatgtatcaatgcccataaaacacgtgggcccaaagtctacaaaaagaagaatggaatgagcacgtggctgtgaccagtaaagaaggaatgttctgatcaaaaagaaaaacaacaaagtccattgctagtgctgcaaaaatcaaacttgcttttgtgtcagaccattacgaaatggtccttccccttgcaaacagattttcaaaagaagtaaagaaaaactgaaacaccttgacaaagtggccctccagaaccagagccctgggacgctggggaggggcggccagtcccagcgggccacggcctccgggacagccgcctgctggtggggcgtgggcacgtgggcacgctgcggcacggcgggaagccgcgagggcagggcagacgccaagaggcccagtggcgtcatcagggtttccctcaaagggatataaagtgctcgcttgctgactcccagccagtgcccccaaggcctttgcaaaggaagaaaaaggctaaaggtccaaggacccacagggagaacacatgaaggaaccctccctgacgtggtcccgcctgcagacgccgaggcagatcctctgccatctgccctggacgcttgctgtggagaagagccgagtgtgtcttcaaagaaaaggctacacagtaatgctctcagcacatttgtgaagctggagtgagctgacagatgaaacgtgcctccccctgccaggcctttgcagagggcgtctccatttgaatgagattagaattaagtccccccactgataacctggccactgagcagtccatgttatcccatcatctgcttaaaaaaaaaaagtgagatgatgcattcctccccataagccacggcggggtaagagggcaggtggcaggatccccagagggctatgcagagaatgaggccaaggaggccagaagagcctgctagctgggccctgccactgctctgtgccatgaatggggaatggaccagctcctcttgccaatctgggcttcagagcaaagagtggccaccagggaggggaaagtcaaacaagtcccaagaccgttctgcctgctctcaaaccactgtctcagagctgaccatcagcagcccagtgaccaagtgaatccaagaatctgcactcatttggtcaaaagtttgagttaatttcagaagctaccctgtaaactttaccaaactccgaaactcggctctgggtccctcctgagcacggtgtgtctgaacttctgcccccaagtctgaacccaatatacactttggaatgaaactggtggcttcatgtgctggaaaataagttaccagtaaaacgtgactgtcagttactgttgaagagaaaaagagtaaagactggctgtcctggtcaggcaatcataccctccctgcaggttcaccaggcaacaagggtccctgggttccttgcagccacaggctccaaaatccagggctggccacgtggctgcagtggaaaaacccaagtgggtaaagagccccacgtgtgccccatgcattgctgacatgctcaaaaggtctttggaaaactcaagttagaattctatcctgacgatgtggtcagagaagtttaaacatgagtttcattaatgctgactgcccccggcatctggcaagcctcccagggtggccgggcatcctaagcaaccctccctgcccttgccacggaggggaaaaacacaccacccctcgtaatactactagtgttgaaagttaaaaagagcccctgggcttctttatacagctcctaggacagaccaggaaagacacaatcgttggtgtcactccgaaaagacctacggtccctcctctcactttctgaaaatagaatctgacagcaacaattctgtacgctgcagaaaactcatcgtacaaaaataaaaacaaaaataattaaaaacctttgaaaggtaaaaaaaaatgtacaagcaagaattcagaaaggaaaaagatttagacattattaccattcagaaaattgctaaatggtgaggaaaaatgtaaaattcataaaacaatgcttattcaggatctttttgtgaaaaaattcatacaaaaatcaacagcaaatttatattctttgctataaaaactcattaggtacatatgtgcatgaaggcttggagacgggagcggttctgttagaaaataattaaaatgaaagtacaaacttgtagggtagttgcccagtggcgaatgtgttggcgatctgaaatctagccaatctggagcttgagaaaacatgaatttcaatcaatcaggatccctttccataagcaccttgagagcaaattcacaagccatccatttgcagggaccttcgcaatctgcattcattttatatatatatatatactttttctataaatgcattataaatattttatcaagatttcataagaatcaagtaagtttcttagcttggaatacattggaatatatattatacatatatatatttatttatacctaaaatttaagcaatacttcatgctacttgcttttaataaaaagcattccgatcgtaacactgcaagtgtgcctaccacatgcttcacgaccagatggagatgctcaatcgtatgtgacgtgtgagaacactttggattcgtttaaaatttgttggacttcaaaacctccaacgggatttgccacttttttggaactacctccatttttcttaaacagcaataaagcaaaacagggaccgccgggctgcagcccctggccccggagatgacggctggtgcccgtgcttgaggcgtcaggccagctcgcggtgccagcactgccaggctcggctggccacaggaaactgtcccaccgattcctgctgtttgttttttcttaaggcattgttcctcagacttcagaaaacccagccacaaaaatccaccagagcaataaaaaaaaaggcacaaactcgcatcttccgatggcttttgagaaactcaagccagctcccccagctcacattcctgtttctgtccagttttgttttctttaaaggtccctctgtcccccacccgggtgcagaccccccgccgcacaccgctatggttcacagaggcgggccacagccgtagaaaacgtcctctttaaaaaaaaataagctacaagatgagtcgagtggtttacacagagactgtggagttgtgggtaataaactttaagcaccagttttaatcaagtttgttttgtattattagatctttgatatttgttttctgtgcctcgtgtcaactgaattcggcagctcggccgcctgttgccacaggctcctttcttccacggcgtcccttgcgggacccgccagagtgtgcttggcttccgcgtgtccgtgtgtctgcgcgtcgccggcgtctgtcccgtgttccctgtgaggctgccacgcccaggcgtgcatgtgcgtctcgagacctgtgggcctgggcggcagaaaggcttcccgtggctgttgcacgctgggtgtccctgggtgctccaagagagccccacggtgggacgcaggcgtgacacgggaaagtttcttggctgagcttcaagacagagacagacagacaagagaacagcagcttcgagggagtgctacaggggcggctcctcttccatgggctcctcatctggtctcttttcggcgggcttcacgcccacggacagcgaggccatggcggtgaccgtctcggcttcttcgttctcgcaagtctgagcctcgatcagagaacgccccgctgtggaggttgtgcgctgcaggcagcgccagtacttgctgtggatctccatgactttctccatggaacggacagcgtttgcattgggtctttgctgtaaaaccttttctgggagaggatcaagctcgtttcccagcaaggcagaaacacatgcttccgaggcgtcgcaaatggcggtcaggtcgtggcctccctcgagggccaggacaatccggccgccagccaggcccatcagctgcttcgtcaggtacccgaagcatctggcggagaggttgtagcccccaagaggggtggggtggccctccacggcatcgaagcctgatgacaccagcaccacatccggggcaaactcgctggcgatcggcatgaccaccgttctgaaggccgccaagtactcagcgtctcccatgggggggtccaggccgccggtgaaagccatgttgacgttgaaacccacgccgggccctgtgcccacctcatcaggagccccgctgcctgggaagaagttcccatcgtcgtagcggtggagggacatgtacaggacgctggggtcgctgtagaaagcctgctgggtcccgtttccatggtgcacgtcccagtccacgatgaggatcttgctcacgctcaacctctgctgcagaagcttggctgccacggccacggagttgaagtagcaaaagcccatgggcgtgctctcctccgcatggtgtccaggggggcggaccacagcaaagccattcttcagctcccctgtggccaccttgaagaccagctctaccacgcagcccacagccaggcgggctgcccccgccgagtgcacctcgttccatatggtgtcactgtccaccccaacaccaccgcaagggagccggacgaacacggaggcgagcgagcctagaagtttcttactgtccagtttctgccggttgagggggttcgtgccatacaggagggtgtgggcttccgagtgcaccgtctgtagctcctccagggtggccttgcgtccgcggatgcactcgcatttgccccggaggcccgtctcctgcaggcgggaccagatgctctggatcctcccggcgtgctcggggtggctgctgctactcccgcaggtgcactggtgcttcagcatcagcgtgtcatacacgaggcctgtcgtgaacctcggcttggtggggggctcctgcacagacacggggaaggtggcagacgcgggtgaggactgcgcccgggacagaggcctgtggccgccgaaggacacggggatgccggcggcctccatggacgcctggtagttcctcagctggtggatccgctgctgctccagcaggagggcttgctgtctgaagagcagctcctgctcactgggctggcgctggcccggctccacctcccgtgggggctctgcctcttcctcatcgctctcaatgggctcctgcttcacctgcacgccggcctgtgcgtgcgcctccttctgccccggcagccggtccaggtagggctcgtccagcagagcctggtgctcacggagctcctcctccgtctcctccgggtggctctccggctgccgggctggctcgcttggcttggggatgatcttgttcatctgcagttgctgctgctggaactgctgcttgtgtttctccagaaactgctgatgctgctgctggatgaccaggtgctgcagagcctgggcgttctggggcagcggggccgactgggtccgccccagtgggcggtgctgccgcagcttgtggatggagggggacacccggtctgcaccaaccaaggactgtgcgtggaggggcagtgctcccaggcctgtgacgaggggtgcttgtgccggcggctgctccagtaagaccatgtgctgcagaagagggctgtgcgctgcccctccgtcccgctccaagggcgaggtgctcaggtagggagtgaggtgggtgccggggaaaagggagagcctctgctggagggcgggaagggtgagtctctcggcgtcctgctggcccgccgtgcccgcagaggggccggtggcaggcaggcccagcgtgatgttgggcaaggatggcgatgtgtagaggggaagtggagcggccgagccttctcgtgccacaagtctgtgcgccaaactcgtctccgccgggatgctggggacggcgggcgcgataccgttctccgcgctgacgctcccggagctgttgttgggtgagctgggtccggagcctggggcgctgctgcacgcggagtctgtgacatccaacggacgcttttttagagcagtgaccactggcccgtctttcctgcgtaacagggggctgctccgtctttcggccactttctgctttagcctggaccgtaatttcagattcggttcagaagctgttttcctaagagggaagtcatctttggcgtcgtacattcccaggaccgggtggttataggaggtcgacactccgctctggggtggagaactctggtcaagggaactgtgctgcgttttcccgtaccagtagcgagggtcgctggaaatgcagtggttcagattccggtgggccagcgccttctttttattgaggacaaattcttgtaacttcatcttcacttctgtgctggccacggcactctctttgcccttctccttgttcttgagctgctgcagcttctgctcccggtgctgcttctccagctcctgctcctggcggtgcctctccagcttccgctggtgttccagcagctcctgctggtgcttcatggccagcatctcctgttgttgcttgatgtgctcgtggagctgcgcctcgtgctgccgggagagctgctcgtgctgcctctggaactcagcgatgaggatctgcctctggatctgctgcttctgcttgagcgccaggagctcctgctgcagctgctgctcccgcagggccggctctgccacaggcagtgagaactggtggtccaggcgcaggtccatgggcactgccgagggggccacttgcagaggcagcgccgtggccacatccaccgtgctgggcatgtggttcacgcgggcaggattcagcagctccactggctggtctcggccagaaagtccatctccatccacagccagatactgcttccggaaccacacttcgtatccaggtgagctcgttttttgtatttcaaaagcacaaagatctatgttcatggtgtagtccaggcagagtgtggttaacaggcctccgggtgtcccccccttccagcccagtgcaggggttcagccgctgcagaaactccgaatctgctaacgtgaagtgccaagactgctgtccgccagcgccctcactcccccagggcctgtacctgtagcaggaggctcacgttccgagtcctcattgctcccagacccaagggcaaggctgtcacaggcgaaagacgggttccccttcctctacacccaagccctcggaagcacgctgcaggcccctggaggtgccacagtgctcccagctcccccagaggctgagttcaaacattctaaacggattcttgataacaagccgccggctcgctggaagacactgagcagttacataacagcacagaaaatcccttacaagtttcttaaaaaagagttaatcgtactgacttggtgctttaccttcagcccagactttcgcttaatcccggaaactgctccaaaggcgtttttctcagggcgttcggcgccgtaactcaggagaaacccaagtcctgctctcccggcggcctcgctggggaagaattcagccgctccaccctgacatctggtttctatttcatatccatgttgtcacattacataacaagcagatgatacgagagatcaccacagtgtttcggctcgagagtcacaaagaacgcccagaacactgtttatattgggggccatgaacgttcaccaaaccagacttagtgcagaggctgcacccttccaggctgaaacccagcacctacagcaaatgcccaaggaagcaagaagcgggaccccgccttctcagccacctctcactaacactcagctccactcctgcttccttcctctcactccacatccgagttagagggaaatacgatttatctctggcctgcatttacttctcctgcacctggcgggaggctctggccttgcaggcgtgcaggagcccctgccagtgagggccagcgaggggcccagggagaagatggaggtcaagtcatagggcctccaccgcaggcagagctccgccagcaagtatcctgggagctggggggcctcaagggaggcaatccccccacacaccatccccttccccttcgctcatctggggaagctgtgaggactggtgttgataaaacattccaaccacacactcagaccatggatgtggccgtgccagcagggaggccagcagcccctagcagaagggtgttctggaagctgccccctcccatgctgctgcctggtcccatggggcatgaagggagggtggccagggtggcccgagccagcatcaggcacaaggcccaaggagtttctccagagcagcctgtcctcttcggtccagaaaaagtcagattccacagcagggttagccgtccagttagggaacccactaaggggctctgtgcgtagaggtgctcagaatcaaaccactaaaccccaggaccccctgctgggggaatggtccgtggcagtcattcagccttggagtgaaccgttctgcccaagtgcaagtgagaacacaatacttcttattatatacagaattgccaaagccaacgtgattagtagaaaaaccgacatgtcagtgacttgggggtctggtttgccccagatgtgggtggaaaccccaggcgtccctcaagcctggtccagagctccacagacagcagatacacaaactctgagtgacagcattggtgtttagcagattctggattttgctcccccccgaaccaagtatagagaatgtttcacagagtagcttcaacagaaaatggccacagtgtgtctgtgagagagtgtgatgttcccggggggatggctggggccaagggaaggcccctcccatgagccctgcctccatgagactgcgtagggcaggactgccaggcagaaagaacacagcacaggcacaagggcagacccaggctggcagggctaaatggcttcaggagctcccccctctgccccccagggagtaaaggcaatgatgcaaatatgataagcaaacagaggtcccaaaacacagaaagggccaggaccctgatgccaaccaagcagacccaaaactgggtctgggagcacagggcagggtcgctgagtgcagaggggcctcactcaatgtccaacacttccctccaaaacagacatgctggtgagaggcttcaacccttccactggcctgacacctggatctctgctgccctgtgccaggttagccacgtccaacaccaccacggccaccggccatttaagaaaacgaaccctgacgttaacctgcttgagccctaatactaagcaagagcagcgccacaattccaaaactgcagagagcgccttttaaacattctgctgagatctgcgcggtcgcggtctgacaggcaggccttcttggctacctgtggtttcattccagcattaacaggcacctaaaaggcctgtgagcttttgtggggtcaagcagcatcagctccactttacaaccccgcagagtgaggtgttagctctgcagctccagggcagagccttgcagccttagggccagggggacggcctggccccttccgagctctcagcagcctgaactccacgtgtcccctgctgtgtcactggcatgctggtcttgcatggcactgagatgtgtggcacaagcaggcaccaagcccggagacacccgacgctcaccgttagactgggtagcatttgtcaagcgccgagcaaacagtggatgaagtgtcctcagccggcgtcagctgttctgatccgcagaacacataactcctggcactcctttccaagcatccgggaaatgtagaatccaagtgttacaccatccagttgaagatgacagatttacgatataaaacggcacccgcgactgaggactttgtaggaatggaggccgctgtcattatttcatgggtgagggggagagggacactgtgacccatgacaggaaaggacagctcagcccctccaaaaccacacacaggggactccgtttctcacaaaacttcaagtttctgttctacgcaaacattacaacacattttaaactacattctgacacgaagctcccgtgctttttaatggcaggtgttacaatgatcatggaacagtgatggggcggtgcttcctcacggtgacatggcagggagaagtctggaccggagccagcagggtccttgacctaagaggccttgggcagcccacggggcagctctgagcaatctcctgtgaaaggaagagctcagaacgggttcctctaaaggttccttccagagcaggggttctgtggttccctggggccctagactaacatgaggaaggggaaacagagaagaatgcccactaaaagccttacccaaaaattgaaagccaagaaaaatcacaccagatcatctcagtttagacttgaggaacctcggcgctgacatcactgtcaccatcacaaaacactggccaccaaggtgccacctaccacactgcaacctggaaggaggggcgggcaggggcacccctgggcagggcaggacaccaggccagccagccacccacgctacagaggaaatgcagcccctcccaactaagagaaccctggtaccatcaccacagccttggtgccagggctcctagcacctgacagggaagatgagaaggacattggctgccgccaagaggcctgctgcccacccccaactgcacggtggtggtgctgccagcaccaccatccatgctggcccaggagcccacacgcagggcacgcacgcacgtagttccacattaggccctttcttcctcaattgttggaaagaaggccaaagccagatgatggtgaaattcacgaggaaaatgtccccgactgtcctccattctaaagcaaacgctaagaatgggctgctgggcttcagcagaagccaagtcacctttcctctatgcgtccaatgaaacgaaaacatccacacttgtctttataaaaacggaaaactgcatctggaacaaggtctgtggcgtttcttccagcgtgtcccatggacatgaagttggtcttcctatgggtcctccaaggcacacccctcgactgcaccacagcactgagggcagaatgtggtggtggcccagctgccgtggcgccggcagactagcctggtacacggagaggggagcctgctgactgtgggtaggccacgttcccccagtgtcttcatctgcagagggagaccgggagcctctgaagaccgctccagctctgcactgtgggggcggccggccagcaggcaggcaatgctctcaggccccacgctcctctcactggctgccgacgggaggcagacgaggtgccgggggcagcctgcagagcaaggagtcaaggtggccagcctggggcagggtgttcccccagccagggagcttcactcaggcttgggctctgtcccgtgcctccccgggggcgttccgaggtggcggaggaggaagctgcagcccgttatccaccgcccagtctctccctctcaccagcacacagatgttctcagcggcagagcctggcttctgcctgaattcatttcatatttttaaatatgctcttaatggaaagcaacaaaagtacttaacaaaatgcgctgatgtaaatgtccctgcagcagccagggactaattttagaaggggctttgaggagaaacccaagggacactcacttgctggaaacggcctcctccccaaagagtgtgaggatctggattagaaccaagtatccccaggctgcccaggagcccgctcctccaattgggggctggccatcccaccgagcactgataccgcaggctggactcttcctaacctcacgagaggtgatgaccggaatcatcccagttttccatggcacttcgcaaacacagctggtcaggcccttagcacctcctgaccccccgatctcccagactctctgctggaagttaaggacacagagaaagtttcttatgaaaataagcgcctcaaaagaaagccaacgtacagcactggtgacagaaaggaagattcagaaaagccttcacgcctggcaatatggcacacgcacttttagagacgtctaattatactcagggctgagttggctgaagagtgaggaatatactccaaagacaggaattcaaggcagggcaaatagaacatgaaagccagcctggagcccagggcctgtcctggggcagccacctgcactgcctcttaccactgcaccgtccctgtgagtgtgcgtggggaggggctgtagttcccttggcaggggaagccagaagacaggcctgcaagggacacatccgggcctgggcttggtgctggctagaaggggtcaaatcgagagaggactcccctcagaactcataatcccagacccctcgcaatggtttggggagaattcagacaacccatgaggcctgatgagcatccctagcacctgcaaacacaggcatgtcccaggtggcacctcccagcaccaggcagaaaccttctctagaggaacacgctatgaacctcaaaaaaacatccaagaaggacggacataaagtcacaatcaagaaccatgggtagcgggagtaagtcccggaaagacctcagttgtaggaaaatcaggcactgacccaaaacacatacgaaggacactcgacaaaacaagagaggtcatccagggtcaggctggagctagaggcctccagatcctgtcacttagtgactgtacaaacctggtggcttcctcaacctccctgtgccttagcttcccatttgccaaaaagggggattagaagagcccacactctccctggagcaaggctaaggaagaaaggagacagatgtctcagctgttattattaataactatcagaagtgtcacatggatctgaatgatccaaatggaacttgtagaaacaaaactgtcatcattaaaatttaaaactaaatgagtgagttaactaatcaagtattaatagacagagctgaagagagaattagtgaacagtaaaatagcacggaagaaataaaccaggatgcaacacataaaggtaaagagatagaaagctggagacgttagaggactggaaggacagaggaagatatgctaacacacatctgtaaaccaaaaataaaattctaagctcccaaccatctgaatggacccctcctctcaagccaagggcattccaacattaacctgaaaagctagttcaggtcgtgatggggacgggcattcagatgtgcctcatgataccctcctcccttttggaattgctgatagaacagactctttaagtctgatgagaaacatttcagtctattctctctgaagcctgctacccggaggcttcgtcggcatggtaaatccttggtctccacaaacccttatcataatccagacattcctttgtgttgataataactctttcaaccaactgccaatcagaacattttaaaatctacctataatctgaaagcctcacacttcgagttgtcccgcgtttctggactggaccaatgttcatcttccacatactgacagacgcctcatgtctccctaaaaatgtatgaaaccaagctgttccccgaccaccttgggcacatgttgtcagcacctc

SEQ ID NO: 10217 - RNA, 7773 nt, Homo sapiens
  source 1..7773: mol_type = other RNA
caggaaggagacaggcagttcactgtgaattctgagtagtttccctaaaacactgtttccacataaatacaataaactctattattggtatgtcacaagtgctagataaactttttttcttaatatgacaaatgtttaagtagtcctttttatttttcttacaataaaaagtacaatttcttaagaataagttcaataagacgcaaacttccccgccctcctctccttcaaggttttgttttacagaaaaatttccatcttttgtatctgcaaatgtcatgagaggggaacagaaaggcatttttcttcttccccaaagctgccgagtttggcgtgcaaaatctgtatacaatataaagtcatgccggtcgtacagtccatgcaacctccaggtgtaggaaacttaaaaaaatatattcatatatatttatatctatatatttatatatgtatcaatgcccataaaacacgtgggcccaaagtctacaaaaagaagaatggaatgagcacgtggctgtgaccagtaaagaaggaatgttctgatcaaaaagaaaaacaacaaagtccattgctagtgctgcaaaaatcaaacttgcttttgtgtcagaccattacgaaatggtccttccccttgcaaacagattttcaaaagaagtaaagaaaaactgaaacaccttgacaaagtggccctccagaaccagagccctgggacgctggggaggggcggccagtcccagcgggccacggcctccgggacagccgcctgctggtggggcgtgggcacgtgggcacgctgcggcacggcgggaagccgcgagggcagggcagacgccaagaggcccagtggcgtcatcagggtttccctcaaagggatataaagtgctcgcttgctgactcccagccagtgcccccaaggcctttgcaaaggaagaaaaaggctaaaggtccaaggacccacagggagaacacatgaaggaaccctccctgacgtggtcccgcctgcagacgccgaggcagatcctctgccatctgccctggacgcttgctgtggagaagagccgagtgtgtcttcaaagaaaaggctacacagtaatgctctcagcacatttgtgaagctggagtgagctgacagatgaaacgtgcctccccctgccaggcctttgcagagggcgtctccatttgaatgagattagaattaagtccccccactgataacctggccactgagcagtccatgttatcccatcatctgcttaaaaaaaaaaagtgagatgatgcattcctccccataagccacggcggggtaagagggcaggtggcaggatccccagagggctatgcagagaatgaggccaaggaggccagaagagcctgctagctgggccctgccactgctctgtgccatgaatggggaatggaccagctcctcttgccaatctgggcttcagagcaaagagtggccaccagggaggggaaagtcaaacaagtcccaagaccgttctgcctgctctcaaaccactgtctcagagctgaccatcagcagcccagtgaccaagtgaatccaagaatctgcactcatttggtcaaaagtttgagttaatttcagaagctaccctgtaaactttaccaaactccgaaactcggctctgggtccctcctgagcacggtgtgtctgaacttctgcccccaagtctgaacccaatatacactttggaatgaaactggtggcttcatgtgctggaaaataagttaccagtaaaacgtgactgtcagttactgttgaagagaaaaagagtaaagactggctgtcctggtcaggcaatcataccctccctgcaggttcaccaggcaacaagggtccctgggttccttgcagccacaggctccaaaatccagggctggccacgtggctgcagtggaaaaacccaagtgggtaaagagccccacgtgtgccccatgcattgctgacatgctcaaaaggtctttggaaaactcaagttagaattctatcctgacgatgtggtcagagaagtttaaacatgagtttcattaatgctgactgcccccggcatctggcaagcctcccagggtggccgggcatcctaagcaaccctccctgcccttgccacggaggggaaaaacacaccacccctcgtaatactactagtgttgaaagttaaaaagagcccctgggcttctttatacagctcctaggacagaccaggaaagacacaatcgttggtgtcactccgaaaagacctacggtccctcctctcactttctgaaaatagaatctgacagcaacaattctgtacgctgcagaaaactcatcgtacaaaaataaaaacaaaaataattaaaaacctttgaaaggtaaaaaaaaatgtacaagcaagaattcagaaaggaaaaagatttagacattattaccattcagaaaattgctaaatggtgaggaaaaatgtaaaattcataaaacaatgcttattcaggatctttttgtgaaaaaattcatacaaaaatcaacagcaaatttatattctttgctataaaaactcattaggtacatatgtgcatgaaggcttggagacgggagcggttctgttagaaaataattaaaatgaaagtacaaacttgtagggtagttgcccagtggcgaatgtgttggcgatctgaaatctagccaatctggagcttgagaaaacatgaatttcaatcaatcaggatccctttccataagcaccttgagagcaaattcacaagccatccatttgcagggaccttcgcaatctgcattcattttatatatatatatatactttttctataaatgcattataaatattttatcaagatttcataagaatcaagtaagtttcttagcttggaatacattggaatatatattatacatatatatatttatttatacctaaaatttaagcaatacttcatgctacttgcttttaataaaaagcattccgatcgtaacactgcaagtgtgcctaccacatgcttcacgaccagatggagatgctcaatcgtatgtgacgtgtgagaacactttggattcgtttaaaatttgttggacttcaaaacctccaacgggatttgccacttttttggaactacctccatttttcttaaacagcaataaagcaaaacagggaccgccgggctgcagcccctggccccggagatgacggctggtgcccgtgcttgaggcgtcaggccagctcgcggtgccagcactgccaggctcggctggccacaggaaactgtcccaccgattcctgctgtttgttttttcttaaggcattgttcctcagacttcagaaaacccagccacaaaaatccaccagagcaataaaaaaaaaggcacaaactcgcatcttccgatggcttttgagaaactcaagccagctcccccagctcacattcctgtttctgtccagttttgttttctttaaaggtccctctgtcccccacccgggtgcagaccccccgccgcacaccgctatggttcacagaggcgggccacagccgtagaaaacgtcctctttaaaaaaaaataagctacaagatgagtcgagtggtttacacagagactgtggagttgtgggtaataaactttaagcaccagttttaatcaagtttgttttgtattattagatctttgatatttgttttctgtgcctcgtgtcaactgaattcggcagctcggccgcctgttgccacaggctcctttcttccacggcgtcccttgcgggacccgccagagtgtgcttggcttccgcgtgtccgtgtgtctgcgcgtcgccggcgtctgtcccgtgttccctgtgaggctgccacgcccaggcgtgcatgtgcgtctcgagacctgtgggcctgggcggcagaaaggcttcccgtggctgttgcacgctgggtgtccctgggtgctccaagagagccccacggtgggacgcaggcgtgacacgggaaagtttcttggctgagcttcaagacagagacagacagacaagagaacagcagcttcgagggagtgctacaggggcggctcctcttccatgggctcctcatctggtctcttttcggcgggcttcacgcccacggacagcgaggccatggcggtgaccgtctcggcttcttcgttctcgcaagtctgagcctcgatcagagaacgccccgctgtggaggttgtgcgctgcaggcagcgccagtacttgctgtggatctccatgactttctccatggaacggacagcgtttgcattgggtctttgctgtaaaaccttttctgggagaggatcaagctcgtttcccagcaaggcagaaacacatgcttccgaggcgtcgcaaatggcggtcaggtcgtggcctccctcgagggccaggacaatccggccgccagccaggcccatcagctgcttcgtcaggtacccgaagcatctggcggagaggttgtagcccccaagaggggtggggtggccctccacggcatcgaagcctgatgacaccagcaccacatccggggcaaactcgctggcgatcggcatgaccaccgttctgaaggccgccaagtactcagcgtctcccatgggggggtccaggccgccggtgaaagccatgttgacgttgaaacccacgccgggccctgtgcccacctcatcaggagccccgctgcctgggaagaagttcccatcgtcgtagcggtggagggacatgtacaggacgctggggtcgctgtagaaagcctgctgggtcccgtttccatggtgcacgtcccagtccacgatgaggatcttgctcacgctcaacctctgctgcagaagcttggctgccacggccacggagttgaagtagcaaaagcccatgggcgtgctctcctccgcatggtgtccaggggggcggaccacagcaaagccattcttcagctcccctgtggccaccttgaagaccagctctaccacgcagcccacagccaggcgggctgcccccgccgagtgcacctcgttccatatggtgtcactgtccaccccaacaccaccgcaagggagccggacgaacacggaggcgagcgagcctagaagtttcttactgtccagtttctgccggttgagggggttcgtgccatacaggagggtgtgggcttccgagtgcaccgtctgtagctcctccagggtggccttgcgtccgcggatgcactcgcatttgccccggaggcccgtctcctgcaggcgggaccagatgctctggatcctcccggcgtgctcggggtggctgctgctactcccgcaggtgcactggtgcttcagcatcagcgtgtcatacacgaggcctgtcgtgaacctcggcttggtggggggctcctgcacagacacggggaaggtggcagacgcgggtgaggactgcgcccgggacagaggcctgtggccgccgaaggacacggggatgccggcggcctccatggacgcctggtagttcctcagctggtggatccgctgctgctccagcaggagggcttgctgtctgaagagcagctcctgctcactgggctggcgctggcccggctccacctcccgtgggggctctgcctcttcctcatcgctctcaatgggctcctgcttcacctgcacgccggcctgtgcgtgcgcctccttctgccccggcagccggtccaggtagggctcgtccagcagagcctggtgctcacggagctcctcctccgtctcctccgggtggctctccggctgccgggctggctcgcttggcttggggatgatcttgttcatctgcagttgctgctgctggaactgctgcttgtgtttctccagaaactgctgatgctgctgctggatgaccaggtgctgcagagcctgggcgttctggggcagcggggccgactgggtccgccccagtgggcggtgctgccgcagcttgtggatggagggggacacccggtctgcaccaaccaaggactgtgcgtggaggggcagtgctcccaggcctgtgacgaggggtgcttgtgccggcggctgctccagtaagaccatgtgctgcagaagagggctgtgcgctgcccctccgtcccgctccaagggcgaggtgctcaggtagggagtgaggtgggtgccggggaaaagggagagcctctgctggagggcgggaagggtgagtctctcggcgtcctgctggcccgccgtgcccgcagaggggccggtggcaggcaggcccagcgtgatgttgggcaaggatggcgatgtgtagaggggaagtggagcggccgagccttctcgtgccacaagtctgtgcgccaaactcgtctccgccgggatgctggggacggcgggcgcgataccgttctccgcgctgacgctcccggagctgttgttgggtgagctgggtccggagcctggggcgctgctgcacgcggagtctgtgacatccaacggacgcttttttagagcagtgaccactggcccgtctttcctgcgtaacagggggctgctccgtctttcggccactttctgctttagcctggaccgtaatttcagattcggttcagaagctgttttcctaagagggaagtcatctttggcgtcgtacattcccaggaccgggtggttataggaggtcgacactccgctctggggtggagaactctggtcaagggaactgtgctgcgttttcccgtaccagtagcgagggtcgctggaaatgcagtggttcagattccggtgggccagcgccttctttttattgaggacaaattcttgtaacttcatcttcacttctgtgctggccacggcactctctttgcccttctccttgttcttgagctgctgcagcttctgctcccggtgctgcttctccagctcctgctcctggcggtgcctctccagcttccgctggtgttccagcagctcctgctggtgcttcatggccagcatctcctgttgttgcttgatgtgctcgtggagctgcgcctcgtgctgccgggagagctgctcgtgctgcctctggaactcagcgatgaggatctgcctctggatctgctgcttctgcttgagcgccaggagctcctgctgcagctgctgctcccgcagggccggctctgccacaggcagtgagaactggtggtccaggcgcaggtccatgggcactgccgagggggccacttgcagaggcagcgccgtggccacatccaccgtgctgggcatgtggttcacgcgggcaggattcagcagctccactggctggtctcggccagaaagtccatctggatggctttgggagctcattgctagcaatgtccactcctttaagtgattcgaaatggctcaaaatttccacggaaacgatagctccaacgagctccaaactcccaccaacacatacaagtaccgggacggtgagggctgggtcacagacgttcaagcgccgagcctcgccggcaaggtctcatgagccaggtaacccacaagttgaacagaggcgtccgctggcttctgcagatgaaccaaaagacgctccaggcgccagccgctgggtgcttcgcggttgaggaggcgcagggaccgggggccagtagtggccgtaaacacgggccccggccgtgtccggtcgcactcggtagcccgcatggctgcctagcggtcagcaccgcatgtctgcgagcctaattcgcgcttagagggcacacaatggggtgcaggctaacgcggggagccggccaggcctcgccgcggcgtccatcttggatactggc

SEQ ID NO: 10218 - RNA, 8169 nt, Homo sapiens
  source 1..8169: mol_type = other RNA
caggaaggagacaggcagttcactgtgaattctgagtagtttccctaaaacactgtttccacataaatacaataaactctattattggtatgtcacaagtgctagataaactttttttcttaatatgacaaatgtttaagtagtcctttttatttttcttacaataaaaagtacaatttcttaagaataagttcaataagacgcaaacttccccgccctcctctccttcaaggttttgttttacagaaaaatttccatcttttgtatctgcaaatgtcatgagaggggaacagaaaggcatttttcttcttccccaaagctgccgagtttggcgtgcaaaatctgtatacaatataaagtcatgccggtcgtacagtccatgcaacctccaggtgtaggaaacttaaaaaaatatattcatatatatttatatctatatatttatatatgtatcaatgcccataaaacacgtgggcccaaagtctacaaaaagaagaatggaatgagcacgtggctgtgaccagtaaagaaggaatgttctgatcaaaaagaaaaacaacaaagtccattgctagtgctgcaaaaatcaaacttgcttttgtgtcagaccattacgaaatggtccttccccttgcaaacagattttcaaaagaagtaaagaaaaactgaaacaccttgacaaagtggccctccagaaccagagccctgggacgctggggaggggcggccagtcccagcgggccacggcctccgggacagccgcctgctggtggggcgtgggcacgtgggcacgctgcggcacggcgggaagccgcgagggcagggcagacgccaagaggcccagtggcgtcatcagggtttccctcaaagggatataaagtgctcgcttgctgactcccagccagtgcccccaaggcctttgcaaaggaagaaaaaggctaaaggtccaaggacccacagggagaacacatgaaggaaccctccctgacgtggtcccgcctgcagacgccgaggcagatcctctgccatctgccctggacgcttgctgtggagaagagccgagtgtgtcttcaaagaaaaggctacacagtaatgctctcagcacatttgtgaagctggagtgagctgacagatgaaacgtgcctccccctgccaggcctttgcagagggcgtctccatttgaatgagattagaattaagtccccccactgataacctggccactgagcagtccatgttatcccatcatctgcttaaaaaaaaaaagtgagatgatgcattcctccccataagccacggcggggtaagagggcaggtggcaggatccccagagggctatgcagagaatgaggccaaggaggccagaagagcctgctagctgggccctgccactgctctgtgccatgaatggggaatggaccagctcctcttgccaatctgggcttcagagcaaagagtggccaccagggaggggaaagtcaaacaagtcccaagaccgttctgcctgctctcaaaccactgtctcagagctgaccatcagcagcccagtgaccaagtgaatccaagaatctgcactcatttggtcaaaagtttgagttaatttcagaagctaccctgtaaactttaccaaactccgaaactcggctctgggtccctcctgagcacggtgtgtctgaacttctgcccccaagtctgaacccaatatacactttggaatgaaactggtggcttcatgtgctggaaaataagttaccagtaaaacgtgactgtcagttactgttgaagagaaaaagagtaaagactggctgtcctggtcaggcaatcataccctccctgcaggttcaccaggcaacaagggtccctgggttccttgcagccacaggctccaaaatccagggctggccacgtggctgcagtggaaaaacccaagtgggtaaagagccccacgtgtgccccatgcattgctgacatgctcaaaaggtctttggaaaactcaagttagaattctatcctgacgatgtggtcagagaagtttaaacatgagtttcattaatgctgactgcccccggcatctggcaagcctcccagggtggccgggcatcctaagcaaccctccctgcccttgccacggaggggaaaaacacaccacccctcgtaatactactagtgttgaaagttaaaaagagcccctgggcttctttatacagctcctaggacagaccaggaaagacacaatcgttggtgtcactccgaaaagacctacggtccctcctctcactttctgaaaatagaatctgacagcaacaattctgtacgctgcagaaaactcatcgtacaaaaataaaaacaaaaataattaaaaacctttgaaaggtaaaaaaaaatgtacaagcaagaattcagaaaggaaaaagatttagacattattaccattcagaaaattgctaaatggtgaggaaaaatgtaaaattcataaaacaatgcttattcaggatctttttgtgaaaaaattcatacaaaaatcaacagcaaatttatattctttgctataaaaactcattaggtacatatgtgcatgaaggcttggagacgggagcggttctgttagaaaataattaaaatgaaagtacaaacttgtagggtagttgcccagtggcgaatgtgttggcgatctgaaatctagccaatctggagcttgagaaaacatgaatttcaatcaatcaggatccctttccataagcaccttgagagcaaattcacaagccatccatttgcagggaccttcgcaatctgcattcattttatatatatatatatactttttctataaatgcattataaatattttatcaagatttcataagaatcaagtaagtttcttagcttggaatacattggaatatatattatacatatatatatttatttatacctaaaatttaagcaatacttcatgctacttgcttttaataaaaagcattccgatcgtaacactgcaagtgtgcctaccacatgcttcacgaccagatggagatgctcaatcgtatgtgacgtgtgagaacactttggattcgtttaaaatttgttggacttcaaaacctccaacgggatttgccacttttttggaactacctccatttttcttaaacagcaataaagcaaaacagggaccgccgggctgcagcccctggccccggagatgacggctggtgcccgtgcttgaggcgtcaggccagctcgcggtgccagcactgccaggctcggctggccacaggaaactgtcccaccgattcctgctgtttgttttttcttaaggcattgttcctcagacttcagaaaacccagccacaaaaatccaccagagcaataaaaaaaaaggcacaaactcgcatcttccgatggcttttgagaaactcaagccagctcccccagctcacattcctgtttctgtccagttttgttttctttaaaggtccctctgtcccccacccgggtgcagaccccccgccgcacaccgctatggttcacagaggcgggccacagccgtagaaaacgtcctctttaaaaaaaaataagctacaagatgagtcgagtggtttacacagagactgtggagttgtgggtaataaactttaagcaccagttttaatcaagtttgttttgtattattagatctttgatatttgttttctgtgcctcgtgtcaactgaattcggcagctcggccgcctgttgccacaggctcctttcttccacggcgtcccttgcgggacccgccagagtgtgcttggcttccgcgtgtccgtgtgtctgcgcgtcgccggcgtctgtcccgtgttccctgtgaggctgccacgcccaggcgtgcatgtgcgtctcgagacctgtgggcctgggcggcagaaaggcttcccgtggctgttgcacgctgggtgtccctgggtgctccaagagagccccacggtgggacgcaggcgtgacacgggaaagtttcttggctgagcttcaagacagagacagacagacaagagaacagcagcttcgagggagtgctacaggggcggctcctcttccatgggctcctcatctggtctcttttcggcgggcttcacgcccacggacagcgaggccatggcggtgaccgtctcggcttcttcgttctcgcaagtctgagcctcgatcagagaacgccccgctgtggaggttgtgcgctgcaggcagcgccagtacttgctgtggatctccatgactttctccatggaacggacagcgtttgcattgggtctttgctgtaaaaccttttctgggagaggatcaagctcgtttcccagcaaggcagaaacacatgcttccgaggcgtcgcaaatggcggtcaggtcgtggcctccctcgagggccaggacaatccggccgccagccaggcccatcagctgcttcgtcaggtacccgaagcatctggcggagaggttgtagcccccaagaggggtggggtggccctccacggcatcgaagcctgatgacaccagcaccacatccggggcaaactcgctggcgatcggcatgaccaccgttctgaaggccgccaagtactcagcgtctcccatgggggggtccaggccgccggtgaaagccatgttgacgttgaaacccacgccgggccctgtgcccacctcatcaggagccccgctgcctgggaagaagttcccatcgtcgtagcggtggagggacatgtacaggacgctggggtcgctgtagaaagcctgctgggtcccgtttccatggtgcacgtcccagtccacgatgaggatcttgctcacgctcaacctctgctgcagaagcttggctgccacggccacggagttgaagtagcaaaagcccatgggcgtgctctcctccgcatggtgtccaggggggcggaccacagcaaagccattcttcagctcccctgtggccaccttgaagaccagctctaccacgcagcccacagccaggcgggctgcccccgccgagtgcacctcgttccatatggtgtcactgtccaccccaacaccaccgcaagggagccggacgaacacggaggcgagcgagcctagaagtttcttactgtccagtttctgccggttgagggggttcgtgccatacaggagggtgtgggcttccgagtgcaccgtctgtagctcctccagggtggccttgcgtccgcggatgcactcgcatttgccccggaggcccgtctcctgcaggcgggaccagatgctctggatcctcccggcgtgctcggggtggctgctgctactcccgcaggtgcactggtgcttcagcatcagcgtgtcatacacgaggcctgtcgtgaacctcggcttggtggggggctcctgcacagacacggggaaggtggcagacgcgggtgaggactgcgcccgggacagaggcctgtggccgccgaaggacacggggatgccggcggcctccatggacgcctggtagttcctcagctggtggatccgctgctgctccagcaggagggcttgctgtctgaagagcagctcctgctcactgggctggcgctggcccggctccacctcccgtgggggctctgcctcttcctcatcgctctcaatgggctcctgcttcacctgcacgccggcctgtgcgtgcgcctccttctgccccggcagccggtccaggtagggctcgtccagcagagcctggtgctcacggagctcctcctccgtctcctccgggtggctctccggctgccgggctggctcgcttggcttggggatgatcttgttcatctgcagttgctgctgctggaactgctgcttgtgtttctccagaaactgctgatgctgctgctggatgaccaggtgctgcagagcctgggcgttctggggcagcggggccgactgggtccgccccagtgggcggtgctgccgcagcttgtggatggagggggacacccggtctgcaccaaccaaggactgtgcgtggaggggcagtgctcccaggcctgtgacgaggggtgcttgtgccggcggctgctccagtaagaccatgtgctgcagaagagggctgtgcgctgcccctccgtcccgctccaagggcgaggtgctcaggtagggagtgaggtgggtgccggggaaaagggagagcctctgctggagggcgggaagggtgagtctctcggcgtcctgctggcccgccgtgcccgcagaggggccggtggcaggcaggcccagcgtgatgttgggcaaggatggcgatgtgtagaggggaagtggagcggccgagccttctcgtgccacaagtctgtgcgccaaactcgtctccgccgggatgctggggacggcgggcgcgataccgttctccgcgctgacgctcccggagctgttgttgggtgagctgggtccggagcctggggcgctgctgcacgcggagtctgtgacatccaacggacgcttttttagagcagtgaccactggcccgtctttcctgcgtaacagggggctgctccgtctttcggccactttctgctttagcctggaccgtaatttcagattcggttcagaagctgttttcctaagagggaagtcatctttggcgtcgtacattcccaggaccgggtggttataggaggtcgacactccgctctggggtggagaactctggtcaagggaactgtgctgcgttttcccgtaccagtagcgagggtcgctggaaatgcagtggttcagattccggtgggccagcgccttctttttattgaggacaaattcttgtaacttcatcttcacttctgtgctggccacggcactctctttgcccttctccttgttcttgagctgctgcagcttctgctcccggtgctgcttctccagctcctgctcctggcggtgcctctccagcttccgctggtgttccagcagctcctgctggtgcttcatggccagcatctcctgttgttgcttgatgtgctcgtggagctgcgcctcgtgctgccgggagagctgctcgtgctgcctctggaactcagcgatgaggatctgcctctggatctgctgcttctgcttgagcgccaggagctcctgctgcagctgctgctcccgcagggccggctctgccacaggcagtgagaactggtggtccaggcgcaggtccatgggcactgccgagggggccacttgcagaggcagcgccgtggccacatccaccgtgctgggcatgtggttcacgcgggcaggattcagcagctccactggctggtctcggccagaaagtccatctggatggctttgggagctcattgctagcaatgtccactcctttaagtgattcgaaatggctcaaaatttccacggaaacgatagctccaacgagctccaaactcccaccaacacatacaagtaccgggacggtgagggctgggtcacagacgttcaagcgccgagcctcgccggcaaggtctcatgagccaggtaacccacaagttgaacagaggcgtccgctggcttctgcagatgaacctgctcggggggcgcgggccccgcaccgggagacggcgccgctgcctgccgtgcccacccccgcgcccccgccccggcgggcgaagccgcctcgcggcgcgggtggaaaggtccagaaggggccgggcggccctggggaccggcgggtcccacggcgcgcggccagcgctggcccccgcctcccacggccgcgcgcggggcgggtgtggaccggcggcgtccacctgccgcgggctccaaggcctgcaggctgcgcggggcgcggggcgggcggcggacaatggcccgcgggcgccgggccggggctgcgcttaccgcggcgggcggcggcggccggctctagccctgctccggcgctccgcgccgcatctcctcagcctgcgccgccacccgccggcgcgcgggctcgggctcgggcggcgacagccgggacgcggccacggcgccgccgggggcccaggctgggaggctgttcgggcggcggcggcggcggcgcgggcgggtgcgcgggctcgggctcgggctcgggcggcggcggggacggtgctccgcggcggcggccccacaacctcccctcctcattcacaaaaaattgacccacgttgaaccatgatgcttctccccactccagcgtcgagccaggc

SEQ ID NO: 10219 - RNA, 7568 nt, Homo sapiens
  source 1..7568: mol_type = other RNA
caggaaggagacaggcagttcactgtgaattctgagtagtttccctaaaacactgtttccacataaatacaataaactctattattggtatgtcacaagtgctagataaactttttttcttaatatgacaaatgtttaagtagtcctttttatttttcttacaataaaaagtacaatttcttaagaataagttcaataagacgcaaacttccccgccctcctctccttcaaggttttgttttacagaaaaatttccatcttttgtatctgcaaatgtcatgagaggggaacagaaaggcatttttcttcttccccaaagctgccgagtttggcgtgcaaaatctgtatacaatataaagtcatgccggtcgtacagtccatgcaacctccaggtgtaggaaacttaaaaaaatatattcatatatatttatatctatatatttatatatgtatcaatgcccataaaacacgtgggcccaaagtctacaaaaagaagaatggaatgagcacgtggctgtgaccagtaaagaaggaatgttctgatcaaaaagaaaaacaacaaagtccattgctagtgctgcaaaaatcaaacttgcttttgtgtcagaccattacgaaatggtccttccccttgcaaacagattttcaaaagaagtaaagaaaaactgaaacaccttgacaaagtggccctccagaaccagagccctgggacgctggggaggggcggccagtcccagcgggccacggcctccgggacagccgcctgctggtggggcgtgggcacgtgggcacgctgcggcacggcgggaagccgcgagggcagggcagacgccaagaggcccagtggcgtcatcagggtttccctcaaagggatataaagtgctcgcttgctgactcccagccagtgcccccaaggcctttgcaaaggaagaaaaaggctaaaggtccaaggacccacagggagaacacatgaaggaaccctccctgacgtggtcccgcctgcagacgccgaggcagatcctctgccatctgccctggacgcttgctgtggagaagagccgagtgtgtcttcaaagaaaaggctacacagtaatgctctcagcacatttgtgaagctggagtgagctgacagatgaaacgtgcctccccctgccaggcctttgcagagggcgtctccatttgaatgagattagaattaagtccccccactgataacctggccactgagcagtccatgttatcccatcatctgcttaaaaaaaaaaagtgagatgatgcattcctccccataagccacggcggggtaagagggcaggtggcaggatccccagagggctatgcagagaatgaggccaaggaggccagaagagcctgctagctgggccctgccactgctctgtgccatgaatggggaatggaccagctcctcttgccaatctgggcttcagagcaaagagtggccaccagggaggggaaagtcaaacaagtcccaagaccgttctgcctgctctcaaaccactgtctcagagctgaccatcagcagcccagtgaccaagtgaatccaagaatctgcactcatttggtcaaaagtttgagttaatttcagaagctaccctgtaaactttaccaaactccgaaactcggctctgggtccctcctgagcacggtgtgtctgaacttctgcccccaagtctgaacccaatatacactttggaatgaaactggtggcttcatgtgctggaaaataagttaccagtaaaacgtgactgtcagttactgttgaagagaaaaagagtaaagactggctgtcctggtcaggcaatcataccctccctgcaggttcaccaggcaacaagggtccctgggttccttgcagccacaggctccaaaatccagggctggccacgtggctgcagtggaaaaacccaagtgggtaaagagccccacgtgtgccccatgcattgctgacatgctcaaaaggtctttggaaaactcaagttagaattctatcctgacgatgtggtcagagaagtttaaacatgagtttcattaatgctgactgcccccggcatctggcaagcctcccagggtggccgggcatcctaagcaaccctccctgcccttgccacggaggggaaaaacacaccacccctcgtaatactactagtgttgaaagttaaaaagagcccctgggcttctttatacagctcctaggacagaccaggaaagacacaatcgttggtgtcactccgaaaagacctacggtccctcctctcactttctgaaaatagaatctgacagcaacaattctgtacgctgcagaaaactcatcgtacaaaaataaaaacaaaaataattaaaaacctttgaaaggtaaaaaaaaatgtacaagcaagaattcagaaaggaaaaagatttagacattattaccattcagaaaattgctaaatggtgaggaaaaatgtaaaattcataaaacaatgcttattcaggatctttttgtgaaaaaattcatacaaaaatcaacagcaaatttatattctttgctataaaaactcattaggtacatatgtgcatgaaggcttggagacgggagcggttctgttagaaaataattaaaatgaaagtacaaacttgtagggtagttgcccagtggcgaatgtgttggcgatctgaaatctagccaatctggagcttgagaaaacatgaatttcaatcaatcaggatccctttccataagcaccttgagagcaaattcacaagccatccatttgcagggaccttcgcaatctgcattcattttatatatatatatatactttttctataaatgcattataaatattttatcaagatttcataagaatcaagtaagtttcttagcttggaatacattggaatatatattatacatatatatatttatttatacctaaaatttaagcaatacttcatgctacttgcttttaataaaaagcattccgatcgtaacactgcaagtgtgcctaccacatgcttcacgaccagatggagatgctcaatcgtatgtgacgtgtgagaacactttggattcgtttaaaatttgttggacttcaaaacctccaacgggatttgccacttttttggaactacctccatttttcttaaacagcaataaagcaaaacagggaccgccgggctgcagcccctggccccggagatgacggctggtgcccgtgcttgaggcgtcaggccagctcgcggtgccagcactgccaggctcggctggccacaggaaactgtcccaccgattcctgctgtttgttttttcttaaggcattgttcctcagacttcagaaaacccagccacaaaaatccaccagagcaataaaaaaaaaggcacaaactcgcatcttccgatggcttttgagaaactcaagccagctcccccagctcacattcctgtttctgtccagttttgttttctttaaaggtccctctgtcccccacccgggtgcagaccccccgccgcacaccgctatggttcacagaggcgggccacagccgtagaaaacgtcctctttaaaaaaaaataagctacaagatgagtcgagtggtttacacagagactgtggagttgtgggtaataaactttaagcaccagttttaatcaagtttgttttgtattattagatctttgatatttgttttctgtgcctcgtgtcaactgaattcggcagctcggccgcctgttgccacaggctcctttcttccacggcgtcccttgcgggacccgccagagtgtgcttggcttccgcgtgtccgtgtgtctgcgcgtcgccggcgtctgtcccgtgttccctgtgaggctgccacgcccaggcgtgcatgtgcgtctcgagacctgtgggcctgggcggcagaaaggcttcccgtggctgttgcacgctgggtgtccctgggtgctccaagagagccccacggtgggacgcaggcgtgacacgggaaagtttcttggctgagcttcaagacagagacagacagacaagagaacagcagcttcgagggagtgctacaggggcggctcctcttccatgggctcctcatctggtctcttttcggcgggcttcacgcccacggacagcgaggccatggcggtgaccgtctcggcttcttcgttctcgcaagtctgagcctcgatcagagaacgccccgctgtggaggttgtgcgctgcaggcagcgccagtacttgctgtggatctccatgactttctccatggaacggacagcgtttgcattgggtctttgctgtaaaaccttttctgggagaggatcaagctcgtttcccagcaaggcagaaacacatgcttccgaggcgtcgcaaatggcggtcaggtcgtggcctccctcgagggccaggacaatccggccgccagccaggcccatcagctgcttcgtcaggtacccgaagcatctggcggagaggttgtagcccccaagaggggtggggtggccctccacggcatcgaagcctgatgacaccagcaccacatccggggcaaactcgctggcgatcggcatgaccaccgttctgaaggccgccaagtactcagcgtctcccatgggggggtccaggccgccggtgaaagccatgttgacgttgaaacccacgccgggccctgtgcccacctcatcaggagccccgctgcctgggaagaagttcccatcgtcgtagcggtggagggacatgtacaggacgctggggtcgctgtagaaagcctgctgggtcccgtttccatggtgcacgtcccagtccacgatgaggatcttgctcacgctcaacctctgctgcagaagcttggctgccacggccacggagttgaagtagcaaaagcccatgggcgtgctctcctccgcatggtgtccaggggggcggaccacagcaaagccattcttcagctcccctgtggccaccttgaagaccagctctaccacgcagcccacagccaggcgggctgcccccgccgagtgcacctcgttccatatggtgtcactgtccaccccaacaccaccgcaagggagccggacgaacacggaggcgagcgagcctagaagtttcttactgtccagtttctgccggttgagggggttcgtgccatacaggagggtgtgggcttccgagtgcaccgtctgtagctcctccagggtggccttgcgtccgcggatgcactcgcatttgccccggaggcccgtctcctgcaggcgggaccagatgctctggatcctcccggcgtgctcggggtggctgctgctactcccgcaggtgcactggtgcttcagcatcagcgtgtcatacacgaggcctgtcgtgaacctcggcttggtggggggctcctgcacagacacggggaaggtggcagacgcgggtgaggactgcgcccgggacagaggcctgtggccgccgaaggacacggggatgccggcggcctccatggacgcctggtagttcctcagctggtggatccgctgctgctccagcaggagggcttgctgtctgaagagcagctcctgctcactgggctggcgctggcccggctccacctcccgtgggggctctgcctcttcctcatcgctctcaatgggctcctgcttcacctgcacgccggcctgtgcgtgcgcctccttctgccccggcagccggtccaggtagggctcgtccagcagagcctggtgctcacggagctcctcctccgtctcctccgggtggctctccggctgccgggctggctcgcttggcttggggatgatcttgttcatctgcagttgctgctgctggaactgctgcttgtgtttctccagaaactgctgatgctgctgctggatgaccaggtgctgcagagcctgggcgttctggggcagcggggccgactgggtccgccccagtgggcggtgctgccgcagcttgtggatggagggggacacccggtctgcaccaaccaaggactgtgcgtggaggggcagtgctcccaggcctgtgacgaggggtgcttgtgccggcggctgctccagtaagaccatgtgctgcagaagagggctgtgcgctgcccctccgtcccgctccaagggcgaggtgctcaggtagggagtgaggtgggtgccggggaaaagggagagcctctgctggagggcgggaagggtgagtctctcggcgtcctgctggcccgccgtgcccgcagaggggccggtggcaggcaggcccagcgtgatgttgggcaaggatggcgatgtgtagaggggaagtggagcggccgagccttctcgtgccacaagtctgtgcgccaaactcgtctccgccgggatgctggggacggcgggcgcgataccgttctccgcgctgacgctcccggagctgttgttgggtgagctgggtccggagcctggggcgctgctgcacgcggagtctgtgacatccaacggacgcttttttagagcagtgaccactggcccgtctttcctgcgtaacagggggctgctccgtctttcggccactttctgctttagcctggaccgtaatttcagattcggttcagaagctgttttcctaagagggaagtcatctttggcgtcgtacattcccaggaccgggtggttataggaggtcgacactccgctctggggtggagaactctggtcaagggaactgtgctgcgttttcccgtaccagtagcgagggtcgctggaaatgcagtggttcagattccggtgggccagcgccttctttttattgaggacaaattcttgtaacttcatcttcacttctgtgctggccacggcactctctttgcccttctccttgttcttgagctgctgcagcttctgctcccggtgctgcttctccagctcctgctcctggcggtgcctctccagcttccgctggtgttccagcagctcctgctggtgcttcatggccagcatctcctgttgttgcttgatgtgctcgtggagctgcgcctcgtgctgccgggagagctgctcgtgctgcctctggaactcagcgatgaggatctgcctctggatctgctgcttctgcttgagcgccaggagctcctgctgcagctgctgctcccgcagggccggctctgccacaggcagtgagaactggtggtccaggcgcaggtccatgggcactgccgagggggccacttgcagaggcagcgccgtggccacatccaccgtgctgggcatgtggttcacgcgggcaggattcagcagctccactggctggtctcggccagaaagtccatctggatggctttgggagctcattgctagcaatgtccactcctttaagtgattcgaaatggctcaaaatttccacggaaacgatagctccaacgagctccaaactcccaccaacacatacaagtaccgggacggtgagggctgggtcacagacgttcaagcgccgagcctcgccggcaaggtctcatgagccaggtaacccacaagttgaacagaggcgtccgctggcttctgcagatgaacgttgaaccatgatgcttctccccactccagcgtcgagccaggc

SEQ ID NO: 10220 - RNA, 14044 nt, Homo sapiens
  source 1..14044: mol_type = other RNA
caggaaggagacaggcagttcactgtgaattctgagtagtttccctaaaacactgtttccacataaatacaataaactctattattggtatgtcacaagtgctagataaactttttttcttaatatgacaaatgtttaagtagtcctttttatttttcttacaataaaaagtacaatttcttaagaataagttcaataagacgcaaacttccccgccctcctctccttcaaggttttgttttacagaaaaatttccatcttttgtatctgcaaatgtcatgagaggggaacagaaaggcatttttcttcttccccaaagctgccgagtttggcgtgcaaaatctgtatacaatataaagtcatgccggtcgtacagtccatgcaacctccaggtgtaggaaacttaaaaaaatatattcatatatatttatatctatatatttatatatgtatcaatgcccataaaacacgtgggcccaaagtctacaaaaagaagaatggaatgagcacgtggctgtgaccagtaaagaaggaatgttctgatcaaaaagaaaaacaacaaagtccattgctagtgctgcaaaaatcaaacttgcttttgtgtcagaccattacgaaatggtccttccccttgcaaacagattttcaaaagaagtaaagaaaaactgaaacaccttgacaaagtggccctccagaaccagagccctgggacgctggggaggggcggccagtcccagcgggccacggcctccgggacagccgcctgctggtggggcgtgggcacgtgggcacgctgcggcacggcgggaagccgcgagggcagggcagacgccaagaggcccagtggcgtcatcagggtttccctcaaagggatataaagtgctcgcttgctgactcccagccagtgcccccaaggcctttgcaaaggaagaaaaaggctaaaggtccaaggacccacagggagaacacatgaaggaaccctccctgacgtggtcccgcctgcagacgccgaggcagatcctctgccatctgccctggacgcttgctgtggagaagagccgagtgtgtcttcaaagaaaaggctacacagtaatgctctcagcacatttgtgaagctggagtgagctgacagatgaaacgtgcctccccctgccaggcctttgcagagggcgtctccatttgaatgagattagaattaagtccccccactgataacctggccactgagcagtccatgttatcccatcatctgcttaaaaaaaaaaagtgagatgatgcattcctccccataagccacggcggggtaagagggcaggtggcaggatccccagagggctatgcagagaatgaggccaaggaggccagaagagcctgctagctgggccctgccactgctctgtgccatgaatggggaatggaccagctcctcttgccaatctgggcttcagagcaaagagtggccaccagggaggggaaagtcaaacaagtcccaagaccgttctgcctgctctcaaaccactgtctcagagctgaccatcagcagcccagtgaccaagtgaatccaagaatctgcactcatttggtcaaaagtttgagttaatttcagaagctaccctgtaaactttaccaaactccgaaactcggctctgggtccctcctgagcacggtgtgtctgaacttctgcccccaagtctgaacccaatatacactttggaatgaaactggtggcttcatgtgctggaaaataagttaccagtaaaacgtgactgtcagttactgttgaagagaaaaagagtaaagactggctgtcctggtcaggcaatcataccctccctgcaggttcaccaggcaacaagggtccctgggttccttgcagccacaggctccaaaatccagggctggccacgtggctgcagtggaaaaacccaagtgggtaaagagccccacgtgtgccccatgcattgctgacatgctcaaaaggtctttggaaaactcaagttagaattctatcctgacgatgtggtcagagaagtttaaacatgagtttcattaatgctgactgcccccggcatctggcaagcctcccagggtggccgggcatcctaagcaaccctccctgcccttgccacggaggggaaaaacacaccacccctcgtaatactactagtgttgaaagttaaaaagagcccctgggcttctttatacagctcctaggacagaccaggaaagacacaatcgttggtgtcactccgaaaagacctacggtccctcctctcactttctgaaaatagaatctgacagcaacaattctgtacgctgcagaaaactcatcgtacaaaaataaaaacaaaaataattaaaaacctttgaaaggtaaaaaaaaatgtacaagcaagaattcagaaaggaaaaagatttagacattattaccattcagaaaattgctaaatggtgaggaaaaatgtaaaattcataaaacaatgcttattcaggatctttttgtgaaaaaattcatacaaaaatcaacagcaaatttatattctttgctataaaaactcattaggtacatatgtgcatgaaggcttggagacgggagcggttctgttagaaaataattaaaatgaaagtacaaacttgtagggtagttgcccagtggcgaatgtgttggcgatctgaaatctagccaatctggagcttgagaaaacatgaatttcaatcaatcaggatccctttccataagcaccttgagagcaaattcacaagccatccatttgcagggaccttcgcaatctgcattcattttatatatatatatatactttttctataaatgcattataaatattttatcaagatttcataagaatcaagtaagtttcttagcttggaatacattggaatatatattatacatatatatatttatttatacctaaaatttaagcaatacttcatgctacttgcttttaataaaaagcattccgatcgtaacactgcaagtgtgcctaccacatgcttcacgaccagatggagatgctcaatcgtatgtgacgtgtgagaacactttggattcgtttaaaatttgttggacttcaaaacctccaacgggatttgccacttttttggaactacctccatttttcttaaacagcaataaagcaaaacagggaccgccgggctgcagcccctggccccggagatgacggctggtgcccgtgcttgaggcgtcaggccagctcgcggtgccagcactgccaggctcggctggccacaggaaactgtcccaccgattcctgctgtttgttttttcttaaggcattgttcctcagacttcagaaaacccagccacaaaaatccaccagagcaataaaaaaaaaggcacaaactcgcatcttccgatggcttttgagaaactcaagccagctcccccagctcacattcctgtttctgtccagttttgttttctttaaaggtccctctgtcccccacccgggtgcagaccccccgccgcacaccgctatggttcacagaggcgggccacagccgtagaaaacgtcctctttaaaaaaaaataagctacaagatgagtcgagtggtttacacagagactgtggagttgtgggtaataaactttaagcaccagttttaatcaagtttgttttgtattattagatctttgatatttgttttctgtgcctcgtgtcaactgaattcggcagctcggccgcctgttgccacaggctcctttcttccacggcgtcccttgcgggacccgccagagtgtgcttggcttccgcgtgtccgtgtgtctgcgcgtcgccggcgtctgtcccgtgttccctgtgaggctgccacgcccaggcgtgcatgtgcgtctcgagacctgtgggcctgggcggcagaaaggcttcccgtggctgttgcacgctgggtgtccctgggtgctccaagagagccccacggtgggacgcaggcgtgacacgggaaagtttcttggctgagcttcaagacagagacagacagacaagagaacagcagcttcgagggagtgctacaggggcggctcctcttccatgggctcctcatctggtctcttttcggcgggcttcacgcccacggacagcgaggccatggcggtgaccgtctcggcttcttcgttctcgcaagtctgagcctcgatcagagaacgccccgctgtggaggttgtgcgctgcaggcagcgccagtacttgctgtggatctccatgactttctccatggaacggacagcgtttgcattgggtctttgctgtaaaaccttttctgggagaggatcaagctcgtttcccagcaaggcagaaacacatgcttccgaggcgtcgcaaatggcggtcaggtcgtggcctccctcgagggccaggacaatccggccgccagccaggcccatcagctgcttcgtcaggtacccgaagcatctggcggagaggttgtagcccccaagaggggtggggtggccctccacggcatcgaagcctgatgacaccagcaccacatccggggcaaactcgctggcgatcggcatgaccaccgttctgaaggccgccaagtactcagcgtctcccatgggggggtccaggccgccggtgaaagccatgttgacgttgaaacccacgccgggccctgtgcccacctcatcaggagccccgctgcctgggaagaagttcccatcgtcgtagcggtggagggacatgtacaggacgctggggtcgctgtagaaagcctgctgggtcccgtttccatggtgcacgtcccagtccacgatgaggatcttgctcacgctcaacctctgctgcagaagcttggctgccacggccacggagttgaagtagcaaaagcccatgggcgtgctctcctccgcatggtgtccaggggggcggaccacagcaaagccattcttcagctcccctgtggccaccttgaagaccagctctaccacgcagcccacagccaggcgggctgcccccgccgagtgcacctcgttccatatggtgtcactgtccaccccaacaccaccgcaagggagccggacgaacacggaggcgagcgagctgtccagtttctgccggttgagggggttcgtgccatacaggagggtgtgggcttccgagtgcaccgtctgtagctcctccagggtggccttgcgtccgcggatgcactcgcatttgccccggaggcccgtctcctgcaggcgggaccagatgctctggatcctcccggcgtgctcggggtggctgctgctactcccgcaggtgcactggtgcttcagcatcagcgtgtcatacacgaggcctgtcgtgaacctcggcttggtggggggctcctgcacagacacggggaaggtggcagacgcgggtgaggactgcgcccgggacagaggcctgtggccgccgaaggacacggggatgccggcggcctccatggacgcctggtagttcctcagctggtggatccgctgctgctccagcaggagggcttgctgtctgaagagcagctcctgctcactgggctggcgctggcccggctccacctcccgtgggggctctgcctcttcctcatcgctctcaatgggctcctgcttcacctgcacgccggcctgtgcgtgcgcctccttctgccccggcagccggtccaggtagggctcgtccagcagagcctggtgctcacggagctcctcctccgtctcctccgggtggctctccggctgccgggctggctcgcttggcttggggatgatcttgttcatctgcagttgctgctgctggaactgctgcttgtgtttctccagaaactgctgatgctgctgctggatgaccaggtgctgcagagcctgggcgttctggggcagcggggccgactgggtccgccccagtgggcggtgctgccgcagcttgtggatggagggggacacccggtctgcaccaaccaaggactgtgcgtggaggggcagtgctcccaggcctgaaagataccagtctgtgacgaggggtgcttgtgccggcggctgctccagtaagaccatgtgctgcagaagagggctgtgcgctgcccctccgtcccgctccaagggcgaggtgctcaggtagggagtgaggtgggtgccggggaaaagggagagcctctgctggagggcgggaagggtgagtctctcggcgtcctgctggcccgccgtgcccgcagaggggccggtggcaggcaggcccagcgtgatgttgggcaaggatggcgatgtgtagaggggaagtggagcggccgagccttctcgtgccacaagtctgtgcgccaaactcgtctccgccgggatgctggggacggcgggcgcgataccgttctccgcgctgacgctcccggagctgttgttgggtgagctgggtccggagcctggggcgctgctgcacgcggagtctgtgacatccaacggacgcttttttagagcagtgaccactggcccgtctttcctgcgtaacagggggctgctccgtctttcggccactttctgctttagcctggaccgtaatttcagattcggttcagaagctgttttcctaagagggaagtcatctttggcgtcgtacattcccaggaccgggtggttataggaggtcgacactccgctctggggtggagaactctggtcaagggaactgtgctgcgttttcccgtaccagtagcgagggtcgctggaaatgcagtggttcagattccggtgggccagcgccttctttttattgaggacaaattcttgtaacttcatcttcacttctgtgctggccacggcactctctttgcccttctccttgttcttgagctgctgcagcttctgctcccggtgctgcttctccagctcctgctcctggcggtgcctctccagcttccgctggtgttccagcagctcctgctggtgcttcatggccagcatctcctgttgttgcttgatgtgctcgtggagctgcgcctcgtgctgccgggagagctgctcgtgctgcctctggaactcagcgatgaggatctgcctctggatctgctgcttctgcttgagcgccaggagctcctgctgcagctgctgctcccgcagggccggctctgccacaggcagtgagaactggtggtccaggcgcaggtccatgggcactgccgagggggccacttgcagaggcagcgccgtggccacatccaccgtgctgggcatgtggttcacgcgggcaggattcagcagctccactggctggtctcggccagaaagtccatctccatccacagccagatactgcttccggaaccacacttcgtatccaggtgagctcgttttttgtatttcaaaagcacaaagatctatgttcatggtgtagtccaggcagagtgtggttaacaggcctccgggtgtcccccccttccagcccagtgcaggggttcagccgctgcagaaactccgaatctgctaacgtgaagtgccaagactgctgtccgccagcgccctcactcccccagggcctgtacctgtagcaggaggctcacgttccgagtcctcattgctcccagacccaagggcaaggctgtcacaggcgaaagacgggttccccttcctctacacccaagccctcggaagcacgctgcaggcccctggaggtgccacagtgctcccagctcccccagaggctgagttcaaacattctaaacggattcttgataacaagccgccggctcgctggaagacactgagcagttacataacagcacagaaaatcccttacaagtttcttaaaaaagagttaatcgtactgacttggtgctttaccttcagcccagactttcgcttaatcccggaaactgctccaaaggcgtttttctcagggcgttcggcgccgtaactcaggagaaacccaagtcctgctctcccggcggcctcgctggggaagaattcagccgctccaccctgacatctggtttctatttcatatccatgttgtcacattacataacaagcagatgatacgagagatcaccacagtgtttcggctcgagagtcacaaagaacgcccagaacactgtttatattgggggccatgaacgttcaccaaaccagacttagtgcagaggctgcacccttccaggctgaaacccagcacctacagcaaatgcccaaggaagcaagaagcgggaccccgccttctcagccacctctcactaacactcagctccactcctgcttccttcctctcactccacatccgagttagagggaaatacgatttatctctggcctgcatttacttctcctgcacctggcgggaggctctggccttgcaggcgtgcaggagcccctgccagtgagggccagcgaggggcccagggagaagatggaggtcaagtcatagggcctccaccgcaggcagagctccgccagcaagtatcctgggagctggggggcctcaagggaggcaatccccccacacaccatccccttccccttcgctcatctggggaagctgtgaggactggtgttgataaaacattccaaccacacactcagaccatggatgtggccgtgccagcagggaggccagcagcccctagcagaagggtgttctggaagctgccccctcccatgctgctgcctggtcccatggggcatgaagggagggtggccagggtggcccgagccagcatcaggcacaaggcccaaggagtttctccagagcagcctgtcctcttcggtccagaaaaagtcagattccacagcagggttagccgtccagttagggaacccactaaggggctctgtgcgtagaggtgctcagaatcaaaccactaaaccccaggaccccctgctgggggaatggtccgtggcagtcattcagccttggagtgaaccgttctgcccaagtgcaagtgagaacacaatacttcttattatatacagaattgccaaagccaacgtgattagtagaaaaaccgacatgtcagtgacttgggggtctggtttgccccagatgtgggtggaaaccccaggcgtccctcaagcctggtccagagctccacagacagcagatacacaaactctgagtgacagcattggtgtttagcagattctggattttgctcccccccgaaccaagtatagagaatgtttcacagagtagcttcaacagaaaatggccacagtgtgtctgtgagagagtgtgatgttcccggggggatggctggggccaagggaaggcccctcccatgagccctgcctccatgagactgcgtagggcaggactgccaggcagaaagaacacagcacaggcacaagggcagacccaggctggcagggctaaatggcttcaggagctcccccctctgccccccagggagtaaaggcaatgatgcaaatatgataagcaaacagaggtcccaaaacacagaaagggccaggaccctgatgccaaccaagcagacccaaaactgggtctgggagcacagggcagggtcgctgagtgcagaggggcctcactcaatgtccaacacttccctccaaaacagacatgctggtgagaggcttcaacccttccactggcctgacacctggatctctgctgccctgtgccaggttagccacgtccaacaccaccacggccaccggccatttaagaaaacgaaccctgacgttaacctgcttgagccctaatactaagcaagagcagcgccacaattccaaaactgcagagagcgccttttaaacattctgctgagatctgcgcggtcgcggtctgacaggcaggccttcttggctacctgtggtttcattccagcattaacaggcacctaaaaggcctgtgagcttttgtggggtcaagcagcatcagctccactttacaaccccgcagagtgaggtgttagctctgcagctccagggcagagccttgcagccttagggccagggggacggcctggccccttccgagctctcagcagcctgaactccacgtgtcccctgctgtgtcactggcatgctggtcttgcatggcactgagatgtgtggcacaagcaggcaccaagcccggagacacccgacgctcaccgttagactgggtagcatttgtcaagcgccgagcaaacagtggatgaagtgtcctcagccggcgtcagctgttctgatccgcagaacacataactcctggcactcctttccaagcatccgggaaatgtagaatccaagtgttacaccatccagttgaagatgacagatttacgatataaaacggcacccgcgactgaggactttgtaggaatggaggccgctgtcattatttcatgggtgagggggagagggacactgtgacccatgacaggaaaggacagctcagcccctccaaaaccacacacaggggactccgtttctcacaaaacttcaagtttctgttctacgcaaacattacaacacattttaaactacattctgacacgaagctcccgtgctttttaatggcaggtgttacaatgatcatggaacagtgatggggcggtgcttcctcacggtgacatggcagggagaagtctggaccggagccagcagggtccttgacctaagaggccttgggcagcccacggggcagctctgagcaatctcctgtgaaaggaagagctcagaacgggttcctctaaaggttccttccagagcaggggttctgtggttccctggggccctagactaacatgaggaaggggaaacagagaagaatgcccactaaaagccttacccaaaaattgaaagccaagaaaaatcacaccagatcatctcagtttagacttgaggaacctcggcgctgacatcactgtcaccatcacaaaacactggccaccaaggtgccacctaccacactgcaacctggaaggaggggcgggcaggggcacccctgggcagggcaggacaccaggccagccagccacccacgctacagaggaaatgcagcccctcccaactaagagaaccctggtaccatcaccacagccttggtgccagggctcctagcacctgacagggaagatgagaaggacattggctgccgccaagaggcctgctgcccacccccaactgcacggtggtggtgctgccagcaccaccatccatgctggcccaggagcccacacgcagggcacgcacgcacgtagttccacattaggccctttcttcctcaattgttggaaagaaggccaaagccagatgatggtgaaattcacgaggaaaatgtccccgactgtcctccattctaaagcaaacgctaagaatgggctgctgggcttcagcagaagccaagtcacctttcctctatgcgtccaatgaaacgaaaacatccacacttgtctttataaaaacggaaaactgcatctggaacaaggtctgtggcgtttcttccagcgtgtcccatggacatgaagttggtcttcctatgggtcctccaaggcacacccctcgactgcaccacagcactgagggcagaatgtggtggtggcccagctgccgtggcgccggcagactagcctggtacacggagaggggagcctgctgactgtgggtaggccacgttcccccagtgtcttcatctgcagagggagaccgggagcctctgaagaccgctccagctctgcactgtgggggcggccggccagcaggcaggcaatgctctcaggccccacgctcctctcactggctgccgacgggaggcagacgaggtgccgggggcagcctgcagagcaaggagtcaaggtggccagcctggggcagggtgttcccccagccagggagcttcactcaggcttgggctctgtcccgtgcctccccgggggcgttccgaggtggcggaggaggaagctgcagcccgttatccaccgcccagtctctccctctcaccagcacacagatgttctcagcggcagagcctggcttctgcctgaattcatttcatatttttaaatatgctcttaatggaaagcaacaaaagtacttaacaaaatgcgctgatgtaaatgtccctgcagcagccagggactaattttagaaggggctttgaggagaaacccaagggacactcacttgctggaaacggcctcctccccaaagagtgtgaggatctggattagaaccaagtatccccaggctgcccaggagcccgctcctccaattgggggctggccatcccaccgagcactgataccgcaggctggactcttcctaacctcacgagaggtgatgaccggaatcatcccagttttccatggcacttcgcaaacacagctggtcaggcccttagcacctcctgaccccccgatctcccagactctctgctggaagttaaggacacagagaaagtttcttatgaaaataagcgcctcaaaagaaagccaacgtacagcactggtgacagaaaggaagattcagaaaagccttcacgcctggcaatatggcacacgcacttttagagacgtctaattatactcagggctgagttggctgaagagtgaggaatatactccaaagacaggaattcaaggcagggcaaatagaacatgaaagccagcctggagcccagggcctgtcctggggcagccacctgcactgcctcttaccactgcaccgtccctgtgagtgtgcgtggggaggggctgtagttcccttggcaggggaagccagaagacaggcctgcaagggacacatccgggcctgggcttggtgctggctagaaggggtcaaatcgagagaggactcccctcagaactcataatcccagacccctcgcaatggtttggggagaattcagacaacccatgaggcctgatgagcatccctagcacctgcaaacacaggcatgtcccaggtggcacctcccagcaccaggcagaaaccttctctagaggaacacgctatgaacctcaaaaaaacatccaagaaggacggacataaagtcacaatcaagaaccatgggtagcgggagtaagtcccggaaagacctcagttgtaggaaaatcaggcactgacccaaaacacatacgaaggacactcgacaaaacaagagaggtcatccagggtcaggctggagctagaggcctccagatcctgtcacttagtgactgtacaaacctggtggcttcctcaacctccctgtgccttagcttcccatttgccaaaaagggggattagaagagcccacactctccctggagcaaggctaaggaagaaaggagacagatgtctcagctgttattattaataactatcagaagtgtcacatggatctgaatgatccaaatggaacttgtagaaacaaaactgtcatcattaaaatttaaaactaaatgagtgagttaactaatcaagtattaatagacagagctgaagagagaattagtgaacagtaaaatagcacggaagaaataaaccaggatgcaacacataaaggtaaagagatagaaagctggagacgttagaggactggaaggacagaggaagatatgctaacacacatctgtaaaccaaaaataaaattctaagctcccaaccatctgaatggacccctcctctcaagccaagggcattccaacattaacctgaaaagctagttcaggtcgtgatggggacgggcattcagatgtgcctcatgataccctcctcccttttggaattgctgatagaacagactctttaagtctgatgagaaacatttcagtctattctctctgaagcctgctacccggaggcttcgtcggcatggtaaatccttggtctccacaaacccttatcataatccagacattcctttgtgttgataataactctttcaaccaactgccaatcagaacattttaaaatctacctataatctgaaagcctcacacttcgagttgtcccgcgtttctggactggaccaatgttcatcttccacatactgacagacgcctcatgtctccctaaaaatgtatgaaaccaagctgttccccgaccaccttgggcacatgttgtcagcacctc

SEQ ID NO: 10221 - RNA, 14029 nt, Homo sapiens
  source 1..14029: mol_type = other RNA
caggaaggagacaggcagttcactgtgaattctgagtagtttccctaaaacactgtttccacataaatacaataaactctattattggtatgtcacaagtgctagataaactttttttcttaatatgacaaatgtttaagtagtcctttttatttttcttacaataaaaagtacaatttcttaagaataagttcaataagacgcaaacttccccgccctcctctccttcaaggttttgttttacagaaaaatttccatcttttgtatctgcaaatgtcatgagaggggaacagaaaggcatttttcttcttccccaaagctgccgagtttggcgtgcaaaatctgtatacaatataaagtcatgccggtcgtacagtccatgcaacctccaggtgtaggaaacttaaaaaaatatattcatatatatttatatctatatatttatatatgtatcaatgcccataaaacacgtgggcccaaagtctacaaaaagaagaatggaatgagcacgtggctgtgaccagtaaagaaggaatgttctgatcaaaaagaaaaacaacaaagtccattgctagtgctgcaaaaatcaaacttgcttttgtgtcagaccattacgaaatggtccttccccttgcaaacagattttcaaaagaagtaaagaaaaactgaaacaccttgacaaagtggccctccagaaccagagccctgggacgctggggaggggcggccagtcccagcgggccacggcctccgggacagccgcctgctggtggggcgtgggcacgtgggcacgctgcggcacggcgggaagccgcgagggcagggcagacgccaagaggcccagtggcgtcatcagggtttccctcaaagggatataaagtgctcgcttgctgactcccagccagtgcccccaaggcctttgcaaaggaagaaaaaggctaaaggtccaaggacccacagggagaacacatgaaggaaccctccctgacgtggtcccgcctgcagacgccgaggcagatcctctgccatctgccctggacgcttgctgtggagaagagccgagtgtgtcttcaaagaaaaggctacacagtaatgctctcagcacatttgtgaagctggagtgagctgacagatgaaacgtgcctccccctgccaggcctttgcagagggcgtctccatttgaatgagattagaattaagtccccccactgataacctggccactgagcagtccatgttatcccatcatctgcttaaaaaaaaaaagtgagatgatgcattcctccccataagccacggcggggtaagagggcaggtggcaggatccccagagggctatgcagagaatgaggccaaggaggccagaagagcctgctagctgggccctgccactgctctgtgccatgaatggggaatggaccagctcctcttgccaatctgggcttcagagcaaagagtggccaccagggaggggaaagtcaaacaagtcccaagaccgttctgcctgctctcaaaccactgtctcagagctgaccatcagcagcccagtgaccaagtgaatccaagaatctgcactcatttggtcaaaagtttgagttaatttcagaagctaccctgtaaactttaccaaactccgaaactcggctctgggtccctcctgagcacggtgtgtctgaacttctgcccccaagtctgaacccaatatacactttggaatgaaactggtggcttcatgtgctggaaaataagttaccagtaaaacgtgactgtcagttactgttgaagagaaaaagagtaaagactggctgtcctggtcaggcaatcataccctccctgcaggttcaccaggcaacaagggtccctgggttccttgcagccacaggctccaaaatccagggctggccacgtggctgcagtggaaaaacccaagtgggtaaagagccccacgtgtgccccatgcattgctgacatgctcaaaaggtctttggaaaactcaagttagaattctatcctgacgatgtggtcagagaagtttaaacatgagtttcattaatgctgactgcccccggcatctggcaagcctcccagggtggccgggcatcctaagcaaccctccctgcccttgccacggaggggaaaaacacaccacccctcgtaatactactagtgttgaaagttaaaaagagcccctgggcttctttatacagctcctaggacagaccaggaaagacacaatcgttggtgtcactccgaaaagacctacggtccctcctctcactttctgaaaatagaatctgacagcaacaattctgtacgctgcagaaaactcatcgtacaaaaataaaaacaaaaataattaaaaacctttgaaaggtaaaaaaaaatgtacaagcaagaattcagaaaggaaaaagatttagacattattaccattcagaaaattgctaaatggtgaggaaaaatgtaaaattcataaaacaatgcttattcaggatctttttgtgaaaaaattcatacaaaaatcaacagcaaatttatattctttgctataaaaactcattaggtacatatgtgcatgaaggcttggagacgggagcggttctgttagaaaataattaaaatgaaagtacaaacttgtagggtagttgcccagtggcgaatgtgttggcgatctgaaatctagccaatctggagcttgagaaaacatgaatttcaatcaatcaggatccctttccataagcaccttgagagcaaattcacaagccatccatttgcagggaccttcgcaatctgcattcattttatatatatatatatactttttctataaatgcattataaatattttatcaagatttcataagaatcaagtaagtttcttagcttggaatacattggaatatatattatacatatatatatttatttatacctaaaatttaagcaatacttcatgctacttgcttttaataaaaagcattccgatcgtaacactgcaagtgtgcctaccacatgcttcacgaccagatggagatgctcaatcgtatgtgacgtgtgagaacactttggattcgtttaaaatttgttggacttcaaaacctccaacgggatttgccacttttttggaactacctccatttttcttaaacagcaataaagcaaaacagggaccgccgggctgcagcccctggccccggagatgacggctggtgcccgtgcttgaggcgtcaggccagctcgcggtgccagcactgccaggctcggctggccacaggaaactgtcccaccgattcctgctgtttgttttttcttaaggcattgttcctcagacttcagaaaacccagccacaaaaatccaccagagcaataaaaaaaaaggcacaaactcgcatcttccgatggcttttgagaaactcaagccagctcccccagctcacattcctgtttctgtccagttttgttttctttaaaggtccctctgtcccccacccgggtgcagaccccccgccgcacaccgctatggttcacagaggcgggccacagccgtagaaaacgtcctctttaaaaaaaaataagctacaagatgagtcgagtggtttacacagagactgtggagttgtgggtaataaactttaagcaccagttttaatcaagtttgttttgtattattagatctttgatatttgttttctgtgcctcgtgtcaactgaattcggcagctcggccgcctgttgccacaggctcctttcttccacggcgtcccttgcgggacccgccagagtgtgcttggcttccgcgtgtccgtgtgtctgcgcgtcgccggcgtctgtcccgtgttccctgtgaggctgccacgcccaggcgtgcatgtgcgtctcgagacctgtgggcctgggcggcagaaaggcttcccgtggctgttgcacgctgggtgtccctgggtgctccaagagagccccacggtgggacgcaggcgtgacacgggaaagtttcttggctgagcttcaagacagagacagacagacaagagaacagcagcttcgagggagtgctacaggggcggctcctcttccatgggctcctcatctggtctcttttcggcgggcttcacgcccacggacagcgaggccatggcggtgaccgtctcggcttcttcgttctcgcaagtctgagcctcgatcagagaacgccccgctgtggaggttgtgcgctgcaggcagcgccagtacttgctgtggatctccatgactttctccatggaacggacagcgtttgcattgggtctttgctgtaaaaccttttctgggagaggatcaagctcgtttcccagcaaggcagaaacacatgcttccgaggcgtcgcaaatggcggtcaggtcgtggcctccctcgagggccaggacaatccggccgccagccaggcccatcagctgcttcgtcaggtacccgaagcatctggcggagaggttgtagcccccaagaggggtggggtggccctccacggcatcgaagcctgatgacaccagcaccacatccggggcaaactcgctggcgatcggcatgaccaccgttctgaaggccgccaagtactcagcgtctcccatgggggggtccaggccgccggtgaaagccatgttgacgttgaaacccacgccgggccctgtgcccacctcatcaggagccccgctgcctgggaagaagttcccatcgtcgtagcggtggagggacatgtacaggacgctggggtcgctgtagaaagcctgctgggtcccgtttccatggtgcacgtcccagtccacgatgaggatcttgctcacgctcaacctctgctgcagaagcttggctgccacggccacggagttgaagtagcaaaagcccatgggcgtgctctcctccgcatggtgtccaggggggcggaccacagcaaagccattcttcagctcccctgtggccaccttgaagaccagctctaccacgcagcccacagccaggcgggctgcccccgccgagtgcacctcgttccatatggtgtcactgtccaccccaacaccaccgcaagggagccggacgaacacggaggcgagcgagctgtccagtttctgccggttgagggggttcgtgccatacaggagggtgtgggcttccgagtgcaccgtctgtagctcctccagggtggccttgcgtccgcggatgcactcgcatttgccccggaggcccgtctcctgcaggcgggaccagatgctctggatcctcccggcgtgctcggggtggctgctgctactcccgcaggtgcactggtgcttcagcatcagcgtgtcatacacgaggcctgtcgtgaacctcggcttggtggggggctcctgcacagacacggggaaggtggcagacgcgggtgaggactgcgcccgggacagaggcctgtggccgccgaaggacacggggatgccggcggcctccatggacgcctggtagttcctcagctggtggatccgctgctgctccagcaggagggcttgctgtctgaagagcagctcctgctcactgggctggcgctggcccggctccacctcccgtgggggctctgcctcttcctcatcgctctcaatgggctcctgcttcacctgcacgccggcctgtgcgtgcgcctccttctgccccggcagccggtccaggtagggctcgtccagcagagcctggtgctcacggagctcctcctccgtctcctccgggtggctctccggctgccgggctggctcgcttggcttggggatgatcttgttcatctgcagttgctgctgctggaactgctgcttgtgtttctccagaaactgctgatgctgctgctggatgaccaggtgctgcagagcctgggcgttctggggcagcggggccgactgggtccgccccagtgggcggtgctgccgcagcttgtggatggagggggacacccggtctgcaccaaccaaggactgtgcgtggaggggcagtgctcccaggcctgtgacgaggggtgcttgtgccggcggctgctccagtaagaccatgtgctgcagaagagggctgtgcgctgcccctccgtcccgctccaagggcgaggtgctcaggtagggagtgaggtgggtgccggggaaaagggagagcctctgctggagggcgggaagggtgagtctctcggcgtcctgctggcccgccgtgcccgcagaggggccggtggcaggcaggcccagcgtgatgttgggcaaggatggcgatgtgtagaggggaagtggagcggccgagccttctcgtgccacaagtctgtgcgccaaactcgtctccgccgggatgctggggacggcgggcgcgataccgttctccgcgctgacgctcccggagctgttgttgggtgagctgggtccggagcctggggcgctgctgcacgcggagtctgtgacatccaacggacgcttttttagagcagtgaccactggcccgtctttcctgcgtaacagggggctgctccgtctttcggccactttctgctttagcctggaccgtaatttcagattcggttcagaagctgttttcctaagagggaagtcatctttggcgtcgtacattcccaggaccgggtggttataggaggtcgacactccgctctggggtggagaactctggtcaagggaactgtgctgcgttttcccgtaccagtagcgagggtcgctggaaatgcagtggttcagattccggtgggccagcgccttctttttattgaggacaaattcttgtaacttcatcttcacttctgtgctggccacggcactctctttgcccttctccttgttcttgagctgctgcagcttctgctcccggtgctgcttctccagctcctgctcctggcggtgcctctccagcttccgctggtgttccagcagctcctgctggtgcttcatggccagcatctcctgttgttgcttgatgtgctcgtggagctgcgcctcgtgctgccgggagagctgctcgtgctgcctctggaactcagcgatgaggatctgcctctggatctgctgcttctgcttgagcgccaggagctcctgctgcagctgctgctcccgcagggccggctctgccacaggcagtgagaactggtggtccaggcgcaggtccatgggcactgccgagggggccacttgcagaggcagcgccgtggccacatccaccgtgctgggcatgtggttcacgcgggcaggattcagcagctccactggctggtctcggccagaaagtccatctccatccacagccagatactgcttccggaaccacacttcgtatccaggtgagctcgttttttgtatttcaaaagcacaaagatctatgttcatggtgtagtccaggcagagtgtggttaacaggcctccgggtgtcccccccttccagcccagtgcaggggttcagccgctgcagaaactccgaatctgctaacgtgaagtgccaagactgctgtccgccagcgccctcactcccccagggcctgtacctgtagcaggaggctcacgttccgagtcctcattgctcccagacccaagggcaaggctgtcacaggcgaaagacgggttccccttcctctacacccaagccctcggaagcacgctgcaggcccctggaggtgccacagtgctcccagctcccccagaggctgagttcaaacattctaaacggattcttgataacaagccgccggctcgctggaagacactgagcagttacataacagcacagaaaatcccttacaagtttcttaaaaaagagttaatcgtactgacttggtgctttaccttcagcccagactttcgcttaatcccggaaactgctccaaaggcgtttttctcagggcgttcggcgccgtaactcaggagaaacccaagtcctgctctcccggcggcctcgctggggaagaattcagccgctccaccctgacatctggtttctatttcatatccatgttgtcacattacataacaagcagatgatacgagagatcaccacagtgtttcggctcgagagtcacaaagaacgcccagaacactgtttatattgggggccatgaacgttcaccaaaccagacttagtgcagaggctgcacccttccaggctgaaacccagcacctacagcaaatgcccaaggaagcaagaagcgggaccccgccttctcagccacctctcactaacactcagctccactcctgcttccttcctctcactccacatccgagttagagggaaatacgatttatctctggcctgcatttacttctcctgcacctggcgggaggctctggccttgcaggcgtgcaggagcccctgccagtgagggccagcgaggggcccagggagaagatggaggtcaagtcatagggcctccaccgcaggcagagctccgccagcaagtatcctgggagctggggggcctcaagggaggcaatccccccacacaccatccccttccccttcgctcatctggggaagctgtgaggactggtgttgataaaacattccaaccacacactcagaccatggatgtggccgtgccagcagggaggccagcagcccctagcagaagggtgttctggaagctgccccctcccatgctgctgcctggtcccatggggcatgaagggagggtggccagggtggcccgagccagcatcaggcacaaggcccaaggagtttctccagagcagcctgtcctcttcggtccagaaaaagtcagattccacagcagggttagccgtccagttagggaacccactaaggggctctgtgcgtagaggtgctcagaatcaaaccactaaaccccaggaccccctgctgggggaatggtccgtggcagtcattcagccttggagtgaaccgttctgcccaagtgcaagtgagaacacaatacttcttattatatacagaattgccaaagccaacgtgattagtagaaaaaccgacatgtcagtgacttgggggtctggtttgccccagatgtgggtggaaaccccaggcgtccctcaagcctggtccagagctccacagacagcagatacacaaactctgagtgacagcattggtgtttagcagattctggattttgctcccccccgaaccaagtatagagaatgtttcacagagtagcttcaacagaaaatggccacagtgtgtctgtgagagagtgtgatgttcccggggggatggctggggccaagggaaggcccctcccatgagccctgcctccatgagactgcgtagggcaggactgccaggcagaaagaacacagcacaggcacaagggcagacccaggctggcagggctaaatggcttcaggagctcccccctctgccccccagggagtaaaggcaatgatgcaaatatgataagcaaacagaggtcccaaaacacagaaagggccaggaccctgatgccaaccaagcagacccaaaactgggtctgggagcacagggcagggtcgctgagtgcagaggggcctcactcaatgtccaacacttccctccaaaacagacatgctggtgagaggcttcaacccttccactggcctgacacctggatctctgctgccctgtgccaggttagccacgtccaacaccaccacggccaccggccatttaagaaaacgaaccctgacgttaacctgcttgagccctaatactaagcaagagcagcgccacaattccaaaactgcagagagcgccttttaaacattctgctgagatctgcgcggtcgcggtctgacaggcaggccttcttggctacctgtggtttcattccagcattaacaggcacctaaaaggcctgtgagcttttgtggggtcaagcagcatcagctccactttacaaccccgcagagtgaggtgttagctctgcagctccagggcagagccttgcagccttagggccagggggacggcctggccccttccgagctctcagcagcctgaactccacgtgtcccctgctgtgtcactggcatgctggtcttgcatggcactgagatgtgtggcacaagcaggcaccaagcccggagacacccgacgctcaccgttagactgggtagcatttgtcaagcgccgagcaaacagtggatgaagtgtcctcagccggcgtcagctgttctgatccgcagaacacataactcctggcactcctttccaagcatccgggaaatgtagaatccaagtgttacaccatccagttgaagatgacagatttacgatataaaacggcacccgcgactgaggactttgtaggaatggaggccgctgtcattatttcatgggtgagggggagagggacactgtgacccatgacaggaaaggacagctcagcccctccaaaaccacacacaggggactccgtttctcacaaaacttcaagtttctgttctacgcaaacattacaacacattttaaactacattctgacacgaagctcccgtgctttttaatggcaggtgttacaatgatcatggaacagtgatggggcggtgcttcctcacggtgacatggcagggagaagtctggaccggagccagcagggtccttgacctaagaggccttgggcagcccacggggcagctctgagcaatctcctgtgaaaggaagagctcagaacgggttcctctaaaggttccttccagagcaggggttctgtggttccctggggccctagactaacatgaggaaggggaaacagagaagaatgcccactaaaagccttacccaaaaattgaaagccaagaaaaatcacaccagatcatctcagtttagacttgaggaacctcggcgctgacatcactgtcaccatcacaaaacactggccaccaaggtgccacctaccacactgcaacctggaaggaggggcgggcaggggcacccctgggcagggcaggacaccaggccagccagccacccacgctacagaggaaatgcagcccctcccaactaagagaaccctggtaccatcaccacagccttggtgccagggctcctagcacctgacagggaagatgagaaggacattggctgccgccaagaggcctgctgcccacccccaactgcacggtggtggtgctgccagcaccaccatccatgctggcccaggagcccacacgcagggcacgcacgcacgtagttccacattaggccctttcttcctcaattgttggaaagaaggccaaagccagatgatggtgaaattcacgaggaaaatgtccccgactgtcctccattctaaagcaaacgctaagaatgggctgctgggcttcagcagaagccaagtcacctttcctctatgcgtccaatgaaacgaaaacatccacacttgtctttataaaaacggaaaactgcatctggaacaaggtctgtggcgtttcttccagcgtgtcccatggacatgaagttggtcttcctatgggtcctccaaggcacacccctcgactgcaccacagcactgagggcagaatgtggtggtggcccagctgccgtggcgccggcagactagcctggtacacggagaggggagcctgctgactgtgggtaggccacgttcccccagtgtcttcatctgcagagggagaccgggagcctctgaagaccgctccagctctgcactgtgggggcggccggccagcaggcaggcaatgctctcaggccccacgctcctctcactggctgccgacgggaggcagacgaggtgccgggggcagcctgcagagcaaggagtcaaggtggccagcctggggcagggtgttcccccagccagggagcttcactcaggcttgggctctgtcccgtgcctccccgggggcgttccgaggtggcggaggaggaagctgcagcccgttatccaccgcccagtctctccctctcaccagcacacagatgttctcagcggcagagcctggcttctgcctgaattcatttcatatttttaaatatgctcttaatggaaagcaacaaaagtacttaacaaaatgcgctgatgtaaatgtccctgcagcagccagggactaattttagaaggggctttgaggagaaacccaagggacactcacttgctggaaacggcctcctccccaaagagtgtgaggatctggattagaaccaagtatccccaggctgcccaggagcccgctcctccaattgggggctggccatcccaccgagcactgataccgcaggctggactcttcctaacctcacgagaggtgatgaccggaatcatcccagttttccatggcacttcgcaaacacagctggtcaggcccttagcacctcctgaccccccgatctcccagactctctgctggaagttaaggacacagagaaagtttcttatgaaaataagcgcctcaaaagaaagccaacgtacagcactggtgacagaaaggaagattcagaaaagccttcacgcctggcaatatggcacacgcacttttagagacgtctaattatactcagggctgagttggctgaagagtgaggaatatactccaaagacaggaattcaaggcagggcaaatagaacatgaaagccagcctggagcccagggcctgtcctggggcagccacctgcactgcctcttaccactgcaccgtccctgtgagtgtgcgtggggaggggctgtagttcccttggcaggggaagccagaagacaggcctgcaagggacacatccgggcctgggcttggtgctggctagaaggggtcaaatcgagagaggactcccctcagaactcataatcccagacccctcgcaatggtttggggagaattcagacaacccatgaggcctgatgagcatccctagcacctgcaaacacaggcatgtcccaggtggcacctcccagcaccaggcagaaaccttctctagaggaacacgctatgaacctcaaaaaaacatccaagaaggacggacataaagtcacaatcaagaaccatgggtagcgggagtaagtcccggaaagacctcagttgtaggaaaatcaggcactgacccaaaacacatacgaaggacactcgacaaaacaagagaggtcatccagggtcaggctggagctagaggcctccagatcctgtcacttagtgactgtacaaacctggtggcttcctcaacctccctgtgccttagcttcccatttgccaaaaagggggattagaagagcccacactctccctggagcaaggctaaggaagaaaggagacagatgtctcagctgttattattaataactatcagaagtgtcacatggatctgaatgatccaaatggaacttgtagaaacaaaactgtcatcattaaaatttaaaactaaatgagtgagttaactaatcaagtattaatagacagagctgaagagagaattagtgaacagtaaaatagcacggaagaaataaaccaggatgcaacacataaaggtaaagagatagaaagctggagacgttagaggactggaaggacagaggaagatatgctaacacacatctgtaaaccaaaaataaaattctaagctcccaaccatctgaatggacccctcctctcaagccaagggcattccaacattaacctgaaaagctagttcaggtcgtgatggggacgggcattcagatgtgcctcatgataccctcctcccttttggaattgctgatagaacagactctttaagtctgatgagaaacatttcagtctattctctctgaagcctgctacccggaggcttcgtcggcatggtaaatccttggtctccacaaacccttatcataatccagacattcctttgtgttgataataactctttcaaccaactgccaatcagaacattttaaaatctacctataatctgaaagcctcacacttcgagttgtcccgcgtttctggactggaccaatgttcatcttccacatactgacagacgcctcatgtctccctaaaaatgtatgaaaccaagctgttccccgaccaccttgggcacatgttgtcagcacctc

SEQ ID NO: 10222 - RNA, 31 nt, Homo sapiens
  source 1..31: mol_type = other RNA
caggagtggggggtgggacgtaaggaggatg

SEQ ID NO: 10223 - RNA, 839 nt, Homo sapiens
  source 1..839: mol_type = other RNA
caggatgccagcatagtaggaacccagtgatggcccttttctgggttacaaactgcagacttactgtatccttacctgatgaaaagagagagagttagctagctctctcggctcttcttataaaggcactaatctcattcatgggggttccaccgtcatgatgtaattgtccttcaaaggccctcacctcctaatactatcacttagggagtgaagatttcaacgtatgaatttaggtggggaggtcacagactttcggtccatagcatgattcaagatgggttccagtatactcagttttccactgcgattgtcttcttctctcattgccagggccgtcagaaaattatcttgtaggtctttaccagcacttgttagcgtcttttgctgagctctttcagccagtcttgcaatctctatagccgctttccttgcttcaaaatcttcccttttcactctctctccagtccctcggtagcctagctccaccaactggcgggccagggtttcatcctccaggtagtacaagtccacagtagtgatctgcgagtccaggaaatcttcataggcgttgaattgagtgacaatattgtccaaggccttcagcccctcttcctgatccattgcggtatcctcggccgaagcgtcccacggcctggagcagacctcacaccgcatctcccctgaatttttgtttcattgtggaggttgttttctttataaatgccctctgagcaagggtgggttttaacaaaattcagtcctttgctgtctagaagaaaaaaaaatgaattaataaatggatcatcaaagatacatttgattaattaagctaatta

SEQ ID NO: 10224 - RNA, 78 nt, Homo sapiens
  source 1..78: mol_type = other RNA
caggcacgggagctcaggtgaggcagggagctgagctcacctgacctcccatgcctgtgcaccctctattatatcact

SEQ ID NO: 10225 - RNA, 2170 nt, Homo sapiens
  source 1..2170: mol_type = other RNA
caggcagggaggtgggaccatgagtgctgcactggggtcgcaggatctctgctgactgctggacacccccggccctcccctatccctgcaggtcctggtggctggcattgaggcgaacatacctgtgacctatggaattggcagccagaggggagacgagagcactggctgtcaattcataggtcagagccctgtgcactcggtctcggcagcccaccgacagccctccactacccgccaccatctggcctgggagcgtcgccacggtagtcctggctggtctgctggccagcacctgcctctccttcttcgtgggtactggccctcgccccagataacagcagccccactggaaccagtgggcacttccacatggagttgctgttacagggggcgggaaccaattggagaccggggccctgcctggcgtccgccttcggcagggctctggagagtgtcccatgcccactcacctgggctccccagtcttcgtggccccaggtccatggtcttttcaccgaggcttcttatcatccggggcccacacctggcgccccgtgtgctgccagcactccttcctgggcaaagtccaggctcaaccccaaatcggcctcataaagccgggagcggctcggatttacaactcctgggcagcctttgcccgctctgatgaccccacgccctctgtccccaagttattttgtttccttgtttctttcccaaccagagctgggcctcagtttcaggtttggccactgtcacctctgccctttgcccaccctccctgctgcagccatggggcagagagacagcaagggacagctggcacttgtcagtccccagggacctcccagtgcctgatttcatgaggatggcctcgtatgggaagctgaagatgagactaagaagaagtgtggggggctgtgtgggggagggcacagaaagagggatagtgaggcagaggggctgagagaggaagagaagagtaaggccgaggatggcggtgcacacctggcatcccagcactttgggagaccaaggtgggaggatctcttgagcccaggagtgcaagaccagcctgggcaacacagtgagaccccatctctacaaaaaataaaaaattagcctggtgtggtgatgcatgcctgtggtcccagctactcaagaggctgaggcgggggatcacttgagcctgggaggtcgaggctccagtgagctgggattgtgccactgcactccagcctcagtgacaaagaaagaccctgtctcaaataaaaataagaggagcaggtagagaactagaaaggaacagagaaaacaaacagggatagtggatgacgaggtgtaggaagggggacgacagggaactggaaaagatgtagatacacaaacctgccgcagaacatgaggaacaggctgtgagcagtggctcgcctggaaggacgcttaggacctcagtggcctggaagacagcaggggcctgggagctgggtgaccttgagcaagtagcgtaacctctctgaaccactgtccatatgtcaatcaggacttacgaggccaccctgcacgctgggctggcctggtgggaagcatccgccctgggacccttgggtctctctccgctgtggggagaggaagcagctgctggccagggtccctgagtgagcccagggctctgtgaggcagagcttcctcttgcaaagcgtgttctcgtccctcccagacaggttccggtgacaggtgccagtcctgcagagacccagcaggcattttgggagactccaaagcttctggagagaaaggggagcttttagagtagacttgggccctgccccctttgccagtggtgcatacaggcctagagagacagagggggccgcccaaggtcacagagcagggccccagggcctgtgctgccccaacaaccttcccgaagtggcgtccccccttctcaggatgcagtcagggtgggatgggggatccctgggctggaatccttctgcctggggggacagacctgcgaaggaagacaccgtagctggtggctggccctccactcagcctggcggcccttcccacagaggcctgggcgagaccagcctcctgcagcgtggtgtccaagtgccctggcctgagtgccgggctggccttcggggcacaaggaggaagt

SEQ ID NO: 10226 - RNA, 8463 nt, Homo sapiens
  source 1..8463: mol_type = other RNA
cagggaaatgggaagaactagaggaaaaagccatgaggtgggaaaacgtgggcattttgggggaatgtcaagctggagtctggagtggctggagcataaagggcatgaagcggagtctaaagagagatgagatgagatacgcgcggattccgaggggcctcacaggacgagtttacactttctttgcccagcgatgatgtcccatggagctttctgagcaagaagtgtcatagtcagaggtgagccatggcacaaaggagcagggagaaatgggagcccctggctggcagagcaaggagggtctggctggtgggagaaggaccatggcagccggaaggccaggcatccgaatcatcccaccccagcctggccactgccctgctctttgccctcccaggctgcctgtcactctgaggaatgtggcacactctccctaagggggaggcaacttgctcatgccacttcctgaacccagactggtcccaggaccatctatttttggctctcccaagccagtgtttgacaagaaaagcacagctgccagtaatttcgccccagtggaatctactgttctataaagggtcatgccagtttctgcacatgaattatggtcacctggacccaaggccaagggaagcacctccgtcttcagcatcacggtgcactggagtctttcccggacctgggaaaagtaggctggtgcctttgttcagcttgcacagaagtagaaacagaagttcagcttgcacagaagtccagttgttcctgggactgtgtttgttcaaggggcaccagggcaccaagagacacactcacttcctagtgcatacagcctgctccgtgcccaataatagctgcatggtgtgagggagaaaactgcaaagccagccagggctacgcttcttatggaatgatccctggagtaaaagggatttatagtcgaggagttatgtttagaaaggacccactcagaacaggaatgagcttagaaacttcataccaactaaagcttcatccctggccagctgagtacccccttctcccctctatcaccctacgaatccattcaccatctttgcttggattttttttttttaaactctcagatttcccagcccccaaactcttgcctctccagtatcttcaaaactggggtccaagatggtgagccccttaacgaaaaggctaggtattaatatcctgtgttacctctacacccagcacagtaaaataaatttgaagcgaatgaataaagaagcaaaccaatgaatgtatgtcccttgggcagctccaccggggcagcgaggcctctccccacaccaacccctgagaaatgtgagtggcactactgtagtcacacagggacagctgaggccgagaggacttgttaacaatgcagtcaggaagagtgaagggaatcaggcagcagtttgaaagaaatgtgcaaatccagcctctctgttgcttttccttttggaatatttctaatgcaccaaatgcggatggtgaagctctagattcattttccccaggaaaacatgttttctttgcttgcttaagtgaagctcagtggcaaaagttttggctgactaggagagttgatgttggcaaatgtgggtagagctgatgaatgccatgatcctcaccaatagtttgtacaccctaagaaattactaataacactgatgacaataatagatgctaccatttaattagtatatactgggtgcaaggcattacgctaagcacttgacatgcattgtataccgaagagtcacagttgtacttaggacatagatactattattatctctggttttagaggaggtttaatgagataaagcctcttgctcaaggtcacatagctagtaagtggcagaacagtgatttaaacccaggataagtgacagcaaatttacttctacacggcagtgccattcaatttttttttccgtggataaatggtcataccctttagggaagaggtagaaagaagaaaggttctgctaactgccagacaacacgctaaggttatttatacaggttgagcatccccagtctgaaatccaaaatgctccaaaatctgaaactttttgagtactgccaagtggagaattccacacttcacctcacgtgatgagttgcagtcaaactgcagtcagcactttgttccatgcacaaaattagttagactattgtatcaaattaccttcaagctatgtgcataaggtgtatatgaaacaaaagaacttcatgttgaggcttgggtcctatcccccaaatatctcatcatgcacatgcacatattccaaaattaaaaaaaaaaattagaaacacttctggtcccaagctttttggggctaaggggtactaaacccgtatatgtaaactcgcttgatgcttaatgatgaaaactgcattatgtcccctttttgcaaatgaggtacctgtatctcagagaagttaactagcaggtctgaagtcataaatgatagttagtacaagtgaagagaattgagaatggcaaaccaattttagtaatcaatcagtgccagaacacaggccaaaatagggtaggtatgagcagtagcttatgctaagtgttgaactagaccagaggttggcaaactttttctgtaaagggccagatatggtcaataggatttggcccgtgggccatagttcgctgacccttgaactagatgatactgatacgtggaaagtttgaacctttgtgagactcctgttcctaacagtagtattcatatatgaatccattaataatttataagtttagtttaatctatctacttagtaaaatcattaacatataataaaaaggtaaacctgggttaataaataaactccaatgggaaaattctaaggcacatgcatgttttagagagggaaaagtaagaaaaatacattccactgaggggggaaaaaagtaacacatttgtactatgagccctgaatacagaacagacgccaaggcttaaactgacatccaaatccttccctcctctttgcagtatggaccagggcttagatgagttggtggcttgggtaattaagaactctaaagatcactgccttcaatctaaaaggccacatgttcacagaaagctttttccttgcgtggatgccagacacttgtgcacagtgccattttcactgaagagtaaaagagcttagttcactgagaaagaaagaattaaaggactggaaatgtctgaatcagaaataatccattttcctaaacagcagtgagaagggagggtaccgcaggatggcctatcatttacaggggggaaaagacctccagtaactgactgaagttctgtctttggtcaatgacctttagcaatgttcctagtcctaggtctacctgcgaaacctgaaaaactccccagaaatgggtgatgggagaaaacaaacaagaagcacagggtggtattcattttgtttggaaaattatctgattcaataatcaattatttcaatattcaggatctgagtcaatactctgtgtttactgagtgcctactcagtgcctggacccatgcaaggttcagggagacaacattagcaagatagccaaggtctttgtcctcaagaacttcagagtttcctgggaggatcatttaggaaatatgtttttaatctcaaccattaaaaagtatttctaataaggtttgcttgcaaaagaccttctctgatttttctttgtcgaggtatcttaggacgctattgtccaaaataaaaacttttgatagtttttggggtacaggtgttttttggattagctctttagtggtggtgtctgagattttagtgcacccatcacccaagcagtgtacattctacccaatatgtagtcctttatccctcacccacctcccaatgtccccacactccagttgccaaagttcgttatatcactctatgcctttatgtcctcatagcttagctcctacttagaagtgagaacatgacatatttggttttccatgtctgagaaccccactttcctagagcacattctcaccatttttccccttcctccctaataaccccaaactgactgaactggctttctctgcagctgccaggagatatcacctctaagtgtgttaccgacaacttggaacgtatcacaacatcctcagacagctccttcgcttctctcaatgagccatgaggatacagaaaggagggtcagcaacatgaggctgaagctcttgggtcatcataatgtagggaagaccagtgcatgtcaccccccaggtggcaatgaggaattgattgctggtctcattgcactgacaaaacctcaggcagtacgtttttgcacaatccatgtatccatccatccaatcattcatgacatgtagcaaaaatttaccactagtgacactgtggtactttcacagtgtttcacaactatcacccctatctagttccagaacactgtcaggattatcaggaagaggaaattcccacctaataaattttggtcagactggttgatctcaaaaccctgtctcctgataagatgttctcaatgacagtggtgcctgaaacttcagtagcaattttaatttcgccccggtcctgtggtcctgtgatctcgccctgcctccctttgccttgtgatattctattaccttgtaaagtacttgatgtctgtgacccacacctatttgcacactccctccccttttgaaactccctaataaaaacttgctggtttttgcggcttgtggggcatcacggaacctaccaacatgtgatgtctcccccggacgcccaactttaaaatttctctcttttgtactctgtccctttatttctcaagctggccggcacttaaggaaaatagaaaagaacctacgtgaatatcggggcagattccccgatatctggtgcccaacgtggattccccgatagagttgaggctactccaaggagaaggaggaaaaagtctcgaagcccaatggcacgtacagaatgcaattggtacatggctacagctgtgttgtccaatgacagccacatgtgactagtgagcacttgcaatgtagctggtctaaagtaaaatacgctgtacattttctactatgttaaaaaaaataaagtagctacatttaaaagtagaaacatgcaaaattaattttaataatatttaatatttaatccaaaatatctgaagtgtcatttcaatgcatggtcaatacaaaagttattaagatattttacagtctttttttggtactaactctttgaaattctctgtgtatagagtttctttgcttccatctatcttctccccagtacagtttgggaccctcatcacaatcaacatccccatttctgctttctagcccaggctgtggatggttggccacacttcaagaaataatgcagcattgctaattattttgaatgtccatcatttgcagagtatctaacattaaaaataataataataaggcacctctacacacactgcctctctctaacaacccaataatcaagtgaggtgctgcaagcaatacagtaccccaggggttatagacaacaaagaggactgcagggctcagtgatctgaccaaggtcacacttcagtgaggtcttttacctctggggccagggttctttcctcactccaccactagcacagctcttcaggctggtgtgtgctagggaaagtaggctgctcctcttgcctgccttggagcgtccaccactgggtggctgtaaggggcaatctcatagttataggaacaggtcaggtggaggcgtaggaaggaggaggctgtgctagcagtgcagacgcacgtctgacaggctgagaggaaggttgtacctggatgcagcttgtctgctggagacagaagctggcagggtgcccccctggccctagaacctgctgccacagaaagtgatcatcaacaagctcctaggctgaacccaacatttgaaatacacagctgcttcataagcagggctctcaccaagtgtgtggcatgacagctgactcagtctgtggctaatcctgccaatggttcctcctgtaacttctgtccgcttaatgcaatcgccagtgtcctctgctctcatgtttagggagccaactgcaggggacactgcatgtgtgttgctggacaggcttgggacaagggggtggggtggaggatggactatgatgaatcatggatcatgccagctccaggcaaaggattcaaattcaattttttaaaatgcgcacctgtcagccaattgcagcacacctaggtaccagttcacaagttcagctctagaacatgacactcttaaagccctttcctctgccttccctaaatggtaaaaagagaataacactggttaactctgagaatttactatattctaggcaccattccaggcactttatttgcactaaatcatttaatctcataaaacacctatgatgcaggaacacttattctactcattttacagataggaactgcagtacagagaaattaagttaactaccccagactgcacacagaggaaccccagaagctgggatgggaacccagacagggaggctcccagagcctggccctctgtaaagggtatctagtgccagcaagatttgctttcttaatgaaggaactgtcttgtctattttgatgctaaatggggacactggcttcatcacacctcttgaagacagggtcacccctaccctatcacagagggactggaaatgaatgtctccgccttcctgccagcacagcacatctttcctctttcggagagattttccctagaagccacagtggacacttgcaggaggcacccaattctctgctccctggggagttccctgtggtcttcccctcaccccacctcccgcctccctgccctgcccacagcacacgcctaccctgcctggctctgcccgctggcaccttttacctcccaccacgctcttccctctgcctggactctcccttcaccttctagtttccagcagtgactcacccagaaaccttcaccctcctctgtttctccaggccaaggtgcccgttgcctcctctggagccctgcagcacttggcaaatactctcaatacaggaatttacacaactcatttttattcatgagtctgtctctgaaaactgcaagttcccccaggatacactgcaaatgctaagaaggcttagagaaataataataataataataataataataataataacaataatgaaaatggtgtccgtttaggtcaggctgacctcctatgaagggacctggctttctggaacctgctgtcctggttcttatccttactgttggaccccaggctgaccttgagccttgagtgatgtcccacatcccgtgagtcttttccagatggctttgggtccacagcctggtttcttaggtccagggacactctctcttgcctgccttgtcacctactggtgcctgctcaccacagaacaggtaccaataggcctggctcacagacaggtcatatcttactgaatatagaaaatgtagaaagaaaagtgaattttgagccaggaatgatggcacatcagaaggaaatacctttatagaagtttctggatatagtttgtaacttttcagcccataacatgctcccaactcaaaccacttcgagagcctgctttccccttaatcaggtattctcaggcttggcattattgacatttggggttggataattctttgttgtggatgccggtcctgtgcaccgatggaggcttgacagcatccgcagcctctccccactagatgccagtagcacttcccctgtgttccaaccctgttatgacagcaaccaaaaatgaatccagacactgccaaacgtcatgaggtgcaaaagcacccaggttgagaagctctgccctaactcgccctcgaatcctgcaatcgctcactcaacttcattcccttcaaacgcaccatgattttagacactcagacaatacaccagcttcagccccccttcttcctgctgttgcatctgtttttccagtcagccaccaactaaagataattgtatcttgacttgtcacaggtttgaatttaaattccaccccttactagctgtgtgtcctctgacaatgcaggtaacctcgctgtgcctgctcttcatcagcagaatggagataatggtatctcagagggctgccgtcaagttcaaagacatccagtgtgaagtgcctgggaggagcaggcacctgagaattcattcgttccttggatatccaagaccacttcttctctgggaaatgagagagcagaggggttgcaatccccacccttttgcctcagttcccctgccccagggcactgcccgttgcccttttcttttctttttgagacggagtcttgctctgttgccagactggagtgcaatggcgtgatctcggctca

SEQ ID NO: 10227 - RNA, 570 nt, Homo sapiens
  source 1..570: mol_type = other RNA
cagggagaaggtggaagtgcagagggttccgtctatggaacaggacggatttgaccagggtgacgacatcccggctggcattgtatccggcgcagacaatagcaacgtggattgtctcgcatttctccacgaccggctgctgcccacactcggagctgttgcctgccacgatgccagcccgaaggttctcgctgtctccagtgccctcctccatggagtaggtcttggagtggttgcctcggcgatgggatggggctcggccctgggccaggctgagctgcctgcggagggcgcggttctcctcctccacctcgcgcatgcgcacctccaggctctcgcgctcccgctggctggaggccgtgtacctggggctgtgtgcctgggactccagcggtgacagagacacgggctttccatcttcgaagctcccagaaaacaggtaaatccaggtgatggctgggatgcagagaagactcaacgaggcagccaagaatttccgtctccccctgcagattcccagcatcctctcagaagtggcaatccctaatcccagcgccgtttctctgtccg

SEQ ID NO: 10228 - RNA, 692 nt, Homo sapiens
  source 1..692: mol_type = other RNA
cagggagaaggtggaagtgcagagggttccgtctatggaacaggacggatttgaccagggtgacgacatcccggctggcattgtatccggcgcagacaatagcaacgtggattgtctcgcatttctccacgaccggctgctgcccacactcggagctgttgcctgccacgatgccagcccgaaggttctcgctgtctccagtgccctcctccatggagtaggtcttggagtggttgcctcggcgatgggatggggctcggccctgggccaggctgagctgcctgcggagggcgcggttctcctcctccacctcgcgcatgcgcacctccaggctctcgcgctcccgctggctggaggccgtgtacctggggctgtgtgcctgggactccagcggtgacagagacacgggctttccatcttcgaagctcccagaaaacaggtaaatccaggtgatggctgggatgcagagaagactcaacgaggcagccaagaatttccgtctccccctgcagattcccagcatcctctcagaagtggcaatccctaatcccagcgccgtttctctgtccggagcatgaagtcctcggcctccctcataatactctctaatctcagcggctgaccgagcccagcagaatgcgaaagggaggcagcggtggtacagcagcgtccccggcgaagaagtaaaagac

SEQ ID NO: 10229 - RNA, 827 nt, Homo sapiens
  source 1..827: mol_type = other RNA
cagggagaaggtggaagtgcagagggttccgtctatggaacaggacggatttgaccagggtgacgacatcccggctggcattgtatccggcgcagacaatagcaacgtggattgtctcgcatttctccacgaccggctgctgcccacactcggagctgttgcctgccacgatgccagcccgaaggttctcgctgtctccagtgccctcctccatggagtaggtcttggagtggttgcctcggcgatgggatggggctcggccctgggccaggctgagctgcctgcggagggcgcggttctcctcctccacctcgcgcatgcgcacctccaggctctcgcgctcccgctggctggaggccgtgtacctggggctgtgtgcctgggactccagcggtgacagagacacgggctttccatcttcgaagctcccagaaaacaggtaaatccaggtgatggctgggatgcagagaagactcaacgaggcagccaagaatttccgtctccccctgcagattcccagcatcctctcagaagtggcaatccctaatcccagcgccgtttctctgtccggagcatgaagtcctcggcctccctcataatactctctctgcccaaaccatccccagcaaaagggaggcccgggaggagggtgcagatttggccagatgatctggagctgggggaatccggccccgatagagcacaccacctcattcctgggtggcctgactttgtatttgggtttattatctctgccctgcccacacccttgggatcaggcctatttctttttttaactcccctggcacgagcagcgcacgacaaag

SEQ ID NO: 10230 - RNA, 809 nt, Homo sapiens
  source 1..809: mol_type = other RNA
cagggagaaggtggaagtgcagagggttccgtctatggaacaggacggatttgaccagggtgacgacatcccggctggcattgtatccggcgcagacaatagcaacgtggattgtctcgcatttctccacgaccggctgctgcccacactcggagctgttgcctgccacgatgccagcccgaaggttctcgctgtctccagtgccctcctccatggagtaggtcttggagtggttgcctcggcgatgggatggggctcggccctgggccaggctgagctgcctgcggagggcgcggttctcctcctccacctcgcgcatgcgcacctccaggctctcgcgctcccgctggctggaggccgtgtacctggggctgtgtgcctgggactccagcggtgacagagacacgggctttccatcttcgaagctcccagaaaacaggtaaatccaggtgatggctgggatgcagagaagactcaacgaggcagccaagaatttccgtctccccctgcagattcccagcatcctctcagaagtggcaatccctaatcccagcgccgtttctctgtccggagcatgaagtcctcggcctccctcataatactctctctgcggcgatgagcctcaccgtgcacgttggcaggcatagcagattctgtttctgatgccattaccgtgtcggagaagaacattatatgaaaaaatactatctaatatcctagagaccattaaagtgtcaaagtttaatgccaagtcttttagctcgaaggctgctcagttcttcctctgacgtgcagctctgttccagaac

SEQ ID NO: 10231 - RNA, 755 nt, Homo sapiens
  source 1..755: mol_type = other RNA
cagggagaaggtggaagtgcagagggttccgtctatggaacaggacggatttgaccagggtgacgacatcccggctggcattgtatccggcgcagacaatagcaacgtggattgtctcgcatttctccacgaccggctgctgcccacactcggagctgttgcctgccacgatgccagcccgaaggttctcgctgtctccagtgccctcctccatggagtaggtcttggagtggttgcctcggcgatgggatggggctcggccctgggccaggctgagctgcctgcggagggcgcggttctcctcctccacctcgcgcatgcgcacctccaggctctcgcgctcccgctggctggaggccgtgtacctggggctgtgtgcctgggactccagcggtgacagagacacgggctttccatcttcgaagctcccagaaaacaggtaaatccaggtgatggctgggatgcagagaagactcaacgaggcagccaagaatttccgtctccccctgcagattcccagcatcctctcagaagtggcaatccctaatcccagcgccgtttctctgtccggagcatgaagtcctcggcctccctcataatactctctggctcacgacaggtgctttacaaacggctgatgcatctgaatgcgtttcttaatgtaggttctaatctcagcggctgaccgagcccagcagaatgcgaaagggaggcagcggtggtacagcagcgtccccggcgaagaagtaaaagac

SEQ ID NO: 10232 - RNA, 890 nt, Homo sapiens
  source 1..890: mol_type = other RNA
cagggagaaggtggaagtgcagagggttccgtctatggaacaggacggatttgaccagggtgacgacatcccggctggcattgtatccggcgcagacaatagcaacgtggattgtctcgcatttctccacgaccggctgctgcccacactcggagctgttgcctgccacgatgccagcccgaaggttctcgctgtctccagtgccctcctccatggagtaggtcttggagtggttgcctcggcgatgggatggggctcggccctgggccaggctgagctgcctgcggagggcgcggttctcctcctccacctcgcgcatgcgcacctccaggctctcgcgctcccgctggctggaggccgtgtacctggggctgtgtgcctgggactccagcggtgacagagacacgggctttccatcttcgaagctcccagaaaacaggtaaatccaggtgatggctgggatgcagagaagactcaacgaggcagccaagaatttccgtctccccctgcagattcccagcatcctctcagaagtggcaatccctaatcccagcgccgtttctctgtccggagcatgaagtcctcggcctccctcataatactctctggctcacgacaggtgctttacaaacggctgatgcatctgaatgcgtttcttaatgtaggttctctgcccaaaccatccccagcaaaagggaggcccgggaggagggtgcagatttggccagatgatctggagctgggggaatccggccccgatagagcacaccacctcattcctgggtggcctgactttgtatttgggtttattatctctgccctgcccacacccttgggatcaggcctatttctttttttaactcccctggcacgagcagcgcacgacaaag

SEQ ID NO: 10233 - RNA, 872 nt, Homo sapiens
  source 1..872: mol_type = other RNA
cagggagaaggtggaagtgcagagggttccgtctatggaacaggacggatttgaccagggtgacgacatcccggctggcattgtatccggcgcagacaatagcaacgtggattgtctcgcatttctccacgaccggctgctgcccacactcggagctgttgcctgccacgatgccagcccgaaggttctcgctgtctccagtgccctcctccatggagtaggtcttggagtggttgcctcggcgatgggatggggctcggccctgggccaggctgagctgcctgcggagggcgcggttctcctcctccacctcgcgcatgcgcacctccaggctctcgcgctcccgctggctggaggccgtgtacctggggctgtgtgcctgggactccagcggtgacagagacacgggctttccatcttcgaagctcccagaaaacaggtaaatccaggtgatggctgggatgcagagaagactcaacgaggcagccaagaatttccgtctccccctgcagattcccagcatcctctcagaagtggcaatccctaatcccagcgccgtttctctgtccggagcatgaagtcctcggcctccctcataatactctctggctcacgacaggtgctttacaaacggctgatgcatctgaatgcgtttcttaatgtaggttctctgcggcgatgagcctcaccgtgcacgttggcaggcatagcagattctgtttctgatgccattaccgtgtcggagaagaacattatatgaaaaaatactatctaatatcctagagaccattaaagtgtcaaagtttaatgccaagtcttttagctcgaaggctgctcagttcttcctctgacgtgcagctctgttccagaac

SEQ ID NO: 10234 - RNA, 1150 nt, Homo sapiens
  source 1..1150: mol_type = other RNA
cagggagaaggtggaagtgcagagggttccgtctatggaacaggacggatttgaccagggtgacgacatcccggctggcattgtatccggcgcagacaatagcaacgtggattgtctcgcatttctccacgaccggctgctgcccacactcggagctgttgcctgccacgatgccagcccgaaggttctcgctgtctccagtgccctcctccatggagtaggtcttggagtggttgcctcggcgatgggatggggctcggccctgggccaggctgagctgcctgcggagggcgcggttctcctcctccacctcgcgcatgcgcacctccaggctctcgcgctcccgctggctggaggccgtgtacctggggctgtgtgcctgggactccagcggtgacagagacacgggctttccatcttcgaagctcccagaaaacaggtaaatccaggtgatggctgggatgcagagaagactcaacgaggcagccaagaatttccgtctccccctgcagattcccagcatcctctcagaagtggcaatccctaatcccagcgccgtttctctgtccggagcatgaagtcctcggcctccctcataatactctctggctcacgacaggtgctttacaaacggctgatgcatctgaatgcgtttcttaatgtaggttcttggccgtgactgccgccaggcagagggagacacggaagaacagggtggcgcggcggcgccgccgcctacgaggcgcagggggtccgggtcagggtcccggcaggcgctgccctactcggagcggcggtgccaagcacagagttcgggactgcccccggctccaaatgccgcggcgagggtccgggtcccccaagctgagcactgtcccttcttcctcttcctccggggccgctgcctggagctgctcccggcccgggggactcttccgagccaggggcgccccgcatgggcaggggcctgggtcagcctcgggttgggtccagggagcgaccgccggggccgactccacctcccgcgctccaagccgattcgtcccttcagggcagggcctgcccgcgaacagcccggcgagacgagcgcggccgcgcccccagcttcgggcgcccgggctccggcgcggcggcggggcaggagcagact

SEQ ID NO: 10235 - RNA, 1087 nt, Homo sapiens
  source 1..1087: mol_type = other RNA
cagggagaaggtggaagtgcagagggttccgtctatggaacaggacggatttgaccagggtgacgacatcccggctggcattgtatccggcgcagacaatagcaacgtggattgtctcgcatttctccacgaccggctgctgcccacactcggagctgttgcctgccacgatgccagcccgaaggttctcgctgtctccagtgccctcctccatggagtaggtcttggagtggttgcctcggcgatgggatggggctcggccctgggccaggctgagctgcctgcggagggcgcggttctcctcctccacctcgcgcatgcgcacctccaggctctcgcgctcccgctggctggaggccgtgtacctggggctgtgtgcctgggactccagcggtgacagagacacgggctttccatcttcgaagctcccagaaaacaggtaaatccaggtgatggctgggatgcagagaagactcaacgaggcagccaagaatttccgtctccccctgcagattcccagcatcctctcagaagtggcaatccctaatcccagcgccgtttctctgtccggagcatgaagtcctcggcctccctcataatactctcttggccgtgactgccgccaggcagagggagacacggaagaacagggtggcgcggcggcgccgccgcctacgaggcgcagggggtccgggtcagggtcccggcaggcgctgccctactcggagcggcggtgccaagcacagagttcgggactgcccccggctccaaatgccgcggcgagggtccgggtcccccaagctgagcactgtcccttcttcctcttcctccggggccgctgcctggagctgctcccggcccgggggactcttccgagccaggggcgccccgcatgggcaggggcctgggtcagcctcgggttgggtccagggagcgaccgccggggccgactccacctcccgcgctccaagccgattcgtcccttcagggcagggcctgcccgcgaacagcccggcgagacgagcgcggccgcgcccccagcttcgggcgcccgggctccggcgcggcggcggggcaggagcagact

SEQ ID NO: 10236 - RNA, 101 nt, Homo sapiens
  source 1..101: mol_type = other RNA
cagggcagagggcacaggaatctgaggtgactggcacagaagactcaggcctgtggctcctccctcaggactgcttcctatccatgacggtctcctggtac

SEQ ID NO: 10237 - RNA, 73 nt, Homo sapiens
  source 1..73: mol_type = other RNA
cagggcagggaaggtgggagagccgagccgagtcagctgtgggaacttgtctccttcaccgagcttggtaact

SEQ ID NO: 10238 - RNA, 1492 nt, Homo sapiens
  source 1..1492: mol_type = other RNA
cagggccaggcacagagtaagactcaaaacatgttttggaatgtatgactggtatgaactacaaaccagtaagctgatgttttcattttgagtctataaatctaattttgtggtggttttgtgtatggctcaaggctcaaattgtaaaatttaatattatgtgaccaaagaaagttatacccagaacctcaatttcctcaccttcaaaatggggcagtttctcactcattggtctgctgtcacgattttaatgagctcatgcacaaacagccctttatataaggtaagtgctggataaatgttggctactataataaaataagcctctaagatacttggtcagcacaagtactacccaagagtatgcactgtaagtaaactgacaaaattgtgtatctaaaactggccagatgaaagagaaacttttaaggggcccttctgcgtgcccgacactgtgctaggcactcacactatcccgacccgagaaaccgatctgcgacccagaggaacttaccaagcctccagcatcttgtgcagccctactcatgggaccatctggatacccacccttgtctttacagggagcagaacacacctcttatgtgtcagaaaacaaagtccaggaagtatatttttacctgaggcaatatctgaaaattgtatgctacagcctccaaagtgagtcttcctctcagtacctctcttctaggcacatggagccctttcttccaagtattatgtttaaccacttaatgaatgaagtcctgaaactgcttacccatgctccctataatctctgagtaatcttccttttccacaacctcaggcataatctcatcttctgtttctattacaatttcaaattctggaaaaaggaagttgtggtctggaattatatggtccagatgatctggttgtgcacaagcctgcttatgtcccaatctccagtctagggtctgatgctccttgctgcagtaatatgctttgtggcatctggagcacgttttggggcctaaacagccacaaaccctgcagagatgagcaccagacttaagctggagacacactgattctcctgtttctgggggaggattctcagaaggtggctcatatgagtaaaaatcgtttttcctgggtagttgattcctaaaaactcgcaggccggcacagcacggctgctcgcggcagcagaagaggaagatgcagcggtggaaggcgtccgggcggccaggcagcggcgcatacacctgcagcaggaaggagagcgggcggccgcacagctcgcaggccagggcctggggccccggcagcccggccgcgcccagccatgccggccgcccgcccaccttgctggggaactgctcgctgcgcagtcgccacgccggcgccgactcggcgaagcccagctccacaggcctggccccggcggcagccatgcggggcgcgggctggcgtggggcgcagcccacagctgggtcggaaggcggaaatc

SEQ ID NO: 10239 - RNA, 1393 nt, Homo sapiens
  source 1..1393: mol_type = other RNA
cagggccaggcacagagtaagactcaaaacatgttttggaatgtatgactggtatgaactacaaaccagtaagctgatgttttcattttgagtctataaatctaattttgtggtggttttgtgtatggctcaaggctcaaattgtaaaatttaatattatgtgaccaaagaaagttatacccagaacctcaatttcctcaccttcaaaatggggcagtttctcactcattggtctgctgtcacgattttaatgagctcatgcacaaacagccctttatataaggtaagtgctggataaatgttggctactataataaaataagcctctaagatacttggtcagcacaagtactacccaagagtatgcactgtaagtaaactgacaaaattgtgtatctaaaactggccagatgaaagagaaacttttaaggggcccttctgcgtgcccgacactgtgctaggcactcacactatcccgacccgagaaaccgatctgcgacccagaggaacttaccaagcctccagcatcttgtgcagccctactcatgggaccatctggatacccacccttgtctttacagggagcagaacacacctcttatgtgtcagaaaacaaagtccaggaagtatatttttacctgaggcaatatctgaaaattgtatgctacagcctccaaagtgagtcttcctctcagtacctctcttctaggcacatggagccctttcttccaagtattatgtttaaccacttaatgaatgaagtcctgaaactgcttacccatgctccctataatctctgagtaatcttccttttccacaacctcaggcataatctcatcttctgtttctattacaatttcaaattctggaaaaaggaagttgtggtctggaattatatggtccagatgatctggttgtgcacaagcctgcttatgtcccaatctccagtctagggtctgatgctccttgctgcagtaatatgctttgtggcatctggagcacgttttggggcctaaacagccacaaaccctgcagagatgagcaccagacttaagctggagacacactgattctcctgtttctgggggaggattctcagaaggtggctcatatgagtaaaaatcgtttttcctgggtagttgattcctaaaaactcgcaggccggcacagcacggctgctcgcggcagcagaagaggaagatgcagcggtggaaggcgtccgggcggccaggcagcggcgcatacaccttgctggggaactgctcgctgcgcagtcgccacgccggcgccgactcggcgaagcccagctccacaggcctggccccggcggcagccatgcggggcgcgggctggcgtggggcgcagcccacagctgggtcggaaggcggaaatc

SEQ ID NO: 10240 - RNA, 631 nt, Homo sapiens
  source 1..631: mol_type = other RNA
cagggccaggcacagagtaagcagcctccaacgtgaccttcagtagattgccccctgagatctgggctgtggtcagtaaaggctctgccactaatactttaacttcaagactgcactgcttagcacttgatctaggagtttctaagggtgagccttgcacagggtgcaatggaactgttgtttgaaatgaactctgtccttccagtaagggaagaaggtccaccacagcctgaccaagaattaaggtcttctcttctttctgtttcttttcctttggtaaaacttcagtcacagttaagaacacaggtttgtgagcgaggtcatctgaagtgattcctccttcaggattaaactcaaaactgctagtgaagttgtattttgcacttccttctggagaaacagtaatttttgcagagtctcccagaaccacttgattgaattctgctcgaataaaggtaactggagtatctcctttaaaacctttcaaatcatatccctctgtcacggtgatctgcacgagtctgcctgctgatggcacttgctccatatcaccaactgggaaaagtccctctgttttctttggtctctgcagcagcctcagttatgtttttgacaactatagcaaccaact

SEQ ID NO: 10241 - RNA, 2075 nt, Homo sapiens
  source 1..2075: mol_type = other RNA
cagggccaggcacagagtaagcagcctccaacgtgaccttcagtagattgccccctgagatctgggctgtggtcagtaaaggctctgccactaatactttaacttcaagactgcactgcttagcacttgatctaggagtttctaagggtgagccttgcacagggtgcaatggaactgttgtttgaaatgaactctgtccttccagtaagggaagaaggtccaccacagcctgaccaagaattaaggtcttctcttctttctgtttcttttcctttggtaaaacttcagtcacagttaagaacacaggtttgtgagcgaggtcatctgaagtgattcctccttcaggattaaactcaaaactgctagtgaagttgtattttgcacttccttctggagaaacagtaatttttgcagagtctcccagaaccacttgattgaattctgctcgaataaaggtaactggagtatctcctttaaaacctttcaaatcatatccctctgtcacggtgatctgcacgagtctgcctgctgatggcacttgctccatatcaccaactgggaaaagtccctctgttttctttggtctcttgccaagagttgggtttaagtgcataggtttccacctttacattttgctttctcgactctttgatttcaatatttctcatttgacaactactgaggaggatgactcaggcaggagtcttcaatggacgctaaggctggtgggtagatgttctatgaggcatagaatactggcgtgattttggaatgcttccatggaatactacttgattacagagggggaaacagtgaatggacgcaaccaacatgatcaggtgatcatggttaacatcaccagtgttgggaggagtctacattgtgagcctcctggtgaaacacactaaaaaaaaacacacacacacacacaaagcatcctttttggttttcctaccatgaaaggaactcaggttgtagaccatccaaggacaagaaagactgggaactgtctctgactgaggttatatgacaactaaattcaatatgtatctctgtatagcattctggaccagaaaggaaaacaacattgttaggacggtgggaaaaatgtgaattagctctgtgaatcgcataccaccccgaacatgcccaatctcatctgaattggatggtagtgttgtaccaatattgatttcctgatgtggaagtttgtttgttgttaggtaggagagtgtccctgtttaggggaaaataaacactagtgtgtttaggagtgatgagacaccatctcttcaatttgctctcttgactttcaaaaggtccagaaaaagactaacaagggatacatacacatgtacacacacatatgcacatgcatgcacacctgcacacatacacacacagtgagcaatggaacaagtgcaataaagtgttaactatttgggaatctgagtgcaggggacatgggacttccttacacgatttgggcaacttttctatacattcgagatcatttcaaaacaattaaaatatatacacacgcataaccactctccctgggaagccctttgcttaggaaatagttaccagagtcaaattttaaaatttttatttatatgaataaagaaacattataaatattgagaaatattttttgaaagttgcagtgttacaggtaataaaggttctcaaaataaaactactgtggcactactgagtaaggatttctctctggattttttttcccaagtgagagttttgggtgaatttgcactgagacagctatcccacttgcaaatgacagactctttctacataataagctgggttaggccaagtctttaatagggagctgttcttccagaaatcgctcatgatcttggtctacttagtactttgcttcaaggtcttaggcaagcaaggataaataacagatgtcacctccttaaacataattaatctccattcaactttagggtacctgagagcaagggctgtatgttacaattttctttttttttttttttaagatggagtctcactctgtagcccaggctggagtgccgtggcgcaat

SEQ ID NO: 10242 - RNA, 673 nt, Homo sapiens
  source 1..673: mol_type = other RNA
cagggccaggcacagagtaagcagcctccaacgtgaccttcagtagattgccccctgagatctgggctgtggtcagtaaaggctctgccactaatactttaacttcaagactgcactgcttagcacttgatctaggagtttctaagggtgagccttgcacagggtgcaatggaactgttgtttgaaatgaactctgtccttccagtaagggaagaaggtccaccacagcctgaccaagaattaaggtcttctcttctttctgtttcttttcctttggtaaaacttcagtcacagttaagaacacaggtttgtgagcgaggtcatctgaagtgattcctccttcaggattaaactcaaaactgctagtgaagttgtattttgcacttccttctggagaaacagtaatttttgcagagtctcccagaaccacttgattgaattctgctcgaataaaggtaactggagtatctcctttaaaacctttcaaatcatatccctctgtcacggtgatctgcacgagtctgcctgctgatggcacttgctccatatcaccaactgggaaaagtccctctgttttctttggtctttttggccatcgcacgagcaagtttattccaagactcgcgataaccctctggggccgggagcagggagcgagacgctgagcttctgc

SEQ ID NO: 10243 - RNA, 2229 nt, Homo sapiens
  source 1..2229: mol_type = other RNA
cagggccaggcacagagtaagcagcctccaacgtgaccttcagtagattgccccctgagatctgggctgtggtcagtaaaggctctgccactaatactttaacttcaagactgcactgcttagcacttgatctaggagtttctaagggtgagccttgcacagggtgcaatggaactgttgtttgaaatgaactctgtccttccagtaagggaagaaggtccaccacagcctgaccaagaattaaggtcttctcttctttctgtttcttttcctttggtaaaacttcagtcacagttaagaacacaggtttgtgagcgaggtcatctgaagtgattcctccttcaggattaaactcaaaactgctagtgaagttgtattttgcacttccttctggagaaacagtaatttttgcagagtctcccagaaccacttgattgaattctgctcgaataaaggtaactggagtatctcctttaaaacctttcaaatcatatccctctgtcacggtgatctgcacgagtctgcctgctgatggcacttgctccatatcaccaactgggaaaagtccctctgttttctttggtctttttggccatcgcacgagcaagtttattccaagactcgcgataaccctctggggccgggagcagggagcgagacgctgagcttctgcgcctgcgccctagcgccggctgcagcctcctcacttcgagagcctgctgtttccgcggatgctttaccttgccaagagttgggtttaagtgcataggtttccacctttacattttgctttctcgactctttgatttcaatatttctcatttgacaactactgaggaggatgactcaggcaggagtcttcaatggacgctaaggctggtgggtagatgttctatgaggcatagaatactggcgtgattttggaatgcttccatggaatactacttgattacagagggggaaacagtgaatggacgcaaccaacatgatcaggtgatcatggttaacatcaccagtgttgggaggagtctacattgtgagcctcctggtgaaacacactaaaaaaaaacacacacacacacacaaagcatcctttttggttttcctaccatgaaaggaactcaggttgtagaccatccaaggacaagaaagactgggaactgtctctgactgaggttatatgacaactaaattcaatatgtatctctgtatagcattctggaccagaaaggaaaacaacattgttaggacggtgggaaaaatgtgaattagctctgtgaatcgcataccaccccgaacatgcccaatctcatctgaattggatggtagtgttgtaccaatattgatttcctgatgtggaagtttgtttgttgttaggtaggagagtgtccctgtttaggggaaaataaacactagtgtgtttaggagtgatgagacaccatctcttcaatttgctctcttgactttcaaaaggtccagaaaaagactaacaagggatacatacacatgtacacacacatatgcacatgcatgcacacctgcacacatacacacacagtgagcaatggaacaagtgcaataaagtgttaactatttgggaatctgagtgcaggggacatgggacttccttacacgatttgggcaacttttctatacattcgagatcatttcaaaacaattaaaatatatacacacgcataaccactctccctgggaagccctttgcttaggaaatagttaccagagtcaaattttaaaatttttatttatatgaataaagaaacattataaatattgagaaatattttttgaaagttgcagtgttacaggtaataaaggttctcaaaataaaactactgtggcactactgagtaaggatttctctctggattttttttcccaagtgagagttttgggtgaatttgcactgagacagctatcccacttgcaaatgacagactctttctacataataagctgggttaggccaagtctttaatagggagctgttcttccagaaatcgctcatgatcttggtctacttagtactttgcttcaaggtcttaggcaagcaaggataaataacagatgtcacctccttaaacataattaatctccattcaactttagggtacctgagagcaagggctgtatgttacaattttctttttttttttttttaagatggagtctcactctgtagcccaggctggagtgccgtggcgcaat

SEQ ID NO: 10244 - RNA, 514 nt, Homo sapiens
  source 1..514: mol_type = other RNA
cagggccaggcacagagtaagcagcctccaacgtgaccttcagtagattgccccctgagatctgggctgtggtcagtaaaggctctgccactaatactttaacttcaagactgcactgcttagcacttgatctaggagtttctaagggtgagccttgcacagggtgcaatggaactgttgtttgaaatgaactctgtccttccagtaagggaagaaggtccaccacagcctgaccaagaattaaggtcttctcttctttctgtttcttttcctttggtaaaacttcagtcacagttaagaacacaggtttgtgagcgaggtcatctgaagtgattcctccttcaggattaaactcaaaactgctagtgaagttgtattttgcacttccttctggagaaacagtaatttttgcagagtctcccagaaccacttgattgaattctgctcgaataaaggtaactggagtatctcctttaaaacctttctgcagcagcctcagttatgtttttgacaa

SEQ ID NO: 10245 - RNA, 554 nt, Homo sapiens
  source 1..554: mol_type = other RNA
cagggccaggcacagagtaagcagcctccaacgtgaccttcagtagattgccccctgagatctgggctgtggtcagtaaaggctctgccactaatactttaacttcaagactgcactgcttagcacttgatctaggagtttctaagggtgagccttgcacagggtgcaatggaactgttgtttgaaatgaactctgtccttccagtaagggaagaaggtccaccacagcctgaccaagaattaaggtcttctcttctttctgtttcttttcctttggtaaaacttcagtcacagttaagaacacaggtttgtgagcgaggtcatctgaagtgattcctccttcaggattaaactcaaaactgctagtgaagttgtattttgcacttccttctggagaaacagtaatttttgcagagtctcccagaaccacttgattgaattctgctcgaataaaggtaactggagtatctcctttaaaacctttttttggccatcgcacgagcaagtttattccaagactcgcgataaccctctggggccgggagcagggagcg

SEQ ID NO: 10246 - RNA, 538 nt, Homo sapiens
  source 1..538: mol_type = other RNA
cagggccaggcacagagtaagcagcctccaacgtgaccttcagtagattgccccctgagatctgggctgtggtcagtaaaggctctgccactaatactttaacttcaagactgcactgcttccagtaagggaagaaggtccaccacagcctgaccaagaattaaggtcttctcttctttctgtttcttttcctttggtaaaacttcagtcacagttaagaacacaggtttgtgagcgaggtcatctgaagtgattcctccttcaggattaaactcaaaactgctagtgaagttgtattttgcacttccttctggagaaacagtaatttttgcagagtctcccagaaccacttgattgaattctgctcgaataaaggtaactggagtatctcctttaaaacctttcaaatcatatccctctgtcacggtgatctgcacgagtctgcctgctgatggcacttgctccatatcaccaactgggaaaagtccctctgttttctttggtctctgcagcagcctcagttatgtttttgacaact

SEQ ID NO: 10247 - RNA, 2149 nt, Homo sapiens
  source 1..2149: mol_type = other RNA
cagggccaggcacagagtaagcagcctccaacgtgaccttcagtagattgccccctgagatctgggctgtggtcagtaaaggctctgccactaatactttaacttcaagactgcactgcttccagtaagggaagaaggtccaccacagcctgaccaagaattaaggtcttctcttctttctgtttcttttcctttggtaaaacttcagtcacagttaagaacacaggtttgtgagcgaggtcatctgaagtgattcctccttcaggattaaactcaaaactgctagtgaagttgtattttgcacttccttctggagaaacagtaatttttgcagagtctcccagaaccacttgattgaattctgctcgaataaaggtaactggagtatctcctttaaaacctttcaaatcatatccctctgtcacggtgatctgcacgagtctgcctgctgatggcacttgctccatatcaccaactgggaaaagtccctctgttttctttggtctttttggccatcgcacgagcaagtttattccaagactcgcgataaccctctggggccgggagcagggagcgagacgctgagcttctgcgcctgcgccctagcgccggctgcagcctcctcacttcgagagcctgctgtttccgcggatgctttaccttgccaagagttgggtttaagtgcataggtttccacctttacattttgctttctcgactctttgatttcaatatttctcatttgacaactactgaggaggatgactcaggcaggagtcttcaatggacgctaaggctggtgggtagatgttctatgaggcatagaatactggcgtgattttggaatgcttccatggaatactacttgattacagagggggaaacagtgaatggacgcaaccaacatgatcaggtgatcatggttaacatcaccagtgttgggaggagtctacattgtgagcctcctggtgaaacacactaaaaaaaaacacacacacacacacaaagcatcctttttggttttcctaccatgaaaggaactcaggttgtagaccatccaaggacaagaaagactgggaactgtctctgactgaggttatatgacaactaaattcaatatgtatctctgtatagcattctggaccagaaaggaaaacaacattgttaggacggtgggaaaaatgtgaattagctctgtgaatcgcataccaccccgaacatgcccaatctcatctgaattggatggtagtgttgtaccaatattgatttcctgatgtggaagtttgtttgttgttaggtaggagagtgtccctgtttaggggaaaataaacactagtgtgtttaggagtgatgagacaccatctcttcaatttgctctcttgactttcaaaaggtccagaaaaagactaacaagggatacatacacatgtacacacacatatgcacatgcatgcacacctgcacacatacacacacagtgagcaatggaacaagtgcaataaagtgttaactatttgggaatctgagtgcaggggacatgggacttccttacacgatttgggcaacttttctatacattcgagatcatttcaaaacaattaaaatatatacacacgcataaccactctccctgggaagccctttgcttaggaaatagttaccagagtcaaattttaaaatttttatttatatgaataaagaaacattataaatattgagaaatattttttgaaagttgcagtgttacaggtaataaaggttctcaaaataaaactactgtggcactactgagtaaggatttctctctggattttttttcccaagtgagagttttgggtgaatttgcactgagacagctatcccacttgcaaatgacagactctttctacataataagctgggttaggccaagtctttaatagggagctgttcttccagaaatcgctcatgatcttggtctacttagtactttgcttcaaggtcttaggcaagcaaggataaataacagatgtcacctccttaaacataattaatctccattcaactttagggtacctgagagcaagggctgtatgttacaattttctttttttttttttttaagatggagtctcactctgtagcccaggctggagtgccgtggcgcaat

SEQ ID NO: 10248 - RNA, 436 nt, Homo sapiens
  source 1..436: mol_type = other RNA
cagggccaggcacagagtaagcagcctccaacgtgaccttcagtagattgccccctgagatctgggctgtggtcagtaaaggctctgccactaatactttaacttcaagactgcactgcttccagtaagggaagaaggtccaccacagcctgaccaagaattaaggtcttctcttctttctgtttcttttcctttggtaaaacttcagtcacagttaagaacacaggtttgtgagcgaggtcatctgaagtgattcctccttcaggattaaactcaaaactgctagtgaagttgtattttgcacttccttctggagaaacagtaatttttgcagagtctcccagaaccacttgattgaattctgctcgaataaaggtaactggagtatctcctttaaaacctttctgcagcagcctcagttatgtttttgacaact

SEQ ID NO: 10249 - RNA, 2047 nt, Homo sapiens
  source 1..2047: mol_type = other RNA
cagggccaggcacagagtaagcagcctccaacgtgaccttcagtagattgccccctgagatctgggctgtggtcagtaaaggctctgccactaatactttaacttcaagactgcactgcttccagtaagggaagaaggtccaccacagcctgaccaagaattaaggtcttctcttctttctgtttcttttcctttggtaaaacttcagtcacagttaagaacacaggtttgtgagcgaggtcatctgaagtgattcctccttcaggattaaactcaaaactgctagtgaagttgtattttgcacttccttctggagaaacagtaatttttgcagagtctcccagaaccacttgattgaattctgctcgaataaaggtaactggagtatctcctttaaaacctttttttggccatcgcacgagcaagtttattccaagactcgcgataaccctctggggccgggagcagggagcgagacgctgagcttctgcgcctgcgccctagcgccggctgcagcctcctcacttcgagagcctgctgtttccgcggatgctttaccttgccaagagttgggtttaagtgcataggtttccacctttacattttgctttctcgactctttgatttcaatatttctcatttgacaactactgaggaggatgactcaggcaggagtcttcaatggacgctaaggctggtgggtagatgttctatgaggcatagaatactggcgtgattttggaatgcttccatggaatactacttgattacagagggggaaacagtgaatggacgcaaccaacatgatcaggtgatcatggttaacatcaccagtgttgggaggagtctacattgtgagcctcctggtgaaacacactaaaaaaaaacacacacacacacacaaagcatcctttttggttttcctaccatgaaaggaactcaggttgtagaccatccaaggacaagaaagactgggaactgtctctgactgaggttatatgacaactaaattcaatatgtatctctgtatagcattctggaccagaaaggaaaacaacattgttaggacggtgggaaaaatgtgaattagctctgtgaatcgcataccaccccgaacatgcccaatctcatctgaattggatggtagtgttgtaccaatattgatttcctgatgtggaagtttgtttgttgttaggtaggagagtgtccctgtttaggggaaaataaacactagtgtgtttaggagtgatgagacaccatctcttcaatttgctctcttgactttcaaaaggtccagaaaaagactaacaagggatacatacacatgtacacacacatatgcacatgcatgcacacctgcacacatacacacacagtgagcaatggaacaagtgcaataaagtgttaactatttgggaatctgagtgcaggggacatgggacttccttacacgatttgggcaacttttctatacattcgagatcatttcaaaacaattaaaatatatacacacgcataaccactctccctgggaagccctttgcttaggaaatagttaccagagtcaaattttaaaatttttatttatatgaataaagaaacattataaatattgagaaatattttttgaaagttgcagtgttacaggtaataaaggttctcaaaataaaactactgtggcactactgagtaaggatttctctctggattttttttcccaagtgagagttttgggtgaatttgcactgagacagctatcccacttgcaaatgacagactctttctacataataagctgggttaggccaagtctttaatagggagctgttcttccagaaatcgctcatgatcttggtctacttagtactttgcttcaaggtcttaggcaagcaaggataaataacagatgtcacctccttaaacataattaatctccattcaactttagggtacctgagagcaagggctgtatgttacaattttctttttttttttttttaagatggagtctcactctgtagcccaggctggagtgccgtggcgcaat

SEQ ID NO: 10250 - RNA, 2072 nt, Homo sapiens
  source 1..2072: mol_type = other RNA
cagggccaggcacagagtaagcagcctccaacgtgaccttcagtagattgccccctgagatctgggctgtggtcagtaaaggctctgccactaatactttaacttcaagactgcacttagcacttgatctaggagtttctaagggtgagccttgcacagggtgcaatggaactgttgtttgaaatgaactctgtccttccagtaagggaagaaggtccaccacagcctgaccaagaattaaggtcttctcttctttctgtttcttttcctttggtaaaacttcagtcacagttaagaacacaggtttgtgagcgaggtcatctgaagtgattcctccttcaggattaaactcaaaactgctagtgaagttgtattttgcacttccttctggagaaacagtaatttttgcagagtctcccagaaccacttgattgaattctgctcgaataaaggtaactggagtatctcctttaaaacctttcaaatcatatccctctgtcacggtgatctgcacgagtctgcctgctgatggcacttgctccatatcaccaactgggaaaagtccctctgttttctttggtctcttgccaagagttgggtttaagtgcataggtttccacctttacattttgctttctcgactctttgatttcaatatttctcatttgacaactactgaggaggatgactcaggcaggagtcttcaatggacgctaaggctggtgggtagatgttctatgaggcatagaatactggcgtgattttggaatgcttccatggaatactacttgattacagagggggaaacagtgaatggacgcaaccaacatgatcaggtgatcatggttaacatcaccagtgttgggaggagtctacattgtgagcctcctggtgaaacacactaaaaaaaaacacacacacacacacaaagcatcctttttggttttcctaccatgaaaggaactcaggttgtagaccatccaaggacaagaaagactgggaactgtctctgactgaggttatatgacaactaaattcaatatgtatctctgtatagcattctggaccagaaaggaaaacaacattgttaggacggtgggaaaaatgtgaattagctctgtgaatcgcataccaccccgaacatgcccaatctcatctgaattggatggtagtgttgtaccaatattgatttcctgatgtggaagtttgtttgttgttaggtaggagagtgtccctgtttaggggaaaataaacactagtgtgtttaggagtgatgagacaccatctcttcaatttgctctcttgactttcaaaaggtccagaaaaagactaacaagggatacatacacatgtacacacacatatgcacatgcatgcacacctgcacacatacacacacagtgagcaatggaacaagtgcaataaagtgttaactatttgggaatctgagtgcaggggacatgggacttccttacacgatttgggcaacttttctatacattcgagatcatttcaaaacaattaaaatatatacacacgcataaccactctccctgggaagccctttgcttaggaaatagttaccagagtcaaattttaaaatttttatttatatgaataaagaaacattataaatattgagaaatattttttgaaagttgcagtgttacaggtaataaaggttctcaaaataaaactactgtggcactactgagtaaggatttctctctggattttttttcccaagtgagagttttgggtgaatttgcactgagacagctatcccacttgcaaatgacagactctttctacataataagctgggttaggccaagtctttaatagggagctgttcttccagaaatcgctcatgatcttggtctacttagtactttgcttcaaggtcttaggcaagcaaggataaataacagatgtcacctccttaaacataattaatctccattcaactttagggtacctgagagcaagggctgtatgttacaattttctttttttttttttttaagatggagtctcactctgtagcccaggctggagtgccgtggcgcaat

SEQ ID NO: 10251 - RNA, 200 nt, Homo sapiens
  source 1..200: mol_type = other RNA
cagggccaggcacagagtaagcagcctccaacgtgaccttcagtagattgccccctgagatctgggctgtggtcagtaaaggctctgccactaatactttaacttcaagactgcacttccagtaagggaagaaggtccaccacagcctgaccaagaattaaggtcttctcttctttctgtttcttttcctttggtaaaac

SEQ ID NO: 10252 - RNA, 132 nt, Homo sapiens
  source 1..132: mol_type = other RNA
cagggcctcactgtatcgcccaggctggagtgcagtggtgcaatctcggctcactgcaacctctgcctcccaggttcaagcaattctcgtgcctcagcctccaaagtagctgggattacaggcacccgtcac

SEQ ID NO: 10253 - RNA, 2551 nt, Homo sapiens
  source 1..2551: mol_type = other RNA
cagggctggcagtgacatgggtgacagccgtgatgccccaaatcatagcttccagttgagcacctgtcacagcagcgcccgaccacaagaggtttacactggcactggcctccaagtcggctgcagctggatccgactgagccctgggggtgacacttgcaggccacagccccatcatgcagcttggcagacatgctgatgatcagcctttcacaggcacccgggagcacttgaggtcccattgctgaggcaatttcaacacagttgtgaagctgatactcatctaagtcctgcttgctgcagaaattctccaatgaattgatttggggaataaggccaagagagtccaccaggacatgtgaatgagcgtgggactctccttgcaaaggctgagaaaaatagacatctatggaatattgtacatctggttctaaacagatgggtgtgggaagcagcatgattctcgtagccgctggtaaggcaaaagactgaggctttgactgtagagtcttgggtatgcagtgctcactccctccaggggggttcaccacaatctggacagtccagtcagctgcagactgggtttcatagtgaatggcaatggtgaagtccacaggaaagggaatgttgttgacagcaaatctcaagccagccccagggagaaccctggcaaatccaggtccagtccatgtaacagggttcccaggaactggctctcctaaaacaacgtgaacagcaggactctggccaaacgtctccgagcccaaaggcgccagtccttggagtgttgtggcttcctctgcctcgtagagatagaaattcaaaggagcaaagaagtagccaggggctggttcagagcagctacggccagtgacatgtgggcggcattcacactgcccattcttgggtgagcacacgttagaataagcacctccaatatcacagtcacagggagaacacccatggagatgatttcccaggccccagtatccaacagtgcattcttcgcagtgtgctccggtgacatatgacaggcacaagcattggcctgtatccacatcacaggtcaagaatggcagactcccaagggggttacagtcgcagggctggcagcccagggggtcggtggcgcttagtccgtagtggttgggtttgcactggtcgcatttggctccttccacgttctctttacaaaggcactggccggccacagaccctaaggcaggatcagagtggctcacacaaatgccaccagatatggtcccatcggggtcacattcacaaggaatgcacgcgtagggatctgagatggtcttgagcgggtccctgtagaagaggggtctgcagcggtcgcagtgctgcccctcagtgttgtgctggcagtcttcacacacgcccccgctgaggccaccgcttgccaggtacgtagtcatgtcaaagtgacagcggctggagtggctattacagctgcacgatctgcaagcgttgtcctggaggtctgcagctggcctccaaggagcatcctggaagaagtccttgcatctctcacagttcggaccatctgtattgtgctgacacacacactgaccgtgaaccattccaggagggctgaaaacatctccccgcatcttctgcatagggcgacattcgctagcatggccattgcaaaagcagcttccccgaacaatcatctcgtacagagcatagtagtatttatcaagggaatcattttgcctccttccaagcaaagcatccccaagggtgtggagcttggtaaagtttatcctcaggtttgtcaatgtcacaaggtcttggatgtaggggctataagggttttcaatttcaaaactgggatccaaaacttttaaaacaacctctccacctgttgagggttcaatatccgagtatttggagtcacaaacaatgtctcccactccctgggcctggccagatgtgatgttaggaaaggaagtggcacagtcttttgcaaaatatttgaacactttccagttgtgtccatagtctgtggaacgttcaactaacattgcagcaggccgaaaagtcttaaaggtcaggataaggtggctgaaccgaaataatgcctctaagtccagtctgatgctgacatgatcaagaccattttcagattgccaccatttcttttctctgtctggttcaaaacttacaatgacattctcaatggtgtggctgttgggttggtcatacggatcatatggaaatctagagtcacagatgaagcatttttgttccccctccaggtaactgaggatgcagtatttctgggctctgctcagcccacaggtagaagaagccataagctgcgtgttcctgcccaccaggagatcaccagtggtgggatgacaggcacccctgttgcagtcatcttgagcttttgagtaactgagccacccaaggtgcaaaaaaagggtcagttgaaattgcattcttttgtcaggagatgattaaattcaattcaggatctgggagtctttgtggagaggttcaggcagcaaacggggcatgtgaagac

SEQ ID NO: 10254 - RNA, 2549 nt, Homo sapiens
  source 1..2549: mol_type = other RNA
cagggctggcagtgacatgggtgacagccgtgatgccccaaatcatagcttccagttgagcacctgtcacagcagcgcccgaccacaagaggtttacactggcactggcctccaagtcggctgcagctggatccgactgagccctgggggtgacacttgcaggccacagccccatcatgcagcttggcagacatgctgatgatcagcctttcacaggcacccgggagcacttgaggtcccattgctgaggcaatttcaacacagttgtgaagctgatactcatctaagtcctgcttgctgcagaaattctccaatgaattgatttggggaataaggccaagagagtccaccaggacatgtgaatgagcgtgggactctccttgcaaaggctgagaaaaatagacatctatggaatattgtacatctggttctaaacagatgggtgtgggaagcagcatgattctcgtagccgctggtaaggcaaaagactgaggctttgactgtagagtcttgggtatgcagtgctcactccctccaggggggttcaccacaatctggacagtccagtcagctgcagactgggtttcatagtgaatggcaatggtgaagtccacaggaaagggaatgttgttgacagcaaatctcaagccagccccagggagaaccctggcaaatccaggtccagtccatgtaacagggttcccaggaactggctctcctaaaacaacgtgaacagcaggactctggccaaacgtctccgagcccaaaggcgccagtccttggagtgttgtggcttcctctgcctcgtagagatagaaattcaaaggagcaaagaagtagccaggggctggttcagagcagctacggccagtgacatgtgggcggcattcacactgcccattcttgggtgagcacacgttagaataagcacctccaatatcacagtcacagggagaacacccatggagatgatttcccaggccccagtatccaacagtgcattcttcgcagtgtgctccggtgacatatgacaggcacaagcattggcctgtatccacatcacaggtcaagaatggcagactcccaagggggttacagtcgcagggctggcagcccagggggtcggtggcgcttagtccgtagtggttgggtttgcactggtcgcatttggctccttccacgttctctttacaaaggcactggccggccacagaccctaaggcaggatcagagtggctcacacaaatgccaccagatatggtcccatcggggtcacattcacaaggaatgcacgcgtagggatctgagatggtcttgagcgggtccctgtagaagaggggtctgcagcggtcgcagtgctgcccctcagtgttgtgctggcagtcttcacacacgcccccgctgaggccaccgcttgccaggtacgtagtcatgtcaaagtgacagcggctggagtggctattacagctgcacgatctgcaagcgttgtcctggaggtctgcagctggcctccaaggagcatcctggaagaagtccttgcatctctcacagttcggaccatctgtattgtgctgacacacacactgaccgtgaaccattccaggagggctgaaaacatctccccgcatcttctgcatagggcgacattcgctagcatggccattgcaaaagcagcttccccgaacaatcatctcgtacagagcatagtagtatttatcaagggaatcattttgcctccttccaagcaaagcatccccaagggtgtggagcttggtaaagtttatcctcaggtttgtcaatgtcacaaggtcttggatgtaggggctataagggttttcaatttcaaaactgggatccaaaacttttaaaacaacctctccacctgttgagggttcaatatccgagtatttggagtcacaaacaatgtctcccactccctgggcctggccagatgtgatgttaggaaaggaagtggcacagtcttttgcaaaatatttgaacactttccagttgtgtccatagtctgtggaacgttcaactaacattgcagcaggccgaaaagtcttaaaggtcaggataaggtggctgaaccgaaataatgcctctaagtccagtctgatgctgacatgatcaagaccattttcagattgccaccatttcttttctctgtctggttcaaaacttacaatgacattctcaatggtgtggctgttgggttggtcatacggatcatatggaaatctagagtcacagatgaagcatttttgttccccctccaggtaactgaggatgcagtatttctgggctctgctcagcccacaggtagaagaagccataagctgcgtgttcctgcccaccaggagatcaccagtggtgggatgacaggcacccctgttgcagtcatcttgagcttttgagtaactgagccacccaaggtgcaaaaaaagggtcagttgaaattgcattcttttgtcaggagatgattaaattcaattctacaggatctgggagtctttgtggagaggttcaggcagcaaacggggcatgtg

SEQ ID NO: 10255 - RNA, 2554 nt, Homo sapiens
  source 1..2554: mol_type = other RNA
cagggctggcagtgacatgggtgacagccgtgatgccccaaatcatagcttccagttgagcacctgtcacagcagcgcccgaccacaagaggtttacactggcactggcctccaagtcggctgcagctggatccgactgagccctgggggtgacacttgcaggccacagccccatcatgcagcttggcagacatgctgatgatcagcctttcacaggcacccgggagcacttgaggtcccattgctgaggcaatttcaacacagttgtgaagctgatactcatctaagtcctgcttgctgcagaaattctccaatgaattgatttggggaataaggccaagagagtccaccaggacatgtgaatgagcgtgggactctccttgcaaaggctgagaaaaatagacatctatggaatattgtacatctggttctaaacagatgggtgtgggaagcagcatgattctcgtagccgctggtaaggcaaaagactgaggctttgactgtagagtcttgggtatgcagtgctcactccctccaggggggttcaccacaatctggacagtccagtcagctgcagactgggtttcatagtgaatggcaatggtgaagtccacaggaaagggaatgttgttgacagcaaatctcaagccagccccagggagaaccctggcaaatccaggtccagtccatgtaacagggttcccaggaactggctctcctaaaacaacgtgaacagcaggactctggccaaacgtctccgagcccaaaggcgccagtccttggagtgttgtggcttcctctgcctcgtagagatagaaattcaaaggagcaaagaagtagccaggggctggttcagagcagctacggccagtgacatgtgggcggcattcacactgcccattcttgggtgagcacacgttagaataagcacctccaatatcacagtcacagggagaacacccatggagatgatttcccaggccccagtatccaacagtgcattcttcgcagtgtgctccggtgacatatgacaggcacaagcattggcctgtatccacatcacaggtcaagaatggcagactcccaagggggttacagtcgcagggctggcagcccagggggtcggtggcgcttagtccgtagtggttgggtttgcactggtcgcatttggctccttccacgttctctttacaaaggcactggccggccacagaccctaaggcaggatcagagtggctcacacaaatgccaccagatatggtcccatcggggtcacattcacaaggaatgcacgcgtagggatctgagatggtcttgagcgggtccctgtagaagaggggtctgcagcggtcgcagtgctgcccctcagtgttgtgctggcagtcttcacacacgcccccgctgaggccaccgcttgccaggtacgtagtcatgtcaaagtgacagcggctggagtggctattacagctgcacgatctgcaagcgttgtcctggaggtctgcagctggcctccaaggagcatcctggaagaagtccttgcatctctcacagttcggaccatctgtattgtgctgacacacacactgaccgtgaaccattccaggagggctgaaaacatctccccgcatcttctgcatagggcgacattcgctagcatggccattgcaaaagcagcttccccgaacaatcatctcgtacagagcatagtagtatttatcaagggaatcattttgcctccttccaagcaaagcatccccaagggtgtggagcttggtaaagtttatcctcaggtttgtcaatgtcacaaggtcttggatgtaggggctataagggttttcaatttcaaaactgggatccaaaacttttaaaacaacctctccacctgttgagggttcaatatccgagtatttggagtcacaaacaatgtctcccactccctgggcctggccagatgtgatgttaggaaaggaagtggcacagtcttttgcaaaatatttgaacactttccagttgtgtccatagtctgtggaacgttcaactaacattgcagcaggccgaaaagtcttaaaggtcaggataaggtggctgaaccgaaataatgcctctaagtccagtctgatgctgacatgatcaagaccattttcagattgccaccatttcttttctctgtctggttcaaaacttacaatgacattctcaatggtgtggctgttgggttggtcatacggatcatatggaaatctagagtcacagatgaagcatttttgttccccctccaggtaactgaggatgcagtatttctgggctctgctcagcccacaggtagaagaagccataagctgcgtgttcctgcccaccaggagatcaccagtggtgggatgacaggcacccctgttgcagtcatcttgagcttttgagtaactgagccacccaaggtgcaaaaaaagggtcagttgaaattgcattcttttgtcaggagatgattaaattcaattctacaggatctgggagtctttgtggagaggttcaggcagcaaacggggcatgtgaagac

SEQ ID NO: 10256 - RNA, 5263 nt, Homo sapiens
  source 1..5263: mol_type = other RNA
cagggtcagctgagcatggaacatggggccaccccaaacgccgtacagcacaaccattaccaacactgtctattgctagagcacagcttcctgcatacataggacactgggcttctgactgcaagtttctcctttccaaaagccagctctaagacttgtctctcttctcatagtcactaagtcatttgcaaagccccagggtccatttcaaattctagagattctagtgagcatcaaggtttacaacccaatcgaggagaacaagatctgtggtgtgctccaccatgccatggttaagcaacgcagacagggcctgtgtctcaggagcaggcgccctctcggtgggccgccagaaccctcggcggactgaaagcaaaggcagcaaggctgggtggcaggcaacgtgggctcaggtgtactcggttttgcggatataattggagggaacgtagcccttcttcccgttaacctcagctaaccaccactctgtatttcctgtaacatctttaaactcgaggatcttgagtttctgattggctgacacgctcagctcatttgggtttcgtgccttgaaggtgtagacagcaaaatagacctggttgccttctgcctcactgccatctggctctgtacttctgtcttccggagcctgggctgttcttgcacatcctttgacgaggtcttgactttgcccatttcgtcctggtacggagtagccaactatttctggatgcctgaagttccggtagctcctcggcgtggcagtgggttgctttacatctctagctacatctgcagagtcccctgaccttggctgggaggtggagtctgggtctgaagggcatctggaaggactactctctgaattactcggatttagggatgcactgagagttccttggtcacattcttttggcggaggagatgcatcttgaggctgcttctggcaagaccccgaggtaaaggatacagccatgctgctggggttgaaggtcagggtgctgccgctgttctggcgtgggaacctgggggaggagctgccgtgctcagactctgtggaggagtggctacccacggaggcatcggagtggctgcggcgaggattgtagggctttaggaaagagctgtacacgaagcctttggtgactccattgtcaatcagccagcggttctggctgcccatggggtcttttttcttaatcacacccaccaggtcaccttccaaaagtgagacatccaagtcttgagcagcattgaagttccgttctgcctggaagagtttttcagggggatacctggccaggagggaggcccggagttcttctgactgtagcatgtaacttggcaggcccaggagtggctttcgagcagactggcggtcaatggttttcctctcaaatggcttcttggtagctggaagagactccgggaagaaggtaaaaacctggagttgctgcagaactctgctgtgctcttcgtggaagatggcaataaggtttccctctctgccagccactttgagtaacgaaagcagtggctttaattgctccagagcctggtgcacaaagtcacagtgggcttcagcatagccgtggacacagttggtgaagaggccctgggcgtactggtggaacttgggcagctcatccagcagctgtgcattcagggcctcatagttgttccgggccgactgcagctcctccagggtcttcttgtcctttagcttttctgcccgttctgtacagttatagaagtccaggagcttgtcaaagcgtttctgtaccagcttatggggccctgtaaacatgctcagtaactgatttaagggggagatgacaagccgctctgtcctctccttaaagtttgtgaagagctggtcactgatgtagcgatgcaccctctcaaactgctccaggtcccggtgtcctctctccatgcacacatcccacatgctcacagcagccaccactttcacacatgcggactcccggatgtgctggaggtagagagacaggtctcggataaaagacttaatcaatctttcttgcattcggaagtttttttctgtttcttcaaatacttcatcttttatctgaggagcaaagccagtgagatgcttcaggtgactgctaactcggttggatttcttgatgatggagtggatgttcagtttggaaattttctccataaggctatcttcatcacccttacggtacttgaggaccaggtcctttcgccgtttatattcattaatgttaacgttgatttccttgaccgcaaggactgcattggttaaaggcactttatctgggtgggattctggggtggaattcagcaactccattagcaacagcgggtaacgcattactctctgtactggtttgatgaggaaggagcccaggttaatataatttgtgcatccccattcgttgtataggctcttcagatctgccaaggagtcctgaagatgcttctggatcttctcatccttctcgtagatttcaagcagcgcaatggcctcatcatgattctggcagtaaatcttgtatgttccctcaagctcatcccggtgaccaagaaacacaggtcctacagcatcgctgatttccagagcagccaataattgcttcgagaccttaatcaccatctgcatatttccaaaaagtccctcaaaatcaatgtttggtacctgtgcctgctgcatgggtaccatgatccgctcaatacacatttccagatcccgaatgtagtctctttctgtctgaagaagttcttctatgaccttggctctcttctccagcatcctctgctctggattttcggcagacacagacccagaaggggccaccagtgatgaagactgggaggagaggagcgtcatttctcttagttgctggagttccatattcaaactttcaatgttactttcacagaacttgagatcctcgagggtctctgctcttgatgattcatcctgcttctcctccagcatgaggtttagctcttcttgagctctactgtacatatccaagtcccgctccatttcctcaatcctcaccagcactaaggggcatggggaggtctggtccagactccttcccatatgaccagggccctccttttctaaggtctcacaggtaggacggtgtcgagataggagcttgggggataccgcattcgttctctgctgtgctgagggaggcaggggagctgggcgagagggtcgcaccaccaagggtggtgcaggttttaggttctggtcaaccagcaaatggggagaagtggataccggagtacagggacgaggtggcggtggccttagggcctttctcctttccggcagctcctgctcggtgattaactttgaggaacctcggacaatatccttctcagagttaaagtccatgattgaaaagtggcgtaaaattttatctggctctgtgccgggccctgccaagctcttctcaaactcgatcagctgttgtgtcagcttcgagtccaggtcagtgctgccgtctccctgtgaatgtgttgctgcttccataacaagcccttgggcttgcggaccaggcttcatctccaatctctctgagatggagtaaacactggacgtgtggtgctttttagtataacttgctaggttgtggagctgaggacttgattgtctgggtttgactacccttgaagctgaaacagaagagcccctgtaaagagggagcactggcttctgaagagtttttagctgggaatacattcttttgggaggtaggctggcatagtctctagtccttgcttctaggggaagaaggtcggggtactgttctgagtgcgggtggctccctcccactgtagaataatactggcttttctgcaagttgggatgaaaagggacctgaggttgggaggaaataccattgactacttctgtagggtcagatgtgggagagtctgtggcaagaggcatttcccactccacgcctgggcttctcgggggccctcctgcggtgtcctcgtcctgataagagtttctgtctgtgtcatactctgaagtcagatgaccgaggggagaagtgggtgcttcagaaataatgcagtcaggctcctcggcctcatggtcactggtttcatgtctttgttcctctactcctaaggtgttctccaaacaatccaaagaagtttccgggatcctggcaaggctgccttcctggggcagagccatggtttcctccacccgtgtgtcaggacataatttcacaaaccggtaaggaaagatgcctgtcctgcccttcagggatccttccagccagccatcttccaaggtcgccagaattcggattttatccccgacctcgaaatccagctcatttggctccagggcttggaatctgtacagggcgaccccataggtccctggctcctcctcatcctcatccggccctatctcttcttctcctacaggggtatctacttcaccattaacaatgcagtcatcttgatttccagaacttactgactcatccacagtcctcaggggccccaacagctctacaaaaccttctggaaaaatgcctcttcggccctctaactccccttcaaaccagcctggttcaggaactccaataatggtgatcacatccccttccctgaagtccagctcttcatccagctgagcagaaagccccattagggcccgggcttgtcccatggaatattccggaatctgaaacagggcgctctgggagtgccactgccggctctgtgaggagaggcagagctcgcggacacatgaagatgggaagaagccccgtgcgccccagcagcttcggccctgcagccagcctgcagtgggaatgccatcgagaatcaccaggtcacctcgatggaggggaagattatccaactcttgggatgtgaattcacaaatgcacacaaacagcctctctccctcttttagactgggaatggtcacaatttccacaaaactgctggggaattgtcctgtaacatcctccttctttcctagaagccaaaattcatccaccactgccagcacctcaataatatctcccacaaagagcggcagttcttctgatacgctagggcagaagtcaaaaatggctcgaaccactgagccagcctccatgttttataacctgctttccgccgcccggcggtccctcggcgcggcaggcagttgcagccgccagtccccagcccgctgtcacctccgcccctggaagcggcgggcgggtcgatcccgtgt

SEQ ID NO: 10257 - RNA, 5340 nt, Homo sapiens
  source 1..5340: mol_type = other RNA
cagggtcagctgagcatggaacatggggccaccccaaacgccgtacagcacaaccattaccaacactgtctattgctagagcacagcttcctgcatacataggacactgggcttctgactgcaagtttctcctttccaaaagccagctctaagacttgtctctcttctcatagtcactaagtcatttgcaaagccccagggtccatttcaaattctagagattctagtgagcatcaaggtttacaacccaatcgaggagaacaagatctgtggtgtgctccaccatgccatggttaagcaacgcagacagggcctgtgtctcaggagcaggcgccctctcggtgggccgccagaaccctcggcggactgaaagcaaaggcagcaaggctgggtggcaggcaacgtgggctcaggtgtactcggttttgcggatataattggagggaacgtagcccttcttcccgttaacctcagctaaccaccactctgtatttcctgtaacatctttaaactcgaggatcttgagtttctgattggctgacacgctcagctcatttgggtttcgtgccttgaaggtgtagacagcaaaatagacctggttgccttctgcctcactgccatctggctctgtacttctgtcttccggagcctgggctgttcttgcacatcctttgacgaggtcttgactttgcccatttcgtcctggtacggagtagccaactatttctggatgcctgaagttccggtagctcctcggcgtggcagtgggttgctttacatctctagctacatctgcagagtcccctgaccttggctgggaggtggagtctgggtctgaagggcatctggaaggactactctctgaattactcggatttagggatgcactgagagttccttggtcacattcttttggcggaggagatgcatcttgaggctgcttctggcaagaccccgaggtaaaggatacagccatgctgctggggttgaaggtcagggtgctgccgctgttctggcgtgggaacctgggggaggagctgccgtgctcagactctgtggaggagtggctacccacggaggcatcggagtggctgcggcgaggattgtagggctttaggaaagagctgtacacgaagcctttggtgactccattgtcaatcagccagcggttctggctgcccatggggtcttttttcttaatcacacccaccaggtcaccttccaaaagtgagacatccaagtcttgagcagcattgaagttccgttctgcctggaagagtttttcagggggatacctggccaggagggaggcccggagttcttctgactgtagcatgtaacttggcaggcccaggagtggctttcgagcagactggcggtcaatggttttcctctcaaatggcttcttggtagctggaagagactccgggaagaaggtaaaaacctggagttgctgcagaactctgctgtgctcttcgtggaagatggcaataaggtttccctctctgccagccactttgagtaacgaaagcagtggctttaattgctccagagcctggtgcacaaagtcacagtgggcttcagcatagccgtggacacagttggtgaagaggccctgggcgtactggtggaacttgggcagctcatccagcagctgtgcattcagggcctcatagttgttccgggccgactgcagctcctccagggtcttcttgtcctttagcttttctgcccgttctgtacagttatagaagtccaggagcttgtcaaagcgtttctgtaccagcttatggggccctgtaaacatgctcagtaactgatttaagggggagatgacaagccgctctgtcctctccttaaagtttgtgaagagctggtcactgatgtagcgatgcaccctctcaaactgctccaggtcccggtgtcctctctccatgcacacatcccacatgctcacagcagccaccactttcacacatgcggactcccggatgtgctggaggtagagagacaggtctcggataaaagacttaatcaatctttcttgcattcggaagtttttttctgtttcttcaaatacttcatcttttatctgaggagcaaagccagtgagatgcttcaggtgactgctaactcggttggatttcttgatgatggagtggatgttcagtttggaaattttctccataaggctatcttcatcacccttacggtacttgaggaccaggtcctttcgccgtttatattcattaatgttaacgttgatttccttgaccgcaaggactgcattggttaaaggcactttatctgggtgggattctggggtggaattcagcaactccattagcaacagcgggtaacgcattactctctgtactggtttgatgaggaaggagcccaggttaatataatttgtgcatccccattcgttgtataggctcttcagatctgccaaggagtcctgaagatgcttctggatcttctcatccttctcgtagatttcaagcagcgcaatggcctcatcatgattctggcagtaaatcttgtatgttccctcaagctcatcccggtgaccaagaaacacaggtcctacagcatcgctgatttccagagcagccaataattgcttcgagaccttaatcaccatctgcatatttccaaaaagtccctcaaaatcaatgtttggtacctgtgcctgctgcatgggtaccatgatccgctcaatacacatttccagatcccgaatgtagtctctttctgtctgaagaagttcttctatgaccttggctctcttctccagcatcctctgctctggattttcggcagacacagacccagaaggggccaccagtgatgaagactgggaggagaggagcgtcatttctcttagttgctggagttccatattcaaactttcaatgttactttcacagaacttgagatcctcgagggtctctgctcttgatgattcatcctgcttctcctccagcatgaggtttagctcttcttgagctctactgtacatatccaagtcccgctccatttcctcaatcctcaccagcactaaggggcatggggaggtctggtccagactccttcccatatgaccagggccctccttttctaaggtctcacaggtaggacggtgtcgagataggagcttgggggataccgcattcgttctctgctgtgctgagggaggcaggggagctgggcgagagggtcgcaccaccaagggtggtgcaggttttaggttctggtcaaccagcaaatggggagaagtggataccggagtacagggacgaggtggcggtggccttagggcctttctcctttccggcagctcctgctcggtgattaactttgaggaacctcggacaatatccttctcagagttaaagtccatgattgaaaagtggcgtaaaattttatctggctctgtgccgggccctgccaagctcttctcaaactcgatcagctgttgtgtcagcttcgagtccaggtcagtgctgccgtctccctgtgaatgtgttgctgcttccataacaagcccttgggcttgcggaccaggcttcatctccaatctctctgagatggagtaaacactggacgtgtggtgctttttagtataacttgctaggttgtggagctgaggacttgattgtctgggtttgactacccttgaagctgaaacagaagagcccctgtaaagagggagcactggcttctgaagagtttttagctgggaatacattcttttgggaggtaggctggcatagtctctagtccttgcttctaggggaagaaggtcggggtactgttctgagtgcgggtggctccctcccactgtagaataatactggcttttctgcaagttgggatgaaaagggacctgaggttgggaggaaataccattgactacttctgtagggtcagatgtgggagagtctgtggcaagaggcatttcccactccacgcctgggcttctcgggggccctcctgcggtgtcctcgtcctgataagagtttctgtctgtgtcatactctgaagtcagatgaccgaggggagaagtgggtgcttcagaaataatgcagtcaggctcctcggcctcatggtcactggtttcatgtctttgttcctctactcctaaggtgttctccaaacaatccaaagaagtttccgggatcctggcaaggctgccttcctggggcagagccatggtttcctccacccgtgtgtcaggacataatttcacaaaccggtaaggaaagatgcctgtcctgcccttcagggatccttccagccagccatcttccaaggtcgccagaattcggattttatccccgacctcgaaatccagctcatttggctccagggcttggaatctgtacagggcgaccccataggtccctggctcctcctcatcctcatccggccctatctcttcttctcctacaggggtatctacttcaccattaacaatgcagtcatcttgatttccagaacttactgactcatccacagtcctcaggggccccaacagctctacaaaaccttctggaaaaatgcctcttcggccctctaactccccttcaaaccagcctggttcaggaactccaataatggtgatcacatccccttccctgaagtccagctcttcatccagctgagcagaaagccccattagggcccgggcttgtcccatggaatattccggaatctgaaacagggcgctctgggagtgccactgccggctctgtgaggagaggcagagctcgcggacacatgaagatgggaagaagccccgtgcgccccagcagcttcggccctgcagccagcctgcagtgggaatgccatcgagaatcaccaggtcacctcgatggaggggaagattatccaactcttgggatgtgaattcacaaatgcacacaaacagcctctctccctcttttagactgggaatggtcacaatttccacaaaactgctggggaattgtcctgtaacatcctccttctttcctagaagccaaaattcatccaccactgccagcacctcaataatatctcccacaaagagcggcagttcttctgatacgctagggcagaagtcaaaaatggctcgaaccactgagccagcctccatgttttataactctttttaagactgagaacaagacaaagatgcccgttagtgtagcagctgttttgacacagttctagtagtcctggccaatgctgctttccgccgcccggcggtccctcggcgcggcaggcagttgcagccgccagtccccagcccgctgtcacctccgcccctggaagcggcgggcgggtcgatcc

SEQ ID NO: 10258 - RNA, 3023 nt, Homo sapiens
  source 1..3023: mol_type = other RNA
cagggtcagctgagcatggaacatggggccaccccaaacgccgtacagcacaaccattaccaacactgtctattgctagagcacagcttcctgcatacataggacactgggcttctgactgcaagtttctcctttccaaaagccagctctaagacttgtctctcttctcatagtcactaagtcatttgcaaagccccagggtccatttcaaattctagagattctagtgagcatcaaggtttacaacccaatcgaggagaacaagatctgtggtgtgctccaccatgccatggttaagcaacgcagacagggcctgtgtctcaggagcaggcgccctctcggtgggccgccagaaccctcggcggactgaaagcaaaggcagcaaggctgggtggcaggcaacgtgggctcaggtgtactcggttttgcggatataattggagggaacgtagcccttcttcccgttaacctcagctaaccaccactctgtatttcctgtaacatctttaaactcgaggatcttgagtttctgattggctgacacgctcagctcatttgggtttcgtgccttgaaggtgtagacagcaaaatagacctggttgccttctgcctcactgccatctggctctgtacttctgtcttccggagcctgggctgttcttgcacatcctttgacgaggtcttgactttgcccatttcgtcctggtacggagtagccaactatttctggatgcctgaagttccggtagctcctcggcgtggcagtgggttgctttacatctctagctacatctgcagagtcccctgaccttggctgggaggtggagtctgggtctgaagggcatctggaaggactactctctgaattactcggatttagggatgcactgagagttccttggtcacattcttttggcggaggagatgcatcttgaggctgcttctggcaagaccccgaggtaaaggatacagccatgctgctggggttgaaggtcagggtgctgccgctgttctggcgtgggaacctgggggaggagctgccgtgctcagactctgtggaggagtggctacccacggaggcatcggagtggctgcggcgaggattgtagggctttaggaaagagctgtacacgaagcctttggtgactccattgtcaatcagccagcggttctggctgcccatggggtcttttttcttaatcacacccaccaggtcaccttccaaaagtgagacatccaagtcttgagcagcattgaagttccgttctgcctggaagagtttttcagggggatacctggccaggagggaggcccggagttcttctgactgtagcatgtaacttggcaggcccaggagtggctttcgagcagactggcggtcaatggttttcctctcaaatggcttcttggtagctggaagagactccgggaagaaggtaaaaacctggagttgctgcagaactctgctgtgctcttcgtggaagatggcaataaggtttccctctctgccagccactttgagtaacgaaagcagtggctttaattgctccagagcctggtgcacaaagtcacagtgggcttcagcatagccgtggacacagttggtgaagaggccctgggcgtactggtggaacttgggcagctcatccagcagctgtgcattcagggcctcatagttgttccgggccgactgcagctcctccagggtcttcttgtcctttagcttttctgcccgttctgtacagttatagaagtccaggagcttgtcaaagcgtttctgtaccagcttatggggccctgtaaacatgctcagtaactgatttaagggggagatgacaagccgctctgtcctctccttaaagtttgtgaagagctggtcactgatgtagcgatgcaccctctcaaactgctccaggtcccggtgtcctctctccatgcacacatcccacatgctcacagcagccaccactttcacacatgcggactcccggatgtgctggaggtagagagacaggtctcggataaaagacttaatcaatctttcttgcattcggaagtttttttctgtttcttcaaatacttcatcttttatctgaggagcaaagccagtgagatgcttcaggtgactgctaactcggttggatttcttgatgatggagtggatgttcagtttggaaattttctccataaggctatcttcatcacccttacggtacttgaggaccaggtcctttcgccgtttatattcattaatgttaacgttgatttccttgaccgcaaggactgcattggttaaaggcactttatctgggtgggattctggggtggaattcagcaactccattagcaacagcgggtaacgcattactctctgtactggtttgatgaggaaggagcccaggttaatataatttgtgcatccccattcgttgtataggctcttcagatctgccaaggagtcctgaagatgcttctggatcttctcatccttctcgtagatttcaagcagcgcaatggcctcatcatgattctggcagtaaatcttgtatgttccctcaagctcatcccggtgaccaagaaacacaggtcctacagcatcgctgatttccagagcagccaataattgcttcgagaccttaatcaccatctgcatatttccaaaaagtccctcaaaatcaatgtttggtacctgtgcctgctgcatgggtaccatgatccgctcaatacacatttccagatcccgaatgtagtctctttctgtctgaagaagttcttctatgaccttggctctcttctccagcatcctctgctctggattttcggcagacacagacccagaaggggccaccagtgatgaagactgggaggagaggagcgtcatttctgcagtgcccagagctggctgtgtgtggaggtgtgggcctgagggtaagcaggcgggacagaatcttcccagagctctggaatgctccacaaccccccaaactcctttgaatagggtcggcatttcccccaggcttccc

SEQ ID NO: 10259 - RNA, 4183 nt, Homo sapiens
  source 1..4183: mol_type = other RNA
cagggtcagctgagcatggaacatggggccaccccaaacgccgtacagcacaaccattaccaacactgtctattgctagagcacagcttcctgcatacataggacactgggcttctgactgcaagtttctcctttccaaaagccagctctaagacttgtctctcttctcatagtcactaagtcatttgcaaagccccagggtccatttcaaattctagagattctagtgagcatcaaggtttacaacccaatcgaggagaacaagatctgtggtgtgctccaccatgccatggttaagcaacgcagacagggcctgtgtctcaggagcaggcgccctctcggtgggccgccagaaccctcggcggactgaaagcaaaggcagcaaggctgggtggcaggcaacgtgggctcaggtgtactcggttttgcggatataattggagggaacgtagcccttcttcccgttaacctcagctaaccaccactctgtatttcctgtaacatctttaaactcgaggatcttgagtttctgattggctgacacgctcagctcatttgggtttcgtgccttgaaggtgtagacagcaaaatagacctggttgccttctgcctcactgccatctggctctgtacttctgtcttccggagcctgggctgttcttgcacatcctttgacgaggtcttgactttgcccatttcgtcctggtacggagtagccaactatttctggatgcctgaagttccggtagctcctcggcgtggcagtgggttgctttacatctctagctacatctgcagagtcccctgaccttggctgggaggtggagtctgggtctgaagggcatctggaaggactactctctgaattactcggatttagggatgcactgagagttccttggtcacattcttttggcggaggagatgcatcttgaggctgcttctggcaagaccccgaggtaaaggatacagccatgctgctggggttgaaggtcagggtgctgccgctgttctggcgtgggaacctgggggaggagctgccgtgctcagactctgtggaggagtggctacccacggaggcatcggagtggctgcggcgaggattgtagggctttaggaaagagctgtacacgaagcctttggtgactccattgtcaatcagccagcggttctggctgcccatggggtcttttttcttaatcacacccaccaggtcaccttccaaaagtgagacatccaagtcttgagcagcattgaagttccgttctgcctggaagagtttttcagggggatacctggccaggagggaggcccggagttcttctgactgtagcatgtaacttggcaggcccaggagtggctttcgagcagactggcggtcaatggttttcctctcaaatggcttcttggtagctggaagagactccgggaagaaggtaaaaacctggagttgctgcagaactctgctgtgctcttcgtggaagatggcaataaggtttccctctctgccagccactttgagtaacgaaagcagtggctttaattgctccagagcctggtgcacaaagtcacagtgggcttcagcatagccgtggacacagttggtgaagaggccctgggcgtactggtggaacttgggcagctcatccagcagctgtgcattcagggcctcatagttgttccgggccgactgcagctcctccagggtcttcttgtcctttagcttttctgcccgttctgtacagttatagaagtccaggagcttgtcaaagcgtttctgtaccagcttatggggccctgtaaacatgctcagtaactgatttaagggggagatgacaagccgctctgtcctctccttaaagtttgtgaagagctggtcactgatgtagcgatgcaccctctcaaactgctccaggtcccggtgtcctctctccatgcacacatcccacatgctcacagcagccaccactttcacacatgcggactcccggatgtgctggaggtagagagacaggtctcggataaaagacttaatcaatctttcttgcattcggaagtttttttctgtttcttcaaatacttcatcttttatctgaggagcaaagccagtgagatgcttcaggtgactgctaactcggttggatttcttgatgatggagtggatgttcagtttggaaattttctccataaggctatcttcatcacccttacggtacttgaggaccaggtcctttcgccgtttatattcattaatgttaacgttgatttccttgaccgcaaggactgcattggttaaaggcactttatctgggtgggattctggggtggaattcagcaactccattagcaacagcgggtaacgcattactctctgtactggtttgatgaggaaggagcccaggttaatataatttgtgcatccccattcgttgtataggctcttcagatctgccaaggagtcctgaagatgcttctggatcttctcatccttctcgtagatttcaagcagcgcaatggcctcatcatgattctggcagtaaatcttgtatgttccctcaagctcatcccggtgaccaagaaacacaggtcctacagcatcgctgatttccagagcagccaataattgcttcgagaccttaatcaccatctgcatatttccaaaaagtccctcaaaatcaatgtttggtacctgtgcctgctgcatgggtaccatgatccgctcaatacacatttccagatcccgaatgtagtctctttctgtctgaagaagttcttctatgaccttggctctcttctccagcatcctctgctctggattttcggcagacacagacccagaaggggccaccagtgatgaagactgggaggagaggagcgtcatttcttgggttttcttgctgttttgcacgaactctgagcgcctcagggtgctgggtgctgtgcggcggaggcaactattccttctccaagtctctgggccatttaattttttctcttcctctaaatgccagatgttcttctctaatgacgagctctgaggaatccccaaatgatgtcctccttgttctcccctggtacactgagtctgcagaccatccagaaggatcctgctgcccccatgtgcctttgttcttggtatgtcagtgccattatactccaaattctccatttgatggagagaatctgtccctctggaattacgagatttatatgcacagtttgcaaataaagcatcatagcctttattttctgtatcaaaatcaccctgatccataatatgagtctttgctttgggatacatgttgtcattttgatgaacattcctgtccccttcatggtatttgataaattccttatcttcattgacaccattcgaatctgaaaagctcacaggctgaccatcaggataactcccaggaacatgatataaattgctgtgttctctacaataaaaattagttgcccaacaatcctcaagattatggttaacattctcatggtctatataccacaactgaggttgacctaaattcgctgaagaatcatccaaacccctacagtcagtcaactgttcagcttttttagagtcctcaggattataattcagattcttacagtctgagtagccatttgcctccccgtatccaccagctttcgaggtcacatctgggcttctcgtaggtgaattatccttcgtcccagggctgagactctcataatctacattttctggactcctataaccatcatgacctccgtggtacacacagccctttccactttcatgtgcttccccacagtccatatagcttggttcactctgttcaaaatcccagtatccacaatccctttttctgtagggctgatgctgtcccttggcccagtacctgggatccaagtcattttctctgtagagtccatccagcactgtaaggttccttttccgtacactcccgtagtcttcatactcccagctggagtcccagtgccttttctcctccacttccctttcttttctagccttctgggtttcacacatattctatgtgcttaaagacaaaggttttactattcttttccatgggcctgggctgggctgtggacaggtgcagtctagcctaaggctggatttgtcctgcttaaaatgtctcccaaccattccagacactcttctcgttgctct

SEQ ID NO: 10260 - RNA, 5135 nt, Homo sapiens
  source 1..5135: mol_type = other RNA
cagggtcagctgagcatggaacatggggccaccccaaacgccgtacagcacaaccattaccaacactgtctattgctagagcacagcttcctgcatacataggacactgggcttctgactgcaagtttctcctttccaaaagccagctctaagacttgtctctcttctcatagtcactaagtcatttgcaaagccccagggtccatttcaaattctagagattctagtgagcatcaaggtttacaacccaatcgaggagaacaagatctgtggtgtgctccaccatgccatggttaagcaacgcagacagggcctgtgtctcaggagcaggcgccctctcggtgggccgccagaaccctcggcggactgaaagcaaaggcagcaaggctgggtggcaggcaacgtgggctcaggtgtactcggttttgcggatataattggagggaacgtagcccttcttcccgttaacctcagctaaccaccactctgtatttcctgtaacatctttaaactcgaggatcttgagtttctgattggctgacacgctcagctcatttgggtttcgtgccttgaaggtgtagacagcaaaatagacctggttgccttctgcctcactgccatctggctctgtacttctgtcttccggagcctgggctgttcttgcacatcctttgacgaggtcttgactttgcccatttcgtcctggtacggagtagccaactatttctggatgcctgaagttccggtagctcctcggcgtggcagtgggttgctttacatctctagctacatctgcagagtcccctgaccttggctgggaggtggagtctgggtctgaagggcatctggaaggactactctctgaattactcggatttagggatgcactgagagttccttggtcacattcttttggcggaggagatgcatcttgaggctgcttctggcaagaccccgaggtaaaggatacagccatgctgctggggttgaaggtcagggtgctgccgctgttctggcgtgggaacctgggggaggagctgccgtgctcagactctgtggaggagtggctacccacggaggcatcggagtggctgcggcgaggattgtagggctttaggaaagagctgtacacgaagcctttggtgactccattgtcaatcagccagcggttctggctgcccatggggtcttttttcttaatcacacccaccaggtcaccttccaaaagtgagacatccaagtcttgagcagcattgaagttccgttctgcctggaagagtttttcagggggatacctggccaggagggaggcccggagttcttctgactgtagcatgtaacttggcaggcccaggagtggctttcgagcagactggcggtcaatggttttcctctcaaatggcttcttggtagctggaagagactccgggaagaaggtaaaaacctggagttgctgcagaactctgctgtgctcttcgtggaagatggcaataaggtttccctctctgccagccactttgagtaacgaaagcagtggctttaattgctccagagcctggtgcacaaagtcacagtgggcttcagcatagccgtggacacagttggtgaagaggccctgggcgtactggtggaacttgggcagctcatccagcagctgtgcattcagggcctcatagttgttccgggccgactgcagctcctccagggtcttcttgtcctttagcttttctgcccgttctgtacagttatagaagtccaggagcttgtcaaagcgtttctgtaccagcttatggggccctgtaaacatgctcagtaactgatttaagggggagatgacaagccgctctgtcctctccttccggatgtgctggaggtagagagacaggtctcggataaaagacttaatcaatctttcttgcattcggaagtttttttctgtttcttcaaatacttcatcttttatctgaggagcaaagccagtgagatgcttcaggtgactgctaactcggttggatttcttgatgatggagtggatgttcagtttggaaattttctccataaggctatcttcatcacccttacggtacttgaggaccaggtcctttcgccgtttatattcattaatgttaacgttgatttccttgaccgcaaggactgcattggttaaaggcactttatctgggtgggattctggggtggaattcagcaactccattagcaacagcgggtaacgcattactctctgtactggtttgatgaggaaggagcccaggttaatataatttgtgcatccccattcgttgtataggctcttcagatctgccaaggagtcctgaagatgcttctggatcttctcatccttctcgtagatttcaagcagcgcaatggcctcatcatgattctggcagtaaatcttgtatgttccctcaagctcatcccggtgaccaagaaacacaggtcctacagcatcgctgatttccagagcagccaataattgcttcgagaccttaatcaccatctgcatatttccaaaaagtccctcaaaatcaatgtttggtacctgtgcctgctgcatgggtaccatgatccgctcaatacacatttccagatcccgaatgtagtctctttctgtctgaagaagttcttctatgaccttggctctcttctccagcatcctctgctctggattttcggcagacacagacccagaaggggccaccagtgatgaagactgggaggagaggagcgtcatttctcttagttgctggagttccatattcaaactttcaatgttactttcacagaacttgagatcctcgagggtctctgctcttgatgattcatcctgcttctcctccagcatgaggtttagctcttcttgagctctactgtacatatccaagtcccgctccatttcctcaatcctcaccagcactaaggggcatggggaggtctggtccagactccttcccatatgaccagggccctccttttctaaggtctcacaggtaggacggtgtcgagataggagcttgggggataccgcattcgttctctgctgtgctgagggaggcaggggagctgggcgagagggtcgcaccaccaagggtggtgcaggttttaggttctggtcaaccagcaaatggggagaagtggataccggagtacagggacgaggtggcggtggccttagggcctttctcctttccggcagctcctgctcggtgattaactttgaggaacctcggacaatatccttctcagagttaaagtccatgattgaaaagtggcgtaaaattttatctggctctgtgccgggccctgccaagctcttctcaaactcgatcagctgttgtgtcagcttcgagtccaggtcagtgctgccgtctccctgtgaatgtgttgctgcttccataacaagcccttgggcttgcggaccaggcttcatctccaatctctctgagatggagtaaacactggacgtgtggtgctttttagtataacttgctaggttgtggagctgaggacttgattgtctgggtttgactacccttgaagctgaaacagaagagcccctgtaaagagggagcactggcttctgaagagtttttagctgggaatacattcttttgggaggtaggctggcatagtctctagtccttgcttctaggggaagaaggtcggggtactgttctgagtgcgggtggctccctcccactgtagaataatactggcttttctgcaagttgggatgaaaagggacctgaggttgggaggaaataccattgactacttctgtagggtcagatgtgggagagtctgtggcaagaggcatttcccactccacgcctgggcttctcgggggccctcctgcggtgtcctcgtcctgataagagtttctgtctgtgtcatactctgaagtcagatgaccgaggggagaagtgggtgcttcagaaataatgcagtcaggctcctcggcctcatggtcactggtttcatgtctttgttcctctactcctaaggtgttctccaaacaatccaaagaagtttccgggatcctggcaaggctgccttcctggggcagagccatggtttcctccacccgtgtgtcaggacataatttcacaaaccggtaaggaaagatgcctgtcctgcccttcagggatccttccagccagccatcttccaaggtcgccagaattcggattttatccccgacctcgaaatccagctcatttggctccagggcttggaatctgtacagggcgaccccataggtccctggctcctcctcatcctcatccggccctatctcttcttctcctacaggggtatctacttcaccattaacaatgcagtcatcttgatttccagaacttactgactcatccacagtcctcaggggccccaacagctctacaaaaccttctggaaaaatgcctcttcggccctctaactccccttcaaaccagcctggttcaggaactccaataatggtgatcacatccccttccctgaagtccagctcttcatccagctgagcagaaagccccattagggcccgggcttgtcccatggaatattccggaatctgaaacagggcgctctgggagtgccactgccggctctgtgaggagaggcagagctcgcggacacatgaagatgggaagaagccccgtgcgccccagcagcttcggccctgcagccagcctgcagtgggaatgccatcgagaatcaccaggtcacctcgatggaggggaagattatccaactcttgggatgtgaattcacaaatgcacacaaacagcctctctccctcttttagactgggaatggtcacaatttccacaaaactgctggggaattgtcctgtaacatcctccttctttcctagaagccaaaattcatccaccactgccagcacctcaataatatctcccacaaagagcggcagttcttctgatacgctagggcagaagtcaaaaatggctcgaaccactgagccagcctccatgttttataacctgctttccgccgcccggcggtccctcggcgcggcaggcagttgcagccgccagtccccagcccgctgtcacctccgcccctggaagcggcgggcgggtcgatcccgtgtg

SEQ ID NO: 10261 - RNA, 4082 nt, Homo sapiens
  source 1..4082: mol_type = other RNA
caggtcgtcttgcagggcttctcgcaagacgacatcctcatcaccaacgacgtgcagctccaggtagcggttctgacgcagggcagggaggtggccctcctggggggtgactctgacaccgaagaactcacacagcgtcagccagaagccaggggtgaactgcaggcctcggtgggcctgggagtgcagagcatttcgctgccagcggccagggcccaggaacagctcagccagctcctgggctgggatggtgtttgcacctacgagagcgggcatctgggtgagcagctgggtgatggctgtcgtgatgctgctgcctgcgatgagggacgaatccaggatgagtcgtagggagcgctggggctggggccgagccacccgcatggcgggtgccggccgcagcgagaggcattgcctcacgcgcagtagcacgaggatggctgccagggctagggtgttcttccagtacaggaggcctcggaagaagtgcagaatgacggccctgatctgggccatgctgaagtgggcgaggaagctgttgaggatctggtcgatgggtatcatggccagcagctcttgccgtaggatctgttcattgagctcatcctgttcttcattctcttcttccccggattccgtcgatggatccctggggaatccccttgaggccagcagcagggtttgcctggcggcagtgttcctctggaaggctctcctccaccggaggtttctcacaggtggcagagctcggccgccgtcttgttctggcagctccatgacgtcaaagttgaagtgggagaagaagaagacccaatgcccggggagaagtacggtgagcctgtcattattcagagaggctagatcctctgtgttgagaaggatcatgatgggctcctcggtgttctccaggtagcggcaccacaccatgaaggcagcccgtattggaagaatcttcatctccgcttgagagtactcaacctcgataggggagatgttgcgggagtagaaagcgcagcaggctctcttgccggtttggtcgtcgatttggatcagggaggcgtgcagggccgtgccggtgacgccggtttccaagtagaatgggttctggggcttggggtggtggaggagaggcgccttgcggaaagccctcttcaggcactcgaaggcctcttgctcctcgactccccagtagaactggtaggagctcagcagctgccgcaccaggggctctgcgatgatgctgaagcgctccacgaagtggcggtaggggaagacgaattcgatgaagtttcgcagagatagcttggagccaggggtagggtaccctgttatgatggtcatgacgttcttgttcagtttcacccctttgggggtgacgacgaagcccaggaattccacggtttggcggtggaactggctcttgtccagggagcagtagacgttgtgatggcggaagcggaccaggacttggcggacgtggtggaggtgctcctcctgactcattgagtagatcaggacttcctggccataagaaagcacaaagaaccctagcatgtcctttaggatgaagtgaatcacgttctgaggtatgatagggtctggggagagcgcaaacggctggtagctcttcatctcttcaagctccaaaccaaacgctgctttccacacatcttcggtgcggtgcccgttcacgctttcctccacaatggtcccacgcagctccagttttgtgaaccactcggctccgtgtaactggtcaaacagttccggaatcatctgtatgtagtcctgtctgttggtcagcatgtcctgcaggtcccagtattcctcctgtagcctggctctttcttgcatcctggcacccacaggttcccaaggcgcggtggagggacactcgtaaaaggtctcgctgtgatcactgtctccagcctgctgaagctcagagggctctgattcagaaagatcatcggatccgtctgagcttggctggtcggaagtctcatcatctgcttccttcgggttaaacacgtcggccaggtctgagtatgggtgtggcagtccgggtagcaggctcatgccgtgcctctctagggcaatgcatggcgggggcgggcggaagcagttcttcaggcagtagggagagtggaaggtgcagcggcctttgatccagtcgacttcgggggcgtggactcggagccagcggatgcctaggaccacagagaagttcggtgaaggtacgatgtcaaattcgatggactcctggtggttctggtggatacacaccaggggctccgtgtagagccagacaggctcgttgccaatcagcgagccgtccacggattggaccggctgtgggtacggcttctcgtagagctcgacgtagtgctcttgggcgaacttctcatccatgaagttgccgtcagctcccgaatccaccagggcctggaccgcgacgctgtggtaggggttcactctcaccatgagcagcaggaagaggtgggcgcgattgatgtccggatggacttcgctgggcaaccagctgctgaccatccacctctctggagcaggtgagtcgatccaggtcaggttccgggggcgggcctcggggggcagcctgagcatagctcttctctctgccagcttctcttctatttgcaggatgagcacaatcagactgtctagggaatccggctgagggacccggaatagatagtgcctgatctcctcgttgagcccctggcacaagtgggcctgcaggacttcatctggccagcccaagatgggtaccaggctctggaactcatcgatgtactcagtggcagagcggccgccctgcctgatggtgaacatggcctcttctgccacacgcagtgcctggcggtactcaaacacttcggacatggcctccaggaaggctgggaagtctccgatcagggggctgttttcctgcagtagagctttggcccattctaatgccaagccggacaggtgattgatgacatagccaactctcagacggtcgttatagaacattcttgggtagctctgtaaggtcagttggcagagtacgatgaactcgtggaattctctgcgatcgccagagaagtgctttggggcgggcagttggcctgcattgatccctttgatcaagatctcttctgctactctctgttgctctttgaggtcttgcattcggaagtacagcgagatgatggacctcaccatggccataagttctgcggttgagtgctcggtctggttttgctcttgaggagtctcctcccttcccgattccttcaggtcagtgtgagcctcttgttcttctcgggctcccgatgggttgactgatgcttctttcatcctatcagatgctccactgagtggatccccccttgcctggtgtgaaccgttgcatgactcctccaggtcttggagtaggtcattgggtggatcctctatttccttacgtgggccactggatggctcctccatgtcttggagtagatcagtgggcagctcttccatttcctggagtgggccactggggggctccttcttttcctgggctgggccgctggctggccctgcctctccccgcactccactgcccgacgtcgcctcggtggtgttggatgagccctcggaggactccatttgttttgatgatggattcttatgctccatcatcgtctcaaatgagtcttcagagggttctatcatttcgtcggatggaaaggagtgtattctgaagattggtaaggttgtgatggcgtccagtcagtagctgggaccgtggagatcagaaccttggctgcaagcgttcaagtggatctcctcccgtcctgtgccactcgatcctcgctgcttgcttccccgggcccagtcccaagcgtgaggctggggatgaagtgatgccggtggcttagtgatgccggtggcttcctgtcctcgaagctcagtcggtcgtctctcagctggtgtgaggctgggccaggatggaaccccagactctccgaggctccccaccacaccctgctgctgaaggctgctcagcgaggctgtgccgagtgctgggggggtgt

SEQ ID NO: 10262 - RNA, 887 nt, Homo sapiens
  source 1..887: mol_type = other RNA
caggtcgtcttgcagggcttctcggggtcggggaagacgagctggttgacaattatattgtgtgtgtcaatcttgcacttggccagctcctggatcagcctctctgtctcatacagggacaggaactcagcaatgcatacgcagatgaaagttgtctgctcagggtccttgaactgttcgctgactgagcggatgacgggcagcgtctcctccagcttggaggccagctggtctgcgttcatgtcccccaggcccagcatgttgcacatctgtgagatgaaagggctgatctggttcttgatctgcataagccggcccaggccccgctccacgatggtggggaagttgagcagcctcagggtgtggcccgtgggtgccgtgtcaaataccaccaccgagaagttcatgcccttcaccagcctcatgacctcggcatagctcatggcctcatcgatgccgggaaatgcgctcatggcctcctgcatcatcttcttgcccatgctcagcatgttgtcctcctcgaagaactcgtcaggcagctccgccacgcccaggctggggtcaatctccatagcaaagaggttgtcatagcctttgaccttggtaggcacctttgagaacttctggtcaaaagcatctgagatgttgtgtgctgggtctgtggagatgatcagaacactctcacgccccttggagagctggactgccaggctgcagctgcaggtggtcttgcccacaccacccttgcccccgacgaagatccacttcaggctgcgctgctcgatgatgttgctaagtgtaggctccagcggctccacatcaggagcatcttcgaactcctctgcctcaaccccccacccggccacccctgccgccattttggaact

SEQ ID NO: 10263 - RNA, 1013 nt, Homo sapiens
  source 1..1013: mol_type = other RNA
caggtcgtcttgcagggcttctcggggtcggggaagacgagctggttgacaattatattgtgtgtgtcaatcttgcacttggccagctcctggatcagcctctctgtctcatacagggacaggaactcagcaatgcatacgcagatgaaagttgtctgctcagggtccttgaactgttcgctgactgagcggatgacgggcagcgtctcctccagcttggaggccagctggtctgcgttcatgtcccccaggcccagcatgttgcacatctgtgagatgaaagggctgatctggttcttgatctgcataagccggcccaggccccgctccacgatggtggggaagttgagcagcctcagggtgtggcccgtgggtgccgtgtcaaataccaccaccgagaagttcatgcccttcaccagcctcatgacctcggcatagctcatggcctcatcgatgccgggaaatgcgctcatggcctcctgcatcatcttcttgcccatgctcagcatgttgtcctcctcgaagaactcgtcaggcagctccgccacgcccaggctggggtcaatctccatagcaaagaggttgtcatagcctttgaccttggtaggcacctttgagaacttctggtcaaaagcatctgagatgttgtgtgctgggtctgtggagatgatcagaacactctcacgccccttggagagctggactgccaggctgcagctgcaggtggtcttgcccacaccacccttgcccccgacgaagatccacttcaggctgcgctgctcgatgatgttgctaagtgtaggctccagcggctccacatcaggagcatcttcgaactcctctgcctcaaccccccacccggccacccctgccgccattttggaactggctcacgtgatccagcggagcgcaccatacgaagaacaccaatcactcttatgttccggtagcgccaacctcaccttagcaaccagccaaacacccagtccatgccctttcggtgaagttagatt

SEQ ID NO: 10264 - RNA, 976 nt, Homo sapiens
  source 1..976: mol_type = other RNA
caggtcgtcttgcagggcttctcggggtcggggaagacgagctggttgacaattatattgtgtgtgtcaatcttgcacttggccagctcctggatcagcctctctgtctcatacagggacaggaactcagcaatgcatacgcagatgaaagttgtctgctcagggtccttgaactgttcgctgactgagcggatgacgggcagcgtctcctccagcttggaggccagctggtctgcgttcatgtcccccaggcccagcatgttgcacatctgtgagatgaaagggctgatctggttcttgatctgcataagccggcccaggccccgctccacgatggtggggaagttgagcagcctcagggtgtggcccgtgggtgccgtgtcaaataccaccaccgagaagttcatgcccttcaccagcctcatgacctcggcatagctcatggcctcatcgatgccgggaaatgcgctcatggcctcctgcatcatcttcttgcccatgctcagcatgttgtcctcctcgaagaactcgtcaggcagctccgccacgcccaggctggggtcaatctccatagcaaagaggttgtcatagcctttgaccttggtaggcacctttgagaacttctggtcaaaagcatctgagatgttgtgtgctgggtctgtggagatgatcagaacactctcacgccccttggagagctggactgccaggctgcagctgcaggtggtcttgcccacaccacccttgcccccgacgaagatccacttcaggctgcgctgctcgatgatgttgctaagtgtaggctccagcggctccacatcaggagcatcttcgaactcctctgcctcaaccccccacccggccacccctgccgccattttggaactggctcacgtgatccagcggagcgcaccatacgaagaaccttagcaaccagccaaacacccagtccatgccctttcggtgaagttagatt

SEQ ID NO: 10265 - RNA, 3383 nt, Homo sapiens
  source 1..3383: mol_type = other RNA
caggtcgtcttgcagggcttctgctttttcatgcaacagcatctttgctgatgaaacaatttgcttggcttggcgtcttgataaatgatcaattgtccttacgagcacttcaggatttgcattagctaagtgcattagacttttgtaacctgcactgtataactgttttgctcgaccctctaaaactccagtaacttccatgagagggattaattctgcctttacacagtaagtcagcttcttggtaagttctaccaaaagggctctgtaaacccaaaactcctcaagctcctcacagaaatgtaacacacaagatgagaatgaggcagttccagtgagaagattttgtatatatcctcgaggcatattaaatttttcagatacagtccaaatgttggtctctttgagcaaggtataaagaacaaaagacagatatagcctgttgacaacgttcttgtccaccttctttccgatggcttggcctgatgctttcttcccaataaagctttcagagactccaagaatggcagctacattttgttctgctggactgagttggctaaactgcctgaagtatatcatccaatcagggttacactgtgaaaccagatcatagggggttgttaggtagattagatgaagaaggctttcaagcacaagtccttcaagacctttcttcaagtctctgtacagaatgtcacaataagctaaatctatagttcccttaaatgaagcacgtcccaactttgtaatatgaaaattatattggacctcttcttcagacttataaatagtgtctttttgtaggagtcctttttctgtcaggtatctaagtgattcaacagttatttcccagagacttttttctttcaataaaaccttttgctgaacaccaaaaaatgtaccattcatgaaatgatagatgtcatcaagattcgttgcaatcttcaaaccaatcaaagagagaaataatgtttggattcccttggtgaattcctgaacaagatggctgtaacagttttccaatggtttagttattaactccaatacctgttgtttgtctttttcttgcaatatgaggatactctccccaatagtatctattccagcacgaccagctctgccaatcatctgtttatattgattcctctttaaaaattccttagcaacatagggagctcttaaaataactcttcgagctggtaggttgacacctgccgctagggtagatgtgcaggtaaaaagacagagcactcctgtggagtaggcctcctccaagagtttcctttcatcacttgttaagccactgtggtgataggcaactccaaatgggatagtgcgctttaaaacaggacacaggttgccattgccaatattcttcaagttcttaatcacctcacatttttctttctccttatgtttcagatattccttgcttaaaaatttgcatatcatttctgctacattttcacagttcttcttactaggacaaaaaactaagcaggaataattgggaataacttctgtcaccaatgctaccaagtgatcaggatccatcttttttagggtatcagaatacttataattaagaagacgtgaaaaagtcatgccattctcagctttgctgtcaacttcatatattgtatcatttattttcagatattcttttaactcaaccttaggtacatactggtctaaattgactggtataatattctgcttgaagaaacttttgtaggtcttcaacattgtttaatgttgcactcataccaataatttgagtcgttttgctagtgtagaggatttttgctagggtcatttccagtgtagctccacggcttccttcaccaatcatgtgcaactcgtctacaacaaccagacccagactgtcaattcttccagtttcaatcaaggagttcaccaagctatgtcctttttcaatagtggcaatatagagtgatttcttttcccttcttttagttggaggaaatcttcctttgcttccagcatattcttcaacaaagaaaccgagttctataccaaaacttgacaaacctgaaatcttttcttggacaattgccacatatggaagaatcattaaaacatctttccgacagcaaagcagttcttgcagcattaaaatctcagccacgagggtttttccaccacttgttggcaaggaatatattaaattttttctttcttgcacagaattcaatgttaaacaagtatgttgccattcatataatttttcaattcccttgaattgggcataaaggtctctcactttgctgggtaatgaataaaaaggaccaaggtcatttgatgatgactcaactgttttcttagcaacattaatttcctcagataggagagtgtctttgagctgtttacttctagaaaatattggtgtctgggccttcgcatttccagtcatggcattttttagatgatctttaatactttttctcctgttcatatctgaactagttctgactttggaagaggactcatcattttgctggggttgctctatgcaattatggggcagttcctcattcacagtgttgtgagaggatgacttccaatccctttctttcatagaatgatcacccaaatcatttgaagagttctgcaaattttcaaagtatatagcctgtgaggaaggtacatcatacaaaagatcagctccaggttcaatagtgacaccttcatatccactctggttctctgtgtgcttatcagtttgtaattcagtaaggttgcctatggtagtaatgctgagtttgtttttgatactttccgagcaaagattttcagtggcaaagtctgtagcatgtttcttatgttcagggagttgcatatatttttgttccaggtcgtcaacttgagctataaaggagttttcagtaaagctatcatagtcaccaaacatgtccacttcactgtcattaggctggtctcccacccctctgtcagtgggcatgtgacgtaggaggtccgggtttgtatcaccacctccaaggacgagacattccggggaatctgagagtagaaggggctgtacctcaaccggcagtacgcccgcggttttccgcctcctgttctcagccaccatttcctcctcctctttcccctcatctccgggcacgagctcggccgcggtgggagcgccaaaaatacaccccaagcttggacggttccttttggggagagacacccgccggcggatgcgggaaccacattcatccatggcaaggacccagggccctattcagacgtcgttctcagtgacccagacgctaagcccatatggaagggagagtgggacgccggagcccgcttctacatccaccttgggaaaagaccccaagttagctctc

SEQ ID NO: 10266 - RNA, 3272 nt, Homo sapiens
  source 1..3272: mol_type = other RNA
caggtcgtcttgcagggcttctgctttttcatgcaacagcatctttgctgatgaaacaatttgcttggcttggcgtcttgataaatgatcaattgtccttacgagcacttcaggatttgcattagctaagtgcattagacttttgtaacctgcactgtataactgttttgctcgaccctctaaaactccagtaacttccatgagagggattaattctgcctttacacagtaagtcagcttcttggtaagttctaccaaaagggctctgtaaacccaaaactcctcaagctcctcacagaaatgtaacacacaagatgagaatgaggcagttccagtgagaagattttgtatatatcctcgaggcatattaaatttttcagatacagtccaaatgttggtctctttgagcaaggtataaagaacaaaagacagatatagcctgttgacaacgttcttgtccaccttctttccgatggcttggcctgatgctttcttcccaataaagctttcagagactccaagaatggcagctacattttgttctgctggactgagttggctaaactgcctgaagtatatcatccaatcagggttacactgtgaaaccagatcatagggggttgttaggtagattagatgaagaaggctttcaagcacaagtccttcaagacctttcttcaagtctctgtacagaatgtcacaataagctaaatctatagttcccttaaatgaagcacgtcccaactttgtaatatgaaaattatattggacctcttcttcagacttataaatagtgtctttttgtaggagtcctttttctgtcaggtatctaagtgattcaacagttatttcccagagacttttttctttcaataaaaccttttgctgaacaccaaaaaatgtaccattcatgaaatgatagatgtcatcaagattcgttgcaatcttcaaaccaatcaaagagagaaataatgtttggattcccttggtgaattcctgaacaagatggctgtaacagttttccaatggtttagttattaactccaatacctgttgtttgtctttttcttgcaatatgaggatactctccccaatagtatctattccagcacgaccagctctgccaatcatctgtttatattgattcctctttaaaaattccttagcaacatagggagctcttaaaataactcttcgagctggtaggttgacacctgccgctagggtagatgtgcaggtaaaaagacagagcactcctgtggagtaggcctcctccaagagtttcctttcatcacttgttaagccactgtggtgataggcaactccaaatgggatagtgcgctttaaaacaggacacaggttgccattgccaatattcttcaagttcttaatcacctcacatttttctttctccttatgtttcagatattccttgcttaaaaatttgcatatcatttctgctacattttcacagttcttcttactaggacaaaaaactaagcaggaataattgggaataacttctgtcaccaatgctaccaagtgatcaggatccatcttttttagggtatcagaatacttataattaagaagacgtgaaaaagtcatgccattctcagctttgctgtcaacttcatatattgtatcatttattttcagatattcttttaactcaactgctagtgtagaggatttttgctagggtcatttccagtgtagctccacggcttccttcaccaatcatgtgcaactcgtctacaacaaccagacccagactgtcaattcttccagtttcaatcaaggagttcaccaagctatgtcctttttcaatagtggcaatatagagtgatttcttttcccttcttttagttggaggaaatcttcctttgcttccagcatattcttcaacaaagaaaccgagttctataccaaaacttgacaaacctgaaatcttttcttggacaattgccacatatggaagaatcattaaaacatctttccgacagcaaagcagttcttgcagcattaaaatctcagccacgagggtttttccaccacttgttggcaaggaatatattaaattttttctttcttgcacagaattcaatgttaaacaagtatgttgccattcatataatttttcaattcccttgaattgggcataaaggtctctcactttgctgggtaatgaataaaaaggaccaaggtcatttgatgatgactcaactgttttcttagcaacattaatttcctcagataggagagtgtctttgagctgtttacttctagaaaatattggtgtctgggccttcgcatttccagtcatggcattttttagatgatctttaatactttttctcctgttcatatctgaactagttctgactttggaagaggactcatcattttgctggggttgctctatgcaattatggggcagttcctcattcacagtgttgtgagaggatgacttccaatccctttctttcatagaatgatcacccaaatcatttgaagagttctgcaaattttcaaagtatatagcctgtgaggaaggtacatcatacaaaagatcagctccaggttcaatagtgacaccttcatatccactctggttctctgtgtgcttatcagtttgtaattcagtaaggttgcctatggtagtaatgctgagtttgtttttgatactttccgagcaaagattttcagtggcaaagtctgtagcatgtttcttatgttcagggagttgcatatatttttgttccaggtcgtcaacttgagctataaaggagttttcagtaaagctatcatagtcaccaaacatgtccacttcactgtcattaggctggtctcccacccctctgtcagtgggcatgtgacgtaggaggtccgggtttgtatcaccacctccaaggacgagacattccggggaatctgagagtagaaggggctgtacctcaaccggcagtacgcccgcggttttccgcctcctgttctcagccaccatttcctcctcctctttcccctcatctccgggcacgagctcggccgcggtgggagcgccaaaaatacaccccaagcttggacggttccttttggggagagacacccgccggcggatgcgggaaccacattcatccatggcaaggacccagggccctattcagacgtcgttctcagtgacccagacgctaagcccatatggaagggagagtgggacgccggagcccgcttctacatccaccttgggaaaagaccccaagttagctctc

SEQ ID NO: 10267 - RNA, 3370 nt, Homo sapiens
  source 1..3370: mol_type = other RNA
caggtcgtcttgcagggcttctgctttttcatgcaacagcatctttgctgatgaaacaatttgcttggcttggcgtcttgataaatgatcaattgtccttacgagcacttcaggatttgcattagctaagtgcattagacttttgtaacctgcactgtataactgttttgctcgaccctctaaaactccagtaacttccatgagagggattaattctgcctttacacagtaagtcagcttcttggtaagttctaccaaaagggctctgtaaacccaaaactcctcaagctcctcacagaaatgtaacacacaagatgagaatgaggcagttccagtgagaagattttgtatatatcctcgaggcatattaaatttttcagatacagtccaaatgttggtctctttgagcaaggtataaagaacaaaagacagatatagcctgttgacaacgttcttgtccaccttctttccgatggcttggcctgatgctttcttcccaataaagctttcagagactccaagaatggcagctacattttgttctgctggactgagttggctaaactgcctgaagtatatcatccaatcagggttacactgtgaaaccagatcatagggggttgttaggtagattagatgaagaaggctttcaagcacaagtccttcaagacctttcttcaagtctctgtacagaatgtcacaataagctaaatctatagttcccttaaatgaagcacgtcccaactttgtaatatgaaaattatattggacctcttcttcagacttataaatagtgtctttttgtaggagtcctttttctgtcaggtatctaagtgattcaacagttatttcccagagacttttttctttcaataaaaccttttgctgaacaccaaaaaatgtaccattcatgaaatgatagatgtcatcaagattcgttgcaatcttcaaaccaatcaaagagagaaataatgtttggattcccttggtgaattcctgaacaagatggctgtaacagttttccaatggtttagttattaactccaatacctgttgtttgtctttttcttgcaatatgaggatactctccccaatagtatctattccagcacgaccagctctgccaatcatctgtttatattgattcctctttaaaaattccttagcaacatagggagctcttaaaataactcttcgagctggtaggttgacacctgccgctagggtagatgtgcaggtaaaaagacagagcactcctgtggagtaggcctcctccaagagtttcctttcatcacttgttaagccactgtggtgataggcaactccaaatgggatagtgcgctttaaaacaggacacaggttgccattgccaatattcttcaagttcttaatcacctcacatttttctttctccttatgtttcagatattccttgcttaaaaatttgcatatcatttctgctacattttcacagttcttcttactaggacaaaaaactaagcaggaataattgggaataacttctgtcaccaatgctaccaagtgatcaggatccatcttttttagggtatcagaatacttataattaagaagacgtgaaaaagtcatgccattctcagctttgctgtcaacttcatatattgtatcatttattttcagatattcttttaactcaactggtctaaattgactggtataatattctgcttgaagaaacttttgtaggtcttcaacattgtttaatgttgcactcataccaataatttgagtcgttttgctagtgtagaggatttttgctagggtcatttccagtgtagctccacggcttccttcaccaatcatgtgcaactcgtctacaacaaccagacccagactgtcaattcttccagtttcaatcaaggagttcaccaagctatgtcctttttcaatagtggcaatatagagtgatttcttttcccttcttttagttggaggaaatcttcctttgcttccagcatattcttcaacaaagaaaccgagttctataccaaaacttgacaaacctgaaatcttttcttggacaattgccacatatggaagaatcattaaaacatctttccgacagcaaagcagttcttgcagcattaaaatctcagccacgagggtttttccaccacttgttggcaaggaatatattaaattttttctttcttgcacagaattcaatgttaaacaagtatgttgccattcatataatttttcaattcccttgaattgggcataaaggtctctcactttgctgggtaatgaataaaaaggaccaaggtcatttgatgatgactcaactgttttcttagcaacattaatttcctcagataggagagtgtctttgagctgtttacttctagaaaatattggtgtctgggccttcgcatttccagtcatggcattttttagatgatctttaatactttttctcctgttcatatctgaactagttctgactttggaagaggactcatcattttgctggggttgctctatgcaattatggggcagttcctcattcacagtgttgtgagaggatgacttccaatccctttctttcatagaatgatcacccaaatcatttgaagagttctgcaaattttcaaagtatatagcctgtgaggaaggtacatcatacaaaagatcagctccaggttcaatagtgacaccttcatatccactctggttctctgtgtgcttatcagtttgtaattcagtaaggttgcctatggtagtaatgctgagtttgtttttgatactttccgagcaaagattttcagtggcaaagtctgtagcatgtttcttatgttcagggagttgcatatatttttgttccaggtcgtcaacttgagctataaaggagttttcagtaaagctatcatagtcaccaaacatgtccacttcactgtcattaggctggtctcccacccctctgtcagtgggcatgtgacgtaggaggtccgggtttgtatcaccacctccaaggacgagacattccggggaatctgagagtagaaggggctgtacctcaaccggcagtacgcccgcggttttccgcctcctgttctcagccaccatttcctcctcctctttcccctcatctccgggcacgagctcggccgcggtgggagcgccaaaaatacaccccaagcttggacggttccttttggggagagacacccgccggcggatgcgggaaccacattcatccatggcaaggacccagggccctattcagacgtcgttctcagtgacccagacgctaagcccatatggaagggagagtgggacgccggagcccgcttctacatccaccttgggaaaagaccccaagttagctctc

SEQ ID NO: 10268 - RNA, 3169 nt, Homo sapiens
  source 1..3169: mol_type = other RNA
caggtcgtcttgcagggcttctgctttttcatgcaacagcatctttgctgatgaaacaatttgcttggcttggcgtcttgataaatgatcaattgtccttacgagcacttcaggatttgcattagctaagtgcattagacttttgtaacctgcactgtataactgttttgctcgaccctctaaaactccagtaacttccatgagagggattaattctgcctttacacagtaagtcagcttcttggtaagttctaccaaaagggctctgtaaacccaaaactcctcaagctcctcacagaaatgtaacacacaagatgagaatgaggcagttccagtgagaagattttgtatatatcctcgaggcatattaaatttttcagatacagtccaaatgttggtctctttgagcaaggtataaagaacaaaagacagatatagcctgttgacaacgttcttgtccaccttctttccgatggcttggcctgatgctttcttcccaataaagctttcagagactccaagaatggcagctacattttgttctgctggactgagttggctaaactgcctgaagtatatcatccaatcagggttacactgtgaaaccagatcatagggggttgttaggtagattagatgaagaaggctttcaagcacaagtccttcaagacctttcttcaagtctctgtacagaatgtcacaataagctaaatctatagttcccttaaatgaagcacgtcccaactttgtaatatgaaaattatattggacctcttcttcagacttataaatagtgtctttttgtaggagtcctttttctgtcaggtatctaagtgattcaacagttatttcccagagacttttttctttcaataaaaccttttgctgaacaccaaaaaatgtaccattcatgaaatgatagatgtcatcaagattcgttgcaatcttcaaaccaatcaaagagagaaataatgtttggattcccttggtgaattcctgaacaagatggctgtaacagttttccaatggtttagttattaactccaatacctgttgtttgtctttttcttgcaatatgaggatactctccccaatagtatctattccagcacgaccagctctgccaatcatctgtttatattgattcctctttaaaaattccttagcaacatagggagctcttaaaataactcttcgagctggtaggttgacacctgccgctagggtagatgtgcaggtaaaaagacagagcactcctgtggagtaggcctcctccaagagtttcctttcatcacttgttaagccactgtggtgataggcaactccaaatgggatagtgcgctttaaaacaggacacaggttgccattgccaatattcttcaagttcttaatcacctcacatttttctttctccttatgtttcagatattccttgcttaaaaatttgcatatcatttctgctacattttcacagttcttcttactaggacaaaaaactaagcaggaataattgggaataacttctgtcaccaatgctaccaagtgatcaggatccatcttttttagggtatcagaatacttataattaagaagacgtgaaaaagtcatgccattctcagctttgctgtcaacttcatatattgtatcatttattttcagatattcttttaactcaactggtctaaattgactggtataatattctgcttgaagaaacttttgtaggtcttcaacattgtttaatgttgcactcataccaataatttgagtcgttttgctagtgtagaggatttttgctagggtcatttccagtgtagctccacggcttccttcaccaatcatgtgcaacttttcttggacaattgccacatatggaagaatcattaaaacatctttccgacagcaaagcagttcttgcagcattaaaatctcagccacgagggtttttccaccacttgttggcaaggaatatattaaattttttctttcttgcacagaattcaatgttaaacaagtatgttgccattcatataatttttcaattcccttgaattgggcataaaggtctctcactttgctgggtaatgaataaaaaggaccaaggtcatttgatgatgactcaactgttttcttagcaacattaatttcctcagataggagagtgtctttgagctgtttacttctagaaaatattggtgtctgggccttcgcatttccagtcatggcattttttagatgatctttaatactttttctcctgttcatatctgaactagttctgactttggaagaggactcatcattttgctggggttgctctatgcaattatggggcagttcctcattcacagtgttgtgagaggatgacttccaatccctttctttcatagaatgatcacccaaatcatttgaagagttctgcaaattttcaaagtatatagcctgtgaggaaggtacatcatacaaaagatcagctccaggttcaatagtgacaccttcatatccactctggttctctgtgtgcttatcagtttgtaattcagtaaggttgcctatggtagtaatgctgagtttgtttttgatactttccgagcaaagattttcagtggcaaagtctgtagcatgtttcttatgttcagggagttgcatatatttttgttccaggtcgtcaacttgagctataaaggagttttcagtaaagctatcatagtcaccaaacatgtccacttcactgtcattaggctggtctcccacccctctgtcagtgggcatgtgacgtaggaggtccgggtttgtatcaccacctccaaggacgagacattccggggaatctgagagtagaaggggctgtacctcaaccggcagtacgcccgcggttttccgcctcctgttctcagccaccatttcctcctcctctttcccctcatctccgggcacgagctcggccgcggtgggagcgccaaaaatacaccccaagcttggacggttccttttggggagagacacccgccggcggatgcgggaaccacattcatccatggcaaggacccagggccctattcagacgtcgttctcagtgacccagacgctaagcccatatggaagggagagtgggacgccggagcccgcttctacatccaccttgggaaaagaccccaagttagctctc

SEQ ID NO: 10269 - RNA, 3253 nt, Homo sapiens
  source 1..3253: mol_type = other RNA
cagtgcaatgttttccttggatggagctgaatctgtgtaaatagctgaggatgagaggcttatattcttggtcacaggatagggttcttgaaacatgtaagtaaccgacgtgccagcctcaaaaacagcagaaacctctacaaacaactggctgttcagctgcagtcgaaaatggccctcctccgacgtctccctggtgctccttggaaggttgtccacctgcagggaggtctccttgaggttcctctcagcccggacatagtgccattggttgtcattcagaagagaaggagactggactacaagctccacaggaccattcccaacatcgatggcaaaggtgatctctgaaggagagcttatttcgagtcgaatgaagtctttaatgccaagattttctaggaaaactccggataatgctgtggttttaaaaaagaaggaaatatcggcactgaattccgcatggaaggtaggaaagtggaggtaagaggcttctgtataaaatgagacggcgttccagaagcgtcggtcaccatagcaacgcaagggaccaattctccaagcggcttctgagtttgatctgtcggtatcagtgataactatctgagtgacaggcaagtggtctttgaaggaaagaaagccagtatcatttgtccattcatccttgtcagcgtcgcaattgcaaaagtgctgaatgtccaggcagctctcgtctaggccacactcacactgctggaccccaggaggggaacctccccagtaagggtgcctttcattggaccgcccaatccaccaggtaaatggtgttccatccggcgtgttgagcaggcgggacctcctgcagtggtaggccacctcctgctcacagtgctcagagccgtcgatcacggcctccagctgttccatgctgcccccgtagtccaaggccatggcatagggcttctcagggttagcgccccgcactcgggtcagctctgtattgttgtgctgcactgatgtccagatcttgtcctcagtgatattgcagtacacctggagaggtcccagtgggccgctgccatctgagtcgatgtagaagaagccggctgtattcccctggtgcctgtacacctcgcaggattgctcgtagatggagttgtggcaggtggcaccagtgtaacttgtgtcactgcagttacaatagaaggtagtccaggactgggagcagcttcctccatgttcacagtagtttggcaaacacctgtctttgatgctacacagatcaatgtgtaaatcactaaaattccccagggaaccttgctgaactgaaatgaggtccttgggctggttatcaataaagatgagcctcatgcagccttggaaagccttaatgggatttaaacattgggaatcggtgagattgtcggggcaccctccaaaatagtagctatttccagaataaatctgcacccaagtgctgtctggagccgggggtgctgcttcatcatccagagtgagcgtgatgcggttcctcctggcgttgatgctaaccgagtgccacaggccatcattcaagttgctgcctgtgaggatttcagctacgcgttctgtcattttctgaatcacgagtctcaggattccaccctccaggctcagcagcagggttcccgagccctcagacagctctgtggacagaagcagaccatccttgttccatgttcgaaactggaaactcactgagagcccatcaatttggggggtgccgggcagcagcaaatagctgccgctggagttgacaaatgtgatgggcacaatctgtggttcggagcaggaaaaagtgacattgcccacagtatagatctgatgctttcgtctcttagccaggtcaattatgtttactccattgtagtaaaggttttcgatgcatccatggaagtttttctttaaaaaggtcccaggttttcctggtactggaattcctccaaaactaagctcatagtcaatgtctaaggcatccgtctcgcccttggtgcggaagtgctgtgtgtgcttgtccaccgtgaagttcacctgcttgcccacccgctcaatgaggaccgagtgccagtgctggtcatccaggaggctgcccagggtggcagagggcaagctgctgctgagccgcgctttgctgtcacccaaattgaggtgtagggcgagcctccccttctggagttccaaggtgatgtggtctccacgctgaccttctccatggaacaggaccccatctccttgcatgctcttgaacttcagggagatcacatctttgagagtactcatcaacttctgattgaacctgtacagaagtgagcttcggccatcaaagtcagcaacatctgatttataggaacatccgtagacctcgactctcatgccaatcttcccactgggattccattccaggggcacaaagcgaacaaatcgggctctcactgagtgcaatagcttgtggtgcaccacgctgtcagcattcatgtttcctgcaaaggtccagatgctgtcttcttgtttgtactgtttccagttgcgtcctgtgtcactgaacatcaggctgtaactcgtcacccagtcagagcttccgtatcttccctgcgtggccactgctgtaatctctactctgtttcccaggtccatctggagccactgttgagcattggaatctgctggggaccaaccgccagttccaactctccagttgagttgagctgggctgtgagtgccagtgaggtctgaggaactggaaaaagccattggagagagcagggatgctagtggatcatcacagttgtagtttgtcgctgttaatcctaaatgccacaagccagagaacagcaaagtcaaaacgctggtcagccgtggtaaagaatccatttcccccgagtgagcggtccctcccaatcgaatcccaaattcgcagtagccagccgcggcttcttctcgctgtctctctcctctgcacagcctgaccccctcccacccccgcttggagaggcactcgctctttcactccatcccgtgcccagacgctccaccgaaaccgtggcgggggattcttcggagctgcagctggggctacggtccccgcaacagccgctagctggactcgccttcctcgcccgcctcttccttctcttcccccctccttaacggtgcaaatccaaacccaattagaacgacaggcgccggagctcggtggacagccaaatccacctcgtcgggcgcgagagctggaatc

SEQ ID NO: 10270 - RNA, 3490 nt, Homo sapiens
  source 1..3490: mol_type = other RNA
cagtgcaatgttttccttggatggagctgaatctgtgtaaatagctgaggatgagaggcttatattcttggtcacaggatagggttcttgaaacatgtaagtaaccgacgtgccagcctcaaaaacagcagaaacctcttttttgcaaaagggcccttcataaggtgaattggtgcaatcacacaggtagccattgtgcttctccacacacttgcccccgttgtggcagatgctgccgtagctgctgcagtggccggggcagcctggcctgactccagatgtgacctttgccctctcttccaggtccattttctgtccattcaagtgtaaggagcgaatgcatcctaggaagcctttctgtctggatgacgttccccctacaaacaactggctgttcagctgcagtcgaaaatggccctcctccgacgtctccctggtgctccttggaaggttgtccacctgcagggaggtctccttgaggttcctctcagcccggacatagtgccattggttgtcattcagaagagaaggagactggactacaagctccacaggaccattcccaacatcgatggcaaaggtgatctctgaaggagagcttatttcgagtcgaatgaagtctttaatgccaagattttctaggaaaactccggataatgctgtggttttaaaaaagaaggaaatatcggcactgaattccgcatggaaggtaggaaagtggaggtaagaggcttctgtataaaatgagacggcgttccagaagcgtcggtcaccatagcaacgcaagggaccaattctccaagcggcttctgagtttgatctgtcggtatcagtgataactatctgagtgacaggcaagtggtctttgaaggaaagaaagccagtatcatttgtccattcatccttgtcagcgtcgcaattgcaaaagtgctgaatgtccaggcagctctcgtctaggccacactcacactgctggaccccaggaggggaacctccccagtaagggtgcctttcattggaccgcccaatccaccaggtaaatggtgttccatccggcgtgttgagcaggcgggacctcctgcagtggtaggccacctcctgctcacagtgctcagagccgtcgatcacggcctccagctgttccatgctgcccccgtagtccaaggccatggcatagggcttctcagggttagcgccccgcactcgggtcagctctgtattgttgtgctgcactgatgtccagatcttgtcctcagtgatattgcagtacacctggagaggtcccagtgggccgctgccatctgagtcgatgtagaagaagccggctgtattcccctggtgcctgtacacctcgcaggattgctcgtagatggagttgtggcaggtggcaccagtgtaacttgtgtcactgcagttacaatagaaggtagtccaggactgggagcagcttcctccatgttcacagtagtttggcaaacacctgtctttgatgctacacagatcaatgtgtaaatcactaaaattccccagggaaccttgctgaactgaaatgaggtccttgggctggttatcaataaagatgagcctcatgcagccttggaaagccttaatgggatttaaacattgggaatcggtgagattgtcggggcaccctccaaaatagtagctatttccagaataaatctgcacccaagtgctgtctggagccgggggtgctgcttcatcatccagagtgagcgtgatgcggttcctcctggcgttgatgctaaccgagtgccacaggccatcattcaagttgctgcctgtgaggatttcagctacgcgttctgtcattttctgaatcacgagtctcaggattccaccctccaggctcagcagcagggttcccgagccctcagacagctctgtggacagaagcagaccatccttgttccatgttcgaaactggaaactcactgagagcccatcaatttggggggtgccgggcagcagcaaatagctgccgctggagttgacaaatgtgatgggcacaatctgtggttcggagcaggaaaaagtgacattgccagtatagatctgatgctttcgtctcttagccaggtcaattatgtttactccattgtagtaaaggttttcgatgcatccatggaagtttttctttaaaaaggtcccaggttttcctggtactggaattcctccaaaactaagctcatagtcaatgtctaaggcatccgtctcgcccttggtgcggaagtgctgtgtgtgcttgtccaccgtgaagttcacctgcttgcccacccgctcaatgaggaccgagtgccagtgctggtcatccaggaggctgcccagggtggcagagggcaagctgctgctgagccgcgctttgctgtcacccaaattgaggtgtagggcgagcctccccttctggagttccaaggtgatgtggtctccacgctgaccttctccatggaacaggaccccatctccttgcatgctcttgaacttcagggagatcacatctttgagagtactcatcaacttctgattgaacctgtacagaagtgagcttcggccatcaaagtcagcaacatctgatttataggaacatccgtagacctcgactctcatgccaatcttcccactgggattccattccaggggcacaaagcgaacaaatcgggctctcactgagtgcaatagcttgtggtgcaccacgctgtcagcattcatgtttcctgcaaaggtccagatgctgtcttcttgtttgtactgtttccagttgcgtcctgtgtcactgaacatcaggctgtaactcgtcacccagtcagagcttccgtatcttccctgcgtggccactgctgtaatctctactctgtttcccaggtccatctggagccactgttgagcattggaatctgctggggaccaaccgccagttccaactctccagttgagttgagctgggctgtgagtgccagtgaggtctgaggaactggaaaaagccattggagagagcagggatgctagtggatcatcacagttgtagtttgtcgctgttaatcctaaatgccacaagccagagaacagcaaagtcaaaacgctggtcagccgtggtaaagaatccatttcccccgagtgagcggtccctcccaatcgaatcccaaattcgcagtagccagccgcggcttcttctcgctgtctctctcctctgcacagcctgaccccctcccacccccgcttggagaggcactcgctctttcactccatcccgtgcccagacgctccaccgaaaccgtggcgggggattcttcggagctgcagctggggctacggtccccgcaacagccgctagctggactcgccttcctcgcccgcctcttccttctcttcccccctccttaacggtgcaaatccaaacccaattagaacgacaggcgccggagctcggtggacagccaaatccacctcgtcgggcgcgagagctggaatc

SEQ ID NO: 10271 - RNA, 3493 nt, Homo sapiens
  source 1..3493: mol_type = other RNA
cagtgcaatgttttccttggatggagctgaatctgtgtaaatagctgaggatgagaggcttatattcttggtcacaggatagggttcttgaaacatgtaagtaaccgacgtgccagcctcaaaaacagcagaaacctcttttttgcaaaagggcccttcataaggtgaattggtgcaatcacacaggtagccattgtgcttctccacacacttgcccccgttgtggcagatgctgccgtagctgctgcagtggccggggcagcctggcctgactccagatgtgacctttgccctctcttccaggtccattttctgtccattcaagtgtaaggagcgaatgcatcctaggaagcctttctgtctggatgacgttccccctacaaacaactggctgttcagctgcagtcgaaaatggccctcctccgacgtctccctggtgctccttggaaggttgtccacctgcagggaggtctccttgaggttcctctcagcccggacatagtgccattggttgtcattcagaagagaaggagactggactacaagctccacaggaccattcccaacatcgatggcaaaggtgatctctgaaggagagcttatttcgagtcgaatgaagtctttaatgccaagattttctaggaaaactccggataatgctgtggttttaaaaaagaaggaaatatcggcactgaattccgcatggaaggtaggaaagtggaggtaagaggcttctgtataaaatgagacggcgttccagaagcgtcggtcaccatagcaacgcaagggaccaattctccaagcggcttctgagtttgatctgtcggtatcagtgataactatctgagtgacaggcaagtggtctttgaaggaaagaaagccagtatcatttgtccattcatccttgtcagcgtcgcaattgcaaaagtgctgaatgtccaggcagctctcgtctaggccacactcacactgctggaccccaggaggggaacctccccagtaagggtgcctttcattggaccgcccaatccaccaggtaaatggtgttccatccggcgtgttgagcaggcgggacctcctgcagtggtaggccacctcctgctcacagtgctcagagccgtcgatcacggcctccagctgttccatgctgcccccgtagtccaaggccatggcatagggcttctcagggttagcgccccgcactcgggtcagctctgtattgttgtgctgcactgatgtccagatcttgtcctcagtgatattgcagtacacctggagaggtcccagtgggccgctgccatctgagtcgatgtagaagaagccggctgtattcccctggtgcctgtacacctcgcaggattgctcgtagatggagttgtggcaggtggcaccagtgtaacttgtgtcactgcagttacaatagaaggtagtccaggactgggagcagcttcctccatgttcacagtagtttggcaaacacctgtctttgatgctacacagatcaatgtgtaaatcactaaaattccccagggaaccttgctgaactgaaatgaggtccttgggctggttatcaataaagatgagcctcatgcagccttggaaagccttaatgggatttaaacattgggaatcggtgagattgtcggggcaccctccaaaatagtagctatttccagaataaatctgcacccaagtgctgtctggagccgggggtgctgcttcatcatccagagtgagcgtgatgcggttcctcctggcgttgatgctaaccgagtgccacaggccatcattcaagttgctgcctgtgaggatttcagctacgcgttctgtcattttctgaatcacgagtctcaggattccaccctccaggctcagcagcagggttcccgagccctcagacagctctgtggacagaagcagaccatccttgttccatgttcgaaactggaaactcactgagagcccatcaatttggggggtgccgggcagcagcaaatagctgccgctggagttgacaaatgtgatgggcacaatctgtggttcggagcaggaaaaagtgacattgcccacagtatagatctgatgctttcgtctcttagccaggtcaattatgtttactccattgtagtaaaggttttcgatgcatccatggaagtttttctttaaaaaggtcccaggttttcctggtactggaattcctccaaaactaagctcatagtcaatgtctaaggcatccgtctcgcccttggtgcggaagtgctgtgtgtgcttgtccaccgtgaagttcacctgcttgcccacccgctcaatgaggaccgagtgccagtgctggtcatccaggaggctgcccagggtggcagagggcaagctgctgctgagccgcgctttgctgtcacccaaattgaggtgtagggcgagcctccccttctggagttccaaggtgatgtggtctccacgctgaccttctccatggaacaggaccccatctccttgcatgctcttgaacttcagggagatcacatctttgagagtactcatcaacttctgattgaacctgtacagaagtgagcttcggccatcaaagtcagcaacatctgatttataggaacatccgtagacctcgactctcatgccaatcttcccactgggattccattccaggggcacaaagcgaacaaatcgggctctcactgagtgcaatagcttgtggtgcaccacgctgtcagcattcatgtttcctgcaaaggtccagatgctgtcttcttgtttgtactgtttccagttgcgtcctgtgtcactgaacatcaggctgtaactcgtcacccagtcagagcttccgtatcttccctgcgtggccactgctgtaatctctactctgtttcccaggtccatctggagccactgttgagcattggaatctgctggggaccaaccgccagttccaactctccagttgagttgagctgggctgtgagtgccagtgaggtctgaggaactggaaaaagccattggagagagcagggatgctagtggatcatcacagttgtagtttgtcgctgttaatcctaaatgccacaagccagagaacagcaaagtcaaaacgctggtcagccgtggtaaagaatccatttcccccgagtgagcggtccctcccaatcgaatcccaaattcgcagtagccagccgcggcttcttctcgctgtctctctcctctgcacagcctgaccccctcccacccccgcttggagaggcactcgctctttcactccatcccgtgcccagacgctccaccgaaaccgtggcgggggattcttcggagctgcagctggggctacggtccccgcaacagccgctagctggactcgccttcctcgcccgcctcttccttctcttcccccctccttaacggtgcaaatccaaacccaattagaacgacaggcgccggagctcggtggacagccaaatccacctcgtcgggcgcgagagctggaatc

SEQ ID NO: 10272 - RNA, 24 nt, Homo sapiens
  source 1..24: mol_type = other RNA
cagtggccagagccctgcagtgct

SEQ ID NO: 10273 - RNA, 768 nt, Homo sapiens
  source 1..768: mol_type = other RNA
cagtggccagagccctgcagtgctaagccttctagcaggcgccgccccagccctctctgattggccgagggtttccggactcgcctccttcccctcctccgcttgagcctccagagcctgcgcccaccatctcttctaagatcaggagcttggtgacttcagagcagacctcgccctccccaggccccacctcccaggcctctcccactgctttagtcctgagggtccacattcccttcatccgaagtacactcactcttgctctttccgggctaccttgtagcaatttgaggctccgtcatcagtttctgctacgtttcaaagatccaggagaagcttagtgttgtgtcaagacgccgatggacccatcacagaagtttaatccaacctacatcccagagtctccacaaatgctcaccgaagaaaattcccgggacgattcaggggcctctcaaatctgctccgagacgttgataaagaaccttagtaacttgactatcaacactagtagcgaatctgtttcccctctatcggaagctttactccgtcgagagtctgtaggagcagaagtcctcagggaaatcgaagatgagtggctttacagcaggagaggagtaagaacattgctgtagatgaaagggaaatgggcctggtccgtgcgtccgagctccacttgacgccgcgccggctcccgtgcctgtcggcctcagcccccgccagccagctcccgagtcttgctagcagtagcttcagggccagaggctgctt

SEQ ID NO: 10274 - RNA, 2577 nt, Homo sapiens
  source 1..2577: mol_type = other RNA
cagtggccagagccctgcagtggccagcaccccaggaggaagggaggggacacggaaagctgttgtgagagatggacagacccacaagtcatcacctctcttgatgcccttggctgggtaggggtgggcctggaattttcactaacatgctccagaccactctctccatgctttgactgtattcttgaaccatgcatgtggtcccaagttttccatcctcttcatgccacttggtcctttactccccactacaccacaacctctgtgttccttgccctcaggatgaccttctcctcaccctggttatgccatcatccttccccttccatggccctgtatataagaactgattataatcacagtatattctgtgttttagcagagcatgtcaacattgctgtacgccatcatcgtgccagctcaacacaaactctaaagaaagtgacattggtgcagtaagagaaagatagacttccccttacctgaaaggaagtggtatcctggctttagggaggagttcatcaattctacagaggagatttcacatctttacacaggtacacaaactacacaaagagggacattcaggaggggaaacactgtggtcgctagaatccctatgtgacaccatggtctctctagagtgtctgtgtgacaccatgttctctctagagtgtctgtgtgacaccgtgttctctctagagtgtctgtgtgacactgtggtctctctggagtgcctgtgtgacgctgtggtctctctagagtgcctgtgtgacgctgtggtctctctagagtgcctgtgtgatgccgtggtctctctagagcgtgtgtgtgacactgtggtctctctagaatgcctgtgtgacactgcagtctctctagaatgtctgtgtgacactgtggtctctctagaatgcctgtgtgacgctgtggtctctctagaatgcctgtgtgacactgtggtctctctagcgtgtcttgtgatgctgtggtctctctagagtgtctgtgtgatgctgcggtcgctagctagaatgactatgtgatgctgtggtctctctagaatgcctatgtgaacttaggaattcacactcctaggctcagtgcaggctgagcaccaaagtgtgatctcatcaagtgaaataacccccttctctcaatttctcttcctgtaaggaggaaaatgccactttccacccacaaagctctctagaggaccaagaagacaattctgtgaaggacgtccaccaggagacaggagctacaagacagctttctggagctgtcctcctaagtccccatgccaatcagtgtatagtaatgtcgccaacttcaaaatcacggaaatatgtttgcatcagacaatggcttcaattccaacacatggtacattcccacaagtttggatttccataggaagaataaataacactggcttccttgaatgtcctggatgaaaaccacacatccttccaaatcctgtggaaaaacatctctggctccctccttcccttagaatcagacccttcaaaatcttgtggtatttccccaaataccataattttgagttgtgacatctggtttccagttctcccaggctggggtttcttgttaaagggacatcggaatctcgacatcccgagctgccaccctgaccttgtgcaggagtctcactgccccacttcctggcatccatgcactctagatggttctggcacttcccccagacaaggaagctacatttttttctaggatgtacctttttagaagcctttgtctcttccagaaggtatgtccggcacgatgggactcccccactctcccttgcctcaaacatcacggaacatctagacatcagtgagcgtcccactagaaaaaggcccctgaatcttcaagaagctccaagaggggagttagattgtctggaaattccccgaagttcttcctgctacacccactggagcccaggatttgagaaccaagcccgccggccgcggcatactaggctcggctttctgtttcgaagctcgaggctgtaccggggagagaggatgtggtccatgggaaggggaagtgccactgctccagggagccaagcatggcttcctcagggcctggctcctcaggcagcaggaggtgggcagcactgtgcagcgggtaagagcacacgctgtgatatcagataggcaggtgttggactcccagctctggccaagtgacctctggcaaacccctttcctcccaagcactggcatcctcacaggtataacaggatacagatggtgggcaaatgccgcggccacatcctacacggggagagacgcttcatcaacaacagccatgaacactgtctggcctgttcatcagggcccagcagacccatcacacagacacatggtaaaagcacgaggaatatttcatttcatggtcacaggtaagtgcttaagctggtagtgaaggaggaagcccaaaggctactgaggcggcatcacagtgacggtcaagaacaggccagaggctggctgcagtggctcaagcctgtaatcccagcactttgggaggcccaggcgggcagat

SEQ ID NO: 10275 - RNA, 541 nt, Homo sapiens
  source 1..541: mol_type = other RNA
cagtggccagagccctgcagtgtccaggatcaggctgcgcagcccagggagctcatgactctgtggccattcggaggtgacccaggaccagaagagttggttcctcttttttaagggctcgatcacagtcttctggatctggttcaccttttcctgattgaaggcatccatccgcttcatggccgtgtccagggccgtcaccatgttcagaaggtcctggtcttgctcacagaggggattggagagtaagtccaaggatatcttcacggcagattttgacatggccaggtctgcgtcggtgctcttcttcatgtctttctgcagcctccgggtctgctcttccagctgctgaagttttccatactccctttcaaagtctctctccactgttttgggcacaatctgtttcttgggctgcccaatcttaaaaggaatccagctcatggtcccgaacctgcgtctgccgccggggtcctcagccacaactcgtttctctagggtcacttccggattcaaccagtctccaggaagtgacgtaagc

SEQ ID NO: 10276 - RNA, 3093 nt, Homo sapiens
  source 1..3093: mol_type = other RNA
cagttctgctgttctgactctagaacaaaaagctacaaatagaggaaataaataagttgaattcaaatgctgctgagaaaaggcaatgtatattatagttctgtggtagtactgataacattcaagtcattcttaggcaccagtcttacgtatatgaagtcactttttcattccattgtacaaaactcatattttgagaaaaatctaatagctaatagtctccaacaccatatgatcataatcctttagcttaagtagagatctacttattaaatgaggcaccatcaacctaaggaaagataagctgtaagagaatgaagacagaggtatatcaagtaacaagaacattcttccttatcaggataaaatgtttatcagtattcaaataaaatatcttaaatggaaagagacaggaaagaacatggttaaatcacagaaaatgaagaaagggagaagctgatcatgatcttgtacaacattatgacagcactaaggtattacgtatccaatacaaggatacttaatagaccaaagaatttaaaatcccagggaactggaataaccagccacaaaagaggcctctctttgttgtggttcacaacacaaaaggccatcaacaaattaggaaatattaaaattaagagagcagcaggtttcttcttggtagacagctcatgctaccatccacaaagtgagcagtggaaggggtatttaatgtcaaggctttattttgaatttctgttccagatgcctctccacagcattcatcacaccttccttcacacttgaagggaaaagtccttaagagttcaccacattttggtgttatttttagcataaacatttgtttttctataagaagtatctctctggattcaaaccacagaaatgtcaatgaatgttatttccattgtataatcatttaaaagtcacctacagagctgggtgcagcagcttgtgcctgtaatctcagttactcaggaggctaaggcaggaggattgtgtgaggtcaggagttcaagaccagcctggacaacatggcaagaccctcatctctacaggaaaaaaaaaaggcacctacaaattgaaactgacttgatagtttaggatcatttatcaccagtcccatgtacttgtagttgatttcaaatgtttggtacaggtgactgtaagacttcaagtattccatgaaaataacattcatgctgggatcataaaattacatttctgggacagtatttttaaagtctgtttttaacttttgtcttcaagagctactttcttcttgctgttctgaccagtgacctttttccacatacttactgtttatccttagctttttctaagaaacattttggagttgtactaatgctctccctttccaatggtttcttaatcatctttttcttttgtttgcttagtagtttctgaaaaccttttatgtattctggtacaggacacccagcctgctgtataacattagcaacgcttcttaataatggcttatcatcctcagtgaaaaatgtaattgcttttcccttattccctgctcttccagttcgacctatcctgtggatatattccactgagctagttggaaagtcatagttgatcaccaagttcacacctttaaaatcaatccctcttgctagcaaggctgtacaaatcagaacccagatttttcctgctctgaaactgtggactgtgttatctctctgttgttgtgttctctctgcatgaataacatccacattaataccttcatatatgagctcatgaaaaagttctttagccctttcaatggactgaacaaaaacaagaacaggtggattgaaaccctttttaacaagttctctcacggccagaagttttccggtctcagatccaacaaagagaagctcttgttctacagtttctactgcagaattccttgctccaatggacacactgatgacattgtccaggttgagtttgcaccactgttcaacatcatatgcaaaagttgcactgaacatagctcttcggaccttgtgggatgtgcaggccaggaaaatggaagccagctggtctctgaacccagttttgccatcttcaaacagtttatctgattcgtctactacaagccactcaacacttgctaggtcgattccggggggatcttgctttaataaatagattagtcgatttggagtagtcacaagaatatcaaactttttagatgatttaggtccaaatttcttggctgccactgctgctttgtggatcatgtgtattctgaatcctgttccctcagaaatttttattaactctctgtgaatctggctggcaagttctcgtgttggtgatataatcagggctctgaagcctttatttgcgggttgtttcagctgcattaaaataggaatgctaaaagctaatgtttttccagatccagttggagcagaagccagaagttcccgaccatgcagcataactgggatggcttgcatttggattggcgtaggcatttggaaacctgcatctagaatgttctgaagtagtcgagaattgattttatattcctggtcaagttgctgaaatgtagcaattgggtcaggaagatcggttccttggacgtgaattttgtgtttattccgcaagaagtttatcttttcttttctgagattctccaactttccggaagttagtttactttctctctgaacttttttgtcttcaatctttgcttctacagatgacatccactgtatagtagcaccttcttcttgggaagcaatttctgaagtcatcgtcttcctttttttcttgctctgctccctcttcctttcagttaggctctcttcttttttctctccattttggggcttctgatgtgtttgtgatgctccacacacacctgggacagacttcttgtttccaaaaaagtccagtccctgaagcacctccgaagaatcaaagtcatatttcctttttcctatctggaatcgagctgcgtctgccgagaagcgtctcgtgtcgaatttggcccccgcgccgagccggcgaaagagatcgtggacgtccatctttacccagaaagcgccacagttctac

SEQ ID NO: 10277 - RNA, 3250 nt, Homo sapiens
  source 1..3250: mol_type = other RNA
cagttctgctgttctgactctagaacaaaaagctacaaatagaggaaataaataagttgaattcaaatgctgctgagaaaaggcaatgtatattatagttctgtggtagtactgataacattcaagtcattcttaggcaccagtcttacgtatatgaagtcactttttcattccattgtacaaaactcatattttgagaaaaatctaatagctaatagtctccaacaccatatgatcataatcctttagcttaagtagagatctacttattaaatgaggcaccatcaacctaaggaaagataagctgtaagagaatgaagacagaggtatatcaagtaacaagaacattcttccttatcaggataaaatgtttatcagtattcaaataaaatatcttaaatggaaagagacaggaaagaacatggttaaatcacagaaaatgaagaaagggagaagctgatcatgatcttgtacaacattatgacagcactaaggtattacgtatccaatacaaggatacttaatagaccaaagaatttaaaatcccagggaactggaataaccagccacaaaagaggcctctctttgttgtggttcacaacacaaaaggccatcaacaaattaggaaatattaaaattaagagagcagcaggtttcttcttggtagacagctcatgctaccatccacaaagtgagcagtggaaggggtatttaatgtcaaggctttattttgaatttctgttccagatgcctctccacagcattcatcacaccttccttcacacttgaagggaaaagtccttaagagttcaccacattttggtgttatttttagcataaacatttgtttttctataagaagtatctctctggattcaaaccacagaaatgtcaatgaatgttatttccattgtataatcatttaaaagtcacctacagagctgggtgcagcagcttgtgcctgtaatctcagttactcaggaggctaaggcaggaggattgtgtgaggtcaggagttcaagaccagcctggacaacatggcaagaccctcatctctacaggaaaaaaaaaaggcacctacaaattgaaactgacttgatagtttaggatcatttatcaccagtcccatgtacttgtagttgatttcaaatgtttggtacaggtgactgtaagacttcaagtattccatgaaaataacattcatgctgggatcataaaattacatttctgggacagtatttttaaagtctgtttttaacttttgtcttcaagagctactttcttcttgctgttctgaccagtgacctttttctgtttatccttagctttttctaagaaacattttggagttgtactaatgctctccctttccaatggtttcttaatcatctttttcttttgtttgcttagtagtttctgaaaaccttttatgtattctggtacaggacacccagcctgctgtataacattagcaacgcttcttaataatggcttatcatcctcagtgaaaaatgtaattgcttttcccttattccctgctcttccagttcgacctatcctgtggatatattccactgagctagttggaaagtcatagttgatcaccaagttcacacctttaaaatcaatccctcttgctagcaaggctgtacaaatcagaacccagatttttcctgctctgaaactgtggactgtgttatctctctgttgttgtgttctctctgcatgaataacatccacattaataccttcatatatgagctcatgaaaaagttctttagccctttcaatggactgaacaaaaacaagaacaggtggattgaaaccctttttaacaagttctctcacggccagaagttttccggtctcagatccaacaaagagaagctcttgttctacagtttctactgcagaattccttgctccaatggacacactgatgacattgtccaggttgagtttgcaccactgttcaacatcatatgcaaaagttgcactgaacatagctcttcggaccttgtgggatgtgcaggccaggaaaatggaagccagctggtctctgaacccagttttgccatcttcaaacagtttatctgattcgtctactacaagccactcaacacttgctaggtcgattccggggggatcttgctttaataaatagattagtcgatttggagtagtcacaagaatatcaaactttttagatgatttaggtccaaatttcttggctgccactgctgctttgtggatcatgtgtattctgaatcctgttccctcagaaatttttattaactctctgtgaatagaaagacttaaaagacttgcccacatggagtaagatccggagcactgtgctgtgtagaggatacttgaccatgacagaagacgtgggccttgctttttaagatctttttattaccttcaaataagaaagatcactgaagtaaaaaccaatcgcatactcttcaaaagctacaagtcatacctggctggcaagttctcgtgttggtgatataatcagggctctgaagcctttatttgcgggttgtttcagctgcattaaaataggaatgctaaaagctaatgtttttccagatccagttggagcagaagccagaagttcccgaccatgcagcataactgggatggcttgcatttggattggcgtaggcatttggaaacctgcatctagaatgttctgaagtagtcgagaattgattttatattcctggtcaagttgctgaaatgtagcaattgggtcaggaagatcggttccttggacgtgaattttgtgtttattccgcaagaagtttatcttttcttttctgagattctccaactttccggaagttagtttactttctctctgaacttttttgtcttcaatctttgcttctacagatgacatccactgtatagtagcaccttcttcttgggaagcaatttctgaagtcatcgtcttcctttttttcttgctctgctccctcttcctttcagttaggctctcttcttttttctctccattttggggcttctgatgtgtttgtgatgctccacacacacctgggacagacttcttgtttccaaaaaagtccagtccctgaagcacctccgaagaatcaaagtcatatttcctttttcctatctggaatcgagctgcgtctgccgagaagcgtctcgtgtcgaatttggcccccgcgccgagccggcgaaagagatcgtggacgtccatctttacccagaaagc

SEQ ID NO: 10278 - RNA, 3080 nt, Homo sapiens
  source 1..3080: mol_type = other RNA
cagttctgctgttctgactctagaacaaaaagctacaaatagaggaaataaataagttgaattcaaatgctgctgagaaaaggcaatgtatattatagttctgtggtagtactgataacattcaagtcattcttaggcaccagtcttacgtatatgaagtcactttttcattccattgtacaaaactcatattttgagaaaaatctaatagctaatagtctccaacaccatatgatcataatcctttagcttaagtagagatctacttattaaatgaggcaccatcaacctaaggaaagataagctgtaagagaatgaagacagaggtatatcaagtaacaagaacattcttccttatcaggataaaatgtttatcagtattcaaataaaatatcttaaatggaaagagacaggaaagaacatggttaaatcacagaaaatgaagaaagggagaagctgatcatgatcttgtacaacattatgacagcactaaggtattacgtatccaatacaaggatacttaatagaccaaagaatttaaaatcccagggaactggaataaccagccacaaaagaggcctctctttgttgtggttcacaacacaaaaggccatcaacaaattaggaaatattaaaattaagagagcagcaggtttcttcttggtagacagctcatgctaccatccacaaagtgagcagtggaaggggtatttaatgtcaaggctttattttgaatttctgttccagatgcctctccacagcattcatcacaccttccttcacacttgaagggaaaagtccttaagagttcaccacattttggtgttatttttagcataaacatttgtttttctataagaagtatctctctggattcaaaccacagaaatgtcaatgaatgttatttccattgtataatcatttaaaagtcacctacagagctgggtgcagcagcttgtgcctgtaatctcagttactcaggaggctaaggcaggaggattgtgtgaggtcaggagttcaagaccagcctggacaacatggcaagaccctcatctctacaggaaaaaaaaaaggcacctacaaattgaaactgacttgatagtttaggatcatttatcaccagtcccatgtacttgtagttgatttcaaatgtttggtacaggtgactgtaagacttcaagtattccatgaaaataacattcatgctgggatcataaaattacatttctgggacagtatttttaaagtctgtttttaacttttgtcttcaagagctactttcttcttgctgttctgaccagtgacctttttctgtttatccttagctttttctaagaaacattttggagttgtactaatgctctccctttccaatggtttcttaatcatctttttcttttgtttgcttagtagtttctgaaaaccttttatgtattctggtacaggacacccagcctgctgtataacattagcaacgcttcttaataatggcttatcatcctcagtgaaaaatgtaattgcttttcccttattccctgctcttccagttcgacctatcctgtggatatattccactgagctagttggaaagtcatagttgatcaccaagttcacacctttaaaatcaatccctcttgctagcaaggctgtacaaatcagaacccagatttttcctgctctgaaactgtggactgtgttatctctctgttgttgtgttctctctgcatgaataacatccacattaataccttcatatatgagctcatgaaaaagttctttagccctttcaatggactgaacaaaaacaagaacaggtggattgaaaccctttttaacaagttctctcacggccagaagttttccggtctcagatccaacaaagagaagctcttgttctacagtttctactgcagaattccttgctccaatggacacactgatgacattgtccaggttgagtttgcaccactgttcaacatcatatgcaaaagttgcactgaacatagctcttcggaccttgtgggatgtgcaggccaggaaaatggaagccagctggtctctgaacccagttttgccatcttcaaacagtttatctgattcgtctactacaagccactcaacacttgctaggtcgattccggggggatcttgctttaataaatagattagtcgatttggagtagtcacaagaatatcaaactttttagatgatttaggtccaaatttcttggctgccactgctgctttgtggatcatgtgtattctgaatcctgttccctcagaaatttttattaactctctgtgaatctggctggcaagttctcgtgttggtgatataatcagggctctgaagcctttatttgcgggttgtttcagctgcattaaaataggaatgctaaaagctaatgtttttccagatccagttggagcagaagccagaagttcccgaccatgcagcataactgggatggcttgcatttggattggcgtaggcatttggaaacctgcatctagaatgttctgaagtagtcgagaattgattttatattcctggtcaagttgctgaaatgtagcaattgggtcaggaagatcggttccttggacgtgaattttgtgtttattccgcaagaagtttatcttttcttttctgagattctccaactttccggaagttagtttactttctctctgaacttttttgtcttcaatctttgcttctacagatgacatccactgtatagtagcaccttcttcttgggaagcaatttctgaagtcatcgtcttcctttttttcttgctctgctccctcttcctttcagttaggctctcttcttttttctctccattttggggcttctgatgtgtttgtgatgctccacacacacctgggacagacttcttgtttccaaaaaagtccagtccctgaagcacctccgaagaatcaaagtcatatttcctttttcctatctggaatcgagctgcgtctgccgagaagcgtctcgtgtcgaatttggcccccgcgccgagccggcgaaagagatcgtggacgtccatctttacccagaaagcgccacagttct

SEQ ID NO: 10279 - RNA, 3195 nt, Homo sapiens
  source 1..3195: mol_type = other RNA
cagttctgctgttctgactctagaacaaaaagctacaaatagaggaaataaataagttgaattcaaatgctgctgagaaaaggcaatgtatattatagttctgtggtagtactgataacattcaagtcattcttaggcaccagtcttacgtatatgaagtcactttttcattccattgtacaaaactcatattttgagaaaaatctaatagctaatagtctccaacaccatatgatcataatcctttagcttaagtagagatctacttattaaatgaggcaccatcaacctaaggaaagataagctgtaagagaatgaagacagaggtatatcaagtaacaagaacattcttccttatcaggataaaatgtttatcagtattcaaataaaatatcttaaatggaaagagacaggaaagaacatggttaaatcacagaaaatgaagaaagggagaagctgatcatgatcttgtacaacattatgacagcactaaggtattacgtatccaatacaaggatacttaatagaccaaagaatttaaaatcccagggaactggaataaccagccacaaaagaggcctctctttgttgtggttcacaacacaaaaggccatcaacaaattaggaaatattaaaattaagagagcagcaggtttcttcttggtagacagctcatgctaccatccacaaagtgagcagtggaaggggtatttaatgtcaaggctttattttgaatttctgttccagatgcctctccacagcattcatcacaccttccttcacacttgaagggaaaagtccttaagagttcaccacattttggtgttatttttagcataaacatttgtttttctataagaagtatctctctggattcaaaccacagaaatgtcaatgaatgttatttccattgtataatcatttaaaagtcacctacagagctgggtgcagcagcttgtgcctgtaatctcagttactcaggaggctaaggcaggaggattgtgtgaggtcaggagttcaagaccagcctggacaacatggcaagaccctcatctctacaggaaaaaaaaaaggcacctacaaattgaaactgacttgatagtttaggatcatttatcaccagtcccatgtacttgtagttgatttcaaatgtttggtacaggtgactgtaagacttcaagtattccatgaaaataacattcatgctgggatcataaaattacatttctgggacagtatttttaaagtctgtttttaacttttgtcttcaagagctactttcttcttgctgttctgaccagtgacctttttctgtttatccttagctttttctaagaaacattttggagttgtactaatgctctccctttccaatggtttcttaatcatctttttcttttgtttgcttagtagtttctgaaaaccttttatgtattctggtacaggacacccagcctgctgtataacattagcaacgcttcttaataatggcttatcatcctcagtgaaaaatgtaattgcttttcccttattccctgctcttccagttcgacctatcctgtggatatattccactgagctagttggaaagtcatagttgatcaccaagttcacacctttaaaatcaatccctcttgctagcaaggctgtacaaatcagaacccagatttttcctgctctgaaactgtggactgtgttatctctctgttgttgtgttctctctgcatgaataacatccacattaataccttcatatatgagctcatgaaaaagttctttagccctttcaatggactgaacaaaaacaagaacaggtggattgaaaccctttttaacaagttctctcacggccagaagttttccggtctcagatccaacaaagagaagctcttgttctacagtttctactgcagaattccttgctccaatggacacactgatgacattgtccaggttgagtttgcaccactgttcaacatcatatgcaaaagttgcactgaacatagctcttcggaccttgtgggatgtgcaggccaggaaaatggaagccagctggtctctgaacccagttttgccatcttcaaacagtttatctgattcgtctactacaagccactcaacacttgctaggtcgattccggggggatcttgctttaataaatagattagtcgatttggagtagtcacaagaatatcaaactttttagatgatttaggtccaaatttcttggctgccactgctgctttgtggatcatgtgtattctgaatcctgttccctcagaaatttttattaactctctgtgaatctggctggcaagttctcgtgttggtgatataatcagggctctgaagcctttatttgcgggttgtttcagctgcattaaaataggaatgctaaaagctaatgtttttccagatccagttggagcagaagccagaagttcccgaccatgcagcataactgggatggcttgcatttggattggcgtaggcatttggaaacctgcatctagaatgttctgaagtagtcgagaattgattttatattcctggtcaagttgctgaaatgtagcaattgggtcaggaagatcggttccttggacgtgaattttgtgtttattccgcaagaagtttatcttttcttttctgagattctccaactttccggaagttagtttactttctctctgaacttttttgtcttcaatctttgcttctacagatgacatccactgtatagtagcaccttcttcttgggaagcaatttctggctgggcgtggtggctcacatctgtaatcccagcactttgggagcccaaggtgggtgaatcacgaggtcaggagatcgagaccatactggctaacatggtgaaaccctgtctctgaagtcatcgtcttcctttttttcttgctctgctccctcttcctttcagttaggctctcttcttttttctctccattttggggcttctgatgtgtttgtgatgctccacacacacctgggacagacttcttgtttccaaaaaagtccagtccctgaagcacctccgaagaatcaaagtcatatttcctttttcctatctggaatcgagctgcgtctgccgagaagcgtctcgtgtcgaatttggcccccgcgccgagccggcgaaagagatcgtggacgtccatctttacccagaaagcgccacagttct

SEQ ID NO: 10280 - RNA, 28 nt, Homo sapiens
  source 1..28: mol_type = other RNA
catacaatctgacatgtatttaagtgat

SEQ ID NO: 10281 - RNA, 4348 nt, Homo sapiens
  source 1..4348: mol_type = other RNA
catacaatctgacatgtatttttccattaaaggtaggcacaactctatgaatatcaaattatatcaatcatttgctttttataatcttgactggaaactgaaaaataagaggaatgtaaagttaagtagccgaaaatgctacttactgcacaaaagcacatcatgaaaaggaatgctagaagtagttctcctcaggaatgggtttttgaaaatttaaaatattattttatcagaaaagttaaagccttcagtgggaaaaccatggtaaatgacatattgactcaatctctaaagccctggcaaattatagattttgtgcaattagtgaccaacatatacatttaagagataatactgactgttgaccagaaccttctgatggttctgaagcatctgctctttagagttacttcagctttacatgtctatgaaatttaagattcctcaatgggatgttatagcttattctgcactagatacaagtaatatgtatagatttagaacaaatgactacttttcaccttccaggagcctgtttttatttatacaaaattagattggtttttcacccacatgtatgcataagtgcttctcaaatttacaccgttcatatctgaaatcccacaataaatgcaaataaatggatactagtttatatatttcatattttcattcatcttttttttttttttttttgagacagagtctccgttgcccaggctggagtgcagtgtcgtgatcttggctcaactgcaacctccacctctcaggtttaagtgattctcatgcctcagcctcctaagtagctgggactacaggcacgcaccaccacgctcggctaatttttgtatttttagtagagacaggttttcaccatgttggccaggctggtttcaaactcctggcctcaagtgatccacctgcctcggcctcccaaagtgctgggattacaggcatgagccaccatgcctggcctttcatccatctttaaacaaattcaatgaccatctagagacagatgtgaccaaagtgttacaaatttctatgcattttctatgaattgctctgtgcagttcacacatgggttcattcaccccgcaggctgtgaacttccttatcctgtaggctgcaggtacttaggtttcagcaactacgcgacccaaaagactaaaggaggacttgtttaaattagtccctctcaaaaattgtttccaatcttataacaaacagatttaatatgcttgtgggttaaattttaaagtagttatgaagccatttactctaatataaatgaatgaaatgtaattaagaaccatacttaaacgagtacttaattttaatgaatggtatttttcatttatatacaaaggaatagccagcagcatttaaatatagaaatagtcccatctcttctctattcccttttataaagtgccattttaattgggtagatttactacccagattttcagtaactacaggataggtatctaattgtcaagaaaagcttggaaaattaagtttagcattttaaacatttgtaaaacattgctacaagtcatagagactaccaatgtattaaaataaaaagtgtaccttacataagaatcattaagttggtttaataattacttcacagaaacatgggctcatgaatacttaggccaatttgtgctaattatttaaaccagaaacagtttctgtaggtaattcagctctaagcaccattaaatagggttatgccaaatagaacaatggttaaataatcctcagaataaacaccccagcaaattcaaacttttagaatagtaacaaaagttagtgagaatccgaaagagaggcaacattttattgaaaactatcataggctgctaagtgttctctttaaataaaattttgtgtagttattaatgtaccttaacactggtgtaccttaatagtggtgttagagataggtggaaaccatactacagaagtgaatgttgcctgtttcttttgttcagtgattaaaactgaaattgcttttaaaaaaataatttaactgctacttacaatacacataaaataccaagaagattcccattttattcacattattctctaattagtatttttgcatttcaactttgatctgaccttcagtagtaccttaaaatgcaaatgcaattagtaaaaacggggcagcctgtcgttttcacacttagaaatacaatgtagtttcattacagtttgcatttttttgttactcttgaaagagtaaccccttataaaatcagatacataaaaactgcattattccttactttgcaggcatccaggaatggttaaagcaaaggaactctcattcattaattcattcattctgttcccccaatttagatacatttctagtctccagaaacggactccagggcagggaagtggagggcagagaagaggtacaggtcaaggtatgatgaatctctgaaaaagacatccacttttcccagaaggctagcctgaagagaactccgccccatccattccgatccctcaagtaagaatgcataatttagcttgtccttctggtctcacttccttacaacacctagtattcaatttattaagacaaataaacctttgcattttctaaaagaagcaatttttacccaaatacattggactttggtctcaatgtgaagggcgagtggcctttaacaggtcgttcctcccccactccctcctcccccctgccctccagcggctgctctgggtccctgaaagagggtgtggtgtggacgatctgggttctgaatcggattttgttgagtctgggttttatacgtccactagagctgcccgaggctttgcgccctggatccttggctttgcctccgacccacccctcagccgagtggtgatggtggtgatggtcccctccatcttctagggcgtgtgagagtttgtaggtgatgagatgcgagggaagcacctttgaaagcctccagcgcccgccgccgctacccgcggcgctttccccgtcaccctcgtccagggctcccaccaggttcttgatctcctcggcgatgctccgactcaggtactgggaggcctttttcccactgtagtccctgatgtccacatcggcgtcgtaggcccccaccagcagcttcaccacctccacgtggccgtgcatggctgccaagtgcagggcggtgtaacccccgctcgtcctggcgtcgatgttcaccggcagctggtgtttgttggcgaagttgactagcatggccagaagctcctgcctgccgtgcttggcggcccagtgcaggcaagtgaagccggtaatgaagtcccgcttgaccagcaggccgggctcgcaggtgagcaagccctccaggctgtcccacttgccatcggaggcagagagcatccacgcgtgctccagggggtccagcgtcacggagcctccgccgctgctctcctcctccgcggacgacgaggccaccgatgcgctgtctgagtcgcccccgcctctgccgcgtcctcccccggaggagctgcccgggctgctgcccccgggacacacgctcctcttcagctgcggggagctgcccatcaccaggtcacggaggttctggcgggccggcctctgtgcggtagcccccacaagggagctgcccctgtccgcctcctcgcagccatgtggcgggagctccaggtcctcgctgggccccggggctggagtccgcggtaggggctgcacgtcgcgccgcgagttcttcctgcgagccccggcgctcaggggcggccagtgcgcgggggcggggggctctccctcgcccagctcgcggccctgtccagggagcgactccggggccgccgcgtcggggagccgatcgcgcgcctcgggcccggcagggccgtcgggggcctcgggctcggcggtcacctggattcgcggcgggtccccggagggctcggacggcccttcacagaacctcttcttgaggtgcacgtacttggcgccgtcggcgggatcgacgcgcacagtggccacggcgttcaccagctccttgaagtgcgcgcgggcgcgggcgcgctgctccggttcgccgcctagggcgcccctgaagtgctgcaccagctcggcgtgcagggcccggcccccgcgctccgccaggaagcgcagcaccgcctcggggcccagcgccgcctcggggccccactctgccggcccctccatcctcgaccgcgctgctcccccgccagcgggcggctcagcgcggtcccatagcgacgggctcccagcggccggctcccgacggcggcggagtctggcgggctcagcgggctgccagcctacgcgtct

SEQ ID NO: 10282 - RNA, 401 nt, Homo sapiens
  source 1..401: mol_type = other RNA
catcatcgtctcaaatgagtcttcagagggttctatcatttcgtcggatggaaaggagtgtattctgaagattggtaaggttgtgatggcgtccagtcagtagctgggaccgtggagatcagaaccttggctgcaagcgttcaagtggatctcctcccgtcctgtgccactcgatcctcgctgcttgcttccccgggcccagtcccaagcgtgaggctggggatgaagtgatgccggtggcttagtgatgccggtggcttcctgtcctcgaagctcagtcggtcgtctctcagctggtgtgaggctgggccaggatggaaccccagactctccgaggctccccaccacaccctgctgctgaaggctgctcagcgaggctgtgccgagtgctgggggggtgt

SEQ ID NO: 10283 - RNA, 831 nt, Homo sapiens
  source 1..831: mol_type = other RNA
catcccttgcatggtggagggtatctctgagccattcttagtcaggtaggttccaaacaagaacatcttcctgtcatttcccacttcagataatgccaaagcttcatggatatctgtaatgtgataggctgcttcaagatcctgtttgtttgcaaacacaaccagaggaagtactgggtttgctgcaattagctgatgaaggtatttcttggcttcaggtaatcggctgtgatctgctgaatccaccacaaagatcagcagcaatcccttggataggtacatttcccagtaggaccgaaaaggtttactgccaccaatctccaggaactccatctggctgtcttcagtgttgatgcaaactgcatggaaaccttgggtgggtgccacactgtgctggactctgtttgaagctagagagtgcaggacactggtttttcctgctccatccaggcccagcactaggatttgcttgtttttctccagcggctcgagcggggtccttgtcaaggtgctgtccttgttctcccctttctcttcttgtcccttaaattgttccttctctttgtttgtctccttcccttgctttgtcctcttttcctctttctcttttccctttctcctctcctgcttctcttgcttttgtttaattttctgctccacctcctttcttttcactttctcttccctacccttttctccgattttctcctcctgcgtctccttttccttctctttcttcttcactttccccctctccatccccagcgccgcggtttccttccctcccgccgcgtgcccgcgtgctgagcggtggctctgggccccaggtgt

SEQ ID NO: 10284 - RNA, 655 nt, Homo sapiens
  source 1..655: mol_type = other RNA
catcccttgcatggtggagggtatctctgagccattcttagtcaggtaggttccaaacaagaacatcttcctgtcatttcccacttcagataatgccaaagcttcatggatatctgtaatgtgataggctgcttcaagatcctgtttgtttgcaaacacaaccagaggaagtactgggtttgctgcaattagctgatgaaggtatttcttggcttcaggtaatcggctgtgatctgctgaatccaccacaaagatcagcagcaatcccttggataggtacatttcccagtaggaccgaaaaggtttactgccaccaatctccaggaactccatctggctgtcttcagtgttgatgcaaactgcatggaaaccttgggtgggtgccacactgtgctggactctgtttgaagctagagagtgcaggacactggtttttcctgctccatccaggcccagcactaggatttgcttgtttttctcctcgcggatgcagggcttcttgcagccgattcgctgaacccgcaggggttcgcaaagagggaagggcggaggcgtacggatggattgagcccagccaagcgaaaccaagaggtcccaaccaggacgtgggacagttcggcggggtatatcattgctgcagaaaaagcgtccctag

SEQ ID NO: 10285 - RNA, 781 nt, Homo sapiens
  source 1..781: mol_type = other RNA
catcccttgcatggtggagggtatctctgagccattcttagtcaggtaggttccaaacaagaacatcttcctgtcatttcccacttcagataatgccaaagcttcatggatatctgtaatgtgataggctgcttcaagatcctgtttgtttgcaaacacaaccagaggaagtactgggtttgctgcaattagctgatgaaggtatttcttggcttcaggtaatcggctgtgatctgctgaatccaccacaaagatcagcagcaatcccttggataggtacatttcccagtaggaccgaaaaggtttactgccaccaatctccaggaactccatctggctgtcttcagtgttgatgcaaactgcatggaaaccttgggtgggtgccacactgtgctggactctgtttgaagctagagagtgcaggacactggtttttcctgctccatccaggcccagcactaggatttgcttgtttttctcctcgggccaggcagggtggctaagagccttccacgtgggccgcagtctaagcaaccttagcgtctgacgtctccggcttcaatcccgagaccggccagcctgtgtgaagaacccctggggcgtcagaatccagaggttccgggaggattctcagccttccctcagctcccaaccatgagcctgtactgctcatgtcatgtatttctccgccctctcccgagtaaactccgctaggagtgtctccagactactacccaggattattagttgactattacccaggattattaaagacaaatag

SEQ ID NO: 10286 - RNA, 963 nt, Homo sapiens
  source 1..963: mol_type = other RNA
catcccttgcatggtggagggtatctctgagccattcttagtcaggtaggttccaaacaagaacatcttcctgtcatttcccacttcagataatgccaaagcttcatggatatctgtaatgtgataggctgcttcaagatcctgtttgtttgcaaacacaaccagaggaagtactgggtttgctgcaattagctgatgaaggtatttcttggcttcaggtaatcggctgtgatctgctgaatccaccacaaagatcagcagcaatcccttggataggtacatttcccagtaggaccgaaaaggtttactgccaccaatctccaggaactccatctggctgtcttcagtgttgatgcaaactgcatggaaaccttgggtgggtgccacactgtgctggactctgtttgaagctagagagtgcaggacactggtttttcctgctccatccaggcccagcactaggatttgcttgtttttctcctgtcagttaaaacttttccgccatccattcatggtactggtggtctgaaaacaactgcagcgtccccaaacacctcctgcgttcaggaaccctgccccttctgacaaagaacgcattcaatgcaaagagggcctgcgtgtggggagggttcggggctggtttctaaatgtggtcaggtggtctgtgcgctagtgttgcgcgctggacagatctaagggcagtagaggggccgttccccatgtccccatgaagaccgagatctcttgtccctcaacaacagacccgactgaggttaagacacaggggtagcgataagggctagggtgggcagggggcccgggaaaaggggatgggtcgttcaaagtttggcgcatctctttcatccataggtaaatagccctcagttgagatccattcgctcccacgcggtcgggggcctccgacgtaacagagacagcgctggggtctgaacggccgacaaa

SEQ ID NO: 10287 - RNA, 285 nt, Homo sapiens
  source 1..285: mol_type = other RNA
catcccttgcatggtggagggtgacgctggtccctgaagggagatggaggaggaggcagagcttttcaagcaattccaggaagctggactcataggaggaatttgtcagaaaagactccttcagcttcagttgcaaagtcatacccggccctgttccatgtgagctgccaaggagggtcaagaggaggacaaggggcagcccagaccccatagtggccactgcgctcctgggatggaggagacactgaagtcccggtggcctctccttaacaggcctgtttctac

SEQ ID NO: 10288 - RNA, 1660 nt, Homo sapiens
  source 1..1660: mol_type = other RNA
catccgtccgtctgtccacatgggcctcagaccccgggggatcctggccgtcactgcccggccatgtgcagcctcggcctgtgtcagacagacttgggctcgaggtccccaggagctccggtcgccgtggtggagcctctcgatgtctcgggctgtctgcggctggagcaccctctgagctggggttgggtcaggtctgaagaaggggccggagctggccctgccaagggcccctcctagcagccgtggcctcctcaggtggggcccagggctccgaggccctgactcctccaggtctgggcagctgctcaggaccggggaaggctctgccaggtgtgatgccccaggctgggagagggtgtggcgggggggctgcctggctcagggcaggttgagcccttcctcctgccctcctgccactgccccagctgtggcaggctcaggacatctggtgtctgctggtgggggggtcgctgtgcctggggacagtccttcccccctgctgcactgggagttcctctggcatcctgggaggcctgtgcctcgagagagaccagccccctagattcctcccaccacgggcggctccccggcacccaaccggctcctgagcccctgccccacctccacattcccgatggctgctctcccagcctcttttccttccttccacccctgtatggtttcgatctgtgtcccctcccaaatcttatgtcgaattgtaattcccagtgttggaggtggggcctggtgggaggtgactggatcatggggtggactctcaggaagggtttactgctatcgcctcggtgctgtcctcatgacagcgagttcccccgagacctggctgtttaaaggtgtgcggcacctccccaccttgctgctgctttcgccatgtgacgtgcctgctcccccttctcttccaccaggattgtgggtttcctggggcctccccggaagccgagcagatgccagcaccacgcttcctgtagagcctgcagaaccgggagccgattaaacttcttttccttaagaatcacccagcctccggtgttccttcacagtagggtgaggggggcgaacgcacaccctgagccttaggggcaactcctgctgctgtgcccaggctgggccgggcagtggctcaggaacgtggcggggaacacggtgccagtgctggggtcagggctctgtcgtggaggcaggatgtctctgtggttccttcctaaccctcatccttttacctcttgtcctggcttactgggctggcaaggacctccaggaagatgttaaacagccttgatgtctgataggccaaacaagggcccggaagccgtctgcatcctcattccggggcctgcaccatgacgtcatggcgaagggctgcgccgagggggccggctgagggtcttgaggtgagaaatcatcctggtcatctgggtgggtccagggtctcaccagggtccatccgcatggccctctgctgtgcactctccttctcgttcgtgtctgtgctgcattctggttggttttccttggcttttttttttttctagttcacgaattctctctttgctgtgtttaatcagctgggagttactctcttgctccctctctccctcccccatcctttctctgtccttgtctctctgtctctgtg

SEQ ID NO: 10289 - RNA, 3244 nt, Homo sapiens
  source 1..3244: mol_type = other RNA
catcttccagtacagtgttggacatagaattatgctttttttttccagtaagaagaaagtcttttaaaataaagaatgaaaattatggggaaaaaacaaaaatgtggaaaggataaatctttacattataagctagaaaactatacaatatgagccaaacgagaaaacaaaacaaaacaaaaggtgaccatcattattttttgtacctcagcttatcttgctcttgaactcttattgattgcaagatacctgtaaatgctcaatcttgtcagtcggaggcagttgggtaattagtcttcctgaatgtctcctctcctcaagaacatcctgcttcttcctactccccagcagcaggtggacactgggaaaggttagggtcctggtgctctgagagagtggctggctccctgctggacccactgtgaaggtaggtgtctgtggctagggggactcatggcctgcaaggctgtgtttcttccccaccaattccactgtcctgctggggctgcctttctttggagagcccaaggctgccatcacacccatcgcatgcccagctccaaggaatagcttgcccaagaccctgggaacctgagaatcacatctcacacccaccgccaagaatcttctctttgcttttgcgtgtcatactgatgcaaggcaggtgaacccaaaatcgaggcttcacctgggagggttgttgcctttgcccaggaaagaatttaagggtgagccagtggtgctagacagcaacttctattgaagcagcagcagaggtgttgtgccttgtggagcagggctaccccagaggcagtgtgcccagagcagcagctcagaagcagttttgtactcacacttatatttactttgaaaattaagggacagattatgcaaaaatttcttgaaaaagagtggtaatttctaggtggttgagtcattgccatggacaaaggtggtaccgctcgagtgttgccctggcaatggtaaaccgacatggcactctgttgggcatatcttatagaaagttgtttttgccccatccgcattttagctagtcctcaatttggtccagtgtccaagctctgccttctaactcaatatgagaagcagcagccccccagatttttctgagaggtgagtaatctttccaggccatgtctgaagatgcatggacaaaccttctgctccaggactcacatgaacccttctggaagcctctgtttatctgcctcctgcccagcaatgaattggggaggtcaaggatgcttacatctatattcttgcctccactctcttcctccacctgggtcactcaaatagaaatattcttcactgcatctcctgtctccacagtcaacagttcagccttggattatttgtttgtgcattagttgtgatcaggttgggctgcaattgagaagaaaacaaacgatgtttttcacttacatacaggctagcctgtccattgtctattgctgcatagcaaatcaccacacatgcagcagctttaaaagacacaaagttattagctcacagcatccatggaccagaagtcctggtacagtgtggcgcagttgcgttctgtgctcagggactctcaaagctaaaatccactttggctttcaaagtgttggctgggctgggctgtctgcagactctggggaagaatccacttacaagtgcatctaggttgttagcagaattcagttcattgcagttgtgaaactgagatccctatctccttgacatgcagatgccctcatcttcaagccaataattgcatggcgaatccttctcatgcttcaaatctctgccttccccttctgcgacgggctggaaaaagatcttccctttcaagggctcatacaatttaaactaggtccacctggtgaatccaggacaatcttccgattttaaggtcaactaattggtaccttaattacattttgccatgtaatgtaacatatccatgaataatgccaagggcaaaagtcatgaggcccaagctctgccttccacagctggtaaggcaactctgccttaagtcctcaggacccaggctcccttctactcaccactccatcacccctggaagggacctctgtcctcgcagcccaggattcaacaactgtatgccaaggcagatgggtatagggttgtatagggttcattctgactaggttttaaggaaggttctcagcagctgccgcacaacgtttctgccttcatcccattggttctacattgtgacatccttgcctggttgtaagggaagctgggcaaggtagctccattctgggtgtcaatgtggctgggtacaaattctgggcaggagctctcctggctaatggcaccctaactggaggactcctggggcacgtgaagacttcgtaaagaagactggtacttcaagcagtttatattttcctgattcctgctaaatgcttctgcaacttgaatcctcctcgtctccaaggcagtgttcatctctgaagtctgcggtggcacagctacaaaccttggcaatcttccaacacagttgtcttttattcttttggatgagttccaactctgttcccacggcagtgctccatccacgggagccgcagcatcggcaggggctgcttttgcacagcaaagcccccttggggagtactgcacactgtccccaagagagcccctgggccaagaggaaggcgccgcctggggttgtggtggttcaacaacgccgttacgcccgggactcagggtcaggccagggggcctggacaagagaggaagcagtgaccctgttcacccacgggagggagaaggcagccttgggccacttcaggaaccaagccaggaggatggggaagttccggtgaggctgttcactcatcagaagaaagaatgttctagaaatcagaacgttctcactgagggaagactcttctagagacatcagttctgtgagagcaggggctgtcgtgtgggcctcaactctatcctccgcggttagaactgtgagcagcgtactgtgaatactccgttgatagctgccaaatgagtgcgtgggtggatggtggaacccagacgatgagctggtgtcgaaggacccctgtgggacccgtatgtatgctaaggcaggggtggctgaagcagtgccctctaaggagcatctccagttcaggacgccaggacccctcaccggcccagggaagctgggaaaaactccccaggagcggccccttcccgctttgtt

SEQ ID NO: 10290 - RNA, 3247 nt, Homo sapiens
  source 1..3247: mol_type = other RNA
catcttccagtacagtgttggacatagaattatgctttttttttccagtaagaagaaagtcttttaaaataaagaatgaaaattatggggaaaaaacaaaaatgtggaaaggataaatctttacattataagctagaaaactatacaatatgagccaaacgagaaaacaaaacaaaacaaaaggtgaccatcattattttttgtacctcagcttatcttgctcttgaactcttattgattgcaagatacctgtaaatgctcaatcttgtcagtcggaggcagttgggtaattagtcttcctgaatgtctcctctcctcaagaacatcctgcttcttcctactccccagcagcaggtggacactgggaaaggttagggtcctggtgctctgagagagtggctggctccctgctggacccactgtgaaggtaggtgtctgtggctagggggactcatggcctgcaaggctgtgtttcttccccaccaattccactgtcctgctggggctgcctttctttggagagcccaaggctgccatcacacccatcgcatgcccagctccaaggaatagcttgcccaagaccctgggaacctgagaatcacatctcacacccaccgccaagaatcttctctttgcttttgcgtgtcatactgatgcaaggcaggtgaacccaaaatcgaggcttcacctgggagggttgttgcctttgcccaggaaagaatttaagggtgagccagtggtgctagacagcaacttctattgaagcagcagcagaggtgttgtgccttgtggagcagggctaccccagaggcagtgtgcccagagcagcagctcagaagcagttttgtactcacacttatatttactttgaaaattaagggacagattatgcaaaaatttcttgaaaaagagtggtaatttctaggtggttgagtcattgccatggacaaaggtggtaccgctcgagtgttgccctggcaatggtaaaccgacatggcactctgttgggcatatcttatagaaagttgtttttgccccatccgcattttagctagtcctcaatttggtccagtgtccaagctctgccttctaactcaatatgagaagcagcagccccccagatttttctgagaggtgagtaatctttccaggccatgtctgaagatgcatggacaaaccttctgctccaggactcacatgaacccttctggaagcctctgtttatctgcctcctgcccagcaatgaattggggaggtcaaggatgcttacatctatattcttgcctccactctcttcctccacctgggtcactcaaatagaaatattcttcactgcatctcctgtctccacagtcaacagttcagccttggattatttgtttgtgcattagttgtgatcaggttgggctgcaattgagaagaaaacaaacgatgtttttcacttacatacaggctagcctgtccattgtctattgctgcatagcaaatcaccacacatgcagcagctttaaaagacacaaagttattagctcacagcatccatggaccagaagtcctggtacagtgtggcgcagttgcgttctgtgctcagggactctcaaagctaaaatccactttggctttcaaagtgttggctgggctgggctgtctgcagactctggggaagaatccacttacaagtgcatctaggttgttagcagaattcagttcattgcagttgtgaaactgagatccctatctccttgacatgcagatgccctcatcttcaagccaataattgcatggcgaatccttctcatgcttcaaatctctgccttccccttctgcgacgggctggaaaaagatcttccctttcaagggctcatacaatttaaactaggtccacctggtgaatccaggacaatcttccgattttaaggtcaactaattggtaccttaattacattttgccatgtaatgtaacatatccatgaataatgccaagggcaaaagtcatgaggcccaagctctgccttccacagctggtaaggcaactctgccttaagtcctcaggacccaggctcccttctactcaccactccatcacccctggaagggacctctgtcctcgcagcccaggattcaacaactgtatgccaaggcagatgggtatagggttgtatagggttcattctgactaggttttaaggaaggttctcagcagctgccgcacaacgtttctgccttcatcccattggttctacattgtgacatccttgcctggttgtaagggaagctgggcaaggtagctccattctgggtgtcaatgtggctgggtacaaattctgggcaggagctctcctggctaatggcaccctaactggaggactcctggggcacgtgaagacttcgtaaagaagactggtacttcaagcagtttatattttcctgattcctgcttctaaatgcttctgcaacttgaatcctcctcgtctccaaggcagtgttcatctctgaagtctgcggtggcacagctacaaaccttggcaatcttccaacacagttgtcttttattcttttggatgagttccaactctgttcccacggcagtgctccatccacgggagccgcagcatcggcaggggctgcttttgcacagcaaagcccccttggggagtactgcacactgtccccaagagagcccctgggccaagaggaaggcgccgcctggggttgtggtggttcaacaacgccgttacgcccgggactcagggtcaggccagggggcctggacaagagaggaagcagtgaccctgttcacccacgggagggagaaggcagccttgggccacttcaggaaccaagccaggaggatggggaagttccggtgaggctgttcactcatcagaagaaagaatgttctagaaatcagaacgttctcactgagggaagactcttctagagacatcagttctgtgagagcaggggctgtcgtgtgggcctcaactctatcctccgcggttagaactgtgagcagcgtactgtgaatactccgttgatagctgccaaatgagtgcgtgggtggatggtggaacccagacgatgagctggtgtcgaaggacccctgtgggacccgtatgtatgctaaggcaggggtggctgaagcagtgccctctaaggagcatctccagttcaggacgccaggacccctcaccggcccagggaagctgggaaaaactccccaggagcggccccttcccgctttgtt

SEQ ID NO: 10291 - RNA, 1538 nt, Homo sapiens
  source 1..1538: mol_type = other RNA
catgctgacctccctcctgccccagcagctccccactgcctgctctgccaccagctggggggcaggctctgcagggttcctgctcccaggatccacaaactgacctcagcttttgcccatggagcacccaagaagggtgaggcatggcctgggctgagctcccccactccagcctcctctacacagggaccttcgccacagaatggcacaggccggggaggccgacgcagcagtctgctggcggggggacaagtgagaggggcactgctccttagggttgcagaccccaccccctgccaggccgtccacctccaccagatccacacgcaacctcctccttgccaggatcccaccagaatcggccacagctggaatcacactaagccggggactcctccctgccaaacacctccacttagccagagcagggctcatcacaggcagccgcagaaccgactggaggtctttgctagtaggggacacgcatctgccgacccccgagatgggcccggcaatggagatgaaggacttgggaccgcaaaaaagccaatgccatgagcccacactgtgatccttctgcagcagggggcgccttctgtctctgcgcccagactctcagccacagccagcttagcccaggccagcggccacacctgcccgacccgctggccatatgccattggacctttccaaaaagacaggggcagggtgccccatgtgtgagccaatgtgtcctgtgctttggcaaatcttgcccttggggggatgggcagagggcagagatgtcggggaggtcaccagcagggcctctgggaatcaagaccaagccttggcggcccccgcgtcacaggggcagtggggtggagtgccaaggccatcagcctgagacagggtagcctgtgccccagactggcacctgtctgcagcatgcccggtatttttagcacagccaggcagctctccagccctggcccacaaacccccaccctcccagaggctgtccctcatggaagcccacctgagttggggcacaactgggctgaacacaggcagggcttcctccctggcctcacttcttgtgcctggaaccagccccccacttgctgagggctgccccaacaagggggacgagcctggacaggggagctgggtgcgcccacccactcccacctctccccgggggctgggatgtgagcacacaggggcctgtagacccggcgcctcctcaaggcctcccctgcagggcccccaccccaagggtctggggtctgtcccacttccaaggcagtcccttctgtccagcatggcactgccctggagtggccgcctcatctgagcggggtctccagccatgcctgcccgcctgccaacccttctgcggtgccagtgtgcagacagaccacatgcgcgtggatcccaggctcaggagctcagtatcctggaccctctggaggggccagcagttttggtttttttgagacgtaatctcgctctgtcgcccaggctggagcgcagtggcgcaatctcagctcactgca

SEQ ID NO: 10292 - RNA, 2001 nt, Homo sapiens
  source 1..2001: mol_type = other RNA
catgctgacctccctcctgccccaggaaaccttcatttccatctcaggttcatcctcttctcaaggttaaatccaaagtgatcggtccttatccacttctgggaaaccattcctagccgacttcacagggtggcggggccagcacacctccgcagctgtgcctctcccctcacctgcccagtgcaccttctgggctgtctccctcctctgttttctcagggtcctgtgtggcctcctggaggctgccatcttgactccctgggactcagtgagtgcttggtggctgccccgcccccctccgcgatctcttgctgggccacactgtgacccatggcactgccccctccctgatttctttctgggccacactgtgatccatggccgcgcaccaggagatgggcacagtttccacttggctgccaggactacagaggaattttccaggagattatccaccagcttctttgggctcatggtcaatatcaaattccaggattcattgttgatctggaaatggcattcatcttttgaagactgttttctgtgaccatgggcccatacttaatctgaggtgagtggtatctgtgtatctaggatggcttggtttttgtaatctgcactaggaaggtaccatctatcgtgctgttctggaagaagccatctgaggcagaggcatcaagcatgaggctgaggacaatgctgaagggctggagcagctcttacccaagctaggtgggcatcccggggggatattgggacttggcagtttgttctccacctggctcctgggctcctggccctgagaacgtcctccagcccagctgcaggaggggagtcctgagccagcttctcatcttcctttcctctgcagccacatcctcttatgtcctacttggaccctggtactctggtcattcattcaggcaacacagaaatatcaagcatttgatgcaagccaggcattgccaggtgctgaaaaaacaaaaataaataaaactccattttgaccctcttggctgtcagacactagcagggtgggtcatgggcaagcagtaagtgttacaacacggtaagtgttttggttgaagtagcaaacaatatagtggaggagacaatatatagtagcaaactatcgtggagaatcagaggtcagacagccactgattcaattctggttcccttaactagctagatgacttaagtcaagttacttaacttcttggagcctcagtttccccaccagtaaaatggggttcttaactcttcctcatagttttgttgtgatgactcggtgggctaataatcacagacttattaaagtgctggcagttgatgaagtcttttaagcaacatggtgatcacatcatctggtcagatttgctcacttttccataagccagtgattctcagacatcactgtgcattaaatcactgttgtatgctaatgaggtgattcagggtggatctctaggtagtttcaggactggggctggttctgggtctcggagaggttcagctggcgggccagctcagtgcgctcgcggcccaccacatactggcagcgctggaactccatctccaggcggtacagctgctcggcagtgaaggatgtacgtgtccgcttgggccggtccaggtccaggcccttaggcaggacaatttcccgaattgtccctttggcatctcgcaccagtatgcggcggcagtggtctgcctcgccgggcccgggctgcccgtcgctgtcggctccactctccctggagcctgcgggactggaggctgaggtcccggccacctccgttgggctgtggccaccgccatcagctcgcaagtcccccgctccgctgcggtctccgcagcgcccaccgccgccaccagactccgcccggcgcgcggggccccggtcgcgctcggcgcccccatcgcccatgctgaccgccactgccaacccctctacggcggagccagcctacgctggccgggagcgccgctccccgcccc

SEQ ID NO: 10293 - RNA, 1541 nt, Homo sapiens
  source 1..1541: mol_type = other RNA
catgctgacctccctcctgccccaggaaaccttcatttccatctcaggttcatcctcttctcaaggttaaatccaaagtgatcggtccttatccacttctgggaaaccattcctagccgacttcacagggtggcggggccagcacacctccgcagctgtgcctctcccctcacctgcccagtgcaccttctgggctgtctccctcctctgttttctcagggtcctgtgtggcctcctggaggctgccatcttgactccctgggactcagtgagtgcttggtggctgccccgcccccctccgcgatctcttgctgggccacactgtgacccatggcactgccccctccctgatttctttctgggccacactgtgatccatggccgcgcaccaggagatgggcacagtttccacttggctgccaggactacagaggaattttccaggagattatccaccagcttctttgggctcatggtcaatatcaaattccaggattcattgttgatctggaaatggcattcatcttttgaagactgttttctgtgaccatgggcccatacttaatctgaggtgagtggtatctgtgtatctaggatggcttggtttttgtaatctgcactaggaaggtaccatctatcgtgctgttctggaagaagccatctgaggcagaggcatcaagcatgaggctgaggacaatgctgaagggctggagcagctcttacccaagctaggtgggcatcccggggggatattgggacttggcagtttgttctccacctggctcctgggctcctggccctgagaacgtcctccagcccagctgcaggaggggagtcctgagccagcttctcatcttcctttcctctgcagccacatcctcttatgtcctacttggaccctggtactctggtcattcattcaggcaacacagaaatatcaagcatttgatgcaagccaggcattgccaggtgtgttgtatgctaatgaggtgattcagggtggatctctaggtagtttcaggactggggctggttctgggtctcggagaggttcagctggcgggccagctcagtgcgctcgcggcccaccacatactggcagcgctggaactccatctccaggcggtacagctgctcggcagtgaaggatgtacgtgtccgcttgggccggtccaggtccaggcccttaggcaggacaatttcccgaattgtccctttggcatctcgcaccagtatgcggcggcagtggtctgcctcgccgggcccgggctgcccgtcgctgtcggctccactctccctggagcctgcgggactggaggctgaggtcccggccacctccgttgggctgtggccaccgccatcagctcgcaagtcccccgctccgctgcggtctccgcagcgcccaccgccgccaccagactccgcccggcgcgcggggccccggtcgcgctcggcgcccccatcgcccatgctgaccgccactgccaacccctctacggcggagccagcctacgctggccgggagcgccgctccccgcccc

SEQ ID NO: 10294 - RNA, 87 nt, Homo sapiens
  source 1..87: mol_type = other RNA
catgctgacctccctcctgccccaggaggaacccaacccgagctcaaccccagccccaacctcaaccgctcagaggagcccaacaac

SEQ ID NO: 10295 - RNA, 979 nt, Homo sapiens
  source 1..979: mol_type = other RNA
cattacagcacagccattctcttcctgatgagggactttgaagacagtgacgctgcttagtccactccctccaagtggtaaccatccaccacttgagtcatctcgggtcatcaccacagctcgcactcgtgcataactattaaagagtgggtttcaaggctgagctgtgagggactgcagaagaattcagaattgaattgctgtagctagagtagagacagcaaatgttattacatcattgctttttcagatgtcttcactgaagtgctccaaatgatatagcaatgtattgcaaattaatcttttataagtatataattatttgtaaatccagtaaactaactcagagttatgtgaacactgaattctaatcactaggacagttgttttcccaatatgaaatgtttttaattatgtgtattaggaaaagatggaaagctttttaaacactaaatcttttcatatgtatatcctatgggcatacgtgcgtgtatgtacactgctgatgtcaaagtgtcaaaatgcagaatgtgtttgttactgtgatgcagtcaaaaagtctgaaagccattgttttagggcataggctttggaatcataagactttaccaagtatgtaatctttgccaagtcatttaactttcctgcacctcagtttccttggctttgtaaatgggagtagtaacattataacaaacacttacatggttattataaagactaaatgcatgaaatgattttaggccaatgctgttacttactcatatatgagctgtcatttaattatgtactgagagctacataaaaccacaaggtaccaaagaacaaaaaaggaatctaagaaatttaagaacaaatttcattacaaataatccacgatagaaaaaaatgtgaattttcagaagtggcagttcatattaagaattttaaaaaaccacttgtactctttgacacacttatcccactcctgtaaatttat

SEQ ID NO: 10296 - RNA, 524 nt, Homo sapiens
  source 1..524: mol_type = other RNA
cattacagcacagccattctcttcctgatgagggactttgaagacagtgacgctgcttagtccactccctccaagtggtaaccatccaccacttgagtcatctcgggtcatcaccacagctcgcactcgtgcataactattatcgttgtcagaagtcgccgtctcctcgctcatctttccctcaccgtgatccgatctggagatggaggagcaacagcaggcgggggagcaacagcagcaccgaggggcaggaggcagcggcggccgggggggcgcgggggcagcggcacaggggcctcaccatggtggatgcctcacccagaacggtacccccccagccgggaaccccggccacccccgcaggggggtggcggcagcaacctccgccgtggcgaccccagcctcttcccccgcctcagtgcccagccaagggatccgaggaggcccggtggaaagggaaaaagagaggggctgcaaaggctgactggagagctgctcctccagccactggggtggagcgcagc

SEQ ID NO: 10297 - RNA, 1309 nt, Homo sapiens
  source 1..1309: mol_type = other RNA
cattacagcacagccattctcttcctgatgagggactttgaagacagtgacgctgcttagtccactccctccaagtggtaaccatccaccacttgagtcatctcgggtcatcaccacagctcgcactcgtgcataactattatgaaaaaagcagattccatcatcatgcccctgacactcgttgtcagaagtcgccgtctcctcgctcatctttccctcaccgtgatccgatctggagatggaggagcaacagcaggcgggggagcaacagcagcaccgaggggcaggaggcagcggcggccgggggggcgcgggggcagcggcacaggggcctcaccatggtggatgcctcacccagaacggtacccccccagccgggaaccccggccacccccgcaggggggtggcggcagcaacctccgccgtggcgaccccagcctcttcccccgcctcagtgcccagccaagggatccgaggaggcccggtggaaagggaaaaagagaggggctgcaaaggctgactggagagctgctcctccagccactggggtggagcgcagcggggtccggccaggaaggagtcggcgggcggagaacccgggagcagaggcggcgcttccctcagggatgcggcgaggaggaagcagagctccgctcggtgggggccggcgggggggtgccgagcccaggctccgggcagcggcggcgcggtcctgccggagcccaccccaccatctcccgcctcgccgccggctgcccctcaacccccggcggcgtctgggtcggtcctcaggcgccggcagagcagggctaggggccccgcggcggcggattcctccagacacgctccagccgggactcctcctcaggggggtggagggggcggcggggagcgtgtgaggcgaggggcaggcaaaccgatcgttcccacccggccggagaagagcgggcgggcccgggtccggggggcaggatcccgagaagcggcgggagaggacaagagcggctgcaggttccccgccagccagtgcccaccagcagctcagcgggccagctcctcacgcccgagagaggggagccgcgaggggggcggcggaagcgctcacgccgcccgctccttccgccgccgcagccgctgcccgaaccgggggcgcccgcgagagaaggaggcgaagtagtccctcgcgacttctcccggccgcccgctttccccggaggccagagcgggcgcggggtggggctgccgagcggggtgcccaggctgtgagggtgtgtgggtaggactaaaagccgcggcctccgggcgaatc

SEQ ID NO: 10298 - RNA, 24149 nt, Homo sapiens
  source 1..24149: mol_type = other RNA
ccaaaactgcagttacttttgccaacactgtttttcacttcaaagctatataatcctttgtcactcatttcggcacaggggattttaagggaagccactttattgatgaatgtaatgtgatgtttgctgtctgcagacaattctcttccatctttgaaccacttggctgagagttctggtgttccagtcactacacactctaatgcaaaaggatttccagtagtgacagtcatgggttcgggcttctctatgattcttgctggttctagtacagtcaagactgcagagcattctctcattccagcatcgtttttgatttggcatatatattttccagaattagatgcttctggactccccagctggagggttgcaatgttatcaatgaatgaaatcctggtattttcactctctctgatgacttcacctctatctttcagccagacaacagaaattggctggaagccctccactatggcccgtaactcaacagcatccccaataagggttgaggtgtcacttagctttttcacgaatcgtggaggttctttgaacttgacagagcaagaacacgtgtcacttcccacctcattagtagctttgcagtgatattccccgacatcggaggcttcaagattaaggatatgaagacttgtatcaaaatgttttgaagtgattttaaatttcttgctgtttctaacctgctttcgatctttaacccatactacttcaaatgggggagttcccgaaatttcacattggagaatcacatcagaacctttaagagctcctactggagaaggcttctgggtgaaaacaggaggtgctttcactgtcaacgctgtgctgcagctggcgtcaccaacaccattatgagcctcacaaatgtagtccccgctgtcttcagcactagcttcattgatcgtaagcaatgccacagaattaatgaatgacatgttgtatttccaactttcatgaagttcgctgtcatttcggaaccatgaaactttgatttctggggagccacttattttacattccagttgaatggattctccctgctttgcaacttttgaagcttctaatttcttaacaaactttggaggttcttttacactgagctgagctgagcacatgtctttgccaacatcattggttgcttggcaagtatattgaccagagtctcctttgcctactttaagaattctcaaatgaggagtgtttcccacacatgtgattgtatagtttcctccaggacggatctccttgttatcttttgaccaagtgattcgcatcggttgagcaccagtaacatgacactcaaaatcagcactttctccagcaataacatctatagatacaggcttgatgtcaaagaagggagatttcttgggttctcttgctgtgagtctagcactagaagatgctgttccaagtgggttggaagctgagcaagagtactggccagagtgactcaagtcagtttgcaaaatttttaaagttgccacattatctacaaatgaagtctgtagattttcatcgtctcttaaaagtactccatctctataccagcacacttggatgggtgcagagccatttaatcgacaagtgagtgtaacaggtaaccccacagtttgttcaatgtcctttaattgtcttgcaaaagaaggtgggagttggcgctcttgaattctgaacacagtcttagaagaagcagttcctatactattttctgctttgcatgtgtactctccactgtcattgatgttcactttattaaaaacaagtgtggccacattgtttgtaaagtaggtcctgtattcaggagttggccgtaatttggtatctcctttgtaccaagacactgtaatttctggtgtcccagcaacttggcattgtaaagaaaccgaatctccaactgctgcctccagaggttccagttccgtaacaaaataaggcggttctaatgtagataccagagctccacaaacatcccttcctgcctcattttcaatctcgcaggaatactgccctgcatctctttttgtgctattcagaatttccaggatacaagttttctctgttgtgactatgttacatttttcagaggtagttatgttaaaaccatcctttttccaagtgacagaaattggaagtgttccagtgtaggtgctctccagaattatggacttccctggttctacagaatgatcacttaatctcttcaaaaatgcagctggttctttcacaaagagacgggtagtgcaagatgcttggccagcgttgttagaaaccacacaggtgtattccccactctgagatatgtcaatattaaataattccagttctgccacagtgtcttcaaaatagatgttgcaccggtctcctttcactagttctctggcacctctgaaccagttgactttgaatggaggggttcctctaataacgcttgtgaaggttacatttttgcctggtagtacttccaaaggttcaggttctttcacaaaagagggtggttcttgtacagttagcactgcacgacattcatcagacccagcgacattagcagccacgcatgtgtaattgcccatatctgaggaatccagagaattcaactgcaatgtgcagacattatctgaaaatgtggtttggtactttgctccactgacaatcttggttttctcatgaaaccaggcaactgaaataggtgatgatccagctactttgcattccaagatgcaagaagcacctaacaccccaccagtatttttcagtcttcgtgtgaaagagggaggaactgctcggtctgaaacatcaaccacagctgtgcagctgcttttcccaacattattttgaacctggaaagtgtatgtgcctgcatcttgcctttcaactgagagaatccttaaggaagagattttgttgtagaagctaaatttgtgtttttggctgctggtcaacagctttccatccttgtaccattcaacagagagttccggagtgccagccaccttacactccagagtgcacgtttctcctacagtcaccgtcatcggtcctgccttctcaacaatgactgcgggctctaagaccatcagtgtggccatgttctccctcattccaccatcattcttgatttggcagatatactttccagcattagctggctctgcttttgcaaactgtagagttgcaacattttccacaaatgtaatcctgatgttttcactttctctaatcacttcttccttctctttaagccactggacaaaaataggctgggcgccttctatggatgcttgtaattcagcaggctctccggctacaacagtgaggctgttcagtttggagacaaatcttggtggttctttcaattttacagtacaaacacaagtatcacttcccacttcattctgtgctttgcagtggtattcaccgatgtctgaagtgtccacattgagaatgtgaatacttgtgtggaagtttttggatgcaatcttgtatttcttgctgcttctgagttgccgcttgtctttgtaccataccacctcaaacggtggtgttcccgaaagttcacattcaagactgacttcagcatttttaagggtttctactataggagggaagctgctaaaaacaggtggctcttttactataaccttggtactgcagcttgtgctgccagcgggattctgagcctcacaaatgaaatctccactgtcctcagtactgagattgttcatctgtatgacggccactgagtcaatgaaagtcattctgtacttatcactggctggaagttcatgttcatttcggaaccacacaactctgatttctggggatccagctatcttgcattcaagtcgtgaagagtcacctgctttcacaattttggaggcttctaatttctttacaaactttggtggttctgtcacaagcaacatcgtagtacaagagtcgctaccaacatcattggtaacatggcaagtatactgtccagtcttagaagcatccactgagtagagatttaagaagctagtcgacccttccaagccaatgaaacatttaggacctgagacaagttccacatcatccttaaaccattttattttaaatggtggtgttccttttagtattgccttaaattccactgtagaatcaggtatggcttgctgtcgcccaggtttcactaggaagcttggtggttctttcacagttaagatgccactgcatgcatcatctcctgctacatttgacactttgcatgtgtaatttgcagtatcttctaattccagattattaacttccagagacacagatctctcatggcacacaagtctgtattttgcacttgtagatatttcttttccatccttaaaccactgagcactaatgggaagtgaaccagacaccttgcactccatatgaatagaagagcccagaactttatccattttggttaattttttggtgaatgatggaggaatattttgatctagcactcttaagtaggcatcacagctactgcttccgaagtcattttccaccttgaaagtgtactgaccgctgtcctgcttcattactgactgaattctaaaactggccacgttattttcaaaactcattgaaaagtatctactgggaactatttgtttcccgtctttaagccatttcactttgagttctggtgttccagccacaacacattccaaggtcatgggatctttctccgtaacatcaactgatttagctttctctacgatttgagctggttcttgtactaaaaggaaagcataacacctctcaactcctgactcattcttggcttgacaggtatatctcccactgtgtccattatccacacttctgatttgaagtgtggccacactgtccacaaatgaaatatagacattatcatcttcatcaagaatctgatcatcctttagccaggttatagaaataggaggagaacctgccacggtactctgaaaggtggcagaacttttcaaaacagtagtggtattttctatcttcttaatgaatgatggtggttctttcagggcaactctagtactgcatgagcagctgccgccttcattggatacaatgcactggtattccccagtgtctgaagggtcacacttggttatatggaggttaaacacagacactctgtcggtcaatgtgtattttttgctgcttcgaatttccctgttattcttcagccaagtgacttcaaacggaggtgttcccgtaacttcacactccagctccacgtcactatattttactacctccacaggcttcagctctctgataaaggtggggggttctttcactttgagttcaatgctgcagctcgccgtgcctgcgtcatttcgagcttcacacacataagtcccactattttctaccctggcaccagaaatctggaaagtggctaaaccatcaatgaaggaaatgccatgtttctgaatggctgttatttcattcccgtctagataccaagacactcggattttaggagtgcctgttatttggcattcaaatgttgttgactgtccattcctcagcactaagactggactgggcttcttaatgaattgaggaggttcttttacaaagagagtggctttgctggttgctgtgccaacatcattgcttagttggcaaatgtaggttccagaatcggtagctttggctgcaaagagctctagactggtagaggtgtcatccttccaaactgagcgggctgctcctgagtgtaactctttgttatctttaaaccactttattgtcatgggtgcagtgccacccacaagagcctttaactgtacccttgtgttgggattgacatcttgtgactgtggcttttccacaaagtaagggggttctttgactgtcagatgcccactgcattggttgtgccctgccttatttgtggcagaacaagtgtatgtcccactgtctgtaccttccagctggctgatttccaagaaggcagtattgtcatgaaaagagaatttgtacttttcactagctgatatttcttggtcatctttgaaccactggatgcttatgggatgtgacccagccactatacattctaaatcaatgaaagaacctttaatgctgtccattttcttcagctttttggtgaatgaaggaggtatgataagatctaatacattaattctagccttgcagctgctcctcccaacatcattttggacctcgaaagtatattctccactatctttcttttctgtagaaataatcttcagtattgagactgtatcagtgacactgattttatattttgagcccagggtcagttcttggccatctttaaaccatttggctgtaatctccttagtccctgaaaatttaacctgcaaagtggctgggtctccttgggtgacatctatagacacagcttcctcggtgattgttgcaggttcttttactgagagtaatgcagaacatctttgtattcctgcatcatttttggcctgacagacatatttcccatcatgcttgacttcaatgccactgaggtacaaactggccacattgttctcaaaggtcattcttatattatcgtcttcagtgatttcatcgctgtcttttagccaagtcaccgtaattggcaaggagcccttcagagtggcctggaaggcagctgtgcctccccggagggagctggtactctcgatcttctttatgaaggatgggggttctcttaaagtcaccctggcactgcagatgctgctgcccacctcattggtcacccgacactggtattcgccagcatctgcagctacaaacttgaggatctgcaggctaaccagatgatcctgaatgaaagtcttatactttctaccacttcgcaggattgtgttatctttgaaccaagtgatctcaaagggaggagtgcctgccacctcagccagcaacatgacatcgtactcctttaagacttcaattggcttaaattccttggtaaaataaggtgactctttgactattacaatgctactgcagtggtcactgccagcctcattttgggcctcacacatatattcaccactgtcttcgatgccaacatctgtcagtcttagaactgcagtagactccacaaaagacattctgtgtttgctgctctccttaatttctctatcatttgcaaaccatgttattttaattggaggggtaccagttactttgcaggctagctgggtggcatctcccttctttaacagctgtgatggctctaacttttcaacaaatgtggcaggttcttttacaaacaagtttgcactgcattccacccctccagcgacattgctgactttacatgtgtacgtgcccgaatcagaggtttttactaaatagagttccagggaactctctaaagcttctttggtaatatagcagcttccaccagaaaccagctctttgttgcccttaaaccatctgattgtgagaggagtagatccttggaaagtgctcttcaggcagactgctgagccaggcagaacatcctttgagccgggtttagttacaaaactgggtggttcttgcacaatcagggctccactgctgtctttgcttcccacggaatttgtggctcgacaagtgaaattccctgcatcattcatgtctactctgatgatctccaaagaggctgtgccttccacaaatgctatcctgtatctgtcagaagcagctatttctttgccatccttaaaccaggacaccctcatggggagggagcctgcaattttgcagtccagtctgcaggtaccattaacaacactatccacgttgcgcaagggtttggtaaaaaatggagcaatgtctcgatctaatacagtgaatgtagtctcacaggagctgctgcccacttcattggaaatctcaaatgtgtattggccactgtcgtgcagctcagctgaataaaatttgagctgggcaacattgtttttaaaacttattcggtattttttactggcgaccaagggtctcccatctttgtaccatttgggcttcagttctggcgtgcctgccactgtgtactccagtgtggcgggatctcctgctgtcacctggatcagttctgctcgctcaatgattttggcaggttctttaactattaattccccaacagatgtttggcttccagcttcattttcagccaggcacgtgtatttgcctccaaaactaatctgaacatcagggattatcaagactgcaacaccattggaaaagctcattttgatttttccgtcttctctgatgacctcttgacctttcatccatgtgacagaaatgggctctgaccctctcacagcagcttgcagggtaacggtttgtcctcctagtgcaatcaaatcatctactttctttacaaaggttggaggttctttgagtaagtgggttgccatgcagccacacttgccgacttcattagcaacaacacattcatattcaccaacatctgcactattaaacgaaaagatctccagacacacaagagacttctgagaaaacaatctgtattttttactacttcgaatttgtttcttgtctttgaaccagctaatttcaaatggtccagtgcctgagacttcacactgaagtagagcatttgttcctctcactatgtctgcaggctcaagagttttgatgaaagaaggaggttctttgataactatttcagtactgcagctatcactgccgacgtcattcactgcttcacatgagtaactcccactgtcttcaacttttacatccgtaatatcaagtatagcctcagaattgacaaaatacattcggactgtgttactttcactgagttctttgttatttttaaaccaagtaacctggatcacaggtgagcctttcagcttgcaatggaggcgtgctgattcacctgggagcattaaataagagggatccaccttcttcacgaaggatggtggctctctgacagtgactgtggctgagcaggagctgcttccagcctcatttgaagctgtacagacataggttcctgaatctttcagtttggccaaaggaatctcaagtgttgctattttatcttcaaaacagatcttataatctttccctggggggagtttttgcccatctttgctccacgtaactgtgacttttctgtcttcatctacttggcactcaaggtggaccttcttattgatagcggactgcacaggctctaattctttaatgaaatgtggcttatcaatgatgatcaactctgcttggcagatgtctgctccaaacttgttggaagccttacaagaataaactcctctatcttgaatggtaaggtttgagagttctaaaatgtgtttgttttctgcgtcggaaatcctccagttaggtgaaggtgagagtgcagcaccatctttctgccaaatggtttctatcacaggagtccctgtcactgtgcagatgaacttggctgccttacccacaaaagttgtaagggacttaggtctggagagaaaggttggtggatatgcctctgtcacagttagtgtggctgtacagctgacactgccatactcattggaagctttgcatgtatactcgccgcagtcaaccacctgggttctcaggatttcaaggctggagatatactttgaagatcgaatagaacacttgtcactctcataaatttctcggccagctttaaaccactggaaccggacattgggagcactttggatctcacaggtgaatttggctaggtggcccagtgctacttccaggggttcgattttcctcttgatcactggggcagctctttttactacagtgagtttggctgaagttgctgtttttccgctgtcattcaaggcctcacagacatactctccttgatggtcttcggtatttactttgtcgatgactagcgtatatgtattttgatcttgtaaacacttgaacttttcatctgaaggcaccagtttattctcaaaataccaattcacctctttagcatttgttatggatgttgtgaggtgtacaatatcaccttcctcagaaacagtgtccactaaaggtgtatgtatcatggggccatcctctttgattaagccaccctcagcttcctgtatctttactgtagcaacctcctcagtaccactttcagaggaagactcctctttttcctctgatggtttcagactctcatcttgtttttcgtcagagacaacagctgaagcaacccctttagtgacaggtgtggcatccaaatatttaaccctactttgcacgttaaaataactgacctcttcagttgagatcagatatttagattcaacttctggttcagtaatgggttcaaccttctgtgaacctgaaaaagaatccatttcttcttgcaaacttgttttggctccttgctgaattctaggaccctcagctgttaggatgtctatttcctcatatataatagcacacaaagcatccctaagttccattttcaggttagccatttgaggatcaacatcttcaataatgatggttacttcttctgttacagactttgccgaagtaacaaggtacatgcacatgatgtgtctgggctcttgggtgatgtttacagcctcgacctccaccttttcaatatttcttagccactcagagaaaagacctggctgctcgctggccacggctgcttgcaaagcccggcagatttgaattttcaggtttaatctctgctcttctggaataccagaaagcaagctttccttagaaagaaggtcccttccctgtacctcctgcactttctttattgccacgggctctcttttagactcaatgatttggtctgggggcatcaccacgttgtcagaatgctcttctttgagcagtacctgcttttcttcaagtgctagtggaaatcttaaggacttgccttcctcaattctgaccgcagaatcttgccctgcattttccagtggatttgcactttctatcaaaattttacctccttctgtgcatgagtgttctgaagggactaggggctcatagtttacctgagagatcatgacatcaggactctggagactctccacgtgtccctcagctaagctctgactcaagatgagcgcactttgtgcctcttgcttttgaagagtcactctttgctctctgttggtgtcagatactgtcttttcttttggtgaaagtacttcctcagccacagaggttagataagaatgcattggaggttctattgaagactgtggataattcccttcaggttcagctaataaagttttcagaggctcaactgttaatgaattaatttgttctatggacatggcacttgggaagattttctcggtatctgatagaactgcctgtgtctcaggctcttcaggcattagaataccttctttggagaaggttttctgggactgtacaatctgcagctgtaggttgggagatggttccttgagaggctgaaagtgaatactgccattgatgcaaagaaattccctggtgctttcaggagtgagcttgtcttgctccaaaatggattgcaattcctgagctcccaaaggaagctgactgctcaattcattggctttagcaatatgctcataagatagttgctggttttcttctgtaattaaagcagctttcaaaatggtgtcttttacaaacgttgcaatttcctgctctgagtcaagtgcttcaactgcgggaccctttaagggtgtctgtggaaaatcctcaggagcctctggtgtggactttgctttgcagggggtatcagtcatgtctgtgtcttccagaagcacaagcagctctgctgcacaggtggactcacccaacatattctctgctttacagatatagaggccactgtcttccctctgagggtcattgacaatgaaagttccagagccattagggttatgaatgatagtgtaataaacactggtgcaaagctgcttgttttctttgaaccatgtaacagtaggggcaggctctccaaccactgtgtactcaaagatggcaggaagcccttgagcacagcgaattggttttaactccttaaggaagtgaggaggacaaggacctcccagcttttccagagattttgccactgctgattctgtttcagtgtctttgtgaccctctcctttggaattaatttttagataggcactacatattgtctttccatagtcattactggccatacatgtatactctccctcatcctccaatttggtgaacagaatgatcaggctatgatcatcaccgtcaaaaacaaatttgtagtcagcagaaggggttaatagcactccattaaagaaccactgaattttaggtttggggatgccaatgacagttacagacagtgtagccacatcccccatgcttatatcagcatttgacacttctttgatgaaaattgggccagtgccttccttttcggaatcaaatttagttgggtaaactggagattcagacaaaagttcaagtgtttcatttattttagataattgaagttcggcgctatgaagtccttcttcctcggcagacagaaaagaactagaaaactctttcatttccatctcaatctcttgttcaatcctctcatgcaaaattgattcaggagcaccttctacacttagtactgctgacgttgtcctctctccacagtcattgtgtacaatgcagctgtatagtccttggtctaccagctgaacattacatatggtaagaaactgaatatttccattttgtgattgtttcagtctctcggattcctctatctttgcaccttcgtgagtccaggttacatcaatgaaagaatcatcttttaaaacacagaggaattgagccgtgtcaccgcactttacagtgacgtcctgaagatgcaggaaaatcttgggcgcctcacccgtggactctttagcacattccttagatagctcagtgctttctgcaatttgtgaaagggatgcagtatggcacaactgtgtatcttgaacagatgcagctgtgtggatggaactttgagatacactttcaaaaacctgcacttcatattcatatgatgatccttgaaatgacttaatttccttttgagatattttgctctcctcctttgtgaaagaggaatctgccactgcctgggacttggtggactctcttacatctttcccagaactttgcctatctagggcttgcacttttggagtcactgtgagtgtagctgcacaagtggcttccccagcactattggctgctttgcaagagtactgcccagcatgctctgagtaagcatcaactataagcattaaagccatgcctgtggactcctcaaaatggaaaactacatcttttgttggtagaattagctgctggttatgaaaccattggatttctggcttgggaatgccagaaaccctcgcatgaaatctgactgtctccccgttgtgcaccctgaggcttgacagaggctggatgaagctgggcttttggccaaggggctccttcttaaatgaaactgataaagagacatgccattgggagtttgatgtattttcttcaaatttgctaaatccttccagactcaggttggctgtgcttgatacttggcctacagcattactagcaacaaacgtgtaagttccttcatcttctggataagcttcggcaatttccagttgataagtgtcttcaaattgagtcattctaaagaaccgagatggcttgattttcttgtctttgctgtaccacgacacttttagatctgttccagaaacccggcattgaaaacgggctggctgcccttcagaagtgacagtgtcctgaagcggggtgatgatggcaggtggataaacaggcatttcctgatcaggagacacaacttctggaacttccactgagagtgaagctgatgttgtggcaacaccatagtcattcttggcttcacaggtatagactgccgcatcctctgggaaggcttcaattagcaaaagcgtgtattcttgcccatcatgaagaaatttgcacttgaagccagtggaaagcagctgctcttccttgtaccaggaaattttgggctgtggtcttccggatatcacggcacagaagcgggcaggcttgccagactgcacagtgacaggctggagctcctgcagaacttggggcggttcaggagcattgacatagagagtgacagaactcctgttccttcctgccacaaaggtgtattctcctgcatcgctctgtctggtctcagagataaacattcggtggattcttctttccactacatatttgtgtcgttcttgaacttggaaattgatttcaatgccatctttataccagtgggcatcaacatcgtcttcattgacctcaaattcaacaacagcacgctgtttctcaatgacctgaacctcctttttaatacttcggatgcgaacatctctgccttctacaaagagttttgcagttgacacgttgcctcctgccaccactgtgtacttcccagcatcagacatccgggtggatgggatcagaaggcggtggacatatttctccttctgaatctttattctgtctgtgatctgcagttcctggtcatctttcatccactgtacagtgatgtcaggttcagaaacttcacattcaaacatggctcgcttcttctccagtaccttaatgtccttaatgtgtttcctaaattctatatgacgagcttccacataaagtgtggctgttgatgttgcttttccagccacaaaggtgtagtcagcagcatccccaaagtgaacattcctgatgttcagtgagtgtgtgagctttttggttctcatctggcacttgtcagttgatttgatttccacaccattctttaaccatttgtaagagatgccttcatagttcactgtcacctcaaaagtaatagtgtctttttcttcagcgttgatgtctttcagcatggaagtaatcatgattggggtgactgtcagggtggcactgacttggtcattgccacagacaaatgtgtattctgccgagtcctctgtgctggtgttcatgatgatcagctgatggagttttccctgcacaactatcttgaacttttcactcatctcaatttccacaccattcttcagccacatggaagggacattgaagtgggacacctcacactcaaaagaggcagttttggtctcaggcacctcgatatttttcatggtttttgtaatatgtaatgtctccacaaacagttttgctttgcattccaattgcccgaccacagctgtgtattccccagcatctgagggggagatgttctgcagcatcagcttgtggactttcctttctgagaccagtctgtgtttgtcacttggcttaatttccacactcttatggaaccattttactggaacagtgtcatgggaaacactaacttcaaaggcaacagtggcattttccaaggctgtcacatcctttggctttttaatgatcttgacagtctccacgtgcagtctggcactggctccaagccttccaagcctgaagccataaacagactcatccacgatggcacagtttttaatcctcagagagtaaattgttcctttgacagagatagcatacttttcattggattccagcacaactccatttttgatccactggacacctttgacattagggtgtgtaagctcgacagtgaaaacagcatcctgtgtttctgtcactgtgaggttcttcagagtcttcttaattttgacagcttcaactttgagtttggcagatgttttggaggtggccaccttgtaggtatattctccaatgtcatctaatttggtggcagcaatgataagtctccttttgtggccatcagactcacttctgatgttgttagtcagtggtaggtgtttgccatccctcaaccattcgcctttggaatctgggttggcaacttcacattcaaacacagcttcctgggattcagctacggtctgatctgtgagtggcttggagatggccccacctgccacagtaagttttccagatgtcatattttctcccgcgtaaaatgtgtattttccttcatcatctttcatcatatttagaactgtcaatttatatatttttccatgtgcttcaattttatatttagaactgggcttgatttccttgtccttaaaattccacaggacatcaattccagagtgggacagctcaacctcaaacaccacattttgagtttctgtacaggtaaggtcacgaagacctctgataattttaattttttctacagagagattacagttggtttcaactctgccaactatcagcttgtaaggtccttcgtctgaagcatgagttcggttaatgactagtcgctgtttagtacctttcacaatggcctgtacacggtcatcaggcttgatttgttcatcatttaagtaccacttaacagaagtcacatcagggactgacaccttacattcaagcacagccttggtgccttcaatcacattaacatcttttagaggtgttatcacgtccacactatagacagagacacgcccactggtggagaggccaagggctggaatggtgaaagagtaatttccagcatcttccttagtcatgtcttcaatgagcagcatatgagattgtttgtctatcacaatgtgaaccctgtcactgggctgcacttcttggccgtctttcatccagacgccttccacactttccaaggagactttaacttcaagctgaacaatgtcaccctcacagactttttggtcactaagtccttgtaggatagcaatggggcggggtttcatctttaatttacaggttgtctttttcccgtcgatgacaaagctgtattctccctggtcctccttggttacatccttgaccgtgaggttctgacgtccacgacgagatgtaattgtatatttgccattggatttaagctccacatcattatgataccattttccttctatattttctggggatacaatgcactctaattctcctgaatatgattctggaacttctatgtcctgaagttctttcacaaactcaacaactgcaccttcaacaataagtttagcagtcgttttgacattttcatcttccacaagtacacagctgtaatcttcagcatcagacgtatcaatggtcagtatggagaggaagtgaacctttctgtcagagtgcatcctgtatttatctccctcatgaacctccataccatctttataccatttcactttgacaaatggttctgaagtttcacattcaaaggttgccatagtgtctttttccttagcaacaacatcttgtaattcctgtgtgaaagtgatcaattgcttggcttggacaagtaagaatgcgtgactggaggtttctccagctatgttgatggcttttaccatgatgctggcagagtcctcagcagtcacatctcttatgaccaattcacaaacattgtcttcgggccagtaccagtagatccggtcagaccgttcaattttgacaccatttttgtaccattcacattcggggtctggtttccccacgactctgacccggaagtgtgcatcagatccttggcccactgtttggctctggattctttcgaagatttttggagcctccatactaggacttagttcaatcttgtcaggtttaaaagttggaatcgtgattttgccttcttcggcaagagctttcttttcctcttcagttaactctttggtccagtggagaagttcatcttttgtcttcctgaggagttcctcataggattcatccttctttcgagacttgagctccacagcggtaatggcttcataatagccctcttctgttctgcgcttgaatttactgcgcagctcttccgactcttcaggcactttttcatgggtaattctttcagcccttttcaacttcacaacttctttggtttcagtggtgtcaacaggtctatccactttttgtacttcaaactgaagctttcctggttcatgtacgtgaaactcaggccttggttcaggagctctcctaaggacagacctaaaatcttccctctgttgaatctcaagcttcactttatgctctatcacaccttcaggattttccgcggtgaccttcacttcacctgtgtcatatgatttgcagtccacgatgtccaggtaatggataccatcatagcgaactctgaaccttttgcttttgcggatgagctgtccattgaggtaccagttgactttgggctgagggtagcctgttaccctgcagcggaaccttgcagtctccccttcaagtactctaactggctctgggtacaagacaatgtctggcttttgcttttctttctgatctgttgttacacctgtaagtgcaccttcatgagccattctctctaattcttcaattctctgtaagcctttcctcccctcaggcaattgggattcttccacaagacttttctcatctttaacaataagggtagcagatgtgtgatctgttccatatttgttagtggctctgcaagtaatgataccactgtctctagaatatgcaacgccataatcaaggctgcagtacccaaattcattgatcatacggagcctgttggctgcttcaagtggctttccatcatggagccactccaccaccatcgttgggtcaccaatgggtgttagcctgcattcaaagtgggcaggcccaaagcgcttaagtcttaaggaagtgagttttttcttgaaaaatggtttctgttgtttctctttgtcatagagatcaccttcttcccattgctcttggccatatcgcaaatggaggggctccagttctggggctgcaatctcctttgctctatatgtcccccgtgggatgattaactttctctctggctcaggctctgcaaactcaacttcaacatttactttgcatcttgtagtgtctctgccagctttattaatagcagtcgcagtataccaggcagaatcttggctgacagtggaatcgattttaagggcagcttctcccttggttccttcaattctgattttgggatatttatgaggcacaatgatgtcactgtttttcaaccatacaatgtcagggttggggttacccgtagctctgactttcatttcaagtcgggaaccttcctttatattgacatttttcagtttttctacaaacatcggttttacctgatgttccacagcttccacagttaaaatcactgaaattgaagatctgcctgccctgttttgggcaaccacagtccattccccagaatcactgggtgtggcagggacaataattagtgattgagtaccatcttctttaatgactactttatgggtatagtcattgacaatttgctggccatcatgaaaccagaacgtctctggcataggtctaccaacaacctttaagtcaaatctggcagtttgcccttctaaacatttgaaagaaacaggttttaacacaaagactggtttatatagtctctcaagttgtgactcatctgtctcctccagcctacgtccaggggacattcttgcaggggacatccgtgcaggagacatccttgcaggtgacatccgtgcaggagacatgcgtataggagacctgctcactgaacgtggagagagagatctgattctgctcactggctctagtgtgggaatgtaagtcggagctccaagtggtgcagcaggctccacatacaatttccctgagcaaattgcatttcctttaatattgctggcaaatgcagtgtagattccttcatcttctggaagaacaacaggtatacgcagactagctctgccatcttgtagaaagtccatttggtatctttctccatgtttgatgcgcttgccatctttgtaccaagcaatctttggtaatggatatccagacatcttgcaatgaaaagtgacacccatcccctcaagaattctataattcttgattcttgaatcaaatcctgattcaacagcttcagattcagaaatgtcaactgccatcttttcttctccatcttcttcaagaagttcttctaatgtagtctttattattctatattcaatttctttaataagtctctcttcaaaggaagaaatatggaattcctgatcttctacataagttctgaccactacagtatctttggccattttcttcctaattaaggcttgttctttttcatactctttttcatactcagagtatacaaatccaggtgctgtttctccaactttaggttcttgaacaaatgcagtcacttgtgtctgataaagcatttcttgctgggacttcatcagtaactcataatcagcttcttcaagcaaggaagcagatgcagaagtttctccatgcttattgcgaacaacaatagtgtattctccagcatcatcagcaaaagtcatagaaatcaccagcttgcattcaccggtttgtttgttgtaactcactttgtatctgtatccagtggttagaggaacaccagattttttccagtatacatggggctttgggttgccgccaacttggcatccaaacaccacgctcccaccttccaccagtttctggaccactggttttgtaataaagtaaggcgcggcaggttctccaggccctgcttgttcctctgtgaggctagtatcagtcataaccacatctcttgactcaacaaagcgtttctcttctgtagtaaatttctcagtcacggctgtggtttccttttcaaattcttctgacacctgcacagccagatagcaggatgtgctgacggttccagcctcatttacagcactgcaagtaaatcgcccgctgtcttccgcaaatgcttcgcgaatcataagacgagcaattccactctggaaggttatctggaagtcaatggaactttcgatttggtagtcttccctgtaccatgtcactgtcggggatgggtatccagagatgtggcactccaaggtgacagattcaccttctatgacagtcacattttttaagcccgagaccaaagttggtggagtaacaggaatttcaacaggtgctggtactcttgctgtttctgttaccttggcttcgcgtccgtgcagtacttcaaagcgctcttcacggacggtggtgccagtgatgctcacccctacttcctttttcacctcaacgccagcttcactcttgtaagtatctggtgtgtcagcgaaggggaactgtggcaagggtgtgggctctgcccttactctagtctcactgggcttcacagtaggagccttcaccgatttggtgatcttctgagcagaagatgtggctgacaactctttttgtaatgtggcaatagcactaccggctattgatgcctcatatccatgttctgtcttaggaacagaaatttttgaaacagtaaagtgagggctagctgtgcgggggcgtttatccacatggactaatctttccgttgttagatctgtagttttcttgatctgtgatgatatgtgcattcccttttgatcagtagttttgatatgagtctcagaaggagcctggattactctaggcttgactgctttagggacaacgtggggttctgaggctggacgttggggaggctcagctacctttgcggcggaaatgcgttccttatatccgtactccaaagtggtctgctgagcataggattcttcaagatgcccaggctctctgggctctctgactcgggcctggtctactgcagcaacaactgttgctacagcttcagccttttttccaacgtccacctttccatgggtaacttggatttgttcttgtctagtagccatagtttctctagttctcagtattgtttcttgttctttggctttagcagtagcaactgctattgtagacaaggcagttttctcggcttcctttctcatcttctcctgagttatttgcacttgttctcttttggtagtaatgccttctctacctcttgatactaaatcttgttctttgactttgggtgtggcaactatgactttaggtacaactgttttcctagtttccttcattatcttttcataacttaggtgcatttgatcttgttgtgtggtagtttcttcttgagctcccgggactgtttctagttttgtggactttgcagtggcaactaccaccatggatgcagcagttatctcagtttcctgtcttattgcttcttgagttacttgtttctgtttcttagtaatttcttcagaaattctagtttcttgttctttggctttagctgcggaaattactacctttggtacaaatgttttttcagtttcttttcttatctgctcatgagttacgtgcatctgctcttgctttgtggtaattacttctttggttcttgattttaattcttgttccttggctttatcggcggccactactaccttagttacagcagtcttctccgcttcctttcttacctgttcttgagcaggttggatgtgcacagcagtcgtggttgtcctctgagcagtctgctctacagcgctgatcactggttctctcactctggccatatcaacggcagcaacaacagtcgcaacagctgcacttttgtcagcatcttgtttcacctctttagcaccagtggcaacagcctctgctgcgtagctagcactggccgacacactggcggcagcacccgcagcaccactgatggtcacttgctcctggacaccgtatctcccttcccatctctcttctgtcctgatctgagtagaggttgtcagcgttgtctctctcatctcagcctcagatgaggaggccacgtagccctcttgcttccaagggggaggcacttcaggacctgtggccacggtggatgcctgagtcttacgcatgagcaatggagacctaacagacctgatgggggatgtggagattcttgctgctggagacacggacctgaccggagatggggtcggtgcccgcacgtgtctgaccggggaaggggagtgtcttatgggcgatggggactgctgccgagccagctgtgctttggcagcaatagacggtggtgttggggatcttgactttggcttcggaggaatcctgggaggtgttttatgtggcagctgttgcccagcggcaccatctatgaccatctcaactgttgcaattgatctggcatcaaagtgggcttcaatcttcttttcaattcgggtttgtcttgattctgagatctgagcagtcgaaacaattgtctttgtctttttagcaggtacttcttcttcaccttgaaccagtaattcagcagtcgaagtagctcttccaacgctattggtggcatttactgaataggtccctgagtcctcagggtatgcttctgcaatcagtaagctgtagaggtcgccttcttgtgaaatttggaaatcaagggagctctggatttcggctccatcccggtagaacttcaccacaggtgtagggattccagtcactctcacttggagtctcacttggcttccttgtctcacggtcatgctctgcagtcgttgaacgaagttgggtggtgctgtctcagctttcacgagaagctcagcagtactagtcgcttgtccagatccattggtggctttcagggaatatcgtccactgttggctttagtcacggcggggatcgtcagtttagcgcggccatcgctaaaggagatctgcacgccgggcagagtggaagtggaaatcacctggccatccctaaaccagctcacctcaggaactggaaaaccactaatgtgagcctcaaaggttgcggtactaccctccagtaccacaacgctttgtaacggctgcgtaaacgtcggtgcttgagttgtcatctttctaggcactctgatttctcaagagtgcctaaaaagggtgggactaagcccaaggttgcttctgaaacgacgtcctatggagagttggtttttctgaccatctccgacatgaatcggtgagcctctaatcctaaaaacaaaactacacagtcaagactgtgtagttttgcttttctatgcaatccctacacccgaggcgaggctgggaatgcacgactgctc

SEQ ID NO: 10299 - RNA, 23201 nt, Homo sapiens
  source 1..23201: mol_type = other RNA
ccaaaactgcagttacttttgccaacactgtttttcacttcaaagctatataatcctttgtcactcatttcggcacaggggattttaagggaagccactttattgatgaatgtaatgtgatgtttgctgtctgcagacaattctcttccatctttgaaccacttggctgagagttctggtgttccagtcactacacactctaatgcaaaaggatttccagtagtgacagtcatgggttcgggcttctctatgattcttgctggttctagtacagtcaagactgcagagcattctctcattccagcatcgtttttgatttggcatatatattttccagaattagatgcttctggactccccagctggagggttgcaatgttatcaatgaatgaaatcctggtattttcactctctctgatgacttcacctctatctttcagccagacaacagaaattggctggaagccctccactatggcccgtaactcaacagcatccccaataagggttgaggtgtcacttagctttttcacgaatcgtggaggttctttgaacttgacagagcaagaacacgtgtcacttcccacctcattagtagctttgcagtgatattccccgacatcggaggcttcaagattaaggatatgaagacttgtatcaaaatgttttgaagtgattttaaatttcttgctgtttctaacctgctttcgatctttaacccatactacttcaaatgggggagttcccgaaatttcacattggagaatcacatcagaacctttaagagctcctactggagaaggcttctgggtgaaaacaggaggtgctttcactgtcaacgctgtgctgcagctggcgtcaccaacaccattatgagcctcacaaatgtagtccccgctgtcttcagcactagcttcattgatcgtaagcaatgccacagaattaatgaatgacatgttgtatttccaactttcatgaagttcgctgtcatttcggaaccatgaaactttgatttctggggagccacttattttacattccagttgaatggattctccctgctttgcaacttttgaagcttctaatttcttaacaaactttggaggttcttttacactgagctgagctgagcacatgtctttgccaacatcattggttgcttggcaagtatattgaccagagtctcctttgcctactttaagaattctcaaatgaggagtgtttcccacacatgtgattgtatagtttcctccaggacggatctccttgttatcttttgaccaagtgattcgcatcggttgagcaccagtaacatgacactcaaaatcagcactttctccagcaataacatctatagatacaggcttgatgtcaaagaagggagatttcttgggttctcttgctgtgagtctagcactagaagatgctgttccaagtgggttggaagctgagcaagagtactggccagagtgactcaagtcagtttgcaaaatttttaaagttgccacattatctacaaatgaagtctgtagattttcatcgtctcttaaaagtactccatctctataccagcacacttggatgggtgcagagccatttaatcgacaagtgagtgtaacaggtaaccccacagtttgttcaatgtcctttaattgtcttgcaaaagaaggtgggagttggcgctcttgaattctgaacacagtcttagaagaagcagttcctatactattttctgctttgcatgtgtactctccactgtcattgatgttcactttattaaaaacaagtgtggccacattgtttgtaaagtaggtcctgtattcaggagttggccgtaatttggtatctcctttgtaccaagacactgtaatttctggtgtcccagcaacttggcattgtaaagaaaccgaatctccaactgctgcctccagaggttccagttccgtaacaaaataaggcggttctaatgtagataccagagctccacaaacatcccttcctgcctcattttcaatctcgcaggaatactgccctgcatctctttttgtgctattcagaatttccaggatacaagttttctctgttgtgactatgttacatttttcagaggtagttatgttaaaaccatcctttttccaagtgacagaaattggaagtgttccagtgtaggtgctctccagaattatggacttccctggttctacagaatgatcacttaatctcttcaaaaatgcagctggttctttcacaaagagacgggtagtgcaagatgcttggccagcgttgttagaaaccacacaggtgtattccccactctgagatatgtcaatattaaataattccagttctgccacagtgtcttcaaaatagatgttgcaccggtctcctttcactagttctctggcacctctgaaccagttgactttgaatggaggggttcctctaataacgcttgtgaaggttacatttttgcctggtagtacttccaaaggttcaggttctttcacaaaagagggtggttcttgtacagttagcactgcacgacattcatcagacccagcgacattagcagccacgcatgtgtaattgcccatatctgaggaatccagagaattcaactgcaatgtgcagacattatctgaaaatgtggtttggtactttgctccactgacaatcttggttttctcatgaaaccaggcaactgaaataggtgatgatccagctactttgcattccaagatgcaagaagcacctaacaccccaccagtatttttcagtcttcgtgtgaaagagggaggaactgctcggtctgaaacatcaaccacagctgtgcagctgcttttcccaacattattttgaacctggaaagtgtatgtgcctgcatcttgcctttcaactgagagaatccttaaggaagagattttgttgtagaagctaaatttgtgtttttggctgctggtcaacagctttccatccttgtaccattcaacagagagttccggagtgccagccaccttacactccagagtgcacgtttctcctacagtcaccgtcatcggtcctgccttctcaacaatgactgcgggctctaagaccatcagtgtggccatgttctccctcattccaccatcattcttgatttggcagatatactttccagcattagctggctctgcttttgcaaactgtagagttgcaacattttccacaaatgtaatcctgatgttttcactttctctaatcacttcttccttctctttaagccactggacaaaaataggctgggcgccttctatggatgcttgtaattcagcaggctctccggctacaacagtgaggctgttcagtttggagacaaatcttggtggttctttcaattttacagtacaaacacaagtatcacttcccacttcattctgtgctttgcagtggtattcaccgatgtctgaagtgtccacattgagaatgtgaatacttgtgtggaagtttttggatgcaatcttgtatttcttgctgcttctgagttgccgcttgtctttgtaccataccacctcaaacggtggtgttcccgaaagttcacattcaagactgacttcagcatttttaagggtttctactataggagggaagctgctaaaaacaggtggctcttttactataaccttggtactgcagcttgtgctgccagcgggattctgagcctcacaaatgaaatctccactgtcctcagtactgagattgttcatctgtatgacggccactgagtcaatgaaagtcattctgtacttatcactggctggaagttcatgttcatttcggaaccacacaactctgatttctggggatccagctatcttgcattcaagtcgtgaagagtcacctgctttcacaattttggaggcttctaatttctttacaaactttggtggttctgtcacaagcaacatcgtagtacaagagtcgctaccaacatcattggtaacatggcaagtatactgtccagtcttagaagcatccactgagtagagatttaagaagctagtcgacccttccaagccaatgaaacatttaggacctgagacaagttccacatcatccttaaaccattttattttaaatggtggtgttccttttagtattgccttaaattccactgtagaatcaggtatggcttgctgtcgcccaggtttcactaggaagcttggtggttctttcacagttaagatgccactgcatgcatcatctcctgctacatttgacactttgcatgtgtaatttgcagtatcttctaattccagattattaacttccagagacacagatctctcatggcacacaagtctgtattttgcacttgtagatatttcttttccatccttaaaccactgagcactaatgggaagtgaaccagacaccttgcactccatatgaatagaagagcccagaactttatccattttggttaattttttggtgaatgatggaggaatattttgatctagcactcttaagtaggcatcacagctactgcttccgaagtcattttccaccttgaaagtgtactgaccgctgtcctgcttcattactgactgaattctaaaactggccacgttattttcaaaactcattgaaaagtatctactgggaactatttgtttcccgtctttaagccatttcactttgagttctggtgttccagccacaacacattccaaggtcatgggatctttctccgtaacatcaactgatttagctttctctacgatttgagctggttcttgtactaaaaggaaagcataacacctctcaactcctgactcattcttggcttgacaggtatatctcccactgtgtccattatccacacttctgatttgaagtgtggccacactgtccacaaatgaaatatagacattatcatcttcatcaagaatctgatcatcctttagccaggttatagaaataggaggagaacctgccacggtactctgaaaggtggcagaacttttcaaaacagtagtggtattttctatcttcttaatgaatgatggtggttctttcagggcaactctagtactgcatgagcagctgccgccttcattggatacaatgcactggtattccccagtgtctgaagggtcacacttggttatatggaggttaaacacagacactctgtcggtcaatgtgtattttttgctgcttcgaatttccctgttattcttcagccaagtgacttcaaacggaggtgttcccgtaacttcacactccagctccacgtcactatattttactacctccacaggcttcagctctctgataaaggtggggggttctttcactttgagttcaatgctgcagctcgccgtgcctgcgtcatttcgagcttcacacacataagtcccactattttctaccctggcaccagaaatctggaaagtggctaaaccatcaatgaaggaaatgccatgtttctgaatggctgttatttcattcccgtctagataccaagacactcggattttaggagtgcctgttatttggcattcaaatgttgttgactgtccattcctcagcactaagactggactgggcttcttaatgaattgaggaggttcttttacaaagagagtggctttgctggttgctgtgccaacatcattgcttagttggcaaatgtaggttccagaatcggtagctttggctgcaaagagctctagactggtagaggtgtcatccttccaaactgagcgggctgctcctgagtgtaactctttgttatctttaaaccactttattgtcatgggtgcagtgccacccacaagagcctttaactgtacccttgtgttgggattgacatcttgtgactgtggcttttccacaaagtaagggggttctttgactgtcagatgcccactgcattggttgtgccctgccttatttgtggcagaacaagtgtatgtcccactgtctgtaccttccagctggctgatttccaagaaggcagtattgtcatgaaaagagaatttgtacttttcactagctgatatttcttggtcatctttgaaccactggatgcttatgggatgtgacccagccactatacattctaaatcaatgaaagaacctttaatgctgtccattttcttcagctttttggtgaatgaaggaggtatgataagatctaatacattaattctagccttgcagctgctcctcccaacatcattttggacctcgaaagtatattctccactatctttcttttctgtagaaataatcttcagtattgagactgtatcagtgacactgattttatattttgagcccagggtcagttcttggccatctttaaaccatttggctgtaatctccttagtccctgaaaatttaacctgcaaagtggctgggtctccttgggtgacatctatagacacagcttcctcggtgattgttgcaggttcttttactgagagtaatgcagaacatctttgtattcctgcatcatttttggcctgacagacatatttcccatcatgcttgacttcaatgccactgaggtacaaactggccacattgttctcaaaggtcattcttatattatcgtcttcagtgatttcatcgctgtcttttagccaagtcaccgtaattggcaaggagcccttcagagtggcctggaaggcagctgtgcctccccggagggagctggtactctcgatcttctttatgaaggatgggggttctcttaaagtcaccctggcactgcagatgctgctgcccacctcattggtcacccgacactggtattcgccagcatctgcagctacaaacttgaggatctgcaggctaaccagatgatcctgaatgaaagtcttatactttctaccacttcgcaggattgtgttatctttgaaccaagtgatctcaaagggaggagtgcctgccacctcagccagcaacatgacatcgtactcctttaagacttcaattggcttaaattccttggtaaaataaggtgactctttgactattacaatgctactgcagtggtcactgccagcctcattttgggcctcacacatatattcaccactgtcttcgatgccaacatctgtcagtcttagaactgcagtagactccacaaaagacattctgtgtttgctgctctccttaatttctctatcatttgcaaaccatgttattttaattggaggggtaccagttactttgcaggctagctgggtggcatctcccttctttaacagctgtgatggctctaacttttcaacaaatgtggcaggttcttttacaaacaagtttgcactgcattccacccctccagcgacattgctgactttacatgtgtacgtgcccgaatcagaggtttttactaaatagagttccagggaactctctaaagcttctttggtaatatagcagcttccaccagaaaccagctctttgttgcccttaaaccatctgattgtgagaggagtagatccttggaaagtgctcttcaggcagactgctgagccaggcagaacatcctttgagccgggtttagttacaaaactgggtggttcttgcacaatcagggctccactgctgtctttgcttcccacggaatttgtggctcgacaagtgaaattccctgcatcattcatgtctactctgatgatctccaaagaggctgtgccttccacaaatgctatcctgtatctgtcagaagcagctatttctttgccatccttaaaccaggacaccctcatggggagggagcctgcaattttgcagtccagtctgcaggtaccattaacaacactatccacgttgcgcaagggtttggtaaaaaatggagcaatgtctcgatctaatacagtgaatgtagtctcacaggagctgctgcccacttcattggaaatctcaaatgtgtattggccactgtcgtgcagctcagctgaataaaatttgagctgggcaacattgtttttaaaacttattcggtattttttactggcgaccaagggtctcccatctttgtaccatttgggcttcagttctggcgtgcctgccactgtgtactccagtgtggcgggatctcctgctgtcacctggatcagttctgctcgctcaatgattttggcaggttctttaactattaattccccaacagatgtttggcttccagcttcattttcagccaggcacgtgtatttgcctccaaaactaatctgaacatcagggattatcaagactgcaacaccattggaaaagctcattttgatttttccgtcttctctgatgacctcttgacctttcatccatgtgacagaaatgggctctgaccctctcacagcagcttgcagggtaacggtttgtcctcctagtgcaatcaaatcatctactttctttacaaaggttggaggttctttgagtaagtgggttgccatgcagccacacttgccgacttcattagcaacaacacattcatattcaccaacatctgcactattaaacgaaaagatctccagacacacaagagacttctgagaaaacaatctgtattttttactacttcgaatttgtttcttgtctttgaaccagctaatttcaaatggtccagtgcctgagacttcacactgaagtagagcatttgttcctctcactatgtctgcaggctcaagagttttgatgaaagaaggaggttctttgataactatttcagtactgcagctatcactgccgacgtcattcactgcttcacatgagtaactcccactgtcttcaacttttacatccgtaatatcaagtatagcctcagaattgacaaaatacattcggactgtgttactttcactgagttctttgttatttttaaaccaagtaacctggatcacaggtgagcctttcagcttgcaatggaggcgtgctgattcacctgggagcattaaataagagggatccaccttcttcacgaaggatggtggctctctgacagtgactgtggctgagcaggagctgcttccagcctcatttgaagctgtacagacataggttcctgaatctttcagtttggccaaaggaatctcaagtgttgctattttatcttcaaaacagatcttataatctttccctggggggagtttttgcccatctttgctccacgtaactgtgacttttctgtcttcatctacttggcactcaaggtggaccttcttattgatagcggactgcacaggctctaattctttaatgaaatgtggcttatcaatgatgatcaactctgcttggcagatgtctgctccaaacttgttggaagccttacaagaataaactcctctatcttgaatggtaaggtttgagagttctaaaatgtgtttgttttctgcgtcggaaatcctccagttaggtgaaggtgagagtgcagcaccatctttctgccaaatggtttctatcacaggagtccctgtcactgtgcagatgaacttggctgccttacccacaaaagttgtaagggacttaggtctggagagaaaggttggtggatatgcctctgtcacagttagtgtggctgtacagctgacactgccatactcattggaagctttgcatgtatactcgccgcagtcaaccacctgggttctcaggatttcaaggctggagatatactttgaagatcgaatagaacacttgtcactctcataaatttctcggccagctttaaaccactggaaccggacattgggagcactttggatctcacaggtgaatttggctaggtggcccagtgctacttccaggggttcgattttcctcttgatcactggggcagctctttttactacagtgagtttggctgaagttgctgtttttccgctgtcattcaaggcctcacagacatactctccttgatggtcttcggtatttactttgtcgatgactagcgtatatgtattttgatcttgtaaacacttgaacttttcatctgaaggcaccagtttattctcaaaataccaattcacctctttagcatttgttatggatgttgtgaggtgtacaatatcaccttcctcagaaacagtgtccactaaaggtgtatgtatcatggggccatcctctttgattaagccaccctcagcttcctgtatctttactgtagcaacctcctcagtaccactttcagaggaagactcctctttttcctctgatggtttcagactctcatcttgtttttcgtcagagacaacagctgaagcaacccctttagtgacaggtgtggcatccaaatatttaaccctactttgcacgttaaaataactgacctcttcagttgagatcagatatttagattcaacttctggttcagtaatgggttcaaccttctgtgaacctgaaaaagaatccatttcttcttgcaaacttgttttggctccttgctgaattctaggaccctcagctgttaggatgtctatttcctcatatataatagcacacaaagcatccctaagttccattttcaggttagccatttgaggatcaacatcttcaataatgatggttacttcttctgttacagactttgccgaagtaacaaggtacatgcacatgatgtgtctgggctcttgggtgatgtttacagcctcgacctccaccttttcaatatttcttagccactcagagaaaagacctggctgctcgctggccacggctgcttgcaaagcccggcagatttgaattttcaggtttaatctctgctcttctggaataccagaaagcaagctttccttagaaagaaggtcccttccctgtacctcctgcactttctttattgccacgggctctcttttagactcaatgatttggtctgggggcatcaccacgttgtcagaatgctcttctttgagcagtacctgcttttcttcaagtgctagtggaaatcttaaggacttgccttcctcaattctgaccgcagaatcttgccctgcattttccagtggatttgcactttctatcaaaattttacctccttctgtgcatgagtgttctgaagggactaggggctcatagtttacctgagagatcatgacatcaggactctggagactctccacgtgtccctcagctaagctctgactcaagatgagcgcactttgtgcctcttgcttttgaagagtcactctttgctctctgttggtgtcagatactgtcttttcttttggtgaaagtacttcctcagccacagaggttagataagaatgcattggaggttctattgaagactgtggataattcccttcaggttcagctaataaagttttcagaggctcaactgttaatgaattaatttgttctatggacatggcacttgggaagattttctcggtatctgatagaactgcctgtgtctcaggctcttcaggcattagaataccttctttggagaaggttttctgggactgtacaatctgcagctgtaggttgggagatggttccttgagaggctgaaagtgaatactgccattgatgcaaagaaattccctggtgctttcaggagtgagcttgtcttgctccaaaatggattgcaattcctgagctcccaaaggaagctgactgctcaattcattggctttagcaatatgctcataagatagttgctggttttcttctgtaattaaagcagctttcaaaatggtgtcttttacaaacgttgcaatttcctgctctgagtcaagtgcttcaactgcgggaccctttaagggtgtctgtggaaaatcctcaggagcctctggtgtggactttgctttgcagggggtatcagtcatgtctgtgtcttccagaagcacaagcagctctgctgcacaggtggactcacccaacatattctctgctttacagatatagaggccactgtcttccctctgagggtcattgacaatgaaagttccagagccattagggttatgaatgatagtgtaataaacactggtgcaaagctgcttgttttctttgaaccatgtaacagtaggggcaggctctccaaccactgtgtactcaaagatggcaggaagcccttgagcacagcgaattggttttaactccttaaggaagtgaggaggacaaggacctcccagcttttccagagattttgccactgctgattctgtttcagtgtctttgtgaccctctcctttggaattaatttttagataggcactacatattgtctttccatagtcattactggccatacatgtatactctccctcatcctccaatttggtgaacagaatgatcaggctatgatcatcaccgtcaaaaacaaatttgtagtcagcagaaggggttaatagcactccattaaagaaccactgaattttaggtttggggatgccaatgacagttacagacagtgtagccacatcccccatgcttatatcagcatttgacacttctttgatgaaaattgggccagtgccttccttttcggaatcaaatttagttgggtaaactggagattcagacaaaagttcaagtgtttcatttattttagataattgaagttcggcgctatgaagtccttcttcctcggcagacagaaaagaactagaaaactctttcatttccatctcaatctcttgttcaatcctctcatgcaaaattgattcaggagcttccagactcaggttggctgtgcttgatacttggcctacagcattactagcaacaaacgtgtaagttccttcatcttctggataagcttcggcaatttccagttgataagtgtcttcaaattgagtcattctaaagaaccgagatggcttgattttcttgtctttgctgtaccacgacacttttagatctgttccagaaacccggcattgaaaacgggctggctgcccttcagaagtgacagtgtcctgaagcggggtgatgatggcaggtggataaacaggcatttcctgatcaggagacacaacttctggaacttccactgagagtgaagctgatgttgtggcaacaccatagtcattcttggcttcacaggtatagactgccgcatcctctgggaaggcttcaattagcaaaagcgtgtattcttgcccatcatgaagaaatttgcacttgaagccagtggaaagcagctgctcttccttgtaccaggaaattttgggctgtggtcttccggatatcacggcacagaagcgggcaggcttgccagactgcacagtgacaggctggagctcctgcagaacttggggcggttcaggagcattgacatagagagtgacagaactcctgttccttcctgccacaaaggtgtattctcctgcatcgctctgtctggtctcagagataaacattcggtggattcttctttccactacatatttgtgtcgttcttgaacttggaaattgatttcaatgccatctttataccagtgggcatcaacatcgtcttcattgacctcaaattcaacaacagcacgctgtttctcaatgacctgaacctcctttttaatacttcggatgcgaacatctctgccttctacaaagagttttgcagttgacacgttgcctcctgccaccactgtgtacttcccagcatcagacatccgggtggatgggatcagaaggcggtggacatatttctccttctgaatctttattctgtctgtgatctgcagttcctggtcatctttcatccactgtacagtgatgtcaggttcagaaacttcacattcaaacatggctcgcttcttctccagtaccttaatgtccttaatgtgtttcctaaattctatatgacgagcttccacataaagtgtggctgttgatgttgcttttccagccacaaaggtgtagtcagcagcatccccaaagtgaacattcctgatgttcagtgagtgtgtgagctttttggttctcatctggcacttgtcagttgatttgatttccacaccattctttaaccatttgtaagagatgccttcatagttcactgtcacctcaaaagtaatagtgtctttttcttcagcgttgatgtctttcagcatggaagtaatcatgattggggtgactgtcagggtggcactgacttggtcattgccacagacaaatgtgtattctgccgagtcctctgtgctggtgttcatgatgatcagctgatggagttttccctgcacaactatcttgaacttttcactcatctcaatttccacaccattcttcagccacatggaagggacattgaagtgggacacctcacactcaaaagaggcagttttggtctcaggcacctcgatatttttcatggtttttgtaatatgtaatgtctccacaaacagttttgctttgcattccaattgcccgaccacagctgtgtattccccagcatctgagggggagatgttctgcagcatcagcttgtggactttcctttctgagaccagtctgtgtttgtcacttggcttaatttccacactcttatggaaccattttactggaacagtgtcatgggaaacactaacttcaaaggcaacagtggcattttccaaggctgtcacatcctttggctttttaatgatcttgacagtctccacgtgcagtctggcactggctccaagccttccaagcctgaagccataaacagactcatccacgatggcacagtttttaatcctcagagagtaaattgttcctttgacagagatagcatacttttcattggattccagcacaactccatttttgatccactggacacctttgacattagggtgtgtaagctcgacagtgaaaacagcatcctgtgtttctgtcactgtgaggttcttcagagtcttcttaattttgacagcttcaactttgagtttggcagatgttttggaggtggccaccttgtaggtatattctccaatgtcatctaatttggtggcagcaatgataagtctccttttgtggccatcagactcacttctgatgttgttagtcagtggtaggtgtttgccatccctcaaccattcgcctttggaatctgggttggcaacttcacattcaaacacagcttcctgggattcagctacggtctgatctgtgagtggcttggagatggccccacctgccacagtaagttttccagatgtcatattttctcccgcgtaaaatgtgtattttccttcatcatctttcatcatatttagaactgtcaatttatatatttttccatgtgcttcaattttatatttagaactgggcttgatttccttgtccttaaaattccacaggacatcaattccagagtgggacagctcaacctcaaacaccacattttgagtttctgtacaggtaaggtcacgaagacctctgataattttaattttttctacagagagattacagttggtttcaactctgccaactatcagcttgtaaggtccttcgtctgaagcatgagttcggttaatgactagtcgctgtttagtacctttcacaatggcctgtacacggtcatcaggcttgatttgttcatcatttaagtaccacttaacagaagtcacatcagggactgacaccttacattcaagcacagccttggtgccttcaatcacattaacatcttttagaggtgttatcacgtccacactatagacagagacacgcccactggtggagaggccaagggctggaatggtgaaagagtaatttccagcatcttccttagtcatgtcttcaatgagcagcatatgagattgtttgtctatcacaatgtgaaccctgtcactgggctgcacttcttggccgtctttcatccagacgccttccacactttccaaggagactttaacttcaagctgaacaatgtcaccctcacagactttttggtcactaagtccttgtaggatagcaatggggcggggtttcatctttaatttacaggttgtctttttcccgtcgatgacaaagctgtattctccctggtcctccttggttacatccttgaccgtgaggttctgacgtccacgacgagatgtaattgtatatttgccattggatttaagctccacatcattatgataccattttccttctatattttctggggatacaatgcactctaattctcctgaatatgattctggaacttctatgtcctgaagttctttcacaaactcaacaactgcaccttcaacaataagtttagcagtcgttttgacattttcatcttccacaagtacacagctgtaatcttcagcatcagacgtatcaatggtcagtatggagaggaagtgaacctttctgtcagagtgcatcctgtatttatctccctcatgaacctccataccatctttataccatttcactttgacaaatggttctgaagtttcacattcaaaggttgccatagtgtctttttccttagcaacaacatcttgtaattcctgtgtgaaagtgatcaattgcttggcttggacaagtaagaatgcgtgactggaggtttctccagctatgttgatggcttttaccatgatgctggcagagtcctcagcagtcacatctcttatgaccaattcacaaacattgtcttcgggccagtaccagtagatccggtcagaccgttcaattttgacaccatttttgtaccattcacattcggggtctggtttccccacgactctgacccggaagtgtgcatcagatccttggcccactgtttggctctggattctttcgaagatttttggagcctccatactaggacttagttcaatcttgtcaggtttaaaagttggaatcgtgattttgccttcttcggcaagagctttcttttcctcttcagttaactctttggtccagtggagaagttcatcttttgtcttcctgaggagttcctcataggattcatccttctttcgagacttgagctccacagcggtaatggcttcataatagccctcttctgttctgcgcttgaatttactgcgcagctcttccgactcttcaggcactttttcatgggtaattctttcagcccttttcaacttcacaacttctttggtttcagtggtgtcaacaggtctatccactttttgtacttcaaactgaagctttcctggttcatgtacgtgaaactcaggccttggttcaggagctctcctaaggacagacctaaaatcttccctctgttgaatctcaagcttcactttatgctctatcacaccttcaggattttccgcggtgaccttcacttcacctgtgtcatatgatttgcagtccacgatgtccaggtaatggataccatcatagcgaactctgaaccttttgcttttgcggatgagctgtccattgaggtaccagttgactttgggctgagggtagcctgttaccctgcagcggaaccttgcagtctccccttcaagtactctaactggctctgggtacaagacaatgtctggcttttgcttttctttctgatctgttgttacacctgtaagtgcaccttcatgagccattctctctaattcttcaattctctgtaagcctttcctcccctcaggcaattgggattcttccacaagacttttctcatctttaacaataagggtagcagatgtgtgatctgttccatatttgttagtggctctgcaagtaatgataccactgtctctagaatatgcaacgccataatcaaggctgcagtacccaaattcattgatcatacggagcctgttggctgcttcaagtggctttccatcatggagccactccaccaccatcgttgggtcaccaatgggtgttagcctgcattcaaagtgggcaggcccaaagcgcttaagtcttaaggaagtgagttttttcttgaaaaatggtttctgttgtttctctttgtcatagagatcaccttcttcccattgctcttggccatatcgcaaatggaggggctccagttctggggctgcaatctcctttgctctatatgtcccccgtgggatgattaactttctctctggctcaggctctgcaaactcaacttcaacatttactttgcatcttgtagtgtctctgccagctttattaatagcagtcgcagtataccaggcagaatcttggctgacagtggaatcgattttaagggcagcttctcccttggttccttcaattctgattttgggatatttatgaggcacaatgatgtcactgtttttcaaccatacaatgtcagggttggggttacccgtagctctgactttcatttcaagtcgggaaccttcctttatattgacatttttcagtttttctacaaacatcggttttacctgatgttccacagcttccacagttaaaatcactgaaattgaagatctgcctgccctgttttgggcaaccacagtccattccccagaatcactgggtgtggcagggacaataattagtgattgagtaccatcttctttaatgactactttatgggtatagtcattgacaatttgctggccatcatgaaaccagaacgtctctggcataggtctaccaacaacctttaagtcaaatctggcagtttgcccttctaaacatttgaaagaaacaggttttaacacaaagactggtttatatagtctctcaagttgtgactcatctgtctcctccagcctacgtccaggggacattcttgcaggggacatccgtgcaggagacatccttgcaggtgacatccgtgcaggagacatgcgtataggagacctgctcactgaacgtggagagagagatctgattctgctcactggctctagtgtgggaatgtaagtcggagctccaagtggtgcagcaggctccacatacaatttccctgagcaaattgcatttcctttaatattgctggcaaatgcagtgtagattccttcatcttctggaagaacaacaggtatacgcagactagctctgccatcttgtagaaagtccatttggtatctttctccatgtttgatgcgcttgccatctttgtaccaagcaatctttggtaatggatatccagacatcttgcaatgaaaagtgacacccatcccctcaagaattctataattcttgattcttgaatcaaatcctgattcaacagcttcagattcagaaatgtcaactgccatcttttcttctccatcttcttcaagaagttcttctaatgtagtctttattattctatattcaatttctttaataagtctctcttcaaaggaagaaatatggaattcctgatcttctacataagttctgaccactacagtatctttggccattttcttcctaattaaggcttgttctttttcatactctttttcatactcagagtatacaaatccaggtgctgtttctccaactttaggttcttgaacaaatgcagtcacttgtgtctgataaagcatttcttgctgggacttcatcagtaactcataatcagcttcttcaagcaaggaagcagatgcagaagtttctccatgcttattgcgaacaacaatagtgtattctccagcatcatcagcaaaagtcatagaaatcaccagcttgcattcaccggtttgtttgttgtaactcactttgtatctgtatccagtggttagaggaacaccagattttttccagtatacatggggctttgggttgccgccaacttggcatccaaacaccacgctcccaccttccaccagtttctggaccactggttttgtaataaagtaaggcgcggcaggttctccaggccctgcttgttcctctgtgaggctagtatcagtcataaccacatctcttgactcaacaaagcgtttctcttctgtagtaaatttctcagtcacggctgtggtttccttttcaaattcttctgacacctgcacagccagatagcaggatgtgctgacggttccagcctcatttacagcactgcaagtaaatcgcccgctgtcttccgcaaatgcttcgcgaatcataagacgagcaattccactctggaaggttatctggaagtcaatggaactttcgatttggtagtcttccctgtaccatgtcactgtcggggatgggtatccagagatgtggcactccaaggtgacagattcaccttctatgacagtcacattttttaagcccgagaccaaagttggtggagtaacaggaatttcaacaggtgctggtactcttgctgtttctgttaccttggcttcgcgtccgtgcagtacttcaaagcgctcttcacggacggtggtgccagtgatgctcacccctacttcctttttcacctcaacgccagcttcactcttgtaagtatctggtgtgtcagcgaaggggaactgtggcaagggtgtgggctctgcccttactctagtctcactgggcttcacagtaggagccttcaccgatttggtgatcttctgagcagaagatgtggctgacaactctttttgtaatgtggcaatagcactaccggctattgatgcctcatatccatgttctgtcttaggaacagaaatttttgaaacagtaaagtgagggctagctgtgcgggggcgtttatccacatggactaatctttccgttgttagatctgtagttttcttgatctgtgatgatatgtgcattcccttttgatcagtagttttgatatgagtctcagaaggagcctggattactctaggcttgactgctttagggacaacgtggggttctgaggctggacgttggggaggctcagctacctttgcggcggaaatgcgttccttatatccgtactccaaagtggtctgctgagcataggattcttcaagatgcccaggctctctgggctctctgactcgggcctggtctactgcagcaacaactgttgctacagcttcagccttttttccaacgtccacctttccatgggtaacttggatttgttcttgtctagtagccatagtttctctagttctcagtattgtttcttgttctttggctttagcagtagcaactgctattgtagacaaggcagttttctcggcttcctttctcatcttctcctgagttatttgcacttgttctcttttggtagtaatgccttctctacctcttgatactaaatcttgttctttgactttgggtgtggcaactatgactttaggtacaactgttttcctagtttccttcattatcttttcataacttaggtgcatttgatcttgttgtgtggtagtttcttcttgagctcccgggactgtttctagttttgtggactttgcagtggcaactaccaccatggatgcagcagttatctcagtttcctgtcttattgcttcttgagttacttgtttctgtttcttagtaatttcttcagaaattctagtttcttgttctttggctttagctgcggaaattactacctttggtacaaatgttttttcagtttcttttcttatctgctcatgagttacgtgcatctgctcttgctttgtggtaattacttctttggttcttgattttaattcttgttccttggctttatcggcggccactactaccttagttacagcagtcttctccgcttcctttcttacctgctgttcttgagcaggttggatgtgcacagcagtcgtggttgtcctctgagcagtctgctctacagcgctgatcactggttctctcactctggccatatcaacggcagcaacaacagtcgcaacagctgcacttttgtcagcatcttgtttcacctctttagcaccagtggcaacagcctctgctgcgtagctagcactggccgacacactggcggcagcacccgcagcaccactgatggtcacttgctcctggacaccgtatctcccttcccatctctcttctgtcctgatctgagtagaggttgtcagcgttgtctctctcatctcagcctcagatgaggaggccacgtagccctcttgcttccaagggggaggcacttcaggacctgtggccacggtggatgcctgagtcttacgcatgagcaatggagacctaacagacctgatgggggatgtggagattcttgctgctggagacacggacctgaccggagatggggtcggtgcccgcacgtgtctgaccggggaaggggagtgtcttatgggcgatggggactgctgccgagccagctgtgctttggcagcaatagacggtggtgttggggatcttgactttggcttcggaggaatcctgggaggtgttttatgtggcagctgttgcccagcggcaccatctatgaccatctcaactgttgcaattgatctggcatcaaagtgggcttcaatcttcttttcaattcgggtttgtcttgattctgagatctgagcagtcgaaacaattgtctttgtctttttagcaggtacttcttcttcaccttgaaccagtaattcagcagtcgaagtagctcttccaacgctattggtggcatttactgaataggtccctgagtcctcagggtatgcttctgcaatcagtaagctgtagaggtcgccttcttgtgaaatttggaaatcaagggagctctggatttcggctccatcccggtagaacttcaccacaggtgtagggattccagtcactctcacttggagtctcacttggcttccttgtctcacggtcatgctctgcagtcgttgaacgaagttgggtggtgctgtctcagctttcacgagaagctcagcagtactagtcgcttgtccagatccattggtggctttcagggaatatcgtccactgttggctttagtcacggcggggatcgtcagtttagcgcggccatcgctaaaggagatctgcacgccgggcagagtggaagtggaaatcacctggccatccctaaaccagctcacctcaggaactggaaaaccactaatgtgagcctcaaaggttgcggtactaccctccagtaccacaacgctttgtaacggctgcgtaaacgtcggtgcttgagttgtcatctttctaggcactctgatttctcaagagtgcctaaaaagggtgggactaagcccaaggttgcttctgaaacgacgtcctatggagagttggtttttctgaccatctccgacatgaatcggtgagcctctaatcctaaaaacaaaactacacagtcaagactgtgtagttttgcttttctatgcaatccctacacccgaggcgaggctgggaatgcacgactgctc

SEQ ID NO: 10300 - RNA, 23198 nt, Homo sapiens
  source 1..23198: mol_type = other RNA
ccaaaactgcagttacttttgccaacactgtttttcacttcaaagctatataatcctttgtcactcatttcggcacaggggattttaagggaagccactttattgatgaatgtaatgtgatgtttgctgtctgcagacaattctcttccatctttgaaccacttggctgagagttctggtgttccagtcactacacactctaatgcaaaaggatttccagtagtgacagtcatgggttcgggcttctctatgattcttgctggttctagtacagtcaagactgcagagcattctctcattccagcatcgtttttgatttggcatatatattttccagaattagatgcttctggactccccagctggagggttgcaatgttatcaatgaatgaaatcctggtattttcactctctctgatgacttcacctctatctttcagccagacaacagaaattggctggaagccctccactatggcccgtaactcaacagcatccccaataagggttgaggtgtcacttagctttttcacgaatcgtggaggttctttgaacttgacagagcaagaacacgtgtcacttcccacctcattagtagctttgcagtgatattccccgacatcggaggcttcaagattaaggatatgaagacttgtatcaaaatgttttgaagtgattttaaatttcttgctgtttctaacctgctttcgatctttaacccatactacttcaaatgggggagttcccgaaatttcacattggagaatcacatcagaacctttaagagctcctactggagaaggcttctgggtgaaaacaggaggtgctttcactgtcaacgctgtgctgcagctggcgtcaccaacaccattatgagcctcacaaatgtagtccccgctgtcttcagcactagcttcattgatcgtaagcaatgccacagaattaatgaatgacatgttgtatttccaactttcatgaagttcgctgtcatttcggaaccatgaaactttgatttctggggagccacttattttacattccagttgaatggattctccctgctttgcaacttttgaagcttctaatttcttaacaaactttggaggttcttttacactgagctgagctgagcacatgtctttgccaacatcattggttgcttggcaagtatattgaccagagtctcctttgcctactttaagaattctcaaatgaggagtgtttcccacacatgtgattgtatagtttcctccaggacggatctccttgttatcttttgaccaagtgattcgcatcggttgagcaccagtaacatgacactcaaaatcagcactttctccagcaataacatctatagatacaggcttgatgtcaaagaagggagatttcttgggttctcttgctgtgagtctagcactagaagatgctgttccaagtgggttggaagctgagcaagagtactggccagagtgactcaagtcagtttgcaaaatttttaaagttgccacattatctacaaatgaagtctgtagattttcatcgtctcttaaaagtactccatctctataccagcacacttggatgggtgcagagccatttaatcgacaagtgagtgtaacaggtaaccccacagtttgttcaatgtcctttaattgtcttgcaaaagaaggtgggagttggcgctcttgaattctgaacacagtcttagaagaagcagttcctatactattttctgctttgcatgtgtactctccactgtcattgatgttcactttattaaaaacaagtgtggccacattgtttgtaaagtaggtcctgtattcaggagttggccgtaatttggtatctcctttgtaccaagacactgtaatttctggtgtcccagcaacttggcattgtaaagaaaccgaatctccaactgctgcctccagaggttccagttccgtaacaaaataaggcggttctaatgtagataccagagctccacaaacatcccttcctgcctcattttcaatctcgcaggaatactgccctgcatctctttttgtgctattcagaatttccaggatacaagttttctctgttgtgactatgttacatttttcagaggtagttatgttaaaaccatcctttttccaagtgacagaaattggaagtgttccagtgtaggtgctctccagaattatggacttccctggttctacagaatgatcacttaatctcttcaaaaatgcagctggttctttcacaaagagacgggtagtgcaagatgcttggccagcgttgttagaaaccacacaggtgtattccccactctgagatatgtcaatattaaataattccagttctgccacagtgtcttcaaaatagatgttgcaccggtctcctttcactagttctctggcacctctgaaccagttgactttgaatggaggggttcctctaataacgcttgtgaaggttacatttttgcctggtagtacttccaaaggttcaggttctttcacaaaagagggtggttcttgtacagttagcactgcacgacattcatcagacccagcgacattagcagccacgcatgtgtaattgcccatatctgaggaatccagagaattcaactgcaatgtgcagacattatctgaaaatgtggtttggtactttgctccactgacaatcttggttttctcatgaaaccaggcaactgaaataggtgatgatccagctactttgcattccaagatgcaagaagcacctaacaccccaccagtatttttcagtcttcgtgtgaaagagggaggaactgctcggtctgaaacatcaaccacagctgtgcagctgcttttcccaacattattttgaacctggaaagtgtatgtgcctgcatcttgcctttcaactgagagaatccttaaggaagagattttgttgtagaagctaaatttgtgtttttggctgctggtcaacagctttccatccttgtaccattcaacagagagttccggagtgccagccaccttacactccagagtgcacgtttctcctacagtcaccgtcatcggtcctgccttctcaacaatgactgcgggctctaagaccatcagtgtggccatgttctccctcattccaccatcattcttgatttggcagatatactttccagcattagctggctctgcttttgcaaactgtagagttgcaacattttccacaaatgtaatcctgatgttttcactttctctaatcacttcttccttctctttaagccactggacaaaaataggctgggcgccttctatggatgcttgtaattcagcaggctctccggctacaacagtgaggctgttcagtttggagacaaatcttggtggttctttcaattttacagtacaaacacaagtatcacttcccacttcattctgtgctttgcagtggtattcaccgatgtctgaagtgtccacattgagaatgtgaatacttgtgtggaagtttttggatgcaatcttgtatttcttgctgcttctgagttgccgcttgtctttgtaccataccacctcaaacggtggtgttcccgaaagttcacattcaagactgacttcagcatttttaagggtttctactataggagggaagctgctaaaaacaggtggctcttttactataaccttggtactgcagcttgtgctgccagcgggattctgagcctcacaaatgaaatctccactgtcctcagtactgagattgttcatctgtatgacggccactgagtcaatgaaagtcattctgtacttatcactggctggaagttcatgttcatttcggaaccacacaactctgatttctggggatccagctatcttgcattcaagtcgtgaagagtcacctgctttcacaattttggaggcttctaatttctttacaaactttggtggttctgtcacaagcaacatcgtagtacaagagtcgctaccaacatcattggtaacatggcaagtatactgtccagtcttagaagcatccactgagtagagatttaagaagctagtcgacccttccaagccaatgaaacatttaggacctgagacaagttccacatcatccttaaaccattttattttaaatggtggtgttccttttagtattgccttaaattccactgtagaatcaggtatggcttgctgtcgcccaggtttcactaggaagcttggtggttctttcacagttaagatgccactgcatgcatcatctcctgctacatttgacactttgcatgtgtaatttgcagtatcttctaattccagattattaacttccagagacacagatctctcatggcacacaagtctgtattttgcacttgtagatatttcttttccatccttaaaccactgagcactaatgggaagtgaaccagacaccttgcactccatatgaatagaagagcccagaactttatccattttggttaattttttggtgaatgatggaggaatattttgatctagcactcttaagtaggcatcacagctactgcttccgaagtcattttccaccttgaaagtgtactgaccgctgtcctgcttcattactgactgaattctaaaactggccacgttattttcaaaactcattgaaaagtatctactgggaactatttgtttcccgtctttaagccatttcactttgagttctggtgttccagccacaacacattccaaggtcatgggatctttctccgtaacatcaactgatttagctttctctacgatttgagctggttcttgtactaaaaggaaagcataacacctctcaactcctgactcattcttggcttgacaggtatatctcccactgtgtccattatccacacttctgatttgaagtgtggccacactgtccacaaatgaaatatagacattatcatcttcatcaagaatctgatcatcctttagccaggttatagaaataggaggagaacctgccacggtactctgaaaggtggcagaacttttcaaaacagtagtggtattttctatcttcttaatgaatgatggtggttctttcagggcaactctagtactgcatgagcagctgccgccttcattggatacaatgcactggtattccccagtgtctgaagggtcacacttggttatatggaggttaaacacagacactctgtcggtcaatgtgtattttttgctgcttcgaatttccctgttattcttcagccaagtgacttcaaacggaggtgttcccgtaacttcacactccagctccacgtcactatattttactacctccacaggcttcagctctctgataaaggtggggggttctttcactttgagttcaatgctgcagctcgccgtgcctgcgtcatttcgagcttcacacacataagtcccactattttctaccctggcaccagaaatctggaaagtggctaaaccatcaatgaaggaaatgccatgtttctgaatggctgttatttcattcccgtctagataccaagacactcggattttaggagtgcctgttatttggcattcaaatgttgttgactgtccattcctcagcactaagactggactgggcttcttaatgaattgaggaggttcttttacaaagagagtggctttgctggttgctgtgccaacatcattgcttagttggcaaatgtaggttccagaatcggtagctttggctgcaaagagctctagactggtagaggtgtcatccttccaaactgagcgggctgctcctgagtgtaactctttgttatctttaaaccactttattgtcatgggtgcagtgccacccacaagagcctttaactgtacccttgtgttgggattgacatcttgtgactgtggcttttccacaaagtaagggggttctttgactgtcagatgcccactgcattggttgtgccctgccttatttgtggcagaacaagtgtatgtcccactgtctgtaccttccagctggctgatttccaagaaggcagtattgtcatgaaaagagaatttgtacttttcactagctgatatttcttggtcatctttgaaccactggatgcttatgggatgtgacccagccactatacattctaaatcaatgaaagaacctttaatgctgtccattttcttcagctttttggtgaatgaaggaggtatgataagatctaatacattaattctagccttgcagctgctcctcccaacatcattttggacctcgaaagtatattctccactatctttcttttctgtagaaataatcttcagtattgagactgtatcagtgacactgattttatattttgagcccagggtcagttcttggccatctttaaaccatttggctgtaatctccttagtccctgaaaatttaacctgcaaagtggctgggtctccttgggtgacatctatagacacagcttcctcggtgattgttgcaggttcttttactgagagtaatgcagaacatctttgtattcctgcatcatttttggcctgacagacatatttcccatcatgcttgacttcaatgccactgaggtacaaactggccacattgttctcaaaggtcattcttatattatcgtcttcagtgatttcatcgctgtcttttagccaagtcaccgtaattggcaaggagcccttcagagtggcctggaaggcagctgtgcctccccggagggagctggtactctcgatcttctttatgaaggatgggggttctcttaaagtcaccctggcactgcagatgctgctgcccacctcattggtcacccgacactggtattcgccagcatctgcagctacaaacttgaggatctgcaggctaaccagatgatcctgaatgaaagtcttatactttctaccacttcgcaggattgtgttatctttgaaccaagtgatctcaaagggaggagtgcctgccacctcagccagcaacatgacatcgtactcctttaagacttcaattggcttaaattccttggtaaaataaggtgactctttgactattacaatgctactgcagtggtcactgccagcctcattttgggcctcacacatatattcaccactgtcttcgatgccaacatctgtcagtcttagaactgcagtagactccacaaaagacattctgtgtttgctgctctccttaatttctctatcatttgcaaaccatgttattttaattggaggggtaccagttactttgcaggctagctgggtggcatctcccttctttaacagctgtgatggctctaacttttcaacaaatgtggcaggttcttttacaaacaagtttgcactgcattccacccctccagcgacattgctgactttacatgtgtacgtgcccgaatcagaggtttttactaaatagagttccagggaactctctaaagcttctttggtaatatagcagcttccaccagaaaccagctctttgttgcccttaaaccatctgattgtgagaggagtagatccttggaaagtgctcttcaggcagactgctgagccaggcagaacatcctttgagccgggtttagttacaaaactgggtggttcttgcacaatcagggctccactgctgtctttgcttcccacggaatttgtggctcgacaagtgaaattccctgcatcattcatgtctactctgatgatctccaaagaggctgtgccttccacaaatgctatcctgtatctgtcagaagcagctatttctttgccatccttaaaccaggacaccctcatggggagggagcctgcaattttgcagtccagtctgcaggtaccattaacaacactatccacgttgcgcaagggtttggtaaaaaatggagcaatgtctcgatctaatacagtgaatgtagtctcacaggagctgctgcccacttcattggaaatctcaaatgtgtattggccactgtcgtgcagctcagctgaataaaatttgagctgggcaacattgtttttaaaacttattcggtattttttactggcgaccaagggtctcccatctttgtaccatttgggcttcagttctggcgtgcctgccactgtgtactccagtgtggcgggatctcctgctgtcacctggatcagttctgctcgctcaatgattttggcaggttctttaactattaattccccaacagatgtttggcttccagcttcattttcagccaggcacgtgtatttgcctccaaaactaatctgaacatcagggattatcaagactgcaacaccattggaaaagctcattttgatttttccgtcttctctgatgacctcttgacctttcatccatgtgacagaaatgggctctgaccctctcacagcagcttgcagggtaacggtttgtcctcctagtgcaatcaaatcatctactttctttacaaaggttggaggttctttgagtaagtgggttgccatgcagccacacttgccgacttcattagcaacaacacattcatattcaccaacatctgcactattaaacgaaaagatctccagacacacaagagacttctgagaaaacaatctgtattttttactacttcgaatttgtttcttgtctttgaaccagctaatttcaaatggtccagtgcctgagacttcacactgaagtagagcatttgttcctctcactatgtctgcaggctcaagagttttgatgaaagaaggaggttctttgataactatttcagtactgcagctatcactgccgacgtcattcactgcttcacatgagtaactcccactgtcttcaacttttacatccgtaatatcaagtatagcctcagaattgacaaaatacattcggactgtgttactttcactgagttctttgttatttttaaaccaagtaacctggatcacaggtgagcctttcagcttgcaatggaggcgtgctgattcacctgggagcattaaataagagggatccaccttcttcacgaaggatggtggctctctgacagtgactgtggctgagcaggagctgcttccagcctcatttgaagctgtacagacataggttcctgaatctttcagtttggccaaaggaatctcaagtgttgctattttatcttcaaaacagatcttataatctttccctggggggagtttttgcccatctttgctccacgtaactgtgacttttctgtcttcatctacttggcactcaaggtggaccttcttattgatagcggactgcacaggctctaattctttaatgaaatgtggcttatcaatgatgatcaactctgcttggcagatgtctgctccaaacttgttggaagccttacaagaataaactcctctatcttgaatggtaaggtttgagagttctaaaatgtgtttgttttctgcgtcggaaatcctccagttaggtgaaggtgagagtgcagcaccatctttctgccaaatggtttctatcacaggagtccctgtcactgtgcagatgaacttggctgccttacccacaaaagttgtaagggacttaggtctggagagaaaggttggtggatatgcctctgtcacagttagtgtggctgtacagctgacactgccatactcattggaagctttgcatgtatactcgccgcagtcaaccacctgggttctcaggatttcaaggctggagatatactttgaagatcgaatagaacacttgtcactctcataaatttctcggccagctttaaaccactggaaccggacattgggagcactttggatctcacaggtgaatttggctaggtggcccagtgctacttccaggggttcgattttcctcttgatcactggggcagctctttttactacagtgagtttggctgaagttgctgtttttccgctgtcattcaaggcctcacagacatactctccttgatggtcttcggtatttactttgtcgatgactagcgtatatgtattttgatcttgtaaacacttgaacttttcatctgaaggcaccagtttattctcaaaataccaattcacctctttagcatttgttatggatgttgtgaggtgtacaatatcaccttcctcagaaacagtgtccactaaaggtgtatgtatcatggggccatcctctttgattaagccaccctcagcttcctgtatctttactgtagcaacctcctcagtaccactttcagaggaagactcctctttttcctctgatggtttcagactctcatcttgtttttcgtcagagacaacagctgaagcaacccctttagtgacaggtgtggcatccaaatatttaaccctactttgcacgttaaaataactgacctcttcagttgagatcagatatttagattcaacttctggttcagtaatgggttcaaccttctgtgaacctgaaaaagaatccatttcttcttgcaaacttgttttggctccttgctgaattctaggaccctcagctgttaggatgtctatttcctcatatataatagcacacaaagcatccctaagttccattttcaggttagccatttgaggatcaacatcttcaataatgatggttacttcttctgttacagactttgccgaagtaacaaggtacatgcacatgatgtgtctgggctcttgggtgatgtttacagcctcgacctccaccttttcaatatttcttagccactcagagaaaagacctggctgctcgctggccacggctgcttgcaaagcccggcagatttgaattttcaggtttaatctctgctcttctggaataccagaaagcaagctttccttagaaagaaggtcccttccctgtacctcctgcactttctttattgccacgggctctcttttagactcaatgatttggtctgggggcatcaccacgttgtcagaatgctcttctttgagcagtacctgcttttcttcaagtgctagtggaaatcttaaggacttgccttcctcaattctgaccgcagaatcttgccctgcattttccagtggatttgcactttctatcaaaattttacctccttctgtgcatgagtgttctgaagggactaggggctcatagtttacctgagagatcatgacatcaggactctggagactctccacgtgtccctcagctaagctctgactcaagatgagcgcactttgtgcctcttgcttttgaagagtcactctttgctctctgttggtgtcagatactgtcttttcttttggtgaaagtacttcctcagccacagaggttagataagaatgcattggaggttctattgaagactgtggataattcccttcaggttcagctaataaagttttcagaggctcaactgttaatgaattaatttgttctatggacatggcacttgggaagattttctcggtatctgatagaactgcctgtgtctcaggctcttcaggcattagaataccttctttggagaaggttttctgggactgtacaatctgcagctgtaggttgggagatggttccttgagaggctgaaagtgaatactgccattgatgcaaagaaattccctggtgctttcaggagtgagcttgtcttgctccaaaatggattgcaattcctgagctcccaaaggaagctgactgctcaattcattggctttagcaatatgctcataagatagttgctggttttcttctgtaattaaagcagctttcaaaatggtgtcttttacaaacgttgcaatttcctgctctgagtcaagtgcttcaactgcgggaccctttaagggtgtctgtggaaaatcctcaggagcctctggtgtggactttgctttgcagggggtatcagtcatgtctgtgtcttccagaagcacaagcagctctgctgcacaggtggactcacccaacatattctctgctttacagatatagaggccactgtcttccctctgagggtcattgacaatgaaagttccagagccattagggttatgaatgatagtgtaataaacactggtgcaaagctgcttgttttctttgaaccatgtaacagtaggggcaggctctccaaccactgtgtactcaaagatggcaggaagcccttgagcacagcgaattggttttaactccttaaggaagtgaggaggacaaggacctcccagcttttccagagattttgccactgctgattctgtttcagtgtctttgtgaccctctcctttggaattaatttttagataggcactacatattgtctttccatagtcattactggccatacatgtatactctccctcatcctccaatttggtgaacagaatgatcaggctatgatcatcaccgtcaaaaacaaatttgtagtcagcagaaggggttaatagcactccattaaagaaccactgaattttaggtttggggatgccaatgacagttacagacagtgtagccacatcccccatgcttatatcagcatttgacacttctttgatgaaaattgggccagtgccttccttttcggaatcaaatttagttgggtaaactggagattcagacaaaagttcaagtgtttcatttattttagataattgaagttcggcgctatgaagtccttcttcctcggcagacagaaaagaactagaaaactctttcatttccatctcaatctcttgttcaatcctctcatgcaaaattgattcaggagcttccagactcaggttggctgtgcttgatacttggcctacagcattactagcaacaaacgtgtaagttccttcatcttctggataagcttcggcaatttccagttgataagtgtcttcaaattgagtcattctaaagaaccgagatggcttgattttcttgtctttgctgtaccacgacacttttagatctgttccagaaacccggcattgaaaacgggctggctgcccttcagaagtgacagtgtcctgaagcggggtgatgatggcaggtggataaacaggcatttcctgatcaggagacacaacttctggaacttccactgagagtgaagctgatgttgtggcaacaccatagtcattcttggcttcacaggtatagactgccgcatcctctgggaaggcttcaattagcaaaagcgtgtattcttgcccatcatgaagaaatttgcacttgaagccagtggaaagcagctgctcttccttgtaccaggaaattttgggctgtggtcttccggatatcacggcacagaagcgggcaggcttgccagactgcacagtgacaggctggagctcctgcagaacttggggcggttcaggagcattgacatagagagtgacagaactcctgttccttcctgccacaaaggtgtattctcctgcatcgctctgtctggtctcagagataaacattcggtggattcttctttccactacatatttgtgtcgttcttgaacttggaaattgatttcaatgccatctttataccagtgggcatcaacatcgtcttcattgacctcaaattcaacaacagcacgctgtttctcaatgacctgaacctcctttttaatacttcggatgcgaacatctctgccttctacaaagagttttgcagttgacacgttgcctcctgccaccactgtgtacttcccagcatcagacatccgggtggatgggatcagaaggcggtggacatatttctccttctgaatctttattctgtctgtgatctgcagttcctggtcatctttcatccactgtacagtgatgtcaggttcagaaacttcacattcaaacatggctcgcttcttctccagtaccttaatgtccttaatgtgtttcctaaattctatatgacgagcttccacataaagtgtggctgttgatgttgcttttccagccacaaaggtgtagtcagcagcatccccaaagtgaacattcctgatgttcagtgagtgtgtgagctttttggttctcatctggcacttgtcagttgatttgatttccacaccattctttaaccatttgtaagagatgccttcatagttcactgtcacctcaaaagtaatagtgtctttttcttcagcgttgatgtctttcagcatggaagtaatcatgattggggtgactgtcagggtggcactgacttggtcattgccacagacaaatgtgtattctgccgagtcctctgtgctggtgttcatgatgatcagctgatggagttttccctgcacaactatcttgaacttttcactcatctcaatttccacaccattcttcagccacatggaagggacattgaagtgggacacctcacactcaaaagaggcagttttggtctcaggcacctcgatatttttcatggtttttgtaatatgtaatgtctccacaaacagttttgctttgcattccaattgcccgaccacagctgtgtattccccagcatctgagggggagatgttctgcagcatcagcttgtggactttcctttctgagaccagtctgtgtttgtcacttggcttaatttccacactcttatggaaccattttactggaacagtgtcatgggaaacactaacttcaaaggcaacagtggcattttccaaggctgtcacatcctttggctttttaatgatcttgacagtctccacgtgcagtctggcactggctccaagccttccaagcctgaagccataaacagactcatccacgatggcacagtttttaatcctcagagagtaaattgttcctttgacagagatagcatacttttcattggattccagcacaactccatttttgatccactggacacctttgacattagggtgtgtaagctcgacagtgaaaacagcatcctgtgtttctgtcactgtgaggttcttcagagtcttcttaattttgacagcttcaactttgagtttggcagatgttttggaggtggccaccttgtaggtatattctccaatgtcatctaatttggtggcagcaatgataagtctccttttgtggccatcagactcacttctgatgttgttagtcagtggtaggtgtttgccatccctcaaccattcgcctttggaatctgggttggcaacttcacattcaaacacagcttcctgggattcagctacggtctgatctgtgagtggcttggagatggccccacctgccacagtaagttttccagatgtcatattttctcccgcgtaaaatgtgtattttccttcatcatctttcatcatatttagaactgtcaatttatatatttttccatgtgcttcaattttatatttagaactgggcttgatttccttgtccttaaaattccacaggacatcaattccagagtgggacagctcaacctcaaacaccacattttgagtttctgtacaggtaaggtcacgaagacctctgataattttaattttttctacagagagattacagttggtttcaactctgccaactatcagcttgtaaggtccttcgtctgaagcatgagttcggttaatgactagtcgctgtttagtacctttcacaatggcctgtacacggtcatcaggcttgatttgttcatcatttaagtaccacttaacagaagtcacatcagggactgacaccttacattcaagcacagccttggtgccttcaatcacattaacatcttttagaggtgttatcacgtccacactatagacagagacacgcccactggtggagaggccaagggctggaatggtgaaagagtaatttccagcatcttccttagtcatgtcttcaatgagcagcatatgagattgtttgtctatcacaatgtgaaccctgtcactgggctgcacttcttggccgtctttcatccagacgccttccacactttccaaggagactttaacttcaagctgaacaatgtcaccctcacagactttttggtcactaagtccttgtaggatagcaatggggcggggtttcatctttaatttacaggttgtctttttcccgtcgatgacaaagctgtattctccctggtcctccttggttacatccttgaccgtgaggttctgacgtccacgacgagatgtaattgtatatttgccattggatttaagctccacatcattatgataccattttccttctatattttctggggatacaatgcactctaattctcctgaatatgattctggaacttctatgtcctgaagttctttcacaaactcaacaactgcaccttcaacaataagtttagcagtcgttttgacattttcatcttccacaagtacacagctgtaatcttcagcatcagacgtatcaatggtcagtatggagaggaagtgaacctttctgtcagagtgcatcctgtatttatctccctcatgaacctccataccatctttataccatttcactttgacaaatggttctgaagtttcacattcaaaggttgccatagtgtctttttccttagcaacaacatcttgtaattcctgtgtgaaagtgatcaattgcttggcttggacaagtaagaatgcgtgactggaggtttctccagctatgttgatggcttttaccatgatgctggcagagtcctcagcagtcacatctcttatgaccaattcacaaacattgtcttcgggccagtaccagtagatccggtcagaccgttcaattttgacaccatttttgtaccattcacattcggggtctggtttccccacgactctgacccggaagtgtgcatcagatccttggcccactgtttggctctggattctttcgaagatttttggagcctccatactaggacttagttcaatcttgtcaggtttaaaagttggaatcgtgattttgccttcttcggcaagagctttcttttcctcttcagttaactctttggtccagtggagaagttcatcttttgtcttcctgaggagttcctcataggattcatccttctttcgagacttgagctccacagcggtaatggcttcataatagccctcttctgttctgcgcttgaatttactgcgcagctcttccgactcttcaggcactttttcatgggtaattctttcagcccttttcaacttcacaacttctttggtttcagtggtgtcaacaggtctatccactttttgtacttcaaactgaagctttcctggttcatgtacgtgaaactcaggccttggttcaggagctctcctaaggacagacctaaaatcttccctctgttgaatctcaagcttcactttatgctctatcacaccttcaggattttccgcggtgaccttcacttcacctgtgtcatatgatttgcagtccacgatgtccaggtaatggataccatcatagcgaactctgaaccttttgcttttgcggatgagctgtccattgaggtaccagttgactttgggctgagggtagcctgttaccctgcagcggaaccttgcagtctccccttcaagtactctaactggctctgggtacaagacaatgtctggcttttgcttttctttctgatctgttgttacacctgtaagtgcaccttcatgagccattctctctaattcttcaattctctgtaagcctttcctcccctcaggcaattgggattcttccacaagacttttctcatctttaacaataagggtagcagatgtgtgatctgttccatatttgttagtggctctgcaagtaatgataccactgtctctagaatatgcaacgccataatcaaggctgcagtacccaaattcattgatcatacggagcctgttggctgcttcaagtggctttccatcatggagccactccaccaccatcgttgggtcaccaatgggtgttagcctgcattcaaagtgggcaggcccaaagcgcttaagtcttaaggaagtgagttttttcttgaaaaatggtttctgttgtttctctttgtcatagagatcaccttcttcccattgctcttggccatatcgcaaatggaggggctccagttctggggctgcaatctcctttgctctatatgtcccccgtgggatgattaactttctctctggctcaggctctgcaaactcaacttcaacatttactttgcatcttgtagtgtctctgccagctttattaatagcagtcgcagtataccaggcagaatcttggctgacagtggaatcgattttaagggcagcttctcccttggttccttcaattctgattttgggatatttatgaggcacaatgatgtcactgtttttcaaccatacaatgtcagggttggggttacccgtagctctgactttcatttcaagtcgggaaccttcctttatattgacatttttcagtttttctacaaacatcggttttacctgatgttccacagcttccacagttaaaatcactgaaattgaagatctgcctgccctgttttgggcaaccacagtccattccccagaatcactgggtgtggcagggacaataattagtgattgagtaccatcttctttaatgactactttatgggtatagtcattgacaatttgctggccatcatgaaaccagaacgtctctggcataggtctaccaacaacctttaagtcaaatctggcagtttgcccttctaaacatttgaaagaaacaggttttaacacaaagactggtttatatagtctctcaagttgtgactcatctgtctcctccagcctacgtccaggggacattcttgcaggggacatccgtgcaggagacatccttgcaggtgacatccgtgcaggagacatgcgtataggagacctgctcactgaacgtggagagagagatctgattctgctcactggctctagtgtgggaatgtaagtcggagctccaagtggtgcagcaggctccacatacaatttccctgagcaaattgcatttcctttaatattgctggcaaatgcagtgtagattccttcatcttctggaagaacaacaggtatacgcagactagctctgccatcttgtagaaagtccatttggtatctttctccatgtttgatgcgcttgccatctttgtaccaagcaatctttggtaatggatatccagacatcttgcaatgaaaagtgacacccatcccctcaagaattctataattcttgattcttgaatcaaatcctgattcaacagcttcagattcagaaatgtcaactgccatcttttcttctccatcttcttcaagaagttcttctaatgtagtctttattattctatattcaatttctttaataagtctctcttcaaaggaagaaatatggaattcctgatcttctacataagttctgaccactacagtatctttggccattttcttcctaattaaggcttgttctttttcatactctttttcatactcagagtatacaaatccaggtgctgtttctccaactttaggttcttgaacaaatgcagtcacttgtgtctgataaagcatttcttgctgggacttcatcagtaactcataatcagcttcttcaagcaaggaagcagatgcagaagtttctccatgcttattgcgaacaacaatagtgtattctccagcatcatcagcaaaagtcatagaaatcaccagcttgcattcaccggtttgtttgttgtaactcactttgtatctgtatccagtggttagaggaacaccagattttttccagtatacatggggctttgggttgccgccaacttggcatccaaacaccacgctcccaccttccaccagtttctggaccactggttttgtaataaagtaaggcgcggcaggttctccaggccctgcttgttcctctgtgaggctagtatcagtcataaccacatctcttgactcaacaaagcgtttctcttctgtagtaaatttctcagtcacggctgtggtttccttttcaaattcttctgacacctgcacagccagatagcaggatgtgctgacggttccagcctcatttacagcactgcaagtaaatcgcccgctgtcttccgcaaatgcttcgcgaatcataagacgagcaattccactctggaaggttatctggaagtcaatggaactttcgatttggtagtcttccctgtaccatgtcactgtcggggatgggtatccagagatgtggcactccaaggtgacagattcaccttctatgacagtcacattttttaagcccgagaccaaagttggtggagtaacaggaatttcaacaggtgctggtactcttgctgtttctgttaccttggcttcgcgtccgtgcagtacttcaaagcgctcttcacggacggtggtgccagtgatgctcacccctacttcctttttcacctcaacgccagcttcactcttgtaagtatctggtgtgtcagcgaaggggaactgtggcaagggtgtgggctctgcccttactctagtctcactgggcttcacagtaggagccttcaccgatttggtgatcttctgagcagaagatgtggctgacaactctttttgtaatgtggcaatagcactaccggctattgatgcctcatatccatgttctgtcttaggaacagaaatttttgaaacagtaaagtgagggctagctgtgcgggggcgtttatccacatggactaatctttccgttgttagatctgtagttttcttgatctgtgatgatatgtgcattcccttttgatcagtagttttgatatgagtctcagaaggagcctggattactctaggcttgactgctttagggacaacgtggggttctgaggctggacgttggggaggctcagctacctttgcggcggaaatgcgttccttatatccgtactccaaagtggtctgctgagcataggattcttcaagatgcccaggctctctgggctctctgactcgggcctggtctactgcagcaacaactgttgctacagcttcagccttttttccaacgtccacctttccatgggtaacttggatttgttcttgtctagtagccatagtttctctagttctcagtattgtttcttgttctttggctttagcagtagcaactgctattgtagacaaggcagttttctcggcttcctttctcatcttctcctgagttatttgcacttgttctcttttggtagtaatgccttctctacctcttgatactaaatcttgttctttgactttgggtgtggcaactatgactttaggtacaactgttttcctagtttccttcattatcttttcataacttaggtgcatttgatcttgttgtgtggtagtttcttcttgagctcccgggactgtttctagttttgtggactttgcagtggcaactaccaccatggatgcagcagttatctcagtttcctgtcttattgcttcttgagttacttgtttctgtttcttagtaatttcttcagaaattctagtttcttgttctttggctttagctgcggaaattactacctttggtacaaatgttttttcagtttcttttcttatctgctcatgagttacgtgcatctgctcttgctttgtggtaattacttctttggttcttgattttaattcttgttccttggctttatcggcggccactactaccttagttacagcagtcttctccgcttcctttcttacctgttcttgagcaggttggatgtgcacagcagtcgtggttgtcctctgagcagtctgctctacagcgctgatcactggttctctcactctggccatatcaacggcagcaacaacagtcgcaacagctgcacttttgtcagcatcttgtttcacctctttagcaccagtggcaacagcctctgctgcgtagctagcactggccgacacactggcggcagcacccgcagcaccactgatggtcacttgctcctggacaccgtatctcccttcccatctctcttctgtcctgatctgagtagaggttgtcagcgttgtctctctcatctcagcctcagatgaggaggccacgtagccctcttgcttccaagggggaggcacttcaggacctgtggccacggtggatgcctgagtcttacgcatgagcaatggagacctaacagacctgatgggggatgtggagattcttgctgctggagacacggacctgaccggagatggggtcggtgcccgcacgtgtctgaccggggaaggggagtgtcttatgggcgatggggactgctgccgagccagctgtgctttggcagcaatagacggtggtgttggggatcttgactttggcttcggaggaatcctgggaggtgttttatgtggcagctgttgcccagcggcaccatctatgaccatctcaactgttgcaattgatctggcatcaaagtgggcttcaatcttcttttcaattcgggtttgtcttgattctgagatctgagcagtcgaaacaattgtctttgtctttttagcaggtacttcttcttcaccttgaaccagtaattcagcagtcgaagtagctcttccaacgctattggtggcatttactgaataggtccctgagtcctcagggtatgcttctgcaatcagtaagctgtagaggtcgccttcttgtgaaatttggaaatcaagggagctctggatttcggctccatcccggtagaacttcaccacaggtgtagggattccagtcactctcacttggagtctcacttggcttccttgtctcacggtcatgctctgcagtcgttgaacgaagttgggtggtgctgtctcagctttcacgagaagctcagcagtactagtcgcttgtccagatccattggtggctttcagggaatatcgtccactgttggctttagtcacggcggggatcgtcagtttagcgcggccatcgctaaaggagatctgcacgccgggcagagtggaagtggaaatcacctggccatccctaaaccagctcacctcaggaactggaaaaccactaatgtgagcctcaaaggttgcggtactaccctccagtaccacaacgctttgtaacggctgcgtaaacgtcggtgcttgagttgtcatctttctaggcactctgatttctcaagagtgcctaaaaagggtgggactaagcccaaggttgcttctgaaacgacgtcctatggagagttggtttttctgaccatctccgacatgaatcggtgagcctctaatcctaaaaacaaaactacacagtcaagactgtgtagttttgcttttctatgcaatccctacacccgaggcgaggctgggaatgcacgactgctc

SEQ ID NO: 10301 - RNA, 20420 nt, Homo sapiens
  source 1..20420: mol_type = other RNA
ccaaaactgcagttacttttgccaacactgtttttcacttcaaagctatataatcctttgtcactcatttcggcacaggggattttaagggaagccactttattgatgaatgtaatgtgatgtttgctgtctgcagacaattctcttccatctttgaaccacttggctgagagttctggtgttccagtcactacacactctaatgcaaaaggatttccagtagtgacagtcatgggttcgggcttctctatgattcttgctggttctagtacagtcaagactgcagagcattctctcattccagcatcgtttttgatttggcatatatattttccagaattagatgcttctggactccccagctggagggttgcaatgttatcaatgaatgaaatcctggtattttcactctctctgatgacttcacctctatctttcagccagacaacagaaattggctggaagccctccactatggcccgtaactcaacagcatccccaataagggttgaggtgtcacttagctttttcacgaatcgtggaggttctttgaacttgacagagcaagaacacgtgtcacttcccacctcattagtagctttgcagtgatattccccgacatcggaggcttcaagattaaggatatgaagacttgtatcaaaatgttttgaagtgattttaaatttcttgctgtttctaacctgctttcgatctttaacccatactacttcaaatgggggagttcccgaaatttcacattggagaatcacatcagaacctttaagagctcctactggagaaggcttctgggtgaaaacaggaggtgctttcactgtcaacgctgtgctgcagctggcgtcaccaacaccattatgagcctcacaaatgtagtccccgctgtcttcagcactagcttcattgatcgtaagcaatgccacagaattaatgaatgacatgttgtatttccaactttcatgaagttcgctgtcatttcggaaccatgaaactttgatttctggggagccacttattttacattccagttgaatggattctccctgctttgcaacttttgaagcttctaatttcttaacaaactttggaggttcttttacactgagctgagctgagcacatgtctttgccaacatcattggttgcttggcaagtatattgaccagagtctcctttgcctactttaagaattctcaaatgaggagtgtttcccacacatgtgattgtatagtttcctccaggacggatctccttgttatcttttgaccaagtgattcgcatcggttgagcaccagtaacatgacactcaaaatcagcactttctccagcaataacatctatagatacaggcttgatgtcaaagaagggagatttcttgggttctcttgctgtgagtctagcactagaagatgctgttccaagtgggttggaagctgagcaagagtactggccagagtgactcaagtcagtttgcaaaatttttaaagttgccacattatctacaaatgaagtctgtagattttcatcgtctcttaaaagtactccatctctataccagcacacttggatgggtgcagagccatttaatcgacaagtgagtgtaacaggtaaccccacagtttgttcaatgtcctttaattgtcttgcaaaagaaggtgggagttggcgctcttgaattctgaacacagtcttagaagaagcagttcctatactattttctgctttgcatgtgtactctccactgtcattgatgttcactttattaaaaacaagtgtggccacattgtttgtaaagtaggtcctgtattcaggagttggccgtaatttggtatctcctttgtaccaagacactgtaatttctggtgtcccagcaacttggcattgtaaagaaaccgaatctccaactgctgcctccagaggttccagttccgtaacaaaataaggcggttctaatgtagataccagagctccacaaacatcccttcctgcctcattttcaatctcgcaggaatactgccctgcatctctttttgtgctattcagaatttccaggatacaagttttctctgttgtgactatgttacatttttcagaggtagttatgttaaaaccatcctttttccaagtgacagaaattggaagtgttccagtgtaggtgctctccagaattatggacttccctggttctacagaatgatcacttaatctcttcaaaaatgcagctggttctttcacaaagagacgggtagtgcaagatgcttggccagcgttgttagaaaccacacaggtgtattccccactctgagatatgtcaatattaaataattccagttctgccacagtgtcttcaaaatagatgttgcaccggtctcctttcactagttctctggcacctctgaaccagttgactttgaatggaggggttcctctaataacgcttgtgaaggttacatttttgcctggtagtacttccaaaggttcaggttctttcacaaaagagggtggttcttgtacagttagcactgcacgacattcatcagacccagcgacattagcagccacgcatgtgtaattgcccatatctgaggaatccagagaattcaactgcaatgtgcagacattatctgaaaatgtggtttggtactttgctccactgacaatcttggttttctcatgaaaccaggcaactgaaataggtgatgatccagctactttgcattccaagatgcaagaagcacctaacaccccaccagtatttttcagtcttcgtgtgaaagagggaggaactgctcggtctgaaacatcaaccacagctgtgcagctgcttttcccaacattattttgaacctggaaagtgtatgtgcctgcatcttgcctttcaactgagagaatccttaaggaagagattttgttgtagaagctaaatttgtgtttttggctgctggtcaacagctttccatccttgtaccattcaacagagagttccggagtgccagccaccttacactccagagtgcacgtttctcctacagtcaccgtcatcggtcctgccttctcaacaatgactgcgggctctaagaccatcagtgtggccatgttctccctcattccaccatcattcttgatttggcagatatactttccagcattagctggctctgcttttgcaaactgtagagttgcaacattttccacaaatgtaatcctgatgttttcactttctctaatcacttcttccttctctttaagccactggacaaaaataggctgggcgccttctatggatgcttgtaattcagcaggctctccggctacaacagtgaggctgttcagtttggagacaaatcttggtggttctttcaattttacagtacaaacacaagtatcacttcccacttcattctgtgctttgcagtggtattcaccgatgtctgaagtgtccacattgagaatgtgaatacttgtgtggaagtttttggatgcaatcttgtatttcttgctgcttctgagttgccgcttgtctttgtaccataccacctcaaacggtggtgttcccgaaagttcacattcaagactgacttcagcatttttaagggtttctactataggagggaagctgctaaaaacaggtggctcttttactataaccttggtactgcagcttgtgctgccagcgggattctgagcctcacaaatgaaatctccactgtcctcagtactgagattgttcatctgtatgacggccactgagtcaatgaaagtcattctgtacttatcactggctggaagttcatgttcatttcggaaccacacaactctgatttctggggatccagctatcttgcattcaagtcgtgaagagtcacctgctttcacaattttggaggcttctaatttctttacaaactttggtggttctgtcacaagcaacatcgtagtacaagagtcgctaccaacatcattggtaacatggcaagtatactgtccagtcttagaagcatccactgagtagagatttaagaagctagtcgacccttccaagccaatgaaacatttaggacctgagacaagttccacatcatccttaaaccattttattttaaatggtggtgttccttttagtattgccttaaattccactgtagaatcaggtatggcttgctgtcgcccaggtttcactaggaagcttggtggttctttcacagttaagatgccactgcatgcatcatctcctgctacatttgacactttgcatgtgtaatttgcagtatcttctaattccagattattaacttccagagacacagatctctcatggcacacaagtctgtattttgcacttgtagatatttcttttccatccttaaaccactgagcactaatgggaagtgaaccagacaccttgcactccatatgaatagaagagcccagaactttatccattttggttaattttttggtgaatgatggaggaatattttgatctagcactcttaagtaggcatcacagctactgcttccgaagtcattttccaccttgaaagtgtactgaccgctgtcctgcttcattactgactgaattctaaaactggccacgttattttcaaaactcattgaaaagtatctactgggaactatttgtttcccgtctttaagccatttcactttgagttctggtgttccagccacaacacattccaaggtcatgggatctttctccgtaacatcaactgatttagctttctctacgatttgagctggttcttgtactaaaaggaaagcataacacctctcaactcctgactcattcttggcttgacaggtatatctcccactgtgtccattatccacacttctgatttgaagtgtggccacactgtccacaaatgaaatatagacattatcatcttcatcaagaatctgatcatcctttagccaggttatagaaataggaggagaacctgccacggtactctgaaaggtggcagaacttttcaaaacagtagtggtattttctatcttcttaatgaatgatggtggttctttcagggcaactctagtactgcatgagcagctgccgccttcattggatacaatgcactggtattccccagtgtctgaagggtcacacttggttatatggaggttaaacacagacactctgtcggtcaatgtgtattttttgctgcttcgaatttccctgttattcttcagccaagtgacttcaaacggaggtgttcccgtaacttcacactccagctccacgtcactatattttactacctccacaggcttcagctctctgataaaggtggggggttctttcactttgagttcaatgctgcagctcgccgtgcctgcgtcatttcgagcttcacacacataagtcccactattttctaccctggcaccagaaatctggaaagtggctaaaccatcaatgaaggaaatgccatgtttctgaatggctgttatttcattcccgtctagataccaagacactcggattttaggagtgcctgttatttggcattcaaatgttgttgactgtccattcctcagcactaagactggactgggcttcttaatgaattgaggaggttcttttacaaagagagtggctttgctggttgctgtgccaacatcattgcttagttggcaaatgtaggttccagaatcggtagctttggctgcaaagagctctagactggtagaggtgtcatccttccaaactgagcgggctgctcctgagtgtaactctttgttatctttaaaccactttattgtcatgggtgcagtgccacccacaagagcctttaactgtacccttgtgttgggattgacatcttgtgactgtggcttttccacaaagtaagggggttctttgactgtcagatgcccactgcattggttgtgccctgccttatttgtggcagaacaagtgtatgtcccactgtctgtaccttccagctggctgatttccaagaaggcagtattgtcatgaaaagagaatttgtacttttcactagctgatatttcttggtcatctttgaaccactggatgcttatgggatgtgacccagccactatacattctaaatcaatgaaagaacctttaatgctgtccattttcttcagctttttggtgaatgaaggaggtatgataagatctaatacattaattctagccttgcagctgctcctcccaacatcattttggacctcgaaagtatattctccactatctttcttttctgtagaaataatcttcagtattgagactgtatcagtgacactgattttatattttgagcccagggtcagttcttggccatctttaaaccatttggctgtaatctccttagtccctgaaaatttaacctgcaaagtggctgggtctccttgggtgacatctatagacacagcttcctcggtgattgttgcaggttcttttactgagagtaatgcagaacatctttgtattcctgcatcatttttggcctgacagacatatttcccatcatgcttgacttcaatgccactgaggtacaaactggccacattgttctcaaaggtcattcttatattatcgtcttcagtgatttcatcgctgtcttttagccaagtcaccgtaattggcaaggagcccttcagagtggcctggaaggcagctgtgcctccccggagggagctggtactctcgatcttctttatgaaggatgggggttctcttaaagtcaccctggcactgcagatgctgctgcccacctcattggtcacccgacactggtattcgccagcatctgcagctacaaacttgaggatctgcaggctaaccagatgatcctgaatgaaagtcttatactttctaccacttcgcaggattgtgttatctttgaaccaagtgatctcaaagggaggagtgcctgccacctcagccagcaacatgacatcgtactcctttaagacttcaattggcttaaattccttggtaaaataaggtgactctttgactattacaatgctactgcagtggtcactgccagcctcattttgggcctcacacatatattcaccactgtcttcgatgccaacatctgtcagtcttagaactgcagtagactccacaaaagacattctgtgtttgctgctctccttaatttctctatcatttgcaaaccatgttattttaattggaggggtaccagttactttgcaggctagctgggtggcatctcccttctttaacagctgtgatggctctaacttttcaacaaatgtggcaggttcttttacaaacaagtttgcactgcattccacccctccagcgacattgctgactttacatgtgtacgtgcccgaatcagaggtttttactaaatagagttccagggaactctctaaagcttctttggtaatatagcagcttccaccagaaaccagctctttgttgcccttaaaccatctgattgtgagaggagtagatccttggaaagtgctcttcaggcagactgctgagccaggcagaacatcctttgagccgggtttagttacaaaactgggtggttcttgcacaatcagggctccactgctgtctttgcttcccacggaatttgtggctcgacaagtgaaattccctgcatcattcatgtctactctgatgatctccaaagaggctgtgccttccacaaatgctatcctgtatctgtcagaagcagctatttctttgccatccttaaaccaggacaccctcatggggagggagcctgcaattttgcagtccagtctgcaggtaccattaacaacactatccacgttgcgcaagggtttggtaaaaaatggagcaatgtctcgatctaatacagtgaatgtagtctcacaggagctgctgcccacttcattggaaatctcaaatgtgtattggccactgtcgtgcagctcagctgaataaaatttgagctgggcaacattgtttttaaaacttattcggtattttttactggcgaccaagggtctcccatctttgtaccatttgggcttcagttctggcgtgcctgccactgtgtactccagtgtggcgggatctcctgctgtcacctggatcagttctgctcgctcaatgattttggcaggttctttaactattaattccccaacagatgtttggcttccagcttcattttcagccaggcacgtgtatttgcctccaaaactaatctgaacatcagggattatcaagactgcaacaccattggaaaagctcattttgatttttccgtcttctctgatgacctcttgacctttcatccatgtgacagaaatgggctctgaccctctcacagcagcttgcagggtaacggtttgtcctcctagtgcaatcaaatcatctactttctttacaaaggttggaggttctttgagtaagtgggttgccatgcagccacacttgccgacttcattagcaacaacacattcatattcaccaacatctgcactattaaacgaaaagatctccagacacacaagagacttctgagaaaacaatctgtattttttactacttcgaatttgtttcttgtctttgaaccagctaatttcaaatggtccagtgcctgagacttcacactgaagtagagcatttgttcctctcactatgtctgcaggctcaagagttttgatgaaagaaggaggttctttgataactatttcagtactgcagctatcactgccgacgtcattcactgcttcacatgagtaactcccactgtcttcaacttttacatccgtaatatcaagtatagcctcagaattgacaaaatacattcggactgtgttactttcactgagttctttgttatttttaaaccaagtaacctggatcacaggtgagcctttcagcttgcaatggaggcgtgctgattcacctgggagcattaaataagagggatccaccttcttcacgaaggatggtggctctctgacagtgactgtggctgagcaggagctgcttccagcctcatttgaagctgtacagacataggttcctgaatctttcagtttggccaaaggaatctcaagtgttgctattttatcttcaaaacagatcttataatctttccctggggggagtttttgcccatctttgctccacgtaactgtgacttttctgtcttcatctacttggcactcaaggtggaccttcttattgatagcggactgcacaggctctaattctttaatgaaatgtggcttatcaatgatgatcaactctgcttggcagatgtctgctccaaacttgttggaagccttacaagaataaactcctctatcttgaatggtaaggtttgagagttctaaaatgtgtttgttttctgcgtcggaaatcctccagttaggtgaaggtgagagtgcagcaccatctttctgccaaatggtttctatcacaggagtccctgtcactgtgcagatgaacttggctgccttacccacaaaagttgtaagggacttaggtctggagagaaaggttggtggatatgcctctgtcacagttagtgtggctgtacagctgacactgccatactcattggaagctttgcatgtatactcgccgcagtcaaccacctgggttctcaggatttcaaggctggagatatactttgaagatcgaatagaacacttgtcactctcataaatttctcggccagctttaaaccactggaaccggacattgggagcactttggatctcacaggtgaatttggctaggtggcccagtgctacttccaggggttcgattttcctcttgatcactggggcagctttcatttccatctcaatctcttgttcaatcctctcatgcaaaattgattcaggagcttccagactcaggttggctgtgcttgatacttggcctacagcattactagcaacaaacgtgtaagttccttcatcttctggataagcttcggcaatttccagttgataagtgtcttcaaattgagtcattctaaagaaccgagatggcttgattttcttgtctttgctgtaccacgacacttttagatctgttccagaaacccggcattgaaaacgggctggctgcccttcagaagtgacagtgtcctgaagcggggtgatgatggcaggtggataaacaggcatttcctgatcaggagacacaacttctggaacttccactgagagtgaagctgatgttgtggcaacaccatagtcattcttggcttcacaggtatagactgccgcatcctctgggaaggcttcaattagcaaaagcgtgtattcttgcccatcatgaagaaatttgcacttgaagccagtggaaagcagctgctcttccttgtaccaggaaattttgggctgtggtcttccggatatcacggcacagaagcgggcaggcttgccagactgcacagtgacaggctggagctcctgcagaacttggggcggttcaggagcattgacatagagagtgacagaactcctgttccttcctgccacaaaggtgtattctcctgcatcgctctgtctggtctcagagataaacattcggtggattcttctttccactacatatttgtgtcgttcttgaacttggaaattgatttcaatgccatctttataccagtgggcatcaacatcgtcttcattgacctcaaattcaacaacagcacgctgtttctcaatgacctgaacctcctttttaatacttcggatgcgaacatctctgccttctacaaagagttttgcagttgacacgttgcctcctgccaccactgtgtacttcccagcatcagacatccgggtggatgggatcagaaggcggtggacatatttctccttctgaatctttattctgtctgtgatctgcagttcctggtcatctttcatccactgtacagtgatgtcaggttcagaaacttcacattcaaacatggctcgcttcttctccagtaccttaatgtccttaatgtgtttcctaaattctatatgacgagcttccacataaagtgtggctgttgatgttgcttttccagccacaaaggtgtagtcagcagcatccccaaagtgaacattcctgatgttcagtgagtgtgtgagctttttggttctcatctggcacttgtcagttgatttgatttccacaccattctttaaccatttgtaagagatgccttcatagttcactgtcacctcaaaagtaatagtgtctttttcttcagcgttgatgtctttcagcatggaagtaatcatgattggggtgactgtcagggtggcactgacttggtcattgccacagacaaatgtgtattctgccgagtcctctgtgctggtgttcatgatgatcagctgatggagttttccctgcacaactatcttgaacttttcactcatctcaatttccacaccattcttcagccacatggaagggacattgaagtgggacacctcacactcaaaagaggcagttttggtctcaggcacctcgatatttttcatggtttttgtaatatgtaatgtctccacaaacagttttgctttgcattccaattgcccgaccacagctgtgtattccccagcatctgagggggagatgttctgcagcatcagcttgtggactttcctttctgagaccagtctgtgtttgtcacttggcttaatttccacactcttatggaaccattttactggaacagtgtcatgggaaacactaacttcaaaggcaacagtggcattttccaaggctgtcacatcctttggctttttaatgatcttgacagtctccacgtgcagtctggcactggctccaagccttccaagcctgaagccataaacagactcatccacgatggcacagtttttaatcctcagagagtaaattgttcctttgacagagatagcatacttttcattggattccagcacaactccatttttgatccactggacacctttgacattagggtgtgtaagctcgacagtgaaaacagcatcctgtgtttctgtcactgtgaggttcttcagagtcttcttaattttgacagcttcaactttgagtttggcagatgttttggaggtggccaccttgtaggtatattctccaatgtcatctaatttggtggcagcaatgataagtctccttttgtggccatcagactcacttctgatgttgttagtcagtggtaggtgtttgccatccctcaaccattcgcctttggaatctgggttggcaacttcacattcaaacacagcttcctgggattcagctacggtctgatctgtgagtggcttggagatggccccacctgccacagtaagttttccagatgtcatattttctcccgcgtaaaatgtgtattttccttcatcatctttcatcatatttagaactgtcaatttatatatttttccatgtgcttcaattttatatttagaactgggcttgatttccttgtccttaaaattccacaggacatcaattccagagtgggacagctcaacctcaaacaccacattttgagtttctgtacaggtaaggtcacgaagacctctgataattttaattttttctacagagagattacagttggtttcaactctgccaactatcagcttgtaaggtccttcgtctgaagcatgagttcggttaatgactagtcgctgtttagtacctttcacaatggcctgtacacggtcatcaggcttgatttgttcatcatttaagtaccacttaacagaagtcacatcagggactgacaccttacattcaagcacagccttggtgccttcaatcacattaacatcttttagaggtgttatcacgtccacactatagacagagacacgcccactggtggagaggccaagggctggaatggtgaaagagtaatttccagcatcttccttagtcatgtcttcaatgagcagcatatgagattgtttgtctatcacaatgtgaaccctgtcactgggctgcacttcttggccgtctttcatccagacgccttccacactttccaaggagactttaacttcaagctgaacaatgtcaccctcacagactttttggtcactaagtccttgtaggatagcaatggggcggggtttcatctttaatttacaggttgtctttttcccgtcgatgacaaagctgtattctccctggtcctccttggttacatccttgaccgtgaggttctgacgtccacgacgagatgtaattgtatatttgccattggatttaagctccacatcattatgataccattttccttctatattttctggggatacaatgcactctaattctcctgaatatgattctggaacttctatgtcctgaagttctttcacaaactcaacaactgcaccttcaacaataagtttagcagtcgttttgacattttcatcttccacaagtacacagctgtaatcttcagcatcagacgtatcaatggtcagtatggagaggaagtgaacctttctgtcagagtgcatcctgtatttatctccctcatgaacctccataccatctttataccatttcactttgacaaatggttctgaagtttcacattcaaaggttgccatagtgtctttttccttagcaacaacatcttgtaattcctgtgtgaaagtgatcaattgcttggcttggacaagtaagaatgcgtgactggaggtttctccagctatgttgatggcttttaccatgatgctggcagagtcctcagcagtcacatctcttatgaccaattcacaaacattgtcttcgggccagtaccagtagatccggtcagaccgttcaattttgacaccatttttgtaccattcacattcggggtctggtttccccacgactctgacccggaagtgtgcatcagatccttggcccactgtttggctctggattctttcgaagatttttggagcctccatactaggacttagttcaatcttgtcaggtttaaaagttggaatcgtgattttgccttcttcggcaagagctttcttttcctcttcagttaactctttggtccagtggagaagttcatcttttgtcttcctgaggagttcctcataggattcatccttctttcgagacttgagctccacagcggtaatggcttcataatagccctcttctgttctgcgcttgaatttactgcgcagctcttccgactcttcaggcactttttcatgggtaattctttcagcccttttcaacttcacaacttctttggtttcagtggtgtcaacaggtctatccactttttgtacttcaaactgaagctttcctggttcatgtacgtgaaactcaggccttggttcaggagctctcctaaggacagacctaaaatcttccctctgttgaatctcaagcttcactttatgctctatcacaccttcaggattttccgcggtgaccttcacttcacctgtgtcatatgatttgcagtccacgatgtccaggtaatggataccatcatagcgaactctgaaccttttgcttttgcggatgagctgtccattgaggtaccagttgactttgggctgagggtagcctgttaccctgcagcggaaccttgcagtctccccttcaagtactctaactggctctgggtacaagacaatgtctggcttttgcttttctttctgatctgttgttacacctgtaagtgcaccttcatgagccattctctctaattcttcaattctctgtaagcctttcctcccctcaggcaattgggattcttccacaagacttttctcatctttaacaataagggtagcagatgtgtgatctgttccatatttgttagtggctctgcaagtaatgataccactgtctctagaatatgcaacgccataatcaaggctgcagtacccaaattcattgatcatacggagcctgttggctgcttcaagtggctttccatcatggagccactccaccaccatcgttgggtcaccaatgggtgttagcctgcattcaaagtgggcaggcccaaagcgcttaagtcttaaggaagtgagttttttcttgaaaaatggtttctgttgtttctctttgtcatagagatcaccttcttcccattgctcttggccatatcgcaaatggaggggctccagttctggggctgcaatctcctttgctctatatgtcccccgtgggatgattaactttctctctggctcaggctctgcaaactcaacttcaacatttactttgcatcttgtagtgtctctgccagctttattaatagcagtcgcagtataccaggcagaatcttggctgacagtggaatcgattttaagggcagcttctcccttggttccttcaattctgattttgggatatttatgaggcacaatgatgtcactgtttttcaaccatacaatgtcagggttggggttacccgtagctctgactttcatttcaagtcgggaaccttcctttatattgacatttttcagtttttctacaaacatcggttttacctgatgttccacagcttccacagttaaaatcactgaaattgaagatctgcctgccctgttttgggcaaccacagtccattccccagaatcactgggtgtggcagggacaataattagtgattgagtaccatcttctttaatgactactttatgggtatagtcattgacaatttgctggccatcatgaaaccagaacgtctctggcataggtctaccaacaacctttaagtcaaatctggcagtttgcccttctaaacatttgaaagaaacaggttttaacacaaagactggtttatatagtctctcaagttgtgactcatctgtctcctccagcctacgtccaggggacattcttgcaggggacatccgtgcaggagacatccttgcaggtgacatccgtgcaggagacatgcgtataggagacctgctcactgaacgtggagagagagatctgattctgctcactggctctagtgtgggaatgtaagtcggagctccaagtggtgcagcaggctccacatacaatttccctgagcaaattgcatttcctttaatattgctggcaaatgcagtgtagattccttcatcttctggaagaacaacaggtatacgcagactagctctgccatcttgtagaaagtccatttggtatctttctccatgtttgatgcgcttgccatctttgtaccaagcaatctttggtaatggatatccagacatcttgcaatgaaaagtgacacccatcccctcaagaattctataattcttgattcttgaatcaaatcctgattcaacagcttcagattcagaaatgtcaactgccatcttttcttctccatcttcttcaagaagttcttctaatgtagtctttattattctatattcaatttctttaataagtctctcttcaaaggaagaaatatggaattcctgatcttctacataagttctgaccactacagtatctttggccattttcttcctaattaaggcttgttctttttcatactctttttcatactcagagtatacaaatccaggtgctgtttctccaactttaggttcttgaacaaatgcagtcacttgtgtctgataaagcatttcttgctgggacttcatcagtaactcataatcagcttcttcaagcaaggaagcagatgcagaagtttctccatgcttattgcgaacaacaatagtgtattctccagcatcatcagcaaaagtcatagaaatcaccagcttgcattcaccggtttgtttgttgtaactcactttgtatctgtatccagtggttagaggaacaccagattttttccagtatacatggggctttgggttgccgccaacttggcatccaaacaccacgctcccaccttccaccagtttctggaccactggttttgtaataaagtaaggcgcggcaggttctccaggccctgcttgttcctctgtgaggctagtatcagtcataaccacatctcttgactcaacaaagcgtttctcttctgtagtaaatttctcagtcacggctgtggtttccttttcaaattcttctgacacctgcacagccagatagcaggatgtgctgacggttccagcctcatttacagcactgcaagtaaatcgcccgctgtcttccgcaaatgcttcgcgaatcataagacgagcaattccactctggaaggttatctggaagtcaatggaactttcgatttggtagtcttccctgtaccatgtcactgtcggggatgggtatccagagatgtggcactccaaggtgacagattcaccttctatgacagtcacattttttaagcccgagaccaaagttggtggagtaacaggaatttcaacaggtgctggtactcttgctgtttctgttaccttggcttcgcgtccgtgcagtacttcaaagcgctcttcacggacggtggtgccagtgatgctcacccctacttcctttttcacctcaacgccagcttcactcttgtaagtatctggtgtgtcagcgaaggggaactgtggcaagggtgtgggctctgcccttactctagtctcactgggcttcacagtaggagccttcaccgatttggtgatcttctgagcagaagatgtggctgacaactctttttgtaatgtggcaatagcactaccggctattgatgcctcatatccatgttctgtcttaggaacagaaatttttgaaacagtaaagtgagggctagctgtgcgggggcgtttatccacatggactaatctttccgttgttagatctgtagttttcttgatctgtgatgatatgtgcattcccttttgatcagtagttttgatatgagtctcagaaggagcctggattactctaggcttgactgctttagggacaacgtggggttctgaggctggacgttggggaggctcagctacctttgcggcggaaatgcgttccttatatccgtactccaaagtggtctgctgagcataggattcttcaagatgcccaggctctctgggctctctgactcgggcctggtctactgcagcaacaactgttgctacagcttcagccttttttccaacgtccacctttccatgggtaacttggatttgttcttgtctagtagccatagtttctctagttctcagtattgtttcttgttctttggctttagcagtagcaactgctattgtagacaaggcagttttctcggcttcctttctcatcttctcctgagttatttgcacttgttctcttttggtagtaatgccttctctacctcttgatactaaatcttgttctttgactttgggtgtggcaactatgactttaggtacaactgttttcctagtttccttcattatcttttcataacttaggtgcatttgatcttgttgtgtggtagtttcttcttgagctcccgggactgtttctagttttgtggactttgcagtggcaactaccaccatggatgcagcagttatctcagtttcctgtcttattgcttcttgagttacttgtttctgtttcttagtaatttcttcagaaattctagtttcttgttctttggctttagctgcggaaattactacctttggtacaaatgttttttcagtttcttttcttatctgctcatgagttacgtgcatctgctcttgctttgtggtaattacttctttggttcttgattttaattcttgttccttggctttatcggcggccactactaccttagttacagcagtcttctccgcttcctttcttacctgctgttcttgagcaggttggatgtgcacagcagtcgtggttgtcctctgagcagtctgctctacagcgctgatcactggttctctcactctggccatatcaacggcagcaacaacagtcgcaacagctgcacttttgtcagcatcttgtttcacctctttagcaccagtggcaacagcctctgctgcgtagctagcactggccgacacactggcggcagcacccgcagcaccactgatggtcacttgctcctggacaccgtatctcccttcccatctctcttctgtcctgatctgagtagaggttgtcagcgttgtctctctcatctcagcctcagatgaggaggccacgtagccctcttgcttccaagggggaggcacttcaggacctgtggccacggtggatgcctgagtcttacgcatgagcaatggagacctaacagacctgatgggggatgtggagattcttgctgctggagacacggacctgaccggagatggggtcggtgcccgcacgtgtctgaccggggaaggggagtgtcttatgggcgatggggactgctgccgagccagctgtgctttggcagcaatagacggtggtgttggggatcttgactttggcttcggaggaatcctgggaggtgttttatgtggcagctgttgcccagcggcaccatctatgaccatctcaactgttgcaattgatctggcatcaaagtgggcttcaatcttcttttcaattcgggtttgtcttgattctgagatctgagcagtcgaaacaattgtctttgtctttttagcaggtacttcttcttcaccttgaaccagtaattcagcagtcgaagtagctcttccaacgctattggtggcatttactgaataggtccctgagtcctcagggtatgcttctgcaatcagtaagctgtagaggtcgccttcttgtgaaatttggaaatcaagggagctctggatttcggctccatcccggtagaacttcaccacaggtgtagggattccagtcactctcacttggagtctcacttggcttccttgtctcacggtcatgctctgcagtcgttgaacgaagttgggtggtgctgtctcagctttcacgagaagctcagcagtactagtcgcttgtccagatccattggtggctttcagggaatatcgtccactgttggctttagtcacggcggggatcgtcagtttagcgcggccatcgctaaaggagatctgcacgccgggcagagtggaagtggaaatcacctggccatccctaaaccagctcacctcaggaactggaaaaccactaatgtgagcctcaaaggttgcggtactaccctccagtaccacaacgctttgtaacggctgcgtaaacgtcggtgcttgagttgtcatctttctaggcactctgatttctcaagagtgcctaaaaagggtgggactaagcccaaggttgcttctgaaacgacgtcctatggagagttggtttttctgaccatctccgacatgaatcggtgagcctctaatcctaaaaacaaaactacacagtcaagactgtgtagttttgcttttctatgcaatccctacacccgaggcgaggctgggaatgcacgactgctc

SEQ ID NO: 10302 - RNA, 20417 nt, Homo sapiens
  source 1..20417: mol_type = other RNA
ccaaaactgcagttacttttgccaacactgtttttcacttcaaagctatataatcctttgtcactcatttcggcacaggggattttaagggaagccactttattgatgaatgtaatgtgatgtttgctgtctgcagacaattctcttccatctttgaaccacttggctgagagttctggtgttccagtcactacacactctaatgcaaaaggatttccagtagtgacagtcatgggttcgggcttctctatgattcttgctggttctagtacagtcaagactgcagagcattctctcattccagcatcgtttttgatttggcatatatattttccagaattagatgcttctggactccccagctggagggttgcaatgttatcaatgaatgaaatcctggtattttcactctctctgatgacttcacctctatctttcagccagacaacagaaattggctggaagccctccactatggcccgtaactcaacagcatccccaataagggttgaggtgtcacttagctttttcacgaatcgtggaggttctttgaacttgacagagcaagaacacgtgtcacttcccacctcattagtagctttgcagtgatattccccgacatcggaggcttcaagattaaggatatgaagacttgtatcaaaatgttttgaagtgattttaaatttcttgctgtttctaacctgctttcgatctttaacccatactacttcaaatgggggagttcccgaaatttcacattggagaatcacatcagaacctttaagagctcctactggagaaggcttctgggtgaaaacaggaggtgctttcactgtcaacgctgtgctgcagctggcgtcaccaacaccattatgagcctcacaaatgtagtccccgctgtcttcagcactagcttcattgatcgtaagcaatgccacagaattaatgaatgacatgttgtatttccaactttcatgaagttcgctgtcatttcggaaccatgaaactttgatttctggggagccacttattttacattccagttgaatggattctccctgctttgcaacttttgaagcttctaatttcttaacaaactttggaggttcttttacactgagctgagctgagcacatgtctttgccaacatcattggttgcttggcaagtatattgaccagagtctcctttgcctactttaagaattctcaaatgaggagtgtttcccacacatgtgattgtatagtttcctccaggacggatctccttgttatcttttgaccaagtgattcgcatcggttgagcaccagtaacatgacactcaaaatcagcactttctccagcaataacatctatagatacaggcttgatgtcaaagaagggagatttcttgggttctcttgctgtgagtctagcactagaagatgctgttccaagtgggttggaagctgagcaagagtactggccagagtgactcaagtcagtttgcaaaatttttaaagttgccacattatctacaaatgaagtctgtagattttcatcgtctcttaaaagtactccatctctataccagcacacttggatgggtgcagagccatttaatcgacaagtgagtgtaacaggtaaccccacagtttgttcaatgtcctttaattgtcttgcaaaagaaggtgggagttggcgctcttgaattctgaacacagtcttagaagaagcagttcctatactattttctgctttgcatgtgtactctccactgtcattgatgttcactttattaaaaacaagtgtggccacattgtttgtaaagtaggtcctgtattcaggagttggccgtaatttggtatctcctttgtaccaagacactgtaatttctggtgtcccagcaacttggcattgtaaagaaaccgaatctccaactgctgcctccagaggttccagttccgtaacaaaataaggcggttctaatgtagataccagagctccacaaacatcccttcctgcctcattttcaatctcgcaggaatactgccctgcatctctttttgtgctattcagaatttccaggatacaagttttctctgttgtgactatgttacatttttcagaggtagttatgttaaaaccatcctttttccaagtgacagaaattggaagtgttccagtgtaggtgctctccagaattatggacttccctggttctacagaatgatcacttaatctcttcaaaaatgcagctggttctttcacaaagagacgggtagtgcaagatgcttggccagcgttgttagaaaccacacaggtgtattccccactctgagatatgtcaatattaaataattccagttctgccacagtgtcttcaaaatagatgttgcaccggtctcctttcactagttctctggcacctctgaaccagttgactttgaatggaggggttcctctaataacgcttgtgaaggttacatttttgcctggtagtacttccaaaggttcaggttctttcacaaaagagggtggttcttgtacagttagcactgcacgacattcatcagacccagcgacattagcagccacgcatgtgtaattgcccatatctgaggaatccagagaattcaactgcaatgtgcagacattatctgaaaatgtggtttggtactttgctccactgacaatcttggttttctcatgaaaccaggcaactgaaataggtgatgatccagctactttgcattccaagatgcaagaagcacctaacaccccaccagtatttttcagtcttcgtgtgaaagagggaggaactgctcggtctgaaacatcaaccacagctgtgcagctgcttttcccaacattattttgaacctggaaagtgtatgtgcctgcatcttgcctttcaactgagagaatccttaaggaagagattttgttgtagaagctaaatttgtgtttttggctgctggtcaacagctttccatccttgtaccattcaacagagagttccggagtgccagccaccttacactccagagtgcacgtttctcctacagtcaccgtcatcggtcctgccttctcaacaatgactgcgggctctaagaccatcagtgtggccatgttctccctcattccaccatcattcttgatttggcagatatactttccagcattagctggctctgcttttgcaaactgtagagttgcaacattttccacaaatgtaatcctgatgttttcactttctctaatcacttcttccttctctttaagccactggacaaaaataggctgggcgccttctatggatgcttgtaattcagcaggctctccggctacaacagtgaggctgttcagtttggagacaaatcttggtggttctttcaattttacagtacaaacacaagtatcacttcccacttcattctgtgctttgcagtggtattcaccgatgtctgaagtgtccacattgagaatgtgaatacttgtgtggaagtttttggatgcaatcttgtatttcttgctgcttctgagttgccgcttgtctttgtaccataccacctcaaacggtggtgttcccgaaagttcacattcaagactgacttcagcatttttaagggtttctactataggagggaagctgctaaaaacaggtggctcttttactataaccttggtactgcagcttgtgctgccagcgggattctgagcctcacaaatgaaatctccactgtcctcagtactgagattgttcatctgtatgacggccactgagtcaatgaaagtcattctgtacttatcactggctggaagttcatgttcatttcggaaccacacaactctgatttctggggatccagctatcttgcattcaagtcgtgaagagtcacctgctttcacaattttggaggcttctaatttctttacaaactttggtggttctgtcacaagcaacatcgtagtacaagagtcgctaccaacatcattggtaacatggcaagtatactgtccagtcttagaagcatccactgagtagagatttaagaagctagtcgacccttccaagccaatgaaacatttaggacctgagacaagttccacatcatccttaaaccattttattttaaatggtggtgttccttttagtattgccttaaattccactgtagaatcaggtatggcttgctgtcgcccaggtttcactaggaagcttggtggttctttcacagttaagatgccactgcatgcatcatctcctgctacatttgacactttgcatgtgtaatttgcagtatcttctaattccagattattaacttccagagacacagatctctcatggcacacaagtctgtattttgcacttgtagatatttcttttccatccttaaaccactgagcactaatgggaagtgaaccagacaccttgcactccatatgaatagaagagcccagaactttatccattttggttaattttttggtgaatgatggaggaatattttgatctagcactcttaagtaggcatcacagctactgcttccgaagtcattttccaccttgaaagtgtactgaccgctgtcctgcttcattactgactgaattctaaaactggccacgttattttcaaaactcattgaaaagtatctactgggaactatttgtttcccgtctttaagccatttcactttgagttctggtgttccagccacaacacattccaaggtcatgggatctttctccgtaacatcaactgatttagctttctctacgatttgagctggttcttgtactaaaaggaaagcataacacctctcaactcctgactcattcttggcttgacaggtatatctcccactgtgtccattatccacacttctgatttgaagtgtggccacactgtccacaaatgaaatatagacattatcatcttcatcaagaatctgatcatcctttagccaggttatagaaataggaggagaacctgccacggtactctgaaaggtggcagaacttttcaaaacagtagtggtattttctatcttcttaatgaatgatggtggttctttcagggcaactctagtactgcatgagcagctgccgccttcattggatacaatgcactggtattccccagtgtctgaagggtcacacttggttatatggaggttaaacacagacactctgtcggtcaatgtgtattttttgctgcttcgaatttccctgttattcttcagccaagtgacttcaaacggaggtgttcccgtaacttcacactccagctccacgtcactatattttactacctccacaggcttcagctctctgataaaggtggggggttctttcactttgagttcaatgctgcagctcgccgtgcctgcgtcatttcgagcttcacacacataagtcccactattttctaccctggcaccagaaatctggaaagtggctaaaccatcaatgaaggaaatgccatgtttctgaatggctgttatttcattcccgtctagataccaagacactcggattttaggagtgcctgttatttggcattcaaatgttgttgactgtccattcctcagcactaagactggactgggcttcttaatgaattgaggaggttcttttacaaagagagtggctttgctggttgctgtgccaacatcattgcttagttggcaaatgtaggttccagaatcggtagctttggctgcaaagagctctagactggtagaggtgtcatccttccaaactgagcgggctgctcctgagtgtaactctttgttatctttaaaccactttattgtcatgggtgcagtgccacccacaagagcctttaactgtacccttgtgttgggattgacatcttgtgactgtggcttttccacaaagtaagggggttctttgactgtcagatgcccactgcattggttgtgccctgccttatttgtggcagaacaagtgtatgtcccactgtctgtaccttccagctggctgatttccaagaaggcagtattgtcatgaaaagagaatttgtacttttcactagctgatatttcttggtcatctttgaaccactggatgcttatgggatgtgacccagccactatacattctaaatcaatgaaagaacctttaatgctgtccattttcttcagctttttggtgaatgaaggaggtatgataagatctaatacattaattctagccttgcagctgctcctcccaacatcattttggacctcgaaagtatattctccactatctttcttttctgtagaaataatcttcagtattgagactgtatcagtgacactgattttatattttgagcccagggtcagttcttggccatctttaaaccatttggctgtaatctccttagtccctgaaaatttaacctgcaaagtggctgggtctccttgggtgacatctatagacacagcttcctcggtgattgttgcaggttcttttactgagagtaatgcagaacatctttgtattcctgcatcatttttggcctgacagacatatttcccatcatgcttgacttcaatgccactgaggtacaaactggccacattgttctcaaaggtcattcttatattatcgtcttcagtgatttcatcgctgtcttttagccaagtcaccgtaattggcaaggagcccttcagagtggcctggaaggcagctgtgcctccccggagggagctggtactctcgatcttctttatgaaggatgggggttctcttaaagtcaccctggcactgcagatgctgctgcccacctcattggtcacccgacactggtattcgccagcatctgcagctacaaacttgaggatctgcaggctaaccagatgatcctgaatgaaagtcttatactttctaccacttcgcaggattgtgttatctttgaaccaagtgatctcaaagggaggagtgcctgccacctcagccagcaacatgacatcgtactcctttaagacttcaattggcttaaattccttggtaaaataaggtgactctttgactattacaatgctactgcagtggtcactgccagcctcattttgggcctcacacatatattcaccactgtcttcgatgccaacatctgtcagtcttagaactgcagtagactccacaaaagacattctgtgtttgctgctctccttaatttctctatcatttgcaaaccatgttattttaattggaggggtaccagttactttgcaggctagctgggtggcatctcccttctttaacagctgtgatggctctaacttttcaacaaatgtggcaggttcttttacaaacaagtttgcactgcattccacccctccagcgacattgctgactttacatgtgtacgtgcccgaatcagaggtttttactaaatagagttccagggaactctctaaagcttctttggtaatatagcagcttccaccagaaaccagctctttgttgcccttaaaccatctgattgtgagaggagtagatccttggaaagtgctcttcaggcagactgctgagccaggcagaacatcctttgagccgggtttagttacaaaactgggtggttcttgcacaatcagggctccactgctgtctttgcttcccacggaatttgtggctcgacaagtgaaattccctgcatcattcatgtctactctgatgatctccaaagaggctgtgccttccacaaatgctatcctgtatctgtcagaagcagctatttctttgccatccttaaaccaggacaccctcatggggagggagcctgcaattttgcagtccagtctgcaggtaccattaacaacactatccacgttgcgcaagggtttggtaaaaaatggagcaatgtctcgatctaatacagtgaatgtagtctcacaggagctgctgcccacttcattggaaatctcaaatgtgtattggccactgtcgtgcagctcagctgaataaaatttgagctgggcaacattgtttttaaaacttattcggtattttttactggcgaccaagggtctcccatctttgtaccatttgggcttcagttctggcgtgcctgccactgtgtactccagtgtggcgggatctcctgctgtcacctggatcagttctgctcgctcaatgattttggcaggttctttaactattaattccccaacagatgtttggcttccagcttcattttcagccaggcacgtgtatttgcctccaaaactaatctgaacatcagggattatcaagactgcaacaccattggaaaagctcattttgatttttccgtcttctctgatgacctcttgacctttcatccatgtgacagaaatgggctctgaccctctcacagcagcttgcagggtaacggtttgtcctcctagtgcaatcaaatcatctactttctttacaaaggttggaggttctttgagtaagtgggttgccatgcagccacacttgccgacttcattagcaacaacacattcatattcaccaacatctgcactattaaacgaaaagatctccagacacacaagagacttctgagaaaacaatctgtattttttactacttcgaatttgtttcttgtctttgaaccagctaatttcaaatggtccagtgcctgagacttcacactgaagtagagcatttgttcctctcactatgtctgcaggctcaagagttttgatgaaagaaggaggttctttgataactatttcagtactgcagctatcactgccgacgtcattcactgcttcacatgagtaactcccactgtcttcaacttttacatccgtaatatcaagtatagcctcagaattgacaaaatacattcggactgtgttactttcactgagttctttgttatttttaaaccaagtaacctggatcacaggtgagcctttcagcttgcaatggaggcgtgctgattcacctgggagcattaaataagagggatccaccttcttcacgaaggatggtggctctctgacagtgactgtggctgagcaggagctgcttccagcctcatttgaagctgtacagacataggttcctgaatctttcagtttggccaaaggaatctcaagtgttgctattttatcttcaaaacagatcttataatctttccctggggggagtttttgcccatctttgctccacgtaactgtgacttttctgtcttcatctacttggcactcaaggtggaccttcttattgatagcggactgcacaggctctaattctttaatgaaatgtggcttatcaatgatgatcaactctgcttggcagatgtctgctccaaacttgttggaagccttacaagaataaactcctctatcttgaatggtaaggtttgagagttctaaaatgtgtttgttttctgcgtcggaaatcctccagttaggtgaaggtgagagtgcagcaccatctttctgccaaatggtttctatcacaggagtccctgtcactgtgcagatgaacttggctgccttacccacaaaagttgtaagggacttaggtctggagagaaaggttggtggatatgcctctgtcacagttagtgtggctgtacagctgacactgccatactcattggaagctttgcatgtatactcgccgcagtcaaccacctgggttctcaggatttcaaggctggagatatactttgaagatcgaatagaacacttgtcactctcataaatttctcggccagctttaaaccactggaaccggacattgggagcactttggatctcacaggtgaatttggctaggtggcccagtgctacttccaggggttcgattttcctcttgatcactggggcagctttcatttccatctcaatctcttgttcaatcctctcatgcaaaattgattcaggagcttccagactcaggttggctgtgcttgatacttggcctacagcattactagcaacaaacgtgtaagttccttcatcttctggataagcttcggcaatttccagttgataagtgtcttcaaattgagtcattctaaagaaccgagatggcttgattttcttgtctttgctgtaccacgacacttttagatctgttccagaaacccggcattgaaaacgggctggctgcccttcagaagtgacagtgtcctgaagcggggtgatgatggcaggtggataaacaggcatttcctgatcaggagacacaacttctggaacttccactgagagtgaagctgatgttgtggcaacaccatagtcattcttggcttcacaggtatagactgccgcatcctctgggaaggcttcaattagcaaaagcgtgtattcttgcccatcatgaagaaatttgcacttgaagccagtggaaagcagctgctcttccttgtaccaggaaattttgggctgtggtcttccggatatcacggcacagaagcgggcaggcttgccagactgcacagtgacaggctggagctcctgcagaacttggggcggttcaggagcattgacatagagagtgacagaactcctgttccttcctgccacaaaggtgtattctcctgcatcgctctgtctggtctcagagataaacattcggtggattcttctttccactacatatttgtgtcgttcttgaacttggaaattgatttcaatgccatctttataccagtgggcatcaacatcgtcttcattgacctcaaattcaacaacagcacgctgtttctcaatgacctgaacctcctttttaatacttcggatgcgaacatctctgccttctacaaagagttttgcagttgacacgttgcctcctgccaccactgtgtacttcccagcatcagacatccgggtggatgggatcagaaggcggtggacatatttctccttctgaatctttattctgtctgtgatctgcagttcctggtcatctttcatccactgtacagtgatgtcaggttcagaaacttcacattcaaacatggctcgcttcttctccagtaccttaatgtccttaatgtgtttcctaaattctatatgacgagcttccacataaagtgtggctgttgatgttgcttttccagccacaaaggtgtagtcagcagcatccccaaagtgaacattcctgatgttcagtgagtgtgtgagctttttggttctcatctggcacttgtcagttgatttgatttccacaccattctttaaccatttgtaagagatgccttcatagttcactgtcacctcaaaagtaatagtgtctttttcttcagcgttgatgtctttcagcatggaagtaatcatgattggggtgactgtcagggtggcactgacttggtcattgccacagacaaatgtgtattctgccgagtcctctgtgctggtgttcatgatgatcagctgatggagttttccctgcacaactatcttgaacttttcactcatctcaatttccacaccattcttcagccacatggaagggacattgaagtgggacacctcacactcaaaagaggcagttttggtctcaggcacctcgatatttttcatggtttttgtaatatgtaatgtctccacaaacagttttgctttgcattccaattgcccgaccacagctgtgtattccccagcatctgagggggagatgttctgcagcatcagcttgtggactttcctttctgagaccagtctgtgtttgtcacttggcttaatttccacactcttatggaaccattttactggaacagtgtcatgggaaacactaacttcaaaggcaacagtggcattttccaaggctgtcacatcctttggctttttaatgatcttgacagtctccacgtgcagtctggcactggctccaagccttccaagcctgaagccataaacagactcatccacgatggcacagtttttaatcctcagagagtaaattgttcctttgacagagatagcatacttttcattggattccagcacaactccatttttgatccactggacacctttgacattagggtgtgtaagctcgacagtgaaaacagcatcctgtgtttctgtcactgtgaggttcttcagagtcttcttaattttgacagcttcaactttgagtttggcagatgttttggaggtggccaccttgtaggtatattctccaatgtcatctaatttggtggcagcaatgataagtctccttttgtggccatcagactcacttctgatgttgttagtcagtggtaggtgtttgccatccctcaaccattcgcctttggaatctgggttggcaacttcacattcaaacacagcttcctgggattcagctacggtctgatctgtgagtggcttggagatggccccacctgccacagtaagttttccagatgtcatattttctcccgcgtaaaatgtgtattttccttcatcatctttcatcatatttagaactgtcaatttatatatttttccatgtgcttcaattttatatttagaactgggcttgatttccttgtccttaaaattccacaggacatcaattccagagtgggacagctcaacctcaaacaccacattttgagtttctgtacaggtaaggtcacgaagacctctgataattttaattttttctacagagagattacagttggtttcaactctgccaactatcagcttgtaaggtccttcgtctgaagcatgagttcggttaatgactagtcgctgtttagtacctttcacaatggcctgtacacggtcatcaggcttgatttgttcatcatttaagtaccacttaacagaagtcacatcagggactgacaccttacattcaagcacagccttggtgccttcaatcacattaacatcttttagaggtgttatcacgtccacactatagacagagacacgcccactggtggagaggccaagggctggaatggtgaaagagtaatttccagcatcttccttagtcatgtcttcaatgagcagcatatgagattgtttgtctatcacaatgtgaaccctgtcactgggctgcacttcttggccgtctttcatccagacgccttccacactttccaaggagactttaacttcaagctgaacaatgtcaccctcacagactttttggtcactaagtccttgtaggatagcaatggggcggggtttcatctttaatttacaggttgtctttttcccgtcgatgacaaagctgtattctccctggtcctccttggttacatccttgaccgtgaggttctgacgtccacgacgagatgtaattgtatatttgccattggatttaagctccacatcattatgataccattttccttctatattttctggggatacaatgcactctaattctcctgaatatgattctggaacttctatgtcctgaagttctttcacaaactcaacaactgcaccttcaacaataagtttagcagtcgttttgacattttcatcttccacaagtacacagctgtaatcttcagcatcagacgtatcaatggtcagtatggagaggaagtgaacctttctgtcagagtgcatcctgtatttatctccctcatgaacctccataccatctttataccatttcactttgacaaatggttctgaagtttcacattcaaaggttgccatagtgtctttttccttagcaacaacatcttgtaattcctgtgtgaaagtgatcaattgcttggcttggacaagtaagaatgcgtgactggaggtttctccagctatgttgatggcttttaccatgatgctggcagagtcctcagcagtcacatctcttatgaccaattcacaaacattgtcttcgggccagtaccagtagatccggtcagaccgttcaattttgacaccatttttgtaccattcacattcggggtctggtttccccacgactctgacccggaagtgtgcatcagatccttggcccactgtttggctctggattctttcgaagatttttggagcctccatactaggacttagttcaatcttgtcaggtttaaaagttggaatcgtgattttgccttcttcggcaagagctttcttttcctcttcagttaactctttggtccagtggagaagttcatcttttgtcttcctgaggagttcctcataggattcatccttctttcgagacttgagctccacagcggtaatggcttcataatagccctcttctgttctgcgcttgaatttactgcgcagctcttccgactcttcaggcactttttcatgggtaattctttcagcccttttcaacttcacaacttctttggtttcagtggtgtcaacaggtctatccactttttgtacttcaaactgaagctttcctggttcatgtacgtgaaactcaggccttggttcaggagctctcctaaggacagacctaaaatcttccctctgttgaatctcaagcttcactttatgctctatcacaccttcaggattttccgcggtgaccttcacttcacctgtgtcatatgatttgcagtccacgatgtccaggtaatggataccatcatagcgaactctgaaccttttgcttttgcggatgagctgtccattgaggtaccagttgactttgggctgagggtagcctgttaccctgcagcggaaccttgcagtctccccttcaagtactctaactggctctgggtacaagacaatgtctggcttttgcttttctttctgatctgttgttacacctgtaagtgcaccttcatgagccattctctctaattcttcaattctctgtaagcctttcctcccctcaggcaattgggattcttccacaagacttttctcatctttaacaataagggtagcagatgtgtgatctgttccatatttgttagtggctctgcaagtaatgataccactgtctctagaatatgcaacgccataatcaaggctgcagtacccaaattcattgatcatacggagcctgttggctgcttcaagtggctttccatcatggagccactccaccaccatcgttgggtcaccaatgggtgttagcctgcattcaaagtgggcaggcccaaagcgcttaagtcttaaggaagtgagttttttcttgaaaaatggtttctgttgtttctctttgtcatagagatcaccttcttcccattgctcttggccatatcgcaaatggaggggctccagttctggggctgcaatctcctttgctctatatgtcccccgtgggatgattaactttctctctggctcaggctctgcaaactcaacttcaacatttactttgcatcttgtagtgtctctgccagctttattaatagcagtcgcagtataccaggcagaatcttggctgacagtggaatcgattttaagggcagcttctcccttggttccttcaattctgattttgggatatttatgaggcacaatgatgtcactgtttttcaaccatacaatgtcagggttggggttacccgtagctctgactttcatttcaagtcgggaaccttcctttatattgacatttttcagtttttctacaaacatcggttttacctgatgttccacagcttccacagttaaaatcactgaaattgaagatctgcctgccctgttttgggcaaccacagtccattccccagaatcactgggtgtggcagggacaataattagtgattgagtaccatcttctttaatgactactttatgggtatagtcattgacaatttgctggccatcatgaaaccagaacgtctctggcataggtctaccaacaacctttaagtcaaatctggcagtttgcccttctaaacatttgaaagaaacaggttttaacacaaagactggtttatatagtctctcaagttgtgactcatctgtctcctccagcctacgtccaggggacattcttgcaggggacatccgtgcaggagacatccttgcaggtgacatccgtgcaggagacatgcgtataggagacctgctcactgaacgtggagagagagatctgattctgctcactggctctagtgtgggaatgtaagtcggagctccaagtggtgcagcaggctccacatacaatttccctgagcaaattgcatttcctttaatattgctggcaaatgcagtgtagattccttcatcttctggaagaacaacaggtatacgcagactagctctgccatcttgtagaaagtccatttggtatctttctccatgtttgatgcgcttgccatctttgtaccaagcaatctttggtaatggatatccagacatcttgcaatgaaaagtgacacccatcccctcaagaattctataattcttgattcttgaatcaaatcctgattcaacagcttcagattcagaaatgtcaactgccatcttttcttctccatcttcttcaagaagttcttctaatgtagtctttattattctatattcaatttctttaataagtctctcttcaaaggaagaaatatggaattcctgatcttctacataagttctgaccactacagtatctttggccattttcttcctaattaaggcttgttctttttcatactctttttcatactcagagtatacaaatccaggtgctgtttctccaactttaggttcttgaacaaatgcagtcacttgtgtctgataaagcatttcttgctgggacttcatcagtaactcataatcagcttcttcaagcaaggaagcagatgcagaagtttctccatgcttattgcgaacaacaatagtgtattctccagcatcatcagcaaaagtcatagaaatcaccagcttgcattcaccggtttgtttgttgtaactcactttgtatctgtatccagtggttagaggaacaccagattttttccagtatacatggggctttgggttgccgccaacttggcatccaaacaccacgctcccaccttccaccagtttctggaccactggttttgtaataaagtaaggcgcggcaggttctccaggccctgcttgttcctctgtgaggctagtatcagtcataaccacatctcttgactcaacaaagcgtttctcttctgtagtaaatttctcagtcacggctgtggtttccttttcaaattcttctgacacctgcacagccagatagcaggatgtgctgacggttccagcctcatttacagcactgcaagtaaatcgcccgctgtcttccgcaaatgcttcgcgaatcataagacgagcaattccactctggaaggttatctggaagtcaatggaactttcgatttggtagtcttccctgtaccatgtcactgtcggggatgggtatccagagatgtggcactccaaggtgacagattcaccttctatgacagtcacattttttaagcccgagaccaaagttggtggagtaacaggaatttcaacaggtgctggtactcttgctgtttctgttaccttggcttcgcgtccgtgcagtacttcaaagcgctcttcacggacggtggtgccagtgatgctcacccctacttcctttttcacctcaacgccagcttcactcttgtaagtatctggtgtgtcagcgaaggggaactgtggcaagggtgtgggctctgcccttactctagtctcactgggcttcacagtaggagccttcaccgatttggtgatcttctgagcagaagatgtggctgacaactctttttgtaatgtggcaatagcactaccggctattgatgcctcatatccatgttctgtcttaggaacagaaatttttgaaacagtaaagtgagggctagctgtgcgggggcgtttatccacatggactaatctttccgttgttagatctgtagttttcttgatctgtgatgatatgtgcattcccttttgatcagtagttttgatatgagtctcagaaggagcctggattactctaggcttgactgctttagggacaacgtggggttctgaggctggacgttggggaggctcagctacctttgcggcggaaatgcgttccttatatccgtactccaaagtggtctgctgagcataggattcttcaagatgcccaggctctctgggctctctgactcgggcctggtctactgcagcaacaactgttgctacagcttcagccttttttccaacgtccacctttccatgggtaacttggatttgttcttgtctagtagccatagtttctctagttctcagtattgtttcttgttctttggctttagcagtagcaactgctattgtagacaaggcagttttctcggcttcctttctcatcttctcctgagttatttgcacttgttctcttttggtagtaatgccttctctacctcttgatactaaatcttgttctttgactttgggtgtggcaactatgactttaggtacaactgttttcctagtttccttcattatcttttcataacttaggtgcatttgatcttgttgtgtggtagtttcttcttgagctcccgggactgtttctagttttgtggactttgcagtggcaactaccaccatggatgcagcagttatctcagtttcctgtcttattgcttcttgagttacttgtttctgtttcttagtaatttcttcagaaattctagtttcttgttctttggctttagctgcggaaattactacctttggtacaaatgttttttcagtttcttttcttatctgctcatgagttacgtgcatctgctcttgctttgtggtaattacttctttggttcttgattttaattcttgttccttggctttatcggcggccactactaccttagttacagcagtcttctccgcttcctttcttacctgttcttgagcaggttggatgtgcacagcagtcgtggttgtcctctgagcagtctgctctacagcgctgatcactggttctctcactctggccatatcaacggcagcaacaacagtcgcaacagctgcacttttgtcagcatcttgtttcacctctttagcaccagtggcaacagcctctgctgcgtagctagcactggccgacacactggcggcagcacccgcagcaccactgatggtcacttgctcctggacaccgtatctcccttcccatctctcttctgtcctgatctgagtagaggttgtcagcgttgtctctctcatctcagcctcagatgaggaggccacgtagccctcttgcttccaagggggaggcacttcaggacctgtggccacggtggatgcctgagtcttacgcatgagcaatggagacctaacagacctgatgggggatgtggagattcttgctgctggagacacggacctgaccggagatggggtcggtgcccgcacgtgtctgaccggggaaggggagtgtcttatgggcgatggggactgctgccgagccagctgtgctttggcagcaatagacggtggtgttggggatcttgactttggcttcggaggaatcctgggaggtgttttatgtggcagctgttgcccagcggcaccatctatgaccatctcaactgttgcaattgatctggcatcaaagtgggcttcaatcttcttttcaattcgggtttgtcttgattctgagatctgagcagtcgaaacaattgtctttgtctttttagcaggtacttcttcttcaccttgaaccagtaattcagcagtcgaagtagctcttccaacgctattggtggcatttactgaataggtccctgagtcctcagggtatgcttctgcaatcagtaagctgtagaggtcgccttcttgtgaaatttggaaatcaagggagctctggatttcggctccatcccggtagaacttcaccacaggtgtagggattccagtcactctcacttggagtctcacttggcttccttgtctcacggtcatgctctgcagtcgttgaacgaagttgggtggtgctgtctcagctttcacgagaagctcagcagtactagtcgcttgtccagatccattggtggctttcagggaatatcgtccactgttggctttagtcacggcggggatcgtcagtttagcgcggccatcgctaaaggagatctgcacgccgggcagagtggaagtggaaatcacctggccatccctaaaccagctcacctcaggaactggaaaaccactaatgtgagcctcaaaggttgcggtactaccctccagtaccacaacgctttgtaacggctgcgtaaacgtcggtgcttgagttgtcatctttctaggcactctgatttctcaagagtgcctaaaaagggtgggactaagcccaaggttgcttctgaaacgacgtcctatggagagttggtttttctgaccatctccgacatgaatcggtgagcctctaatcctaaaaacaaaactacacagtcaagactgtgtagttttgcttttctatgcaatccctacacccgaggcgaggctgggaatgcacgactgctc

SEQ ID NO: 10303 - RNA, 29 nt, Homo sapiens
  source 1..29: mol_type = other RNA
ccaaaccagtcgtgcctgtgggcacaacc

SEQ ID NO: 10304 - RNA, 66 nt, Homo sapiens
  source 1..66: mol_type = other RNA
ccaaatcttgatcagaagccttcctagcttctgatcaaggcttctgatcaagatttggggtatcag

SEQ ID NO: 10305 - RNA, 2824 nt, Homo sapiens
  source 1..2824: mol_type = other RNA
ccaatattggctgtgctgctccagggcaccaggccacctccaggcatgcagagctgctgcagactgtgcctggtctgcagaggaggcctctgccctctgggagcagctccaggctccggtctcagggcagggcccagggtggcttgagcgggccctccttcccggcctccttcagagggaacctgtccacagcacccccacgcacaccaagtccacctccatctcccctgccctccagttcccatgtgctcctgatgaccagccaggtcaggctgactctaccctccccgaagggagagggccttcaggtatcctctggattgaattaccccagttctgacctggttccaagacacatttgaggacctcactgaccaaatcagaccttggcccctgcctagccatgtgtgtgtcctctggaatcaacatgccaggaaccagccccttatgtcagctggaggccccagcaggattataaacagcacctgctggttttaaggttgctacatggcctgggaagtggagttgggaggactgtgtgctaacaatggaggacaaatgacagcaaagtaacactcaggcttgggtgatgccctgatgcaggtaacagggtggctcctggcctgtgcatgggaccaggagccagggcccatgggccacgtcccgcgtgtctgcagcccctggcctcagcctgggcctctggcccacagcccctgctggctgcctggcagtccccggacacctctgcactcctctccacccttttgtcccttaggcccatgagagatgttttcagaagacggttttcctgtcttccgatcattagaacttgtgggggcagctcctcttctggcgtttcacagagcccttgggccctcactgtacacctgctgtctcggaccctcccttcccacctgtccagctgttccccgggcatgacgtagcctgacatgtgcccttttcacccagtcactcatgcattcatccacaatgtgctttcctagcctgtgccggcatcgcgctgcatcctggggtgtaaggcccctgcccacaaggctagcacactgggcgcagagagactctgagtaaggacatggtttaatgggataactagagatggcggtaaaccaatgcagtggctgagaagcctctccaggtgggtgaagtgaggaacgggggtgcaaagaccatgggtgggaatataacttggccgtggtgagtgagaattggggggtgaaggccgaccatgcacagcctcaggctagggtagggcatagggatttcactctctgtgtctctgcagcgtggtaagcaggggaacggtatgatgtggcttaggttttaagtcatcccgtctggctgctgtgtggagtggttacaggggagcaggagtccagctgggggcccacagtgcccaccaggagctgctgagagaacatgttcaacgaggtccgggaagtgactgctcgattctgccaaaagagggatggcgcatgggtgacctgacaggagaattcagtggcatcctggtaacaagtggcagagtttgccaggggggaggcaaaggagtggatgaggaagtgaaggggcgttgatctaggggtatattcgtgtactgatgggtggcttcctggtgctgctctgacaaagccccacaaacctagtggcttaaaacaagcagggcgagaaggctgacttccaggtgtgggccacgctcctgccagaggttccaaaggaggatctgttgcctcttccagcttctggtggccatccttcattccttggctgtggcctccaccttcaaacggccttctctgcagatttatcttctaagagtgcaaatgcattaagaggccgcccagataatccaaataagctccttctctcaagatccacagaaagcagtatttgtggggttttggttggttgttttttgttttggccatataagggaatagtcagaggttctgggaattaaaatatggacatacgttttgcagggggccatcatccaacccattaccatgggaatgatctgagcgggacacagatggccaggtatctgtcgactgccacggccagaaggctgaagatggagctctgcgtgagcaccagcacgaagcaggcgaggaagaggcagccgtagaagtcagtgcagaagcccaggctgatggtgatggcaaaggggatggcgaagagccccacggccacgtcggccgcagccagggacaccaggaagtagttggtgggcgtctgcagagtgttcgccgtgcccaccgcggcgcacaccagcacgttgcccgccaccgaaagcgcggcgatgaccagctccagcgccacgtacagcgcgtcctgtgtctccagcagcatggccgggccagctgggccccgggcgccccctaccgaaggcgcgccgggcgaggggcagccgcgtgagacccgccgggcatggccatagcgcccggaccgcgcctccgcctgccgcttctgagcctcggggctggggcgctggtggccgggacccacgggtcggggccccccgcggccaagaggcggcacccattggcccgcgcgcccgcccgtctcgggctgggcggagcaccacccactcgcccgagcccaaagttcgcgcccgcgcggggcccctccggtccaggcgccgtgccgcgtcttggtggcggcggataactaacaaattgccccaacttcccgtcacgctcgagctcggaggctgtgtcccagtgctcgcactgccttccagtccgggcgactcctgggatggggccgggctctgcccggggcgccagcaggtcccaggagccgc

SEQ ID NO: 10306 - RNA, 1088 nt, Homo sapiens
  source 1..1088: mol_type = other RNA
ccaatattggctgtgctgctcccctttcagtggcaggcctttgatggcttcagaaagctttgagtggacagaggcctggttcctgctttctaccacatcctgcatattttggagaagcccagtgttctgaggggctggagtgcccagtttctgctgcctgcttctcatttccagctcttctgtttcaggatctgaaaaccccaggtagattttctctgtcgccttctggagtttctccagaccctgctgatcacctaattctctcctgcattgggctggggccctgcctaagattttctccatgtcagcaaagacctggtggatttgggaaggttggcctttggagagtggctgcagctttctgggaagggcacccatgaaacgccagggagtgtcacccagcatgcctgggctctttcctttgttataggatccctcacttatagcctgcatctcttgatctaggtccagatcagcaagcccaggtgctgacggaggagacaagctgcagagaaaggatgaaggaggcagaagtccctcctcaggctgcgtttccagcgaacttttgggggggtctctgtccttcttgtctttcttttcctttttttttttcttcttcttaatggccccagaagttgacagctttgcccgctcttggatcaccaagctccgatagtgttcgtcacatggatggtcccacatagactgcccgttggcgaagttgaaatagtaaatgtcacctgtgatgtcctggcatggtttccactctccaggcagtggggccacgatgccctctcgcgccagccacatcagttctggttccttgatgggatcaataccaatctcccgggcaaattcaagaatttccgccagacccccagcccgggcccggtggcccgctcaggagccggcgagatttcaaacggaggaactgtcgcctggcagtccgattttcacttcttccctcagtccccgcccacactcgagcgcatcacgctcgttggctcgagagcgtgcctcgggtcccccgccacgctcgctcccttccccgccgcccaacccctccctcgatgaggtcctcaactatc

SEQ ID NO: 10307 - RNA, 1164 nt, Homo sapiens
  source 1..1164: mol_type = other RNA
ccaatattggctgtgctgctcccctttcagtggcaggcctttgatggcttcagaaagctttgagtggacagaggcctggttcctgctttctaccacatcctgcatattttggagaagcccagtgttctgaggggctggagtgcccagtttctgctgcctgcttctcatttccagctcttctgtttcaggatctgaaaaccccaggtagattttctctgtcgccttctggagtttctccagaccctgctgatcacctaattctctcctgcattgggctggggccctgcctaagattttctccatgtcagcaaagacctggtggatttgggaaggttggcctttggagagtggctgcagctttctgggaagggcacccatgaaacgccagggagtgtcacccagcatgcctgggctctttcctttgttataggatccctcacttatagcctgcatctcttgatctaggtccagatcagcaagcccaggtgctgacggaggagacaagctgcagagaaaggatgaaggaggcagaagtccctcctcaggctgcgtttccagcgaacttttgggggggtctctgtccttcttgtctttcttttcctttttttttttcttcttcttaatggccccagaagttgacagctttgcccgctcttggatcaccaagctccgatagtgttcgtcacatggatggtcccacatagactgcccgttggcgaagttgaaatagtaaatgtcacctgtgatgtcctggcatggtttccactctccaggcagtggggccacgatgccctctcgcgccagccacatcagttctggttccttgatgggatcaataccaatctcccgggcaaattcaagaatttctctcctccttagcccaatatactctcaggtcctattctcattctccagctctcagtccaaataaagttatttctcccgccagacccccagcccgggcccggtggcccgctcaggagccggcgagatttcaaacggaggaactgtcgcctggcagtccgattttcacttcttccctcagtccccgcccacactcgagcgcatcacgctcgttggctcgagagcgtgcctcgggtcccccgccacgctcgctcccttccccgccgcccaacccctccctcgatgaggtcctcaactatc

SEQ ID NO: 10308 - RNA, 961 nt, Homo sapiens
  source 1..961: mol_type = other RNA
ccaatattggctgtgctgctcccctttcagtggcaggcctttgatggcttcagaaagctttgagtggacagaggcctggttcctgctttctaccacatcctgcatattttggagaagcccagtgttctgaggggctggagtgcccagtttctgctgcctgcttctcatttccagctcttctgtttcaggatctgaaaaccccaggtagattttctctgtcgccttctggagtttctccagaccctgctgatcacctaattctctcctgcattgggctggggccctgcctaagattttctccatgtcagcaaagacctggtggatttgggaaggttggcctttggagagtggctgcagctttctgggaagggcacccatgaaacgccagggagtgtcacccagcatgcctgggctctttcctttgttataggatccctcacttatagcctgcatctcttgatctaggtccagatcagcaagcccaggtgctgacggaggagacaagctgcagagaaaggatgaaggaggcagaagtccctcctcaggctgcgtttccagcgaacttttgggggggtctctgtccttcttgtctttcttttcctttttttttttcttcttcttaatggccccagaagttgacagctttgcccgctcttggatcaccaagctccgatagtgttcgtcacatggatggtcccacatagactgcccgttggcgaagttgaaatagtaaatgtcacctgtgatgtcctggcatggtttccactctccaggcagtggggccacgatgccctctcgcgccagccacatcagttctggttccttgatgggatcaataccaatctcccgggcaaattcaagaatttctctcctccttagcccaatatactctcaggtcctattctcattctccagctctcagtccaaataaagttatttctcccgctcccccagcttccag

SEQ ID NO: 10309 - RNA, 1294 nt, Homo sapiens
  source 1..1294: mol_type = other RNA
ccaatattggctgtgctgctcccctttcagtggcaggcctttgatggcttcagaaagctttgagtggacagaggcctggttcctgctttctaccacatcctgcatattttggagaagcccagtgttctgaggggctggagtgcccagtttctgctgcctgcttctcatttccagctcttctgtttcaggatctgaaaaccccaggtagattttctctgtcgccttctggagtttctccagaccctgctgatcacctaattctctcctgcattgggctggggccctgcctaagattttctccatgtcagcaaagacctggtggatttgggaaggttggcctttggagagtggctgcagctttctgggaagggcacccatgaaacgccagggagtgtcacccagcatgcctgggctctttcctttgttataggatccctcacttatagcctgcatctcttgatctaggtccagatcagcaagcccaggtgctgacggaggagacaagctgcagagaaaggatgaaggaggcagaagtccctcctcaggctgcgtttccagcgaacttttgggggggtctctgtccttcttgtctttcttttcctttttttttttcttcttcttaatggccccagaagttgacagctttgcccgctcttggatcaccaagctccgatagtgttcgtcacatggatggtcccacatagactgcccgttggcgaagttgaaatagtaaatgtcacctgtgatgtcctggcatggtttccactctccaggcagtggggccacgatgccctctcgcgccagccacatcagttctggttccttgatgggatcaataccaatctcccgggcaaattcaagaatttcttgctcactaggaatgtaggtctcatcataatcttcttccagaaccagctgatctcctatgcggaggggtcgtccagccatgactcatctgggctcaaacacccgccagacccccagcccgggcccggtggcccgctcaggagccggcgagatttcaaacggaggaactgtcgcctggcagtccgattttcacttcttccctcagtccccgcccacactcgagcgcatcacgctcgttggctcgagagcgtgcctcgggtcccccgccacgctcgctcccttccccgccgcccaacccctccctcgatgaggtcctcaactatcccccaccccggaaggctccgggcgaggctccgggcgaggctctgggcgaggcgcagctcccccaacgccacccaacacccacccgctcccccagcttccaggg

SEQ ID NO: 10310 - RNA, 1366 nt, Homo sapiens
  source 1..1366: mol_type = other RNA
ccaatattggctgtgctgctcccctttcagtggcaggcctttgatggcttcagaaagctttgagtggacagaggcctggttcctgctttctaccacatcctgcatattttggagaagcccagtgttctgaggggctggagtgcccagtttctgctgcctgcttctcatttccagctcttctgtttcaggatctgaaaaccccaggtagattttctctgtcgccttctggagtttctccagaccctgctgatcacctaattctctcctgcattgggctggggccctgcctaagattttctccatgtcagcaaagacctggtggatttgggaaggttggcctttggagagtggctgcagctttctgggaagggcacccatgaaacgccagggagtgtcacccagcatgcctgggctctttcctttgttataggatccctcacttatagcctgcatctcttgatctaggtccagatcagcaagcccaggtgctgacggaggagacaagctgcagagaaaggatgaaggaggcagaagtccctcctcaggctgcgtttccagcgaacttttgggggggtctctgtccttcttgtctttcttttcctttttttttttcttcttcttaatggccccagaagttgacagctttgcccgctcttggatcaccaagctccgatagtgttcgtcacatggatggtcccacatagactgcccgttggcgaagttgaaatagtaaatgtcacctgtgatgtcctggcatggtttccactctccaggcagtggggccacgatgccctctcgcgccagccacatcagttctggttccttgatgggatcaataccaatctcccgggcaaattcaagaatttcttgctcactaggaatgtaggtctcatcataatcttcttccagaaccagctgatctcctatgcggaggggtcgtccagccatgactcatctgggctcaaacacctctcctccttagcccaatatactctcaggtcctattctcattctccagctctcagtccaaataaagttatttctcccgccagacccccagcccgggcccggtggcccgctcaggagccggcgagatttcaaacggaggaactgtcgcctggcagtccgattttcacttcttccctcagtccccgcccacactcgagcgcatcacgctcgttggctcgagagcgtgcctcgggtcccccgccacgctcgctcccttccccgccgcccaacccctccctcgatgaggtcctcaactatcccccaccccggaaggctccgggcgaggctccgggcgaggctctgggcgaggcgcagctcccccaacgccacccaacacccacccgctcccccagcttcc

SEQ ID NO: 10311 - RNA, 1385 nt, Homo sapiens
  source 1..1385: mol_type = other RNA
ccaatattggctgtgctgctcccctttcagtggcaggcctttgatggcttcagaaagctttgagtggacagaggcctggttcctgctttctaccacatcctgcatattttggagaagcccagtgttctgaggggctggagtgcccagtttctgctgcctgcttctcatttccagctcttctgtttcaggatctgaaaaccccaggtagattttctctgtcgccttctggagtttctccagaccctgctgatcacctaattctctcctgcattgggctggggccctgcctaagattttctccatgtcagcaaagacctggtggatttgggaaggttggcctttggagagtggctgcagctttctgggaagggcacccatgaaacgccagggagtgtcacccagcatgcctgggctctttcctttgttataggatccctcacttatagcctgcatctcttgatctaggtccagatcagcaagcccaggtgctgacggaggagacaagctgcagagaaaggatgaaggaggcagaagtccctcctcaggctgcgtttccagcgaacttttgggggggtctctgtccttcttgtctttcttttcctttttttttttcttcttcttaatggccccagaagttgacagctttgcccgctcttggatcaccaagctccgatagtgttcgtcacatggatggtcccacatagactgcccgttggcgaagttgaaatagtaaatgtcacctgtgatgtcctggcatggtttccactctccaggcagtggggccacgatgccctctcgcgccagccacatcagttctggttccttgatgggatcaataccaatctcccgggcaaattcaagaatttcttgctcactaggaatgtaggtctcatcataatcttcttccagaaccagctgatctcctatgcggaggggtcgtccagccatgactcatctgggctcaaacacctctcctccttagcccaatatactctcaggtcctattctcattctccagctctcagtccaaataaagttatttctcccgctcccccagcttccagggacgccggggtgttgccctgcagcgcgcaacaaacacttccggaaaaggtaccgcctagcaaccgggagtcccgcctccagcaggagccaataggtcgccggctgagagctgtgacaatggattggctcgaagtcccttcggtgcacgcaggagctctgtccgttttccgttgcacgatgggagtgtagtttaagatagataatgggaatccgcaagaggttgaaagagtgtagtttaagatagataatgggaatccgcaagaggttgaaagagaacctcatcggctgggcgcggtggctcacgcctgtaattccagcaa

SEQ ID NO: 10312 - RNA, 1233 nt, Homo sapiens
  source 1..1233: mol_type = other RNA
ccaatattggctgtgctgctcccctttcagtggcaggcctttgatggcttcagaaagctttgagtggacagaggcctggttcctgctttctaccacatcctgcatattttggagaagcccagtgttctgaggggctggagtgcccagtttctgctgcctgcttctcatttccagctcttctgtttcaggatctgaaaaccccaggtagattttctctgtcgccttctggagtttctccagaccctgctgatcacctaattctctcctgcattgggctggggccctgcctaagattttctccatgtcagcaaagacctggtggatttgggaaggttggcctttggagagtggctgcagctttctgggaagggcacccatgaaacgccagggagtgtcacccagcatgcctgggctctttcctttgttataggatccctcacttatagcctgcatctcttgatctaggtccagatcagcaagcccaggtgctgacggaggagacaagctgcagagaaaggatgaaggaggcagaagtccctcctcaggctgcgtttccagcgaacttttgggggggtctctgtccttcttgtctttcttttcctttttttttttcttcttcttaatggccccagaagttgacagctttgcccgctcttggatcaccaagctccgatagtgttcgtcacatggatggtcccacatagactgcccgttggcgaagttgaaatagtaaatgtcacctgtgatgtcctggcatggtttccactctccaggcagtggggccacgatgccctctcgcgccagccacatcagttctggttccttgatgggatcaataccaatctcccgggcaaattcaagaatttcttgctcactaggaatgtaggtctcatcataatcttcttccagaaccagctgatctcctatgcggaggggtcgtccagccatgactcatctgggctcaaacacctctcctccttagcccaatatactctcaggtcctattctcattctccagctctcagtccaaataaagttatttctccgtttatttctctctgtatctccagcgcctggcagtgtgcctggcatacagtgggtgctccttccatgctgaaagaaagactgacagacgggaggtgtgcccctctccatccgtctggcccttcccgccagggccttgcagggcggactccacctcggcagagggcatcccagacccctctccagccc

SEQ ID NO: 10313 - RNA, 1168 nt, Homo sapiens
  source 1..1168: mol_type = other RNA
ccaatattggctgtgctgctcccctttcagtggcaggcctttgatggcttcagaaagctttgagtggacagaggcctggttcctgctttctaccacatcctgcatattttggagaagcccagtgttctgaggggctggagtgcccagtttctgctgcctgcttctcatttccagctcttctgtttcaggatctgaaaaccccaggtagattttctctgtcgccttctggagtttctccagaccctgctgatcacctaattctctcctgcattgggctggggccctgcctaagattttctccatgtcagcaaagacctggtggatttgggaaggttggcctttggagagtggctgcagctttctgggaagggcacccatgaaacgccagggagtgtcacccagcatgcctgggctctttcctttgttataggatccctcacttatagcctgcatctcttgatctaggtccagatcagcaagcccaggtgctgacggaggagacaagctgcagagaaaggatgaaggaggcagaagtccctcctcaggctgcgtttccagcgaacttttgggggggtctctgtccttcttgtctttcttttcctttttttttttcttcttcttaatggccccagaagttgacagctttgcccgctcttggatcaccaagctccgatagtgttcgtcacatggatggtcccacatagactgcccgttggcgaagttgaaatagtaaatgtcacctgtgatgtcctggcatggtttccactctccaggcagtggggccacgatgccctctcgcgccagccacatcagttctggttccttgatgggatcaataccaatctcccgggcaaattcaagaatttcttgctcactaggaatgtaggtctcatcataatcttcttccagaaccagctgatctcctatgcggaggggtcgtccagccatgactcatctgggctcaaacacctctcctccttagcccaatatactctcaggtcctattctcattctccagctctcagtccaaataaagttatttctcctgtagtctcatctacagaggctgatgtggaagggtcacttgagcacaggaggtcaaggctgtagtgagccatgatcatgccactgcactgcagcctgagtgacagagcaagaccccatctct

SEQ ID NO: 10314 - RNA, 1323 nt, Homo sapiens
  source 1..1323: mol_type = other RNA
ccaatattggctgtgctgctcccctttcagtggcaggcctttgatggcttcagaaagctttgagtggacagaggcctggttcctgctttctaccacatcctgcatattttggagaagcccagtgttctgaggggctggagtgcccagtttctgctgcctgcttctcatttccagctcttctgtttcaggatctgaaaaccccaggtagattttctctgtcgccttctggagtttctccagaccctgctgatcacctaattctctcctgcattgggctggggccctgcctaagattttctccatgtcagcaaagacctggtggatttgggaaggttggcctttggagagtggctgcagctttctgggaagggcacccatgaaacgccagggagtgtcacccagcatgcctgggctctttcctttgttataggatccctcacttatagcctgcatctcttgatctaggtccagatcagcaagcccaggtgctgacggaggagacaagctgcagagaaaggatgaaggaggcagaagtccctcctcaggctgcgtttccagcgaacttttgggggggtctctgtccttcttgtctttcttttcctttttttttttcttcttcttaatggccccagaagttgacagctttgcccgctcttggatcaccaagctccgatagtgttcgtcacatggatggtcccacatagactgcccgttggcgaagttgaaatagtaaatgtcacctgtgatgtcctggctaatctctagatgttgatgtataatcactggagttcttgagaatgcaggctggacatggtttccactctccaggcagtggggccacgatgccctctcgcgccagccacatcagttctggttccttgatgggatcaataccaatctcccgggcaaattcaagaatttcttgctcactaggaatgtaggtctcatcataatcttcttccagaaccagctgatctcctatgcggaggggtcgtccagccatgactcatctgggctcaaacacctctcctccttagcccaatatactctcaggtcctattctcattctccagctctcagtccaaataaagttatttctcccgccagacccccagcccgggcccggtggcccgctcaggagccggcgagatttcaaacggaggaactgtcgcctggcagtccgattttcacttcttccctcagtccccgcccacactcgagcgcatcacgctcgttggctcgagagcgtgcctcgggtcccccgccacgctcgctcccttccccgccgcccaacccctccctcgatgaggtcctcaactatcc

SEQ ID NO: 10315 - RNA, 2365 nt, Homo sapiens
  source 1..2365: mol_type = other RNA
ccaatattggctgtgctgctcctcactgaccccggctgtcatttcctggatctctgcgagagaggcttggcatcttcctttgatgcatttcaggaggcccccaccttgcccagcttctttcctggggctgctttctgccttttaactcagtggacctggactcttagcgtttggtgtaatttaggatcaggtctgagtgtgggccttgaacactagctctggaagcacctcagtggtcaagaacggcctcctattttatacgggaggaaactggtgcacggcctcggcgctctggcctctggtcctgacctgggtgcagggctcctgacgagtggcttggctgtcaccacgtgtgctggggtggctgcggctggtcctggggctggaggacggctccttctcatggagcccgtggacctccaagggcacgtccacagacatctctctggattccctgagccaggagttggccttgatgcctgacgtgtaggaactgccgtggctgtcggcggagtggcgtgagaggcagtgggggcagtgctggctgctgaccccactgcccgggaagctcctgctggccaggtccagctccagctcatcgctgatataggactcccggtagtgctgcttctcttctgcctcctcccgctgccgcagctgttgcagagtgggccgcacgcggaggtggagctggtggctggcgcgcagcaggtgcagcaggtgcctggaccgccaggtgcaccccgtgtagtaaaccagcttctgtgctgcgggcagcccatccagctggatctccagcttctttcccagaaatgccagcttcccaacgtggggccaggggaggtcgtacagcagctgcggagcacggtccacctcctggtagatgtgcactcccctgagggccagtcccaggatcacggtgggacgaccttccttcttatccttgtgcagcctgaagaagtgcacgggcacgtcctccagccggcaggcctcctggatgaagcacagcatggcctccttggggctcaggccctggcgctcacggtgcagggtaggcatgtgccggaggatgtagtcaatccccctcttggtgatgatccactgtgggaagtaggagtgtggctcgaagtacctcccggcatgggccgactcccggtgctcgcccaggtcagcctgcagcgcgcaggcagccagcaggaagtaggcttcctcccggtgagcgcactgtgacctcagcacgcgctccttcaagtggcagtagtacaggtgccgtgccctgtggtcgccctgaagctctgttctggaagtaagtctcaggatcctcctgagggacgtctttgttaccctagaagctctaaggcagctctgtaatcccagcactttgggaggtcgaggcgggtggatcacctgaggtcgggagtttgagaccagcttgaccaacacagagaaaccccgtctctacttatgacccttccgttttccacgtagtgctgcactcggaggaaggccacgaagggggctctgggtttctcatttccctagtggggaaaatgcaagaaagagcaagtgagccgcagggaggtgccgctggctgtcctgtcttcccagttgggggggcctggattgcttcacactcagcttaaagtcgaagctcaggtgtctgcagccatagctgacaattcgactcatggtattttctacccggagaaccctgagtgggacgtggtctacagcgttcaagaacatctgcaaaggcgggcttcgggcgggcacacctgcttgcagcctcagggctcaccacagtccccctgcggacagcccctctggacggagcagttcatttctttctttcttccaatcttttgagaagtacttgctgagcttttgctccaaatccataaatatatactcattgtttctgaccacacagaggccaaagaactgcgcgtctctgatgctcgccacgttgcacacttgctggaaaagctcgcggccagtagccttcacccccacggccagccgcagttgctcccggctgggcagcagcacgaggacatccctgtgttccgaggccatcgcgtccattcccagggtcggctcctgctgactgcatgcaggcctctcaggactgggttccatacatcgcgcccctctgaatgtcttgtcttctcgactggcctgttcgtgatggaagaggctggcctgccacgttcgtgatgtcagggccgggcagtggacgggcagaggccgcgaggaagaggagaccaccgcccagatctcctcatggctgagccctggagtcctcctcggcccaactctctcttcttctggacggctggtttccatcctctatcatgagatagat

SEQ ID NO: 10316 - RNA, 2295 nt, Homo sapiens
  source 1..2295: mol_type = other RNA
ccaatattggctgtgctgctcctcactgaccccggctgtcatttcctggatctggtgcacggcctcggcgctctggcctctggtcctgacctgggtgcagggctcctgacgagtggcttggctgtcaccacgtgtgctggggtggctgcggctggtcctggggctggaggacggctccttctcatggagcccgtggacctccaagggcacgtccacagacatctctctggattccctgagccaggagttggccttgatgcctgacgtgtaggaactgccgtggctgtcggcggagtggcgtgagaggcagtgggggcagtgctggctgctgaccccactgcccgggaagctcctgctggccaggtccagctccagctcatcgctgatataggactcccggtagtgctgcttctcttctgcctcctcccgctgccgcagctgttgcagagtgggccgcacgcggaggtggagctggtggctggcgcgcagcaggtgcagcaggtgcctggaccgccaggtgcaccccgtgtagtaaaccagcttctgtgctgcgggcagcccatccagctggatctccagcttctttcccagaaatgccagcttcccaacgtggggccaggggaggtcgtacagcagctgcggagcacggtccacctcctggtagatgtgcactcccctgagggccagtcccaggatcacggtgggacgaccttccttcttatccttgtgcagcctgaagaagtgcacgggcacgtcctccagccggcaggcctcctggatgaagcacagcatggcctccttggggctcaggccctggcgctcacggtgcagggtaggcatgtgccggaggatgtagtcaatccccctcttggtgatgatccactgtgggaagtaggagtgtggctcgaagtacctcccggcatgggccgactcccggtgctcgcccaggtcagcctgcagcgcgcaggcagccagcaggaagtaggcttcctcccggtgagcgcactgtgacctcagcacgcgctccttcaagtggcagtagtacaggtgccgtgccctgtggtcgctggaaggtggcagggagtgagttccaggacgaccggtgtggggactgctggcccctctggccctgccttgtccctccccacaccagctcccagggctgtcctgagcccctggtacctagttcctgtcttgttatacccacagctgtgtccctgcagggccagcacggcacaggcccacactcttcctggagcggggcacaggtgacttgctgccaccaaggagccactagatgaggctccacctgccgaggtcccactccttccccagtgagcttggccttcaccaaaccaagccccagtgcaggagaggtgcacagagcccgggcgactcgaatccctggaggtgcacagggcctggacaacttgaatccctggatgtggacagacctggctcccagagctcaccgcccagcacggggcttggccatggctggtattcattaatcacaggccaggtggaggctcgcccaagatgcaggtgcaagatcttctcatataattcccccgaactggccccatagcaccaggtagctccatccatcaacccaacactttccagacctcccctccaaggctatccagaaccttccacatattcacacacccctcactctccagaacctgccacacaaccacataccagtgtctccagggctctccacacaaccacacacctttcactctccagaaccctcccacacaaccacacgcccctcaccccctagaaccttccacacaaccgcacacatgccttttggaactggcagggattgtgcctgcttagggaattcctgggaaacccccttaggttttcccccagggtaaaccctgttcacgcacccctgaagctctgttctggaagtaagtctcaggatcctcctgagggacgtctttgttaccctagaagctctaaggcagctctggaagaagcagcccccgttggtttagagtgcagcccaccagatgtacaacttacccactcctgtcggggaaagcttcccactagacacctgcagagtgggcagtgaacagcgagaaccgccacgcagcaagcatagcagcccttagcccagcgacctccagaagcctcgcccacccccggatggtatacccaccctagagagtacgagtcctggcatttgaggaagtaccactttaggccgggcacggtggctcacacctgtaatcccagcactttgggaggtcgaggcgggtggatcacctgagg

SEQ ID NO: 10317 - RNA, 1403 nt, Homo sapiens
  source 1..1403: mol_type = other RNA
ccaatattggctgtgctgctcctcactgaccccggctgtcatttcctggatctggtgcacggcctcggcgctctggcctctggtcctgacctgggtgcagggctcctgacgagtggcttggctgtcaccacgtgtgctggggtggctgcggctggtcctggggctggaggacggctccttctcatggagcccgtggacctccaagggcacgtccacagacatctctctggattccctgagccaggagttggccttgatgcctgacgtgtaggaactgccgtggctgtcggcggagtggcgtgagaggcagtgggggcagtgctggctgctgaccccactgcccgggaagctcctgctggccaggtccagctccagctcatcgctgatataggactcccggtagtgctgcttctcttctgcctcctcccgctgccgcagctgttgcagagtgggccgcacgcggaggtggagctggtggctggcgcgcagcaggtgcagcaggtgcctggaccgccaggtgcaccccgtgtagtaaaccagcttctgtgctgcgggcagcccatccagctggatctccagcttctttcccagaaatgccagcttcccaacgtggggccaggggaggtcgtacagcagctgcggagcacggtccacctcctggtagatgtgcactcccctgagggccagtcccaggatcacggtgggacgaccttccttcttatccttgtgcagcctgaagaagtgcacgggcacgtcctccagccggcaggcctcctggatgaagcacagcatggcctccttggggctcaggccctggcgctcacggtgcagggtaggcatgtgccggaggatgtagtcaatccccctcttggtgatgatccactgtgggaagtaggagtgtggctcgaagtacctcccggcatgggccgactcccggtgctcgcccaggtcagcctgcagcgcgcaggcagccagcaggaagtaggcttcctcccggtgagcgcactgtgacctcagcacgcgctccttcaagtggcagtagtacaggtgccgtgccctgtggtcgcttatgacccttccgttttccacgtagtgctgcactcggaggaaggccacgaagggggctctgggtttctcatttccttcatttctttctttcttccaatcttttgagaagtacttgctgagcttttgctccaaatccataaatatatactcattgtccccacggccagccgcagttgctcccggctgggcagcagcacgaggacatccctgtgttccgaggccatcgcgtccattcccagggtcggctcctgctgactgcatgcaggcctctcaggactgggttccatacatcgcgcccagttccacatggctggggaagcctcacaatcgtggtg

SEQ ID NO: 10318 - RNA, 1467 nt, Homo sapiens
  source 1..1467: mol_type = other RNA
ccaatattggctgtgctgctcctcactgaccccggctgtcatttcctggatctggtgcacggcctcggcgctctggcctctggtcctgacctgggtgcagggctcctgacgagtggcttggctgtcaccacgtgtgctggggtggctgcggctggtcctggggctggaggacggctccttctcatggagcccgtggacctccaagggcacgtccacagacatctctctggattccctgagccaggagttggccttgatgcctgacgtgtaggaactgccgtggctgtcggcggagtggcgtgagaggcagtgggggcagtgctggctgctgaccccactgcccgggaagctcctgctggccaggtccagctccagctcatcgctgatataggactcccggtagtgctgcttctcttctgcctcctcccgctgccgcagctgttgcagagtgggccgcacgcggaggtggagctggtggctggcgcgcagcaggtgcagcaggtgcctggaccgccaggtgcaccccgtgtagtaaaccagcttctgtgctgcgggcagcccatccagctggatctccagcttctttcccagaaatgccagcttcccaacgtggggccaggggaggtcgtacagcagctgcggagcacggtccacctcctggtagatgtgcactcccctgagggccagtcccaggatcacggtgggacgaccttccttcttatccttgtgcagcctgaagaagtgcacgggcacgtcctccagccggcaggcctcctggatgaagcacagcatggcctccttggggctcaggccctggcgctcacggtgcagggtaggcatgtgccggaggatgtagtcaatccccctcttggtgatgatccactgtgggaagtaggagtgtggctcgaagtacctcccggcatgggccgactcccggtgctcgcccaggtcagcctgcagcgcgcaggcagccagcaggaagtaggcttcctcccggtgagcgcactgtgacctcagcacgcgctccttcaagtggcagtagtacaggtgccgtgccctgtggtcgcttatgacccttccgttttccacgtagtgctgcactcggaggaaggccacgaagggggctctgggtttctcatttccttcatttctttctttcttccaatcttttgagaagtacttgctgagcttttgctccaaatccataaatatatactcattgtccccacggccagccgcagttgctcccggctgggcagcagcacgaggacatccctgtgttccgaggccatcgcgtccattcccagggtcggctcctgctgactgcatgcaggcctctcaggactgggttccatacatcgcgcccctcccagatcacagctgtgctttccgggacccgcccttgccgagcttctcactgggaagggaattgagagggaagcctgggctgggaatccagcatggcca

SEQ ID NO: 10319 - RNA, 1505 nt, Homo sapiens
  source 1..1505: mol_type = other RNA
ccaatattggctgtgctgctcctcactgaccccggctgtcatttcctggatctggtgcacggcctcggcgctctggcctctggtcctgacctgggtgcagggctcctgacgagtggcttggctgtcaccacgtgtgctggggtggctgcggctggtcctggggctggaggacggctccttctcatggagcccgtggacctccaagggcacgtccacagacatctctctggattccctgagccaggagttggccttgatgcctgacgtgtaggaactgccgtggctgtcggcggagtggcgtgagaggcagtgggggcagtgctggctgctgaccccactgcccgggaagctcctgctggccaggtccagctccagctcatcgctgatataggactcccggtagtgctgcttctcttctgcctcctcccgctgccgcagctgttgcagagtgggccgcacgcggaggtggagctggtggctggcgcgcagcaggtgcagcaggtgcctggaccgccaggtgcaccccgtgtagtaaaccagcttctgtgctgcgggcagcccatccagctggatctccagcttctttcccagaaatgccagcttcccaacgtggggccaggggaggtcgtacagcagctgcggagcacggtccacctcctggtagatgtgcactcccctgagggccagtcccaggatcacggtgggacgaccttccttcttatccttgtgcagcctgaagaagtgcacgggcacgtcctccagccggcaggcctcctggatgaagcacagcatggcctccttggggctcaggccctggcgctcacggtgcagggtaggcatgtgccggaggatgtagtcaatccccctcttggtgatgatccactgtgggaagtaggagtgtggctcgaagtacctcccggcatgggccgactcccggtgctcgcccaggtcagcctgcagcgcgcaggcagccagcaggaagtaggcttcctcccggtgagcgcactgtgacctcagcacgcgctccttcaagtggcagtagtacaggtgccgtgccctgtggtcgcttatgacccttccgttttccacgtagtgctgcactcggaggaaggccacgaagggggctctgggtttctcatttccttcatttctttctttcttccaatcttttgagaagtacttgctgagcttttgctccaaatccataaatatatactcattgtccccacggccagccgcagttgctcccggctgggcagcagcacgaggacatccctgtgttccgaggccatcgcgtccattcccagggtcggctcctgctgactgcatgcaggcctctcaggactgggttccatacatcgcgccctcggccctcccccgccatgggtcgcaggtgggtgctcagcacctcccagatcacagctgtgctttccgggacccgcccttgccgagcttctcactgggaagggaattgagagggaagcctgggctgggaatccagcatg

SEQ ID NO: 10320 - RNA, 1442 nt, Homo sapiens
  source 1..1442: mol_type = other RNA
ccaatattggctgtgctgctcctcactgaccccggctgtcatttcctggatctggtgcacggcctcggcgctctggcctctggtcctgacctgggtgcagggctcctgacgagtggcttggctgtcaccacgtgtgctggggtggctgcggctggtcctggggctggaggacggctccttctcatggagcccgtggacctccaagggcacgtccacagacatctctctggattccctgagccaggagttggccttgatgcctgacgtgtaggaactgccgtggctgtcggcggagtggcgtgagaggcagtgggggcagtgctggctgctgaccccactgcccgggaagctcctgctggccaggtccagctccagctcatcgctgatataggactcccggtagtgctgcttctcttctgcctcctcccgctgccgcagctgttgcagagtgggccgcacgcggaggtggagctggtggctggcgcgcagcaggtgcagcaggtgcctggaccgccaggtgcaccccgtgtagtaaaccagcttctgtgctgcgggcagcccatccagctggatctccagcttctttcccagaaatgccagcttcccaacgtggggccaggggaggtcgtacagcagctgcggagcacggtccacctcctggtagatgtgcactcccctgagggccagtcccaggatcacggtgggacgaccttccttcttatccttgtgcagcctgaagaagtgcacgggcacgtcctccagccggcaggcctcctggatgaagcacagcatggcctccttggggctcaggccctggcgctcacggtgcagggtaggcatgtgccggaggatgtagtcaatccccctcttggtgatgatccactgtgggaagtaggagtgtggctcgaagtacctcccggcatgggccgactcccggtgctcgcccaggtcagcctgcagcgcgcaggcagccagcaggaagtaggcttcctcccggtgagcgcactgtgacctcagcacgcgctccttcaagtggcagtagtacaggtgccgtgccctgtggtcgcttatgacccttccgttttccacgtagtgctgcactcggaggaaggccacgaagggggctctgggtttctcatttccttcatttctttctttcttccaatcttttgagaagtacttgctgagcttttgctccaaatccataaatatatactcattgtttctgaccacacagaggccaaagaactgcgcgtctctgatgctcgccacgttgcacacttgctggaaaagctcgcggccagtagccttcacatcatccatcgcccaactgatgcgagtgatcccaacagtgttcctacagctgagcctctcacggcagcctctaaacacccagcgtctggtgcgtgtccctgtttccggcgtcccgtgtccacatttcc

SEQ ID NO: 10321 - RNA, 1488 nt, Homo sapiens
  source 1..1488: mol_type = other RNA
ccaatattggctgtgctgctcctcactgaccccggctgtcatttcctggatctggtgcacggcctcggcgctctggcctctggtcctgacctgggtgcagggctcctgacgagtggcttggctgtcaccacgtgtgctggggtggctgcggctggtcctggggctggaggacggctccttctcatggagcccgtggacctccaagggcacgtccacagacatctctctggattccctgagccaggagttggccttgatgcctgacgtgtaggaactgccgtggctgtcggcggagtggcgtgagaggcagtgggggcagtgctggctgctgaccccactgcccgggaagctcctgctggccaggtccagctccagctcatcgctgatataggactcccggtagtgctgcttctcttctgcctcctcccgctgccgcagctgttgcagagtgggccgcacgcggaggtggagctggtggctggcgcgcagcaggtgcagcaggtgcctggaccgccaggtgcaccccgtgtagtaaaccagcttctgtgctgcgggcagcccatccagctggatctccagcttctttcccagaaatgccagcttcccaacgtggggccaggggaggtcgtacagcagctgcggagcacggtccacctcctggtagatgtgcactcccctgagggccagtcccaggatcacggtgggacgaccttccttcttatccttgtgcagcctgaagaagtgcacgggcacgtcctccagccggcaggcctcctggatgaagcacagcatggcctccttggggctcaggccctggcgctcacggtgcagggtaggcatgtgccggaggatgtagtcaatccccctcttggtgatgatccactgtgggaagtaggagtgtggctcgaagtacctcccggcatgggccgactcccggtgctcgcccaggtcagcctgcagcgcgcaggcagccagcaggaagtaggcttcctcccggtgagcgcactgtgacctcagcacgcgctccttcaagtggcagtagtacaggtgccgtgccctgtggtcgcttatgacccttccgttttccacgtagtgctgcactcggaggaaggccacgaagggggctctgggtttctcatttccttcatttctttctttcttccaatcttttgagaagtacttgctgagcttttgctccaaatccataaatatatactcattgtttctgaccacacagaggccaaagaactgcgcgtctctgatgctcgccacgttgcacacttgctggaaaagctcgcggccagtagccttcacccccacggccagccgcagttgctcccggctgggcagcagcacgaggacatccctgtgttccgaggccatcgcgtccattcccagggtcggctcctgctgactgcatgcaggcctctcaggactgggttccatacatcgcgcccagttccacatggctggggaagcctcacaatc

SEQ ID NO: 10322 - RNA, 1672 nt, Homo sapiens
  source 1..1672: mol_type = other RNA
ccaatattggctgtgctgctcctcactgaccccggctgtcatttcctggatctggtgcacggcctcggcgctctggcctctggtcctgacctgggtgcagggctcctgacgagtggcttggctgtcaccacgtgtgctggggtggctgcggctggtcctggggctggaggacggctccttctcatggagcccgtggacctccaagggcacgtccacagacatctctctggattccctgagccaggagttggccttgatgcctgacgtgtaggaactgccgtggctgtcggcggagtggcgtgagaggcagtgggggcagtgctggctgctgaccccactgcccgggaagctcctgctggccaggtccagctccagctcatcgctgatataggactcccggtagtgctgcttctcttctgcctcctcccgctgccgcagctgttgcagagtgggccgcacgcggaggtggagctggtggctggcgcgcagcaggtgcagcaggtgcctggaccgccaggtgcaccccgtgtagtaaaccagcttctgtgctgcgggcagcccatccagctggatctccagcttctttcccagaaatgccagcttcccaacgtggggccaggggaggtcgtacagcagctgcggagcacggtccacctcctggtagatgtgcactcccctgagggccagtcccaggatcacggtgggacgaccttccttcttatccttgtgcagcctgaagaagtgcacgggcacgtcctccagccggcaggcctcctggatgaagcacagcatggcctccttggggctcaggccctggcgctcacggtgcagggtaggcatgtgccggaggatgtagtcaatccccctcttggtgatgatccactgtgggaagtaggagtgtggctcgaagtacctcccggcatgggccgactcccggtgctcgcccaggtcagcctgcagcgcgcaggcagccagcaggaagtaggcttcctcccggtgagcgcactgtgacctcagcacgcgctccttcaagtggcagtagtacaggtgccgtgccctgtggtcgcttatgacccttccgttttccacgtagtgctgcactcggaggaaggccacgaagggggctctgggtttctcatttccttcatttctttctttcttccaatcttttgagaagtacttgctgagcttttgctccaaatccataaatatatactcattgtttctgaccacacagaggccaaagaactgcgcgtctctgatgctcgccacgttgcacacttgctggaaaagctcgcggccagtagccttcacccccacggccagccgcagttgctcccggctgggcagcagcacgaggacatccctgtgttccgaggccatcgcgtccattcccagggtcggctcctgctgactgcatgcaggcctctcaggactgggttccatacatcgcgcccctctgaatgtcttgtcttctcgactggcctgttcgtgatggaagaggctggcctgccacgttcgtgatgtcagggccgggcagtggacgggcagaggccgcgaggaagaggagaccaccgcccagatctcctcatggctgagccctggagtcctcctcggcccaactctctcttcttctggacggctggtttccatcctctatcatgagatagat

SEQ ID NO: 10323 - RNA, 1527 nt, Homo sapiens
  source 1..1527: mol_type = other RNA
ccaatattggctgtgctgctcctcactgaccccggctgtcatttcctggatctggtgcacggcctcggcgctctggcctctggtcctgacctgggtgcagggctcctgacgagtggcttggctgtcaccacgtgtgctggggtggctgcggctggtcctggggctggaggacggctccttctcatggagcccgtggacctccaagggcacgtccacagacatctctctggattccctgagccaggagttggccttgatgcctgacgtgtaggaactgccgtggctgtcggcggagtggcgtgagaggcagtgggggcagtgctggctgctgaccccactgcccgggaagctcctgctggccaggtccagctccagctcatcgctgatataggactcccggtagtgctgcttctcttctgcctcctcccgctgccgcagctgttgcagagtgggccgcacgcggaggtggagctggtggctggcgcgcagcaggtgcagcaggtgcctggaccgccaggtgcaccccgtgtagtaaaccagcttctgtgctgcgggcagcccatccagctggatctccagcttctttcccagaaatgccagcttcccaacgtggggccaggggaggtcgtacagcagctgcggagcacggtccacctcctggtagatgtgcactcccctgagggccagtcccaggatcacggtgggacgaccttccttcttatccttgtgcagcctgaagaagtgcacgggcacgtcctccagccggcaggcctcctggatgaagcacagcatggcctccttggggctcaggccctggcgctcacggtgcagggtaggcatgtgccggaggatgtagtcaatccccctcttggtgatgatccactgtgggaagtaggagtgtggctcgaagtacctcccggcatgggccgactcccggtgctcgcccaggtcagcctgcagcgcgcaggcagccagcaggaagtaggcttcctcccggtgagcgcactgtgacctcagcacgcgctccttcaagtggcagtagtacaggtgccgtgccctgtggtcgcttatgacccttccgttttccacgtagtgctgcactcggaggaaggccacgaagggggctctgggtttctcatttccttcatttctttctttcttccaatcttttgagaagtacttgctgagcttttgctccaaatccataaatatatactcattgtttctgaccacacagaggccaaagaactgcgcgtctctgatgctcgccacgttgcacacttgctggaaaagctcgcggccagtagccttcacctgtgagtgccgggaagtgagggtggagggggtggggtgctctggacagtggatcagggctgccccctccatccctgtctgtctctggtgtgaggatttcccgagaccagtcagggacacacgatgcagcgtcaactccagggccgccctctgggctctgtcctcgcacggcacaaatgaatgcttggttccccatgagcgcgagcatcggtg

SEQ ID NO: 10324 - RNA, 2261 nt, Homo sapiens
  source 1..2261: mol_type = other RNA
ccaatattggctgtgctgctcctcactgaccccggctgtcatttcctggatctggtgcacggcctcggcgctctggcctctggtcctgacctgggtgcagggctcctgacgagtggcttggctgtcaccacgtgtgctggggtggctgcggctggtcctggggctggaggacggctccttctcatggagcccgtggacctccaagggcacgtccacagacatctctctggattccctgagccaggagttggccttgatgcctgacgtgtaggaactgccgtggctgtcggcggagtggcgtgagaggcagtgggggcagtgctggctgctgaccccactgcccgggaagctcctgctggccaggtccagctccagctcatcgctgatataggactcccggtagtgctgcttctcttctgcctcctcccgctgccgcagctgttgcagagtgggccgcacgcggaggtggagctggtggctggcgcgcagcaggtgcagcaggtgcctggaccgccaggtgcaccccgtgtagtaaaccagcttctgtgctgcgggcagcccatccagctggatctccagcttctttcccagaaatgccagcttcccaacgtggggccaggggaggtcgtacagcagctgcggagcacggtccacctcctggtagatgtgcactcccctgagggccagtcccaggatcacggtgggacgaccttccttcttatccttgtgcagcctgaagaagtgcacgggcacgtcctccagccggcaggcctcctggatgaagcacagcatggcctccttggggctcaggccctggcgctcacggtgcagggtaggcatgtgccggaggatgtagtcaatccccctcttggtgatgatctcccggcatgggccgactcccggtgctcgcccaggtcagcctgcagcgcgcaggcagccagcaggaagtaggcttcctcccggtgagcgcactgtgacctcagcacgcgctccttcaagtggcagtagtacaggtgccgtgccctgtggtcgctggaaggtggcagggagtgagttccaggacgaccggtgtggggactgctggcccctctggccctgccttgtccctccccacaccagctcccagggctgtcctgagcccctggtacctagttcctgtcttgttatacccacagctgtgtccctgcagggccagcacggcacaggcccacactcttcctggagcggggcacaggtgacttgctgccaccaaggagccactagatgaggctccacctgccgaggtcccactccttccccagtgagcttggccttcaccaaaccaagccccagtgcaggagaggtgcacagagcccgggcgactcgaatccctggaggtgcacagggcctggacaacttgaatccctggatgtggacagacctggctcccagagctcaccgcccagcacggggcttggccatggctggtattcattaatcacaggccaggtggaggctcgcccaagatgcaggtgcaagatcttctcatataattcccccgaactggccccatagcaccaggtagctccatccatcaacccaacactttccagacctcccctccaaggctatccagaaccttccacatattcacacacccctcactctccagaacctgccacacaaccacataccagtgtctccagggctctccacacaaccacacacctttcactctccagaaccctcccacacaaccacacgcccctcaccccctagaaccttccacacaaccgcacacatgccttttggaactggcagggattgtgcctgcttagggaattcctgggaaacccccttaggttttcccccagggtaaaccctgttcacgcacccctgaagctctgttctggaagtaagtctcaggatcctcctgagggacgtctttgttaccctagaagctctaaggcagctctggaagaagcagcccccgttggtttagagtgcagcccaccagatgtacaacttacccactcctgtcggggaaagcttcccactagacacctgcagagtgggcagtgaacagcgagaaccgccacgcagcaagcatagcagcccttagcccagcgacctccagaagcctcgcccacccccggatggtatacccaccctagagagtacgagtcctggcatttgaggaagtaccactttaggccgggcacggtggctcacacctgtaatcccagcactttgggaggtcgaggcgggtggatcacctgagg

SEQ ID NO: 10325 - RNA, 1342 nt, Homo sapiens
  source 1..1342: mol_type = other RNA
ccaatattggctgtgctgctcctcactgaccccggctgtcatttcctggatctggtgcacggcctcggcgctctggcctctggtcctgacctgggtgcagggctcctgacgagtggcttggctgtcaccacgtgtgctggggtggctgcggctggtcctggggctggaggacggctccttctcatggagcccgtggacctccaagggcacgtccacagacatctctctggattccctgagccaggagttggccttgatgcctgacgtgtaggaactgccgtggctgtcggcggagtggcgtgagaggcagtgggggcagtgctggctgctgaccccactgcccgggaagctcctgctggccaggtccagctccagctcatcgctgatataggactcccggtagtgctgcttctcttctgcctcctcccgctgccgcagctgttgcagagtgggccgcacgcggaggtggagctggtggctggcgcgcagcaggtgcagcaggtgcctggaccgccaggtgcaccccgtgtagtaaaccagcttctgtgctgcgggcagcccatccagctggatctccagcttctttccctggtagatgtgcactcccctgagggccagtcccaggatcacggtgggacgaccttccttcttatccttgtgcagcctgaagaagtgcacgggcacgtcctccagccggcaggcctcctggatgaagcacagcatggcctccttggggctcaggccctggcgctcacggtgcagggtaggcatgtgccggaggatgtagtcaatccccctcttggtgatgatccactgtgggaagtaggagtgtggctcgaagtacctcccggcatgggccgactcccggtgctcgcccaggtcagcctgcagcgcgcaggcagccagcaggaagtaggcttcctcccggtgagcgcactgtgacctcagcacgcgctccttcaagtggcagtagtacaggtgccgtgccctgtggtcgcttatgacccttccgttttccacgtagtgctgcactcggaggaaggccacgaagggggctctgggtttctcatttccttcatttctttctttcttccaatcttttgagaagtacttgctgagcttttgctccaaatccataaatatatactcattgtttctgaccacacagaggccaaagaactgcgcgtctctgatgctcgccacgttgcacacttgctggaaaagctcgcggccagtagccttcacatcatccatcgcccaactgatgcgagtgatcccaacagtgttcctacagctgagcctctcacggcagcctctaaacacccagcgtctggtgcgtgtc

SEQ ID NO: 10326 - RNA, 1603 nt, Homo sapiens
  source 1..1603: mol_type = other RNA
ccaatattggctgtgctgctcctcactgaccccggctgtcatttcctggatctggtgcacggcctcggcgctctggcctctggtcctgacctgggtgcagggctcctgacgagtggcttggctgtcaccacgtgtgctggggtggctgcggctggtcctggggctggaggacggctccttctcatggagcccgtggacctccaagggcacgtccacagacatctctctggattccctgagccaggagttggccttgatgcctgacgtgtaggaactgccgtggctgtcggcggagtggcgtgagaggcagtgggggcagtgctggctgctgaccccactgcccgggaagctcctgctggccaggtccagctccagctcatcgctgatataggactcccggtagtgctgcttctcttctgcctcctcccgctgccgcagctgttgcagagtgggccgcacgcggaggtggagctggtggctggcgcgcagcaggtgcagcaggtgcctggaccgccaggtgcaccccgtgtagtaaaccagcttctgtgctgcgggcagcccatccagctggatctccagcttctttccctggtagatgtgcactcccctgagggccagtcccaggatcacggtgggacgaccttccttcttatccttgtgcagcctgaagaagtgcacgggcacgtcctccagccggcaggcctcctggatgaagcacagcatggcctccttggggctcaggccctggcgctcacggtgcagggtaggcatgtgccggaggatgtagtcaatccccctcttggtgatgatccactgtgggaagtaggagtgtggctcgaagtacctcccggcatgggccgactcccggtgctcgcccaggtcagcctgcagcgcgcaggcagccagcaggaagtaggcttcctcccggtgagcgcactgtgacctcagcacgcgctccttcaagtggcagtagtacaggtgccgtgccctgtggtcgcttatgacccttccgttttccacgtagtgctgcactcggaggaaggccacgaagggggctctgggtttctcatttccttcatttctttctttcttccaatcttttgagaagtacttgctgagcttttgctccaaatccataaatatatactcattgtttctgaccacacagaggccaaagaactgcgcgtctctgatgctcgccacgttgcacacttgctggaaaagctcgcggccagtagccttcacccccacggccagccgcagttgctcccggctgggcagcagcacgaggacatccctgtgttccgaggccatcgcgtccattcccagggtcggctcctgctgactgcatgcaggcctctcaggactgggttccatacatcgcgcccctctgaatgtcttgtcttctcgactggcctgttcgtgatggaagaggctggcctgccacgttcgtgatgtcagggccgggcagtggacgggcagaggccgcgaggaagaggagaccaccgcccagatctcctcatggctgagccctggagtcctcctcggcccaactctctcttcttctggacggctggtttccatcctctatcatgagatagat

SEQ ID NO: 10327 - RNA, 1576 nt, Homo sapiens
  source 1..1576: mol_type = other RNA
ccaatattggctgtgctgctcctcactgaccccggctgtcatttcctggatctggtgcacggcctcggcgctctggcctctggtcctgacctgggtgcagggctcctgacgagtggcttggctgtcaccacgtgtgctggggtggctgcggctggtcctggggctggaggacggctccttctcatggagcccgtggacctccaagggcacgtccacagacatctctctggattccctgagccaggagttggccttgatgcctgacgtgtaggaactgccgtggctgtcggcggagtggcgtgagaggcagtgggggcagtgctggctgctgaccccactgcccgggaagctcctgctggccaggtccagctccagctcatcgctgatataggactcccggtagtgctgcttctcttctgcctcctcccgctgccgcagctgttgcagagtgggccgcacgcggaggtggagctggtggctggcgcgcagcaggtgcagcaggtgcctggaccgccaggtgcaccccgtgtagtaaaccagcttctgtgctgcgggcagcccatccagctggatctccagcttctttccctggtagatgtgcactcccctgagggccagtcccaggatcacggtgggacgaccttccttcttatccttgtgcagcctgaagaagtgcacgggcacgtcctccagccggcaggcctcctggatgaagcacagcatggcctccttggggctcaggccctggcgctcacggtgcagggtaggcatgtgccggaggatgtagtcaatccccctcttggtgatgatccactgtgggaagtaggagtgtggctcgaagtacctcccggcatgggccgactcccggtgctcgcccaggtcagcctgcagcgcgcaggcagccagcaggaagtaggcttcctcccggtgagcgcactgtgacctcagcacgcgctccttcaagtggcagtagtacaggtgccgtgccctgtggtcgcttatgacccttccgttttccacgtagtgctgcactcggaggaaggccacgaagggggctctgggtttctcatttccttcatttctttctttcttccaatcttttgagaagtacttgctgagcttttgctccaaatccataaatatatactcattgtttctgaccacacagaggccaaagaactgcgcgtctctgatgctcgccacgttgcacacttgctggaaaagctcgcggccagtagccttcacccccacggccagccgcagttgctcccggctgggcagcagcacgaggacatccctgtgttccgaggccatcgcgtccattcccagggtcggctcctgctgactgcatgcaggcctctcaggactgggttccatacatcgcgcccctgaaggagggaacgtgtcagggtttgtccgggcggggtctatgcccctccctctcgggggcaccgccatgctgtcgttactcggccctcccccgccatgggtcgcaggtgggtgctcagcacctcccagatcacagctgtgctttccgggacccgcccttgccgagcttctcactgggaagggaatt

SEQ ID NO: 10328 - RNA, 895 nt, Homo sapiens
  source 1..895: mol_type = other RNA
ccaatattggctgtgctgctcctggggaacagacggccgcctccgtgcccccaccgtcgggggaggccccgtggcctgggatccccggcctgcagcctcgggttccgcctcctccgagggcacatcctgtcgccaggctttcactggctgcttctgtaggtcctccaccaaggcgacagcctcctcaccgcttcccgggtgctgctcacgcacccagccctggatctcccctggcagcactgtcaggaactgctccagcaccagcagctccaggatctgctccttggtacgcagctcgggccgcagccagcggcagcagagctcccagagctggctgaaggcctcatgaggcccatgcacatccccgtagcagaattgccggaagcgctggcggcaggcttcggaatccctgccatcctcatgctgggcagattcctgttcccaggaggaatcttccactttcacaatcagaagcccttctccctccccaggggcctggtcctgggcctccaagggggctgccattcccctggcctgaggctcagggttggtcggcttcaacctgggccccagaacctgtactttcagtctcccagagggatcccctgtggtagctgggctggcatctggatgtgtactccagggtcgctcagcaggacacggcaggcgggaaggcgagccagccggagccccgcgctgtccaccgcagcctcgcccgcggggcgagcggcgatcgtacaggggcgtctgccgggggaccaagctggcagagcggcgcgggggaccagcacttcctagcagtgcgcgcgccctccggcctctgcctcggggcgctgatcccggccactcggagcccggtgcttgatgttggagccaggcggccagaggccccgtc

SEQ ID NO: 10329 - RNA, 999 nt, Homo sapiens
  source 1..999: mol_type = other RNA
ccaatattggctgtgctgctcctggggaacagacggccgcctccgtgcccccaccgtcgggggaggccccgtggcctgggatccccggcctgcagcctcgggttccgcctcctccgagggcacatcctgtcgccaggctttcactggctgcttctgtaggtcctccaccaaggcgacagcctcctcaccgcttcccgggtgctgctcacgcacccagccctggatctcccctggcagcactgtcaggaactgctccagcaccagcagctccaggatctgctccttggtacgcagctcgggccgcagccagcggcagcagagctcccagagctggctgaaggcctcatgaggcccatgcacatccccgtagcagaattgccggaagcgctggcggcaggcttcggaatccctgccatcctcatgctgggcagattcctgttcccaggaggaatcttccactttcacaatcagaagcccttctccctccccaggggcctggtcctgggcctccaagggggctgccattcccctggcctgaggctcagggttggtcggcttcaacctgggccccagaacctgtactttcagtctcccagagggatcccctgtggtagctgggctggcatctggatgtgtactccagggtcgctcagcaggacacggcaggcgggaaggcgagccagccggagccccgcgctgtccaccgcagcctcgcccgcggggcgagcggcgatcgtacaggggcgtctgccgggggaccaagctggcagagcggcgcgggggaccagcacttcctagcagtgcgcgcgccctccggcctctgcctcggggcgctgatcccggccactcggagcccggtgcttgatgttggagccaggcggccagaggccccgtccccgccccggcccccgcccccgcccccgcccccgaaacacacaacgcccactacggcccaggagatcccacttccgccgcgagctcccggcgccggaagtcctc

SEQ ID NO: 10330 - RNA, 1057 nt, Homo sapiens
  source 1..1057: mol_type = other RNA
ccaatattggctgtgctgctcctggggaacagacggccgcctccgtgcccccaccgtcgggggaggccccgtggcctgggatccccggcctgcagcctcgggttccgcctcctccgagggcacatcctgtcgccaggctttcactggctgcttctgtaggtcctccaccaaggcgacagcctcctcaccgcttcccgggtgctgctcacgcacccagccctggatctcccctggcagcactgtcaggaactgctccagcaccagcagctccaggatctgctccttggtacgcagctcgggccgcagccagcggcagcagagctcccagagctggctgaaggcctcatgaggcccatgcacatccccgtagcagaattgccggaagcgctggcggcaggcttcggaatccctgccatcctcatgctgggcagattcctgttcccaggaggaatcttccactttcacaatcagaagcccttctccctccccaggggcctggtcctgggcctccaagggggctgccattcccctggcctgaggctcagggttggtcggcttcaacctgggccccagaacctgtactttcagtctcccagagggatcccctgtggtagctgggctggcatctggatgtgtactccattctcatcctctggtgacttcgaagaagactttcctcgaagagggccaggactcaccagggtcgctcagcaggacacggcaggcgggaaggcgagccagccggagccccgcgctgtccaccgcagcctcgcccgcggggcgagcggcgatcgtacaggggcgtctgccgggggaccaagctggcagagcggcgcgggggaccagcacttcctagcagtgcgcgcgccctccggcctctgcctcggggcgctgatcccggccactcggagcccggtgcttgatgttggagccaggcggccagaggccccgtccccgccccggcccccgcccccgcccccgcccccgaaacacacaacgcccactacggcccaggagatcccacttccgccgcgagctcccggcgccggaagtcctc

SEQ ID NO: 10331 - RNA, 1063 nt, Homo sapiens
  source 1..1063: mol_type = other RNA
ccaatattggctgtgctgctcctggggaacagacggccgcctccgtgcccccaccgtcgggggaggccccgtggcctgggatccccggcctgcagcctcgggttccgcctcctccgagggcacatcctgtgcaggaaccacaacatgctcatcagcccgagaccagaccgggggagacagagtttactccctgtcgccaggctttcactggctgcttctgtaggtcctccaccaaggcgacagcctcctcaccgcttcccgggtgctgctcacgcacccagccctggatctcccctggcagcactgtcaggaactgctccagcaccagcagctccaggatctgctccttggtacgcagctcgggccgcagccagcggcagcagagctcccagagctggctgaaggcctcatgaggcccatgcacatccccgtagcagaattgccggaagcgctggcggcaggcttcggaatccctgccatcctcatgctgggcagattcctgttcccaggaggaatcttccactttcacaatcagaagcccttctccctccccaggggcctggtcctgggcctccaagggggctgccattcccctggcctgaggctcagggttggtcggcttcaacctgggccccagaacctgtactttcagtctcccagagggatcccctgtggtagctgggctggcatctggatgtgtactccagggtcgctcagcaggacacggcaggcgggaaggcgagccagccggagccccgcgctgtccaccgcagcctcgcccgcggggcgagcggcgatcgtacaggggcgtctgccgggggaccaagctggcagagcggcgcgggggaccagcacttcctagcagtgcgcgcgccctccggcctctgcctcggggcgctgatcccggccactcggagcccggtgcttgatgttggagccaggcggccagaggccccgtccccgccccggcccccgcccccgcccccgcccccgaaacacacaacgcccactacggcccaggagatcccacttccgccgcgagctcccggcgccggaagtcctc

SEQ ID NO: 10332 - RNA, 32 nt, Homo sapiens
  source 1..32: mol_type = other RNA
ccaccaggtctagcattgggatttaagcgacc

SEQ ID NO: 10333 - RNA, 512 nt, Homo sapiens
  source 1..512: mol_type = other RNA
ccagaggtggggactgagagccagccccttttcaccccctggcttttaggacccccatcgcagcacggggaggcatcccccgcgaggcggggactgagaaccagcccctcttcccccgctggctgttgggaccccaatcgcaggggggggaggcatcccccacgaggcgtggactgagagccagcccctcttccccccctgtctcttgggacccccatcgcaggcggaggaggtacccccgggaggaggggactgagagccagcccctctcccctccctcggtcttgggacccccatgggaaggggtggaggcacctcccgcgaggcggggactgagagccagcccctcttccctccctggctcttgggacccccatcgcagtggggggaggcacctcccgcgaggcggggactgagagccagcccctcttccccccccccggctcttaggacccccatcgcagttgggggaggcaccccccgcgagacagggactgcgagccagctccttt

SEQ ID NO: 10334 - RNA, 457 nt, Homo sapiens
  source 1..457: mol_type = other RNA
ccagaggtggggactgagagccagccccttttcaccccctggcttttaggacccccatcgcagcacggggaggcatcccccgcgaggcggggactgagaaccagcccctcttcccccgctggctgttgggaccccaatcgcaggggggggaggcatcccccacgaggcgtggactgagagccagcccctcttccccccctgtctcttgggacccccatcgcaggcggaggaggtacccccgggaggaggggactgagagccagcccctctcccctccctgggtcttgggacccccatcggaaggggcggaggcacctcccgcgaggcggggactgagagccagcccctcttccctccctggctcttgggacccccatcgcagtggggggaggcacctcccgcgaggcggggactgagagccagcccctcttccccccccggctcttaggacccccat

SEQ ID NO: 10335 - RNA, 2311 nt, Homo sapiens
  source 1..2311: mol_type = other RNA
ccaggctctgcagtgggagatgctcctcatgggagtctggaacctggttgttctgaaatggtgtgtgtggggtggaggtctccttgctcagggactctctgggggaaacaaggcagggctgtactcaaattggagttttccttgggctcctgccgtcttttctgagtccctgtgcactagtggctttgtggtacctgcttgtggctcctcggccgacagatgaaatcttgtctcaccatttttggtgaggagggacccagtcgtctgtggagctgagaccctttctctgcgcgcagggttcggggctacggtgaagtgggagggggagggaagaatgtggagctggccttggccgccgtgtgcaccggcagctgcgccatggccagaggtgagctggcacaggcgccggctagtgggggctccccaagctgtgttttcgtttttccgggtctggccggaaaaccgaagaggctcaaagccctggctgagcagggcggaggcagagaagagtcggtaaacaccgccccaaaaaccccacgaaggcaccaaaaaattctgggcagccgaacagagtcagaggcgagaattttaaaaagagagagaaaattaagagtgaggggatgtgggcaatgggccttttgctgctgcctgtgtctctacgctcgcatggcagttctcatgctggctggactgcaactttcaacttgaccttggcctccagccgtgtctgaccagtatgtaaaaccgccttcaagtccccaggaacaggggcctagaaccctactctgtctctttgtcactgtgagttttacaatgccacttggagggaggaaggggggtggtgaaacggccagaaagtaacagaaaaatcaagtccctacagaggctagttcctgagtctgcaaatggccagtcagggagaaggtaaactgggggcaaatcaatatttacccagaactgctaaaaagtcaagaaggaaagggcacacttggtgggggggtggctggtgtgggggtcatagaaggttttattgggcgacacttacattggtcaggacaaatccaggatcaggacagataaaagcccaagcccagccacattggtctggatcctgcaggaagcccaggggccttagacagcagatggtggggtgtgtgtgaggggtggtatgcgtgctgctctgagtttagggctgagtgtgcaagctaggagcagaggacaggtccaagcctggcttctcaccagtccgcctggggtggaaaagaatccagcactctccccagcactattccggtaatgtgcccactttcactttgaacgcttgttcctcttctaggcatctgaccagctcacagtagtgaatcaggaagtggaagtatgtggctctaaagcagcaggacccccagaacccctcgacaaaacatggcagctacaagacgggtcgctgcttggttcttcagcaccaacaccctaccatgctcccaagaaaaggttgcatttcccaggcacagaggaaaggcttcttggactggttcttgggcaaagaaggactaggcaccctctgcaggctggagatcctacttgaggggaaggcaggaagtggccccaaagagcccctttttcttgtcccaaaatagagtgaaatagcgggttcccagattcctggagagtcaggtccggtccacaaagaagcgtggctttagggcccagaaggggggtttaagtcccagccagaagcacagctggggcttgttcctcttaagccccttccagaactaagccagccatactggcgaggtgggagcatggatgaatggtgcacagggatcgctcgctctatctcaaagtctctggaggaggaagcgttgttaccaggtcagagcaaggatcaggctgtatacctaagtgtgcgaatgtgagtgtgtcagtgtacactgtgtgtgtgtgtgatgagtcgttctgagtctatgggtctaaatgcaaacatatgaaattgctcactaacagtgtggacagggaagggataggggctcctaaatgcagtccaagcctccagtggaatgtcctgggacccaggcatatccgcaggaaccgataagcagcaaacaccctgccactgtttccctggaaagagcaaaatcgcaactccatcgaagccgaaggcgccgatgtccgtcctgtggtctcactgcagaaatacgcgccggttcctgacctgtccccactgctccagatcgcaacccaatcgcgcgcccacctcccctccccgcctggttgcgcgggtctgggccccactgggataaaggaaggg

SEQ ID NO: 10336 - RNA, 31 nt, Homo sapiens
  source 1..31: mol_type = other RNA
ccaggctctgcagtgggaggtgatgcccgga

SEQ ID NO: 10337 - RNA, 1469 nt, Homo sapiens
  source 1..1469: mol_type = other RNA
ccagggaggctggtttggaggaatactccctgagcctggatactgggattctaagtctggttcgctgctctctgaggtgggagatgggctgtggccatccagggatttggaggccttgatgctgaaaggaaacctgcgtccccctgatgccaaggtgtgtttcttaatcatcaggtgcaggctttctgcgctgtccatactctctacgctttctacaatgggctgcggccttggtcggtcagccttcctcactggggtagtcttggggtcctcagagttgttggagtctgtgtcagactcactcagtgacctctgcatcagctgtctcagcctggctaacttcagttccctcttctccagtgggatctttttagaatttctagaggaagcctgagcatcctggaattccaaggacagtttttcctgggtgcagacattttctgagatttcctttcccaataactggcgtaagattttatcagaatcttcatcttttgctttgggtctagcccggctggaggctgacaggcttccaagaacctgaatcccctcttggactcctggcttgcttttggctacagaatcatcatctgcatctggagatttccactgggactttctggaggcaggtgaggatggtgaactgggtgaagaagggagtgacttgccctctgatttctgggcttctagaaattgttggagttggttctgcagcgtgacacgttctactgtttgttcctttagctgcttggttaacttcaccacttgagaggccagcgacatgcaggtctccaccaccaccaggtacctggagcacagggtgtgcccctgccgctcggcgctctgggagggcttttccccagcgtggttctgcatggtgacatttgctccatattcaaccaaggtctgtatgcatccaaggtagccatgctgtgaggctacgtgaacggcactgttgccatcctggtctacttcatccaacgagatgccctgttcttgcataaactgaagaagccacagaagaatcttttccgtagcaagagaaaattctcattcagatgtgaattgaaaatccttgaatctctgactggccatagcaacctgcgtaatgaataaggcttggaaaatccttagaacaactcagttctgcaatggcttctgtttcgctcaccatccagcgtacgcactccaactgaccattctgatctgtcttcgttttgcgtatcacatcttcggcacagttctgggatcgtcttgagtgatgtgactgaataagatatgtcatcactaaagtcaatttcatccaaatcaaggtattcaggggcttccattattcttccttgcacattttgagtacggtcaaatacttataaattcctttcgctctttttacctcgactgccgttgcttttccccagctggggctctcctctcctccccgcctactttttgtccgcgcttcccacttt

SEQ ID NO: 10338 - RNA, 1256 nt, Homo sapiens
  source 1..1256: mol_type = other RNA
ccagggaggctggtttggaggaatactccctgagcctggatactgggattctaagtctggttcgctgctctctgaggtgggagatgggctgtggccatccagggatttggaggccttgatgctgaaaggaaacctgcgtccccctgatgccaaggtgtgtttcttaatcatcaggtgcaggctttctgcgctgtccatactctctacgctttctacaatgggctgcggccttggtcggtcagccttcctcactggggtagtcttggggtcctcagagttgttggagtctgtgtcagactcactcagtgacctctgcatcagctgtctcagcctggctaacttcagttccctcttctccagtgggatctttttagaatttctagaggaagcctgagcatcctggaattccaaggacagtttttcctgggtgcagacattttctgagatttcctttcccaataactggcgtaagattttatcagaatcttcatcttttgctttgggtctagcccggctggaggctgacaggcttccaagaacctgaatcccctcttggactcctggcttgcttttggctacagaatcatcatctgcatctggagatttccactgggactttctggaggcaggtgaggatggtgaactgggtgaagaagggagtgacttgccctctgatttctgggcttctagaaattgttggagttggttctgcagcgtgacacgttctactgtttgttcctttagctgcttggttaacttcaccacttgagaggccagcgacatgcaggtctccaccaccaccaggtacctggagcacagggtgtgcccctgccgctcggcgctctgggagggcttttccccagcgtggttctgcatggtgacatttgctccatattcaaccaaggtctgtatgcatccaaggtagccatgctgtgaggctacgtgaacggcactgttgccatcctggtctacttcatccaacgagatgccctgttcttgcataaactgaagaagccacagaagaatcttttcctgatctgtcttcgttttgcgtatcacatcttcggcacagttctgggatcgtcttgagtgatgtgactgaataagatatgtcatcactaaagtcaatttcatccaaatcaaggtattcaggggcttccattattcttccttgcacattttgagtacggtcaaatacttataaattcccggggcgcccggcgcgccggcggctcaggagcgcgaagggactgact

SEQ ID NO: 10339 - RNA, 2194 nt, Homo sapiens
  source 1..2194: mol_type = other RNA
ccagggaggctggtttggaggaatactccctgagcctggatactgggattctaagtctggttcgctgctctctgaggtgggagatgggctgtggccatccagggatttggaggccttgatgctgaaaggaaacctgcgtccccctgatgccaaggtgtgtttcttaatcatcaggtgcaggctttctgcgctgtccatactctctacgctttctacaatgggctgcggccttggtcggtcagccttcctcactggggtagtcttggggtcctcagagttgttggagtctgtgtcagactcactcagtgacctctgcatcagctgtctcagcctggctaacttcagttccctcttctccagtgggatctttttagaatttctagaggaagcctgagcatcctggaattccaaggacagtttttcctgggtgcagacattttctgagatttcctttcccaataactggcgtaagattttatcagaatcttcatcttttgctttgggtctagcccggctggaggctgacaggcttccaagaacctgaatcccctcttggactcctggcttgcttttggctacagaatcatcatctgcatctggagatttccactgggactttctggaggcaggtgaggatggtgaactgggtgaagaagggagtgacttgccctctgatttctgggcttctagaaattgttggagttggttctgcagcgtgacacgttctactgtttgttcctttagctgcttggttaacttcaccacttgagaggccagcgacatgcaggtctccaccaccaccaggtacctggagcacagggtgtgcccctgccgctcggcgctctgggagggcttttccccagcgtggttctgcatggtgacatttgctccatattcaaccaaggtctgtatgcatccaaggtagccatgctgtgaggctacgtgaacggcactgttgccatcctggtctacttcatccaacgagatgccctgttcttgcataaactgaagaagccacagaagaatcttttcctggccatagcaacctgcgtaatgaataaggcttggaaaatccttagaacaactcagttctgcaatggcttctgtttcgctcaccatccagcgtacgcactccaactgaccattcaggagagagatctgtccttctttaacaatgttcaagatgcttttcacttttttcagatactcactcctttcttctgggccttgggagctggtccggtttaggccactgacctgctcttctggtttggattctgctgctgaggattgtaggtggaaggccctgagctggcagtctggtgttgtcttctcaacttttcgaccatgaggatcactaaatgtcttgtttaggaagtctttactctggttttcaggctcatatgcagagccacatttaaccagaggaggtgagatctcggtttcttcagtggacagcttgtgctggtcgtggatgacagctgatgcttttctcaagtgagggcttttcacgggagaaagaacacaaaatggtgccatgttggatgatgagctctcagaacttcctgtagagcaggctttgccagaaaggccattgatggttgtgcataagcccaaaattcttttttctgaagtcaccttggtaaaagaggcaagctgctgactggatttaatataaggcacatccagaatctcatccatgtcgaggtcgtagtgctccagttcacccagcgatgtgctgggctcagagctcttacctggtgggccgcccactccatctccagggccaagctcctgaggctgggggcccaggtcagactcaccccctttctggtactcaaccactttctggttcttttggtcatcactttcattgttctccagagtctctggctgatgtttcagtggcgaaacccgcttcactgggcggaacttactgtacacatcagcgattcctgtgggcttttgcgtgtttgtaataagagttgagatgccacaattccagctagagctagaaactgatctgtcttcgttttgcgtatcacatcttcggcacagttctgggatcgtcttgagtgatgtgactgaataagatatgtcatcactaaagtcaatttcatccaaatcaaggtattcaggggcttccattattcttccttgcacattttgagtacggtcaaatacttataaattc

SEQ ID NO: 10340 - RNA, 1828 nt, Homo sapiens
  source 1..1828: mol_type = other RNA
ccagggaggctggtttggaggaatactccctgagcctggatactgggattctaagtctggttcgctgctctctgaggtgggagatgggctgtggccatccagggatttggaggccttgatgctgaaaggaaacctgcgtccccctgatgccaaggtgtgtttcttaatcatcaggtgcaggctttctgcgctgtccatactctctacgctttctacaatgggctgcggccttggtcggtcagccttcctcactggggtagtcttggggtcctcagagttgttggagtctgtgtcagactcactcagtgacctctgcatcagctgtctcagcctggctaacttcagttccctcttctccagtgggatctttttagaatttctagaggaagcctgagcatcctggaattccaaggacagtttttcctgggtgcagacattttctgagatttcctttcccaataactggcgtaagattttatcagaatcttcatcttttgctttgggtctagcccggctggaggctgacaggcttccaagaacctgaatcccctcttggactcctggcttgcttttggctacagaatcatcatctgcatctggagatttccactgggactttctggaggcaggtgaggatggtgaactgggtgaagaagggagtgacttgccctctgatttctgggcttctagaaattgttggagttggttctgcagcgtgacacgttctactgtttgttcctttagctgcttggttaacttcaccacttgagaggccagcgacatgcaggtctccaccaccaccaggtacctggagcacagggtgtgcccctgccgctcggcgctctgggagggcttttccccagcgtggttctgcatggtgacatttgctccatattcaaccaaggtctgtatgcatccaaggtagccatgctgtgaggctacgtgaacggcactgttgccatcctggtctacttcatccaacgagatgccctgttcttgcataaactgaagaagccacagaagaatcttttcctggccatagcaacctgcgtaatgaataaggcttggaaaatccttagaacaactcagttctgcaatggcttctgtttcgctcaccatccagcgtacgcactccaactgaccattctgatctgtcttcgttttgcgtatcacatcttcggcacagttctgggatcgtcttgagtgatgtgactgaataagatatgtcatcactaaagtcaatttcatccaaatcaaggtattcaggggcttccattattcttccttgcacattttgagtacggtcaaatacttataaattccacctgcagatgaaagtcatcgccaagagacaaggccaagagagaaacattcccctctgaaatccacgcggaccagcctgggacgcagaacagcactagagggaggctggcggagcccgggctggacagggcagtcggggagctggtgctgatgagcgaggggcggcagcaacaccagacgtcccttttctacagctattattaccgttgttagtactgtcgctattactattacttcgcccctccttatctcagcttttccgagccgcggaactgcccatccctgcctgcgataagatcccgggtgacagcaagaataagaaccacatgaggcgggcaaatgaaaagaacaatcctttggaaaccgaggcgggggttgtttccccctttccccagtaaagcagccgctgccgccaccactgttactgttactatagagacctccccctcaaaccctttctgcagaggcgcctctgctgcccggagcagccgagactcgcggcaca

SEQ ID NO: 10341 - RNA, 1370 nt, Homo sapiens
  source 1..1370: mol_type = other RNA
ccagggaggctggtttggaggaatactccctgagcctggatactgggattctaagtctggttcgctgctctctgaggtgggagatgggctgtggccatccagggatttggaggccttgatgctgaaaggaaacctgcgtccccctgatgccaaggtgtgtttcttaatcatcaggtgcaggctttctgcgctgtccatactctctacgctttctacaatgggctgcggccttggtcggtcagccttcctcactggggtagtcttggggtcctcagagttgttggagtctgtgtcagactcactcagtgacctctgcatcagctgtctcagcctggctaacttcagttccctcttctccagtgggatctttttagaatttctagaggaagcctgagcatcctggaattccaaggacagtttttcctgggtgcagacattttctgagatttcctttcccaataactggcgtaagattttatcagaatcttcatcttttgctttgggtctagcccggctggaggctgacaggcttccaagaacctgaatcccctcttggactcctggcttgcttttggctacagaatcatcatctgcatctggagatttccactgggactttctggaggcaggtgaggatggtgaactgggtgaagaagggagtgacttgccctctgatttctgggcttctagaaattgttggagttggttctgcagcgtgacacgttctactgtttgttcctttagctgcttggttaacttcaccacttgagaggccagcgacatgcaggtctccaccaccaccaggtacctggagcacagggtgtgcccctgccgctcggcgctctgggagggcttttccccagcgtggttctgcatggtgacatttgctccatattcaaccaaggtctgtatgcatccaaggtagccatgctgtgaggctacgtgaacggcactgttgccatcctggtctacttcatccaacgagatgccctgttcttgcataaactgaagaagccacagaagaatcttttcctggccatagcaacctgcgtaatgaataaggcttggaaaatccttagaacaactcagttctgcaatggcttctgtttcgctcaccatccagcgtacgcactccaactgaccattctgatctgtcttcgttttgcgtatcacatcttcggcacagttctgggatcgtcttgagtgatgtgactgaataagatatgtcatcactaaagtcaatttcatccaaatcaaggtattcaggggcttccattattcttccttgcacattttgagtacggtcaaatacttataaattcccggggcgcccggcgcgccggcggctcaggagcgcgaagggactgact

SEQ ID NO: 10342 - RNA, 1452 nt, Homo sapiens
  source 1..1452: mol_type = other RNA
ccagggaggctggtttggaggaatactccctgagcctggatactgggattctaagtctggttcgctgctctctgaggtgggagatgggctgtggccatccagggatttggaggccttgatgctgaaaggaaacctgcgtccccctgatgccaaggtgtgtttcttaatcatcaggtgcaggctttctgcgctgtccatactctctacgctttctacaatgggctgcggccttggtcggtcagccttcctcactggggtagtcttggggtcctcagagttgttggagtctgtgtcagactcactcagtgacctctgcatcagctgtctcagcctggctaacttcagttccctcttctccagtgggatctttttagaatttctagaggaagcctgagcatcctggaattccaaggacagtttttcctgggtgcagacattttctgagatttcctttcccaataactggcgtaagattttatcagaatcttcatcttttgctttgggtctagcccggctggaggctgacaggcttccaagaacctgaatcccctcttggactcctggcttgcttttggctacagaatcatcatctgcatctggagatttccactgggactttctggaggcaggtgaggatggtgaactgggtgaagaagggagtgacttgccctctgatttctgggcttctagaaattgttggagttggttctgcagcgtgacacgttctactgtttgttcctttagctgcttggttaacttcaccacttgagaggccagcgacatgcaggtctccaccaccaccaggtacctggagcacagggtgtgcccctgccgctcggcgctctgggagggcttttccccagcgtggttctgcatggtgacatttgctccatattcaaccaaggtctgtatgcatccaaggtagccatgctgtgaggctacgtgaacggcactgttgccatcctggtctacttcatccaacgagatgccctgttcttgcataaactgaagaagccacagaagaatcttttcctggccatagcaacctgcgtaatgaataaggcttggaaaatccttagaacaactcagttctgcaatggcttctgtttcgctcaccatccagcgtacgcactccaactgaccattctgatctgtcttcgttttgcgtatcacatcttcggcacagttctgggatcgtcttgagtgatgtgactgaataagatatgtcatcactaaagtcaatttcatccaaatcaaggtattcaggggcttccattattcttccttgcacattttgagtacggtcaaatacttataaattcctttcgctctttttacctcgactgccgttgcttttccccagctggggctctcctctcctccccgcctactttttgtccgcgcttcccacttttctcctcctgccccccacccccttccttgcttcttggc

SEQ ID NO: 10343 - RNA, 1454 nt, Homo sapiens
  source 1..1454: mol_type = other RNA
ccagggaggctggtttggaggaatactccctgagcctggatactgggattctaagtctggttcgctgctctctgaggtgggagatgggctgtggccatccagggatttggaggccttgatgctgaaaggaaacctgcgtccccctgatgccaaggtgtgtttcttaatcatcaggtgcaggctttctgcgctgtccatactctctacgctttctacaatgggctgcggccttggtcggtcagccttcctcactggggtagtcttggggtcctcagagttgttggagtctgtgtcagactcactcagtgacctctgcatcagctgtctcagcctggctaacttcagttccctcttctccagtgggatctttttagaatttctagaggaagcctgagcatcctggaattccaaggacagtttttcctgggtgcagacattttctgagatttcctttcccaataactggcgtaagattttatcagaatcttcatcttttgctttgggtctagcccggctggaggctgacaggcttccaagaacctgaatcccctcttggactcctggcttgcttttggctacagaatcatcatctgcatctggagatttccactgggactttctggaggcaggtgaggatggtgaactgggtgaagaagggagtgacttgccctctgatttctgggcttctagaaattgttggagttggttctgcagcgtgacacgttctactgtttgttcctttagctgcttggttaacttcaccacttgagaggccagcgacatgcaggtctccaccaccaccaggtacctggagcacagggtgtgcccctgccgctcggcgctctgggagggcttttccccagcgtggttctgcatggtgacatttgctccatattcaaccaaggtctgtatgcatccaaggtagccatgctgtgaggctacgtgaacggcactgttgccatcctggtctacttcatccaacgagatgccctgttcttgcataaactgaagaagccacagaagaatcttttcctggccatagcaacctgcgtaatgaataaggcttggaaaatccttagaacaactcagttctgcaatggcttctgtttcgctcaccatccagcgtacgcactccaactgaccattctgatctgtcttcgttttgcgtatcacatcttcggcacagttctgggatcgtcttgagtgatgtgactgaataagatatgtcatcactaaagtcaatttcatccaaatcaaggtattcaggggcttccattattcttccttgcacattttgagtacggtcaaatacttataaattcctttcgctctttttacctcgactgccgttgcttttccccagctggggctctcctctcctccccgcctactttttgtccgcgcttcccacttttctcctcctgccccccacccccttccttgcttcttggcct

SEQ ID NO: 10344 - RNA, 1306 nt, Homo sapiens
  source 1..1306: mol_type = other RNA
ccagggaggctggtttggaggaatactccctgagcctggatactgggattctaagtctggttcgctgctctctgaggtgggagatgggctgtggccatccagggatttggaggccttgatgctgaaaggaaacctgcgtccccctgatgccaaggtgtgtttcttaatcatcaggtgcaggctttctgcgctgtccatactctctacgctttctacaatgggctgcggccttggtcggtcagccttcctcactggggtagtcttggggtcctcagagttgttggagtctgtgtcagactcactcagtgacctctgcatcagctgtctcagcctggctaacttcagttccctcttctccagtgggatctttttagaatttctagaggaagcctgagcatcctggaattccaaggacagtttttcctgggtgcagacattttctgagatttcctttcccaataactggcgtaagattttatcagaatcttcatcttttgctttgggtctagcccggctggaggctgacaggcttccaagaacctgaatcccctcttggactcctggcttgcttttggctacagaatcatcatctgcatctggagatttccactgggactttctggaggcaggtgaggatggtgaactgggtgaagaagggagtgacttgccctctgatttctgggcttctagaaattgttggagttggttctgcagcgtgacacgttctactgtttgttcctttagctgcttggttaacttcaccacttgagaggccagcgacatgcaggtctccaccaccaccaggtacctggagcacagggtgtgcccctgccgctcggcgctctgggagggcttttccccagcgtggttctgcatggtgacatttgctccatattcaaccaaggtctgtatgcatccaaggtagccatgctgtgaggctacgtgaacggcactgttgccatcctggtctacttcatccaacgagatgccctgttcttgcataaactgaagaagccacagaagaatcttttcctggccatagcaacctgcgtaatgaataaggcttggaaaatccttagaacaactcagttctgcaatggcttctgtttcgctcaccatccagcgtacgcactccaactgaccattctgatctgtcttcgttttgcgtatcacatcttcggcacagttctgggatcgtcttgagtgatgtgactgaatactcattctcaggacaatggcaagctcccagggcagcaactactgtcagtttggccctatgggaaccaaagcccattgcatcttccct

SEQ ID NO: 10345 - RNA, 1463 nt, Homo sapiens
  source 1..1463: mol_type = other RNA
ccagggaggctggtttggaggaatactccctgagcctggatactgggattctaagtctggttcgctgctctctgaggtgggagatgggctgtggccatccagggatttggaggccttgatgctgaaaggaaacctgcgtccccctgatgccaaggtgtgtttcttaatcatcaggtgcaggctttctgcgctgtccatactctctacgctttctacaatgggctgcggccttggtcggtcagccttcctcactggggtagtcttggggtcctcagagttgttggagtctgtgtcagactcactcagtgacctctgcatcagctgtctcagcctggctaacttcagttccctcttctccagtgggatctttttagaatttctagaggaagcctgagcatcctggaattccaaggacagtttttcctgggtgcagacattttctgagatttcctttcccaataactggcgtaagattttatcagaatcttcatcttttgctttgggtctagcccggctggaggctgacaggcttccaagaacctgaatcccctcttggactcctggcttgcttttggctacagaatcatcatctgcatctggagatttccactgggactttctggaggcaggtgaggatggtgaactgggtgaagaagggagtgacttgccctctgatttctgggcttctagaaattgttggagttggttctgcagcgtgacacgttctactgtttgttcctttagctgcttggttaacttcaccacttgagaggccagcgacatgcaggtctccaccaccaccaggtacctggagcacagggtgtgcccctgccgctcggcgctctgggagggcttttccccagcgtggttctgcatggtgacatttgctccatattcaaccaaggtctgtatgcatccaaggtagccatgctgtgaggctacgtgaacggcactgttgccatcctggtctacttcatccaacgagatgccctgttcttgcataaactgaagaagccacagaagaatcttttcctggccatagcaacctgcgtaatgaataaggcttggaaaatccttagaacaactcagttctgcaatggcttctgtttcgctcaccatccagcgtacgcactccaactgaccattctgatctgtcttcgttttgcgtatcacatcttcggcacagttctgggatcgtcttgagtgatgtgactgaatactcattctcaggacaatggcaagctcccagggcagcaactactgtcagtttggccctatgggaaccaaagcccattgcatcttccctgtctgtgtcctccaatccaagcttttgtagcctgttcccttgactcctattgtcagatatgtcatcactaaagtcaatttcatccaaatcaaggtattcaggggcttccattattcttccttgcacattttgagtacggtcaaatacttataaattc

SEQ ID NO: 10346 - RNA, 1533 nt, Homo sapiens
  source 1..1533: mol_type = other RNA
ccagggaggctggtttggaggaatactccctgagcctggatactgggattctaagtctggttcgctgctctctgaggtgggagatgggctgtggccatccagggatttggaggccttgatgctgaaaggaaacctgcgtccccctgatgccaaggtgtgtttcttaatcatcaggtgcaggctttctgcgctgtccatactctctacgctttctacaatgggctgcggccttggtcggtcagccttcctcactggggtagtcttggggtcctcagagttgttggagtctgtgtcagactcactcagtgacctctgcatcagctgtctcagcctggctaacttcagttccctcttctccagtgggatctttttagaatttctagaggaagcctgagcatcctggaattccaaggacagtttttcctgggtgcagacattttctgagatttcctttcccaataactggcgtaagattttatcagaatcttcatcttttgctttgggtctagcccggctggaggctgacaggcttccaagaacctgaatcccctcttggactcctggcttgcttttggctacagaatcatcatctgcatctggagatttccactgggactttctggaggcaggtgaggatggtgaactgggtgaagaagggagtgacttgccctctgatttctgggcttctagaaattgttggagttggttctgcagcgtgacacgttctactgtttgttcctttagctgcttggttaacttcaccacttgagaggccagcgacatgcaggtctccaccaccaccaggtacctggagcacagggtgtgcccctgccgctcggcgctctgggagggcttttccccagcgtggttctgcatggtgacatttgctccatattcaaccaaggtctgtatgcatccaaggtagccatgctgtgaggctacgtgaacggcactgttgccatcctggtctacttcatccaacgagatgccctgttcttgcataaactgaagaagccacagaagaatcttttcctggccatagcaacctgcgtaatgaataaggcttggaaaatccttagaacaactcagttctgcaatggcttctgtttcgctcaccatccagcgtacgcactccaactgaccattctgatctgtcttcgttttgcgtatcacatcttcggcacagttctgggatcgtcttgagtgatgtgactgaatactcattctcaggacaatggcaagctcccagggcagcaactactgtcagtttggccctatgggaaccaaagcccattgcatcttccctgtctgtgtcctccaatccaagcttttgtagcctgttcccttgactcctattgtcagatatgtcatcactaaagtcaatttcatccaaatcaaggtattcaggggcttccattattcttccttgcacattttgagtacggtcaaatacttataaattccagggatcccccggcctgcccgccggctcctgtccacgaacctgctctttctttacctttcgctcttttt

SEQ ID NO: 10347 - RNA, 2477 nt, Homo sapiens
  source 1..2477: mol_type = other RNA
ccagggaggctggtttggaggaatactccctgagcctggatactgggattctaagtctggttcgctgctctctgaggtgggagatgggctgtggccatccagggatttggaggccttgatgctgaaaggaaacctgcgtccccctgatgccaaggtgtgtttcttaatcatcaggtgcaggctttctgcgctgtccatactctctacgctttctacaatgggctgcggccttggtcggtcagccttcctcactggggtagtcttggggtcctcagagttgttggagtctgtgtcagactcactcagtgacctctgcatcagctgtctcagcctggctaacttcagttccctcttctccagtgggatctttttagaatttctagaggaagcctgagcatcctggaattccaaggacagtttttcctgggtgcagacattttctgagatttcctttcccaataactggcgtaagattttatcagaatcttcatcttttgctttgggtctagcccggctggaggctgacaggcttccaagaacctgaatcccctcttggactcctggcttgcttttggctacagaatcatcatctgcatctggagatttccactgggactttctggaggcaggtgaggatggtgaactgggtgaagaagggagtgacttgccctctgatttctgggcttctagaaattgttggagttggttctgcagcgtgacacgttctactgtttgttcctttagctgcttggttaacttcaccacttgagaggccagcgacatgcaggtctccaccaccaccaggtacctggagcacagggtgtgcccctgccgctcggcgctctgggagggcttttccccagcgtggttctgcatggtgacatttgctccatattcaaccaaggtctgtatgcatccaaggtagccatgctgtgaggctacgtgaacggcactgttgccatcctggtctacttcatccaacgagatgccctgttcttgcataaactgaagaagccacagaagaatcttttcctggccatagcaacctgcgtaatgaataaggcttggaaaatccttagaacaactcagttctgcaatggcttctgtttcgctcaccatccagcgtacgcactccaactgaccattcttaatggccaggcctgctggagtcaacttctcagtgttgcgctcattgaggcagtcttctcccatcaaagaagtgaggtgctgtagacactctgcgtgtccctgtgacgccgcaatatgtaatagattgtttccattttcgtcgtgaattttgtctagattgtctgcagctaggtgtggcaggagagagatctgtccttctttaacaatgttcaagatgcttttcacttttttcagatactcactcctttcttctgggccttgggagctggtccggtttaggccactgacctgctcttctggtttggattctgctgctgaggattgtaggtggaaggccctgagctggcagtctggtgttgtcttctcaacttttcgaccatgaggatcactaaatgtcttgtttaggaagtctttactctggttttcaggctcatatgcagagccacatttaaccagaggaggtgagatctcggtttcttcagtggacagcttgtgctggtcgtggatgacagctgatgcttttctcaagtgagggcttttcacgggagaaagaacacaaaatggtgccatgttggatgatgagctctcagaacttcctgtagagcaggctttgccagaaaggccattgatggttgtgcataagcccaaaattcttttttctgaagtcaccttggtaaaagaggcaagctgctgactggatttaatataaggcacatccagaatctcatccatgtcgaggtcgtagtgctccagttcacccagcgatgtgctgggctcagagctcttacctggtgggccgcccactccatctccagggccaagctcctgaggctgggggcccaggtcagactcaccccctttctggtactcaaccactttctggttcttttggtcatcactttcattgttctccagagtctctggctgatgtttcagtggcgaaacccgcttcactgggcggaacttactgtacacatcagcgattcctgtgggcttttgcgtgtttgtaataagagttgagatgccacaattccagctagagctagaaactgatctgtcttcgttttgcgtatcacatcttcggcacagttctgggatcgtcttgagtgatgtgactgaataagatatgtcatcactaaagtcaatttcatccaaatcaaggtattcaggggcttccattattcttccttgcacattttgagtacggtcaaatacttataaattccacctgcagatgaaagtcatcgccaagagacaaggccaagagagaaacattcccctctgaaatccacgcggaccagcctgggacgcagaacagcactagaggg

SEQ ID NO: 10348 - RNA, 2453 nt, Homo sapiens
  source 1..2453: mol_type = other RNA
ccagggaggctggtttggaggaatactccctgagcctggatactgggattctaagtctggttcgctgctctctgaggtgggagatgggctgtggccatccagggatttggaggccttgatgctgaaaggaaacctgcgtccccctgatgccaaggtgtgtttcttaatcatcaggtgcaggctttctgcgctgtccatactctctacgctttctacaatgggctgcggccttggtcggtcagccttcctcactggggtagtcttggggtcctcagagttgttggagtctgtgtcagactcactcagtgacctctgcatcagctgtctcagcctggctaacttcagttccctcttctccagtgggatctttttagaatttctagaggaagcctgagcatcctggaattccaaggacagtttttcctgggtgcagacattttctgagatttcctttcccaataactggcgtaagattttatcagaatcttcatcttttgctttgggtctagcccggctggaggctgacaggcttccaagaacctgaatcccctcttggactcctggcttgcttttggctacagaatcatcatctgcatctggagatttccactgggactttctggaggcaggtgaggatggtgaactgggtgaagaagggagtgacttgccctctgatttctgggcttctagaaattgttggagttggttctgcagcgtgacacgttctactgtttgttcctttagctgcttggttaacttcaccacttgagaggccagcgacatgcaggtctccaccaccaccaggtacctggagcacagggtgtgcccctgccgctcggcgctctgggagggcttttccccagcgtggttctgcatggtgacatttgctccatattcaaccaaggtctgtatgcatccaaggtagccatgctgtgaggctacgtgaacggcactgttgccatcctggtctacttcatccaacgagatgccctgttcttgcataaactgaagaagccacagaagaatcttttcctggccatagcaacctgcgtaatgaataaggcttggaaaatccttagaacaactcagttctgcaatggcttctgtttcgctcaccatccagcgtacgcactccaactgaccattcttaatggccaggcctgctggagtcaacttctcagtgttgcgctcattgaggcagtcttctcccatcaaagaagtgaggtgctgtagacactctgcgtgtccctgtgacgccgcaatatgtaatagattgtttccattttcgtcgtgaattttgtctagattgtctgcagctaggtgtggcaggagagagatctgtccttctttaacaatgttcaagatgcttttcacttttttcagatactcactcctttcttctgggccttgggagctggtccggtttaggccactgacctgctcttctggtttggattctgctgctgaggattgtaggtggaaggccctgagctggcagtctggtgttgtcttctcaacttttcgaccatgaggatcactaaatgtcttgtttaggaagtctttactctggttttcaggctcatatgcagagccacatttaaccagaggaggtgagatctcggtttcttcagtggacagcttgtgctggtcgtggatgacagctgatgcttttctcaagtgagggcttttcacgggagaaagaacacaaaatggtgccatgttggatgatgagctctcagaacttcctgtagagcaggctttgccagaaaggccattgatggttgtgcataagcccaaaattcttttttctgaagtcaccttggtaaaagaggcaagctgctgactggatttaatataaggcacatccagaatctcatccatgtcgaggtcgtagtgctccagttcacccagcgatgtgctgggctcagagctcttacctggtgggccgcccactccatctccagggccaagctcctgaggctgggggcccaggtcagactcaccccctttctggtactcaaccactttctggttcttttggtcatcactttcattgttctccagagtctctggctgatgtttcagtggcgaaacccgcttcactgggcggaacttactgtacacatcagcgattcctgtgggcttttgcgtgtttgtaataagagttgagatgccacaattccagctagagctagaaactgatctgtcttcgttttgcgtatcacatcttcggcacagttctgggatcgtcttgagtgatgtgactgaataagatatgtcatcactaaagtcaatttcatccaaatcaaggtattcaggggcttccattattcttccttgcacattttgagtacggtcaaatacttataaattccagggatcccccggcctgcccgccggctcctgtccacgaacctgctctttctttacctttcgctctttttacctcgact

SEQ ID NO: 10349 - RNA, 2422 nt, Homo sapiens
  source 1..2422: mol_type = other RNA
ccagggaggctggtttggaggaatactccctgagcctggatactgggattctaagtctggttcgctgctctctgaggtgggagatgggctgtggccatccagggatttggaggccttgatgctgaaaggaaacctgcgtccccctgatgccaaggtgtgtttcttaatcatcaggtgcaggctttctgcgctgtccatactctctacgctttctacaatgggctgcggccttggtcggtcagccttcctcactggggtagtcttggggtcctcagagttgttggagtctgtgtcagactcactcagtgacctctgcatcagctgtctcagcctggctaacttcagttccctcttctccagtgggatctttttagaatttctagaggaagcctgagcatcctggaattccaaggacagtttttcctgggtgcagacattttctgagatttcctttcccaataactggcgtaagattttatcagaatcttcatcttttgctttgggtctagcccggctggaggctgacaggcttccaagaacctgaatcccctcttggactcctggcttgcttttggctacagaatcatcatctgcatctggagatttccactgggactttctggaggcaggtgaggatggtgaactgggtgaagaagggagtgacttgccctctgatttctgggcttctagaaattgttggagttggttctgcagcgtgacacgttctactgtttgttcctttagctgcttggttaacttcaccacttgagaggccagcgacatgcaggtctccaccaccaccaggtacctggagcacagggtgtgcccctgccgctcggcgctctgggagggcttttccccagcgtggttctgcatggtgacatttgctccatattcaaccaaggtctgtatgcatccaaggtagccatgctgtgaggctacgtgaacggcactgttgccatcctggtctacttcatccaacgagatgccctgttcttgcataaactgaagaagccacagaagaatcttttcctggccatagcaacctgcgtaatgaataaggcttggaaaatccttagaacaactcagttctgcaatggcttctgtttcgctcaccatccagcgtacgcactccaactgaccattcttaatggccaggcctgctggagtcaacttctcagtgttgcgctcattgaggcagtcttctcccatcaaagaagtgaggtgctgtagacactctgcgtgtccctgtgacgccgcaatatgtaatagattgtttccattttcgtcgtgaattttgtctagattgtctgcagctaggtgtggcaggagagagatctgtccttctttaacaatgttcaagatgcttttcacttttttcagatactcactcctttcttctgggccttgggagctggtccggtttaggccactgacctgctcttctggtttggattctgctgctgaggattgtaggtggaaggccctgagctggcagtctggtgttgtcttctcaacttttcgaccatgaggatcactaaatgtcttgtttaggaagtctttactctggttttcaggctcatatgcagagccacatttaaccagaggaggtgagatctcggtttcttcagtggacagcttgtgctggtcgtggatgacagctgatgcttttctcaagtgagggcttttcacgggagaaagaacacaaaatggtgccatgttggatgatgagctctcagaacttcctgtagagcaggctttgccagaaaggccattgatggttgtgcataagcccaaaattcttttttctgaagtcaccttggtaaaagaggcaagctgctgactggatttaatataaggcacatccagaatctcatccatgtcgaggtcgtagtgctccagttcacccagcgatgtgctgggctcagagctcttacctggtgggccgcccactccatctccagggccaagctcctgaggctgggggcccaggtcagactcaccccctttctggtactcaaccactttctggttcttttggtcatcactttcattgttctccagagtctctggctgatgtttcagtggcgaaacccgcttcactgggcggaacttactgtacacatcagcgattcctgtgggcttttgcgtgtttgtaataagagttgagatgccacaattccagctagagctagaaactgatctgtcttcgttttgcgtatcacatcttcggcacagttctgggatcgtcttgagtgatgtgactgaataagatatgtcatcactaaagtcaatttcatccaaatcaaggtattcaggggcttccattattcttccttgcacattttgagtacggtcaaatacttataaattcccggggcgcccggcgcgccggcggctcaggagcgcgaagggactgact

SEQ ID NO: 10350 - RNA, 2492 nt, Homo sapiens
  source 1..2492: mol_type = other RNA
ccagggaggctggtttggaggaatactccctgagcctggatactgggattctaagtctggttcgctgctctctgaggtgggagatgggctgtggccatccagggatttggaggccttgatgctgaaaggaaacctgcgtccccctgatgccaaggtgtgtttcttaatcatcaggtgcaggctttctgcgctgtccatactctctacgctttctacaatgggctgcggccttggtcggtcagccttcctcactggggtagtcttggggtcctcagagttgttggagtctgtgtcagactcactcagtgacctctgcatcagctgtctcagcctggctaacttcagttccctcttctccagtgggatctttttagaatttctagaggaagcctgagcatcctggaattccaaggacagtttttcctgggtgcagacattttctgagatttcctttcccaataactggcgtaagattttatcagaatcttcatcttttgctttgggtctagcccggctggaggctgacaggcttccaagaacctgaatcccctcttggactcctggcttgcttttggctacagaatcatcatctgcatctggagatttccactgggactttctggaggcaggtgaggatggtgaactgggtgaagaagggagtgacttgccctctgatttctgggcttctagaaattgttggagttggttctgcagcgtgacacgttctactgtttgttcctttagctgcttggttaacttcaccacttgagaggccagcgacatgcaggtctccaccaccaccaggtacctggagcacagggtgtgcccctgccgctcggcgctctgggagggcttttccccagcgtggttctgcatggtgacatttgctccatattcaaccaaggtctgtatgcatccaaggtagccatgctgtgaggctacgtgaacggcactgttgccatcctggtctacttcatccaacgagatgccctgttcttgcataaactgaagaagccacagaagaatcttttcctggccatagcaacctgcgtaatgaataaggcttggaaaatccttagaacaactcagttctgcaatggcttctgtttcgctcaccatccagcgtacgcactccaactgaccattcttaatggccaggcctgctggagtcaacttctcagtgttgcgctcattgaggcagtcttctcccatcaaagaagtgaggtgctgtagacactctgcgtgtccctgtgacgccgcaatatgtaatagattgtttccattttcgtcgtgaattttgtctagattgtctgcagctaggtgtggcaggagagagatctgtccttctttaacaatgttcaagatgcttttcacttttttcagatactcactcctttcttctgggccttgggagctggtccggtttaggccactgacctgctcttctggtttggattctgctgctgaggattgtaggtggaaggccctgagctggcagtctggtgttgtcttctcaacttttcgaccatgaggatcactaaatgtcttgtttaggaagtctttactctggttttcaggctcatatgcagagccacatttaaccagaggaggtgagatctcggtttcttcagtggacagcttgtgctggtcgtggatgacagctgatgcttttctcaagtgagggcttttcacgggagaaagaacacaaaatggtgccatgttggatgatgagctctcagaacttcctgtagagcaggctttgccagaaaggccattgatggttgtgcataagcccaaaattcttttttctgaagtcaccttggtaaaagaggcaagctgctgactggatttaatataaggcacatccagaatctcatccatgtcgaggtcgtagtgctccagttcacccagcgatgtgctgggctcagagctcttacctggtgggccgcccactccatctccagggccaagctcctgaggctgggggcccaggtcagactcaccccctttctggtactcaaccactttctggttcttttggtcatcactttcattgttctccagagtctctggctgatgtttcagtggcgaaacccgcttcactgggcggaacttactgtacacatcagcgattcctgtgggcttttgcgtgtttgtaataagagttgagatgccacaattccagctagagctagaaactgatctgtcttcgttttgcgtatcacatcttcggcacagttctgggatcgtcttgagtgatgtgactgaataagatatgtcatcactaaagtcaatttcatccaaatcaaggtattcaggggcttccattattcttccttgcacattttgagtacggtcaaatacttataaattcccggggcgcccggcgcgccggcggctcaggagcgcgaagggactgactgaccgaccgacggaccgcagcggcaggagcagaacagcctcagccgaagtaggcgggcggtggaggcgct

SEQ ID NO: 10351 - RNA, 2646 nt, Homo sapiens
  source 1..2646: mol_type = other RNA
ccagggaggctggtttggaggaatactccctgagcctggatactgggattctaagtctggttcgctgctctctgaggtgggagatgggctgtggccatccagggatttggaggccttgatgctgaaaggaaacctgcgtccccctgatgccaaggtgtgtttcttaatcatcaggtgcaggctttctgcgctgtccatactctctacgctttctacaatgggctgcggccttggtcggtcagccttcctcactggggtagtcttggggtcctcagagttgttggagtctgtgtcagactcactcagtgacctctgcatcagctgtctcagcctggctaacttcagttccctcttctccagtgggatctttttagaatttctagaggaagcctgagcatcctggaattccaaggacagtttttcctgggtgcagacattttctgagatttcctttcccaataactggcgtaagattttatcagaatcttcatcttttgctttgggtctagcccggctggaggctgacaggcttccaagaacctgaatcccctcttggactcctggcttgcttttggctacagaatcatcatctgcatctggagatttccactgggactttctggaggcaggtgaggatggtgaactgggtgaagaagggagtgacttgccctctgatttctgggcttctagaaattgttggagttggttctgcagcgtgacacgttctactgtttgttcctttagctgcttggttaacttcaccacttgagaggccagcgacatgcaggtctccaccaccaccaggtacctggagcacagggtgtgcccctgccgctcggcgctctgggagggcttttccccagcgtggttctgcatggtgacatttgctccatattcaaccaaggtctgtatgcatccaaggtagccatgctgtgaggctacgtgaacggcactgttgccatcctggtctacttcatccaacgagatgccctgttcttgcataaactgaagaagccacagaagaatcttttcctggccatagcaacctgcgtaatgaataaggcttggaaaatccttagaacaactcagttctgcaatggcttctgtttcgctcaccatccagcgtacgcactccaactgaccattcttaatggccaggcctgctggagtcaacttctcagtgttgcgctcattgaggcagtcttctcccatcaaagaagtgaggtgctgtagacactctgcgtgtccctgtgacgccgcaatatgtaatagattgtttccattttcgtcgtgaattttgtctagattgtctgcagctaggtgtggcaggagagagatctgtccttctttaacaatgttcaagatgcttttcacttttttcagatactcactcctttcttctgggccttgggagctggtccggtttaggccactgacctgctcttctggtttggattctgctgctgaggattgtaggtggaaggccctgagctggcagtctggtgttgtcttctcaacttttcgaccatgaggatcactaaatgtcttgtttaggaagtctttactctggttttcaggctcatatgcagagccacatttaaccagaggaggtgagatctcggtttcttcagtggacagcttgtgctggtcgtggatgacagctgatgcttttctcaagtgagggcttttcacgggagaaagaacacaaaatggtgccatgttggatgatgagctctcagaacttcctgtagagcaggctttgccagaaaggccattgatggttgtgcataagcccaaaattcttttttctgaagtcaccttggtaaaagaggcaagctgctgactggatttaatataaggcacatccagaatctcatccatgtcgaggtcgtagtgctccagttcacccagcgatgtgctgggctcagagctcttacctggtgggccgcccactccatctccagggccaagctcctgaggctgggggcccaggtcagactcaccccctttctggtactcaaccactttctggttcttttggtcatcactttcattgttctccagagtctctggctgatgtttcagtggcgaaacccgcttcactgggcggaacttactgtacacatcagcgattcctgtgggcttttgcgtgtttgtaataagagttgagatgccacaattccagctagagctagaaactgatctgtcttcgttttgcgtatcacatcttcggcacagttctgggatcgtcttgagtgatgtgactgaataagatatgtcatcactaaagtcaatttcatccaaatcaaggtattcaggggcttccattattcttccttgcacattttgagtacggtcaaatacttataaattccgtgatccaagcgttaaccgctgccatctcattggtccccagaccattccagggttccagcataaactgggagaagagactcgggaaggcggggaacggaaggtgggcattgccctgggaaactcatgtctgagaagccttttggcagagtattttgcgttggcacggagtcttcacccccacccctccccccgaagctcgcccacccctgaggacgtggccaaggagaggagggcaagggtggctttgcctgcctggaatgttctgtgctc

SEQ ID NO: 10352 - RNA, 2517 nt, Homo sapiens
  source 1..2517: mol_type = other RNA
ccagggaggctggtttggaggaatactccctgagcctggatactgggattctaagtctggttcgctgctctctgaggtgggagatgggctgtggccatccagggatttggaggccttgatgctgaaaggaaacctgcgtccccctgatgccaaggtgtgtttcttaatcatcaggtgcaggctttctgcgctgtccatactctctacgctttctacaatgggctgcggccttggtcggtcagccttcctcactggggtagtcttggggtcctcagagttgttggagtctgtgtcagactcactcagtgacctctgcatcagctgtctcagcctggctaacttcagttccctcttctccagtgggatctttttagaatttctagaggaagcctgagcatcctggaattccaaggacagtttttcctgggtgcagacattttctgagatttcctttcccaataactggcgtaagattttatcagaatcttcatcttttgctttgggtctagcccggctggaggctgacaggcttccaagaacctgaatcccctcttggactcctggcttgcttttggctacagaatcatcatctgcatctggagatttccactgggactttctggaggcaggtgaggatggtgaactgggtgaagaagggagtgacttgccctctgatttctgggcttctagaaattgttggagttggttctgcagcgtgacacgttctactgtttgttcctttagctgcttggttaacttcaccacttgagaggccagcgacatgcaggtctccaccaccaccaggtacctggagcacagggtgtgcccctgccgctcggcgctctgggagggcttttccccagcgtggttctgcatggtgacatttgctccatattcaaccaaggtctgtatgcatccaaggtagccatgctgtgaggctacgtgaacggcactgttgccatcctggtctacttcatccaacgagatgccctgttcttgcataaactgaagaagccacagaagaatcttttcctggccatagcaacctgcgtaatgaataaggcttggaaaatccttagaacaactcagttctgcaatggcttctgtttcgctcaccatccagcgtacgcactccaactgaccattcttaatggccaggcctgctggagtcaacttctcagtgttgcgctcattgaggcagtcttctcccatcaaagaagtgaggtgctgtagacactctgcgtgtccctgtgacgccgcaatatgtaatagattgtttccattttcgtcgtgaattttgtctagattgtctgcagctaggtgtggcaggagagagatctgtccttctttaacaatgttcaagatgcttttcacttttttcagatactcactcctttcttctgggccttgggagctggtccggtttaggccactgacctgctcttctggtttggattctgctgctgaggattgtaggtggaaggccctgagctggcagtctggtgttgtcttctcaacttttcgaccatgaggatcactaaatgtcttgtttaggaagtctttactctggttttcaggctcatatgcagagccacatttaaccagaggaggtgagatctcggtttcttcagtggacagcttgtgctggtcgtggatgacagctgatgcttttctcaagtgagggcttttcacgggagaaagaacacaaaatggtgccatgttggatgatgagctctcagaacttcctgtagagcaggctttgccagaaaggccattgatggttgtgcataagcccaaaattcttttttctgaagtcaccttggtaaaagaggcaagctgctgactggatttaatataaggcacatccagaatctcatccatgtcgaggtcgtagtgctccagttcacccagcgatgtgctgggctcagagctcttacctggtgggccgcccactccatctccagggccaagctcctgaggctgggggcccaggtcagactcaccccctttctggtactcaaccactttctggttcttttggtcatcactttcattgttctccagagtctctggctgatgtttcagtggcgaaacccgcttcactgggcggaacttactgtacacatcagcgattcctgtgggcttttgcgtgtttgtaataagagttgagatgccacaattccagctagagctagaaactgatctgtcttcgttttgcgtatcacatcttcggcacagttctgggatcgtcttgagtgatgtgactgaataagatatgtcatcactaaagtcaatttcatccaaatcaaggtattcaggggcttccattattcttccttgcacattttgagtacggtcaaatacttataaattcctgctctttctttacctttcgctctttttacctcgactgccgttgcttttccccagctggggctctcctctcctccccgcctactttttgtccgcgcttcccacttttctcctcctgccccccacccccttccttgcttcttg

SEQ ID NO: 10353 - RNA, 2502 nt, Homo sapiens
  source 1..2502: mol_type = other RNA
ccagggaggctggtttggaggaatactccctgagcctggatactgggattctaagtctggttcgctgctctctgaggtgggagatgggctgtggccatccagggatttggaggccttgatgctgaaaggaaacctgcgtccccctgatgccaaggtgtgtttcttaatcatcaggtgcaggctttctgcgctgtccatactctctacgctttctacaatgggctgcggccttggtcggtcagccttcctcactggggtagtcttggggtcctcagagttgttggagtctgtgtcagactcactcagtgacctctgcatcagctgtctcagcctggctaacttcagttccctcttctccagtgggatctttttagaatttctagaggaagcctgagcatcctggaattccaaggacagtttttcctgggtgcagacattttctgagatttcctttcccaataactggcgtaagattttatcagaatcttcatcttttgctttgggtctagcccggctggaggctgacaggcttccaagaacctgaatcccctcttggactcctggcttgcttttggctacagaatcatcatctgcatctggagatttccactgggactttctggaggcaggtgaggatggtgaactgggtgaagaagggagtgacttgccctctgatttctgggcttctagaaattgttggagttggttctgcagcgtgacacgttctactgtttgttcctttagctgcttggttaacttcaccacttgagaggccagcgacatgcaggtctccaccaccaccaggtacctggagcacagggtgtgcccctgccgctcggcgctctgggagggcttttccccagcgtggttctgcatggtgacatttgctccatattcaaccaaggtctgtatgcatccaaggtagccatgctgtgaggctacgtgaacggcactgttgccatcctggtctacttcatccaacgagatgccctgttcttgcataaactgaagaagccacagaagaatcttttcctggccatagcaacctgcgtaatgaataaggcttggaaaatccttagaacaactcagttctgcaatggcttctgtttcgctcaccatccagcgtacgcactccaactgaccattcttaatggccaggcctgctggagtcaacttctcagtgttgcgctcattgaggcagtcttctcccatcaaagaagtgaggtgctgtagacactctgcgtgtccctgtgacgccgcaatatgtaatagattgtttccattttcgtcgtgaattttgtctagattgtctgcagctaggtgtggcaggagagagatctgtccttctttaacaatgttcaagatgcttttcacttttttcagatactcactcctttcttctgggccttgggagctggtccggtttaggccactgacctgctcttctggtttggattctgctgctgaggattgtaggtggaaggccctgagctggcagtctggtgttgtcttctcaacttttcgaccatgaggatcactaaatgtcttgtttaggaagtctttactctggttttcaggctcatatgcagagccacatttaaccagaggaggtgagatctcggtttcttcagtggacagcttgtgctggtcgtggatgacagctgatgcttttctcaagtgagggcttttcacgggagaaagaacacaaaatggtgccatgttggatgatgagctctcagaacttcctgtagagcaggctttgccagaaaggccattgatggttgtgcataagcccaaaattcttttttctgaagtcaccttggtaaaagaggcaagctgctgactggatttaatataaggcacatccagaatctcatccatgtcgaggtcgtagtgctccagttcacccagcgatgtgctgggctcagagctcttacctggtgggccgcccactccatctccagggccaagctcctgaggctgggggcccaggtcagactcaccccctttctggtactcaaccactttctggttcttttggtcatcactttcattgttctccagagtctctggctgatgtttcagtggcgaaacccgcttcactgggcggaacttactgtacacatcagcgattcctgtgggcttttgcgtgtttgtaataagagttgagatgccacaattccagctagagctagaaactgatctgtcttcgttttgcgtatcacatcttcggcacagttctgggatcgtcttgagtgatgtgactgaataagatatgtcatcactaaagtcaatttcatccaaatcaaggtattcaggggcttccattattcttccttgcacattttgagtacggtcaaatacttataaattcctttcgctctttttacctcgactgccgttgcttttccccagctggggctctcctctcctccccgcctactttttgtccgcgcttcccacttttctcctcctgccccccacccccttccttgcttcttg

SEQ ID NO: 10354 - RNA, 2503 nt, Homo sapiens
  source 1..2503: mol_type = other RNA
ccagggaggctggtttggaggaatactccctgagcctggatactgggattctaagtctggttcgctgctctctgaggtgggagatgggctgtggccatccagggatttggaggccttgatgctgaaaggaaacctgcgtccccctgatgccaaggtgtgtttcttaatcatcaggtgcaggctttctgcgctgtccatactctctacgctttctacaatgggctgcggccttggtcggtcagccttcctcactggggtagtcttggggtcctcagagttgttggagtctgtgtcagactcactcagtgacctctgcatcagctgtctcagcctggctaacttcagttccctcttctccagtgggatctttttagaatttctagaggaagcctgagcatcctggaattccaaggacagtttttcctgggtgcagacattttctgagatttcctttcccaataactggcgtaagattttatcagaatcttcatcttttgctttgggtctagcccggctggaggctgacaggcttccaagaacctgaatcccctcttggactcctggcttgcttttggctacagaatcatcatctgcatctggagatttccactgggactttctggaggcaggtgaggatggtgaactgggtgaagaagggagtgacttgccctctgatttctgggcttctagaaattgttggagttggttctgcagcgtgacacgttctactgtttgttcctttagctgcttggttaacttcaccacttgagaggccagcgacatgcaggtctccaccaccaccaggtacctggagcacagggtgtgcccctgccgctcggcgctctgggagggcttttccccagcgtggttctgcatggtgacatttgctccatattcaaccaaggtctgtatgcatccaaggtagccatgctgtgaggctacgtgaacggcactgttgccatcctggtctacttcatccaacgagatgccctgttcttgcataaactgaagaagccacagaagaatcttttcctggccatagcaacctgcgtaatgaataaggcttggaaaatccttagaacaactcagttctgcaatggcttctgtttcgctcaccatccagcgtacgcactccaactgaccattcttaatggccaggcctgctggagtcaacttctcagtgttgcgctcattgaggcagtcttctcccatcaaagaagtgaggtgctgtagacactctgcgtgtccctgtgacgccgcaatatgtaatagattgtttccattttcgtcgtgaattttgtctagattgtctgcagctaggtgtggcaggagagagatctgtccttctttaacaatgttcaagatgcttttcacttttttcagatactcactcctttcttctgggccttgggagctggtccggtttaggccactgacctgctcttctggtttggattctgctgctgaggattgtaggtggaaggccctgagctggcagtctggtgttgtcttctcaacttttcgaccatgaggatcactaaatgtcttgtttaggaagtctttactctggttttcaggctcatatgcagagccacatttaaccagaggaggtgagatctcggtttcttcagtggacagcttgtgctggtcgtggatgacagctgatgcttttctcaagtgagggcttttcacgggagaaagaacacaaaatggtgccatgttggatgatgagctctcagaacttcctgtagagcaggctttgccagaaaggccattgatggttgtgcataagcccaaaattcttttttctgaagtcaccttggtaaaagaggcaagctgctgactggatttaatataaggcacatccagaatctcatccatgtcgaggtcgtagtgctccagttcacccagcgatgtgctgggctcagagctcttacctggtgggccgcccactccatctccagggccaagctcctgaggctgggggcccaggtcagactcaccccctttctggtactcaaccactttctggttcttttggtcatcactttcattgttctccagagtctctggctgatgtttcagtggcgaaacccgcttcactgggcggaacttactgtacacatcagcgattcctgtgggcttttgcgtgtttgtaataagagttgagatgccacaattccagctagagctagaaactgatctgtcttcgttttgcgtatcacatcttcggcacagttctgggatcgtcttgagtgatgtgactgaataagatatgtcatcactaaagtcaatttcatccaaatcaaggtattcaggggcttccattattcttccttgcacattttgagtacggtcaaatacttataaattcctttcgctctttttacctcgactgccgttgcttttccccagctggggctctcctctcctccccgcctactttttgtccgcgcttcccacttttctcctcctgccccccacccccttccttgcttcttgg

SEQ ID NO: 10355 - RNA, 3022 nt, Homo sapiens
  source 1..3022: mol_type = other RNA
ccagggaggctggtttggaggaatactccctgagcctggatactgggattctaagtctggttcgctgctctctgaggtgggagatgggctgtggccatccagggatttggaggccttgatgctgaaaggaaacctgcgtccccctgatgccaaggtgtgtttcttaatcatcaggtgcaggctttctgcgctgtccatactctctacgctttctacaatgggctgcggccttggtcggtcagccttcctcactggggtagtcttggggtcctcagagttgttggagtctgtgtcagactcactcagtgacctctgcatcagctgtctcagcctggctaacttcagttccctcttctccagtgggatctttttagaatttctagaggaagcctgagcatcctggaattccaaggacagtttttcctgggtgcagacattttctgagatttcctttcccaataactggcgtaagattttatcagaatcttcatcttttgctttgggtctagcccggctggaggctgacaggcttccaagaacctgaatcccctcttggactcctggcttgcttttggctacagaatcatcatctgcatctggagatttccactgggactttctggaggcaggtgaggatggtgaactgggtgaagaagggagtgacttgccctctgatttctgggcttctagaaattgttggagttggttctgcagcgtgacacgttctactgtttgttcctttagctgcttggttaacttcaccacttgagaggccagcgacatgcaggtctccaccaccaccaggtacctggagcacagggtgtgcccctgccgctcggcgctctgggagggcttttccccagcgtggttctgcatggtgacatttgctccatattcaaccaaggtctgtatgcatccaaggtagccatgctgtgaggctacgtgaacggcactgttgccatcctggtctacttcatccaacgagatgccctgttcttgcataaactgaagaagccacagaagaatcttttcctggccatagcaacctgcgtaatgaataaggcttggaaaatccttagaacaactcagttctgcaatggcttctgtttcgctcaccatccagcgtacgcactccaactgaccattcttaatggccaggcctgctggagtcaacttctcagtgttgcgctcattgaggcagtcttctcccatcaaagaagtgaggtgctgtagacactctgcgtgtccctgtgacgccgcaatatgtaatagattgtttccattttcgtcgtgaattttgtctagattgtctgcagctaggtgtggcaggagagagatctgtccttctttaacaatgttcaagatgcttttcacttttttcagatactcactcctttcttctgggccttgggagctggtccggtttaggccactgacctgctcttctggtttggattctgctgctgaggattgtaggtggaaggccctgagctggcagtctggtgttgtcttctcaacttttcgaccatgaggatcactaaatgtcttgtttaggaagtctttactctggttttcaggctcatatgcagagccacatttaaccagaggaggtgagatctcggtttcttcagtggacagcttgtgctggtcgtggatgacagctgatgcttttctcaagtgagggcttttcacgggagaaagaacacaaaatggtgccatgttggatgatgagctctcagaacttcctgtagagcaggctttgccagaaaggccattgatggttgtgcataagcccaaaattcttttttctgaagtcaccttggtaaaagaggcaagctgctgactggatttaatataaggcacatccagaatctcatccatgtcgaggtcgtagtgctccagttcacccagcgatgtgctgggctcagagctcttacctggtgggccgcccactccatctccagggccaagctcctgaggctgggggcccaggtcagactcaccccctttctggtactcaaccactttctggttcttttggtcatcactttcattgttctccagagtctctggctgatgtttcagtggcgaaacccgcttcactgggcggaacttactgtacacatcagcgattcctgtgggcttttgcgtgtttgtaataagagttgagatgccacaattccagctagagctagaaactgatctgtcttcgttttgcgtatcacatcttcggcacagttctgggatcgtcttgagtgatgtgactgaatactcattctcaggacaatggcaagctcccagggcagcaactactgtcagtttggccctatgggaaccaaagcccattgcatcttccctgtctgtgtcctccaatccaagcttttgtagcctgttcccttgactcctattgtcagatatgtcatcactaaagtcaatttcatccaaatcaaggtattcaggggcttccattattcttccttgcacattttgagtacggtcaaatacttataaattccacctgcagatgaaagtcatcgccaagagacaaggccaagagagaaacattcccctctgaaatccacgcggaccagcctgggacgcagaacagcactagagggaggctggcggagcccgggctggacagggcagtcggggagctggtgctgatgagcgaggggcggcagcaacaccagacgtcccttttctacagctattattaccgttgttagtactgtcgctattactattacttcgcccctccttatctcagcttttccgagccgcggaactgcccatccctgcctgcgataagatcccgggtgacagcaagaataagaaccacatgaggcgggcaaatgaaaagaacaatcctttggaaaccgaggcgggggttgtttccccctttccccagtaaagcagccgctgccgccaccactgttactgttactatagagacctccccctcaaaccctttctgcagaggcgcctctgctgcccggagcagccgagactcgcggcacaa

SEQ ID NO: 10356 - RNA, 2646 nt, Homo sapiens
  source 1..2646: mol_type = other RNA
ccagggaggctggtttggaggaatactccctgagcctggatactgggattctaagtctggttcgctgctctctgaggtgggagatgggctgtggccatccagggatttggaggccttgatgctgaaaggaaacctgcgtccccctgatgccaaggtgtgtttcttaatcatcaggtgcaggctttctgcgctgtccatactctctacgctttctacaatgggctgcggccttggtcggtcagccttcctcactggggtagtcttggggtcctcagagttgttggagtctgtgtcagactcactcagtgacctctgcatcagctgtctcagcctggctaacttcagttccctcttctccagtgggatctttttagaatttctagaggaagcctgagcatcctggaattccaaggacagtttttcctgggtgcagacattttctgagatttcctttcccaataactggcgtaagattttatcagaatcttcatcttttgctttgggtctagcccggctggaggctgacaggcttccaagaacctgaatcccctcttggactcctggcttgcttttggctacagaatcatcatctgcatctggagatttccactgggactttctggaggcaggtgaggatggtgaactgggtgaagaagggagtgacttgccctctgatttctgggcttctagaaattgttggagttggttctgcagcgtgacacgttctactgtttgttcctttagctgcttggttaacttcaccacttgagaggccagcgacatgcaggtctccaccaccaccaggtacctggagcacagggtgtgcccctgccgctcggcgctctgggagggcttttccccagcgtggttctgcatggtgacatttgctccatattcaaccaaggtctgtatgcatccaaggtagccatgctgtgaggctacgtgaacggcactgttgccatcctggtctacttcatccaacgagatgccctgttcttgcataaactgaagaagccacagaagaatcttttcctggccatagcaacctgcgtaatgaataaggcttggaaaatccttagaacaactcagttctgcaatggcttctgtttcgctcaccatccagcgtacgcactccaactgaccattcttaatggccaggcctgctggagtcaacttctcagtgttgcgctcattgaggcagtcttctcccatcaaagaagtgaggtgctgtagacactctgcgtgtccctgtgacgccgcaatatgtaatagattgtttccattttcgtcgtgaattttgtctagattgtctgcagctaggtgtggcaggagagagatctgtccttctttaacaatgttcaagatgcttttcacttttttcagatactcactcctttcttctgggccttgggagctggtccggtttaggccactgacctgctcttctggtttggattctgctgctgaggattgtaggtggaaggccctgagctggcagtctggtgttgtcttctcaacttttcgaccatgaggatcactaaatgtcttgtttaggaagtctttactctggttttcaggctcatatgcagagccacatttaaccagaggaggtgagatctcggtttcttcagtggacagcttgtgctggtcgtggatgacagctgatgcttttctcaagtgagggcttttcacgggagaaagaacacaaaatggtgccatgttggatgatgagctctcagaacttcctgtagagcaggctttgccagaaaggccattgatggttgtgcataagcccaaaattcttttttctgaagtcaccttggtaaaagaggcaagctgctgactggatttaatataaggcacatccagaatctcatccatgtcgaggtcgtagtgctccagttcacccagcgatgtgctgggctcagagctcttacctggtgggccgcccactccatctccagggccaagctcctgaggctgggggcccaggtcagactcaccccctttctggtactcaaccactttctggttcttttggtcatcactttcattgttctccagagtctctggctgatgtttcagtggcgaaacccgcttcactgggcggaacttactgtacacatcagcgattcctgtgggcttttgcgtgtttgtaataagagttgagatgccacaattccagctagagctagaaactgatctgtcttcgttttgcgtatcacatcttcggcacagttctgggatcgtcttgagtgatgtgactgaatactcattctcaggacaatggcaagctcccagggcagcaactactgtcagtttggccctatgggaaccaaagcccattgcatcttccctgtctgtgtcctccaatccaagcttttgtagcctgttcccttgactcctattgtcagatatgtcatcactaaagtcaatttcatccaaatcaaggtattcaggggcttccattattcttccttgcacattttgagtacggtcaaatacttataaattcccggggcgcccggcgcgccggcggctcaggagcgcgaagggactgactgaccgaccgacggaccgcagcggcaggagcagaacagcctcagccgaagtaggcgggcggtggaggcgctgccgcggccccgc

SEQ ID NO: 10357 - RNA, 2648 nt, Homo sapiens
  source 1..2648: mol_type = other RNA
ccagggaggctggtttggaggaatactccctgagcctggatactgggattctaagtctggttcgctgctctctgaggtgggagatgggctgtggccatccagggatttggaggccttgatgctgaaaggaaacctgcgtccccctgatgccaaggtgtgtttcttaatcatcaggtgcaggctttctgcgctgtccatactctctacgctttctacaatgggctgcggccttggtcggtcagccttcctcactggggtagtcttggggtcctcagagttgttggagtctgtgtcagactcactcagtgacctctgcatcagctgtctcagcctggctaacttcagttccctcttctccagtgggatctttttagaatttctagaggaagcctgagcatcctggaattccaaggacagtttttcctgggtgcagacattttctgagatttcctttcccaataactggcgtaagattttatcagaatcttcatcttttgctttgggtctagcccggctggaggctgacaggcttccaagaacctgaatcccctcttggactcctggcttgcttttggctacagaatcatcatctgcatctggagatttccactgggactttctggaggcaggtgaggatggtgaactgggtgaagaagggagtgacttgccctctgatttctgggcttctagaaattgttggagttggttctgcagcgtgacacgttctactgtttgttcctttagctgcttggttaacttcaccacttgagaggccagcgacatgcaggtctccaccaccaccaggtacctggagcacagggtgtgcccctgccgctcggcgctctgggagggcttttccccagcgtggttctgcatggtgacatttgctccatattcaaccaaggtctgtatgcatccaaggtagccatgctgtgaggctacgtgaacggcactgttgccatcctggtctacttcatccaacgagatgccctgttcttgcataaactgaagaagccacagaagaatcttttcctggccatagcaacctgcgtaatgaataaggcttggaaaatccttagaacaactcagttctgcaatggcttctgtttcgctcaccatccagcgtacgcactccaactgaccattcttaatggccaggcctgctggagtcaacttctcagtgttgcgctcattgaggcagtcttctcccatcaaagaagtgaggtgctgtagacactctgcgtgtccctgtgacgccgcaatatgtaatagattgtttccattttcgtcgtgaattttgtctagattgtctgcagctaggtgtggcaggagagagatctgtccttctttaacaatgttcaagatgcttttcacttttttcagatactcactcctttcttctgggccttgggagctggtccggtttaggccactgacctgctcttctggtttggattctgctgctgaggattgtaggtggaaggccctgagctggcagtctggtgttgtcttctcaacttttcgaccatgaggatcactaaatgtcttgtttaggaagtctttactctggttttcaggctcatatgcagagccacatttaaccagaggaggtgagatctcggtttcttcagtggacagcttgtgctggtcgtggatgacagctgatgcttttctcaagtgagggcttttcacgggagaaagaacacaaaatggtgccatgttggatgatgagctctcagaacttcctgtagagcaggctttgccagaaaggccattgatggttgtgcataagcccaaaattcttttttctgaagtcaccttggtaaaagaggcaagctgctgactggatttaatataaggcacatccagaatctcatccatgtcgaggtcgtagtgctccagttcacccagcgatgtgctgggctcagagctcttacctggtgggccgcccactccatctccagggccaagctcctgaggctgggggcccaggtcagactcaccccctttctggtactcaaccactttctggttcttttggtcatcactttcattgttctccagagtctctggctgatgtttcagtggcgaaacccgcttcactgggcggaacttactgtacacatcagcgattcctgtgggcttttgcgtgtttgtaataagagttgagatgccacaattccagctagagctagaaactgatctgtcttcgttttgcgtatcacatcttcggcacagttctgggatcgtcttgagtgatgtgactgaatactcattctcaggacaatggcaagctcccagggcagcaactactgtcagtttggccctatgggaaccaaagcccattgcatcttccctgtctgtgtcctccaatccaagcttttgtagcctgttcccttgactcctattgtcagatatgtcatcactaaagtcaatttcatccaaatcaaggtattcaggggcttccattattcttccttgcacattttgagtacggtcaaatacttataaattcccggggcgcccggcgcgccggcggctcaggagcgcgaagggactgactgaccgaccgacggaccgcagcggcaggagcagaacagcctcagccgaagtaggcgggcggtggaggcgctgccgcggccccgcta

SEQ ID NO: 10358 - RNA, 3867 nt, Homo sapiens
  source 1..3867: mol_type = other RNA
ccagggaggctggtttggaggaatactccctgagcctggatactgggattctaagtctggttcgctgctctctgaggtgggagatgggctgtggccatccagggatttggaggccttgatgctgaaaggaaacctgcgtccccctgatgccaaggtgtgtttcttaatcatcaggtgcaggctttctgcgctgtccatactctctacgctttctacaatgggctgcggccttggtcggtcagccttcctcactggggtagtcttggggtcctcagagttgttggagtctgtgtcagactcactcagtgacctctgcatcagctgtctcagcctggctaacttcagttccctcttctccagtgggatctttttagaatttctagaggaagcctgagcatcctggaattccaaggacagtttttcctgggtgcagacattttctgagatttcctttcccaataactggcgtaagattttatcagaatcttcatcttttgctttgggtctagcccggctggaggctgacaggcttccaagaacctgaatcccctcttggactcctggcttgcttttggctacagaatcatcatctgcatctggagatttccactgggactttctggaggcaggtgaggatggtgaactgggtgaagaagggagtgacttgccctctgatttctgggcttctagaaattgttggagttggttctgcagcgtgacacgttctactgtttgttcctttagctgcttggttaacttcaccacttgagaggccagcgacatgcaggtctccaccaccaccaggtacctggagcacagggtgtgcccctgccgctcggcgctctgggagggcttttccccagcgtggttctgcatggtgacatttgctccatattcaaccaaggtctgtatgcatccaaggtagccatgctgtgaggctacgtgaacggcactgttgccatcctggtctacttcatccaacgagatgccctgttcttgcataaactgaagaagccacagaagaatcttttcctggccatagcaacctgcgtaatgaataaggcttggaaaatccttagaacaactcagttctgcaatggcttctgtttcgctcaccatccagcgtacgcactccaactgaccattcttaatggccaggcctgctggagtcaacttctcagtgttgcgctcattgaggcagtcttctcccatcaaagaagtgaggtgctgtagacactctgcgtgtccctgtgacgccgcaatatgtaatagattgtttccattttcgtcgtgaattttgtctagattgtctgcagctaggtgtggcaggagagagatctgtccttctttaacaatgttcaagatgcttttcacttttttcagatactcactcctttcttctgggccttgggagctggtccggtttaggccactgacctgctcttctggtttggattctgctgctgaggattgtaggtggaaggccctgagctggcagtctggtgttgtcttctcaacttttcgaccatgaggatcactaaatgtcttgtttaggaagtctttactctggttttcaggctcatatgcagagccacatttaaccagaggaggtgagatctcggtttcttcagtggacagcttgtgctggtcgtggatgacagctgatgcttttctcaagtgagggcttttcacgggagaaagaacacaaaatggtgccatgttggatgatgagctctcagaacttcctgtagagcaggctttgccagaaaggccattgatggttgtgcataagcccaaaattcttttttctgaagtcaccttggtaaaagaggcaagctgctgactggatttaatataaggcacatccagaatctcatccatgtcgaggtcgtagtgctccagttcacccagcgatgtgctgggctcagagctcttacctggtgggccgcccactccatctccagggccaagctcctgaggctgggggcccaggtcagactcaccccctttctggtactcaaccactttctggttcttttggtcatcactttcattgttctccagagtctctggctgatgtttcagtggcgaaacccgcttcactgggcggaacttactgtacacatcagcgattcctgtgggcttttgcgtgtttgtaataagagttgagatgccacaattccagctagagctagaaactgatctgtcttcgttttgcgtatcacatcttcggcacagttctgggatcgtcttgagtgatgtgactgaatactcattctcaggacaatggcaagctcccagggcagcaactactgtcagtttggccctatgggaaccaaagcccattgcatcttccctgtctgtgtcctccaatccaagcttttgtagcctgttcccttgactcctattgtcagatatgtcatcactaaagtcaatttcatccaaatcaaggtattcaggggcttccattattcttccttgcacattttgagtacggtcaaatacttataaattcctcaaacccatcacttgatttaattttcctgtttcctctcctttttttcccatatgtatataccatttttaaagtcttaattacaatagatacagagtccatccaagaaaggattaggatgttacttccatgtttaaatgagattatccatttagcaaatgttaaaaattcttctgaaatcacagtaaggcttacaatgaaaagaaaaccaacttgtatttgtaaaaaatatttaaaatcagaaattttattatttgtagaaatctgaaaataggttatcaaacaaattgcttggtataaaaatgtcacttttcttcaatttacaaagattttcagaggaaaatatatgtactctgcttggaaattactcaaaacaacattctctcctactgtgatggattctgatacaatccagactctttggatactagcgtgttcactaggagactttcttccaatccaatttcttttcatgaaatctgtactccgtgatgaactattgatttacagactctgttcccacggccttggtgaacaacacacagatgatgctgggtgccaggatatggtataaacatcagcaggaacatggaaatatggggagatgaagcagagaaacatgcatcgaagctggggaccaaatggatctttaaataaatgaaactataaaatgtggatgaacatgtcttaattaagtaaattaacaaataaccattgcacccctgtttgaggtgctccaacaatatagacagcaatatccagttgagtgtagccattccaatagaatataaccagcggataataactcatggcatcacaacaggaatctttcaatttgcacttgcaggatggtagtgaggttctttattctataggcaagaacacaagacttacaacaggtgcagctcattataggaagtcttgggccactgcccatatttatttctgtgggttggatggccccaccttagactaaggctcctaggcatctggaatttgcctctacttcccagcaggcctccacatgctatctcctttaagatgtctcattctgttcatgatccaatttattttgtctggtttcaatgcttgtctctttcagggtgccactttaagaatatttacattctcaattataatgtgcagaaatccccgtggttttccaatcctgactacattccccaacattaactgcttctttacaggtaagagtgagtctgcagttgtcccagtggccaatacaatgcctcctcttctctcgtctgcccttccaccaagcctctggcactctcaggcactcttttccggggcgcccggcgcgccggcggctcaggagcgcgaagggactgact

SEQ ID NO: 10359 - RNA, 4975 nt, Homo sapiens
  source 1..4975: mol_type = other RNA
ccagggaggctggtttggaggaatactccctgagcctggatactgggattctaagtctggttcgctgctctctgaggtgggagatgggctgtggccatccagggatttggaggccttgatgctgaaaggaaacctgcgtccccctgatgccaaggtgtgtttcttaatcatcaggtgcaggctttctgcgctgtccatactctctacgctttctacaatgggctgcggccttggtcggtcagccttcctcactggggtagtcttggggtcctcagagttgttggagtctgtgtcagactcactcagtgacctctgcatcagctgtctcagcctggctaacttcagttccctcttctccagtgggatctttttagaatttctagaggaagcctgagcatcctggaattccaaggacagtttttcctgggtgcagacattttctgagatttcctttcccaataactggcgtaagattttatcagaatcttcatcttttgctttgggtctagcccggctggaggctgacaggcttccaagaacctgaatcccctcttggactcctggcttgcttttggctacagaatcatcatctgcatctggagatttccactgggactttctggaggcaggtgaggatggtgaactgggtgaagaagggagtgacttgccctctgatttctgggcttctagaaattgttggagttggttctgcagcgtgacacgttctactgtttgttcctttagctgcttggttaacttcaccacttgagaggccagcgacatgcaggtctccaccaccaccaggtacctggagcacagggtgtgcccctgccgctcggcgctctgggagggcttttccccagcgtggttctgcatggtgacatttgctccatattcaaccaaggtctgtatgcatccaaggtagccatgctgtgaggctacgtgaacggcactgttgccatcctggtctacttcatccaacgagatgccctgttcttgcataaactgaagaagccacagaagaatcttttcctggccatagcaacctgcgtaatgaataaggcttggaaaatccttagaacaactcagttctgcaatggcttctgtttcgctcaccatccagcgtacgcactccaactgaccattcttaatggccaggcctgctggagtcaacttctcagtgttgcgctcattgaggcagtcttctcccatcaaagaagtgaggtgctgtagacactctgcgtgtccctgtgacgccgcaatatgtaatagattgtttccattttcgtcgtgaattttgtctagattgtctgcagctaggtgtggcaggagagagatctgtccttctttaacaatgttcaagatgcttttcacttttttcagatactcactcctttcttctgggccttgggagctggtccggtttaggccactgacctgctcttctggtttggattctgctgctgaggattgtaggtggaaggccctgagctggcagtctggtgttgtcttctcaacttttcgaccatgaggatcactaaatgtcttgtttaggaagtctttactctggttttcaggctcatatgcagagccacatttaaccagaggaggtgagatctcggtttcttcagtggacagcttgtgctggtcgtggatgacagctgatgcttttctcaagtgagggcttttcacgggagaaagaacacaaaatggtgccatgttggatgatgagctctcagaacttcctgtagagcaggctttgccagaaaggccattgatggttgtgcataagcccaaaattcttttttctgaagtcaccttggtaaaagaggcaagctgctgactggatttaatataaggcacatccagaatctcatccatgtcgaggtcgtagtgctccagttcacccagcgatgtgctgggctcagagctcttacctggtgggccgcccactccatctccagggccaagctcctgaggctgggggcccaggtcagactcaccccctttctggtactcaaccactttctggttcttttggtcatcactttcattgttctccagagtctctggctgatgtttcagtggcgaaacccgcttcactgggcggaacttactgtacacatcagcgattcctgtgggcttttgcgtgtttgtaataagagttgagatgccacaattccagctagagctagaaactgatctgtcttcgttttgcgtatcacatcttcggcacagttctgggatcgtcttgagtgatgtgactgaatactcattctcaggacaatggcaagctcccagggcagcaactactgtcagtttggccctatgggaaccaaagcccattgcatcttccctgtctgtgtcctccaatccaagcttttgtagcctgttcccttgactcctattgtcagatatgtcatcactaaagtcaatttcatccaaatcaaggtattcaggggcttccattattcttccttgcacattttgagtacggtcaaatacttataaattcctcaaacccatcacttgatttaattttcctgtttcctctcctttttttcccatatgtatataccatttttaaagtcttaattacaatagatacagagtccatccaagaaaggattaggatgttacttccatgtttaaatgagattatccatttagcaaatgttaaaaattcttctgaaatcacagtaaggcttacaatgaaaagaaaaccaacttgtatttgtaaaaaatatttaaaatcagaaattttattatttgtagaaatctgaaaataggttatcaaacaaattgcttggtataaaaatgtcacttttcttcaatttacaaagattttcagaggaaaatatatgtactctgcttggaaattactcaaaacaacattctctcctactgtgatggattctgatacaatccagactctttggatactagcgtgttcactaggagactttcttccaatccaatttcttttcatgaaatctgtactccgtgatgaactattgatttacagactctgttcccacggccttggtgaacaacacacagatgatgctgggtgccaggatatggtataaacatcagcaggaacatggaaatatggggagatgaagcagagaaacatgcatcgaagctggggaccaaatggatctttaaataaatgaaactataaaatgtggatgaacatgtcttaattaagtaaattaacaaataaccattgcacccctgtttgaggtgctccaacaatatagacagcaatatccagttgagtgtagccattccaatagaatataaccagcggataataactcatggcatcacaacaggaatctttcaatttgcacttgcaggatggtagtgaggttctttattctataggcaagaacacaagacttacaacaggtgcagctcattataggaagtcttgggccactgcccatatttatttctgtgggttggatggccccaccttagactaaggctcctaggcatctggaatttgcctctacttcccagcaggcctccacatgctatctcctttaagatgtctcattctgttcatgatccaatttattttgtctggtttcaatgcttgtctctttcagggtgccactttaagaatatttacattctcaattataatgtgcagaaatccccgtggttttccaatcctgactacattccccaacattaactgcttctttacaggtaagagtgagtctgcagttgtcccagtggccaatacaatgcctcctcttctctcgtctgcccttccaccaagcctctggcactctcaggcactcttttctaaggaatcagtgacaagataggaagcaataaggtcaggttagagtagctgctgcaaatgatcaaacatgataaggacaatgaggtgaactgtggttgcttttctcatcctgctcttctgacacctcccactctgcacaccaatccactatggaaaccaataagccttctttcagacccatggcaaacatgctgtaacagaaagcacagctacagagggcatgcattggaggcctgtgagctgaatctggcccacagatgtgatttgtttgaccccaacagtgttaaagaaaaaaaaaaaattgaatcagttgccaacttgcagaccttgggtgatttcacataaaattctggatttctggctttgttttaaatacctgaagctctggcaacaggggtctgcagtccccatggcaacaactagctggagctaagccgcagctgctcctacctgtccatggggcctgtgctccccattttcccagagcctctccaaggctgctctactcaccaacatgccttggggacatttgagtgttcgacccttcaaaggaattcagtattaaacataagtacaaccattacccccaattttgtattggtgcctcctgccaaaaatgttgacttcatttgtattctaagatttaatttgtattctaagatcattttaaattatcataccacaacagcaacaaaatacaatttcctacaaataaactattggcacatcacaatttgtgctttcacagaatgtccactttatctcttagtactaggaaaagaaaacctttgcaaacttaataaaatgttacgaagtggggattatgtttccttcactttacaactgggggaaggaagggttcttcttgctttgtgtgattggtgtggatttacatggtgacacttcactgctgtgactccaggggaagggaggaagccgtgccaagtgcaaacccagaaaaagtcctgaagccatcctctgtctggcccaaaccagcagctgggaggcaagagagccaacctactgaggccaacaagagtgggtttatacctaagcaaaatacattttttacgctttccagaaagggcaggccagcttaaaatcctttatgtagggtcgggcatggtgactcacacctgtaatcccagcactttg

SEQ ID NO: 10360 - RNA, 2573 nt, Homo sapiens
  source 1..2573: mol_type = other RNA
ccagggaggctggtttggaggaatactccctgagcctggatactgggattctaagtctggttcgctgctctctgaggtgggagatgggctgtggccatccagggatttggaggccttgatgctgaaaggaaacctgcgtccccctgatgccaaggtgtgtttcttaatcatcaggtgcaggctttctgcgctgtccatactctctacgctttctacaatgggctgcggccttggtcggtcagccttcctcactggggtagtcttggggtcctcagagttgttggagtctgtgtcagactcactcagtgacctctgcatcagctgtctcagcctggctaacttcagttccctcttctccagtgggatctttttagaatttctagaggaagcctgagcatcctggaattccaaggacagtttttcctgggtgcagacattttctgagatttcctttcccaataactggcgtaagattttatcagaatcttcatcttttgctttgggtctagcccggctggaggctgacaggcttccaagaacctgaatcccctcttggactcctggcttgcttttggctacagaatcatcatctgcatctggagatttccactgggactttctggaggcaggtgaggatggtgaactgggtgaagaagggagtgacttgccctctgatttctgggcttctagaaattgttggagttggttctgcagcgtgacacgttctactgtttgttcctttagctgcttggttaacttcaccacttgagaggccagcgacatgcaggtctccaccaccaccaggtacctggagcacagggtgtgcccctgccgctcggcgctctgggagggcttttccccagcgtggttctgcatggtgacatttgctccatattcaaccaaggtctgtatgcatccaaggtagccatgctgtgaggctacgtgaacggcactgttgccatcctggtctacttcatccaacgagatgccctgttcttgcataaactgaagaagccacagaagaatcttttcctggccatagcaacctgcgtaatgaataaggcttggaaaatccttagaacaactcagttctgcaatggcttctgtttcgctcaccatccagcgtacgcactccaactgaccattcttaatggccaggcctgctggagtcaacttctcagtgttgcgctcattgaggcagtcttctcccatcaaagaagtgaggtgctgtagacactctgcgtgtccctgtgacgccgcaatatgtaatagattgtttccattttcgtcgtgaattttgtctagattgtctgcagctaggtgtggcaggagagagatctgtccttctttaacaatgttcaagatgcttttcacttttttcagatactcactcctttcttctgggccttgggagctggtccggtttaggccactgacctgctcttctggtttggattctgctgctgaggattgtaggtggaaggccctgagctggcagtctggtgttgtcttctcaacttttcgaccatgaggatcactaaatgtcttgtttaggaagtctttactctggttttcaggctcatatgcagagccacatttaaccagaggaggtgagatctcggtttcttcagtggacagcttgtgctggtcgtggatgacagctgatgcttttctcaagtgagggcttttcacgggagaaagaacacaaaatggtgccatgttggatgatgagctctcagaacttcctgtagagcaggctttgccagaaaggccattgatggttgtgcataagcccaaaattcttttttctgaagtcaccttggtaaaagaggcaagctgctgactggatttaatataaggcacatccagaatctcatccatgtcgaggtcgtagtgctccagttcacccagcgatgtgctgggctcagagctcttacctggtgggccgcccactccatctccagggccaagctcctgaggctgggggcccaggtcagactcaccccctttctggtactcaaccactttctggttcttttggtcatcactttcattgttctccagagtctctggctgatgtttcagtggcgaaacccgcttcactgggcggaacttactgtacacatcagcgattcctgtgggcttttgcgtgtttgtaataagagttgagatgccacaattccagctagagctagaaactgatctgtcttcgttttgcgtatcacatcttcggcacagttctgggatcgtcttgagtgatgtgactgaatactcattctcaggacaatggcaagctcccagggcagcaactactgtcagtttggccctatgggaaccaaagcccattgcatcttccctgtctgtgtcctccaatccaagcttttgtagcctgttcccttgactcctattgtcagatatgtcatcactaaagtcaatttcatccaaatcaaggtattcaggggcttccattattcttccttgcacattttgagtacggtcaaatacttataaattcctgctctttctttacctttcgctctttttacctcgactgccgttgcttttccccagct

SEQ ID NO: 10361 - RNA, 2597 nt, Homo sapiens
  source 1..2597: mol_type = other RNA
ccagggaggctggtttggaggaatactccctgagcctggatactgggattctaagtctggttcgctgctctctgaggtgggagatgggctgtggccatccagggatttggaggccttgatgctgaaaggaaacctgcgtccccctgatgccaaggtgtgtttcttaatcatcaggtgcaggctttctgcgctgtccatactctctacgctttctacaatgggctgcggccttggtcggtcagccttcctcactggggtagtcttggggtcctcagagttgttggagtctgtgtcagactcactcagtgacctctgcatcagctgtctcagcctggctaacttcagttccctcttctccagtgggatctttttagaatttctagaggaagcctgagcatcctggaattccaaggacagtttttcctgggtgcagacattttctgagatttcctttcccaataactggcgtaagattttatcagaatcttcatcttttgctttgggtctagcccggctggaggctgacaggcttccaagaacctgaatcccctcttggactcctggcttgcttttggctacagaatcatcatctgcatctggagatttccactgggactttctggaggcaggtgaggatggtgaactgggtgaagaagggagtgacttgccctctgatttctgggcttctagaaattgttggagttggttctgcagcgtgacacgttctactgtttgttcctttagctgcttggttaacttcaccacttgagaggccagcgacatgcaggtctccaccaccaccaggtacctggagcacagggtgtgcccctgccgctcggcgctctgggagggcttttccccagcgtggttctgcatggtgacatttgctccatattcaaccaaggtctgtatgcatccaaggtagccatgctgtgaggctacgtgaacggcactgttgccatcctggtctacttcatccaacgagatgccctgttcttgcataaactgaagaagccacagaagaatcttttcctggccatagcaacctgcgtaatgaataaggcttggaaaatccttagaacaactcagttctgcaatggcttctgtttcgctcaccatccagcgtacgcactccaactgaccattcttaatggccaggcctgctggagtcaacttctcagtgttgcgctcattgaggcagtcttctcccatcaaagaagtgaggtgctgtagacactctgcgtgtccctgtgacgccgcaatatgtaatagattgtttccattttcgtcgtgaattttgtctagattgtctgcagctaggtgtggcaggagagagatctgtccttctttaacaatgttcaagatgcttttcacttttttcagatactcactcctttcttctgggccttgggagctggtccggtttaggccactgacctgctcttctggtttggattctgctgctgaggattgtaggtggaaggccctgagctggcagtctggtgttgtcttctcaacttttcgaccatgaggatcactaaatgtcttgtttaggaagtctttactctggttttcaggctcatatgcagagccacatttaaccagaggaggtgagatctcggtttcttcagtggacagcttgtgctggtcgtggatgacagctgatgcttttctcaagtgagggcttttcacgggagaaagaacacaaaatggtgccatgttggatgatgagctctcagaacttcctgtagagcaggctttgccagaaaggccattgatggttgtgcataagcccaaaattcttttttctgaagtcaccttggtaaaagaggcaagctgctgactggatttaatataaggcacatccagaatctcatccatgtcgaggtcgtagtgctccagttcacccagcgatgtgctgggctcagagctcttacctggtgggccgcccactccatctccagggccaagctcctgaggctgggggcccaggtcagactcaccccctttctggtactcaaccactttctggttcttttggtcatcactttcattgttctccagagtctctggctgatgtttcagtggcgaaacccgcttcactgggcggaacttactgtacacatcagcgattcctgtgggcttttgcgtgtttgtaataagagttgagatgccacaattccagctagagctagaaactgatctgtcttcgttttgcgtatcacatcttcggcacagttctgggatcgtcttgagtgatgtgactgaatactcattctcaggacaatggcaagctcccagggcagcaactactgtcagtttggccctatgggaaccaaagcccattgcatcttccctgtctgtgtcctccaatccaagcttttgtagcctgttcccttgactcctattgtcagatatgtcatcactaaagtcaatttcatccaaatcaaggtattcaggggcttccattattcttccttgcacattttgagtacggtcaaatacttataaattcctttaaatctgatctctcgaggagccaagatggccgaataggaacagctccggtctacagctcccagcgtgagcgacacaga

SEQ ID NO: 10362 - RNA, 2647 nt, Homo sapiens
  source 1..2647: mol_type = other RNA
ccagggaggctggtttggaggaatactccctgagcctggatactgggattctaagtctggttcgctgctctctgaggtgggagatgggctgtggccatccagggatttggaggccttgatgctgaaaggaaacctgcgtccccctgatgccaaggtgtgtttcttaatcatcaggtgcaggctttctgcgctgtccatactctctacgctttctacaatgggctgcggccttggtcggtcagccttcctcactggggtagtcttggggtcctcagagttgttggagtctgtgtcagactcactcagtgacctctgcatcagctgtctcagcctggctaacttcagttccctcttctccagtgggatctttttagaatttctagaggaagcctgagcatcctggaattccaaggacagtttttcctgggtgcagacattttctgagatttcctttcccaataactggcgtaagattttatcagaatcttcatcttttgctttgggtctagcccggctggaggctgacaggcttccaagaacctgaatcccctcttggactcctggcttgcttttggctacagaatcatcatctgcatctggagatttccactgggactttctggaggcaggtgaggatggtgaactgggtgaagaagggagtgacttgccctctgatttctgggcttctagaaattgttggagttggttctgcagcgtgacacgttctactgtttgttcctttagctgcttggttaacttcaccacttgagaggccagcgacatgcaggtctccaccaccaccaggtacctggagcacagggtgtgcccctgccgctcggcgctctgggagggcttttccccagcgtggttctgcatggtgacatttgctccatattcaaccaaggtctgtatgcatccaaggtagccatgctgtgaggctacgtgaacggcactgttgccatcctggtctacttcatccaacgagatgccctgttcttgcataaactgaagaagccacagaagaatcttttcctggccatagcaacctgcgtaatgaataaggcttggaaaatccttagaacaactcagttctgcaatggcttctgtttcgctcaccatccagcgtacgcactccaactgaccattcttaatggccaggcctgctggagtcaacttctcagtgttgcgctcattgaggcagtcttctcccatcaaagaagtgaggtgctgtagacactctgcgtgtccctgtgacgccgcaatatgtaatagattgtttccattttcgtcgtgaattttgtctagattgtctgcagctaggtgtggcaggagagagatctgtccttctttaacaatgttcaagatgcttttcacttttttcagatactcactcctttcttctgggccttgggagctggtccggtttaggccactgacctgctcttctggtttggattctgctgctgaggattgtaggtggaaggccctgagctggcagtctggtgttgtcttctcaacttttcgaccatgaggatcactaaatgtcttgtttaggaagtctttactctggttttcaggctcatatgcagagccacatttaaccagaggaggtgagatctcggtttcttcagtggacagcttgtgctggtcgtggatgacagctgatgcttttctcaagtgagggcttttcacgggagaaagaacacaaaatggtgccatgttggatgatgagctctcagaacttcctgtagagcaggctttgccagaaaggccattgatggttgtgcataagcccaaaattcttttttctgaagtcaccttggtaaaagaggcaagctgctgactggatttaatataaggcacatccagaatctcatccatgtcgaggtcgtagtgctccagttcacccagcgatgtgctgggctcagagctcttacctggtgggccgcccactccatctccagggccaagctcctgaggctgggggcccaggtcagactcaccccctttctggtactcaaccactttctggttcttttggtcatcactttcattgttctccagagtctctggctgatgtttcagtggcgaaacccgcttcactgggcggaacttactgtacacatcagcgattcctgtgggcttttgcgtgtttgtaataagagttgagatgccacaattccagctagagctagaaactgatctgtcttcgttttgcgtatcacatcttcggcacagttctgggatcgtcttgagtgatgtgactgaatactcattctcaggacaatggcaagctcccagggcagcaactactgtcagtttggccctatgggaaccaaagcccattgcatcttccctgtctgtgtcctccaatccaagcttttgtagcctgttcccttgactcctattgtcagatatgtcatcactaaagtcaatttcatccaaatcaaggtattcaggggcttccattattcttccttgcacattttgagtacggtcaaatacttataaattcctttcgctctttttacctcgactgccgttgcttttccccagctggggctctcctctcctccccgcctactttttgtccgcgcttcccacttttctcctcctgccccccacccccttccttgcttcttggcct

SEQ ID NO: 10363 - RNA, 1502 nt, Homo sapiens
  source 1..1502: mol_type = other RNA
ccagggaggctggtttggaggaatactccctgagcctggatactgggattctaagtctggttcgctgctctctgaggtgggagatgggctgtggccatccagggatttggaggccttgatgctgaaaggaaacctgcgtccccctgatgccaaggtgtgtttcttaatcatcaggtgcaggctttctgcgctgtccatactctctacgctttctacaatgggctgcggccttggtcggtcagccttcctcactggggtagtcttggggtcctcagagttgttggagtctgtgtcagactcactcagtgacctctgcatcagctgtctcagcctggctaacttcagttccctcttctccagtgggatctttttagaatttctagaggaagcctgagcatcctggaattccaaggacagtttttcctgggtgcagacattttctgagatttcctttcccaataactggcgtaagattttatcagaatcttcatcttttgctttgggtctagcccggctggaggctgacaggcttccaagaacctgaatcccctcttggactcctggcttgcttttggctacagaatcatcatctgcatctggagatttccactgggactttctggaggcaggtgaggatggtgaactgggtgaagaagggagtgacttgccctctgatttctgggcttctagaaattgttggagttggttctgcagcgtgacacgttctactgtttgttcctttagctgcttggttaacttcaccacttgagaggccagcgacatgcaggtctccaccaccaccaggtacctggagcacagggtgtgcccctgccgctcggcgctctgggagggcttttccccagcgtggttctgcatggtgacatttgctccatattcaaccaaggtctgtatgcatccaaggtagccatgctgtgaggctacgtgaacggcactgttgccatcctggtctacttcatccaacgagatgccctgttcttgcataaactgaagaagccacagaagaatcttttcctggccatagcaacctgcgtaatgaataaggcttggaaaatccttagaacaactcagttctgcaatggcttctgtttcgctcaccatccagcgtacgcactccaactgaccattcttaatggccaggcctgctggagtcaacttctcagtgttgcgctcattgaggcagtcttctcccatcaaagaagtgaggtgctgtagacactctgcgtgtccctgtgacgccgcaatatgtaatagattgtttccattttcgtcgtgaattttgtctagattgtctgcagctaggtgtggctgatctgtcttcgttttgcgtatcacatcttcggcacagttctgggatcgtcttgagtgatgtgactgaataagatatgtcatcactaaagtcaatttcatccaaatcaaggtattcaggggcttccattattcttccttgcacattttgagtacggtcaaatacttataaattc

SEQ ID NO: 10364 - RNA, 2740 nt, Homo sapiens
  source 1..2740: mol_type = other RNA
ccagggaggctggtttggaggaatactccctgagcctggatactgggattctaagtctggttcgctgctctctgaggtgggagatgggctgtggccatccagggatttggaggccttgatgctgaaaggaaacctgcgtccccctgatgccaaggtgtgtttcttaatcatcaggtgcaggctttctgcgctgtccatactctctacgctttctacaatgggctgcggccttggtcggtcagccttcctcactggggtagtcttggggtcctcagagttgttggagtctgtgtcagactcactcagtgacctctgcatcagctgtctcagcctggctaacttcagttccctcttctccagtgggatctttttagaatttctagaggaagcctgagcatcctggaattccaaggacagtttttcctgggtgcagacattttctgagatttcctttcccaataactggcgtaagattttatcagaatcttcatcttttgctttgggtctagcccggctggaggctgacaggcttccaagaacctgaatcccctcttggactcctggcttgcttttggctacagaatcatcatctgcatctggagatttccactgggactttctggaggcaggtgaggatggtgaactgggtgaagaagggagtgacttgccctctgatttctgggcttctagaaattgttggagttggttctgcagcgtgacacgttctactgtttgttcctttagctgcttggttaacttcaccacttgagaggccagcgacatgcaggtctccaccaccaccaggtacctggagcacagggtgtgcccctgccgctcggcgctctgggagggcttttccccagcgtggttctgcatggtgacatttgctccatattcaaccaaggtctgttctcatttgcttgggctctagtaactggatttggtctctggtaattggttttgaaataacacctgtttatttgttgctgcgccaacctgatcaggaataaaaagaactccttcttgtccttgacactgcagcccagaagagatagggggataggagctaaagtggtgtgtaaaaaggcatgtctcactcccattccaagtcccttgaatcttgagtctagtctgtatgcatccaaggtagccatgctgtgaggctacgtgaacggcactgttgccatcctggtctacttcatccaacgagatgccctgttcttgcataaactgaagaagccacagaagaatcttttcctggccatagcaacctgcgtaatgaataaggcttggaaaatccttagaacaactcagttctgcaatggcttctgtttcgctcaccatccagcgtacgcactccaactgaccattcttaatggccaggcctgctggagtcaacttctcagtgttgcgctcattgaggcagtcttctcccatcaaagaagtgaggtgctgtagacactctgcgtgtccctgtgacgccgcaatatgtaatagattgtttccattttcgtcgtgaattttgtctagattgtctgcagctaggtgtggcaggagagagatctgtccttctttaacaatgttcaagatgcttttcacttttttcagatactcactcctttcttctgggccttgggagctggtccggtttaggccactgacctgctcttctggtttggattctgctgctgaggattgtaggtggaaggccctgagctggcagtctggtgttgtcttctcaacttttcgaccatgaggatcactaaatgtcttgtttaggaagtctttactctggttttcaggctcatatgcagagccacatttaaccagaggaggtgagatctcggtttcttcagtggacagcttgtgctggtcgtggatgacagctgatgcttttctcaagtgagggcttttcacgggagaaagaacacaaaatggtgccatgttggatgatgagctctcagaacttcctgtagagcaggctttgccagaaaggccattgatggttgtgcataagcccaaaattcttttttctgaagtcaccttggtaaaagaggcaagctgctgactggatttaatataaggcacatccagaatctcatccatgtcgaggtcgtagtgctccagttcacccagcgatgtgctgggctcagagctcttacctggtgggccgcccactccatctccagggccaagctcctgaggctgggggcccaggtcagactcaccccctttctggtactcaaccactttctggttcttttggtcatcactttcattgttctccagagtctctggctgatgtttcagtggcgaaacccgcttcactgggcggaacttactgtacacatcagcgattcctgtgggcttttgcgtgtttgtaataagagttgagatgccacaattccagctagagctagaaactgatctgtcttcgttttgcgtatcacatcttcggcacagttctgggatcgtcttgagtgatgtgactgaatactcattctcaggacaatggcaagctcccagggcagcaactactgtcagtttggccctatgggaaccaaagcccattgcatcttccctgtctgtgtcctccaatccaagcttttgtagcctgttcccttgactcctattgtcagatatgtcatcactaaagtcaatttcatccaaatcaaggtattcaggggcttccattattcttccttgcacattttgagtacggtcaaatacttataaattc

SEQ ID NO: 10365 - RNA, 2882 nt, Homo sapiens
  source 1..2882: mol_type = other RNA
ccagggaggctggtttggaggaatactccctgagcctggatactgggattctaagtctggttcgctgctctctgaggtgggagatgggctgtggccatccagggatttggaggccttgatgctgaaaggaaacctgcgtccccctgatgccaaggtgtgtttcttaatcatcaggtgcaggctttctgcgctgtccatactctctacgctttctacaatgggctgcggccttggtcggtcagccttcctcactggggtagtcttggggtcctcagagttgttggagtctgtgtcagactcactcagtgacctctgcatcagctgtctcagcctggctaacttcagttccctcttctccagtgggatctttttagaatttctagaggaagcctgagcatcctggaattccaaggacagtttttcctgggtgcagacattttctgagatttcctttcccaataactggcgtaagattttatcagaatcttcatcttttgctttgggtctagcccggctggaggctgacaggcttccaagaacctgaatcccctcttggactcctggcttgcttttggctacagaatcatcatctgcatctggagatttccactgggactttctggaggcaggtgaggatggtgaactgggtgaagaagggagtgacttgccctctgatttctgggcttctagaaattgttggagttggttctgcagcgtgacacgttctactgtttgttcctttagctgcttggttaacttcaccacttgagaggccagcgacatgcaggtctccaccaccaccaggtacctggagcacagggtgtgcccctgccgctcggcgctctgggagggcttttccccagcgtggttctgcatggtgacatttgctccatattcaaccaaggtctgttctcatttgcttgggctctagtaactggatttggtctctggtaattggttttgaaataacacctgtttatttgttgctgcgccaacctgatcaggaataaaaagaactccttcttgtccttgacactgcagcccagaagagatagggggataggagctaaagtggtgtgtaaaaaggcatgtctcactcccattccaagtcccttgaatcttgagtctagtctgtatgcatccaaggtagccatgctgtgaggctacgtgaacggcactgttgccatcctggtctacttcatccaacgagatgccctgttcttgcataaactgaagaagccacagaagaatcttttcctggccatagcaacctgcgtaatgaataaggcttggaaaatccttagaacaactcagttctgcaatggcttctgtttcgctcaccatccagcgtacgcactccaactgaccattcttaatggccaggcctgctggagtcaacttctcagtgttgcgctcattgaggcagtcttctcccatcaaagaagtgaggtgctgtagacactctgcgtgtccctgtgacgccgcaatatgtaatagattgtttccattttcgtcgtgaattttgtctagattgtctgcagctaggtgtggcaggagagagatctgtccttctttaacaatgttcaagatgcttttcacttttttcagatactcactcctttcttctgggccttgggagctggtccggtttaggccactgacctgctcttctggtttggattctgctgctgaggattgtaggtggaaggccctgagctggcagtctggtgttgtcttctcaacttttcgaccatgaggatcactaaatgtcttgtttaggaagtctttactctggttttcaggctcatatgcagagccacatttaaccagaggaggtgagatctcggtttcttcagtggacagcttgtgctggtcgtggatgacagctgatgcttttctcaagtgagggcttttcacgggagaaagaacacaaaatggtgccatgttggatgatgagctctcagaacttcctgtagagcaggctttgccagaaaggccattgatggttgtgcataagcccaaaattcttttttctgaagtcaccttggtaaaagaggcaagctgctgactggatttaatataaggcacatccagaatctcatccatgtcgaggtcgtagtgctccagttcacccagcgatgtgctgggctcagagctcttacctggtgggccgcccactccatctccagggccaagctcctgaggctgggggcccaggtcagactcaccccctttctggtactcaaccactttctggttcttttggtcatcactttcattgttctccagagtctctggctgatgtttcagtggcgaaacccgcttcactgggcggaacttactgtacacatcagcgattcctgtgggcttttgcgtgtttgtaataagagttgagatgccacaattccagctagagctagaaactgatctgtcttcgttttgcgtatcacatcttcggcacagttctgggatcgtcttgagtgatgtgactgaatactcattctcaggacaatggcaagctcccagggcagcaactactgtcagtttggccctatgggaaccaaagcccattgcatcttccctgtctgtgtcctccaatccaagcttttgtagcctgttcccttgactcctattgtcagatatgtcatcactaaagtcaatttcatccaaatcaaggtattcaggggcttccattattcttccttgcacattttgagtacggtcaaatacttataaattcccggggcgcccggcgcgccggcggctcaggagcgcgaagggactgactgaccgaccgacggaccgcagcggcaggagcagaacagcctcagccgaagtaggcgggcggtggaggcgctgccgcggccccgctacgtcacaat

SEQ ID NO: 10366 - RNA, 151 nt, Homo sapiens
  source 1..151: mol_type = other RNA
ccagggaggctggtttggaggacaggattgacttgttctcatcctcccgccaagagcccagctgggaaaacgtcttacccattcttcaggggcgggggtttcaccgcggacgactgcagcgacagaaacggaagagagtggaatcgaaaat

SEQ ID NO: 10367 - RNA, 319 nt, Homo sapiens
  source 1..319: mol_type = other RNA
ccagggaggctggtttggaggacaggattgacttgttctcatcctcccgccaagagcccagctgggaaaacgtcttacccattcttcaggggcgggggtttcacttgttcaggtctgggatcccaggctcctcagccgcacgagggcgagacttctggagtgcgtctttggggagaagggcctctaagggcagagtgggctgggctgggctgagctgagctgggcggtggtggggagaagcaccgcctggggccggcaaccggccggagtcccgcggacgactgcagcgacagaaacggaagagagtggaatcgaaaat

SEQ ID NO: 10368 - RNA, 341 nt, Homo sapiens
  source 1..341: mol_type = other RNA
ccagggaggctggtttggaggacaggattgacttgttctcatcctcccgccaagagcccagctgggaaaacgtcttacccattcttcaggggcgggggtttcacttgttcaggtctgggatcccaggctcctcagccgcacgagggcgagacttctggagtgcgtctttggggagaagggcctctaagggcagagtgggctgggctgggctgagctgagctgggcggtggtggggagaagcaccgcctggggccggcaaccggccggagtcctaggggaacgaatgtgccgcaccgcggacgactgcagcgacagaaacggaagagagtggaatcgaaaat

SEQ ID NO: 10369 - RNA, 3919 nt, Homo sapiens
  source 1..3919: mol_type = other RNA
ccagtattaactgtgctgctgactggctcctcctcctgtttcctgacttcctcctaatgctaggagaaaaagtttctgtctctgtgttcctggtggaaatggagtgaatgcggctcaccacggcctgtgggtggcttactgactgctacagaccctccccagctaaacaggcatctctatctgcccaggattcaaactgcaatcacaggccactctgctcagcgcccaggaaaatattcccatgaacagcagccaggaacaatccaaacagggtctctttggcattccacatctatgaatgaacttactatgacgtacaatgtattgtgcagcacaaatcgtatgtggcccggtgcgggggtgggggaaggtcaaagacaatgcttcagtaggatagggaaacagaagagtgaaaggaaaaaatgaagagagaagatgcatgtgttttaattttaatgagctcaggaggctaaggagaaactcgctgtaacctacattgccggcagctctcatcggaggatgtgtttccagagagctggtctatttcagactgacaggccactgcctcgcatcacgcagttttcacgatcctattaattgggtgaggctgttagacgctgtggaggaaaggtggtcaactgtatgcattgctttgctgttggcttatttggggatggggctgtatgatttccttggtgtggattttcctataatggacaagggctgaaagatgccgaaacacccacaactcacccgtggaaggctaagcaatagtcaagggccgttacagaggcttgtggtctcagacctggaagcctctcagagcagggccccagcctggccacgccctaatcatggggtcttaagcaattcagaccatgtctctgtgcttccgatacctcctccgaactggagatggtcatcccacctcccagcacccctgtccctgttagggttgtggaggtaataagaggcataaactatataggttagagtttaatagtcacatggtaattgctggatcaataaacactattgtttataatcacttacctagcatgcacaagccattattatttaatactttacattgcaagtacttgattctggcttctctctttcttactcccaaatcagtttagtcacccagttttatcctcctggcctgtcccctttccttcacccccactaccaacagcagatccaggccaccatcaccccacctggctcacagcaggagactcttctgcagttctggtcctgttattccctcggggctccccaaagatctctagataaaatgcaaaacccgtaaccaagttggcaagcccttccccatggggaccttgtttgcccctctagtctcatcttattctaaagccccctactctcctgccccgaccctaccagcccaaatccacgctccagcccctgcgtttcttacaggtctctgaacgcttcactgtctcatgctggtgggactttgtctatgctgttccctagcagaggccaccaggagccagcactcctccatgtcaccttgctaaactcaactaagattctatttctgcagaaagatttcgtcctgcgtctccccatctcagggtctgtgttgcgttagatatcccttctgagttacccatagtatgctttccgcctggctcttggcttgacctattgtaattagttggtcttcctcaaaatgaaagaagcagatcataggcacacatggggaaaaggcacccaccaagagtcctcaaggcgacggcccagaggaaaataaccaaagcatcaagaagcacagctgagcttctcaacaatctggaggcacttatgctttcctcctggctcttgccttaacctattgtaatgagttgcctgttttcttgcctggggccagatcttgaacttgagcttgccaggtcaggggccatgtctgcctggctaattgctgaccccagggctttatctggtgctcagtttgtccagtgaatgagtgagtgagacagtgagtgagtgagcagatagtgagtctagcagagaaagtcagggtctcatgataatgtagatgggtggtgtggtggccattcaccctgtattagtgtgggcttcagccacaagaaagaagcatctgtccctgggcttcagcaggggcctcacacctgcaatgggtgcctggggagagggtgcagatgttgcgtggcagctggcctcctggggtggaggtggagaggacccacaatgggagagaagttgctcgagcaccctaggacttaccctcaactgcacacacagccatcgggggtcacgtggcagagcccacatctgccagcaggattgggtagaacccagcgcgttctgtgtctttatttgtgtggcaaggtggggatggaaatggacacagggaaccagacctagagcgcattgtcttgtcccacagctttgttgacatcccccctccaaagcccagatttggtgtttttggggctcttttggaatcaaagtgagctctaaacacctggggcagcagcatgggatcccagagggcaggctgaggggcatggcgtagcagctcctccaagaggccctgccacaggggcattgggaccagctgggaggaggcttcggggtcgctcccttggagtctgcatcttatcatcacaccagacccctaaggaaggcggatcccttgtcagacacacatacaccctcccagctctgctcgggaatgcggggaacccacttacgctggcatccaagacaccccacatgcccgggaccagcagaccaagctcagctttgtcagagtttcacttggcacctttagttttagccacacaatattatagtgcaggagctaagttttgatttcatgaaggacttcagaggtagaagatgcctggaaggggtgtgtgtgtgcttttggcactgtgagatgttctctctcgatttggaagacagcaagaaaaagcacagcaatttgctcccccagggttcttctgtgttttgaaggtacctgaagcttattgatttgctcacggttgccaggccattgaaaaagggtatttctttctttgcataggtacttctgggttcttggcaatcagttacagttcgtttgactcccaatggaagctttaaaagccaatggtagctacaaaagattaggtattctcttgatgcagtgaaatgaacacctatcttttttttttttttatgactcaaattctgggataacttctgctactcacttgattgtgagacctggaacacggtccttaaattgtctatatctcagtttccttgtttgtctaacatattaaaaaatgttaaccattccaacttttcagcactattatgaagaggtagcaagagagtagaattgtaagtgatttggaaattttaaatgcaaaatacaaaggccaatccccacaaaactcagcagctcaggtgatgtcattgctcctgagacatttttatgagattacgcgagaaaggcacaaaacagctcagtgtaaatataagtttctcggttttttatttcttaggcacctggtgtgtctttattgaggtttttaaaatgaggggactgtaaatagatcgatgcctatggtggccagtgttttcttctttgaggcaagtgatgattcatggattatagttttatgattagattttatgattccaaagtaagacttgtagatcagtgtaacactttaccttaagcattttttaatagaagaaaatgtgacggagatgacaaattcctctaggtgggcacatttctcctggggccaaaggtgctcctgcagtggaagaagtgttgctattaataaccaatgaccctgagcctcatggtgaatctcttcatgttctttttcttgatgcagcttataacaggtcttgttgcttcctctgg

SEQ ID NO: 10370 - RNA, 2004 nt, Homo sapiens
  source 1..2004: mol_type = other RNA
ccagtcctgtgcctgccgcctctgttggctttcatcttcctggcgactcaaatgtgaccctccaggacctgagggctctgtgcttccctcggttctggaaggttctgacgacgacaccagggactcgccataggcatcctcttttctctgtgttgcatcctgagaggtctttccaggtccacgttccaggcaccaacgcactccacagcttctgtccttcctgacccttctgaggggaggttgtctgcctgatgccccctcatccagagtctgtggcatgcactttctacacacgaagactctgaccagcaccccaaaatcggggcacccctgtggacagaagcctcccgcgggcctcagcccactcaagccccgtcctcatgggcacagagggctgttccgggcctgtggttgctcagctgtcttgtctctcgggcctccgtcatcccagcggctccgcgggttcttgacgttcaggacctgtgagggaatgtgaggtaggggcacccgcccattgacctgcacgctctcctgcatctccctgcggtgctgcttacggatcctgtatggggggatcccatccacgctgctgtccgtgagggacagggtgtctgcatcgctggacaggctctgctgctcgctgtcgttggcactggtggctggggccagggcatagccggcattgacataataggggttgactggctcccgccaggatccatacctgaactctctgccttcgctgtaccgtctactggaggagaccctcggggcagctgtctccaggagcagcttctgagggagtcttccggggggagcagcgtctctgccatcgtcctcatccatgtcctggtcacacttccattcctcatcttcatttaaggtcggcaggtatccagatatgcccttccctgtccctgacccagagctctggtcactacagactttggggctctccgagcctgtcctcgtatattccaaataaatatcagacttaaggaaggagggataggtgttttcctccatagtggcctggatttcggtctgggcctggtcaaacatggcaggatcgatcagctgcttcatgatgcagccctttatgaagctcttggtggctggcttggtctgccgggacacgatgccattgttatcaagaatgtactttcggtagatggctctcgccagcttcagcctcttctcctcgttcgagtcacagggctccagcttcctgaagccagtgcaggcaaaccagaagtccagcaagtcggcacagccctcctgcttcaggaaagtcctgaacaggcttatcccatcttggtcatccagcagggaatgcagtgactcagcccacttcaagtatggtggggtgggggaggcactgccctcaggctcataccccaggtccagatccgagcgcctcggagtggccgtcgaagtctcacctttaatgccaacacctttcccggagcagaaactgtagctggcgggcctcgggtctgtggacaccagttctccctcctcaccaggcactgggggtcggggagcatcttcggtgaaacttgctccgaggtccaaggggaaaccctgctcttggatattcattttgggactctgcgtcaaggaacaatgagcgctgcaccctaatacatcagtacttacagctccaaagtgaatcaatctgtcccgcgcgcggtggtggcgggaccccgggcccggctcccggagcggcgcggcgcggtccgggcccatgcgctcagcggcagcgcggcgggcgggacccggcgggggcgcggcccggggcggcccccatctcggcggctgcggctcggcggcccggaggcggacgcggggcaggccgcgggggcgccgcaggggcccagccgccagctcccacccgcccgctccgcgtggacgcggctccgggccgactccggccggctctggcggcggcagcggccacgatcgcctcccgagccagagcccgagccagagcgccgaagccca

SEQ ID NO: 10371 - RNA, 843 nt, Homo sapiens
  source 1..843: mol_type = other RNA
ccagtcctgtgcctgccgcctgcctgctcctgccctggctcctcctaccctcaccagcctggggctgcagacacagagcccatgtgttaccactcctggccccatcacagcctgcttttcctgcccagtagttgtctgtggggtgctggtgttgaagacaaagagttggtgcctctttggcgagtttttctgcctggtcgtagaagttggtttccatcaagccaaaagagtagatgcctttcacatagctgcttagggggatgtcaggtgtccagaaggggtaaattcgagcaacagaatctctcatctgttcctgatagcccaggtaaaaataagcatcatgggaaaatttcagggccaacatgtctgtcgggtggtcctggagaatctgttcccatagttcacaggctttcggaaagttcccattggcaaatgtctctactgcagacacgtgcagctgctcccgccttgtcagcggctgggttcttgaaatctccaccattgtcttcacagccaggtccagctctttgtccagcttcacggagcttccagtgccaatcagcacaaggccagtagccatggcgtggcccatcacaaaggttggatctgctgctttgagctttgacaggcagccctcgatgccaccgagactcttgtcattggtccattttacatactgggtcagcgtggcatcgaacagcttgcaggcttcgttgcttgtggtggagagcgggagcctcgcatccttccaggcctggcagtcgcgcagaggcgaggctgcggccatgttgcgccgggtcggagtccaccgcgagctctgggcacccgggccttcctgggagt

SEQ ID NO: 10372 - RNA, 3233 nt, Homo sapiens
  source 1..3233: mol_type = other RNA
ccatgtgtctgggctgggaaacactggctggtgctaccaagacactatgtaactgttgtccattcacaaagtattatctacactacatacagaatacattttcccctacattttaactgatgctcgctttagagcaactccctttgtttggacaagaaaggaatcccatctccctgtgagtggaatccagaatctattaagaaaaatcaaccttttccacacagttttagtttaataaaaggaaggaaaacccaccaagtacatttcatgtcgaaagagaagcaaaaaatttgtactgcaagtagtcgtgtgagttaccttgattcccaggaaaagaaattttaaatgctggtacatttgcaagttgcagcatcactcattgtaccttaaggactggcaaagcctttccaataaggaagcatcctggttctagcttattttaaaacaaagtgacaggacaccaactgaagtcaacgtggctcgatctagaggcggtaggcatttgaaacattttgaggctgcatggggtgccaaattggttgagttctttttctgagactctcaggcaaaatacatcgtgtgctgggtatcatggtggatttgcacagccttagccaaggcctgaggatcccggccgttgctctgtcctgacacatgactgccttccgcactgtcatgatctttatccaccagatgataccttgccctaaatgctacaagccgggcataatatgcaggggctggaatagagactgagcgagtgcacctcacataggtgtgacacagctggtaagtcagtagctggagttcatctgcagtgaagcagttgtcatcccacaagacctggtaatgtgagggacggctggttccctgaattcctgcatgactacagaggtaaaagtcaaactcagatggatgtgtgatggtactatccactgtagtgcctgctggtacattgccacttttccctaccctttctgttttatctgcacagaagagtcgtgtgtgatgtcttttttgcaccacaatataagttattcctggccggtaatcttcttccaagctaatacatgcctttcgaattgctattagttctggccaagctacctgtttcatttgtccctcagatacccctccacggtaatagatgatccgagtgggtttgaagcgtgtggatttgtagaactgaatcagcagctctcgaaccatgttagtcaggtcctggatgacctcttgactgtagaggagctcttgggagatctcctgccgggaagtctgcacccgaacggtggcacagtaccggctggggtggccatccatactgccaaccacagcagcaatggaaggtttcttcccatcccctgctggggggtgtgtgacatccgctcccaggaagatgacaggctgctggaacaccgagggcctttgatgaggcacaagcacattgttaattcctccaagttttgcatttatcttcaggcaaagattggaaagggtttgaggtgaggtcttcactacattttttacctggacacactgtgtggccatacctagaagggtatctccaacacgtttcacctccgcatatactggtgtctttccaggcaggataaccactattagctgtaggcccacataagtcattttcagatgtttaaacataggctccacactgtctgcaccttgtgcatacttgcagaaacatggctgaccctggatgggcattcctgcatccttagagattttacgcagctggtcagtgaaactctttagtaaatcttccctacattgtttctgaggtgcaaaacaagcaactgcccaaactttaatttcaatgccagcataaaactgctttcctcgcatgtcccagacaccctggttgggtgtggctactgttttattccggcctccatattgcagcattggtgctggaagtaccctgcctgtgagctctgtcatttcattgtggacaacaataccaaattctttaaggtatggatcaggtccacccaccatactgttgctcttcaccagtctactgatctcttcctgtctgtcaggagcagatcttgctgtagctttgatcattgtggaagtctgattgtctgtgagcttcttgatacatcgctgtcctgccactatattacagacctcgagtggcaagtatgtatgcttttgttcttgtcccacttggagacagggaagatgggggtatttcagttgcagactatacttttgcttaaaatattgagctactgtacattccatagcttgaccgttttctagctgcaaaggaaaagtttgatgactggctggccgtctagtcacattacaaactcggtattttcgtttcatctgtccacagtgggtcacctcaactttgagacctctgatttctttggtaaatttgacacgctgggagtctgttagaggtttggtctgttcattgatgttctgaatgtctaaaacctcacacatgaactcaatgataggctgagcccggtagaaagcagttgcagatacatcaatgttgagcatcatattccacatggcaggtctcacagactgatgaaaaccaaaccagacctccctgccccctcccagagggtggtagtaaccttccgggggtgagaaaaaggaacggcccactggggtgtacctcatggagggaaggtgtcttgtgataacatcaagtgcttgtactgagtcatctgggacttcattcaagtgcccagccaaagcttctaaaagcaactgaaggctcacaactgacacccactgaacagacactttaaatgtttggtctttaccctcgcctggaagagtcacctccatatcaaccctatcccgtccaattggtagtggatgtgctgtgtacatgtttcttttgccatcatacccaggctgccgatcaccaaatatttgcatcttgaagtgccgcaccattgtatctactacctccctgttgactctacgaggccgtttttcaggcttaatatccacatcatagtgatacacatctattttaggaatctgaacctgaaaatgattggctaacagtcgaattggttttccaacagttccaaggccaggacgacgaggtggctgaaacaggctagccggaggtccgggtcccagcgcctccatggcggcggcgggggccgcctcgccccggtccccggcgcctcccgctccgggccccgccgccgccgccgccgccgccgcgtaacgct

SEQ ID NO: 10373 - RNA, 4073 nt, Homo sapiens
  source 1..4073: mol_type = other RNA
ccatgtgtctgggctgggaaacactggctggtgctaccaagacactatgtaactgttgtccattcacaaagtattatctacactacatacagaatacattttcccctacattttaactgatgctcgctttagagcaactccctttgtttggacaagaaaggaatcccatctccctgtgagtggaatccagaatctattaagaaaaatcaaccttttccacacagttttagtttaataaaaggaaggaaaacccaccaagtacatttcatgtcgaaagagaagcaaaaaatttgtactgcaagtagtcgtgtgagttaccttgattcccaggaaaagaaattttaaatgctggtacatttgcaagttgcagcatcactcattgtaccttaaggactggcaaagcctttccaataaggaagcatcctggttctagcttattttaaaacaaagtgacaggacaccaactgtgaatataaaacaggtaaaaataattctttaaaaaggcatggaaatatatgtcttttctgactggtttcagaaattgccagattatgatatataagaaatagctgataaaatcatactgaaatctcatctagaaaactacattgttggggaaggaagaggagagaccttaaaaaatgtttattgccaaagttaagtttctatgagaaaagtttaaaaatcatttagatttaacaaaccacacagcagcataaaatgggcacttttgaaaacttggaaaaatactaaaagcaatttttttttccaaataggggaaacatgagtacttttatcatggcagtgttatctccgtcactgtgacatgcattacatctgtttatgtcacacattcacaaaagtcgaccaaataagagaactgcctatttgaatctgcagccaaatatagtgcaaattgcctgtcagcatgtacttgcaccagcacaagtctgcagagatcaataagataaagtagtaaaactaataaaactctgtaaaactttcaaaaattaatgctcattaaaggcatttacagtggcaaagtcagaaatcttcattaaaaagtctatggacccacacaattaaatagttacactgaactgaagtagattgtttggtttttctctcccacttatgcatataccccactcaatgactacagaaaaaaggaataatcttctcttctaagactagagggatgcggtgaacaccacagctagcaaaatattccatagaaacccttcttgtaaagtcctttagaaagttcaggctgatcagcctttgcacattgaggtaaaaattcagtccagtgcatcagaaaagataatctattagtatctattactttaaaaaaatggctcaattttgttgacgcatcagacagtgctgcaaagtatagattcagtgcaactattccgagctgctggtagaagaccacctgaagtcaacgtggctcgatctagaggcggtaggcatttgaaacattttgaggctgcatggggtgccaaattggttgagttctttttctgagactctcaggcaaaatacatcgtgtgctgggtatcatggtggatttgcacagccttagccaaggcctgaggatcccggccgttgctctgtcctgacacatgactgccttccgcactgtcatgatctttatccaccagatgataccttgccctaaatgctacaagccgggcataatatgcaggggctggaatagagactgagcgagtgcacctcacataggtgtgacacagctggtaagtcagtagctggagttcatctgcagtgaagcagttgtcatcccacaagacctggtaatgtgagggacggctggttccctgaattcctgcatgactacagaggtaaaagtcaaactcagatggatgtgtgatggtactatccactgtagtgcctgctggtacattgccacttttccctaccctttctgttttatctgcacagaagagtcgtgtgtgatgtcttttttgcaccacaatataagttattcctggccggtaatcttcttccaagctaatacatgcctttcgaattgctattagttctggccaagctacctgtttcatttgtccctcagatacccctccacggtaatagatgatccgagtgggtttgaagcgtgtggatttgtagaactgaatcagcagctctcgaaccatgttagtcaggtcctggatgacctcttgactgtagaggagctcttgggagatctcctgccgggaagtctgcacccgaacggtggcacagtaccggctggggtggccatccatactgccaaccacagcagcaatggaaggtttcttcccatcccctgctggggggtgtgtgacatccgctcccaggaagatgacaggctgctggaacaccgagggcctttgatgaggcacaagcacattgttaattcctccaagttttgcatttatcttcaggcaaagattggaaagggtttgaggtgaggtcttcactacattttttacctggacacactgtgtggccatacctagaagggtatctccaacacgtttcacctccgcatatactggtgtctttccaggcaggataaccactattagctgtaggcccacataagtcattttcagatgtttaaacataggctccacactgtctgcaccttgtgcatacttgcagaaacatggctgaccctggatgggcattcctgcatccttagagattttacgcagctggtcagtgaaactcccggcctccatattgcagcattggtgctggaagtaccctgcctgtgagctctgtcatttcattgtggacaacaataccaaattctttaaggtatggatcaggtccacccaccatactgttgctcttcaccagtctactgatctcttcctgtctgtcaggagcagatcttgctgtagctttgatcattgtggaagtctgattgtctgtgagcttcttgatacatcgctgtcctgccactatattacagacctcgagtggcaagtatgtatgcttttgttcttgtcccacttggagacagggaagatgggggtatttcagttgcagactatacttttgcttaaaatattgagctactgtacattccatagcttgaccgttttctagctgcaaaggaaaagtttgatgactggctggccgtctagtcacattacaaactcggtattttcgtttcatctgtccacagtgggtcacctcaactttgagacctctgatttctttggtaaatttgacacgctgggagtctgttagaggtttggtctgttcattgatgttctgaatgtctaaaacctcacacatgaactcaatgataggctgagcccggtagaaagcagttgcagatacatcaatgttgagcatcatattccacatggcaggtctcacagactgatgaaaaccaaaccagacctccctgccccctcccagagggtggtagtaaccttccgggggtgagaaaaaggaacggcccactggggtgtacctcatggagggaaggtgtcttgtgataacatcaagtgcttgtactgagtcatctgggacttcattcaagtgcccagccaaagcttctaaaagcaactgaaggctcacaactgacacccactgaacagacactttaaatgtttggtctttaccctcgcctggaagagtcacctccatatcaaccctatcccgtccaattggtagtggatgtgctgtgtacatgtttcttttgccatcatacccaggctgccgatcaccaaatatttgcatcttgaagtgccgcaccattgtatctactacctccctgttgactctacgaggccgtttttcaggcttaatatccacatcatagtgatacacatctattttaggaatctgaacctgaaaatgattggctaacagtcgaattggttttccaacagttccaaggccaggacgacgaggtggctgaaacaggctagccggaggtccgggtcccagcgcctccatggcggcggcgggggccgcctcgccccggtccccggcgcctcccgctccgggccccgccgccgccgccgccgccgccgcgtaacgct

SEQ ID NO: 10374 - RNA, 4522 nt, Homo sapiens
  source 1..4522: mol_type = other RNA
ccatgtgtctgggctgggaaacactggctggtgctaccaagacactatgtaactgttgtccattcacaaagtattatctacactacatacagaatacattttcccctacattttaactgatgctcgctttagagcaactccctttgtttggacaagaaaggaatcccatctccctgtgagtggaatccagaatctattaagaaaaatcaaccttttccacacagttttagtttaataaaaggaaggaaaacccaccaagtacatttcatgtcgaaagagaagcaaaaaatttgtactgcaagtagtcgtgtgagttaccttgattcccaggaaaagaaattttaaatgctggtacatttgcaagttgcagcatcactcattgtaccttaaggactggcaaagcctttccaataaggaagcatcctggttctagcttattttaaaacaaagtgacaggacaccaactgtgaatataaaacaggtaaaaataattctttaaaaaggcatggaaatatatgtcttttctgactggtttcagaaattgccagattatgatatataagaaatagctgataaaatcatactgaaatctcatctagaaaactacattgttggggaaggaagaggagagaccttaaaaaatgtttattgccaaagttaagtttctatgagaaaagtttaaaaatcatttagatttaacaaaccacacagcagcataaaatgggcacttttgaaaacttggaaaaatactaaaagcaatttttttttccaaataggggaaacatgagtacttttatcatggcagtgttatctccgtcactgtgacatgcattacatctgtttatgtcacacattcacaaaagtcgaccaaataagagaactgcctatttgaatctgcagccaaatatagtgcaaattgcctgtcagcatgtacttgcaccagcacaagtctgcagagatcaataagataaagtagtaaaactaataaaactctgtaaaactttcaaaaattaatgctcattaaaggcatttacagtggcaaagtcagaaatcttcattaaaaagtctatggacccacacaattaaatagttacactgaactgaagtagattgtttggtttttctctcccacttatgcatataccccactcaatgactacagaaaaaaggaataatcttctcttctaagactagagggatgcggtgaacaccacagctagcaaaatattccatagaaacccttcttgtaaagtcctttagaaagttcaggctgatcagcctttgcacattgaggtaaaaattcagtccagtgcatcagaaaagataatctattagtatctattactttaaaaaaatggctcaattttgttgacgcatcagacagtgctgcaaagtatagattcagtgcaactattccgagctgctggtagaagaccacctgaagtcaacgtggctcgatctagaggcggtaggcatttgaaacattttgaggctgcatggggtgccaaattggttgagttctttttctgagactctcaggcaaaatacatcgtgtgctgggtatcatggtggatttgcacagccttagccaaggcctgaggatcccggccgttgctctgtcctgacacatgactgccttccgcactgtcatgatctttatccaccagatgataccttgccctaaatgctacaagccgggcataatatgcaggggctggaatagagactgagcgagtgcacctcacataggtgtgacacagctggtaagtcagtagctggagttcatctgcagtgaagcagttgtcatcccacaagacctggtaatgtgagggacggctggttccctgaattcctgcatgactacagaggtaaaagtcaaactcagatggatgtgtgatggtactatccactgtagtgcctgctggtacattgccacttttccctaccctttctgttttatctgcacagaagagtcgtgtgtgatgtcttttttgcaccacaatataagttattcctggccggtaatcttcttccaagctaatacatgcctttcgaattgctattagttctggccaagctacctgtttcatttgtccctcagatacccctccacggtaatagatgatccgagtgggtttgaagcgtgtggatttgtagaactgaatcagcagctctcgaaccatgttagtcaggtcctggatgacctcttgactgtagaggagctcttgggagatctcctgccgggaagtctgcacccgaacggtggcacagtaccggctggggtggccatccatactgccaaccacagcagcaatggaaggtttcttcccatcccctgctggggggtgtgtgacatccgctcccaggaagatgacaggctgctggaacaccgagggcctttgatgaggcacaagcacattgttaattcctccaagttttgcatttatcttcaggcaaagattggaaagggtttgaggtgaggtcttcactacattttttacctggacacactgtgtggccatacctagaagggtatctccaacacgtttcacctccgcatatactggtgtctttccaggcaggataaccactattagctgtaggcccacataagtcattttcagatgtttaaacataggctccacactgtctgcaccttgtgcatacttgcagaaacatggctgaccctggatgggcattcctgcatccttagagattttacgcagctggtcagtgaaactctttagtaaatcttccctacattgtttctgaggtgcaaaacaagcaactgcccaaactttaatttcaatgccagcataaaactgctttcctcgcatgtcccagacaccctggttgggtgtggctactgttttattccggcctccatattgcagcattggtgctggaagtaccctgcctgtgagctctgtcatttcattgtggacaacaataccaaattctttaaggtatggatcaggtccacccaccatactgttgctcttcaccagtctactgatctcttcctgtctgtcaggagcagatcttgctgtagctttgatcattgtggaagtctgattgtctgtgagcttcttgatacatcgctgtcctgccactatattacagacctcgagtggcaagtatgtatgcttttgttcttgtcccacttggagacagggaagatgggggtatttcagttgcagactatacttttgcttaaaatattgagctactgtacattccatagcttgaccgttttctagctgcaaaggaaaagtttgatgactggctggccgtctagtcacattacaaactcggtattttcgtttcatctgtccacagtgggtcacctcaactttgagacctctgatttctttggtaaatttgacacgctgggagtctgttagaggtttggtctgttcattgatgttctgaatgtctaaaacctcacacatgaactcaatgataggctgagcccggtagaaagcagttgcagatacatcaatgttgagcatcatattccacatggcaggtctcacagactgatgaaaaccaaaccagacctccctgccccctcccagagggtggtagtaaccttccgggggtgagaaaaaggaacggcccactggggtgtacctcatggagggaaggtgtcttgtgataacatcaagtgcttgtactgagtcatctgggacttcattcaagtgcccagccaaagcttctaaaagcaactgaaggctcacaactgacacccactgaacagacactttaaatgtttggtctttaccctcgcctggaagagtcacctccatatcaaccctatcccgtccaattggtagtggatgtgctgtgtacatgtttcttttgccatcatacccaggctgccgatcaccaaatatttgcatcttgaagtgccgcaccattgtatctactacctccctgttgactctacgaggccgtttttcaggcttaatatccacatcatagtgatacacatctattttaggaatctgaacctgaaaatgattggctaacagtcgaattggttttccaacagttccaaggccaggacgacgaggtggctgaaacaggctagccggaggtccgggtcccagcgcctccatggcggcggcgggggccgcctcgccccggtccccggcgcctcccgctccgggccccgccgccgccgccgccgccgccgcgtaacgcttgatctccggaatattggcgctggggtggcgccgcggagacgcgggcgctgggcagggggcggcggcggcgcccggcccggggacagggacccggctccggctcttccggcctcagcgacaacaaaaacaatccccgccgccgccgccgccgccgccgccaacgggagcgggagcgggagccagcgcgcgcgcccgccgggagggaagggggcgcggggtgcgcggacccagggtcccggcgggcggagggggcgtgcgcggccccgggcgcggggtccacagagcccggcaggcggcgaggcgggtcggggaac

SEQ ID NO: 10375 - RNA, 4196 nt, Homo sapiens
  source 1..4196: mol_type = other RNA
ccatgtgtctgggctgggaaacactggctggtgctaccaagacactatgtaactgttgtccattcacaaagtattatctacactacatacagaatacattttcccctacattttaactgatgctcgctttagagcaactccctttgtttggacaagaaaggaatcccatctccctgtgagtggaatccagaatctattaagaaaaatcaaccttttccacacagttttagtttaataaaaggaaggaaaacccaccaagtacatttcatgtcgaaagagaagcaaaaaatttgtactgcaagtagtcgtgtgagttaccttgattcccaggaaaagaaattttaaatgctggtacatttgcaagttgcagcatcactcattgtaccttaaggactggcaaagcctttccaataaggaagcatcctggttctagcttattttaaaacaaagtgacaggacaccaactgtgaatataaaacaggtaaaaataattctttaaaaaggcatggaaatatatgtcttttctgactggtttcagaaattgccagattatgatatataagaaatagctgataaaatcatactgaaatctcatctagaaaactacattgttggggaaggaagaggagagaccttaaaaaatgtttattgccaaagttaagtttctatgagaaaagtttaaaaatcatttagatttaacaaaccacacagcagcataaaatgggcacttttgaaaacttggaaaaatactaaaagcaatttttttttccaaataggggaaacatgagtacttttatcatggcagtgttatctccgtcactgtgacatgcattacatctgtttatgtcacacattcacaaaagtcgaccaaataagagaactgcctatttgaatctgcagccaaatatagtgcaaattgcctgtcagcatgtacttgcaccagcacaagtctgcagagatcaataagataaagtagtaaaactaataaaactctgtaaaactttcaaaaattaatgctcattaaaggcatttacagtggcaaagtcagaaatcttcattaaaaagtctatggacccacacaattaaatagttacactgaactgaagtagattgtttggtttttctctcccacttatgcatataccccactcaatgactacagaaaaaaggaataatcttctcttctaagactagagggatgcggtgaacaccacagctagcaaaatattccatagaaacccttcttgtaaagtcctttagaaagttcaggctgatcagcctttgcacattgaggtaaaaattcagtccagtgcatcagaaaagataatctattagtatctattactttaaaaaaatggctcaattttgttgacgcatcagacagtgctgcaaagtatagattcagtgcaactattccgagctgctggtagaagaccacctgaagtcaacgtggctcgatctagaggcggtaggcatttgaaacattttgaggctgcatggggtgccaaattggttgagttctttttctgagactctcaggcaaaatacatcgtgtgctgggtatcatggtggatttgcacagccttagccaaggcctgaggatcccggccgttgctctgtcctgacacatgactgccttccgcactgtcatgatctttatccaccagatgataccttgccctaaatgctacaagccgggcataatatgcaggggctggaatagagactgagcgagtgcacctcacataggtgtgacacagctggtaagtcagtagctggagttcatctgcagtgaagcagttgtcatcccacaagacctggtaatgtgagggacggctggttccctgaattcctgcatgactacagaggtaaaagtcaaactcagatggatgtgtgatggtactatccactgtagtgcctgctggtacattgccacttttccctaccctttctgttttatctgcacagaagagtcgtgtgtgatgtcttttttgcaccacaatataagttattcctggccggtaatcttcttccaagctaatacatgcctttcgaattgctattagttctggccaagctacctgtttcatttgtccctcagatacccctccacggtaatagatgatccgagtgggtttgaagcgtgtggatttgtagaactgaatcagcagctctcgaaccatgttagtcaggtcctggatgacctcttgactgtagaggagctcttgggagatctcctgccgggaagtctgcacccgaacggtggcacagtaccggctggggtggccatccatactgccaaccacagcagcaatggaaggtttcttcccatcccctgctggggggtgtgtgacatccgctcccaggaagatgacaggctgctggaacaccgagggcctttgatgaggcacaagcacattgttaattcctccaagttttgcatttatcttcaggcaaagattggaaagggtttgaggtgaggtcttcactacattttttacctggacacactgtgtggccatacctagaagggtatctccaacacgtttcacctccgcatatactggtgtctttccaggcaggataaccactattagctgtaggcccacataagtcattttcagatgtttaaacataggctccacactgtctgcaccttgtgcatacttgcagaaacatggctgaccctggatgggcattcctgcatccttagagattttacgcagctggtcagtgaaactctttagtaaatcttccctacattgtttctgaggtgcaaaacaagcaactgcccaaactttaatttcaatgccagcataaaactgctttcctcgcatgtcccagacaccctggttgggtgtggctactgttttattccggcctccatattgcagcattggtgctggaagtaccctgcctgtgagctctgtcatttcattgtggacaacaataccaaattctttaaggtatggatcaggtccacccaccatactgttgctcttcaccagtctactgatctcttcctgtctgtcaggagcagatcttgctgtagctttgatcattgtggaagtctgattgtctgtgagcttcttgatacatcgctgtcctgccactatattacagacctcgagtggcaagtatgtatgcttttgttcttgtcccacttggagacagggaagatgggggtatttcagttgcagactatacttttgcttaaaatattgagctactgtacattccatagcttgaccgttttctagctgcaaaggaaaagtttgatgactggctggccgtctagtcacattacaaactcggtattttcgtttcatctgtccacagtgggtcacctcaactttgagacctctgatttctttggtaaatttgacacgctgggagtctgttagaggtttggtctgttcattgatgttctgaatgtctaaaacctcacacatgaactcaatgataggctgagcccggtagaaagcagttgcagatacatcaatgttgagcatcatattccacatggcaggtctcacagactgatgaaaaccaaaccagacctccctgccccctcccagagggtggtagtaaccttccgggggtgagaaaaaggaacggcccactggggtgtacctcatggagggaaggtgtcttgtgataacatcaagtgcttgtactgagtcatctgggacttcattcaagtgcccagccaaagcttctaaaagcaactgaaggctcacaactgacacccactgaacagacactttaaatgtttggtctttaccctcgcctggaagagtcacctccatatcaaccctatcccgtccaattggtagtggatgtgctgtgtacatgtttcttttgccatcatacccaggctgccgatcaccaaatatttgcatcttgaagtgccgcaccattgtatctactacctccctgttgactctacgaggccgtttttcaggcttaatatccacatcatagtgatacacatctattttaggaatctgaacctgaaaatgattggctaacagtcgaattggttttccaacagttccaaggccaggacgacgaggtggctgaaacaggctagccggaggtccttagacgctagcagtcctccttcatcccttcattcagcaccacacacccaactgcgcgtccctctccgtatagccggaaggcaccacgggaat

SEQ ID NO: 10376 - RNA, 4004 nt, Homo sapiens
  source 1..4004: mol_type = other RNA
ccatgtgtctgggctgggaaacactggctggtgctaccaagacactatgtaactgttgtccattcacaaagtattatctacactacatacagaatacattttcccctacattttaactgatgctcgctttagagcaactccctttgtttggacaagaaaggaatcccatctccctgtgagtggaatccagaatctattaagaaaaatcaaccttttccacacagttttagtttaataaaaggaaggaaaacccaccaagtacatttcatgtcgaaagagaagcaaaaaatttgtactgcaagtagtcgtgtgagttaccttgattcccaggaaaagaaattttaaatgctggtacatttgcaagttgcagcatcactcattgtaccttaaggactggcaaagcctttccaataaggaagcatcctggttctagcttattttaaaacaaagtgacaggacaccaactgtgaatataaaacaggtaaaaataattctttaaaaaggcatggaaatatatgtcttttctgactggtttcagaaattgccagattatgatatataagaaatagctgataaaatcatactgaaatctcatctagaaaactacattgttggggaaggaagaggagagaccttaaaaaatgtttattgccaaagttaagtttctatgagaaaagtttaaaaatcatttagatttaacaaaccacacagcagcataaaatgggcacttttgaaaacttggaaaaatactaaaagcaatttttttttccaaataggggaaacatgagtacttttatcatggcagtgttatctccgtcactgtgacatgcattacatctgtttatgtcacacattcacaaaagtcgaccaaataagagaactgcctatttgaatctgcagccaaatatagtgcaaattgcctgtcagcatgtacttgcaccagcacaagtctgcagagatcaataagataaagtagtaaaactaataaaactctgtaaaactttcaaaaattaatgctcattaaaggcatttacagtggcaaagtcagaaatcttcattaaaaagtctatggacccacacaattaaatagttacactgaactgaagtagattgtttggtttttctctcccacttatgcatataccccactcaatgactacagaaaaaaggaataatcttctcttctaagactagagggatgcggtgaacaccacagctagcaaaatattccatagaaacccttcttgtaaagtcctttagaaagttcaggctgatcagcctttgcacattgaggtaaaaattcagtccagtgcatcagaaaagataatctattagtatctattactttaaaaaaatggctcaattttgttgacgcatcagacagtgctgcaaagtatagattcagtgcaactattccgagctgctggtagaagaccacctgaagtcaacgtggctcgatctagaggcggtaggcatttgaaacattttgaggctgcatggggtgccaaattggttgagttctttttctgagactctcaggcaaaatacatcgtgtgctgggtatcatggtggatttgcacagccttagccaaggcctgaggatcccggccgttgctctgtcctgacacatgactgccttccgcactgtcatgatctttatccaccagatgataccttgccctaaatgctacaagccgggcataatatgcaggggctggaatagagactgagcgagtgcacctcacataggtgtgacacagctggtaagtcagtagctggagttcatctgcagtgaagcagttgtcatcccacaagacctggtaatgtgagggacggctggttccctgaattcctgcatgactacagaggtaaaagtcaaactcagatggatgtgtgatggtactatccactgtagtgcctgctggtacattgccacttttccctaccctttctgttttatctgcacagaagagtcgtgtgtgatgtcttttttgcaccacaatataagttattcctggccggtaatcttcttccaagctaatacatgcctttcgaattgctattagttctggccaagctacctgtttcatttgtccctcagatacccctccacggtaatagatgatccgagtgggtttgaagcgtgtggatttgtagaactgaatcagcagctctcgaaccatgttagtcaggtcctggatgacctcttgactgtagaggagctcttgggagatctcctgccgggaagtctgcacccgaacggtggcacagtaccggctggggtggccatccatactgccaaccacagcagcaatggaaggtttcttcccatcccctgctggggggtgtgtgacatccgctcccaggaagatgacaggctgctggaacaccgagggcctttgatgaggcacaagcacattgttaattcctccaagttttgcatttatcttcaggcaaagattggaaagggtttgaggtgaggtcttcactacattttttacctggacacactgtgtggccatacctagaagggtatctccaacacgtttcacctccgcatatactggtgtctttccaggcaggataaccactattagctgtaggcccacataagtcattttcagatgtttaaacataggctccacactgtctgcaccttgtgcatacttgcagaaacatggctgaccctggatgggcattcctgcatccttagagattttacgcagctggtcagtgaaactctttagtaaatcttccctacattgtttctgaggtgcaaaacaagcaactgcccaaactttaatttcaatgccagcataaaactgctttcctcgcatgtcccagacaccctggttgggtgtggctactgttttattccggcctccatattgcagcattggtgctggaagtaccctgcctgtgagctctgtcatttcattgtggacaacaataccaaattctttaaggtatggatcaggtccacccaccatactgttgctcttcaccagtctactgatctcttcctgtctgtcaggagcagatcttgctgtagctttgatcattgtggaagtctgattgtctgtgagcttcttgatacatcgctgtcctgccactatattacagacctcgagtggcaagtatgtatgcttttgttcttgtcccacttggagacagggaagatgggggtatttcagttgcagactatacttttgcttaaaatattgagctactgtacattccatagcttgaccgttttctagctgcaaaggaaaagtttgatgactggctggccgtctagtcacattacaaactcggtattttcgtttcatctgtccacagtgggtcacctcaactttgagacctctgatttctttggtaaatttgacacgctgggagtctgttagaggtttggtctgttcattgatgttctgaatgtctaaaacctcacacatgaactcaatgataggctgagcccggtagaaagcagttgcagatacatcaatgttgagcatcatattccacatggcaggtctcacagactgatgaaaaccaaaccagacctccctgccccctcccagagggtggtagtaaccttccgggggtgagaaaaaggaacggcccactggggtgtacctcatggagggaaggtgtcttgtgataacatcaagtgcttgtactgagtcatctgggacttcattcaagtgcccagccaaagcttctaaaagcaactgaaggctcacaactgacacccactgaacagacactttaaatgtttggtctttaccctcgcctggaagagtcacctccatatcaaccctatcccgtccaattggtagtggatgtgctgtgtacatgtttcttttgccatcatacccaggctgccgatcaccaaatatttgcatcttgaagtgccgcaccattgtatctactacctcccttcactgttgactctacgaggccgtttttcaggcttaatatccacatcatagtgatacacatctatt

SEQ ID NO: 10377 - RNA, 3800 nt, Homo sapiens
  source 1..3800: mol_type = other RNA
ccatgtgtctgggctgggaaacactggctggtgctaccaagacactatgtaactgttgtccattcacaaagtattatctacactacatacagaatacattttcccctacattttaactgatgctcgctttagagcaactccctttgtttggacaagaaaggaatcccatctccctgtgagtggaatccagaatctattaagaaaaatcaaccttttccacacagttttagtttaataaaaggaaggaaaacccaccaagtacatttcatgtcgaaagagaagcaaaaaatttgtactgcaagtagtcgtgtgagttaccttgattcccaggaaaagaaattttaaatgctggtacatttgcaagttgcagcatcactcattgtaccttaaggactggcaaagcctttccaataaggaagcatcctggttctagcttattttaaaacaaagtgacaggacaccaactgtgaatataaaacaggtaaaaataattctttaaaaaggcatggaaatatatgtcttttctgactggtttcagaaattgccagattatgatatataagaaatagctgataaaatcatactgaaatctcatctagaaaactacattgttggggaaggaagaggagagaccttaaaaaatgtttattgccaaagttaagtttctatgagaaaagtttaaaaatcatttagatttaacaaaccacacagcagcataaaatgggcacttttgaaaacttggaaaaatactaaaagcaatttttttttccaaataggggaaacatgagtacttttatcatggcagtgttatctccgtcactgtgacatgcattacatctgtttatgtcacacattcacaaaagtcgaccaaataagagaactgcctatttgaatctgcagccaaatatagtgcaaattgcctgtcagcatgtacttgcaccagcacaagtctgcagagatcaataagataaagtagtaaaactaataaaactctgtaaaactttcaaaaattaatgctcattaaaggcatttacagtggcaaagtcagaaatcttcattaaaaagtctatggacccacacaattaaatagttacactgaactgaagtagattgtttggtttttctctcccacttatgcatataccccactcaatgactacagaaaaaaggaataatcttctcttctaagactagagggatgcggtgaacaccacagctagcaaaatattccatagaaacccttcttgtaaagtcctttagaaagttcaggctgatcagcctttgcacattgaggtaaaaattcagtccagtgcatcagaaaagataatctattagtatctattactttaaaaaaatggctcaattttgttgacgcatcagacagtgctgcaaagtatagattcagtgcaactattccgagctgctggtagaagaccacctgaagtcaacgtggctcgatctagaggcggtaggcatttgaaacattttgaggctgcatggggtgccaaattggttgagttctttttctgagactctcaggcaaaatacatcgtgtgctgggtatcatggtggatttgcacagccttagccaaggcctgaggatcccggccgttgctctgtcctgacacatgactgccttccgcactgtcatgatctttatccaccagatgataccttgccctaaatgctacaagccgggcataatatgcaggggctggaatagagactgagcgagtgcacctcacataggtgtgacacagctggtaagtcagtagctggagttcatctgcagtgaagcagttgtcatcccacaagacctggtaatgtgagggacggctggttccctgaattcctgcatgactacagaggtaaaagtcaaactcagatggatgtgtgatggtactatccactgtagtgcctgctggtacattgccacttttccctaccctttctgttttatctgcacagaagagtcgtgtgtgatgtcttttttgcaccacaatataagttattcctggccggtaatcttcttccaagctaatacatgcctttcgaattgctattagttctggccaagctacctgtttcatttgtccctcagatacccctccacggtaatagatgatccgagtgggtttgaagcgtgtggatttgtagaactgaatcagcagctctcgaaccatgttagtcaggtcctggatgacctcttgactgtagaggagctcttgggagatctcctgccgggaagtctgcacccgaacggtggcacagtaccggctggggtggccatccatactgccaaccacagcagcaatggaaggtttcttcccatcccctgctggggggtgtgtgacatccgctcccaggaagatgacaggctgctggaacaccgagggcctttgatgaggcacaagcacattgttaattcctccaagttttgcatttatcttcaggcaaagattggaaagggtttgaggtgaggtcttcactacattttttacctggacacactgtgtggccatacctagaagggtatctccaacacgtttcacctccgcatatactggtgtctttccaggcaggataaccactattagctgtaggcccacataagtcattttcagatgtttaaacataggctccacactgtctgcaccttgtgcatacttgcagaaacatggctgaccctggatgggcattcctgcatccttagagattttacgcagctggtcagtgaaactctttagtaaatcttccctacattgtttctgaggtgcaaaacaagcaactgcccaaactttaatttcaatgccagcataaaactgctttcctcgcatgtcccagacaccctggttgggtgtggctactgttttattccggcctccatattgcagcattggtgctggaagtaccctgcctgtgagctctgtcatttcattgtggacaacaataccaaattctttaaggtatggatcaggtccacccaccatactgttgctcttcaccagtctactgatctcttcctgtctgtcaggagcagatcttgctgtagctttgatcattgtggaagtctgattgtctgtgagcttcttgatacatcgctgtcctgccactatattacagacctcgagtggcaagtatgtatgcttttgttcttgtcccacttggagacagggaagatgggggtatttcagttgcagactatacttttgcttaaaatattgagctactgtacattccatagcttgaccgttttctagctgcaaaggaaaagtttgatgactggctggccgtctagtcacattacaaactcggtattttcgtttcatctgtccacagtgggtcacctcaactttgagacctctgatttctttggtaaatttgacacgctgggagtctgttagaggtttggtctgttcattgatgttctgaatgtctaaaacctcacacatgaactcaatgataggctgagcccggtagaaagcagttgcagatacatcaatgttgagcatcatattccacatggcaggtctcacagactgatgaaaaccaaaccagacctccctgccccctcccagagggtggtagtaaccttccgggggtgagaaaaaggaacggcccactggggtgtacctgaagaaataagagtttgcatgtgtcacattaaacatgtgaaaggtccttcatttcactctcaactctgggagctcatggagggaaggtgtcttgtgataacatcaagtgcttgtactgagtcatctgggacttcattcaagtgcccagccaaagcttctaaaagc

SEQ ID NO: 10378 - RNA, 3663 nt, Homo sapiens
  source 1..3663: mol_type = other RNA
ccatgtgtctgggctgggaaacactggctggtgctaccaagacactatgtaactgttgtccattcacaaagtattatctacactacatacagaatacattttcccctacattttaactgatgctcgctttagagcaactccctttgtttggacaagaaaggaatcccatctccctgtgagtggaatccagaatctattaagaaaaatcaaccttttccacacagttttagtttaataaaaggaaggaaaacccaccaagtacatttcatgtcgaaagagaagcaaaaaatttgtactgcaagtagtcgtgtgagttaccttgattcccaggaaaagaaattttaaatgctggtacatttgcaagttgcagcatcactcattgtaccttaaggactggcaaagcctttccaataaggaagcatcctggttctagcttattttaaaacaaagtgacaggacaccaactgtgaatataaaacaggtaaaaataattctttaaaaaggcatggaaatatatgtcttttctgactggtttcagaaattgccagattatgatatataagaaatagctgataaaatcatactgaaatctcatctagaaaactacattgttggggaaggaagaggagagaccttaaaaaatgtttattgccaaagttaagtttctatgagaaaagtttaaaaatcatttagatttaacaaaccacacagcagcataaaatgggcacttttgaaaacttggaaaaatactaaaagcaatttttttttccaaataggggaaacatgagtacttttatcatggcagtgttatctccgtcactgtgacatgcattacatctgtttatgtcacacattcacaaaagtcgaccaaataagagaactgcctatttgaatctgcagccaaatatagtgcaaattgcctgtcagcatgtacttgcaccagcacaagtctgcagagatcaataagataaagtagtaaaactaataaaactctgtaaaactttcaaaaattaatgctcattaaaggcatttacagtggcaaagtcagaaatcttcattaaaaagtctatggacccacacaattaaatagttacactgaactgaagtagattgtttggtttttctctcccacttatgcatataccccactcaatgactacagaaaaaaggaataatcttctcttctaagactagagggatgcggtgaacaccacagctagcaaaatattccatagaaacccttcttgtaaagtcctttagaaagttcaggctgatcagcctttgcacattgaggtaaaaattcagtccagtgcatcagaaaagataatctattagtatctattactttaaaaaaatggctcaattttgttgacgcatcagacagtgctgcaaagtatagattcagtgcaactattccgagctgctggtagaagaccacctgaagtcaacgtggctcgatctagaggcggtaggcatttgaaacattttgaggctgcatggggtgccaaattggttgagttctttttctgagactctcaggcaaaatacatcgtgtgctgggtatcatggtggatttgcacagccttagccaaggcctgaggatcccggccgttgctctgtcctgacacatgactgccttccgcactgtcatgatctttatccaccagatgataccttgccctaaatgctacaagccgggcataatatgcaggggctggaatagagactgagcgagtgcacctcacataggtgtgacacagctggtaagtcagtagctggagttcatctgcagtgaagcagttgtcatcccacaagacctggtaatgtgagggacggctggttccctgaattcctgcatgactacagaggtaaaagtcaaactcagatggatgtgtgatggtactatccactgtagtgcctgctggtacattgccacttttccctaccctttctgttttatctgcacagaagagtcgtgtgtgatgtcttttttgcaccacaatataagttattcctggccggtaatcttcttccaagctaatacatgcctttcgaattgctattagttctggccaagctacctgtttcatttgtccctcagatacccctccacggtaatagatgatccgagtgggtttgaagcgtgtggatttgtagaactgaatcagcagctctcgaaccatgttagtcaggtcctggatgacctcttgactgtagaggagctcttgggagatctcctgccgggaagtctgcacccgaacggtggcacagtaccggctggggtggccatccatactgccaaccacagcagcaatggaaggtttcttcccatcccctgctggggggtgtgtgacatccgctcccaggaagatgacaggctgctggaacaccgagggcctttgatgaggcacaagcacattgttaattcctccaagttttgcatttatcttcaggcaaagattggaaagggtttgaggtgaggtcttcactacattttttacctggacacactgtgtggccatacctagaagggtatctccaacacgtttcacctccgcatatactggtgtctttccaggcaggataaccactattagctgtaggcccacataagtcattttcagatgtttaaacataggctccacactgtctgcaccttgtgcatacttgcagaaacatggctgaccctggatgggcattcctgcatccttagagattttacgcagctggtcagtgaaactctttagtaaatcttccctacattgtttctgaggtgcaaaacaagcaactgcccaaactttaatttcaatgccagcataaaactgctttcctcgcatgtcccagacaccctggttgggtgtggctactgttttattccggcctccatattgcagcattggtgctggaagtaccctgcctgtgagctctgtcatttcattgtggacaacaataccaaattctttaaggtatggatcaggtccacccaccatactgttgctcttcaccagtctactgatctcttcctgtctgtcaggagcagatcttgctgtagctttgatcattgtggaagtctgattgtctgtgagcttcttgatacatcgctgtcctgccactatattacagacctcgagtggcaagtatgtatgcttttgttcttgtcccacttggagacagggaagatgggggtatttcagttgcagactatacttttgcttaaaatattgagctactgtacattccatagcttgaccgttttctagctgcaaaggaaaagtttgatgactggctggccgtctagtcacattacaaactcggtattttcgtttcatctgtccacagtgggtcacctcaactttgagacctctgatttctttggtaaatttgacacgctgggagtctgttagaggtttggtctgttcattgatgttctgaatgtctaaaacctcacacatgaactcaatgataggctgagcccggtagaaagcagttgcagatactgaagaaataagagtttgcatgtgtcacattaaacatgtgaaaggtccttcatttcactctcaactctgggagctcatggagggaaggtgtcttgtgataacatcaagtgcttgtactgagtcatctgggacttcattcaagtgcccagccaaagcttctaaaagc

SEQ ID NO: 10379 - RNA, 4807 nt, Homo sapiens
  source 1..4807: mol_type = other RNA
ccatgtgtctgggctgggaaacactggctggtgctaccaagacactatgtaactgttgtccattcacaaagtattatctacactacatacagaatacattttcccctacattttaactgatgctcgctttagagcaactccctttgtttggacaagaaaggaatcccatctccctgtgagtggaatccagaatctattaagaaaaatcaaccttttccacacagttttagtttaataaaaggaaggaaaacccaccaagtacatttcatgtcgaaagagaagcaaaaaatttgtactgcaagtagtcgtgtgagttaccttgattcccaggaaaagaaattttaaatgctggtacatttgcaagttgcagcatcactcattgtaccttaaggactggcaaagcctttccaataaggaagcatcctggttctagcttattttaaaacaaagtgacaggacaccaactgtgaatataaaacaggtaaaaataattctttaaaaaggcatggaaatatatgtcttttctgactggtttcagaaattgccagattatgatatataagaaatagctgataaaatcatactgaaatctcatctagaaaactacattgttggggaaggaagaggagagaccttaaaaaatgtttattgccaaagttaagtttctatgagaaaagtttaaaaatcatttagatttaacaaaccacacagcagcataaaatgggcacttttgaaaacttggaaaaatactaaaagcaatttttttttccaaataggggaaacatgagtacttttatcatggcagtgttatctccgtcactgtgacatgcattacatctgtttatgtcacacattcacaaaagtcgaccaaataagagaactgcctatttgaatctgcagccaaatatagtgcaaattgcctgtcagcatgtacttgcaccagcacaagtctgcagagatcaataagataaagtagtaaaactaataaaactctgtaaaactttcaaaaattaatgctcattaaaggcatttacagtggcaaagtcagaaatcttcattaaaaagtctatggacccacacaattaaatagttacactgaactgaagtagattgtttggtttttctctcccacttatgcatataccccactcaatgactacagaaaaaaggaataatcttctcttctaagactagagggatgcggtgaacaccacagctagcaaaatattccatagaaacccttcttgtaaagtcctttagaaagttcaggctgatcagcctttgcacattgaggtaaaaattcagtccagtgcatcagaaaagataatctattagtatctattactttaaaaaaatggctcaattttgttgacgcatcagacagtgctgcaaagtatagattcagtgcaactattccgagctgctggtagaagaccacctgaagtcaacgtggctcgatctagaggcggtaggcatttgaaacattttgaggctgcatggggtgccaaattggttgagttctttttctgagactctcaggcaaaatacatcgtgtgctgggtatcatggtggatttgcacagccttagccaaggcctgaggatcccggccgttgctctgtcctgacacatgactgccttccgcactgtcatgatctttatccaccagatgataccttgccctaaatgctacaagccgggcataatatgcaggggctggaatagagactgagcgagtgcacctcacataggtgtgacacagctggtaagtcagtagctggagttcatctgcagtgaagcagttgtcatcccacaagacctggtaatgtgagggacggctggttccctgaattcctgcatgactacagaggtaaaagtcaaactcagatggatgtgtgatggtactatccactgtagtgcctgctggtacattgccacttttccctaccctttctgttttatctgcacagaagagtcgtgtgtgatgtcttttttgcaccacaatataagttattcctggccggtaatcttcttccaagctaatacatgcctttcgaattgctattagttctggccaagctacctgtttcatttgtccctcagatacccctccacggtaatagatgatccgagtgggtttgaagcgtgtggatttgtagaactgaatcagcagctctcgaaccatgttagtcaggtcctggatgacctcttgactgtagaggagctcttgggagatctcctgccgggaagtctgcacccgaacggtggcacagtaccggctggggtggccatccatactgccaaccacagcagcaatggaaggtttcttcccatcccctgctggggggtgtgtgacatccgctcccaggaagatgacaggctgctggaacaccgagggcctttgatgaggcacaagcacattgttaattcctccaagttttgcatttatcttcaggcaaagattggaaagggtttgaggtgaggtcttcactacattttttacctggacacactgtgtggccatacctagaagggtatctccaacacgtttcacctccgcatatactggtgtctttccaggcaggataaccactattagctgtaggcccacataagtcattttcagatgtttaaacataggctccacactgtctgcaccttgtgcatacttgcagaaacatggctgaccctggatgggcattcctgcatccttagagattttacgcagctggtcagtgaaactctttagtaaatcttccctacattgtttctgaggtgcaaaacaagcaactgcccaaactttaatttcaatgccagcataaaactgctttcctcgcatgtcccagacaccctggttgggtgtggctactgttttattccggcctccatattgcagcattggtgctggaagtaccctgcctgtgagctctgtcatttcattgtggacaacaataccaaattctttaaggtatggatcaggtccacccaccatactgttgctcttcaccagtctactgatctcttcctgtctgtcaggagcagatcttgctgtagctttgatcattgtggaagtctgattgtctgtgagcttcttgatacatcgctgtcctgccactatattacagacctcgagtggcaagtatgtatgcttttgttcttgtcccacttggagacagggaagatgggggtatttcagttgcagactatacttttgcttaaaatattgagctactgtacattccatagcttgaccgttttctagctgcaaaggaaaagtttgatgactggctggccgtctagtcacattacaaactcggtattttcgtttcatctgtccacagtgggtcacctcaactttgagacctgaaattttttttaaaaggcaaaacatcagttaattaaaatcacagtggcaaaaacagattcaaatgttgtcttcaaaatgtcatgacattgtacaggataaaaattgcaagaatatggggacaatttcatcgttataggcaaaaaacctgagttaagcagaataaattagaactcagattacctaagatgctcaatctcctttagtttattatttcatccaataaatatttattaagcatcaactatgttctgatgcttattttcaggtctggagacagctttcgtgaagtttatattctagtgagggaaactaactaataacaagaagaaaagaaatcccagaaggataataaatgaatttatgttattttattaaaatggaagttcttaagtgggtaagcatagcatttactgagtgcctgatatgtgacaggtactatgctagaaagctttataagcctaattgcatttaattctcacaacaactctacaaggtatatattattatctttaccttagagatgaatacactaaggttcacagtggttaaggaacttgaccaaggtcccattgatagaagtggttagcctgagaccgaagcccaggtctgtgtgactccagagcacaggcaacgtgcagcatgctgagctgcttctccaagactacattaatgcaaacacttacctctgatttctttggtaaatttgacacgctgggagtctgttagaggtttggtctgttcattgatgttctgaatgtctaaaacctcacacatgaactcaatgataggctgagcccggtagaaagcagttgcagatactaacaaacagagaaggatacttcacttcagggaaaagggaagggccaaaacaaacaaacaaacaaaaaccagcccaaagagttattggataaagagagttccatcctaccatcaatgttgagcatcatattccacatggcaggtctcacagactgatgaaaaccaaaccagacctccctgccccctcccagagggtggtagtaaccttccgggggtgagaaaaaggaacggcccactggggtgtacctgaagaaataagagtttgcatgtgtcacattaaacatgtgaaaggtccttcatttcactctcaactctgggagctcatggagggaaggtgtcttgtgataacatcaagtgcttgtactgagtcatctgggacttcattcaagtgcccagccaaagcttctaaaagcaactgaaggctcacaactgacacccactgaacagacactttaaatgtttggtctttaccctcgcctggaagagtcacctccatatcaaccctatcccgtccaattggtagtggatgtgctgtgtacatgtttcttttgccatcatacccaggctgccgatcaccaaatatttgcatcttgaagtgccgcaccattgtatctactacctcc

SEQ ID NO: 10380 - RNA, 4022 nt, Homo sapiens
  source 1..4022: mol_type = other RNA
ccatgtgtctgggctgggaaacactggctggtgctaccaagacactatgtaactgttgtccattcacaaagtattatctacactacatacagaatacattttcccctacattttaactgatgctcgctttagagcaactccctttgtttggacaagaaaggaatcccatctccctgtgagtggaatccagaatctattaagaaaaatcaaccttttccacacagttttagtttaataaaaggaaggaaaacccaccaagtacatttcatgtcgaaagagaagcaaaaaatttgtactgcaagtagtcgtgtgagttaccttgattcccaggaaaagaaattttaaatgctggtacatttgcaagttgcagcatcactcattgtaccttaaggactggcaaagcctttccaataaggaagcatcctggttctagcttattttaaaacaaagtgacaggacaccaactgtgaatataaaacaggtaaaaataattctttaaaaaggcatggaaatatatgtcttttctgactggtttcagaaattgccagattatgatatataagaaatagctgataaaatcatactgaaatctcatctagaaaactacattgttggggaaggaagaggagagaccttaaaaaatgtttattgccaaagttaagtttctatgagaaaagtttaaaaatcatttagatttaacaaaccacacagcagcataaaatgggcacttttgaaaacttggaaaaatactaaaagcaatttttttttccaaataggggaaacatgagtacttttatcatggcagtgttatctccgtcactgtgacatgcattacatctgtttatgtcacacattcacaaaagtcgaccaaataagagaactgcctatttgaatctgcagccaaatatagtgcaaattgcctgtcagcatgtacttgcaccagcacaagtctgcagagatcaataagataaagtagtaaaactaataaaactctgtaaaactttcaaaaattaatgctcattaaaggcatttacagtggcaaagtcagaaatcttcattaaaaagtctatggacccacacaattaaatagttacactgaactgaagtagattgtttggtttttctctcccacttatgcatataccccactcaatgactacagaaaaaaggaataatcttctcttctaagactagagggatgcggtgaacaccacagctagcaaaatattccatagaaacccttcttgtaaagtcctttagaaagttcaggctgatcagcctttgcacattgaggtaaaaattcagtccagtgcatcagaaaagataatctattagtatctattactttaaaaaaatggctcaattttgttgacgcatcagacagtgctgcaaagtatagattcagtgcaactattccgagctgctggtagaagaccacctgaagtcaacgtggctcgatctagaggcggtaggcatttgaaacattttgaggctgcatggggtgccaaattggttgagttctttttctgagactctcaggcaaaatacatcgtgtgctgggtatcatggtggatttgcacagccttagccaaggcctgaggatcccggccgttgctctgtcctgacacatgactgccttccgcactgtcatgatctttatccaccagatgataccttgccctaaatgctacaagccgggcataatatgcaggggctggaatagagactgagcgagtgcacctcacataggtgtgacacagctggtaagtcagtagctggagttcatctgcagtgaagcagttgtcatcccacaagacctggtaatgtgagggacggctggttccctgaattcctgcatgactacagaggtaaaagtcaaactcagatggatgtgtgatggtactatccactgtagtgcctgctggtacattgccacttttccctaccctttctgttttatctgcacagaagagtcgtgtgtgatgtcttttttgcaccacaatataagttattcctggccggtaatcttcttccaagctaatacatgcctttcgaattgctattagttctggccaagctacctgtttcatttgtccctcagatacccctccacggtaatagatgatccgagtgggtttgaagcgtgtggatttgtagaactgaatcagcagctctcgaaccatgttagtcaggtcctggatgacctcttgactgtagaggagctcttgggagatctcctgccgggaagtctgcacccgaacggtggcacagtaccggctggggtggccatccatactgccaaccacagcagcaatggaaggtttcttcccatcccctgctggggggtgtgtgacatccgctcccaggaagatgacaggctgctggaacaccgagggcctttgatgaggcacaagcacattgttaattcctccaagttttgcatttatcttcaggcaaagattggaaagggtttgaggtgaggtcttcactacattttttacctggacacactgtgtggccatacctagaagggtatctccaacacgtttcacctccgtttagtaaatcttccctacattgtttctgaggtgcaaaacaagcaactgcccaaactttaatttcaatgccagcataaaactgctttcctcgcatgtcccagacaccctggttgggtgtggctactgttttattccggcctccatattgcagcattggtgctggaagtaccctgcctgtgagctctgtcatttcattgtggacaacaataccaaattctttaaggtatggatcaggtccacccaccatactgttgctcttcaccagtctactgatctcttcctgtctgtcaggagcagatcttgctgtagctttgatcattgtggaagtctgattgtctgtgagcttcttgatacatcgctgtcctgccactatattacagacctcgagtggcaagtatgtatgcttttgttcttgtcccacttggagacagggaagatgggggtatttcagttgcagactatacttttgcttaaaatattgagctactgtacattccatagcttgaccgttttctagctgcaaaggaaaagtttgatgactggctggccgtctagtcacattacaaactcggtattttcgtttcatctgtccacagtgggtcacctcaactttgagacctctgatttctttggtaaatttgacacgctgggagtctgttagaggtttggtctgttcattgatgttctgaatgtctaaaacctcacacatgaactcaatgataggctgagcccggtagaaagcagttgcagatacatcaatgttgagcatcatattccacatggcaggtctcacagactgatgaaaaccaaaccagacctccctgccccctcccagagggtggtagtaaccttccgggggtgagaaaaaggaacggcccactggggtgtacctcatggagggaaggtgtcttgtgataacatcaagtgcttgtactgagtcatctgggacttcattcaagtgcccagccaaagcttctaaaagcaactgaaggctcacaactgacacccactgaacagacactttaaatgtttggtctttaccctcgcctggaagagtcacctccatatcaaccctatcccgtccaattggtagtggatgtgctgtgtacatgtttcttttgccatcatacccaggctgccgatcaccaaatatttgcatcttgaagtgccgcaccattgtatctactacctccctgttgactctacgaggccgtttttcaggcttaatatccacatcatagtgatacacatctattttaggaatctgaacctgaaaatgattggctaacagtcgaattggttttccaacagttccaaggccaggacgacgaggtggctgaaacaggctagccggaggtccgggtcccagcgcctccatggcggcggcgggggccgcctcgccccggtccccggcgcctcccgctccgggccccgccgccgccgccgccgccgccgcgtaacgct

SEQ ID NO: 10381 - RNA, 7433 nt, Homo sapiens
  source 1..7433: mol_type = other RNA
cccactgccccaggtgctgctggcctcagtcaagggtggattcccccagggcaccgaagtgagtgccaatccttctggtcatgaggagaggtggtaaggaaggtcactttctctgccttctctggtcacagccaggtttccctgaggcaagaactgtggttacatctgagccaccactgggattaaatttcagccgcttggttgcctggctcagcctggctggcctcaagccctgtagagccagtgtggaggtaggctggacacatgcatccatgctgagactgtcctgaggaaggggggttttcttgcagctctgaaatgcaacttctaaggggagcaaaaagacatcctaaggctgcccagatctgtccccgaaggccttctcagatccgctctttctactagaagaattggaactgcatttccaggcctcgagcagttcctggtccacagctggaattcaattcaactcatattggtctaacgaagtaaatagatcgaggtcccttcctccccagactgtcccaggcaccttcctctgtccccttcagtcttgcatcctttctggggcatttttcttttcttttcttttcttttcttttttttttttttttttttgagagggagcctcactctatcacccaggatataatgcagtggcacgatctcagctcactgcaacctccacttcccaggttcaagcaatcctccctgcctcagcctcccaagtagctgggattacaggtgtccaccaccacaccggctaatttttgtatttttttagtagagatggggtttcgctatgttcactaggctggtcttgaactcccgacttcaggtgatccgcccaccttggccttccaatgctgggattataggcatgagacaccgcacctggctggcatttttcttggtaaggaaatttaccatctacccctccctaccccccaggtcttcttttcctgtccctacagtagatgggtctctgggaaggggccagaatcttccctttagaccctcaaagatttggagtgggtttttatgtgaggttctcaaagccctttggaaccaagtccatggcactgggagtgaaagccaggcagtggtgagtgggggcgttggcacattcagtggggagcagtccagagttcccaagagggacctagggtgcagtctagatggaaggctggggatctgccttgaggttgcatttgcattgaatgcaccttactttacttggggtattttgaagatgctgtggagattatgaggatcaaagccctccaaagctatccttggtgccaatattggtatccaggggagggaatctaggcatctggctgtcctgcccactgtccgtgccaggggctttgcctacagtcccaggagggaggagggaaaagcaaagagagcctgggaaaggagagggaagcagaggccctggagctgggggaaaggagggtcattggtattctgggcgctgaggagttcctggctgggcagcactcaaggcccaccccctggcatcaggctgcacattcagcatcgacagccctggccagtaggccttctgggctcccagcaacgcctgcattttgcacattggtttgcatgactggtaatgtcccttcacagggccaccctcaccccacccccaccccaggtctagagatttcctgaattgctttgcttaacccatgattctgctgtctaacctccatccttccagctgcaaagtcagctcctcctctgtgcagggagtgggagcaccacaggagccaatgcccaatcatagctgcctccagggaggtagctacggtcctttgcaccccattctgcctccagaaaagagttttccattttttttattagaaagggtgtctcttttcaggagcaaagcccccattctcccttcatccacttcttacagtctaattgactccctcctccttcttctttgaacaacgagaagactctccagttgtccaacttccacccctccagctgcaacatcgtcatcctttagctcagcgaacgctgggcgaacgctccctccccgcccctcctgcccctcctccctactccaagccctcggcttctcatccgctgaacgatgtcctacttcgctcgtccttgctctcgccgctgctgccggagccgaagcagagaaggcagcgggtcccgtgaccgtcccgagagccccgcgctcccgaccagggggcgggggcggccccggggagggcggggcaggggcggggggaagaaagggggttttgtgctgcgccgggagggccggcgccctcttccgaatgtcctgcggccccagcctctcctcacgctcgcgcagtctccgccgcagtctcagctgcagctgcaggactgagccgtgcacccggaggagacccccggaggaggcgacaaacttcgcagtgccgcgacccaaccccagccctgggtaggtgagtgcctccgcagccccgccgcccgccgtggggtcggggacagggagaagggagtgcctgcctggtctgcgccccccgcctgtcagcccttgcctcgaggctctggggcacccaactcgtcgactcctgacaccgcagcggggtaggctgctggacagccccgagcgcctgcagctgctgctgccatctctgatctacatgcttccagctctgccagtggcagcccccctgctgctcgcagtctgatcagcaacccctcgggtcctcgcatcttccctgctgcgcgctcctgtcccagcgcggccgccgagatttccgaccttgtcccaggcagggcggtagcgttccggatcagtccttgcctccgtgcccccacgcacaggcagctccaggagcagcggccagcaacccttctggggacaccttactgtagtccggcaggacagccgatcagagccgctctagggggtggtcggagtgcccatttcggctggaatcccaactcggctccttgctctgtgaccttggggtagttagttgacttctctgaacctcgggttcctcatcggtgtaatgagcaaaacataaacaatctttttctcacagttgaggttatccacaggaagcatttaggagaactggctcaggtagacatcagtaactattagctggaattcggttaccactattgcattccttcctagcactgccaggggcctgggaattccctctcccaggtatttccatatcctgtcaggtattcccccacctattggaatagctctgcctacatggttctaataggaccaagagattggcgtcaagtccaaggggcaccattattatctgcattacttagattgcagatgatgacagtaagatcagggaacagtgttacccttagacccacccacagtattaccagtgcctatgttgctatggctaactttgctatttataacagcatcatccacatttcagattctatacgagagggatctgcaactgctcggctggtgtcattgctaatagtattattagttttgcttccaataaaaaggactatttatatgatgattgcaattacttctacaggccctaaggccctgcttatattgtgtaggctcatgttgctcctcatgaagccgttaagggggtagcagagagcttccctcctgctatagccaaagctctggcttcttgtgcctccctgctgaccctgctgagtgctggagctcagttcctatgggacagaccttggctgccggctgatgggcattcagcatggaggtggtgggtgttgttagatgtgtgtacacacgtgcatgcctacacacacacacacacacacacacacagagagagagagagagagagagagagagagagacctggtcttaactctctgggttgggtctatgaagactgtgagggagatggacatcccgggtcagacagaaatgatgtgacaagaggaaagtttcctgaacagctcaagaaattcaaaacaagggcagagatacagacgctggagctgaaacagagagggggatgttgtggcgtcaagggaacggaccgcatgactgctgagctctcagggttagagttggagaggtgtggcctgctctggaggaagagaagaggaagtggagatgagtggtgtgtgggatagagaaggccacagaaccctggacccctgggttctgaggctggtaccggatgtggggaagtctgagtttcctcagggctcctagctgcaattgggaggctgaggcccgagactggagagacagagctctctcagaactgcacggggctaccctcttggcctcactggtcagtgactcccatttttggggtcaagggtaggttgccctccatgttccagagcagttaggtcctcattggccttaggccctcttccctcactctcccactgtcagacagaggtgaaagggtggtccagggtgttggccccaaaatgactccaactatatgggtctctgggctgcccgtcagagagatgggagccaggtctgtgagcagctccagctccagcccagagagaagggagggagggcaccagaagggggccaggcccaggccctggcacagctcagatgcatggcaaacagtcttcccagcacccggtgggcactggctgctcctgcccaatggtccccactccagccccagaacagtcctcccaagcaccccaatgcctggagctggtctccgcacctctaatctggccccatcaagaacctcctccctctgaaaggtcagagagaggccctaagcatctggttgtgccactcctctcccaactctgaccctagggaatgatatccagacacagtgggggagatgggggttatgatggcagggaggtgggaggatctgggaaaagtaggaaatttcccatcatctcaggcttaggaaagtgcagggacaggtatgaaggcagatgctgagagggcagggaagatgggggataaacagtgggcctggaatgggagtgcacagccagtggaataaacctgatctctaggaagtcctgcctgtagtctaaccttcaattctcttgctgcatcattggcctattccatggcatacctggatctccatgctcttctaagtttagcccaacccttaaagatgatgtagctctgagtcttctctcctgggagcacattgccctcgtgcctgacttggctttactagggatccagggtcagccctatccttctctgagcctcagtctccatttctcaatgtcacaacacatcctttttatgagagtgtaagtgcttcgagatctttggaggaatattctgggttctagagcttctgatagccaggggtaggaaggggtagcccctcccatttattctccccccccttagtccaccctccagcccaaggctttcacaaaaggtagggtgggggaagggaggggctggatagaggccagactggcagagacaggggctttgtcccaactgatttctgagccaagagttccggtgggaaagcccgtgccaggcagaaaggagaggctgggaagaagaagggaggaggcagccaaggaagggggatggagaatgttggggagtaaagagaggagtttccttacaaataatggtggggaggaagtagaggagagggtgggctcaggagaagctgtgcttacttgcgttcggtctaggaggccctcctggaaaaggccaggtgagtatggtgtccctggaggcagggacagtctagaaggcagaagaggctaaagagatactatgggagaaggctctgggttcgaggaaggagtctggcactgggaggagcagatggaattctgagtataagagcacccaccattcatgctgtaaactgagctcctactgtctgcctggtgctatgcatttgtacaggagttttaagatactaaacactctcaaagcacatggtcctatctcaactcatgagatagtaatgatgatgcttttttataagtaagaaaataaaggctcagagaaggtaaggagcttggcttaggtcacacagtgagttgactaggactcgggttttggttctgagaagaaatcacttgctgggaagatggggatcagaaacagagagtccatggtgatgtgaaggtaggggacttctggagccaggatatgtgtgaacccacatgggtgtggtagggagcaggggggaagtccatcctgaagtctaaccccatctttccttctcatgtccctctgtcagcctgcagcatggcccagctgttcctgcccctgctggcagccctggtcctggcccaggctcctgcagctttagcagatgttctggaaggagacagctcaggtaagcaaccccacttggggtcaccgtctctgtcttgttcagccctaaccaactgcttccaggcttaggggccccaggaagagagagaattggagggctgtggggaagcgtccaggctggaacacttggaaataagggctgagctgtgagcatctggtgggttggagaaatcatggggcaggactagggaagggcactgggtgcaaggctttgggcccctaaggtggaggataggggatcctgaagctaggaggtgggaaaggggtggaactgggagaaaccctgaaggaggccctaaagggagcagactgggaaactgggctggaggactcagggggcgaggttggaggaccctggggtgtggtctaggaattttggagaggaagtggaagactctgagagcagggcaaggaatcctgggggctgaattgactgggagactttgggggatgggtctggagaccgtcggggtggtcctggaggacctagaggtagggctgcaggaccctggcccctggcccctggcccctggtcctaggggggccggggaatcctggggccggaaggagggatcctggagcggggcttggaggccaccgggtgggactctgagggtcgacagcgttaagttccagccggctccacccgttcacagaggaccgcgcttttcgcgtgcgcatcgcgggcgacgcgccactgcagggcgtgctcggcggcgccctcaccatcccttgccacgtccactacctgcggccaccgccgagccgccgggctgtgctgggctctccgcgggtcaagtggactttcctgtcccggggccgggaggcagaggtgctggtggcgcggggagtgcgcgtcaaggtgaacgaggcctaccggttccgcgtggcactgcctgcgtacccagcgtcgctcaccgacgtctccctggcgctgagcgagctgcgccccaacgactcaggtatctatcgctgtgaggtccagcacggcatcgatgacagcagcgacgcaactctccccaagagcggcaggagggctccatcatcttctctgatgtattgatcaggagagctccagaggtagacaggctgaagctggaatact

SEQ ID NO: 10382 - RNA, 10262 nt, Homo sapiens
  source 1..10262: mol_type = other RNA
ccccacctcctctctcctcagatatttggaaactttctgtaatgccgaaaatgaaaataactcgcctctgggcaccagctctgcacttgacccaggttcagaattgtgtgcacactggatccttgttataatattgcaaggcagctatcactaacccccttttaaaggcgaggaaactgaggctgagggaacccaatacatccaagtttcaggggtgggacacttcctaaacattcccactggcttctcctcaacacagtcacctggatgtgcctcctggccacccaactttccaagaatccccaggatctgactacttttcatgcctcatttggaagagaacacctgcacctcgtgcatccacaagggtccttggccagcttggtggatgggatgtgaacagaggtgctgataggccacatgaggcctggtttatggcagcatccctggttatggcagcactgaagaaagatcttcagtcctttcttcccccagatggcagagaactattaaacgcacactggactttgcatgaactggcaagaggttcttattgtccttagctgttgaaaatcagggttatctgtgctgtgctggtgcgttgatcaccaagatgaacaccacagtagctaggctctattcattctctacactaaaccctaactggtttctctgtttccactctggttcctacagtttagtctccacccaaaggccaaagggatccttgacaaatgaagcaagatcatattgtccctccgctcaaaacccactatatctagaaagcaagccagactgtggtgacttacacggtacctggggccgtgacacatgacacatgacagatgtgaccactctgtcatcatcatttcccccctcactccctcttctccatttacacaaacttctccccacttgctgcccctcaaacacaccgcacgctggaacctcagagcctttgtgcgtgctgctcctgctggctgcagtgctcttcccttgattttcctgtgcactctcctttgattacttcttgcctctgctcagacgtcccctcctcagaaatgtcttccctgaccagcctatccaaaatggcacccctccatcacgctttagccctcaccgaatttatttctcctcatggtatttaacactacctgagatatgacatattcctttacttcttgtcctccttcccttcactttagaaaggtccttgcttctgcagtgccagcacctagaacaatgtctgacacattgtaagcatttataaaaaatatttgctaaatgagcaaatggataaatttaaatttaaagtgagtccaaggcaagtccttaggtctcttcactctcaaacaaattgccagctgtgagtctgtcctatggaaaacttctgggaccacctccaccatgttcacagatggggacttggacactggtctgtctaattcctgagtatcccttctttctgttccactaggctgatctgctgcattctgtgaatcagcaaacgttctgtgaaggtccagcaaatgttctgtggaggtccagatagtgcgtggtttttctttgttggccatatggtctctgttgcaactactgaactctgctatgtagagataaagcagttatagatgatatgtaaatgaatgggtgagggtatgtgccaataacattttatttacgaaacagatggtggtctagggtttcccttgctggccaattgttggctaacccctgtgctagaggttttagaaaagggaggaggctcttgtagattccttgtgtcattagtacctctgggcagagggctggctggctgaataattaatccacagcctatgctgcatagcatctaaataggagcacctaaatcttcctgaagatgtttgctttctaatctcctttcttttgttcatgtattgctgattgtctaggctttgtcctttctgtttccagtgactagctccaattggcatagttgtatctttctgtctatccatctacttacttacctgtctgtctaaaacatcctgaagttattgtaaaagactgccaaatttagggctaatttgcataccaatcaaatgtagcctgaattttcagacagtcatgcatgcaaatgtgctaatctgaatccttgaaaatggcttcagatttatgccattgtaatcgttgacctttagtaggaaaatgttgcagtgcctggaacctgcttcattatactgctagaatcatctgggatgattgccagagttgtgctgaaagatgtcctcttggtacctgtgagcacccagtgtctagaatccacctgagaggttgttaagggctggatggagacccacagactggagtggggggttctgagccccaagggacattctctggggactgaaatgggcagacagggctgatacaggcctgggtgggatggtggtgcctgggcaaagcatgagtcaaagctcctcttgctcatgggtgttgtccacagagcctacaggaagattctggaagcaatgttctaaagaaatgcaaggtctgtggcagggccgacagtatggagcccagacttcagtccaaaagggcccaaccaagacaaaaaacaagccaaagggtgaggggttcaagagtagctgatccatgagaagcaactattgaggtgatggacctggatggattcctgacctgggactcacgcacttcctatgattgtaggaggatcccacattgcaatgagcccaagagaacagtcagcctaggcagaacgaccactgggggatggacattaagaaaagtcgccaagaaaaaaggaccaaagttgagataatgaatgtgttgaataggagttatgaatgaaaataaaaattagaaagcaaacagggaatgcagtggttgggggaacagaaggtgaggtgggcgggacagttcagggctaatcaaaagggtagacagtgaacttggtgcctgtttgtgcagtttctggcctgtagcttgggggaaatgcttggaggcttggcaaaagtatagcagtcaggattgtacagatcaaagtgtcacctaaaacaatactgttcatttgtttccctggcgtctatcaaagtacctcgcacacagcttcgccatgactcctgatgctaactagccatttaggccaaacttcacaggttaagagcacagccgttcacaagactggccttacttcagacaccagcgacaggctcaggggttccgtgaacatatggtaacacatttgggggttctcactaccccttctggtttgataatttgctcaaatgactcacagaactcaggaagtgctatgcttagaattacagctttattatagcaaaaaggatacgaatcagaataagccacaagaagagatcacagggcaaggtctggaaggattccagctctggtgttctctctcctcccacagagtgttgtctaccagggaagctcacccaagcttcagtgttccaaatttttattggggtttcatcatgtagatgtgattgatcaaatcattggccataaggttgaactcaatctttggtcctcctctcttccctggaggtagggctgatgtcacttggctcaaagccccaaccctctatcacatggctggtctttcttgcatggccaacccccatcctgagttatcttgttaacatacactatcaagggattctgagaggtctgccatgaataactcaagaaatcccaagaattcacaggctacatcccaagaaccagggacaaaggccagccaaactttattatacagttgtctactgtgtatataagatttacattacacaaatgcatattataaacagaaaatactcaaaaaatgtttgtaaaatgaattagtgagtgagagaaggaaggagtgagaaagaatgaatgagaacttaactttaggagtctaactcattggccccacaccatccaatataaattaggacttatttgaaacaacactggcagccacagaaataatactgaatggcttggctttgataagaaattactcacttttccagtggtttttgagttagccatgttttgtcttcttgggaggggagacacagactcttgtccttcatggtgttagtatttaagcccagggtttctgtagagcaattaagttgactcaatgcatttcccagcataaatggtatattctattattttctcctgtctgctccttccctaaaggcagataaacaaatgataataaaaagcaaaatcaacatttccctctataagggtagagctgcccagttagccacagatgttagaacctgatcaaacaagattcaagtgaaccaacagagagagaacccaaaagcaagttctggtgctttcagttaatcccaccccataatgccatcttagcaggctgctctgggaacccaggcgctcttagagaaagaagcatgtcgcctggcaggtgcctctggtgtggcctgagacccattctcaaggaaaccaggagggaatgatgagcagagactgtgtcaaacgacataagttctggttggggtgagggggaggcatagcagggctcaagactttggtggaagagggctgagattacaggaggaccctgtgcattgtgtcactgcagaaacaacgggcaattatgtctatgaaatgggtatctctgaatcccagagttttgtcccctcaccccccgctcttttcagttttactcttgcttttgtctcactttatctcagtaactataaaagcaacagacttccattaggaaaaaaaaaaaaaaaaaccaccgcacagaaatttgataatgaagctacacatacaaacattcttctgtgagtgagagatgatctctctcatttgtataccagccccacatggcagatttatgctgataaccctgtattacaaataagggagagattgagtgactggcctaaggctacctagctaatagatggtacacttgggcctgaacacagtcaaaacccagactccatccagaggccgcttttaatgtgtcatctaaatccactcttttttctgaagatcatcatatatactgtttaatactctcttttttggcttactatttatttgtaagcacctttctatgctattggaagttctgcatcaccaggatgtttaacagcagtgtggagctgcctcctgtgatgtcctatcttcctaatgtgggcctctgaggttgtttccaatttttctctaatatgagatgctgctgcattgtttaaattgggatctgtgagtcattgtttggtttggtttgatttgatcagagccagcacagctgctgactgatgagggcccagggaccttttccagcctggggcgttggtgtccaggtgtcccaggctgtgagtgccaactccccccgcaccatgccctggaggtcccagcgattagagctggacagcctgcctctttgatatagaattttctcatttcataaagtttctccaagaaaaatgcctttgttgagccaaatggggaaaggaactcggtcccatcaaatctccaggaagctcagcttagtgcagtgggggcagtggttgctgcagccagagagctggggatagctgatccagcaagatgggaggtagggaaacttggagggctgtgttggagttgcacagctggtgtgaacaaaccagacaagtgaaactagaagcaccctatttctgacccataggggaagaccctgaaatttattgagcacctgctgtatgctgacatcatgctcgggacttcacacacctcatttcatccttctggcggcctcatctacaagctaggggttcttattcccattctataaatgagttattccagaattgatgttgcagacggggcccctgctacctcaagcatccagaagtgaattgactggtaatgaaaacaatttgcccttttcattccggccaaccggaggatatgcaaaaaggagagcaaaatatcatctcaagtctgcgaaaatgcactgttccctgtaaacacagctatgcaacctctcaaaagaatgttccagcaggaggaaggctcaggactgtgattgaataagaataatattgggagtgcattcacttctctgcttctgcctggggccaaatagacaatgaaacttaccttctttatgtttcaactaattaaacccaagcatttggctgccccctcactgcaaaggtggctgaggggaaacccaggaggctctgaaagccttacttgcctggctgttgcttgtaattgatgtttcctctttcatcatgtttcatttcattctgaaagctaactgtgggaacaaaatagtctcaggtgtctggaggcacaggagcctctttcccagtgagtcagccaggctcctctgggagaatcacttggggaggaggaaaaaacaccacaaacctgcaaacctaatgctcaagtcaagccaaaatgggagctgagttttttccttaggacaagggaggtgtactggggtcacccaacaccaccttcaggtaggataattcactggcatgagtcacaggcgttggcacaggaatgcggtagtactcacagctatgactgatcacagtggtggaacacaatgctaagtcagcaaaggaaaaaggtgcaggggtgaagtccagaggaaaccaggggcaagctccaaagaactcttctagcagagcctcacgggacgcgcttcatccccacagcaacgagttgtgacaactcttgtgaaatttgtctaacaaggaaactcattagagacttggagtccagggtttttctcggggggtggtcacataggcactctctgcttggcaagcagaaaattccagattcccagaaagaaagcagatataaaccacactgagacagcataaaccacactgtttgcacagtttaggtacactgagtcactcttaccagatctgggaacggtggcaacccttccaacatccaagttcccagatgcaagcccgggacttaccctgcagcaggcttttctaggaagagaagtctcaggcgtgctgtgagagctcttttctacacaggaggccttacctcggggagccaggcgacattaggtagcactgctgggattgtggaattttgttcttgtggggccctaacttcagagggcctggttcaacaatgggtacttttttaaggacttctggactgcgttcttccctgtgccagtgtgttcagtggtgcagactgtctttataaagccctaaggcattgtggcatgacttcctctcttatgcaatggtgtgtgtactctggcccagctaccaagtgttacttccgtgtatttttacaggactcctgagaatcgttccaagtgagttcacgggaggctctgtgtgaatcagtaaggcacattaatattgttaaacgggctacgaggtaatttgcctcccattgtctggcaatttcttttattatttggagatgctctaagccagtcttggctgggaattgcagagttcaattttatgtccagaggcttggtccccaggttcctggcctgggagataatggtaagtgattcatggattcttgaatctgacaaataaatgagcctaggccccttattttacaaatatagcagtaaaaatatcaacaacactaccaccaaccaccccaatttccggtttttattgtgtacttcatatcgacccagcactgtgctgtatcttcattctctcattaaatcttcacagtaactcttcaaggagggcaatgatttaacagatgaggaacctgaggcgcagagaggttaagtaacttactcaaggtcacccagcaaagaagtggcagagctgagagtggaaaaaagccaattccaactacctttaacattgacagcacttccagagaggcacacagattgcttaagatcacccaaggccacagaaagactcagtgatgcaagcaagtgttaaatccagaactcttggctctttcttaagcttcctttgctttaaccatgtagccttttattcagttgtttgcagtttaggctgtagttagtactagccgtaacatcaatgcttctggagcaactcataacaattttgatcagactcatcatctcataccaattgcaggagcttcctaacaggcctagcatcctctagtctaatccctgaaatgtccttcacactgcacctatgaagaacattcttaaccacaaattagagctatcaattccgtgctaaaaccctccaatggctccccagtgcccatggaattttgtgtagactcctgaggctggcaggcaaagccaggtacaggcagcctccaaccttctactgggccacctttcaacccactgcgtcttttatacctcctgtgtggcaacctgtggtctccggtttctgcaccttcaagaattctgttaactctgcctgtcgtcctgtaactgagcccactccgtctgcccttcttgcttgcttgacttggattccacagcctttcttggcttcctattgtcatggcatttttattccatgttataattgtatgtttacttgactactgtctccactagatcttgaactccttgaaggcaagaaacagcagaatttgtatctagaagaaaggatgggaagctgggcccctggtagtgaggaagcagacctgtaaagtcagatagaaagatacaagaatgtgcctcgtggctgttggctgaatgaaaaagtaaaacaaggaatcccaagtaagataggaatgagtgagatgtcccaaagcaggcctagaggttacctaccacagtgatcttaaagcaaatttttattgcagattgttttcttcaaacaggatcgagttctcccaacacataaaaggaaagctctaggtaaaggtttatatctccaagccttcatgacttggcctaaatctctcctccttcttgaagcctcaggtcacagtgcaattgtgatggcatgggctctgtagttacgttgattgtgtcagcagggcaaacttgctgctgtaataaacaagccctgtatctcagtggcttaacacagtgaaaattcccatttatatcacctcatttgaaggagatgagcaggaacactctgctccatgaagccattcagggacccaggttccttaagtgaagtggttccaccattctctaggactttggagtcctctgctagatcctctgtggctggccagctgacaggagcaagcgtggagcaggcaaacacattctcagcgtcttggtggaggtcacacatgtcccttgtacttacactccttgcttgagaagtagtcatatggccccacctagatgcaaggaactgggtaaggtggcctggcagtatgtccaggaagaggagagcactgtgaggtctagcaggccctgcagttctaccatctttggcatggctgtgggatgtgtttctccactccagacttctctgttgtgaatgaaacttctcaggatggctacaagggttgaatgagatgagatatccaaatgtctgatacatacttagcagtcaaccaatcttcattccatgtctcctcttctcccctgtagtcgtctgtctcagctactcgggaggctgaagtaccaggacctcctgaccccaggggatcaaatctgcagtgagctgtgatcatgccactgcactccagccttcaatctctaagtaatggaggagtcataaagaagtgaggatgcagaaaaagatcagatcaaaggatgtgttggttgttatgccccaagcagctgccagtttccttttcatcattatgagagtaaaagttgatttgggctgaagtttcagcttgaagagcaactctcattggctttatttgagacgggtcattccatcacttgacagagtcaattgtgcatctgttctttcaattgcactgaaattattcttcttacacatatcattggatctggttcttccgtctgttgtggtagctccccagctggtctccctgctttcacacttgtcccctgcagtccaggagcaacagagaagacaagatgtagtgatcttgttcaagtattagccggtgtcattcctctccttggaatctcccagtggctgctatctcccccaggggggaaacgctagttcttatggtggcatagaagactctctgagttcttcttttctcttctcaactttcactttctactgcttgctccctggctccctactgcctccagccaggctggcctcactgatgtttctttctttctttttcttttcttt

SEQ ID NO: 10383 - RNA, 7053 nt, Homo sapiens
  source 1..7053: mol_type = other RNA
ccccacctcctctctcctcagatatttggaaactttctgtaatgccgaaaatgaaaataactcgcctctgggcaccagctctgcacttgacccaggttcagaattgtgtgcacactggatccttgttataatattgcaaggcagctatcactaacccccttttaaaggcgaggaaactgaggctgagggaacccaatacatccaagtttcaggggtgggacacttcctaaacattcccactggcttctcctcaacacagtcacctggatgtgcctcctggccacccaactttccaagaatccccaggatctgactacttttcatgcctcatttggaagagaacacctgcacctcgtgcatccacaagggtccttggccagcttggtggatgggatgtgaacagaggtgctgataggccacatgaggcctggtttatggcagcatccctggttatggcagcactgaagaaagatcttcagtcctttcttcccccagatggcagagaactattaaacgcacactggactttgcatgaactggcaagaggttcttattgtccttagctgttgaaaatcagggttatctgtgctgtgctggtgcgttgatcaccaagatgaacaccacagtagctaggctctattcattctctacactaaaccctaactggtttctctgtttccactctggttcctacagtttagtctccacccaaaggccaaagggatccttgacaaatgaagcaagatcatattgtccctccgctcaaaacccactatatctagaaagcaagccagactgtggtgacttacacggtacctggggccgtgacacatgacacatgacagatgtgaccactctgtcatcatcatttcccccctcactccctcttctccatttacacaaacttctccccacttgctgcccctcaaacacaccgcacgctggaacctcagagcctttgtgcgtgctgctcctgctggctgcagtgctcttcccttgattttcctgtgcactctcctttgattacttcttgcctctgctcagacgtcccctcctcagaaatgtcttccctgaccagcctatccaaaatggcacccctccatcacgctttagccctcaccgaatttatttctcctcatggtatttaacactacctgagatatgacatattcctttacttcttgtcctccttcccttcactttagaaaggtccttgcttctgcagtgccagcacctagaacaatgtctgacacattgtaagcatttataaaaaatatttgctaaatgagcaaatggataaatttaaatttaaagtgagtccaaggcaagtccttaggtctcttcactctcaaacaaattgccagctgtgagtctgtcctatggaaaacttctgggaccacctccaccatgttcacagatggggacttggacactggtctgtctaattcctgagtatcccttctttctgttccactaggctgatctgctgcattctgtgaatcagcaaacgttctgtgaaggtccagcaaatgttctgtggaggtccagatagtgcgtggtttttctttgttggccatatggtctctgttgcaactactgaactctgctatgtagagataaagcagttatagatgatatgtaaatgaatgggtgagggtatgtgccaataacattttatttacgaaacagatggtggtctagggtttcccttgctggccaattgttggctaacccctgtgctagaggttttagaaaagggaggaggctcttgtagattccttgtgtcattagtacctctgggcagagggctggctggctgaataattaatccacagcctatgctgcatagcatctaaataggagcacctaaatcttcctgaagatgtttgctttctaatctcctttcttttgttcatgtattgctgattgtctaggctttgtcctttctgtttccagtgactagctccaattggcatagttgtatctttctgtctatccatctacttacttacctgtctgtctaaaacatcctgaagttattgtaaaagactgccaaatttagggctaatttgcataccaatcaaatgtagcctgaattttcagacagtcatgcatgcaaatgtgctaatctgaatccttgaaaatggcttcagatttatgccattgtaatcgttgacctttagtaggaaaatgttgcagtgcctggaacctgcttcattatactgctagaatcatctgggatgattgccagagttgtgctgaaagatgtcctcttggtacctgtgagcacccagtgtctagaatccacctgagaggttgttaagggctggatggagacccacagactggagtggggggttctgagccccaagggacattctctggggactgaaatgggcagacagggctgatacaggcctgggtgggatggtggtgcctgggcaaagcatgagtcaaagctcctcttgctcatgggtgttgtccacagagcctacaggaagattctggaagcaatgttctaaagaaatgcaaggtctgtggcagggccgacagtatggagcccagacttcagtccaaaagggcccaaccaagacaaaaaacaagccaaagggtgaggggttcaagagtagctgatccatgagaagcaactattgaggtgatggacctggatggattcctgacctgggactcacgcacttcctatgattgtaggaggatcccacattgcaatgagcccaagagaacagtcagcctaggcagaacgaccactgggggatggacattaagaaaagtcgccaagaaaaaaggaccaaagttgagataatgaatgtgttgaataggagttatgaatgaaaataaaaattagaaagcaaacagggaatgcagtggttgggggaacagaaggtgaggtgggcgggacagttcagggctaatcaaaagggtagacagtgaacttggtgcctgtttgtgcagtttctggcctgtagcttgggggaaatgcttggaggcttggcaaaagtatagcagtcaggattgtacagatcaaagtgtcacctaaaacaatactgttcatttgtttccctggcgtctatcaaagtacctcgcacacagcttcgccatgactcctgatgctaactagccatttaggccaaacttcacaggttaagagcacagccgttcacaagactggccttacttcagacaccagcgacaggctcaggggttccgtgaacatatggtaacacatttgggggttctcactaccccttctggtttgataatttgctcaaatgactcacagaactcaggaagtgctatgcttagaattacagctttattatagcaaaaaggatacgaatcagaataagccacaagaagagatcacagggcaaggtctggaaggattccagctctggtgttctctctcctcccacagagtgttgtctaccagggaagctcacccaagcttcagtgttccaaatttttattggggtttcatcatgtagatgtgattgatcaaatcattggccataaggttgaactcaatctttggtcctcctctcttccctggaggtagggctgatgtcacttggctcaaagccccaaccctctatcacatggctggtctttcttgcatggccaacccccatcctgagttatcttgttaacatacactatcaagggattctgagaggtctgccatgaataactcaagaaatcccaagaattcacaggctacatcccaagaaccagggacaaaggccagccaaactttattatacagttgtctactgtgtatataagatttacattacacaaatgcatattataaacagaaaatactcaaaaaatgtttgtaaaatgaattagtgagtgagagaaggaaggagtgagaaagaatgaatgagaacttaactttaggagtctaactcattggccccacaccatccaatataaattaggacttatttgaaacaacactggcagccacagaaataatactgaatggcttggctttgataagaaattactcacttttccagtggtttttgagttagccatgttttgtcttcttgggaggggagacacagactcttgtccttcatggtgttagtatttaagcccagggtttctgtagagcaattaagttgactcaatgcatttcccagcataaatggtatattctattattttctcctgtctgctccttccctcggggagccaggcgacattaggtagcactgctgggattgtggaattttgttcttgtggggccctaacttcagagggcctggttcaacaatgggtacttttttaaggacttctggactgcgttcttccctgtgccagtgtgttcagtggtgcagactgtctttataaagccctaaggcattgtggcatgacttcctctcttatgcaatggtgtgtgtactctggcccagctaccaagtgttacttccgtgtatttttacaggactcctgagaatcgttccaagtgagttcacgggaggctctgtgtgaatcagtaaggcacattaatattgttaaacgggctacgaggtaatttgcctcccattgtctggcaatttcttttattatttggagatgctctaagccagtcttggctgggaattgcagagttcaattttatgtccagaggcttggtccccaggttcctggcctgggagataatggtaagtgattcatggattcttgaatctgacaaataaatgagcctaggccccttattttacaaatatagcagtaaaaatatcaacaacactaccaccaaccaccccaatttccggtttttattgtgtacttcatatcgacccagcactgtgctgtatcttcattctctcattaaatcttcacagtaactcttcaaggagggcaatgatttaacagatgaggaacctgaggcgcagagaggttaagtaacttactcaaggtcacccagcaaagaagtggcagagctgagagtggaaaaaagccaattccaactacctttaacattgacagcacttccagagaggcacacagattgcttaagatcacccaaggccacagaaagactcagtgatgcaagcaagtgttaaatccagaactcttggctctttcttaagcttcctttgctttaaccatgtagccttttattcagttgtttgcagtttaggctgtagttagtactagccgtaacatcaatgcttctggagcaactcataacaattttgatcagactcatcatctcataccaattgcaggagcttcctaacaggcctagcatcctctagtctaatccctgaaatgtccttcacactgcacctatgaagaacattcttaaccacaaattagagctatcaattccgtgctaaaaccctccaatggctccccagtgcccatggaattttgtgtagactcctgaggctggcaggcaaagccaggtacaggcagcctccaaccttctactgggccacctttcaacccactgcgtcttttatacctcctgtgtggcaacctgtggtctccggtttctgcaccttcaagaattctgttaactctgcctgtcgtcctgtaactgagcccactccgtctgcccttcttgcttgcttgacttggattccacagcctttcttggcttcctattgtcatggcatttttattccatgttataattgtatgtttacttgactactgtctccactagatcttgaactccttgaaggcaagaaacagcagaatttgtatctagaagaaaggatgggaagctgggcccctggtagtgaggaagcagacctgtaaagtcagatagaaagatacaagaatgtgcctcgtggctgttggctgaatgaaaaagtaaaacaaggaatcccaagtaagataggaatgagtgagatgtcccaaagcaggcctagaggttacctaccacagtgatcttaaagcaaatttttattgcagattgttttcttcaaacaggatcgagttctcccaacacataaaaggaaagctctaggtaaaggtttatatctccaagccttcatgacttggcctaaatctctcctccttcttgaagcctcaggtcacagtgcaattgtgatggcatgggctctgtagttacgttgattgtgtcagcagggcaaacttgctgctgtaataaacaagccctgtatctcagtggcttaacacagtgaaaattcccatttatatcacctcatttgaaggagatgagcaggaacactctgctccatgaagccattcagggacccaggttccttaagtgaagtggttccaccattctctaggactttggagtcctctgctagatcctctgtggctggccagctgacaggagcaagcgtggagcaggcaaacacattctcagcgtcttggtggaggtcacacatgtcccttgtacttacactccttgcttgagaagtagtcatatggccccacctagatgcaaggaactgggtaaggtggcctggcagtatgtccaggaagaggagagcactgtgaggtctagcaggccctgcagttctaccatctttggcatggctgtgggatgtgtttctccactccagacttctctgttgtgaatgaaacttctcaggatggctacaagggttgaatgagatgagatatccaaatgtctgatacatacttagcagtcaaccaatcttcattccatgtctcctcttctcccctgtagtcgtctgtctcagctactcgggaggctgaagtaccaggacctcctgaccccaggggatcaaatctgcagtgagctgtgatcatgccactgcactccagccttcaatctctaagtaatggaggagtcataaagaagtgaggatgcagaaaaagatcagatcaaaggatgtgttggttgttatgccccaagcagctgccagtttccttttcatcattatgagagtaaaagttgatttgggctgaagtttcagcttgaagagcaactctcattggctttatttgagacgggtcattccatcacttgacagagtcaattgtgcatctgttctttcaattgcactgaaa

SEQ ID NO: 10384 - RNA, 187 nt, Homo sapiens
  source 1..187: mol_type = other RNA
ccccacctcctctctcctcagccgctcgggtcctccgctccactcgcagttaccgggtgctgtccctgcagtctgggaggggaggccaggcaccgcggcaggggcgctcgcggcctggggaggggctgggggcgccctggcaagcctggccgaggctcctctgcggatgaagctggacggggtgagc

SEQ ID NO: 10385 - RNA, 105 nt, Homo sapiens
  source 1..105: mol_type = other RNA
ccccacctcctctctcctcaggcaggcggcggcaccgactcagtctctttgccaccctccctctctctccccgagccctgaagccacagagcccggccgctgccc

SEQ ID NO: 10386 - RNA, 992 nt, Homo sapiens
  source 1..992: mol_type = other RNA
ccccacctcctctctcctcagggacatcactcttctggaagtgaggcatgtgccagagggtgtccagcttcacgggcggcttgtacttcctcagctgactgctccgggtctcatacagcttcccaaggaccaccttctgcttcttctccagtttgatggctttctgggtggccttttgttcctgtacccacagctgcaggtaccggtgctgcagcagatcaaagaagggtgtggaaggccgtgcccggatcccaaatgtcatgtttggagggagagggggcggctctttcttcatgcgccggtcatcctggtcactgatgcggatgtcattgagctgacggtagagcaagttctcccgggcagtcaccaggccggctttcaccgccccgcggttcattgcgatataattccgggtcagctcgtgggggcaggtgggctgctgcttgaacacgttccagcgtccgatggcttcagggactcctccgtcaagccctcggatgtagagtccataattaaaattaatgccgggcagactgtagcttctttcccggggcttgccgagttcagccttgacgatgagagggttctgaaacatggagtcccgcacgacccccagccgctcgttctccatgccggaacggatgtccgccacggtcaggggccgccgcgggggcgggcagacctggctgaccgtgcggcgcacaggctgctgctgcttcctccatcgcgtgaggtccgggccggagctcctggcctctggcatccttgaggtcgccggggagccggcccgcgggctggtttgggcgcgcttccccacgtcgggcacagcctggagctccgaagggcctgccgggcggcccgggccgcaccaccgggatcctgagggggaaactcagatgccaggacccctccggagccaggcgcgccccgctcgcgccggcccctcatcgcaaagagccccggagcaatgcaggagccccgcgggatcctca

SEQ ID NO: 10387 - RNA, 776 nt, Homo sapiens
  source 1..776: mol_type = other RNA
ccccagggcgacgcggcgggcagcgcggggcccaggccgccactgccccgcccggccgcccccgccgcggccgccgtgtccagcgccggcgagttgaggcagaaataggacgcgaagcccgagccgccgcggcccacgccctgcgaggtctcccagatctgcatccacagggcattggccggccccttctgctcgggctggatccaggccacgcgcggatccatccacgcgccgcccccgcggggcccgcgcgcccgcccgccccgacgcggccccgcccccgccgcgccccgaggcccggccgcgcgcgcacggacggacggacgggcctgggccggtggcggcggcggcggcggcggcggcgggcgggccgagccccggcctcctgctctagccgcgctcccgtcgggctccggcgtggggcggcggcggcggtgatgggccccggcaggccgcggcgggcggctccggcgcttggcgcgtcccagcgggcggctgcggtctccgggctcccgcttcacgcggcgcggggcgggcgcgggggccgcggcggcggcggcgttccactcgggccgcggggagaggccatcggagaagggcgggcggcggggccgagggggcgggcccaggcgccgagcggctgaaggacccgcgggaggcgccgccgcccgtgcggctagccctcagtcacgctcgcgccgctggctcggcgctcctgcggcggcggcggcggcggcggtgaaaagacactctcggcggcgacagcgcgggggaag

SEQ ID NO: 10388 - RNA, 283 nt, Homo sapiens
  source 1..283: mol_type = other RNA
ccccgccaccgccttggcgtgttccccatacagttccatgggctcgaagcgctggtggttgaggaattccaggaagtcgaaggggtagctctggaagtgcaccccgtcctcgcccccgatgccgctgctcccgccacccccggcgccgctgcccgctgggttcgcctccatctccggcgggtgggagacgggagacccggcgccggggtctccgccgggaggaggccgaggaggcggaggaggcgccgccgctccggggagacccgagggcccgaccggaagt

SEQ ID NO: 10389 - RNA, 38 nt, Homo sapiens
  source 1..38: mol_type = other RNA
cccctgggccggccttggctcggaggggctcaggaaga

SEQ ID NO: 10390 - RNA, 7592 nt, Homo sapiens
  source 1..7592: mol_type = other RNA
cccgcaggtgagatgagggctactgaatggactctcagatttcatcaacatagttaaccagaagcaagtttatttaagagatcagttcagcacaggctactgtagaatgtcttaccccaccatattgtaatggtatgcacaaaaggcctaaaatcagagctatatatctaggaacaagacagatatgttggatgctgttgtacatgcaccaataatattttaaaacaagacaaactattccagtgaccataattgcctaccatagactccagagaagatcagcattttagaattagaaacacacttgaatagatggaaaagaaacaagctgttctacctgtgacaagagcaccagtattgagtgatgaggacaaaaagaggaagaatatattcaaggaaatgtttagcacttttgttcaaagctagaacccactgttggaagagcagcgtatgggctggtgtcttgtcagttgttaagcagtttgtttgcattttgaaatgcttactgcagttgaggattccaagattgcttgaagattgatttgactccggtcaaatcaagacttgaccagcaacatccctaaaggtctcttttccttcactttctggggataattaattgctggtcatcctcttgagcctttcacacctcgtttagtggctatagtgcccccaagacctgaggctgtccaccaacagctataccctgaagcatggctgcagaacactgcagggaaggcagccccatgcaggccatgtgtggatgcaggtggataggaggacaagaaattaggctaaaaaatctgagtttagcaaaaaagtatgtaacattgcttcagcacttgtagatgagtaaggatggctcataaattaggtcataatagtgttccagtagcagctataagaaaggcattaaacaaccctcatttgtgacattctagggcagcccatggatgagttaaaataattcaaatcctggctgggcgcagtggctcaggcctgtaatcccagcattttgggaggccgaggcgagtgaattgcttgagcccagaggttcgagatcagcctgggcaacgtgatgaaaccccatctctacaaaaaaaaaacaaaatttggctgggcttggtgatgtgtgcctatagtcccagctacttgggaggctgaggtgggaggatcacctgagcctggggaggtagaggctgcagtgagccgtgattgtgccactgcactccagcctgagatcctgtctcaaaaaataataactcaaatcctactaacaaatgttaccagactttgacattaaatttttaaaatgtattaatttttaatatgaactaaaggaaaatagtattttgtttagagttccttaaatgtgtgaatacctaaggctttcccattgtgctatgcagcatatttaaaggttccagaaagtgtttaaggccaagaaccaaaattacaggcctaataaagtatttcttctcagatgctaaacagttctctacctttcaaacttaagcctttgtcttaccctttaaagtgtaagggctttgtaggtccacaaagttggtaaatttgttccagttctctcctgtcactatctttggaaataatttaaaatgtacacagtcttgaaatcttgatataacattttacaaaatcacccaaaagctgctaattaggcaacctgtttaagcagctaccaaaaatgaaaggcaagaaatgaaaggaggacaaattattggtttaaagctatgatagtcttttgaaacgatgagtaagttctctgagtcatggcagcatgatttaaggttgaatttagaatcaatgaaggaggagtcgatccactttccagtctggtcttccatcagcattgtcctttttaagaaataaggtggctggaaggacctccagaagattcttcttccttctttgttcaggtatataggaccatggcttcccacacttgtgtaaacttctctttgctgacagtgttgaggataatgtgattttgatcatactgtgtgccccctttaatgtctaaaactaaatttggcttcaacttgctgtaaatcctgccatcggacttcaagctccagaactggctgtcagcattctggtccagggccaggcctagcttggagccagatgttaccaggctgcccacaatcgtcaggcagcagtcttctgctatcctgcatttgatacatccttcttgatagatccaaatctgatcatcggccccgacatcctccatgacctgtatcctcagaagcttcagatcctctaagtttccattggttgacatgaataaccctgttgctttgtttcgaagtctgaaataaattcgcttctgaacaaaaggtcgtagagaacctatttggcgacagccactgaattcataccaattaggtacttctgcaggtgacaataggaactgtcgccctctgtaactgccatattcataagtaacccatatgccaccaataacctgaacagagcgtatttgtgtgttgaatcccagggatcggagattgacagtttctgcattaagttcaatcttttttcctttgaagtcttctctttcaaagagaataattgttggttcagaaaattcaacatctataaaacgaagagacttgaaagttgctccaggcgggcatcccattgcagacagacaaggataatggccttcttccaacacgtattgattaccagtgaaattttctccatcatatacaacccagctgcctcctgaaactctgcaagacttggtagaaaatgaatcatcaatttgacttgttgtttcttcaaaactttgactgtgaccttgaaactgtggttctgaaaacaagtgaatctgatttcgtctccttgggccagtgaaagaatccaaacatataggttgaacagaagagatcttacaatttttgcctccccagtcctcaaaactggtataaaatcctttatccagtatatactgttctcctgtgaagtcaggattttcataggctacccatactccactcagtacattaatagactgtgtcttcactccatatccagtctcctttaaattagcaacaattcccaatacatcaatactggaacctttggatccaaagtttttttcactgtacattatcatgtgagcatttgaaaaatcacctaatataggtcgtaaagactgaagctctccattgtaacctccccaggctttccagtccctgtattctccttcttctagcaaatactgatgaccggtaaatccaggtttctcatatgcaacccaaatgcctcttagaactttcatagaccccactgacgtaaacggcaaatgatcgtctccagtcgcctcttctgtttcacctccctccatgacaaaactacacattcctgtttctagttccacacattttccttcaaagaaaggcttttcataaacaactacctttggatctgtagggaattcaactttacggccacccattttcagaggccgcatggatccaatgtacgcttcttctgtatcccagaaggacaagtcagggtattcaccaggttccaggatgaaaggaacaccctgaaatccaggttcttcataaatcagccacgtgccccaatgtactttcatggaacaagtcttctgcattacaccaaatccctgcatttcttcagtatcatcaaagtaggaacttaggattcctaacccttctggttcagtaaataagtcaatgtgactaactctgtaatcctgaaccacatgtctgatggaaccaatcaccactggcttatcagactctgcttcttcgtgcctttccaaaatgtcttctataccccagagaccagagagttccaattctccttcttctaaggggatggagtgcccttcaaaatttggttgctcatacaaaatccaacatcctctaacaacttttatgagtatcactggagagaggctccaagaactgcaatcctgaatgtcactgaaaacttcaatgcacttctcagagacgtcgggttcactatatatcactacctttccaggtcggggattgagtttattttggacacttcctctaagtgtcattgtgtctgataatgacattccagaaaaagaaatgcttgggtcataccggcttgatttgaaaagacccatgaagtcggtgtcactgtttgcacagtttggcaagtttgatttaataacactttcaatatgattagccttttccatatcatcattcttcagttttgacaattcagaaaatttagtttctggcaagtgtaggttgcttcgtgaatccagatcttctttggttttctctttttgcgggtatttttccatgtggcttggacttttcaaactggagtgtgatgtacttgacgagttgaaattgaagacctttaaggagttgtcgggcagaagatttgactgttctttgttcaaaccacagggcggggcaccctcagtcgtgggctgtgacactgaagactgagatagggaaccgttctgagaagtactgaaagccgtggtcatagtgttgactgatgtcacagaaggagaaaagattttgtcttgtggtaaagaagataacaagcttgagaaaagtgcacttttttctagtctcgatctcttaatgccaccatttgtgacgtccctgttctctttgtcattgatttccggcatcaccagaggctcactgttcccattagtgttggtgtgcagggacttgaagaggacgctctgttcagcagatgcacgtttgggtctcagtttggattttgtgtcaaggttctgcatcaaatgtaaagccggtgacatttctggctgactttccttcttcttccccaaaccaaaggtaaacactttgggatcaaacaccttttctaaatggtcttcgtgaataggaggcatggcaaagtgaggagcaggagagtttggcatcctggccttctttcttttcatgggcatacaaactgcgctatccatctgttttataatttcagtgaatttttccatatcagaagaagaatcaaatacactatcatcactaccagcagaaatgttcaaaaggctggcagggctatcctggccatttgtaacagtctgatctggcctttgaggagtggctaagtgatttccgctgctgggagagttggtgggactggattcagccatcaggggtgttctgctgccctgactttgagcctgaataggcagagttttctctgatgctggcggtatgacttgtgggccagattttgccgcgagctctgctgtgcaatgagagtgttcattgcccagtacttcctcttgtgggggagcacaacttgcaacggaaaccacttcaggttcattactgtgacaagttggcaactgcacttctctaacttcagagctctctgggatgacctgggagctcacatcctgggtgctctccacggggagcacgaaggacctgacctggacgaggactctggatggacactcacttcccacagcttctggactacgctctgtggacaaaggaggggttgtttctcctccaagttctaaaagtggcattttctcattgttctgacgagacacaggcaaaacacatcctttatggttttctgacacttttagatcagtgcatgggaaactgcttatgggtgattgaacacatgtgtctttgggaacatccccaggagcgggtgcagacagtgaaagagaaggcccaggagatgactcagcaggggactgtgagtcagaaaatgtatgctgtggctttggcatggccgttggaggtaaatctttggtatccacagtggtggggatgtcttgtgctgtatcggttacattttcaagtacaaggcttttgctgtctgcagcctctgagtcctccttctctaagagcttatgatccttgacaggaatcagagcagaagccactggttctgaaaggcagccagcatctgtttgtacatctgctttatcatcttggttaggctgaggaccaagagcttgattctcagaagagtctccattcattcctctggttgctggcagaatctcttcttccgagacggtaactttggtttctatagcagtttccttaaccagcacaccattctggggactgtttggcattactttcttttcaggttgctccatttctttggcttttttggctaaattcagctttgccctcccaacaaacgttttactagaggcaggagtattcctttggcctcgaatgtcagtgtgtcttgggctactgtttgtccgtttgttttcaaataaggagattttggtggcagtgttgcctttgtgaactggctggctaaatggattgtgctcatttcccaaactgtcaagattcttaggggttttaagatttagttccacatgtttgggcttggcagggagggtcactttagtggtcactgtcgacctgcccacgccgaaatggttcctgggcttcaagccgtcggcgtcagaagctccaggcgctccggccgctctgcccagctctctgcttcgacctccctctgcccggccgttgaagtggttggggagcgggcccctcttgtgctcgggcttgatctccggcagcagcgagctgctcttgaccgggagctcgcgggggatggcccgcgccgcctcctccccgctctcggccgcagtgcccttggtgactgggctgggatcgggcaccctcttgggtggggactccttggcgggagcccgggggccgctggcgggcggggcgggcacggcctcgagggcacggctcctgcccttcctcttcgtgggggacgaagccgggggtggctgtttgctccggtccgactcccctcggagctgccctttggtaccggggctgggcttggactctgggctcgcagcggaggcaacgcccccgtcgagggctgcccgcggagatttcactttcttttccgccgaggcgttatcgctggccgcgtttggcgccacctcgtcgtcgaacaccgcgtcgtccctggcagcgctctcagggagctcggcgtccgcgccgggggagtcggtggatttctgcgaccccctccgcctccccgacctacggccgctggacctcttctccatgtcgtcccagtcaccgcaatcttccgctctgggagtaatcacgaccggctcgtccacttgtgccccctcagtcttactcaagtagatgtccaaagttagcaccttagcagggtgggcgtgacccttggggcgggctgtgcagtctgcctgcgcggagctggccgtgtgcgctgcgccctcggccggaggctcacctggcaaatcagacgcgcccttggggggctggctgcgggcgttgcggggccccagggagccttcttcggcacacacactgggggctccgttaggggcctcgcctagtcctcccgcgggccgctcctgggtgggcgaccctggcgcacccctcacacccaggaaagcctcctgttcgtggccagcacctggtgaagcgtcctcccccggactgcgggcgggcgtctctgcgttctcttgcctggaggaatttcccggcgaggaatgcagctgcttggcagtggtggtggcatct

SEQ ID NO: 10391 - RNA, 8521 nt, Homo sapiens
  source 1..8521: mol_type = other RNA
cccgcaggtgagatgagggctactgaatggactctcagatttcatcaacatagttaaccagaagcaagtttatttaagagatcagttcagcacaggctactgtagaatgtcttaccccaccatattgtaatggtatgcacaaaaggcctaaaatcagagctatatatctaggaacaagacagatatgttggatgctgttgtacatgcaccaataatattttaaaacaagacaaactattccagtgaccataattgcctaccatagactccagagaagatcagcattttagaattagaaacacacttgaatagatggaaaagaaacaagctgttctacctgtgacaagagcaccagtattgagtgatgaggacaaaaagaggaagaatatattcaaggaaatgtttagcacttttgttcaaagctagaacccactgttggaagagcagcgtatgggctggtgtcttgtcagttgttaagcagtttgtttgcattttgaaatgcttactgcagttgaggattccaagattgcttgaagattgatttgactccggtcaaatcaagacttgaccagcaacatccctaaaggtctcttttccttcactttctggggataattaattgctggtcatcctcttgagcctttcacacctcgtttagtggctatagtgcccccaagacctgaggctgtccaccaacagctataccctgaagcatggctgcagaacactgcagggaaggcagccccatgcaggccatgtgtggatgcaggtggataggaggacaagaaattaggctaaaaaatctgagtttagcaaaaaagtatgtaacattgcttcagcacttgtagatgagtaaggatggctcataaattaggtcataatagtgttccagtagcagctataagaaaggcattaaacaaccctcatttgtgacattctagggcagcccatggatgagttaaaataattcaaatcctggctgggcgcagtggctcaggcctgtaatcccagcattttgggaggccgaggcgagtgaattgcttgagcccagaggttcgagatcagcctgggcaacgtgatgaaaccccatctctacaaaaaaaaaacaaaatttggctgggcttggtgatgtgtgcctatagtcccagctacttgggaggctgaggtgggaggatcacctgagcctggggaggtagaggctgcagtgagccgtgattgtgccactgcactccagcctgagatcctgtctcaaaaaataataactcaaatcctactaacaaatgttaccagactttgacattaaatttttaaaatgtattaatttttaatatgaactaaaggaaaatagtattttgtttagagttccttaaatgtgtgaatacctaaggctttcccattgtgctatgcagcatatttaaaggttccagaaagtgtttaaggccaagaaccaaaattacaggcctaataaagtatttcttctcagatgctaaacagttctctacctttcaaacttaagcctttgtcttaccctttaaagtgtaagggctttgtaggtccacaaagttggtaaatttgttccagttctctcctgtcactatctttggaaataatttaaaatgtacacagtcttgaaatcttgatataacattttacaaaatcacccaaaagctgctaattaggcaacctgtttaagcagctaccaaaaatgaaaggcaagaaatgaaaggaggacaaattattggtttaaagctatgatagtcttttgaaacgatgagtaagttctctgagtcatggcagcatgatttaaggttgaatttagaatcaatgaaggaggagtcgatccactttccagtctggtcttccatcagcattgtcctttttaagaaataaggtggctggaaggacctccagaagattcttcttccttctttgttcaggtatataggaccatggcttcccacacttgtgtaaacttctctttgctgacagtgttgaggataatgtgattttgatcatactgtgtgccccctttaatgtctaaaactaaatttggcttcaacttgctgtaaatcctgccatcggacttcaagctccagaactggctgtcagcattctggtccagggccaggcctagcttggagccagatgttaccaggctgcccacaatcgtcaggcagcagtcttctgctatcctgcatttgatacatccttcttgatagatccaaatctgatcatcggccccgacatcctccatgacctgtatcctcagaagcttcagatcctctaagtttccattggttgacatgaataaccctgttgctttgtttcgaagtctgaaataaattcgcttctgaacaaaaggtcgtagagaacctatttggcgacagccactgaattcataccaattaggtacttctgcaggtgacaataggaactgtcgccctctgtaactgccatattcataagtaacccatatgccaccaataacctgaacagagcgtatttgtgtgttgaatcccagggatcggagattgacagtttctgcattaagttcaatcttttttcctttgaagtcttctctttcaaagagaataattgttggttcagaaaattcaacatctataaaacgaagagacttgaaagttgctccaggcgggcatcccattgcagacagacaaggataatggccttcttccaacacgtattgattaccagtgaaattttctccatcatatacaacccagctgcctcctgaaactctgcaagacttggtagaaaatgaatcatcaatttgacttgttgtttcttcaaaactttgactgtgaccttgaaactgtggttctgaaaacaagtgaatctgatttcgtctccttgggccagtgaaagaatccaaacatataggttgaacagaagagatcttacaatttttgcctccccagtcctcaaaactggtataaaatcctttatccagtatatactgttctcctgtgaagtcaggattttcataggctacccatactccactcagtacattaatagactgtgtcttcactccatatccagtctcctttaaattagcaacaattcccaatacatcaatactggaacctttggatccaaagtttttttcactgtacattatcatgtgagcatttgaaaaatcacctaatataggtcgtaaagactgaagctctccattgtaacctccccaggctttccagtccctgtattctccttcttctagcaaatactgatgaccggtaaatccaggtttctcatatgcaacccaaatgcctcttagaactttcatagaccccactgacgtaaacggcaaatgatcgtctccagtcgcctcttctgtttcacctccctccatgacaaaactacacattcctgtttctagttccacacattttccttcaaagaaaggcttttcataaacaactacctttggatctgtagggaattcaactttacggccacccattttcagaggccgcatggatccaatgtacgcttcttctgtatcccagaaggacaagtcagggtattcaccaggttccaggatgaaaggaacaccctgaaatccaggttcttcataaatcagccacgtgccccaatgtactttcatggaacaagtcttctgcattacaccaaatccctgcatttcttcagtatcatcaaagtaggaacttaggattcctaacccttctggttcagtaaataagtcaatgtgactaactctgtaatcctgaaccacatgtctgatggaaccaatcaccactggcttatcagactctgcttcttcgtgcctttccaaaatgtcttctataccccagagaccagagagttccaattctccttcttctaaggggatggagtgcccttcaaaatttggttgctcatacaaaatccaacatcctctaacaacttttatgagtatcactggagagaggctccaagaactgcaatcctgaatgtcactgaaaacttcaatgcacttctcagagacgtcgggttcactatatatcactacctttccaggtcggggattgagtttattttggacacttcctctaagtgtcattgtgtctgataatgacattccagaaaaagaaatgcttgggtcataccggcttgatttgaaaagacccatgaagtcggtgtcactgtttgcacagtttggcaagtttgatttaataacactttcaatatgattagccttttccatatcatcattcttcagttttgacaattcagaaaatttagtttctggcaagtgtaggttgcttcgtgaatccagatcttctttggttttctctttttgcgggtatttttccatgtggcttggacttttcaaactggagtgtgatgtacttgacgagttgaaattgaagacctttaaggagttgtcgggcagaagatttgactgttctttgttcaaaccacagggcggggcaccctcagtcgtgggctgtgacactgaagactgagatagggaaccgttctgagaagtactgaaagccgtggtcatagtgttgactgatgtcacagaaggagaaaagattttgtcttgtggtaaagaagataacaagcttgagaaaagtgcacttttttctagtctcgatctcttaatgccaccatttgtgacgtccctgttctctttgtcattgatttccggcatcaccagaggctcactgttcccattagtgttggtgtgcagggacttgaagaggacgctctgttcagcagatgcacgtttgggtctcagtttggattttgtgtcaaggttctgcatcaaatgtaaagccggtgacatttctggctgactttccttcttcttccccaaaccaaaggtaaacactttgggatcaaacaccttttctaaatggtcttcgtgaataggaggcatggcaaagtgaggagcaggagagtttggcatcctggccttctttcttttcatgggcatacaaactgcgctatccatctgttttataatttcagtgaatttttccatatcagaagaagaatcaaatacactatcatcactaccagcagaaatgttcaaaaggctggcagggctatcctggccatttgtaacagtctgatctggcctttgaggagtggctaagtgatttccgctgctgggagagttggtgggactggattcagccatcaggggtgttctgctgccctgactttgagcctgaataggcagagttttctctgatgctggcggtatgacttgtgggccagattttgccgcgagctctgctgtgcaatgagagtgttcattgcccagtacttcctcttgtgggggagcacaacttgcaacggaaaccacttcaggttcattactgtgacaagttggcaactgcacttctctaacttcagagctctctgggatgacctgggagctcacatcctgggtgctctccacggggagcacgaaggacctgacctggacgaggactctggatggacactcacttcccacagcttctggactacgctctgtggacaaaggaggggttgtttctcctccaagttctaaaagtggcattttctcattgttctgacgagacacaggcaaaacacatcctttatggttttctgacacttttagatcagtgcatgggaaactgcttatgggtgattgaacacatgtgtctttgggaacatccccaggagcgggtgcagacagtgaaagagaaggcccaggagatgactcagcaggggactgtgagtcagaaaatgtatgctgtggctttggcatggccgttggaggtaaatctttggtatccacagtggtggggatgtcttgtgctgtatcggttacattttcaagtacaaggcttttgctgtctgcagcctctgagtcctccttctctaagagcttatgatccttgacaggaatcagagcagaagccactggttctgaaaggcagccagcatctgtttgtacatctgctttatcatcttggttaggctgaggaccaagagcttgattctcagaagagtctccattcattcctctggttgctggcagaatctcttcttccgagacggtaactttggtttctatagcagtttccttaaccagcacaccattctggggactgtttggcattactttcttttcaggttgctccatttctttggcttttttggctaaattcagctttgccctcccaacaaacgttttactagaggcaggagtattcctttggcctcgaatgtcagtgtgtcttgggctactgtttgtccgtttgttttcaaataaggagattttggtggcagtgttgcctttgtgaactggctggctaaatggattgtgctcatttcccaaactgtcaagattcttaggggttttaagatttagttccacatgtttgggcttggcagggagggtcactttagtggtcactgtcgacctgcccacgccgaaatggttcctgggcttcaagccgtcggcgtcagaagctccaggcgctccggccgctctgcccagctctctgcttcgacctccctctgcccggccgttgaagtggttggggagcgggcccctcttgtgctcgggcttgatctccggcagcagcgagctgctcttgaccgggagctcgcgggggatggcccgcgccgcctcctccccgctctcggccgcagtgcccttggtgactgggctgggatcgggcaccctcttgggtggggactccttggcgggagcccgggggccgctggcgggcggggcgggcacggcctcgagggcacggctcctgcccttcctcttcgtgggggacgaagccgggggtggctgtttgctccggtccgactcccctcggagctgccctttggtaccggggctgggcttggactctgggctcgcagcggaggcaacgcccccgtcgagggctgcccgcggagatttcactttcttttccgccgaggcgttatcgctggccgcgtttggcgccacctcgtcgtcgaacaccgcgtcgtccctggcagcgctctcagggagctcggcgtccgcgccgggggagtcggtggatttctgcgaccccctccgcctccccgacctacggccgctggacctcttctccatgtcgtcccagtcaccgcaatcttccgctctgggagtaatcacgaccggctcgtccacttgtgccccctcagtcttactcaagtagatgtccaaagttagcaccttagcagggtgggcgtgacccttggggcgggctgtgcagtctgcctgcgcggagctggccgtgtgcgctgcgccctcggccggaggctcacctggcaaatcagacgcgcccttggggggctggctgcgggcgttgcggggccccagggagccttcttcggcacacacactgggggctccgttaggggcctcgcctagtcctcccgcgggccgctcctgggtgggcgaccctggcgcacccctcacacccaggaaagcctcctgttcgtggccagcacctggtgaagcgtcctcccccggactgcgggcgggcgtctctgcgttctcttgcctggaggaatttcccggcgaggaatgcagctgcttggcagtggtggtggcatctgggaaaggctctccctctgcctccagaggttctaattggggtgaatcattttcatggcactgctgcacagccacagccgctgcactgctgctccagcgaggtgacagctcggcgtcagggggggctgcggggccaccgctctcggggagctcgccctctgcctctcggggattctcccgcggggagccctcctcgcttgtgtccgtttgcttcagttggctgctctgagatctgctcctctcactctctctctctgggagcttaggagaggctaccacatctttgggagagagtggtttggcatttgatctggtgggactctctaacccgtttctactgtttcttctccttcctgcagtgaatagagtgccaagtttccccaaaactggcttccttctgttgtcttctggaggttgtgctctggactttttaaatattccagactctagaagtaaggaaccaagcgcctcactggtggtgtggaagaactgggattccccacagtgcagtggaaattcctgggagtctcgaaccacatattttccatcgactacatccaaagctctggcctctccggcaggcgccgggagcgggtgcggaacgaacaccccacagtcaggcggcgccggctgctgcttctttttggagcgccagaggtggaaggtggtgtgcttcttagggggcctgcacgggctgggctccccggggtcgccctgggctggcggggacagcggcatcgtcttgtcctcctcccgctccgactgccgggacgcggtcctctctgccgcccgggccctatggaagaacacacctgagcgccagctcgcccgcctttctcagcgcgccgtgggaccccgccccctcgtcgcggatgcggggggacggccgcgggttgcagaaccagcacccagcgcagcgcgagcagcact

SEQ ID NO: 10392 - RNA, 171 nt, Homo sapiens
  source 1..171: mol_type = other RNA
ccctctctggctcctccccaaaccctttcccttggcctctggaatgtgtttttcttgtcacatttgcatatgggtgtgtaggtctggctggagtttctggacatttaaacaaacagtgagaagtcacacactggaatcctgactcaggagcctctgggaagctgccagctt

SEQ ID NO: 10393 - RNA, 2034 nt, Homo sapiens
  source 1..2034: mol_type = other RNA
ccctctctggctcctccccaaatgtccccagctcatcctttcagagtcctaggagctgggcagacccaggggagactccacattcaatcccagctcaccacttcctcaatccatgcccttggggaaatcacagaactttgtgtgccaggtttctcctctgtaaaacggagtgggaggaataatgtatccacctcccagggcttacctgaggatagaaaatgggcacctagtgttctggggcactaggaagggaacttggagaccttttgggcagggcccacacggcaggcactctgagtggggaccctgatgccagggagtggggcctgggcacagagggcaggatggtatggtaactgggaggggaggtggaaacatgggcccagggaggatcagagttggaaatggagaaacagagtggtttggtcgtggggagatactgcctggagggagttgcagtataggggaggtcctcccctgaaggtgaaggtggggagaaaacctggtcaaatcaccctgagtatgagcaatgaagccacctggccctgacaggctggagaaaagatctctgacaccccctgcccacagcatggtcatcgttttatacctgagtcgaaagtaccagatacggggacactggtacccacctgagctgcaagcccgcacctgcgtggatgagtacttggcgtggaagcatgtcaccatccagctgcctgccaccaatgtctacctgtgcaaggtgagcttcctaggccctgtcatgcaggctggggcaggggcctggacccccagagatggaaggcaccagttggtacatattacatattagcttcacttccactgtcctcagcagacataactaatctatcacagtactccttcccctaagcctgaatgaatccttagaaaccttctgaacacagagccccagaggacatcactaatgagtggcagccgggaagggatggagaggaggcccaagaggcttccaagagtctgggttaagttgctcctctcctcccagcccagtctctcctgccccacttctccggacagcctgcagatgctgcacagctggagcggctgttggggaggctgatgccagccctgcagcacctggattggggggtgctggtggccaggcccttcctggcaatggagcagatctccctggaagacttggtgctgacggaggtgatgcaggtgaagctttcctacccacctgccctctggggggactctgggcatggggctgagccccaaccccagctgccctgtcttcccagcccactgccgttggctgcgacctcttccaagactgccccggctggcagtgtggcaggcccgtgtggcggctgcccttggtactgagctcttgctggaggcccacaagctcatactccagcctctgaaccacagtgaggcttggcgggacccccagctggcccagaagcaggtgcagtgggtgcagcccactccactgcaccctgctgtctgcaataaacacactgcatgctcttcgcttgtctccaggcttactctgtcaccagaagtggggtcagtcccatttctcagcctagacctattagatcacagcatagagtgagtggcactcagtcctctacgtggggctctagttaccttccttggccaccaggtacacagtctggccactgcagccccaaccaaggccaggaagtttctaggctcctctgtgtggcacacaccggctgagtgccccctgacttcctggtggtggtgtccccattgctcccaaagctcacagtttcctgtgtctctttctcccagttcctttctagtcatagttcaggctcgattcacctgtgtctctttctcccaattcctttctagtcatagttcaggctcgatttacctgtggatactcccagcctctacttctagaatcctccagggataattctcattgcctcctcttcattctggaccctgcaaagcccctttcgtcaggttctttgccacgggcctctccccagcctactcctgggcctcctt

SEQ ID NO: 10394 - RNA, 1521 nt, Homo sapiens
  source 1..1521: mol_type = other RNA
cccttccctcactcttctctcagcatttctattacctaaaagtgaggtgcaacatgatatctgtggccaactggcaattcagacattcccctgacggagagttggcaatactctacctagaagcataaacactggctgaactgtagctaatgggggatgtgaaagaagtaggagcttcactctgctagagatgtgttcatttgcaattaacatagggtgacggtgatcctttcagaatttctggcttggaggttcacaatttagacttggaccttgctcctacccatagttgaaaaccctggtgatgtatgttatataatttcccctactaccagaaattcatccaaattgagtttttccctaaactgcatctctctaaattctcatcccagaggaagcaaaaattacatattatggcaactaaattttctacctaataattataagtaatcttttaaagccaaaatattaagccttttatcccaacttggatgggctctttcctttactctcgccggttttttctttactgtctctttaagatttctctctctatttatactttttttttaactacttcatcaaccttttcccccaatgacctttaattcttaagcatcttgtccttccccattgtcccctccacaatttctctaatgtaatcaacaggaccagaaacttggctcaaccataaaatgtgacttctttacacagacacgcagcaaaaatggccagaggtgaaattcagagaggactgatacagaatatacctatgatttggaagtctttgttgttgtcattctaacatttctcaaaaacattctagaaacaacaacttaatgtgtgtttttgagaactgagtatttttttctcttgattgattgtcaatgttatataagcaggtacactaggaatcagagtaaccaagtgtgactttgcagtttgtgcccagcaaaatgtttctaaaaaataaaccatgatgcattgtctggttttgggtctttgtgtctgcagagctatgtcatcccagagggaataccttgttcttattcatataaaagtgcttaaacaggctagggtactcctgctgggatatataacaactaatgatgcattatgaacaactgcttactagatagcttcactttgctacctaataggcatctccaacaacatggctaaatcaccatgaaaatggtgctattttccacccatttgctcaagcaaagatcctaggagatatctttcatccttttcttttcctttctaatcacgtctaatccatcaaaagagctggcagttctaacttcaaaacatatttccaaactttcttcccttgatgtctattgctatctaattttagataccatatgtgtttcttatatgttcttatatgtaagaaaaaagactagggagtatcatatgttgcttcttgtcttttttctttcatataaaagcagaattcacccagcaggtagaattatattacaactcagctttcaaaaagcttaggaggcatct

SEQ ID NO: 10395 - RNA, 394 nt, Homo sapiens
  source 1..394: mol_type = other RNA
ccgcactgtgggtacttgctgctgcagctcagggatctcatcagaagctccctggtttggagatttgggtgcacaggctcctggtttttggctgcttggcaactcatagggaatggctggaggcggagatggtatatgatgagcgcacacctccacgccctgggatttctgcagactcggtcttgtccgtcccttggcggacttgggccttatcatgtgcatatttagtgagtttggctgccaaatgaggctgtcaactgctgtgctgacaacagtgctacactcaggtggtgctatattcacaggggcttctgtggccattgcttctcaagacccctagccgttccgctccatccgccgcctgcgcccgggctctgtcctgctggtaaacaac

SEQ ID NO: 10396 - RNA, 916 nt, Homo sapiens
  source 1..916: mol_type = other RNA
ccgcactgtgggtacttgctgctgcagctcagggatctcatcagaagctccctggtttggagatttgggtgcacaggctcctggtttttggctgcttggcaactcatagggaatggctggaggcggagatggtatatgatgagcgcacacctccacgccctgggatttctgcagactcggtcttgtccgtcccttggcggacttgggccttatcatgtgcatatttagtgagtttggctgccaaatgaggctgtcaactgctgtgctgacaacagtgctacactcaggtggtgctatattcacaggggcttctgtggccattgcttctcaagacccctcagattcacttcctgcagaatgatttgcacttcctgcaaattcactcctttcatcacaaaatcttgaacaatgtaatctgagcctctcagggtttgtattctaacctcaccattctgcacatgtaaccactgctgcctaattttaaggagtatctgcttcctctccactcagaccaggaccaaacgcaacacattatccctatatcttcctgatgtcctgctcaattcaaaatcttggacaaagctaccctcttttaaaggcctctatgtctgctgcattccactcacagcctgagtctctctccactcccattttccacttctccctcgtctttcacacccagtctggctgctagtagctcaggagccttctccttagcaaacttttggcatcaaaaaagactgcccatctccttgttaatttcatctattttctgatcaactgtgaagaatgtgtttttccccctttagtctccttctcaagtctttctctggcaattagcagctctgcactttcactcaggatggcaggagaaggtcataactgtccaactgttctgccaaagataagctccaca

SEQ ID NO: 10397 - RNA, 719 nt, Homo sapiens
  source 1..719: mol_type = other RNA
ccgcactgtgggtacttgctgctgcagctcagggatctcatcagaagctccctggtttggagatttgggtgcacaggctcctggtttttggctgcttggcaactcatagggaatggctggaggcggagatggtatatgatgagcgcacacctccacgccctgggatttctgcagactcggtcttgtccgtcccttggcggacttgggccttatcatgtgcatatttagtgagtttggctgccaaatgaggctgtcaactgctgtgctgacaacagtgctacactcaggtggtgctatattcacaggggcttctgtggccattgcttctcaagacccctgcgtgttcccccatggcccttatctgtgctgtccgttgcactggtcgtggggactgcaggcatggcctctgacgtcaaagcttgagtatcaatcctggctccaccacttgccagctgaagacgttaggtaaatgatttaccttcgctggatgtcagtttccgcatctctagaatggtgatgataagcacaggattgttgtgcggctgaaatgaggtaacacacgtgccaagtgcttagtgagggctactaactcttgttgcatcatcttcacttacagtgtacatctccttcagtaggttatgagctccttgaaggcaggaacttgcctgtctcggaatcccctgccttgtccacacaatgcttactttgtgatacgtgct

SEQ ID NO: 10398 - RNA, 230 nt, Homo sapiens
  source 1..230: mol_type = other RNA
ccgccttctctcctcccccagaggtggtgggtgggcttgaaagatccaatcttctaatcacttggttggttcccaaggcaactggcccccatactgaggctgtccagaagcccccagccaccagtcatttcattggcacacaagacacttttgtcgctccagagaggccaagggtctttcttggtatgtgccaggaaccggggacagaaaccaaatatacatttcttatt

SEQ ID NO: 10399 - RNA, 6518 nt, Homo sapiens
  source 1..6518: mol_type = other RNA
ccgccttctctcctcccccagctcttagtttgagtcctgtatccccaagccacctcgagaatttggaccatccagacaatggctcggctggactctttgaagagcaaggtttggagggaaaggcaatgtgtgtgggtgggaagagtgaggtcagaggctgccccactggcaaggttaaggggaacccctgcccccagccgaaggcacgatggcacctctaagttcttcacattgaccaaacatggactgtccatgggaacagatgtaaaggccaaggtgctttgaggtgaggaccagcaccagaagatacacactgcacacaaatctccaattccaggcaagggatatagcagcacaaccaggacttctaaagattggcatccttctcctcttccctgcacagtctaccttcaccgttgcagcattcagatcttggtttatttgctttaaacctcagacagagccagacagtcctgatttcatactgacaacaaaaataaagagggcgcaagtgttctcatctcccctttggttcccagatctggtgccctttgacatattcagttttctcccaaatggaggcatctgagaggtctcctgacagccagggtaaactaggtgggtgctgggtcgcattcttcaactgtagattatcactgaatgttaatctggtaataatccagtgtttgttgatggaaaattgacaaacatttctcattttaaaaatccctgtttttcaaaggcctatgtatctttagccaatttggttaaactcttcttcttttatctggattttcttcaaactcttcaaaagaataatcactagtgttcttcttgaattctcttcctgctgacaaaatggccaattgatgatttgttcaagcacctgctatgctccaaaagtgttcagagctgtagggggtgctgtcaacatctcagagaggtacactgagggttccagcagagattcccggctcagcaggctttggtttgtctcccagctctgcctctgaaaagctgtggaatcttactcaagctctgggcctccaggtcctcatgcagaaaatgtgagtaagaagaatgcccacttcatagggttgcacgagaggagtctgcaggtaacctctctcctccttcaaaacaagcggaagctgacatccagagagaggagagcttgctgtgatttctcagggcacaaccagccctgttctcagcacctggaacatctggaacatctctgcttcatcttcctgcctccattttattattgggttaaaaaaataaaataagaagacgtaccttcactgtccttttaacaataggaggcctttgcttttctgggtaggaggtgtagtattgggctcaaatgatatgtttgtggttgtgtgtgtgttgtctcctcctggaacaatttatttcataccttgaagccttgtgctgggtttttttttttttgttataaatgatccccatttcataaggagcctcaagcaacaattagtcctgcatgtaatttctgaatcaaatggtgggtttgggtgagaaccgtgctgagcagtttggaagcagatgtagcccgaggtgaagtcactccctgtgtttgaagggaatccgggagggcatggagggaaggagggcaggtgcacagcctggtgtatggcccagggctctaaattgggagccctcaaagatgtgcctgactaattccctggaacctgttcatatgttaccttaacgtggcacaagggactttgtaggtgtgcttaaggttaaggaccataacatggtgagattaccctggattatctggtgatcacactctaatcacacgagtccttaaaaggggagaccctttcctgactgcagttagagagagatgtgaccacagaagagctgtccaagagaagcaacatagttggttttgaagatggaagaaggaagccatgagccaaggaatgcgggtggctgctagaagattgagaaggcaagggaatggtttttagccggcagcctctggaaggaacacagccctgctggcatcctgactagcccagtgagacccgggtctggctcttggaagatacgaaatgtatgttgtgttcagccactaagtcagtggtaatttgttacagccacgtaggaaatgaacacagcctggccccagctctgcctttgattagccctaacactttggccgtggcattgaactctctgtgagctttggtgccttaatcaataaaacggggacgtattcctgttttatcacccaaaacgctctaagcctcgccagcccatggggactggtaaagtcagtttaacaacaacatacaaacgtgtgccactgtcctggacctgagtcagtgggcacctggcaagcctcttccctctgtcccagaagacagaggacctacctcccaagcactctgaggaagtaagtcatttcctttctctttctgggtttcatttcttctcatttgtaacctgaaagtgttgaactagatgatttctaagattccttcaatcactaaagatatttcacatacaattgtatctttctttcattttctgaagacattttaggactttaccccaatgcagggccattgtggtaagtgtcagttttctctgtacaaggctgtcattgtagactatggactcttgagtgaatctaaactcagactgtggcagagccctgaatttgtcttaaaatgtgtaaataaatttttagtttgtaaaaaggtgaaataaaaatagctctacccacctttctgatgaacatccggagatggaaactattgcttgaacatgtacaattggtgccaggcatgaaagcgtagtggggtggggatgaagtgggaaaccaggaacgcagaggagtcatccttctccaacctcaacaagtggaaagttcacctgctcttccatttcctcaggttagtgtgaaaagacacacagaggtctatgtggacctattgtataaaagttgcatgcgactctttcttttccctcctttctgagtgtaggctcagccttccaggacgatgtcaccatgtcaagagaaaagtgaagaccagagaagaaacgtgactggttcaaaatcacatcttcttctctgatagccagtcattcatctaaatcatgaccattgtatcagtcagaatgggctaagctatgctatagtaacaaacagcccccaaacacagtgacttaaaataacatgatttatctctttgcccatcctccaagttcatcatggttggcagggggttctgttcatcgtaatcacggaggggcctagagtggcagagcagctatcatttcaaacaatatagtcactgtatcagagagaatgagagggctttggagggtctagtgctctggcccaaaagtgacacaggtcacgtctgcccacacgcattggtcagaactaaccacaaggctacacagggacaacaaaggaaatacaagcctagcatggatggcaaagagctgagaaattcggcaaacagcatacagcctatacattggtcctttgggccccaccacccttcacgctacctcctctacaaagcctttcctcatccccatagactgcattcttgaaagttctatttgtgatgttctcacctgggagatggggaaagaggaagcatgaattgtgttgttgaactgcaagagctataagcgggaagcatatgtcccaagtatgtgctgagctgcagaggccgcttgcttaactggtgtgccaggagctggctgtgtttagttagttctcaccaatgattgtgggcagaagtgacctgtgcactttcagtcctttggctttttgctttggagaaatagggtcccagcaggcatgggactgtggtccgggagaggtcactaataccgcatccagcatctgctgtaaccctcctgggactgaacccctcgaccagaagagcaccctgccttgggacccaggatggatgctgggatggcagactgtgcgagtttctacttccttctttgttatctatctctttcctttattaaaaatgtgtggtaataaaggctcaatttgattttctcatgtggatgggctaggaagtcttgggagaaactgtcccctctgcccttatttttttctggctaactcaggtgctacctgcaacagtttcaaccccacctccaaggtggaagagccatctcttgcctctgccttcccttctgagtcctggtatagatttctttcatgacatgcctcagtctccacttgtgttcagtaagttgcctgcatacttgcacttctccatgggctgagactatttcaaggacaggatgacatcctctaactctaccccagagggagcccagtgcctagcagaaactgttcccagcctggattctcacataatatttgttgactaaatattatcagtgtcagagtgggaaagtgtaaggcccagtgttgatagtttttaaaagccccctaggtgatttgaatgaggagccaggatgaagaaacactgtcatagtccaataccctcatttcaaatgagacaggagaatggggtgtgggggcagggaacctaaggctgatttgcactgacttcctggaactgaattgaaaggaaaaccccaactttccatgttcaagtaacaaaacgatcagaggctactccctttgcactccctgctttctatgtcatagatgaaaaaatggaaagtcctgttgcgggcctagtcttcatttgcatacaggtgaaactttgtaacttcacttcagtctctggtcccctcccacaatcaatcagacatttgcataggatgtaactttgtaatttcatttgcgttggatgtaacttcaccttccatgaccaatcagactggtcacgggccaccacttcatttacacagggtgtaaatcaagtagccaatgagaatcctctagagggtattaaaaccccagaaagttctgtaaccagcactcttgagccacttgctgaagcccgctcccactctgtagagtacactctgtggagtgtactttcctttgaataaatctgctttggtgcttcattctttcgtttgtgcattttgtccaattctttgttcaaaacaacaagaacctggacatcctccaccagtaacacaaagatggggaaacagactcaggatggggaacggacatttgccagggcttcacagctggggaataataaggtagttgcttaaacctcagcctgccttcacctctgctccctagtaactgtatatatgccacaattggaactccatttctgcacctctgacacctagcactgggcaagggtgctgaataaaataggtacgggataaattaatcctgcttccaaatctacacaacatttgatttaatttttatttaacaattataatgcaccaacactatataaatattttacaaatatcactgaatccttaaaactatcctttgtggtaattacaacttatttccctcattctatagttgaaaacatggaggcacagagaggttaagcaacttcaccagggtcacaaagctaccaagtggtggaatggggactcaaactcaggttagctaacccgagggtccaagtgcacaataactacactctgttgtgtcttgttgcaccagcggggagggccccttaccactgtgattccaacagctcaactcagtaactctgtgctcagcaggctcctgtagggcccatctttttgttgttgttgttgttgttgttgttgttgttgtagcaccttagactttgtgcccagtttccttttctgtcaaaacttacctgccctgtgccccacccacttccctcagggacttgttgtctacagaccagataacttccggagagctgggaggtgccaaaggtaatgattttcagtgttgacagttttacctcaggctggcccaaagcagataacacacctggggtagcagtgagtgggtggtataggcggcttagcatgtggcaatgcaaatgcacacagtctgtgtgtgcttatttggagcaacatcttctaggaatcaacttcaagatcagccggaaggtgccttgctccggcctgcaggcgccacaagatggcagcatttctgaacattccagatgggcccggggccgcgcatcagggtgtcggggggccttggccctgtgtcaggcgcacatcctcccttaggttaggaggattaagagtcccgaccccaggatgctctcgtcttcagccagagacagagagaagggatccagagcagaagggccgggtctgcctggtgcacattcagctgtttcaacaaaatcagtcttgaacccaagtgcctgttggccggtggccaggttggaagttgggctggattgtctttgtttatctgagaaatgaaggctttggggccagacgttgtgtgggggccaaggaactttgtggtgctttagaaagttcgtccctgccagcctcagtctgtgtgccccagaggacttcatcgatggggcatggccgggcaccaatgc

SEQ ID NO: 10400 - RNA, 2453 nt, Homo sapiens
  source 1..2453: mol_type = other RNA
ccgccttctctcctcccccaggtctgctataaagtcaaatgaaagagcacatgcaaatgttccttgccaactgggcagtgtgtgtgcagggaatgagcgagcttattgaccggtgggtgtcctgatttggaaggtgtcctcggaggtaaggcagatgaaggcctgcaaatcaatctgccaccgctggacatccaggctggtctggttggtgaggtcctgcagcctggctttccgcagtgggtatctcttggcagctggcatggggtcacttgccatggtggctcttgggaggggcttgtgattggtgatctggttggtgctgtatgccctccgtcgctgagagaggttcagatcgtgcttggtggtagagtctccgctggctagccgggcatttttggcctgccctaggatgaagggtgcccccgagttcttggcacagtctccaccttccagcccgggtccgtcatcctgagagtggtagaagacagagctgccagactcctgagagtgcagcatgctgtaccggcgcctcttgtcagatctgggattggagatgtgcaaagaagcatcacatacaatgccataccccaccagccgttctccagggaagagggagctggcgctgacgggtgagaccaggacctcagtggtctcagggaagatccactccacagtcacatcgctcaggactggggccatggccttcttcaaggatttgaccatcttgggttgcagccgctccccctccatcaggagctcagcactgccctcggacacagatgccagtcctttcaccagtctgtggcagacgttgggtccaattccaaagctatagcacctggtggagaaggcgtgatttcgcaccagctccagcaccttccctgtgttgttgacagcgccatctgtgatcacgaagaggagccgcgggtggcctcggtgcactggctgcctgatgacccacttgagaggggaaaggatgttggtcccacccatgtcggccttcattctctggatgtcatcacaagccatggccaagctgtcctcactgtaggtctggctggaaggaaaaaggctcttaaatgtggatccaaacccaatgatattgaagaggcaggctggcatgaggctcttaagggccaccaacatggcatccttgactcggtgcatgctgatcccgctcatgctgctgctcctgtcaatgaggaagatgaactccccgtgggcctttctcaggcacggctggactgactggaggtcgggacagaagttgagcatgatgacggagtggtggggaatgtctttgtggaggcgttttcgaatgatttctgtcttccgctctgctctgctcttcttcttcatccctttaatgaaatctgttcttcccttcaagtgctggtcaaactctcccagggtcatgtcccctttctctatcaggacatggggcatatggggctcgctggggtggatgaggatctccacaggccggtcaaaggtgtgcttgttggccaaggtgatgatgatgctcttggccgagcgggcagatggggcggcgtcggcacgaatctcatgagtgggactctccacccctgcgagcagacatggcccacggatctccagctggaagttgaactcatactccatggggttggacacttcggtgttcaggagagtcgccaggcacaacttattccaggagcccggggcccaggcaccgaagcagtgcctgtctttgccctgggcctgttggttggaggtgccagtgctcttggtgcagaactggggcacggttggggcacagacagcaggcagaaggaccctcacagccccgctgggcagcgttgggagctccgaggaggtgctgatgaagatggtgacattctccatgggggcaatggtccccaggttggccacgaacaggatccgctccaaatcctcgtccaaggtcacctttcccggtgtgcaggaatgaggggctatggaaaccccgtcttgcagaatgttccctgtgactgttggggatcgaacatgggaggcatcgaagtggccgctctccagcttggctttgtccttgatctgtactgtcacgacacggtcggcaatgactgcctcaaagccgatcaccgtggtgcactcatccagggggtacacgaagaggccctggaagggctgggcttccaggttgccataggtgagggaggcagttaggcccagggcataaccgctgacacaggaggtaacatcagacgcggtgaggggcagggctgcccccgtgatccaattcagcaagccgggcatcccgctggctactcagccttcagaacctggggctaggggcctttgcttcttttcttatctccagccccctctaggaagtcctgctttcatgtcccctttagaagcccgtgctctaagggccacccaatcaccaatagcaccaacactcttatcaaagt

SEQ ID NO: 10401 - RNA, 3778 nt, Homo sapiens
  source 1..3778: mol_type = other RNA
ccgccttctctcctcccccagtccaacagatttaattaagctgctaaagctttggaaaaacagaattatttgagctaagaggaaatgtgattgtcacattttctagttaacctgtcactcatttgatttggcaaaggcagtgctcctattacacattcagtcttaaaaccccatgtaccaggagggcacgagtcttagatttttgcctaggcaaaatcctgtcccttcactccttgggttttctgtagggaactagactacagttccctactgtagctgcaatgctagctattccaactacatttaattttaactatgctatggtcccaaaggtggatgtttggcatgtctcactccatcaacctaatttagggcagcctggagaagtgaccgatgtagtaaatgccaagtaggctaactaaaataatagatttcaactactgcctttgaatagaacttctcctttgcattttggccccagaatttaaaacaaatgttcaaggaaaagcaaatccttgactggataaaaacagtaaacacttagggacattcacctaaatttattgttggcttaaatgaccaagcgttccccacgtccgtttctaaagtggggtaggatgtttagaatgcattactcacacagaaagatgggattgatgaaatcacaaaactaaacacaggctatagcaactatgaacagccttcacagagaatgaacaatagcacaaatgccagactgcaacacttcctaaaatgatgtctatagctatctgtaaagagagaataaccggccaggtgcagtggctcatgcctgtaatcccagcactttaggaggccgaggtgggcagatcacctgaggtcaggagttcaagaccagcctgaccaacatggagaaatcctgtctctactaaaaaatatgaaattagccaggcatggtggcgcatgcctgtaatcacagctactcaggaggctaagacaggagaatcccttgaacccaggaggcggaggttgtggtgagtggagatacgccattgcactccagcctgggcaacaacagcgaaactccgtctcaaaaaaaaaagagagaataaccaactcctaagacatccattaagacagacgcacagtctgtcaactttggttagaataccaaaccttaagatcaggtaatgcttttgtgcataggctgtcacaactatattacatccacgttagcatccatgtgaaactaggtatcaggggcttgaccaaatgagatggtaacatccagggcctaaagacacctcttgttaactaatatggagaaaaaagagtgcctttccacactctcccacagaatggaggctccctaactaacactcaaatttggggttcagcaaatgaaactaaatatcaactgacaccacaatagcactagcctgccctagagtcaagactctgggtgggcagctcttcaataaagacagcaaggaggccatcctgaagaggtatatccacgtctaacaggttacaagaatactgccactagaatcctaaagagcagagtggtcactggggggtaaaaagaaaaaggaaaatccttgaagaaaggcaaaggagacaaccagtctcaagaccacaaggtattataagtcttctgtcaaagtaagatgtataagatttgtaaacactattgtgcaaaataagttcaataaggaatgaaaaaatcccccccacccacaaaaaaaaatcaaggcagctagtacctacagaagggagaggagaggatttactattttaatttgtcctttcaataggattcttctcctgctccatcctacttataatgtcctggattgccaactttaaaatactgacaggtattcagaggattcaaataaaaaagtaagaggggttgttaaaagtaacttatatccattcacaagttatctaacactggctcacagcctggtaaagaatctcttccttatggaagattgaacaatgatttctttgaggtaccagaaagtagactttgcctctgcagagaggtgggtcttttgcttgaacctgggtgttctggcttaatgctggctttcaggaggcagctaccttcaatttaaattaaaaaaacaaaaaaaaactataccaaccgaacgcttgcttaaacacagacacacacacacaaaatcaggagggacttcatacaaaaaaattcaagtcggcaatgggcatttccaaaaggtgacgagttttttaaataaaaattttgtgaaaaataaaatccaaaatcggcaaagcacaaaacagcaaaagaacatgaaatgctgctccaagcaggaccctggatagggaccttcattgctgatgggatgacacaaattaactgtacgagaagtctgggagacgctggaaccgatggtggcttcgcatgttcctgtcaacccactgagtcagactgtatctttgcagatgtttctgtcggcgggcgtagtttcgcgtggtgaggtccgaaggatgctgccattttgagtgctgcatatgatgaacttgatccatcaaggcacaaagctcccccgagatacccagcaattccacttctagggattcatccttcatttatcaacattttatcaaagctgtttccagtattttttggcttggttagtgtcctctgggtcttctatatgagcaatgacactcctgagataaagctgcttctgctgttctagatttgactgtgaaaacgtcggaacattagtcctggtcttagtttgtagaacaggaatgactttgcctagtcttctctcatggcctttcatcttcccagaatccttgttaagaacatctttgtttgatgaggtggaaacaaccagagatctcatttcacaacttgacttgtgtgaaccaccatttctgcaggataactccatattaggagtctctgaatggtctgagatccgagagaatacagacgtagggttctcactgtcaggcatatttttatcagagacagtctgttgaaagttattgtttgaagaagagagctggggcccattccaggcagagttattggggctgatcccttcagattcagtacaaagtttgctttcatttgggctaagaccatcttctctcatctcttctccaagggaagagagtttttcagtatctttggacgaatcagtctcgtccttatcaagcagagcatcacaaactgttggattaaatggtgcaacagttacttttataagattcttttctagtacagagcgtctgtttaatggtttagtatgagctggtccatgaccacttgatgtacttagctgaggtagtttgaagaggtcaggagtctcagctactggtcccaggctgtacgatgaatttttctctcggggagtatcaagtagaatttgactccctctttctcccttctcaacatgcccaccatcatcttccccagaagactgctcatatgatgggtcatcttccttcaacagtgcatcaatctcttcctctgtgtaatttacatcaccatcatcttcttctccctctgacagctccagcaaggagtcatccaatccatcctcatccaaggaatcccaagaaaatggggcaccgtctttaggcaagagagaggtaccagaagactgttcagagggcacccgtgagcacatcattttgtgtggagctgctggagcaatctctgcctttgccacgagaccaaatggaaaaaggtttcagttcctgctagctgttcctttcaggagacttgtcaaaatgattgactcccaccttc

SEQ ID NO: 10402 - RNA, 3735 nt, Homo sapiens
  source 1..3735: mol_type = other RNA
ccgccttctctcctcccccagtccaacagatttaattaagctgctaaagctttggaaaaacagaattatttgagctaagaggaaatgtgattgtcacattttctagttaacctgtcactcatttgatttggcaaaggcagtgctcctattacacattcagtcttaaaaccccatgtaccaggagggcacgagtcttagatttttgcctaggcaaaatcctgtcccttcactccttgggttttctgtagggaactagactacagttccctactgtagctgcaatgctagctattccaactacatttaattttaactatgctatggtcccaaaggtggatgtttggcatgtctcactccatcaacctaatttagggcagcctggagaagtgaccgatgtagtaaatgccaagtaggctaactaaaataatagatttcaactactgcctttgaatagaacttctcctttgcattttggccccagaatttaaaacaaatgttcaaggaaaagcaaatccttgactggataaaaacagtaaacacttagggacattcacctaaatttattgttggcttaaatgaccaagcgttccccacgtccgtttctaaagtggggtaggatgtttagaatgcattactcacacagaaagatgggattgatgaaatcacaaaactaaacacaggctatagcaactatgaacagccttcacagagaatgaacaatagcacaaatgccagactgcaacacttcctaaaatgatgtctatagctatctgtaaagagagaataaccggccaggtgcagtggctcatgcctgtaatcccagcactttaggaggccgaggtgggcagatcacctgaggtcaggagttcaagaccagcctgaccaacatggagaaatcctgtctctactaaaaaatatgaaattagccaggcatggtggcgcatgcctgtaatcacagctactcaggaggctaagacaggagaatcccttgaacccaggaggcggaggttgtggtgagtggagatacgccattgcactccagcctgggcaacaacagcgaaactccgtctcaaaaaaaaaagagagaataaccaactcctaagacatccattaagacagacgcacagtctgtcaactttggttagaataccaaaccttaagatcaggtaatgcttttgtgcataggctgtcacaactatattacatccacgttagcatccatgtgaaactaggtatcaggggcttgaccaaatgagatggtaacatccagggcctaaagacacctcttgttaactaatatggagaaaaaagagtgcctttccacactctcccacagaatggaggctccctaactaacactcaaatttggggttcagcaaatgaaactaaatatcaactgacaccacaatagcactagcctgccctagagtcaagactctgggtgggcagctcttcaataaagacagcaaggaggccatcctgaagaggtatatccacgtctaacaggttacaagaatactgccactagaatcctaaagagcagagtggtcactggggggtaaaaagaaaaaggaaaatccttgaagaaaggcaaaggagacaaccagtctcaagaccacaaggtattataagtcttctgtcaaagtaagatgtataagatttgtaaacactattgtgcaaaataagttcaataaggaatgaaaaaatcccccccacccacaaaaaaaaatcaaggcagctagtacctacagaagggagaggagaggatttactattttaatttgtcctttcaataggattcttctcctgctccatcctacttataatgtcctggattgccaactttaaaatactgacaggtattcagaggattcaaataaaaaagtaagaggggttgttaaaagtaacttatatccattcacaagttatctaacactggctcacagcctggtaaagaatctcttccttatggaagattgaacaatgatttctttgaggtaccagaaagtagactttgcctctgcagagaggtgggtcttttgcttgaacctgggtgttctggcttaatgctggctttcaggaggcagctaccttcaatttaaattaaaaaaacaaaaaaaaactataccaaccgaacgcttgcttaaacacagacacacacacacaaaatcaggagggacttcatacaaaaaaattcaagtcggcaatgggcatttccaaaaggtgacgagttttttaaataaaaattttgtgaaaaataaaatccaaaatcggcaaagcacaaaacagcaaaagaacatgaaatgctgctccaagcaggaccctggatagggaccttcattgctgatgggatgacacaaattaactgtacgagaagtctgggagacgctggaaccgatggtggcttcgcatgttcctgtcaacccactgagtcagactgtatctttgcagatgtttctgtcggcgggcgtagtttcgcgtggtgaggtccgaaggatgctgccattttgagtgctgcatatgatgaacttgatccatcaaggcacaaagctcccccgagatacccagcaattccacttctagggattcatccttggttagtgtcctctgggtcttctatatgagcaatgacactcctgagataaagctgcttctgctgttctagatttgactgtgaaaacgtcggaacattagtcctggtcttagtttgtagaacaggaatgactttgcctagtcttctctcatggcctttcatcttcccagaatccttgttaagaacatcctgtttgtttgatgaggtggaaacaaccagagatctcatttcacaacttgacttgtgtgaaccaccatttctgcaggataactccatattaggagtctctgaatggtctgagatccgagagaatacagacgtagggttctcactgtcaggcatatttttatcagagacagtctgttgaaagttattgtttgaagaagagagctggggcccattccaggcagagttattggggctgatcccttcagattcagtacaaagtttgctttcatttgggctaagaccatcttctctcatctcttctccaagggaagagagtttttcagtatctttggacgaatcagtctcgtccttatcaagcagagcatcacaaactgttggattaaatggtgcaacagttacttttataagattcttttctagtacagagcgtctgtttaatggtttagtatgagctggtccatgaccacttgatgtacttagctgaggtagtttgaagaggtcaggagtctcagctactggtcccaggctgtacgatgaatttttctctcggggagtatcaagtagaatttgactccctctttctcccttctcaacatgcccaccatcatcttccccagaagactgctcatatgatgggtcatcttccttcaacagtgcatcaatctcttcctctgtgtaatttacatcaccatcatcttcttctccctctgacagctccagcaaggagtcatccaatccatcctcatccaaggaatcccaagaaaatggggcaccgtctttaggcaagagagaggtaccagaagactgttcagagggcacccgtgagcacatcattttgtgtggagctgctggagcaatctctgcctttgccacgagaccaaatggaaaaaggtttcagttcctgctagctgttcctttcaggagacttgtcaaaatgattgactcccaccttc

SEQ ID NO: 10403 - RNA, 3870 nt, Homo sapiens
  source 1..3870: mol_type = other RNA
ccgccttctctcctcccccagtccaacagatttaattaagctgctaaagctttggaaaaacagaattatttgagctaagaggaaatgtgattgtcacattttctagttaacctgtcactcatttgatttggcaaaggcagtgctcctattacacattcagtcttaaaaccccatgtaccaggagggcacgagtcttagatttttgcctaggcaaaatcctgtcccttcactccttgggttttctgtagggaactagactacagttccctactgtagctgcaatgctagctattccaactacatttaattttaactatgctatggtcccaaaggtggatgtttggcatgtctcactccatcaacctaatttagggcagcctggagaagtgaccgatgtagtaaatgccaagtaggctaactaaaataatagatttcaactactgcctttgaatagaacttctcctttgcattttggccccagaatttaaaacaaatgttcaaggaaaagcaaatccttgactggataaaaacagtaaacacttagggacattcacctaaatttattgttggcttaaatgaccaagcgttccccacgtccgtttctaaagtggggtaggatgtttagaatgcattactcacacagaaagatgggattgatgaaatcacaaaactaaacacaggctatagcaactatgaacagccttcacagagaatgaacaatagcacaaatgccagactgcaacacttcctaaaatgatgtctatagctatctgtaaagagagaataaccggccaggtgcagtggctcatgcctgtaatcccagcactttaggaggccgaggtgggcagatcacctgaggtcaggagttcaagaccagcctgaccaacatggagaaatcctgtctctactaaaaaatatgaaattagccaggcatggtggcgcatgcctgtaatcacagctactcaggaggctaagacaggagaatcccttgaacccaggaggcggaggttgtggtgagtggagatacgccattgcactccagcctgggcaacaacagcgaaactccgtctcaaaaaaaaaagagagaataaccaactcctaagacatccattaagacagacgcacagtctgtcaactttggttagaataccaaaccttaagatcaggtaatgcttttgtgcataggctgtcacaactatattacatccacgttagcatccatgtgaaactaggtatcaggggcttgaccaaatgagatggtaacatccagggcctaaagacacctcttgttaactaatatggagaaaaaagagtgcctttccacactctcccacagaatggaggctccctaactaacactcaaatttggggttcagcaaatgaaactaaatatcaactgacaccacaatagcactagcctgccctagagtcaagactctgggtgggcagctcttcaataaagacagcaaggaggccatcctgaagaggtatatccacgtctaacaggttacaagaatactgccactagaatcctaaagagcagagtggtcactggggggtaaaaagaaaaaggaaaatccttgaagaaaggcaaaggagacaaccagtctcaagaccacaaggtattataagtcttctgtcaaagtaagatgtataagatttgtaaacactattgtgcaaaataagttcaataaggaatgaaaaaatcccccccacccacaaaaaaaaatcaaggcagctagtacctacagaagggagaggagaggatttactattttaatttgtcctttcaataggattcttctcctgctccatcctacttataatgtcctggattgccaactttaaaatactgacaggtattcagaggattcaaataaaaaagtaagaggggttgttaaaagtaacttatatccattcacaagttatctaacactggctcacagcctggtaaagaatctcttccttatggaagattgaacaatgatttctttgaggtaccagaaagtagactttgcctctgcagagaggtgggtcttttgcttgaacctgggtgttctggcttaatgctggctttcaggaggcagctaccttcaatttaaattaaaaaaacaaaaaaaaactataccaaccgaacgcttgcttaaacacagacacacacacacaaaatcaggagggacttcatacaaaaaaattcaagtcggcaatgggcatttccaaaaggtgacgagttttttaaataaaaattttgtgaaaaataaaatccaaaatcggcaaagcacaaaacagcaaaagaacatgaaatgctgctccaagcaggaccctggatagggaccttcattgctgatgggatgacacaaattaactgtacgagaagtctgggagacgctggaaccgatggtggcttcgcatgttcctgtcaacccactgagtcagactgtatctttgcagatgtttctgtcggcgggcgtagtttcgcgtggtgaggtccgaaggatgctgccattttgagtgctgcatatgatgaacttgatccatcaaggcacaaagctcccccgagatacccagcaattccacttctagggattcatccttggttagtgtcctctgggtcttctatatgagcaatgacactcctgagataaagctgcttctgctgttctagatttgactgtgaaaacgtcggaacattagtcctggtcttagtttgtagaacaggaatgactttgcctagtcttctctcatggcctttcatcttcccagaatccttgttaagaacatcctgtttgtttgatgaggtggaaacaaccagagatctcatttcacaacttgacttgtgtgaaccaccatttctgcaggataactccatattaggagtctctgaatggtctgagatccgagagaatacagacgtagggttctcactgtcaggcatatttttatcagagacagtctgttgaaagttattgtttgaagaagagagctggggcccattccaggcagagttattggggctgatcccttcagattcagtacaaagtttgctttcatttgggctaagaccatcttctctcatctcttctccaagggaagagagtttttcagtatctttggacgaatcagtctcgtccttatcaagcagagcatcacaaactgttggattaaatggtgcaacagttacttttataagattcttttctagtacagagcgtctgtttaatggtttagtatgagctggtccatgaccacttgatgtacttagctgaggtagtttgaagaggtcaggagtctcagctactggtcccaggctgtacgatgaatttttctctcggggagtatcaagtagaatttgactccctctttctcccttctcaacatgcccaccatcatcttccccagaagactgctcatatgatgggtcatcttccttcaacagtgcatcaatctcttcctctgtgtaatttacatcaccatcatcttcttctccctctgacagctccagcaaggagtcatccaatccatcctcatccaaggaatcccaagaaaatggggcaccgtctttaggcaagagagaggtaccagaagactgttcagagggcacccgtgagcacatcattttgtgtggagctgctggagcaatctctgcctttgccacgagaccaaatggaaaaaggtttcagttcctgctagctgttcctttcaggagacttgtcaaaatgattgactcccaccttcctccggaagccgggccaaagcctgggcgaacgactgcgcctcactccgccccctgcgccattttatcgccccctccccgacctcccctaccccgagtcagccgggccaacaccagggggagggcaaaccagcagt

SEQ ID NO: 10404 - RNA, 3893 nt, Homo sapiens
  source 1..3893: mol_type = other RNA
ccgccttctctcctcccccagtccaacagatttaattaagctgctaaagctttggaaaaacagaattatttgagctaagaggaaatgtgattgtcacattttctagttaacctgtcactcatttgatttggcaaaggcagtgctcctattacacattcagtcttaaaaccccatgtaccaggagggcacgagtcttagatttttgcctaggcaaaatcctgtcccttcactccttgggttttctgtagggaactagactacagttccctactgtagctgcaatgctagctattccaactacatttaattttaactatgctatggtcccaaaggtggatgtttggcatgtctcactccatcaacctaatttagggcagcctggagaagtgaccgatgtagtaaatgccaagtaggctaactaaaataatagatttcaactactgcctttgaatagaacttctcctttgcattttggccccagaatttaaaacaaatgttcaaggaaaagcaaatccttgactggataaaaacagtaaacacttagggacattcacctaaatttattgttggcttaaatgaccaagcgttccccacgtccgtttctaaagtggggtaggatgtttagaatgcattactcacacagaaagatgggattgatgaaatcacaaaactaaacacaggctatagcaactatgaacagccttcacagagaatgaacaatagcacaaatgccagactgcaacacttcctaaaatgatgtctatagctatctgtaaagagagaataaccggccaggtgcagtggctcatgcctgtaatcccagcactttaggaggccgaggtgggcagatcacctgaggtcaggagttcaagaccagcctgaccaacatggagaaatcctgtctctactaaaaaatatgaaattagccaggcatggtggcgcatgcctgtaatcacagctactcaggaggctaagacaggagaatcccttgaacccaggaggcggaggttgtggtgagtggagatacgccattgcactccagcctgggcaacaacagcgaaactccgtctcaaaaaaaaaagagagaataaccaactcctaagacatccattaagacagacgcacagtctgtcaactttggttagaataccaaaccttaagatcaggtaatgcttttgtgcataggctgtcacaactatattacatccacgttagcatccatgtgaaactaggtatcaggggcttgaccaaatgagatggtaacatccagggcctaaagacacctcttgttaactaatatggagaaaaaagagtgcctttccacactctcccacagaatggaggctccctaactaacactcaaatttggggttcagcaaatgaaactaaatatcaactgacaccacaatagcactagcctgccctagagtcaagactctgggtgggcagctcttcaataaagacagcaaggaggccatcctgaagaggtatatccacgtctaacaggttacaagaatactgccactagaatcctaaagagcagagtggtcactggggggtaaaaagaaaaaggaaaatccttgaagaaaggcaaaggagacaaccagtctcaagaccacaaggtattataagtcttctgtcaaagtaagatgtataagatttgtaaacactattgtgcaaaataagttcaataaggaatgaaaaaatcccccccacccacaaaaaaaaatcaaggcagctagtacctacagaagggagaggagaggatttactattttaatttgtcctttcaataggattcttctcctgctccatcctacttataatgtcctggattgccaactttaaaatactgacaggtattcagaggattcaaataaaaaagtaagaggggttgttaaaagtaacttatatccattcacaagttatctaacactggctcacagcctggtaaagaatctcttccttatggaagattgaacaatgatttctttgaggtaccagaaagtagactttgcctctgcagagaggtgggtcttttgcttgaacctgggtgttctggcttaatgctggctttcaggaggcagctaccttcaatttaaattaaaaaaacaaaaaaaaactataccaaccgaacgcttgcttaaacacagacacacacacacaaaatcaggagggacttcatacaaaaaaattcaagtcggcaatgggcatttccaaaaggtgacgagttttttaaataaaaattttgtgaaaaataaaatccaaaatcggcaaagcacaaaacagcaaaagaacatgaaatgctgctccaagcaggaccctggatagggaccttcattgctgatgggatgacacaaattaactgtacgagaagtctgggagacgctggaaccgatggtggcttcgcatgttcctgtcaacccactgagtcagactgtatctttgcagatgtttctgtcggcgggcgtagtttcgcgtggtgaggtccgaaggatgctgccattttgagtgctgcatatgatgaacttgatccatcaaggcacaaagctcccccgagatacctctaggtcaacaaaactgcgatgatctagtagaaatcttgactgattttccttggttagtgtcctctgggtcttctatatgagcaatgacactcctgagataaagctgcttctgctgttctagatttgactgtgaaaacgtcggaacattagtcctggtcttagtttgtagaacaggaatgactttgcctagtcttctctcatggcctttcatcttcccagaatccttgttaagaacatcctgtttgtttgatgaggtggaaacaaccagagatctcatttcacaacttgacttgtgtgaaccaccatttctgcaggataactccatattaggagtctctgaatggtctgagatccgagagaatacagacgtagggttctcactgtcaggcatatttttatcagagacagtctgttgaaagttattgtttgaagaagagagctggggcccattccaggcagagttattggggctgatcccttcagattcagtacaaagtttgctttcatttgggctaagaccatcttctctcatctcttctccaagggaagagagtttttcagtatctttggacgaatcagtctcgtccttatcaagcagagcatcacaaactgttggattaaatggtgcaacagttacttttataagattcttttctagtacagagcgtctgtttaatggtttagtatgagctggtccatgaccacttgatgtacttagctgaggtagtttgaagaggtcaggagtctcagctactggtcccaggctgtacgatgaatttttctctcggggagtatcaagtagaatttgactccctctttctcccttctcaacatgcccaccatcatcttccccagaagactgctcatatgatgggtcatcttccttcaacagtgcatcaatctcttcctctgtgtaatttacatcaccatcatcttcttctccctctgacagctccagcaaggagtcatccaatccatcctcatccaaggaatcccaagaaaatggggcaccgtctttaggcaagagagaggtaccagaagactgttcagagggcacccgtgagcacatcattttgtgtggagctgctggagcaatctctgcctttgccacgagaccaaatggaaaaaggtttcagttcctgctagctgttcctttcaggagacttgtcaaaatgattgactcccaccttcctccggaagccgggccaaagcctgggcgaacgactgcgcctcactccgccccctgcgccattttatcgccccctccccgacctcccctaccccgagtcagccgggccaacaccagggggagggcaaaccagcagt

SEQ ID NO: 10405 - RNA, 3888 nt, Homo sapiens
  source 1..3888: mol_type = other RNA
ccgccttctctcctcccccagtccaacagatttaattaagctgctaaagctttggaaaaacagaattatttgagctaagaggaaatgtgattgtcacattttctagttaacctgtcactcatttgatttggcaaaggcagtgctcctattacacattcagtcttaaaaccccatgtaccaggagggcacgagtcttagatttttgcctaggcaaaatcctgtcccttcactccttgggttttctgtagggaactagactacagttccctactgtagctgcaatgctagctattccaactacatttaattttaactatgctatggtcccaaaggtggatgtttggcatgtctcactccatcaacctaatttagggcagcctggagaagtgaccgatgtagtaaatgccaagtaggctaactaaaataatagatttcaactactgcctttgaatagaacttctcctttgcattttggccccagaatttaaaacaaatgttcaaggaaaagcaaatccttgactggataaaaacagtaaacacttagggacattcacctaaatttattgttggcttaaatgaccaagcgttccccacgtccgtttctaaagtggggtaggatgtttagaatgcattactcacacagaaagatgggattgatgaaatcacaaaactaaacacaggctatagcaactatgaacagccttcacagagaatgaacaatagcacaaatgccagactgcaacacttcctaaaatgatgtctatagctatctgtaaagagagaataaccggccaggtgcagtggctcatgcctgtaatcccagcactttaggaggccgaggtgggcagatcacctgaggtcaggagttcaagaccagcctgaccaacatggagaaatcctgtctctactaaaaaatatgaaattagccaggcatggtggcgcatgcctgtaatcacagctactcaggaggctaagacaggagaatcccttgaacccaggaggcggaggttgtggtgagtggagatacgccattgcactccagcctgggcaacaacagcgaaactccgtctcaaaaaaaaaagagagaataaccaactcctaagacatccattaagacagacgcacagtctgtcaactttggttagaataccaaaccttaagatcaggtaatgcttttgtgcataggctgtcacaactatattacatccacgttagcatccatgtgaaactaggtatcaggggcttgaccaaatgagatggtaacatccagggcctaaagacacctcttgttaactaatatggagaaaaaagagtgcctttccacactctcccacagaatggaggctccctaactaacactcaaatttggggttcagcaaatgaaactaaatatcaactgacaccacaatagcactagcctgccctagagtcaagactctgggtgggcagctcttcaataaagacagcaaggaggccatcctgaagaggtatatccacgtctaacaggttacaagaatactgccactagaatcctaaagagcagagtggtcactggggggtaaaaagaaaaaggaaaatccttgaagaaaggcaaaggagacaaccagtctcaagaccacaaggtattataagtcttctgtcaaagtaagatgtataagatttgtaaacactattgtgcaaaataagttcaataaggaatgaaaaaatcccccccacccacaaaaaaaaatcaaggcagctagtacctacagaagggagaggagaggatttactattttaatttgtcctttcaataggattcttctcctgctccatcctacttataatgtcctggattgccaactttaaaatactgacaggtattcagaggattcaaataaaaaagtaagaggggttgttaaaagtaacttatatccattcacaagttatctaacactggctcacagcctggtaaagaatctcttccttatggaagattgaacaatgatttctttgaggtaccagaaagtagactttgcctctgcagagaggtgggtcttttgcttgaacctgggtgttctggcttaatgctggctttcaggaggcagctaccttcaatttaaattaaaaaaacaaaaaaaaactataccaaccgaacgcttgcttaaacacagacacacacacacaaaatcaggagggacttcatacaaaaaaattcaagtcggcaatgggcatttccaaaaggtgacgagttttttaaataaaaattttgtgaaaaataaaatccaaaatcggcaaagcacaaaacagcaaaagaacatgaaatgctgctccaagcaggaccctggatagggaccttcattgctgatgggatgacacaaattaactgtacgagaagtctgggagacgctggaaccgatggtggcttcgcatgttcctgtcaacccactgagtcagactgtatctttgcagatgtttctgtcggcgggcgtagtttcgcgtggtgaggtccgaaggatgctgccattttgagtgctgcatatgatgaacttgatccatcaaggcacaaagctcccccgagataccttcatttatcaacattttatcaaagctgtttccagtattttttggcttggttagtgtcctctgggtcttctatatgagcaatgacactcctgagataaagctgcttctgctgttctagatttgactgtgaaaacgtcggaacattagtcctggtcttagtttgtagaacaggaatgactttgcctagtcttctctcatggcctttcatcttcccagaatccttgttaagaacatcctgtttgtttgatgaggtggaaacaaccagagatctcatttcacaacttgacttgtgtgaaccaccatttctgcaggataactccatattaggagtctctgaatggtctgagatccgagagaatacagacgtagggttctcactgtcaggcatatttttatcagagacagtctgttgaaagttattgtttgaagaagagagctggggcccattccaggcagagttattggggctgatcccttcagattcagtacaaagtttgctttcatttgggctaagaccatcttctctcatctcttctccaagggaagagagtttttcagtatctttggacgaatcagtctcgtccttatcaagcagagcatcacaaactgttggattaaatggtgcaacagttacttttataagattcttttctagtacagagcgtctgtttaatggtttagtatgagctggtccatgaccacttgatgtacttagctgaggtagtttgaagaggtcaggagtctcagctactggtcccaggctgtacgatgaatttttctctcggggagtatcaagtagaatttgactccctctttctcccttctcaacatgcccaccatcatcttccccagaagactgctcatatgatgggtcatcttccttcaacagtgcatcaatctcttcctctgtgtaatttacatcaccatcatcttcttctccctctgacagctccagcaaggagtcatccaatccatcctcatccaaggaatcccaagaaaatggggcaccgtctttaggcaagagagaggtaccagaagactgttcagagggcacccgtgagcacatcattttgtgtggagctgctggagcaatctctgcctttgccacgagaccaaatggaaaaaggtttcagttcctgctagctgttcctttcaggagacttgtcaaaatgattgactcccaccttcctccggaagccgggccaaagcctgggcgaacgactgcgcctcactccgccccctgcgccattttatcgccccctccccgacctcccctaccccgagtcagccgggccaacaccagggggagggcaaaccagcagt

SEQ ID NO: 10406 - RNA, 4004 nt, Homo sapiens
  source 1..4004: mol_type = other RNA
ccgccttctctcctcccccagtccaacagatttaattaagctgctaaagctttggaaaaacagaattatttgagctaagaggaaatgtgattgtcacattttctagttaacctgtcactcatttgatttggcaaaggcagtgctcctattacacattcagtcttaaaaccccatgtaccaggagggcacgagtcttagatttttgcctaggcaaaatcctgtcccttcactccttgggttttctgtagggaactagactacagttccctactgtagctgcaatgctagctattccaactacatttaattttaactatgctatggtcccaaaggtggatgtttggcatgtctcactccatcaacctaatttagggcagcctggagaagtgaccgatgtagtaaatgccaagtaggctaactaaaataatagatttcaactactgcctttgaatagaacttctcctttgcattttggccccagaatttaaaacaaatgttcaaggaaaagcaaatccttgactggataaaaacagtaaacacttagggacattcacctaaatttattgttggcttaaatgaccaagcgttccccacgtccgtttctaaagtggggtaggatgtttagaatgcattactcacacagaaagatgggattgatgaaatcacaaaactaaacacaggctatagcaactatgaacagccttcacagagaatgaacaatagcacaaatgccagactgcaacacttcctaaaatgatgtctatagctatctgtaaagagagaataaccggccaggtgcagtggctcatgcctgtaatcccagcactttaggaggccgaggtgggcagatcacctgaggtcaggagttcaagaccagcctgaccaacatggagaaatcctgtctctactaaaaaatatgaaattagccaggcatggtggcgcatgcctgtaatcacagctactcaggaggctaagacaggagaatcccttgaacccaggaggcggaggttgtggtgagtggagatacgccattgcactccagcctgggcaacaacagcgaaactccgtctcaaaaaaaaaagagagaataaccaactcctaagacatccattaagacagacgcacagtctgtcaactttggttagaataccaaaccttaagatcaggtaatgcttttgtgcataggctgtcacaactatattacatccacgttagcatccatgtgaaactaggtatcaggggcttgaccaaatgagatggtaacatccagggcctaaagacacctcttgttaactaatatggagaaaaaagagtgcctttccacactctcccacagaatggaggctccctaactaacactcaaatttggggttcagcaaatgaaactaaatatcaactgacaccacaatagcactagcctgccctagagtcaagactctgggtgggcagctcttcaataaagacagcaaggaggccatcctgaagaggtatatccacgtctaacaggttacaagaatactgccactagaatcctaaagagcagagtggtcactggggggtaaaaagaaaaaggaaaatccttgaagaaaggcaaaggagacaaccagtctcaagaccacaaggtattataagtcttctgtcaaagtaagatgtataagatttgtaaacactattgtgcaaaataagttcaataaggaatgaaaaaatcccccccacccacaaaaaaaaatcaaggcagctagtacctacagaagggagaggagaggatttactattttaatttgtcctttcaataggattcttctcctgctccatcctacttataatgtcctggattgccaactttaaaatactgacaggtattcagaggattcaaataaaaaagtaagaggggttgttaaaagtaacttatatccattcacaagttatctaacactggctcacagcctggtaaagaatctcttccttatggaagattgaacaatgatttctttgaggtaccagaaagtagactttgcctctgcagagaggtgggtcttttgcttgaacctgggtgttctggcttaatgctggctttcaggaggcagctaccttcaatttaaattaaaaaaacaaaaaaaaactataccaaccgaacgcttgcttaaacacagacacacacacacaaaatcaggagggacttcatacaaaaaaattcaagtcggcaatgggcatttccaaaaggtgacgagttttttaaataaaaattttgtgaaaaataaaatccaaaatcggcaaagcacaaaacagcaaaagaacatgaaatgctgctccaagcaggaccctggatagggaccttcattgctgatgggatgacacaaattaactgtacgagaagtctgggagacgctggaaccgatggtggcttcgcatgttcctgtcaacccactgagtcagactgtatctttgcagatgtttctgtcggcgggcgtagtttcgcgtggtgaggtccgaaggatgctgccattttgagtgctgcatatgatgaacttgatccatcaaggcacaaagctcccccgagataccttggttagtgtcctctgggtcttctatatgagcaatgacactcctgagataaagctgcttctgctgttctagatttgactgtgaaaacgtcggaacattagtcctggtcttagtttgtagaacaggaatgactttgcctagtcttctctcatggcctttcatcttcccagaatccttgttaagaacatcctgtttgtttgatgaggtggaaacaaccagagatctcatttcacaacttgacttgtgtgaaccaccatttctgcaggataactccatattaggagtctctgaatggtctgagatccgagagaatacagacgtagggttctcactgtcaggcatatttttatcagagacagtctgttgaaagttattgtttgaagaagagagctggggcccattccaggcagagttattggggctgatcccttcagattcagtacaaagtttgctttcatttgggctaagaccatcttctctcatctcttctccaagggaagagagtttttcagtatctttggacgaatcagtctcgtccttatcaagcagagcatcacaaactgttggattaaatggtgcaacagttacttttataagattcttttctagtacagagcgtctgtttaatggtttagtatgagctggtccatgaccacttgatgtacttagctgaggtagtttgaagaggtcaggagtctcagctactggtcccaggctgtacgatgaatttttctctcggggagtatcaagtagaatttgactccctctttctcccttctcaacatgcccaccatcatcttccccagaagactgctcatatgatgggtcatcttccttcaacagtgcatcaatctcttcctctgtgtaatttacatcaccatcatcttcttctccctctgacagctccagcaaggagtcatccaatccatcctcatccaaggaatcccaagaaaatggggcaccgtctttaggcaagagagaggtaccagaagactgttcagagggcacccgtgagcacatcattttgtgtggagctgctggagcaatctctgcctttgccacgagaccaaatggaaaaaggtttcagttcctgctagctgttcctttcaggagacttgtcaaaatgattgactcccaccttccagattgttttgaagcaaatcccaggcattgtatcatttcatctgtaaataacaagaattccttatcataaaatatacagttcagatttccaattatcttatgtcatatttttttttaaggctaaaaaataatcagtatccaagtaaggtccatacaatgtgactggctgataatgtcttatgtgtattttaatctaaaaatttcagatcttttccccctgcaattactttattaaaaaaacaatacgcgagatggcttacgcctgtaatcccagcactttcggaggctaagttggg

SEQ ID NO: 10407 - RNA, 3769 nt, Homo sapiens
  source 1..3769: mol_type = other RNA
ccgccttctctcctcccccagtccaacagatttaattaagctgctaaagctttggaaaaacagaattatttgagctaagaggaaatgtgattgtcacattttctagttaacctgtcactcatttgatttggcaaaggcagtgctcctattacacattcagtcttaaaaccccatgtaccaggagggcacgagtcttagatttttgcctaggcaaaatcctgtcccttcactccttgggttttctgtagggaactagactacagttccctactgtagctgcaatgctagctattccaactacatttaattttaactatgctatggtcccaaaggtggatgtttggcatgtctcactccatcaacctaatttagggcagcctggagaagtgaccgatgtagtaaatgccaagtaggctaactaaaataatagatttcaactactgcctttgaatagaacttctcctttgcattttggccccagaatttaaaacaaatgttcaaggaaaagcaaatccttgactggataaaaacagtaaacacttagggacattcacctaaatttattgttggcttaaatgaccaagcgttccccacgtccgtttctaaagtggggtaggatgtttagaatgcattactcacacagaaagatgggattgatgaaatcacaaaactaaacacaggctatagcaactatgaacagccttcacagagaatgaacaatagcacaaatgccagactgcaacacttcctaaaatgatgtctatagctatctgtaaagagagaataaccggccaggtgcagtggctcatgcctgtaatcccagcactttaggaggccgaggtgggcagatcacctgaggtcaggagttcaagaccagcctgaccaacatggagaaatcctgtctctactaaaaaatatgaaattagccaggcatggtggcgcatgcctgtaatcacagctactcaggaggctaagacaggagaatcccttgaacccaggaggcggaggttgtggtgagtggagatacgccattgcactccagcctgggcaacaacagcgaaactccgtctcaaaaaaaaaagagagaataaccaactcctaagacatccattaagacagacgcacagtctgtcaactttggttagaataccaaaccttaagatcaggtaatgcttttgtgcataggctgtcacaactatattacatccacgttagcatccatgtgaaactaggtatcaggggcttgaccaaatgagatggtaacatccagggcctaaagacacctcttgttaactaatatggagaaaaaagagtgcctttccacactctcccacagaatggaggctccctaactaacactcaaatttggggttcagcaaatgaaactaaatatcaactgacaccacaatagcactagcctgccctagagtcaagactctgggtgggcagctcttcaataaagacagcaaggaggccatcctgaagaggtatatccacgtctaacaggttacaagaatactgccactagaatcctaaagagcagagtggtcactggggggtaaaaagaaaaaggaaaatccttgaagaaaggcaaaggagacaaccagtctcaagaccacaaggtattataagtcttctgtcaaagtaagatgtataagatttgtaaacactattgtgcaaaataagttcaataaggaatgaaaaaatcccccccacccacaaaaaaaaatcaaggcagctagtacctacagaagggagaggagaggatttactattttaatttgtcctttcaataggattcttctcctgctccatcctacttataatgtcctggattgccaactttaaaatactgacaggtattcagaggattcaaataaaaaagtaagaggggttgttaaaagtaacttatatccattcacaagttatctaacactggctcacagcctggtaaagaatctcttccttatggaagattgaacaatgatttctttgaggtaccagaaagtagactttgcctctgcagagaggtgggtcttttgcttgaacctgggtgttctggcttaatgctggctttcaggaggcagctaccttcaatttaaattaaaaaaacaaaaaaaaactataccaaccgaacgcttgcttaaacacagacacacacacacaaaatcaggagggacttcatacaaaaaaattcaagtcggcaatgggcatttccaaaaggtgacgagttttttaaataaaaattttgtgaaaaataaaatccaaaatcggcaaagcacaaaacagcaaaagaacatgaaatgctgctccaagcaggaccctggatagggaccttcattgctgatgggatgacacaaattaactgtacgagaagtctgggagacgctggaaccgatggtggcttcgcatgttcctgtcaacccactgagtcagactgtatctttgcagatgtttctgtcggcgggcgtagtttcgcgtggtgaggtccgaaggatgctgccattttgagtgctgcatatgatgaacttgatccatcaaggcacaaagctcccccgagataccttggttagtgtcctctgggtcttctatatgagcaatgacactcctgagataaagctgcttctgctgttctagatttgactgtgaaaacgtcggaacattagtcctggtcttagtttgtagaacaggaatgactttgcctagtcttctctcatggcctttcatcttcccagaatccttgttaagaacatcctgtttgtttgatgaggtggaaacaaccagagatctcatttcacaacttgacttgtgtgaaccaccatttctgcaggataactccatattaggagtctctgaatggtctgagatccgagagaatacagacgtagggttctcactgtcaggcatatttttatcagagacagtctgttgaaagttattgtttgaagaagagagctggggcccattccaggcagagttattggggctgatcccttcagattcagtacaaagtttgctttcatttgggctaagaccatcttctctcatctcttctccaagggaagagagtttttcagtatctttggacgaatcagtctcgtccttatcaagcagagcatcacaaactgttggattaaatggtgcaacagttacttttataagattcttttctagtacagagcgtctgtttaatggtttagtatgagctggtccatgaccacttgatgtacttagctgaggtagtttgaagaggtcaggagtctcagctactggtcccaggctgtacgatgaatttttctctcggggagtatcaagtagaatttgactccctctttctcccttctcaacatgcccaccatcatcttccccagaagactgctcatatgatgggtcatcttccttcaacagtgcatcaatctcttcctctgtgtaatttacatcaccatcatcttcttctccctctgacagctccagcaaggagtcatccaatccatcctcatccaaggaatcccaagaaaatggggcaccgtctttaggcaagagagaggtaccagaagactgttcagagggcacccgtgagcacatcattttgtgtggagctgctggagcaatctctgcctttgccacgagaccaaatggaaaaaggtttcagttcctgctagctgttcctttcaggagacttgtcaaaatgattgactcccaccttccattctctttctgatgtctgatgttacttcctctttttttttttttttttttgaaacggagt

SEQ ID NO: 10408 - RNA, 3865 nt, Homo sapiens
  source 1..3865: mol_type = other RNA
ccgccttctctcctcccccagtccaacagatttaattaagctgctaaagctttggaaaaacagaattatttgagctaagaggaaatgtgattgtcacattttctagttaacctgtcactcatttgatttggcaaaggcagtgctcctattacacattcagtcttaaaaccccatgtaccaggagggcacgagtcttagatttttgcctaggcaaaatcctgtcccttcactccttgggttttctgtagggaactagactacagttccctactgtagctgcaatgctagctattccaactacatttaattttaactatgctatggtcccaaaggtggatgtttggcatgtctcactccatcaacctaatttagggcagcctggagaagtgaccgatgtagtaaatgccaagtaggctaactaaaataatagatttcaactactgcctttgaatagaacttctcctttgcattttggccccagaatttaaaacaaatgttcaaggaaaagcaaatccttgactggataaaaacagtaaacacttagggacattcacctaaatttattgttggcttaaatgaccaagcgttccccacgtccgtttctaaagtggggtaggatgtttagaatgcattactcacacagaaagatgggattgatgaaatcacaaaactaaacacaggctatagcaactatgaacagccttcacagagaatgaacaatagcacaaatgccagactgcaacacttcctaaaatgatgtctatagctatctgtaaagagagaataaccggccaggtgcagtggctcatgcctgtaatcccagcactttaggaggccgaggtgggcagatcacctgaggtcaggagttcaagaccagcctgaccaacatggagaaatcctgtctctactaaaaaatatgaaattagccaggcatggtggcgcatgcctgtaatcacagctactcaggaggctaagacaggagaatcccttgaacccaggaggcggaggttgtggtgagtggagatacgccattgcactccagcctgggcaacaacagcgaaactccgtctcaaaaaaaaaagagagaataaccaactcctaagacatccattaagacagacgcacagtctgtcaactttggttagaataccaaaccttaagatcaggtaatgcttttgtgcataggctgtcacaactatattacatccacgttagcatccatgtgaaactaggtatcaggggcttgaccaaatgagatggtaacatccagggcctaaagacacctcttgttaactaatatggagaaaaaagagtgcctttccacactctcccacagaatggaggctccctaactaacactcaaatttggggttcagcaaatgaaactaaatatcaactgacaccacaatagcactagcctgccctagagtcaagactctgggtgggcagctcttcaataaagacagcaaggaggccatcctgaagaggtatatccacgtctaacaggttacaagaatactgccactagaatcctaaagagcagagtggtcactggggggtaaaaagaaaaaggaaaatccttgaagaaaggcaaaggagacaaccagtctcaagaccacaaggtattataagtcttctgtcaaagtaagatgtataagatttgtaaacactattgtgcaaaataagttcaataaggaatgaaaaaatcccccccacccacaaaaaaaaatcaaggcagctagtacctacagaagggagaggagaggatttactattttaatttgtcctttcaataggattcttctcctgctccatcctacttataatgtcctggattgccaactttaaaatactgacaggtattcagaggattcaaataaaaaagtaagaggggttgttaaaagtaacttatatccattcacaagttatctaacactggctcacagcctggtaaagaatctcttccttatggaagattgaacaatgatttctttgaggtaccagaaagtagactttgcctctgcagagaggtgggtcttttgcttgaacctgggtgttctggcttaatgctggctttcaggaggcagctaccttcaatttaaattaaaaaaacaaaaaaaaactataccaaccgaacgcttgcttaaacacagacacacacacacaaaatcaggagggacttcatacaaaaaaattcaagtcggcaatgggcatttccaaaaggtgacgagttttttaaataaaaattttgtgaaaaataaaatccaaaatcggcaaagcacaaaacagcaaaagaacatgaaatgctgctccaagcaggaccctggatagggaccttcattgctgatgggatgacacaaattaactgtacgagaagtctgggagacgctggaaccgatggtggcttcgcatgttcctgtcaacccactgagtcagactgtatctttgcagatgtttctgtcggcgggcgtagtttcgcgtggtgaggtccgaaggatgctgccattttgagtgctgcatatgatgaacttgatccatcaaggcacaaagctcccccgagataccttggttagtgtcctctgggtcttctatatgagcaatgacactcctgagataaagctgcttctgctgttctagatttgactgtgaaaacgtcggaacattagtcctggtcttagtttgtagaacaggaatgactttgcctagtcttctctcatggcctttcatcttcccagaatccttgttaagaacatcctgtttgtttgatgaggtggaaacaaccagagatctcatttcacaacttgacttgtgtgaaccaccatttctgcaggataactccatattaggagtctctgaatggtctgagatccgagagaatacagacgtagggttctcactgtcaggcatatttttatcagagacagtctgttgaaagttattgtttgaagaagagagctggggcccattccaggcagagttattggggctgatcccttcagattcagtacaaagtttgctttcatttgggctaagaccatcttctctcatctcttctccaagggaagagagtttttcagtatctttggacgaatcagtctcgtccttatcaagcagagcatcacaaactgttggattaaatggtgcaacagttacttttataagattcttttctagtacagagcgtctgtttaatggtttagtatgagctggtccatgaccacttgatgtacttagctgaggtagtttgaagaggtcaggagtctcagctactggtcccaggctgtacgatgaatttttctctcggggagtatcaagtagaatttgactccctctttctcccttctcaacatgcccaccatcatcttccccagaagactgctcatatgatgggtcatcttccttcaacagtgcatcaatctcttcctctgtgtaatttacatcaccatcatcttcttctccctctgacagctccagcaaggagtcatccaatccatcctcatccaaggaatcccaagaaaatggggcaccgtctttaggcaagagagaggtaccagaagactgttcagagggcacccgtgagcacatcattttgtgtggagctgctggagcaatctctgcctttgccacgagaccaaatggaaaaaggtttcagttcctgctagctgttcctttcaggagacttgtcaaaatgattgactcccaccttccccgagtcagccgggccaacaccagggggagggcaaaccagcagtgattggcaggaaaccgtcccgcctctaggagggttgtgccccgctcaggcgcctcagccccgccctccgcaccgcccaccgtgcccactggctccaccttttcccgtctcatc

SEQ ID NO: 10409 - RNA, 3814 nt, Homo sapiens
  source 1..3814: mol_type = other RNA
ccgccttctctcctcccccagtccaacagatttaattaagctgctaaagctttggaaaaacagaattatttgagctaagaggaaatgtgattgtcacattttctagttaacctgtcactcatttgatttggcaaaggcagtgctcctattacacattcagtcttaaaaccccatgtaccaggagggcacgagtcttagatttttgcctaggcaaaatcctgtcccttcactccttgggttttctgtagggaactagactacagttccctactgtagctgcaatgctagctattccaactacatttaattttaactatgctatggtcccaaaggtggatgtttggcatgtctcactccatcaacctaatttagggcagcctggagaagtgaccgatgtagtaaatgccaagtaggctaactaaaataatagatttcaactactgcctttgaatagaacttctcctttgcattttggccccagaatttaaaacaaatgttcaaggaaaagcaaatccttgactggataaaaacagtaaacacttagggacattcacctaaatttattgttggcttaaatgaccaagcgttccccacgtccgtttctaaagtggggtaggatgtttagaatgcattactcacacagaaagatgggattgatgaaatcacaaaactaaacacaggctatagcaactatgaacagccttcacagagaatgaacaatagcacaaatgccagactgcaacacttcctaaaatgatgtctatagctatctgtaaagagagaataaccggccaggtgcagtggctcatgcctgtaatcccagcactttaggaggccgaggtgggcagatcacctgaggtcaggagttcaagaccagcctgaccaacatggagaaatcctgtctctactaaaaaatatgaaattagccaggcatggtggcgcatgcctgtaatcacagctactcaggaggctaagacaggagaatcccttgaacccaggaggcggaggttgtggtgagtggagatacgccattgcactccagcctgggcaacaacagcgaaactccgtctcaaaaaaaaaagagagaataaccaactcctaagacatccattaagacagacgcacagtctgtcaactttggttagaataccaaaccttaagatcaggtaatgcttttgtgcataggctgtcacaactatattacatccacgttagcatccatgtgaaactaggtatcaggggcttgaccaaatgagatggtaacatccagggcctaaagacacctcttgttaactaatatggagaaaaaagagtgcctttccacactctcccacagaatggaggctccctaactaacactcaaatttggggttcagcaaatgaaactaaatatcaactgacaccacaatagcactagcctgccctagagtcaagactctgggtgggcagctcttcaataaagacagcaaggaggccatcctgaagaggtatatccacgtctaacaggttacaagaatactgccactagaatcctaaagagcagagtggtcactggggggtaaaaagaaaaaggaaaatccttgaagaaaggcaaaggagacaaccagtctcaagaccacaaggtattataagtcttctgtcaaagtaagatgtataagatttgtaaacactattgtgcaaaataagttcaataaggaatgaaaaaatcccccccacccacaaaaaaaaatcaaggcagctagtacctacagaagggagaggagaggatttactattttaatttgtcctttcaataggattcttctcctgctccatcctacttataatgtcctggattgccaactttaaaatactgacaggtattcagaggattcaaataaaaaagtaagaggggttgttaaaagtaacttatatccattcacaagttatctaacactggctcacagcctggtaaagaatctcttccttatggaagattgaacaatgatttctttgaggtaccagaaagtagactttgcctctgcagagaggtgggtcttttgcttgaacctgggtgttctggcttaatgctggctttcaggaggcagctaccttcaatttaaattaaaaaaacaaaaaaaaactataccaaccgaacgcttgcttaaacacagacacacacacacaaaatcaggagggacttcatacaaaaaaattcaagtcggcaatgggcatttccaaaaggtgacgagttttttaaataaaaattttgtgaaaaataaaatccaaaatcggcaaagcacaaaacagcaaaagaacatgaaatgctgctccaagcaggaccctggatagggaccttcattgctgatgggatgacacaaattaactgtacgagaagtctgggagacgctggaaccgatggtggcttcgcatgttcctgtcaacccactgagtcagactgtatctttgcagatgtttctgtcggcgggcgtagtttcgcgtggtgaggtccgaaggatgctgccattttgagtgctgcatatgatgaacttgatccatcaaggcacaaagctcccccgagataccttggttagtgtcctctgggtcttctatatgagcaatgacactcctgagataaagctgcttctgctgttctagatttgactgtgaaaacgtcggaacattagtcctggtcttagtttgtagaacaggaatgactttgcctagtcttctctcatggcctttcatcttcccagaatccttgttaagaacatcctgtttgtttgatgaggtggaaacaaccagagatctcatttcacaacttgacttgtgtgaaccaccatttctgcaggataactccatattaggagtctctgaatggtctgagatccgagagaatacagacgtagggttctcactgtcaggcatatttttatcagagacagtctgttgaaagttattgtttgaagaagagagctggggcccattccaggcagagttattggggctgatcccttcagattcagtacaaagtttgctttcatttgggctaagaccatcttctctcatctcttctccaagggaagagagtttttcagtatctttggacgaatcagtctcgtccttatcaagcagagcatcacaaactgttggattaaatggtgcaacagttacttttataagattcttttctagtacagagcgtctgtttaatggtttagtatgagctggtccatgaccacttgatgtacttagctgaggtagtttgaagaggtcaggagtctcagctactggtcccaggctgtacgatgaatttttctctcggggagtatcaagtagaatttgactccctctttctcccttctcaacatgcccaccatcatcttccccagaagactgctcatatgatgggtcatcttccttcaacagtgcatcaatctcttcctctgtgtaatttacatcaccatcatcttcttctccctctgacagctccagcaaggagtcatccaatccatcctcatccaaggaatcccaagaaaatggggcaccgtctttaggcaagagagaggtaccagaagactgttcagagggcacccgtgagcacatcattttgtgtggagctgctggagcaatctctgcctttgccacgagaccaaatggaaaaaggtttcagttcctgctagctgttcctttcaggagacttgtcaaaatgattgactcccaccttcctcaggagctagaacgcgcccttctcgcagcagggcgtgggcctcccaatccctccaaggggcggacggcgtgcgcaaccccctggagaagcaacaggcgcccccat

SEQ ID NO: 10410 - RNA, 3744 nt, Homo sapiens
  source 1..3744: mol_type = other RNA
ccgccttctctcctcccccagtccaacagatttaattaagctgctaaagctttggaaaaacagaattatttgagctaagaggaaatgtgattgtcacattttctagttaacctgtcactcatttgatttggcaaaggcagtgctcctattacacattcagtcttaaaaccccatgtaccaggagggcacgagtcttagatttttgcctaggcaaaatcctgtcccttcactccttgggttttctgtagggaactagactacagttccctactgtagctgcaatgctagctattccaactacatttaattttaactatgctatggtcccaaaggtggatgtttggcatgtctcactccatcaacctaatttagggcagcctggagaagtgaccgatgtagtaaatgccaagtaggctaactaaaataatagatttcaactactgcctttgaatagaacttctcctttgcattttggccccagaatttaaaacaaatgttcaaggaaaagcaaatccttgactggataaaaacagtaaacacttagggacattcacctaaatttattgttggcttaaatgaccaagcgttccccacgtccgtttctaaagtggggtaggatgtttagaatgcattactcacacagaaagatgggattgatgaaatcacaaaactaaacacaggctatagcaactatgaacagccttcacagagaatgaacaatagcacaaatgccagactgcaacacttcctaaaatgatgtctatagctatctgtaaagagagaataaccggccaggtgcagtggctcatgcctgtaatcccagcactttaggaggccgaggtgggcagatcacctgaggtcaggagttcaagaccagcctgaccaacatggagaaatcctgtctctactaaaaaatatgaaattagccaggcatggtggcgcatgcctgtaatcacagctactcaggaggctaagacaggagaatcccttgaacccaggaggcggaggttgtggtgagtggagatacgccattgcactccagcctgggcaacaacagcgaaactccgtctcaaaaaaaaaagagagaataaccaactcctaagacatccattaagacagacgcacagtctgtcaactttggttagaataccaaaccttaagatcaggtaatgcttttgtgcataggctgtcacaactatattacatccacgttagcatccatgtgaaactaggtatcaggggcttgaccaaatgagatggtaacatccagggcctaaagacacctcttgttaactaatatggagaaaaaagagtgcctttccacactctcccacagaatggaggctccctaactaacactcaaatttggggttcagcaaatgaaactaaatatcaactgacaccacaatagcactagcctgccctagagtcaagactctgggtgggcagctcttcaataaagacagcaaggaggccatcctgaagaggtatatccacgtctaacaggttacaagaatactgccactagaatcctaaagagcagagtggtcactggggggtaaaaagaaaaaggaaaatccttgaagaaaggcaaaggagacaaccagtctcaagaccacaaggtattataagtcttctgtcaaagtaagatgtataagatttgtaaacactattgtgcaaaataagttcaataaggaatgaaaaaatcccccccacccacaaaaaaaaatcaaggcagctagtacctacagaagggagaggagaggatttactattttaatttgtcctttcaataggattcttctcctgctccatcctacttataatgtcctggattgccaactttaaaatactgacaggtattcagaggattcaaataaaaaagtaagaggggttgttaaaagtaacttatatccattcacaagttatctaacactggctcacagcctggtaaagaatctcttccttatggaagattgaacaatgatttctttgaggtaccagaaagtagactttgcctctgcagagaggtgggtcttttgcttgaacctgggtgttctggcttaatgctggctttcaggaggcagctaccttcaatttaaattaaaaaaacaaaaaaaaactataccaaccgaacgcttgcttaaacacagacacacacacacaaaatcaggagggacttcatacaaaaaaattcaagtcggcaatgggcatttccaaaaggtgacgagttttttaaataaaaattttgtgaaaaataaaatccaaaatcggcaaagcacaaaacagcaaaagaacatgaaatgctgctccaagcaggaccctggatagggaccttcattgctgatgggatgacacaaattaactgtacgagaagtctgggagacgctggaaccgatggtggcttcgcatgttcctgtcaacccactgagtcagactgtatctttgcagatgtttctgtcggcgggcgtagtttcgcgtggtgaggtccgaaggatgctgccattttgagtgctgcatatgatgaacttgatccatcaaggcacaaagctcccccgagataccttggttagtgtcctctgggtcttctatatgagcaatgacactcctgagataaagctgcttctgctgttctagatttgactgtgaaaacgtcggaacattagtcctggtcttagtttgtagaacaggaatgactttgcctagtcttctctcatggcctttcatcttcccagaatccttgttaagaacatcctgtttgtttgatgaggtggaaacaaccagagatctcatttcacaacttgacttgtgtgaaccaccatttctgcaggataactccatattaggagtctctgaatggtctgagatccgagagaatacagacgtagggttctcactgtcaggcatatttttatcagagacagtctgttgaaagttattgtttgaagaagagagctggggcccattccaggcagagttattggggctgatcccttcagattcagtacaaagtttgctttcatttgggctaagaccatcttctctcatctcttctccaagggaagagagtttttcagtatctttggacgaatcagtctcgtccttatcaagcagagcatcacaaactgttggattaaatggtgcaacagttacttttataagattcttttctagtacagagcgtctgtttaatggtttagtatgagctggtccatgaccacttgatgtacttagctgaggtagtttgaagaggtcaggagtctcagctactggtcccaggctgtacgatgaatttttctctcggggagtatcaagtagaatttgactccctctttctcccttctcaacatgcccaccatcatcttccccagaagactgctcatatgatgggtcatcttccttcaacagtgcatcaatctcttcctctgtgtaatttacatcaccatcatcttcttctccctctgacagctccagcaaggagtcatccaatccatcctcatccaaggaatcccaagaaaatggggcaccgtctttaggcaagagagaggtaccagaagactgttcagagggcacccgtgagcacatcattttgtgtggagctgctggagcaatctctgcctttgccacgagaccaaatggaaaaaggtttcagttcctgctagctgttcctttcaggagacttgtcaaaatgattgactcccaccttcctccggaagccgggccaaagcctgggcgaacgactgc

SEQ ID NO: 10411 - RNA, 3923 nt, Homo sapiens
  source 1..3923: mol_type = other RNA
ccgccttctctcctcccccagtccaacagatttaattaagctgctaaagctttggaaaaacagaattatttgagctaagaggaaatgtgattgtcacattttctagttaacctgtcactcatttgatttggcaaaggcagtgctcctattacacattcagtcttaaaaccccatgtaccaggagggcacgagtcttagatttttgcctaggcaaaatcctgtcccttcactccttgggttttctgtagggaactagactacagttccctactgtagctgcaatgctagctattccaactacatttaattttaactatgctatggtcccaaaggtggatgtttggcatgtctcactccatcaacctaatttagggcagcctggagaagtgaccgatgtagtaaatgccaagtaggctaactaaaataatagatttcaactactgcctttgaatagaacttctcctttgcattttggccccagaatttaaaacaaatgttcaaggaaaagcaaatccttgactggataaaaacagtaaacacttagggacattcacctaaatttattgttggcttaaatgaccaagcgttccccacgtccgtttctaaagtggggtaggatgtttagaatgcattactcacacagaaagatgggattgatgaaatcacaaaactaaacacaggctatagcaactatgaacagccttcacagagaatgaacaatagcacaaatgccagactgcaacacttcctaaaatgatgtctatagctatctgtaaagagagaataaccggccaggtgcagtggctcatgcctgtaatcccagcactttaggaggccgaggtgggcagatcacctgaggtcaggagttcaagaccagcctgaccaacatggagaaatcctgtctctactaaaaaatatgaaattagccaggcatggtggcgcatgcctgtaatcacagctactcaggaggctaagacaggagaatcccttgaacccaggaggcggaggttgtggtgagtggagatacgccattgcactccagcctgggcaacaacagcgaaactccgtctcaaaaaaaaaagagagaataaccaactcctaagacatccattaagacagacgcacagtctgtcaactttggttagaataccaaaccttaagatcaggtaatgcttttgtgcataggctgtcacaactatattacatccacgttagcatccatgtgaaactaggtatcaggggcttgaccaaatgagatggtaacatccagggcctaaagacacctcttgttaactaatatggagaaaaaagagtgcctttccacactctcccacagaatggaggctccctaactaacactcaaatttggggttcagcaaatgaaactaaatatcaactgacaccacaatagcactagcctgccctagagtcaagactctgggtgggcagctcttcaataaagacagcaaggaggccatcctgaagaggtatatccacgtctaacaggttacaagaatactgccactagaatcctaaagagcagagtggtcactggggggtaaaaagaaaaaggaaaatccttgaagaaaggcaaaggagacaaccagtctcaagaccacaaggtattataagtcttctgtcaaagtaagatgtataagatttgtaaacactattgtgcaaaataagttcaataaggaatgaaaaaatcccccccacccacaaaaaaaaatcaaggcagctagtacctacagaagggagaggagaggatttactattttaatttgtcctttcaataggattcttctcctgctccatcctacttataatgtcctggattgccaactttaaaatactgacaggtattcagaggattcaaataaaaaagtaagaggggttgttaaaagtaacttatatccattcacaagttatctaacactggctcacagcctggtaaagaatctcttccttatggaagattgaacaatgatttctttgaggtaccagaaagtagactttgcctctgcagagaggtgggtcttttgcttgaacctgggtgttctggcttaatgctggctttcaggaggcagctaccttcaatttaaattaaaaaaacaaaaaaaaactataccaaccgaacgcttgcttaaacacagacacacacacacaaaatcaggagggacttcatacaaaaaaattcaagtcggcaatgggcatttccaaaaggtgacgagttttttaaataaaaattttgtgaaaaataaaatccaaaatcggcaaagcacaaaacagcaaaagaacatgaaatgctgctccaagcaggaccctggatagggaccttcattgctgatgggatgacacaaattaactgtacgagaagtctgggagacgctggaaccgatggtggcttcgcatgttcctgtcaacccactgagtcagactgtatctttgcagatgtttctgtcggcgggcgtagtttcgcgtggtgaggtccgaaggatgctgccattttgagtgctgcatatgatgaacttgatccatcaaggcacaaagctcccccgagataccttggttagtgtcctctgggtcttctatatgagcaatgacactcctgagataaagctgcttctgctgttctagatttgactgtgaaaacgtcggaacattagtcctggtcttagtttgtagaacaggaatgactttgcctagtcttctctcatggcctttcatcttcccagaatccttgttaagaacatcctgtttgtttgatgaggtggaaacaaccagagatctcatttcacaacttgacttgtgtgaaccaccatttctgcaggataactccatattaggagtctctgaatggtctgagatccgagagaatacagacgtagggttctcactgtcaggcatatttttatcagagacagtctgttgaaagttattgtttgaagaagagagctggggcccattccaggcagagttattggggctgatcccttcagattcagtacaaagtttgctttcatttgggctaagaccatcttctctcatctcttctccaagggaagagagtttttcagtatctttggacgaatcagtctcgtccttatcaagcagagcatcacaaactgttggattaaatggtgcaacagttacttttataagattcttttctagtacagagcgtctgtttaatggtttagtatgagctggtccatgaccacttgatgtacttagctgaggtagtttgaagaggtcaggagtctcagctactggtcccaggctgtacgatgaatttttctctcggggagtatcaagtagaatttgactccctctttctcccttctcaacatgcccaccatcatcttccccagaagactgctcatatgatgggtcatcttccttcaacagtgcatcaatctcttcctctgtgtaatttacatcaccatcatcttcttctccctctgacagctccagcaaggagtcatccaatccatcctcatccaaggaatcccaagaaaatggggcaccgtctttaggcaagagagaggtaccagaagactgttcagagggcacccgtgagcacatcattttgtgtggagctgctggagcaatctctgcctttgccacgagaccaaatggaaaaaggtttcagttcctgctagctgttcctttcaggagacttgtcaaaatgattgactcccaccttcctcttgcgtccagttgtcttgtgttggagccaaactttgaatccaggactcccattccacccccctattaagtgccagacgtggtgcttagtcgctggggatacgtcaagggcctgccagagcttgtctgaaggggatcagacgttaaaaatgacccattacggttcaagtaagtactggaagatgctatactgggagctttaaagggaaagagag

SEQ ID NO: 10412 - RNA, 3952 nt, Homo sapiens
  source 1..3952: mol_type = other RNA
ccgccttctctcctcccccagtccaacagatttaattaagctgctaaagctttggaaaaacagaattatttgagctaagaggaaatgtgattgtcacattttctagttaacctgtcactcatttgatttggcaaaggcagtgctcctattacacattcagtcttaaaaccccatgtaccaggagggcacgagtcttagatttttgcctaggcaaaatcctgtcccttcactccttgggttttctgtagggaactagactacagttccctactgtagctgcaatgctagctattccaactacatttaattttaactatgctatggtcccaaaggtggatgtttggcatgtctcactccatcaacctaatttagggcagcctggagaagtgaccgatgtagtaaatgccaagtaggctaactaaaataatagatttcaactactgcctttgaatagaacttctcctttgcattttggccccagaatttaaaacaaatgttcaaggaaaagcaaatccttgactggataaaaacagtaaacacttagggacattcacctaaatttattgttggcttaaatgaccaagcgttccccacgtccgtttctaaagtggggtaggatgtttagaatgcattactcacacagaaagatgggattgatgaaatcacaaaactaaacacaggctatagcaactatgaacagccttcacagagaatgaacaatagcacaaatgccagactgcaacacttcctaaaatgatgtctatagctatctgtaaagagagaataaccggccaggtgcagtggctcatgcctgtaatcccagcactttaggaggccgaggtgggcagatcacctgaggtcaggagttcaagaccagcctgaccaacatggagaaatcctgtctctactaaaaaatatgaaattagccaggcatggtggcgcatgcctgtaatcacagctactcaggaggctaagacaggagaatcccttgaacccaggaggcggaggttgtggtgagtggagatacgccattgcactccagcctgggcaacaacagcgaaactccgtctcaaaaaaaaaagagagaataaccaactcctaagacatccattaagacagacgcacagtctgtcaactttggttagaataccaaaccttaagatcaggtaatgcttttgtgcataggctgtcacaactatattacatccacgttagcatccatgtgaaactaggtatcaggggcttgaccaaatgagatggtaacatccagggcctaaagacacctcttgttaactaatatggagaaaaaagagtgcctttccacactctcccacagaatggaggctccctaactaacactcaaatttggggttcagcaaatgaaactaaatatcaactgacaccacaatagcactagcctgccctagagtcaagactctgggtgggcagctcttcaataaagacagcaaggaggccatcctgaagaggtatatccacgtctaacaggttacaagaatactgccactagaatcctaaagagcagagtggtcactggggggtaaaaagaaaaaggaaaatccttgaagaaaggcaaaggagacaaccagtctcaagaccacaaggtattataagtcttctgtcaaagtaagatgtataagatttgtaaacactattgtgcaaaataagttcaataaggaatgaaaaaatcccccccacccacaaaaaaaaatcaaggcagctagtacctacagaagggagaggagaggatttactattttaatttgtcctttcaataggattcttctcctgctccatcctacttataatgtcctggattgccaactttaaaatactgacaggtattcagaggattcaaataaaaaagtaagaggggttgttaaaagtaacttatatccattcacaagttatctaacactggctcacagcctggtaaagaatctcttccttatggaagattgaacaatgatttctttgaggtaccagaaagtagactttgcctctgcagagaggtgggtcttttgcttgaacctgggtgttctggcttaatgctggctttcaggaggcagctaccttcaatttaaattaaaaaaacaaaaaaaaactataccaaccgaacgcttgcttaaacacagacacacacacacaaaatcaggagggacttcatacaaaaaaattcaagtcggcaatgggcatttccaaaaggtgacgagttttttaaataaaaattttgtgaaaaataaaatccaaaatcggcaaagcacaaaacagcaaaagaacatgaaatgctgctccaagcaggaccctggatagggaccttcattgctgatgggatgacacaaattaactgtacgagaagtctgggagacgctggaaccgatggtggcttcgcatgttcctgtcaacccactgagtcagactgtatctttgcagatgtttctgtcggcgggcgtagtttcgcgtggtgaggtccgaaggatgctgccattttgagtgctgcatatgatgaacttgatccatcaaggcacaaagctcccccgagataccttggttagtgtcctctgggtcttctatatgagcaatgacactcctgagataaagctgcttctgctgttctagatttgactgtgaaaacgtcggaacattagtcctggtcttagtttgtagaacaggaatgactttgcctagtcttctctcatggcctttcatcttcccagaatccttgttaagaacatcctgtttgtttgatgaggtggaaacaaccagagatctcatttcacaacttgacttgtgtgaaccaccatttctgcaggataactccatattaggagtctctgaatggtctgagatccgagagaatacagacgtagggttctcactgtcaggcatatttttatcagagacagtctgttgaaagttattgtttgaagaagagagctggggcccattccaggcagagttattggggctgatcccttcagattcagtacaaagtttgctttcatttgggctaagaccatcttctctcatctcttctccaagggaagagagtttttcagtatctttggacgaatcagtctcgtccttatcaagcagagcatcacaaactgttggattaaatggtgcaacagttacttttataagattcttttctagtacagagcgtctgtttaatggtttagtatgagctggtccatgaccacttgatgtacttagctgaggtagtttgaagaggtcaggagtctcagctactggtcccaggctgtacgatgaatttttctctcggggagtatcaagtagaatttgactccctctttctcccttctcaacatgcccaccatcatcttccccagaagactgctcatatgatgggtcatcttccttcaacagtgcatcaatctcttcctctgtgtaatttacatcaccatcatcttcttctccctctgacagctccagcaaggagtcatccaatccatcctcatccaaggaatcccaagaaaatggggcaccgtctttaggcaagagagaggtaccagaagactgttcagagggcacccgtgagcacatcattttgtgtggagctgctggagcaatctctgcctttgccacgagaccaaatggaaaaaggtttcagttcctgctagctgttcctttcaggagacttgtcaaaatgattgactcccaccttcctgatagggttgtggcaagaattaaatgagatcgtgaacataaatgtggcacactagaggcatggcataagagacaaataactggtggccatagttattatttcaccccaccaccatcattgccccgatccctggagtcttaagagaagcatagggccaggcgcagaggctgattcctgtaatcccagcactttgggaggctgaggtgggtggatcacctgaggtcaggagttcaagaccagcct

SEQ ID NO: 10413 - RNA, 800 nt, Homo sapiens
  source 1..800: mol_type = other RNA
ccggcatgtccagggcaccgggccctaaacttgtctctagctgtgattttacaaaaacgtcaaaagatgttcacagcagcaccactcataatacacgaaaggtggagagagcccaaatatccatcaactaatgaatggataaagaaaatgttgtaaatccacacaatggaatattattcaaccataaaaaggattgaagtaccaacacatgccacagtgtggccgcactgtgaaaacactatgctaagtgaaagaagacaaacacaaaaagtcacaatagtgtgggattccatttacatgaaatatccagaataggtaaatccatagagacagcagaccaggggtggggggaggaggaaatggggagtgatggtttatagatatggggttttatttaggtgtgatgagaatgttttggaattagatggagatggtggctgcagaatctcgtaaatgtgctaaaatgccactgaattggtcacattaaaatggttaattttatatcatgtaaatttcacaaaaaatttttaggtatcatcaattgttattaatgaatggaagaagaaactaaggtgatggtcaggttctcctggtggtcattcaagggccagcactcgctcggggtcgggagcatctccttgctcagcgggacctccctgactgacacctttgccccaagacatcctgtgttctgtttgctggtttagcactttaaaatacatttgttaaattttactatggtaagaacatgtaacatgagatctacccttgtaacaatcttttttttttagatggagtct

SEQ ID NO: 10414 - RNA, 1149 nt, Homo sapiens
  source 1..1149: mol_type = other RNA
ccgggagaaggaggtggcctggaccagagccgcctccaggctggcccgaaccttctgctcattagccagttcctgctgtagccgctgcaaatccacctgctgctgctccagctgcaggctcagctggtctctctggctcctgcagctgcagggatctctgctccaactggctcagcaggaggcgcagctcctcggcctccttggtgtcctgctgctgctcctggcacttcttagtcagcatgaggatgatcttctggtggcctcttttgtgcctggccatgaccttctgggtgttctccagcagctccagctgtttgcacagattgttctgtcttcccttgagctgctcattctcctgcagcagcttcatgccttgctgggagaccctggccatctgcagggtaatgccgttgttctctttgatggcccgcttggttgtctcccacatccggttcgtggtcaccttgtggaactcattggccacgaggttcacgcgctggatgatctctttcctcagtctgtccttgtccagcaccgacttcttctccaggttgtatgcatagtccctgaactcattctcctgcttccgcacctgctcctccagcaatgtgaacttgtccgtgacctcctctttctgcagccggaactcctccagggctgccagcttccccccaaggatgatgttctccgtggtgagctggtccttggtctcctggaactcgtggcgcacctgggccagctgcgcctcgaaggcatccttctccatctctttggctagctgcaagttctggagctgctcgttgaggtctgtgatctcatccacctgctggttgagcgtgcgcttgaggaaggccacaatctccttcttgttattggccagctgctcaaactcctggcggaacatcttctcctgcacagccagctcatcccacttccgctggtaccgggctagccggtcctccaggtctcggatctggatgtggtagaactccttcatctccttggccagaggcggctccacggccaccaccggctccttcttgccccctttcttcttgacttcaagctccttgcctgccttgctcacactctttttgggagccatggctgatggcaaccagggctccaggccccaggaagaggccaggt

SEQ ID NO: 10415 - RNA, 1169 nt, Homo sapiens
  source 1..1169: mol_type = other RNA
ccgggagaaggaggtggcctggaccagagccgcctccaggctggcccgaaccttctgctcattagccagttcctgctgtagccgctgcaaatccacctgctgctgctccagctgcaggctcagctggtctctctggctcttcagtgcctggttatccacctgcagctgcagggatctctgctccaactggctcagcaggaggcgcagctcctcggcctccttggtgtcctgctgctgctcctggcacttcttagtcagcatgaggatgatcttctggtggcctcttttgtgcctggccatgaccttctgggtgttctccagcagctccagctgtttgcacagattgttctgtcttcccttgagctgctcattctcctgcagcagcttcatgccttgctgggagaccctggccatctgcagggtaatgccgttgttctctttgatggcccgcttggttgtctcccacatccggttcgtggtcaccttgtggaactcattggccacgaggttcacgcgctggatgatctctttcctcagtctgtccttgtccagcaccgacttcttctccaggttgtatgcatagtccctgaactcattctcctgcttccgcacctgctcctccagcaatgtgaacttgtccgtgacctcctctttctgcagccggaactcctccagggctgccagcttccccccaaggatgatgttctccgtggtgagctggtccttggtctcctggaactcgtggcgcacctgggccagctgcgcctcgaaggcatccttctccatctctttggctagctgcaagttctggagctgctcgttgaggtctgtgatctcatccacctgctggttgagcgtgcgcttgaggaaggccacaatctccttcttgttattggccagctgctcaaactcctggcggaacatcttctcctgcacagccagctcatcccacttccgctggtaccgggctagccggtcctccaggtctcggatctggatgtggtagaactccttcatctccttggccagaggcggctccacggccaccaccggctccttcttgccccctttcttcttgacttcaagctccttgcctgccttgctcacactctttttgggagccatggctgatggcaaccagggctccaggccccaggaagaggccaggt

SEQ ID NO: 10416 - RNA, 115 nt, Homo sapiens
  source 1..115: mol_type = other RNA
ccgggagaaggaggtggcctggccccaactcagctctggggcctgacagatcctcagaggcccaggagccataggaatgacctcagggagcaaactcaacaccttcaattcacag

SEQ ID NO: 10417 - RNA, 117 nt, Homo sapiens
  source 1..117: mol_type = other RNA
ccgggagaaggaggtggcctggccccaactcagctctggggcctgacagatcctcagaggcccaggagccataggaatgacctcagggagcaaactcaacaccttcaattcacaggt

SEQ ID NO: 10418 - RNA, 181 nt, Homo sapiens
  source 1..181: mol_type = other RNA
ccgtcgccgccacccgagccgccaggacgccggaagccggacgcccgagaggggcgcgcggggccaggtgcggacgcaggaaggggcctggccgcccgcagctcctaccgcgcgctgccccagatttatcggctgggaccgagtgctgggtgcgcgcgcctagcgcccgcggttcccagct

SEQ ID NO: 10419 - RNA, 9141 nt, Homo sapiens
  source 1..9141: mol_type = other RNA
cctcaccaccccttctgcctgcagtcctgtgtgaagcccctcacctatgccatctccataagcaccctaggcactgactacgtgcacaagtttgtgggcaaagagccaagtggcctgcgctacaacaagctctccctcaatgaggaaggtgagcactaccaaggctcagaccgtacttacagctgtccccttctccttatccccaccccatctcccagccttttttgtttctctgcccttcctgattagccctgtcatgcctttctccctagcagtctttcttgtctaacccacaaagtgagcgggctgtcagggaggctttgttcagtggctaagactcttggtggtttgtatttccccaggaatcccccataaccccatggtcaatgctggtgccattgttgtcagctccctgatcaaggtcagtgccaccttaaccttctgataggtattatcctctaagctcctgtgttcctgtatccctcatatttgttcagctctccagggagactggtggggctctgattcctttgagggtccccagaaggcacatgaggcacagcagggacccacatgttatgctgacaatgtcagtataagagactgcaccacctccgtcatccccactcagtactgttccctgcccccacccatgagtctagagcctagagctttctgacccttagagaagtgagcaggtcctgacccctgcctaggaccaagggccaaatgccagagacaaggggaggacagcactattgggcactgattggccacttctgggtgtgggacacctgcaggcaagggtgaatggccaggccagggcagttattcacgtcacctggaactgtgagttggccttgaacagggtgtcagactagcccatcagctgtaggtctcccagggcttgagcaagaacctgggagcagctgggcagcaacaccctggagccaatcacagcccctcctggggaaggtggtgttaggaatcctcccctcagggactcaggtatcagagtccctgtggtattgactctgtagttgacacatgagtaagcaatgagtctgggtgaggaaaagaggctgagtctctccccttgttctgtgatggctccatctacaaacctgtatctgggacctgcctcatcccattcccatctaagtaggaccttttttaaaaaatatagaggccaggcgcggtggctcacgcctgtaatcccaacactttgggaggccgaggtgggcaaatcacgaggtcaggagatcgagaccatcctggctagcacggtgaaaccccgtctctactaaaaatacaaaaaattagccaggcttggtggtgggcacctgtggtcccagctgctcgggaggctaaggcaggagaatggtatgaacccgggaggcggagcttgcagttgagccgagatcctgccactgcactccagcctgggcgacagagcaagactccatctcaaaaaaaaaaaaaaaaaaaaattgaggcagggtctctcctatgttgcctaggctggtctcaaacccctggtctcaagcgatcctcctgcctcagccccccaaattgctgagattacaggcatgaaccatcatgctggccaatgggatggagtaaagctccagcatggggtgtaaggaatggggatggagatcagggatagggtggggctaggagacaggattcgagtcaggaaaatgaacgtgggagtcagggatgagggtttggattgagaatggaagtgggatggcccagcaagctggctcatgcctgtaatccgagctacttggaggctgaagtgggaggatcgcttgagcctgggaggtcaaagctgcagtgagccatgatcgtgccactgcactccagcctgggtgacaagggtgacaaagcaagactgtctcaaaaaaaagaaagagaaagagaggagccaatggaagtgcggtgttttcagaaggataaaaaaagggccattataaaattgaacacatttgcagcagcaggaccagactaacactagaactccactagatccttctgacccttccctctgtcatcctcctacacttagaatgctgacatctctctctttctctgcagatggactgtaacaaagcagagaagtttgattttgtaagttcccttgctacttagcccctggctgcatttcgccatggcatgctgtcctctccagctgccccagtggctctctaaccccactaccaggtgcaccagcccatactagaagccttatttccagaaatgtggaaatctgctggcctcagagaggaaagcctcttgacaagacctgagttcagaagggctagtcaacctgtgaggtattaatagagcttcttaaccaagtggagcctcaatgtccctttttctcttccaggtgttgcagtatctcaacaaaatggctgggaatgaatacatgggtttcagcaatgccacgtaagtccctactcagaggactgactgaaagcattgtggtgtatgtgtgtgtacttaggatggggacaagaggaatgggggagagagaatcttaggaggaagaaatcccaggggaactttggccctccagcttcctctgagtcccttcataaacatttgtttatcttgtaaaataatttgttccatttctaattagtacataatgagagaggcagtgtgatggtttgtgcctaagccctttcttgccaagactttcaaagccaaaaacttcaccagttttcctagatgactagacagtttggggtgtttggtttgggtttactttataacaaaactatgctgagtgtttgctcaggttcagaaatttcctctaatattactgtgagaagttataaaggggttcatttagtttgtggtgtgatgtagttctgtctctccagggaaggtaatttttccccttctcccaacacccactcctccaacttcaagtactaaattgggtgtttgcttcagattccagtcagagaaggaaacaggggatcggaattatgccatcggctattatctcaaggaaaagaaggtaaccagaagaggccggaagagaaagtccctgggaattctgctgctagtggaagggcagtaggggttgggggcttcagctgagaccctgacagtgtgaaagggctgatgtcctgaagagaaatgctctcccctctcttccttgcagtgctttcctaagggggtggacatgatggctgcccttgatctctacttccaggtaagaaaacactgctcagggccgagggaacaggacagactgtccttgcccttgccctttccctacacccgagggtcccatgtgcaggttcacgtcacatcttcacctattctttgttttcatagctgtgttctgtggaggtcacttgtgaatcaggcagtgtcatggcagccaccctcgccaacggtgggatctgccccatcacaggcgagagtgtgctgagtgctgaagcagtgcgcaacaccctcagcctcatgcattcctgcggcatgtatgacttctctggccagtttgccttccacgtgagtttctggctctgctatccatctgtcatgagcccagtgctaagaagagagaacactgactctctcaagatagaggtggaagcttgttcctgcctctcattcactaacttccaggaaggcaattaggttgagactccttagacgagtttctcaaaaacaccaagttcctcgaatatataaagagatgtctttgggaggccgaggcaggtggatcacctgaggtcaggagttcgagaccagcctgacctacatggtgaaaccccatctctactaaatacaaaaaattagccgggggtggtggtgtgcacctgtaatcccagctacttgggaggctgaggcagaagtgcttgaacctgggaggcagaggttgcactgagccgagattgtgccattgcactgtagcctgggcaacaagagcaaaactccatctcaaaaaaaaagaaaaaaagaaaaagaaaaacaaccagaggtgttgcagctcctgaattgtgcttcacattgctggctcttctccttggggtctcagcttagatgtcatttccaaagaaagacttttctgaccaccctatctcatgtggcccccctctacctctatttacagcaccctacttctcactatttatcacaattactttaaacattacgtgtctatttatttacctgtttattacctatctcctaacaccagaatggaagttcctagttctagcacagcatctagcacagaatgctgtaagtatttcaaaaaatattttctagctgaatcaatgaatttaagggaaggaaaggacaggagtaataaaagaagctaattaacaagccaaaaggttgaggtggattgtggtcatgcagtcatttgtaaacttgttaagagtacagcctaacttgtttattttctgatttggggcacacccactttatcctcagcttcagttctgttccccaggtgggcctgccagccaagtcagctgtatcaggagccatcctcctggtggtacccaatgtcatgggaatgatgtgcctgtcacccccattggacaagctggggaacagccatagggggaccagcttctgccaggtgagatgctttgcatatagtacttactatttttgaagcaataaatttgtttaatggtaccacttttactataataaagcaattttgagctcctactaagtgtaaggagtaaataaacaatatatttggcttacaattctagaagttggtgtctctcttcaatttccacaactatgacaacctgaggcactgtgctcggaagttagacccacggcgtgaaggggcagaaattcgggtaaggaaaactccaggtggcttgtaagaatatttcaaaggccaggtgcggtggctcacgcctgtaatccctgcactttgagaggccaaggcgggcggatcacaaggtcaggagatcaagaccatcctggctaacacggtgaaacctggtctctattgaaaatacaaaaaattagccagacgtggtggcacgcgcctgtggtcccagctacttgggaggctgaggcaggagaatcgcttgaaaccgggaggcagaggttgcagtgagccaagaccgcgcgccactacacttcagcctgaacgacagagcgagactccgtctcaaaaaaaaaaaaaaaaaaaagaatatttcagagtagcacattccataacacttcagcaatacccttggactaagcatccatggaggagggtcacagggcacagctggcataggtgagttcaattaatgtcatgtgggtatgatttgtgttccagaacaagactgtggtcaacctgttatttgctgcctatagtggcgatgtctcagctcttcgaaggtaatgctactgtgaccaaatatacacaataaaatactcctggtcagagattttactaggaggcagcgtaacaaaatagttaagtgcttcagctttggaattagaatggatatagattgcatttaaatgaaatttttttaaaaaaggagattttttttaaaaaaagtaaactgtctgctctatgataattaatgttagccattgttattgagtgttaagagcagtgtcctaggaagtaggtaccctgcctcaaatgggcacttaccacaggtaggcagtgagtgatatttctggaaggatcacattcccatctctctaatatgagtataacagtctcatctggatatggaaaaaagattattcagagccaacaaatctggctataggctgtttcactttctctgaaactcatccagtctgacaccagttcacaaagaacacctgtgattccagtctgatctaggcaactctagctgctttcccactaccctcaggtttgccttgtcagccatggatatggaacagaaagactatgactcgcgcacagctctgcatgttgctgcagctgaaggtactgaagggttaaggaggggaggaggagggtaatcataagaccctttctttttcaccaaaagtaccttcattatatgtgccctcaaggttataggggcagcaactagttttatctagacacccttcggtttgcagctagactatgactgagtgctgcagggtacaaaatgggaagaggccttttcccctcccctcttggtaaagacttcagtggctaagtgtctgcaccaaagggttcaagacctgcgccttctcattttccttctgcccatattcctaggacacatcgaagttgttaaattcctgatcgaggcttgcaaagtgaatccttttgccaaggacaggtgaggaataggctaaaagtggaggagggtgggcacagcttctccacctaccctccagccaccatgcaaatatatacaaccaccactctccacgtctcctttgcctgatcatatcattattcctctcaggtggggcaacattcccctggatgatgctgtgcagttcaaccatctggaggtggtcaaactgcttcaagattaccaggactcctacacactctctgaaactcaggctgaggcagcagctgaggccctgtccaaagagaacttagaaagcatggtatgagcacaggtcatggacagcccctgctcaagaaaaagcatgagctggccacacatgtaatccataaccaccaaaaatactatggagagctacactgcttcagtggggaccaagcagtcatttggtgacttaggctagtgctttctatgggagtcaaaataccccattccctcagcagacagagtacagagaagggcctcagaggacacctgcagtacagctatccagagagactgggcttcaaggtacagcctaatggcttgccccactcaaaaccatcccagctcttcacccaggtctcctcttcctctccctgaagaaaccatcatgagagagatactctggtggagggactctagctaccatgcacatgtacatatccacagaatatgggaagtgggaatggctatatacatggctttagtagtctggagaaatctactccccttggccaggacatgctgctgctactgctaacagccaattttatagacagagaaagtattttgtgttcaaataaactttaattaccaaatcatttttgctaaacccagtccttctttcttccctaggggtatctagcttcatcaccatcatagaaggtagaaaaagatggaatcacagggtcaaagcacagcttctctacctaccctaccaaacagtacatattcacttaccccaccaggtttttctcaactccaaatactgctttaggttaagtgtattctgctgccaagggaagcataggtttgagtctaaacaggctctgaaacagattgtgcaaaacctcaggcctccttccttcctcgggaagttccaactgtggcagaaatgaagatggaacttctcaagaataaacagttttggccgggtgtggtggctcacgcctgaaatcccagcactttgggaggccaaggtgggctgatcacatgaggccaggagttcgagaccagcctggccaatatggcaaaaccccatctctactaaaaatataaaaatgagacgggcatggtggcacacacctgtaatcctagctactcaggaggctgaggcacgagagtcgcttgaacccaaaaggcagagtttgcagtgagccaagatcatgccactgcactccagcctgggtgacagagtgagactctgtctcaaaaataaataaatagtttctagcactcatcccctagatatcccccaagtgtctctcttcccctttggtcaaggttataactgggataatgattatgacagactggctgggtgtcagaggtacagatttaaggtagatggactcagggtaaggatagctacagctgtgtggggctgaaggtctgtggcactgagctactggggaaggagggctctgttttcattttgacacactgagttaataaagcacttactgagggagccagagcccaaactctaaatgtgctgtagaaaaagggccaagtcattgactgcaccactccttcagccagaggtagaaaggatttactcttcagccatctggtagagccccaagaacaagttacatgtggacaaagggagggagaggtatcatggtgattaataaattcaaacaaagctgaatgataagaccccaggatggaatacagtctgagaaaggcctgggcaaagggaggcagagggactgaaggaagcaggtcaaggaagatacacccatggtagcctaggaaattggcagtagttggtgggtggggaaaaggagggtttggctgtatgcctagctttcacaaggtaggggatgaggaagatgatcatgatattgcacagaggacccaacactgaattgtgggagctagaggttgcttgaggcaaagtaaaaaggcttcggacactttcaaaaggaggctggccaaaggcgtgattagggactccagtaatggacatactagaggccctcgggcacctcaagccctgaatgggtcagcagctccccatcccagagagcaaaggcaggcaccactggaccccggaaatctgtctgtagcgtgtgaaccacagagacctggctcacatccaccaggctcagcttctgggcctcatactccagcaacagccccaccttctctggctgcccaataccctcaactggggctttctcgttggccaacatggtgtaccacttgcgctgggcataggtgaacacccaggaacgatcatcaacaccaatgcagctatcccgggacatgtccacatctgccactcctatccggaactgctgggagcgcttcactgtcacttcccagtagtgtctgccactggtgaccgctgtgtctgccagcaccactgcccactcccggaagcgctccacattcaaggccaccttggtgggctccaatcccaccaagccatatttgacacccgtatcatctctgaagagtgccaggctgctgtgggcggttttttcttccagtttgaaactgacgcctctctgggcctctgtggaggcaactcccaatcgtttggctccccagcggcacaagcgcaaagaacgtgcaaaaagcagcgccatcttgcgccttggat

SEQ ID NO: 10420 - RNA, 3452 nt, Homo sapiens
  source 1..3452: mol_type = other RNA
cctcaccaccccttctgcctgcatcccaagaaaaccagtctctgggagcttcaccggggccttccaaggagacttgagttcagtcttaaagaagggggcaggccttggggaccggcacccctgaaatctgggcagagagagagcagtgggcgggaggttgagcatgttccactctgaggacagtcagggacctgtggaagccagagctggcccaggccacaccatgacgggcatcttgagaaacagcctctgcagattcagggccttgtgtaaatgtgccctggaggtgccacccagtcacagaaggcagtacagtgtggcagaaggcagtacagtctggctctagagcccaacttcccagattcaaatcctagctcatcactttcatgctgtgtgacctcaggaaggcaacttcactcctctgagcctctggttcctcatctgtgcactggggcgatgatgctgtgtggtgattgtaaggagttagtgtgcatgcaagtctagtggcacctggacacaaaacttaagcagtgaggaccggcatctttttcccctttccaaactgctaagacggaccccggctgaggcaggagggagagtgcagctcgctgtggccagaaatccagcctttgctccttaatcagacactaatgggcatatctatcttcattgttatttgagagatgctggtaaaaaaaaagctgatgaagaaaccacaggagaccaagatggggcaaccccgaggaagtcactgtaatctgcaatgcagagtggtcgaggcctccaatgccctggaccatctactgctctgacactgaaaagggagagaggcttgaaaactgaatttaaccgacatttatgttagggctggaggctgaggggcctccatagggaaaactgcagccagaagcacccggtgcctgggatgctggagtcctcttcagggctagaagccatcctttttcctcctgccttctcctcccttcaccgcagcaaacacagaaccctgtctcccgactgccatctccatgggccatttggaggccagggagctgcctcctgtatctttacaggggtcaggccctcctagggatgtggggccagagggaagatttgagcatgtggggcagagtgactccatgaggacgtcaagcaaccccgccatggctctgggcttctcgccttgggttttctcatggagacatccatctgttaaagatcttgcttatggggcagacctggggtttgatggagagagacttgctggagacagagccattcacgcacaccgcggctaactccccagcccagcctccaccctgccagtgattccaggaattccagacaggtggtccatgtcccttctccctcattgtcaagggtcaggttcttttgcactcgtgacctccccttaagctgatgcactggcagatgatatacggtggcagtgacagatgtgatcggtaagaactggcagccatgagcaggcactgtctggagccaggctagtaatcctattaacatggcggcttccagggaagagtgccgcttctggacaactaagatgtccctttgcctgtcatcaagaacactcatttctcctgagaccacagcggcaagtccagctttcttgtaattgtctctaaatatacacgagagcttcctaaccagctttttaagtttctccactacagagggtgttattgacacaattcttctgtttttgcagtgtataaagtgaggagaaagcctctctgggcctagaggtgagtgagcccccttctgggacctttcccactctatctgcactgggatgctgccttgggaaggtgtggggggtgggggtgggggtggttcctgtgcaataagatttcctaatgaagaaagaaaagtgtgcccttctctctggtttttacttggaagcttccttgcttgccaggaccccagatgctgatatttcagaatttaaggaagtggcttgggcagaagcactttcacagcttcaggagaatgcacggtatccacactgaatgtaaaggacgggtatctgagcagcctgccaatctcgcacccaccttcaagatgcctggacattctcctgagggcagcttctcagcaacctcctcagggaagtgcttagttggggcagagagctcagtgagctgagagtgaggacacatctttctgttccgactcctccacaaacctgcctggtgaccacaggcaaatcacccccctttctgacccatccgttgaataattcagtggatgtgaatcttgttcatctttaaaattccacgattcctcagagaagaaacagcattctcacgtgggtggcctgaagagtccactgcctggcacatctagctcttaaagacatcctctcctcttcttaaaaagaagagaaagtccgaccaggagataaaaaccaccaacaacacccccagaaaccccacctattaccagtaaccccccatccctgggtctcccaatgcacttgggtcttggaagggaccaggtgtctggtggcaaaggtgccatttcaaagtcaaactaggaacatccaatggccctactagatggccaagggactgaatgtgaaaccagaattgggtcaggaacactgaagttctgagggctgctcttgccccagcaccccacgccctaggttcgataagtttgcataaaaacaagacacacgagtgattatttaccaccagcaagcgatcatcaaatcatgtctatgttttaaacttaactagctgtctcatctggtcccatgttcctggaatgtagtttcaaggatccccaatctgccctctgaaggccttgccccgtcatgcctctaggggcaggaggcccatacttccatgtcttctgactcagcttgaccacaacatgggatatttgaaatcagggctgctggggagaaattccagaaggacggccgccgcccctggtcaaaactcctggttctagaacacaggagaagccaaaggccgacagcaagtcagagctacgtgccaagcctcaccccatggtggtgcagggtgtgccgtcctcagaaggtgaaggcatacaccacgcccaccaccacgatgttccccagcgtagctatgatggcaatccatagcaagacggcgtcgttggaggaccgaggaggatcttccggctggccctggccattggcagccgcgtggacattggcagaggagttaaacagggagtactcggtgctgaagtcctcgttgggcgagtccatgaaagctccccccatcatgggcagctgcgcggccataaaggagagatccatggtgtcgctgcagccagcgctcgagtcctcgctgctgccgctgccgctgcgggtcagccgcctgcacagttggcggggatcgggctgagcagcgagcgtccggagaccgcacggcgcactcggctgtctctgggcttct

SEQ ID NO: 10421 - RNA, 3551 nt, Homo sapiens
  source 1..3551: mol_type = other RNA
cctcaccaccccttctgcctgcatcccaagaaaaccagtctctgggagcttcaccggggccttccaaggagacttgagttcagtcttaaagaagggggcaggccttggggaccggcacccctgaaatctgggcagagagagagcagtgggcgggaggttgagcatgttccactctgaggacagtcagggacctgtggaagccagagctggcccaggccacaccatgacgggcatcttgagaaacagcctctgcagattcagggccttgtgtaaatgtgccctggaggtgccacccagtcacagaaggcagtacagtgtggcagaaggcagtacagtctggctctagagcccaacttcccagattcaaatcctagctcatcactttcatgctgtgtgacctcaggaaggcaacttcactcctctgagcctctggttcctcatctgtgcactggggcgatgatgctgtgtggtgattgtaaggagttagtgtgcatgcaagtctagtggcacctggacacaaaacttaagcagtgaggaccggcatctttttcccctttccaaactgctaagacggaccccggctgaggcaggagggagagtgcagctcgctgtggccagaaatccagcctttgctccttaatcagacactaatgggcatatctatcttcattgttatttgagagatgctggtaaaaaaaaagctgatgaagaaaccacaggagaccaagatggggcaaccccgaggaagtcactgtaatctgcaatgcagagtggtcgaggcctccaatgccctggaccatctactgctctgacactgaaaagggagagaggcttgaaaactgaatttaaccgacatttatgttagggctggaggctgaggggcctccatagggaaaactgcagccagaagcacccggtgcctgggatgctggagtcctcttcagggctagaagccatcctttttcctcctgccttctcctcccttcaccgcagcaaacacagaaccctgtctcccgactgccatctccatgggccatttggaggccagggagctgcctcctgtatctttacaggggtcaggccctcctagggatgtggggccagagggaagatttgagcatgtggggcagagtgactccatgaggacgtcaagcaaccccgccatggctctgggcttctcgccttgggttttctcatggagacatccatctgttaaagatcttgcttatggggcagacctggggtttgatggagagagacttgctggagacagagccattcacgcacaccgcggctaactccccagcccagcctccaccctgccagtgattccaggaattccagacaggtggtccatgtcccttctccctcattgtcaagggtcaggttcttttgcactcgtgacctccccttaagctgatgcactggcagatgatatacggtggcagtgacagatgtgatcggtaagaactggcagccatgagcaggcactgtctggagccaggctagtaatcctattaacatggcggcttccagggaagagtgccgcttctggacaactaagatgtccctttgcctgtcatcaagaacactcatttctcctgagaccacagcggcaagtccagctttcttgtaattgtctctaaatatacacgagagcttcctaaccagctttttaagtttctccactacagagggtgttattgacacaattcttctgtttttgcagtgtataaagtgaggagaaagcctctctgggcctagaggtgagtgagcccccttctgggacctttcccactctatctgcactgggatgctgccttgggaaggtgtggggggtgggggtgggggtggttcctgtgcaataagatttcctaatgaagaaagaaaagtgtgcccttctctctggtttttacttggaagcttccttgcttgccaggaccccagatgctgatatttcagaatttaaggaagtggcttgggcagaagcactttcacagcttcaggagaatgcacggtatccacactgaatgtaaaggacgggtatctgagcagcctgccaatctcgcacccaccttcaagatgcctggacattctcctgagggcagcttctcagcaacctcctcagggaagtgcttagttggggcagagagctcagtgagctgagagtgaggacacatctttctgttccgactcctccacaaacctgcctggtgaccacaggcaaatcacccccctttctgacccatccgttgaataattcagtggatgtgaatcttgttcatctttaaaattccacgattcctcagagaagaaacagcattctcacgtgggtggcctgaagagtccactgcctggcacatctagctcttaaagacatcctctcctcttcttaaaaagaagagaaagtccgaccaggagataaaaaccaccaacaacacccccagaaaccccacctattaccagtaaccccccatccctgggtctcccaatgcacttgggtcttggaagggaccaggtgtctggtggcaaaggtgccatttcaaagtcaaactaggaacatccaatggccctactagatggccaagggactgaatgtgaaaccagaattgggtcaggaacactgaagttctgagggctgctcttgccccagcaccccacgccctaggttcgataagtttgcataaaaacaagacacacgagtgattatttaccaccagcaagcgatcatcaaatcatgtctatgttttaaacttaactagctgtctcatctggtcccatgttcctggaatgtagtttcaaggatccccaatctgccctctgaaggccttgccccgtcatgcctctaggggcaggaggcccatacttccatgtcttctgactcagcttgaccacaacatgggatatttgaaatcagggctgctggggagaaattccagaaggacggccgccgcccctggtcaaaactcctggttctagaacacaggagaagccaaaggccgacagcaagtcagagctacgtgccaagcctcaccccatggtggtgcagggtgtgccgtcctcagaaggtgaaggcatacaccacgcccaccaccacgatgttccccagcgtagctatgatggcaatccatagcaagacggcgtcgttggaggaccgaggaggatcttccggctggccctggccattggcagccgcgtggacattggcagaggagttaaacagggagtactcggtgctgaagtcctcgttgggcgagtccatgaaagctccccccatcatgggcagctggaagaactccaagtggcaacggcagactggaaaggagttaggctggtccatgcatgatttggcatcctcacttgttattccccaggctcacttgacctgcgcggccataaaggagagatccatggtgtcgctgcagccagcgctcgagtcctcgctgctgccgctgccgctgcgggtcagccgcctgcacagttggcggggatcgggctgagcagcgagcgtccggagaccgcacggcgcactcggctgtctctgggcttct

SEQ ID NO: 10422 - RNA, 4822 nt, Homo sapiens
  source 1..4822: mol_type = other RNA
cctcaccaccccttctgcctgcatcccaagaaaaccagtctctgggagcttcaccggggccttccaaggagacttgagttcagtcttaaagaagggggcaggccttggggaccggcacccctgaaatctgggcagagagagagcagtgggcgggaggttgagcatgttccactctgaggacagtcagggacctgtggaagccagagctggcccaggccacaccatgacgggcatcttgagaaacagcctctgcagattcagggccttgtgtaaatgtgccctggaggtgccacccagtcacagaaggcagtacagtgtggcagaaggcagtacagtctggctctagagcccaacttcccagattcaaatcctagctcatcactttcatgctgtgtgacctcaggaaggcaacttcactcctctgagcctctggttcctcatctgtgcactggggcgatgatgctgtgtggtgattgtaaggagttagtgtgcatgcaagtctagtggcacctggacacaaaacttaagcagtgaggaccggcatctttttcccctttccaaactgctaagacggaccccggctgaggcaggagggagagtgcagctcgctgtggccagaaatccagcctttgctccttaatcagacactaatgggcatatctatcttcattgttatttgagagatgctggtaaaaaaaaagctgatgaagaaaccacaggagaccaagatggggcaaccccgaggaagtcactgtaatctgcaatgcagagtggtcgaggcctccaatgccctggaccatctactgctctgacactgaaaagggagagaggcttgaaaactgaatttaaccgacatttatgttagggctggaggctgaggggcctccatagggaaaactgcagccagaagcacccggtgcctgggatgctggagtcctcttcagggctagaagccatcctttttcctcctgccttctcctcccttcaccgcagcaaacacagaaccctgtctcccgactgccatctccatgggccatttggaggccagggagctgcctcctgtatctttacaggggtcaggccctcctagggatgtggggccagagggaagatttgagcatgtggggcagagtgactccatgaggacgtcaagcaaccccgccatggctctgggcttctcgccttgggttttctcatggagacatccatctgttaaagatcttgcttatggggcagacctggggtttgatggagagagacttgctggagacagagccattcacgcacaccgcggctaactccccagcccagcctccaccctgccagtgattccaggaattccagacaggtggtccatgtcccttctccctcattgtcaagggtcaggttcttttgcactcgtgacctccccttaagctgatgcactggcagatgatatacggtggcagtgacagatgtgatcggtaagaactggcagccatgagcaggcactgtctggagccaggctagtaatcctattaacatggcggcttccagggaagagtgccgcttctggacaactaagatgtccctttgcctgtcatcaagaacactcatttctcctgagaccacagcggcaagtccagctttcttgtaattgtctctaaatatacacgagagcttcctaaccagctttttaagtttctccactacagagggtgttattgacacaattcttctgtttttgcagtgtataaagtgaggagaaagcctctctgggcctagaggtgagtgagcccccttctgggacctttcccactctatctgcactgggatgctgccttgggaaggtgtggggggtgggggtgggggtggttcctgtgcaataagatttcctaatgaagaaagaaaagtgtgcccttctctctggtttttacttggaagcttccttgcttgccaggaccccagatgctgatatttcagaatttaaggaagtggcttgggcagaagcactttcacagcttcaggagaatgcacggtatccacactgaatgtaaaggacgggtatctgagcagcctgccaatctcgcacccaccttcaagatgcctggacattctcctgagggcagcttctcagcaacctcctcagggaagtgcttagttggggcagagagctcagtgagctgagagtgaggacacatctttctgttccgactcctccacaaacctgcctggtgaccacaggcaaatcacccccctttctgacccatccgttgaataattcagtggatgtgaatcttgttcatctttaaaattccacgattcctcagagaagaaacagcattctcacgtgggtggcctgaagagtccactgcctggcacatctagctcttaaagacatcctctcctcttcttaaaaagaagagaaagtccgaccaggagataaaaaccaccaacaacacccccagaaaccccacctattaccagtaaccccccatccctgggtctcccaatgcacttgggtcttggaagggaccaggtgtctggtggcaaaggtgccatttcaaagtcaaactaggaacatccaatggccctactagatggccaagggactgaatgtgaaaccagaattgggtcaggaacactgaagttctgagggctgctcttgccccagcaccccacgccctaggttcgataagtttgcataaaaacaagacacacgagtgattatttaccaccagcaagcgatcatcaaatcatgtctatgttttaaacttaactagctgtctcatctggtcccatgttcctggaatgtagtttcaaggatccccaatctgccctctgaaggccttgccccgtcatgcctctaggggcaggaggcccatacttccatgtcttctgactcagcttgaccacaacatgggatatttgaaatcagggctgctggggagaaattccagaaggacggccgccgcccctggtcaaaactcctggttctagaacacaggagaagccaaaggccgacagcaagtcagagctacgtgccaagcctcaccccatggtggtgcagggtgtgccgtcctcagaaggtgaaggcatacaccacgcccaccaccacgatgttccccagcgtagctatgatggcaatccatagcaagacggcgtcgttggaggaccgaggaggatcttccggctggccctggccattggcagccgcgtggacattggcagaggagttaaacagggagtactcggtgctgaagtcctcgttgggcgagtccatgaaagctccccccatcatgggcagctggaagaactccaagtggcaacggcagactggaaaggagttaggctggtccatgcatgatttggcatcctcacttgttattccccaggctcacttgacctgtagagtatgtatgtatgttactcacattttgtggcatttgggagacagggagaaagagaaatgctggctggatcaggggcccatagctgggaggtaggggtaatggtctagatttagattcaagtgtcaacattccttttcccacaacgggagaaaaggaggaacggtggaaatatagctgttaaaagcacagccttatgaaaattccacatccagccaaaatggagtaatagggaatagatttaccctcccaactgaaacaactgaaaaaccagataaaatacatgaaaatgattttcaagacaccggacatcagacaatgaaggacagtgaccctcgagagatgggaaattggcaagatgagccatacaggtgctccggtttactgcctatggaaagtttccaggccatggagcagtaaactcaggcagggctcaatggactctctgagttgaagaatggaagtgagagtctgaggagagtgaggcagctggagaccacatggcagagtatggagagaagacagccgcccacagagagaaccctggggtttgagagagggaccactcaaacattcaacaaaggacagatgaatgcatgtttgtacagaaactgcctgaggcagggaaagaatcacccaaaaaattatagaaaatagtgcctggaacccatatagggccagaaatagtgcctgtttccatcacccatcttgaaaatctcatcatttatgagacactgagcaggtagaatactcagaacagcattgcctttgtgatggggaataattactcttagattaaatttggcttgatcctgcctaacaaatcttaaaaacagtacttgcaaaaatcaaactgttctcaagcatctgaactgcatcccagaacaaagcacaagaatatttatgggaatacaaaaatatctagcatacaccacagttaaattcacaatgtttggcatccaaccaagaattatcaggcatgtaaagcagcaggaaaatatgaaccatatgaggagaaaaggcaatcaatcaaaaccaatccagaattgacatatttagaattaataagtgaggacattaaaacagttgttataactgtattccatatgtccaaaaagctacaggtaacaatgaacatgttaagaagagaatggaagagatatgtttttatataaaagatccaaattagcttctagagatgaaaactataatatctagtatcaaaagtacattgggtggggctattattaatagcagattagatattgcagaagaaaaccttgttaacttgaagacatatcaataataactatccaaataaaacacaaacagaaacaaagaccaaaaaaaaaaaaaatgaagagactatcagtgagctctaagacaacttcaggtgacctaatatatgtgtattagtcccaaaagaagaggag

SEQ ID NO: 10423 - RNA, 3545 nt, Homo sapiens
  source 1..3545: mol_type = other RNA
cctcaccaccccttctgcctgcatcccaagaaaaccagtctctgggagcttcaccggggccttccaaggagacttgagttcagtcttaaagaagggggcaggccttggggaccggcacccctgaaatctgggcagagagagagcagtgggcgggaggttgagcatgttccactctgaggacagtcagggacctgtggaagccagagctggcccaggccacaccatgacgggcatcttgagaaacagcctctgcagattcagggccttgtgtaaatgtgccctggaggtgccacccagtcacagaaggcagtacagtgtggcagaaggcagtacagtctggctctagagcccaacttcccagattcaaatcctagctcatcactttcatgctgtgtgacctcaggaaggcaacttcactcctctgagcctctggttcctcatctgtgcactggggcgatgatgctgtgtggtgattgtaaggagttagtgtgcatgcaagtctagtggcacctggacacaaaacttaagcagtgaggaccggcatctttttcccctttccaaactgctaagacggaccccggctgaggcaggagggagagtgcagctcgctgtggccagaaatccagcctttgctccttaatcagacactaatgggcatatctatcttcattgttatttgagagatgctggtaaaaaaaaagctgatgaagaaaccacaggagaccaagatggggcaaccccgaggaagtcactgtaatctgcaatgcagagtggtcgaggcctccaatgccctggaccatctactgctctgacactgaaaagggagagaggcttgaaaactgaatttaaccgacatttatgttagggctggaggctgaggggcctccatagggaaaactgcagccagaagcacccggtgcctgggatgctggagtcctcttcagggctagaagccatcctttttcctcctgccttctcctcccttcaccgcagcaaacacagaaccctgtctcccgactgccatctccatgggccatttggaggccagggagctgcctcctgtatctttacaggggtcaggccctcctagggatgtggggccagagggaagatttgagcatgtggggcagagtgactccatgaggacgtcaagcaaccccgccatggctctgggcttctcgccttgggttttctcatggagacatccatctgttaaagatcttgcttatggggcagacctggggtttgatggagagagacttgctggagacagagccattcacgcacaccgcggctaactccccagcccagcctccaccctgccagtgattccaggaattccagacaggtggtccatgtcccttctccctcattgtcaagggtcaggttcttttgcactcgtgacctccccttaagctgatgcactggcagatgatatacggtggcagtgacagatgtgatcggtaagaactggcagccatgagcaggcactgtctggagccaggctagtaatcctattaacatggcggcttccagggaagagtgccgcttctggacaactaagatgtccctttgcctgtcatcaagaacactcatttctcctgagaccacagcggcaagtccagctttcttgtaattgtctctaaatatacacgagagcttcctaaccagctttttaagtttctccactacagagggtgttattgacacaattcttctgtttttgcagtgtataaagtgaggagaaagcctctctgggcctagaggtgagtgagcccccttctgggacctttcccactctatctgcactgggatgctgccttgggaaggtgtggggggtgggggtgggggtggttcctgtgcaataagatttcctaatgaagaaagaaaagtgtgcccttctctctggtttttacttggaagcttccttgcttgccaggaccccagatgctgatatttcagaatttaaggaagtggcttgggcagaagcactttcacagcttcaggagaatgcacggtatccacactgaatgtaaaggacgggtatctgagcagcctgccaatctcgcacccaccttcaagatgcctggacattctcctgagggcagcttctcagcaacctcctcagggaagtgcttagttggggcagagagctcagtgagctgagagtgaggacacatctttctgttccgactcctccacaaacctgcctggtgaccacaggcaaatcacccccctttctgacccatccgttgaataattcagtggatgtgaatcttgttcatctttaaaattccacgattcctcagagaagaaacagcattctcacgtgggtggcctgaagagtccactgcctggcacatctagctcttaaagacatcctctcctcttcttaaaaagaagagaaagtccgaccaggagataaaaaccaccaacaacacccccagaaaccccacctattaccagtaaccccccatccctgggtctcccaatgcacttgggtcttggaagggaccaggtgtctggtggcaaaggtgccatttcaaagtcaaactaggaacatccaatggccctactagatggccaagggactgaatgtgaaaccagaattgggtcaggaacactgaagttctgagggctgctcttgccccagcaccccacgccctaggttcgataagtttgcataaaaacaagacacacgagtgattatttaccaccagcaagcgatcatcaaatcatgtctatgttttaaacttaactagctgtctcatctggtcccatgttcctggaatgtagtttcaaggatccccaatctgccctctgaaggccttgccccgtcatgcctctaggggcaggaggcccatacttccatgtcttctgactcagcttgaccacaacatgggatatttgaaatcagggctgctggggagaaattccagaaggacggccgccgcccctggtcaaaactcctggttctagaacacaggagaagccaaaggccgacagcaagtcagagctacgtgccaagcctcaccccatggtggtgcagggtgtgccgtcctcagaaggtgaaggcatacaccacgcccaccaccacgatgttccccagcgtagctatgatggcaatccatagcaagacggcgtcgttggaggaccgaggaggatcttccggctggccctggccattggcagccgcgtggacattggcagaggagttaaacagggagtactcggtgctgaagtcctcgttgggcgagtccatgaaagctccccccatcatgggcagtctcccaggccaaacgcagcccttccctggagccagctctgggtcttctctagggtcacagactgatggagaaatccgggatttgtctttgttctgcgcggccataaaggagagatccatggtgtcgctgcagccagcgctcgagtcctcgctgctgccgctgccgctgcgggtcagccgcctgcacagttggcggggatcgggctgagcagcgagcgtccggagaccgcacggcgcactcggctgtctctgggcttct

SEQ ID NO: 10424 - RNA, 789 nt, Homo sapiens
  source 1..789: mol_type = other RNA
cctcaccatcccttctgcctgcgcggcctggctgggcaggagcacagggacggccctcaatccatggctcacgaaagcccactgtgggagagcatgtgtggtgcaggaagcccctttccccatgcgccagtgtgggcaaaggcgacccacgagagagcagggtgtcacccaattggggctgcattgcaccggatgcttgcctgcgtgggcgccctgccagactgtccccggtgcctggctcttcgattctgaaaccagatctgaatcctggactccgggaggcccgtctctctggccagctcttccctggcagcaatgcctggaaagcgatccttctcaaaggctcggaggagcagggcggtttgggatccggtgatggcagtccgctttcgtctgcctttttgcgggtcacgtctcccgggccagggccgagattgccgccggtgctgcctcaactggcatgatctctcattctgaaaccaaatctggaccctgggctccggaatgtcgatgccctgggccagctcttctttggtggcaatgcccgggtacaggttccgctcaaagcaggctcgcagggcatcactttgactcggggtcgaaaggagtatcattcgccttcccggtccctgggcttcctcggggagggtgtcgtccaaagctgtcaggagggccatctcagggagccccggccggaatttcacggactgacacgggcagagagaggcgggcgggctcccgtgcacctcagccagcctgttcactgcgcaggtgctgccaggaggcctg

SEQ ID NO: 10425 - RNA, 544 nt, Homo sapiens
  source 1..544: mol_type = other RNA
cctcacccagctctctggccctctggagtttcatcccctccaatcagtactctgtctgggttctttaggtccttgatggctgttccctctgccagaaactcagggttggacagcacagaaataaatacaagatcagcttctttgatggcatcatcaatattggtagaaaaaaaaagattttttcctcgacaggattctaccacttcttttagtcctggctcataaataggaagtgtaggagaattccacgcattgattcttgattcattgacatcaacaaccgttaccctgatttcaggacacatatgagcaatgacactacatgtgggtcctccaacatagcctgcaccgatgcaacagatcttcttaatttcaaacatgattgtaccacttcccagcagcaagcgcagggaccgctcctatcccgatcgttcggacagcaccttcctacgggccgcgccgccgcagcttctccacccgcgccccgctcgatctgagctccctctcggcgcacgcccctccctcaggctgccacgcgttacac

SEQ ID NO: 10426 - RNA, 576 nt, Homo sapiens
  source 1..576: mol_type = other RNA
cctcacccagctctctggccctctggagtttcatcccctccaatcagtactctgtctgggttctttaggtccttgatggctgttccctctgccagaaactcagggttggacagcacctgtaaattcaagttgggttttgtgtttgcatcaaatatgcgacggatactttctgctgcccgcactggaactgtgcttttctcagtcacaattttgtacccatttgagttttgcacaatgcgtctagcacaagcttcaatatacttcagatctgctgcccggcctttccccattccataggtttttgttggagtattcacagaaataaatacaagatcagcttctttgatggcatcatcaatattggtagaaaaaaaaagattttttcctcgacaggattctaccacttcttttagtcctggccacttcccagcagcaagcgcagggaccgctcctatcccgatcgttcggacagcaccttcctacgggccgcgccgccgcagcttctccacccgcgccccgctcgatctgagctccctctcggcgcacgcccctccctcaggctgccacgcgttacac

SEQ ID NO: 10427 - RNA, 745 nt, Homo sapiens
  source 1..745: mol_type = other RNA
cctcacccagctctctggccctctggagtttcatcccctccaatcagtactctgtctgggttctttaggtccttgatggctgttccctctgccagaaactcagggttggacagcacctgtaaattcaagttgggttttgtgtttgcatcaaatatgcgacggatactttctgctgcccgcactggaactgtgcttttctcagtcacaattttgtacccatttgagttttgcacaatgcgtctagcacaagcttcaatatacttcagatctgctgcccggcctttccccattccataggtttttgttggagtattcacagaaataaatacaagatcagcttctttgatggcatcatcaatattggtagaaaaaaaaagattttttcctcgacaggattctaccacttcttttagtcctggctcataaataggaagtgtaggagaattccacgcattgattcttgattcattgacatcaacaaccgttaccctgatttcaggacacatatgagcaatgacactacatgtgggtcctccaacatagcctgcaccgatgcaacagatcttcttaatttcaaacatgattgtaccacttcccagcagcaagcgcagggaccgctcctatcccgatcgttcggacagcaccttcctacgggccgcgccgccgcagcttctccacccgcgccccgctcgatctgagctccctctcggcgcacgcccctccctcaggctgccacgcgttacac

SEQ ID NO: 10428 - RNA, 643 nt, Homo sapiens
  source 1..643: mol_type = other RNA
cctcacccagctctctggccctctggagtttcatcccctccaatcagtactctgtctgggttctttaggtccttgatggctgttccctctgccagaaactcagggttggacagcacctgtaaattcaagttgggttttgtgtttgcatcaaatatgcgacggatactttctgctgcccgcactggaactgtgcttttctcagtcacaattttgtacccatttgagttttgcacaatgcgtctagcacaagcttcaatatacttcagatctgctgcccggcctttccccattccataggtttttgttggagtattcacagaaataaatacaagatcagcttctttgatggcatcatcaatattggtagaaaaaaaaagattttttcctcgacaggattctaccacttcttttagtcctggctcataaataggaagtgtaggagaattccacgcattgattcttgattcattgacatcaacaaccgttaccctgatttcaggacacatatgagcaatgacactacatgtgggtcctccaacatagcctgcaccgatgcaacagatcttcttaatttcaaacatgattgtagagtcttgaataagaagcccagacgaccacatccccaggacagcagttccaaaat

SEQ ID NO: 10429 - RNA, 3491 nt, Homo sapiens
  source 1..3491: mol_type = other RNA
cctcctgccctccttgctgtcactttgggaaagagatcctcctgaggcacgtgtcatgttttattcttgagtgaattatctgaccatcacggcccttgctccccttttatgacatgtgcctgttatttcttttgttgcttatgatgacaagaaggcagtcccgggaggggagtctggcacagctgcccttgggaaggaactggtgtttctgagggggagggggctggtggggtgtagcaaatgcttatgtacggttatccatactcagtcaattgtgaagggaacagtatacccacaattccacccaaagactctacaaaataaatctttctctccatctcccttacatttagggcctttcatttttaaggcactgggttgtgaagacttgaagacatacaaggtcagtaaaactgaagaccttgcatcctgcttgcttcaaatgtggagaggcaaacacaggctactggaccagacgggaacggttacccacggtgacaaaagcaggtctccaaagcacagcattttggttagtgcattccagatgtgttagctacaactggggacaccaacttgaataacacatttttcttttaacaaaacaaaagtttaccctgcttggatgatgctaaatgcccttaagcactaggccttcggttgccactgagaaagcacaccatttccattccactgtgtgtgaagccacaaccctactaattccttcattaactcaacaagatttgcatcccttaataaatccaagccgatgcggagacatcaggggagactttatcagatgtcccccaagggagggcaagtctggaagtagtggggttatgcttcacaggggagagatactgttctaggaaaaaaaaacacccacattttctggaaggaaaactgagtttttttaagagcagtgtttcatcccgagctaaggtcaggattaatgcctatttttcatttggtttgcatcagaagagctcgttttccttcccagcagctccagtggaattactttttggaattagaactgagaccaaacaaagtgatgatgtcagtcattgcttctttcaggtgccttccaaagcgatgagaatccgtctcagggcaagagaacttggaagaaatgtggaaattgatgaggttctctcccacaaggatgtacgacacaccatagccgtcatcagcaaccggtccaaagccccctccgctggacacgtactctgggttattctccaagtcaaacagctccacttgctgctgaggggtctggcttgttgataatctccaaggctcagataaaacttccttaaggaaaggggactccacagcgagatatttagacaccacgtaaaggcagaagaggtgacgatcgatcccagagccggtcatggcgaggcgatacatatgctgatgcttctcagacgccaacttgaacaacttcagcctctgttccaccgtctgggccgggtccaccatggcccgcacgaagtcgcatgactcagtggtgcaggagcgcacggtctccgtcctcccctctcggaagagccgggtcatggaggcctcgtatgtgaggcaaaacttgcccatgtccttgtagtgcgccagctggagggccagctgcacaaaggcgtctgggctcgtgcgacatttcttgatgattcctttaccaaaggctacgaatgggaaggaatggaaatccacgtcgtttgccagaagatttgcggtgttcagggaggtctctataacctcttgacattcccccgggatgtcccactgcagcctggtggggtacggaatgttcggattgatgtcgcctttgcagtgcccatcctccgcatagcccagctggaggctgtcaatggacatgacgtactcccaaaggtgggccacgatcggcgcatctgcccaggagtgttcagcgttgaggcccatcttcccgtttttgaagacaacaaacgtgaacgacttgtcaaaccacctgtcgtaacatcggccgtgtagtagagatttggcgtagctgtccattgacgtatccgggtcttcacttctgtatccttcttcagtttcatctaacgtcacaaagaacgctgctttctccacagcatcaagagactgcttatttttcccacgtccaaaataggcctgacgacacctggcccagggaactctgtctcctgcggtgagggctgccagcctggcctccccgggctgaggctccgaggtattgtccaggatcctctgcatctgctgctccatctcccggggcttcagcagccgcccatcatggtagagccagaccttgaagtagcgtcctcgatggtacacgacgatgtgcttgctgtctctcatgtgctggatggtgtctgtctcctctcctgggatccgggaagtattaaacatccgctcccactgagcggagcagagtggaatcgtggatcccaaaagacgaattggtttgatttcctcccggtccagtttgcgcctgtaaagcaggatggcatggatggcgttgccggctcttgctgcctgaatgtgagttggaaggatatacagcagatccatggcataatagttgctgttcaccatgagcggccctcgtcctcggaggtagatgtactcctcccaccagtcgctcacgtaatttgtagcccaccaggattttaacttcaaataccactgtaatcttggtccaagaccgacagcaaaatcttgagcaagtgctgtcatccgtttgaagtcttcttccttcataagaggcctcaccgactgtagatacctgttcacagtgtctttgacagccgggaccggcaggcgaggcagcgatgtctggaagctgtacaacatgggttttcggcctgaaaagatcttgaccatacccatccagatcttggtggcacgactcatcttgccgtgctcagtgaacatccacccgtggtaggagagcagcactttcagggagtagcgcatggtgacgatgagggccacccacaggccggtgccaaacagcacgccgctgaccacgttcttcgtctggctggacatgcagttggccgtttccagagtccgattgatttttgcaattattcctaacgaggggtcgatcttggcgtacatcgttgtcatcacgcccaccaccacgataagccaactggaggggcttgccgggtacacgccagtgatgatgccgttcttgaatctgatgaacttctttttccaggaatgaagtccagagagatagatttgtctaagagcttcatggctcagccgcaggtcaatcccgtccggagtgaccgtgaactgaaaggccacagcttggtgagcttctgccatcttcagagagtaccgagtcagctacggaggtgcggcagcggcagcggcagcggcggcggcggcggcggcggtggagtgaacgagcggcgagcgggagccggggaaggagggccgcgggcgaggccgagcgcacccgacgccggcagcagcggatt

SEQ ID NO: 10430 - RNA, 3482 nt, Homo sapiens
  source 1..3482: mol_type = other RNA
cctcctgccctccttgctgtcactttgggaaagagatcctcctgaggcacgtgtcatgttttattcttgagtgaattatctgaccatcacggcccttgctccccttttatgacatgtgcctgttatttcttttgttgcttatgatgacaagaaggcagtcccgggaggggagtctggcacagctgcccttgggaaggaactggtgtttctgagggggagggggctggtggggtgtagcaaatgcttatgtacggttatccatactcagtcaattgtgaagggaacagtatacccacaattccacccaaagactctacaaaataaatctttctctccatctcccttacatttagggcctttcatttttaaggcactgggttgtgaagacttgaagacatacaaggtcagtaaaactgaagaccttgcatcctgcttgcttcaaatgtggagaggcaaacacaggctactggaccagacgggaacggttacccacggtgacaaaagcaggtctccaaagcacagcattttggttagtgcattccagatgtgttagctacaactggggacaccaacttgaataacacatttttcttttaacaaaacaaaagtttaccctgcttggatgatgctaaatgcccttaagcactaggccttcggttgccactgagaaagcacaccatttccattccactgtgtgtgaagccacaaccctactaattccttcattaactcaacaagatttgcatcccttaataaatccaagccgatgcggagacatcaggggagactttatcagatgtcccccaagggagggcaagtctggaagtagtggggttatgcttcacaggggagagatactgttctaggaaaaaaaaacacccacattttctggaaggaaaactgagtttttttaagagcagtgtttcatcccgagctaaggtcaggattaatgcctatttttcatttggtttgcatcagaagagctcgttttccttcccagcagctccagtggaattactttttggaattagaactgagaccaaacaaagtgatgatgtcagtcattgcttctttcaggtgccttccaaagcgatgagaatccgtctcagggcaagagaacttggaagaaatgtggaaattgatgaggttctctcccacaaggatgtacgacacaccatagccgtcatcagcaaccggtccaaagccccctccgctggacacgtactctgggttattctccaagtcaaacagctccacttgctgctgaggggtctggcttgttgataatctccaaggctcagataaaacttccttaaggaaaggggactccacagcgagatatttagacaccacgtaaaggcagaagaggtgacgatcgatcccagagccggtcatggcgaggcgatacatatgctgatgcttctcagacgccaacttgaacaacttcagcctctgttccaccgtctgggccgggtccaccatggcccgcacgaagtcgcatgactcagtggtgcaggagcgcacggtctccgtcctcccctctcggaagagccgggtcatggaggcctcgtatgtgaggcaaaacttgcccatgtccttgtagtgcgccagctggagggccagctgcacaaaggcgtctgggctcgtgcgacatttcttgatgattcctttaccaaaggctacgaatgggaaggaatggaaatccacgtcgtttgccagaagatttgcggtgttcagggaggtctctataacctcttgacattcccccgggatgtcccactgcagcctggtggggtacggaatgttcggattgatgtcgcctttgcagtgcccatcctccgcatagcccagctggaggctgtcaatggacatgacgtactcccaaaggtgggccacgatcggcgcatctgcccaggagtgttcagcgttgaggcccatcttcccgtttttgaagacaacaaacgtgaacgacttgtcaaaccacctgtcgtaacatcggccgtgtagtagagatttggcgtagctgtccattgacgtatccgggtcttcacttctgtatccttcttcagtttcatctaacgtcacaaagaacgctgctttctccacagcatcaagagactgcttatttttcccacgtccaaaataggcctgacgacacctggcccagggaactctgtctcctgcggtgagggctgccagcctggcctccccgggctgaggctccgaggtattgtccaggatcctctgcatctgctgctccatctcccggggcttcagcagccgcccatcatggtagagccagaccttgaagtagcgtcctcgatggtacacgacgatgtgcttgctgtctctcatgtgctggatggtgtctgtctcctctcctgggatccgggaagtattaaacatccgctcccactgagcggagcagagtggaatcgtggatcccaaaagacgaattggtttgatttcctcccggtccagtttgcgcctgtaaagcaggatggcatggatggcgttgccggctcttgctgcctgaatgtgagttggaaggatatacagcagatccatggcataatagttgctgttcaccatgagcggccctcgtcctcggaggtagatgtactcctcccaccagtcgctcacgtaatttgtagcccaccaggattttaacttcaaataccactgtaatcttggtccaagaccgacagcaaaatcttgagcaagtgctgtcatccgtttgaagtcttcttccttcataagaggcctcaccgactgtagatacctgttcacagtgtctttgacagccgggaccggcaggcgaggcagcgatgtctggaagctgtacaacatgggttttcggcctgaaaagatcttgaccatacccatccagatcttggtggcacgactcatcttgccgtgctcagtgaacatccacccgtggtaggagagcagcactttcagggagtagcgcatggtgacgatgagggccacccacaggccggtgccaaacagcacgccgctgaccacgttcttcgtctggctggacatgcagttggccgtttccagagtccgattgatttttgcaattattcctaacgaggggtcgatcttggcgtacatcgttgtcatcacgcccaccaccacgataagccaactggaggggcttgccgggtacacgccagtgatgatgccgttcttgaatctgatgaacttctttttccaggaatgaagtccagagagatagatttgtctaagagcttcatggctcagccgcaggtcaatcccgtccggagtgaccgtgaactgaaaggccacagcttggtgagcttctgccatcttcagagagtacctctccgtgggaaggtcgagccctgcggtgcccagctgtggggacagctcggtgctcagtgcttctgatgacagatgctgcatccaacgagccagaaacgcaggcaccgcgctcaagagcccagggcgcgtct

SEQ ID NO: 10431 - RNA, 325 nt, Homo sapiens
  source 1..325: mol_type = other RNA
cctcctgccctccttgctgttcctggaacttgccagttatcttgcatttgcctcagggccgttgcattagctgcttctgtgcctggagcacctttcccttaccgatgggcaaggcgctctccccgctttctttgggcctctgctccaaggccactttcttaggcacaatcctgtcttctgggtcctcagcttctttgccctcttgcctctccaaagaggaacttacttgttcagcttacttgttctttgttctctattttcaaagcctaacttccttgttctttgtacctccttacccctagttacggtaaacaaccttcccgcg

SEQ ID NO: 10432 - RNA, 71 nt, Homo sapiens
  source 1..71: mol_type = other RNA
cctctaaagggaagcgctttctcttctttcagacaacagaaagggcttccctttgcagtcacagcttgaga

SEQ ID NO: 10433 - RNA, 72 nt, Homo sapiens
  source 1..72: mol_type = other RNA
cctctaaagggaagcgctttctcttctttctgacaacagaaagcgctttcctttgtagactcatagcttgag

SEQ ID NO: 10434 - RNA, 73 nt, Homo sapiens
  source 1..73: mol_type = other RNA
cctctaaagggaagcgctttctcttcttttagacaacagaaagggcttccctttgcagacccacagcttgaga

SEQ ID NO: 10435 - RNA, 73 nt, Homo sapiens
  source 1..73: mol_type = other RNA
cctctaaagggaagcgctttcttttcttttagccaacagaaagcgcttccctctagagggtcacagcctgaga

SEQ ID NO: 10436 - RNA, 3963 nt, Homo sapiens
  source 1..3963: mol_type = other RNA
cctctagatggaagcactgtctgagtgatccacttttgttgaaggaatgctcataggagacattatctgtgtggctattccttttgaaataggtggtagagctggatttagatttggatgtaagataggttgagttggaaccaatggagcttgaagacaaagattttcctagattatcagaacttttcttgatgatattggtagctgtcttactccaatctgagttatctgctaaccgaaatctaccacagcagagatgctgccgccactgtttctgaacattctccttcatagcacagtggaagatgaatataaataagccttgtaatgaattgaagatggagaagaggtacatgaaggggatatttaagggtccccaggcaaagaatgcaaaaccccatgtcatgcccaacagaaaggtcaagctaaccacactgcgcaggttccttaacacttcttctctcagggtccggttgcttctcttgccattcctcccacagatctgcaccattaccacaatgaacatggcaatgttcagaaaaaacatgactccaaaatacccagcacaggtcacataaaatatgactggatcttgaatccaacagaattcatcacctttttctttcccataactttcttttccatagacttcattgttgtttctgctcgctagaacaactgacaccactaaggcaggcaaaccccagccaatgatgcagaattttagaatgtatcggcgaatgtaagtgttaaatactttaactagagcaatgtacatgtgaattgcttctagccccatccaggtaaaggttgccagaaggaagaaatgcaacaggactgcaacagcaatgcaaagtccatccacattgaaggaggtgatccagccatctaggaggaagaggagattcaggaacagcagggctgtgctcaggttcatcaagattttggagggataatcccttcgcaatttctcaaaagcaacatatgtcaggagagttgctgctgaaaaaatagcagatattccacacccaatatagctgatgaaagtgaggactttagtgtttcttgcatctaactgtgaggcacttcttggaaggtccatcagaactccaaagtgtgtgaagtggttacacaggcagactgtctcacttgcatctgaatctctgtgtgcaacacatcctgacgtgttccatcctccaaaacttttgtttttgttcagatcccagaaggcacagatgggatgatgcacttcctgagttcttgtatgtttgatttttatttgaacaggatccttcagattctggatagtaatgtttccaatactgcacgccatcacataactcactaaagtttttctttggggtcctacatcctggaaaagtccagttttgttgaagaaagtaaactgtgctcttctaactaatacagaatcttctggacttaaattctcaagtaagtttggaggcaaaattacagatgccagtggatccacttgtccactctcaaaatccatctggaaatacgattcattattgcttggaagaccaatgctaaaatttgaaattgcatttgtccctggtaacagggatgatacgctgagagccaagttccgagttgtaatattcacatgtgatgtgctatttaggtctatcttgaaggccaattcatcaattgtttttaaagcttcagaagatgactcaagcaagtcactgtctgaactgcttaagatattagaaaatatattcattagagttgagccaagtgttatatcaatgttttcttctttattcacaattcttttgacctgttccacaatgttggtaatattggctgaggttaagttctgcccatcagcagttaaatttaaaatctggttagcaacttcatttgcttcttttaaacagttggagatatcaacaggtccccagtaggttaccaatgggttggtagcattgtaaaaacatatccgagaagcagaaaagccaggcttgtctggacaaggaagaacgtattcagaaggttggatagatggccagtagtagcctttgggttcctccatggcaagacaatgacccagttgtctcacattcactgtatgtagcctcaagccttcatccaaggactcattattttttaggagcttctgctgaatgatttttccttccaaattagtattgttggtagcattgtaaactagaagggcccaaagcaccaaccttggctcatcctcaaggcttctcttgactttaatcttgtcctctccagcactcaggtgaaaactgatattaacgacataaaccgtgtagttccaattttggaaggttgaattgagccattctgccaccttgctctgtacttttacctcagggtgacgaaggatgttctgaatcactacggatattctatagataattccatcattcctttgtttatcgattctgttagtaacaggcatgttagtggtgacagtgggtggtgtagtactaggagagtttacagtagcttgacagagggtccccaggtctgcacagctggccagttctgctgctgggagcgggatcaggtaggaaccacagcttaggttgctttcagctttcagagctaggtttgggatattccagaagtcattttgccagtcgactacattccctttcacattacagctgaggttggagaggattttggcattcatggtaaaattccaaagtcgaaagttataaatgtccccttttagagagacaatttcattttgattggagcccaacaacaatttcccattcccaggaataactttactaatggtagaatcacatggaactgtttcatagtttcttttgaaatttacaccaatagagcccaaagaattattccaaacaaggcagagctgttcaaagctttctgcaaaaatgtcttctttttctttgacaggtaatgcattattcaacaaacattttgaatcagaaatggatagaaagtagccactcttggcctttccaaaactgagcaattgtgtgaaggatgcatttgagtaggagaaagctgtccaatcactgtcttcatggccaactttggttgcttcaaagcagagtgtgaaagcactgagctctggaatagagatgctttttgcaacagatacctggtaagcatctgatgtctggggtaaaatgaccttttgattccttaaggacacggcaactctgatgtagctggcattgaaacctttcttctggatgctaaagtcacttgaaaaggacacatgcatctcattcgcacttgagttaaatgataggcctttggcagttgctccacaaaatttagtctggctctctccattatcaagggataatgagtcataaatgcaattgggagcttcttcaatgtcaaagtcgttaaatgttatctgaatgatataaccggtgggggctcggagcgtccacatgcaagcctggctgtttgggtagtcgttagggtagcatggagaagtaaaggtcccagaagggttggacaaaaccactcggcagttggcacatccccacactgagtgaggaacacacatgatatataaagcaaataagaacaggagaggactgggcttccatttccaatggcagctccacattcgatctgagcgaaacatcatgttgacattactgcgccgaggtcccctttggccgcaagatcatcctccaccactttcccgctctgctgccgctgctccacccagggggaacccaggcgccccagccctgcgccgcggcgggaccctcctttacgccgtttctggagagttcatgggctttcccgacggcgcaaggtgaaccctgggcgcggcagcgttcagcgcagggcctgcggacgaggaagcaggctggcggcaggtccctcctcgcagggaagttggcagggtgagggcgagaagctgaggaagtagggtgtgcgtggggctggtgctgaggagaccgg

SEQ ID NO: 10437 - RNA, 3952 nt, Homo sapiens
  source 1..3952: mol_type = other RNA
cctctagatggaagcactgtctgagtgatccacttttgttgaaggaatgctcataggagacattatctgtgtggctattccttttgaaataggtggtagagctggatttagatttggatgtaagataggttgagttggaaccaatggagcttgaagacaaagattttcctagattatcagaacttttcttgatgatattggtagctgtcttactccaatctgagttatctgctaaccgaaatctaccacagcagagatgctgccgccactgtttctgaacattctccttcatagcacagtggaagatgaatataaataagccttgtaatgaattgaagatggagaagaggtacatgaaggggatatttaagggtccccaggcaaagaatgcaaaaccccatgtcatgcccaacagaaaggtcaagctaaccacactgcgcaggttccttaacacttcttctctcagggtccggttgcttctcttgccattcctcccacagatctgcaccattaccacaatgaacatggcaatgttcagaaaaaacatgactccaaaatacccagcacaggtcacataaaatatgactggatcttgaatccaacagaattcatcacctttttctttcccataactttcttttccatagacttcattgttgtttctgctcgctagaacaactgacaccactaaggcaggcaaaccccagccaatgatgcagaattttagaatgtatcggcgaatgtaagtgttaaatactttaactagagcaatgtacatgtgaattgcttctagccccatccaggtaaaggttgccagaaggaagaaatgcaacaggactgcaacagcaatgcaaagtccatccacattgaaggaggtgatccagccatctaggaggaagaggagattcaggaacagcagggctgtgctcaggttcatcaagattttggagggataatcccttcgcaatttctcaaaagcaacatatgtcaggagagttgctgctgaaaaaatagcagatattccacacccaatatagctgatgaaagtgaggactttagtgtttcttgcatctaactgtgaggcacttcttggaaggtccatcagaactccaaagtgtgtgaagtggttacacaggcagactgtctcacttgcatctgaatctctgtgtgcaacacatcctgacgtgttccatcctccaaaacttttgtttttgttcagatcccagaaggcacagatgggatgatgcacttcctgagttcttgtatgtttgatttttatttgaacaggatccttcagattctggatagtaatgtttccaatactgcacgccatcacataactcactaaagtttttctttggggtcctacatcctggaaaagtccagttttgttgaagaaagtaaactgtgctcttctaactaatacagaatcttctggacttaaattctcaagtaagtttggaggcaaaattacagatgccagtggatccacttgtccactctcaaaatccatctggaaatacgattcattattgcttggaagaccaatgctaaaatttgaaattgcatttgtccctggtaacagggatgatacgctgagagccaagttccgagttgtaatattcacatgtgatgtgctatttaggtctatcttgaaggccaattcatcaattgtttttaaagcttcagaagatgactcaagcaagtcactgtctgaactgcttaagatattagaaaatatattcattagagttgagccaagtgttatatcaatgttttcttctttattcacaattcttttgacctgttccacaatgttggtaatattggctgaggttaagttctgcccatcagcagttaaatttaaaatctggttagcaacttcatttgcttcttttaaacagttggagatatcaacaggtccccagtaggttaccaatgggttggtagcattgtaaaaacatatccgagaagcagaaaagccaggcttgtctggacaaggaagaacgtattcagaaggttggatagatggccagtagtagcctttgggttcctccatggcaagacaatgacccagttgtctcacattcactgtatgtagcctcaagccttcatccaaggactcattattttttaggagcttctgctgaatgatttttccttccaaattagtattgttggtagcattgtaaactagaagggcccaaagcaccaaccttggctcatcctcaaggcttctcttgactttaatcttgtcctctccagcactcaggtgaaaactgatattaacgacataaaccgtgtagttccaattttggaaggttgaattgagccattctgccaccttgctctgtacttttacctcagggtgacgaaggatgttctgaatcactacggatattctatagataattccatcattcctttgtttatcgattctgttagtaacaggcatgttagtggtgacagtgggtggtgtagtactaggagagtttacagtagcttgacagagggtccccaggtctgcacagctggccagttctgctgctgggagcgggatcaggtaggaaccacagcttaggttgctttcagctttcagagctaggtttgggatattccagaagtcattttgccagtcgactacattccctttcacattacagctgaggttggagaggattttggcattcatggtaaaattccaaagtcgaaagttataaatgtccccttttagagagacaatttcattttgattggagcccaacaacaatttcccattcccaggaataactttactaatggtagaatcacatggaactgtttcatagtttcttttgaaatttacaccaatagagcccaaagaattattccaaacaaggcagagctgttcaaagctttctgcaaaaatgtcttctttttctttgacaggtaatgcattattcaacaaacattttgaatcagaaatggatagaaagtagccactcttggcctttccaaaactgagcaattgtgtgaaggatgcatttgagtaggagaaagctgtccaatcactgtcttcatggccaactttggttgcttcaaagcagagtgtgaaagcactgagctctggaatagagatgctttttgcaacagatacctggtaagcatctgatgtctggggtaaaatgaccttttgattccttaaggacacggcaactctgatgtagctggcattgaaacctttcttctggatgctaaagtcacttgaaaaggacacatgcatctcattcgcacttgagttaaatgataggcctttggcagttgctccacaaaatttagtctggctctctccattatcaagggataatgagtcataaatgcaattgggagcttcttcaatgtcaaagtcgttaaatgttatctgaatgatataaccggtgggggctcggagcgtccacatgcaagcctggctgtttgggtagtcgttagggtagcatggagaagtaaaggtcccagaagggttggacaaaaccactcggcagttggcacatccccacactgctgagtgaggaacacacatgatatataaagcaaataagaacaggagaggactgggcttccatttccaatggcagctccacattcgatctgagcgaaacatcatgttgacattactgcgccgaggtcccctttggccgcaagatcatcctccaccactttcccgctctgctgccgctgctccacccagggggaacccaggcgccccagccctgcgccgcggcgggaccctcctttacgccgtttctggagagttcatgggctttcccgacggcgcaaggtgaaccctgggcgcggcagcgttcagcgcagggcctgcggacgaggaagcaggctggcggcaggtccctcctcgcagggaagttggcagggtgagggcgagaagctgaggaagtagggtgtgcgtggggctggt

SEQ ID NO: 10438 - RNA, 3879 nt, Homo sapiens
  source 1..3879: mol_type = other RNA
cctctagatggaagcactgtctgagtgatccacttttgttgaaggaatgctcataggagacattatctgtgtggctattccttttgaaataggtggtagagctggatttagatttggatgtaagataggttgagttggaaccaatggagcttgaagacaaagattttcctagattatcagaacttttcttgatgatattggtagctgtcttactccaatctgagttatctgctaaccgaaatctaccacagcagagatgctgccgccactgtttctgaacattctccttcatagcacagtggaagatgaatataaataagccttgtaatgaattgaagatggagaagaggtacatgaaggggatatttaagggtccccaggcaaagaatgcaaaaccccatgtcatgcccaacagaaaggtcaagctaaccacactgcgcaggttccttaacacttcttctctcagggtccggttgcttctcttgccattcctcccacagatctgcaccattaccacaatgaacatggcaatgttcagaaaaaacatgactccaaaatacccagcacaggtcacataaaatatgactggatcttgaatccaacagaattcatcacctttttctttcccataactttcttttccatagacttcattgttgtttctgctcgctagaacaactgacaccactaaggcaggcaaaccccagccaatgatgcagaattttagaatgtatcggcgaatgtaagtgttaaatactttaactagagcaatgtacatgtgaattgcttctagccccatccaggtaaaggttgccagaaggaagaaatgcaacaggactgcaacagcaatgcaaagtccatccacattgaaggaggtgatccagccatctaggaggaagaggagattcaggaacagcagggctgtgctcaggttcatcaagattttggagggataatcccttcgcaatttctcaaaagcaacatatgtcaggagagttgctgctgaaaaaatagcagatattccacacccaatatagctgatgaaagtgaggactttagtgtttcttgcatctaactgtgaggcacttcttggaaggtccatcagaactccaaagtgtgtgaagtggttacacaggcagactgtctcacttgcatctgaatctctgtgtgcaacacatcctgacgtgttccatcctccaaaacttttgtttttgttcagatcccagaaggcacagatgggatgatgcacttcctgagttcttgtatgtttgatttttatttgaacaggatccttcagattctggatagtaatgtttccaatactgcacgccatcacataactcactaaagtttttctttggggtcctacatcctggaaaagtccagttttgttgaagaaagtaaactgtgctcttctaactaatacagaatcttctggacttaaattctcaagtaagtttggaggcaaaattacagatgccagtggatccacttgtccactctcaaaatccatctggaaatacgattcattattgcttggaagaccaatgctaaaatttgaaattgcatttgtccctggtaacagggatgatacgctgagagccaagttccgagttgtaatattcacatgtgatgtgctatttaggtctatcttgaaggccaattcatcaattgtttttaaagcttcagaagatgactcaagcaagtcactgtctgaactgcttaagatattagaaaatatattcattagagttgagccaagtgttatatcaatgttttcttctttattcacaattcttttgacctgttccacaatgttggtaatattggctgaggttaagttctgcccatcagcagttaaatttaaaatctggttagcaacttcatttgcttcttttaaacagttggagatatcaacaggtccccagtaggttaccaatgggttggtagcattgtaaaaacatatccgagaagcagaaaagccaggcttgtctggacaaggaagaacgtattcagaaggttggatagatggccagtagtagcctttgggttcctccatggcaagacaatgacccagttgtctcacattcactgtatgtagcctcaagccttcatccaaggactcattattttttaggagcttctgctgaatgatttttccttccaaattagtattgttggtagcattgtaaactagaagggcccaaagcaccaaccttggctcatcctcaaggcttctcttgactttaatcttgtcctctccagcactcaggtgaaaactgatattaacgacataaaccgtgtagttccaattttggaaggttgaattgagccattctgccaccttgctctgtacttttacctcagggtgacgaaggatgttctgaatcactacggatattctatagataattccatcttgacagagggtccccaggtctgcacagctggccagttctgctgctgggagcgggatcaggtaggaaccacagcttaggttgctttcagctttcagagctaggtttgggatattccagaagtcattttgccagtcgactacattccctttcacattacagctgaggttggagaggattttggcattcatggtaaaattccaaagtcgaaagttataaatgtccccttttagagagacaatttcattttgattggagcccaacaacaatttcccattcccaggaataactttactaatggtagaatcacatggaactgtttcatagtttcttttgaaatttacaccaatagagcccaaagaattattccaaacaaggcagagctgttcaaagctttctgcaaaaatgtcttctttttctttgacaggtaatgcattattcaacaaacattttgaatcagaaatggatagaaagtagccactcttggcctttccaaaactgagcaattgtgtgaaggatgcatttgagtaggagaaagctgtccaatcactgtcttcatggccaactttggttgcttcaaagcagagtgtgaaagcactgagctctggaatagagatgctttttgcaacagatacctggtaagcatctgatgtctggggtaaaatgaccttttgattccttaaggacacggcaactctgatgtagctggcattgaaacctttcttctggatgctaaagtcacttgaaaaggacacatgcatctcattcgcacttgagttaaatgataggcctttggcagttgctccacaaaatttagtctggctctctccattatcaagggataatgagtcataaatgcaattgggagcttcttcaatgtcaaagtcgttaaatgttatctgaatgatataaccggtgggggctcggagcgtccacatgcaagcctggctgtttgggtagtcgttagggtagcatggagaagtaaaggtcccagaagggttggacaaaaccactcggcagttggcacatccccacactgagtgaggaacacacatgatatataaagcaaataagaacaggagaggactgggcttccatttccaatggcagctccacattcgatctgagcgaaacatcatgttgacattactgcgccgaggtcccctttggccgcaagatcatcctccaccactttcccgctctgctgccgctgctccacccagggggaacccaggcgccccagccctgcgccgcggcgggaccctcctttacgccgtttctggagagttcatgggctttcccgacggcgcaaggtgaaccctgggcgcggcagcgttcagcgcagggcctgcggacgaggaagcaggctggcggcaggtccctcctcgcagggaagttggcagggtgagggcgagaagctgaggaagtagggtgtgcgtggggctggtgctgaggagaccgg

SEQ ID NO: 10439 - RNA, 3917 nt, Homo sapiens
  source 1..3917: mol_type = other RNA
cctctagatggaagcactgtctgtgtggctattccttttgaaataggtggtagagctggatttagatttggatgtaagataggttgagttggaaccaatggagcttgaagacaaagattttcctagattatcagaacttttcttgatgatattggtagctgtcttactccaatctgagttatctgctaaccgaaatctaccacagcagagatgctgccgccactgtttctgaacattctccttcatagcacagtggaagatgaatataaataagccttgtaatgaattgaagatggagaagaggtacatgaaggggatatttaagggtccccaggcaaagaatgcaaaaccccatgtcatgcccaacagaaaggtcaagctaaccacactgcgcaggttccttaacacttcttctctcagggtccggttgcttctcttgccattcctcccacagatctgcaccattaccacaatgaacatggcaatgttcagaaaaaacatgactccaaaatacccagcacaggtcacataaaatatgactggatcttgaatccaacagaattcatcacctttttctttcccataactttcttttccatagacttcattgttgtttctgctcgctagaacaactgacaccactaaggcaggcaaaccccagccaatgatgcagaattttagaatgtatcggcgaatgtaagtgttaaatactttaactagagcaatgtacatgtgaattgcttctagccccatccaggtaaaggttgccagaaggaagaaatgcaacaggactgcaacagcaatgcaaagtccatccacattgaaggaggtgatccagccatctaggaggaagaggagattcaggaacagcagggctgtgctcaggttcatcaagattttggagggataatcccttcgcaatttctcaaaagcaacatatgtcaggagagttgctgctgaaaaaatagcagatattccacacccaatatagctgatgaaagtgaggactttagtgtttcttgcatctaactgtgaggcacttcttggaaggtccatcagaactccaaagtgtgtgaagtggttacacaggcagactgtctcacttgcatctgaatctctgtgtgcaacacatcctgacgtgttccatcctccaaaacttttgtttttgttcagatcccagaaggcacagatgggatgatgcacttcctgagttcttgtatgtttgatttttatttgaacaggatccttcagattctggatagtaatgtttccaatactgcacgccatcacataactcactaaagtttttctttggggtcctacatcctggaaaagtccagttttgttgaagaaagtaaactgtgctcttctaactaatacagaatcttctggacttaaattctcaagtaagtttggaggcaaaattacagatgccagtggatccacttgtccactctcaaaatccatctggaaatacgattcattattgcttggaagaccaatgctaaaatttgaaattgcatttgtccctggtaacagggatgatacgctgagagccaagttccgagttgtaatattcacatgtgatgtgctatttaggtctatcttgaaggccaattcatcaattgtttttaaagcttcagaagatgactcaagcaagtcactgtctgaactgcttaagatattagaaaatatattcattagagttgagccaagtgttatatcaatgttttcttctttattcacaattcttttgacctgttccacaatgttggtaatattggctgaggttaagttctgcccatcagcagttaaatttaaaatctggttagcaacttcatttgcttcttttaaacagttggagatatcaacaggtccccagtaggttaccaatgggttggtagcattgtaaaaacatatccgagaagcagaaaagccaggcttgtctggacaaggaagaacgtattcagaaggttggatagatggccagtagtagcctttgggttcctccatggcaagacaatgacccagttgtctcacattcactgtatgtagcctcaagccttcatccaaggactcattattttttaggagcttctgctgaatgatttttccttccaaattagtattgttggtagcattgtaaactagaagggcccaaagcaccaaccttggctcatcctcaaggcttctcttgactttaatcttgtcctctccagcactcaggtgaaaactgatattaacgacataaaccgtgtagttccaattttggaaggttgaattgagccattctgccaccttgctctgtacttttacctcagggtgacgaaggatgttctgaatcactacggatattctatagataattccatcattcctttgtttatcgattctgttagtaacaggcatgttagtggtgacagtgggtggtgtagtactaggagagtttacagtagcttgacagagggtccccaggtctgcacagctggccagttctgctgctgggagcgggatcaggtaggaaccacagcttaggttgctttcagctttcagagctaggtttgggatattccagaagtcattttgccagtcgactacattccctttcacattacagctgaggttggagaggattttggcattcatggtaaaattccaaagtcgaaagttataaatgtccccttttagagagacaatttcattttgattggagcccaacaacaatttcccattcccaggaataactttactaatggtagaatcacatggaactgtttcatagtttcttttgaaatttacaccaatagagcccaaagaattattccaaacaaggcagagctgttcaaagctttctgcaaaaatgtcttctttttctttgacaggtaatgcattattcaacaaacattttgaatcagaaatggatagaaagtagccactcttggcctttccaaaactgagcaattgtgtgaaggatgcatttgagtaggagaaagctgtccaatcactgtcttcatggccaactttggttgcttcaaagcagagtgtgaaagcactgagctctggaatagagatgctttttgcaacagatacctggtaagcatctgatgtctggggtaaaatgaccttttgattccttaaggacacggcaactctgatgtagctggcattgaaacctttcttctggatgctaaagtcacttgaaaaggacacatgcatctcattcgcacttgagttaaatgataggcctttggcagttgctccacaaaatttagtctggctctctccattatcaagggataatgagtcataaatgcaattgggagcttcttcaatgtcaaagtcgttaaatgttatctgaatgatataaccggtgggggctcggagcgtccacatgcaagcctggctgtttgggtagtcgttagggtagcatggagaagtaaaggtcccagaagggttggacaaaaccactcggcagttggcacatccccacactgagtgaggaacacacatgatatataaagcaaataagaacaggagaggactgggcttccatttccaatggcagctccacattcgatctgagcgaaacatcatgttgacattactgcgccgaggtcccctttggccgcaagatcatcctccaccactttcccgctctgctgccgctgctccacccagggggaacccaggcgccccagccctgcgccgcggcgggaccctcctttacgccgtttctggagagttcatgggctttcccgacggcgcaaggtgaaccctgggcgcggcagcgttcagcgcagggcctgcggacgaggaagcaggctggcggcaggtccctcctcgcagggaagttggcagggtgagggcgagaagctgaggaagtagggtgtgcgtggggctggtgctgaggagaccgg

SEQ ID NO: 10440 - RNA, 3706 nt, Homo sapiens
  source 1..3706: mol_type = other RNA
cctctagatggaagcactgtctgtgtggctattccttttgaaataggtggtagagctggatttagatttggatgtaagataggttgagttggaaccaatggagcttgaagacaaagattttcctagattatcagaacttttcttgatgatattggtagctgtcttactccaatctgagttatctgctaaccgaaatctaccacagcagagatgctgccgccactgtttctgaacattctccttcatagcacagtggaagatgaatataaataagccttgtaatgaattgaagatggagaagaggtacatgaaggggatatttaagggtccccaggcaaagaatgcaaaaccccatgtcatgcccaacagaaaggtcaagctaaccacactgcgcaggttccttaacacttcttctctcagggtccggttgcttctcttgccattcctcccacagatctgcaccattaccacaatgaacatggcaatgttcagaaaaaacatgactccaaaatacccagcacaggtcacataaaatatgactggatcttgaatccaacagaattcatcacctttttctttcccataactttcttttccatagacttcattgttgtttctgctcgctagaacaactgacaccactaaggcaggcaaaccccagccaatgatgcagaattttagaatgtatcggcgaatgtaagtgttaaatactttaactagagcaatgtacatgtgaattgcttctagccccatccaggtaaaggttgccagaaggaagaaatgcaacaggactgcaacagcaatgcaaagtccatccacattgaaggaggtgatccagccatctaggaggaagaggagattcaggaacagcagggctgtgctcaggttcatcaagattttggagggataatcccttcgcaatttctcaaaagcaacatatgtcaggagagttgctgctgaaaaaatagcagatattccacacccaatatagctgatgaaagtgaggactttagtgtttcttgcatctaactgtgaggcacttcttggaaggtccatcagaactccaaagtgtgtgaagtggttacacaggcagactgtctcacttgcatctgaatctctgtgtgcaacacatcctgacgtgttccatcctccaaaacttttgtttttgttcagatcccagaaggcacagatgggatgatgcacttcctgagttcttgtatgtttgatttttatttgaacaggatccttcagattctggatagtaatgtttccaatactgcacgccatcacataactcactaaagtttttctttggggtcctacatcctggaaaagtccagttttgttgaagaaagtaaactgtgctcttctaactaatacagaatcttctggacttaaattctcaagtaagtttggaggcaaaattacagatgccagtggatccacttgtccactctcaaaatccatctggaaatacgattcattattgcttggaagaccaatgctaaaatttgaaattgcatttgtccctggtaacagggatgatacgctgagagccaagttccgagttgtaatattcacatgtgatgtgctatttaggtctatcttgaaggccaattcatcaattgtttttaaagcttcagaagatgactcaagcaagtcactgtctgaactgcttaagatattagaaaatatattcattagagttgagccaagtgttatatcaatgttttcttctttattcacaattcttttgacctgttccacaatgttggtaatattggctgaggttaagttctgcccatcagcagttaaatttaaaatctggttagcaacttcatttgcttcttttaaacagttggagatatcaacaggtccccagtaggttaccaatgggttggtagcattgtaaaaacatatccgagaagcagaaaagccaggcttgtctggacaaggaagaacgtattcagaaggttggatagatggccagtagtagcctttgggttcctccatggcaagacaatgacccagttgtctcacattcactgtatgtagcctcaagccttcatccaaggactcattattttttaggagcttctgctgaatgatttttccttccaaattagtattgttggtagcattgtaaactagaagggcccaaagcaccaaccttggctcatcctcaaggcttctcttgactttaatcttgtcctctccagcactcaggtgaaaactgatattaacgacataaaccgtgtagttccaattttggaaggttgaattgagccattctgccaccttgctctgtacttttacctcagggtgacgaaggatgttctgaatcactacggatattctatagataattccatcattcctttgtttatcgattctgttagtaacaggcatgttagtggtgacagtgggtggtgtagtactaggagagtttacagtagcttgacagagggtccccaggtctgcacagctggccagttctgctgctgggagcgggatcaggtaggaaccacagcttaggttgctttcagctttcagagctaggtttgggatattccagaagtcattttgccagtcgactacattccctttcacattacagctgaggttggagaggattttggcattcatggtaaaattccaaagtcgaaagttataaatgtccccttttagagagacaatttcattttgattggagcccaacaacaatttcccattcccaggaataactttactaatggtagaatcacatggaactgtttcatagtttcttttgaaatttacaccaatagagcccaaagaattattccaaacaaggcagagctgttcaaagctttctgcaaaaatgtcttctttttctttgacaggtaatgcattattcaacaaacattttgaatcagaaatggatagaaagtagccactcttggcctttccaaaactgagcaattgtgtgaaggatgcatttgagtaggagaaagctgtccaatcactgtcttcatggccaactttggttgcttcaaagcagagtgtgaaagcactgagctctggaatagagatgctttttgcaacagatacctggtaagcatctgatgtctggggtaaaatgaccttttgattccttaaggacacggcaactctgatgtagctggcattgaaacctttcttctggatgctaaagtcacttgaaaaggacacatgcatctcattcgcacttgagttaaatgataggcctttggcagttgctccacaaaatttagtctggctctctccattatcaagggataatgagtcataaatgcaattgggagcttcttcaatgtcaaagtcgttaaatgttatctgaatgatataaccggtgggggctcggagcgtccacatgcaagcctggctgtttgggtagtcgttagggtagcatggagaagtaaaggtcccagaagggttggacaaaaccactcggcagttggcacatccccacactgagtgaggaacacacatgatatataaagcaaataagaacaggagaggactgggcttccatttccaatggcagctccacattcgatctgagcgaaacatccttccaagcccccaggtgttgattccggagagcgccttcttggcagggccaggcctctggactgaggagcggtgcctgttactccttgtttaatttgaattgaaaacacgtttt

SEQ ID NO: 10441 - RNA, 3906 nt, Homo sapiens
  source 1..3906: mol_type = other RNA
cctctagatggaagcactgtctgtgtggctattccttttgaaataggtggtagagctggatttagatttggatgtaagataggttgagttggaaccaatggagcttgaagacaaagattttcctagattatcagaacttttcttgatgatattggtagctgtcttactccaatctgagttatctgctaaccgaaatctaccacagcagagatgctgccgccactgtttctgaacattctccttcatagcacagtggaagatgaatataaataagccttgtaatgaattgaagatggagaagaggtacatgaaggggatatttaagggtccccaggcaaagaatgcaaaaccccatgtcatgcccaacagaaaggtcaagctaaccacactgcgcaggttccttaacacttcttctctcagggtccggttgcttctcttgccattcctcccacagatctgcaccattaccacaatgaacatggcaatgttcagaaaaaacatgactccaaaatacccagcacaggtcacataaaatatgactggatcttgaatccaacagaattcatcacctttttctttcccataactttcttttccatagacttcattgttgtttctgctcgctagaacaactgacaccactaaggcaggcaaaccccagccaatgatgcagaattttagaatgtatcggcgaatgtaagtgttaaatactttaactagagcaatgtacatgtgaattgcttctagccccatccaggtaaaggttgccagaaggaagaaatgcaacaggactgcaacagcaatgcaaagtccatccacattgaaggaggtgatccagccatctaggaggaagaggagattcaggaacagcagggctgtgctcaggttcatcaagattttggagggataatcccttcgcaatttctcaaaagcaacatatgtcaggagagttgctgctgaaaaaatagcagatattccacacccaatatagctgatgaaagtgaggactttagtgtttcttgcatctaactgtgaggcacttcttggaaggtccatcagaactccaaagtgtgtgaagtggttacacaggcagactgtctcacttgcatctgaatctctgtgtgcaacacatcctgacgtgttccatcctccaaaacttttgtttttgttcagatcccagaaggcacagatgggatgatgcacttcctgagttcttgtatgtttgatttttatttgaacaggatccttcagattctggatagtaatgtttccaatactgcacgccatcacataactcactaaagtttttctttggggtcctacatcctggaaaagtccagttttgttgaagaaagtaaactgtgctcttctaactaatacagaatcttctggacttaaattctcaagtaagtttggaggcaaaattacagatgccagtggatccacttgtccactctcaaaatccatctggaaatacgattcattattgcttggaagaccaatgctaaaatttgaaattgcatttgtccctggtaacagggatgatacgctgagagccaagttccgagttgtaatattcacatgtgatgtgctatttaggtctatcttgaaggccaattcatcaattgtttttaaagcttcagaagatgactcaagcaagtcactgtctgaactgcttaagatattagaaaatatattcattagagttgagccaagtgttatatcaatgttttcttctttattcacaattcttttgacctgttccacaatgttggtaatattggctgaggttaagttctgcccatcagcagttaaatttaaaatctggttagcaacttcatttgcttcttttaaacagttggagatatcaacaggtccccagtaggttaccaatgggttggtagcattgtaaaaacatatccgagaagcagaaaagccaggcttgtctggacaaggaagaacgtattcagaaggttggatagatggccagtagtagcctttgggttcctccatggcaagacaatgacccagttgtctcacattcactgtatgtagcctcaagccttcatccaaggactcattattttttaggagcttctgctgaatgatttttccttccaaattagtattgttggtagcattgtaaactagaagggcccaaagcaccaaccttggctcatcctcaaggcttctcttgactttaatcttgtcctctccagcactcaggtgaaaactgatattaacgacataaaccgtgtagttccaattttggaaggttgaattgagccattctgccaccttgctctgtacttttacctcagggtgacgaaggatgttctgaatcactacggatattctatagataattccatcattcctttgtttatcgattctgttagtaacaggcatgttagtggtgacagtgggtggtgtagtactaggagagtttacagtagcttgacagagggtccccaggtctgcacagctggccagttctgctgctgggagcgggatcaggtaggaaccacagcttaggttgctttcagctttcagagctaggtttgggatattccagaagtcattttgccagtcgactacattccctttcacattacagctgaggttggagaggattttggcattcatggtaaaattccaaagtcgaaagttataaatgtccccttttagagagacaatttcattttgattggagcccaacaacaatttcccattcccaggaataactttactaatggtagaatcacatggaactgtttcatagtttcttttgaaatttacaccaatagagcccaaagaattattccaaacaaggcagagctgttcaaagctttctgcaaaaatgtcttctttttctttgacaggtaatgcattattcaacaaacattttgaatcagaaatggatagaaagtagccactcttggcctttccaaaactgagcaattgtgtgaaggatgcatttgagtaggagaaagctgtccaatcactgtcttcatggccaactttggttgcttcaaagcagagtgtgaaagcactgagctctggaatagagatgctttttgcaacagatacctggtaagcatctgatgtctggggtaaaatgaccttttgattccttaaggacacggcaactctgatgtagctggcattgaaacctttcttctggatgctaaagtcacttgaaaaggacacatgcatctcattcgcacttgagttaaatgataggcctttggcagttgctccacaaaatttagtctggctctctccattatcaagggataatgagtcataaatgcaattgggagcttcttcaatgtcaaagtcgttaaatgttatctgaatgatataaccggtgggggctcggagcgtccacatgcaagcctggctgtttgggtagtcgttagggtagcatggagaagtaaaggtcccagaagggttggacaaaaccactcggcagttggcacatccccacactgctgagtgaggaacacacatgatatataaagcaaataagaacaggagaggactgggcttccatttccaatggcagctccacattcgatctgagcgaaacatcatgttgacattactgcgccgaggtcccctttggccgcaagatcatcctccaccactttcccgctctgctgccgctgctccacccagggggaacccaggcgccccagccctgcgccgcggcgggaccctcctttacgccgtttctggagagttcatgggctttcccgacggcgcaaggtgaaccctgggcgcggcagcgttcagcgcagggcctgcggacgaggaagcaggctggcggcaggtccctcctcgcagggaagttggcagggtgagggcgagaagctgaggaagtagggtgtgcgtggggctggt

SEQ ID NO: 10442 - RNA, 3709 nt, Homo sapiens
  source 1..3709: mol_type = other RNA
cctctagatggaagcactgtctgtgtggctattccttttgaaataggtggtagagctggatttagatttggatgtaagataggttgagttggaaccaatggagcttgaagacaaagattttcctagattatcagaacttttcttgatgatattggtagctgtcttactccaatctgagttatctgctaaccgaaatctaccacagcagagatgctgccgccactgtttctgaacattctccttcatagcacagtggaagatgaatataaataagccttgtaatgaattgaagatggagaagaggtacatgaaggggatatttaagggtccccaggcaaagaatgcaaaaccccatgtcatgcccaacagaaaggtcaagctaaccacactgcgcaggttccttaacacttcttctctcagggtccggttgcttctcttgccattcctcccacagatctgcaccattaccacaatgaacatggcaatgttcagaaaaaacatgactccaaaatacccagcacaggtcacataaaatatgactggatcttgaatccaacagaattcatcacctttttctttcccataactttcttttccatagacttcattgttgtttctgctcgctagaacaactgacaccactaaggcaggcaaaccccagccaatgatgcagaattttagaatgtatcggcgaatgtaagtgttaaatactttaactagagcaatgtacatgtgaattgcttctagccccatccaggtaaaggttgccagaaggaagaaatgcaacaggactgcaacagcaatgcaaagtccatccacattgaaggaggtgatccagccatctaggaggaagaggagattcaggaacagcagggctgtgctcaggttcatcaagattttggagggataatcccttcgcaatttctcaaaagcaacatatgtcaggagagttgctgctgaaaaaatagcagatattccacacccaatatagctgatgaaagtgaggactttagtgtttcttgcatctaactgtgaggcacttcttggaaggtccatcagaactccaaagtgtgtgaagtggttacacaggcagactgtctcacttgcatctgaatctctgtgtgcaacacatcctgacgtgttccatcctccaaaacttttgtttttgttcagatcccagaaggcacagatgggatgatgcacttcctgagttcttgtatgtttgatttttatttgaacaggatccttcagattctggatagtaatgtttccaatactgcacgccatcacataactcactaaagtttttctttggggtcctacatcctggaaaagtccagttttgttgaagaaagtaaactgtgctcttctaactaatacagaatcttctggacttaaattctcaagtaagtttggaggcaaaattacagatgccagtggatccacttgtccactctcaaaatccatctggaaatacgattcattattgcttggaagaccaatgctaaaatttgaaattgcatttgtccctggtaacagggatgatacgctgagagccaagttccgagttgtaatattcacatgtgatgtgctatttaggtctatcttgaaggccaattcatcaattgtttttaaagcttcagaagatgactcaagcaagtcactgtctgaactgcttaagatattagaaaatatattcattagagttgagccaagtgttatatcaatgttttcttctttattcacaattcttttgacctgttccacaatgttggtaatattggctgaggttaagttctgcccatcagcagttaaatttaaaatctggttagcaacttcatttgcttcttttaaacagttggagatatcaacaggtccccagtaggttaccaatgggttggtagcattgtaaaaacatatccgagaagcagaaaagccaggcttgtctggacaaggaagaacgtattcagaaggttggatagatggccagtagtagcctttgggttcctccatggcaagacaatgacccagttgtctcacattcactgtatgtagcctcaagccttcatccaaggactcattattttttaggagcttctgctgaatgatttttccttccaaattagtattgttggtagcattgtaaactagaagggcccaaagcaccaaccttggctcatcctcaaggcttctcttgactttaatcttgtcctctccagcactcaggtgaaaactgatattaacgacataaaccgtgtagttccaattttggaaggttgaattgagccattctgccaccttgctctgtacttttacctcagggtgacgaaggatgttctgaatcactacggatattctatagataattccatcattcctttgtttatcgattctgttagtaacaggcatgttagtggtgacagtgggtggtgtagtactaggagagtttacagtagcttgacagagggtccccaggtctgcacagctggccagttctgctgctgggagcgggatcaggtaggaaccacagcttaggttgctttcagctttcagagctaggtttgggatattccagaagtcattttgccagtcgactacattccctttcacattacagctgaggttggagaggattttggcattcatggtaaaattccaaagtcgaaagttataaatgtccccttttagagagacaatttcattttgattggagcccaacaacaatttcccattcccaggaataactttactaatggtagaatcacatggaactgtttcatagtttcttttgaaatttacaccaatagagcccaaagaattattccaaacaaggcagagctgttcaaagctttctgcaaaaatgtcttctttttctttgacaggtaatgcattattcaacaaacattttgaatcagaaatggatagaaagtagccactcttggcctttccaaaactgagcaattgtgtgaaggatgcatttgagtaggagaaagctgtccaatcactgtcttcatggccaactttggttgcttcaaagcagagtgtgaaagcactgagctctggaatagagatgctttttgcaacagatacctggtaagcatctgatgtctggggtaaaatgaccttttgattccttaaggacacggcaactctgatgtagctggcattgaaacctttcttctggatgctaaagtcacttgaaaaggacacatgcatctcattcgcacttgagttaaatgataggcctttggcagttgctccacaaaatttagtctggctctctccattatcaagggataatgagtcataaatgcaattgggagcttcttcaatgtcaaagtcgttaaatgttatctgaatgatataaccggtgggggctcggagcgtccacatgcaagcctggctgtttgggtagtcgttagggtagcatggagaagtaaaggtcccagaagggttggacaaaaccactcggcagttggcacatccccacactgctgagtgaggaacacacatgatatataaagcaaataagaacaggagaggactgggcttccatttccaatggcagctccacattcgatctgagcgaaacatccttccaagcccccaggtgttgattccggagagcgccttcttggcagggccaggcctctggactgaggagcggtgcctgttactccttgtttaatttgaattgaaaacacgtttt

SEQ ID NO: 10443 - RNA, 3833 nt, Homo sapiens
  source 1..3833: mol_type = other RNA
cctctagatggaagcactgtctgtgtggctattccttttgaaataggtggtagagctggatttagatttggatgtaagataggttgagttggaaccaatggagcttgaagacaaagattttcctagattatcagaacttttcttgatgatattggtagctgtcttactccaatctgagttatctgctaaccgaaatctaccacagcagagatgctgccgccactgtttctgaacattctccttcatagcacagtggaagatgaatataaataagccttgtaatgaattgaagatggagaagaggtacatgaaggggatatttaagggtccccaggcaaagaatgcaaaaccccatgtcatgcccaacagaaaggtcaagctaaccacactgcgcaggttccttaacacttcttctctcagggtccggttgcttctcttgccattcctcccacagatctgcaccattaccacaatgaacatggcaatgttcagaaaaaacatgactccaaaatacccagcacaggtcacataaaatatgactggatcttgaatccaacagaattcatcacctttttctttcccataactttcttttccatagacttcattgttgtttctgctcgctagaacaactgacaccactaaggcaggcaaaccccagccaatgatgcagaattttagaatgtatcggcgaatgtaagtgttaaatactttaactagagcaatgtacatgtgaattgcttctagccccatccaggtaaaggttgccagaaggaagaaatgcaacaggactgcaacagcaatgcaaagtccatccacattgaaggaggtgatccagccatctaggaggaagaggagattcaggaacagcagggctgtgctcaggttcatcaagattttggagggataatcccttcgcaatttctcaaaagcaacatatgtcaggagagttgctgctgaaaaaatagcagatattccacacccaatatagctgatgaaagtgaggactttagtgtttcttgcatctaactgtgaggcacttcttggaaggtccatcagaactccaaagtgtgtgaagtggttacacaggcagactgtctcacttgcatctgaatctctgtgtgcaacacatcctgacgtgttccatcctccaaaacttttgtttttgttcagatcccagaaggcacagatgggatgatgcacttcctgagttcttgtatgtttgatttttatttgaacaggatccttcagattctggatagtaatgtttccaatactgcacgccatcacataactcactaaagtttttctttggggtcctacatcctggaaaagtccagttttgttgaagaaagtaaactgtgctcttctaactaatacagaatcttctggacttaaattctcaagtaagtttggaggcaaaattacagatgccagtggatccacttgtccactctcaaaatccatctggaaatacgattcattattgcttggaagaccaatgctaaaatttgaaattgcatttgtccctggtaacagggatgatacgctgagagccaagttccgagttgtaatattcacatgtgatgtgctatttaggtctatcttgaaggccaattcatcaattgtttttaaagcttcagaagatgactcaagcaagtcactgtctgaactgcttaagatattagaaaatatattcattagagttgagccaagtgttatatcaatgttttcttctttattcacaattcttttgacctgttccacaatgttggtaatattggctgaggttaagttctgcccatcagcagttaaatttaaaatctggttagcaacttcatttgcttcttttaaacagttggagatatcaacaggtccccagtaggttaccaatgggttggtagcattgtaaaaacatatccgagaagcagaaaagccaggcttgtctggacaaggaagaacgtattcagaaggttggatagatggccagtagtagcctttgggttcctccatggcaagacaatgacccagttgtctcacattcactgtatgtagcctcaagccttcatccaaggactcattattttttaggagcttctgctgaatgatttttccttccaaattagtattgttggtagcattgtaaactagaagggcccaaagcaccaaccttggctcatcctcaaggcttctcttgactttaatcttgtcctctccagcactcaggtgaaaactgatattaacgacataaaccgtgtagttccaattttggaaggttgaattgagccattctgccaccttgctctgtacttttacctcagggtgacgaaggatgttctgaatcactacggatattctatagataattccatcttgacagagggtccccaggtctgcacagctggccagttctgctgctgggagcgggatcaggtaggaaccacagcttaggttgctttcagctttcagagctaggtttgggatattccagaagtcattttgccagtcgactacattccctttcacattacagctgaggttggagaggattttggcattcatggtaaaattccaaagtcgaaagttataaatgtccccttttagagagacaatttcattttgattggagcccaacaacaatttcccattcccaggaataactttactaatggtagaatcacatggaactgtttcatagtttcttttgaaatttacaccaatagagcccaaagaattattccaaacaaggcagagctgttcaaagctttctgcaaaaatgtcttctttttctttgacaggtaatgcattattcaacaaacattttgaatcagaaatggatagaaagtagccactcttggcctttccaaaactgagcaattgtgtgaaggatgcatttgagtaggagaaagctgtccaatcactgtcttcatggccaactttggttgcttcaaagcagagtgtgaaagcactgagctctggaatagagatgctttttgcaacagatacctggtaagcatctgatgtctggggtaaaatgaccttttgattccttaaggacacggcaactctgatgtagctggcattgaaacctttcttctggatgctaaagtcacttgaaaaggacacatgcatctcattcgcacttgagttaaatgataggcctttggcagttgctccacaaaatttagtctggctctctccattatcaagggataatgagtcataaatgcaattgggagcttcttcaatgtcaaagtcgttaaatgttatctgaatgatataaccggtgggggctcggagcgtccacatgcaagcctggctgtttgggtagtcgttagggtagcatggagaagtaaaggtcccagaagggttggacaaaaccactcggcagttggcacatccccacactgagtgaggaacacacatgatatataaagcaaataagaacaggagaggactgggcttccatttccaatggcagctccacattcgatctgagcgaaacatcatgttgacattactgcgccgaggtcccctttggccgcaagatcatcctccaccactttcccgctctgctgccgctgctccacccagggggaacccaggcgccccagccctgcgccgcggcgggaccctcctttacgccgtttctggagagttcatgggctttcccgacggcgcaaggtgaaccctgggcgcggcagcgttcagcgcagggcctgcggacgaggaagcaggctggcggcaggtccctcctcgcagggaagttggcagggtgagggcgagaagctgaggaagtagggtgtgcgtggggctggtgctgaggagaccgg

SEQ ID NO: 10444 - RNA, 3822 nt, Homo sapiens
  source 1..3822: mol_type = other RNA
cctctagatggaagcactgtctgtgtggctattccttttgaaataggtggtagagctggatttagatttggatgtaagataggttgagttggaaccaatggagcttgaagacaaagattttcctagattatcagaacttttcttgatgatattggtagctgtcttactccaatctgagttatctgctaaccgaaatctaccacagcagagatgctgccgccactgtttctgaacattctccttcatagcacagtggaagatgaatataaataagccttgtaatgaattgaagatggagaagaggtacatgaaggggatatttaagggtccccaggcaaagaatgcaaaaccccatgtcatgcccaacagaaaggtcaagctaaccacactgcgcaggttccttaacacttcttctctcagggtccggttgcttctcttgccattcctcccacagatctgcaccattaccacaatgaacatggcaatgttcagaaaaaacatgactccaaaatacccagcacaggtcacataaaatatgactggatcttgaatccaacagaattcatcacctttttctttcccataactttcttttccatagacttcattgttgtttctgctcgctagaacaactgacaccactaaggcaggcaaaccccagccaatgatgcagaattttagaatgtatcggcgaatgtaagtgttaaatactttaactagagcaatgtacatgtgaattgcttctagccccatccaggtaaaggttgccagaaggaagaaatgcaacaggactgcaacagcaatgcaaagtccatccacattgaaggaggtgatccagccatctaggaggaagaggagattcaggaacagcagggctgtgctcaggttcatcaagattttggagggataatcccttcgcaatttctcaaaagcaacatatgtcaggagagttgctgctgaaaaaatagcagatattccacacccaatatagctgatgaaagtgaggactttagtgtttcttgcatctaactgtgaggcacttcttggaaggtccatcagaactccaaagtgtgtgaagtggttacacaggcagactgtctcacttgcatctgaatctctgtgtgcaacacatcctgacgtgttccatcctccaaaacttttgtttttgttcagatcccagaaggcacagatgggatgatgcacttcctgagttcttgtatgtttgatttttatttgaacaggatccttcagattctggatagtaatgtttccaatactgcacgccatcacataactcactaaagtttttctttggggtcctacatcctggaaaagtccagttttgttgaagaaagtaaactgtgctcttctaactaatacagaatcttctggacttaaattctcaagtaagtttggaggcaaaattacagatgccagtggatccacttgtccactctcaaaatccatctggaaatacgattcattattgcttggaagaccaatgctaaaatttgaaattgcatttgtccctggtaacagggatgatacgctgagagccaagttccgagttgtaatattcacatgtgatgtgctatttaggtctatcttgaaggccaattcatcaattgtttttaaagcttcagaagatgactcaagcaagtcactgtctgaactgcttaagatattagaaaatatattcattagagttgagccaagtgttatatcaatgttttcttctttattcacaattcttttgacctgttccacaatgttggtaatattggctgaggttaagttctgcccatcagcagttaaatttaaaatctggttagcaacttcatttgcttcttttaaacagttggagatatcaacaggtccccagtaggttaccaatgggttggtagcattgtaaaaacatatccgagaagcagaaaagccaggcttgtctggacaaggaagaacgtattcagaaggttggatagatggccagtagtagcctttgggttcctccatggcaagacaatgacccagttgtctcacattcactgtatgtagcctcaagccttcatccaaggactcattattttttaggagcttctgctgaatgatttttccttccaaattagtattgttggtagcattgtaaactagaagggcccaaagcaccaaccttggctcatcctcaaggcttctcttgactttaatcttgtcctctccagcactcaggtgaaaactgatattaacgacataaaccgtgtagttccaattttggaaggttgaattgagccattctgccaccttgctctgtacttttacctcagggtgacgaaggatgttctgaatcactacggatattctatagataattccatcttgacagagggtccccaggtctgcacagctggccagttctgctgctgggagcgggatcaggtaggaaccacagcttaggttgctttcagctttcagagctaggtttgggatattccagaagtcattttgccagtcgactacattccctttcacattacagctgaggttggagaggattttggcattcatggtaaaattccaaagtcgaaagttataaatgtccccttttagagagacaatttcattttgattggagcccaacaacaatttcccattcccaggaataactttactaatggtagaatcacatggaactgtttcatagtttcttttgaaatttacaccaatagagcccaaagaattattccaaacaaggcagagctgttcaaagctttctgcaaaaatgtcttctttttctttgacaggtaatgcattattcaacaaacattttgaatcagaaatggatagaaagtagccactcttggcctttccaaaactgagcaattgtgtgaaggatgcatttgagtaggagaaagctgtccaatcactgtcttcatggccaactttggttgcttcaaagcagagtgtgaaagcactgagctctggaatagagatgctttttgcaacagatacctggtaagcatctgatgtctggggtaaaatgaccttttgattccttaaggacacggcaactctgatgtagctggcattgaaacctttcttctggatgctaaagtcacttgaaaaggacacatgcatctcattcgcacttgagttaaatgataggcctttggcagttgctccacaaaatttagtctggctctctccattatcaagggataatgagtcataaatgcaattgggagcttcttcaatgtcaaagtcgttaaatgttatctgaatgatataaccggtgggggctcggagcgtccacatgcaagcctggctgtttgggtagtcgttagggtagcatggagaagtaaaggtcccagaagggttggacaaaaccactcggcagttggcacatccccacactgctgagtgaggaacacacatgatatataaagcaaataagaacaggagaggactgggcttccatttccaatggcagctccacattcgatctgagcgaaacatcatgttgacattactgcgccgaggtcccctttggccgcaagatcatcctccaccactttcccgctctgctgccgctgctccacccagggggaacccaggcgccccagccctgcgccgcggcgggaccctcctttacgccgtttctggagagttcatgggctttcccgacggcgcaaggtgaaccctgggcgcggcagcgttcagcgcagggcctgcggacgaggaagcaggctggcggcaggtccctcctcgcagggaagttggcagggtgagggcgagaagctgaggaagtagggtgtgcgtggggctggt

SEQ ID NO: 10445 - RNA, 4285 nt, Homo sapiens
  source 1..4285: mol_type = other RNA
cctctagggaagagaaggttggactagtgtgttaccctgatgtgacctcaacattcaccctaacatggaacccaaatgccagagctaagaccaccattagcccttccaatccttaacccaatactaaatcctgccttgaccccaatcatttttctaaatgagagatgacaacaaagtcttactcctaaactccaacatcaaaccccaaccctaaatgccaaatgtaatcccagccttaaagcccagacatctccaaaaacctaatgcccacatcaatccccaaccatgactccccaaattcaactttagtactatccaacactttccaacccaggctccaaatcccaacttcatcgaaacatacactacagccctctccccaaactcaatgctaaggctaaacccagtctcagctccaatcctgtccccactaatcctaacaacaaccccagctccagcacccctagtcctaacagtcatcctggtgcaaactgaatcccaacctcactggtcacctgcaaccactgccattcaccagaatgtggtcagtggctggaaaatcacttcctctctccacccccacttcatcccctgtaaacctcacatctcccagccaggctctagccaggatttacagccatccctggccccagtgagaaatcagggttcaagaaagcagaagacatgcttaaggccccatgagtgaatagtgcagcctagattcaaacccaggtcccctcaagcacctactctttctactcagcctaaaagttctcaaaatccaactctagccctaccataaattccacccaagccaaacatgctgaatttagccttgctctaacatcaaccaaatcggaccccagattccaaccctaacccctacactgattgtagctaactctgaatgtcagttctattggaagtactcttcatcttaaccctgggccagggcttccaagctttgtctcccactgttcccacggtgattcttcctgaagcatagtgatgatctgcagcagtcatttctcttaaagctggcactcttattaaaataacttttgatttcaggagactttcaggtcaccatcaaacttgacgttgagcacaaagtccttgtagaggcggcgcccgttaactggccgcatcgcgtcacagagccgggtggtgttggggcagagggcacggtgcatgttgtggagcgcatgggccatggcgtacactgcattgaccacaaacatgatcttggactcctgctcaaagggcacagcccggagagagtgggctgcgcagtctcgctgccggaagctgcagcggaacctctgctcccagaattcacggaaccaggggttccggctgttgttccaagggtccaggctctggaagtaggaggcaaagtcactgatggggtaggaggccagctcgatggtgatagcaccctcagcagccccctcactgcctgccaccacactctccagggccccccaaccatcactggccacccaggtgaagctggcattgaggcgctggctggcagcaagcagctcccgggcatcctcagaacgggtgaacaggacagccacgcgggcactgggcttctgcagcagggctcgcaccacaccctcaaaggccgcgcggctcatggcacggcccactttctccgaggtggccacacagatgttgcgggcacgagcctctagctcaaaggcctcaatgcctgtctcgccatagtcgccctcagacgccacagtggacacataggtccagttgaagaagcggagaatctcagccatggccttggcttggaagaagtcaggaggcactgtgcgggcaaagtagtcatagcgggacttgtcactcagcttggcactggtagaggcgtagctaatctgtgggatctgaaatagcctcaagaggttggccacctggatggagacatcactgtaggaaccgccaataacaccagtgatggcagtgggagcatcaccatgggtcgcataagagccgtcggggcagatgtggcgtgagccatcagcaccacggctgagtgaggcacgcacaaagtccagtgcctgctccagcgcatgtgtgtccttggagcaactgtcgaggatgtgtgcacccaggcgcacgccaggcagcaggtgcgggtcacggttgatgcggtccagtgcaaaaagcatggcctccaggcgctggatgccacggtgctcattgacaggaccacagtcctctgctgggccgcccttctggtgcactgggaacagcccacccagcaccaagtctccctccagggtcagcaccttcttggctgggccctcagccacagcaccccacagcagcagcagtgccaggagcgcaagcagcgatcccatggccccaaaggggatggatgggtcccgcagacctgggtctccaggggatgagattagaagcagcgaaggcaaagagaggaggaaacagggaccaggaaaggacagacaagaagagagatgcgaagggacccagctcctgcagagagatagaaagacagaaaaacagaccaggaaaagtggaacctgagagcagctgccccttctgactctgcctccccacgagcccctttcctaggtactcaaaagccagggagggacaggatggtgtcattaagtaggttgagaagctcctgggactcccctggacctgtctctcagccctggcctcagcttggtgagagatgggccatattcccctaccaaactcagcagtggggagagatgcaagcagtgaagtcccaggcagaggacaggagaccccagccaatgctgacccctctgtaattcaaagggtgtccaagaacagcacaaacctcccaggaccccgaggtcaatacctttggaacagactatgtcacagtcacaaactcagaggtccccatcctgagccttggatttccagagagaaggaactgctgtctcaggacccaccagggaagaggaagggaagcatctctaagggacagtctccaacccgtggggagactggagcccatgtgaacacccaagggttctaacctttggttcttaaaaagccatccccacagtttgctgactgaggaaggaatagagacactaagccctgggaatgagacagcaaggtggaatggctggcctcagggagggtacccaagtggctcaaggtcctaagtcaacagggcaagcagatgttcacgtatgtgtgtgtcagggttgggggctagagtctccaaacagtgctgagggtgagagtgcgggactctctagctctgtgtagaacactgcttgagattttgtgcctctgttttctcttcactcccgacccagcagagaaagtcaccatttccaatctccccatcctcagcttcagggccctgcccaccctagccatggccctcagagaccccctccctgtctcttccccactgcgtccaatcatttgtaccccagttgccttcccaaacacacaccccacaaaggctctcacaatcacacaggcttggaaaggctgggagagggacatacctctttcctcagaacaggaaaggaaactgagtttgaagaagggcagcaactaactcaaggaccccatgtgctggccacggaggctgagcctcttcattttgccccctcagctccccagggcaggggcactgggctcctctggggatcaggaaagcagcagcttacccaggcaagcgagggagaagcagggaggaagaccagcacagatggagacagggacccagatgggggctgaagccaaaactggtcaagtcgcaagtctcccagaggggaggcccagacggaagctcagaggcaggaaggggacagaaacccggagtcagacagccaggagcctgggccacaaaatctgggcagggagcgagcaagcctgagaggttgagacaaagacggaggcacagacagaaagaaggaccagaggacgctggagcaggaggaacgggggagtgcgatgtggggcgtgcgttttctggagaagaaaggcgggacgcccggggctgtcttcccgcttcccggagctctcagggaacgctgtctggacacagcagcgcgggcgccccacaacttgagggcccgcaggaccctgggacgtgaggtaagggccaaaaaggtcggcagcggcagcggcaccaccaccaccggctcaccctacctggcgcgctggctctggcgcggagagaatcggagtggagcggggggcgcgaggctccggctcccgctcgctcgctcgctggctcgctggctct

SEQ ID NO: 10446 - RNA, 2837 nt, Homo sapiens
  source 1..2837: mol_type = other RNA
cctctagggaagagaaggttgggctacaaatggcccatgttagtgcaaactgggtataatgttcctactattctaagattgagtccagttagatgaataactggccataccctcctatcacataagtagagaatcttgtgaaatcacaagagttcaacaggtaaagtactatggccatgaaatccacaccaatttgaaagataggcataggctcagaccatttaaatccatctagttatacacatgaattaagttagactagcaccagccacctgtgaatatgagcacttttccagattttcacaaaagagacagtgttagcacttgaaaaagtcatcgacagaaaactgccactttaaaactttagcttaacttaaaattacatgggaaatggaaacaatcagactaaaagctctttctgagactaattttttcttcgatctactctaataatagaacacatttaaatctcagtacacttgaaaacagtacacaaaaatagatacatataaatattaagaatgaggatctaagttagtgcttctctgtgttagagaggtcacagctaaagtcctagtgatattgcctcagattgttacccgtatttaaaattaaaagtcacatcaaacaagtttagacgtctttacccaataataccctaaatgctcttataagagtgcatagttgtcctgattcatctggtacctcagttactatttatcacaaaattataaaatgaaatgattaattttatgccaggaaaaaaaaatgctgataattgcactttgttatcttttccttactgaaatgaaatgtcacaaggatgaaggaaaatccctccctaccctgcaatctttaagcatacccattttccatgtataaaactctctcagctttctgaaatactgtcagcactcttttgtatcaaagacaagtttcctaagaatgagatgccagtgatgcactaaggcctgctactcatttagagtactttctgaagacactgaggatacagtttagcaacagcacattcaaaatgccggccaaggtcccagagccgatctggggtctcatacactttcatccactggtcagcaatgtcatcatattggtaaagggaattttttctgctggttctgaagacgtgttcttcaacagtcacttgagtagctcgaacaaataaatggagtttgttctggaaaagtaccagtttaaggtatggatttatggactgatcacatggaaagtctttcttacgagtccatttatttagctcaatatcataggcttctacagtaaacatacgttgatgatttccacaggttccagctatgtagtagatagagtccttgtatacagctgctaagccctggattctaggcacagtcatgggggttaagaaaccccagtagtctttttgaggctcatagaagagaaaaaattctccctgtaaaacatagatcttctctttgtactccacagcattatgaaattccattgcaactggcatcgcgcaaacagtcgtccaacaattctctctactgtcgtagcactcaacagattttagtgagtttctcccatcaccttcataaacacgacctccgattgcatacattttaccacagcaatagacaagtttgcagcctattctggctcgaagcaaggatggtttggatagccatctattggtggaatgatcatacatccagaaatcattttctgccttatggtcgatggagacctcactgctgcttggcctgtaccctcctgcaatgtaaatgtcattatctggtgatacaagaatcccaacttctctcaggtcatttggtggtttgcatagtttaaacacccttcctgtgactatatctagacaaggcactgtttgcttctttcctgagtgtttgtgggcagcatcaaaacatatgatcatttcagaagcagtcattccaagcctctgtgtacagccattggtgttggatggtcccttttctacacagcttttggctatagcctgtgcaaactgaggtggaattttctctataaaggtatcttccatcagaggaaaacgtatgcatttagcaaaaatttctggaaggtgcacttctctttcattctgttcatgctcaaaccaccttataatgctttcataaacatgctcttctcggtctacatttaaatcgtcactgtctagtatacttatcagttggtcttttgtcaactggagaaactcttgttctttggtgacacacagaaactttttacgaatgtattcttttgatcgatctccgagttcctgatgaccataatgatcagcaaagataaagaccccaatagaattctgtgggtccaaatgactgatcatatacttagcacattggtcttggatggaaggaatctggaagatgctagctgcagtgaacaaggcttgaacattggcctctgtaagaataactctggaagtgtaggcatagttcaacactaaatccatcgattcagcttcaacaccaactattcgaacttctttttgagtactttctgtaaggccgctagtgaacatggatctgaagtaagggctgattgcagcaagaacgtttctatgacaggaaaatgttttcccgtgatccacttccactacaatgtctgtcaactgtccttcatcgtacattgttttgagttgcttaagaatactgcaagcatggaaggggtccatggcatcgctggctgggtctgaagatggaatcccattcggtgttggggaagacttacttaaatctgccgacgcggccatttctcgatggggccccgactccagctatttaaaaaggaaatgtcatttc

SEQ ID NO: 10447 - RNA, 2626 nt, Homo sapiens
  source 1..2626: mol_type = other RNA
cctctagggaagagaaggttgggctacaaatggcccatgttagtgcaaactgggtataatgttcctactattctaagattgagtccagttagatgaataactggccataccctcctatcacataagtagagaatcttgtgaaatcacaagagttcaacaggtaaagtactatggccatgaaatccacaccaatttgaaagataggcataggctcagaccatttaaatccatctagttatacacatgaattaagttagactagcaccagccacctgtgaatatgagcacttttccagattttcacaaaagagacagtgttagcacttgaaaaagtcatcgacagaaaactgccactttaaaactttagcttaacttaaaattacatgggaaatggaaacaatcagactaaaagctctttctgagactaattttttcttcgatctactctaataatagaacacatttaaatctcagtacacttgaaaacagtacacaaaaatagatacatataaatattaagaatgaggatctaagttagtgcttctctgtgttagagaggtcacagctaaagtcctagtgatattgcctcagattgttacccgtatttaaaattaaaagtcacatcaaacaagtttagacgtctttacccaataataccctaaatgctcttataagagtgcatagttgtcctgattcatctggtacctcagttactatttatcacaaaattataaaatgaaatgattaattttatgccaggaaaaaaaaatgctgataattgcactttgttatcttttccttactgaaatgaaatgtcacaaggatgaaggaaaatccctccctaccctgcaatctttaagcatacccattttccatgtataaaactctctcagctttctgaaatactgtcagcactcttttgtatcaaagacaagtttcctaagaatgagatgccagtgatgcactaaggcctgctactcatttagagtactttctgaagacactgaggatacagtttagcaacagcacattcaaaatgccggccaaggtcccagagccgatctggggtctcatacactttcatccactggtcagcaatgtcatcatattggtaaagggaattttttctgctggttctgaagacgtgttcttcaacagtcacttgagtagctcgaacaaataaatggagtttgttctggaaaagtaccagtttaaggtatggatttatggactgatcacatggaaagtctttcttacgagtccatttatttagctcaatatcataggcttctacagtaaacatacgttgatgatttccacaggttccagctatgtagtagatagagtccttgtatacagctgctaagccctggattctaggcacagtcatgggggttaagaaaccccagtagtctttttgaggctcatagaagagaaaaaattctccctgtaaaacatagatcttctctttgtactccacagcattatgaaattccattgcaactggcatcgcgcaaacagtcgtccaacaattctctctactgtcgtagcactcaacagattttagtgagtttctcccatcaccttcataaacacgacctccgattgcatacattttaccacagcaatagacaagtttgcagcctattctggctcgaagcaaggatggtttggatagccatctattggtggaatgatcatacatccagaaatcattttctgccttatggtcgatggagacctcactgctgcttggcctgtaccctcctgcaatgtaaatgtcattatctggtgatacaagaatcccaacttctctcaggtcatttggtggtttgcatagtttaaacacccttcctgtgactatatctagacaaggcactgtttgcttctttcctgagtgtttgtgggcagcatcaaaacatatgatcatttcagaagcagtcattccaagcctctgtgtacagccattggtgttggatggtcccttttctacacagcttttggctatagcctgtgcaaactgaggtggaattttctctataaaggtatcttccatcagaggaaaacgtatgcatttagcaaaaatttctggaaggtgcacttctctttcattctgttcatgctcaaaccaccttataatgctttcataaacatgctcttctcggtctacatttaaatcgtcactgtctagtatacttatcagttggtcttttgtcaactggagaaactcttgttctttggtgacacacagaaactttttacgaatgtattcttttgatcgatctccgagttcctgatgaccataatgatcagcaaagataaagaccccaatagaattctgtgggtccaaatgactgatcatatacttagcacattggtcttggatggaaggaatctggaagatgctagctgcagtgaacaaggcttgaacattggcctctgtaagaataactctggaagtgtaggcatagttcaacactaaatccatcgattcagcttcaacaccaactattcgaacttctttttgagtactttctgtaaggccgctagtgaacatggatctgccgacgcggccatttctcgatggggccccgactccagctatttaaaaaggaaatgtcatttc

SEQ ID NO: 10448 - RNA, 327 nt, Homo sapiens
  source 1..327: mol_type = other RNA
cctctcctccctgtgccccagaatctcgggttggttcttcaaaaacccaaccaagacgactgaggacacactggctggacggttcagacgaggcccgcagccctccattatgaagtgcgggcccacgaaccctgactacaagtgccccaggataaaacagagcctgcattatacttggcaacgatgtctggggctcagtactgtaaccatgcaacgctggacttccgccgaatgggcttttagtgggcaagcagagcggtgaaccccgaggtccagctcccggactgtgctagagcgggcggtgcccgcctccttcctggagcgcga

SEQ ID NO: 10449 - RNA, 1889 nt, Homo sapiens
  source 1..1889: mol_type = other RNA
cctctcctccctgtgccccagcaaggtggggtggggaccggacccaccaccgtcccacagctctgagacgtggtgggctctgtcctgtgtctcctgcgtgccctcctcccccgattccccagcgggccacgcgggccacaccacctgacctttgttcaggctgggtcctgctgggaagtccttccactttttcttcctgttaaaatcttgctcttccagaaaggtctgtcccacccagtgctctagcgtccctgccaggacaaggttctcagttctctctcctccagggagctcagcccgtctgttctgagctccaggtctcatcccctgaccccactacagacgtcccaggtcgaaggcccagggctggccgggtgtctcttcagtggagggcgtgaacctgtcccaggtggtggctgaggcaggccctctggacaggctctctcagcacccctggagtgagggccttgggttctagccacacaaggctctgtagcccagacaggctggagaagcttcccgggcggctccgtctggtggggggctcttttagggagggggacggccactcccggaggtgagcactttcggagcagagtgtggcggctgcacccaagcacaggacaaggggccgtgagcctggggtcttggcgtgcccggccccagcatgccacctggcaaaggtgggagttctggaagcttccttctaccctgggaccagaagccccctcctgcttcaagggatctcgtgggtgaggaggggtgggccagggtcgggaggagggggtctcttctcaaaccaggactgggacctgcacaggtgggagctggaagggcaccacctccacccaggcatggcagggccactcatttgcatgcaggggccaccgaggcgagagccgccaccaccgccaccgctgaacggatttgagcagaagctccgttttccttctgttcttgtctctctcaaggtcagagcccaagcagggacgggaacaaaggcggtgcgtcccccattcaacctccccgcgcccgctggccgctcctagaggaaggacctggggaagggaggggagggcagggcgtctccgaggcctggccctgggcgaggctgccccggcaaacccctgcctggcaggggggccactgtgggggtccaagaagccctgttccctcctggggctgggagctgtcccggctttgggacgcagccgcggccggaggtcactctagagtaagcttcctgtggagccaagggtcagaaatcaggctcactctgggaacaggtgtccgccaaggtcaggggttatccagggtcgccctcagtccctggtctggagccagtacagggcttgatggggtctggccccgccccctgctctgcactgctgggactggggtctacccagactcaggaagggacttgtccagcccgtgcccagcacccactgcccacatggccaggccacagggcttgggatcagcgtcccgcagcccctcagccttcaaaggccgcgacgccaggaggaagctaaaaatatgcggggagaatttctcattacagaataaattggacccaatgcgctgcctgccctggtgccggcagccttcagaagccccatctcagccaggcaaggatcaggcggcaggggtcacggggcgctggggcccgggcaggtcacaggctccactcagggcgggagccccaccgctgtccatcgccccccacctgcgaagcacggagctggggtctgcgcttagccccaggggccaggggcgtttcccctgggctgggtcgctgtccttgaaaataaaaatgtatccctttctccagtgggtaacatgaaaatccccacccccatccagccatggacccaagattcctgcaa

SEQ ID NO: 10450 - RNA, 1331 nt, Homo sapiens
  source 1..1331: mol_type = other RNA
cctctgaaattcagttcttcagacacaccaggtacatttcaagtactcagtaggcacatgcagctagtggctaccttattgaacagtggatcctggctattcaaatggaaatgcttccaccagtagacacagtaggagccccactgaattacgagccatggctgataactgaattacaagtcatgggaaccttgggttcattcctcctgctatggctgtgggactaagcaggtgtaaagaagagtagccactctgtcaggggtattggctctgatcatcaggaggaggcagggttgttcttacacactgtgaacagagaaggatatatttggcacccaggtgatccatttgaatgtctcctaataattccctgcccaatttttatggtaaatggacacatgcaatttccacagtctgagaagggcacggggaccatgggctcagaaacaatcctcagggataaaggtctgttactcgaccagccaggtcactgagaacggcagacatggtggctgagactgagggtactctctgcttctgctccctaacagcaagcagtgtgcgccccgagccgcgtttctttcctcactggcaggagacctgacaccacccgcctgtacgacttcaactcctactggagggtgcacgctggaaacttctccaccatcccccagtacttcaaggagaatggctatgtgaccatgtcggtgggaaaagtctttcaccctggtactgctccacgtccagagtctgggttctcttggtttgtggtgtctgaatccagcattcccatcctggggatggggctgtctttgcagagccctcttctggctgggcgagtccttcgctagtcagtgcttcctttctaaaaaaccgacttgtcaacccagccacatgttttcacccaaagtgaaaaagggtagaaagaactttgcttcctttcagaaaccactgagggtgtgctgttgggtccttcagctcctcgggtggtagggaggacacaggctggggaggtggcagtgttgggtggagtccagctcagggccccaccctctcccctgcagggtacctgtcagtaaacctaggggtggggtgaggacacctgagggcctcccgtgtggccagcattgctgttgctgacttattgcccagtgagggggctgtgcttaggtgggggctgctatccactctgtgaattaggtcagaaagatgagtgtaatctggtttctgcacctggtctcagaagctcccaggtctgggaatgggaaagcgcacttcaacaggtgtctcaggtggtctggccacctctctttgagttcatccttcccttg

SEQ ID NO: 10451 - RNA, 2127 nt, Homo sapiens
  source 1..2127: mol_type = other RNA
cctctgggcccttcctccaggcgtaagagggcatagcgagccgcactgagagacagacctcgtatcccatcgccccactccttctctgccccacggtactcaatgtacttgtagatgagtccagcaatgagcatggctaccagtgcataataccaggagcagatgaacatgagggccaggcagaggctcatgcccaggaaggagagggtccagtggtaatatcgaaagcgtggcctccagttgggtgtcctcagcagcgtctgcactgcacaggccagattcacaaacatgtagcacatcaggaagaacatagagaggatgggggccacctcgtcgagggatgcaatgaggatgccaatctcgcagatgcaggcagtcaggagcagggcccaggtcggctctccattggccttgccatggccaaagacctgcaggaagggcacaatgccatccctcgagatggcctgcagcaggcgtggggcccccgtgaggctctgcagcccagccccacaggtggagaagaaggatccgatgacaattacccatggagatggccaggccagagtgcccaccacgaggttgccattcacagcttcgccaaacttgtcccgcaggacgaccccctcaatgcaggccccaaacagaacaacggagctgatgtagacagcagaggtggtggcgatggccaggatggtgccagtggggattgacttctgggcatccctcaggtccccagagcggttagaaccagccatgatccctgtgactgaggggaagtagatgccaaccagcagggtgaagtaggaggtcatatcactgaagacataagggtggtccatgtcgataggagtgccatcggccaggcccaccgaggtcatcccactcctctccacaatcacgcccttggtcaggtaggagctccagaggttctctttgatgaggccactggcagcaccagggatgccctggatctctgtgacattgtttcgggtgaagtattcatcacaggtggcgttgaggaagcgagaggagcagaaaaggccccatagccgtgtggtcaccgtctcatttccttcccaagccagcttggcacagacatcaaagccatggcgagacagcgtgcggttacccaggaggcagatcgggaagttgggtgggtcgaaggcagacttgatgaccccagcatagatggccaggatggagaggatgacacaacccaggaagacaagggcaaacttgttgacatacttgacacccacaaacaccacagtggccatgcaggtgagcacacaggtgccgtaaacacgcatgttgttcagcatggctgctgcctccccactggcatcttctgccttgaagatggccatggctgggaagaggtaagccagcaggatttcgatggtgcccaggatgtacatggctcctgcaaaggtagtgcccaggtagaagcagaggcccacggcacccccaaactctgggcccagagacctggaaatcatgtagtaggagccaccagcaggcacaacaccattcgttgcaattgcactcatggagatggccgtgagcatcgtacaggagcagcagatgaacaccatgcagaaggactccatgatgcctgcaatgcccaccacccaggtgagccgcaggaagaggatgacgccaaagatgttctgcaggcacggcaggtacacgcccatgaaggtgcccatgcgtggggcctgcaccggcttcttttttccaccctcattgttttctgcctcttcatgctccctacttccctggggcaggttggtgtagttggccaggccactgagcaaggaggacaccatagggctggtgtccatctcctcctcaaacaaggccatgttcttgccatcatactcctttcccttctctgtgtcggtgctgttgatgaagggactgctttccttggggttgccatcacccgggttggctcccccatcgccgtcctcgcagtccgtcaggttgtttagcatggtggcggcgcggcccctggtccggggatggctgcgccgcctcgcccgcgcccctctacccgccttcgccgctctctcgttcgctgtagctctgtctcgctctccgctccacggaggaagaagctgcagt

SEQ ID NO: 10452 - RNA, 2146 nt, Homo sapiens
  source 1..2146: mol_type = other RNA
cctctgggcccttcctccaggcgtaagagggcatagcgagccgcactgagagacagacctcgtatcccatcgccccactccttctctgccccacggtactcaatgtacttgtagatgagtccagcaatgagcatggctaccagtgcataataccaggagcagatgaacatgagggccaggcagaggctcatgcccaggaaggagagggtccagtggtaatatcgaaagcgtggcctccagttgggtgtcctcagcagcgtctgcactgcacaggccagattcacaaacatgtagcacatcaggaagaacatagagaggatgggggccacctcgtcgagggatgcaatgaggatgccaatctcgcagatgcaggcagtcaggagcagggcccaggtcggctctccattggccttgccatggccaaagacctgcaggaagggcacaatgccatccctcgagatggcctgcagcaggcgtggggcccccgtgaggctctgcagcccagccccacaggtggagaagaaggatccgatgacaattacccatggagatggccaggccagagtgcccaccacgaggttgccattcacagcttcgccaaacttgtcccgcaggacgaccccctcaatgcaggccccaaacagaacaacggagctgatgtagacagcagaggtggtggcgatggccaggatggtgccagtggggattgacttctgggcatccctcaggtccccagagcggttagaaccagccatgatccctgtgactgaggggaagtagatgccaaccagcagggtgaagtaggaggtcatatcactgaagacataagggtggtccatgtcgataggagtgccatcggccaggcccaccgaggtcatcccactcctctccacaatcacgcccttggtcaggtaggagctccagaggttctctttgatgaggccactggcagcaccagggatgccctggatctctgtgacattgtttcgggtgaagtattcatcacaggtggcgttgaggaagcgagaggagcagaaaaggccccatagccgtgtggtcaccgtctcatttccttcccaagccagcttggcacagacatcaaagccatggcgagacagcgtgcggttacccaggaggcagatcgggaagttgggtgggtcgaaggcagacttgatgaccccagcatagatggccaggatggagaggatgacacaacccaggaagacaagggcaaacttgttgacatacttgacacccacaaacaccacagtggccatgcaggtgagcacacaggtgccgtaaacacgcatgttgttcagcatggctgctgcctccccactggcatcttctgccttgaagatggccatggctgggaagaggtaagccagcaggatttcgatggtgcccaggatgtacatggctcctgcaaaggtagtgcccaggtagaagcagaggcccacggcacccccaaactctgggcccagagacctggaaatcatgtagtaggagccaccagcaggcacaacaccattcgttgcaattgcactcatggagatggccgtgagcatcgtacaggagcagcagatgaacaccatgcagaaggactccatgatgcctgcaatgcccaccacccaggtgagccgcaggaagaggatgacgccaaagatgttctgcaggcacggcaggtacacgcccatgaaggtgcccatgcgtggggcctgcaccggcttcttttttccaccctcattgttttctgcctcttcatgctccctacttccctggggcaggttggtgtagttggccaggccactgagcaaggaggacaccatagggctggtgtccatctcctcctcaaacaaggccatgttcttgccatcatactcctttcccttctctgtgtcggtgctgttgatgaagggactgctttccttggggttgccatcacctttgacgtcttcccccgggaggtggcgggggtctgcgaccgaatgccggcgggactctgggtcagggcttctggcgggccctgcggggggcagcgaggtgaccgtgaacctgcggctcatggcgcggaaaggagccaggcggccgcggcaaggtccgggatcgcacaagtggctgcaaccaggctctaggagggagaaag

SEQ ID NO: 10453 - RNA, 791 nt, Homo sapiens
  source 1..791: mol_type = other RNA
cctctgggcccttcctccaggggcgctgctccgccctgtctgcttgagctgagtcaggactggccgttctagctgcggcagccacccttactcctgccgctgtcccatcctctctgcaggtcctcagtgcttttcctctgaatggagcctgccacctccctcctctctttttgggccattatttatgaggcttccttcctgggatttctctgcgccctctctgctcagcagtgagctcctgtgcaaagactatgggctgcatgtgctggttctaatcctgcttctccaaccctaataaagtatgacctgccacactttcctcacctgtgacatgaggatgacaatccttccgcatttatcaggtaagcctgataaatggccactctggataaatgtcagctcccactcctccagcttggttcccatcccatcttgcactccacctgtggtcccagttttcttgctttggcaaatgtccctcccaggtctagagtggtcccctaacctctagcctggaggctgggtggcagtgctccctgctgcaggggccagttcctcccgctcttctttccacctgggcctggctcctgccatccctgttgtttcatcttgacagacagatgaaatatatatctagatgaaatctagatagactatctatgaagatatagatgtaaatatttatatttcatatagatgaaatatctatgtatttcaagatgaagcaacacagaccagcatttcaaaagaggaaataaagccaattagtaaacttgaaaaaatatttgaca

SEQ ID NO: 10454 - RNA, 2447 nt, Homo sapiens
  source 1..2447: mol_type = other RNA
cctctgggcccttcctccaggtgtcctcgacttccccggcacgggctgatttgcctaattaccaggtgtgtttccagcccgccttcctcctaaatggggcctcaaccttatctggagtcccaatgccctctgaggagtcagagtgaatgatcagagccgaaaccttctgtcttcctgcactgagacccactgatatgtttgcttaaatgggctgcaaaccaggaccagaccaaccagtccctacaggctgtgggagccggctctcaccagcactccaatacccctgttgctgaattaggaagacatagcagattctttcctatctggggcagagaaactactctctgtgaacatcaggctggtggtgagtcggtgtaggagggcctggaaggtggcagtgaggacggggccacattcccaccattaaccgaatctcaacagtagcacagggaccccaagcctttgcccaaaagcacaaggcagaacttgcaagagctgcccaagccagggctcagcgaaaaatcacacgggctatgcttatccacgcttctaagacggccaaccgcgagcgcaggcaggttcacagattcacacgggctatgcttatccacgcttctacgacggccaaccgtgagtgcgggcaggttcacagattcacacgggctatgcttatctaggcttctacgacggccaactgcgagtgcgggcaggttcacagattcacacgggctatgcttatccacgcttctacgacggccaaccgcgagtgcgggcaggttcacagattcacccgggctatgcttatggggccttctacgacggccagccgcgagtgcgggcaggttcacagattcacacgggctatgcttgtggggccttctacgacggccagctgcgagtgcgggcaggttcacagattcacacgggctatgcttatggggccttctacgacggccaaccgcgaatgcgggcaggttcacagattcacatgggctatgcttatccacacttctacgatggccaaccgcgagtgcgggcaggttcacagattcacacgggctatgcttatccaggcttctacgacggccaaccgcgagtgcgggcaggttcacagattcacacgggctatgcttatccaggcttctacaacggccaaccgcgagtgcgggcaggttcacagattcacacgggctatgcttatggggccttctacgacggccaaccgcgaatgcgggcaggttcacagattcacatgggctatgcttatccacacttctacgatggccaaccgcgagtgcgggcaggttcacagattcacacgggctatgcttatccaggcttctacgatggccaaccgcgagtgcgggcaggttcacagattcacacgggctatgcttatccaggcttctacgacggccaaccgtgagcacaggcaggttcacagattcacacgggctatgcttatggggccttctacgacggccaaccgcgagcgcgggcaggttcacagattcacacgggctatgcttatccatgcttctacgacggccaaccgtgagcacaggcaggttcacagattcacacgggctatgcttatccaggcttctacgacggccaaccgcgagcgcaggcaggttcacagattcacacgggctatgcttatccatgcttctacgacggccaaccgcgagcgcaggcaggttcacagatgtctccgtaaagagaagagtcttgctgcaggactgccttccagacagtcctggccactgaggaggcccagccagcccagatccagcggcagaacaggcaggctggctgcgggctcgaggccacggtgctcctcggcaaaggtggactccagcacagacacacaaacgggcttccgtgggtgaaaaggatgccccttcacatgggccgtaaccatggggtgcttcctgggcccagagcccctctcttgcctcacgcgggcacgcgctgccatcactccgccttgaggaggaatgggagcaagaagctggggcctgctcatcagcacggcgcgggatggagggaaccagaggagggaagagcttcgccctctgcagagctctggacgtggacacggtgccccgtgctgcctagatcactatggatgtttctgtttagaacacaggccgcgagatgaacaggttgggaaggcttagacatctgggagtgcgcggggctgcgaaacagcagaaccccagagccagtgctctaagggtgccttagaggcagatggcctgagagccgggcagaagggggaggggcaggagaaagggcgggggatacctggaggaccagcaacgtggggcatcctagcgtaaagagcggggcctgcctgtgaaaaagtttagcatccaggccaggcgtggtggcttacgcctgtaatcccagcactttgggaggccgaggtgggcggatcatga

SEQ ID NO: 10455 - RNA, 8459 nt, Homo sapiens
  source 1..8459: mol_type = other RNA
cctcttccccttgtctctccagcccctaacacaggggatgcctgaccccaaactagacgagttacttgacctctctgacccaagacaaaatgggaggaaagtgccaaatttccaagattggccaggggattaaataagataaatatgcaagtctcttatctgggggtctggcttggtaaatataaagttcttttttcttttcttcctttttcttttttttttttctttctttttgagacagggtcttactctgtcaccaaggctggagtgcagtggcatgatcatggctcaatgaaacatcgacttcctgggctcaggcgatcctcccacctcagccccctgagtctcttggactccaggcgtgcaccaccatgactggctaattttttgtatttttagtaaagacagggtttcgacatgttgcctaggctggtctcgaactcctaggctaaagtgatccacttgtctcagcctcccaaagtgctgggattatagacatgagccaccatgcccagctaaaagttcctttttaaaatctgcttgttagatacactcatagaaaggtaactggccacagaagggagaggaatggcagtccatccagggatcactggagtgtcatatgaaatgttataggaatcacaggccttagaacttgaaaggaacccaaggatcatctaggctactttatgcaggtaaaacagccacctgtgcccatcacatagctggggcacagctggagaccccaacagagaggagagctgatgggtgacgagaaatcaggcctctccgccacggcagcctagctaatgggtcttggctggaagctaacaggaaggcctctttccagaaacactgtaagccagtgtttctcagattgctgggtgtaattcataggcagatcatgaaatcagtttaatagctttgaccagcattaacctatttatgcctagcgttcccttattggaacactaagtctgtgagagttatttacatcctactgcttaaggtcatcgccaaaatctgattttttacacaaaaaatttgcaacctccagcataaatgggttaaaacaagacaaaacaaaacaataccagaatggaaaatagtgcatgatctgtacagtatagttgtagaaaacttcttgttttatcatttgatgtcatgaaagtccctgctgtagataaaagatggagcttgtgcttctgagtggtcatgctcaacagggtggggagcccaggggagtggggagtgatcgtatagacagaggtgggtggggccagtgtgagcctgatggtcaattacttctcatttctagggaaaattgaaggaaaagaaggagggggatgtggaggggagagaaggcctcagtagagtttgcactattattagggcaagtaagctgcttctgaaaagaaggggtttgcaaagccaacccaggcaaaagcaatctgctggaagaacttcatccccagctgacactgtgggaaggaccccatgcagaagcaatagggcagcctggtcccatatcctcatgaaatgcctcttataattgtgacatcttgcaattgtggaggactttacacttttcggagttcctagcccctcacttatttctcgtaagaccgctgggaggtggggggatggtatcatcatcccactttagagatgaggaaacaggatcagagtgagctaaatgactgccagatccaaaactagaattcagacctcctagtttctaagtggacgctctttctacaccaccataatgtgagtgttctgtgtttacagggtgtattcaagtccatgactgcccattagaatccccccaaaaaattccaggactggcctgagttgctccttagaccaatgaaatcagactcctgggagtacggcccgggcctcgggatcctttaaagctccatttggagagcctcgggcacagccaggttggatccatctcccagtcccccagccttggctcagcctggccaagctgcccaggaggtcccttggtgccctgggctctgtttcactgttgttttgtagagcaacttcccagtgatgctgccactgggccccatcctaacagtgaagtcccccgggccctcctgagaggaggtgtgaactggaagatggggaggcaggcggctctgacagacagaaagcaaacagctcagaggggtggcaggctgcattttattcatcgttaatttaaacacccttcaagtcctctcttggaatgctgctcagaaaaatagatgtattgtttgagaaaccctgcaggcttgtcccgcatgctctagccccctcctgagagaacagatagcataaaaaatgatttgtaaagcaagggggagcttccttagggaagaaggggaaggggaagagggtttggggccaggtccgagtgcagaaatcctcaatgcatgagactagcgtggaaggtgtagcaattgtgctctggggtgcctgaaagtgccagagctgcttcaggggcaagagtccaggccccaagtccatgctgatgagcccaccctgggggtcaggaatggcctcagcaggccctccctccctccctctccaccctacaaagtgaggagccttgagtcaccaccagcacattatacaacaatacaagaaccctgcaacagataaagccccagcgcctcttctggactcagatgccctaggctggctgtctggctgtgctttccagacagtgtgtatgtggaattgtgctttttgttttttaagaatgtaaaaagttacagtaagatcgaaccacagggcccgtcgctcctatggtctctgcctgactgggctgccgtctgcctcagttccccagaagcttctcctttggccatgagggctcagtcatccctcaccccagagtccacaggaagagggggtctgctgggaggcctgtctgaaggacggaggatcctgggtcaatttagcagctattttccagggtttggcttgggtttggatgctggcttctgtgtgaaacctgaatacatgcaaattgtacataaaactcccccaaggcagagagggattttccaggccctggtacatctctagagagttaaaaatgggaaatctttcttcttaaagtggcccagactgagacttttccttggggaaaagggttagtagctctttgtaaggctggtgtgtatgtgtgtgtgtatatatatatacatatatgcatgatgctgtgcaaatgcccagggctgtctggcattttccacaaaatgagagcctgagattgcctaagccttctgatgccttctccaggcctggaggcactgcttcattcagaggacacaaaggcctgaccacctggctttagcaagctaggacacccagggtggcttctttacctttctcctcagctctgagaaggctgctagccaagactctggattctctgtggccacagtcatatggtgagggcctcttggagttcattcaaactttaagggagccccacagcaccggcatgatgggtaagtccaggcctaaggttaggaagcaaatcctggagcatgaggaaattgtaggctacagtgagctaccagtggtgtgcaaactggagacccccaagacagtgagagaggccacagcatctgagggaatggagctctttcttggcctgaggttcagaagaacctgcaccaaagaaaggcatccctatcaatgtcactgttcctgaaatgatgggagaaccacatccctgcttcagggaagcagtccctgtcgtctggggcgctgagccctttggcctgagatgaaggatgatggtgtgatgtatcatggcagtgtgactgagactggattgggggatggggacaggggaacataggcaaaaatacacatgtgccactggatcctgagctgccattgtaccttggaggactggcgtttctctgggaagttgggaggtgggaagaggaagggtctcattttcctgccccttgaaaccatgcttaccattcctttagaagattgctcaagctgcctccaattgcctctttccaaaaccaaagcataggaaaacaagtaaaaacagctgaggctgcagcataagcaacttaggatagagtctaggaagcaccgccaacagagaagactgccaagaaacattttgagtttttcttctctggaggtgggtcctggttcctcccatggagaccacgattctgtgtagtcctgcacgctgggcgggggattgcctggaggtttctttagacctgtctagctcacacagtcttgatgcctgggttttaggctgctgtactgttgctggggctcacttcctgtgggtaggctgttattttgcccgcagatcaagtcctcactgtctagatgcctctatcatggggatctcttcttccctctctggatggctctgatccccaagttatttcctgttgcctaggtaacacctctaattggatgccttttaatcgttcccttttttaaagggataaatgtggattttatttccaggtcctgtcagagggccctgccctagagaacacgtgcgcccctgcgtgggcaatcccttcactgtgaccgcaaccatgggttggatggggggcactcactgggctggcctgacagtcacagtgaatcctgaaagcatggttttcacaggaacccaccttcaggatttagcaagactgacgtctctcctggccagcgctgcttcactggcttcaccccagattagggcctgtgtttaaaaaccaatcccaactcaaatcagaaattacccaaaatagctggagagtcactgagatctcaggtaagctttcccttcctgccatgaactagaaggggaaagaagagtttgacattcaagtttgactctaatgctgggtgcgtgagcgcatgcgtgcatgtttgtgtgtgtgtgtgttccacgcacatttgccagggagagagatttcacagcatggctccagctggaggcggtgaggcggtgcttttctaagacttcctatcagaagctgtgcatactggtgggtcacgccgtgcctgtataaactctggcacctgtccttgccctcatcatatatgagaaaaatgggcagagagagtgttcgtttacacccccagaccactatcctttcaatgaagcctgggtatctggccttcctccaggtcagggaccccctatgctgcagaaggcaagtctgggagaatctgtccctcagcccgagagcaaaactgtaatcctaacattacttccatccaccagtttcaccagctacctccctcctgccttcctctgcctccaataggctgtgcatggagaagacaaatcctcttgataaacaatatttagaaagggattctatctttcctgaccccaaacacatcatggcctctggagccaaataccctgacatttgcaagatggcttcttttgggttcctggtgctgcaggccctggttcccaaggacgcagctggcagaggtgcctccttcagaggaggaggaggagaagctggagggctgcgcccggcaaccccatgatctcttaaagggggaaaagttgaactgatcaacagtagttaagaaaaaaaaaatccacaccaacaaataaatatcttgtctgagaagactcagatattcctggttaatattgaaaagcactgctgtggatgagcttgtgaaagaaaggacggttgggggattcaagatctgccgatccgagcctggagatcagccagctaaaagcccagcagggctcctgcagcctcaccgctcccctcctcacaggtgccctggaccgcccaccattagaagtagctgccctgtgctctgtgctaaatggactaactctgagctgagaaaggccagctaagcccctcaccactgcaatttccaaatctgggggaaatgccacagtccgcaagttggtgctatgtttcatctcattgcataatactacaccattctctgtgtgtagtggctgttctatatatatacatcgggaggcaacatatggctgtcccaacccccacctgtcaaaactgtgactatatcacttctgacgaccagaaggaagctgctaggctgggccaggattctaaatgctgaggaggtaattcagagccacgaaaagttgcaccatatgctttggggttgccggctgcttctgtgcatggggacggggtttagtgccagtctgcaaaaccctcctcgctgcggtatgccctgggtgtgggcctggggggccacgttttctctccctgaaggagaatctgctgggggccacggttctccaagaggggactcacaaggaacacaggcgtccccaaaacctgcccttgataacatcaggcctggccaaatagtatttctttaaaaaaattttttttgtttcattttattggataaagattaagaaagcgccagcagtgactgagagaagcaaaccacgcccggcggccccgcggcctggagagggtccccggcgcgggcggacgggcggtctacctggaggcgctggtctcggccagccggttgttcatgatgcccagcgcgcccacgccgcccgagaagccgttctggcgcgtgttgacgcacacgctgcgcgggtagccgttggccgtctccgacagctgcttctgcagcagcgccagcgacaccttgttggaggccgtgaggtcgcgcatggagatgagctcgcccgagaggcggcggccctcggcgtcgctgtcgcgggccgcggggtcggcaccgagcgcggccaggcggcggcgcagccgggagcctggggtgatggcattgcgccgggccaggggcgcgccaggagccgggcagcagcgcgcgcagcagcggcagctcagcttgcgcagcatccagttgagcacctgcttgatgaggatggagatgacgttgaagagcgagtaaatgcagcacacgccgagcaggatgaagaggaagttgcccaggcggtagagcccctggttccggtaggcggcgtgctggctgctcaccaggtccccgaagccgatggtgctgaaggtgacgaagcagaagtagagcgagtccacgtagtcccagccctccacgctggtgtacatggccgaggcgcagcaggacagcagcacggcgaacaggcccaggatgagcagcacgtggtacaccgagggcttccagcccgccaggctgtcggcctccgagagcgcggagccgcggcggaaggtggcgggcagcaggccgctgcggcgcagctggcgctcccggcaggcgcgcatgatgaaggccagcagcgagatgatgcgctccaggaagaggttgaagaacaggatggtcccagcgcagccgaacagcccgtaggcgatgaggaaggccttcccgcccaccgtcgcgggggtggtcatgccgaaacctatggttgacaccacggtgcccacgaagtagaaggcgccggggaagtcccagcgcgggcgcagcgcgtcggcgcggacgccggcggccagcgcggcctcgtagtgccggaggaaggcgcgcagctctggctcggccacgccgtgcgcagcgctgaagttgcgcagcgtggcgccccagcgcgcccgcgcctccgcctcgccggggctctcgagcgccgagaagactgtggcacccgccaccaggtagaggccgatgagcgccgccagcagcacgaagcggccggtgtcctcgttgaggtgcgaacggcggcagcagcagcagcagcaggaggggcgcggcaggcggcggcggctacggcggggcgggggccgggggctgcgggaggacatggtccggagctcagccccggggccggggcggcgctcggggcccgggccacgacatccccccggcgggagcaggagcgtgaggatggtggccaggggtccggggccgccgcggagcccctcgccgccttcgcagagcccctcgtcgccttcccagagcccggacagaggggcgcctccgcctcctccccggcgctcaggccacacgcgagtcccgtggcccagcgggtgcccgggcaggggcgctcctctgcgcgccccgacgcctcgccggctcccgcggctccttacccgccgctctcgggcgcggggctccgcagctaggcccctgccgcccggtggccggcgtccgcggggccccgggcctcatactcctctccagacaggccgcgggctgcgggcggggtgggccgtggatcccgggcgcctaggaccgggacgcggcagcaaggcgtggagagagcccccgggggcgtcccatgaggcgttcgggatcggcgcctcctaggtgcgggctgtgcgggcagtcctgctcccgcccccggggctgagctggcggcgtcggcttcagagcctcggagccgagccgagtccggggaagcgctcctttctcagctccagccgaagagccgcccggcagggagaggcggagtcact

SEQ ID NO: 10456 - RNA, 2964 nt, Homo sapiens
  source 1..2964: mol_type = other RNA
cctcttccccttgtctctccagcctttgaagattgggctcctaagctcctgctctgctggatgctgcctgtgaggctgtacgtgaggggcttagatggccacctgccctcctgtccagctggaggaggcttcaagggttcatgatcattccaagatgggattcctcgcggtgccctctggaactgcttccatgcaggtgaggaggccagaagactctctggcatgtgatcagatgctttggtcagcacctgctttctcagacttgccattggtggctttctaaggaacatgtccacctcaacttctgagccagccccagattcacaggtggctgaggagggaccagcaagctgtgtaagggacaaggatgaaaccttttccagtttaaagcactgaatgggcttgaggaccctgaggggtagaccccacctgtgtttggcccaaaacctcacaatatgggctcccaacccctgctgagtacacggctcgaggaaggaaagcacctgggctgtgttcacacaggctttcccacttttcggggctgctagattgctggttttcacatgggtgttggacacgggaagagcctggttgacagcaagccaggatcgacgcacacacacggggatcaagccctcgttggtctggcccaagttcctgcccatgtgggctttcaggatgttttctatatgagtcctctctgtgcatcttaataaatcacttcccgagtcactcctcaagggcttcctcaagttcctttccaactcctcagaagtcacccccagaaccttccgtgggaagcttttcatatccctggatagattttgtggggtctcacccagaatttgccccagatgtgggcacgggtccctctctagctggaacttcaccttctgtgcctccttgctgccttcacctgtggacatggaggactgccagggactgggtttgcccttggcctgacttgtccctggtgattcatcccgaagctgcatcagatccagagactcttggatccttcccaggttgccccagtgttggatgatccacttttttatgtgttgctccagttgtctccggagttcaggactgactggaaagttctcaggcagaatggatgtcaaactttcctggggaaggttaggagtggagacactaaagacgtcctgagatttttggaccctagagggtaaagccaacctaccttctagttgtctcctcaacaaaggccattcagggtgctgagtttcaggtagggagagagcttgcactttattctgcgatgcagggcaagctactccagtgttctgaatcagggatggaaaagcaggagataggactgggaaagaagattgaagatgggcctgagcctcggcctgagccataggtgtgggccggaattggggtgtggatgaaataaagggttggcactcgggccccagatgggacaggggctgggcctggaaaagcagtggggacattgtagtctccctttgaattgggcagacattggacatttcattgaacaagaaaggaggagactgtaaagtataagacctgtcagttacccaggcgttagccaccagggactcgctgtgcagagaggggaggccccagaaaagctggctataattcttccaaaaactttcctgccagagcctaggatctgagagcttctgaggtccgggcagctgtttcgagttctctcccatgttccagaagggttttgggtttgtggtgtcctgctcagcatccaatgatttagccaaattccgcaaagaatttaagtgcttttctggggtcattcgatttgtaaatgatccaacattttctttttcttcccaaatgttgaccttggctgtttctgtgacttgtatccccacgacattctggccatcagagctgagcaaaaacaggctaccagcttccatctgacaggtctctggtgggtggcgggaaagatgatcttgctggactgatgagttaaaggcgcacgaggttctggcagtctcctgccaccgggaggaggcagaaacatgactgtttgagccaccaaggcctgagatggctgggacagaagccaccaaatcctcatgtggagacaagctttgagggacggtgcccagtggaaatgccactgagtcacagtgagatggagttatcagtgtggagtcccgcaggggaggagcagtgaagccttttggaggaggcagagagcaggccagaggatcaggggtgtgtggtgggtgagggaaaagtgcaggtggctcgggtgaggggtgttctaggggaagggaaggttctggtggctgggaggcacttagggaggagactgaggtggtcattgggcctggtgatggggtggaggccagatcctgaggatgcttggcttgaggatccggggaagctaacggggagagaatgggagcagcatcttccataggctcatgagaggactgggaggctccatcaggtgctctttcgcccacctcacctggggggtctggaccggagagctgaccaaagtcacctttgtcaaggtgtggccccaggaggctctgcagttgtgaaagcaggtccgaagtctcctccaggcctctccggcactctctaccagctctcagactgtggtttttcatcctgcctctgggcctccgcctccgccctactggacactgggagacacgatgacgtacggagacaagatgacgctttctcttcccaggcgatggtgagggtgggtcatcacaacggaagtaagataagtaggggagtaataggaagaagaaccccagggcaaacaccaaagtgaggaagatatccaacacccatggtgtggaactgggggcgtttagcgatgaggcactaagtaattttaaaggaaagggaagattctccatgtgaataggcgcgttgctttcaagcaactgagctctgggcatccccgtggggactagggactgg

SEQ ID NO: 10457 - RNA, 2893 nt, Homo sapiens
  source 1..2893: mol_type = other RNA
cctcttccccttgtctctccagcctttgaagattgggctcctaagctcctgctctgctggatgctgcctgtgaggctgtacgtgaggggcttagatggccacctgccctcctgtccagctggaggaggcttcaagggttcatgatcattccaagatgggattcctcgcggtgccctctggaactgcttccatgcaggtgaggaggccagaagactctctggcatgtgatcagatgctttggtcagcacctgctttctcagacttgccattggtggctttctaaggaacatgtccacctcaacttctgagccagccccagattcacaggtggctgaggagggaccagcaagctgtgtaagggacaaggatgaaaccttttccagtttaaagcactgaatgggcttgaggaccctgaggggtagaccccacctgtgtttggcccaaaacctcacaatatgggctcccaacccctgctgagtacacggctcgaggaaggaaagcacctgggctgtgttcacacaggctttcccacttttcggggctgctagattgctggttttcacatgggtgttggacacgggaagagcctggttgacagcaagccaggatcgacgcacacacacggggatcaagccctcgttggtctggcccaagttcctgcccatgtgggctttcaggatgttttctatatgagtcctctctgtgcatcttaataaatcacttcccgagtcactcctcaagggcttcctcaagttcctttccaactcctcagaagtcacccccagaaccttccgtgggaagcttttcatatccctggatagattttgtggggtctcacccagaatttgccccagatgtgggcacgggtccctctctagctggaacttcaccttctgtgcctccttgctgccttcacctgtggacatggaggactgccagggactgggtttgcccttggcctgacttgtccctggtgattcatcccgaagctgcatcagatccagagactcttggatccttcccaggttgccccagtgttggatgatccacttttttatgtgttgctccagttgtctccggagttcaggactgactggaaagttctcaggcagaatggatgtcaaactttcctggggaaggttaggagtggagacactaaagacgtcctgagatttttggaccctagagggtaaagccaacctaccttctagttgtctcctcaacaaaggccattcagggtgctgagtttcaggtagggagagagcttgcactttattctgcgatgcagggcaagctactccagtgttctgaatcagggatggaaaagcaggagataggactgggaaagaagattgaagatgggcctgagcctcggcctgagccataggtgtgggccggaattggggtgtggatgaaataaagggttggcactcgggccccagatgggacaggggctgggcctggaaaagcagtggggacattgtagtctccctttgaattgggcagacattggacatttcattgaacaagaaaggaggagactgtaaagtataagacctgtcagttacccaggcgttagccaccagggactcgctgtgcagagaggggaggccccagaaaagctggctataattcttccaaaaactttcctgccagagcctaggatctgagagcttctgaggtccgggcagctgtttcgagttctctcccatgttccagaagggttttgggtttgtggtgtcctgctcagcatccaatgatttagccaaattccgcaaagaatttaagtgcttttctggggtcattcgatttgtaaatgatccaacattttctttttcttcccaaatgttgaccttggctgtttctgtgacttgtatccccacgacattctggccatcagagctgagcaaaaacaggctaccagcttccatctgacaggtctctggtgggtggcgggaaagatgatcttgctggactgatgagttaaaggcgcacgaggttctggcagtctcctgccaccgggaggaggcagaaacatgactgtttgagccaccaaggcctgagatggctgggacagaagccaccaaatcctcatgtggagacaagctttgagggacggtgcccagtggaaatgccactgagtcacagtgagatggagttatcagtgtggagtcccgcaggggaggagcagtgaagccttttggaggaggcagagagcaggccagaggatcaggggtgtgtggtgggtgagggaaaagtgcaggtggctcgggtgaggggtgttctaggggaagggaaggttctggtggctgggaggcacttagggaggagactgaggtggtcattgggcctggtgatggggtggaggccagatcctgaggatgcttggcttgaggatccggggaagctaacggggagagaatgggagcagcatcttccataggctcatgagaggactgggaggctccatcaggtgctctttcgcccacctcacctggggggtctggaccggagagctgaccaaagtcacctttgtcaaggtgtggccccaggaggctctgcagttgtgaaagcaggtccgaagtctcctccaggcctctccggcactctctaccagctctcagactgtggtttttcatcctgcctctgggcctccgcctccgccctactggacactttctcttcccaggcgatggtgagggtgggtcatcacaacggaagtaagataagtaggggagtaataggaagaagaaccccagggcaaacaccaaagtgaggaagatatccaacacccatggtgtggaactgggggcgtttagcgatgaggcactaagtaattttaaaggaaagggaagattctccatgtgaataggcgcgttgctttcaagcaact

SEQ ID NO: 10458 - RNA, 2893 nt, Homo sapiens
  source 1..2893: mol_type = other RNA
cctcttccccttgtctctccagcctttgaagattgggctcctaagctcctgctctgctggatgctgcctgtgaggctgtacgtgaggggcttagatggccacctgccctcctgtccagctggaggaggcttcaagggttcatgatcattccaagatgggattcctcgcggtgccctctggaactgcttccatgcaggtgaggaggccagaagactctctggcatgtgatcagatgctttggtcagcacctgctttctcagacttgccattggtggctttctaaggaacatgtccacctcaacttctgagccagccccagattcacaggtggctgaggagggaccagcaagctgtgtaagggacaaggatgaaaccttttccagtttaaagcactgaatgggcttgaggaccctgaggggtagaccccacctgtgtttggcccaaaacctcacaatatgggctcccaacccctgctgagtacacggctcgaggaaggaaagcacctgggctgtgttcacacaggctttcccacttttcggggctgctagattgctggttttcacatgggtgttggacacgggaagagcctggttgacagcaagccaggatcgacgcacacacacggggatcaagccctcgttggtctggcccaagttcctgcccatgtgggctttcaggatgttttctatatgagtcctctctgtgcatcttaataaatcacttcccgagtcactcctcaagggcttcctcaagttcctttccaactcctcagaagtcacccccagaaccttccgtgggaagcttttcatatccctggatagattttgtggggtctcacccagaatttgccccagatgtgggcacgggtccctctctagctggaacttcaccttctgtgcctccttgctgctttcacctgtggacatggaggactgccagggactgggtttgcccttggcctgacttgtccctggtgattcatcccgaagctgcatcagatccagagactcttggatccttcccaggttgccccagtgttggatgatccacttttttatgtgttgctccagttgtctccggagttcaggactgactggaaagttctcaggcagaatggatgtcaaactttcctggggaaggttaggagtggagacactaaagacgtcctgagatttttggaccctagagggtaaagccaacctaccttctagttgtctcctcaacaaaggccattcagggtgctgagtttcaggtagggagagagcttgcactttattctgcgatgcagggcaagctactccagtgttctgaatcagggatggaaaagcaggagataggactgggaaagaagattgaagatgggcctgagcctcggcctgagccataggtgtgggccggaattggggtgtggatgaaataaagggttggcactcgggccccagatgggacaggggctgggcctggaaaagcagtggggacattgtagtctccctttgaattgggcagacattggacatttcattgaacaagaaaggaggagactgtaaagtataagacctgtcagttacccaggcgttagccaccagggactcgctgtgcagagaggggaggccccagaaaagctggctataattcttccaaaaactttcctgccagagcctaggatctgagagcttctgaggtccgggcagctgtttcgagttctctcccatgttccagaagggttttgggtttgtggtgtcctgctcagcatccaatgatttagccaaattccgcaaataatttaagtgcttttctggggtcattcgatttgtaaatgatccaacattttctttttcttcccaaatgttgaccttggctgtttctgtgacttgtatccccacgacattctggccatcagagctgagcaaaaacaggctaccagcttccatctgacaggtctctggtgggtggcgggaaagatgatcttgctggactgatgagttaaaggcgcacgaggttctggcagtctcctgccaccgggaggaggcagaaacatgactgtttgagccaccaaggcctgagatggctgggacagaagccaccaaatcctcatgtggagacaagctttgagggacggtgcccagtggaaatgccactgagtcacagtgagatggagttatcagtgtggagtcccgcaggggaggagcagtgaagccttttggaggaggcagagagcaggccagaggatcaggggtgtgtggtgggtgagggaaaagtgcaggtggctcgggtgaggggtgttctaggggaagggaaggttctggtggctgggaggcacttagggaggagactgaggtggtcattgggcctggtgatggggtggaggccagatcctgaggatgcttggcttgaggatccggggaagctaacggggagagaatgggagcagcatcttccataggctcatgagaggactgggaggctccatcaggtgctctttcacccacctcacctggggggtctggaccggagagctgaccaaagtcacctttgtcaaggtgtggccccaggaggctctgcagttgtgaaagcaggtccgaagtctcctccaggcctctcgggcactctctaccagctctcagactgtggtttttcatcctgcctctgggcctccgcctccgccctactggacactttctcttcccaggcgatggtgagggtgggtcatcacaacggaagtaagataagtaggggagtaataggaagaagaaccccagggcaaacaccaaagtgaggaagatatccaacacccatggtgtggaactgggggcgtttagcgatgaggcactaagtaattttaaaggaaagggaagattctccatgtgaataggcgcgttgctttcaagcaact

SEQ ID NO: 10459 - RNA, 2888 nt, Homo sapiens
  source 1..2888: mol_type = other RNA
cctcttccccttgtctctccagcctttgaagattgggctcctaagctcctgctctgctgggtgctgcctgtgaggctgtacgtgaggggcttagatggccacctgccctcctgtccagctggaggaggcttcaagggcccatgatcattccaagatgggattcctcgcggtgccctctggaactgcttccatgcaggtgaggaggccagaagactctctggcatgtgatcagatgctttggtcagcacctgctttctcagacttgccattggtggctttctaaggaacatgtccacctcaacttctgagccagccccagattcacaggtggctgaggagggaccagcaagctgcgtaagggacaaggatgaaaccttttccagtttaaagcactgaatgggcttgaggaccctgaggggtagaccccacctgtgtttggcccaaaacctcacaatatgggctcccaacccctgctgagtacacggctcgaggaaggaaagcacctgggctgtgttcacacaggctttcccacttttcggggctgctagattgctggttttcacatgggtgttggacacgggaagagcctggttgacagcaagccaggatcgacgcacacgcacggggatcaagccctcgttggtctggcccaagttcctgcccatgtgggctttcaggatgttttctatatgagtcctctctgtgcatcttaataaatcacttcccgagtcactcctcaagggcttcctcaagttcctttccgactcctcagaagtcacccccagaaccttccgtgggaagcttttcatgtccctggatagattttgtggggtctcacccagaatttgccccagatgtgggcacaggtccctctctagctggaacttcaccttctgtgcctccttgctgctttcacctgtggacgtggaggactgccagggactgggtttgcccttggcctgacttgtccctggtgattcgtcccgaagctgcatcagatccagagactcttggatccttcccaggttgccccagtgttggatgatccacttttttatgtgttgctccagttgtctccggagttcaggactgactggaaagttctcaggcagaatggatgtcaaactttcctggggaaggttaggagtggagacactaaagacgtcctgagatttttggaccctagagggtaaagccaacctaccttctagttgtttcctcaacaaaggccattcagggtgctgagtttcaggtagggagagagcttgcactttattctgcgatgcagggcaagctactccagtgttcttaatcagggatggaaaagcaggagataggactgggaaagaagactgaagatgggcctgagcctcggcctgagccataggtgtgggcaggaattggggtgtggatgaaataaagggttggcggtgggacaggggctgggcctggaaaagcagtggggacattgtagtctccctttgaattgggcagacattggacatttcattgaacaagaaaggaggagactgtaaagtataagacctgtcagttacccaggcgttagccaccagggactcgctgtgcagagaggggaggccccagaaaagctggctataattcttccaaaaactttcctgcaagagcctaggatctgagcacttctgaggtccgggcagctgtttcgagttctctcccatgttccagaagggttttgggtttgtggtgtcctgctcagcatccaatgatttagccaaattccccaaagaatttaagtgcttttctggggtcatttgatttgtaaatgatccaacattttctttttcttcccaaatgttgaccttggctgtttctgtgacttgtatccccacgacattctggccatcagagctgagcaaaaacaggctaccagcttccatctgacaggtctctggtgggtggcgggaaagaggatcttgctggactgatgagttaaaggcgcacgaggttctggcagtctcctgccaccgggaggaggcagaaacatgactgtttgagccaccaaggcctgagatggctgggacagaagccaccaaatcctcatgtggagacaagctttgagggacggtgcccagtggaagtgccactgagtcacagtgagatggagttatcagtgtggagtcccgcaggggaggagcagtgaagccttttggaggaggcggagagcaggccagaggatcaggggtgtgtggtgggtgagggaaaagtgcaggtggctcgggtgaggggtgttctaggggaagggaaggttctggtggctgggaggcacttagggaggagactgaggtggtcattgggcctggtgatggggtggaggccagatcctgaggatgcttggcttgaggatccggggaagctaacggggagagaatgggagcagcatcttccataggctcatgagaggactgggaggctccatcaggtgctctttcgcccacctcacctggggggtctggaccggagagctgaccaaagtcacctttgtcaaggtgtggccccaggaggctctgcagttgtgaaagaaggtccgaagtctcctccaggcctctcgggcactctctaccagctctcagactgtggtttttcatcctgcctctgggcctccgcctccgccctactggacactgggagacatgatgacgtacggagacaagatgacgctttctcttcccaggcgatggtgagggtgggtcatcacaatggaagtaagataagtaggggagtaataggaagaagaaccccagggcaaacaccaaggtgaggaagatatccaacacccatggtgtggagctgggggcgtttagcgatgaggcactaagtaattttaaaggaaagggaagattctccat

SEQ ID NO: 10460 - RNA, 2881 nt, Homo sapiens
  source 1..2881: mol_type = other RNA
cctcttccccttgtctctccagcctttgaagattgggctcctaagctcctgctctgctgggtgctgcctgtgaggctgtacgtgaggggcttagatggccacctgccctcctgtccagctggaggaggcttcaagggcccatgatcattccaagatgggattcctcgcggtgccctctggaactgcttccatgcaggtgaggaggccagaagactctctggcatgtgatcagatgctttggtcagcacctgctttctcagacttgccattggtggctttctaaggaacatgtccacctcaacttctgagccagccccagattcacaggtggctgaggagggaccagcaagctgcgtaagggacaaggatgaaaccttttccagtttaaagcactgaatgggcttgaggaccctgaggggtagaccccacctgtgtttggcccaaaacctcacaatatgggctcccaacccctgctgagtacacggctcgaggaaggaaagcacctgggctgtgttcacacaggctttcccacttttcggggctgctagattgctggttttcacatgggtgttggacacgggaagagcctggttgacagcaagccaggatcgacgcacacgcacggggatcaagccctcgttggtctggcccaagttcctgcccatgtgggctttcaggatgttttctatatgagtcctctctgtgcatcttaataaatcacttcccgagtcactcctcaagggcttcctcaagttcctttccgactcctcagaagtcacccccagaaccttccgtgggaagcttttcatgtccctggatagattttgtggggtctcacccagaatttgccccagatgtgggcacaggtccctctctagctggaacttcaccttctgtgcctccttgctgctttcacctgtggacgtggaggactgccagggactgggtttgcccttggcctgacttgtccctggtgattcgtcccgaagctgcatcagatccagagactcttggatccttcccaggttgccccagtgttggatgatccacttttttatgtgttgctccagttgtctccggagttcaggactgactggaaagttctcaggcagaatggatgtcaaactttcctggggaaggttaggagtggagacactaaagacgtcctgagatttttggaccctagagggtaaagccaacctaccttctagttgtttcctcaacaaaggccattcagggtgctgagtttcaggtagggagagagcttgcactttattctgcgatgcagggcaagctactccagtgttcttaatcagggatggaaaagcaggagataggactgggaaagaagactgaagatgggcctgagcctcggcctgagccataggtgtgggcaggaattggggtgtggatgaaataaagggttggcggtgggacaggggctgggcctggaaaagcagtggggacattgtagtctccctttgaattgggcagacattggacatttcattgaacaagaaaggaggagactgtaaagtataagacctgtcagttacccaggcgttagccaccagggactcgctgtgcagagaggggaggccccagaaaagctggctataattcttccaaaaactttcctgcaagagcctaggatctgagcacttctgaggtccgggcagctgtttcgagttctctcccatgttccagaagggttttgggtttgtggtgtcctgctcagcatccaatgatttagccaaattccccaaagaatttaagtgcttttctggggtcatttgatttgtaaatgatccaacattttctttttcttcccaaatgttgaccttggctgtttctgtgacttgtatccccacgacattctggccatcagagctgagcaaaaacaggctaccagcttccatctgacaggtctctggtgggtggcgggaaagaggatcttgctggactgatgagttaaaggcgcacgaggttctggcagtctcctgccaccgggaggaggcagaaacatgactgtttgagccaccaaggcctgagatggctgggacagaagccaccaaatcctcatgtggagacaagctttgagggacggtgcccagtggaagtgccactgagtcacagtgagatggagttatcagtgtggagtcccgcaggggaggagcagtgaagccttttggaggaggcggagagcaggccagaggatcaggggtgtgtggtgggtgagggaaaagtgcaggtggctcgggtgaggggtgttctaggggaagggaaggttctggtggctgggaggcacttagggaggagactgaggtggtcattgggcctggtgatggggtggaggccagatcctgaggatgcttggcttgaggatccggggaagctaacggggagagaatgggagcagcatcttccataggctcatgagaggactgggaggctccatcaggtgctctttcgcccacctcacctggggggtctggaccggagagctgaccaaagtcacctttgtcaaggtgtggccccaggaggctctgcagttgtgaaagaaggtccgaagtctcctccaggcctctcgggcactctctaccagctctcagactgtggtttttcatcctgcctctgggcctccgcctccgccctactggacactttctcttcccaggcgatggtgagggtgggtcatcacaatggaagtaagataagtaggggagtaataggaagaagaaccccagggcaaacaccaaggtgaggaagatatccaacacccatggtgtggagctgggggcgtttagcgatgaggcactaagtaattttaaaggaaagggaagattctccatgtgaataggcacgttgctttcaagcaact

SEQ ID NO: 10461 - RNA, 2964 nt, Homo sapiens
  source 1..2964: mol_type = other RNA
cctcttccccttgtctctccagcctttgaagattgggctcctaagctcctgctctgctgggtgctgcctgtgaggctgtacgtgaggggcttagatggccacctgccctcctgtccagctggaggaggcttcaagggcccatgatcattccaagatgggattcctcgcggtgccctctggaactgcttccatgcaggtgaggaggccagaagactctctggcatgtgatcagatgctttggtcagcacctgctttctcagacttgccattggtggctttctaaggaacatgtccacctcaacttctgagccagccccagattcacaggtggctgaggagggaccagcaagctgtgtaagggacaaggatgaaaccttttccagtttaaagcactgaatgggcttgaggaccctgaggggtagaccccacctgtgtttggcccaaaacctcacaatatgggctcccaacccctgctgagtacacggctcgaggaaggaaagcacctgggctgtgttcacacaggctttcccacttttcggggctgctagattgctggttttcacatgggtgttggacacgggaagagcctggttgacagcaagccaggatcgacgcacacgcacggggatcaagccctcgttggtctggcccaagttcctgcccatgtgggctttcaggatgttttctatatgagtcctctctgtgcatcttaataaatcacttcccgagtcactcctcaagggcttcctcaagttcctttccgactcctcagaagtcacccccagaaccttccgtgggaagcttttcatgtccctggatagattttgtggggtctcacccagaatttgccccagatgtgggcacgggtccctctctagctggaacttcaccttctgtgcctccttgctgctttcacctgtggacatggaggactgccagggactgggtttgcccttggcctgacttgtccctggtgattcgtcccgaagctgcatcagatccagagactcttggatccttcccaggttgccccagtgttggatgatccacttttttatgtgttgctccagttgtctccggagttcaggactgactggaaagttctcaggcagaatggatgtcaaactttcctggggaaggttaggagtggagacactaaagacgtcctgagatttttggaccctagagggtaaagccaacctaccttctagttgtctcctcaacaaaggccattcagggtgctgagtttcaggtagggagagagcttgcactttattctgcgatgcagggcaagctactccagtgttcttaatcagggatggaaaagcaggagataggactgggaaagaagattgaagatgggcctgagcctcggcctgagccataggtgtgggccggaattggggtgtggatgaaataaagggttggcactcgggccccagatgggacgggggctgggcctggaaaagcagtggggacattgtagtctccctttgaattgggcagacattggacatttcattgaacaagaaaggaggagactgtaaagtataagacctgtcagttacccaggcgttagccaccagggactcgctgtgcagagaggggaggccccagaaaagctggctataattcttccaaaaactttcctgccagagcctaggatctgagagcttctgaggtccgggcagctgtttcgagttctctcccatgttccagaagggttttgggtttgtggtgtcctgctcagcatccaatgatttagccaaattccgcaaagaatttaagtgcttttctggggtcattcgatctgtaaatgatccaacattttctttttcttcccaaatgttgaccttggctgtttctgtgacttgtatccccacggcattctggccatcagagctgagcaaaaacaggctaccagcttccatctggtaggtctctggtgggtggcgggaaagatgatcttgctggactgatgagttaaaggcgcacgaggttctggcagtctcctgccaccgggaggaggcagaaacatgactgtttgagccaccaaggcctgagatggctgggacagaagccaccaaatcctcatgtggagacaagctttgagggacggtgcccagtggaagtgccactgagtcacagtgagatggagttatcagtgtggagtcccgcaggggaggagcagtgaagccttttggaggaggcggagagcaggccagaggatcaggggtgtgtggtgggtgagggaaaagtgcaggtggctcgggtgaggggtgttctaggggaagggaaggttctggtggctgggaggcacttagggaggagactgaggtggtcattgggcctggtgatggggtggaggccagatcctgaggatgcttggcttgaggatccggggaagctaacggggagagaatgggagcagcatcttccataggctcatgagaggactgggaggctccatcaggtgctctttcgcccacttcacctggggggtctggaccggagagctgaccaaagtcacctttgtcaaggtgtggccccaggaggctctgcagttgtgaaagcaggtccgaagtctcctgcaggcctctcgggcactctctaccagctctcagactgtggtttttcatcctgcctctgggcctccgcctccgccctactggacactgggagacacgatgacgtacggagacaagatgacgctttctcttcccaggcgatggtgagggtgggtcatcacaacggaagtaagataagtaggggagtaataggaagaagaaccccagggcaaacaccaaagtgaggaagatatccaacacccatggtgtggaactgggggcgtttagcgatgaggcactaagtaattttaaaggaaagggaagattctccatgtgaataggcgcgttgctttcaagcaactgagctctgggcatccccgtggggactagggactgg

SEQ ID NO: 10462 - RNA, 2926 nt, Homo sapiens
  source 1..2926: mol_type = other RNA
cctcttccccttgtctctccagcctttgaagattgggctcctaagctcctgctctgctgggtgctgcctgtgaggctgtacgtgaggggcttagatggccacctgccctcctgtccagctggaggaggcttcaagggcccatgatcattccaagatgggattcctcgcggtgccctctggaactgcttccatgcaggtgaggaggccagaagactctctggcatgtgatcagatgctttggtcagcacctgctttctcagacttgccattggtggctttctaaggaacatgtccacctcaacttctgagccagccccagattcacaggtggctgaggagggaccagcaagctgtgtaagggacaaggatgaaaccttttccagtttaaagcactgaatgggcttgaggaccctgaggggtagaccccacctgtgtttggcccaaaacctcacaatatgggctcccaacccctgctgagtacacggctcgaggaaggaaagcacctgggctgtgttcacacaggctttcccacttttcggggctgctagattgctggttttcacatgggtgttggacacgggaagagcctggttgacagcaagccaggatcgacgcacacgcacggggatcaagccctcgttggtctggcccaagttcctgcccatgtgggctttcaggatgttttctatatgagtcctctctgtgcatcttaataaatcacttcccgagtcactcctcaagggcttcctcaagttcctttccgactcctcagaagtcacccccagaaccttccgtgggaagcttttcatgtccctggatagattttgtggggtctcacccagaatttgccccagatgtgggcacgggtccctctctagctggaacttcaccttctgtgcctccttgctgctttcacctgtggacatggaggactgccagggactgggtttgcccttggcctgacttgtccctggtgattcgtcccgaagctgcatcagatccagagactcttggatccttcccaggttgccccagtgttggatgatccacttttttatgtgttgctccagttgtctccggagttcaggactgactggaaagttctcaggcagaatggatgtcaaactttcctggggaaggttaggagtggagacactaaagacgtcctgagatttttggaccctagagggtaaagccaacctaccttctagttgtctcctcaacaaaggccattcagggtgctgagtttcaggtagggagagagcttgcactttattctgcgatgcagggcaagctactccagtgttcttaatcagggatggaaaagcaggagataggactgggaaagaagattgaagatgggcctgagcctcggcctgagccataggtgtgggccggaattggggtgtggatgaaataaagggttggcactcgggccccagatgggacgggggctgggcctggaaaagcagtggggacattgtagtctccctttgaattgggcagacattggacatttcattgaacaagaaaggaggagactgtaaagtataagacctgtcagttacccaggcgttagccaccagggactcgctgtgcagagaggggaggccccagaaaagctggctataattcttccaaaaactttcctgccagagcctaggatctgagagcttctgaggtccgggcagctgtttcgagttctctcccatgttccagaagggttttgggtttgtggtgtcctgctcagcatccaatgatttagccaaattccgcaaagaatttaagtgcttttctggggtcattcgatctgtaaatgatccaacattttctttttcttcccaaatgttgaccttggctgtttctgtgacttgtatccccacggcattctggccatcagagctgagcaaaaacaggctaccagcttccatctggtaggtctctggtgggtggcgggaaagatgatcttgctggactgatgagttaaaggcgcacgaggttctggcagtctcctgccaccgggaggaggcagaaacatgactgtttgagccaccaaggcctgagatggctgggacagaagccaccaaatcctcatgtggagacaagctttgagggacggtgcccagtggaagtgccactgagtcacagtgagatggagttatcagtgtggagtcccgcaggggaggagcagtgaagccttttggaggaggcggagagcaggccagaggatcaggggtgtgtggtgggtgagggaaaagtgcaggtggctcgggtgaggggtgttctaggggaagggaaggttctggtggctgggaggcacttagggaggagactgaggtggtcattgggcctggtgatggggtggaggccagatcctgaggatgcttggcttgaggatccggggaagctaacggggagagaatgggagcagcatcttccataggctcatgagaggactgggaggctccatcaggtgctctttcgcccacttcacctggggggtctggaccggagagctgaccaaagtcacctttgtcaaggtgtggccccaggaggctctgcagttgtgaaagcaggtccgaagtctcctgcaggcctctcgggcactctctaccagctctcagactgtggtttttcatcctgcctctgggcctccgcctccgccctactggacactttctcttcccaggcgatggtgagggtgggtcatcacaacggaagtaagataagtaggggagtaataggaagaagaaccccagggcaaacaccaaagtgaggaagatatccaacacccatggtgtggaactgggggcgtttagcgatgaggcactaagtaattttaaaggaaagggaagattctccatgtgaataggcgcgttgctttcaagcaactgagctctgggcatccccgtggggactagggact

SEQ ID NO: 10463 - RNA, 2811 nt, Homo sapiens
  source 1..2811: mol_type = other RNA
cctcttccccttgtctctccagcctttgaagattgggctcctaagctcctgctctgctgggtgctgcctgtgaggctgtacgtgaggggcttagatggccacctgccctcctgtccagctggaggaggcttcaagggttcatgatcattccaagatgggattcctcgcggtgccctctggaactgcttccatgcaggtgaggaggccagaagactctctggcatgtgatcagatgctttggtcagcacctgctttctcagacttgccattggtggctttctaaggaacatgtccacctcaacttctgagccagccccagattcacaggtggctgaggagggaccagcaagctgtgtaagggacaaggatgaaaccttttccagtttaaagcactgaatgggcttgaggaccctgaggggtagaccccacctgtgtttggcccaaaacctcacaatatgggctcccaacccctgctgagtacacggctcgaggaaggaaagcacctgggctgtgttcacacaggctttcccacttttcggggctgctagattgctggttttcacatgggtgttggacacgggaagagcctggttgacagcaagccaggatcgacgcacacgcacggggatcaagccctcgttggtctggcccaagttcctgcccatgtgggctttcaggatgttttctatatgagtcctctctgtgcatcttaataaatcacttcccgagtcactcctcaagggcttcctcaagttcctttccaactcctcagaagtcacccccagaaccttccgtgggaagcttttcatatccctggatagattttgtggggtctcacccagaatttgccccagatgtgggcacgggtccctctctagctggaacttcaccttctgtgcctccttgctgctttcacctgtggacatggaggactgccagggactgggtttgcccttggcctgacttgtccctggtgattcgtcctgaagctgcatcagatccagagactcttggatccttcccaggttgccccagtgttggatgatccacttttttatgtgttgctccagttgtctccggagttcaggactgactggaaagttctcaggcagaatggatgtcaaactttcctggggaaggttaggagtggagacactaaagacgtcctgagatttttggaccctagagggtaaagccaacctaccttctagttgtctcctcaacaaaggccattcagggtgctgagtttcaggtagggagagagcttgcactttattctgcgatgcagggcaagctactccagtgttctgaatcagggatggaaaagcaggagataggactgggaaagaagattgaagatgggcctgagcctcggcctgagccataggtgtgggccggaattggggtgtggatgaaataaagggttggcactcgggccccagatgggacaggggctgggcctggaaaagcagtggggacattgtagtctccctttgaattgggcagacattggacatttcattgaacaagaaaggaggagactgtaaagtataagacctgtcagttacccaggcgttagccaccagggactcgctgtgcagagaggggaggccccagaaaagctggctataattcttccaaaaactttcctgccagagcctaggatctgagagcttctgaggtccgggcagctgtttcgagttctctcccatgttccagaagggttttgggtttgtggtgtcctgctcagcatccaatgatttagccaaattccgcaaagaatttaagtgcttttctggggtcattcgatttgtaaatgatccaacattttctttttcttcccaaatgttgaccttggctgtttctgtgacttgtatccccacgacattctggccatcagagctgagcaaaaacaggctaccagcttccatctgacaggtctctggtgggtggcgggaaagatgatcttgctggactgatgagttaaaggcgcacgaggttctggcagtctcctgccaccgggaggaggcagaaacatgactgtttgagccaccaaggcctgagatggctgggacagaagccaccaaatcctcatgtggagacaagctttgagggacggtgcccagtggaagtgccactgagtcacagtgagatggagttatcagtgtggagtcccgcaggggaggagcagtgaagccttttggaggaggcagagagcaggccagaggatcaggggtgtgtggtgggtgagggaaaagtgcaggtggctcgggtgaggggtgttctaggggaagggaaggttctggtggctgggaggcacttagggaggagactgaggtggtcattgggcctggtgatggggtggaggccagatcctgaggatgcttggcttgaggatccggggaagctaacagggagagaatgggagcagcatcttccataggctcatgagaggactgggaggctccatcaggtgctctttcgcccacctcacctggggggtctggaccggagagctgaccaaagtcacctttgtcaaggtgtggccccaggaggctctgcagttgtgaaagcaggtccgaagtctcctccaggcctctccggcactctctaccagccccctccgcatccaggcaggcattggtctccccaggacacacacactgccccctgctgggtaacgcccagtccctggcccaccatggcttcattcccgcatggaatctgagaaggacccggggttctgatttccttcctaggagcccccacctcaggcttcttcaactgacttcttcagagtcagttcccttc

SEQ ID NO: 10464 - RNA, 2893 nt, Homo sapiens
  source 1..2893: mol_type = other RNA
cctcttccccttgtctctccagcctttgaagattgggctcctaagctcctgctctgctgggtgctgcctgtgaggctgtacgtgaggggcttagatggccacctgccctcctgtccagctggaggaggcttcaagggttcatgatcattccaagatgggattcctcgcggtgccctctggaactgcttccatgcaggtgaggaggccagaagactctctggcatgtgatcagatgctttggtcagcacctgctttctcagacttgccattggtggctttctaaggaacatgtccacctcaacttctgagccagccccagattcacaggtggctgaggagggaccagcaagctgtgtaagggacaaggatgaaaccttttccagtttaaagcactgaatgggcttgaggaccctgaggggtagaccccacctgtgtttggcccaaaacctcacaatatgggctcccaacccctgctgagtacacggctcgaggaaggaaagcacctgggctgtgttcacacaggctttcccacttttcggggctgctagattgctggttttcacatgggtgttggacacgggaagagcctggttgacagcaagccaggatcgacgcacacgcacggggatcaagccctcgttggtctggcccaagttcctgcccatgtgggctttcaggatgttttctatatgagtcctctctgtgcatcttaataaatcacttcccgagtcactcctcaagggcttcctcaagttcctttccaactcctcagaagtcacccccagaaccttccgtgggaagcttttcatatccctggatagattttgtggggtctcacccagaatttgccccagatgtgggcacgggtccctctctagctggaacttcaccttctgtgcctccttgctgctttcacctgtggacatggaggactgccagggactgggtttgcccttggcctgacttgtccctggtgattcgtcctgaagctgcatcagatccagagactcttggatccttcccaggttgccccagtgttggatgatccacttttttatgtgttgctccagttgtctccggagttcaggactgactggaaagttctcaggcagaatggatgtcaaactttcctggggaaggttaggagtggagacactaaagacgtcctgagatttttggaccctagagggtaaagccaacctaccttctagttgtctcctcaacaaaggccattcagggtgctgagtttcaggtagggagagagcttgcactttattctgcgatgcagggcaagctactccagtgttctgaatcagggatggaaaagcaggagataggactgggaaagaagattgaagatgggcctgagcctcggcctgagccataggtgtgggccggaattggggtgtggatgaaataaagggttggcactcgggccccagatgggacaggggctgggcctggaaaagcagtggggacattgtagtctccctttgaattgggcagacattggacatttcattgaacaagaaaggaggagactgtaaagtataagacctgtcagttacccaggcgttagccaccagggactcgctgtgcagagaggggaggccccagaaaagctggctataattcttccaaaaactttcctgccagagcctaggatctgagagcttctgaggtccgggcagctgtttcgagttctctcccatgttccagaagggttttgggtttgtggtgtcctgctcagcatccaatgatttagccaaattccgcaaagaatttaagtgcttttctggggtcattcgatttgtaaatgatccaacattttctttttcttcccaaatgttgaccttggctgtttctgtgacttgtatccccacgacattctggccatcagagctgagcaaaaacaggctaccagcttccatctgacaggtctctggtgggtggcgggaaagatgatcttgctggactgatgagttaaaggcgcacgaggttctggcagtctcctgccaccgggaggaggcagaaacatgactgtttgagccaccaaggcctgagatggctgggacagaagccaccaaatcctcatgtggagacaagctttgagggacggtgcccagtggaagtgccactgagtcacagtgagatggagttatcagtgtggagtcccgcaggggaggagcagtgaagccttttggaggaggcagagagcaggccagaggatcaggggtgtgtggtgggtgagggaaaagtgcaggtggctcgggtgaggggtgttctaggggaagggaaggttctggtggctgggaggcacttagggaggagactgaggtggtcattgggcctggtgatggggtggaggccagatcctgaggatgcttggcttgaggatccggggaagctaacagggagagaatgggagcagcatcttccataggctcatgagaggactgggaggctccatcaggtgctctttcgcccacctcacctggggggtctggaccggagagctgaccaaagtcacctttgtcaaggtgtggccccaggaggctctgcagttgtgaaagcaggtccgaagtctcctccaggcctctccggcactctctaccagctctcagactgtggtttttcatcctgcctctgggcctccgcctccgccctactggacactttctcttcccaggcgatggtgagggtgggtcatcacaacggaagtaagataagtaggggagtaataggaagaagaaccccagggcaaacaccaaagtgaggaagatatccaacacccatggtgtggaactgggggcgtttagcgatgaggcactaagtaattttaaaggaaagggaagattctccatgtgaataggcgcgttgctttcaagcaact

SEQ ID NO: 10465 - RNA, 910 nt, Homo sapiens
  source 1..910: mol_type = other RNA
cctgagaaaagggccaactatgatttttttttaattagcaagttttaaagagtcatagtgtagaggattataaactctgcttgaattactttcagaattaaccaatgattcaatttaaaacatctcttaaaggtaaaataaactatttgtggtatttggaaagcagccacatttgaagaaacatgtaatactgaacaaagttacaattattagcagtttcataaaagccctttttgtttaaaaaagaataagttgctgcaaatataaaattcatggaagcagagtgatcttcactttagaatttcctgatttgttttaaattgataaaaataatttttcttccaaggaaatgaaaaaagaagtaaattgttttaatcgaatataatcaaacacaattactatgtaaaaaagtggaagaatcaaggcaagattaaattatcctagttaagtaaaaaaataaacaccagcaaaattgaatatgtgtctatttgcatttccataaaagttctataacgtaaaaggggtctagctttatcaaggatatgcaatccagttaggatctatgattctaaaagaaaagaaaaattcactctttaaggacagcaagtcaatataggcatcttacagtcacctttcttaaatcactaagacttaatgaagagcaaaagtaactattcaatgagattcttatctgttcctgataccatgcagtcaccaaagccaaagttccaaggaaaaagaatgaacaaaaaaggccaggcgcagtggctcacgcctgtaattccaacactttgggaggccgaggtgggcggatcacttgaggtcaggagttccagaccagcctgaccaacatgctgaaactctgtctctattaaaaatacaaaaattagctgggtgtggtagtgcgcac

SEQ ID NO: 10466 - RNA, 69 nt, Homo sapiens
  source 1..69: mol_type = other RNA
cctgcagagaggaagcccttccaatacctgtaagcagaagggcttcctctctgcaggaccggcctgaat

SEQ ID NO: 10467 - RNA, 69 nt, Homo sapiens
  source 1..69: mol_type = other RNA
cctgcagagaggaagcccttctgcttacaggtattggaagggcttcctctctgcaggaccggcctgaat

SEQ ID NO: 10468 - RNA, 1044 nt, Homo sapiens
  source 1..1044: mol_type = other RNA
cctgcagcgacttgatggcttccgtgtccttttcgtgggtagccatgaccaaagactggagcagcagaaagagctcctcgggaagctggccgctgctctcctgcccgtggctgtcaaaagcctcccaggagtacttctccagggtctgggcgtgctccggcagcagcttggcgggcggtggttgcaggaggagcagcagcagcacgcgggacacctcgcagcggaccagcacgtccgagaaggcgcccagggcggcgggagagggcgccgccgagccggagttcggaggaagcagcgcggccggtagggcgggcgtcgccccgggcccgggctggggtgccggcggcgggggcggcggcagtgactgcaccgggtggctgccgtgctcccgcgccaggcgctgcatgcgcgtgaagaccgccagggcgccggtgtagtcgcgcgccagcagctggcaggaggcggcctcgccaagcgcctgcagcgcggccaggggcagctggggcagctggagctgggcggcgcgctggaagtgaccggcggcggcggccggctggcccaggtcgcgcagggcggcggccagctcgaggcagagggcggcggcggcggccggctggcccagctcgaggtgcagacgcaccgcggcgcccagggcgctggcggcggcctgcagcggctccccgtaggcggcggggcagaccaggcgctggcgcgcgtcgcgctcctgccgcaggaagaggcgggcggcctcggtgagggccagcgcctccccgggcccgtggaagagcgcctgctggcagcgcgccaccgccagctggcaccaggccgcgtagggcagacactcctgggcgcgcagctcccggcccagctgtccgaactgctcgccggcctccgccacgttcggcttccgcaggaaccgcttcttcagcttgttcgataccagccggtagcgggccaggaagtccccggcctcgggtcccgggccggcgccgccgccgcccaggcctgcagccgctgccgccatgctcgccgccccaagcactt

SEQ ID NO: 10469 - RNA, 53 nt, Homo sapiens
  source 1..53: mol_type = other RNA
cctgcgtgttttctgtccaaatcagaaaaggatttggacagaaaacacgcagg

SEQ ID NO: 10470 - RNA, 61 nt, Homo sapiens
  source 1..61: mol_type = other RNA
cctgcgtgttttctgtccaaatccttttctgatttggacagaaaacacgcaggtggcacac

SEQ ID NO: 10471 - RNA, 1421 nt, Homo sapiens
  source 1..1421: mol_type = other RNA
cctggcatatttggtataacttcacatttttggtatatagaaattttattttcttaatgcagcacagtagacatacaatcaatattattccctagaatgtgcaatatataaattattcacattaaaaaattaacagaaagcctcatatgcagtaaatatttaaaaatgtatatctaactttgattctgtttctgactatacactactagctttataaatctgaatgaatatgacatttacacatttgaatgaagtacacggatgggtccattccagatgcttattacaccgtatgaataatctgctcttcactttggtcattaaggttccatgtgctgaggcatatagtggatccgaaagacacttccaggaagtacatttattacattggcatcttaagaatttctgttccttttattctcctttatagcgagggggccttttctctttaaaagcaagaagaccttcaagtctgtcttttgttggaatggtctccatcccttgattaattgctaattttgccactctcattgcaacaggtccctgaggtaaaaactctctcgccaggtccaaggccttcctgtaggccgcgtctccctcctggttctgttccagaacgtggctgattaagcccactgctttggcttctttgccatcgaggactcgcgcagagaatatgagctccttggccagggacattccaatggcgcgtggcaatcgctgtgtcccccctccaccaggaataatcgccaattttgtttcaaccaggcccatttttgcagaggaagctgctactcgtatatcacaggctaaagccagttcaagaccaccacctaaagcgagtccatctattgctgcaattgttggtactggaagattagcaatatcgttaatcactgctcttattttggagacaaaaggaccaacttcactggaactcattttggctctttccttaaggtcagcaccagcacagaatatccctgggacttcactcctgattattatggtccgtactttcttatcagatttcaaagcatccacagcttttgatagcatttttataagatttttactgagtgaatttttgccataagctctgtttattccaagcaccacaattcctcggttctcctcctccaggtgccgcacccgcagctcgtcctccgtcttcatctcagagctgtagccccttttcggggcgggacccccggccgcaggtacccagccctgggcccagatcgccgggcccgctcgccggcctgccaacgagccgggcagcctcaaccccgggcagagccacgcactgcaagcggccaccaggcgggcgccgccagcatgcagggatcccaaggccccaggtgccgccgccaccgcggccgccatgttgtctgtttacggcgtggacctgcgacggccgc

SEQ ID NO: 10472 - RNA, 1485 nt, Homo sapiens
  source 1..1485: mol_type = other RNA
cctggcatatttggtataacttcacatttttggtatatagaaattttattttcttaatgcagcacagtagacatacaatcaatattattccctagaatgtgcaatatataaattattcacattaaaaaattaacagaaagcctcatatgcagtaaatatttaaaaatgtatatctaactttgattctgtttctgactatacactactagctttataaatctgaatgaatatgacatttacacatttgaatgaagtacacggatgggtccattccagatgcttattacaccgtatgaataatctgctcttcactttggtcattaaggttccatgtgctgaggcatatagtggatccgaaagacacttccaggaagtacatttattacattggcatcttaagaatttctgttccttttattctcctttatagcgagggggccttttctctttaaaagcaagaagaccttcaagtctgtcttttgttggaatggtctccatcccttgattaattgctaattttgccactctcattgcaacaggtccctgaggtaaaaactctctcgccaggtccaaggccttcctgtaggccgcgtctccctcctggttctgttccagaacgtggctgattaagcccactgctttggcttctttgccatcgaggactcgcgcagagaatatgagctccttggccagggacattccaatggcgcgtggcaatcgctgtgtcccccctccaccaggaataatcgccaattttgtttcaaccaggcccatttttgcagaggaagctgctactcgtatatcacaggctaaagccagttcaagaccaccacctaaagcgagtccatctattgctgcaattgttggtactggaagattagcaatatcgttaatcactgctcttattttggagacaaaaggaccaacttcactggaactcattttggctctttccttaaggtcagcaccagcacagaatatccctgggacttcactcctgattattatggtccgtactttcttatcagatttcaaagcatccacagcttttgatagcatttttataagatttttactgagtgaatttttgccataagctctgtttattccaagcaccacaattccttatgttacgtcccaaatacaccacacatgttcacatctccatgcctttgaccatgttcttgtctctgtctcggttctcctcctccaggtgccgcacccgcagctcgtcctccgtcttcatctcagagctgtagccccttttcggggcgggacccccggccgcaggtacccagccctgggcccagatcgccgggcccgctcgccggcctgccaacgagccgggcagcctcaaccccgggcagagccacgcactgcaagcggccaccaggcgggcgccgccagcatgcagggatcccaaggccccaggtgccgccgccaccgcggccgccatgttgtctgtttacggcgtggacctgcgac

SEQ ID NO: 10473 - RNA, 1466 nt, Homo sapiens
  source 1..1466: mol_type = other RNA
cctggcatatttggtataacttcacatttttggtatatagaaattttattttcttaatgcagcacagtagacatacaatcaatattattccctagaatgtgcaatatataaattattcacattaaaaaattaacagaaagcctcatatgcagtaaatatttaaaaatgtatatctaactttgattctgtttctgactatacactactagctttataaatctgaatgaatatgacatttacacatttgaatgaagtacacggatgggtccattccagatgcttattacaccgtatgaataatctgctcttcactttggtcattaaggttccatgtgctgaggcatatagtggatccgaaagacacttccaggaagtacatttattacattggcatcttaagaatttctgttccttttattctcctttatagcgagggggccttttctctttaaaagcaagaagaccttcaagtctgtcttttgttggaatggtctccatcccttgattaattgctaattttgccactctcattgcaacaggtccctgaggtaaaaactctctcgccaggtccaaggccttcctgtaggccgcgtctccctcctggttctgttccagaacgtggctgattaagcccactgctttggcttctttgccatcgaggactcgcgcagagaatatgagctccttggccagggacattccaatggcgcgtggcaatcgctgtgtcccccctccaccaggaataatcgccaattttgtttcaaccaggcccatttttgcagaggaagctgctactcgtatatcacaggctaaagccagttcaagaccaccacctaaagcgagtccatctattgctgcaattgttggtactggaagattagcaatatcgttaatcactgctcttattttggagacaaaaggaccaacttcactggaactcattttggctctttccttaaggtcagcaccagcacagaatatccctgggacttcactcctgattattatggtccgtactttcttatcagatttcaaagcatccacagcttttgatagcatttttataagatttttactgagtgaatttttgccataagctctgtttattccaagcaccacaattctatagtgatcagcagccatggaactagagtctcggttctcctcctccaggtgccgcacccgcagctcgtcctccgtcttcatctcagagctgtagccccttttcggggcgggacccccggccgcaggtacccagccctgggcccagatcgccgggcccgctcgccggcctgccaacgagccgggcagcctcaaccccgggcagagccacgcactgcaagcggccaccaggcgggcgccgccagcatgcagggatcccaaggccccaggtgccgccgccaccgcggccgccatgttgtctgtttacggcgtggacctgcgacggccgctccgcccccgcccgg

SEQ ID NO: 10474 - RNA, 1625 nt, Homo sapiens
  source 1..1625: mol_type = other RNA
cctggcatatttggtataacttcacatttttggtatatagaaattttattttcttaatgcagcacagtagacatacaatcaatattattccctagaatgtgcaatatataaattattcacattaaaaaattaacagaaagcctcatatgcagtaaatatttaaaaatgtatatctaactttgattctgtttctgactatacactactagctttataaatctgaatgaatatgacatttacacatttgaatgaagtacacggatgggtccattccagatgcttattacaccgtatgaataatctgctcttcactttggtcattaaggttccatgtgctgaggcatatagtggatccgaaagacacttccaggaagtacatttattacattggcatcttaagaatttctgttccttttattctcctttatagcgagggggccttttctctttaaaagcaagaagaccttcaagtctgtcttttgttggaatggtctgagcataacaagcttcttctatggctaaccctgttactaaatcgacctccatcccttgattaattgctaattttgccactctcattgcaacaggtccctgaggtaaaaactctctcgccaggtccaaggccttcctgtaggccgcgtctccctcctggttctgttccagaacgtggctgattaagcccactgctttggcttctttgccatcgaggactcgcgcagagaatatgagctccttggccagggacattccaatggcgcgtggcaatcgctgtgtcccccctccaccaggaataatcgccaattttgtttcaaccaggcccatttttgcagaggaagctgctactcgtatatcacaggctaaagccagttcaagaccaccacctaaagcgagtccatctattgctgcaattgttggtactggaagattagcaatatcgttaatcactgctcttattttggagacaaaaggaccaacttcactggaactcattttggctctttccttaaggtcagcaccagcacagaatatccctgggacttcactcctgattattatggtccgtactttcttatcagatttcaaagcatccacagcttttgatagcatttttataagatttttactgagtgaatttttgccataagctctgtttattccaagcaccacaattcccaaaagatgatggcattcaggctctaatcactccagtgctagtctatgcttccagctgaatttcttactattctgcttatgccacacttgccttatgttacgtcccaaatacaccacacatgttcacatctccatgcctttgaccatgttcttgtctctgtctcggttctcctcctccaggtgccgcacccgcagctcgtcctccgtcttcatctcagagctgtagccccttttcggggcgggacccccggccgcaggtacccagccctgggcccagatcgccgggcccgctcgccggcctgccaacgagccgggcagcctcaaccccgggcagagccacgcactgcaagcggccaccaggcgggcgccgccagcatgcagggatcccaaggccccaggtgccgccgccaccgcggccgccatgttgtctgtttacggcgtggacctgcgac

SEQ ID NO: 10475 - RNA, 1463 nt, Homo sapiens
  source 1..1463: mol_type = other RNA
cctggcatatttggtataacttcacatttttggtatatagaaattttattttcttaatgcagcacagtagacatacaatcaatattattccctagaatgtgcaatatataaattattcacattaaaaaattaacagaaagcctcatatgcagtaaatatttaaaaatgtatatctaactttgattctgtttctgactatacactactagctttataaatctgaatgaatatgacatttacacatttgaatgaagtacacggatgggtccattccagatgcttattacaccgtatgaataatctgctcttcactttggtcattaaggttccatgtgctgaggcatatagtggatccgaaagacacttccaggaagtacatttattacattggcatcttaagaatttctgttccttttattctcctttatagcgagggggccttttctctttaaaagcaagaagaccttcaagtctgtcttttgttggaatggtctgagcataacaagcttcttctatggctaaccctgttactaaatcgacctccatcccttgattaattgctaattttgccactctcattgcaacaggtccctgaggtaaaaactctctcgccaggtccaaggccttcctgtaggccgcgtctccctcctggttctgttccagaacgtggctgattaagcccactgctttggcttctttgccatcgaggactcgcgcagagaatatgagctccttggccagggacattccaatggcgcgtggcaatcgctgtgtcccccctccaccaggaataatcgccaattttgtttcaaccaggcccatttttgcagaggaagctgctactcgtatatcacaggctaaagccagttcaagaccaccacctaaagcgagtccatctattgctgcaattgttggtactggaagattagcaatatcgttaatcactgctcttattttggagacaaaaggaccaacttcactggaactcattttggctctttccttaaggtcagcaccagcacagaatatccctgggacttcactcctgattattatggtccgtactttcttatcagatttcaaagcatccacagcttttgatagcatttttataagatttttactgagtgaatttttgccataagctctgtttattccaagcaccacaattcctcggttctcctcctccaggtgccgcacccgcagctcgtcctccgtcttcatctcagagctgtagccccttttcggggcgggacccccggccgcaggtacccagccctgggcccagatcgccgggcccgctcgccggcctgccaacgagccgggcagcctcaaccccgggcagagccacgcactgcaagcggccaccaggcgggcgccgccagcatgcagggatcccaaggccccaggtgccgccgccaccgcggccgccatgttgtctgtttacggcgtggacctgcgac

SEQ ID NO: 10476 - RNA, 1533 nt, Homo sapiens
  source 1..1533: mol_type = other RNA
cctggcatatttggtataacttcacatttttggtatatagaaattttattttcttaatgcagcacagtagacatacaatcaatattattccctagaatgtgcaatatataaattattcacattaaaaaattaacagaaagcctcatatgcagtaaatatttaaaaatgtatatctaactttgattctgtttctgactatacactactagctttataaatctgaatgaatatgacatttacacatttgaatgaagtacacggatgggtccattccagatgcttattacaccgtatgaataatctgctcttcactttggtcattaaggttccatgtgctgaggcatatagtggatccgaaagacacttccaggaagtacatttattacattggcatcttaagaatttctgttccttttattctcctttatagcgagggggccttttctctttaaaagcaagaagaccttcaagtctgtcttttgttggaatggtctgagcataacaagcttcttctatggctaaccctgttactaaatcgacctccatcccttgattaattgctaattttgccactctcattgcaacaggtccctgaggtaaaaactctctcgccaggtccaaggccttcctgtaggccgcgtctccctcctggttctgttccagaacgtggctgattaagcccactgctttggcttctttgccatcgaggactcgcgcagagaatatgagctccttggccagggacattccaatggcgcgtggcaatcgctgtgtcccccctccaccaggaataatcgccaattttgtttcaaccaggcccatttttgcagaggaagctgctactcgtatatcacaggctaaagccagttcaagaccaccacctaaagcgagtccatctattgctgcaattgttggtactggaagattagcaatatcgttaatcactgctcttattttggagacaaaaggaccaacttcactggaactcattttggctctttccttaaggtcagcaccagcacagaatatccctgggacttcactcctgattattatggtccgtactttcttatcagatttcaaagcatccacagcttttgatagcatttttataagatttttactgagtgaatttttgccataagctctgtttattccaagcaccacaattccttatgttacgtcccaaatacaccacacatgttcacatctccatgcctttgaccatgttcttgtctctgtctcggttctcctcctccaggtgccgcacccgcagctcgtcctccgtcttcatctcagagctgtagccccttttcggggcgggacccccggccgcaggtacccagccctgggcccagatcgccgggcccgctcgccggcctgccaacgagccgggcagcctcaaccccgggcagagccacgcactgcaagcggccaccaggcgggcgccgccagcatgcagggatcccaaggccccaggtgccgccgccaccgcggccgccatgttgtctgtttacggcgtggacctgcgac

SEQ ID NO: 10477 - RNA, 1512 nt, Homo sapiens
  source 1..1512: mol_type = other RNA
cctggcatatttggtataacttcacatttttggtatatagaaattttattttcttaatgcagcacagtagacatacaatcaatattattccctagaatgtgcaatatataaattattcacattaaaaaattaacagaaagcctcatatgcagtaaatatttaaaaatgtatatctaactttgattctgtttctgactatacactactagctttataaatctgaatgaatatgacatttacacatttgaatgaagtacacggatgggtccattccagatgcttattacaccgtatgaataatctgctcttcactttggtcattaaggttccatgtgctgaggcatatagtggatccgaaagacacttccaggaagtacatttattacattggcatcttaagaatttctgttccttttattctcctttatagcgagggggccttttctctttaaaagcaagaagaccttcaagtctgtcttttgttggaatggtctgagcataacaagcttcttctatggctaaccctgttactaaatcgacctccatcccttgattaattgctaattttgccactctcattgcaacaggtccctgaggtaaaaactctctcgccaggtccaaggccttcctgtaggccgcgtctccctcctggttctgttccagaacgtggctgattaagcccactgctttggcttctttgccatcgaggactcgcgcagagaatatgagctccttggccagggacattccaatggcgcgtggcaatcgctgtgtcccccctccaccaggaataatcgccaattttgtttcaaccaggcccatttttgcagaggaagctgctactcgtatatcacaggctaaagccagttcaagaccaccacctaaagcgagtccatctattgctgcaattgttggtactggaagattagcaatatcgttaatcactgctcttattttggagacaaaaggaccaacttcactggaactcattttggctctttccttaaggtcagcaccagcacagaatatccctgggacttcactcctgattattatggtccgtactttcttatcagatttcaaagcatccacagcttttgatagcatttttataagatttttactgagtgaatttttgccataagctctgtttattccaagcaccacaattctatagtgatcagcagccatggaactagagtctcggttctcctcctccaggtgccgcacccgcagctcgtcctccgtcttcatctcagagctgtagccccttttcggggcgggacccccggccgcaggtacccagccctgggcccagatcgccgggcccgctcgccggcctgccaacgagccgggcagcctcaaccccgggcagagccacgcactgcaagcggccaccaggcgggcgccgccagcatgcagggatcccaaggccccaggtgccgccgccaccgcggccgccatgttgtctgtttacggcgtggacctgcgacggccgctccgcccccgccc

SEQ ID NO: 10478 - RNA, 1376 nt, Homo sapiens
  source 1..1376: mol_type = other RNA
cctggcatatttggtataacttcacatttttggtatatagaaattttattttcttaatgcagcacagtagacatacaatcaatattattccctagaatgtgcaatatataaattattcacattaaaaaattaacagaaagcctcatatgcagtaaatatttaaaaatgtatatctaactttgattctgtttctgactatacactactagctttataaatctgaatgaatatgacatttacacatttgaatgaagtacacggatgggtccattccagatgcttattacaccgtatgaataatctgctcttcactttggtcattaaggttccatgtgctgaggcatatagtggatccgaaagacacttccaggaagtacatttattacattggcatcttaagaatttctgttccttttattctcctttatagcgagggggccttttctctttaaaagcaagaagaccttcaagtctgtcttttgttggaatggtctgagcataacaagcttcttctatggctaaccctgttactaaatcgacctccatcccttgattaattgctaattttgccactctcattgcaacaggtccctgaggtaaaaactctctcgccaggtccaaggccttcctgtaggccgcgtctccctcctggttctgttccagaacgtggctgattaagcccactgctttggcttctttgccatcgaggactcgcgcagagaatatgagctccttggccagggacattccaatggcgcgtggcaatcgctgtgtcccccctccaccaggaataatcgccaattttgtttcaaccaggcccatttttgcagaggaagctgctactcgtatatcacaggctaaagccagttcaagaccaccacctaaagcgagtccatctattgctgcaattgttggtactggaagattagcagcacagaatatccctgggacttcactcctgattattatggtccgtactttcttatcagatttcaaagcatccacagcttttgatagcatttttataagatttttactgagtgaatttttgccataagctctgtttattccaagcaccacaattcctcggttctcctcctccaggtgccgcacccgcagctcgtcctccgtcttcatctcagagctgtagccccttttcggggcgggacccccggccgcaggtacccagccctgggcccagatcgccgggcccgctcgccggcctgccaacgagccgggcagcctcaaccccgggcagagccacgcactgcaagcggccaccaggcgggcgccgccagcatgcagggatcccaaggccccaggtgccgccgccaccgcggccgccatgttgtctgtttacggcgtggacctgcgac

SEQ ID NO: 10479 - RNA, 1428 nt, Homo sapiens
  source 1..1428: mol_type = other RNA
cctggcatatttggtataacttcacatttttggtatatagaaattttattttcttaatgcagcacagtagacatacaatcaatattattccctagaatgtgcaatatataaattattcacattaaaaaattaacagaaagcctcatatgcagtaaatatttaaaaatgtatatctaactttgattctgtttctgactatacactactagctttataaatctgaatgaatatgacatttacacatttgaatgaagtacacggatgggtccattccagatgcttattacaccgtatgaataatctgctcttcactttggtcattaaggttccatgtgctgaggcatatagtggatccgaaagacacttccaggaagtacatttattacattggcatcttaagaatttctgttccttttattctcctttatagcgagggggccttttctctttaaaagcaagaagaccttcaagtctgtcttttgttggaatggtctgagcataacaagcttcttctatggctaaccctgttactaaatcgacctccatcccttgattaattgctaattttgccactctcattgcaacaggtccctgaggtaaaaactctctcgccaggtccaaggccttcctgtaggccgcgtctccctcctggttctgttccagaacgtggctgattaagcccactgctttggcttctttgccatcgaggactcgcgcagagaatatgagctccttggccagggacattccaatggcgcgtggcaatcgctgtgtcccccctccaccaggaataatcgccaattttgtttcaaccaggcccatttttgcagaggaagctgctactcgtatatcacaggctaaagccagttcaagaccaccacctaaagcgagtccatctattgctgcaattgttggtactggaagattagcagcacagaatatccctgggacttcactcctgattattatggtccgtactttcttatcagatttcaaagcatccacagcttttgatagcatttttataagatttttactgagtgaatttttgccataagctctgtttattccaagcaccacaattctatagtgatcagcagccatggaactagagtctcggttctcctcctccaggtgccgcacccgcagctcgtcctccgtcttcatctcagagctgtagccccttttcggggcgggacccccggccgcaggtacccagccctgggcccagatcgccgggcccgctcgccggcctgccaacgagccgggcagcctcaaccccgggcagagccacgcactgcaagcggccaccaggcgggcgccgccagcatgcagggatcccaaggccccaggtgccgccgccaccgcggccgccatgttgtctgtttacggcgtggacctgcgacggccgctccgcccccgcccggc

SEQ ID NO: 10480 - RNA, 1611 nt, Homo sapiens
  source 1..1611: mol_type = other RNA
cctggcatatttggtataacttcacatttttggtatatagaaattttattttcttaatgcagcacagtagacatacaatcaatattattccctagaatgtgcaatatataaattattcacattaaaaaattaacagaaagcctcatatgcagtaaatatttaaaaatgtatatctaactttgattctgtttctgactatacactactagctttataaatctgaatgaatatgacatttacacatttgaatgaagtacacggatgggtccattccagatgcttattacaccgtatgaataatctgctcttcactttggtcattaaggttccatgtgctgaggcatatagtggatccgaaagacacttccaggaagtacatttattacattggcatcttaagaatttctgttccttttattctcctttatagcgagggggccttttctctttaaaagcaagaagaccttcaagtctgtcttttgttggaatggtctgagcataacaagcttcttctatggctaaccctgttactaaatcgacctccatcccttgattaattgctaattttgccactctcattgcaacaggtccctgaggtaaaaactctctcgccaggtccaaggccttcctgtaggccgcgtctccctcctggttctgttccagaacgtggctgattaagcccactgctttggcttctttgccatcgaggactcgcgcagagaatatgagctccttggccagggacattccaatggcgcgtggcaatcgctgtgtcccccctttgggttttgtaggcaatgcttatagcatccatgttgctgatgaaacaactgatgccagcttaatacttcttcacacacaggcaacttgtttttcttcctctctgaaatcttttatgatcttctcttaatcctccgagcactccaccaggaataatcgccaattttgtttcaaccaggcccatttttgcagaggaagctgctactcgtatatcacaggctaaagccagttcaagaccaccacctaaagcgagtccatctattgctgcaattgttggtactggaagattagcaatatcgttaatcactgctcttattttggagacaaaaggaccaacttcactggaactcattttggctctttccttaaggtcagcaccagcacagaatatccctgggacttcactcctgattattatggtccgtactttcttatcagatttcaaagcatccacagcttttgatagcatttttataagatttttactgagtgaatttttgccataagctctgtttattccaagcaccacaattcctcggttctcctcctccaggtgccgcacccgcagctcgtcctccgtcttcatctcagagctgtagccccttttcggggcgggacccccggccgcaggtacccagccctgggcccagatcgccgggcccgctcgccggcctgccaacgagccgggcagcctcaaccccgggcagagccacgcactgcaagcggccaccaggcgggcgccgccagcatgcagggatcccaaggccccaggtgccgccgccaccgcggccgccatgttgtctgtttacggcgtggacctgcgacggccgc

SEQ ID NO: 10481 - RNA, 1659 nt, Homo sapiens
  source 1..1659: mol_type = other RNA
cctggcatatttggtataacttcacatttttggtatatagaaattttattttcttaatgcagcacagtagacatacaatcaatattattccctagaatgtgcaatatataaattattcacattaaaaaattaacagaaagcctcatatgcagtaaatatttaaaaatgtatatctaactttgattctgtttctgactatacactactagctttataaatctgaatgaatatgacatttacacatttgaatgaagtacacggatgggtccattccagatgcttattacaccgtatgaataatctgctcttcactttggtcattaaggttccatgtgctgaggcatatagtggatccgaaagacacttccaggaagtacatttattacattggcatcttaagaatttctgttccttttattctcctttatagcgagggggccttttctctttaaaagcaagaagaccttcaagtctgtcttttgttggaatggtctgagcataacaagcttcttctatggctaaccctgttactaaatcgacctccatcccttgattaattgctaattttgccactctcattgcaacaggtccctgaggtaaaaactctctcgccaggtccaaggccttcctgtaggccgcgtctccctcctggttctgttccagaacgtggctgattaagcccactgctttggcttctttgccatcgaggactcgcgcagagaatatgagctccttggccagggacattccaatggcgcgtggcaatcgctgtgtcccccctttgggttttgtaggcaatgcttatagcatccatgttgctgatgaaacaactgatgccagcttaatacttcttcacacacaggcaacttgtttttcttcctctctgaaatcttttatgatcttctcttaatcctccgagcactccaccaggaataatcgccaattttgtttcaaccaggcccatttttgcagaggaagctgctactcgtatatcacaggctaaagccagttcaagaccaccacctaaagcgagtccatctattgctgcaattgttggtactggaagattagcaatatcgttaatcactgctcttattttggagacaaaaggaccaacttcactggaactcattttggctctttccttaaggtcagcaccagcacagaatatccctgggacttcactcctgattattatggtccgtactttcttatcagatttcaaagcatccacagcttttgatagcatttttataagatttttactgagtgaatttttgccataagctctgtttattccaagcaccacaattctatagtgatcagcagccatggaactagagtctcggttctcctcctccaggtgccgcacccgcagctcgtcctccgtcttcatctcagagctgtagccccttttcggggcgggacccccggccgcaggtacccagccctgggcccagatcgccgggcccgctcgccggcctgccaacgagccgggcagcctcaaccccgggcagagccacgcactgcaagcggccaccaggcgggcgccgccagcatgcagggatcccaaggccccaggtgccgccgccaccgcggccgccatgttgtctgtttacggcgtggacctgcgacggccgctccgcccccgcccggcgc

SEQ ID NO: 10482 - RNA, 2606 nt, Homo sapiens
  source 1..2606: mol_type = other RNA
cctgggcagcgtgtggctgaagggagtgaagaacaggaaggccaggtggacatcagggccctagtagaccaacaggcccacagtgccctggaagctgaggctcatctatgccaagcagcaacttcgggcactatccttcgggtagtagagcccggccacgttcatcaactctctaaggatcttcttcttgttttccctgacattcttcttggctaatgccaagagtagcaccaccacatctagagtgtaggtgtcagcaagcttgaatgtgtcgtatgtgtcactccatgcctcaatatcacctccacaggcatctatgttgaacaggggaaaatgcatcaccactggtccagtttctcctttcaggatgtagcagctggcgggggccttggaccacaaatccagctcagcctcttctacttggggaaaggggatcttgtggcggcggcagtagtcagtggtagcccggatggtctcgaaaggatctccggcactgaagtcgaaggagaggatgaggtgaacctcccgcgtcgggggcagcacgagtgggaagggagtgttgatggctaaaccagcatccaccaggtggaggtgcttccggctgctcattatcttgtcccggatgccaccgtgtttgtacaggaagttgtgagtggtcccccattcccactttgaagcgcaaatgcctgttttcttcacaaaatccatcaagttactgagtgagcctttcctttcggggtcctcatggggctgctcctgcttttccagggaggtcctggtccaattctcgagcatctcagtcagccaggtgtgttcaggctcaccgccttcatcaaaaataaggtgtccaatgcttttagcattagcaacagcccttctccataaacctttcagggtcagattccttaactggtcaaaaatgtattccctaatgacttcagtgttaccaagagcacttccccataaacctctcaggaaagtcaggtctctctcagggtgagttctgaccagtcttcccttcttgaatttgcttccgaagtgggttatggaaacaaaggcccccagtgcagagaagccagcgtggtgaggggtgaactcgaaccaggtctctggtgctcttgcctcctgccaggaaggttgcaggtcattgtcaatggctgcaaatattgggtagggtagtgtcccttcttccacgggcttcttcatattggacaaatgagactccggcagttctctggtttgcttagagataaccatgtaggcccagaagtcggtcagagagtaattctcagacctcgctgcttggatggttttctgtaggctcttagccaagtcccactcctgtcgggtaaatcgatgtttcaggtcagcctcgagagcttccatgtcaccatcattggtgtagagagaagatattgcccaagtggatccagagacccctgcgaggtacgtgacggcatccaacaggccctgttctttcatctcactcaggaccccaaggcaggcaatgtgagcccgcagtcctccgcctgagcccagcacagcaacaactggggcctcatcagcctcaatccttagcttcttcagagctttcagcacatgaagtcttcgtctctccacggccgccttttcttctttctggagcccaggaattatggaaacttcagagcttcccatggtgcactgcggtcagaaaattctcagtcctcctgagcctgggtctggggcgtgtgcgcatgcgcggtggagcttgtgctccggaatccggtgcggaggcttgggctccctgcgcttagcggtgtagtcgctggacagctccttcagccggaatctccgcgggtgaagactgcggggatcctcggtgccaaagcttctgtggtcctcctgctttccttttccccctgtgggaggaggtcgcgggctggaggtgtttcctcctggtcctgagcagggccaacctggaggtaaaatggcccctgcgcctttaaacagccctcctcggcttgtaggccctgcttggttgctccagctttttcagctgttccagagctcacccggagctattttcatccgtgggatcacgtggagggctgggactttccaggcttccttagtgatgtcacccttctgtcattaggcacccgagaccagtattcaaaaaaagaatgttgtcgttatataactatattggagataagtattcctcaaaacagattagctaatcctcctatgcatctggctgtctaataaccatcatatataatatcatactcaaatacccagaaaaagaaatattgaggccaggcgtggtggcttacgcctgtaatcctagcactttgggaggctgaggcaggcggatcatgtgaagtcaggagttcgagaccagcctggccaacatggtgaaacaccttctctactaaaaatacaaaaattagctcggtatggtggcgtgtgcctgtaatcccagctactactcgggaggctgaggcaggtgcttcatcctgggaggtggaggttgcagtgagccagatccttagggccaactctggttcatttaatgtccatttttagaaaacctgtgagctccattcacagtgaaggtttga

SEQ ID NO: 10483 - RNA, 3089 nt, Homo sapiens
  source 1..3089: mol_type = other RNA
cctgggcagcgtgtggctgaagggagtgaagaacaggaaggccaggtggacatcagggccctagtagaccaacaggcccacagtgccctggaagctgaggctcatctatgccaagcagcaacttcgggcactatccttcgggtagtagagcccggccacgttcatcaactctctaaggatcttcttcttgttttccctgacattcttcttggctaatgccaagagtagcaccaccacatctagagtgtaggtgtcagcaagcttgaatgtgtcgtatgtgtcactccatgcctcaatatcacctccacaggcatctatgttgaacaggggaaaatgcatcaccactggtccagtttctcctttcaggatgtagcagctggcgggggccttggaccacaaatccagctcagcctcttctacttggggaaaggggatcttgtggcggcggcagtagtcagtggtagcccggatggtctcgaaaggatctccggcactgaagtcgaaggagaggatgaggtgaacctcccgcgtcgggggcagcacgagtgggaagggagtgttgatggctaaaccagcatccaccaggtggaggtgcttccggctgctcattatcttgtcccggatgccaccgtgtttgtacaggaagttgtgagtggtcccccattcccactttgaagcgcaaatgcctgttttcttcacaaaatccatcaagttactgagtgagcctttcctttcggggtcctcatggggctgctcctgcttttccagggaggtcctggtccaattctcgagcatctcagtcagccaggtgtgttcaggctcaccgccttcatcttctgggggaggatgttccccttgtgaactttcttgcagcctcagtaatcgggcaaaaataaggtgtccaatgcttttagcattagcaacagcccttctccataaacctttcagggtcagattccttaactggtcaaaaatgtattccctaatgacttcagtgttaccaagagcacttccccataaacctctcaggaaagtcaggtctctctcagggtgagttctgaccagtcttcccttcttgaatttgcttccgaagtgggttatggaaacaaaggcccccagtgcagagaagccagcgtggtgaggggtgaactcgaaccaggtctcaggacacagttgctgaacaagtgagtgcattttatgcttaggaaatagggtaaggaggtctggatctcaggagagagatgagctcaaaagagaaactggaatgtctggagagctgccagcatttgggtgataatcggacctatggagaaggaagacatctaaaaagtgagagatggccgggtgcggtggctcatgcctgtaatcccagcactttgggaggccgaggcgggtggatcacctgaggtcaggagttcgagaccagcctgaccaacagggagaaaccacgtctctactaaaaatacaaaattcgctgggcgtgatggcgcatgcctgtaatcccagctactcgggaggctggggcaggagaatcgcttgaacctgggaggcggaggttgtggtgagccgagatcgtgccattgcactctaacctggtgctcttgcctcctgccaggaaggttgcaggtcattgtcaatggctgcaaatattgggtagggtagtgtcccttcttccacgggcttcttcatattggacaaatgagactccggcagttctctggtttgcttagagataaccatgtaggcccagaagtcggtcagagagtaattctcagacctcgctgcttggatggttttctgtaggctcttagccaagtcccactcctgtcgggtaaatcgatgtttcaggtcagcctcgagagcttccatgtcaccatcattggtgtagagagaagatattgcccaagtggatccagagacccctgcgaggtacgtgacggcatccaacaggccctgttctttcatctcactcaggaccccaaggcaggcaatgtgagcccgcagtcctccgcctgagcccagcacagcaacaactggggcctcatcagcctcaatccttagcttcttcagagctttcagcacatgaagtcttcgtctctccacggccgccttttcttctttctggagcccaggaattatggaaacttcagagcttcccatggtgcactgcggtcagaaaattctcagtcctcctgagcctgggtctggggcgtgtgcgcatgcgcggtggagcttgtgctccggaatccggtgcggaggcttgggctccctgcgcttagcggtgtagtcgctggacagctccttcagccggaatctccgcgggtgaagactgcggggatcctcggtgccaaagcttctgtggtcctcctgctttccttttccccctgtgggaggaggtcgcgggctggaggtgtttcctcctggtcctgagcagggccaacctggaggtaaaatggcccctgcgcctttaaacagccctcctcggcttgtaggccctgcttggttgctccagctttttcagctgttccagagctcacccggagctattttcatccgtgggatcacgtggagggctgggactttccaggcttccttagtgatgtcacccttctgtcattaggcacccgagaccagtattcaaaaaaagaatgttgtcgttatataactatattggagataagtattcctcaaaacagattagctaatcctcctatgcatctggctgtctaataaccatcatatataatatcatactcaaatacccagaaaaagaaatattgaggccaggcgtggtggcttacgcctgtaatcctagcactttgggaggctgaggcaggcggatcatgtgaagtcaggagttcgagaccagcctggccaacatggtgaaacaccttctctactaaaaatacaaaaattagctcggtatggtggcgtgtgcctgtaatcccagctactactcgggaggctgaggcaggtgcttcatcctgggaggtggaggttgcagtgagccagatccttagggccaactctggttcatttaatgtccatttttagaaaacctgtgagctccattcacagtgaaggtttga

SEQ ID NO: 10484 - RNA, 2094 nt, Homo sapiens
  source 1..2094: mol_type = other RNA
cctgggcagcgtgtggctgaagggagtgaagaacaggaaggccaggtggacatcagggccctagtagaccaacaggcccacagtgccctggaagctgaggctcatctatgccaagcagcaacttcgggcactatccttcgggtagtagagcccggccacgttcatcaactctctaaggatcttcttcttgttttccctgacattcttcttggctaatgccaagagtagcaccaccacatctagagtgtaggtgtcagcaagcttgaatgtgtcgtatgtgtcactccatgcctcaatatcacctccacaggcatctatgttgaacaggggaaaatgcatcaccactggtccagtttctcctttcaggatgtagcagctggcgggggccttggaccacaaatccagctcagcctcttctacttggggaaaggggatcttgtggcggcggcagtagtcagtggtagcccggatggtctcgaaaggatctccggcactgaagtcgaaggagaggatgaggtgaacctcccgcgtcgggggcagcacgagtgggaagggagtgttgatggctaaaccagcatccaccaggtggaggtgcttccggctgctcattatcttgtcccggatgccaccgtgtttgtacaggaagttgtgagtggtcccccattcccactttgaagcgcaaatgcctgttttcttcacaaaatccatcaagttactgagtgagcctttcctttcggggtcctcatggggctgctcctgcttttccagggaggtcctggtccaattctcgagcatctcagtcagccaggtgtgttcaggctcaccgccttcatcttctgggggaggatgttccccttgtgaactttcttgcagcctcagtaatcgggcaaaaataaggtgtccaatgcttttagcattagcaacagcccttctccataaacctttcagggtcagattccttaactggtcaaaaatgtattccctaatgacttcagtgttaccaagagcacttccccataaacctctcaggaaagtcaggtctctctcagggtgagttctgaccagtcttcccttcttgaatttgcttccgaagtgggttatggaaacaaaggcccccagtgcagagaagccagcgtggtgaggggtgaactcgaaccaggtctctggtgctcttgcctcctgccaggaaggttgcaggtcattgtcaatggctgcaaatattgggtagggtagtgtcccttcttccacgggcttcttcatattggacaaatgagactccggcagttctctggtttgcttagagataaccatgtaggcccagaagtcggtcagagagtaattctcagacctcgctgcttggatggttttctgtaggctcttagccaagtcccactcctgtcgggtaaatcgatgtttcaggtcagcctcgagagcttccatgtcaccatcattggtgtagagagaagatattgcccaagtggatccagagacccctgcgaggtacgtgacggcatccaacaggccctgttctttcatctcactcaggaccccaaggcaggcaatgtgagcccgcagtcctccgcctgagcccagcacagcaacaactggggcctcatcagcctcaatccttagcttcttcagagctttcagcacatgaagtcttcgtctctccacggccgccttttcttctttctggagcccaggaattatggaaacttcagagcttcccatggtgcactgcggtcagaaaattctcagtcctcctgagcctgggtctggggcgtgtgcgcatgcgcggtggagcttgtgctccggaatccggtgcggaggcttgggctccctgcgcttagcggtgtagtcgctggacagctccttcagccggaatctccgcgggtgaagactgcggggatcctcggtgccaaagcttctgtggtcctcctgctttccttttccccctgtgggaggaggtcgcgggctggaggtgtttcctcctggtcctgagcagggccaacctggaggtaaaatggcccctgcgcctttaaacagccctcctcggcttgtaggccctgcttggttgctccagctttttcagct

SEQ ID NO: 10485 - RNA, 2063 nt, Homo sapiens
  source 1..2063: mol_type = other RNA
cctgggcagcgtgtggctgaagggagtgaagaacaggaaggccaggtggacatcagggccctagtagaccaacaggcccacagtgccctggaagctgaggctcatctatgccaagcagcaacttcgggcactatccttcgggtagtagagcccggccacgttcatcaactctctaaggatcttcttcttgttttccctgacattcttcttggctaatgccaagagtagcaccaccacatctagagtgtaggtgtcagcaagcttgaatgtgtcgtatgtgtcactccatgcctcaatatcacctccacaggcatctatgttgaacaggggaaaatgcatcaccactggtccagtttctcctttcaggatgtagcagctggcgggggccttggaccacaaatccagctcagcctcttctacttggggaaaggggatcttgtggcggcggcagtagtcagtggtagcccggatggtctcgaaaggatctccggcactgaagtcgaaggagaggatgaggtgaacctcccgcgtcgggggcagcacgagtgggaagggagtgttgatggctaaaccagcatccaccaggtggaggtgcttccggctgctcattatcttgtcccggatgccaccgtgtttgtacaggaagttgtgagtggtcccccattcccactttgaagcgcaaatgcctgttttcttcacaaaatccatcaagttactgagtgagcctttcctttcggggtcctcatggggctgctcctgcttttccagggaggtcctggtccaattctcgagcatctcagtcagccaggtgtgttcaggctcaccgccttcatcttctgggggaggatgttccccttgtgaactttcttgcagcctcagtaatcgggcaaaaataaggtgtccaatgcttttagcattagcaacagcccttctccataaacctttcagggtcagattccttaactggtcaaaaatgtattccctaatgacttcagtgttaccaagagcacttccccataaacctctcaggaaagtcaggtctctctcagggtgagttctgaccagtcttcccttcttgaatttgcttccgaagtgggttatggaaacaaaggcccccagtgcagagaagccagcgtggtgaggggtgaactcgaaccaggtctctggtgctcttgcctcctgccaggaaggttgcaggtcattgtcaatggctgcaaatattgggtagggtagtgtcccttcttccacgggcttcttcatattggacaaatgagactccggcagttctctggtttgcttagagataaccatgtaggcccagaagtcggtcagagagtaattctcagacctcgctgcttggatggttttctgtaggctcttagccaagtcccactcctgtcgggtaaatcgatgtttcaggtcagcctcgagagcttccatgtcaccatcattggtgtagagagaagatattgcccaagtggatccagagacccctgcgaggtacgtgacggcatccaacaggccctgttctttcatctcactcaggaccccaaggcaggcaatgtgagcccgcagtcctccgcctgagcccagcacagcaacaactggggcctcatcagcctcaatccttagcttcttcagagctttcagcacatgaagtcttcgtctctccacggccgccttttcttctttcttcccatggtgcactgcggtcagaaaattctcagtcctcctgagcctgggtctggggcgtgtgcgcatgcgcggtggagcttgtgctccggaatccggtgcggaggcttgggctccctgcgcttagcggtgtagtcgctggacagctccttcagccggaatctccgcgggtgaagactgcggggatcctcggtgccaaagcttctgtggtcctcctgctttccttttccccctgtgggaggaggtcgcgggctggaggtgtttcctcctggtcctgagcagggccaacctggaggtaaaatggcccctgcgcctttaaacagccctcctcggcttgtaggccctgcttggttgctccagctttttcagct

SEQ ID NO: 10486 - RNA, 2649 nt, Homo sapiens
  source 1..2649: mol_type = other RNA
cctgggcagcgtgtggctgaagggagtgaagaacaggaaggccaggtggacatcagggccctagtagaccaacaggcccacagtgccctggaagctgaggctcatctatgccaagcagcaacttcgggcactatccttcgggtagtagagctgaacgagcataggcatcagagcgactatggtctcccacctacccggccacgttcatcaactctctaaggatcttcttcttgttttccctgacattcttcttggctaatgccaagagtagcaccaccacatctagagtgtaggtgtcagcaagcttgaatgtgtcgtatgtgtcactccatgcctcaatatcacctccacaggcatctatgttgaacaggggaaaatgcatcaccactggtccagtttctcctttcaggatgtagcagctggcgggggccttggaccacaaatccagctcagcctcttctacttggggaaaggggatcttgtggcggcggcagtagtcagtggtagcccggatggtctcgaaaggatctccggcactgaagtcgaaggagaggatgaggtgaacctcccgcgtcgggggcagcacgagtgggaagggagtgttgatggctaaaccagcatccaccaggtggaggtgcttccggctgctcattatcttgtcccggatgccaccgtgtttgtacaggaagttgtgagtggtcccccattcccactttgaagcgcaaatgcctgttttcttcacaaaatccatcaagttactgagtgagcctttcctttcggggtcctcatggggctgctcctgcttttccagggaggtcctggtccaattctcgagcatctcagtcagccaggtgtgttcaggctcaccgccttcatcaaaaataaggtgtccaatgcttttagcattagcaacagcccttctccataaacctttcagggtcagattccttaactggtcaaaaatgtattccctaatgacttcagtgttaccaagagcacttccccataaacctctcaggaaagtcaggtctctctcagggtgagttctgaccagtcttcccttcttgaatttgcttccgaagtgggttatggaaacaaaggcccccagtgcagagaagccagcgtggtgaggggtgaactcgaaccaggtctctggtgctcttgcctcctgccaggaaggttgcaggtcattgtcaatggctgcaaatattgggtagggtagtgtcccttcttccacgggcttcttcatattggacaaatgagactccggcagttctctggtttgcttagagataaccatgtaggcccagaagtcggtcagagagtaattctcagacctcgctgcttggatggttttctgtaggctcttagccaagtcccactcctgtcgggtaaatcgatgtttcaggtcagcctcgagagcttccatgtcaccatcattggtgtagagagaagatattgcccaagtggatccagagacccctgcgaggtacgtgacggcatccaacaggccctgttctttcatctcactcaggaccccaaggcaggcaatgtgagcccgcagtcctccgcctgagcccagcacagcaacaactggggcctcatcagcctcaatccttagcttcttcagagctttcagcacatgaagtcttcgtctctccacggccgccttttcttctttctggagcccaggaattatggaaacttcagagcttcccatggtgcactgcggtcagaaaattctcagtcctcctgagcctgggtctggggcgtgtgcgcatgcgcggtggagcttgtgctccggaatccggtgcggaggcttgggctccctgcgcttagcggtgtagtcgctggacagctccttcagccggaatctccgcgggtgaagactgcggggatcctcggtgccaaagcttctgtggtcctcctgctttccttttccccctgtgggaggaggtcgcgggctggaggtgtttcctcctggtcctgagcagggccaacctggaggtaaaatggcccctgcgcctttaaacagccctcctcggcttgtaggccctgcttggttgctccagctttttcagctgttccagagctcacccggagctattttcatccgtgggatcacgtggagggctgggactttccaggcttccttagtgatgtcacccttctgtcattaggcacccgagaccagtattcaaaaaaagaatgttgtcgttatataactatattggagataagtattcctcaaaacagattagctaatcctcctatgcatctggctgtctaataaccatcatatataatatcatactcaaatacccagaaaaagaaatattgaggccaggcgtggtggcttacgcctgtaatcctagcactttgggaggctgaggcaggcggatcatgtgaagtcaggagttcgagaccagcctggccaacatggtgaaacaccttctctactaaaaatacaaaaattagctcggtatggtggcgtgtgcctgtaatcccagctactactcgggaggctgaggcaggtgcttcatcctgggaggtggaggttgcagtgagccagatccttagggccaactctggttcatttaatgtccatttttagaaaacctgtgagctccattcacagtgaaggtttga

SEQ ID NO: 10487 - RNA, 3132 nt, Homo sapiens
  source 1..3132: mol_type = other RNA
cctgggcagcgtgtggctgaagggagtgaagaacaggaaggccaggtggacatcagggccctagtagaccaacaggcccacagtgccctggaagctgaggctcatctatgccaagcagcaacttcgggcactatccttcgggtagtagagctgaacgagcataggcatcagagcgactatggtctcccacctacccggccacgttcatcaactctctaaggatcttcttcttgttttccctgacattcttcttggctaatgccaagagtagcaccaccacatctagagtgtaggtgtcagcaagcttgaatgtgtcgtatgtgtcactccatgcctcaatatcacctccacaggcatctatgttgaacaggggaaaatgcatcaccactggtccagtttctcctttcaggatgtagcagctggcgggggccttggaccacaaatccagctcagcctcttctacttggggaaaggggatcttgtggcggcggcagtagtcagtggtagcccggatggtctcgaaaggatctccggcactgaagtcgaaggagaggatgaggtgaacctcccgcgtcgggggcagcacgagtgggaagggagtgttgatggctaaaccagcatccaccaggtggaggtgcttccggctgctcattatcttgtcccggatgccaccgtgtttgtacaggaagttgtgagtggtcccccattcccactttgaagcgcaaatgcctgttttcttcacaaaatccatcaagttactgagtgagcctttcctttcggggtcctcatggggctgctcctgcttttccagggaggtcctggtccaattctcgagcatctcagtcagccaggtgtgttcaggctcaccgccttcatcttctgggggaggatgttccccttgtgaactttcttgcagcctcagtaatcgggcaaaaataaggtgtccaatgcttttagcattagcaacagcccttctccataaacctttcagggtcagattccttaactggtcaaaaatgtattccctaatgacttcagtgttaccaagagcacttccccataaacctctcaggaaagtcaggtctctctcagggtgagttctgaccagtcttcccttcttgaatttgcttccgaagtgggttatggaaacaaaggcccccagtgcagagaagccagcgtggtgaggggtgaactcgaaccaggtctcaggacacagttgctgaacaagtgagtgcattttatgcttaggaaatagggtaaggaggtctggatctcaggagagagatgagctcaaaagagaaactggaatgtctggagagctgccagcatttgggtgataatcggacctatggagaaggaagacatctaaaaagtgagagatggccgggtgcggtggctcatgcctgtaatcccagcactttgggaggccgaggcgggtggatcacctgaggtcaggagttcgagaccagcctgaccaacagggagaaaccacgtctctactaaaaatacaaaattcgctgggcgtgatggcgcatgcctgtaatcccagctactcgggaggctggggcaggagaatcgcttgaacctgggaggcggaggttgtggtgagccgagatcgtgccattgcactctaacctggtgctcttgcctcctgccaggaaggttgcaggtcattgtcaatggctgcaaatattgggtagggtagtgtcccttcttccacgggcttcttcatattggacaaatgagactccggcagttctctggtttgcttagagataaccatgtaggcccagaagtcggtcagagagtaattctcagacctcgctgcttggatggttttctgtaggctcttagccaagtcccactcctgtcgggtaaatcgatgtttcaggtcagcctcgagagcttccatgtcaccatcattggtgtagagagaagatattgcccaagtggatccagagacccctgcgaggtacgtgacggcatccaacaggccctgttctttcatctcactcaggaccccaaggcaggcaatgtgagcccgcagtcctccgcctgagcccagcacagcaacaactggggcctcatcagcctcaatccttagcttcttcagagctttcagcacatgaagtcttcgtctctccacggccgccttttcttctttctggagcccaggaattatggaaacttcagagcttcccatggtgcactgcggtcagaaaattctcagtcctcctgagcctgggtctggggcgtgtgcgcatgcgcggtggagcttgtgctccggaatccggtgcggaggcttgggctccctgcgcttagcggtgtagtcgctggacagctccttcagccggaatctccgcgggtgaagactgcggggatcctcggtgccaaagcttctgtggtcctcctgctttccttttccccctgtgggaggaggtcgcgggctggaggtgtttcctcctggtcctgagcagggccaacctggaggtaaaatggcccctgcgcctttaaacagccctcctcggcttgtaggccctgcttggttgctccagctttttcagctgttccagagctcacccggagctattttcatccgtgggatcacgtggagggctgggactttccaggcttccttagtgatgtcacccttctgtcattaggcacccgagaccagtattcaaaaaaagaatgttgtcgttatataactatattggagataagtattcctcaaaacagattagctaatcctcctatgcatctggctgtctaataaccatcatatataatatcatactcaaatacccagaaaaagaaatattgaggccaggcgtggtggcttacgcctgtaatcctagcactttgggaggctgaggcaggcggatcatgtgaagtcaggagttcgagaccagcctggccaacatggtgaaacaccttctctactaaaaatacaaaaattagctcggtatggtggcgtgtgcctgtaatcccagctactactcgggaggctgaggcaggtgcttcatcctgggaggtggaggttgcagtgagccagatccttagggccaactctggttcatttaatgtccatttttagaaaacctgtgagctccattcacagtgaaggtttga

SEQ ID NO: 10488 - RNA, 2137 nt, Homo sapiens
  source 1..2137: mol_type = other RNA
cctgggcagcgtgtggctgaagggagtgaagaacaggaaggccaggtggacatcagggccctagtagaccaacaggcccacagtgccctggaagctgaggctcatctatgccaagcagcaacttcgggcactatccttcgggtagtagagctgaacgagcataggcatcagagcgactatggtctcccacctacccggccacgttcatcaactctctaaggatcttcttcttgttttccctgacattcttcttggctaatgccaagagtagcaccaccacatctagagtgtaggtgtcagcaagcttgaatgtgtcgtatgtgtcactccatgcctcaatatcacctccacaggcatctatgttgaacaggggaaaatgcatcaccactggtccagtttctcctttcaggatgtagcagctggcgggggccttggaccacaaatccagctcagcctcttctacttggggaaaggggatcttgtggcggcggcagtagtcagtggtagcccggatggtctcgaaaggatctccggcactgaagtcgaaggagaggatgaggtgaacctcccgcgtcgggggcagcacgagtgggaagggagtgttgatggctaaaccagcatccaccaggtggaggtgcttccggctgctcattatcttgtcccggatgccaccgtgtttgtacaggaagttgtgagtggtcccccattcccactttgaagcgcaaatgcctgttttcttcacaaaatccatcaagttactgagtgagcctttcctttcggggtcctcatggggctgctcctgcttttccagggaggtcctggtccaattctcgagcatctcagtcagccaggtgtgttcaggctcaccgccttcatcttctgggggaggatgttccccttgtgaactttcttgcagcctcagtaatcgggcaaaaataaggtgtccaatgcttttagcattagcaacagcccttctccataaacctttcagggtcagattccttaactggtcaaaaatgtattccctaatgacttcagtgttaccaagagcacttccccataaacctctcaggaaagtcaggtctctctcagggtgagttctgaccagtcttcccttcttgaatttgcttccgaagtgggttatggaaacaaaggcccccagtgcagagaagccagcgtggtgaggggtgaactcgaaccaggtctctggtgctcttgcctcctgccaggaaggttgcaggtcattgtcaatggctgcaaatattgggtagggtagtgtcccttcttccacgggcttcttcatattggacaaatgagactccggcagttctctggtttgcttagagataaccatgtaggcccagaagtcggtcagagagtaattctcagacctcgctgcttggatggttttctgtaggctcttagccaagtcccactcctgtcgggtaaatcgatgtttcaggtcagcctcgagagcttccatgtcaccatcattggtgtagagagaagatattgcccaagtggatccagagacccctgcgaggtacgtgacggcatccaacaggccctgttctttcatctcactcaggaccccaaggcaggcaatgtgagcccgcagtcctccgcctgagcccagcacagcaacaactggggcctcatcagcctcaatccttagcttcttcagagctttcagcacatgaagtcttcgtctctccacggccgccttttcttctttctggagcccaggaattatggaaacttcagagcttcccatggtgcactgcggtcagaaaattctcagtcctcctgagcctgggtctggggcgtgtgcgcatgcgcggtggagcttgtgctccggaatccggtgcggaggcttgggctccctgcgcttagcggtgtagtcgctggacagctccttcagccggaatctccgcgggtgaagactgcggggatcctcggtgccaaagcttctgtggtcctcctgctttccttttccccctgtgggaggaggtcgcgggctggaggtgtttcctcctggtcctgagcagggccaacctggaggtaaaatggcccctgcgcctttaaacagccctcctcggcttgtaggccctgcttggttgctccagctttttcagct

SEQ ID NO: 10489 - RNA, 1204 nt, Homo sapiens
  source 1..1204: mol_type = other RNA
cctgggcagcgtgtggctgaaggtcaccatgttctccttggccatggggctgcgcggggccagcaggtccacgtccacgctggcgcgcttcaggctgcccagcgaggtcttctcgcgggccacgggccggggcgcgccctccagccgccctgggggccccagctcgtcggtgctcaccgacttattctgctgataaaccgagtcgtggccccgctgcgtcagggcccgcagcgcgtccttggcgggggccggggccgcgggcttctctgcaggtggggcctggaagttgcccaccgcgtggcaggccaggtaggcagcgatgcccgccccgatgaggaagccggcatacacgtccacagggtggctgcggtactgcgtgatctgcgtgagcccgcatacgcccgcggcgatggcaaaggcgaagaccaggatgggcttcagcagcttggtggtgtccgagatgaccgagttgaagtacatcgacacatagaccgcggcgaaggctgacagcgtggcgtgctgggacgggaaggtcttccgtgcagacaggatggcgtggatgtcgtggccggagcagatgtcctgcgtgatgtaggggttgacctcgcaggacgtgcccaggagagtgtagttgggcttgcagacggtgaggaagaagggagtgtggtaacccgtggccagctggatcacgtccgtcaccagggctgtggcacacaggccgaacacgtggacacccacaaaccgcaccgtacgccgcaggaaggagttgaagttgcagccgccggcgttgatgctgccctccgccccggcgggccccccggcacggccccacagccgggactgcagacagtacaacatgccctcggccaccatgatcgaggcggcaggggccgcgaaggccaagctgagcagcatcagcagcgggatgagctcctcgttggtctccacgtagggcatggagagagtgcggtcatagcactggaagcccaccttggccggcttgaagaggtcggtcagctccaggaagtacaaggatacgatggaagaagccactatgggcagctccacgaagtagaagcagggcagaagcgtcatgctgtccttcgggatcttgttcttctccttggtggagatcatggtgccgcgggcgccgcaggccgtggctggcgcggccggcgcccagcacaaagcgcgtctcctccgt

SEQ ID NO: 10490 - RNA, 1288 nt, Homo sapiens
  source 1..1288: mol_type = other RNA
cctgggcagcgtgtggctgaaggtcaccatgttctccttggccatggggctgcgcggggccagcaggtccacgtccacgctggcgcgcttcaggctgcccagcgaggtcttctcgcgggccacgggccggggcgcgccctccagccgccctgggggccccagctcgtcggtgctcaccgacttattctgctgataaaccgagtcgtggccccgctgcgtcagggcccgcagcgcgtccttggcgggggccggggccgcgggcttctctgcaggtggggcctggaagttgcccaccgcgtggcaggccaggtaggcagcgatgcccgccccgatgaggaagccggcatacacgtccacagggtggctgcggtactgcgtgatctgcgtgagcccgcatacgcccgcggcgatggcaaaggcgaagaccaggatgggcttcagcagcttggtggtgtccgagatgaccgagttgaagtacatctggggcatgggggttggggtcagggagggctccccacgggtcagcaagagggcctgggaagggcagtgaggggccggactcaccgacacatagaccgcggcgaaggctgacagcgtggcgtgctgggacgggaaggtcttccgtgcagacaggatggcgtggatgtcgtggccggagcagatgtcctgcgtgatgtaggggttgacctcgcaggacgtgcccaggagagtgtagttgggcttgcagacggtgaggaagaagggagtgtggtaacccgtggccagctggatcacgtccgtcaccagggctgtggcacacaggccgaacacgtggacacccacaaaccgcaccgtacgccgcaggaaggagttgaagttgcagccgccggcgttgatgctgccctccgccccggcgggccccccggcacggccccacagccgggactgcagacagtacaacatgccctcggccaccatgatcgaggcggcaggggccgcgaaggccaagctgagcagcatcagcagcgggatgagctcctcgttggtctccacgtagggcatggagagagtgcggtcatagcactggaagcccaccttggccggcttgaagaggtcggtcagctccaggaagtacaaggatacgatggaagaagccactatgggcagctccacgaagtagaagcagggcagaagcgtcatgctgtccttcgggatcttgttcttctccttggtggagatcatggtgccgcgggcgccgcaggccgtggctggcgcggccggcgcccagcacaaagcgcgtctcctccgt

SEQ ID NO: 10491 - RNA, 1877 nt, Homo sapiens
  source 1..1877: mol_type = other RNA
cctgggcagcgtgtggctgaaggtcaccatgttctccttggccatggggctgcgcggggccagcaggtccacgtccacgctggcgcgcttcaggctgcccagcgaggtcttctcgcgggccacgggccggggcgcgccctccagccgccctgggggccccagctcgtcggtgctcaccgacttattctgctgataaaccgagtcgtggccccgctgcgtcagggcccgcagcgcgtccttggcgggggccggggccgcgggcttctctgcaggtggggcctggaagttgcccaccgcgtggcaggccaggtaggcagcgatgcccgccccgatgaggaagccggcatacacgtccacagggtggctgcggtactgcgtgatctgcgtgagcccgcatacgcccgcggcgatggcaaaggcgaagaccaggatgggcttcagcagcttggtggtgtccgagatgaccgagttgaagtacatctggggcatgggggttggggtcagggagggctccccacgggtcagcaagagggcctgggaagggcagtgaggggccggactcaccgacacatagaccgcggcgaaggctgacagcgtggcgtgctgggacgggaaggtcttccgtgcagacaggatggcgtggatgtcgtggccggagcagatgtcctgcgtgatgtaggggttgacctcgcaggacgtgcccaggagagtgtagttgggcttgcagacggtgaggaagaagggagtgtggtaacccgtggccagctggatcacgtccgtcaccagggctgtggcacacaggccgaacacgtggacacccacaaaccgcaccgtacgccgcaggaaggagttgaagttgcagccgccggcgttgatgctgccctccgccccggcgggccccccggcacggccccacagccgggactgcagacagtacaacatgccctcggccaccatgatcgaggcggcaggggccgcgaaggccaagctgagcagcatcagcagcgggatgagctcctcgttggtctccacgtagggcatggagagagtgcggtcatagcactggaagcccaccttggccggcttgaagaggtcggtcagctccaggaagtacaaggatacgatggaagaagccactatgggcagctccacgaagtagaagcagggcagaagcgtcatgctgtccttcgggatcttgttcttctccttggtggagatcatggtgccgcgggcgccgcaggccgtggctttggatggactcggaggcagcccagcttcctgggacaggactgcacggactgcctggggaggggtctttggccccccggttcctgcaggggggctcggggaggccctgtgagcagttggtcacaggtgggtcccattcgatgcgatcctgttcctccccaacagccctggagaagggggacgttgcctgctgtggctgcggctgttttcctggcctgtgagaggcggggccagagtggccgttgggaatctgggtgttgcaaggtgaccacaaacagctctctgggggaggaggaggaaaatgcaattgattttcaggagccttctgaggtcaggagtgggagagtgtgcagggggaccctcctggcagcttgggggtccaacagaagatctgggggagtctcagggtcttctccccctaggatcaccagtggtggagatggggcaggcctggccatggagggcacgttgcttggctgaggggcctgggcttgagtgtggggcctgggcttgagtgatgggagagttccgagcaggccggaggggttgagcgtaccagacgctgctcaaaacttttatttaaaaatgattattattattattactattattttgagatggactcttgc

SEQ ID NO: 10492 - RNA, 2318 nt, Homo sapiens
  source 1..2318: mol_type = other RNA
cctggggacaggggattggggcaggtaaggccccagtccctcgcaggcctgcagttttgtgttcaggctttccctccccatcttccaggccaagtcagaccacatccaccacaaagacacttccctcgaggatttttccagcaggtagactgaaacagaggccaagtcctctcatttttctgagtgacttgaaggggaaacatgtacaagtaagaaaagaggatgcttaagatatcagaatgtattttgccctggattgtctaaattggctgtttgcgtggctctaataatctataaaatcattatgatttttgcatttttctattcaaatgaccagggccatggagtaaagattttttttcaagtcaatgaggtaaacaagaaagaagaaatgtttcacattttaaaaatgatttctttgtcagttagcaatgaatatcatgctctaaagtaaggaagagaagaaattagcatgggttgtagatgccaggaacttgaccttccaaatcctcacagcaatctaatgagggctgtgcctccaaagtgcacagtggggcagctaggttgtcctccctgggtgtggggagaatcctggaattttaccatcttggtgtctcagagatgtgcccacacaggccttcaagaactctctgttgaattgcattatgagcaaaaattgtgtgttcctgtggtttccttgcaggcctcttccagcccaggctcagaaaacattgggcagatttcctgtgtggcctgactaaacggggttttaagcgccaccaacacctctgtgggaaatgccattcctgtcgccaagagacaccccctccagataggcatctgcaaggaaaaagcagctgttctggcggctttgtgaaccttcacctcggtttagagcacctgagggcagatcgagatgtgcgtccccacctggctgctagagagccggcccagagaaacaggagattcaggtagccatcagcaatgccagagaagccctcgctccactgcctttcacccaggatgtcacagacccacctcctggcccacacacgtgcatgccaccagcatcaacatgcaggcagacacagccactcccagatgcacctcccctggtgccaagaagagttttcagatacaaggagggaaaggaacaggggtttgggcattgcagacctgagtttgtttgcatcttagctctgccattttaccttgctgggcattctcttcctcatctgactccaactgagaactgaacatgggtcataaaagatgggttttgtccccttcccagtggaatgatccagaaacagcctgcgccccctgatgcacgggctccttgtggtggccccgcctacgccaccccactcctgggtttttctcctgcttgagttgcggaatggcaggcatgactgcagggaacaagtgagagagcgtccctgccgccttctatttctgccaattccctcttcttttctctcaggtctgagtcgtgcaggaaaagagtgatgaaaccattccctcactctctcctgccactgagaattattcgttttgttccaaagagtctcgtgggctggaggcagccacagggcttggatggagttcattatcgggcacagacccagggcagaacataaaagattcagccttgacattttacagatggaaacaaatttctgcgctgtcatggtggggctcagagagagcacattttaacacagacacaggatgaaaactctttacagtcctggactggtgggagcagcagcacagctcgcaggagaccaacattggcacgatcggcctcatgaccctcaacaaggctctcatgctccatgagcctcagttcccctatatatacaagaggggacactaaacacctgctgtagggctgttggtgcctagcgctcccatggcacacagcctatctggacctacctctaggttatcagctgtgtcacactttgccggggaccacggatgtgtactattataaatagctattgtttattgaaatgttactatgttctgagaatttttaatcatgcatatagaagactttggtggtgccccagccatcccccctccccactaaccatttccatacatgttgtcccaacttccgaatgccatcatttccgaatctatctgaggatcctctctggttgctggtgcccaccgtgcccacgtgtcaaataatgagagagctgaggcattaaggcaccccaggagtggtcctcccacagtgaatgatgggaatctgtggataaataccccagctcccttgcccctcaggcaaggtcctactgagaggg

SEQ ID NO: 10493 - RNA, 1683 nt, Homo sapiens
  source 1..1683: mol_type = other RNA
cctggggacaggggattggggcaggtaaggccccagtccctcgcaggcctgcagttttgtgttcaggctttccctccccatcttccaggccaagtcagaccacatccaccacaaagacacttccctcgaggatttttccagcaggtagactgaaacagaggccaagtcctctcatttttctgagtgacttgaaggggaaacatgtacaagtaagaaaagaggatgcttaagatatcagaatgtattttgccctggattgtctaaattggctgtttgcgtggctctaataatctataaaatcattatgatttttgcatttttctattcaaatgaccagggccatggagtaaagattttttttcaagtcaatgaggtaaacaagaaagaagaaatgtttcacattttaaaaatgatttctttgtcagttagcaatgaatatcatgctctaaagtaaggaagagaagaaattagcatgggttgtagatgccaggaacttgaccttccaaatcctcacagcaatctaatgagggctgtgcctccaaagtgcacagtggggcagctaggttgtcctccctgggtgtggggagaatcctggaattttaccatcttggtgtctcagagatgtgcccacacaggccttcaagaactctctgttgaattgcattatgagcaaaaattgtgtgttcctgtggtttccttgcaggcctcttccagcccaggctcagaaaacattgggcagatttcctgtgtggcctgactaaacggggttttaagcgccaccaacacctctgtgggaaatgccattcctgtcgccaagagacaccccctccagataggcatctgcaaggaaaaagcagctgttctggcggctttgtgaaccttcacctcggtttagagcacctgagggcagatcgagatgtgcgtccccacctggctgctagagagccggcccagagaaacaggagattcaggtagccatcagcaatgccagagaagccctcgctccactgcctttcacccaggatgtcacagacccacctcctggcccacacacgtgcatgccaccagcatcaacatgcaggcagacacagccactcccagatgcacctcccctggtgccaagaagagttttcagatacaaggagggaaaggaacaggggtttgggcattgcagacctgagtttgtttgcatcttagctctgccattttaccttgctgggcattctcttcctcatctgactccaactgagaactgaacatgggtcataaaagatgggttttgtccccttcccagtggaatgatccagaaacagcctgcgccccctgatgcacgggctccttgtggtggccccgcctacgccaccccactcctgggtttttctcctgcttgagttgcggaatggcccgggactttctcactctccctctgtttcttgtctctgctgctctcagctccttggcttcttctataagtctcaggaagatgctgagcacctctctgtgccatgctctcctgggaattaggaatgagaaatgatggtgttgctcagggcctggtagggaggatagtgcgcccaagtcatcttgatcccaagccatcttgatgatgctgcaatggaagcatgtccctggcatctgcagcctcaaaggataagagtgcatctgcttgagagagaaggcctg

SEQ ID NO: 10494 - RNA, 1686 nt, Homo sapiens
  source 1..1686: mol_type = other RNA
cctggggacaggggattggggcaggtaaggccccagtccctcgcaggcctgcagttttgtgttcaggctttccctccccatcttccaggccaagtcagaccacatccaccacaaagacacttccctcgaggatttttccagcaggtagactgaaacagaggccaagtcctctcatttttctgagtgacttgaaggggaaacatgtacaagtaagaaaagaggatgcttaagatatcagaatgtattttgccctggattgtctaaattggctgtttgcgtggctctaataatctataaaatcattatgatttttgcatttttctattcaaatgaccagggccatggagtaaagattttttttcaagtcaatgaggtaaacaagaaagaagaaatgtttcacattttaaaaatgatttctttgtcagttagcaatgaatatcatgctctaaagtaaggaagagaagaaattagcatgggttgtagatgccaggaacttgaccttccaaatcctcacagcaatctaatgagggctgtgcctccaaagtgcacagtggggcagctaggttgtcctccctgggtgtggggagaatcctggaattttaccatcttggtgtctcagagatgtgcccacacaggccttcaagaactctctgttgaattgcattatgagcaaaaattgtgtgttcctgtggtttccttgcaggcctcttccagcccaggctcagaaaacattgggcagatttcctgtgtggcctgactaaacggggttttaagcgccaccaacacctctgtgggaaatgccattcctgtcgccaagagacaccccctccagataggcatctgcaaggaaaaagcagctgttctggcggctttgtgaaccttcacctcggtttagagcacctgagggcagatcgagatgtgcgtccccacctggctgctagagagccggcccagagaaacaggagattcaggtagccatcagcaatgccagagaagccctcgctccactgcctttcacccaggatgtcacagacccacctcctggcccacacacgtgcatgccaccagcatcaacatgcaggcagacacagccactcccagatgcacctcccctggtgccaagaagagttttcagatacaaggagggaaaggaacaggggtttgggcattgcagacctgagtttgtttgcatcttagctctgccattttaccttgctgggcattctcttcctcatctgactccaactgagaactgaacatgggtcataaaagatgggttttgtccccttcccagtggaatgatccagaaacagcctgcgccccctgatgcacgggctccttgtggtggccccgcctacgccaccccactcctgggtttttctcctgcttgagttgcggaatggcctagtgcagtacaaaggagacagttgaggcttctctctctttcgtcaccagcacagacagatgtggcaatggtgttcaggaaagagagctgagagcagactcgatgccccgccatgaggcaggtgatggaaccccaggtttctgctcccagtgtacccaaagcagcccccctggtccagcaaactcccaaattccatacaggcatgactgcagggaacaagtgagagagcgtccctgccgccttctatttctgccaattccctcttcttttctctcaggtct

SEQ ID NO: 10495 - RNA, 915 nt, Homo sapiens
  source 1..915: mol_type = other RNA
cctggtggcttccttttcgactgtgaaatcctgggccagctggtcagccacgcagggcagcacccagtagtgagggaggagaggcccgtgtgctaaggctgcttcctgagcccaaagaaggggccaacccagctccgaagaccaggttagaagtggacttgagcagaggagagcagaggaaaggccaggagagggtgagggctgggatccacaaccagcccttgccaagtggctgctgagagagcaggtttgtgctccctgctctgcagacgtgcaagccccagggcagaggaagggttgtcgggagaggaccccagcttccctctggtgggatgctccagctcgaggggctgtggaggggcagtttgggccgtgaggctgggctggagggcactgagcttagaggaagacccctgcaggctggaaccagtgtgcgaggcaaacaggagagggctgggggacagctggacaggaggttcagcaaccacagcggggccaagggacagtgagggcagggggcactggaggaggctgggagaatcatgaggctgtggacctggagagagcggctgagctgggtaacaggaacccggggtctggaacagctccagctgctcccggcagccatgttgtccctgtgggccagggcccaggagcccctcagcctggtcccagcagcccaggagccctggagctgagcaggaggcacaatccatggggcacaggcgctcatgcacgtgcagggtccggctccaccacgccagctcggcctgcagggactggatctccttccgcagggcgaggttgtctttttccagagactcgtgctgcaaattccctgtggtagaattccaggcctgtgtagtggctgcagctcagacctccggtctcctctctctcgccttctttcttgct

SEQ ID NO: 10496 - RNA, 1034 nt, Homo sapiens
  source 1..1034: mol_type = other RNA
cctggtggcttccttttcgactgtgaaatcctgggccagctggtcagccacgcagggcagcacccagtagtgagggaggagaggcccgtgtgctaaggctgcttcctgagcccaaagaaggggccaacccagctccgaagaccaggttagaagtggacttgagcagaggagagcagaggaaaggccaggagagggtgagggctgggatccacaaccagcccttgccaagtggctgctgagagagcaggtttgtgctccctgctctgcagacgtgcaagccccagggcagaggaagggttgtcgggagaggaccccagcttccctctggtgggatgctccagctcgaggggctgtggaggggcagtttgggccgtgaggctgggctggagggcactgagcttagaggaagacccctgcaggctggaaccagtgtgcgaggcaaacaggagagggctgggggacagctggacaggaggttcagcaaccacagcggggccaagggacagtgagggcagggggcactggaggaggctgggagaatcatgaggctgtggacctggagagagcggctgagctgggtaacaggaacccggggtctggaacagctccagctgctcccggcagccatgttgtccctgtgggccagggcccaggagcccctcagcctggtcccagcagcccaggagccctggagctgagcaggaggcacaatccatggggcacaggcgctcatgcacgtgcagggtccggctccaccacgccagctcggcctgcagggactggatctccttccgcagggcgaggttgtctttttccagagactcgtgctgctgggatatgcacgggcctccaacccgtgtgtcccccaaaccacctattctcttgcccacaggagccattcagcaaccatgtcattaattgcaggttaaagccctttagaggcacccaccaaattccctgtggtagaattccaggcctgtgtagtggctgcagctcagacctccggtctcctctctctcgccttctttcttgct

SEQ ID NO: 10497 - RNA, 1028 nt, Homo sapiens
  source 1..1028: mol_type = other RNA
cctggtggcttccttttcgactgtgaaatcctgggccagctggtcagccacgcagggcagcacccagtagtgagggaggagaggcccgtgtgctaaggctgcttcctgagcccaaagaaggggccaacccagctccgaagaccaggttagaagtggacttgagcagaggagagcagaggaaaggccaggagagggtgagggctgggatccacaaccagcccttgccaagtggctgctgagagagcaggtttgtgctccctgctctgcagacgtgcaagccccagggcagaggaagggttgtcgggagaggaccccagcttccctctggtgggatgctccagctcgaggggctgtggaggggcagtttgggccgtgaggctgggctggagggcactgagcttagaggaagacccctgcaggctggaaccagtgtgcgaggcaaacaggagagggctgggggacagctggacaggaggttcagcaaccacagcggggccaagggacagtgagggcagggggcactggaggaggctgggagaatcatgaggctgtggacctggagagagcggctgagctgggtaacaggaacccggggtctggaacagctccagctgctcccggcagccatgttgtccctgtgggccagggcccaggagcccctcagcctggtcccagcagcccaggagccctggagctgagcaggaggcacaatccatggggcacaggcgctcatgcacgtgcagggtccggctccaccacgccagctcggcctgcagggactggatctccttccgcagggcgaggttgtctttttccagagactcgtgctgctggtgcagggcgtctgccttgtctgtgtgcttctgccggcttcgctgggcggctgcccggttcttctgcttcttcagctgcctttgttgctccttggggtctgtctgggtcagcagcccattgcccccacagaggtgcatggcttaggcgggggagcagagtggtccctcagcagctgtgacttcccagtgccctct

SEQ ID NO: 10498 - RNA, 88 nt, Homo sapiens
  source 1..88: mol_type = other RNA
cctgtctgtgcctgctgtacaggtgagcggatgttctgcacagcaagtgtagacaggcagacacatgacaactctgtccagccaggcc

SEQ ID NO: 10499 - RNA, 2110 nt, Homo sapiens
  source 1..2110: mol_type = other RNA
cctgtctgtgcctgctgtacaggtgagcggatgttctgcacagcaagtgtagacaggcagacacatgacaactctgtccagccaggcccttggttccttcaggtttcctttgctcatagacagatacaatcagcctgttttccagatttggtgattttggagagtaaggggaaagggagaaaaatacacaatataattaaacattaaaacattatggaactaaaaacaagttagacttttgactttattcagaaagtacatttatacatttgttccaaatgtgctaacatggataatttgcgtaacagaaaactcacattaaaattttaaggaaaaaaagagattaaacacaaggtttattcttaagtccaattcatattattactggcccacatgtagtcagagttcagcgtaattgaaccagatgtttttcctctttgcaaaaaactgcatattttaatactgaagttaaagataaaaactatgtttatgcatgtttcttttagtagataagtaccataaccttgtccatgaaaaagaaaattatcatttacatggaaacagcagcccttttcaaaataattaatgagcctaatttatttggcaacccaagttgctgactttggtatttgatgctctgataataggatcctacaagggaatatgtttttaccaattatatgtgaaacaacaggaacctatttaaatgtctcattttccttttaaatgcaaagtttataactgtggatgtgaaatcaaattaaaggcagttgtgagcttaagttatccacctcttaattaactatagggccatgctgtgaatcaaaagggtacaaactggaaggctgttactcacagtgatgctcagaatgtgttttggatatagttagtgcaatatagttacaaaatagtacttaagaaaaggcagaaaaggcaaattcatttcatatccaaaaaattaaaaccagatcctttgaaaatttttcttataatttatatgagctaatagtgttaaatatgcagatataaaatttaattctggtgagttgagagtaattctattttaatatcaattatcaattcacatctttagaagtattaagcaaattcccctccccttttaaaaacaaaaatatccaaatagtcaaaattccagtaagtaggacttcttaaaaaacacagcaccaaaaaaacacagtattgtccaaggattgtataattagacattttctcaaagaactttaagaaaaacaaacagtttgtgatttatctttaattgtaaaattctgagaaaatagcaaatagaaacttaatggaaagcaaaatagttttagatactgagaaaattacaattttctacaaatctggacttttatgcagtgattaggtaaggtaatgttttaacaaaagctaataagtgccattttctgtgtatttatgtaatttcaagaaaacaaatttccgattctgtttcggccatcactttcgagtaaaggaactttttttttttcttgacagaatcaaaaacatgagtaaacttggctgttatttaaataattacaaggttagagtatgccaaaaaccagtgccttaaaatactattgtgttattgttgctgcattcagtgcaacagaaagtaattatagagtgattcacttacaaagagtatattggtggaaattaaaaattactataattctttataacttttcctctctctcccataaataatttgatccagttaactctgctcaattaaaggaatgatgcatgcaacacttattacatccaggggtagttttagttgaagatgctcactgttggttagtttcctctggaatagattccatgatccccgctggtcttcccttcggcagtcttttctcagcagtgtccccgagggcttcttggtccctagtgtgcaaaacttaaaatcctctcccggtcctcaggaaaagcctcccttcctgcaccaggggttgcattcagctttcccccctgaattctgctgcgctgactgagacacactcaagggctgtgatttccagtcttgacgtggcacatttgctgcagactggggaactggcaatgaatttaggaccaggaaaag

SEQ ID NO: 10500 - RNA, 6016 nt, Homo sapiens
  source 1..6016: mol_type = other RNA
cctgtctgtgcctgctgtacaggtgagcggatgttctgcacagcaagtgtagacaggcagacacatgacaactctgtccagccaggcccttggttccttcaggtttcctttgctcatagacagatacaatcagcctgttttccagatttggtgattttggagagtaaggggaaagggagaaaaatacacaatataattaaacattaaaacattatggaactaaaaacaagttagacttttgactttattcagaaagtacatttatacatttgttccaaatgtgctaacatggataatttgcgtaacagaaaactcacattaaaattttaaggaaaaaaagagattaaacacaaggtttattcttaagtccaattcatattattactggcccacatgtagtcagagttcagcgtaattgaaccagatgtttttcctctttgcaaaaaactgcatattttaatactgaagttaaagataaaaactatgtttatgcatgtttcttttagtagataagtaccataaccttgtccatgaaaaagaaaattatcatttacatggaaacagcagcccttttcaaaataattaatgagcctaatttatttggcaacccaagttgctgactttggtatttgatgctctgataataggatcctacaagggaatatgtttttaccaattatatgtgaaacaacaggaacctatttaaatgtctcattttccttttaaatgcaaagtttataactgtggatgtgaaatcaaattaaaggcagttgtgagcttaagttatccacctcttaattaactatagggccatgctgtgaatcaaaagggtacaaactggaaggctgttactcacagtgatgctcagaatgtgttttggatatagttagtgcaatatagttacaaaatagtacttaagaaaaggcagaaaaggcaaattcatttcatatccaaaaaattaaaaccagatcctttgaaaatttttcttataatttatatgagctaatagtgttaaatatgcagatataaaatttaattctggtgagttgagagtaattctattttaatatcaattatcaattcacatctttagaagtattaagcaaattcccctccccttttaaaaacaaaaatatccaaatagtcaaaattccagtaagtaggacttcttaaaaaacacagcaccaaaaaaacacagtattgtccaaggattgtataattagacattttctcaaagaactttaagaaaaacaaacagtttgtgatttatctttaattgtaaaattctgagaaaatagcaaatagaaacttaatggaaagcaaaatagttttagatactgagaaaattacaattttctacaaatctggacttttatgcagtgattaggtaaggtaatgttttaacaaaagctaataagtgccattttctgtgtatttatgtaatttcaagaaaacaaatttccgattctgtttcggccatcactttcgagtaaaggaactttttttttttcttgacagaatcaaaaacatgagtaaacttggctgttatttaaataattacaaggttagagtatgccaaaaaccagtgccttaaaatactattgtgttattgttgctgcattcagtgcaacagaaagtaattatagagtgattcacttacaaagagtatattggtggaaattaaaaattactataattctttataacttttcctctctctcccataaataatttgatccagttaactctgctcaattaaaggaatgatgcatgcaacctgaaaaaataaaaagaaatatttgtgagtttgtatgttatgctttaatataaaacagttttattaaggcaagatataaaaattttttgagccagaaaaaccacaacagtttttcaggggaaaaaaaaaatcttgctgaaaacaattgttctattcataaggcttttggacaatttatgtttctgatagatttttaaaacacacttacagtaactatgtgacatatgcacacttcattgttatgttgaacctgcccctaaacttgttaaaaagatgaaagactgaaaaccatattgacctttttttaatctcccaaattataggttgaatattagtttattattacttaaaatactagctaaaacataaaagagctatttgtattattatcataccatgtaatttttagtgtggttattacaccttgttttctttttgtcttttatttcttaaggaaaaaaatgtaagaaaagaattgtcttctaagtcttctgtagtgaaattaaaccaaagcaactccaggaaactggctgtcacgctaagtcaaaaaattcaaaatgaagatttaattatttttcctaatttacttcgttatctctaactattaaaactgataaaaattatttgtaagagacctttgaaaatgagtaaatatttatttctacttaatttacagaacatgaaagtaagaagggatttgaagtaagaaagtttctatcttaactcaggaatttcctgtctcaggttaaagcctgaccttctagttattttaagccaggatttctgagtgatggtctcttagttattattttgacgttattgtgatgggtgggctattctccttagagcagagtaaagtgcattgtttataaagagcagatcccttacagagtaagtgaaagctttggcgtctctttaccgagcatggatgcttgtggatgagtgaattttttcacattaccaagttgtactttttatatcttataacagcttaagacttcaaccaaaaaagtggggagaattctttcgttaggatttttatgcctaaactgtttcccacagagtgaaatacatgggtggtctgtaggcgagaggtgggggtagatagtatattttggtcttttacaaacataaacatattatctgggccgaaagcccgaatgccaagcaggaaggatattaagcctattgactaactacaggaaagtgatcagtgtgaaactttgtcctatagtaaacagtctttctttgattttgagatctgtggcctaaaagaaaaatgagtttgaaaatttaagtccaccgttttagattgatccttttccagttaagaaattgtggtgttgaagctaaggctctgaacttcctttctcttagatggtggaaaagtccttttaacccagtacctagtccaatttatcaatcattcacatgctaaaatgaaaaataattatgaaatttctatgaagtgtagtttggacagaccctgaaacaattttctcttcatgaccacatataatgtttaattttaatacttacacttattacatccaggggtagttttagttgaagatgctcactgttggttagtttcctctggaatagattccatgatccctaaaatatttgtatatctccttataaagtaatatgaaaataaaattaaacatttttctaatttacctggatatagatatggctataatgtatataaatgtgggcgtgtgtaccagcgcataaactacaatcctgccttcattcagcagagctttataaaatgagcttttacctttgatctttaatttagcccatataattgaaaaataagtactattcgttttcatttgttaaaactttgcctcgaaaataagtcgctagagccacatcaagcatgtgcaggaactccttggttatccttttacaaagtaattcttatatttctactcctgtacttatgccagaggcacccttatgtcccttctatctccagactaaaagtcatcctgagggagaaaataggtgagggacccatagggattcatttctttgaaacaaaaagaccgtttaacatgaagaaagaaattgaaattaaatatacattaaatgaaagcaaattttgaaatgtaatcatttctagagtaaaaaaaaaaaaaaaacccagaaaatttgagaaaaacattaccaaagtaccttgttagctatttttcctcttcagtaattgtatcaattagaaaaaatatatttcttgaaaaaatgagctcctctaagttactttttttagttttcttatgtaaaagaaactatatagatttttaacatctcatttgttctactaaaaataattaatatggaactctccaagtcacaatagaaaatgaaaggataactttactatatcatctaagtgaaagtagctaaatttctccttgctgtttatattttaactaataatcatgaatatatgagaatacttaatgttttctttatacacattttggggtgatcagaagggtaatttttaaagtaagttgttttgacaaaagaaaacttagggaatcttttataataaaatattttgctaaagagaacttgagtcaatttttgaattgttgcaaaatgtataacttagaaaagaatttgttcaggaaccactgtaactttaaaggaggacaaaagagattatgtttatttttcacaaaccctgtagaagagatgttttcattatatagaattgtttcggaatagaaattaatgggggttaagaaaattagggatgaggcaataacatttttccagaactttctttaaggggccgacctctaaagttcagcacagatcacattgcaatccagacttgctctattattttctctattaggatttcattcagcttgagggttttcttccctcccaccttcctccccctctcccaccctctttcacctccaggacagctggaaactgaccaaagaaaacttctgccttcgtttacaaattccttttttatcagtgggtttctagacaaagtgccttattttaaatgctcagagaagtggaagcattgtaagctataggcaagagggctcagctgagcagcaattattaaccactctttgatttaaaaaaaatgtaaaacagatatttacaggggtatctaaagatagaggtttttattccctgatttactcagttgctgactcaataagttgtgggtcggtgctcttctctgggcaaatcccatctgcattgtctggtaggcaagacttggcaggttcttcttttattgttaggtactattattcctgttgtttatattacagaaggaaatcttcagaaaagcactatccatatagcatttaaaaaccagcaagtattctttactttggggaaaaatgacttcagtcctgggatgttaaaagttatacatacagccttcatccatataagtttttaaatctttgaattattattaaacaattcaaaagtagcctcattaaactattcttaagtgtctggaatgagttttttcatatttcattttgaagtgggaaaacctttaagaaaacacttgaattatcaatcttcagaaataaaaaaaaaaaaaacagtaaatcgctatataccacacacttttgctcttttaaaattaaatacatctctacccatcacacatgtacctctgtttcccttgcatgttaacacaaatcatgggctccccacctaggttcccttggtcacagaccaggtgagcagtcaagaaggccttacccgctggtcttcccttcggcagtcttttctcagcagtgtccccgagggcttcttggtccctagtgtgcaaaacctgtgaagaaaaacactggatatgagattcaaaaaaggagcaaacaaatgtcttctccttggaaacagcccattttgtccccagcggtccatggcgttgctctcccttgcccagtctaaccaatgtgcagactactgtacaacggcattgtcctgaacaggtagtctgaacactggggcgacggagcaggatctccagaagcttccttctatgtacttaaaatcctctcccggtcctcaggaaaagcctcccttcctgcaccaggggttgcattcagctttcccccctgaattctgctgcgctgactgagacacactcaagggctgtgatttccagtcttgacgtggcacatttgctgcagactggggaactggcaatgaatttaggaccaggaaaag

SEQ ID NO: 10501 - RNA, 1377 nt, Homo sapiens
  source 1..1377: mol_type = other RNA
cctgtgccttttacttctttaagaaataggaagctcaagccatcactggttatttctccagctctatgctttgagtctattagggttttatcccttttttcttgaattccatattttcttcctccttgatttatttcttccttttgtgggagtacatctttcagtaattctttcacagaagatttttggctggcaaattttctaaggctttgcagatctgaaaatgtctttatttcaccatcacatttaaatgctaatttaacttcacacagaaatttaggttcaaaatcattttctctcagaatgttgaagacattactccattgcttactaatatccagtgttgctgatgaaaggtcggctaccagggtaagtactgctccttcatccatcaacactttttcttctctggaggcttttaaaacctcctctttattcttcaatttctgaaattttctttcctctctcatttctttgacaaattcatcctctccatccttcctactctctctttctgtaaattctaaatggacattgcgatttccatctctgtcatctatattgcataaggtttcttccatacttcccatgacttcgtaacttcgtgattcaccctggggtaatttcttaccatcattactattgtattcgttagtgttgtctaatttaccactcagctcatttacttctaatttaaaggttaaattttcattatcatcacctattttagagttttctccttctattttccctaccatccctgttttttgtaatgctaaattgattatttgctgaaactctgtcctactactggagttctctgaattctttacctcaggtattgtagcttttccccctaaaactgcttttaggtcatttttaagagtttccctcatctcctcaaacatcaggtcttgaatttccattaagaccttaaacttattcataattgctgatacgtccttgcattttaaatctaataccggagctatgtccttatcagtttctgttaactgctctcttttcatataggtgatattttcctttttctttgcaagtctagcaaattttgattgtacactagtagatacatcagacattgtggatatgttgtcaagactggattctgtttttaattcctacagaatgatttttgttcttacaggcctgctagacttcagaagttaaaaaaatcttaaaatacgtcaatcaagtctcagcagttcatccgcctctgtaccttcgctgggaagacgaactccgcagagcaggactcgggtctactctaagctgtgccttggtgcctggcgaaaaaggaatccgcctggacgactgaggagcgaacaaagtgaggatggagccttgtaactaaggact

SEQ ID NO: 10502 - RNA, 1488 nt, Homo sapiens
  source 1..1488: mol_type = other RNA
cctgtgccttttacttctttaagaaataggaagctcaagccatcactggttatttctccagctctatgctttgagtctattagggttttatcccttttttcttgaattccatattttcttcctccttgatttatttcttccttttgtgggagtacatctttcagtaattctttcacagaagatttttggctggcaaattttctaaggctttgcagatctgaaaatgtctttatttcaccatcacatttaaatgctaatttaacttcacacagaaatttaggttcaaaatcattttctctcagaatgttgaagacattactccattgcttactaatatccagtgttgctgatgaaaggtcggctaccagggtaagtactgctccttcatccatcaacactttttcttctctggaggcttttaaaacctcctctttattcttcaatttctgaaattttctttcctctctcatttctttgacaaattcatcctctccatccttcctactctctctttctgtaaattctaaatggacattgcgatttccatctctgtcatctatattgcataaggtttcttccatacttcccatgacttcgtaacttcgtgattcaccctggggtaatttcttaccatcattactattgtattcgttagtgttgtctaatttaccactcagctcatttacttctaatttaaaggttaaattttcattatcatcacctattttagagttttctccttctattttccctaccatccctgttttttgtaatgctaaattgattatttgctgaaactctgtcctactactggagttctctgaattctttacctcaggtattgtagcttttccccctaaaactgcttttaggtcatttttaagagtttccctcatctcctcaaacatcaggtcttgaatttccattaagaccttaaacttattcataattgctgatacgtccttgcattttaaatctaataccggagctatgtccttatcagtttctgttaactgctctcttttcatataggtgatattttcctttttctttgcaagtctagcaaattttgattgtacactagtagatacatcagacattgtggatatgttgtcaagactggattctgtttttaattcctacagaatgatttttgttcttacaggcctgctagacttcagaagttaaaaaaatcttaaaatacgtcaatctgtagtcccagctactcaggaggctgaggtataagaatcacttgaacctgggaggtggaggttgcagtgagccaagatcacgccactgtaccgggcgacagagtgagacccaagtctcagcagttcatccgcctctgtaccttcgctgggaagacgaactccgcagagcaggactcgggtctactctaagctgtgccttggtgcctggcgaaaaaggaatccgcctggacgactgaggagcgaacaaagtgaggatggagccttgtaactaaggact

SEQ ID NO: 10503 - RNA, 22796 nt, Homo sapiens
  source 1..22796: mol_type = other RNA
cctgtgccttttacttctttaagcctgagaagcagcaggctaccaattgctcccatttaaggatgtggctgccatgataatctttcacttgttcagcagtatttctttttctttccattgacaagctaggatacgagcacagtccctgctctgccaaaggaaaccatgtcttttgttaaagtttaagctactgataaatatttaagggagtgcaggggtagatgttaatattacctagcaaagaattcatgggcaaacaactttcaaatgtatcagtaagtttaccttaaaatgacttactagataatgagatacatctaatatatttgcaactgaaacacttgaagctttcaaggtctacctgaactaatttcttccctccctccctcctttccttccttcctttgtcaaatatttattgaatgcctaacatgtgcctggcacccttcagggtactgggcttatagcagtttacagagcagaaaaatatctctgcccccttagagctttcaatttactggggacagacagacaataaacaaatcccatgacaaatatgaaagaagggaggagatttactatattttcatgagattgtcaggaaaggcctctctaatgcatacttatttaatatttaagaagaaaccaaaaagatgtgagggaggaagatctgtggctaactgggggaagaagagcattcagggtggtgggaactgcaatgacaaaagaccaaagggggtgcatggttgatgcagagagaacaaagggggcagtggctggagaagtggtcagagcaggagacaggggaacagactgggtggggcttcccctctttcgtgaatctcccacccaagttaatgtctgtgaagagatggttcttttgtttaggcagataaaatgccttcttcaaggcctatttgaagctgcatttccttcttgaagtattcccctttaatgccaatagttccctatacccagattctcttaactctaaagtatgaatcatgcaatcatttcttgtgctttattgtgagtgactatttcttctgtcagcatctttaaagagattgcaagcaatttaaaggtagaaaacacatcatactttttcttcatcccatatagcacatgatgttaaactcaaggtaatcaagaaagaaatgaaagaaatatataaaactgtcaattaagaaaagacaaagaaatatatgactctaaaaacaaattcaggtattttgagaatatagccatgaaaacaaaaacattaaggtagaactcagtggataagacacatgatctgattttgtttagtaatctacatcattgcttatcccaacttagagcttatacctatacatctgtagatctcttcttcctgtcctacagaaaatgtaatccctcatccatgcagccttctttctttctttacattagcactactgcccattcttcacaatgtctatcttcctttatgattttttttctctgaactcatatcttcaatttcctagagtattgttacctagcagggtcagggctattagtggagcagaaattataaacatttgagagacataggtagagggttaaaaacccactagtctactagtttatttcactcattgcttgggatttatctacttaagcaaagcaattaggttacaaatgaactggcgataaaatactttcataaaaattatttatcctgagataaactctttatgatttttagacttgaaataattttatatacttttaaaaatcagttctgtatctaaggtagtatagtccaactaagaaacagagttgatgtgctccatgctgaggtcgaatgaagaagatagaaagtgcccctggatgcctctctaatcattattttagtggaacatttcaatcgcagtctaattattgagctctcccaatccctccagtgctaaatttcaaacatgttggaacttggcgtgaagaagggcaagattgtttttctccatctgtagatgaattcttctttttacctaaactacttagtcctgatttttctttaggccatccttctaaatatgtcttagtcattgctgtgctaaatagaagaggtggcaacagggtagaaaacgactcattaacactccttgctgatgttctttcataaaactattttttaaaaaaattttatttgtgtctcaattcttgcctgactgtttacttactagtatttatttcttttgggtaaaattatgagtttgggaacctatttacacttacattcactaatttgtttaagtgtattaatttcaaacaaaaagatgtataccctcaaggctgtatctgctgtgtttaatacactaatcaatcattaggcatccttgccttcctatcttaccattttgtccaaaacacatctagtactcattgacatttatgtccaacaaacaaaaaaatcagtatagcaacttctatttattatggaagacatgttaactaagaatcttgaacaatttttagattaatagcaggttaattaggttaatagcaggcaaataaataataactctagttttgccaatgtctcataacaaatgtttcagtgaaagcaaatagttactttcttctttttatgagacattaaagtattccgctgagcaatttgaactgctttgtccctcacacaggactttgtacatcacttggcacattataggttcttaatccatgtttgttggatggattaatgaatgaatgatatggctagttcatcaggtcattttattttcctagttcctaggtaactgtccatatttcctgttatcgaaaaagttcttccaatcagttattctctttgtcgacttttagctgtgacttcctattattgaacataacccagtactctaagtattcgaatttaatacaaaaagaaaatctattggaacatttggtaagagatatttgacttacatattgtgtgtaactctgattggagtttcagcacttctttattgtataggtatgaccaagttggcctttaggaggcctgatggatttttaatgaattatcggttttgccaatcattacttttgttgcattatggctttttttttaatatcttgggtctggcgtatatcatagtttagtagctgtgctgttgggaccaaagatctacttacaaccattttcaacacatactaaattttttttgtaggctgctttcccccttttcccttcattgaagttctccaagaaataaccttcctgaagtcttttattcaagatcaaaatttttcaattattctagaatgctatatcattttcaaaagaatgaaaaataaaatatcaacctgtttatttatttggtttcctggccatttgtcaatttttttcttcatattttactatttatggtctagtttaacttggtttccatttgcttacttctcattccctgaaattgtactgggacagaagggaaaaattagttctgtgttattttaattgaaattcatgctgatgaatcatttttccttaagtattcttttcttctattaggttataaattactcaaatagctagaaatcagcaatattgtttagaaaataagaactgatttccacacagacccattaatactgtttcctttggaattgtaatactcatctgctcttcagtaacaaagacaggcttctctaacatgacattatcaatgtttgcttcctggaacactagttctttaagatgctccatgaacataatgacccatggtcaattatatctgggaaatcaaatactgtctttatgctactggaacattaatttcacacattgagggtaattcaaagaataggcttcattttgccagtgttgaagccattttaatttcaagtagcatttcgtgataatataggaacaaaaagatcttcaaattctctgggcattcattgtacttaactttttacttaagagttggtatttatcaatatgatttttgtgttgtatctgagacttatgtggtcccacatgcaggggcagatcaaaattttgttgagcctgaagtgtatacatttttggagtccccttttaaggaaaagaatgcaaaaatatcatacatttgaaaattttatataaacataagatgtgaacatactgctaaggactgtcctagggcctccaaaagacttatgtaagcaatgggctcagaaatttaagcttcattagctacatgctacacttgcatatcccacatgaaaaatagtactttactattatttggcctaataatataatagtgtttcagcctcattatttctggttcttttctccacctgacacataccctacattcttagggttgtgagatttagcaagtaaaaatgcaatatgcccagttaaatttgaatttcagagaaacaagtatttttagtatagtagattccaaatattgcatgaaacatacttgtactaaaaatttcattcactgattattggaaattcaaacttaactcatgtcctacatgaatctagttctagtatagagtgctagttctagtatacagtggttctagttaaaccagtctataacaggacttctctgaaaatgacacattcttttatactctacgccttggttccatgttcctaaattttcttcatgaaaagactgtccagagcaacttattacaaatagagattactaaggccatcccttcaagagtttaaaaagtcttctagatgagttctaccaacaggtagacttgtcagatatggccttagttcaggtaatttcttttcttcaaactggaatgtctttgcactcttcaactatgcagcctttcaggcctagtggtgagaagctgacctttgtcctcaccttcttccctggacagatttaatccaactattctcagaatgtctgttgctgttcacaaacttagatttcagagattttcaaagtccaagtgtggttcctcagactagtagcattagcatcacctgaaaacttgttagaaatgtaaattttcaggcctcactccagatctattgaatcagaacctctggagatggggatatgcaggctgtgctttgacaagccctccaggtgattttgatacatgcttaagtgggagaatcgctgctctataaatggagcccattatttttgagatatatatatacacacacacacacatatatatatatggctatttcacctactagtttgctttgctaaaatccttgatgggtagtggctgcctctcatttctctttgcatttactctctatgtgtctggcacatagaagatgtttaaaattcttcttgaatgaaagatttggagaataaaggggttaatagataattacattttttttgagtaagctacctggtgaaagccatgacccaaagggcatcgcataaagctacgtggatgatcaagctgctgtgtggccccattgcatggcactgtggctccaagttccaactcttttacattttctcaagttgttatctgcttcctcatcctcacgtattttagttctatgactgtagaagaatacaaagagttcatatggattattttcacaggtcattttaatgctaatgttaaaaccatgtatgtgtgaaatatttgacaggacaattataccataggaaaagttttgaattagagacaggccatccaatgaatgtgtaactatgtgtaaggatatgttgtgaaaattacattttacatatatatccatctttgtccagtgctgacataacattgcaatactacatctttatggtagaataaaagcatgtgccttatacataactttcatagaagatgactgcagagcagatctctgattgtgggaggaacagtgatcttgtttctaagcataaatcacctgaactgctaaattccctgaaatgcaaataaatctcaagaattatttgctaattaaattgatgtttatatatgtagattaatctagatactattgtagtgtctctagctataatacgtgcatgtagataagagttatatatacctgagtatccagtaattttacatggaaaaaagtataaaagattagactgcctatttatgttcctaagatattcgtttcttcctctttgactcatcttttatttactgaatttaattaatgcaatataaaccatttttccccaagttagatatgcagaaaaccaaatcaactgttctgtaaagataaagcaatttcctgaaaatttgtggtaaagctttacaaatgttataaaaatgggccacgctgcatgtcaaaaccacaggaatgtgaagattaaactatacattagagtattgtagtaaatagatcacacagagctaataactagttactgttataccacattaaattcactaatgtgaatattgttgtgttttagacactcaaagttcttgggtgttcaggccatcttacagatataagttttgtgaattgtatttatttcttcctttttatattcagtgccacaactctatttcaggccaatattaccttcattgctgatgaccacaacagcctcctaacttaattctttggttcaggtctctcatctccagtctaacctacacttagaacattgcagattaatacttctaaattttgaatctaataataataataataaaaagtaatctgagtccatcaaatcaaatataaattctgcagcatgatgtttgcaggtccttatatgaaactttctggtttgtacaaattcaactcctgtactggaaatgtaccctcaagctaaattgagttcgttgacccaggaacatattctgtgcttttgttgcatgttatggctttgctcagtctggtcccgtcacatggggtgctcaggccaataatcttacctcatcttaagtgctatcttaatgcaacacactcataccaggtttggctctactagaaatcatctctctaccctctggatatctccttttggactctgtacaagttctggcttatattctagttatagatgtcacagacgcttttgtcttgtgactttttaaaacttcacttaataaaaggctctatcagtatttattggattaaatgtgttgacttggttgtctaagccactgtttttcaaattgagccacacattgaaatcactatgggaactcccagaagtactgaggttgggtctcgctataggatatattgatttaagtagtctggcatgaagtctgggcattgagactttaaacatctctctaggtcattccaaagtacagcaaattttgagaaccactagctttgttactcctagggttatccaaaatgtctcttagagtgtgtttgttgaccatggtctcgtatggccacttggttgttggatttatctccattctacttctgtgaacagatgtcctcctcgtgaaccagttggaaaatggggcctccccaggccaactccaaccttatctataactctaaaaagcataattaggaaatgcttttttcaggtttaaagtttaaaatatattcctccaaacatcttgtaatatgattgctggttttggggagcaccactattataattaaaactttaactattaaaaaggacaagggtaatgtataaatcagttaggtttatgcttaaaaactaagtgcatatgtaccttatgtgatcttcaaagaaagcatcagtgaatcataaggaagtgaatttaaaaaatagttttaagcattttaacaaactcattgtcttaaaatttacatttagaaaaggatagatggggagaaaatctatgcagttatttttcatcacatataatttacatttggacttctctgtacatgcacctttcatactgatttatgatgaaaagatgatatattttaccatagggacatagtacttgtttacaatgttttctttctgggaacaatctataaatcagggacaataatacctattctattaggcaggtattatttgaattgttaattaaaataatattaacagagatagttaattggagtgtattagtttgagctgtttgttctggagagtttgggttcccagcaatccatgtcagtctcttactctcacactttgagggcttttgtgccagaacgtggacggtgttccatcatcaggagaatcaaactcatgctctaaactggctcttgcaaccactacatttcaaagcaagagagattataaatttatgtgatattgctcagttttgggatccttgattttaacagttaaaattcaaaaatagagactgtgtatttacattttgtaaaccattcactgcatttaagcccaaggatacatcataaaaagagctttttctttatgatccctctccaaaatccaagtaactccccatatcctggcaatgctttataataccactcacaatgggcgcttcctttttattcccatctgtaacaagtctcttctgggttgctatcatctcatctgttatagccttcatcctggacaacctgctttcctgcccttgtatatttcactttttctccctgactgttgagcccatcctccatctctatctattagaatcttacccacacttcaatgtggatcagttcataattccttccttactttccttgaatactccagctgcaaatttcctcaacagatcatgcatacctcaaagtcaggaactatgaatagtttagtggtattttcttctgagcctagcacagagaccaatataggtgctcctaaatatgaggtaagtaaataggtacaatcacaagccatctaggggtacttcagaaacccatctacatcaaatcttgatcctaaaatgggactgaatttctagttctatctttttaaagagtaacaaactttttggagacttagatatgtcagggtttttctgaaactttccaatgtgttcctttgtttttaaagcctaactaagctaatgaacagaaactaaataaaaaaaaggtttcagttcagttgtttagtcccttcttcaacagttttagatccgttttaaaattttttctcactttacctttttttttaaaaaaacacccttgtccttaatttttctttatgttggatcacattctcccttattttactatcaagatgtgtatagctctaggttgtagcatttcaacttataggaaaggacagttattaccaacaaacttgaaattcttcctttatatggggccttattattgtgtaactggctatataggaaaattcaagaaaatgaaacaaaacaacaacaaaagcttctgaatatgggctctcaaagattgaaattattaaataacctccttttcattaggtcatgagcaggcaactgataagctggagaagtcttttatatttttcttcactgaatggataattactgaacgtctgcaaagcagacattgtgtgcttcatagtttggcatgtcagttgccatttttaaaataaaatcagtggagaatttcaacttgaagcacatataaatgacaataaatagtacttttgcaaactttatttagtatttgcaaataggttccaaatgtccagcttaatttttctgagttcttatttcattcctttctagccatgcttatttttatgtaaaggagaaaacatgcttaattactctaaagaaaagttattttagaaatgataaaagttgaacatatttaaaggaaaaaagcagaataaaattaataattaaaatactaaatttggacaggaaaatggctattgaataagtccaaacatttccaggaaagacataaaggcatccttgtttttaagaaaacatacggcaaactatataaaatgaaatattactaagacttctttggtctcctcatcatacgtcaataatgaggagagctttgcaatgataaagcttttgaagtggcttgtggaatattaaattgtttaagtataattttggcatcaagtgaccttacatattttgaatgttggttatctatgcgttatgtataatgccaccacattattcatcaaaatacagtggacttggatattgaaatatttaacatgattggttttagtgacttagaagtggtgctgatagcccctgaacaattatgccccagcttgaaactgtatagcgtgcagccaaagggatgtgctttgtgattaatctctgggtactactgaggagccgctggctcactcattgtctccatcttctgcagctctcatatggtgagaaaaatgttggttcaagtatttttatagttaatattactacaataatgcaatgtaatgcagtgataaattttaggtagaatttatttgacccgattataaattgctgtagatttgaaggtaacataattattaaggggtgttaaagtgctatctgaatcttttagtaatgctttagtaatttatgtgttttagagacatttgtgaacttagggattcataaaaatatctctcaggaatgccaagacattttgtatttgcttcagaatgctttatcttaaccacggagagataattgatatatatcatcacagtattattttaatgtatgtattcttgaatgtttaaaggataaaaaattacattataagttttagaacttgtgattcaataaaatactaaaaaaacatagattatgttattttacattgtgatgttataagatgttttgtttaggaagtttaattcttagcctagaattaaaaggtagcatgctcgaagttctcactgaggttagaggaataagttgcatattataatattctgtggggcatttaatactaacaataaagaatgaagaaaaatctggcgaatttaagaataacctagcttttacagcatttgtgattgtgattttaaaagacctcatatttgaccctaagaactatagaatatacacctgtataatttatcactactttaatatataaattatttctattattatgactaatggaactagatttcttttgttgttaaaataaaaagttgagatagccagaaatgctgtttaactttgcctagtggcactgtagtaaatatgattttgatgacttttttttccaagtagctaagatttaattgttatttttcttaagatttgtacctgtaagctttagataatagatttgtcatgcagataaattatgagcaatttaactaaaattattgtatttcagtgtgtccaaaacatgaaaataatgatgaaccgaacaaggaaatatttggaacataatttcccttgactgaggtatgagattcatttaattattaaatgtgtgtttacacatgcaaatctatgggaaataatttgttctttatttgtttctattatagttaagaaaaacctgttttgcaaaatgttttttcactgatcaacatagaggtaaattttgataatggaccaaattcaggtgaattggaaactttggaaactttggaaggacttttggtttgggttcttagtaagatcaaaaataggtacttttagaatattttcttctttgtgagatctaaaatggctacacagcagtcttctatttcacaggagatatttttggatggaaatacaacttgggtaatgtttttttgatttgacatttttgttcacaattcgtttttaagctttcctcagtaaggtagctttagttgtagagcccaaggtacagaactacagagcagaaacctaaaatggctttgtttgtactattttgggagtgataaatgaggctgttttcatgaatgggatgaacctatatgtaatagagtattttagaaggaatattgttatgggtaaagacatctggaattgatggtttgccatgaggtttgtagtgttaatacatcaaagtttcataatttcatacatttagtcacccttctttgctgtagaaactggtattttgtctagctaggattaagaacaagtgggttttgttttaggaaagaaaataaaaatgctcaacttttactctcatttctacaatttgtctatgcatgggtgaagactgtttctccctaggagttttcttttcactgatgctaatgtttccgtaagtgacttgtgttttaaaaaccccgatttagcagaaaataatagcaatgccttccagaggaaaagaaaacttaagtaaaatgccaaataatggtaactttgtctctttctatttgcctagaataaacaaacaaacacccgaacagattttttcctccaagaaaagtgataagtgaaatgcacttggaatttttctgaagttattcacagattatttgtgcatcttactgggtagactgctgcctctaatcaaagtcagattactctctttctgagtcaatttttgagctctgggatatctgtagggagacaactaacaactgccttgaaagatttcatattaatgaatattatgttaaccagaatgtataagtgggactgcatataggagtgctcattttacattttgccttgtctaatttgataaagtgaatgagcatcaaggaaaggtgataaataatattgctttgtggctttaatatattgccatttaatcaaagattgcatgccattttgtctttaaatacccttatgaggtagcttggagagatctctgcccttttcaatctgtgacagatttcctagttcagagcaaaaaagtctactgctgaaaaatatgcataattaacaggaaagtataataaagttgttgcttaaactactaaaactttgggatatttgcattgactagtttaaggtctagtttatcagtttgtagcacatttatgtttgtgaagaaaagatgccagaattcccttattctacttgaaaatagatgctacagactgtaccaggagatgcaagaatatgacggcttattcttttttttttttccccagctctatcagtgttgctaccaacaaccagtgaattcatcagataaaatgatagaaggtgtttccgtgtccagggagagattctagtaaccatattacattagataatttaaatgctccccataacatactgtagactgccgctactgagaatataagttaaatttatatagcactgaaaagttatacatttttattaaacaccagtaatctttcgtccatgagagtgtttcctagttattcctaggaaattcttcaatgcagtcttccaaagcattagaatttttttccccctctggtttgacagagccttgtgggcaatgtgcttactctacaaactgtggcaacagagggaaagaaaaccgtaatgctcctctattagaccatgccattagctgttgggaaaccagagctcagctacaaatggcttctaaaaacctcagctcagataagtgcaatgaaatcatacacagcaggaatcacacaccatcagtggtgattcctactctgttcctaaagtttctttctgatttttaagattttataattaccatgacctgtgagacctttcttaagggaaattttcaactggggaaaaatagtagaagctggctttctataatttaagatagtgcaaaatcagtgatagtttcctttataaatactttattatattaaaaatatctaccttatagaggttttcagtttaaggtacactcccatttaatttttacatctttagagatgcagaagacataaaatgtgatttgtagactaggaagttatactataaatatattcttaaccctatatattgctcttttgagttgttttccgttttataagaaaagcaagtggcttctctatcagcaatagagagtcctcattaagtatgaaaaaaactgattagaaaaagtgttcattatgactcaaagactcacaaaatatagtcaatgagagccactctgggaatgaatgatgcttatgtcggtgcttactttaagcttctttacaaagagtctccctagcttttcactttcactaacaaaagggtctacggctcttcctttgtgcttggaaattcaggagcacctcccactgcaaagattaggttatgaatctaacaaatgagaacccagtcttcaagtgcaatgtatttgcctatgatcaagtttgctagcagttgagaatctatagttttgcaacaccacgtgattctctctgctgtattctaaatcacagaatatgtggtattattccacttgttctatcacacctacttacagacatcttgatttctgagatgtgggctcatctctcaatatccttccagtgtcatttcaaatgttgcctgatctaactccacaacacttcaaacacagaacaccacctcttgtgctcctaagttaaacgtgatggtggattaatcttggtcctttagttgataaatcaaggtaatttactgctgctatacccatacacagtccctcccctgctggatctcatgcagtgtggctttgttgctttcacttatgattttgctgctttcatttgggtcaatatcattgtagttattttgtagacaaagtagtaaaaaacttgatttttccctatcctatatatctgcagctcactgatttaaaatattagcataaaggtccgcaccacagtgatgatgttcaatttcatattgagattgaagatggggaaatagcaagggcataccaattcagccataaatatgttttgggtcaatgtcataaaattgtcacaaaattttggtaattgagaaaaagctaaaactttttttgtttgttttttgtttgtaaagggaagaaaagtgcttctgaggctcttttggaataagtaacagttttcagattcacttttgcaaagattgccaatatccttcgcagacaccaacaaaccagactgaacagaaagatccctgtagtaggatgccgagcaaatcattgacttctccaatctctaagagacaatatctaaatgtcagtctcatggcattgtattttctgcttcaccataagattagcaaacacaagacataaaattatgtttatttactaaccaatacagaatatactaggccctttgcctggaagccagatttcacttctgagattttccgaagtccattctagaagaggtggttgttactgatacccagggaaggcaattcttaaattgcttacctggggatggaactttctgtggactttaggcccttaagaccaaaagccatgaggcatttatgaataggtgatgtaagaaattttaataaaagttgcaataaccctgaaaatagtgtctttaataacctatgtactattaataacaaagcatgcatagtgccgtgcattcataactatttggtcataaaaatatgtgactgtaattatgatatttacagtcaacttataaaaatacatgtaattctgaatggcaatagttaatccttagctctaaccacaagcctagaaggattagcttattacggggaaatgtgatagataattacaaaatggacaaagcttttactgtcttgaatttaacattcaagaataactataatagcatcataaaacatttgtcatcattattcttctcacctcacaaggtaaaaacctaaattctgtggaaataaatgggaatcaaataggaaagggccacttacatgatacaacaacagaggagaatagttctttcatagaatactcatgcacagccttcaaagaggttcatagtaactgcaagaattcctgggaagacatctaaacatgactttcattaaaaagaattaaggctggtctaaagaatcaaatctctaaggtatgattacctttaaccataaacggtaaaaaatcttttagctgatctctctgtaatttaggtgagtacctctttgaagtttattaacatcaaagagagtggagctcacatggcactttccaattcaaatttaaattctgatggaaggaaataaatccacattccagtttacatacagaaaaagagtagttttttcaaactttataacctcttactttaagggcatatatgtttcaattaaataaaatattacacaaagctaacatatttcccacaaatttcttctcttctaggagttgattggtcatctgctgacaacagataagttcctaatttgaatggcattagtacttcataaatgaacaaaacaatgagtgcaaactggaaaaactagggagaggtgcatacaagctaccaaaaaaggttgggattgggggtgacctgcaagtcatgatctcatatcttaggatgtatcttagtattcaggaaatggaattcttggaaacatctgtttcacagtgaggttgggaggtcagacgatgctctgttagattcttcttaggattaaattacttcctaggactgcattaagacactttaggtggtatattaactcttccagaacaaataattccatttcagtaaattattgctacagttctctaaagagtactacggtgtcctggaaaagataatgttccttccaaaatgccctctagtcactcgaacaatgagaaattcatatttatcttagacactttgatccttgaagacataaactaaaaaagaactgtttttccctatctaaacagagactatctggatggagacataatattagatctgccctggtcatttggcagtgtataccatttcctccatgtgcttttgacaactggcatgcttgattctttccctgtaaatcagcctgccattcttctttgcatgcagaatggtctataggaaccaagaaaaaaccaaccccaatagccaatcttttaaaaaataggtgaatgagtggagcatggcacacaatgggaagaaaaggagtgatagttaattaactttctcagtgattatctcccatattttgatatgggagataaaaatcttccatatcaaatctttacaaatgatgggtaatctgtaagaggaattctcctcctccctgcacccccactacaaaactcccacccaaacaaaaaatcaaaacccaaccaaaaacctcctctgaaacttctacttcagatatgagatcatggtctggaggctactcgtaccaaataccagttcattctagtacagcagttcatgaggcaaaaggctaggagtatttgtgacatgactttacaaataatgtaaaaacaataaccctatgattatgggcaataattttccccactcaaatctatagatattgcactgaaactgacacaatggagaagacatagatcatttcctgttgaaacccaattacctcaaggtaaaacaaaacaaactccatttaataaatgaaatattacttaaatgttttcattttagggtctgttccctttcccctttatattctggaaagttatatgtctaagtatacttgttttgttacttcattagtctatcaacttcatttccagagactataacgagaatggaatggtttgtaccttttttctgaacataattgagtcaaggagttttgttattttaggtattattaatttgattaaaacatagaaccaaagttgatgggaagtagtagctttcttctaggtaaaagagcttactagcagattttataatcatcggacatttattctgtcctacctggaaataaattatgttactgcttggcatgggaaaaggcattttctagtaatttcctgtgacaggaggcacagcaatagtccaagtaagcacccaacaggtgcttgggagtagttttaaactttaacttaatgaaaacatttacctcagtacttttgtttgagaaagaattcagcagcagttatagttaatatcccacctgtggagagctgcgatcaccctaggaggtgggccaaccgaggagcactttccaggtaacaagagcaacactattgtgagaagctacaaatggtactgcagtaggtgtagtgaacactactatagtgatcatggcctgggttatgttccaaatactaatgcaaggaatacactagagtttataggattagaatagtttccttatgctaagaactagtagatggcatgtgatgagtgggtatggtccattttattctatttcactctacgagtttcctagttatgtctcctttctcctatgttaattatctatattccatgacagttattttccctatctaaaataagaacggtgtaactatggagtaccccaactcacatacacatacttgtgcacccttagactcatgtatggataatctgtgtaaagcgctcatttgcaattgggtgagctcactgaaagcagccatatcagtcttccaaatacagtaaaagccaacgaaaatccatatcaactgtttatttctaatatgaaacagtaaaccttgtccatgtggtaattaattcaaatgccttttgtgttttcttgtgaagtcatccaaagcaaaagtctagatgactgctgacatgatatgcataatctaatgaactcacatctctgtttattttgctcatcccacagttgaatgacacactgactgctgagacacttgggttgatttagaacggctattaatgaatctataaatttggctaaggttgatttgactttctagggaaaagccagcctatcttcaaatggacagctccctccacataaacgtcaatgtaccctaaagacaaaactaagtatatgtatatacgggatatatacatatatatgtacacataaaatggattgggaagtcctttggtttagacagtattaaatatgtacttcccaagtgcataggtttcctttgaccaacctgttcaaaaaacaagcatgaaaagtgccatggcacatttcccatgtctttccccctatttgaaggacacctttccttgcttctccatcactcctaagcattttatttttaaaagaagctggttattttggccttctatcttaacactccattgattcatccattccttggaagagctctcagattacatccagaaacttgtttttagaggagaacaaggttgcaaataactttttcctctttttttattccctcttccccccaagaagcaggcaccttgaagtgtcatgaataatgcactcttgatctgacttgccttgttacccctggccagcccaagcagctgaggtctgagctttacttgccctgcatcattgtgcaatactggaaaagaaaaataatccactggtctatacccctcatactgtggtgacgtgatccgggttctcttgaatttctatgcattcaatttcctctctctcctttcgcttggcacgtttctttttcttgtggtgctttttggaaggggggaaaaacgttaggaacacaggtaaaataacaaaacagtgcagaagtgtgcaacccccagtgagcagcaagcatttgaacagtgtgaaggtcaggttcgaaggcacaaatagaagggggactaacccaataagaaaagaagtaacattttgcaaaatggctgtcccatggtcttgcaaggagctttttatacattgtgttcgggtgtgctcagttgctaatacaaatgtgaaaagcagtggtgcacagtggtcaatggcgaaattcaaggtgtagataaggcacaagatagaaatgcaatccatgtcgacgttccataatgtcattaagcccagaacgcccagctcaattgaggtgacgctaagaattagccagaagtttcccagagggtggatcactaggaaaaaagtcaggattaacaccaggagaacaccaaagcctgcaatcagaacaggcactgtgacagacaagctgtaatggtccatgaagacaaaggaggggttgaacacgatgaatcggatgctctttgagagggataggggcctcagcttttccaacacttctgtgatttctttctgcttgtctctgctagtcctggccaccagatacaagcgagaagcaatgatattgctttcatcccctgccttggagaagatgatatcatttcgaaaatgctggaattctggcttttttaaaaatgagctttgcaggacactgatgaagtcacttttgttattggcactgacgttgctgactttcaggaactggtagtactgctccacccaggacactgcagtgaatccactacagagtcttcttaggtcatcctggacgctgctgttccagtactctaggggctcatagacgtagaatcctatcacagggctatagttgctgaaatatttctgctgaaccatggcataggaaacacttggcgaatcactggctagtagattgatgatgttggctccgtcactgatctgtaagcaccccatgaaggagaaggaggcataaatgagatagaggatgacaacaaatggcttcacatatatattggtaatccattcattataatgttcacggaggaagtgctgaatgaagtggtgctggtaggggttcgtctcatgatgggacgtctgttgatgcccatcactcatcactgtctggaaccacacaggtttgcgatccaggtattctgcagaagggatcttacagcaaaagatgctgtggtagcggttttgctctagttggccagcaaagaccagacaggagccaaagaaggagaaaatgtagaagtagttcaacagaatagagacacacatgttttgacagaagaccttcacagcctctatgtttgtgaatgggctggcacccatgccaaaagtgatgaagtacagggagctggtcatggtataggtgaccatcacatcagaataggcatctgctatcctgtctttgaagggcaagttctctttggttctccgccatccggacagaagctcaaacactcctttagttccatgacccatggcgaagaacgggattcccagcagggtggagttgtactttccatcggtgatgaagaagatccctgctgctgtgatgatggagatgcatactgtgagcacccccaggaggcccaggaagggcttactgcgcaagcagtccttcatggagctggagagggtggctgtggtcaggatcagcacgaggctcaccaggaccttgcttctggccaggatgctggtcttatgaaagtccctccagaggctaaaggatgctaaagagtagagctggagttcttgatgctcctcctggagcttccttataagcttacagaactcattctcccacttctcccctatgaggtcttgggtggcagagccataggtctggaggtagtaggtgatttgaatggctctggctgacttgacccgctgatctttgctgtttggcacttccactaccccgcccagttggtgtccaataaaactgttcctcccatccttcatttccagcacggctcggtgggtctgcaggatcccctcagcctggagcaaaatattgtccccggttggggagaggaggatcaccctgccatacctcccaggggtgtgtaagtccgaatagagctggcttttggactggtccagggggaaaaggctgctggccaggctgcgctcgatcttggccaggctgtggctgggagcgaccaggcgctccaggtcgccctcgggctggaagcggttgagcgcgctgaggccgaaggtgattgtcaggactgcgggcacggtgaggaaaaagaccgggtgccggctcacgcacaaacccagcctgtggcagaacgactggagccctctgcgaagcacctgccgcagcatcctccaccagatccagctcgcaggcgctcccggccgtcgcatgagcagcgttccctcggtctagcccttcatctcggtgctgcagtcccctggcctccctcgctggaggtggttccgtgtggagcgtcccacagatgtggatttcctctctgtcttggtggggttcggtgcctaactggaaccatgtgcctcggtgttgtaagaagcagacatgtgccccataaagggggggggggctgagggggggagaggagggagaagggcgggagcacgttgggggtgggggggcagataagcttttttctttttttaagatgctgacagttatttttagagttttgtgttccctcttccctccccgctggagtgaattgaagaggaaataaatggtgaaggtgctgctggcccattggagcaagggcaattagagcccaaggagtggggcatggagggagacagccccagggctccaggagacagccttctcgcccctccagtttccctgtgccctcgaattctgcttttcagcgaagaaaaggagcagagaggatgatgctgcatttttaacacaccacacagcatgcaagggatttcctcgcaacaccttcctcgctgtgattccacagaccagtccgctgcagctgagggctgcggagactccatctatccctggtgcgttgggaccgtctggatagcttctttcctctgatggctggagaggaggcatttgccaatagcagtagcctgtgtgcgtgtgcgtgtgcgtgtgtgtgtattgaaagtgaagatctacaggcaatatgaggtttctcataacatgttacattcactttctgtattcttgagattaaaggacagaaagttcctaaagctgatttcagtccccttttccagtgtctccttccacccctcacccatgaggactgtttcaagccatctggttcaggctaattttcccctgtgagtggaattccagaaacagacacttccagacacaccaggtagttttgccttctggctttcggtttggattggcgcatggaggcaacaacagaattggagagtgagaggggatttcttttatttcttctctgctacttctctgccatactgtggttggtagtggctgcatccctctaccgatggccagacttctcact

SEQ ID NO: 10504 - RNA, 21862 nt, Homo sapiens
  source 1..21862: mol_type = other RNA
cctgtgccttttacttctttaagcctgagaagcagcaggctaccaattgctcccatttaaggatgtggctgccatgataatctttcacttgttcagcagtatttctttttctttccattgacaagctaggatacgagcacagtccctgctctgccaaaggaaaccatgtcttttgttaaagtttaagctactgataaatatttaagggagtgcaggggtagatgttaatattacctagcaaagaattcatgggcaaacaactttcaaatgtatcagtaagtttaccttaaaatgacttactagataatgagatacatctaatatatttgcaactgaaacacttgaagctttcaaggtctacctgaactaatttcttccctccctccctcctttccttccttcctttgtcaaatatttattgaatgcctaacatgtgcctggcacccttcagggtactgggcttatagcagtttacagagcagaaaaatatctctgcccccttagagctttcaatttactggggacagacagacaataaacaaatcccatgacaaatatgaaagaagggaggagatttactatattttcatgagattgtcaggaaaggcctctctaatgcatacttatttaatatttaagaagaaaccaaaaagatgtgagggaggaagatctgtggctaactgggggaagaagagcattcagggtggtgggaactgcaatgacaaaagaccaaagggggtgcatggttgatgcagagagaacaaagggggcagtggctggagaagtggtcagagcaggagacaggggaacagactgggtggggcttcccctctttcgtgaatctcccacccaagttaatgtctgtgaagagatggttcttttgtttaggcagataaaatgccttcttcaaggcctatttgaagctgcatttccttcttgaagtattcccctttaatgccaatagttccctatacccagattctcttaactctaaagtatgaatcatgcaatcatttcttgtgctttattgtgagtgactatttcttctgtcagcatctttaaagagattgcaagcaatttaaaggtagaaaacacatcatactttttcttcatcccatatagcacatgatgttaaactcaaggtaatcaagaaagaaatgaaagaaatatataaaactgtcaattaagaaaagacaaagaaatatatgactctaaaaacaaattcaggtattttgagaatatagccatgaaaacaaaaacattaaggtagaactcagtggataagacacatgatctgattttgtttagtaatctacatcattgcttatcccaacttagagcttatacctatacatctgtagatctcttcttcctgtcctacagaaaatgtaatccctcatccatgcagccttctttctttctttacattagcactactgcccattcttcacaatgtctatcttcctttatgattttttttctctgaactcatatcttcaatttcctagagtattgttacctagcagggtcagggctattagtggagcagaaattataaacatttgagagacataggtagagggttaaaaacccactagtctactagtttatttcactcattgcttgggatttatctacttaagcaaagcaattaggttacaaatgaactggcgataaaatactttcataaaaattatttatcctgagataaactctttatgatttttagacttgaaataattttatatacttttaaaaatcagttctgtatctaaggtagtatagtccaactaagaaacagagttgatgtgctccatgctgaggtcgaatgaagaagatagaaagtgcccctggatgcctctctaatcattattttagtggaacatttcaatcgcagtctaattattgagctctcccaatccctccagtgctaaatttcaaacatgttggaacttggcgtgaagaagggcaagattgtttttctccatctgtagatgaattcttctttttacctaaactacttagtcctgatttttctttaggccatccttctaaatatgtcttagtcattgctgtgctaaatagaagaggtggcaacagggtagaaaacgactcattaacactccttgctgatgttctttcataaaactattttttaaaaaaattttatttgtgtctcaattcttgcctgactgtttacttactagtatttatttcttttgggtaaaattatgagtttgggaacctatttacacttacattcactaatttgtttaagtgtattaatttcaaacaaaaagatgtataccctcaaggctgtatctgctgtgtttaatacactaatcaatcattaggcatccttgccttcctatcttaccattttgtccaaaacacatctagtactcattgacatttatgtccaacaaacaaaaaaatcagtatagcaacttctatttattatggaagacatgttaactaagaatcttgaacaatttttagattaatagcaggttaattaggttaatagcaggcaaataaataataactctagttttgccaatgtctcataacaaatgtttcagtgaaagcaaatagttactttcttctttttatgagacattaaagtattccgctgagcaatttgaactgctttgtccctcacacaggactttgtacatcacttggcacattataggttcttaatccatgtttgttggatggattaatgaatgaatgatatggctagttcatcaggtcattttattttcctagttcctaggtaactgtccatatttcctgttatcgaaaaagttcttccaatcagttattctctttgtcgacttttagctgtgacttcctattattgaacataacccagtactctaagtattcgaatttaatacaaaaagaaaatctattggaacatttggtaagagatatttgacttacatattgtgtgtaactctgattggagtttcagcacttctttattgtataggtatgaccaagttggcctttaggaggcctgatggatttttaatgaattatcggttttgccaatcattacttttgttgcattatggctttttttttaatatcttgggtctggcgtatatcatagtttagtagctgtgctgttgggaccaaagatctacttacaaccattttcaacacatactaaattttttttgtaggctgctttcccccttttcccttcattgaagttctccaagaaataaccttcctgaagtcttttattcaagatcaaaatttttcaattattctagaatgctatatcattttcaaaagaatgaaaaataaaatatcaacctgtttatttatttggtttcctggccatttgtcaatttttttcttcatattttactatttatggtctagtttaacttggtttccatttgcttacttctcattccctgaaattgtactgggacagaagggaaaaattagttctgtgttattttaattgaaattcatgctgatgaatcatttttccttaagtattcttttcttctattaggttataaattactcaaatagctagaaatcagcaatattgtttagaaaataagaactgatttccacacagacccattaatactgtttcctttggaattgtaatactcatctgctcttcagtaacaaagacaggcttctctaacatgacattatcaatgtttgcttcctggaacactagttctttaagatgctccatgaacataatgacccatggtcaattatatctgggaaatcaaatactgtctttatgctactggaacattaatttcacacattgagggtaattcaaagaataggcttcattttgccagtgttgaagccattttaatttcaagtagcatttcgtgataatataggaacaaaaagatcttcaaattctctgggcattcattgtacttaactttttacttaagagttggtatttatcaatatgatttttgtgttgtatctgagacttatgtggtcccacatgcaggggcagatcaaaattttgttgagcctgaagtgtatacatttttggagtccccttttaaggaaaagaatgcaaaaatatcatacatttgaaaattttatataaacataagatgtgaacatactgctaaggactgtcctagggcctccaaaagacttatgtaagcaatgggctcagaaatttaagcttcattagctacatgctacacttgcatatcccacatgaaaaatagtactttactattatttggcctaataatataatagtgtttcagcctcattatttctggttcttttctccacctgacacataccctacattcttagggttgtgagatttagcaagtaaaaatgcaatatgcccagttaaatttgaatttcagagaaacaagtatttttagtatagtagattccaaatattgcatgaaacatacttgtactaaaaatttcattcactgattattggaaattcaaacttaactcatgtcctacatgaatctagttctagtatagagtgctagttctagtatacagtggttctagttaaaccagtctataacaggacttctctgaaaatgacacattcttttatactctacgccttggttccatgttcctaaattttcttcatgaaaagactgtccagagcaacttattacaaatagagattactaaggccatcccttcaagagtttaaaaagtcttctagatgagttctaccaacaggtagacttgtcagatatggccttagttcaggtaatttcttttcttcaaactggaatgtctttgcactcttcaactatgcagcctttcaggcctagtggtgagaagctgacctttgtcctcaccttcttccctggacagatttaatccaactattctcagaatgtctgttgctgttcacaaacttagatttcagagattttcaaagtccaagtgtggttcctcagactagtagcattagcatcacctgaaaacttgttagaaatgtaaattttcaggcctcactccagatctattgaatcagaacctctggagatggggatatgcaggctgtgctttgacaagccctccaggtgattttgatacatgcttaagtgggagaatcgctgctctataaatggagcccattatttttgagatatatatatacacacacacacacatatatatatatggctatttcacctactagtttgctttgctaaaatccttgatgggtagtggctgcctctcatttctctttgcatttactctctatgtgtctggcacatagaagatgtttaaaattcttcttgaatgaaagatttggagaataaaggggttaatagataattacattttttttgagtaagctacctggtgaaagccatgacccaaagggcatcgcataaagctacgtggatgatcaagctgctgtgtggccccattgcatggcactgtggctccaagttccaactcttttacattttctcaagttgttatctgcttcctcatcctcacgtattttagttctatgactgtagaagaatacaaagagttcatatggattattttcacaggtcattttaatgctaatgttaaaaccatgtatgtgtgaaatatttgacaggacaattataccataggaaaagttttgaattagagacaggccatccaatgaatgtgtaactatgtgtaaggatatgttgtgaaaattacattttacatatatatccatctttgtccagtgctgacataacattgcaatactacatctttatggtagaataaaagcatgtgccttatacataactttcatagaagatgactgcagagcagatctctgattgtgggaggaacagtgatcttgtttctaagcataaatcacctgaactgctaaattccctgaaatgcaaataaatctcaagaattatttgctaattaaattgatgtttatatatgtagattaatctagatactattgtagtgtctctagctataatacgtgcatgtagataagagttatatatacctgagtatccagtaattttacatggaaaaaagtataaaagattagactgcctatttatgttcctaagatattcgtttcttcctctttgactcatcttttatttactgaatttaattaatgcaatataaaccatttttccccaagttagatatgcagaaaaccaaatcaactgttctgtaaagataaagcaatttcctgaaaatttgtggtaaagctttacaaatgttataaaaatgggccacgctgcatgtcaaaaccacaggaatgtgaagattaaactatacattagagtattgtagtaaatagatcacacagagctaataactagttactgttataccacattaaattcactaatgtgaatattgttgtgttttagacactcaaagttcttgggtgttcaggccatcttacagatataagttttgtgaattgtatttatttcttcctttttatattcagtgccacaactctatttcaggccaatattaccttcattgctgatgaccacaacagcctcctaacttaattctttggttcaggtctctcatctccagtctaacctacacttagaacattgcagattaatacttctaaattttgaatctaataataataataataaaaagtaatctgagtccatcaaatcaaatataaattctgcagcatgatgtttgcaggtccttatatgaaactttctggtttgtacaaattcaactcctgtactggaaatgtaccctcaagctaaattgagttcgttgacccaggaacatattctgtgcttttgttgcatgttatggctttgctcagtctggtcccgtcacatggggtgctcaggccaataatcttacctcatcttaagtgctatcttaatgcaacacactcataccaggtttggctctactagaaatcatctctctaccctctggatatctccttttggactctgtacaagttctggcttatattctagttatagatgtcacagacgcttttgtcttgtgactttttaaaacttcacttaataaaaggctctatcagtatttattggattaaatgtgttgacttggttgtctaagccactgtttttcaaattgagccacacattgaaatcactatgggaactcccagaagtactgaggttgggtctcgctataggatatattgatttaagtagtctggcatgaagtctgggcattgagactttaaacatctctctaggtcattccaaagtacagcaaattttgagaaccactagctttgttactcctagggttatccaaaatgtctcttagagtgtgtttgttgaccatggtctcgtatggccacttggttgttggatttatctccattctacttctgtgaacagatgtcctcctcgtgaaccagttggaaaatggggcctccccaggccaactccaaccttatctataactctaaaaagcataattaggaaatgcttttttcaggtttaaagtttaaaatatattcctccaaacatcttgtaatatgattgctggttttggggagcaccactattataattaaaactttaactattaaaaaggacaagggtaatgtataaatcagttaggtttatgcttaaaaactaagtgcatatgtaccttatgtgatcttcaaagaaagcatcagtgaatcataaggaagtgaatttaaaaaatagttttaagcattttaacaaactcattgtcttaaaatttacatttagaaaaggatagatggggagaaaatctatgcagttatttttcatcacatataatttacatttggacttctctgtacatgcacctttcatactgatttatgatgaaaagatgatatattttaccatagggacatagtacttgtttacaatgttttctttctgggaacaatctataaatcagggacaataatacctattctattaggcaggtattatttgaattgttaattaaaataatattaacagagatagttaattggagtgtattagtttgagctgtttgttctggagagtttgggttcccagcaatccatgtcagtctcttactctcacactttgagggcttttgtgccagaacgtggacggtgttccatcatcaggagaatcaaactcatgctctaaactggctcttgcaaccactacatttcaaagcaagagagattataaatttatgtgatattgctcagttttgggatccttgattttaacagttaaaattcaaaaatagagactgtgtatttacattttgtaaaccattcactgcatttaagcccaaggatacatcataaaaagagctttttctttatgatccctctccaaaatccaagtaactccccatatcctggcaatgctttataataccactcacaatgggcgcttcctttttattcccatctgtaacaagtctcttctgggttgctatcatctcatctgttatagccttcatcctggacaacctgctttcctgcccttgtatatttcactttttctccctgactgttgagcccatcctccatctctatctattagaatcttacccacacttcaatgtggatcagttcataattccttccttactttccttgaatactccagctgcaaatttcctcaacagatcatgcatacctcaaagtcaggaactatgaatagtttagtggtattttcttctgagcctagcacagagaccaatataggtgctcctaaatatgaggtaagtaaataggtacaatcacaagccatctaggggtacttcagaaacccatctacatcaaatcttgatcctaaaatgggactgaatttctagttctatctttttaaagagtaacaaactttttggagacttagatatgtcagggtttttctgaaactttccaatgtgttcctttgtttttaaagcctaactaagctaatgaacagaaactaaataaaaaaaaggtttcagttcagttgtttagtcccttcttcaacagttttagatccgttttaaaattttttctcactttacctttttttttaaaaaaacacccttgtccttaatttttctttatgttggatcacattctcccttattttactatcaagatgtgtatagctctaggttgtagcatttcaacttataggaaaggacagttattaccaacaaacttgaaattcttcctttatatggggccttattattgtgtaactggctatataggaaaattcaagaaaatgaaacaaaacaacaacaaaagcttctgaatatgggctctcaaagattgaaattattaaataacctccttttcattaggtcatgagcaggcaactgataagctggagaagtcttttatatttttcttcactgaatggataattactgaacgtctgcaaagcagacattgtgtgcttcatagtttggcatgtcagttgccatttttaaaataaaatcagtggagaatttcaacttgaagcacatataaatgacaataaatagtacttttgcaaactttatttagtatttgcaaataggttccaaatgtccagcttaatttttctgagttcttatttcattcctttctagccatgcttatttttatgtaaaggagaaaacatgcttaattactctaaagaaaagttattttagaaatgataaaagttgaacatatttaaaggaaaaaagcagaataaaattaataattaaaatactaaatttggacaggaaaatggctattgaataagtccaaacatttccaggaaagacataaaggcatccttgtttttaagaaaacatacggcaaactatataaaatgaaatattactaagacttctttggtctcctcatcatacgtcaataatgaggagagctttgcaatgataaagcttttgaagtggcttgtggaatattaaattgtttaagtataattttggcatcaagtgaccttacatattttgaatgttggttatctatgcgttatgtataatgccaccacattattcatcaaaatacagtggacttggatattgaaatatttaacatgattggttttagtgacttagaagtggtgctgatagcccctgaacaattatgccccagcttgaaactgtatagcgtgcagccaaagggatgtgctttgtgattaatctctgggtactactgaggagccgctggctcactcattgtctccatcttctgcagctctcatatggtgagaaaaatgttggttcaagtatttttatagttaatattactacaataatgcaatgtaatgcagtgataaattttaggtagaatttatttgacccgattataaattgctgtagatttgaaggtaacataattattaaggggtgttaaagtgctatctgaatcttttagtaatgctttagtaatttatgtgttttagagacatttgtgaacttagggattcataaaaatatctctcaggaatgccaagacattttgtatttgcttcagaatgctttatcttaaccacggagagataattgatatatatcatcacagtattattttaatgtatgtattcttgaatgtttaaaggataaaaaattacattataagttttagaacttgtgattcaataaaatactaaaaaaacatagattatgttattttacattgtgatgttataagatgttttgtttaggaagtttaattcttagcctagaattaaaaggtagcatgctcgaagttctcactgaggttagaggaataagttgcatattataatattctgtggggcatttaatactaacaataaagaatgaagaaaaatctggcgaatttaagaataacctagcttttacagcatttgtgattgtgattttaaaagacctcatatttgaccctaagaactatagaatatacacctgtataatttatcactactttaatatataaattatttctattattatgactaatggaactagatttcttttgttgttaaaataaaaagttgagatagccagaaatgctgtttaactttgcctagtggcactgtagtaaatatgattttgatgacttttttttccaagtagctaagatttaattgttatttttcttaagatttgtacctgtaagctttagataatagatttgtcatgcagataaattatgagcaatttaactaaaattattgtatttcagtgtgtccaaaacatgaaaataatgatgaaccgaacaaggaaatatttggaacataatttcccttgactgaggtatgagattcatttaattattaaatgtgtgtttacacatgcaaatctatgggaaataatttgttctttatttgtttctattatagttaagaaaaacctgttttgcaaaatgttttttcactgatcaacatagaggtaaattttgataatggaccaaattcaggtgaattggaaactttggaaactttggaaggacttttggtttgggttcttagtaagatcaaaaataggtacttttagaatattttcttctttgtgagatctaaaatggctacacagcagtcttctatttcacaggagatatttttggatggaaatacaacttgggtaatgtttttttgatttgacatttttgttcacaattcgtttttaagctttcctcagtaaggtagctttagttgtagagcccaaggtacagaactacagagcagaaacctaaaatggctttgtttgtactattttgggagtgataaatgaggctgttttcatgaatgggatgaacctatatgtaatagagtattttagaaggaatattgttatgggtaaagacatctggaattgatggtttgccatgaggtttgtagtgttaatacatcaaagtttcataatttcatacatttagtcacccttctttgctgtagaaactggtattttgtctagctaggattaagaacaagtgggttttgttttaggaaagaaaataaaaatgctcaacttttactctcatttctacaatttgtctatgcatgggtgaagactgtttctccctaggagttttcttttcactgatgctaatgtttccgtaagtgacttgtgttttaaaaaccccgatttagcagaaaataatagcaatgccttccagaggaaaagaaaacttaagtaaaatgccaaataatggtaactttgtctctttctatttgcctagaataaacaaacaaacacccgaacagattttttcctccaagaaaagtgataagtgaaatgcacttggaatttttctgaagttattcacagattatttgtgcatcttactgggtagactgctgcctctaatcaaagtcagattactctctttctgagtcaatttttgagctctgggatatctgtagggagacaactaacaactgccttgaaagatttcatattaatgaatattatgttaaccagaatgtataagtgggactgcatataggagtgctcattttacattttgccttgtctaatttgataaagtgaatgagcatcaaggaaaggtgataaataatattgctttgtggctttaatatattgccatttaatcaaagattgcatgccattttgtctttaaatacccttatgaggtagcttggagagatctctgcccttttcaatctgtgacagatttcctagttcagagcaaaaaagtctactgctgaaaaatatgcataattaacaggaaagtataataaagttgttgcttaaactactaaaactttgggatatttgcattgactagtttaaggtctagtttatcagtttgtagcacatttatgtttgtgaagaaaagatgccagaattcccttattctacttgaaaatagatgctacagactgtaccaggagatgcaagaatatgacggcttattcttttttttttttccccagctctatcagtgttgctaccaacaaccagtgaattcatcagataaaatgatagaaggtgtttccgtgtccagggagagattctagtaaccatattacattagataatttaaatgctccccataacatactgtagactgccgctactgagaatataagttaaatttatatagcactgaaaagttatacatttttattaaacaccagtaatctttcgtccatgagagtgtttcctagttattcctaggaaattcttcaatgcagtcttccaaagcattagaatttttttccccctctggtttgacagagccttgtgggcaatgtgcttactctacaaactgtggcaacagagggaaagaaaaccgtaatgctcctctattagaccatgccattagctgttgggaaaccagagctcagctacaaatggcttctaaaaacctcagctcagataagtgcaatgaaatcatacacagcaggaatcacacaccatcagtggtgattcctactctgttcctaaagtttctttctgatttttaagattttataattaccatgacctgtgagacctttcttaagggaaattttcaactggggaaaaatagtagaagctggctttctataatttaagatagtgcaaaatcagtgatagtttcctttataaatactttattatattaaaaatatctaccttatagaggttttcagtttaaggtacactcccatttaatttttacatctttagagatgcagaagacataaaatgtgatttgtagactaggaagttatactataaatatattcttaaccctatatattgctcttttgagttgttttccgttttataagaaaagcaagtggcttctctatcagcaatagagagtcctcattaagtatgaaaaaaactgattagaaaaagtgttcattatgactcaaagactcacaaaatatagtcaatgagagccactctgggaatgaatgatgcttatgtcggtgcttactttaagcttctttacaaagagtctccctagcttttcactttcactaacaaaagggtctacggctcttcctttgtgcttggaaattcaggagcacctcccactgcaaagattaggttatgaatctaacaaatgagaacccagtcttcaagtgcaatgtatttgcctatgatcaagtttgctagcagttgagaatctatagttttgcaacaccacgtgattctctctgctgtattctaaatcacagaatatgtggtattattccacttgttctatcacacctacttacagacatcttgatttctgagatgtgggctcatctctcaatatccttccagtgtcatttcaaatgttgcctgatctaactccacaacacttcaaacacagaacaccacctcttgtgctcctaagttaaacgtgatggtggattaatcttggtcctttagttgataaatcaaggtaatttactgctgctatacccatacacagtccctcccctgctggatctcatgcagtgtggctttgttgctttcacttatgattttgctgctttcatttgggtcaatatcattgtagttattttgtagacaaagtagtaaaaaacttgatttttccctatcctatatatctgcagctcactgatttaaaatattagcataaaggtccgcaccacagtgatgatgttcaatttcatattgagattgaagatggggaaatagcaagggcataccaattcagccataaatatgttttgggtcaatgtcataaaattgtcacaaaattttggtaattgagaaaaagctaaaactttttttgtttgttttttgtttgtaaagggaagaaaagtgcttctgaggctcttttggaataagtaacagttttcagattcacttttgcaaagattgccaatatccttcgcagacaccaacaaaccagactgaacagaaagatccctgtagtaggatgccgagcaaatcattgacttctccaatctctaagagacaatatctaaatgtcagtctcatggcattgtattttctgcttcaccataagattagcaaacacaagacataaaattatgtttatttactaaccaatacagaatatactaggccctttgcctggaagccagatttcacttctgagattttccgaagtccattctagaagaggtggttgttactgatacccagggaaggcaattcttaaattgcttacctggggatggaactttctgtggactttaggcccttaagaccaaaagccatgaggcatttatgaataggtgatgtaagaaattttaataaaagttgcaataaccctgaaaatagtgtctttaataacctatgtactattaataacaaagcatgcatagtgccgtgcattcataactatttggtcataaaaatatgtgactgtaattatgatatttacagtcaacttataaaaatacatgtaattctgaatggcaatagttaatccttagctctaaccacaagcctagaaggattagcttattacggggaaatgtgatagataattacaaaatggacaaagcttttactgtcttgaatttaacattcaagaataactataatagcatcataaaacatttgtcatcattattcttctcacctcacaaggtaaaaacctaaattctgtggaaataaatgggaatcaaataggaaagggccacttacatgatacaacaacagaggagaatagttctttcatagaatactcatgcacagccttcaaagaggttcatagtaactgcaagaattcctgggaagacatctaaacatgactttcattaaaaagaattaaggctggtctaaagaatcaaatctctaaggtatgattacctttaaccataaacggtaaaaaatcttttagctgatctctctgtaatttaggtgagtacctctttgaagtttattaacatcaaagagagtggagctcacatggcactttccaattcaaatttaaattctgatggaaggaaataaatccacattccagtttacatacagaaaaagagtagttttttcaaactttataacctcttactttaagggcatatatgtttcaattaaataaaatattacacaaagctaacatatttcccacaaatttcttctcttctaggagttgattggtcatctgctgacaacagataagttcctaatttgaatggcattagtacttcataaatgaacaaaacaatgagtgcaaactggaaaaactagggagaggtgcatacaagctaccaaaaaaggttgggattgggggtgacctgcaagtcatgatctcatatcttaggatgtatcttagtattcaggaaatggaattcttggaaacatctgtttcacagtgaggttgggaggtcagacgatgctctgttagattcttcttaggattaaattacttcctaggactgcattaagacactttaggtggtatattaactcttccagaacaaataattccatttcagtaaattattgctacagttctctaaagagtactacggtgtcctggaaaagataatgttccttccaaaatgccctctagtcactcgaacaatgagaaattcatatttatcttagacactttgatccttgaagacataaactaaaaaagaactgtttttccctatctaaacagagactatctggatggagacataatattagatctgccctggtcatttggcagtgtataccatttcctccatgtgcttttgacaactggcatgcttgattctttccctgtaaatcagcctgccattcttctttgcatgcagaatggtctataggaaccaagaaaaaaccaaccccaatagccaatcttttaaaaaataggtgaatgagtggagcatggcacacaatgggaagaaaaggagtgatagttaattaactttctcagtgattatctcccatattttgatatgggagataaaaatcttccatatcaaatctttacaaatgatgggtaatctgtaagaggaattctcctcctccctgcacccccactacaaaactcccacccaaacaaaaaatcaaaacccaaccaaaaacctcctctgaaacttctacttcagatatgagatcatggtctggaggctactcgtaccaaataccagttcattctagtacagcagttcatgaggcaaaaggctaggagtatttgtgacatgactttacaaataatgtaaaaacaataaccctatgattatgggcaataattttccccactcaaatctatagatattgcactgaaactgacacaatggagaagacatagatcatttcctgttgaaacccaattacctcaaggtaaaacaaaacaaactccatttaataaatgaaatattacttaaatgttttcattttagggtctgttccctttcccctttatattctggaaagttatatgtctaagtatacttgttttgttacttcattagtctatcaacttcatttccagagactataacgagaatggaatggtttgtaccttttttctgaacataattgagtcaaggagttttgttattttaggtattattaatttgattaaaacatagaaccaaagttgatgggaagtagtagctttcttctaggtaaaagagcttactagcagattttataatcatcggacatttattctgtcctacctggaaataaattatgttactgcttggcatgggaaaaggcattttctagtaatttcctgtgacaggaggcacagcaatagtccaagtaagcacccaacaggtgcttgggagtagttttaaactttaacttaatgaaaacatttacctcagtacttttgtttgagaaagaattcagcagcagttatagttaatatcccacctgtggagagctgcgatcaccctaggaggtgggccaaccgaggagcactttccaggtaacaagagcaacactattgtgagaagctacaaatggtactgcagtaggtgtagtgaacactactatagtgatcatggcctgggttatgttccaaatactaatgcaaggaatacactagagtttataggattagaatagtttccttatgctaagaactagtagatggcatgtgatgagtgggtatggtccattttattctatttcactctacgagtttcctagttatgtctcctttctcctatgttaattatctatattccatgacagttattttccctatctaaaataagaacggtgtaactatggagtaccccaactcacatacacatacttgtgcacccttagactcatgtatggataatctgtgtaaagcgctcatttgcaattgggtgagctcactgaaagcagccatatcagtcttccaaatacagtaaaagccaacgaaaatccatatcaactgtttatttctaatatgaaacagtaaaccttgtccatgtggtaattaattcaaatgccttttgtgttttcttgtgaagtcatccaaagcaaaagtctagatgactgctgacatgatatgcataatctaatgaactcacatctctgtttattttgctcatcccacagttgaatgacacactgactgctgagacacttgggttgatttagaacggctattaatgaatctataaatttggctaaggttgatttgactttctagggaaaagccagcctatcttcaaatggacagctccctccacataaacgtcaatgtaccctaaagacaaaactaagtatatgtatatacgggatatatacatatatatgtacacataaaatggattgggaagtcctttggtttagacagtattaaatatgtacttcccaagtgcataggtttcctttgaccaacctgttcaaaaaacaagcatgaaaagtgccatggcacatttcccatgtctttccccctatttgaaggacacctttccttgcttctccatcactcctaagcattttatttttaaaagaagctggttattttggccttctatcttaacactccattgattcatccattccttggaagagctctcagattacatccagaaacttgtttttagaggagaacaaggttgcaaataactttttcctctttttttattccctcttccccccaagaagcaggcaccttgaagtgtcatgaataatgcactcttgatctgacttgccttgttacccctggccagcccaagcagctgaggtctgagctttacttgccctgcatcattgtgcaatactggaaaagaaaaataatccactggtctatacccctcatactgtggtgacgtgatccgggttctcttgaatttctatgcattcaatttcctctctctcctttcgcttggcacgtttctttttcttgtggtgctttttggaaggggggaaaaacgttaggaacacaggtaaaataacaaaacagtgcagaagtgtgcaacccccagtgagcagcaagcatttgaacagtgtgaaggtcaggttcgaaggcacaaatagaagggggactaacccaataagaaaagaagtaacattttgcaaaatggctgtcccatggtcttgcaaggagctttttatacattgtgttcgggtgtgctcagttgctaatacaaatgtgaaaagcagtggtgcacagtggtcaatggcgaaattcaaggtgtagataaggcacaagatagaaatgcaatccatgtcgacgttccataatgtcattaagcccagaacgcccagctcaattgaggtgacgctaagaattagccagaagtttcccagagggtggatcactaggaaaaaagtcaggattaacaccaggagaacaccaaagcctgcaatcagaacaggcactgtgacagacaagctgtaatggtccatgaagacaaaggaggggttgaacacgatgaatcggatgctctttgagagggataggggcctcagcttttccaacacttctgtgatttctttctgcttgtctctgctagtcctggccaccagatacaagcgagaagcaatgatattgctttcatcccctgccttggagaagatgatatcatttcgaaaatgctggaattctggcttttttaaaaatgagctttgcaggacactgatgaagtcacttttgttattggcactgacgttgctgactttcaggaactggtagtactgctccacccaggacactgcagtgaatccactacagagtcttcttaggtcatcctggacgctgctgttccagtactctaggggctcatagacgtagaatcctatcacagggctatagttgctgaaatatttctgctgaaccatggcataggaaacacttggcgaatcactggctagtagattgatgatgttggctccgtcactgatctgtaagcaccccatgaaggagaaggaggcataaatgagatagaggatgacaacaaatggcttcacatatatattggtaatccattcattataatgttcacggaggaagtgctgaatgaagtggtgctggtaggggttcgtctcatgatgggacgtctgttgatgcccatcactcatcactgtctggaaccacacaggtttgcgatccaggtattctgcagaagggatcttacagcaaaagatgctgtggtagcggttttgctctagttggccagcaaagaccagacaggagccaaagaaggagaaaatgtagaagtagttcaacagaatagagacacacatgttttgacagaagaccttcacagcctctatgtttgtgaatgggctggcacccatgccaaaagtgatgaagtacagggagctggtcatggtataggtgaccatcacatcagaataggcatctgctatcctgtctttgaagggcaagttctctttggttctccgccatccggacagaagctcaaacactcctttagttccatgacccatggcgaagaacgggattcccagcagggtggagttgtactttccatcggtgatgaagaagatccctgctgctgtgatgatggagatgcatactgtgagcacccccaggaggcccaggaagggcttactgcgcaagcagtccttcatggagctggagagggtggctgtggtcaggatcagcacgaggctcaccaggaccttgcttctggccaggatgctggtcttatgaaagtccctccagaggctaaaggatgctaaagagtagagctggagttcttgatgctcctcctggagcttccttataagcttacagaactcattctcccacttctcccctatgaggtcttgggtggcagagccataggtctggaggtagtaggtgatttgaatggctctggctgacttgacccgctgatctttgctgtttggcacttccactaccccgcccagttggtgtccaataaaactgttcctcccatccttcatttccagcacggctcggtgggtctgcaggatcccctcagcctggagcaaaatattgtccccggttggggagaggaggatcaccctgccatacctcccaggggtgtgtaagtccgaatagagctggcttttggactggtccagggggaaaaggctgctggccaggctgcgctcgatcttggccaggctgtggctgggagcgaccaggcgctccaggtcgccctcgggctggaagcggttgagcgcgctgaggccgaaggtgattgtcaggactgcgggcacggtgaggaaaaagaccgggtgccggctcacgcacaaacccagcctgtggcagaacgactggagccctctgcgaagcacctgccgcagcatcctccaccagatccagctcgcaggcgctcccggccgtcttaaaaagcacatgtgacatgtgtaagcgccgggctaccccgttctcccccatcccaccccctggggccagtcccccctccccaccgccgccgcctccccacccactccgcgctcaccccacaaccactccgcctggtctttccccggccccacctccatgcgctcctactactctttcaaacactgc

SEQ ID NO: 10505 - RNA, 21330 nt, Homo sapiens
  source 1..21330: mol_type = other RNA
cctgtgccttttacttctttaagcctgagaagcagcaggctaccaattgctcccatttaaggatgtggctgccatgataatctttcacttgttcagcagtatttctttttctttccattgacaagctaggatacgagcacagtccctgctctgccaaaggaaaccatgtcttttgttaaagtttaagctactgataaatatttaagggagtgcaggggtagatgttaatattacctagcaaagaattcatgggcaaacaactttcaaatgtatcagtaagtttaccttaaaatgacttactagataatgagatacatctaatatatttgcaactgaaacacttgaagctttcaaggtctacctgaactaatttcttccctccctccctcctttccttccttcctttgtcaaatatttattgaatgcctaacatgtgcctggcacccttcagggtactgggcttatagcagtttacagagcagaaaaatatctctgcccccttagagctttcaatttactggggacagacagacaataaacaaatcccatgacaaatatgaaagaagggaggagatttactatattttcatgagattgtcaggaaaggcctctctaatgcatacttatttaatatttaagaagaaaccaaaaagatgtgagggaggaagatctgtggctaactgggggaagaagagcattcagggtggtgggaactgcaatgacaaaagaccaaagggggtgcatggttgatgcagagagaacaaagggggcagtggctggagaagtggtcagagcaggagacaggggaacagactgggtggggcttcccctctttcgtgaatctcccacccaagttaatgtctgtgaagagatggttcttttgtttaggcagataaaatgccttcttcaaggcctatttgaagctgcatttccttcttgaagtattcccctttaatgccaatagttccctatacccagattctcttaactctaaagtatgaatcatgcaatcatttcttgtgctttattgtgagtgactatttcttctgtcagcatctttaaagagattgcaagcaatttaaaggtagaaaacacatcatactttttcttcatcccatatagcacatgatgttaaactcaaggtaatcaagaaagaaatgaaagaaatatataaaactgtcaattaagaaaagacaaagaaatatatgactctaaaaacaaattcaggtattttgagaatatagccatgaaaacaaaaacattaaggtagaactcagtggataagacacatgatctgattttgtttagtaatctacatcattgcttatcccaacttagagcttatacctatacatctgtagatctcttcttcctgtcctacagaaaatgtaatccctcatccatgcagccttctttctttctttacattagcactactgcccattcttcacaatgtctatcttcctttatgattttttttctctgaactcatatcttcaatttcctagagtattgttacctagcagggtcagggctattagtggagcagaaattataaacatttgagagacataggtagagggttaaaaacccactagtctactagtttatttcactcattgcttgggatttatctacttaagcaaagcaattaggttacaaatgaactggcgataaaatactttcataaaaattatttatcctgagataaactctttatgatttttagacttgaaataattttatatacttttaaaaatcagttctgtatctaaggtagtatagtccaactaagaaacagagttgatgtgctccatgctgaggtcgaatgaagaagatagaaagtgcccctggatgcctctctaatcattattttagtggaacatttcaatcgcagtctaattattgagctctcccaatccctccagtgctaaatttcaaacatgttggaacttggcgtgaagaagggcaagattgtttttctccatctgtagatgaattcttctttttacctaaactacttagtcctgatttttctttaggccatccttctaaatatgtcttagtcattgctgtgctaaatagaagaggtggcaacagggtagaaaacgactcattaacactccttgctgatgttctttcataaaactattttttaaaaaaattttatttgtgtctcaattcttgcctgactgtttacttactagtatttatttcttttgggtaaaattatgagtttgggaacctatttacacttacattcactaatttgtttaagtgtattaatttcaaacaaaaagatgtataccctcaaggctgtatctgctgtgtttaatacactaatcaatcattaggcatccttgccttcctatcttaccattttgtccaaaacacatctagtactcattgacatttatgtccaacaaacaaaaaaatcagtatagcaacttctatttattatggaagacatgttaactaagaatcttgaacaatttttagattaatagcaggttaattaggttaatagcaggcaaataaataataactctagttttgccaatgtctcataacaaatgtttcagtgaaagcaaatagttactttcttctttttatgagacattaaagtattccgctgagcaatttgaactgctttgtccctcacacaggactttgtacatcacttggcacattataggttcttaatccatgtttgttggatggattaatgaatgaatgatatggctagttcatcaggtcattttattttcctagttcctaggtaactgtccatatttcctgttatcgaaaaagttcttccaatcagttattctctttgtcgacttttagctgtgacttcctattattgaacataacccagtactctaagtattcgaatttaatacaaaaagaaaatctattggaacatttggtaagagatatttgacttacatattgtgtgtaactctgattggagtttcagcacttctttattgtataggtatgaccaagttggcctttaggaggcctgatggatttttaatgaattatcggttttgccaatcattacttttgttgcattatggctttttttttaatatcttgggtctggcgtatatcatagtttagtagctgtgctgttgggaccaaagatctacttacaaccattttcaacacatactaaattttttttgtaggctgctttcccccttttcccttcattgaagttctccaagaaataaccttcctgaagtcttttattcaagatcaaaatttttcaattattctagaatgctatatcattttcaaaagaatgaaaaataaaatatcaacctgtttatttatttggtttcctggccatttgtcaatttttttcttcatattttactatttatggtctagtttaacttggtttccatttgcttacttctcattccctgaaattgtactgggacagaagggaaaaattagttctgtgttattttaattgaaattcatgctgatgaatcatttttccttaagtattcttttcttctattaggttataaattactcaaatagctagaaatcagcaatattgtttagaaaataagaactgatttccacacagacccattaatactgtttcctttggaattgtaatactcatctgctcttcagtaacaaagacaggcttctctaacatgacattatcaatgtttgcttcctggaacactagttctttaagatgctccatgaacataatgacccatggtcaattatatctgggaaatcaaatactgtctttatgctactggaacattaatttcacacattgagggtaattcaaagaataggcttcattttgccagtgttgaagccattttaatttcaagtagcatttcgtgataatataggaacaaaaagatcttcaaattctctgggcattcattgtacttaactttttacttaagagttggtatttatcaatatgatttttgtgttgtatctgagacttatgtggtcccacatgcaggggcagatcaaaattttgttgagcctgaagtgtatacatttttggagtccccttttaaggaaaagaatgcaaaaatatcatacatttgaaaattttatataaacataagatgtgaacatactgctaaggactgtcctagggcctccaaaagacttatgtaagcaatgggctcagaaatttaagcttcattagctacatgctacacttgcatatcccacatgaaaaatagtactttactattatttggcctaataatataatagtgtttcagcctcattatttctggttcttttctccacctgacacataccctacattcttagggttgtgagatttagcaagtaaaaatgcaatatgcccagttaaatttgaatttcagagaaacaagtatttttagtatagtagattccaaatattgcatgaaacatacttgtactaaaaatttcattcactgattattggaaattcaaacttaactcatgtcctacatgaatctagttctagtatagagtgctagttctagtatacagtggttctagttaaaccagtctataacaggacttctctgaaaatgacacattcttttatactctacgccttggttccatgttcctaaattttcttcatgaaaagactgtccagagcaacttattacaaatagagattactaaggccatcccttcaagagtttaaaaagtcttctagatgagttctaccaacaggtagacttgtcagatatggccttagttcaggtaatttcttttcttcaaactggaatgtctttgcactcttcaactatgcagcctttcaggcctagtggtgagaagctgacctttgtcctcaccttcttccctggacagatttaatccaactattctcagaatgtctgttgctgttcacaaacttagatttcagagattttcaaagtccaagtgtggttcctcagactagtagcattagcatcacctgaaaacttgttagaaatgtaaattttcaggcctcactccagatctattgaatcagaacctctggagatggggatatgcaggctgtgctttgacaagccctccaggtgattttgatacatgcttaagtgggagaatcgctgctctataaatggagcccattatttttgagatatatatatacacacacacacacatatatatatatggctatttcacctactagtttgctttgctaaaatccttgatgggtagtggctgcctctcatttctctttgcatttactctctatgtgtctggcacatagaagatgtttaaaattcttcttgaatgaaagatttggagaataaaggggttaatagataattacattttttttgagtaagctacctggtgaaagccatgacccaaagggcatcgcataaagctacgtggatgatcaagctgctgtgtggccccattgcatggcactgtggctccaagttccaactcttttacattttctcaagttgttatctgcttcctcatcctcacgtattttagttctatgactgtagaagaatacaaagagttcatatggattattttcacaggtcattttaatgctaatgttaaaaccatgtatgtgtgaaatatttgacaggacaattataccataggaaaagttttgaattagagacaggccatccaatgaatgtgtaactatgtgtaaggatatgttgtgaaaattacattttacatatatatccatctttgtccagtgctgacataacattgcaatactacatctttatggtagaataaaagcatgtgccttatacataactttcatagaagatgactgcagagcagatctctgattgtgggaggaacagtgatcttgtttctaagcataaatcacctgaactgctaaattccctgaaatgcaaataaatctcaagaattatttgctaattaaattgatgtttatatatgtagattaatctagatactattgtagtgtctctagctataatacgtgcatgtagataagagttatatatacctgagtatccagtaattttacatggaaaaaagtataaaagattagactgcctatttatgttcctaagatattcgtttcttcctctttgactcatcttttatttactgaatttaattaatgcaatataaaccatttttccccaagttagatatgcagaaaaccaaatcaactgttctgtaaagataaagcaatttcctgaaaatttgtggtaaagctttacaaatgttataaaaatgggccacgctgcatgtcaaaaccacaggaatgtgaagattaaactatacattagagtattgtagtaaatagatcacacagagctaataactagttactgttataccacattaaattcactaatgtgaatattgttgtgttttagacactcaaagttcttgggtgttcaggccatcttacagatataagttttgtgaattgtatttatttcttcctttttatattcagtgccacaactctatttcaggccaatattaccttcattgctgatgaccacaacagcctcctaacttaattctttggttcaggtctctcatctccagtctaacctacacttagaacattgcagattaatacttctaaattttgaatctaataataataataataaaaagtaatctgagtccatcaaatcaaatataaattctgcagcatgatgtttgcaggtccttatatgaaactttctggtttgtacaaattcaactcctgtactggaaatgtaccctcaagctaaattgagttcgttgacccaggaacatattctgtgcttttgttgcatgttatggctttgctcagtctggtcccgtcacatggggtgctcaggccaataatcttacctcatcttaagtgctatcttaatgcaacacactcataccaggtttggctctactagaaatcatctctctaccctctggatatctccttttggactctgtacaagttctggcttatattctagttatagatgtcacagacgcttttgtcttgtgactttttaaaacttcacttaataaaaggctctatcagtatttattggattaaatgtgttgacttggttgtctaagccactgtttttcaaattgagccacacattgaaatcactatgggaactcccagaagtactgaggttgggtctcgctataggatatattgatttaagtagtctggcatgaagtctgggcattgagactttaaacatctctctaggtcattccaaagtacagcaaattttgagaaccactagctttgttactcctagggttatccaaaatgtctcttagagtgtgtttgttgaccatggtctcgtatggccacttggttgttggatttatctccattctacttctgtgaacagatgtcctcctcgtgaaccagttggaaaatggggcctccccaggccaactccaaccttatctataactctaaaaagcataattaggaaatgcttttttcaggtttaaagtttaaaatatattcctccaaacatcttgtaatatgattgctggttttggggagcaccactattataattaaaactttaactattaaaaaggacaagggtaatgtataaatcagttaggtttatgcttaaaaactaagtgcatatgtaccttatgtgatcttcaaagaaagcatcagtgaatcataaggaagtgaatttaaaaaatagttttaagcattttaacaaactcattgtcttaaaatttacatttagaaaaggatagatggggagaaaatctatgcagttatttttcatcacatataatttacatttggacttctctgtacatgcacctttcatactgatttatgatgaaaagatgatatattttaccatagggacatagtacttgtttacaatgttttctttctgggaacaatctataaatcagggacaataatacctattctattaggcaggtattatttgaattgttaattaaaataatattaacagagatagttaattggagtgtattagtttgagctgtttgttctggagagtttgggttcccagcaatccatgtcagtctcttactctcacactttgagggcttttgtgccagaacgtggacggtgttccatcatcaggagaatcaaactcatgctctaaactggctcttgcaaccactacatttcaaagcaagagagattataaatttatgtgatattgctcagttttgggatccttgattttaacagttaaaattcaaaaatagagactgtgtatttacattttgtaaaccattcactgcatttaagcccaaggatacatcataaaaagagctttttctttatgatccctctccaaaatccaagtaactccccatatcctggcaatgctttataataccactcacaatgggcgcttcctttttattcccatctgtaacaagtctcttctgggttgctatcatctcatctgttatagccttcatcctggacaacctgctttcctgcccttgtatatttcactttttctccctgactgttgagcccatcctccatctctatctattagaatcttacccacacttcaatgtggatcagttcataattccttccttactttccttgaatactccagctgcaaatttcctcaacagatcatgcatacctcaaagtcaggaactatgaatagtttagtggtattttcttctgagcctagcacagagaccaatataggtgctcctaaatatgaggtaagtaaataggtacaatcacaagccatctaggggtacttcagaaacccatctacatcaaatcttgatcctaaaatgggactgaatttctagttctatctttttaaagagtaacaaactttttggagacttagatatgtcagggtttttctgaaactttccaatgtgttcctttgtttttaaagcctaactaagctaatgaacagaaactaaataaaaaaaaggtttcagttcagttgtttagtcccttcttcaacagttttagatccgttttaaaattttttctcactttacctttttttttaaaaaaacacccttgtccttaatttttctttatgttggatcacattctcccttattttactatcaagatgtgtatagctctaggttgtagcatttcaacttataggaaaggacagttattaccaacaaacttgaaattcttcctttatatggggccttattattgtgtaactggctatataggaaaattcaagaaaatgaaacaaaacaacaacaaaagcttctgaatatgggctctcaaagattgaaattattaaataacctccttttcattaggtcatgagcaggcaactgataagctggagaagtcttttatatttttcttcactgaatggataattactgaacgtctgcaaagcagacattgtgtgcttcatagtttggcatgtcagttgccatttttaaaataaaatcagtggagaatttcaacttgaagcacatataaatgacaataaatagtacttttgcaaactttatttagtatttgcaaataggttccaaatgtccagcttaatttttctgagttcttatttcattcctttctagccatgcttatttttatgtaaaggagaaaacatgcttaattactctaaagaaaagttattttagaaatgataaaagttgaacatatttaaaggaaaaaagcagaataaaattaataattaaaatactaaatttggacaggaaaatggctattgaataagtccaaacatttccaggaaagacataaaggcatccttgtttttaagaaaacatacggcaaactatataaaatgaaatattactaagacttctttggtctcctcatcatacgtcaataatgaggagagctttgcaatgataaagcttttgaagtggcttgtggaatattaaattgtttaagtataattttggcatcaagtgaccttacatattttgaatgttggttatctatgcgttatgtataatgccaccacattattcatcaaaatacagtggacttggatattgaaatatttaacatgattggttttagtgacttagaagtggtgctgatagcccctgaacaattatgccccagcttgaaactgtatagcgtgcagccaaagggatgtgctttgtgattaatctctgggtactactgaggagccgctggctcactcattgtctccatcttctgcagctctcatatggtgagaaaaatgttggttcaagtatttttatagttaatattactacaataatgcaatgtaatgcagtgataaattttaggtagaatttatttgacccgattataaattgctgtagatttgaaggtaacataattattaaggggtgttaaagtgctatctgaatcttttagtaatgctttagtaatttatgtgttttagagacatttgtgaacttagggattcataaaaatatctctcaggaatgccaagacattttgtatttgcttcagaatgctttatcttaaccacggagagataattgatatatatcatcacagtattattttaatgtatgtattcttgaatgtttaaaggataaaaaattacattataagttttagaacttgtgattcaataaaatactaaaaaaacatagattatgttattttacattgtgatgttataagatgttttgtttaggaagtttaattcttagcctagaattaaaaggtagcatgctcgaagttctcactgaggttagaggaataagttgcatattataatattctgtggggcatttaatactaacaataaagaatgaagaaaaatctggcgaatttaagaataacctagcttttacagcatttgtgattgtgattttaaaagacctcatatttgaccctaagaactatagaatatacacctgtataatttatcactactttaatatataaattatttctattattatgactaatggaactagatttcttttgttgttaaaataaaaagttgagatagccagaaatgctgtttaactttgcctagtggcactgtagtaaatatgattttgatgacttttttttccaagtagctaagatttaattgttatttttcttaagatttgtacctgtaagctttagataatagatttgtcatgcagataaattatgagcaatttaactaaaattattgtatttcagtgtgtccaaaacatgaaaataatgatgaaccgaacaaggaaatatttggaacataatttcccttgactgaggtatgagattcatttaattattaaatgtgtgtttacacatgcaaatctatgggaaataatttgttctttatttgtttctattatagttaagaaaaacctgttttgcaaaatgttttttcactgatcaacatagaggtaaattttgataatggaccaaattcaggtgaattggaaactttggaaactttggaaggacttttggtttgggttcttagtaagatcaaaaataggtacttttagaatattttcttctttgtgagatctaaaatggctacacagcagtcttctatttcacaggagatatttttggatggaaatacaacttgggtaatgtttttttgatttgacatttttgttcacaattcgtttttaagctttcctcagtaaggtagctttagttgtagagcccaaggtacagaactacagagcagaaacctaaaatggctttgtttgtactattttgggagtgataaatgaggctgttttcatgaatgggatgaacctatatgtaatagagtattttagaaggaatattgttatgggtaaagacatctggaattgatggtttgccatgaggtttgtagtgttaatacatcaaagtttcataatttcatacatttagtcacccttctttgctgtagaaactggtattttgtctagctaggattaagaacaagtgggttttgttttaggaaagaaaataaaaatgctcaacttttactctcatttctacaatttgtctatgcatgggtgaagactgtttctccctaggagttttcttttcactgatgctaatgtttccgtaagtgacttgtgttttaaaaaccccgatttagcagaaaataatagcaatgccttccagaggaaaagaaaacttaagtaaaatgccaaataatggtaactttgtctctttctatttgcctagaataaacaaacaaacacccgaacagattttttcctccaagaaaagtgataagtgaaatgcacttggaatttttctgaagttattcacagattatttgtgcatcttactgggtagactgctgcctctaatcaaagtcagattactctctttctgagtcaatttttgagctctgggatatctgtagggagacaactaacaactgccttgaaagatttcatattaatgaatattatgttaaccagaatgtataagtgggactgcatataggagtgctcattttacattttgccttgtctaatttgataaagtgaatgagcatcaaggaaaggtgataaataatattgctttgtggctttaatatattgccatttaatcaaagattgcatgccattttgtctttaaatacccttatgaggtagcttggagagatctctgcccttttcaatctgtgacagatttcctagttcagagcaaaaaagtctactgctgaaaaatatgcataattaacaggaaagtataataaagttgttgcttaaactactaaaactttgggatatttgcattgactagtttaaggtctagtttatcagtttgtagcacatttatgtttgtgaagaaaagatgccagaattcccttattctacttgaaaatagatgctacagactgtaccaggagatgcaagaatatgacggcttattcttttttttttttccccagctctatcagtgttgctaccaacaaccagtgaattcatcagataaaatgatagaaggtgtttccgtgtccagggagagattctagtaaccatattacattagataatttaaatgctccccataacatactgtagactgccgctactgagaatataagttaaatttatatagcactgaaaagttatacatttttattaaacaccagtaatctttcgtccatgagagtgtttcctagttattcctaggaaattcttcaatgcagtcttccaaagcattagaatttttttccccctctggtttgacagagccttgtgggcaatgtgcttactctacaaactgtggcaacagagggaaagaaaaccgtaatgctcctctattagaccatgccattagctgttgggaaaccagagctcagctacaaatggcttctaaaaacctcagctcagataagtgcaatgaaatcatacacagcaggaatcacacaccatcagtggtgattcctactctgttcctaaagtttctttctgatttttaagattttataattaccatgacctgtgagacctttcttaagggaaattttcaactggggaaaaatagtagaagctggctttctataatttaagatagtgcaaaatcagtgatagtttcctttataaatactttattatattaaaaatatctaccttatagaggttttcagtttaaggtacactcccatttaatttttacatctttagagatgcagaagacataaaatgtgatttgtagactaggaagttatactataaatatattcttaaccctatatattgctcttttgagttgttttccgttttataagaaaagcaagtggcttctctatcagcaatagagagtcctcattaagtatgaaaaaaactgattagaaaaagtgttcattatgactcaaagactcacaaaatatagtcaatgagagccactctgggaatgaatgatgcttatgtcggtgcttactttaagcttctttacaaagagtctccctagcttttcactttcactaacaaaagggtctacggctcttcctttgtgcttggaaattcaggagcacctcccactgcaaagattaggttatgaatctaacaaatgagaacccagtcttcaagtgcaatgtatttgcctatgatcaagtttgctagcagttgagaatctatagttttgcaacaccacgtgattctctctgctgtattctaaatcacagaatatgtggtattattccacttgttctatcacacctacttacagacatcttgatttctgagatgtgggctcatctctcaatatccttccagtgtcatttcaaatgttgcctgatctaactccacaacacttcaaacacagaacaccacctcttgtgctcctaagttaaacgtgatggtggattaatcttggtcctttagttgataaatcaaggtaatttactgctgctatacccatacacagtccctcccctgctggatctcatgcagtgtggctttgttgctttcacttatgattttgctgctttcatttgggtcaatatcattgtagttattttgtagacaaagtagtaaaaaacttgatttttccctatcctatatatctgcagctcactgatttaaaatattagcataaaggtccgcaccacagtgatgatgttcaatttcatattgagattgaagatggggaaatagcaagggcataccaattcagccataaatatgttttgggtcaatgtcataaaattgtcacaaaattttggtaattgagaaaaagctaaaactttttttgtttgttttttgtttgtaaagggaagaaaagtgcttctgaggctcttttggaataagtaacagttttcagattcacttttgcaaagattgccaatatccttcgcagacaccaacaaaccagactgaacagaaagatccctgtagtaggatgccgagcaaatcattgacttctccaatctctaagagacaatatctaaatgtcagtctcatggcattgtattttctgcttcaccataagattagcaaacacaagacataaaattatgtttatttactaaccaatacagaatatactaggccctttgcctggaagccagatttcacttctgagattttccgaagtccattctagaagaggtggttgttactgatacccagggaaggcaattcttaaattgcttacctggggatggaactttctgtggactttaggcccttaagaccaaaagccatgaggcatttatgaataggtgatgtaagaaattttaataaaagttgcaataaccctgaaaatagtgtctttaataacctatgtactattaataacaaagcatgcatagtgccgtgcattcataactatttggtcataaaaatatgtgactgtaattatgatatttacagtcaacttataaaaatacatgtaattctgaatggcaatagttaatccttagctctaaccacaagcctagaaggattagcttattacggggaaatgtgatagataattacaaaatggacaaagcttttactgtcttgaatttaacattcaagaataactataatagcatcataaaacatttgtcatcattattcttctcacctcacaaggtaaaaacctaaattctgtggaaataaatgggaatcaaataggaaagggccacttacatgatacaacaacagaggagaatagttctttcatagaatactcatgcacagccttcaaagaggttcatagtaactgcaagaattcctgggaagacatctaaacatgactttcattaaaaagaattaaggctggtctaaagaatcaaatctctaaggtatgattacctttaaccataaacggtaaaaaatcttttagctgatctctctgtaatttaggtgagtacctctttgaagtttattaacatcaaagagagtggagctcacatggcactttccaattcaaatttaaattctgatggaaggaaataaatccacattccagtttacatacagaaaaagagtagttttttcaaactttataacctcttactttaagggcatatatgtttcaattaaataaaatattacacaaagctaacatatttcccacaaatttcttctcttctaggagttgattggtcatctgctgacaacagataagttcctaatttgaatggcattagtacttcataaatgaacaaaacaatgagtgcaaactggaaaaactagggagaggtgcatacaagctaccaaaaaaggttgggattgggggtgacctgcaagtcatgatctcatatcttaggatgtatcttagtattcaggaaatggaattcttggaaacatctgtttcacagtgaggttgggaggtcagacgatgctctgttagattcttcttaggattaaattacttcctaggactgcattaagacactttaggtggtatattaactcttccagaacaaataattccatttcagtaaattattgctacagttctctaaagagtactacggtgtcctggaaaagataatgttccttccaaaatgccctctagtcactcgaacaatgagaaattcatatttatcttagacactttgatccttgaagacataaactaaaaaagaactgtttttccctatctaaacagagactatctggatggagacataatattagatctgccctggtcatttggcagtgtataccatttcctccatgtgcttttgacaactggcatgcttgattctttccctgtaaatcagcctgccattcttctttgcatgcagaatggtctataggaaccaagaaaaaaccaaccccaatagccaatcttttaaaaaataggtgaatgagtggagcatggcacacaatgggaagaaaaggagtgatagttaattaactttctcagtgattatctcccatattttgatatgggagataaaaatcttccatatcaaatctttacaaatgatgggtaatctgtaagaggaattctcctcctccctgcacccccactacaaaactcccacccaaacaaaaaatcaaaacccaaccaaaaacctcctctgaaacttctacttcagatatgagatcatggtctggaggctactcgtaccaaataccagttcattctagtacagcagttcatgaggcaaaaggctaggagtatttgtgacatgactttacaaataatgtaaaaacaataaccctatgattatgggcaataattttccccactcaaatctatagatattgcactgaaactgacacaatggagaagacatagatcatttcctgttgaaacccaattacctcaaggtaaaacaaaacaaactccatttaataaatgaaatattacttaaatgttttcattttagggtctgttccctttcccctttatattctggaaagttatatgtctaagtatacttgttttgttacttcattagtctatcaacttcatttccagagactataacgagaatggaatggtttgtaccttttttctgaacataattgagtcaaggagttttgttattttaggtattattaatttgattaaaacatagaaccaaagttgatgggaagtagtagctttcttctaggtaaaagagcttactagcagattttataatcatcggacatttattctgtcctacctggaaataaattatgttactgcttggcatgggaaaaggcattttctagtaatttcctgtgacaggaggcacagcaatagtccaagtaagcacccaacaggtgcttgggagtagttttaaactttaacttaatgaaaacatttacctcagtacttttgtttgagaaagaattcagcagcagttatagttaatatcccacctgtggagagctgcgatcaccctaggaggtgggccaaccgaggagcactttccaggtaacaagagcaacactattgtgagaagctacaaatggtactgcagtaggtgtagtgaacactactatagtgatcatggcctgggttatgttccaaatactaatgcaaggaatacactagagtttataggattagaatagtttccttatgctaagaactagtagatggcatgtgatgagtgggtatggtccattttattctatttcactctacgagtttcctagttatgtctcctttctcctatgttaattatctatattccatgacagttattttccctatctaaaataagaacggtgtaactatggagtaccccaactcacatacacatacttgtgcacccttagactcatgtatggataatctgtgtaaagcgctcatttgcaattgggtgagctcactgaaagcagccatatcagtcttccaaatacagtaaaagccaacgaaaatccatatcaactgtttatttctaatatgaaacagtaaaccttgtccatgtggtaattaattcaaatgccttttgtgttttcttgtgaagtcatccaaagcaaaagtctagatgactgctgacatgatatgcataatctaatgaactcacatctctgtttattttgctcatcccacagttgaatgacacactgactgctgagacacttgggttgatttagaacggctattaatgaatctataaatttggctaaggttgatttgactttctagggaaaagccagcctatcttcaaatggacagctccctccacataaacgtcaatgtaccctaaagacaaaactaagtatatgtatatacgggatatatacatatatatgtacacataaaatggattgggaagtcctttggtttagacagtattaaatatgtacttcccaagtgcataggtttcctttgaccaacctgttcaaaaaacaagcatgaaaagtgccatggcacatttcccatgtctttccccctatttgaaggacacctttccttgcttctccatcactcctaagcattttatttttaaaagaagctggttattttggccttctatcttaacactccattgattcatccattccttggaagagctctcagattacatccagaaacttgtttttagaggagaacaaggttgcaaataactttttcctctttttttattccctcttccccccaagaagcaggcaccttgaagtgtcatgaataatgcactcttgatctgacttgccttgttacccctggccagcccaagcagctgaggtctgagctttacttgccctgcatcattgtgcaatactggaaaagaaaaataatccactggtctatacccctcatactgtggtgacgtgatccgggttctcttgaatttctatgcattcaatttcctctctctcctttcgcttggcacgtttctttttcttgtggtgctttttggaaggggggaaaaacgttaggaacacaggtaaaataacaaaacagtgcagaagtgtgcaacccccagtgagcagcaagcatttgaacagtgtgaaggtcaggttcgaaggcacaaatagaagggggactaacccaataagaaaagaagtaacattttgcaaaatggctgtcccatggtcttgcaaggagctttttatacattgtgttcgggtgtgctcagttgctaatacaaatgtgaaaagcagtggtgcacagtggtcaatggcgaaattcaaggtgtagataaggcacaagatagaaatgcaatccatgtcgacgttccataatgtcattaagcccagaacgcccagctcaattgaggtgacgctaagaattagccagaagtttcccagagggtggatcactaggaaaaaagtcaggattaacaccaggagaacaccaaagcctgcaatcagaacaggcactgtgacagacaagctgtaatggtccatgaagacaaaggaggggttgaacacgatgaatcggatgctctttgagagggataggggcctcagcttttccaacacttctgtgatttctttctgcttgtctctgctagtcctggccaccagatacaagcgagaagcaatgatattgctttcatcccctgccttggagaagatgatatcatttcgaaaatgctggaattctggcttttttaaaaatgagctttgcaggacactgatgaagtcacttttgttattggcactgacgttgctgactttcaggaactggtagtactgctccacccaggacactgcagtgaatccactacagagtcttcttaggtcatcctggacgctgctgttccagtactctaggggctcatagacgtagaatcctatcacagggctatagttgctgaaatatttctgctgaaccatggcataggaaacacttggcgaatcactggctagtagattgatgatgttggctccgtcactgatctgtaagcaccccatgaaggagaaggaggcataaatgagatagaggatgacaacaaatggcttcacatatatattggtaatccattcattataatgttcacggaggaagtgctgaatgaagtggtgctggtaggggttcgtctcatgatgggacgtctgttgatgcccatcactcatcactgtctggaaccacacaggtttgcgatccaggtattctgcagaagggatcttacagcaaaagatgctgtggtagcggttttgctctagttggccagcaaagaccagacaggagccaaagaaggagaaaatgtagaagtagttcaacagaatagagacacacatgttttgacagaagaccttcacagcctctatgtttgtgaatgggctggcacccatgccaaaagtgatgaagtacagggagctggtcatggtataggtgaccatcacatcagaataggcatctgctatcctgtctttgaagggcaagttctctttggttctccgccatccggacagaagctcaaacactcctttagttccatgacccatggcgaagaacgggattcccagcagggtggagttgtactttccatcggtgatgaagaagatccctgctgctgtgatgatggagatgcatactgtgagcacccccaggaggcccaggaagggcttactgcgcaagcagtccttcatggagctggagagggtggctgtggtcaggatcagcacgaggctcaccaggaccttgcttctggccaggatgctggtcttatgaaagtccctccagaggctaaaggatgctaaagagtagagctggagttcttgatgctcctcctggagcttccttataagcttacagaactcattctcccacttctcccctatgaggtcttgggtggcagagccataggtctggaggtagtaggtgatttgaatggctctggctgacttgacccgctgatctttgctgtttggcacttccactaccccgcccagttggtgtccaataaaactgttcctcccatccttctggctttcggtttggattggcgcatggaggcaacaacagaattggagagtgagaggggatttctt

SEQ ID NO: 10506 - RNA, 22905 nt, Homo sapiens
  source 1..22905: mol_type = other RNA
cctgtgccttttacttctttaagcctgagaagcagcaggctaccaattgctcccatttaaggatgtggctgccatgataatctttcacttgttcagcagtatttctttttctttccattgacaagctaggatacgagcacagtccctgctctgccaaaggaaaccatgtcttttgttaaagtttaagctactgataaatatttaagggagtgcaggggtagatgttaatattacctagcaaagaattcatgggcaaacaactttcaaatgtatcagtaagtttaccttaaaatgacttactagataatgagatacatctaatatatttgcaactgaaacacttgaagctttcaaggtctacctgaactaatttcttccctccctccctcctttccttccttcctttgtcaaatatttattgaatgcctaacatgtgcctggcacccttcagggtactgggcttatagcagtttacagagcagaaaaatatctctgcccccttagagctttcaatttactggggacagacagacaataaacaaatcccatgacaaatatgaaagaagggaggagatttactatattttcatgagattgtcaggaaaggcctctctaatgcatacttatttaatatttaagaagaaaccaaaaagatgtgagggaggaagatctgtggctaactgggggaagaagagcattcagggtggtgggaactgcaatgacaaaagaccaaagggggtgcatggttgatgcagagagaacaaagggggcagtggctggagaagtggtcagagcaggagacaggggaacagactgggtggggcttcccctctttcgtgaatctcccacccaagttaatgtctgtgaagagatggttcttttgtttaggcagataaaatgccttcttcaaggcctatttgaagctgcatttccttcttgaagtattcccctttaatgccaatagttccctatacccagattctcttaactctaaagtatgaatcatgcaatcatttcttgtgctttattgtgagtgactatttcttctgtcagcatctttaaagagattgcaagcaatttaaaggtagaaaacacatcatactttttcttcatcccatatagcacatgatgttaaactcaaggtaatcaagaaagaaatgaaagaaatatataaaactgtcaattaagaaaagacaaagaaatatatgactctaaaaacaaattcaggtattttgagaatatagccatgaaaacaaaaacattaaggtagaactcagtggataagacacatgatctgattttgtttagtaatctacatcattgcttatcccaacttagagcttatacctatacatctgtagatctcttcttcctgtcctacagaaaatgtaatccctcatccatgcagccttctttctttctttacattagcactactgcccattcttcacaatgtctatcttcctttatgattttttttctctgaactcatatcttcaatttcctagagtattgttacctagcagggtcagggctattagtggagcagaaattataaacatttgagagacataggtagagggttaaaaacccactagtctactagtttatttcactcattgcttgggatttatctacttaagcaaagcaattaggttacaaatgaactggcgataaaatactttcataaaaattatttatcctgagataaactctttatgatttttagacttgaaataattttatatacttttaaaaatcagttctgtatctaaggtagtatagtccaactaagaaacagagttgatgtgctccatgctgaggtcgaatgaagaagatagaaagtgcccctggatgcctctctaatcattattttagtggaacatttcaatcgcagtctaattattgagctctcccaatccctccagtgctaaatttcaaacatgttggaacttggcgtgaagaagggcaagattgtttttctccatctgtagatgaattcttctttttacctaaactacttagtcctgatttttctttaggccatccttctaaatatgtcttagtcattgctgtgctaaatagaagaggtggcaacagggtagaaaacgactcattaacactccttgctgatgttctttcataaaactattttttaaaaaaattttatttgtgtctcaattcttgcctgactgtttacttactagtatttatttcttttgggtaaaattatgagtttgggaacctatttacacttacattcactaatttgtttaagtgtattaatttcaaacaaaaagatgtataccctcaaggctgtatctgctgtgtttaatacactaatcaatcattaggcatccttgccttcctatcttaccattttgtccaaaacacatctagtactcattgacatttatgtccaacaaacaaaaaaatcagtatagcaacttctatttattatggaagacatgttaactaagaatcttgaacaatttttagattaatagcaggttaattaggttaatagcaggcaaataaataataactctagttttgccaatgtctcataacaaatgtttcagtgaaagcaaatagttactttcttctttttatgagacattaaagtattccgctgagcaatttgaactgctttgtccctcacacaggactttgtacatcacttggcacattataggttcttaatccatgtttgttggatggattaatgaatgaatgatatggctagttcatcaggtcattttattttcctagttcctaggtaactgtccatatttcctgttatcgaaaaagttcttccaatcagttattctctttgtcgacttttagctgtgacttcctattattgaacataacccagtactctaagtattcgaatttaatacaaaaagaaaatctattggaacatttggtaagagatatttgacttacatattgtgtgtaactctgattggagtttcagcacttctttattgtataggtatgaccaagttggcctttaggaggcctgatggatttttaatgaattatcggttttgccaatcattacttttgttgcattatggctttttttttaatatcttgggtctggcgtatatcatagtttagtagctgtgctgttgggaccaaagatctacttacaaccattttcaacacatactaaattttttttgtaggctgctttcccccttttcccttcattgaagttctccaagaaataaccttcctgaagtcttttattcaagatcaaaatttttcaattattctagaatgctatatcattttcaaaagaatgaaaaataaaatatcaacctgtttatttatttggtttcctggccatttgtcaatttttttcttcatattttactatttatggtctagtttaacttggtttccatttgcttacttctcattccctgaaattgtactgggacagaagggaaaaattagttctgtgttattttaattgaaattcatgctgatgaatcatttttccttaagtattcttttcttctattaggttataaattactcaaatagctagaaatcagcaatattgtttagaaaataagaactgatttccacacagacccattaatactgtttcctttggaattgtaatactcatctgctcttcagtaacaaagacaggcttctctaacatgacattatcaatgtttgcttcctggaacactagttctttaagatgctccatgaacataatgacccatggtcaattatatctgggaaatcaaatactgtctttatgctactggaacattaatttcacacattgagggtaattcaaagaataggcttcattttgccagtgttgaagccattttaatttcaagtagcatttcgtgataatataggaacaaaaagatcttcaaattctctgggcattcattgtacttaactttttacttaagagttggtatttatcaatatgatttttgtgttgtatctgagacttatgtggtcccacatgcaggggcagatcaaaattttgttgagcctgaagtgtatacatttttggagtccccttttaaggaaaagaatgcaaaaatatcatacatttgaaaattttatataaacataagatgtgaacatactgctaaggactgtcctagggcctccaaaagacttatgtaagcaatgggctcagaaatttaagcttcattagctacatgctacacttgcatatcccacatgaaaaatagtactttactattatttggcctaataatataatagtgtttcagcctcattatttctggttcttttctccacctgacacataccctacattcttagggttgtgagatttagcaagtaaaaatgcaatatgcccagttaaatttgaatttcagagaaacaagtatttttagtatagtagattccaaatattgcatgaaacatacttgtactaaaaatttcattcactgattattggaaattcaaacttaactcatgtcctacatgaatctagttctagtatagagtgctagttctagtatacagtggttctagttaaaccagtctataacaggacttctctgaaaatgacacattcttttatactctacgccttggttccatgttcctaaattttcttcatgaaaagactgtccagagcaacttattacaaatagagattactaaggccatcccttcaagagtttaaaaagtcttctagatgagttctaccaacaggtagacttgtcagatatggccttagttcaggtaatttcttttcttcaaactggaatgtctttgcactcttcaactatgcagcctttcaggcctagtggtgagaagctgacctttgtcctcaccttcttccctggacagatttaatccaactattctcagaatgtctgttgctgttcacaaacttagatttcagagattttcaaagtccaagtgtggttcctcagactagtagcattagcatcacctgaaaacttgttagaaatgtaaattttcaggcctcactccagatctattgaatcagaacctctggagatggggatatgcaggctgtgctttgacaagccctccaggtgattttgatacatgcttaagtgggagaatcgctgctctataaatggagcccattatttttgagatatatatatacacacacacacacatatatatatatggctatttcacctactagtttgctttgctaaaatccttgatgggtagtggctgcctctcatttctctttgcatttactctctatgtgtctggcacatagaagatgtttaaaattcttcttgaatgaaagatttggagaataaaggggttaatagataattacattttttttgagtaagctacctggtgaaagccatgacccaaagggcatcgcataaagctacgtggatgatcaagctgctgtgtggccccattgcatggcactgtggctccaagttccaactcttttacattttctcaagttgttatctgcttcctcatcctcacgtattttagttctatgactgtagaagaatacaaagagttcatatggattattttcacaggtcattttaatgctaatgttaaaaccatgtatgtgtgaaatatttgacaggacaattataccataggaaaagttttgaattagagacaggccatccaatgaatgtgtaactatgtgtaaggatatgttgtgaaaattacattttacatatatatccatctttgtccagtgctgacataacattgcaatactacatctttatggtagaataaaagcatgtgccttatacataactttcatagaagatgactgcagagcagatctctgattgtgggaggaacagtgatcttgtttctaagcataaatcacctgaactgctaaattccctgaaatgcaaataaatctcaagaattatttgctaattaaattgatgtttatatatgtagattaatctagatactattgtagtgtctctagctataatacgtgcatgtagataagagttatatatacctgagtatccagtaattttacatggaaaaaagtataaaagattagactgcctatttatgttcctaagatattcgtttcttcctctttgactcatcttttatttactgaatttaattaatgcaatataaaccatttttccccaagttagatatgcagaaaaccaaatcaactgttctgtaaagataaagcaatttcctgaaaatttgtggtaaagctttacaaatgttataaaaatgggccacgctgcatgtcaaaaccacaggaatgtgaagattaaactatacattagagtattgtagtaaatagatcacacagagctaataactagttactgttataccacattaaattcactaatgtgaatattgttgtgttttagacactcaaagttcttgggtgttcaggccatcttacagatataagttttgtgaattgtatttatttcttcctttttatattcagtgccacaactctatttcaggccaatattaccttcattgctgatgaccacaacagcctcctaacttaattctttggttcaggtctctcatctccagtctaacctacacttagaacattgcagattaatacttctaaattttgaatctaataataataataataaaaagtaatctgagtccatcaaatcaaatataaattctgcagcatgatgtttgcaggtccttatatgaaactttctggtttgtacaaattcaactcctgtactggaaatgtaccctcaagctaaattgagttcgttgacccaggaacatattctgtgcttttgttgcatgttatggctttgctcagtctggtcccgtcacatggggtgctcaggccaataatcttacctcatcttaagtgctatcttaatgcaacacactcataccaggtttggctctactagaaatcatctctctaccctctggatatctccttttggactctgtacaagttctggcttatattctagttatagatgtcacagacgcttttgtcttgtgactttttaaaacttcacttaataaaaggctctatcagtatttattggattaaatgtgttgacttggttgtctaagccactgtttttcaaattgagccacacattgaaatcactatgggaactcccagaagtactgaggttgggtctcgctataggatatattgatttaagtagtctggcatgaagtctgggcattgagactttaaacatctctctaggtcattccaaagtacagcaaattttgagaaccactagctttgttactcctagggttatccaaaatgtctcttagagtgtgtttgttgaccatggtctcgtatggccacttggttgttggatttatctccattctacttctgtgaacagatgtcctcctcgtgaaccagttggaaaatggggcctccccaggccaactccaaccttatctataactctaaaaagcataattaggaaatgcttttttcaggtttaaagtttaaaatatattcctccaaacatcttgtaatatgattgctggttttggggagcaccactattataattaaaactttaactattaaaaaggacaagggtaatgtataaatcagttaggtttatgcttaaaaactaagtgcatatgtaccttatgtgatcttcaaagaaagcatcagtgaatcataaggaagtgaatttaaaaaatagttttaagcattttaacaaactcattgtcttaaaatttacatttagaaaaggatagatggggagaaaatctatgcagttatttttcatcacatataatttacatttggacttctctgtacatgcacctttcatactgatttatgatgaaaagatgatatattttaccatagggacatagtacttgtttacaatgttttctttctgggaacaatctataaatcagggacaataatacctattctattaggcaggtattatttgaattgttaattaaaataatattaacagagatagttaattggagtgtattagtttgagctgtttgttctggagagtttgggttcccagcaatccatgtcagtctcttactctcacactttgagggcttttgtgccagaacgtggacggtgttccatcatcaggagaatcaaactcatgctctaaactggctcttgcaaccactacatttcaaagcaagagagattataaatttatgtgatattgctcagttttgggatccttgattttaacagttaaaattcaaaaatagagactgtgtatttacattttgtaaaccattcactgcatttaagcccaaggatacatcataaaaagagctttttctttatgatccctctccaaaatccaagtaactccccatatcctggcaatgctttataataccactcacaatgggcgcttcctttttattcccatctgtaacaagtctcttctgggttgctatcatctcatctgttatagccttcatcctggacaacctgctttcctgcccttgtatatttcactttttctccctgactgttgagcccatcctccatctctatctattagaatcttacccacacttcaatgtggatcagttcataattccttccttactttccttgaatactccagctgcaaatttcctcaacagatcatgcatacctcaaagtcaggaactatgaatagtttagtggtattttcttctgagcctagcacagagaccaatataggtgctcctaaatatgaggtaagtaaataggtacaatcacaagccatctaggggtacttcagaaacccatctacatcaaatcttgatcctaaaatgggactgaatttctagttctatctttttaaagagtaacaaactttttggagacttagatatgtcagggtttttctgaaactttccaatgtgttcctttgtttttaaagcctaactaagctaatgaacagaaactaaataaaaaaaaggtttcagttcagttgtttagtcccttcttcaacagttttagatccgttttaaaattttttctcactttacctttttttttaaaaaaacacccttgtccttaatttttctttatgttggatcacattctcccttattttactatcaagatgtgtatagctctaggttgtagcatttcaacttataggaaaggacagttattaccaacaaacttgaaattcttcctttatatggggccttattattgtgtaactggctatataggaaaattcaagaaaatgaaacaaaacaacaacaaaagcttctgaatatgggctctcaaagattgaaattattaaataacctccttttcattaggtcatgagcaggcaactgataagctggagaagtcttttatatttttcttcactgaatggataattactgaacgtctgcaaagcagacattgtgtgcttcatagtttggcatgtcagttgccatttttaaaataaaatcagtggagaatttcaacttgaagcacatataaatgacaataaatagtacttttgcaaactttatttagtatttgcaaataggttccaaatgtccagcttaatttttctgagttcttatttcattcctttctagccatgcttatttttatgtaaaggagaaaacatgcttaattactctaaagaaaagttattttagaaatgataaaagttgaacatatttaaaggaaaaaagcagaataaaattaataattaaaatactaaatttggacaggaaaatggctattgaataagtccaaacatttccaggaaagacataaaggcatccttgtttttaagaaaacatacggcaaactatataaaatgaaatattactaagacttctttggtctcctcatcatacgtcaataatgaggagagctttgcaatgataaagcttttgaagtggcttgtggaatattaaattgtttaagtataattttggcatcaagtgaccttacatattttgaatgttggttatctatgcgttatgtataatgccaccacattattcatcaaaatacagtggacttggatattgaaatatttaacatgattggttttagtgacttagaagtggtgctgatagcccctgaacaattatgccccagcttgaaactgtatagcgtgcagccaaagggatgtgctttgtgattaatctctgggtactactgaggagccgctggctcactcattgtctccatcttctgcagctctcatatggtgagaaaaatgttggttcaagtatttttatagttaatattactacaataatgcaatgtaatgcagtgataaattttaggtagaatttatttgacccgattataaattgctgtagatttgaaggtaacataattattaaggggtgttaaagtgctatctgaatcttttagtaatgctttagtaatttatgtgttttagagacatttgtgaacttagggattcataaaaatatctctcaggaatgccaagacattttgtatttgcttcagaatgctttatcttaaccacggagagataattgatatatatcatcacagtattattttaatgtatgtattcttgaatgtttaaaggataaaaaattacattataagttttagaacttgtgattcaataaaatactaaaaaaacatagattatgttattttacattgtgatgttataagatgttttgtttaggaagtttaattcttagcctagaattaaaaggtagcatgctcgaagttctcactgaggttagaggaataagttgcatattataatattctgtggggcatttaatactaacaataaagaatgaagaaaaatctggcgaatttaagaataacctagcttttacagcatttgtgattgtgattttaaaagacctcatatttgaccctaagaactatagaatatacacctgtataatttatcactactttaatatataaattatttctattattatgactaatggaactagatttcttttgttgttaaaataaaaagttgagatagccagaaatgctgtttaactttgcctagtggcactgtagtaaatatgattttgatgacttttttttccaagtagctaagatttaattgttatttttcttaagatttgtacctgtaagctttagataatagatttgtcatgcagataaattatgagcaatttaactaaaattattgtatttcagtgtgtccaaaacatgaaaataatgatgaaccgaacaaggaaatatttggaacataatttcccttgactgaggtatgagattcatttaattattaaatgtgtgtttacacatgcaaatctatgggaaataatttgttctttatttgtttctattatagttaagaaaaacctgttttgcaaaatgttttttcactgatcaacatagaggtaaattttgataatggaccaaattcaggtgaattggaaactttggaaactttggaaggacttttggtttgggttcttagtaagatcaaaaataggtacttttagaatattttcttctttgtgagatctaaaatggctacacagcagtcttctatttcacaggagatatttttggatggaaatacaacttgggtaatgtttttttgatttgacatttttgttcacaattcgtttttaagctttcctcagtaaggtagctttagttgtagagcccaaggtacagaactacagagcagaaacctaaaatggctttgtttgtactattttgggagtgataaatgaggctgttttcatgaatgggatgaacctatatgtaatagagtattttagaaggaatattgttatgggtaaagacatctggaattgatggtttgccatgaggtttgtagtgttaatacatcaaagtttcataatttcatacatttagtcacccttctttgctgtagaaactggtattttgtctagctaggattaagaacaagtgggttttgttttaggaaagaaaataaaaatgctcaacttttactctcatttctacaatttgtctatgcatgggtgaagactgtttctccctaggagttttcttttcactgatgctaatgtttccgtaagtgacttgtgttttaaaaaccccgatttagcagaaaataatagcaatgccttccagaggaaaagaaaacttaagtaaaatgccaaataatggtaactttgtctctttctatttgcctagaataaacaaacaaacacccgaacagattttttcctccaagaaaagtgataagtgaaatgcacttggaatttttctgaagttattcacagattatttgtgcatcttactgggtagactgctgcctctaatcaaagtcagattactctctttctgagtcaatttttgagctctgggatatctgtagggagacaactaacaactgccttgaaagatttcatattaatgaatattatgttaaccagaatgtataagtgggactgcatataggagtgctcattttacattttgccttgtctaatttgataaagtgaatgagcatcaaggaaaggtgataaataatattgctttgtggctttaatatattgccatttaatcaaagattgcatgccattttgtctttaaatacccttatgaggtagcttggagagatctctgcccttttcaatctgtgacagatttcctagttcagagcaaaaaagtctactgctgaaaaatatgcataattaacaggaaagtataataaagttgttgcttaaactactaaaactttgggatatttgcattgactagtttaaggtctagtttatcagtttgtagcacatttatgtttgtgaagaaaagatgccagaattcccttattctacttgaaaatagatgctacagactgtaccaggagatgcaagaatatgacggcttattcttttttttttttccccagctctatcagtgttgctaccaacaaccagtgaattcatcagataaaatgatagaaggtgtttccgtgtccagggagagattctagtaaccatattacattagataatttaaatgctccccataacatactgtagactgccgctactgagaatataagttaaatttatatagcactgaaaagttatacatttttattaaacaccagtaatctttcgtccatgagagtgtttcctagttattcctaggaaattcttcaatgcagtcttccaaagcattagaatttttttccccctctggtttgacagagccttgtgggcaatgtgcttactctacaaactgtggcaacagagggaaagaaaaccgtaatgctcctctattagaccatgccattagctgttgggaaaccagagctcagctacaaatggcttctaaaaacctcagctcagataagtgcaatgaaatcatacacagcaggaatcacacaccatcagtggtgattcctactctgttcctaaagtttctttctgatttttaagattttataattaccatgacctgtgagacctttcttaagggaaattttcaactggggaaaaatagtagaagctggctttctataatttaagatagtgcaaaatcagtgatagtttcctttataaatactttattatattaaaaatatctaccttatagaggttttcagtttaaggtacactcccatttaatttttacatctttagagatgcagaagacataaaatgtgatttgtagactaggaagttatactataaatatattcttaaccctatatattgctcttttgagttgttttccgttttataagaaaagcaagtggcttctctatcagcaatagagagtcctcattaagtatgaaaaaaactgattagaaaaagtgttcattatgactcaaagactcacaaaatatagtcaatgagagccactctgggaatgaatgatgcttatgtcggtgcttactttaagcttctttacaaagagtctccctagcttttcactttcactaacaaaagggtctacggctcttcctttgtgcttggaaattcaggagcacctcccactgcaaagattaggttatgaatctaacaaatgagaacccagtcttcaagtgcaatgtatttgcctatgatcaagtttgctagcagttgagaatctatagttttgcaacaccacgtgattctctctgctgtattctaaatcacagaatatgtggtattattccacttgttctatcacacctacttacagacatcttgatttctgagatgtgggctcatctctcaatatccttccagtgtcatttcaaatgttgcctgatctaactccacaacacttcaaacacagaacaccacctcttgtgctcctaagttaaacgtgatggtggattaatcttggtcctttagttgataaatcaaggtaatttactgctgctatacccatacacagtccctcccctgctggatctcatgcagtgtggctttgttgctttcacttatgattttgctgctttcatttgggtcaatatcattgtagttattttgtagacaaagtagtaaaaaacttgatttttccctatcctatatatctgcagctcactgatttaaaatattagcataaaggtccgcaccacagtgatgatgttcaatttcatattgagattgaagatggggaaatagcaagggcataccaattcagccataaatatgttttgggtcaatgtcataaaattgtcacaaaattttggtaattgagaaaaagctaaaactttttttgtttgttttttgtttgtaaagggaagaaaagtgcttctgaggctcttttggaataagtaacagttttcagattcacttttgcaaagattgccaatatccttcgcagacaccaacaaaccagactgaacagaaagatccctgtagtaggatgccgagcaaatcattgacttctccaatctctaagagacaatatctaaatgtcagtctcatggcattgtattttctgcttcaccataagattagcaaacacaagacataaaattatgtttatttactaaccaatacagaatatactaggccctttgcctggaagccagatttcacttctgagattttccgaagtccattctagaagaggtggttgttactgatacccagggaaggcaattcttaaattgcttacctggggatggaactttctgtggactttaggcccttaagaccaaaagccatgaggcatttatgaataggtgatgtaagaaattttaataaaagttgcaataaccctgaaaatagtgtctttaataacctatgtactattaataacaaagcatgcatagtgccgtgcattcataactatttggtcataaaaatatgtgactgtaattatgatatttacagtcaacttataaaaatacatgtaattctgaatggcaatagttaatccttagctctaaccacaagcctagaaggattagcttattacggggaaatgtgatagataattacaaaatggacaaagcttttactgtcttgaatttaacattcaagaataactataatagcatcataaaacatttgtcatcattattcttctcacctcacaaggtaaaaacctaaattctgtggaaataaatgggaatcaaataggaaagggccacttacatgatacaacaacagaggagaatagttctttcatagaatactcatgcacagccttcaaagaggttcatagtaactgcaagaattcctgggaagacatctaaacatgactttcattaaaaagaattaaggctggtctaaagaatcaaatctctaaggtatgattacctttaaccataaacggtaaaaaatcttttagctgatctctctgtaatttaggtgagtacctctttgaagtttattaacatcaaagagagtggagctcacatggcactttccaattcaaatttaaattctgatggaaggaaataaatccacattccagtttacatacagaaaaagagtagttttttcaaactttataacctcttactttaagggcatatatgtttcaattaaataaaatattacacaaagctaacatatttcccacaaatttcttctcttctaggagttgattggtcatctgctgacaacagataagttcctaatttgaatggcattagtacttcataaatgaacaaaacaatgagtgcaaactggaaaaactagggagaggtgcatacaagctaccaaaaaaggttgggattgggggtgacctgcaagtcatgatctcatatcttaggatgtatcttagtattcaggaaatggaattcttggaaacatctgtttcacagtgaggttgggaggtcagacgatgctctgttagattcttcttaggattaaattacttcctaggactgcattaagacactttaggtggtatattaactcttccagaacaaataattccatttcagtaaattattgctacagttctctaaagagtactacggtgtcctggaaaagataatgttccttccaaaatgccctctagtcactcgaacaatgagaaattcatatttatcttagacactttgatccttgaagacataaactaaaaaagaactgtttttccctatctaaacagagactatctggatggagacataatattagatctgccctggtcatttggcagtgtataccatttcctccatgtgcttttgacaactggcatgcttgattctttccctgtaaatcagcctgccattcttctttgcatgcagaatggtctataggaaccaagaaaaaaccaaccccaatagccaatcttttaaaaaataggtgaatgagtggagcatggcacacaatgggaagaaaaggagtgatagttaattaactttctcagtgattatctcccatattttgatatgggagataaaaatcttccatatcaaatctttacaaatgatgggtaatctgtaagaggaattctcctcctccctgcacccccactacaaaactcccacccaaacaaaaaatcaaaacccaaccaaaaacctcctctgaaacttctacttcagatatgagatcatggtctggaggctactcgtaccaaataccagttcattctagtacagcagttcatgaggcaaaaggctaggagtatttgtgacatgactttacaaataatgtaaaaacaataaccctatgattatgggcaataattttccccactcaaatctatagatattgcactgaaactgacacaatggagaagacatagatcatttcctgttgaaacccaattacctcaaggtaaaacaaaacaaactccatttaataaatgaaatattacttaaatgttttcattttagggtctgttccctttcccctttatattctggaaagttatatgtctaagtatacttgttttgttacttcattagtctatcaacttcatttccagagactataacgagaatggaatggtttgtaccttttttctgaacataattgagtcaaggagttttgttattttaggtattattaatttgattaaaacatagaaccaaagttgatgggaagtagtagctttcttctaggtaaaagagcttactagcagattttataatcatcggacatttattctgtcctacctggaaataaattatgttactgcttggcatgggaaaaggcattttctagtaatttcctgtgacaggaggcacagcaatagtccaagtaagcacccaacaggtgcttgggagtagttttaaactttaacttaatgaaaacatttacctcagtacttttgtttgagaaagaattcagcagcagttatagttaatatcccacctgtggagagctgcgatcaccctaggaggtgggccaaccgaggagcactttccaggtaacaagagcaacactattgtgagaagctacaaatggtactgcagtaggtgtagtgaacactactatagtgatcatggcctgggttatgttccaaatactaatgcaaggaatacactagagtttataggattagaatagtttccttatgctaagaactagtagatggcatgtgatgagtgggtatggtccattttattctatttcactctacgagtttcctagttatgtctcctttctcctatgttaattatctatattccatgacagttattttccctatctaaaataagaacggtgtaactatggagtaccccaactcacatacacatacttgtgcacccttagactcatgtatggataatctgtgtaaagcgctcatttgcaattgggtgagctcactgaaagcagccatatcagtcttccaaatacagtaaaagccaacgaaaatccatatcaactgtttatttctaatatgaaacagtaaaccttgtccatgtggtaattaattcaaatgccttttgtgttttcttgtgaagtcatccaaagcaaaagtctagatgactgctgacatgatatgcataatctaatgaactcacatctctgtttattttgctcatcccacagttgaatgacacactgactgctgagacacttgggttgatttagaacggctattaatgaatctataaatttggctaaggttgatttgactttctagggaaaagccagcctatcttcaaatggacagctccctccacataaacgtcaatgtaccctaaagacaaaactaagtatatgtatatacgggatatatacatatatatgtacacataaaatggattgggaagtcctttggtttagacagtattaaatatgtacttcccaagtgcataggtttcctttgaccaacctgttcaaaaaacaagcatgaaaagtgccatggcacatttcccatgtctttccccctatttgaaggacacctttccttgcttctccatcactcctaagcattttatttttaaaagaagctggttattttggccttctatcttaacactccattgattcatccattccttggaagagctctcagattacatccagaaacttgtttttagaggagaacaaggttgcaaataactttttcctctttttttattccctcttccccccaagaagcaggcaccttgaagtgtcatgaataatgcactcttgatctgacttgccttgttacccctggccagcccaagcagctgaggtctgagctttacttgccctgcatcattgtgcaatactggaaaagaaaaataatccactggtctatacccctcatactgtggtgacgtgatccgggttctcttgaatttctatgcattcaatttcctctctctcctttcgcttggcacgtttctttttcttgtggtgctttttggaaggggggaaaaacgttaggaacacaggtaaaataacaaaacagtgcagaagtgtgcaacccccagtgagcagcaagcatttgaacagtgtgaaggtcaggttcgaaggcacaaatagaagggggactaacccaataagaaaagaagtaacattttgcaaaatggctgtcccatggtcttgcaaggagctttttatacattgtgttcgggtgtgctcagttgctaatacaaatgtgaaaagcagtggtgcacagtggtcaatggcgaaattcaaggtgtagataaggcacaagatagaaatgcaatccatgtcgacgttccataatgtcattaagcccagaacgcccagctcaattgaggtgacgctaagaattagccagaagtttcccagagggtggatcactaggaaaaaagtcaggattaacaccaggagaacaccaaagcctgcaatcagaacaggcactgtgacagacaagctgtaatggtccatgaagacaaaggaggggttgaacacgatgaatcggatgctctttgagagggataggggcctcagcttttccaacacttctgtgatttctttctgcttgtctctgctagtcctggccaccagatacaagcgagaagcaatgatattgctttcatcccctgccttggagaagatgatatcatttcgaaaatgctggaattctggcttttttaaaaatgagctttgcaggacactgatgaagtcacttttgttattggcactgacgttgctgactttcaggaactggtagtactgctccacccaggacactgcagtgaatccactacagagtcttcttaggtcatcctggacgctgctgttccagtactctaggggctcatagacgtagaatcctatcacagggctatagttgctgaaatatttctgctgaaccatggcataggaaacacttggcgaatcactggctagtagattgatgatgttggctccgtcactgatctgtaagcaccccatgaaggagaaggaggcataaatgagatagaggatgacaacaaatggcttcacatatatattggtaatccattcattataatgttcacggaggaagtgctgaatgaagtggtgctggtaggggttcgtctcatgatgggacgtctgttgatgcccatcactcatcactgtctggaaccacacaggtttgcgatccaggtattctgcagaagggatcttacagcaaaagatgctgtggtagcggttttgctctagttggccagcaaagaccagacaggagccaaagaaggagaaaatgtagaagtagttcaacagaatagagacacacatgttttgacagaagaccttcacagcctctatgtttgtgaatgggctggcacccatgccaaaagtgatgaagtacagggagctggtcatggtataggtgaccatcacatcagaataggcatctgctatcctgtctttgaagggcaagttctctttggttctccgccatccggacagaagctcaaacactcctttagttccatgacccatggcgaagaacgggattcccagcagggtggagttgtactttccatcggtgatgaagaagatccctgctgctgtgatgatggagatgcatactgtgagcacccccaggaggcccaggaagggcttactgcgcaagcagtccttcatggagctggagagggtggctgtggtcaggatcagcacgaggctcaccaggaccttgcttctggccaggatgctggtcttatgaaagtccctccagaggctaaaggatgctaaagagtagagctggagttcttgatgctcctcctggagcttccttataagcttacagaactcattctcccacttctcccctatgaggtcttgggtggcagagccataggtctggaggtagtaggtgatttgaatggctctggctgacttgacccgctgatctttgctgtttggcacttccactaccccgcccagttggtgtccaataaaactgttcctcccatcctttaatttagtgttgggatacctcacttgcaccctggctgttgtcttattggagacggcagcctgcctgagatcctctagcactgaaataatatcatccagcacgcatttcttatcctgatttctcaacacacacagatgggaaaaagtataattatagcccttgtggttcaccttcatttccagcacggctcggtgggtctgcaggatcccctcagcctggagcaaaatattgtccccggttggggagaggaggatcaccctgccatacctcccaggggtgtgtaagtccgaatagagctggcttttggactggtccagggggaaaaggctgctggccaggctgcgctcgatcttggccaggctgtggctgggagcgaccaggcgctccaggtcgccctcgggctggaagcggttgagcgcgctgaggccgaaggtgattgtcaggactgcgggcacggtgaggaaaaagaccgggtgccggctcacgcacaaacccagcctgtggcagaacgactggagccctctgcgaagcacctgccgcagcatcctccaccagatccagctcgcaggcgctcccggccgtcgcatgagcagcgttccctcggtctagcccttcatctcggtgctgcagtcccctggcctccctcgctggaggtggttccgtgtggagcgtcccacagatgtggatttcctctctgtcttggtggggttcggtgcctaactggaaccatgtgcctcggtgttgtaagaagcagacatgtgccccataaagggggggggggctgagggggggagaggagggagaagggcgggagcacgttgggggtgggggggcagataagcttttttctttttttaagatgctgacagttatttttagagttttgtgttccctcttccctccccgctggagtgaattgaagaggaaataaatggtgaaggtgctgctggcccattggagcaagggcaattagagcccaaggagtggggcatggagggagacagccccagggctccaggagacagccttctcgcccctccagtttccctgtgccctcgaattctgcttttcagcgaagaaaaggagcagagaggatgatgctgcatttttaacacaccacacagcatgcaagggatttcctcgcaacaccttcctcgctgtgattccacagaccagtccgctgcagctgagggctgcggagactccatctatccctggtgcgttgggaccgtctggatagcttctttcctctgatggctggagaggaggcatttgccaatagcagtagcctgtgtgcgtgtgcgtgtgcgtgtgtgtgtattgaaagtgaagatctacaggcaatatgaggtttctcataacatgttacattcactttctgtattcttgagattaaaggacagaaagttcctaaagctgatttcagtccccttttccagtgtctccttccacccctcacccatgaggactgtttcaagccatctggttcaggctaattttcccctgtgagtggaattccagaaacagacacttccagacacaccaggtagttttgccttctggctttcggtttggattggcgcatggaggcaacaacagaattggagagtgagaggggatttcttttatttcttctctgc

SEQ ID NO: 10507 - RNA, 21861 nt, Homo sapiens
  source 1..21861: mol_type = other RNA
cctgtgccttttacttctttaagcctgagaagcagcaggctaccaattgctcccatttaaggatgtggctgccatgataatctttcacttgttcagcagtatttctttttctttccattgacaagctaggatacgagcacagtccctgctctgccaaaggaaaccatgtcttttgttaaagtttaagctactgataaatatttaagggagtgcaggggtagatgttaatattacctagcaaagaattcatgggcaaacaactttcaaatgtatcagtaagtttaccttaaaatgacttactagataatgagatacatctaatatatttgcaactgaaacacttgaagctttcaaggtctacctgaactaatttcttccctccctccctcctttccttccttcctttgtcaaatatttattgaatgcctaacatgtgcctggcacccttcagggtactgggcttatagcagtttacagagcagaaaaatatctctgcccccttagagctttcaatttactggggacagacagacaataaacaaatcccatgacaaatatgaaagaagggaggagatttactatattttcatgagattgtcaggaaaggcctctctaatgcatacttatttaatatttaagaagaaaccaaaaagatgtgagggaggaagatctgtggctaactgggggaagaagagcattcagggtggtgggaactgcaatgacaaaagaccaaagggggtgcatggttgatgcagagagaacaaagggggcagtggctggagaagtggtcagagcaggagacaggggaacagactgggtggggcttcccctctttcgtgaatctcccacccaagttaatgtctgtgaagagatggttcttttgtttaggcagataaaatgccttcttcaaggcctatttgaagctgcatttccttcttgaagtattcccctttaatgccaatagttccctatacccagattctcttaactctaaagtatgaatcatgcaatcatttcttgtgctttattgtgagtgactatttcttctgtcagcatctttaaagagattgcaagcaatttaaaggtagaaaacacatcatactttttcttcatcccatatagcacatgatgttaaactcaaggtaatcaagaaagaaatgaaagaaatatataaaactgtcaattaagaaaagacaaagaaatatatgactctaaaaacaaattcaggtattttgagaatatagccatgaaaacaaaaacattaaggtagaactcagtggataagacacatgatctgattttgtttagtaatctacatcattgcttatcccaacttagagcttatacctatacatctgtagatctcttcttcctgtcctacagaaaatgtaatccctcatccatgcagccttctttctttctttacattagcactactgcccattcttcacaatgtctatcttcctttatgattttttttctctgaactcatatcttcaatttcctagagtattgttacctagcagggtcagggctattagtggagcagaaattataaacatttgagagacataggtagagggttaaaaacccactagtctactagtttatttcactcattgcttgggatttatctacttaagcaaagcaattaggttacaaatgaactggcgataaaatactttcataaaaattatttatcctgagataaactctttatgatttttagacttgaaataattttatatacttttaaaaatcagttctgtatctaaggtagtatagtccaactaagaaacagagttgatgtgctccatgctgaggtcgaatgaagaagatagaaagtgcccctggatgcctctctaatcattattttagtggaacatttcaatcgcagtctaattattgagctctcccaatccctccagtgctaaatttcaaacatgttggaacttggcgtgaagaagggcaagattgtttttctccatctgtagatgaattcttctttttacctaaactacttagtcctgatttttctttaggccatccttctaaatatgtcttagtcattgctgtgctaaatagaagaggtggcaacagggtagaaaacgactcattaacactccttgctgatgttctttcataaaactattttttaaaaaaattttatttgtgtctcaattcttgcctgactgtttacttactagtatttatttcttttgggtaaaattatgagtttgggaacctatttacacttacattcactaatttgtttaagtgtattaatttcaaacaaaaagatgtataccctcaaggctgtatctgctgtgtttaatacactaatcaatcattaggcatccttgccttcctatcttaccattttgtccaaaacacatctagtactcattgacatttatgtccaacaaacaaaaaaatcagtatagcaacttctatttattatggaagacatgttaactaagaatcttgaacaatttttagattaatagcaggttaattaggttaatagcaggcaaataaataataactctagttttgccaatgtctcataacaaatgtttcagtgaaagcaaatagttactttcttctttttatgagacattaaagtattccgctgagcaatttgaactgctttgtccctcacacaggactttgtacatcacttggcacattataggttcttaatccatgtttgttggatggattaatgaatgaatgatatggctagttcatcaggtcattttattttcctagttcctaggtaactgtccatatttcctgttatcgaaaaagttcttccaatcagttattctctttgtcgacttttagctgtgacttcctattattgaacataacccagtactctaagtattcgaatttaatacaaaaagaaaatctattggaacatttggtaagagatatttgacttacatattgtgtgtaactctgattggagtttcagcacttctttattgtataggtatgaccaagttggcctttaggaggcctgatggatttttaatgaattatcggttttgccaatcattacttttgttgcattatggctttttttttaatatcttgggtctggcgtatatcatagtttagtagctgtgctgttgggaccaaagatctacttacaaccattttcaacacatactaaattttttttgtaggctgctttcccccttttcccttcattgaagttctccaagaaataaccttcctgaagtcttttattcaagatcaaaatttttcaattattctagaatgctatatcattttcaaaagaatgaaaaataaaatatcaacctgtttatttatttggtttcctggccatttgtcaatttttttcttcatattttactatttatggtctagtttaacttggtttccatttgcttacttctcattccctgaaattgtactgggacagaagggaaaaattagttctgtgttattttaattgaaattcatgctgatgaatcatttttccttaagtattcttttcttctattaggttataaattactcaaatagctagaaatcagcaatattgtttagaaaataagaactgatttccacacagacccattaatactgtttcctttggaattgtaatactcatctgctcttcagtaacaaagacaggcttctctaacatgacattatcaatgtttgcttcctggaacactagttctttaagatgctccatgaacataatgacccatggtcaattatatctgggaaatcaaatactgtctttatgctactggaacattaatttcacacattgagggtaattcaaagaataggcttcattttgccagtgttgaagccattttaatttcaagtagcatttcgtgataatataggaacaaaaagatcttcaaattctctgggcattcattgtacttaactttttacttaagagttggtatttatcaatatgatttttgtgttgtatctgagacttatgtggtcccacatgcaggggcagatcaaaattttgttgagcctgaagtgtatacatttttggagtccccttttaaggaaaagaatgcaaaaatatcatacatttgaaaattttatataaacataagatgtgaacatactgctaaggactgtcctagggcctccaaaagacttatgtaagcaatgggctcagaaatttaagcttcattagctacatgctacacttgcatatcccacatgaaaaatagtactttactattatttggcctaataatataatagtgtttcagcctcattatttctggttcttttctccacctgacacataccctacattcttagggttgtgagatttagcaagtaaaaatgcaatatgcccagttaaatttgaatttcagagaaacaagtatttttagtatagtagattccaaatattgcatgaaacatacttgtactaaaaatttcattcactgattattggaaattcaaacttaactcatgtcctacatgaatctagttctagtatagagtgctagttctagtatacagtggttctagttaaaccagtctataacaggacttctctgaaaatgacacattcttttatactctacgccttggttccatgttcctaaattttcttcatgaaaagactgtccagagcaacttattacaaatagagattactaaggccatcccttcaagagtttaaaaagtcttctagatgagttctaccaacaggtagacttgtcagatatggccttagttcaggtaatttcttttcttcaaactggaatgtctttgcactcttcaactatgcagcctttcaggcctagtggtgagaagctgacctttgtcctcaccttcttccctggacagatttaatccaactattctcagaatgtctgttgctgttcacaaacttagatttcagagattttcaaagtccaagtgtggttcctcagactagtagcattagcatcacctgaaaacttgttagaaatgtaaattttcaggcctcactccagatctattgaatcagaacctctggagatggggatatgcaggctgtgctttgacaagccctccaggtgattttgatacatgcttaagtgggagaatcgctgctctataaatggagcccattatttttgagatatatatatacacacacacacacatatatatatatggctatttcacctactagtttgctttgctaaaatccttgatgggtagtggctgcctctcatttctctttgcatttactctctatgtgtctggcacatagaagatgtttaaaattcttcttgaatgaaagatttggagaataaaggggttaatagataattacattttttttgagtaagctacctggtgaaagccatgacccaaagggcatcgcataaagctacgtggatgatcaagctgctgtgtggccccattgcatggcactgtggctccaagttccaactcttttacattttctcaagttgttatctgcttcctcatcctcacgtattttagttctatgactgtagaagaatacaaagagttcatatggattattttcacaggtcattttaatgctaatgttaaaaccatgtatgtgtgaaatatttgacaggacaattataccataggaaaagttttgaattagagacaggccatccaatgaatgtgtaactatgtgtaaggatatgttgtgaaaattacattttacatatatatccatctttgtccagtgctgacataacattgcaatactacatctttatggtagaataaaagcatgtgccttatacataactttcatagaagatgactgcagagcagatctctgattgtgggaggaacagtgatcttgtttctaagcataaatcacctgaactgctaaattccctgaaatgcaaataaatctcaagaattatttgctaattaaattgatgtttatatatgtagattaatctagatactattgtagtgtctctagctataatacgtgcatgtagataagagttatatatacctgagtatccagtaattttacatggaaaaaagtataaaagattagactgcctatttatgttcctaagatattcgtttcttcctctttgactcatcttttatttactgaatttaattaatgcaatataaaccatttttccccaagttagatatgcagaaaaccaaatcaactgttctgtaaagataaagcaatttcctgaaaatttgtggtaaagctttacaaatgttataaaaatgggccacgctgcatgtcaaaaccacaggaatgtgaagattaaactatacattagagtattgtagtaaatagatcacacagagctaataactagttactgttataccacattaaattcactaatgtgaatattgttgtgttttagacactcaaagttcttgggtgttcaggccatcttacagatataagttttgtgaattgtatttatttcttcctttttatattcagtgccacaactctatttcaggccaatattaccttcattgctgatgaccacaacagcctcctaacttaattctttggttcaggtctctcatctccagtctaacctacacttagaacattgcagattaatacttctaaattttgaatctaataataataataataaaaagtaatctgagtccatcaaatcaaatataaattctgcagcatgatgtttgcaggtccttatatgaaactttctggtttgtacaaattcaactcctgtactggaaatgtaccctcaagctaaattgagttcgttgacccaggaacatattctgtgcttttgttgcatgttatggctttgctcagtctggtcccgtcacatggggtgctcaggccaataatcttacctcatcttaagtgctatcttaatgcaacacactcataccaggtttggctctactagaaatcatctctctaccctctggatatctccttttggactctgtacaagttctggcttatattctagttatagatgtcacagacgcttttgtcttgtgactttttaaaacttcacttaataaaaggctctatcagtatttattggattaaatgtgttgacttggttgtctaagccactgtttttcaaattgagccacacattgaaatcactatgggaactcccagaagtactgaggttgggtctcgctataggatatattgatttaagtagtctggcatgaagtctgggcattgagactttaaacatctctctaggtcattccaaagtacagcaaattttgagaaccactagctttgttactcctagggttatccaaaatgtctcttagagtgtgtttgttgaccatggtctcgtatggccacttggttgttggatttatctccattctacttctgtgaacagatgtcctcctcgtgaaccagttggaaaatggggcctccccaggccaactccaaccttatctataactctaaaaagcataattaggaaatgcttttttcaggtttaaagtttaaaatatattcctccaaacatcttgtaatatgattgctggttttggggagcaccactattataattaaaactttaactattaaaaaggacaagggtaatgtataaatcagttaggtttatgcttaaaaactaagtgcatatgtaccttatgtgatcttcaaagaaagcatcagtgaatcataaggaagtgaatttaaaaaatagttttaagcattttaacaaactcattgtcttaaaatttacatttagaaaaggatagatggggagaaaatctatgcagttatttttcatcacatataatttacatttggacttctctgtacatgcacctttcatactgatttatgatgaaaagatgatatattttaccatagggacatagtacttgtttacaatgttttctttctgggaacaatctataaatcagggacaataatacctattctattaggcaggtattatttgaattgttaattaaaataatattaacagagatagttaattggagtgtattagtttgagctgtttgttctggagagtttgggttcccagcaatccatgtcagtctcttactctcacactttgagggcttttgtgccagaacgtggacggtgttccatcatcaggagaatcaaactcatgctctaaactggctcttgcaaccactacatttcaaagcaagagagattataaatttatgtgatattgctcagttttgggatccttgattttaacagttaaaattcaaaaatagagactgtgtatttacattttgtaaaccattcactgcatttaagcccaaggatacatcataaaaagagctttttctttatgatccctctccaaaatccaagtaactccccatatcctggcaatgctttataataccactcacaatgggcgcttcctttttattcccatctgtaacaagtctcttctgggttgctatcatctcatctgttatagccttcatcctggacaacctgctttcctgcccttgtatatttcactttttctccctgactgttgagcccatcctccatctctatctattagaatcttacccacacttcaatgtggatcagttcataattccttccttactttccttgaatactccagctgcaaatttcctcaacagatcatgcatacctcaaagtcaggaactatgaatagtttagtggtattttcttctgagcctagcacagagaccaatataggtgctcctaaatatgaggtaagtaaataggtacaatcacaagccatctaggggtacttcagaaacccatctacatcaaatcttgatcctaaaatgggactgaatttctagttctatctttttaaagagtaacaaactttttggagacttagatatgtcagggtttttctgaaactttccaatgtgttcctttgtttttaaagcctaactaagctaatgaacagaaactaaataaaaaaaaggtttcagttcagttgtttagtcccttcttcaacagttttagatccgttttaaaattttttctcactttacctttttttttaaaaaaacacccttgtccttaatttttctttatgttggatcacattctcccttattttactatcaagatgtgtatagctctaggttgtagcatttcaacttataggaaaggacagttattaccaacaaacttgaaattcttcctttatatggggccttattattgtgtaactggctatataggaaaattcaagaaaatgaaacaaaacaacaacaaaagcttctgaatatgggctctcaaagattgaaattattaaataacctccttttcattaggtcatgagcaggcaactgataagctggagaagtcttttatatttttcttcactgaatggataattactgaacgtctgcaaagcagacattgtgtgcttcatagtttggcatgtcagttgccatttttaaaataaaatcagtggagaatttcaacttgaagcacatataaatgacaataaatagtacttttgcaaactttatttagtatttgcaaataggttccaaatgtccagcttaatttttctgagttcttatttcattcctttctagccatgcttatttttatgtaaaggagaaaacatgcttaattactctaaagaaaagttattttagaaatgataaaagttgaacatatttaaaggaaaaaagcagaataaaattaataattaaaatactaaatttggacaggaaaatggctattgaataagtccaaacatttccaggaaagacataaaggcatccttgtttttaagaaaacatacggcaaactatataaaatgaaatattactaagacttctttggtctcctcatcatacgtcaataatgaggagagctttgcaatgataaagcttttgaagtggcttgtggaatattaaattgtttaagtataattttggcatcaagtgaccttacatattttgaatgttggttatctatgcgttatgtataatgccaccacattattcatcaaaatacagtggacttggatattgaaatatttaacatgattggttttagtgacttagaagtggtgctgatagcccctgaacaattatgccccagcttgaaactgtatagcgtgcagccaaagggatgtgctttgtgattaatctctgggtactactgaggagccgctggctcactcattgtctccatcttctgcagctctcatatggtgagaaaaatgttggttcaagtatttttatagttaatattactacaataatgcaatgtaatgcagtgataaattttaggtagaatttatttgacccgattataaattgctgtagatttgaaggtaacataattattaaggggtgttaaagtgctatctgaatcttttagtaatgctttagtaatttatgtgttttagagacatttgtgaacttagggattcataaaaatatctctcaggaatgccaagacattttgtatttgcttcagaatgctttatcttaaccacggagagataattgatatatatcatcacagtattattttaatgtatgtattcttgaatgtttaaaggataaaaaattacattataagttttagaacttgtgattcaataaaatactaaaaaaacatagattatgttattttacattgtgatgttataagatgttttgtttaggaagtttaattcttagcctagaattaaaaggtagcatgctcgaagttctcactgaggttagaggaataagttgcatattataatattctgtggggcatttaatactaacaataaagaatgaagaaaaatctggcgaatttaagaataacctagcttttacagcatttgtgattgtgattttaaaagacctcatatttgaccctaagaactatagaatatacacctgtataatttatcactactttaatatataaattatttctattattatgactaatggaactagatttcttttgttgttaaaataaaaagttgagatagccagaaatgctgtttaactttgcctagtggcactgtagtaaatatgattttgatgacttttttttccaagtagctaagatttaattgttatttttcttaagatttgtacctgtaagctttagataatagatttgtcatgcagataaattatgagcaatttaactaaaattattgtatttcagtgtgtccaaaacatgaaaataatgatgaaccgaacaaggaaatatttggaacataatttcccttgactgaggtatgagattcatttaattattaaatgtgtgtttacacatgcaaatctatgggaaataatttgttctttatttgtttctattatagttaagaaaaacctgttttgcaaaatgttttttcactgatcaacatagaggtaaattttgataatggaccaaattcaggtgaattggaaactttggaaactttggaaggacttttggtttgggttcttagtaagatcaaaaataggtacttttagaatattttcttctttgtgagatctaaaatggctacacagcagtcttctatttcacaggagatatttttggatggaaatacaacttgggtaatgtttttttgatttgacatttttgttcacaattcgtttttaagctttcctcagtaaggtagctttagttgtagagcccaaggtacagaactacagagcagaaacctaaaatggctttgtttgtactattttgggagtgataaatgaggctgttttcatgaatgggatgaacctatatgtaatagagtattttagaaggaatattgttatgggtaaagacatctggaattgatggtttgccatgaggtttgtagtgttaatacatcaaagtttcataatttcatacatttagtcacccttctttgctgtagaaactggtattttgtctagctaggattaagaacaagtgggttttgttttaggaaagaaaataaaaatgctcaacttttactctcatttctacaatttgtctatgcatgggtgaagactgtttctccctaggagttttcttttcactgatgctaatgtttccgtaagtgacttgtgttttaaaaaccccgatttagcagaaaataatagcaatgccttccagaggaaaagaaaacttaagtaaaatgccaaataatggtaactttgtctctttctatttgcctagaataaacaaacaaacacccgaacagattttttcctccaagaaaagtgataagtgaaatgcacttggaatttttctgaagttattcacagattatttgtgcatcttactgggtagactgctgcctctaatcaaagtcagattactctctttctgagtcaatttttgagctctgggatatctgtagggagacaactaacaactgccttgaaagatttcatattaatgaatattatgttaaccagaatgtataagtgggactgcatataggagtgctcattttacattttgccttgtctaatttgataaagtgaatgagcatcaaggaaaggtgataaataatattgctttgtggctttaatatattgccatttaatcaaagattgcatgccattttgtctttaaatacccttatgaggtagcttggagagatctctgcccttttcaatctgtgacagatttcctagttcagagcaaaaaagtctactgctgaaaaatatgcataattaacaggaaagtataataaagttgttgcttaaactactaaaactttgggatatttgcattgactagtttaaggtctagtttatcagtttgtagcacatttatgtttgtgaagaaaagatgccagaattcccttattctacttgaaaatagatgctacagactgtaccaggagatgcaagaatatgacggcttattcttttttttttttccccagctctatcagtgttgctaccaacaaccagtgaattcatcagataaaatgatagaaggtgtttccgtgtccagggagagattctagtaaccatattacattagataatttaaatgctccccataacatactgtagactgccgctactgagaatataagttaaatttatatagcactgaaaagttatacatttttattaaacaccagtaatctttcgtccatgagagtgtttcctagttattcctaggaaattcttcaatgcagtcttccaaagcattagaatttttttccccctctggtttgacagagccttgtgggcaatgtgcttactctacaaactgtggcaacagagggaaagaaaaccgtaatgctcctctattagaccatgccattagctgttgggaaaccagagctcagctacaaatggcttctaaaaacctcagctcagataagtgcaatgaaatcatacacagcaggaatcacacaccatcagtggtgattcctactctgttcctaaagtttctttctgatttttaagattttataattaccatgacctgtgagacctttcttaagggaaattttcaactggggaaaaatagtagaagctggctttctataatttaagatagtgcaaaatcagtgatagtttcctttataaatactttattatattaaaaatatctaccttatagaggttttcagtttaaggtacactcccatttaatttttacatctttagagatgcagaagacataaaatgtgatttgtagactaggaagttatactataaatatattcttaaccctatatattgctcttttgagttgttttccgttttataagaaaagcaagtggcttctctatcagcaatagagagtcctcattaagtatgaaaaaaactgattagaaaaagtgttcattatgactcaaagactcacaaaatatagtcaatgagagccactctgggaatgaatgatgcttatgtcggtgcttactttaagcttctttacaaagagtctccctagcttttcactttcactaacaaaagggtctacggctcttcctttgtgcttggaaattcaggagcacctcccactgcaaagattaggttatgaatctaacaaatgagaacccagtcttcaagtgcaatgtatttgcctatgatcaagtttgctagcagttgagaatctatagttttgcaacaccacgtgattctctctgctgtattctaaatcacagaatatgtggtattattccacttgttctatcacacctacttacagacatcttgatttctgagatgtgggctcatctctcaatatccttccagtgtcatttcaaatgttgcctgatctaactccacaacacttcaaacacagaacaccacctcttgtgctcctaagttaaacgtgatggtggattaatcttggtcctttagttgataaatcaaggtaatttactgctgctatacccatacacagtccctcccctgctggatctcatgcagtgtggctttgttgctttcacttatgattttgctgctttcatttgggtcaatatcattgtagttattttgtagacaaagtagtaaaaaacttgatttttccctatcctatatatctgcagctcactgatttaaaatattagcataaaggtccgcaccacagtgatgatgttcaatttcatattgagattgaagatggggaaatagcaagggcataccaattcagccataaatatgttttgggtcaatgtcataaaattgtcacaaaattttggtaattgagaaaaagctaaaactttttttgtttgttttttgtttgtaaagggaagaaaagtgcttctgaggctcttttggaataagtaacagttttcagattcacttttgcaaagattgccaatatccttcgcagacaccaacaaaccagactgaacagaaagatccctgtagtaggatgccgagcaaatcattgacttctccaatctctaagagacaatatctaaatgtcagtctcatggcattgtattttctgcttcaccataagattagcaaacacaagacataaaattatgtttatttactaaccaatacagaatatactaggccctttgcctggaagccagatttcacttctgagattttccgaagtccattctagaagaggtggttgttactgatacccagggaaggcaattcttaaattgcttacctggggatggaactttctgtggactttaggcccttaagaccaaaagccatgaggcatttatgaataggtgatgtaagaaattttaataaaagttgcaataaccctgaaaatagtgtctttaataacctatgtactattaataacaaagcatgcatagtgccgtgcattcataactatttggtcataaaaatatgtgactgtaattatgatatttacagtcaacttataaaaatacatgtaattctgaatggcaatagttaatccttagctctaaccacaagcctagaaggattagcttattacggggaaatgtgatagataattacaaaatggacaaagcttttactgtcttgaatttaacattcaagaataactataatagcatcataaaacatttgtcatcattattcttctcacctcacaaggtaaaaacctaaattctgtggaaataaatgggaatcaaataggaaagggccacttacatgatacaacaacagaggagaatagttctttcatagaatactcatgcacagccttcaaagaggttcatagtaactgcaagaattcctgggaagacatctaaacatgactttcattaaaaagaattaaggctggtctaaagaatcaaatctctaaggtatgattacctttaaccataaacggtaaaaaatcttttagctgatctctctgtaatttaggtgagtacctctttgaagtttattaacatcaaagagagtggagctcacatggcactttccaattcaaatttaaattctgatggaaggaaataaatccacattccagtttacatacagaaaaagagtagttttttcaaactttataacctcttactttaagggcatatatgtttcaattaaataaaatattacacaaagctaacatatttcccacaaatttcttctcttctaggagttgattggtcatctgctgacaacagataagttcctaatttgaatggcattagtacttcataaatgaacaaaacaatgagtgcaaactggaaaaactagggagaggtgcatacaagctaccaaaaaaggttgggattgggggtgacctgcaagtcatgatctcatatcttaggatgtatcttagtattcaggaaatggaattcttggaaacatctgtttcacagtgaggttgggaggtcagacgatgctctgttagattcttcttaggattaaattacttcctaggactgcattaagacactttaggtggtatattaactcttccagaacaaataattccatttcagtaaattattgctacagttctctaaagagtactacggtgtcctggaaaagataatgttccttccaaaatgccctctagtcactcgaacaatgagaaattcatatttatcttagacactttgatccttgaagacataaactaaaaaagaactgtttttccctatctaaacagagactatctggatggagacataatattagatctgccctggtcatttggcagtgtataccatttcctccatgtgcttttgacaactggcatgcttgattctttccctgtaaatcagcctgccattcttctttgcatgcagaatggtctataggaaccaagaaaaaaccaaccccaatagccaatcttttaaaaaataggtgaatgagtggagcatggcacacaatgggaagaaaaggagtgatagttaattaactttctcagtgattatctcccatattttgatatgggagataaaaatcttccatatcaaatctttacaaatgatgggtaatctgtaagaggaattctcctcctccctgcacccccactacaaaactcccacccaaacaaaaaatcaaaacccaaccaaaaacctcctctgaaacttctacttcagatatgagatcatggtctggaggctactcgtaccaaataccagttcattctagtacagcagttcatgaggcaaaaggctaggagtatttgtgacatgactttacaaataatgtaaaaacaataaccctatgattatgggcaataattttccccactcaaatctatagatattgcactgaaactgacacaatggagaagacatagatcatttcctgttgaaacccaattacctcaaggtaaaacaaaacaaactccatttaataaatgaaatattacttaaatgttttcattttagggtctgttccctttcccctttatattctggaaagttatatgtctaagtatacttgttttgttacttcattagtctatcaacttcatttccagagactataacgagaatggaatggtttgtaccttttttctgaacataattgagtcaaggagttttgttattttaggtattattaatttgattaaaacatagaaccaaagttgatgggaagtagtagctttcttctaggtaaaagagcttactagcagattttataatcatcggacatttattctgtcctacctggaaataaattatgttactgcttggcatgggaaaaggcattttctagtaatttcctgtgacaggaggcacagcaatagtccaagtaagcacccaacaggtgcttgggagtagttttaaactttaacttaatgaaaacatttacctcagtacttttgtttgagaaagaattcagcagcagttatagttaatatcccacctgtggagagctgcgatcaccctaggaggtgggccaaccgaggagcactttccaggtaacaagagcaacactattgtgagaagctacaaatggtactgcagtaggtgtagtgaacactactatagtgatcatggcctgggttatgttccaaatactaatgcaaggaatacactagagtttataggattagaatagtttccttatgctaagaactagtagatggcatgtgatgagtgggtatggtccattttattctatttcactctacgagtttcctagttatgtctcctttctcctatgttaattatctatattccatgacagttattttccctatctaaaataagaacggtgtaactatggagtaccccaactcacatacacatacttgtgcacccttagactcatgtatggataatctgtgtaaagcgctcatttgcaattgggtgagctcactgaaagcagccatatcagtcttccaaatacagtaaaagccaacgaaaatccatatcaactgtttatttctaatatgaaacagtaaaccttgtccatgtggtaattaattcaaatgccttttgtgttttcttgtgaagtcatccaaagcaaaagtctagatgactgctgacatgatatgcataatctaatgaactcacatctctgtttattttgctcatcccacagttgaatgacacactgactgctgagacacttgggttgatttagaacggctattaatgaatctataaatttggctaaggttgatttgactttctagggaaaagccagcctatcttcaaatggacagctccctccacataaacgtcaatgtaccctaaagacaaaactaagtatatgtatatacgggatatatacatatatatgtacacataaaatggattgggaagtcctttggtttagacagtattaaatatgtacttcccaagtgcataggtttcctttgaccaacctgttcaaaaaacaagcatgaaaagtgccatggcacatttcccatgtctttccccctatttgaaggacacctttccttgcttctccatcactcctaagcattttatttttaaaagaagctggttattttggccttctatcttaacactccattgattcatccattccttggaagagctctcagattacatccagaaacttgtttttagaggagaacaaggttgcaaataactttttcctctttttttattccctcttccccccaagaagcaggcaccttgaagtgtcatgaataatgcactcttgatctgacttgccttgttacccctggccagcccaagcagctgaggtctgagctttacttgccctgcatcattgtgcaatactggaaaagaaaaataatccactggtctatacccctcatactgtggtgacgtgatccgggttctcttgaatttctatgcattcaatttcctctctctcctttcgcttggcacgtttctttttcttgtggtgctttttggaaggggggaaaaacgttaggaacacaggtaaaataacaaaacagtgcagaagtgtgcaacccccagtgagcagcaagcatttgaacagtgtgaaggtcaggttcgaaggcacaaatagaagggggactaacccaataagaaaagaagtaacattttgcaaaatggctgtcccatggtcttgcaaggagctttttatacattgtgttcgggtgtgctcagttgctaatacaaatgtgaaaagcagtggtgcacagtggtcaatggcgaaattcaaggtgtagataaggcacaagatagaaatgcaatccatgtcgacgttccataatgtcattaagcccagaacgcccagctcaattgaggtgacgctaagaattagccagaagtttcccagagggtggatcactaggaaaaaagtcaggattaacaccaggagaacaccaaagcctgcaatcagaacaggcactgtgacagacaagctgtaatggtccatgaagacaaaggaggggttgaacacgatgaatcggatgctctttgagagggataggggcctcagcttttccaacacttctgtgatttctttctgcttgtctctgctagtcctggccaccagatacaagcgagaagcaatgatattgctttcatcccctgccttggagaagatgatatcatttcgaaaatgctggaattctggcttttttaaaaatgagctttgcaggacactgatgaagtcacttttgttattggcactgacgttgctgactttcaggaactggtagtactgctccacccaggacactgcagtgaatccactacagagtcttcttaggtcatcctggacgctgctgttccagtactctaggggctcatagacgtagaatcctatcacagggctatagttgctgaaatatttctgctgaaccatggcataggaaacacttggcgaatcactggctagtagattgatgatgttggctccgtcactgatctgtaagcaccccatgaaggagaaggaggcataaatgagatagaggatgacaacaaatggcttcacatatatattggtaatccattcattataatgttcacggaggaagtgctgaatgaagtggtgctggtaggggttcgtctcatgatgggacgtctgttgatgcccatcactcatcactgtctggaaccacacaggtttgcgatccaggtattctgcagaagggatcttacagcaaaagatgctgtggtagcggttttgctctagttggccagcaaagaccagacaggagccaaagaaggagaaaatgtagaagtagttcaacagaatagagacacacatgttttgacagaagaccttcacagcctctatgtttgtgaatgggctggcacccatgccaaaagtgatgaagtacagggagctggtcatggtataggtgaccatcacatcagaataggcatctgctatcctgtctttgaagggcaagttctctttggttctccgccatccggacagaagctcaaacactcctttagttccatgacccatggcgaagaacgggattcccagcagggtggagttgtactttccatcggtgatgaagaagatccctgctgctgtgatgatggagatgcatactgtgagcacccccaggaggcccaggaagggcttactgcgcaagcagtccttcatggagctggagagggtggctgtggtcaggatcagcacgaggctcaccaggaccttgcttctggccaggatgctggtcttatgaaagtccctccagaggctaaaggatgctaaagagtagagctggagttcttgatgctcctcctggagcttccttataagcttacagaactcattctcccacttctcccctatgaggtcttgggtggcagagccataggtctggaggtagtaggtgatttgaatggctctggctgacttgacccgctgatctttgctgtttggcacttccactaccccgcccagttggtgtccaataaaactgttcctcccatcctttaatttagtgttgggatacctcacttgcaccctggctgttgtcttattggagacggcagcctgcctgagatcctctagcactgaaataatatcatccagcacgcatttcttatcctgatttctcaacacacacagatgggaaaaagtataattatagcccttgtggttcaccttcatttccagcacggctcggtgggtctgcaggatcccctcagcctggagcaaaatattgtccccggttggggagaggaggatcaccctgccatacctcccaggggtgtgtaagtccgaatagagctggcttttggactggtccagggggaaaaggctgctggccaggctgcgctcgatcttggccaggctgtggctgggagcgaccaggcgctccaggtcgccctcgggctggaagcggttgagcgcgctgaggccgaaggtgattgtcaggactgcgggcacggtgaggaaaaagaccgggtgccggctcacgcacaaacccagcctgtggcagaacgactggagccctctgcgaagcacctgccgcagcatcctccaccagatccagctcgcaggcgctcccggccgtcttaaaaagcacat

SEQ ID NO: 10508 - RNA, 21574 nt, Homo sapiens
  source 1..21574: mol_type = other RNA
cctgtgccttttacttctttaagcctgagaagcagcaggctaccaattgctcccatttaaggatgtggctgccatgataatctttcacttgttcagcagtatttctttttctttccattgacaagctaggatacgagcacagtccctgctctgccaaaggaaaccatgtcttttgttaaagtttaagctactgataaatatttaagggagtgcaggggtagatgttaatattacctagcaaagaattcatgggcaaacaactttcaaatgtatcagtaagtttaccttaaaatgacttactagataatgagatacatctaatatatttgcaactgaaacacttgaagctttcaaggtctacctgaactaatttcttccctccctccctcctttccttccttcctttgtcaaatatttattgaatgcctaacatgtgcctggcacccttcagggtactgggcttatagcagtttacagagcagaaaaatatctctgcccccttagagctttcaatttactggggacagacagacaataaacaaatcccatgacaaatatgaaagaagggaggagatttactatattttcatgagattgtcaggaaaggcctctctaatgcatacttatttaatatttaagaagaaaccaaaaagatgtgagggaggaagatctgtggctaactgggggaagaagagcattcagggtggtgggaactgcaatgacaaaagaccaaagggggtgcatggttgatgcagagagaacaaagggggcagtggctggagaagtggtcagagcaggagacaggggaacagactgggtggggcttcccctctttcgtgaatctcccacccaagttaatgtctgtgaagagatggttcttttgtttaggcagataaaatgccttcttcaaggcctatttgaagctgcatttccttcttgaagtattcccctttaatgccaatagttccctatacccagattctcttaactctaaagtatgaatcatgcaatcatttcttgtgctttattgtgagtgactatttcttctgtcagcatctttaaagagattgcaagcaatttaaaggtagaaaacacatcatactttttcttcatcccatatagcacatgatgttaaactcaaggtaatcaagaaagaaatgaaagaaatatataaaactgtcaattaagaaaagacaaagaaatatatgactctaaaaacaaattcaggtattttgagaatatagccatgaaaacaaaaacattaaggtagaactcagtggataagacacatgatctgattttgtttagtaatctacatcattgcttatcccaacttagagcttatacctatacatctgtagatctcttcttcctgtcctacagaaaatgtaatccctcatccatgcagccttctttctttctttacattagcactactgcccattcttcacaatgtctatcttcctttatgattttttttctctgaactcatatcttcaatttcctagagtattgttacctagcagggtcagggctattagtggagcagaaattataaacatttgagagacataggtagagggttaaaaacccactagtctactagtttatttcactcattgcttgggatttatctacttaagcaaagcaattaggttacaaatgaactggcgataaaatactttcataaaaattatttatcctgagataaactctttatgatttttagacttgaaataattttatatacttttaaaaatcagttctgtatctaaggtagtatagtccaactaagaaacagagttgatgtgctccatgctgaggtcgaatgaagaagatagaaagtgcccctggatgcctctctaatcattattttagtggaacatttcaatcgcagtctaattattgagctctcccaatccctccagtgctaaatttcaaacatgttggaacttggcgtgaagaagggcaagattgtttttctccatctgtagatgaattcttctttttacctaaactacttagtcctgatttttctttaggccatccttctaaatatgtcttagtcattgctgtgctaaatagaagaggtggcaacagggtagaaaacgactcattaacactccttgctgatgttctttcataaaactattttttaaaaaaattttatttgtgtctcaattcttgcctgactgtttacttactagtatttatttcttttgggtaaaattatgagtttgggaacctatttacacttacattcactaatttgtttaagtgtattaatttcaaacaaaaagatgtataccctcaaggctgtatctgctgtgtttaatacactaatcaatcattaggcatccttgccttcctatcttaccattttgtccaaaacacatctagtactcattgacatttatgtccaacaaacaaaaaaatcagtatagcaacttctatttattatggaagacatgttaactaagaatcttgaacaatttttagattaatagcaggttaattaggttaatagcaggcaaataaataataactctagttttgccaatgtctcataacaaatgtttcagtgaaagcaaatagttactttcttctttttatgagacattaaagtattccgctgagcaatttgaactgctttgtccctcacacaggactttgtacatcacttggcacattataggttcttaatccatgtttgttggatggattaatgaatgaatgatatggctagttcatcaggtcattttattttcctagttcctaggtaactgtccatatttcctgttatcgaaaaagttcttccaatcagttattctctttgtcgacttttagctgtgacttcctattattgaacataacccagtactctaagtattcgaatttaatacaaaaagaaaatctattggaacatttggtaagagatatttgacttacatattgtgtgtaactctgattggagtttcagcacttctttattgtataggtatgaccaagttggcctttaggaggcctgatggatttttaatgaattatcggttttgccaatcattacttttgttgcattatggctttttttttaatatcttgggtctggcgtatatcatagtttagtagctgtgctgttgggaccaaagatctacttacaaccattttcaacacatactaaattttttttgtaggctgctttcccccttttcccttcattgaagttctccaagaaataaccttcctgaagtcttttattcaagatcaaaatttttcaattattctagaatgctatatcattttcaaaagaatgaaaaataaaatatcaacctgtttatttatttggtttcctggccatttgtcaatttttttcttcatattttactatttatggtctagtttaacttggtttccatttgcttacttctcattccctgaaattgtactgggacagaagggaaaaattagttctgtgttattttaattgaaattcatgctgatgaatcatttttccttaagtattcttttcttctattaggttataaattactcaaatagctagaaatcagcaatattgtttagaaaataagaactgatttccacacagacccattaatactgtttcctttggaattgtaatactcatctgctcttcagtaacaaagacaggcttctctaacatgacattatcaatgtttgcttcctggaacactagttctttaagatgctccatgaacataatgacccatggtcaattatatctgggaaatcaaatactgtctttatgctactggaacattaatttcacacattgagggtaattcaaagaataggcttcattttgccagtgttgaagccattttaatttcaagtagcatttcgtgataatataggaacaaaaagatcttcaaattctctgggcattcattgtacttaactttttacttaagagttggtatttatcaatatgatttttgtgttgtatctgagacttatgtggtcccacatgcaggggcagatcaaaattttgttgagcctgaagtgtatacatttttggagtccccttttaaggaaaagaatgcaaaaatatcatacatttgaaaattttatataaacataagatgtgaacatactgctaaggactgtcctagggcctccaaaagacttatgtaagcaatgggctcagaaatttaagcttcattagctacatgctacacttgcatatcccacatgaaaaatagtactttactattatttggcctaataatataatagtgtttcagcctcattatttctggttcttttctccacctgacacataccctacattcttagggttgtgagatttagcaagtaaaaatgcaatatgcccagttaaatttgaatttcagagaaacaagtatttttagtatagtagattccaaatattgcatgaaacatacttgtactaaaaatttcattcactgattattggaaattcaaacttaactcatgtcctacatgaatctagttctagtatagagtgctagttctagtatacagtggttctagttaaaccagtctataacaggacttctctgaaaatgacacattcttttatactctacgccttggttccatgttcctaaattttcttcatgaaaagactgtccagagcaacttattacaaatagagattactaaggccatcccttcaagagtttaaaaagtcttctagatgagttctaccaacaggtagacttgtcagatatggccttagttcaggtaatttcttttcttcaaactggaatgtctttgcactcttcaactatgcagcctttcaggcctagtggtgagaagctgacctttgtcctcaccttcttccctggacagatttaatccaactattctcagaatgtctgttgctgttcacaaacttagatttcagagattttcaaagtccaagtgtggttcctcagactagtagcattagcatcacctgaaaacttgttagaaatgtaaattttcaggcctcactccagatctattgaatcagaacctctggagatggggatatgcaggctgtgctttgacaagccctccaggtgattttgatacatgcttaagtgggagaatcgctgctctataaatggagcccattatttttgagatatatatatacacacacacacacatatatatatatggctatttcacctactagtttgctttgctaaaatccttgatgggtagtggctgcctctcatttctctttgcatttactctctatgtgtctggcacatagaagatgtttaaaattcttcttgaatgaaagatttggagaataaaggggttaatagataattacattttttttgagtaagctacctggtgaaagccatgacccaaagggcatcgcataaagctacgtggatgatcaagctgctgtgtggccccattgcatggcactgtggctccaagttccaactcttttacattttctcaagttgttatctgcttcctcatcctcacgtattttagttctatgactgtagaagaatacaaagagttcatatggattattttcacaggtcattttaatgctaatgttaaaaccatgtatgtgtgaaatatttgacaggacaattataccataggaaaagttttgaattagagacaggccatccaatgaatgtgtaactatgtgtaaggatatgttgtgaaaattacattttacatatatatccatctttgtccagtgctgacataacattgcaatactacatctttatggtagaataaaagcatgtgccttatacataactttcatagaagatgactgcagagcagatctctgattgtgggaggaacagtgatcttgtttctaagcataaatcacctgaactgctaaattccctgaaatgcaaataaatctcaagaattatttgctaattaaattgatgtttatatatgtagattaatctagatactattgtagtgtctctagctataatacgtgcatgtagataagagttatatatacctgagtatccagtaattttacatggaaaaaagtataaaagattagactgcctatttatgttcctaagatattcgtttcttcctctttgactcatcttttatttactgaatttaattaatgcaatataaaccatttttccccaagttagatatgcagaaaaccaaatcaactgttctgtaaagataaagcaatttcctgaaaatttgtggtaaagctttacaaatgttataaaaatgggccacgctgcatgtcaaaaccacaggaatgtgaagattaaactatacattagagtattgtagtaaatagatcacacagagctaataactagttactgttataccacattaaattcactaatgtgaatattgttgtgttttagacactcaaagttcttgggtgttcaggccatcttacagatataagttttgtgaattgtatttatttcttcctttttatattcagtgccacaactctatttcaggccaatattaccttcattgctgatgaccacaacagcctcctaacttaattctttggttcaggtctctcatctccagtctaacctacacttagaacattgcagattaatacttctaaattttgaatctaataataataataataaaaagtaatctgagtccatcaaatcaaatataaattctgcagcatgatgtttgcaggtccttatatgaaactttctggtttgtacaaattcaactcctgtactggaaatgtaccctcaagctaaattgagttcgttgacccaggaacatattctgtgcttttgttgcatgttatggctttgctcagtctggtcccgtcacatggggtgctcaggccaataatcttacctcatcttaagtgctatcttaatgcaacacactcataccaggtttggctctactagaaatcatctctctaccctctggatatctccttttggactctgtacaagttctggcttatattctagttatagatgtcacagacgcttttgtcttgtgactttttaaaacttcacttaataaaaggctctatcagtatttattggattaaatgtgttgacttggttgtctaagccactgtttttcaaattgagccacacattgaaatcactatgggaactcccagaagtactgaggttgggtctcgctataggatatattgatttaagtagtctggcatgaagtctgggcattgagactttaaacatctctctaggtcattccaaagtacagcaaattttgagaaccactagctttgttactcctagggttatccaaaatgtctcttagagtgtgtttgttgaccatggtctcgtatggccacttggttgttggatttatctccattctacttctgtgaacagatgtcctcctcgtgaaccagttggaaaatggggcctccccaggccaactccaaccttatctataactctaaaaagcataattaggaaatgcttttttcaggtttaaagtttaaaatatattcctccaaacatcttgtaatatgattgctggttttggggagcaccactattataattaaaactttaactattaaaaaggacaagggtaatgtataaatcagttaggtttatgcttaaaaactaagtgcatatgtaccttatgtgatcttcaaagaaagcatcagtgaatcataaggaagtgaatttaaaaaatagttttaagcattttaacaaactcattgtcttaaaatttacatttagaaaaggatagatggggagaaaatctatgcagttatttttcatcacatataatttacatttggacttctctgtacatgcacctttcatactgatttatgatgaaaagatgatatattttaccatagggacatagtacttgtttacaatgttttctttctgggaacaatctataaatcagggacaataatacctattctattaggcaggtattatttgaattgttaattaaaataatattaacagagatagttaattggagtgtattagtttgagctgtttgttctggagagtttgggttcccagcaatccatgtcagtctcttactctcacactttgagggcttttgtgccagaacgtggacggtgttccatcatcaggagaatcaaactcatgctctaaactggctcttgcaaccactacatttcaaagcaagagagattataaatttatgtgatattgctcagttttgggatccttgattttaacagttaaaattcaaaaatagagactgtgtatttacattttgtaaaccattcactgcatttaagcccaaggatacatcataaaaagagctttttctttatgatccctctccaaaatccaagtaactccccatatcctggcaatgctttataataccactcacaatgggcgcttcctttttattcccatctgtaacaagtctcttctgggttgctatcatctcatctgttatagccttcatcctggacaacctgctttcctgcccttgtatatttcactttttctccctgactgttgagcccatcctccatctctatctattagaatcttacccacacttcaatgtggatcagttcataattccttccttactttccttgaatactccagctgcaaatttcctcaacagatcatgcatacctcaaagtcaggaactatgaatagtttagtggtattttcttctgagcctagcacagagaccaatataggtgctcctaaatatgaggtaagtaaataggtacaatcacaagccatctaggggtacttcagaaacccatctacatcaaatcttgatcctaaaatgggactgaatttctagttctatctttttaaagagtaacaaactttttggagacttagatatgtcagggtttttctgaaactttccaatgtgttcctttgtttttaaagcctaactaagctaatgaacagaaactaaataaaaaaaaggtttcagttcagttgtttagtcccttcttcaacagttttagatccgttttaaaattttttctcactttacctttttttttaaaaaaacacccttgtccttaatttttctttatgttggatcacattctcccttattttactatcaagatgtgtatagctctaggttgtagcatttcaacttataggaaaggacagttattaccaacaaacttgaaattcttcctttatatggggccttattattgtgtaactggctatataggaaaattcaagaaaatgaaacaaaacaacaacaaaagcttctgaatatgggctctcaaagattgaaattattaaataacctccttttcattaggtcatgagcaggcaactgataagctggagaagtcttttatatttttcttcactgaatggataattactgaacgtctgcaaagcagacattgtgtgcttcatagtttggcatgtcagttgccatttttaaaataaaatcagtggagaatttcaacttgaagcacatataaatgacaataaatagtacttttgcaaactttatttagtatttgcaaataggttccaaatgtccagcttaatttttctgagttcttatttcattcctttctagccatgcttatttttatgtaaaggagaaaacatgcttaattactctaaagaaaagttattttagaaatgataaaagttgaacatatttaaaggaaaaaagcagaataaaattaataattaaaatactaaatttggacaggaaaatggctattgaataagtccaaacatttccaggaaagacataaaggcatccttgtttttaagaaaacatacggcaaactatataaaatgaaatattactaagacttctttggtctcctcatcatacgtcaataatgaggagagctttgcaatgataaagcttttgaagtggcttgtggaatattaaattgtttaagtataattttggcatcaagtgaccttacatattttgaatgttggttatctatgcgttatgtataatgccaccacattattcatcaaaatacagtggacttggatattgaaatatttaacatgattggttttagtgacttagaagtggtgctgatagcccctgaacaattatgccccagcttgaaactgtatagcgtgcagccaaagggatgtgctttgtgattaatctctgggtactactgaggagccgctggctcactcattgtctccatcttctgcagctctcatatggtgagaaaaatgttggttcaagtatttttatagttaatattactacaataatgcaatgtaatgcagtgataaattttaggtagaatttatttgacccgattataaattgctgtagatttgaaggtaacataattattaaggggtgttaaagtgctatctgaatcttttagtaatgctttagtaatttatgtgttttagagacatttgtgaacttagggattcataaaaatatctctcaggaatgccaagacattttgtatttgcttcagaatgctttatcttaaccacggagagataattgatatatatcatcacagtattattttaatgtatgtattcttgaatgtttaaaggataaaaaattacattataagttttagaacttgtgattcaataaaatactaaaaaaacatagattatgttattttacattgtgatgttataagatgttttgtttaggaagtttaattcttagcctagaattaaaaggtagcatgctcgaagttctcactgaggttagaggaataagttgcatattataatattctgtggggcatttaatactaacaataaagaatgaagaaaaatctggcgaatttaagaataacctagcttttacagcatttgtgattgtgattttaaaagacctcatatttgaccctaagaactatagaatatacacctgtataatttatcactactttaatatataaattatttctattattatgactaatggaactagatttcttttgttgttaaaataaaaagttgagatagccagaaatgctgtttaactttgcctagtggcactgtagtaaatatgattttgatgacttttttttccaagtagctaagatttaattgttatttttcttaagatttgtacctgtaagctttagataatagatttgtcatgcagataaattatgagcaatttaactaaaattattgtatttcagtgtgtccaaaacatgaaaataatgatgaaccgaacaaggaaatatttggaacataatttcccttgactgaggtatgagattcatttaattattaaatgtgtgtttacacatgcaaatctatgggaaataatttgttctttatttgtttctattatagttaagaaaaacctgttttgcaaaatgttttttcactgatcaacatagaggtaaattttgataatggaccaaattcaggtgaattggaaactttggaaactttggaaggacttttggtttgggttcttagtaagatcaaaaataggtacttttagaatattttcttctttgtgagatctaaaatggctacacagcagtcttctatttcacaggagatatttttggatggaaatacaacttgggtaatgtttttttgatttgacatttttgttcacaattcgtttttaagctttcctcagtaaggtagctttagttgtagagcccaaggtacagaactacagagcagaaacctaaaatggctttgtttgtactattttgggagtgataaatgaggctgttttcatgaatgggatgaacctatatgtaatagagtattttagaaggaatattgttatgggtaaagacatctggaattgatggtttgccatgaggtttgtagtgttaatacatcaaagtttcataatttcatacatttagtcacccttctttgctgtagaaactggtattttgtctagctaggattaagaacaagtgggttttgttttaggaaagaaaataaaaatgctcaacttttactctcatttctacaatttgtctatgcatgggtgaagactgtttctccctaggagttttcttttcactgatgctaatgtttccgtaagtgacttgtgttttaaaaaccccgatttagcagaaaataatagcaatgccttccagaggaaaagaaaacttaagtaaaatgccaaataatggtaactttgtctctttctatttgcctagaataaacaaacaaacacccgaacagattttttcctccaagaaaagtgataagtgaaatgcacttggaatttttctgaagttattcacagattatttgtgcatcttactgggtagactgctgcctctaatcaaagtcagattactctctttctgagtcaatttttgagctctgggatatctgtagggagacaactaacaactgccttgaaagatttcatattaatgaatattatgttaaccagaatgtataagtgggactgcatataggagtgctcattttacattttgccttgtctaatttgataaagtgaatgagcatcaaggaaaggtgataaataatattgctttgtggctttaatatattgccatttaatcaaagattgcatgccattttgtctttaaatacccttatgaggtagcttggagagatctctgcccttttcaatctgtgacagatttcctagttcagagcaaaaaagtctactgctgaaaaatatgcataattaacaggaaagtataataaagttgttgcttaaactactaaaactttgggatatttgcattgactagtttaaggtctagtttatcagtttgtagcacatttatgtttgtgaagaaaagatgccagaattcccttattctacttgaaaatagatgctacagactgtaccaggagatgcaagaatatgacggcttattcttttttttttttccccagctctatcagtgttgctaccaacaaccagtgaattcatcagataaaatgatagaaggtgtttccgtgtccagggagagattctagtaaccatattacattagataatttaaatgctccccataacatactgtagactgccgctactgagaatataagttaaatttatatagcactgaaaagttatacatttttattaaacaccagtaatctttcgtccatgagagtgtttcctagttattcctaggaaattcttcaatgcagtcttccaaagcattagaatttttttccccctctggtttgacagagccttgtgggcaatgtgcttactctacaaactgtggcaacagagggaaagaaaaccgtaatgctcctctattagaccatgccattagctgttgggaaaccagagctcagctacaaatggcttctaaaaacctcagctcagataagtgcaatgaaatcatacacagcaggaatcacacaccatcagtggtgattcctactctgttcctaaagtttctttctgatttttaagattttataattaccatgacctgtgagacctttcttaagggaaattttcaactggggaaaaatagtagaagctggctttctataatttaagatagtgcaaaatcagtgatagtttcctttataaatactttattatattaaaaatatctaccttatagaggttttcagtttaaggtacactcccatttaatttttacatctttagagatgcagaagacataaaatgtgatttgtagactaggaagttatactataaatatattcttaaccctatatattgctcttttgagttgttttccgttttataagaaaagcaagtggcttctctatcagcaatagagagtcctcattaagtatgaaaaaaactgattagaaaaagtgttcattatgactcaaagactcacaaaatatagtcaatgagagccactctgggaatgaatgatgcttatgtcggtgcttactttaagcttctttacaaagagtctccctagcttttcactttcactaacaaaagggtctacggctcttcctttgtgcttggaaattcaggagcacctcccactgcaaagattaggttatgaatctaacaaatgagaacccagtcttcaagtgcaatgtatttgcctatgatcaagtttgctagcagttgagaatctatagttttgcaacaccacgtgattctctctgctgtattctaaatcacagaatatgtggtattattccacttgttctatcacacctacttacagacatcttgatttctgagatgtgggctcatctctcaatatccttccagtgtcatttcaaatgttgcctgatctaactccacaacacttcaaacacagaacaccacctcttgtgctcctaagttaaacgtgatggtggattaatcttggtcctttagttgataaatcaaggtaatttactgctgctatacccatacacagtccctcccctgctggatctcatgcagtgtggctttgttgctttcacttatgattttgctgctttcatttgggtcaatatcattgtagttattttgtagacaaagtagtaaaaaacttgatttttccctatcctatatatctgcagctcactgatttaaaatattagcataaaggtccgcaccacagtgatgatgttcaatttcatattgagattgaagatggggaaatagcaagggcataccaattcagccataaatatgttttgggtcaatgtcataaaattgtcacaaaattttggtaattgagaaaaagctaaaactttttttgtttgttttttgtttgtaaagggaagaaaagtgcttctgaggctcttttggaataagtaacagttttcagattcacttttgcaaagattgccaatatccttcgcagacaccaacaaaccagactgaacagaaagatccctgtagtaggatgccgagcaaatcattgacttctccaatctctaagagacaatatctaaatgtcagtctcatggcattgtattttctgcttcaccataagattagcaaacacaagacataaaattatgtttatttactaaccaatacagaatatactaggccctttgcctggaagccagatttcacttctgagattttccgaagtccattctagaagaggtggttgttactgatacccagggaaggcaattcttaaattgcttacctggggatggaactttctgtggactttaggcccttaagaccaaaagccatgaggcatttatgaataggtgatgtaagaaattttaataaaagttgcaataaccctgaaaatagtgtctttaataacctatgtactattaataacaaagcatgcatagtgccgtgcattcataactatttggtcataaaaatatgtgactgtaattatgatatttacagtcaacttataaaaatacatgtaattctgaatggcaatagttaatccttagctctaaccacaagcctagaaggattagcttattacggggaaatgtgatagataattacaaaatggacaaagcttttactgtcttgaatttaacattcaagaataactataatagcatcataaaacatttgtcatcattattcttctcacctcacaaggtaaaaacctaaattctgtggaaataaatgggaatcaaataggaaagggccacttacatgatacaacaacagaggagaatagttctttcatagaatactcatgcacagccttcaaagaggttcatagtaactgcaagaattcctgggaagacatctaaacatgactttcattaaaaagaattaaggctggtctaaagaatcaaatctctaaggtatgattacctttaaccataaacggtaaaaaatcttttagctgatctctctgtaatttaggtgagtacctctttgaagtttattaacatcaaagagagtggagctcacatggcactttccaattcaaatttaaattctgatggaaggaaataaatccacattccagtttacatacagaaaaagagtagttttttcaaactttataacctcttactttaagggcatatatgtttcaattaaataaaatattacacaaagctaacatatttcccacaaatttcttctcttctaggagttgattggtcatctgctgacaacagataagttcctaatttgaatggcattagtacttcataaatgaacaaaacaatgagtgcaaactggaaaaactagggagaggtgcatacaagctaccaaaaaaggttgggattgggggtgacctgcaagtcatgatctcatatcttaggatgtatcttagtattcaggaaatggaattcttggaaacatctgtttcacagtgaggttgggaggtcagacgatgctctgttagattcttcttaggattaaattacttcctaggactgcattaagacactttaggtggtatattaactcttccagaacaaataattccatttcagtaaattattgctacagttctctaaagagtactacggtgtcctggaaaagataatgttccttccaaaatgccctctagtcactcgaacaatgagaaattcatatttatcttagacactttgatccttgaagacataaactaaaaaagaactgtttttccctatctaaacagagactatctggatggagacataatattagatctgccctggtcatttggcagtgtataccatttcctccatgtgcttttgacaactggcatgcttgattctttccctgtaaatcagcctgccattcttctttgcatgcagaatggtctataggaaccaagaaaaaaccaaccccaatagccaatcttttaaaaaataggtgaatgagtggagcatggcacacaatgggaagaaaaggagtgatagttaattaactttctcagtgattatctcccatattttgatatgggagataaaaatcttccatatcaaatctttacaaatgatgggtaatctgtaagaggaattctcctcctccctgcacccccactacaaaactcccacccaaacaaaaaatcaaaacccaaccaaaaacctcctctgaaacttctacttcagatatgagatcatggtctggaggctactcgtaccaaataccagttcattctagtacagcagttcatgaggcaaaaggctaggagtatttgtgacatgactttacaaataatgtaaaaacaataaccctatgattatgggcaataattttccccactcaaatctatagatattgcactgaaactgacacaatggagaagacatagatcatttcctgttgaaacccaattacctcaaggtaaaacaaaacaaactccatttaataaatgaaatattacttaaatgttttcattttagggtctgttccctttcccctttatattctggaaagttatatgtctaagtatacttgttttgttacttcattagtctatcaacttcatttccagagactataacgagaatggaatggtttgtaccttttttctgaacataattgagtcaaggagttttgttattttaggtattattaatttgattaaaacatagaaccaaagttgatgggaagtagtagctttcttctaggtaaaagagcttactagcagattttataatcatcggacatttattctgtcctacctggaaataaattatgttactgcttggcatgggaaaaggcattttctagtaatttcctgtgacaggaggcacagcaatagtccaagtaagcacccaacaggtgcttgggagtagttttaaactttaacttaatgaaaacatttacctcagtacttttgtttgagaaagaattcagcagcagttatagttaatatcccacctgtggagagctgcgatcaccctaggaggtgggccaaccgaggagcactttccaggtaacaagagcaacactattgtgagaagctacaaatggtactgcagtaggtgtagtgaacactactatagtgatcatggcctgggttatgttccaaatactaatgcaaggaatacactagagtttataggattagaatagtttccttatgctaagaactagtagatggcatgtgatgagtgggtatggtccattttattctatttcactctacgagtttcctagttatgtctcctttctcctatgttaattatctatattccatgacagttattttccctatctaaaataagaacggtgtaactatggagtaccccaactcacatacacatacttgtgcacccttagactcatgtatggataatctgtgtaaagcgctcatttgcaattgggtgagctcactgaaagcagccatatcagtcttccaaatacagtaaaagccaacgaaaatccatatcaactgtttatttctaatatgaaacagtaaaccttgtccatgtggtaattaattcaaatgccttttgtgttttcttgtgaagtcatccaaagcaaaagtctagatgactgctgacatgatatgcataatctaatgaactcacatctctgtttattttgctcatcccacagttgaatgacacactgactgctgagacacttgggttgatttagaacggctattaatgaatctataaatttggctaaggttgatttgactttctagggaaaagccagcctatcttcaaatggacagctccctccacataaacgtcaatgtaccctaaagacaaaactaagtatatgtatatacgggatatatacatatatatgtacacataaaatggattgggaagtcctttggtttagacagtattaaatatgtacttcccaagtgcataggtttcctttgaccaacctgttcaaaaaacaagcatgaaaagtgccatggcacatttcccatgtctttccccctatttgaaggacacctttccttgcttctccatcactcctaagcattttatttttaaaagaagctggttattttggccttctatcttaacactccattgattcatccattccttggaagagctctcagattacatccagaaacttgtttttagaggagaacaaggttgcaaataactttttcctctttttttattccctcttccccccaagaagcaggcaccttgaagtgtcatgaataatgcactcttgatctgacttgccttgttacccctggccagcccaagcagctgaggtctgagctttacttgccctgcatcattgtgcaatactggaaaagaaaaataatccactggtctatacccctcatactgtggtgacgtgatccgggttctcttgaatttctatgcattcaatttcctctctctcctttcgcttggcacgtttctttttcttgtggtgctttttggaaggggggaaaaacgttaggaacacaggtaaaataacaaaacagtgcagaagtgtgcaacccccagtgagcagcaagcatttgaacagtgtgaaggtcaggttcgaaggcacaaatagaagggggactaacccaataagaaaagaagtaacattttgcaaaatggctgtcccatggtcttgcaaggagctttttatacattgtgttcgggtgtgctcagttgctaatacaaatgtgaaaagcagtggtgcacagtggtcaatggcgaaattcaaggtgtagataaggcacaagatagaaatgcaatccatgtcgacgttccataatgtcattaagcccagaacgcccagctcaattgaggtgacgctaagaattagccagaagtttcccagagggtggatcactaggaaaaaagtcaggattaacaccaggagaacaccaaagcctgcaatcagaacaggcactgtgacagacaagctgtaatggtccatgaagacaaaggaggggttgaacacgatgaatcggatgctctttgagagggataggggcctcagcttttccaacacttctgtgatttctttctgcttgtctctgctagtcctggccaccagatacaagcgagaagcaatgatattgctttcatcccctgccttggagaagatgatatcatttcgaaaatgctggaattctggcttttttaaaaatgagctttgcaggacactgatgaagtcacttttgttattggcactgacgttgctgactttcaggaactggtagtactgctccacccaggacactgcagtgaatccactacagagtcttcttaggtcatcctggacgctgctgttccagtactctaggggctcatagacgtagaatcctatcacagggctatagttgctgaaatatttctgctgaaccatggcataggaaacacttggcgaatcactggctagtagattgatgatgttggctccgtcactgatctgtaagcaccccatgaaggagaaggaggcataaatgagatagaggatgacaacaaatggcttcacatatatattggtaatccattcattataatgttcacggaggaagtgctgaatgaagtggtgctggtaggggttcgtctcatgatgggacgtctgttgatgcccatcactcatcactgtctggaaccacacaggtttgcgatccaggtattctgcagaagggatcttacagcaaaagatgctgtggtagcggttttgctctagttggccagcaaagaccagacaggagccaaagaaggagaaaatgtagaagtagttcaacagaatagagacacacatgttttgacagaagaccttcacagcctctatgtttgtgaatgggctggcacccatgccaaaagtgatgaagtacagggagctggtcatggtataggtgaccatcacatcagaataggcatctgctatcctgtctttgaagggcaagttctctttggttctccgccatccggacagaagctcaaacactcctttagttccatgaccttgccccaaaccggtaagaatccgattaccacaaggatggatagttacccatggcgaagaacgggattcccagcagggtggagttgtactttccatcggtgatgaagaagatccctgctgctgtgatgatggagatgcatactgtgagcacccccaggaggcccaggaagggcttactgcgcaagcagtccttcatggagctggagagggtggctgtggtcaggatcagcacgaggctcaccaggaccttgcttctggccaggatgctggtcttatgaaagtccctccagaggctaaaggatgctaaagagtagagctggagttcttgatgctcctcctggagcttccttataagcttacagaactcattctcccacttctcccctatgaggtcttgggtggcagagccataggtctggaggtagtaggtgatttgaatggctctggctgacttgacccgctgatctttgctgtttggcacttccactaccccgcccagttggtgtccaataaaactgttcctcccatccttcatttccagcacggctcggtgggtctgcaggatcccctcagcctggagcaaaatattgtccccggttggggagaggaggatcaccctgccatacctcccaggggtgtgtaagtccgaatagagctggcttttggactggtccagggggaaaaggctgctggccaggctgcgctcgatcttggccaggctgtggctgggagcgaccaggcgctccaggtcgccctcgggctggaagcggttgagcgcgctgaggccgaaggt

SEQ ID NO: 10509 - RNA, 21896 nt, Homo sapiens
  source 1..21896: mol_type = other RNA
cctgtgccttttacttctttaagcctgagaagcagcaggctaccaattgctcccatttaaggatgtggctgccatgataatctttcacttgttcagcagtatttctttttctttccattgacaagctaggatacgagcacagtccctgctctgccaaaggaaaccatgtcttttgttaaagtttaagctactgataaatatttaagggagtgcaggggtagatgttaatattacctagcaaagaattcatgggcaaacaactttcaaatgtatcagtaagtttaccttaaaatgacttactagataatgagatacatctaatatatttgcaactgaaacacttgaagctttcaaggtctacctgaactaatttcttccctccctccctcctttccttccttcctttgtcaaatatttattgaatgcctaacatgtgcctggcacccttcagggtactgggcttatagcagtttacagagcagaaaaatatctctgcccccttagagctttcaatttactggggacagacagacaataaacaaatcccatgacaaatatgaaagaagggaggagatttactatattttcatgagattgtcaggaaaggcctctctaatgcatacttatttaatatttaagaagaaaccaaaaagatgtgagggaggaagatctgtggctaactgggggaagaagagcattcagggtggtgggaactgcaatgacaaaagaccaaagggggtgcatggttgatgcagagagaacaaagggggcagtggctggagaagtggtcagagcaggagacaggggaacagactgggtggggcttcccctctttcgtgaatctcccacccaagttaatgtctgtgaagagatggttcttttgtttaggcagataaaatgccttcttcaaggcctatttgaagctgcatttccttcttgaagtattcccctttaatgccaatagttccctatacccagattctcttaactctaaagtatgaatcatgcaatcatttcttgtgctttattgtgagtgactatttcttctgtcagcatctttaaagagattgcaagcaatttaaaggtagaaaacacatcatactttttcttcatcccatatagcacatgatgttaaactcaaggtaatcaagaaagaaatgaaagaaatatataaaactgtcaattaagaaaagacaaagaaatatatgactctaaaaacaaattcaggtattttgagaatatagccatgaaaacaaaaacattaaggtagaactcagtggataagacacatgatctgattttgtttagtaatctacatcattgcttatcccaacttagagcttatacctatacatctgtagatctcttcttcctgtcctacagaaaatgtaatccctcatccatgcagccttctttctttctttacattagcactactgcccattcttcacaatgtctatcttcctttatgattttttttctctgaactcatatcttcaatttcctagagtattgttacctagcagggtcagggctattagtggagcagaaattataaacatttgagagacataggtagagggttaaaaacccactagtctactagtttatttcactcattgcttgggatttatctacttaagcaaagcaattaggttacaaatgaactggcgataaaatactttcataaaaattatttatcctgagataaactctttatgatttttagacttgaaataattttatatacttttaaaaatcagttctgtatctaaggtagtatagtccaactaagaaacagagttgatgtgctccatgctgaggtcgaatgaagaagatagaaagtgcccctggatgcctctctaatcattattttagtggaacatttcaatcgcagtctaattattgagctctcccaatccctccagtgctaaatttcaaacatgttggaacttggcgtgaagaagggcaagattgtttttctccatctgtagatgaattcttctttttacctaaactacttagtcctgatttttctttaggccatccttctaaatatgtcttagtcattgctgtgctaaatagaagaggtggcaacagggtagaaaacgactcattaacactccttgctgatgttctttcataaaactattttttaaaaaaattttatttgtgtctcaattcttgcctgactgtttacttactagtatttatttcttttgggtaaaattatgagtttgggaacctatttacacttacattcactaatttgtttaagtgtattaatttcaaacaaaaagatgtataccctcaaggctgtatctgctgtgtttaatacactaatcaatcattaggcatccttgccttcctatcttaccattttgtccaaaacacatctagtactcattgacatttatgtccaacaaacaaaaaaatcagtatagcaacttctatttattatggaagacatgttaactaagaatcttgaacaatttttagattaatagcaggttaattaggttaatagcaggcaaataaataataactctagttttgccaatgtctcataacaaatgtttcagtgaaagcaaatagttactttcttctttttatgagacattaaagtattccgctgagcaatttgaactgctttgtccctcacacaggactttgtacatcacttggcacattataggttcttaatccatgtttgttggatggattaatgaatgaatgatatggctagttcatcaggtcattttattttcctagttcctaggtaactgtccatatttcctgttatcgaaaaagttcttccaatcagttattctctttgtcgacttttagctgtgacttcctattattgaacataacccagtactctaagtattcgaatttaatacaaaaagaaaatctattggaacatttggtaagagatatttgacttacatattgtgtgtaactctgattggagtttcagcacttctttattgtataggtatgaccaagttggcctttaggaggcctgatggatttttaatgaattatcggttttgccaatcattacttttgttgcattatggctttttttttaatatcttgggtctggcgtatatcatagtttagtagctgtgctgttgggaccaaagatctacttacaaccattttcaacacatactaaattttttttgtaggctgctttcccccttttcccttcattgaagttctccaagaaataaccttcctgaagtcttttattcaagatcaaaatttttcaattattctagaatgctatatcattttcaaaagaatgaaaaataaaatatcaacctgtttatttatttggtttcctggccatttgtcaatttttttcttcatattttactatttatggtctagtttaacttggtttccatttgcttacttctcattccctgaaattgtactgggacagaagggaaaaattagttctgtgttattttaattgaaattcatgctgatgaatcatttttccttaagtattcttttcttctattaggttataaattactcaaatagctagaaatcagcaatattgtttagaaaataagaactgatttccacacagacccattaatactgtttcctttggaattgtaatactcatctgctcttcagtaacaaagacaggcttctctaacatgacattatcaatgtttgcttcctggaacactagttctttaagatgctccatgaacataatgacccatggtcaattatatctgggaaatcaaatactgtctttatgctactggaacattaatttcacacattgagggtaattcaaagaataggcttcattttgccagtgttgaagccattttaatttcaagtagcatttcgtgataatataggaacaaaaagatcttcaaattctctgggcattcattgtacttaactttttacttaagagttggtatttatcaatatgatttttgtgttgtatctgagacttatgtggtcccacatgcaggggcagatcaaaattttgttgagcctgaagtgtatacatttttggagtccccttttaaggaaaagaatgcaaaaatatcatacatttgaaaattttatataaacataagatgtgaacatactgctaaggactgtcctagggcctccaaaagacttatgtaagcaatgggctcagaaatttaagcttcattagctacatgctacacttgcatatcccacatgaaaaatagtactttactattatttggcctaataatataatagtgtttcagcctcattatttctggttcttttctccacctgacacataccctacattcttagggttgtgagatttagcaagtaaaaatgcaatatgcccagttaaatttgaatttcagagaaacaagtatttttagtatagtagattccaaatattgcatgaaacatacttgtactaaaaatttcattcactgattattggaaattcaaacttaactcatgtcctacatgaatctagttctagtatagagtgctagttctagtatacagtggttctagttaaaccagtctataacaggacttctctgaaaatgacacattcttttatactctacgccttggttccatgttcctaaattttcttcatgaaaagactgtccagagcaacttattacaaatagagattactaaggccatcccttcaagagtttaaaaagtcttctagatgagttctaccaacaggtagacttgtcagatatggccttagttcaggtaatttcttttcttcaaactggaatgtctttgcactcttcaactatgcagcctttcaggcctagtggtgagaagctgacctttgtcctcaccttcttccctggacagatttaatccaactattctcagaatgtctgttgctgttcacaaacttagatttcagagattttcaaagtccaagtgtggttcctcagactagtagcattagcatcacctgaaaacttgttagaaatgtaaattttcaggcctcactccagatctattgaatcagaacctctggagatggggatatgcaggctgtgctttgacaagccctccaggtgattttgatacatgcttaagtgggagaatcgctgctctataaatggagcccattatttttgagatatatatatacacacacacacacatatatatatatggctatttcacctactagtttgctttgctaaaatccttgatgggtagtggctgcctctcatttctctttgcatttactctctatgtgtctggcacatagaagatgtttaaaattcttcttgaatgaaagatttggagaataaaggggttaatagataattacattttttttgagtaagctacctggtgaaagccatgacccaaagggcatcgcataaagctacgtggatgatcaagctgctgtgtggccccattgcatggcactgtggctccaagttccaactcttttacattttctcaagttgttatctgcttcctcatcctcacgtattttagttctatgactgtagaagaatacaaagagttcatatggattattttcacaggtcattttaatgctaatgttaaaaccatgtatgtgtgaaatatttgacaggacaattataccataggaaaagttttgaattagagacaggccatccaatgaatgtgtaactatgtgtaaggatatgttgtgaaaattacattttacatatatatccatctttgtccagtgctgacataacattgcaatactacatctttatggtagaataaaagcatgtgccttatacataactttcatagaagatgactgcagagcagatctctgattgtgggaggaacagtgatcttgtttctaagcataaatcacctgaactgctaaattccctgaaatgcaaataaatctcaagaattatttgctaattaaattgatgtttatatatgtagattaatctagatactattgtagtgtctctagctataatacgtgcatgtagataagagttatatatacctgagtatccagtaattttacatggaaaaaagtataaaagattagactgcctatttatgttcctaagatattcgtttcttcctctttgactcatcttttatttactgaatttaattaatgcaatataaaccatttttccccaagttagatatgcagaaaaccaaatcaactgttctgtaaagataaagcaatttcctgaaaatttgtggtaaagctttacaaatgttataaaaatgggccacgctgcatgtcaaaaccacaggaatgtgaagattaaactatacattagagtattgtagtaaatagatcacacagagctaataactagttactgttataccacattaaattcactaatgtgaatattgttgtgttttagacactcaaagttcttgggtgttcaggccatcttacagatataagttttgtgaattgtatttatttcttcctttttatattcagtgccacaactctatttcaggccaatattaccttcattgctgatgaccacaacagcctcctaacttaattctttggttcaggtctctcatctccagtctaacctacacttagaacattgcagattaatacttctaaattttgaatctaataataataataataaaaagtaatctgagtccatcaaatcaaatataaattctgcagcatgatgtttgcaggtccttatatgaaactttctggtttgtacaaattcaactcctgtactggaaatgtaccctcaagctaaattgagttcgttgacccaggaacatattctgtgcttttgttgcatgttatggctttgctcagtctggtcccgtcacatggggtgctcaggccaataatcttacctcatcttaagtgctatcttaatgcaacacactcataccaggtttggctctactagaaatcatctctctaccctctggatatctccttttggactctgtacaagttctggcttatattctagttatagatgtcacagacgcttttgtcttgtgactttttaaaacttcacttaataaaaggctctatcagtatttattggattaaatgtgttgacttggttgtctaagccactgtttttcaaattgagccacacattgaaatcactatgggaactcccagaagtactgaggttgggtctcgctataggatatattgatttaagtagtctggcatgaagtctgggcattgagactttaaacatctctctaggtcattccaaagtacagcaaattttgagaaccactagctttgttactcctagggttatccaaaatgtctcttagagtgtgtttgttgaccatggtctcgtatggccacttggttgttggatttatctccattctacttctgtgaacagatgtcctcctcgtgaaccagttggaaaatggggcctccccaggccaactccaaccttatctataactctaaaaagcataattaggaaatgcttttttcaggtttaaagtttaaaatatattcctccaaacatcttgtaatatgattgctggttttggggagcaccactattataattaaaactttaactattaaaaaggacaagggtaatgtataaatcagttaggtttatgcttaaaaactaagtgcatatgtaccttatgtgatcttcaaagaaagcatcagtgaatcataaggaagtgaatttaaaaaatagttttaagcattttaacaaactcattgtcttaaaatttacatttagaaaaggatagatggggagaaaatctatgcagttatttttcatcacatataatttacatttggacttctctgtacatgcacctttcatactgatttatgatgaaaagatgatatattttaccatagggacatagtacttgtttacaatgttttctttctgggaacaatctataaatcagggacaataatacctattctattaggcaggtattatttgaattgttaattaaaataatattaacagagatagttaattggagtgtattagtttgagctgtttgttctggagagtttgggttcccagcaatccatgtcagtctcttactctcacactttgagggcttttgtgccagaacgtggacggtgttccatcatcaggagaatcaaactcatgctctaaactggctcttgcaaccactacatttcaaagcaagagagattataaatttatgtgatattgctcagttttgggatccttgattttaacagttaaaattcaaaaatagagactgtgtatttacattttgtaaaccattcactgcatttaagcccaaggatacatcataaaaagagctttttctttatgatccctctccaaaatccaagtaactccccatatcctggcaatgctttataataccactcacaatgggcgcttcctttttattcccatctgtaacaagtctcttctgggttgctatcatctcatctgttatagccttcatcctggacaacctgctttcctgcccttgtatatttcactttttctccctgactgttgagcccatcctccatctctatctattagaatcttacccacacttcaatgtggatcagttcataattccttccttactttccttgaatactccagctgcaaatttcctcaacagatcatgcatacctcaaagtcaggaactatgaatagtttagtggtattttcttctgagcctagcacagagaccaatataggtgctcctaaatatgaggtaagtaaataggtacaatcacaagccatctaggggtacttcagaaacccatctacatcaaatcttgatcctaaaatgggactgaatttctagttctatctttttaaagagtaacaaactttttggagacttagatatgtcagggtttttctgaaactttccaatgtgttcctttgtttttaaagcctaactaagctaatgaacagaaactaaataaaaaaaaggtttcagttcagttgtttagtcccttcttcaacagttttagatccgttttaaaattttttctcactttacctttttttttaaaaaaacacccttgtccttaatttttctttatgttggatcacattctcccttattttactatcaagatgtgtatagctctaggttgtagcatttcaacttataggaaaggacagttattaccaacaaacttgaaattcttcctttatatggggccttattattgtgtaactggctatataggaaaattcaagaaaatgaaacaaaacaacaacaaaagcttctgaatatgggctctcaaagattgaaattattaaataacctccttttcattaggtcatgagcaggcaactgataagctggagaagtcttttatatttttcttcactgaatggataattactgaacgtctgcaaagcagacattgtgtgcttcatagtttggcatgtcagttgccatttttaaaataaaatcagtggagaatttcaacttgaagcacatataaatgacaataaatagtacttttgcaaactttatttagtatttgcaaataggttccaaatgtccagcttaatttttctgagttcttatttcattcctttctagccatgcttatttttatgtaaaggagaaaacatgcttaattactctaaagaaaagttattttagaaatgataaaagttgaacatatttaaaggaaaaaagcagaataaaattaataattaaaatactaaatttggacaggaaaatggctattgaataagtccaaacatttccaggaaagacataaaggcatccttgtttttaagaaaacatacggcaaactatataaaatgaaatattactaagacttctttggtctcctcatcatacgtcaataatgaggagagctttgcaatgataaagcttttgaagtggcttgtggaatattaaattgtttaagtataattttggcatcaagtgaccttacatattttgaatgttggttatctatgcgttatgtataatgccaccacattattcatcaaaatacagtggacttggatattgaaatatttaacatgattggttttagtgacttagaagtggtgctgatagcccctgaacaattatgccccagcttgaaactgtatagcgtgcagccaaagggatgtgctttgtgattaatctctgggtactactgaggagccgctggctcactcattgtctccatcttctgcagctctcatatggtgagaaaaatgttggttcaagtatttttatagttaatattactacaataatgcaatgtaatgcagtgataaattttaggtagaatttatttgacccgattataaattgctgtagatttgaaggtaacataattattaaggggtgttaaagtgctatctgaatcttttagtaatgctttagtaatttatgtgttttagagacatttgtgaacttagggattcataaaaatatctctcaggaatgccaagacattttgtatttgcttcagaatgctttatcttaaccacggagagataattgatatatatcatcacagtattattttaatgtatgtattcttgaatgtttaaaggataaaaaattacattataagttttagaacttgtgattcaataaaatactaaaaaaacatagattatgttattttacattgtgatgttataagatgttttgtttaggaagtttaattcttagcctagaattaaaaggtagcatgctcgaagttctcactgaggttagaggaataagttgcatattataatattctgtggggcatttaatactaacaataaagaatgaagaaaaatctggcgaatttaagaataacctagcttttacagcatttgtgattgtgattttaaaagacctcatatttgaccctaagaactatagaatatacacctgtataatttatcactactttaatatataaattatttctattattatgactaatggaactagatttcttttgttgttaaaataaaaagttgagatagccagaaatgctgtttaactttgcctagtggcactgtagtaaatatgattttgatgacttttttttccaagtagctaagatttaattgttatttttcttaagatttgtacctgtaagctttagataatagatttgtcatgcagataaattatgagcaatttaactaaaattattgtatttcagtgtgtccaaaacatgaaaataatgatgaaccgaacaaggaaatatttggaacataatttcccttgactgaggtatgagattcatttaattattaaatgtgtgtttacacatgcaaatctatgggaaataatttgttctttatttgtttctattatagttaagaaaaacctgttttgcaaaatgttttttcactgatcaacatagaggtaaattttgataatggaccaaattcaggtgaattggaaactttggaaactttggaaggacttttggtttgggttcttagtaagatcaaaaataggtacttttagaatattttcttctttgtgagatctaaaatggctacacagcagtcttctatttcacaggagatatttttggatggaaatacaacttgggtaatgtttttttgatttgacatttttgttcacaattcgtttttaagctttcctcagtaaggtagctttagttgtagagcccaaggtacagaactacagagcagaaacctaaaatggctttgtttgtactattttgggagtgataaatgaggctgttttcatgaatgggatgaacctatatgtaatagagtattttagaaggaatattgttatgggtaaagacatctggaattgatggtttgccatgaggtttgtagtgttaatacatcaaagtttcataatttcatacatttagtcacccttctttgctgtagaaactggtattttgtctagctaggattaagaacaagtgggttttgttttaggaaagaaaataaaaatgctcaacttttactctcatttctacaatttgtctatgcatgggtgaagactgtttctccctaggagttttcttttcactgatgctaatgtttccgtaagtgacttgtgttttaaaaaccccgatttagcagaaaataatagcaatgccttccagaggaaaagaaaacttaagtaaaatgccaaataatggtaactttgtctctttctatttgcctagaataaacaaacaaacacccgaacagattttttcctccaagaaaagtgataagtgaaatgcacttggaatttttctgaagttattcacagattatttgtgcatcttactgggtagactgctgcctctaatcaaagtcagattactctctttctgagtcaatttttgagctctgggatatctgtagggagacaactaacaactgccttgaaagatttcatattaatgaatattatgttaaccagaatgtataagtgggactgcatataggagtgctcattttacattttgccttgtctaatttgataaagtgaatgagcatcaaggaaaggtgataaataatattgctttgtggctttaatatattgccatttaatcaaagattgcatgccattttgtctttaaatacccttatgaggtagcttggagagatctctgcccttttcaatctgtgacagatttcctagttcagagcaaaaaagtctactgctgaaaaatatgcataattaacaggaaagtataataaagttgttgcttaaactactaaaactttgggatatttgcattgactagtttaaggtctagtttatcagtttgtagcacatttatgtttgtgaagaaaagatgccagaattcccttattctacttgaaaatagatgctacagactgtaccaggagatgcaagaatatgacggcttattcttttttttttttccccagctctatcagtgttgctaccaacaaccagtgaattcatcagataaaatgatagaaggtgtttccgtgtccagggagagattctagtaaccatattacattagataatttaaatgctccccataacatactgtagactgccgctactgagaatataagttaaatttatatagcactgaaaagttatacatttttattaaacaccagtaatctttcgtccatgagagtgtttcctagttattcctaggaaattcttcaatgcagtcttccaaagcattagaatttttttccccctctggtttgacagagccttgtgggcaatgtgcttactctacaaactgtggcaacagagggaaagaaaaccgtaatgctcctctattagaccatgccattagctgttgggaaaccagagctcagctacaaatggcttctaaaaacctcagctcagataagtgcaatgaaatcatacacagcaggaatcacacaccatcagtggtgattcctactctgttcctaaagtttctttctgatttttaagattttataattaccatgacctgtgagacctttcttaagggaaattttcaactggggaaaaatagtagaagctggctttctataatttaagatagtgcaaaatcagtgatagtttcctttataaatactttattatattaaaaatatctaccttatagaggttttcagtttaaggtacactcccatttaatttttacatctttagagatgcagaagacataaaatgtgatttgtagactaggaagttatactataaatatattcttaaccctatatattgctcttttgagttgttttccgttttataagaaaagcaagtggcttctctatcagcaatagagagtcctcattaagtatgaaaaaaactgattagaaaaagtgttcattatgactcaaagactcacaaaatatagtcaatgagagccactctgggaatgaatgatgcttatgtcggtgcttactttaagcttctttacaaagagtctccctagcttttcactttcactaacaaaagggtctacggctcttcctttgtgcttggaaattcaggagcacctcccactgcaaagattaggttatgaatctaacaaatgagaacccagtcttcaagtgcaatgtatttgcctatgatcaagtttgctagcagttgagaatctatagttttgcaacaccacgtgattctctctgctgtattctaaatcacagaatatgtggtattattccacttgttctatcacacctacttacagacatcttgatttctgagatgtgggctcatctctcaatatccttccagtgtcatttcaaatgttgcctgatctaactccacaacacttcaaacacagaacaccacctcttgtgctcctaagttaaacgtgatggtggattaatcttggtcctttagttgataaatcaaggtaatttactgctgctatacccatacacagtccctcccctgctggatctcatgcagtgtggctttgttgctttcacttatgattttgctgctttcatttgggtcaatatcattgtagttattttgtagacaaagtagtaaaaaacttgatttttccctatcctatatatctgcagctcactgatttaaaatattagcataaaggtccgcaccacagtgatgatgttcaatttcatattgagattgaagatggggaaatagcaagggcataccaattcagccataaatatgttttgggtcaatgtcataaaattgtcacaaaattttggtaattgagaaaaagctaaaactttttttgtttgttttttgtttgtaaagggaagaaaagtgcttctgaggctcttttggaataagtaacagttttcagattcacttttgcaaagattgccaatatccttcgcagacaccaacaaaccagactgaacagaaagatccctgtagtaggatgccgagcaaatcattgacttctccaatctctaagagacaatatctaaatgtcagtctcatggcattgtattttctgcttcaccataagattagcaaacacaagacataaaattatgtttatttactaaccaatacagaatatactaggccctttgcctggaagccagatttcacttctgagattttccgaagtccattctagaagaggtggttgttactgatacccagggaaggcaattcttaaattgcttacctggggatggaactttctgtggactttaggcccttaagaccaaaagccatgaggcatttatgaataggtgatgtaagaaattttaataaaagttgcaataaccctgaaaatagtgtctttaataacctatgtactattaataacaaagcatgcatagtgccgtgcattcataactatttggtcataaaaatatgtgactgtaattatgatatttacagtcaacttataaaaatacatgtaattctgaatggcaatagttaatccttagctctaaccacaagcctagaaggattagcttattacggggaaatgtgatagataattacaaaatggacaaagcttttactgtcttgaatttaacattcaagaataactataatagcatcataaaacatttgtcatcattattcttctcacctcacaaggtaaaaacctaaattctgtggaaataaatgggaatcaaataggaaagggccacttacatgatacaacaacagaggagaatagttctttcatagaatactcatgcacagccttcaaagaggttcatagtaactgcaagaattcctgggaagacatctaaacatgactttcattaaaaagaattaaggctggtctaaagaatcaaatctctaaggtatgattacctttaaccataaacggtaaaaaatcttttagctgatctctctgtaatttaggtgagtacctctttgaagtttattaacatcaaagagagtggagctcacatggcactttccaattcaaatttaaattctgatggaaggaaataaatccacattccagtttacatacagaaaaagagtagttttttcaaactttataacctcttactttaagggcatatatgtttcaattaaataaaatattacacaaagctaacatatttcccacaaatttcttctcttctaggagttgattggtcatctgctgacaacagataagttcctaatttgaatggcattagtacttcataaatgaacaaaacaatgagtgcaaactggaaaaactagggagaggtgcatacaagctaccaaaaaaggttgggattgggggtgacctgcaagtcatgatctcatatcttaggatgtatcttagtattcaggaaatggaattcttggaaacatctgtttcacagtgaggttgggaggtcagacgatgctctgttagattcttcttaggattaaattacttcctaggactgcattaagacactttaggtggtatattaactcttccagaacaaataattccatttcagtaaattattgctacagttctctaaagagtactacggtgtcctggaaaagataatgttccttccaaaatgccctctagtcactcgaacaatgagaaattcatatttatcttagacactttgatccttgaagacataaactaaaaaagaactgtttttccctatctaaacagagactatctggatggagacataatattagatctgccctggtcatttggcagtgtataccatttcctccatgtgcttttgacaactggcatgcttgattctttccctgtaaatcagcctgccattcttctttgcatgcagaatggtctataggaaccaagaaaaaaccaaccccaatagccaatcttttaaaaaataggtgaatgagtggagcatggcacacaatgggaagaaaaggagtgatagttaattaactttctcagtgattatctcccatattttgatatgggagataaaaatcttccatatcaaatctttacaaatgatgggtaatctgtaagaggaattctcctcctccctgcacccccactacaaaactcccacccaaacaaaaaatcaaaacccaaccaaaaacctcctctgaaacttctacttcagatatgagatcatggtctggaggctactcgtaccaaataccagttcattctagtacagcagttcatgaggcaaaaggctaggagtatttgtgacatgactttacaaataatgtaaaaacaataaccctatgattatgggcaataattttccccactcaaatctatagatattgcactgaaactgacacaatggagaagacatagatcatttcctgttgaaacccaattacctcaaggtaaaacaaaacaaactccatttaataaatgaaatattacttaaatgttttcattttagggtctgttccctttcccctttatattctggaaagttatatgtctaagtatacttgttttgttacttcattagtctatcaacttcatttccagagactataacgagaatggaatggtttgtaccttttttctgaacataattgagtcaaggagttttgttattttaggtattattaatttgattaaaacatagaaccaaagttgatgggaagtagtagctttcttctaggtaaaagagcttactagcagattttataatcatcggacatttattctgtcctacctggaaataaattatgttactgcttggcatgggaaaaggcattttctagtaatttcctgtgacaggaggcacagcaatagtccaagtaagcacccaacaggtgcttgggagtagttttaaactttaacttaatgaaaacatttacctcagtacttttgtttgagaaagaattcagcagcagttatagttaatatcccacctgtggagagctgcgatcaccctaggaggtgggccaaccgaggagcactttccaggtaacaagagcaacactattgtgagaagctacaaatggtactgcagtaggtgtagtgaacactactatagtgatcatggcctgggttatgttccaaatactaatgcaaggaatacactagagtttataggattagaatagtttccttatgctaagaactagtagatggcatgtgatgagtgggtatggtccattttattctatttcactctacgagtttcctagttatgtctcctttctcctatgttaattatctatattccatgacagttattttccctatctaaaataagaacggtgtaactatggagtaccccaactcacatacacatacttgtgcacccttagactcatgtatggataatctgtgtaaagcgctcatttgcaattgggtgagctcactgaaagcagccatatcagtcttccaaatacagtaaaagccaacgaaaatccatatcaactgtttatttctaatatgaaacagtaaaccttgtccatgtggtaattaattcaaatgccttttgtgttttcttgtgaagtcatccaaagcaaaagtctagatgactgctgacatgatatgcataatctaatgaactcacatctctgtttattttgctcatcccacagttgaatgacacactgactgctgagacacttgggttgatttagaacggctattaatgaatctataaatttggctaaggttgatttgactttctagggaaaagccagcctatcttcaaatggacagctccctccacataaacgtcaatgtaccctaaagacaaaactaagtatatgtatatacgggatatatacatatatatgtacacataaaatggattgggaagtcctttggtttagacagtattaaatatgtacttcccaagtgcataggtttcctttgaccaacctgttcaaaaaacaagcatgaaaagtgccatggcacatttcccatgtctttccccctatttgaaggacacctttccttgcttctccatcactcctaagcattttatttttaaaagaagctggttattttggccttctatcttaacactccattgattcatccattccttggaagagctctcagattacatccagaaacttgtttttagaggagaacaaggttgcaaataactttttcctctttttttattccctcttccccccaagaagcaggcaccttgaagtgtcatgaataatgcactcttgatctgacttgccttgttacccctggccagcccaagcagctgaggtctgagctttacttgccctgcatcattgtgcaatactggaaaagaaaaataatccactggtctatacccctcatactgtggtgacgtgatccgggttctcttgaatttctatgcattcaatttcctctctctcctttcgcttggcacgtttctttttcttgtggtgctttttggaaggggggaaaaacgttaggaacacaggtaaaataacaaaacagtgcagaagtgtgcaacccccagtgagcagcaagcatttgaacagtgtgaaggtcaggttcgaaggcacaaatagaagggggactaacccaataagaaaagaagtaacattttgcaaaatggctgtcccatggtcttgcaaggagctttttatacattgtgttcgggtgtgctcagttgctaatacaaatgtgaaaagcagtggtgcacagtggtcaatggcgaaattcaaggtgtagataaggcacaagatagaaatgcaatccatgtcgacgttccataatgtcattaagcccagaacgcccagctcaattgaggtgacgctaagaattagccagaagtttcccagagggtggatcactaggaaaaaagtcaggattaacaccaggagaacaccaaagcctgcaatcagaacaggcactgtgacagacaagctgtaatggtccatgaagacaaaggaggggttgaacacgatgaatcggatgctctttgagagggataggggcctcagcttttccaacacttctgtgatttctttctgcttgtctctgctagtcctggccaccagatacaagcgagaagcaatgatattgctttcatcccctgccttggagaagatgatatcatttcgaaaatgctggaattctggcttttttaaaaatgagctttgcaggacactgatgaagtcacttttgttattggcactgacgttgctgactttcaggaactggtagtactgctccacccaggacactgcagtgaatccactacagagtcttcttaggtcatcctggacgctgctgttccagtactctaggggctcatagacgtagaatcctatcacagggctatagttgctgaaatatttctgctgaaccatggcataggaaacacttggcgaatcactggctagtagattgatgatgttggctccgtcactgatctgtaagcaccccatgaaggagaaggaggcataaatgagatagaggatgacaacaaatggcttcacatatatattggtaatccattcattataatgttcacggaggaagtgctgaatgaagtggtgctggtaggggttcgtctcatgatgggacgtctgttgatgcccatcactcatcactgtctggaaccacacaggtttgcgatccaggtattctgcagaagggatcttacagcaaaagatgctgtggtagcggttttgctctagttggccagcaaagaccagacaggagccaaagaaggagaaaatgtagaagtagttcaacagaatagagacacacatgttttgacagaagaccttcacagcctctatgtttgtgaatgggctggcacccatgccaaaagtgatgaagtacagggagctggtcatggtataggtgaccatcacatcagaataggcatctgctatcctgtctttgaagggcaagttctctttggttctccgccatccggacagaagctcaaacactcctttagttccatgaccttgccccaaaccggtaagaatccgattaccacaaggatggatagttacccatggcgaagaacgggattcccagcagggtggagttgtactttccatcggtgatgaagaagatccctgctgctgtgatgatggagatgcatactgtgagcacccccaggaggcccaggaagggcttactgcgcaagcagtccttcatggagctggagagggtggctgtggtcaggatcagcacgaggctcaccaggaccttgcttctggccaggatgctggtcttatgaaagtccctccagaggctaaaggatgctaaagagtagagctggagttcttgatgctcctcctggagcttccttataagcttacagaactcattctcccacttctcccctatgaggtcttgggtggcagagccataggtctggaggtagtaggtgatttgaatggctctggctgacttgacccgctgatctttgctgtttggcacttccactaccccgcccagttggtgtccaataaaactgttcctcccatcctttaatttagtgttgggatacctcacttgcaccctggctgttgtcttattggagacggcagcctgcctgagatcctctagcactgaaataatatcatccagcacgcatttcttatcctgatttctcaacacacacagatgggaaaaagtataattatagcccttgtggttcaccttcatttccagcacggctcggtgggtctgcaggatcccctcagcctggagcaaaatattgtccccggttggggagaggaggatcaccctgccatacctcccaggggtgtgtaagtccgaatagagctggcttttggactggtccagggggaaaaggctgctggccaggctgcgctcgatcttggccaggctgtggctgggagcgaccaggcgctccaggtcgccctcgggctggaagcggttgagcgcgctgaggccgaaggtgattgtcaggactgcgggcacggtgaggaaaaagaccgggtgccggctcacgcacaaacccagcctgtggcagaacgactggagccctctgcgaagcacctgccgcagcatcctccaccagatccagctcgcaggcgctcccggccgt

SEQ ID NO: 10510 - RNA, 1037 nt, Homo sapiens
  source 1..1037: mol_type = other RNA
cctgttgaagtgtaatccccaacgttggaagtgggacctggtgggaagggattggatcatggtggtggtccttcacaagtgggttagcgccagcttcttggtgctgttctcatgatagtgagttatcgttagatctggttgtttcaaagtgtgcggcaccccctctttttctctctctactgctcccatgtgagacgccttgtcccgccttcaccttccaccatgactataagtttcctgaggcctccctagaagtggaagctgctatgcttcctgtaaagcctgcagaaccgtgagccaattaaacctcttttcttcatgaagtgcccagtcttaggtatgtctttatagcagtgtgagaatggatgaatgcacgaggtcttcaggacaagcccgatttcattggttacgagatgcatgtttttcattctagcccccagagacctggatacgttgcacagatgctgacagcaggtggcagtgtggagcagcggtgtgacacctgcagggccctccggggacaccacataagggcagccacagtgtcccggagcccatgcagtgtgacagccccaggtaactctccagccagcactccacccgtggaattacagccgactgaagcacctctgctacattcgtcagcttgataaatgtccaaggaatgaaccaagcacagggaccatctcttccggtagcttctcaccatcacacacactttgcagggccgagggctcttcctggcccatatctagcacctagatattttattcacttatgttttgaatatttcatgggtccttctcccccagaggcctcagagcactcccagaattggaatggaaatacacagtgtgtccttgtcagctgtccgggccgccgcgttcaaagggcaggacatagtagcttctgctcaaattagaatgatctgtctcgtcaagcggaagatggttgttgagactttgtgtctttaaagtattgcagttccacatggctggggaggcctcagaatcatggcggcagcaagagaaaatgag

SEQ ID NO: 10511 - RNA, 1565 nt, Homo sapiens
  source 1..1565: mol_type = other RNA
ccttcactgtgactctgctgcagctttctgaggacctctcaaagccccacagtctctgtttcaactacaggagagaaaagttagggcttgctccccagggccttacgactcttcatggctaacgtgacagtgcagtatcatttgggagaatttttttagtacagttcagagtctggaacagtctccttcctcctctgtctttcctgccttctgactttccatggggaaaggaggacatttaggaagagggaacaggtgaggatttccagtaccttgctggtgtattttaatttatttaaatttagagaaacagtggtctaatcaggcagtaattaattccctcttcattaggggccttcatgtttgccttttgcatatggatgagccacgggtcacactgtccctttgaagagagatccttgctgaaggtgagagcccagtgtgctctccggcacttgagctccttccccttctgtgccaatgcttctcttttctccccaccctcacctgacaaggactagattccggttcaactggaaggctggagcccccttggggtggggcatcccaggccggggtccccctcggggctcctcatggtcaggggtgggggtaggtgagtccccgaaggcccccagcacagtgactccagccggggacaggtctgtcagtggctgctggctctcctcctgcctcagggcaccttgctgccctgagggtctgcgtcgcttctggctgcggtcccagcagaacttgaagatgatgccagtggccacgagaacaatgatgatggagatggtaattgtgacatagagctgggggtccacaccttccccacggcccccgaacaggaatggccgcagggtggcaggtgcctctccaaggataagcccatctccatcacctcgcatggagtctgagttggggtgtggggttgcgagcccatgaggggctgcaaaaccatagtccagaaatccgggattggcagagttggggtcccctccatcctctcgagacacggtgggaccccacacgatagcccaggggtattgggatgagggcggcccctcctcaaagcctgatggggtggctgggggtgcagtgccaggcaggacttgccgacgtgatcttgggacccgaggagatcggcttggtggaggtgctcgctcccacacgcacacatgacgtggggccgaggggcctcccctggcacacggggggcgggctggggctggtggggttcgaggggaggatgaagagccctgagcaggcggtgggaggggcagcaacagcagtggccagagagggaggaggtgggacagcagcagcgcaggccacatcctggactccatgtctgaggtcttcctcagctgtgacccagattttcagcctttactgcatgcttggcgcggcggcgcgacgactgcgggcgctcgggactgagcggggctggggggtcgcaggagcgggcggggtgcggggcatggtggggaggtttggcccgcggcagggcgctggagcgggtggggggcgggcgcctggggcgcggggcggcggcggtggga

SEQ ID NO: 10512 - RNA, 1388 nt, Homo sapiens
  source 1..1388: mol_type = other RNA
cgaatcattatttgctgctctattcacagccagtggattattatcaccagcaatatggaaacagtcagaccattcagtggccccctctattggtattgccccagttccacacattggatcgactattatatcataaggtagaggatcacagagcctgagcatcccataggcaagagttgatctaagagttgtaggtccaaaatgtgttatatttcttcggtggagactctcttcagtcaatgcaatgcccacaatgacttcattatcatggatgttcaaaagaacctccacatcaaagttggtcatgtcggccttccacttaaaataatcttgaacagcacccccaaaatctcttgcagcctcatttgaggtaaagcaatgtttctctcctgccctgttgcatgtgactctaaacttcagcacttgaggctcagtttcttcttttgagctttcatcagtctcatctttgcaagatgccaaatcatcacctattaatgttgatacatcctctttgatggctggattttcataataatctaagatatgagaatctaaagcatggctagtgaactcttttttaacatttctctgatcgattttgacttcttgtccattattaatcttctctttacttgaattctgatttatctttttgcgctttgcttttttctttttaaaactggcattaattttccacacttttaaggggtttgaccatgggagttttccagccaagtcttcaaaatcctttagaacttcttcctttgtttgtttgaactggtaatcttgaaactcctgaaccaccacaaataagttatcaactgatctcagacaatgaacctgtgccagactttccactgaaatgacaaaatatatcttgccacggtctctgctgattttgcatgatgacccaagtttctctctgacttcatctgcagctgtttgctcaaagccagtaggtacagtggctccaatagtgactagaagctcagattcacttccgaggtcactttctgtcacttgtacagacttctggttctcatgaaggttcacatctaggagttggttagtggcttcttcaatgtcacacatgttggctgtgcttccaagatccctaacactgtctctttaaaagcagtactgtcagggcccgggaatcctagggagcgggtaaaggcctgggagagggagcaagatgggctccgccacgagatccgcctgaagtccggctcggcgccggcctcaactgcaagaggaaggccacccctctctccccaagctgaaacaccagaagagccacactcggccgttcccaaccgccgccagttaccggccgccagcgaagaccctttcagctcccacactccattggcctcttgcggtcaggt

SEQ ID NO: 10513 - RNA, 2005 nt, Homo sapiens
  source 1..2005: mol_type = other RNA
cgaatcattatttgctgctctattcacagccagtggattattatcaccagcaatatggaaacagtcagaccattcagtggccccctctattggtattgccccagttccacacattggatcgactattatatcataaggtagaggatcacagagcctgagcatcccataggcaagagttgatctaagagttgtaggtccaaaatgtgttatatttcttcggtggagactctcttcagtcaatgcaatgcccacaatgacttcattatcatggatgttcaaaagaacctccacatcaaagttggtcatgtcggccttccacttaaaataatcttgaacagcacccccaaaatctcttgcagcctcatttgaggtaaagcaatgtttctctcctgccctgttgcatgtgactctaaacttcagcacttgaggctcagtttcttcttttgagctttcatcagtctcatctttgcaagatgccaaatcatcacctattaatgttgatacatcctctttgatggctggattttcataataatctaagatatgagaatctaaagcatggctagtgaactcttttttaacatttctctgatcgattttgacttcttgtccattattaatcttctctttacttgaattctgatttatctttttgcgctttgcttttttctttttaaaactggcattaattttccacacttttaaggggtttgaccatgggagttttccagccaagtcttcaaaatcctttagaacttcttcctttgtttgtttgaactggtaatcttgaaactcctgaaccaccacaaataagttatcaactgatctcagacaatgaacctgtgccagactttccactgaaatgacaaaatatatcttgccacggtctctgctgattttgcatgatgacccaagtttctctctgacttcatctgcagctgtttgctcaaagccagtaggtacagtggctccaatagtgactagaagctcagattcacttccgaggtcactttctgtcacttgtacagacttctggttctcatgaaggttcacatctaggagttggttagtggcttcttcaatgtcacacatgttggctgtgcttccaagatccctaacactgtctctttaaaagcagtactgtccagactctgggatccatagatgggcatcaggagagagatcttggaagtaatccgaaatagtaaaacaaatttcctatgcataagcttttgtgtgtgcttggggtgggggccgggggaagtattagagaggtggaggggccatagcttacacgagattttcaaaaggtctgtgactcaaaataacttaattgagtacagaatacctataatgtccttgtgctgtgccagcgatacacgacagtgtttaacactacgtcagttcccgccgttaaaaagctgacagtcactgtgaatacaatctccatcttctaaaaaatgcagctgaggtcagctaaaggacgcgttccgcacaaggtcagagagccaatgagaggcgcagaatgaaagagaactcacgtctcccaactcccacctacagggcccgggaatcctagggagcgggtaaaggcctgggagagggagcaagatgggctccgccacgagatccgcctgaagtccggctcggcgccggcctcaactgcaagaggaaggccacccctctctccccaagctgaaacaccagaagagccacactcggccgttcccaaccgccgccagttaccggccgccagcgaagaccctttcagctcccacactccattggcctcttgcggtcaggtcacgccgccggaagccgcccccggaaacggaagtcaggctacgagtcacggtggctccgcgctggcggcgggttcccccacaaggtcttggggaaaggagcatgcgctggaagctgtgtgctgttggttttgaggatcttcagtaagctgaaagcggagagtcaggggccttgtgtcctaccatggtatttgctaacgttt

SEQ ID NO: 10514 - RNA, 1219 nt, Homo sapiens
  source 1..1219: mol_type = other RNA
cgaatcattatttgctgctctattcacagccagtggattattatcaccagcaatatggaaacagtcagaccattcagtggccccctctattggtattgccccagttccacacattggatcgactattatatcataaggtagaggatcacagagcctgagcatcccataggcaagagttgatctaagagttgtaggtccaaaatgtgttatatttcttcggtggagactctcttcagtcaatgcaatgcccacaatgacttcattatcatggatgttcaaaagaacctccacatcaaagttggtcatgtcggccttccacttaaaataatcttgaacagcacccccaaaatctcttgcagcctcatttgaggtaaagcaatgtttctctcctgccctgttgcatgtgactctaaacttcagcacttgaggctcagtttcttcttttgagctttcatcagtctcatctttgcaagatgccaaatcatcacctattaatgttgatacatcctctttgatggctggattttcataataatctaagatatgagaatctaaagcatggctagtgaactcttttttaacatttctctgatcgattttgacttcttgtccattattaatcttctctttacttgaattctgatttatctttttgcgctttgcttttttctttttaaaactggcattaattttccacacttttaaggggtttgaccatgggagttttccagccaagtcttcaaaatcctttagaacttcttcctttgtttgtttgaactggtaatcttgaaactcctgaaccaccacaaataagttatcaactgatctcagacaatgaacctgtgccagactttccactgaaatgacaaaatatatcttgccacggtctctgctgattttgcatgatgacccaagtttctctctgacttcatctgcagctgtttgctcaaagccagtaggtacagtggctccaatagtgactagaagctcagattcacttccgaggtcactttctgtcacttgtacagacttctggttctcatgaaggttcacatctaggagttggttagtggcttcttcaatgtcacacatgttggctgtgcttccaagatccctaacactgtctctttaaaagcagtactgtccggccgccagcgaagaccctttcagctcccacactccattggcctcttgcggtcaggtcacgccgccggaagcc

SEQ ID NO: 10515 - RNA, 1414 nt, Homo sapiens
  source 1..1414: mol_type = other RNA
cgaatcattatttgctgctctattcacagccagtggattattatcaccagcaatatggaaacagtcagaccattcagtggccccctctattggtattgccccagttccacacattggatcgactattatatcataaggtagaggatcacagagcctgagcatcccataggcaagagttgatctaagagttgtaggtccaaaatgtgttatatttcttcggtggagactctcttcagtcaatgcaatgcccacaatgacttcattatcatggatgttcaaaagaacctccacatcaaagttggtcatgtcggccttccacttaaaataatcttgaacagcacccccaaaatctcttgcagcctcatttgaggtaaagcaatgtttctctcctgccctgttgcatgtgactctaaacttcagcacttgaggctcagtttcttcttttgagctttcatcagtctcatctttgcaagatgccaaatcatcacctattaatgttgatacatcctctttgatggctggattttcataataatctaagatatgagaatctaaagcatggctagtgaactcttttttaacatttctctgatcgattttgacttcttgtccattattaatcttctctttacttgaattctgatttatctttttgcgctttgcttttttctttttaaaactggcattaattttccacacttttaaggggtttgaccatgggagttttccagccaagtcttcaaaatcctttagaacttcttcctttgtttgtttgaactggtaatcttgaaactcctgaaccaccacaaataagttatcaactgatctcagacaatgaacctgtgccagactttccactgaaatgacaaaatatatcttgccacggtctctgctgattttgcatgatgacccaagtttctctctgacttcatctgcagctgtttgctcaaagccagtaggtacagtggctccaatagtgactagaagctcagattcacttccgaggtcactttctgtcacttgtacagacttctggttctcatgaaggttcacatctaggagttggttagtggcttcttcaatgtcacacatgttggctgtgcttccaagatccctaacactgtctctttaaaagcagtactgtcctacagggcccgggaatcctagggagcgggtaaaggcctgggagagggagcaagatgggctccgccacgagatccgcctgaagtccggctcggcgccggcctcaactgcaagaggaaggccacccctctctccccaagctgaaacaccagaagagccacactcggccgttcccaaccgccgccagttaccggccgccagcgaagaccctttcagctcccacactccattggcctcttgcggtcaggtcacgccgccggaagccgccccc

SEQ ID NO: 10516 - RNA, 1802 nt, Homo sapiens
  source 1..1802: mol_type = other RNA
cgaatcattatttgctgctctattcacagccagtggattattatcaccagcaatatggaaacagtcagaccattcagtggccccctctattggtattgccccagttccacacattggatcgactattatatcataaggtagaggatcacagagcctgagcatcccataggcaagagttgatctaagagttgtaggtccaaaatgtgttatatttcttcggtggagactctcttcagtcaatgcaatgcccacaatgacttcattatcatggatgttcaaaagaacctccacatcaaagttggtcatgtcggccttccacttaaaataatcttgaacagcacccccaaaatctcttgcagcctcatttgaggtaaagcaatgtttctctcctgccctgttgcatgtgactctaaacttcagcacttgaggctcagtttcttcttttgagctttcatcagtctcatctttgcaagatgccaaatcatcacctattaatgttgatacatcctctttgatggctggattttcataataatctaagatatgagaatctaaagcatggctagtgaactcttttttaacatttctctgatcgattttgacttcttgtccattattaatcttctctttacttgaattctgatttatctttttgcgctttgcttttttctttttaaaactggcattaattttccacacttttaaggggtttgaccatgggagttttccagccaagtcttcaaaatcctttagaacttcttcctttgtttgtttgaactggtaatcttgaaactcctgaaccaccacaaataagttatcaactgatctcagacaatgaacctgtgccagactttccactgaaatgacaaaatatatcttgccacggtctctgctgattttgcatgatgacccaagtttctctctgacttcatctgcagctgtttgctcaaagccagtaggtacagtggctccaatagtgactagaagctcagattcacttccgaggtcactttctgtcacttgtacagacttctggttctcatgaaggttcacatctaggagttggttagtggcttcttcaatgtcacacatgttggctgtgcttccaagatccctaacactgtctctttaaaagcagtactgtcctataatgtccttgtgctgtgccagcgatacacgacagtgtttaacactacgtcagttcccgccgttaaaaagctgacagtcactgtgaatacaatctccatcttctaaaaaatgcagctgaggtcagctaaaggacgcgttccgcacaaggtcagagagccaatgagaggcgcagaatgaaagagaactcacgtctcccaactcccacctacagggcccgggaatcctagggagcgggtaaaggcctgggagagggagcaagatgggctccgccacgagatccgcctgaagtccggctcggcgccggcctcaactgcaagaggaaggccacccctctctccccaagctgaaacaccagaagagccacactcggccgttcccaaccgccgccagttaccggccgccagcgaagaccctttcagctcccacactccattggcctcttgcggtcaggtcacgccgccggaagccgcccccggaaacggaagtcaggctacgagtcacggtggctccgcgctggcggcgggttcccccacaaggtcttggggaaaggagcatgcgctggaagctgtgtgctgttggttttgaggatcttcagtaagctgaaagcggagagtcaggggccttgtgtcctaccatggtatttgctaacgttt

SEQ ID NO: 10517 - RNA, 1508 nt, Homo sapiens
  source 1..1508: mol_type = other RNA
cgaatcattatttgctgctctattcacagccagtggattattatcaccagcaatatggaaacagtcagaccattcagtggccccctctattggtattgccccagttccacacattggatcgactattatatcataaggtagaggatcacagagcctgagcatcccataggcaagagttgatctaagagttgtaggtccaaaatgtgttatatttcttcggtggagactctcttcagtcaatgcaatgcccacaatgacttcattatcatggatgttcaaaagaacctccacatcaaagttggtcatgtcggccttccacttaaaataatcttgaacagcacccccaaaatctcttgcagcctcatttgaggtaaagcaatgtttctctcctgccctgttgcatgtgactctaaacttcagcacttgaggctcagtttcttcttttgagctttcatcagtctcatctttgcaagatgccaaatcatcacctattaatgttgatacatcctctttgatggctggattttcataataatctaagatatgagaatctaaagcatggctagtgaactcttttttaacatttctctgatcgattttgacttcttgtccattattaatcttctctttacttgaattctgatttatctttttgcgctttgcttttttctttttaaaactggcattaattttccacacttttaaggggtttgaccatgggagttttccagccaagtcttcaaaatcctttagaacttcttcctttgtttgtttgaactggtaatcttgaaactcctgaaccaccacaaataagttatcaactgatctcagacaatgaacctgtgccagactttccactgaaatgacaaaatatatcttgccacggtctctgctgattttgcatgatgacccaagtttctctctgacttcatctgcagctgtttgctcaaagccagtaggtacagtggctccaatagtgactagaagctcagattcacttccgaggtcactttctgtcacttgtacagacttctggttctcatgaaggttcacatctaggagttggttagtggcttcttcaatgtcacacatgttggctgtgcttccaagatccctaacactgtctctttaaaagcagtactgtcctctttcctagagtcgttaggagacaagtgagagtagtacctggttaggccaataattaaaacttattaataggctatctatcttcttccctcctgtgaaatagcatttcatgcatttaaaaatgattaactgggctgggcacactggctcatgcctgtaatcccagcactttagggagctgaggtgagtagattgcttgaggccaagagttcgagaccaatctgcgtaagatggcaaaatctcatctctaccaaaaacacaaaaaatagctgggcgtggtggtgggcgcctggagtccagctacttgggaggctgaggtgggaggactgcactccagcctgggtgacacagtgaggccctgt

SEQ ID NO: 10518 - RNA, 1424 nt, Homo sapiens
  source 1..1424: mol_type = other RNA
cgaatcattatttgctgctctattcacagccagtggattattatcaccagcaatatggaaacagtcagaccattcagtggccccctctattggtattgccccagttccacacattggatcgactattatatcataaggtagaggatcacagagcctgagcatcccataggcaagagttgatctaagagttgtaggtccaaaatgtgttatatttcttcggtggagactctcttcagtcaatgcaatgcccacaatgacttcattatcatggatgttcaaaagaacctccacatcaaagttggtcatgtcggccttccacttaaaataatcttgaacagcacccccaaaatctcttgcagcctcatttgaggtaaagcaatgtttctctcctgccctgttgcatgtgactctaaacttcagcacttgaggctcagtttcttcttttgagctttcatcagtctcatctttgcaagatgccaaatcatcacctattaatgttgatacatcctctttgatggctggattttcataataatctaagatatgagaatctaaagcatggctagtgaactcttttttaacatttctctgatcgattttgacttcttgtccattattaatcttctctttacttgaattctgatttatctttttgcgctttgcttttttctttttaaaactggcattaattttccacacttttaaggggtttgaccatgggagttttccagccaagtcttcaaaatcctttagaacttcttcctttgtttgtttgaactggtaatcttgaaactcctgaaccaccacaaataagttatcaactgatctcagacaatgaacctgtgccagactttccactgaaatgacaaaatatatcttgccacggtctctgctgattttgcatgatgacccaagtttctctctgacttcatctgcagctgtttgctcaaagccagtaggtacagtggctccaatagtgactagaagctcagattcacttccgaggtcactttctgtcacttgtacagacttctggttctcatgaaggttcacatctaggagttggttagtggcttcttcaatgtcacacatgttggctgtgcttccaagatccctaacactgtctctttaaaagcagtactgtcgtctcccaactcccacctacagggcccgggaatcctagggagcgggtaaaggcctgggagagggagcaagatgggctccgccacgagatccgcctgaagtccggctcggcgccggcctcaactgcaagaggaaggccacccctctctccccaagctgaaacaccagaagagccacactcggccgttcccaaccgccgccagttaccggccgccagcgaagaccctttcagctcccacactccattggcctcttgcggtcaggtcacgccgccggaagcc

SEQ ID NO: 10519 - RNA, 2044 nt, Homo sapiens
  source 1..2044: mol_type = other RNA
cgaatcattatttgctgctctattcacagccagtggattattatcaccagcaatatggaaacagtcagaccattcagtggccccctctattggtattgccccagttccacacattggatcgactattatatcataaggtagaggatcacagagcctgagcatcccataggcaagagttgatctaagagttgtaggtccaaaatgtgttatatttcttcggtggagactctcttcagtcaatgcaatgcccacaatgacttcattatcatggatgttcaaaagaacctccacatcaaagttggtcatgtcggccttccacttaaaataatcttgaacagcacccccaaaatctcttgcagcctcatttgaggtaaagcaatgtttctctcctgccctgttgcatgtgactctaaacttcagcacttgaggctcagtttcttcttttgagctttcatcagtctcatctttgcaagatgccaaatcatcacctattaatgttgatacatcctctttgatggctggattttcataataatctaagatatgagaatctaaagcatggctagtgaactcttttttaacatttctctgatcgattttgacttcttgtccattattaatcttctctttacttgaattctgatttatctttttgcgctttgcttttttctttttaaaactggcattaattttccacacttttaaggggtttgaccatgggagttttccagccaagtcttcaaaatcctttagaacttcttcctttgtttgtttgaactggtaatcttgaaactcctgaaccaccacaaataagttatcaactgatctcagacaatgaacctgtgccagactttccactgaaatgacaaaatatatcttgccacggtctctgctgattttgcatgatgacccaagtttctctctgacttcatctgcagctgtttgctcaaagccagtaggtacagtggctccaatagtgactagaagctcagattcacttccgaggtcactttctgtcacttgtacagacttctggttctcatgaaggttcacatctaggagttggttagtggcttcttcaatgtcacacatgttggctgtgcttccaagatccctaacactgtctctttaaaagcagtactgtctatctaatgattacaaatgttcaaacgcctactacttgccagactctgggatccatagatgggcatcaggagagagatcttggaagtaatccgaaatagtaaaacaaatttcctatgcataagcttttgtgtgtgcttggggtgggggccgggggaagtattagagaggtggaggggccatagcttacacgagattttcaaaaggtctgtgactcaaaataacttaattgagtacagaatacctataatgtccttgtgctgtgccagcgatacacgacagtgtttaacactacgtcagttcccgccgttaaaaagctgacagtcactgtgaatacaatctccatcttctaaaaaatgcagctgaggtcagctaaaggacgcgttccgcacaaggtcagagagccaatgagaggcgcagaatgaaagagaactcacgtctcccaactcccacctacagggcccgggaatcctagggagcgggtaaaggcctgggagagggagcaagatgggctccgccacgagatccgcctgaagtccggctcggcgccggcctcaactgcaagaggaaggccacccctctctccccaagctgaaacaccagaagagccacactcggccgttcccaaccgccgccagttaccggccgccagcgaagaccctttcagctcccacactccattggcctcttgcggtcaggtcacgccgccggaagccgcccccggaaacggaagtcaggctacgagtcacggtggctccgcgctggcggcgggttcccccacaaggtcttggggaaaggagcatgcgctggaagctgtgtgctgttggttttgaggatcttcagtaagctgaaagcggagagtcaggggccttgtgtcctaccatggtatttgctaacgttt

SEQ ID NO: 10520 - RNA, 1074 nt, Homo sapiens
  source 1..1074: mol_type = other RNA
cgaggggtagaagagcacaggggaaactgctcccatgatgcaattacctccacctgatccctcccctgacacatggggattatggggattatgggatttacaattcaagatgagatttgaatgaggacacaaagcctaaccgtatcagggttcttccagtgagacaggatgcgtatagagagatatattagaaggaattggctcacagaattagaggctgataagtccccaaatctgcagggtgagtcagcaagcaagacccaagagaacggatggtgcacttacagtctgggtccaaaggcccaagaaccaagagagctgatggtataaacttcaatctgaagcctggcaggttgaagatctaggaagagctgatgtttctattcaagtccaaaggcaggaaaaagttgacgtcctagtttgaatgcagtcaagcagacgaaatttcctcctactgagggagggttggcctttttgttccattcaggctttcaatggattggatgaggcctggccatatcatagagggccatctgctttactcagtctaccaatttaaatgttaatctcacccaaaacgccctcacagaaacacccagaataatgtttgaccaaatatctgggtacccctgggcccagtcaagttgacacataaaatcaaccatcacaatggagtcagaggcagcactgagtactggaaaaaacaccatttctggaggtcaacagcccaacgtcaagttccagctctcttacttcctagttgtgtgatccgcaggttactcgaactctctgaagctgcctcagttgcctcatcagtagaataaggatgacagaagaatcagtgtctgacacatagcaggcaccaaagcgttggctgttttggatgcaaaaagtacttttcaatggttccatttgccctttgcatttaatgtacatcactattttagacaaaaggggcttgtctcatttgttcacaaagaatccaaagccagcaacatcgatcagcttcttgctttttgtccaactacttgcctacaactctagaaaaacaacagaggtctgccaagaatctgc

SEQ ID NO: 10521 - RNA, 206 nt, Homo sapiens
  source 1..206: mol_type = other RNA
cgaggggtagaagagcacaggggttccagagtctctgaaggatagaggatccacgtcggcgaagagaaacagcagccccaaccgaaggcaaaaggaaatcccaccgcagcctccaaaggcgcgtgggcgggactggagaatggggccctgcgcactaggcgcggaagtcaagaagcagccccaccacccgtgccgcgagaaaagca

SEQ ID NO: 10522 - RNA, 212 nt, Homo sapiens
  source 1..212: mol_type = other RNA
cgcaggggccgggtgctcaccgaggagcggccgccgcggcagctcaggccccggcccagccgcctccccgcctcggccaccgccgccgccgcttccttcctccccgccgcgctccgggactggaggtttcgggtttcagcccaccgagccccgcttcgctcctcccgcgggccagccaccagcacgcggacccgggcgggcgcaggccaagt

SEQ ID NO: 10523 - RNA, 1150 nt, Homo sapiens
  source 1..1150: mol_type = other RNA
cgcatcccctagggcattggtgacgttgcagattaaagttgtgttgattggtttgtccacaggacggatcaggagctgggcgccctgggccacagcaaagggtggcaggggacccatggtcgtgctccaattatagcctgtgggctctgggttgctgcgagcatcgcaggtcagggtggcctcattctggccaaggtaccagttgttatcatagccagagatggatacctctggggggtagtacacggtgaggttcacagtcagcagctgaggcttctcaaagctctcgtgctccaccttgcaggtcacattcttgccgtccacctggcttgagggcaccaatatccagaggctggtgacagtgactgtgccagacaggaaccctggcacctggctcgtattgggcatcccgcccaggtctgagtgccaggtgatttgggctggcgggcgaccccctgtggagacgcagcgggccatgggcactggctctccagtgagctggaccttctgaacctcagctgtgttctggggcttggcaagcactcggagccagatatccacgctcctgctgccctgcgggaacgtgacgaacaggcaggtgtagttgccttcatcctctacgcgcaacccgaacatcctcagcgaggcattccgcagctccgcgcccagtctggctgccacgaattccagccgtttggactccgaatagctggggccctgcgtttggtggaagacggccatgctgccagattcaccatgccgcgcccaagtcagctgtgacacatgcgtcacctccatgttgggcacctgtaggtagcagggcagcgtcacggagtcgcccaagaagccgggcacctgggtgggcgcctgcacgacgacgtccccggttcctgggggtggccaggacagcaccagtagcgccaccagcagcagcggccacgcggcggccatggctcgggccatgccagttgctccgagcagctgggcctcccgcgggcgtctcctcgcttcccggcgcccgctcgctctgccgcggtcgctgcgagtccagctcccggagctcaggtcctggaatccccggggggccgctcctccagtgcctggggtgggaaggggaatacccacttcttcaagctccagacaagtgact

SEQ ID NO: 10524 - RNA, 1255 nt, Homo sapiens
  source 1..1255: mol_type = other RNA
cgcccctcctgcccccacagtgttcccaagtcttgtctgaggcgtcagggccactgttaccgtgcactccttctgggctgcagcctttgatcttcccaatgagaatctcatctaggaatggatgaaacaccacgcagcgaaaatggaacctgagcccagattctgagccatcagtggctccaaagtcaatttcaacctccctccaggctctccttcagctcctaaaaagggcagaagcaactggtaaagaacgcagggtttggaaactcccacctcctgctgagcagcaaagtcggccccaggcacagctctgacctggagaggaggctaaaaatgccctggtgttgtgaggcgcaggccagcagcccagcaaaaatgcctctgtgggttctcaggccatgctgcaggtggtccccactcacctgactgcaaggaaaacaccaggtggggtctgtgcccacatcgcacactctgaccccaggccctggcattagctgtatgtcaccttgtcactcaggcccttgctcgaagccccaaagtaggagtccaacgctgacctgagaatcagcacgcggctgccccctgcagacagggccaccgggtcgaatcttgccttcctcagacaggtttaatcccaaacacaggcttccacgatgccgtcaaccatttagtcggccaacatgccccccaggacggcagggaccctggcatcagcagggcatgaggagaggcagccgatggacctctcaccctttggtgtgtgatgcgccatccccagggaatacataggcatcctccagtttggtgatatcaaacagacaaatgcagagtcccacgttgtacacgaccttgttggccaacttcttgttcagctcctcggcaatggagtcgttgagcttcctctcaaactgccaaggggggatccggacggtgtccaccatttccaccaggacgaacatcccggcctgcgctgggggctctgggaacaggagggtcagtcacgcaccagggccgggggcagggagaatccccgagccccttggtcccgtcccagtcgctgaggcccccaggctggcggtgaggttgcacggggcggtctcgggggcccggtccgggccatgctccgctactacaacatgaggaaactgaggccagagggaggcactctccgtccacagctccgggtgcgcgcccgcgccgcgagaccccgccacgccacgccactccacgccacgccactccacgccccgcaccc

SEQ ID NO: 10525 - RNA, 817 nt, Homo sapiens
  source 1..817: mol_type = other RNA
cgcccctcctgcccccacagtgttcccaagtcttgtctgaggcgtcagggccactgttaccgtgcactccttctgggctgcagcctttgatcttcccaatgagaatctcatctaggaatggatgaaacaccacgcagcgaaaatggacagacagggccaccgggtcgaatcttgccttcctcagacaggtttaatcccaaacacaggcttccacgatgccgtcaaccatttagtcggccaacatgccccccaggacggcagggaccctggcatcagcagggcatgaggagaggcagccgatggacctctcaccctttggtgtgtgatgcgccatccccagggaatacataggcatcctccagtttggtgatatcaaacagacaaatgcagagtcccacgttgtacacgaccttgttggccaacttcttgttcagctcctcggcaatggagtcgttgagcttcctctcaaactgccaaggggggatccggacggtgtccaccatttccaccaggacgaacatcccggcctgcgctgggggctctgggaacaggagggtcagtcacgcaccagggccgggggcagggagaatccccgagccccttggtcccgtcccagtcgctgaggcccccaggctggcggtgaggttgcacggggcggtctcgggggcccggtccgggccatgctccgctactacaacatgaggaaactgaggccagagggaggcactctccgtccacagctccgggtgcgcgcccgcgccgcgagaccccgccacgccacgccactccacgccacgccactccacgccccgcaccc

SEQ ID NO: 10526 - RNA, 705 nt, Homo sapiens
  source 1..705: mol_type = other RNA
cgcccctcctgcccccacagtgttcccaagtcttgtctgaggcgtcagggccactgttaccgtgcactccttctgggctgcagcctttgatcttcccaatgagaatctcatctaggaatggatgaaacaccacgcagcgaaaatggactttggtgtgtgatgcgccatccccagggaatacataggcatcctccagtttggtgatatcaaacagacaaatgcagagtcccacgttgtacacgaccttgttggccaacttcttgttcagctcctcggcaatggagtcgttgagcttcctctcaaactgccaaggggggatccggacggtgtccaccatttccaccaggacgaacatcccggcctgcgctgggggctctgggaacaggagggtcagtcacgcaccagggccgggggcagggagaatccccgagccccttggtcccgtcccagtcgctgaggcccccaggctggcggtgaggttgcacggggcggtctcgggggcccggtccgggccatgctccgctactacaacatgaggaaactgaggccagagggaggcactctccgtccacagctccgggtgcgcgcccgcgccgcgagaccccgccacgccacgccactccacgccacgccactccacgccccgcacccgcgccacgtgccgccgctcgtatcacgcaccacgcaccacgcaccgcgcacagc

SEQ ID NO: 10527 - RNA, 993 nt, Homo sapiens
  source 1..993: mol_type = other RNA
cgcctgcccagccctcctgctcaccgaaggtcactacccccatatgtctccttgggcttcttccccctctctttctggaacctgaccaggcagaacgcagcaactgacagcaacagcacgcccaggagcaccccaatcagagctccggccactcggccttgggagggttcggtcacagagagggtcagctcacaggatgcactgcccatctggttggtggccacacagcggtaggtgcccgaggaggtcagggagaggttggtgagaatgagctggccagacacctcatcttgaaccatgctgccaggagaaggtgtaggaaaagttccaagacgcacccagttgtacactggcttaggagccccctcggaagagctgcatctcagtgcagtagagcctcccacagaggtttgtccactctgactgcataagggattactggggggaaccagcacagtaaggttgattagccccaacccattggtgtagaaatctggtgggttgttgacttggcagaggtaggttccagtatctgaggggtggacgtcagtcagtttcagtgtggccacccccactgtgggggggttctgaagcaggctgacccgctttgacttagaaccagttggatacagatggccattggtgaagtacaggattggatgggactcagagatgggtttcccaggctgcacaaagctccactccagggcgaagctgtctcccaccgacgtgctgtaggtgcaggtcagctcggctgtcttccccaggggcgtgctcagcggctctgtgggtaccttcacctccacggccagcccactcaggcacaggaagcctagcagggccccgcagagaaagggccccgggagctcggccatggccgcgtccggccgtcctgtcctgctcctgccaggtgggcggtcaaggtcggtctgggtgtcgggcagggaagggagcacccaagggcagccgcccgggctgggcaggagcgagact

SEQ ID NO: 10528 - RNA, 814 nt, Homo sapiens
  source 1..814: mol_type = other RNA
cgcctgcccagccctcctgctttccttgggaggcttccaggcccttggatgacttgatgggaccatttcttgccacaggagccagagggtccagacggcccctccccaatgacacagtgagaagggaggtggcatgtgaatgaaccctgacctctgagatgctcactcctgaaactgtgactcttgagataaggacacaaggaaatgccctgctaactgcttctgcccagccgtctccagcatagcagcccagctcgtcacctcggaaagtgccttagctctctgctgtcagcccacattgctgcagctcccaggccctgatatcctaacagcacgttccctttggtaattggccagcagcttctgctgtttgcatctagaaaccccaaatgacaaaacggctcacagcctgttcaagacagagggcaacgccacacctctaggaagccacccctccaggcggaaggttttccatgcagagctgtgttatatgtgcagtcttctccctgaaatatgggtgtgatgtacggagcacacgcagccaccctgcagcatgagatgactgttgagtacaggacacgcagaacgaagcttggaaagctgcagagctgacttcaggttgtgccaattcctgtgctgcctcatccctcatgtacataaagcgtgaggcgcgcaggcctgcacctgcgccatccctcatccacctaaagcgcgtggcgcgcaggcctgcgccggcgccatccctcatctacgcaaagcgtgcgacgctcaggcctgtgcctgcgtcatccctcatctacgcaaagcgtgcgac

SEQ ID NO: 10529 - RNA, 1070 nt, Homo sapiens
  source 1..1070: mol_type = other RNA
cgcgccgggcccgggttggccgctgacccccgcggggcccccggcggccggggcgggggcgggggctgccccggcgctgcccccgttctgggcggcggcggggggcggcacggcgggcgcggcggtcgggggtccggcggggtggccgggcggccgggccagagtggcgggcgcggggggtggcgggggcggggcggcggcgggggcggcgggcgcgggggcggcggggggcgagggcgcggcgggcgcggggggcgcggcggcgcccacgaaggggggcgtctggatgacagtgccgggggcggcgggcttgggcagcggcagcagcgcggcgggcccgttgttgaccaggctgacagcaggtgcggcggcgtggtgcgagttcagcagcgcggcgctcccattcaaagtttgcgcggcgccggggccggcgggcttgccagggccagggccggggccggggccggggccgggcccggggccggggccggcgcgggcggccagcgcggcggggccggcgggcttggcggggccggcgggggcgggctcgggccccgcggcgacggcggcggcggcgggcaccggggcgcaggaccccgcgctgccctcgggcggcggcctcagcttcgcggcgggcggcgcgggccctgcggggacaagggggcggcgcggtgagggggggcccgggcgctgcggccccccgccccccggccgcgctctacctgcggggggcggctccggcgccgctccgggcgcgccctcggcgggggcggccggccctgcgcccgcggctccggccgggctgccgctcacaacatggttcccgagcgcgccggcggccgcggcccgcacctcgggcgtgcgcggcgcgaggtggtggtggtgggccgcgctggccgccagctgcgactccagcgagcccaccaggtcgctcaccactttctcgtccacctcgctgttgaagaagacctcgtccagcagatccgagcccgccgccatcttttttcctcggccgccgccgccgccgccgctcgggccgagcgcgcctgggcgaggaggaggttccgact

SEQ ID NO: 10530 - RNA, 285 nt, Homo sapiens
  source 1..285: mol_type = other RNA
cgcgcctgcaggaactggtagatctcgctcagcgtcaggcgcttggtgggtgaactctggatggccatgacgatgagcgcgatgtaggaatagggcggcttctccgggcgccggatgccggcgttggtcttcttggccttggacgggccggacgacgcggggtccatggccgcgccgcctcccccgccgccgccgccgccgccgccgtgcggtggctgctgcttctcgggcgccgaagacatcgggtggctgctgccgccgccgccgctgccgccgctgctctgc

SEQ ID NO: 10531 - RNA, 770 nt, Homo sapiens
  source 1..770: mol_type = other RNA
cgcgcctgcaggaactggtagatctcgctgagcgtcaggcgcttgctgggcgagctctggatggccatgacgatgagcgcgatgtacgagtagggcggcttctcgggccgccgcagccccgagctcgccttcttggcgcccccgctcccggcgcccgcgccgccgccgcccgcgctcttgcaggcagccgagggggcgctggccgaattggaggaggacgaggacgaggcgcaggaggcggaggacgacgacgaggaggaggaggtggtctccggggcggcggcggcggcggcggcggcggcgggcggcgggctcatcagggcggcctggagcgcgccggggaccgggctgcacgcgcggcggagcggggccggcggcggcccgccctcggtggtcatctgggacccgggagcgaggccgggccgcgagggcgggccccgggcgggaagcggaggcgccggagcggggtcggcccagaagccctgcgagcgccctagcccgccgcccgggctgcagccgtggccactccgggccagcgcttcggcgtcgcctccctcagctcctctggggcttctggcggcggcggcggcggcgggcgggaggcaacgcccggcgcatccctccccgagccgcgggccctgccttgcgcaacggcctcccaggccgcggggccgagcggccggcgccgggcgactgcgcccgcgagtgggaccgcggcctggaccccggggacgagcccgacgtctcccttcaggagcgctcctcgctct

SEQ ID NO: 10532 - RNA, 69 nt, Homo sapiens
  source 1..69: mol_type = other RNA
cgcgggcgctcctggccgccgcccgcgcggctgtgcgctggccgtcatagcgcgcgggaggacgcgcct

SEQ ID NO: 10533 - RNA, 361 nt, Homo sapiens
  source 1..361: mol_type = other RNA
cgcgggcgctcctggccgccgcctcctcctcgttctcctcctcctcctcgagctccacagcgcccactgcctccaggccggcccccgaggttaggcgaagggtcggggcttctctgaagtctcgcgcctcccgggctgccacctgggctgccattgggcaaccgtccgagggaacgcgaggccggctggctcctcacccgagactctgggccccccgaagtgagcgaggacacctccgcaggcgcccaccctcctccgcggtcgccgcgagcgcagaccctagtctcccacctgctgctacttagcagccgcgccactgcgcacagctgtagcctcgcaggccgaagcgaaggcctgggac

SEQ ID NO: 10534 - RNA, 52 nt, Homo sapiens
  source 1..52: mol_type = other RNA
cgctggcagtgttggtgacactgggacacccggcgagcgcggcgagaccgac

SEQ ID NO: 10535 - RNA, 53 nt, Homo sapiens
  source 1..53: mol_type = other RNA
cgctggcagtgttggtgacactgggacacccggcgagcgcggcgagaccgact

SEQ ID NO: 10536 - RNA, 3900 nt, Homo sapiens
  source 1..3900: mol_type = other RNA
cggatgagcaaagaaagtggttgcttgagatgaaatctactcctggtgaagatgctgtgaacgttgttgaaataaaaacaaaagatttagaatattccataaacctatttgataaagcagtaactgagttttagagatttaagaggattgaaagaagttctactgtggataaaatgctatgaaacagcatcacatgctacagagaaatctcttgtgaaaggaggagtcaatcaatctagcaaactttattgtcttattttaagaaattgctacagcacccaggaattcgatgccacggtaagctataatcccaccactgccctccagcataggtgacggagcaagaccctatctagaaaaaaaaaagaaggaaaaaaaagagtgagaaagaaaatgctacagctttcagtaataaccagcctgatcaatcagcagctatcaccatcaagacaagacattcctttagcaaaaagattatgattcaccaaaggctcagttgattgtagtgaaaacataacttttatgcactgggaaaccaaaatatttgtgtgacttgctttattgtgatattagttttagtgctgtcatctggaatcaaacctgcaatatcttcgaggtatacctctaaatgtccatgggtgatttcataattggccaagtgttcctgttgtatggtgccttccctgattcacacagttacaaatgattaccctttcttttgctctcattttatcttagttagtattattttttttgtatcaattttcatgtttcctttattatgccatgtgctttgaccattccttatacatttagacaaaagaaacagacatatgatcaagagaattcagcatgcaaattacactcagaaagcaaagcaattcagtgtggtcaaagcaaaagttgcactatggtcttgtatagcctattattttatcctgaaattggatttgaagccaaagtgtgatatgaggaggtttgtctctttagaatactttggcagatagtattggctgaaatcagatatggggcaactaataaggaatcttctgcagtaatccagggaagaaatggtgaggatcttaatgtagtcacaatgaggaacctggagatatttggaaaataaactagagcagtacttctcaaacttccctgtactttaggaccacctagagagacttgaaaaactctgatgcctgcacctcactccatacaaggtaacacagaatccttggaattattattattttttaactctctaggtaatttcaatgctcagccaagtacttggttaatcactggatgtgggcgacaaagataggtattcctagttttctgatctgggacaaaagagtgaaacaaaagcatatatagtgtggataaataagcaaatttagagtggagaaatttaagtttggttttggacaaatggaaattaagtgctaacgggtagtcgtatatgcaattcttgcacttaggaaaaagatgcagtttagaggtatacactttcgagattttctgcatgtattaatagatattatttacagtcattgcgaatatgatgtctagtgaatgcatgtgaaatgagactaaaagaggactgtgagtggactctgggagcatcaacatgtgagaaattgacagaggtagaaaaagaacaccaaaaaaaaaaaaaaaaagaggaaaagtaagtggtatctccaaagctcagttagaagaggggttcaagaaactggaggtggttagtagtcttaaatgctgaagagagtttagtacagatctgggctgaaaagtatataatatatttggtgaggtcactgttaaccttggggagatcagttcctaagcatattggggacagaaactaaataaaaatatattatggagtgatcaaaaggggaggaaaaagcaagttactgtagctcctagagtggtacagtggttgtttcctgttgtgttggaaaacatctctgattttttatagaaactcttgtatattgtttaaatgttacttttctatatttgaaatagttgtgtaaataagacatttgtcagccccaaaataaaccaaaaaatgatgaatttttaaataattttaaaagacaacttgtaagcatactagtctcatttatgaccattaagtaagcaatgaacaaataaaattagaaaagcttattatttcaccttaaatgtcttatagtcaatgtatatatttcaggaatattgcaccaatctcactttcactaaatttgaactaaggcataaaggacatctaaaatttgaatgttgtatggttaattaacatttaataaacttattttctttgtttaaatgtctttgaaaatcaaatgtctcatgctgtttttcctcatcaatgtaatcccagtagtcttaggaatgattttgttgaattgtttgacaaaacctaacttggctgcttgtaatttatagttgttcacccccgtcactttgcagtttttccctactaaaaaatttagattgtcttgaagctgaattgttgactggatttcctatgtagttcacagtatggttacagaataccaaaatagcattgtcaatgtgttttaaaaagcatagacctgaagtcaatgggaatttgacaagacagcctgcatgttattgtaagccattgcaagttttatgttgttcttcaccttaatttttaatgtgtaaactttaatgaaattcagtttttaaaagctacttaataaaataattttatttattccctaaggaaatggaattgtcaaaacaaaaaaagttgaccattaaatttgattcttttatttaaaatttcaaaggatgacaatggaagccatatagcactactttttttttttttgccaaataagcatctgcacattgtttttcacctttgagataccataatgtatctctcccatctgtggtcacccctccccagtcagaggctgccccaccagcattcagtggcatgattctcgcaatgtcctgaacaactctctgtatgatatttatttcccttcatcaagtccaattgtagtgcctcatgcttctcagcaacgtgtatcaagtatgtgctttgggctagcaaaacctagtcgttaaaagcacagactcttgctcagtcacactgcctggctctgggtcctggcgctgttccttatcagctatatgactgtcaggtgtcattgccttggcgtcttcatcgcatgacatggttttgagacaggtcatattatccacagttgacacttgagcagctggagacaaagaagattgactgacttgtccaaatcatccccaattccttagctacaggcgtaagattagaactcagggttcagcaggctgtgctcatccatgctcactaccaaaccatcaaggaaagagcagcatggttttcagcaactctcaaataacatgaagacctttaaaatcggattaggaaagcaaaaccataaggaaaccatgttaaaaacaggctcaatgatcaaatggactttaacaaatgtgcagaagaaaaagcagactcactaatgaataaagataggcaagactatcaaccgattaatgactagctggagttcttaaatttgttgaggtcctacttaaaattcacaaagcaggaaaaaataggctaaaatcttaaacaattaggaaggaaagagaaagaagaaacaactgttgccctaaagaaaggtctggtgtacttagaaagtagtgaactattttttaagcctttgcatgtgataaacctgttaaaatactcttataaccaattcaagcttctagttggccttaccgaaaaataaaccgcggcactggaaaaattatagaagttaggtaaaagaatataaaatttgaatcagctagtttattcctccatctctaaaatta

SEQ ID NO: 10537 - RNA, 763 nt, Homo sapiens
  source 1..763: mol_type = other RNA
cggatgagcaaagaaagtggttgtttgaaaaggaatctattcatggtgaagactctgtaaatattgttgaaatgacaacaaaggatgtggaatagtgcataaacttagttgaccaagcagagacaaggtttgagagaattgactccaattttgaaagaagttctactatgggtaaaatgctatcaaacagcattgcatgatatggagaaatcctttgtgaaagggagtcaatcaatgcagcaaacttcattgttgtcttattttaagaaattgccatagccattcccaacattcagaaactaccattctgatcagtcagcaacctgaccctgatcagtcagcacctatcaacattgaggcaagaccttccacaagcaaaatgactgtgaatctagtgggcatggtgatgtgggcctgtagtcccagctcctcaggaggctgaagcaggaggactgcttgaccccgggagtttgaggctgtagtgtagtatgatcacatctgtgaataagccactgtactcaatcctggagaacacagcaagactccatctatttctgcctttgaatcacggatccttcatctcccaaggccttagagttagaagacagatttctacttctggaaatctgccttgggcacacaaaagagcaggcgcgacctcggaccagctccgaggcaaaattcactcagcgcgggacagcgacagggaatccggccgcacctgtgcctgcagtctcattgctcggaacggcgcgccactgtg

SEQ ID NO: 10538 - RNA, 2767 nt, Homo sapiens
  source 1..2767: mol_type = other RNA
cggatgagcaaagaaagtggtttcctgaaatgaaatctactcctgaagatgctgtgaacattgttgaaaagacaacagacttagaatattacatcaacttagttgatcaagcagtggcgaagtttgagaggattaagtccaattctaaaagaagttccactatgcgtaaaatgttatcaaacagcgtcgaatgctaaagagaagtttttcatgtaatgaagagtcaatcaatgcagcaatcttcactgctgtcttattttaagaaactgccacagccaccctgatcaacagccatcaacactgaggcaagacctaccacaagcaaaaagattacaactcaccaaagtctcacatgatcattagcactttttggcaataaagtattttaaactaaggtactttacttagacataacacaactgcacacaagagactaccatatgatgtaaacctaacttatatgcactgggaaaccaaaacatttgtatgattcatgttattgtgatattcactttatagtggtagtctggaacaaaactcacaatatctacagggcatgcctgtatcttgtatcaatagggtttctcttctccattgcaacatcttatatacttagaaaggcctaaggaaataatgagggctttctgtgttttctacattgtatggccccatggtgagttctcaaatgttggattgtgaccacaatccaatcccttgagaaaagaatgtgtattaacaacgacttacaaaaaaaaaaaaaaaaaaaaaaaaaaaaaaaaaaggccaggagcagtggctcactcctataatcccagcactttgggaggccaaggcgggtggatcacctgaggtcaggagctcgagaccagcctggccaacatggtgaaaccccatctctactaaaaatacaaaaattagctgggtgtggttgacggcacctgtaatccaagctacttgaaggctgaggcagaatcgcctgaacccaggagacaaaggttgcagtgagctgggatcatgccattgcactccagcctgtgtgatgacaacagcaaaactctgtctcaaataaaataaaataaaataaaataaaataaaataaaataaaataaaataataaaaaaagattccattggctccctaacattcctaaaatttataggggacacatagagtatgagttctttcatgtcttcgaagtgaatggggataactgaaggcctcctcacattctttgtaccaataaaatttctcttcagtgtgaattcaaatgtggtaattatggtatgagaaattcctaaaagatttccacattccttacattcagagtttttcttcagtgtgtttttaaatgtttagtaagtaaataaaatctattgtaggctttcccacattcgttacatatatagggtttctctccagtgtgaattctaacatgtttctgtagatgtgaagaagcacggaaggttttcccacattccttacatatatacggtttctctccagtgtgagttcttatatgttcaatgagttgtgaagatgtagcaaaggctttcccacagtccttacattcatagggcttctctccagtatggatttttacatgattatgtaagcttgaggaaacagtgaatgctttcccacactccttacatttatagggttttattccagtgtgaattctaaagtgattcttaaggcatgaagagcttctgaaggattttccacataccttacattcaaagggcttctcctctgtgtgagttttaaaatgttcagttagtagataaaacctattgtaggctttcccacattcgttacattcatagggcttctctccagtgtgtattcgtacatgtttagtaaggcctgagcgcccagcgaaggctcttccacattccttacattgataaggtttctctccagtatgaattcttacatgttcaactaggtgtgaagaaacagtgaagcatttcccacattccttacattcatagggtttctccccagtatgggttcgcatgtgactattaagatatgaagaatatctaaagaattttccacattccttacattcgtagggtttttctacagtatgcattttaacagacacagcatggcttgtggagtaagtaaaagctctcccacattgcttctgttcatagagtgtttctccattgtgagttatcctatttgcctgaagatgtgactgatcaacaaaggcttcctcacagtcactgtattcaaaggatttgtctcctatccacgttctctggtgaacatttggtggcaggctgaaggcttttctgcactgattcaacacagaaagtgtctctccagcaggggcactgttgtgtaacatgggaaagttttctccatactcatcacagtcataagtgtcccctgtattttcagttcccatgtgtgcattaaggcatgagtgttcactgaagatttctccattttccataaagtcacagagttcccctccattgtggatttctgccataaaataggatcagcaggaggcctgagcttgttttcctgcaactagacagtcccatcatttgtatgccgtttgatgttttgttaagccaaaaaaaaatgttgttgaggtgctgacactttggttttaacttgccattcttggggaactccggttggcaatgtgctcaacttttccttctcctcctccagtcaagagacagactgagtttgaataggtccacagccagggtggactccaccacgataaaggcgaaatggcact

SEQ ID NO: 10539 - RNA, 2709 nt, Homo sapiens
  source 1..2709: mol_type = other RNA
cggatgagcaaagaaagtggtttcctgaaatgaaatctactcctgaagatgctgtgaacattgttgaaaagacaacagacttagaatattacatcaacttagttgatcaagcagtggcgaagtttgagaggattaagtccaattctaaaagaagttccactatgcgtaaaatgttatcaaacagcgtcgaatgctaaagagaagtttttcatgtaatgaagagtcaatcaatgcagcaatcttcactgctgtcttattttaagaaactgccacagccaccctgatcaacagccatcaacactgaggcaagacctaccacaagcaaaaagattacaactcaccaaagtctcacatgatcattagcactttttggcaataaagtattttaaactaaggtactttacttagacataacacaactgcacacaagagactaccatatgatgtaaacctaacttatatgcactgggaaaccaaaacatttgtatgattcatgttattgtgatattcactttatagtggtagtctggaacaaaactcacaatatctacagggcatgcctgtatcttgtatcaatagggtttctcttctccattgcaacatcttatatacttagaaaggcctaaggaaataatgagggctttctgtgttttctacattgtatggccccatggtgagttctcaaatgttggattgtgaccacaatccaatcccttgagaaaagaatgtgtattaacaacgacttacaaaaaaaaaaaaaaaaaaaaaaaaaaaaaaaaaaggccaggagcagtggctcactcctataatcccagcactttgggaggccaaggcgggtggatcacctgaggtcaggagctcgagaccagcctggccaacatggtgaaaccccatctctactaaaaatacaaaaattagctgggtgtggttgacggcacctgtaatccaagctacttgaaggctgaggcagaatcgcctgaacccaggagacaaaggttgcagtgagctgggatcatgccattgcactccagcctgtgtgatgacaacagcaaaactctgtctcaaataaaataaaataaaataaaataaaataaaataaaataaaataaaataataaaaaaagattccattggctccctaacattcctaaaatttataggggacacatagagtatgagttctttcatgtcttcgaagtgaatggggataactgaaggcctcctcacattctttgtaccaataaaatttctcttcagtgtgaattcaaatgtggtaattatggtatgagaaattcctaaaagatttccacattccttacattcagagtttttcttcagtgtgtttttaaatgtttagtaagtaaataaaatctattgtaggctttcccacattcgttacatatatagggtttctctccagtgtgaattctaacatgtttctgtagatgtgaagaagcacggaaggttttcccacattccttacatatatacggtttctctccagtgtgagttcttatatgttcaatgagttgtgaagatgtagcaaaggctttcccacagtccttacattcatagggcttctctccagtatggatttttacatgattatgtaagcttgaggaaacagtgaatgctttcccacactccttacatttatagggttttattccagtgtgaattctaaagtgattcttaaggcatgaagagcttctgaaggattttccacataccttacattcaaagggcttctcctctgtgtgagttttaaaatgttcagttagtagataaaacctattgtaggctttcccacattcgttacattcatagggcttctctccagtgtgtattcgtacatgtttagtaaggcctgagcgcccagcgaaggctcttccacattccttacattgataaggtttctctccagtatgaattcttacatgttcaactaggtgtgaagaaacagtgaagcatttcccacattccttacattcatagggtttctccccagtatgggttcgcatgtgactattaagatatgaagaatatctaaagaattttccacattccttacattcgtagggtttttctacagtatgcattttaacagacacagcatggcttgtggagtaagtaaaagctctcccacattgcttctgttcatagagtgtttctccattgtgagttatcctatttgcctgaagatgtgactgatcaacaaaggcttcctcacagtcactgtattcaaaggatttgtctcctatccacgttctctggtgaacatttggtggcaggctgaaggcttttctgcactgattcaacacagaaagtgtctctccagcaggggcactgttgtgtaacatgggaaagttttctccatactcatcacagtcataagtgtcccctgtattttcagttcccatgtgtgcattaaggcatgagtgttcactgaagatttctccattttccataaagtcacagagttcccctccattgtggatttctgccatttgtatgccgtttgatgttttgttaagccaaaaaaaaatgttgttgaggtgctgacactttggttttaacttgccattcttggggaactccggttggcaatgtgctcaacttttccttctcctcctccagtcaagagacagactgagtttgaataggtccacagccagggtggactccaccacgataaaggcgaaatggcact

SEQ ID NO: 10540 - RNA, 630 nt, Homo sapiens
  source 1..630: mol_type = other RNA
cggatgagcaaagaaagtggtttcctgagatggaatctattcctagggaacatgctgtgagcatgtcaaaattacaacaaaggattcagaataaacttaattgacaaagacgtggcagggtttgagggaactgactcctattctgaaagaagtcctactgtgggcaaaatgctaaacagcaacgcatgctacaaagaaatcttttgtgaaaggaagagtccatcaatgtggcaaatttcattgttgtcttcttttaagaaactgtcgcagccaccacctcaaccttcaaccaccaccaccgtcatcagtcagcagccatcaacatctgggcaaaaagactatgactcgacttgctaaaaactcagatgatccttagcatttttcagtaataaaatattttaaaattaagatccgtacattgtttaggcataaggctactgccctattcacagacggcaatacagtgtaaacataactttgtatgcactaggaaaccaaaaactgtgtgtgacttgctttactgccgtatttgctttatgtgatggcctgaaatcaaacccacaattttctcagacgtgtgtctgtacatttgtccaaacccatagaatgtacaaaagcaagagtgaaccc

SEQ ID NO: 10541 - RNA, 555 nt, Homo sapiens
  source 1..555: mol_type = other RNA
cggatgagcaaagaaagtggtttcttcagatggcatctatactcctggtgaagatgtaagtgaaagtggatcatcaaaggtcttcatcctcattatcttcacgttaaagcaggctaagtgggaggaggggttggtcttgctatctcagggatggcagaggcggaagaaaatccacatgtaagtggacccacacagctcaaacccatgttgttcaagggtcaactgtactttgatttcttctgagctgcagtctcccctttctctaccctcacttccctccaccactagctccattcctgactactttcttctactgttctcaagcccaggatacatcagctctccctggcagatggttggtgctccatgaatgtcgggtccatttcttggatttatgcaggtcccagttttctattaaagagtaagctccacatggtcaaacatgttcttacttcctgtattttgtgtcagcagtttgtcagcttagcacaaaaagtacctgatgaataatttctgccaccaaagtcatgttgttttttctaaccaatttttttt

SEQ ID NO: 10542 - RNA, 349 nt, Homo sapiens
  source 1..349: mol_type = other RNA
cggatgagcaaagaaagtggtttcttcagatggcatctatactcctggtgaagatgtaagtgaaagtggatcatcaaaggtcttcatcctcattatcttcacgttaaagcaggctaagtgggaggaggggttggtcttgctggcagatggttggtgctccatgaatgtcgggtccatttcttggatttatgcaggtcccagttttctattaaagagtaagctccacatggtcaaacatgttcttacttcctgtattttgtgtcagcagtttgtcagcttagcacaaaaagtacctgatgaataatttctgccaccaaagtcatgttgttttttctaaccaatttttttt

SEQ ID NO: 10543 - RNA, 61 nt, Homo sapiens
  source 1..61: mol_type = other RNA
cggatgagcaaagaaagtggtttcttgaggcgcaaaccactttctttgctcatccgtaaga

SEQ ID NO: 10544 - RNA, 37 nt, Homo sapiens
  source 1..37: mol_type = other RNA
cggatgagcaaagaaagtggtttcttttttctttttt

SEQ ID NO: 10545 - RNA, 1736 nt, Homo sapiens
  source 1..1736: mol_type = other RNA
cggcccgggctgctgctgttcctctcactgctttcatagccagattccattcgctggattagtcgggggtgctgctctaaaaggtgagagcctggccgtgctgggccccagcgcttgtactgggggcttggtccaccaaatttaatgtcgtaagaaggtggcttgcttggttcatctggtataaattctttagctgaatcctcagaaaaggggctaagctgggtatagccacagtgcttccttttgtccttactaaagatactgtcaatattcagagattctcgtttgggtctccatgtgggacgatacttgctggaagaactggattttgactcactgctggtactctctatttcccagtcacgagagtgtaaaggcagggtcctaggaggttttttgtcaggctggtctcctcctctgcccctgcagtgagagcctacattggtctgagaagccagggatggtctgttatggatcatattgctgactgtctctttaaaatctctcagcctgttggtgctgctggatggtttggaggcatttctaggagcctgcttctctttcagtgtttctccttcactgtggtatcccgaggcctggggctcatcgcctttcctcctaacccgaccagagctcctcttgcgctctatcagtgaccctttcttggatgtgtgtttctgattacattcactatcagtcaggtgtcctgaatcttcactgtcgtagcatgtcctgctgtatgactggaactcagcttggggaggcaggtcctgggtggaaactggggtaccctggggatctgcataaagcagcagcaggggctgataatgccccttgatgcatttggtcaccacatccttccatttgggcccaatctccttgacatgagcatcatcaaaatacatccatttgcgaatctttgtttgaaaaaagaatgtagaataatgtttgccatagtaacagatcattccaactaagtacagttcagattgcttggcccggtcatccgtcactctgaaaaacagatcacccagcttaaggcaggttcccaggctgtggataacatcttctgctaagtctgagtggtctgagtcccataccagcccaatcgtgataatctgtggagcattcatcaacacacggcgaatcctgatcctctctccacagttgcttggacagttccgcagatcccccatggtgctggcattctgcagcagctcaccaaacatgcttggtgaaggtttctctcgtctttccagcatacaaatagcctgattgcaaagggaagtggtggagatataatgtaccatctggatgaaaggcagcggatcagaagtggcaccacagctagtacatacacactgctcaaacaatgtcattgcaaatttctgatgggaaatgcagtgttgggcagtacatatatcctctttggtttcatcagcaatgtggaagtgaattctcatcaggaggttttcaaagcactctgcagcatcatccataattcccagctggaaacgttgttcatcctggaaagtctttgccagagcactgcggagagtgtcagatggaagcactttttcactactacactgaaactggttaaagattccctcttaattacaggcagccttcctcatacacactgagaatctgaatgcattcagaatggcctctgactacatcttctttattctcttattttaattattgttgtcagtcttgctctgctattgtta

SEQ ID NO: 10546 - RNA, 1932 nt, Homo sapiens
  source 1..1932: mol_type = other RNA
cggcccgggctgctgctgttcctctcactgctttcatagccagattccattcgctggattagtcgggggtgctgctctaaaaggtgagagcctggccgtgctgggccccagcgcttgtactgggggcttggtccaccaaatttaatgtcgtaagaaggtggcttgcttggttcatctggtataaattctttagctgaatcctcagaaaaggggctaagctgggtatagccacagtgcttccttttgtccttactaaagatactgtcaatattcagagattctcgtttgggtctccatgtgggacgatacttgctggaagaactggattttgactcactgctggtactctctatttcccagtcacgagagtgtaaaggcagggtcctaggaggttttttgtcaggctggtctcctcctctgcccctgcagtgagagcctacattggtctgagaagccagggatggtctgttatggatcatattgctgactgtctctttaaaatctctcagcctgttggtgctgctggatggtttggaggcatttctaggagcctgcttctctttcagtgtttctccttcactgtggtatcccgaggcctggggctcatcgcctttcctcctaacccgaccagagctcctcttgcgctctatcagtgaccctttcttggatgtgtgtttctgattacattcactatcagtcaggtgtcctgaatcttcactgtcgtagcatgtcctgctgtatgactggaactcagcttggggaggcaggtcctgggtggaaactggggtaccctggggatctgcataaagcagcagcaggggctgataatgccccttgatgcatttggtcaccacatccttccatttgggcccaatctccttgacatgagcatcatcaaaatacatccatttgcgaatctttgtttgaaaaaagaatgtagaataatgtttgccatagtaacagatcattccaactaagtacagttcagattgcttggcccggtcatccgtcactctgaaaaacagatcacccagcttaaggcaggttcccaggctgtggataacatcttctgctaagtctgagtggtctgagtcccataccagcccaatcgtgataatctgtggagcattcatcaacacacggcgaatcctgatcctctctccacagttgcttggacagttccgcagatcccccatggtgctggcattctgcagcagctcaccaaacatgcttggtgaaggtttctctcgtctttccagcatacaaatagcctgattgcaaagggaagtggtggagatataatgtaccatctggatgaaaggcagcggatcagaagtggcaccacagctagtacatacacactgctcaaacaatgtcattgcaaatttctgatgggaaatgcagtgttgggcagtacatatatcctctttggtttcatcagcaatgtggaagtgaattctcatcaggaggttttcaaagcactctgcagcatcatccataattcccagctggaaacgttgttcatcctggaaagtctttgccagagcactgcggagagtgtcagatggaagcactttttcactactacactgaaactggttaaagattcccttgagagcgcaaaagatgcaggaatctcccatgcacttgtgagttgtaagctgcctaaagctacgtcggaagatatccaagtgccacaaaacctgcagggcactgttgaggaagcagctgttttgccctggctcattgctgaggcctttgctgggggctatggaggttgagcttcgaggtgcaaacatcccttgtacactaccacgaccccctgaaaaataatttctcttccaagacattattgttcacatttagccagacagcacagtcaacctccagcaaaagacctctaatcacgagggtatctgtggggcaagtgat

SEQ ID NO: 10547 - RNA, 2138 nt, Homo sapiens
  source 1..2138: mol_type = other RNA
cggcccgggctgctgctgttcctctcactgctttcatagccagattccattcgctggattagtcgggggtgctgctctaaaaggtgagagcctggccgtgctgggccccagcgcttgtactgggggcttggtccaccaaatttaatgtcgtaagaaggtggcttgcttggttcatctggtataaattctttagctgaatcctcagaaaaggggctaagctgggtatagccacagtgcttccttttgtccttactaaagatactgtcaatattcagagattctcgtttgggtctccatgtgggacgatacttgctggaagaactggattttgactcactgctggtactctctatttcccagtcacgagagtgtaaaggcagggtcctaggaggttttttgtcaggctggtctcctcctctgcccctgcagtgagagcctacattggtctgagaagccagggatggtctgttatggatcatattgctgactgtctctttaaaatctctcagcctgttggtgctgctggatggtttggaggcatttctaggagcctgcttctctttcagtgtttctccttcactgtggtatcccgaggcctggggctcatcgcctttcctcctaacccgaccagagctcctcttgcgctctatcagtgaccctttcttggatgtgtgtttctgattacattcactatcagtcaggtgtcctgaatcttcactgtcgtagcatgtcctgctgtatgactggaactcagcttggggaggcaggtcctgggtggaaactggggtaccctggggatctgcataaagcagcagcaggggctgataatgccccttgatgcatttggtcaccacatccttccatttgggcccaatctccttgacatgagcatcatcaaaatacatccatttgcgaatctttgtttgaaaaaagaatgtagaataatgtttgccatagtaacagatcattccaactaagtacagttcagattgcttggcccggtcatccgtcactctgaaaaacagatcacccagcttaaggcaggttcccaggctgtggataacatcttctgctaagtctgagtggtctgagtcccataccagcccaatcgtgataatctgtggagcattcatcaacacacggcgaatcctgatcctctctccacagttgcttggacagttccgcagatcccccatggtgctggcattctgcagcagctcaccaaacatgcttggtgaaggtttctctcgtctttccagcatacaaatagcctgattgcaaagggaagtggtggagatataatgtaccatctggatgaaaggcagcggatcagaagtggcaccacagctagtacatacacactgctcaaacaatgtcattgcaaatttctgatgggaaatgcagtgttgggcagtacatatatcctctttggtttcatcagcaatgtggaagtgaattctcatcaggaggttttcaaagcactctgcagcatcatccataattcccagctggaaacgttgttcatcctggaaagtctttgccagagcactgcggagagtgtcagatggaagcactttttcactactacactgaaactggttaaagattcccttgagagcgcaaaagatgcaggaatctcccatgcacttgtgagttgtaagctgcctaaagctacgtcggaagatatccaagtgccacaaaacctgcagggcactgttgaggaagcagctgttttgccctggctcattgctgaggcctttgctgggggctatggaggttgagcttcgaggtgcaaacatcccttgtacactaccacgaccccctgaaaaataatttctcttccaagacattattgttcacatttagccctctattgccttgtctcatcatcctctgaagcaaaaactcaaattctgagcaactgcaaaaggttccacaaagccaagaagaagcctgtttgaatcatctgaggtttttgttgatgttcttgctgcttctttttaatgtgccccaaacttctattgtcccatccagatcttcagcaagtctctcctctttcttctgggactagaatagccagctgtgtcagagagagctcctggcgccgcatacttaaccgccgcggctgctatagctac

SEQ ID NO: 10548 - RNA, 2598 nt, Homo sapiens
  source 1..2598: mol_type = other RNA
cggcccgggctgctgctgttcctctcactgctttcatagccagattccattcgctggattagtcgggggtgctgctctaaaaggtgagagcctggccgtgctgggccccagcgcttgtactgggggcttggtccaccaaatttaatgtcgtaagaaggtggcttgcttggttcatctggtataaattctttagctgaatcctcagaaaaggggctaagctgggtatagccacagtgcttccttttgtccttactaaagatactgtcaatattcagagattctcgtttgggtctccatgtgggacgatacttgctggaagaactggattttgactcactgctggtactctctatttcccagtcacgagagtgtaaaggcagggtcctaggaggttttttgtcaggctggtctcctcctctgcccctgcagtgagagcctacattggtctgagaagccagggatggtctgttatggatcatattgctgactgtctctttaaaatctctcagcctgttggtgctgctggatggtttggaggcatttctaggagcctgcttctctttcagtgtttctccttcactgtggtatcccgaggcctggggctcatcgcctttcctcctaacccgaccagagctcctcttgcgctctatcagtgaccctttcttggatgtgtgtttctgattacattcactatcagtcaggtgtcctgaatcttcactgtcgtagcatgtcctgctgtatgactggaactcagcttggggaggcaggtcctgggtggaaactggggtaccctggggatctgcataaagcagcagcaggggctgataatgccccttgatgcatttggtcaccacatccttccatttgggcccaatctccttgacatgagcatcatcaaaatacatccatttgcgaatctttgtttgaaaaaagaatgtagaataatgtttgccatagtaacagatcattccaactaagtacagttcagattgcttggcccggtcatccgtcactctgaaaaacagatcacccagcttaaggcaggttcccaggctgtggataacatcttctgctaagtctgagtggtctgagtcccataccagcccaatcgtgataatctgtggagcattcatcaacacacggcgaatcctgatcctctctccacagttgcttggacagttccgcagatcccccatggtgctggcattctgcagcagctcaccaaacatgcttggtgaaggtttctctcgtctttccagcatacaaatagcctgattgcaaagggaagtggtggagatataatgtaccatctggatgaaaggcagcggatcagaagtggcaccacagctagtacatacacactgctcaaacaatgtcattgcaaatttctgatgggaaatgcagtgttgggcagtacatatatcctctttggtttcatcagcaatgtggaagtgaattctcatcaggaggttttcaaagcactctgcagcatcatccataattcccagctggaaacgttgttcatcctggaaagtctttgccagagcactgcggagagtgtcagatggaagcactttttcactactacactgaaactggttaaagattcccttgagagcgcaaaagatgcaggaatctcccatgcacttgtgagttgtaagctgcctaaagctacgtcggaagatatccaagtgccacaaaacctgcagggcactgttgaggaagcagctgttttgccctggctcattgctgaggcctttgctgggggctatggaggttgagcttcgaggtgcaaacatcccttgtacactaccacgaccccctgaaaaataatttctcttccaagacattattgttcacatttagcctgaaaaaaaaatggagaaggatttgtgcctttttggcaggaatttctgtctgctaaagttctaaaaggaaagggaatccagaatttagtgaatttattttggaagattttgactttaccaccttccaaatatcatctgtgtagtcaagggactcaggtatcctcctagatcaagatgacagagccctccctcacttgttccaaacaatctccaaaatgtaacatggcacaggactaatgcaaacagagaaatccttaagtattgcttccttctatttttcttgaacagcctccataaagtcctggtgaagtggatgtaattctcaactccaacagcatccaggatcagggtaagatgtgttcttcaggcttgttgataatgcttcttatggactgaagatttttccaactggaaggagaggcagacagagaagcaagaatccaacatgatcctcctcaccctctattgccttgtctcatcatcctctgaagcaaaaactcaaattctgagcaactgcaaaaggttccacaaagccaagaagaagcctgtttgaatcatctgaggtttttgttgatgttcttgctgcttctttttaatgtgccccaaacttctattgtcccatccagatcttcagcaagtctctcctctttcttctgggactagaatagccagctgtgtcagagagagctcctggcgccgcatacttaaccgccgcggctgctatagctac

SEQ ID NO: 10549 - RNA, 2643 nt, Homo sapiens
  source 1..2643: mol_type = other RNA
cggcccgggctgctgctgttcctctcactgctttcatagccagattccattcgctggattagtcgggggtgctgctctaaaaggtgagagcctggccgtgctgggccccagcgcttgtactgggggcttggtccaccaaatttaatgtcgtaagaaggtggcttgcttggttcatctggtataaattctttagctgaatcctcagaaaaggggctaagctgggtatagccacagtgcttccttttgtccttactaaagatactgtcaatattcagagattctcgtttgggtctccatgtgggacgatacttgctggaagaactggattttgactcactgctggtactctctatttcccagtcacgagagtgtaaaggcagggtcctaggaggttttttgtcaggctggtctcctcctctgcccctgcagtgagagcctacattggtctgagaagccagggatggtctgttatggatcatattgctgactgtctctttaaaatctctcagcctgttggtgctgctggatggtttggaggcatttctaggagcctgcttctctttcagtgtttctccttcactgtggtatcccgaggcctggggctcatcgcctttcctcctaacccgaccagagctcctcttgcgctctatcagtgaccctttcttggatgtgtgtttctgattacattcactatcagtcaggtgtcctgaatcttcactgtcgtagcatgtcctgctgtatgactggaactcagcttggggaggcaggtcctgggtggaaactggggtaccctggggatctgcataaagcagcagcaggggctgataatgccccttgatgcatttggtcaccacatccttccatttgggcccaatctccttgacatgagcatcatcaaaatacatccatttgcgaatctttgtttgaaaaaagaatgtagaataatgtttgccatagtaacagatcattccaactaagtacagttcagattgcttggcccggtcatccgtcactctgaaaaacagatcacccagcttaaggcaggttcccaggctgtggataacatcttctgctaagtctgagtggtctgagtcccataccagcccaatcgtgataatctgtggagcattcatcaacacacggcgaatcctgatcctctctccacagttgcttggacagttccgcagatcccccatggtgctggcattctgcagcagctcaccaaacatgcttggtgaaggtttctctcgtctttccagcatacaaatagcctgattgcaaagggaagtggtggagatataatgtaccatctggatgaaaggcagcggatcagaagtggcaccacagctagtacatacacactgctcaaacaatgtcattgcaaatttctgatgggaaatgcagtgttgggcagtacatatatcctctttggtttcatcagcaatgtggaagtgaattctcatcaggaggttttcaaagcactctgcagcatcatccataattcccagctggaaacgttgttcatcctggaaagtctttgccagagcactgcggagagtgtcagatggaagcactttttcactactacactgaaactggttaaagattcccttgagagcgcaaaagatgcaggaatctcccatgcacttgtgagttgtaagctgcctaaagctacgtcggaagatatccaagtgccacaaaacctgcagggcactgttgaggaagcagctgttttgccctggctcattgctgaggcctttgctgggggctatggaggttgagcttcgaggtgcaaacatcccttgtacactaccacgaccccctgaaaaataatttctcttccaagacattattgttcacatttagcctgaaaaaaaaatggagaaggatttgtgcctttttggcaggaatttctgtctgctaaagttctaaaaggaaagggaatccagaatttagtgaatttattttggaagattttgactttaccaccttccaaatatcatctgtgtagtcaagggactcaggtatcctcctagatcaagatgacagagccctccctcacttgttccaaacaatctccaaaatgtaacatggcacaggactaatgcaaacagagaaatccttaagtattgcttccttctatttttcttgaacagcctccataaagtcctggtgaagtggatgtaattctcaactccaacagcatccaggatcagggtaagatgtgttcttcaggcttgttgataatgcttcttatggactgaagatttttccaactggaaggagaggcagacagagaagcaagaatccaacatgatcctcctcaccctctattgccttgtctcatcatcctctgaagcaaaaactcaaattctgagcaactgcaaaaggttccacaaagccaagaagaagcctgtttgaatcatctgaggtttttgttgatgttcttgctgcttctttttaatgtgccccaaacttctattgtcccatccagatcttcagcaagtctctcctctttcttctgggactagaatagccagctgtgtcagagagcaagtgcctgaagtgtcaatcatttcctgcttctcccagctgcaggacttggaactaggaaaacattcagtcagcgtctagagcaggtct

SEQ ID NO: 10550 - RNA, 5116 nt, Homo sapiens
  source 1..5116: mol_type = other RNA
cggcccgggctgctgctgttcctctcactgctttcatagccagattccattcgctggattagtcgggggtgctgctctaaaaggtgagagcctggccgtgctgggccccagcgcttgtactgggggcttggtccaccaaatttaatgtcgtaagaaggtggcttgcttggttcatctggtataaattctttagctgaatcctcagaaaaggggctaagctgggtatagccacagtgcttccttttgtccttactaaagatactgtcaatattcagagattctcgtttgggtctccatgtgggacgatacttgctggaagaactggattttgactcactgctggtactctctatttcccagtcacgagagtgtaaaggcagggtcctaggaggttttttgtcaggctggtctcctcctctgcccctgcagtgagagcctacattggtctgagaagccagggatggtctgttatggatcatattgctgactgtctctttaaaatctctcagcctgttggtgctgctggatggtttggaggcatttctaggagcctgcttctctttcagtgtttctccttcactgtggtatcccgaggcctggggctcatcgcctttcctcctaacccgaccagagctcctcttgcgctctatcagtgaccctttcttggatgtgtgtttctgattacattcactatcagtcaggtgtcctgaatcttcactgtcgtagcatgtcctgctgtatgactggaactcagcttggggaggcaggtcctgggtggaaactggggtaccctggggatctgcataaagcagcagcaggggctgataatgccccttgatgcatttggtcaccacatccttccatttgggcccaatctccttgacatgagcatcatcaaaatacatccatttgcgaatctttgtttgaaaaaagaatgtagaataatgtttgccatagtaacagatcattccaactaagtacagttcagattgcttggcccggtcatccgtcactctgaaaaacagatcacccagcttaaggcaggttcccaggctgtggataacatcttctgctaagtctgagtggtctgagtcccataccagcccaatcgtgataatctgtggagcattcatcaacacacggcgaatcctgatcctctctccacagttgcttggacagttccgcagatcccccatggtgctggcattctgcagcagctcaccaaacatgcttggtgaaggtttctctcgtctttccagcatacaaatagcctgattgcaaagggaagtggtggagatataatgtaccatctggatgaaaggcagcggatcagaagtggcaccacagctagtacatacacactgctcaaacaatgtcattgcaaatttctgatgggaaatgcagtgttgggcagtacatatatcctctttggtttcatcagcaatgtggaagtgaattctcatcaggaggttttcaaagcactctgcagcatcatccataattcccagctggaaacgttgttcatcctggaaagtctttgccagagcactgcggagagtgtcagatggaagcactttttcactactacactgaaactggttaaagattcccttgagagcgcaaaagatgcaggaatctcccatgcacttgtgagttgtaagctgcctaaagctacgtcggaagatatccaagtgccacaaaacctgcagggcactgttgaggaagcagctgttttgccctggctcattgctgaggcctttgctgggggctatggaggttgagcttcgaggtgcaaacatcccttgtacactaccacgaccccctgaaaaataatttctcttccaagacattattgttcacatttagcctgaaaaaaaaatggagaaggatttgtgcctttttggcaggaatttctgtctgctaaagttctaaaaggaaagggaatccagaatttagtgaatttattttggaagattttgactttaccaccttccaaatatcatctgtgtagtcaagggactcaggtatcctcctagatcaagatgacagagccctccctcacttgttccaaacaatctccaaaatgtaacatggcacaggactaatgcaaacagagaaatccttaagtattgcttccttctatttttcttgaacagcctccataaagtcctggtgaagtggatgtaattctcaactccaacagcatccaggatcagggtaagatgtgttcttcaggcttgttgataatgcttcttatggactgaagatttttccaactggaaggagaggcagacagagaagcaagaatccaacatgatcctcctcaccctctattgccttgtctcatcatcctctgaagcaaaaactcaaattctgagcaactgcaaaaggttccacaaagccaagaagaagcctgtttgaatcatctgaggtttttgttgatgttcttgctgcttctttttaatgtgccccaaacttctattgtcccatccagatcttcagcaagtctctcctctttcttctgggactagaatagccagctgtgtcagagagctttaacagaaataaaaaaaatcaaaagcttgcgtcacttaatgactctactggctttggactgttctgccaagatcaacgttgcctcacttctcactataaacttgaaaccttggcaaacaatgccaaaaaaaaagaaaaaaagaaaaaaaaaaaaaagagagagacacccaaactaaagagaaggaaaaaaaggtatgaacagctttactttcaggggaaaattctctgaaattttcttgaagcagaagaaagttgatctggatagaaataaaaacaaaatacaaactttccagtatcaggctaacacaaaacaaatcaccaagtaagcacacacaaactaggaactgaaagttccttttggacattgtgaataaagcactttttaaaaggtgttttccatgaatatgcttatgaaaacgtgcttaaaggtgggaaggccatgttagcagtctaagatctgttctgagtaaagatgttccatccagagaaacactgatggcgagtaaaccacatgtccttaacatgcagtccaagagaactaaatcttctcctgccctgtttgtttgtttgtttcatttttgccagaggatcagagagataatttgggttacaaatcatttaatctccagattatatccaagggctcacaatcagaggcaatccattgaccaactttagttttcaactaattaaaatgccagtgaggcaacagagagtaataccaaagcaagtatgttccctggaaggaaatcaccacatctccagctttaagttttcctataaggctgccatgtccatctacataaggaaaaatttttaaatgttaagtgttaaatttgccaacatcaacaattcctcattctcccttccttctcaccatcatatgcaccatctaaaaacacaaaaatgctttaacatcttaatcattctctgggagatcacctagcattgtctacagcatgtccaatggaaaaactgaggtacaggaatattaaatggttgcataagactgttctttcccttctgtaaattcccagactatttataatctacatgtcccaattaaagtatttgattatacagcctactgtcacattattctctatttttattactctctgttttatatcgtatccgtcataatatgactacatgaaatgaaatagtagctacagtcaggtatgtgctaaacacgatacttatgtcctttatttaatattcacaacagtcctatcagatagctattaatagttccattttacagaaaagtaaagagaggcttaaagacattaacttgcccaattcaacactggtaagtggcagatctagaaatgtttgactattaaacaatgacttaattatatattttattattctattccaaaagctcctattacagtgccagtcataagaaggcagtcaataaatactgcctgatgattaacatgacactagaaaagaacccatatctcccacacagactataagaccctcacctttctacacacaccctcatacacaccccactcaaggccactaagcaacttccaacaagccatgcagcattccttcagctcaactgctgcaaaggaatgacaagtaccaagcctccactttgctcacagccaaaaggacttggcaggcaggtggggtttccaatatccacattaggagctaactgaaactcagcctgccctatgacacacactcctgagtacagggagcaaaaggagaaaaacgcagtagcagagaaaagattctcaggctctgaatggcagtattatgtagggtaaagcagtaagttctcagacctgttctagatgtgtcaccaactagaagtgagagcataaaggaccagacaagagaggcagtaacaagtggtccagagaaatactaacaccaaaaacatttcacttaaattgtagatatagcattaaacaatgtaatccttctccaataccatttactgaagatatgtgaggaggggaattatagttttatctgtatggctctcactacctagttttgttttttgggttttgttttgttttgttttgttttgtttctgaggcagaatctcactgtcacccaggctggagtgcagtcgcgcaatattggctcactgcagcctccgcctcttaggttcaagcaatcctcctgcctcagcctcccgagtagctgggattacaggcatgtgccactatgcctggctaatttttgtatttttagtagagacgggatttcaccaggggctggtctcaaacccctgacttcaggtgatccacctgccttgacttcccaaatgctgggattacaggcatgagccaccgcacccagccagtcaattgatttttgatgaaagtaccaaggccatttaattgagaaatgacagtcttttcaacaaatgatgttggaacaattgggacacccatatgcaaaaaactgaacattgagtcataccttacatcttatacaaaaataattcaatacatcacagtcctaaacaaaaaacctaaaactataaattctaggagaagacaggagaaaattttataacctt

SEQ ID NO: 10551 - RNA, 2496 nt, Homo sapiens
  source 1..2496: mol_type = other RNA
cggcccgggctgctgctgttcctctcactgctttcatagccagattccattcgctggattagtcgggggtgctgctctaaaaggtgagagcctggccgtgctgggccccagcgcttgtactgggggcttggtccaccaaatttaatgtcgtaagaaggtggcttgcttggttcatctggtataaattctttagctgaatcctcagaaaaggggctaagctgggtatagccacagtgcttccttttgtccttactaaagatactgtcaatattcagagattctcgtttgggtctccatgtgggacgatacttgctggaagaactggattttgactcactgctggtactctctatttcccagtcacgagagtgtaaaggcagggtcctaggaggttttttgtcaggctggtctcctcctctgcccctgcagtgagagcctacattggtctgagaagccagggatggtctgttatggatcatattgctgactgtctctttaaaatctctcagcctgttggtgctgctggatggtttggaggcatttctaggagcctgcttctctttcagtgtttctccttcactgtggtatcccgaggcctggggctcatcgcctttcctcctaacccgaccagagctcctcttgcgctctatcagtgaccctttcttggatgtgtgtttctgattacattcactatcagtcaggtgtcctgaatcttcactgtcgtagcatgtcctgctgtatgactggaactcagcttggggaggcaggtcctgggtggaaactggggtaccctggggatctgcataaagcagcagcaggggctgataatgccccttgatgcatttggtcaccacatccttccatttgggcccaatctccttgacatgagcatcatcaaaatacatccatttgcgaatctttgtttgaaaaaagaatgtagaataatgtttgccatagtaacagatcattccaactaagtacagttcagattgcttggcccggtcatccgtcactctgaaaaacagatcacccagcttaaggcaggttcccaggctgtggataacatcttctgctaagtctgagtggtctgagtcccataccagcccaatcgtgataatctgtggagcattcatcaacacacggcgaatcctgatcctctctccacagttgcttggacagttccgcagatcccccatggtgctggcattctgcagcagctcaccaaacatgcttggtgaaggtttctctcgtctttccagcatacaaatagcctgattgcaaagggaagtggtggagatataatgtaccatctggatgaaaggcagcggatcagaagtggcaccacagctagtacatacacactgctcaaacaatgtcattgcaaatttctgatgggaaatgcagtgttgggcagtacatatatcctctttggtttcatcagcaatgtggaagtgaattctcatcaggaggttttcaaagcactctgcagcatcatccataattcccagctggaaacgttgttcatcctggaaagtctttgccagagcactgcggagagtgtcagatggaagcactttttcactactacactgaaactggttaaagattcccttgagagcgcaaaagatgcaggaatctcccatgcacttgtgagttgtaagctgcctaaagctacgtcggaagatatccaagtgccacaaaacctgcagggcactgttgaggaagcagctgttttgccctggctcattgctgaggcctttgctgggggctatggaggttgagcttcgaggtgcaaacatcccttgtacactaccacgaccccctgaaaaataatttctcttccaagacattattgttcacatttagccttccaaatatcatctgtgtagtcaagggactcaggtatcctcctagatcaagatgacagagccctccctcacttgttccaaacaatctccaaaatgtaacatggcacaggactaatgcaaacagagaaatccttaagtattgcttccttctatttttcttgaacagcctccataaagtcctggtgaagtggatgtaattctcaactccaacagcatccaggatcagggtaagatgtgttcttcaggcttgttgataatgcttcttatggactgaagatttttccaactggaaggagaggcagacagagaagcaagaatccaacatgatcctcctcaccctctattgccttgtctcatcatcctctgaagcaaaaactcaaattctgagcaactgcaaaaggttccacaaagccaagaagaagcctgtttgaatcatctgaggtttttgttgatgttcttgctgcttctttttaatgtgccccaaacttctattgtcccatccagatcttcagcaagtctctcctctttcttctgggactagaatagccagctgtgtcagagagcagacagcacagtcaacctccagcaaaagacctctaatcacgagggtatctgtggggcaagtgat

SEQ ID NO: 10552 - RNA, 3986 nt, Homo sapiens
  source 1..3986: mol_type = other RNA
cggcccgggctgctgctgttcctctcactgctttcatagccagattccattcgctggattagtcgggggtgctgctctaaaaggtgagagcctggccgtgctgggccccagcgcttgtactgggggcttggtccaccaaatttaatgtcgtaagaaggtggcttgcttggttcatctggtataaattctttagctgaatcctcagaaaaggggctaagctgggtatagccacagtgcttccttttgtccttactaaagatactgtcaatattcagagattctcgtttgggtctccatgtgggacgatacttgctggaagaactggattttgactcactgctggtactctctatttcccagtcacgagagtgtaaaggcagggtcctaggaggttttttgtcaggctggtctcctcctctgcccctgcagtgagagcctacattggtctgagaagccagggatggtctgttatggatcatattgctgactgtctctttaaaatctctcagcctgttggtgctgctggatggtttggaggcatttctaggagcctgcttctctttcagtgtttctccttcactgtggtatcccgaggcctggggctcatcgcctttcctcctaacccgaccagagctcctcttgcgctctatcagtgaccctttcttggatgtgtgtttctgattacattcactatcagtcaggtgtcctgaatcttcactgtcgtagcatgtcctgctgtatgactggaactcagcttggggaggcaggtcctgggtggaaactggggtaccctggggatctgcataaagcagcagcaggggctgataatgccccttgatgcatttggtcaccacatccttccatttgggcccaatctccttgacatgagcatcatcaaaatacatccatttgcgaatctttgtttgaaaaaagaatgtagaataatgtttgccatagtaacagatcattccaactaagtacagttcagattgcttggcccggtcatccgtcactctgaaaaacagatcacccagcttaaggcaggttcccaggctgtggataacatcttctgctaagtctgagtggtctgagtcccataccagcccaatcgtgataatctgtggagcattcatcaacacacggcgaatcctgatcctctctccacagttgcttggacagttccgcagatcccccatggtgctggcattctgcagcagctcaccaaacatgcttggtgaaggtttctctcgtctttccagcatacaaatagcctgattgcaaagggaagtggtggagatataatgtaccatctggatgaaaggcagcggatcagaagtggcaccacagctagtacatacacactgctcaaacaatgtcattgcaaatttctgatgggaaatgcagtgttgggcagtacatatatcctctttggtttcatcagcaatgtggaagtgaattctcatcaggaggttttcaaagcactctgcagcatcatccataattcccagctggaaacgttgttcatcctggaaagtctttgccagagcactgcggagagtgtcagatggaagcactttttcactactacactgaaactggttaaagattcccttgagagcgcaaaagatgcaggaatctcccatgcacttgtgagttgtaagctgcctaaagctacgtcggaagatatccaagtgccacaaaacctgcagggcactgttgaggaagcagctgttttgccctggctcattgctgaggcctttgctgggggctatggaggttgagcttcgaggtgcaaacatcccttgtacactaccacgaccccctgaaaaataatttctcttccaagacattattgttcacatttagccttccaaatatcatctgtgtagtcaagggactcaggtatcctcctagatcaagatgacagagccctccctcacttgttccaaacaatctccaaaatgtaacatggcacaggactaatgcaaacagagaaatccttaagtattgcttccttctatttttcttgaacagcctccataaagtcctggtgaagtggatgtaattctcaactccaacagcatccaggatcagggtaagatgtgttcttcaggcttgttgataatgcttcttatggactgaagatttttccaactggaaggagaggcagacagagaagcaagaatccaacatgatcctcctcaccctctattgccttgtctcatcatcctctgaagcaaaaactcaaattctgagcaactgcaaaaggttccacaaagccaagaagaagcctgtttgaatcatctgaggtttttgttgatgttcttgctgcttctttttaatgtgccccaaacttctattgtcccatccagatcttcagcaagtctctcctctttcttctgggactagaatagccagctgtgtcagagagcagacagcacagtcaacctccagcaaaagacctctaatcacgagggtatctgtggggcaagtgatacaagaatggggagggatatgggaatagctagagctgtggggagggaaggctaggagggaggagacgactgtagctagcaacaatgagaaactgtgaatctaaaccacaaggacttcccgcagaacaggatatcagagagaaggcaattctttttaccaactaccaggaactcagcactgacaattcatgacaaagttaaaaaggtggagcttccaattaaaaacaaagtaaacttaagaaactaaccaaaagtaacttgaaaggacgttatcacaaacttcacctgaggcttaagaaaaacaattatgaagctgtttcctggggcattcctgatgacaaaggtcattaaacaataaggtttgcagggtggctgctgcttccaaagaagggccagtcccccacaaaaaaattcctttgcactgcagtcaaaaggagcacgagaagacaacatttttgtagttgtttacagaataatcaaaacaatgttattgttggaatccctaattcagaattccaagactgggcttaaattaaatcaaatcattttaataggcaaaactcctccaactgtcttaaacgagccacactattaaagaaaattattatttaaactgagccattggaatctactgagtcaattttaaaatgcttgggatctaagggttctcaaccccaaagtccacaacagggaaagatctccacccctctctcggggaagagacctagttacatcaccaagaacaaacagcaggcagagtcccacccccaaacatgtgatcagtcaaccgagaacttgcatttgcaggcagggcacaaaggccccagaggaccaacacacacccttctatgtattacctgaggttataaaacagttttattgaaagaagttgttttataagcatactgatgaaaaaaactcatcagcagaatccttgccaaatatgaaggtctgttgtgtttctataggttgagagaaaatatacgagttgactaaaaaaaagatgtaattaagatttattggtaaaatttaacaaacatgggcaatgtccaaaactaattaagctcttacattttaacaatacagtatattaaattgaagtagtcctttggccacaaggaaagtgccacaaaaaaaaaaaaaaaaaaaaagatactgttgcttttcttgttaaccattagcattctaactcaggtctcctagtggtgctaggtggaggaggaggtagtaatgccatttcaaagtgtgaaacacaaaatttctactgataagtgctgactgcaaataaagacatacaaacatcaagaccaagctcttcaatcaagtcattaaaatataggtatatattcattgtgaaactaatcaaataaaactagagtactgggacagagttacagagcttcaaccctgattacaactagacaacattacttttcatgtctcatccaggtaagggaagtgatccacagggaaatctcactctaatagatt

SEQ ID NO: 10553 - RNA, 5182 nt, Homo sapiens
  source 1..5182: mol_type = other RNA
cggcccgggctgctgctgttcctctcactgctttcatagccagattccattcgctggattagtcgggggtgctgctctaaaaggtgagagcctggccgtgctgggccccagcgcttgtactgggggcttggtccaccaaatttaatgtcgtaagaaggtggcttgcttggttcatctggtataaattctttagctgaatcctcagaaaaggggctaagctgggtatagccacagtgcttccttttgtccttactaaagatactgtcaatattcagagattctcgtttgggtctccatgtgggacgatacttgctggaagaactggattttgactcactgctggtactctctatttcccagtcacgagagtgtaaaggcagggtcctaggaggttttttgtcaggctggtctcctcctctgcccctgcagtgagagcctacattggtctgagaagccagggatggtctgttatggatcatattgctgactgtctctttaaaatctctcagcctgttggtgctgctggatggtttggaggcatttctaggagcctgcttctctttcagtgtttctccttcactgtggtatcccgaggcctggggctcatcgcctttcctcctaacccgaccagagctcctcttgcgctctatcagtgaccctttcttggatgtgtgtttctgattacattcactatcagtcaggtgtcctgaatcttcactgtcgtagcatgtcctgctgtatgactggaactcagcttggggaggcaggtcctgggtggaaactggggtaccctggggatctgcataaagcagcagcaggggctgataatgccccttgatgcatttggtcaccacatccttccatttgggcccaatctccttgacatgagcatcatcaaaatacatccatttgcgaatctttgtttgaaaaaagaatgtagaataatgtttgccatagtaacagatcattccaactaagtacagttcagattgcttggcccggtcatccgtcactctgaaaaacagatcacccagcttaaggcaggttcccaggctgtggataacatcttctgctaagtctgagtggtctgagtcccataccagcccaatcgtgataatctgtggagcattcatcaacacacggcgaatcctgatcctctctccacagttgcttggacagttccgcagatcccccatggtgctggcattctgcagcagctcaccaaacatgcttggtgaaggtttctctcgtctttccagcatacaaatagcctgattgctgtccccagatccaaagctcatagaatccccactcctcctcccactttgctggccagtactgagccaaagggaagtggtggagatataatgtaccatctggatgaaaggcagcggatcagaagtggcaccacagctagtacatacacactgctcaaacaatgtcattgcaaatttctgatgggaaatgcagtgttgggcagtacatatatcctctttggtttcatcagcaatgtggaagtgaattctcatcaggaggttttcaaagcactctgcagcatcatccataattcccagctggaaacgttgttcatcctggaaagtctttgccagagcactgcggagagtgtcagatggaagcactttttcactactacactgaaactggttaaagattcccttgagagcgcaaaagatgcaggaatctcccatgcacttgtgagttgtaagctgcctaaagctacgtcggaagatatccaagtgccacaaaacctgcagggcactgttgaggaagcagctgttttgccctggctcattgctgaggcctttgctgggggctatggaggttgagcttcgaggtgcaaacatcccttgtacactaccacgaccccctgaaaaataatttctcttccaagacattattgttcacatttagcctgaaaaaaaaatggagaaggatttgtgcctttttggcaggaatttctgtctgctaaagttctaaaaggaaagggaatccagaatttagtgaatttattttggaagattttgactttaccaccttccaaatatcatctgtgtagtcaagggactcaggtatcctcctagatcaagatgacagagccctccctcacttgttccaaacaatctccaaaatgtaacatggcacaggactaatgcaaacagagaaatccttaagtattgcttccttctatttttcttgaacagcctccataaagtcctggtgaagtggatgtaattctcaactccaacagcatccaggatcagggtaagatgtgttcttcaggcttgttgataatgcttcttatggactgaagatttttccaactggaaggagaggcagacagagaagcaagaatccaacatgatcctcctcaccctctattgccttgtctcatcatcctctgaagcaaaaactcaaattctgagcaactgcaaaaggttccacaaagccaagaagaagcctgtttgaatcatctgaggtttttgttgatgttcttgctgcttctttttaatgtgccccaaacttctattgtcccatccagatcttcagcaagtctctcctctttcttctgggactagaatagccagctgtgtcagagagctttaacagaaataaaaaaaatcaaaagcttgcgtcacttaatgactctactggctttggactgttctgccaagatcaacgttgcctcacttctcactataaacttgaaaccttggcaaacaatgccaaaaaaaaagaaaaaaagaaaaaaaaaaaaaagagagagacacccaaactaaagagaaggaaaaaaaggtatgaacagctttactttcaggggaaaattctctgaaattttcttgaagcagaagaaagttgatctggatagaaataaaaacaaaatacaaactttccagtatcaggctaacacaaaacaaatcaccaagtaagcacacacaaactaggaactgaaagttccttttggacattgtgaataaagcactttttaaaaggtgttttccatgaatatgcttatgaaaacgtgcttaaaggtgggaaggccatgttagcagtctaagatctgttctgagtaaagatgttccatccagagaaacactgatggcgagtaaaccacatgtccttaacatgcagtccaagagaactaaatcttctcctgccctgtttgtttgtttgtttcatttttgccagaggatcagagagataatttgggttacaaatcatttaatctccagattatatccaagggctcacaatcagaggcaatccattgaccaactttagttttcaactaattaaaatgccagtgaggcaacagagagtaataccaaagcaagtatgttccctggaaggaaatcaccacatctccagctttaagttttcctataaggctgccatgtccatctacataaggaaaaatttttaaatgttaagtgttaaatttgccaacatcaacaattcctcattctcccttccttctcaccatcatatgcaccatctaaaaacacaaaaatgctttaacatcttaatcattctctgggagatcacctagcattgtctacagcatgtccaatggaaaaactgaggtacaggaatattaaatggttgcataagactgttctttcccttctgtaaattcccagactatttataatctacatgtcccaattaaagtatttgattatacagcctactgtcacattattctctatttttattactctctgttttatatcgtatccgtcataatatgactacatgaaatgaaatagtagctacagtcaggtatgtgctaaacacgatacttatgtcctttatttaatattcacaacagtcctatcagatagctattaatagttccattttacagaaaagtaaagagaggcttaaagacattaacttgcccaattcaacactggtaagtggcagatctagaaatgtttgactattaaacaatgacttaattatatattttattattctattccaaaagctcctattacagtgccagtcataagaaggcagtcaataaatactgcctgatgattaacatgacactagaaaagaacccatatctcccacacagactataagaccctcacctttctacacacaccctcatacacaccccactcaaggccactaagcaacttccaacaagccatgcagcattccttcagctcaactgctgcaaaggaatgacaagtaccaagcctccactttgctcacagccaaaaggacttggcaggcaggtggggtttccaatatccacattaggagctaactgaaactcagcctgccctatgacacacactcctgagtacagggagcaaaaggagaaaaacgcagtagcagagaaaagattctcaggctctgaatggcagtattatgtagggtaaagcagtaagttctcagacctgttctagatgtgtcaccaactagaagtgagagcataaaggaccagacaagagaggcagtaacaagtggtccagagaaatactaacaccaaaaacatttcacttaaattgtagatatagcattaaacaatgtaatccttctccaataccatttactgaagatatgtgaggaggggaattatagttttatctgtatggctctcactacctagttttgttttttgggttttgttttgttttgttttgttttgtttctgaggcagaatctcactgtcacccaggctggagtgcagtcgcgcaatattggctcactgcagcctccgcctcttaggttcaagcaatcctcctgcctcagcctcccgagtagctgggattacaggcatgtgccactatgcctggctaatttttgtatttttagtagagacgggatttcaccaggggctggtctcaaacccctgacttcaggtgatccacctgccttgacttcccaaatgctgggattacaggcatgagccaccgcacccagccagtcaattgatttttgatgaaagtaccaaggccatttaattgagaaatgacagtcttttcaacaaatgatgttggaacaattgggacacccatatgcaaaaaactgaacattgagtcataccttacatcttatacaaaaataattcaatacatcacagtcctaaacaaaaaacctaaaactataaattctaggagaagacaggagaaaattttataacctt

SEQ ID NO: 10554 - RNA, 2083 nt, Homo sapiens
  source 1..2083: mol_type = other RNA
cggcccgggctgctgctgttcctctcactgctttcatagccagattccattcgctggattagtcgggggtgctgctctaaaaggtgagagcctggccgtgctgggccccagcgcttgtactgggggcttggtccaccaaatttaatgtcgtaagaaggtggcttgcttggttcatctggtataaattctttagctgaatcctcagaaaaggggctaagctgggtatagccacagtgcttccttttgtccttactaaagatactgtcaatattcagagattctcgtttgggtctccatgtgggacgatacttgctggaagaactggattttgactcactgctggtactctctatttcccagtcacgagagtgtaaaggcagggtcctaggaggttttttgtcaggctggtctcctcctctgcccctgcagtgagagcctacattggtctgagaagccagggatggtctgttatggatcatattgctgactgtctctttaaaatctctcagcctgttggtgctgctggatggtttggaggcatttctaggagcctgcttctctttcagtgtttctccttcactgtggtatcccgaggcctggggctcatcgcctttcctcctaacccgaccagagctcctcttgcgctctatcagtgaccctttcttggatgtgtgtttctgattacattcactatcagtcaggtgtcctgtgtcccgactgctctgagacatggaatcattttccacattatagatgactgtcccctgagaatcagaagagaagtgactgaccacagactcatggtgggaatgtttgtagggatagctctccgttgaggaatctgttcgagtgtcacttgagatggagggctccctccctgaatcttcactgtcgtagcatgtcctgctgtatgactggaactcagcttggggaggcaggtcctgggtggaaactggggtaccctggggatctgcataaagcagcagcaggggctgataatgccccttgatgcatttggtcaccacatccttccatttgggcccaatctccttgacatgagcatcatcaaaatacatccatttgcgaatctttgtttgaaaaaagaatgtagaataatgtttgccatagtaacagatcattccaactaagtacagttcagattgcttggcccggtcatccgtcactctgaaaaacagatcacccagcttaaggcaggttcccaggctgtggataacatcttctgctaagtctgagtggtctgagtcccataccagcccaatcgtgataatctgtggagcattcatcaacacacggcgaatcctgatcctctctccacagttgcttggacagttccgcagatcccccatggtgctggcattctgcagcagctcaccaaacatgcttggtgaaggtttctctcgtctttccagcatacaaatagcctgattgcaaagggaagtggtggagatataatgtaccatctggatgaaaggcagcggatcagaagtggcaccacagctagtacatacacactgctcaaacaatgtcattgcaaatttctgatgggaaatgcagtgttgggcagtacatatatcctctttggtttcatcagcaatgtggaagtgaattctcatcaggaggttttcaaagcactctgcagcatcatccataattcccagctggaaacgttgttcatcctggaaagtctttgccagagcactgcggagagtgtcagatggaagcactttttcactactacactgaaactggttaaagattcccttgagagcgcaaaagatgcaggaatctcccatgcacttgtgagttgtaagctgcctaaagctacgtcggaagatatccaagtgccacaaaacctgcagggcactgttgaggaagcagctgttttgccctggctcattgctgaggcctttgctgggggctatggaggttgagcttcgaggtgcaaacatcccttgtacactaccacgaccccctgaaaaataatttctcttccaagacattattgttcacatttagcagctcctggcgccgcatacttaaccgccgcggctgctatagctac

SEQ ID NO: 10555 - RNA, 3008 nt, Homo sapiens
  source 1..3008: mol_type = other RNA
cggcccgggctgctgctgttcctctcactgctttcatagccagattccattcgctggattagtcgggggtgctgctctaaaaggtgagagcctggccgtgctgggccccagcgcttgtactgggggcttggtccaccaaatttaatgtcgtaagaaggtggcttgcttggttcatctggtataaattctttagctgaatcctcagaaaaggggctaagctgggtatagccacagtgcttccttttgtccttactaaagatactgtcaatattcagagattctcgtttgggtctccatgtgggacgatacttgctggaagaactggattttgactcactgctggtactctctatttcccagtcacgagagtgtaaaggcagggtcctaggaggttttttgtcaggctggtctcctcctctgcccctgcagtgagagcctacattggtctgagaagccagggatggtctgttatggatcatattgctgactgtctctttaaaatctctcagcctgttggtgctgctggatggtttggaggcatttctaggagcctgcttctctttcagtgtttctccttcactgtggtatcccgaggcctggggctcatcgcctttcctcctaacccgaccagagctcctcttgcgctctatcagtgaccctttcttggatgtgtgtttctgattacattcactatcagtcaggtgtcctgtgtcccgactgctctgagacatggaatcattttccacattatagatgactgtcccctgagaatcagaagagaagtgactgaccacagactcatggtgggaatgtttgtagggatagctctccgttgaggaatctgttcgagtgtcacttgagatggagggctccctccctgaatcttcactgtcgtagcatgtcctgctgtatgactggaactcagcttggggaggcaggtcctgggtggaaactggggtaccctggggatctgcataaagcagcagcaggggctgataatgccccttgatgcatttggtcaccacatccttccatttgggcccaatctccttgacatgagcatcatcaaaatacatccatttgcgaatctttgtttgaaaaaagaatgtagaataatgtttgccatagtaacagatcattccaactaagtacagttcagattgcttggcccggtcatccgtcactctgaaaaacagatcacccagcttaaggcaggttcccaggctgtggataacatcttctgctaagtctgagtggtctgagtcccataccagcccaatcgtgataatctgtggagcattcatcaacacacggcgaatcctgatcctctctccacagttgcttggacagttccgcagatcccccatggtgctggcattctgcagcagctcaccaaacatgcttggtgaaggtttctctcgtctttccagcatacaaatagcctgattgcaaagggaagtggtggagatataatgtaccatctggatgaaaggcagcggatcagaagtggcaccacagctagtacatacacactgctcaaacaatgtcattgcaaatttctgatgggaaatgcagtgttgggcagtacatatatcctctttggtttcatcagcaatgtggaagtgaattctcatcaggaggttttcaaagcactctgcagcatcatccataattcccagctggaaacgttgttcatcctggaaagtctttgccagagcactgcggagagtgtcagatggaagcactttttcactactacactgaaactggttaaagattcccttgagagcgcaaaagatgcaggaatctcccatgcacttgtgagttgtaagctgcctaaagctacgtcggaagatatccaagtgccacaaaacctgcagggcactgttgaggaagcagctgttttgccctggctcattgctgaggcctttgctgggggctatggaggttgagcttcgaggtgcaaacatcccttgtacactaccacgaccccctgaaaaataatttctcttccaagacattattgttcacatttagcagctcctggcgccgcatacttaaccgccgcggctgctatagctacagggagccaaggcaaccagctctcgcgacactttccttggccatggcgagagcacacgagaagagactctcgcaagaaagtaaatgagtcaggctggaaacagcgaagtatatctcgcgatagcactgtttaaaatggcggcttcaaggcgtttcacgggtgtcccggacaggcgtggaggtggggcgcaggcgaggatgaagcttgagttggccaggagtcggaaaacgattgcaggcgggaccgcgtccgtcggggctgaggaaacttagcgtggcagaccctaaactgggataactttagggatatggccttcttttcccagttgcctcaaacttagagcagcgtcgtctttagccgaagattcattttcccagcattttccttctccaggcggagtagttggagacagagggcaagccagaaactgaccttcccatctcctcattcccttccatcaagaacttttcatcgttctttccccaccctggtttgtaaatggtatttggcttcataaaaacgtttgtccacaggtgccctgctccatcagttcgctccagcaatataggaagttaccaaaaaaaaaatttttttttattgaccttggatgcagaaaggaaccgcgttggtgtgtgatttgaattttggacttcttgtttcctgccttgtggccacgtcccccttacttggtgactctcagcacttagttgtggggctttttctctctgctctcagacaactataaaagcagactaattgaacagcatctagaacagaaggtggatgtaaagaacattggtcggccgggcgctgtggctcacgcctgtaatcccagcacttgagaggccgaggcgggcagatcacgaggtcaggagatcgagaccatcctgaccaacattgtgaaaccccgtctctactaaaaata

SEQ ID NO: 10556 - RNA, 2103 nt, Homo sapiens
  source 1..2103: mol_type = other RNA
cggcccgggctgctgctgttcctctcactgctttcatagccagattccattcgctggattagtcgggggtgctgctctaaaaggtgagagcctggccgtgctgggccccagcgcttgtactgggggcttggtccaccaaatttaatgtcgtaagaaggtggcttgcttggttcatctggtataaattctttagctgaatcctcagaaaaggggctaagctgggtatagccacagtgcttccttttgtccttactaaagatactgtcaatattcagagattctcgtttgggtctccatgtgggacgatacttgctggaagaactggattttgactcactgctggtactctctatttcccagtcacgagagtgtaaaggcagggtcctaggaggttttttgtcaggctggtctcctcctctgcccctgcagtgagagcctacattggtctgagaagccagggatggtctgttatggatcatattgctgactgtctctttaaaatctctcagcctgttggtgctgctggatggtttggaggcatttctaggagcctgcttctctttcagtgtttctccttcactgtggtatcccgaggcctggggctcatcgcctttcctcctaacccgaccagagctcctcttgcgctctatcagtgaccctttcttggatgtgtgtttctgattacattcactatcagtcaggtgtcctgtgtcccgactgctctgagacatggaatcattttccacattatagatgactgtcccctgagaatcagaagagaagtgactgaccacagactcatggtgggaatgtttgtagggatagctctccgttgaggaatctgttcgagtgtcacttgagatggagggctccctccctgaatcttcactgtcgtagcatgtcctgctgtatgactggaactcagcttggggaggcaggtcctgggtggaaactggggtaccctggggatctgcataaagcagcagcaggggctgataatgccccttgatgcatttggtcaccacatccttccatttgggcccaatctccttgacatgagcatcatcaaaatacatccatttgcgaatctttgtttgaaaaaagaatgtagaataatgtttgccatagtaacagatcattccaactaagtacagttcagattgcttggcccggtcatccgtcactctgaaaaacagatcacccagcttaaggcaggttcccaggctgtggataacatcttctgctaagtctgagtggtctgagtcccataccagcccaatcgtgataatctgtggagcattcatcaacacacggcgaatcctgatcctctctccacagttgcttggacagttccgcagatcccccatggtgctggcattctgcagcagctcaccaaacatgcttggtgaaggtttctctcgtctttccagcatacaaatagcctgattgcaaagggaagtggtggagatataatgtaccatctggatgaaaggcagcggatcagaagtggcaccacagctagtacatacacactgctcaaacaatgtcattgcaaatttctgatgggaaatgcagtgttgggcagtacatatatcctctttggtttcatcagcaatgtggaagtgaattctcatcaggaggttttcaaagcactctgcagcatcatccataattcccagctggaaacgttgttcatcctggaaagtctttgccagagcactgcggagagtgtcagatggaagcactttttcactactacactgaaactggttaaagattcccttgagagcgcaaaagatgcaggaatctcccatgcacttgtgagttgtaagctgcctaaagctacgtcggaagatatccaagtgccacaaaacctgcagggcactgttgaggaagcagctgttttgccctggctcattgctgaggcctttgctgggggctatggaggttgagcttcgaggtgcaaacatcccttgtacactaccacgaccccctgaaaaataatttctcttccaagacattattgttcacatttagccagacagcacagtcaacctccagcaaaagacctctaatcacgagggtatctgtggggcaagtgat

SEQ ID NO: 10557 - RNA, 2329 nt, Homo sapiens
  source 1..2329: mol_type = other RNA
cggcccgggctgctgctgttcctctcactgctttcatagccagattccattcgctggattagtcgggggtgctgctctaaaaggtgagagcctggccgtgctgggccccagcgcttgtactgggggcttggtccaccaaatttaatgtcgtaagaaggtggcttgcttggttcatctggtataaattctttagctgaatcctcagaaaaggggctaagctgggtatagccacagtgcttccttttgtccttactaaagatactgtcaatattcagagattctcgtttgggtctccatgtgggacgatacttgctggaagaactggattttgactcactgctggtactctctatttcccagtcacgagagtgtaaaggcagggtcctaggaggttttttgtcaggctggtctcctcctctgcccctgcagtgagagcctacattggtctgagaagccagggatggtctgttatggatcatattgctgactgtctctttaaaatctctcagcctgttggtgctgctggatggtttggaggcatttctaggagcctgcttctctttcagtgtttctccttcactgtggtatcccgaggcctggggctcatcgcctttcctcctaacccgaccagagctcctcttgcgctctatcagtgaccctttcttggatgtgtgtttctgattacattcactatcagtcaggtgtcctgtgtcccgactgctctgagacatggaatcattttccacattatagatgactgtcccctgagaatcagaagagaagtgactgaccacagactcatggtgggaatgtttgtagggatagctctccgttgaggaatctgttcgagtgtcacttgagatggagggctccctccctgaatcttcactgtcgtagcatgtcctgctgtatgactggaactcagcttggggaggcaggtcctgggtggaaactggggtaccctggggatctgcataaagcagcagcaggggctgataatgccccttgatgcatttggtcaccacatccttccatttgggcccaatctccttgacatgagcatcatcaaaatacatccatttgcgaatctttgtttgaaaaaagaatgtagaataatgtttgccatagtaacagatcattccaactaagtacagttcagattgcttggcccggtcatccgtcactctgaaaaacagatcacccagcttaaggcaggttcccaggctgtggataacatcttctgctaagtctgagtggtctgagtcccataccagcccaatcgtgataatctgtggagcattcatcaacacacggcgaatcctgatcctctctccacagttgcttggacagttccgcagatcccccatggtgctggcattctgcagcagctcaccaaacatgcttggtgaaggtttctctcgtctttccagcatacaaatagcctgattgcaaagggaagtggtggagatataatgtaccatctggatgaaaggcagcggatcagaagtggcaccacagctagtacatacacactgctcaaacaatgtcattgcaaatttctgatgggaaatgcagtgttgggcagtacatatatcctctttggtttcatcagcaatgtggaagtgaattctcatcaggaggttttcaaagcactctgcagcatcatccataattcccagctggaaacgttgttcatcctggaaagtctttgccagagcactgcggagagtgtcagatggaagcactttttcactactacactgaaactggttaaagattcccttgagagcgcaaaagatgcaggaatctcccatgcacttgtgagttgtaagctgcctaaagctacgtcggaagatatccaagtgccacaaaacctgcagggcactgttgaggaagcagctgttttgccctggctcattgctgaggcctttgctgggggctatggaggttgagcttcgaggtgcaaacatcccttgtacactaccacgaccccctgaaaaataatttctcttccaagacattattgttcacatttagccctctattgccttgtctcatcatcctctgaagcaaaaactcaaattctgagcaactgcaaaaggttccacaaagccaagaagaagcctgtttgaatcatctgaggtttttgttgatgttcttgctgcttctttttaatgtgccccaaacttctattgtcccatccagatcttcagcaagtctctcctctttcttctgggactagaatagccagctgtgtcagagagcagacagcacagtcaacctccagcaaaagacctctaatcacgagggtatctgtggggcaagtgat

SEQ ID NO: 10558 - RNA, 4321 nt, Homo sapiens
  source 1..4321: mol_type = other RNA
cggcccgggctgctgctgttcctctcactgctttcatagccagattccattcgctggattagtcgggggtgctgctctaaaaggtgagagcctggccgtgctgggccccagcgcttgtactgggggcttggtccaccaaatttaatgtcgtaagaaggtggcttgcttggttcatctggtataaattctttagctgaatcctcagaaaaggggctaagctgggtatagccacagtgcttccttttgtccttactaaagatactgtcaatattcagagattctcgtttgggtctccatgtgggacgatacttgctggaagaactggattttgactcactgctggtactctctatttcccagtcacgagagtgtaaaggcagggtcctaggaggttttttgtcaggctggtctcctcctctgcccctgcagtgagagcctacattggtctgagaagccagggatggtctgttatggatcatattgctgactgtctctttaaaatctctcagcctgttggtgctgctggatggtttggaggcatttctaggagcctgcttctctttcagtgtttctccttcactgtggtatcccgaggcctggggctcatcgcctttcctcctaacccgaccagagctcctcttgcgctctatcagtgaccctttcttggatgtgtgtttctgattacattcactatcagtcaggtgtcctgtgtcccgactgctctgagacatggaatcattttccacattatagatgactgtcccctgagaatcagaagagaagtgactgaccacagactcatggtgggaatgtttgtagggatagctctccgttgaggaatctgttcgagtgtcacttgagatggagggctccctccctgaatcttcactgtcgtagcatgtcctgctgtatgactggaactcagcttggggaggcaggtcctgggtggaaactggggtaccctggggatctgcataaagcagcagcaggggctgataatgccccttgatgcatttggtcaccacatccttccatttgggcccaatctccttgacatgagcatcatcaaaatacatccatttgcgaatctttgtttgaaaaaagaatgtagaataatgtttgccatagtaacagatcattccaactaagtacagttcagattgcttggcccggtcatccgtcactctgaaaaacagatcacccagcttaaggcaggttcccaggctgtggataacatcttctgctaagtctgagtggtctgagtcccataccagcccaatcgtgataatctgtggagcattcatcaacacacggcgaatcctgatcctctctccacagttgcttggacagttccgcagatcccccatggtgctggcattctgcagcagctcaccaaacatgcttggtgaaggtttctctcgtctttccagcatacaaatagcctgattgcaaagggaagtggtggagatataatgtaccatctggatgaaaggcagcggatcagaagtggcaccacagctagtacatacacactgctcaaacaatgtcattgcaaatttctgatgggaaatgcagtgttgggcagtacatatatcctctttggtttcatcagcaatgtggaagtgaattctcatcaggaggttttcaaagcactctgcagcatcatccataattcccagctggaaacgttgttcatcctggaaagtctttgccagagcactgcggagagtgtcagatggaagcactttttcactactacactgaaactggttaaagattcccttgagagcgcaaaagatgcaggaatctcccatgcacttgtgagttgtaagctgcctaaagctacgtcggaagatatccaagtgccacaaaacctgcagggcactgttgaggaagcagctgttttgccctggctcattgctgaggcctttgctgggggctatggaggttgagcttcgaggtgcaaacatcccttgtacactaccacgaccccctgaaaaataatttctcttccaagacattattgttcacatttagccctctattgccttgtctcatcatcctctgaagcaaaaactcaaattctgagcaactgcaaaaggttccacaaagccaagaagaagcctgtttgaatcatctgaggtttttgttgatgttcttgctgcttctttttaatgtgccccaaacttctattgtcccatccagatcttcagcaagtctctcctctttcttctgggactagaatagccagctgtgtcagagagctttaacagaaataaaaaaaatcaaaagcttgcgtcacttaatgactctactggctttggactgttctgccaagatcaacgttgcctcacttctcactataaacttgaaaccttggcaaacaatgccaaaaaaaaagaaaaaaagaaaaaaaaaaaaaagagagagacacccaaactaaagagaaggaaaaaaaggtatgaacagctttactttcaggggaaaattctctgaaattttcttgaagcagaagaaagttgatctggatagaaataaaaacaaaatacaaactttccagtatcaggctaacacaaaacaaatcaccaagtaagcacacacaaactaggaactgaaagttccttttggacattgtgaataaagcactttttaaaaggtgttttccatgaatatgcttatgaaaacgtgcttaaaggtgggaaggccatgttagcagtctaagatctgttctgagtaaagatgttccatccagagaaacactgatggcgagtaaaccacatgtccttaacatgcagtccaagagaactaaatcttctcctgccctgtttgtttgtttgtttcatttttgccagaggatcagagagataatttgggttacaaatcatttaatctccagattatatccaagggctcacaatcagaggcaatccattgaccaactttagttttcaactaattaaaatgccagtgaggcaacagagagtaataccaaagcaagtatgttccctggaaggaaatcaccacatctccagctttaagttttcctataaggctgccatgtccatctacataaggaaaaatttttaaatgttaagtgttaaatttgccaacatcaacaattcctcattctcccttccttctcaccatcatatgcaccatctaaaaacacaaaaatgctttaacatcttaatcattctctgggagatcacctagcattgtctacagcatgtccaatggaaaaactgaggtacaggaatattaaatggttgcataagactgttctttcccttctgtaaattcccagactatttataatctacatgtcccaattaaagtatttgattatacagcctactgtcacattattctctatttttattactctctgttttatatcgtatccgtcataatatgactacatgaaatgaaatagtagctacagtcaggtatgtgctaaacacgatacttatgtcctttatttaatattcacaacagtcctatcagatagctattaatagttccattttacagaaaagtaaagagaggcttaaagacattaacttgcccaattcaacactggtaagtggcagatctagaaatgtttgactattaaacaatgacttaattatatattttattattctattccaaaagctcctattacagtgccagtcataagaaggcagtcaataaatactgcctgatgattaacatgacactagaaaagaacccatatctcccacacagactataagaccctcacctttctacacacaccctcatacacaccccactcaaggccactaagcaacttccaacaagccatgcagcattccttcagctcaactgctgcaaaggaatgacaagtaccaagcctccactttgctcacagccaaaaggacttggcaggcaggtggggtttccaatatccacattaggagctaactgaaactcagcctgccctatgacacacactcctgagtacagggagcaaaaggagaaaaacgcagtagcagagaaaagattctcaggctctgaatggcagtattatgtagggtaaagcagtaagttctcagacctgttctagatgtgtcaccaactagaagtgagagcataaaggaccagacaagagaggcagtaacaagtggtccagagaaatactaacaccaaaaacatttcacttaaattgtagatatagcattaaacaatgtaatccttctccaataccatttactgaagatatgtgaggaggggaattatagttttatctgtatggctctcactacctagttttgttttttgggttttgttttgttttgtt

SEQ ID NO: 10559 - RNA, 3694 nt, Homo sapiens
  source 1..3694: mol_type = other RNA
cggcccgggctgctgctgttcctctcactgctttcatagccagattccattcgctggattagtcgggggtgctgctctaaaaggtgagagcctggccgtgctgggccccagcgcttgtactgggggcttggtccaccaaatttaatgtcgtaagaaggtggcttgcttggttcatctggtataaattctttagctgaatcctcagaaaaggggctaagctgggtatagccacagtgcttccttttgtccttactaaagatactgtcaatattcagagattctcgtttgggtctccatgtgggacgatacttgctggaagaactggattttgactcactgctggtactctctatttcccagtcacgagagtgtaaaggcagggtcctaggaggttttttgtcaggctggtctcctcctctgcccctgcagtgagagcctacattggtctgagaagccagggatggtctgttatggatcatattgctgactgtctctttaaaatctctcagcctgttggtgctgctggatggtttggaggcatttctaggagcctgcttctctttcagtgtttctccttcactgtggtatcccgaggcctggggctcatcgcctttcctcctaacccgaccagagctcctcttgcgctctatcagtgaccctttcttggatgtgtgtttctgattacattcactatcagtcaggtgtcctgtgtcccgactgctctgagacatggaatcattttccacattatagatgactgtcccctgagaatcagaagagaagtgactgaccacagactcatggtgggaatgtttgtagggatagctctccgttgaggaatctgttcgagtgtcacttgagatggagggctccctccctgaatcttcactgtcgtagcatgtcctgctgtatgactggaactcagcttggggaggcaggtcctgggtggaaactggggtaccctggggatctgcataaagcagcagcaggggctgataatgccccttgatgcatttggtcaccacatccttccatttgggcccaatctccttgacatgagcatcatcaaaatacatccatttgcgaatctttgtttgaaaaaagaatgtagaataatgtttgccatagtaacagatcattccaactaagtacagttcagattgcttggcccggtcatccgtcactctgaaaaacagatcacccagcttaaggcaggttcccaggctgtggataacatcttctgctaagtctgagtggtctgagtcccataccagcccaatcgtgataatctgtggagcattcatcaacacacggcgaatcctgatcctctctccacagttgcttggacagttccgcagatcccccatggtgctggcattctgcagcagctcaccaaacatgcttggtgaaggtttctctcgtctttccagcatacaaatagcctgattgcaaagggaagtggtggagatataatgtaccatctggatgaaaggcagcggatcagaagtggcaccacagctagtacatacacactgctcaaacaatgtcattgcaaatttctgatgggaaatgcagtgttgggcagtacatatatcctctttggtttcatcagcaatgtggaagtgaattctcatcaggaggttttcaaagcactctgcagcatcatccataattcccagctggaaacgttgttcatcctggaaagtctttgccagagcactgcggagagtgtcagatggaagcactttttcactactacactgaaactggttaaagattcccttgagagcgcaaaagatgcaggaatctcccatgcacttgtgagttgtaagctgcctaaagctacgtcggaagatatccaagtgccacaaaacctgcagggcactgttgaggaagcagctgttttgccctggctcattgctgaggcctttgctgggggctatggaggttgagcttcgaggtgcaaacatcccttgtacactaccacgaccccctgaaaaataatttctcttccaagacattattgttcacatttagcctgaaaaaaaaatggagaaggatttgtgcctttttggcaggaatttctgtctgctaaagttctaaaaggaaagggaatccagaatttagtgaatttattttggaagattttgactttaccaccttccaaatatcatctgtgtagtcaagggactcaggtatcctcctagatcaagatgacagagccctccctcacttgttccaaacaatctccaaaatgtaacatggcacaggactaatgcaaacagagaaatccttaagtattgcttccttctatttttcttgaacagcctccataaagtcctggtgaagtggatgtaattctcaactccaacagcatccaggatcagggtaagatgtgttcttcaggcttgttgataatgcttcttatggactgaagatttttccaactggaaggagaggcagacagagaagcaagaatccaacatgatcctcctcaccctctattgccttgtctcatcatcctctgaagcaaaaactcaaattctgagcaactgcaaaaggttccacaaagccaagaagaagcctgtttgaatcatctgaggtttttgttgatgttcttgctgcttctttttaatgtgccccaaacttctattgtcccatccagatcttcagcaagtctctcctctttcttctgggactagaatagccagctgtgtcagagagagctcctggcgccgcatacttaaccgccgcggctgctatagctacagggagccaaggcaaccagctctcgcgacactttccttggccatggcgagagcacacgagaagagactctcgcaagaaagtaaatgagtcaggctggaaacagcgaagtatatctcgcgatagcactgtttaaaatggcggcttcaaggcgtttcacgggtgtcccggacaggcgtggaggtggggcgcaggcgaggatgaagcttgagttggccaggagtcggaaaacgattgcaggcgggaccgcgtccgtcggggctgaggaaacttagcgtggcagaccctaaactgggataactttagggatatggccttcttttcccagttgcctcaaacttagagcagcgtcgtctttagccgaagattcattttcccagcattttccttctccaggcggagtagttggagacagagggcaagccagaaactgaccttcccatctcctcattcccttccatcaagaacttttcatcgttctttccccaccctggtttgtaaatggtatttggcttcataaaaacgtttgtccacaggtgccctgctccatcagttcgctccagcaatataggaagttaccaaaaaaaaaatttttttttattgaccttggatgcagaaaggaaccgcgttggtgtgtgatttgaattttggacttcttgtttcctgccttgtggccacgtcccccttacttggtgactctcagcacttagttgtggggctttttctctctgctctcagacaactataaaagcagactaattgaacagcatctagaacagaaggtggatgtaaagaacattggtcggccgggcgctgtggctcacgcctgtaatcccagcacttgagaggccgaggcgggcagatcacgaggtcaggagatcgagaccatcctgaccaacattgtgaaaccccgtctctactaaaaata

SEQ ID NO: 10560 - RNA, 4279 nt, Homo sapiens
  source 1..4279: mol_type = other RNA
cggcccgggctgctgctgttcctctcactgctttcatagccagattccattcgctggattagtcgggggtgctgctctaaaaggtgagagcctggccgtgctgggccccagcgcttgtactgggggcttggtccaccaaatttaatgtcgtaagaaggtggcttgcttggttcatctggtataaattctttagctgaatcctcagaaaaggggctaagctgggtatagccacagtgcttccttttgtccttactaaagatactgtcaatattcagagattctcgtttgggtctccatgtgggacgatacttgctggaagaactggattttgactcactgctggtactctctatttcccagtcacgagagtgtaaaggcagggtcctaggaggttttttgtcaggctggtctcctcctctgcccctgcagtgagagcctacattggtctgagaagccagggatggtctgttatggatcatattgctgactgtctctttaaaatctctcagcctgttggtgctgctggatggtttggaggcatttctaggagcctgcttctctttcagtgtttctccttcactgtggtatcccgaggcctggggctcatcgcctttcctcctaacccgaccagagctcctcttgcgctctatcagtgaccctttcttggatgtgtgtttctgattacattcactatcagtcaggtgtcctgtgtcccgactgctctgagacatggaatcattttccacattatagatgactgtcccctgagaatcagaagagaagtgactgaccacagactcatggtgggaatgtttgtagggatagctctccgttgaggaatctgttcgagtgtcacttgagatggagggctccctccctgaatcttcactgtcgtagcatgtcctgctgtatgactggaactcagcttggggaggcaggtcctgggtggaaactggggtaccctggggatctgcataaagcagcagcaggggctgataatgccccttgatgcatttggtcaccacatccttccatttgggcccaatctccttgacatgagcatcatcaaaatacatccatttgcgaatctttgtttgaaaaaagaatgtagaataatgtttgccatagtaacagatcattccaactaagtacagttcagattgcttggcccggtcatccgtcactctgaaaaacagatcacccagcttaaggcaggttcccaggctgtggataacatcttctgctaagtctgagtggtctgagtcccataccagcccaatcgtgataatctgtggagcattcatcaacacacggcgaatcctgatcctctctccacagttgcttggacagttccgcagatcccccatggtgctggcattctgcagcagctcaccaaacatgcttggtgaaggtttctctcgtctttccagcatacaaatagcctgattgcaaagggaagtggtggagatataatgtaccatctggatgaaaggcagcggatcagaagtggcaccacagctagtacatacacactgctcaaacaatgtcattgcaaatttctgatgggaaatgcagtgttgggcagtacatatatcctctttggtttcatcagcaatgtggaagtgaattctcatcaggaggttttcaaagcactctgcagcatcatccataattcccagctggaaacgttgttcatcctggaaagtctttgccagagcactgcggagagtgtcagatggaagcactttttcactactacactgaaactggttaaagattcccttgagagcgcaaaagatgcaggaatctcccatgcacttgtgagttgtaagctgcctaaagctacgtcggaagatatccaagtgccacaaaacctgcagggcactgttgaggaagcagctgttttgccctggctcattgctgaggcctttgctgggggctatggaggttgagcttcgaggtgcaaacatcccttgtacactaccacgaccccctgaaaaataatttctcttccaagacattattgttcacatttagcctgaaaaaaaaatggagaaggatttgtgcctttttggcaggaatttctgtctgctaaagttctaaaaggaaagggaatccagaatttagtgaatttattttggaagattttgactttaccaccttccaaatatcatctgtgtagtcaagggactcaggtatcctcctagatcaagatgacagagccctccctcacttgttccaaacaatctccaaaatgtaacatggcacaggactaatgcaaacagagaaatccttaagtattgcttccttctatttttcttgaacagcctccataaagtcctggtgaagtggatgtaattctcaactccaacagcatccaggatcagggtaagatgtgttcttcaggcttgttgataatgcttcttatggactgaagatttttccaactggaaggagaggcagacagagaagcaagaatccaacatgatcctcctcaccctctattgccttgtctcatcatcctctgaagcaaaaactcaaattctgagcaactgcaaaaggttccacaaagccaagaagaagcctgtttgaatcatctgaggtttttgttgatgttcttgctgcttctttttaatgtgccccaaacttctattgtcccatccagatcttcagcaagtctctcctctttcttctgggactagaatagccagctgtgtcagagagcagacagcacagtcaacctccagcaaaagacctctaatcacgagggtatctgtggggcaagtgatacaagaatggggagggatatgggaatagctagagctgtggggagggaaggctaggagggaggagacgactgtagctagcaacaatgagaaactgtgaatctaaaccacaaggacttcccgcagaacaggatatcagagagaaggcaattctttttaccaactaccaggaactcagcactgacaattcatgacaaagttaaaaaggtggagcttccaattaaaaacaaagtaaacttaagaaactaaccaaaagtaacttgaaaggacgttatcacaaacttcacctgaggcttaagaaaaacaattatgaagctgtttcctggggcattcctgatgacaaaggtcattaaacaataaggtttgcagggtggctgctgcttccaaagaagggccagtcccccacaaaaaaattcctttgcactgcagtcaaaaggagcacgagaagacaacatttttgtagttgtttacagaataatcaaaacaatgttattgttggaatccctaattcagaattccaagactgggcttaaattaaatcaaatcattttaataggcaaaactcctccaactgtcttaaacgagccacactattaaagaaaattattatttaaactgagccattggaatctactgagtcaattttaaaatgcttgggatctaagggttctcaaccccaaagtccacaacagggaaagatctccacccctctctcggggaagagacctagttacatcaccaagaacaaacagcaggcagagtcccacccccaaacatgtgatcagtcaaccgagaacttgcatttgcaggcagggcacaaaggccccagaggaccaacacacacccttctatgtattacctgaggttataaaacagttttattgaaagaagttgttttataagcatactgatgaaaaaaactcatcagcagaatccttgccaaatatgaaggtctgttgtgtttctataggttgagagaaaatatacgagttgactaaaaaaaagatgtaattaagatttattggtaaaatttaacaaacatgggcaatgtccaaaactaattaagctcttacattttaacaatacagtatattaaattgaagtagtcctttggccacaaggaaagtgccacaaaaaaaaaaaaaaaaaaaaagatactgttgcttttcttgttaaccattagcattctaactcaggtctcctagtggtgctaggtggaggaggaggtagtaatgccatttcaaagtgtgaaacacaaaatttctactgataagtgctgactgcaaataaagacatacaaacatcaagaccaagctcttcaatcaagtcattaaaatataggtatatattcattgtgaaactaatcaaataaaactagagtactgggacagagttacagagcttcaaccctgattacaactagacaacattacttttcatgtctcatccaggtaagggaagtgatccacagggaaatctcactctaatagatt

SEQ ID NO: 10561 - RNA, 5287 nt, Homo sapiens
  source 1..5287: mol_type = other RNA
cggcccgggctgctgctgttcctctcactgctttcatagccagattccattcgctggattagtcgggggtgctgctctaaaaggtgagagcctggccgtgctgggccccagcgcttgtactgggggcttggtccaccaaatttaatgtcgtaagaaggtggcttgcttggttcatctggtataaattctttagctgaatcctcagaaaaggggctaagctgggtatagccacagtgcttccttttgtccttactaaagatactgtcaatattcagagattctcgtttgggtctccatgtgggacgatacttgctggaagaactggattttgactcactgctggtactctctatttcccagtcacgagagtgtaaaggcagggtcctaggaggttttttgtcaggctggtctcctcctctgcccctgcagtgagagcctacattggtctgagaagccagggatggtctgttatggatcatattgctgactgtctctttaaaatctctcagcctgttggtgctgctggatggtttggaggcatttctaggagcctgcttctctttcagtgtttctccttcactgtggtatcccgaggcctggggctcatcgcctttcctcctaacccgaccagagctcctcttgcgctctatcagtgaccctttcttggatgtgtgtttctgattacattcactatcagtcaggtgtcctgtgtcccgactgctctgagacatggaatcattttccacattatagatgactgtcccctgagaatcagaagagaagtgactgaccacagactcatggtgggaatgtttgtagggatagctctccgttgaggaatctgttcgagtgtcacttgagatggagggctccctccctgaatcttcactgtcgtagcatgtcctgctgtatgactggaactcagcttggggaggcaggtcctgggtggaaactggggtaccctggggatctgcataaagcagcagcaggggctgataatgccccttgatgcatttggtcaccacatccttccatttgggcccaatctccttgacatgagcatcatcaaaatacatccatttgcgaatctttgtttgaaaaaagaatgtagaataatgtttgccatagtaacagatcattccaactaagtacagttcagattgcttggcccggtcatccgtcactctgaaaaacagatcacccagcttaaggcaggttcccaggctgtggataacatcttctgctaagtctgagtggtctgagtcccataccagcccaatcgtgataatctgtggagcattcatcaacacacggcgaatcctgatcctctctccacagttgcttggacagttccgcagatcccccatggtgctggcattctgcagcagctcaccaaacatgcttggtgaaggtttctctcgtctttccagcatacaaatagcctgattgcaaagggaagtggtggagatataatgtaccatctggatgaaaggcagcggatcagaagtggcaccacagctagtacatacacactgctcaaacaatgtcattgcaaatttctgatgggaaatgcagtgttgggcagtacatatatcctctttggtttcatcagcaatgtggaagtgaattctcatcaggaggttttcaaagcactctgcagcatcatccataattcccagctggaaacgttgttcatcctggaaagtctttgccagagcactgcggagagtgtcagatggaagcactttttcactactacactgaaactggttaaagattcccttgagagcgcaaaagatgcaggaatctcccatgcacttgtgagttgtaagctgcctaaagctacgtcggaagatatccaagtgccacaaaacctgcagggcactgttgaggaagcagctgttttgccctggctcattgctgaggcctttgctgggggctatggaggttgagcttcgaggtgcaaacatcccttgtacactaccacgaccccctgaaaaataatttctcttccaagacattattgttcacatttagcctgaaaaaaaaatggagaaggatttgtgcctttttggcaggaatttctgtctgctaaagttctaaaaggaaagggaatccagaatttagtgaatttattttggaagattttgactttaccaccttccaaatatcatctgtgtagtcaagggactcaggtatcctcctagatcaagatgacagagccctccctcacttgttccaaacaatctccaaaatgtaacatggcacaggactaatgcaaacagagaaatccttaagtattgcttccttctatttttcttgaacagcctccataaagtcctggtgaagtggatgtaattctcaactccaacagcatccaggatcagggtaagatgtgttcttcaggcttgttgataatgcttcttatggactgaagatttttccaactggaaggagaggcagacagagaagcaagaatccaacatgatcctcctcaccctctattgccttgtctcatcatcctctgaagcaaaaactcaaattctgagcaactgcaaaaggttccacaaagccaagaagaagcctgtttgaatcatctgaggtttttgttgatgttcttgctgcttctttttaatgtgccccaaacttctattgtcccatccagatcttcagcaagtctctcctctttcttctgggactagaatagccagctgtgtcagagagctttaacagaaataaaaaaaatcaaaagcttgcgtcacttaatgactctactggctttggactgttctgccaagatcaacgttgcctcacttctcactataaacttgaaaccttggcaaacaatgccaaaaaaaaagaaaaaaagaaaaaaaaaaaaaagagagagacacccaaactaaagagaaggaaaaaaaggtatgaacagctttactttcaggggaaaattctctgaaattttcttgaagcagaagaaagttgatctggatagaaataaaaacaaaatacaaactttccagtatcaggctaacacaaaacaaatcaccaagtaagcacacacaaactaggaactgaaagttccttttggacattgtgaataaagcactttttaaaaggtgttttccatgaatatgcttatgaaaacgtgcttaaaggtgggaaggccatgttagcagtctaagatctgttctgagtaaagatgttccatccagagaaacactgatggcgagtaaaccacatgtccttaacatgcagtccaagagaactaaatcttctcctgccctgtttgtttgtttgtttcatttttgccagaggatcagagagataatttgggttacaaatcatttaatctccagattatatccaagggctcacaatcagaggcaatccattgaccaactttagttttcaactaattaaaatgccagtgaggcaacagagagtaataccaaagcaagtatgttccctggaaggaaatcaccacatctccagctttaagttttcctataaggctgccatgtccatctacataaggaaaaatttttaaatgttaagtgttaaatttgccaacatcaacaattcctcattctcccttccttctcaccatcatatgcaccatctaaaaacacaaaaatgctttaacatcttaatcattctctgggagatcacctagcattgtctacagcatgtccaatggaaaaactgaggtacaggaatattaaatggttgcataagactgttctttcccttctgtaaattcccagactatttataatctacatgtcccaattaaagtatttgattatacagcctactgtcacattattctctatttttattactctctgttttatatcgtatccgtcataatatgactacatgaaatgaaatagtagctacagtcaggtatgtgctaaacacgatacttatgtcctttatttaatattcacaacagtcctatcagatagctattaatagttccattttacagaaaagtaaagagaggcttaaagacattaacttgcccaattcaacactggtaagtggcagatctagaaatgtttgactattaaacaatgacttaattatatattttattattctattccaaaagctcctattacagtgccagtcataagaaggcagtcaataaatactgcctgatgattaacatgacactagaaaagaacccatatctcccacacagactataagaccctcacctttctacacacaccctcatacacaccccactcaaggccactaagcaacttccaacaagccatgcagcattccttcagctcaactgctgcaaaggaatgacaagtaccaagcctccactttgctcacagccaaaaggacttggcaggcaggtggggtttccaatatccacattaggagctaactgaaactcagcctgccctatgacacacactcctgagtacagggagcaaaaggagaaaaacgcagtagcagagaaaagattctcaggctctgaatggcagtattatgtagggtaaagcagtaagttctcagacctgttctagatgtgtcaccaactagaagtgagagcataaaggaccagacaagagaggcagtaacaagtggtccagagaaatactaacaccaaaaacatttcacttaaattgtagatatagcattaaacaatgtaatccttctccaataccatttactgaagatatgtgaggaggggaattatagttttatctgtatggctctcactacctagttttgttttttgggttttgttttgttttgttttgttttgtttctgaggcagaatctcactgtcacccaggctggagtgcagtcgcgcaatattggctcactgcagcctccgcctcttaggttcaagcaatcctcctgcctcagcctcccgagtagctgggattacaggcatgtgccactatgcctggctaatttttgtatttttagtagagacgggatttcaccaggggctggtctcaaacccctgacttcaggtgatccacctgccttgacttcccaaatgctgggattacaggcatgagccaccgcacccagccagtcaattgatttttgatgaaagtaccaaggccatttaattgagaaatgacagtcttttcaacaaatgatgttggaacaattgggacacccatatgcaaaaaactgaacattgagtcataccttacatcttatacaaaaataattcaatacatcacagtcctaaacaaaaaacctaaaactataaattctaggagaagacaggagaaaattttataacctt

SEQ ID NO: 10562 - RNA, 3572 nt, Homo sapiens
  source 1..3572: mol_type = other RNA
cggcccgggctgctgctgttcctctcactgctttcatagccagattccattcgctggattagtcgggggtgctgctctaaaaggtgagagcctggccgtgctgggccccagcgcttgtactgggggcttggtccaccaaatttaatgtcgtaagaaggtggcttgcttggttcatctggtataaattctttagctgaatcctcagaaaaggggctaagctgggtatagccacagtgcttccttttgtccttactaaagatactgtcaatattcagagattctcgtttgggtctccatgtgggacgatacttgctggaagaactggattttgactcactgctggtactctctatttcccagtcacgagagtgtaaaggcagggtcctaggaggttttttgtcaggctggtctcctcctctgcccctgcagtgagagcctacattggtctgagaagccagggatggtctgttatggatcatattgctgactgtctctttaaaatctctcagcctgttggtgctgctggatggtttggaggcatttctaggagcctgcttctctttcagtgtttctccttcactgtggtatcccgaggcctggggctcatcgcctttcctcctaacccgaccagagctcctcttgcgctctatcagtgaccctttcttggatgtgtgtttctgattacattcactatcagtcaggtgtcctgtgtcccgactgctctgagacatggaatcattttccacattatagatgactgtcccctgagaatcagaagagaagtgactgaccacagactcatggtgggaatgtttgtagggatagctctccgttgaggaatctgttcgagtgtcacttgagatggagggctccctccctgaatcttcactgtcgtagcatgtcctgctgtatgactggaactcagcttggggaggcaggtcctgggtggaaactggggtaccctggggatctgcataaagcagcagcaggggctgataatgccccttgatgcatttggtcaccacatccttccatttgggcccaatctccttgacatgagcatcatcaaaatacatccatttgcgaatctttgtttgaaaaaagaatgtagaataatgtttgccatagtaacagatcattccaactaagtacagttcagattgcttggcccggtcatccgtcactctgaaaaacagatcacccagcttaaggcaggttcccaggctgtggataacatcttctgctaagtctgagtggtctgagtcccataccagcccaatcgtgataatctgtggagcattcatcaacacacggcgaatcctgatcctctctccacagttgcttggacagttccgcagatcccccatggtgctggcattctgcagcagctcaccaaacatgcttggtgaaggtttctctcgtctttccagcatacaaatagcctgattgcaaagggaagtggtggagatataatgtaccatctggatgaaaggcagcggatcagaagtggcaccacagctagtacatacacactgctcaaacaatgtcattgcaaatttctgatgggaaatgcagtgttgggcagtacatatatcctctttggtttcatcagcaatgtggaagtgaattctcatcaggaggttttcaaagcactctgcagcatcatccataattcccagctggaaacgttgttcatcctggaaagtctttgccagagcactgcggagagtgtcagatggaagcactttttcactactacactgaaactggttaaagattcccttgagagcgcaaaagatgcaggaatctcccatgcacttgtgagttgtaagctgcctaaagctacgtcggaagatatccaagtgccacaaaacctgcagggcactgttgaggaagcagctgttttgccctggctcattgctgaggcctttgctgggggctatggaggttgagcttcgaggtgcaaacatcccttgtacactaccacgaccccctgaaaaataatttctcttccaagacattattgttcacatttagccttccaaatatcatctgtgtagtcaagggactcaggtatcctcctagatcaagatgacagagccctccctcacttgttccaaacaatctccaaaatgtaacatggcacaggactaatgcaaacagagaaatccttaagtattgcttccttctatttttcttgaacagcctccataaagtcctggtgaagtggatgtaattctcaactccaacagcatccaggatcagggtaagatgtgttcttcaggcttgttgataatgcttcttatggactgaagatttttccaactggaaggagaggcagacagagaagcaagaatccaacatgatcctcctcaccctctattgccttgtctcatcatcctctgaagcaaaaactcaaattctgagcaactgcaaaaggttccacaaagccaagaagaagcctgtttgaatcatctgaggtttttgttgatgttcttgctgcttctttttaatgtgccccaaacttctattgtcccatccagatcttcagcaagtctctcctctttcttctgggactagaatagccagctgtgtcagagagagctcctggcgccgcatacttaaccgccgcggctgctatagctacagggagccaaggcaaccagctctcgcgacactttccttggccatggcgagagcacacgagaagagactctcgcaagaaagtaaatgagtcaggctggaaacagcgaagtatatctcgcgatagcactgtttaaaatggcggcttcaaggcgtttcacgggtgtcccggacaggcgtggaggtggggcgcaggcgaggatgaagcttgagttggccaggagtcggaaaacgattgcaggcgggaccgcgtccgtcggggctgaggaaacttagcgtggcagaccctaaactgggataactttagggatatggccttcttttcccagttgcctcaaacttagagcagcgtcgtctttagccgaagattcattttcccagcattttccttctccaggcggagtagttggagacagagggcaagccagaaactgaccttcccatctcctcattcccttccatcaagaacttttcatcgttctttccccaccctggtttgtaaatggtatttggcttcataaaaacgtttgtccacaggtgccctgctccatcagttcgctccagcaatataggaagttaccaaaaaaaaaatttttttttattgaccttggatgcagaaaggaaccgcgttggtgtgtgatttgaattttggacttcttgtttcctgccttgtggccacgtcccccttacttggtgactctcagcacttagttgtggggctttttctctctgctctcagacaactataaaagcagactaattgaacagcatctagaacagaaggtggatgtaaagaacattggtcggccgggcgctgtggctcacgcctgtaatcccagcacttgagaggccgaggcgggcagatcacgaggtcaggagatcgagaccatcctgaccaacattgtgaaaccccgtctctactaaaaata

SEQ ID NO: 10563 - RNA, 2656 nt, Homo sapiens
  source 1..2656: mol_type = other RNA
cggcccgggctgctgctgttcctctcactgctttcatagccagattccattcgctggattagtcgggggtgctgctctaaaaggtgagagcctggccgtgctgggccccagcgcttgtactgggggcttggtccaccaaatttaatgtcgtaagaaggtggcttgcttggttcatctggtataaattctttagctgaatcctcagaaaaggggctaagctgggtatagccacagtgcttccttttgtccttactaaagatactgtcaatattcagagattctcgtttgggtctccatgtgggacgatacttgctggaagaactggattttgactcactgctggtactctctatttcccagtcacgagagtgtaaaggcagggtcctaggaggttttttgtcaggctggtctcctcctctgcccctgcagtgagagcctacattggtctgagaagccagggatggtctgttatggatcatattgctgactgtctctttaaaatctctcagcctgttggtgctgctggatggtttggaggcatttctaggagcctgcttctctttcagtgtttctccttcactgtggtatcccgaggcctggggctcatcgcctttcctcctaacccgaccagagctcctcttgcgctctatcagtgaccctttcttggatgtgtgtttctgattacattcactatcagtcaggtgtcctgtgtcccgactgctctgagacatggaatcattttccacattatagatgactgtcccctgagaatcagaagagaagtgactgaccacagactcatggtgggaatgtttgtagggatagctctccgttgaggaatctgttcgagtgtcacttgagatggagggctccctccctgaatcttcactgtcgtagcatgtcctgctgtatgactggaactcagcttggggaggcaggtcctgggtggaaactggggtaccctggggatctgcataaagcagcagcaggggctgataatgccccttgatgcatttggtcaccacatccttccatttgggcccaatctccttgacatgagcatcatcaaaatacatccatttgcgaatctttgtttgaaaaaagaatgtagaataatgtttgccatagtaacagatcattccaactaagtacagttcagattgcttggcccggtcatccgtcactctgaaaaacagatcacccagcttaaggcaggttcccaggctgtggataacatcttctgctaagtctgagtggtctgagtcccataccagcccaatcgtgataatctgtggagcattcatcaacacacggcgaatcctgatcctctctccacagttgcttggacagttccgcagatcccccatggtgctggcattctgcagcagctcaccaaacatgcttggtgaaggtttctctcgtctttccagcatacaaatagcctgattgcaaagggaagtggtggagatataatgtaccatctggatgaaaggcagcggatcagaagtggcaccacagctagtacatacacactgctcaaacaatgtcattgcaaatttctgatgggaaatgcagtgttgggcagtacatatatcctctttggtttcatcagcaatgtggaagtgaattctcatcaggaggttttcaaagcactctgcagcatcatccataattcccagctggaaacgttgttcatcctggaaagtctttgccagagcactgcggagagtgtcagatggaagcactttttcactactacactgaaactggttaaagattcccttgagagcgcaaaagatgcaggaatctcccatgcacttgtgagttgtaagctgcctaaagctacgtcggaagatatccaagtgccacaaaacctgcagggcactgttgaggaagcagctgttttgccctggctcattgctgaggcctttgctgggggctatggaggttgagcttcgaggtgcaaacatcccttgtacactaccacgaccccctgaaaaataatttctcttccaagacattattgttcacatttagccttccaaatatcatctgtgtagtcaagggactcaggtatcctcctagatcaagatgacagagccctccctcacttgttccaaacaatctccaaaatgtaacatggcacaggactaatgcaaacagagaaatccttaagtattgcttccttctatttttcttgaacagcctccataaagtcctggtgaagtggatgtaattctcaactccaacagcatccaggatcagggtaagatgtgttcttcaggcttgttgataatgcttcttatggactgaagatttttccaactggaaggagaggcagacagagaagcaagaatccaacatgatcctcctcaccctctattgccttgtctcatcatcctctgaagcaaaaactcaaattctgagcaactgcaaaaggttccacaaagccaagaagaagcctgtttgaatcatctgaggtttttgttgatgttcttgctgcttctttttaatgtgccccaaacttctattgtcccatccagatcttcagcaagtctctcctctttcttctgggactagaatagccagctgtgtcagagagaggacccaggtcctgccccacacgtcacactcaggtccattcctcccgcgacct

SEQ ID NO: 10564 - RNA, 2667 nt, Homo sapiens
  source 1..2667: mol_type = other RNA
cggcccgggctgctgctgttcctctcactgctttcatagccagattccattcgctggattagtcgggggtgctgctctaaaaggtgagagcctggccgtgctgggccccagcgcttgtactgggggcttggtccaccaaatttaatgtcgtaagaaggtggcttgcttggttcatctggtataaattctttagctgaatcctcagaaaaggggctaagctgggtatagccacagtgcttccttttgtccttactaaagatactgtcaatattcagagattctcgtttgggtctccatgtgggacgatacttgctggaagaactggattttgactcactgctggtactctctatttcccagtcacgagagtgtaaaggcagggtcctaggaggttttttgtcaggctggtctcctcctctgcccctgcagtgagagcctacattggtctgagaagccagggatggtctgttatggatcatattgctgactgtctctttaaaatctctcagcctgttggtgctgctggatggtttggaggcatttctaggagcctgcttctctttcagtgtttctccttcactgtggtatcccgaggcctggggctcatcgcctttcctcctaacccgaccagagctcctcttgcgctctatcagtgaccctttcttggatgtgtgtttctgattacattcactatcagtcaggtgtcctgtgtcccgactgctctgagacatggaatcattttccacattatagatgactgtcccctgagaatcagaagagaagtgactgaccacagactcatggtgggaatgtttgtagggatagctctccgttgaggaatctgttcgagtgtcacttgagatggagggctccctccctgaatcttcactgtcgtagcatgtcctgctgtatgactggaactcagcttggggaggcaggtcctgggtggaaactggggtaccctggggatctgcataaagcagcagcaggggctgataatgccccttgatgcatttggtcaccacatccttccatttgggcccaatctccttgacatgagcatcatcaaaatacatccatttgcgaatctttgtttgaaaaaagaatgtagaataatgtttgccatagtaacagatcattccaactaagtacagttcagattgcttggcccggtcatccgtcactctgaaaaacagatcacccagcttaaggcaggttcccaggctgtggataacatcttctgctaagtctgagtggtctgagtcccataccagcccaatcgtgataatctgtggagcattcatcaacacacggcgaatcctgatcctctctccacagttgcttggacagttccgcagatcccccatggtgctggcattctgcagcagctcaccaaacatgcttggtgaaggtttctctcgtctttccagcatacaaatagcctgattgcaaagggaagtggtggagatataatgtaccatctggatgaaaggcagcggatcagaagtggcaccacagctagtacatacacactgctcaaacaatgtcattgcaaatttctgatgggaaatgcagtgttgggcagtacatatatcctctttggtttcatcagcaatgtggaagtgaattctcatcaggaggttttcaaagcactctgcagcatcatccataattcccagctggaaacgttgttcatcctggaaagtctttgccagagcactgcggagagtgtcagatggaagcactttttcactactacactgaaactggttaaagattcccttgagagcgcaaaagatgcaggaatctcccatgcacttgtgagttgtaagctgcctaaagctacgtcggaagatatccaagtgccacaaaacctgcagggcactgttgaggaagcagctgttttgccctggctcattgctgaggcctttgctgggggctatggaggttgagcttcgaggtgcaaacatcccttgtacactaccacgaccccctgaaaaataatttctcttccaagacattattgttcacatttagccttccaaatatcatctgtgtagtcaagggactcaggtatcctcctagatcaagatgacagagccctccctcacttgttccaaacaatctccaaaatgtaacatggcacaggactaatgcaaacagagaaatccttaagtattgcttccttctatttttcttgaacagcctccataaagtcctggtgaagtggatgtaattctcaactccaacagcatccaggatcagggtaagatgtgttcttcaggcttgttgataatgcttcttatggactgaagatttttccaactggaaggagaggcagacagagaagcaagaatccaacatgatcctcctcaccctctattgccttgtctcatcatcctctgaagcaaaaactcaaattctgagcaactgcaaaaggttccacaaagccaagaagaagcctgtttgaatcatctgaggtttttgttgatgttcttgctgcttctttttaatgtgccccaaacttctattgtcccatccagatcttcagcaagtctctcctctttcttctgggactagaatagccagctgtgtcagagagcagacagcacagtcaacctccagcaaaagacctctaatcacgagggtatctgtggggcaagtgat

SEQ ID NO: 10565 - RNA, 4157 nt, Homo sapiens
  source 1..4157: mol_type = other RNA
cggcccgggctgctgctgttcctctcactgctttcatagccagattccattcgctggattagtcgggggtgctgctctaaaaggtgagagcctggccgtgctgggccccagcgcttgtactgggggcttggtccaccaaatttaatgtcgtaagaaggtggcttgcttggttcatctggtataaattctttagctgaatcctcagaaaaggggctaagctgggtatagccacagtgcttccttttgtccttactaaagatactgtcaatattcagagattctcgtttgggtctccatgtgggacgatacttgctggaagaactggattttgactcactgctggtactctctatttcccagtcacgagagtgtaaaggcagggtcctaggaggttttttgtcaggctggtctcctcctctgcccctgcagtgagagcctacattggtctgagaagccagggatggtctgttatggatcatattgctgactgtctctttaaaatctctcagcctgttggtgctgctggatggtttggaggcatttctaggagcctgcttctctttcagtgtttctccttcactgtggtatcccgaggcctggggctcatcgcctttcctcctaacccgaccagagctcctcttgcgctctatcagtgaccctttcttggatgtgtgtttctgattacattcactatcagtcaggtgtcctgtgtcccgactgctctgagacatggaatcattttccacattatagatgactgtcccctgagaatcagaagagaagtgactgaccacagactcatggtgggaatgtttgtagggatagctctccgttgaggaatctgttcgagtgtcacttgagatggagggctccctccctgaatcttcactgtcgtagcatgtcctgctgtatgactggaactcagcttggggaggcaggtcctgggtggaaactggggtaccctggggatctgcataaagcagcagcaggggctgataatgccccttgatgcatttggtcaccacatccttccatttgggcccaatctccttgacatgagcatcatcaaaatacatccatttgcgaatctttgtttgaaaaaagaatgtagaataatgtttgccatagtaacagatcattccaactaagtacagttcagattgcttggcccggtcatccgtcactctgaaaaacagatcacccagcttaaggcaggttcccaggctgtggataacatcttctgctaagtctgagtggtctgagtcccataccagcccaatcgtgataatctgtggagcattcatcaacacacggcgaatcctgatcctctctccacagttgcttggacagttccgcagatcccccatggtgctggcattctgcagcagctcaccaaacatgcttggtgaaggtttctctcgtctttccagcatacaaatagcctgattgcaaagggaagtggtggagatataatgtaccatctggatgaaaggcagcggatcagaagtggcaccacagctagtacatacacactgctcaaacaatgtcattgcaaatttctgatgggaaatgcagtgttgggcagtacatatatcctctttggtttcatcagcaatgtggaagtgaattctcatcaggaggttttcaaagcactctgcagcatcatccataattcccagctggaaacgttgttcatcctggaaagtctttgccagagcactgcggagagtgtcagatggaagcactttttcactactacactgaaactggttaaagattcccttgagagcgcaaaagatgcaggaatctcccatgcacttgtgagttgtaagctgcctaaagctacgtcggaagatatccaagtgccacaaaacctgcagggcactgttgaggaagcagctgttttgccctggctcattgctgaggcctttgctgggggctatggaggttgagcttcgaggtgcaaacatcccttgtacactaccacgaccccctgaaaaataatttctcttccaagacattattgttcacatttagccttccaaatatcatctgtgtagtcaagggactcaggtatcctcctagatcaagatgacagagccctccctcacttgttccaaacaatctccaaaatgtaacatggcacaggactaatgcaaacagagaaatccttaagtattgcttccttctatttttcttgaacagcctccataaagtcctggtgaagtggatgtaattctcaactccaacagcatccaggatcagggtaagatgtgttcttcaggcttgttgataatgcttcttatggactgaagatttttccaactggaaggagaggcagacagagaagcaagaatccaacatgatcctcctcaccctctattgccttgtctcatcatcctctgaagcaaaaactcaaattctgagcaactgcaaaaggttccacaaagccaagaagaagcctgtttgaatcatctgaggtttttgttgatgttcttgctgcttctttttaatgtgccccaaacttctattgtcccatccagatcttcagcaagtctctcctctttcttctgggactagaatagccagctgtgtcagagagcagacagcacagtcaacctccagcaaaagacctctaatcacgagggtatctgtggggcaagtgatacaagaatggggagggatatgggaatagctagagctgtggggagggaaggctaggagggaggagacgactgtagctagcaacaatgagaaactgtgaatctaaaccacaaggacttcccgcagaacaggatatcagagagaaggcaattctttttaccaactaccaggaactcagcactgacaattcatgacaaagttaaaaaggtggagcttccaattaaaaacaaagtaaacttaagaaactaaccaaaagtaacttgaaaggacgttatcacaaacttcacctgaggcttaagaaaaacaattatgaagctgtttcctggggcattcctgatgacaaaggtcattaaacaataaggtttgcagggtggctgctgcttccaaagaagggccagtcccccacaaaaaaattcctttgcactgcagtcaaaaggagcacgagaagacaacatttttgtagttgtttacagaataatcaaaacaatgttattgttggaatccctaattcagaattccaagactgggcttaaattaaatcaaatcattttaataggcaaaactcctccaactgtcttaaacgagccacactattaaagaaaattattatttaaactgagccattggaatctactgagtcaattttaaaatgcttgggatctaagggttctcaaccccaaagtccacaacagggaaagatctccacccctctctcggggaagagacctagttacatcaccaagaacaaacagcaggcagagtcccacccccaaacatgtgatcagtcaaccgagaacttgcatttgcaggcagggcacaaaggccccagaggaccaacacacacccttctatgtattacctgaggttataaaacagttttattgaaagaagttgttttataagcatactgatgaaaaaaactcatcagcagaatccttgccaaatatgaaggtctgttgtgtttctataggttgagagaaaatatacgagttgactaaaaaaaagatgtaattaagatttattggtaaaatttaacaaacatgggcaatgtccaaaactaattaagctcttacattttaacaatacagtatattaaattgaagtagtcctttggccacaaggaaagtgccacaaaaaaaaaaaaaaaaaaaaagatactgttgcttttcttgttaaccattagcattctaactcaggtctcctagtggtgctaggtggaggaggaggtagtaatgccatttcaaagtgtgaaacacaaaatttctactgataagtgctgactgcaaataaagacatacaaacatcaagaccaagctcttcaatcaagtcattaaaatataggtatatattcattgtgaaactaatcaaataaaactagagtactgggacagagttacagagcttcaaccctgattacaactagacaacattacttttcatgtctcatccaggtaagggaagtgatccacagggaaatctcactctaatagatt

SEQ ID NO: 10566 - RNA, 4656 nt, Homo sapiens
  source 1..4656: mol_type = other RNA
cggcccgggctgctgctgttcctctcactgctttcatagccagattccattcgctggattagtcgggggtgctgctctaaaaggtgagagcctggccgtgctgggccccagcgcttgtactgggggcttggtccaccaaatttaatgtcgtaagaaggtggcttgcttggttcatctggtataaattctttagctgaatcctcagaaaaggggctaagctgggtatagccacagtgcttccttttgtccttactaaagatactgtcaatattcagagattctcgtttgggtctccatgtgggacgatacttgctggaagaactggattttgactcactgctggtactctctatttcccagtcacgagagtgtaaaggcagggtcctaggaggttttttgtcaggctggtctcctcctctgcccctgcagtgagagcctacattggtctgagaagccagggatggtctgttatggatcatattgctgactgtctctttaaaatctctcagcctgttggtgctgctggatggtttggaggcatttctaggagcctgcttctctttcagtgtttctccttcactgtggtatcccgaggcctggggctcatcgcctttcctcctaacccgaccagagctcctcttgcgctctatcagtgaccctttcttggatgtgtgtttctgattacattcactatcagtcaggtgtcctgtgtcccgactgctctgagacatggaatcattttccacattatagatgactgtcccctgagaatcagaagagaagtgactgaccacagactcatggtgggaatgtttgtagggatagctctccgttgaggaatctgttcgagtgtcacttgagatggagggctccctccctgaatcttcactgtcgtagcatgtcctgctgtatgactggaactcagcttggggaggcaggtcctgggtggaaactggggtaccctggggatctgcataaagcagcagcaggggctgataatgccccttgatgcatttggtcaccacatccttccatttgggcccaatctccttgacatgagcatcatcaaaatacatccatttgcgaatctttgtttgaaaaaagaatgtagaataatgtttgccatagtaacagatcattccaactaagtacagttcagattgcttggcccggtcatccgtcactctgaaaaacagatcacccagcttaaggcaggttcccaggctgtggataacatcttctgctaagtctgagtggtctgagtcccataccagcccaatcgtgataatctgtggagcattcatcaacacacggcgaatcctgatcctctctccacagttgcttggacagttccgcagatcccccatggtgctggcattctgcagcagctcaccaaacatgcttggtgaaggtttctctcgtctttccagcatacaaatagcctgattgcaaagggaagtggtggagatataatgtaccatctggatgaaaggcagcggatcagaagtggcaccacagctagtacatacacactgctcaaacaatgtcattgcaaatttctgatgggaaatgcagtgttgggcagtacatatatcctctttggtttcatcagcaatgtggaagtgaattctcatcaggaggttttcaaagcactctgcagcatcatccataattcccagctggaaacgttgttcatcctggaaagtctttgccagagcactgcggagagtgtcagatggaagcactttttcactactacactgaaactggttaaagattcccttgagagcgcaaaagatgcaggaatctcccatgcacttgtgagttgtaagctgcctaaagctacgtcggaagatatccaagtgccacaaaacctgcagggcactgttgaggaagcagctgttttgccctggctcattgctgaggcctttgctgggggctatggaggttgagcttcgaggtgcaaacatcccttgtacactaccacgaccccctgaaaaataatttctcttccaagacattattgttcacatttagccttccaaatatcatctgtgtagtcaagggactcaggtatcctcctagatcaagatgacagagccctccctcacttgttccaaacaatctccaaaatgtaacatggcacaggactaatgcaaacagagaaatccttaagtattgcttccttctatttttcttgaacagcctccataaagtcctggtgaagtggatgtaattctcaactccaacagcatccaggatcagggtaagatgtgttcttcaggcttgttgataatgcttcttatggactgaagatttttccaactggaaggagaggcagacagagaagcaagaatccaacatgatcctcctcaccctctattgccttgtctcatcatcctctgaagcaaaaactcaaattctgagcaactgcaaaaggttccacaaagccaagaagaagcctgtttgaatcatctgaggtttttgttgatgttcttgctgcttctttttaatgtgccccaaacttctattgtcccatccagatcttcagcaagtctctcctctttcttctgggactagaatagccagctgtgtcagagagctttaacagaaataaaaaaaatcaaaagcttgcgtcacttaatgactctactggctttggactgttctgccaagatcaacgttgcctcacttctcactataaacttgaaaccttggcaaacaatgccaaaaaaaaagaaaaaaagaaaaaaaaaaaaaagagagagacacccaaactaaagagaaggaaaaaaaggtatgaacagctttactttcaggggaaaattctctgaaattttcttgaagcagaagaaagttgatctggatagaaataaaaacaaaatacaaactttccagtatcaggctaacacaaaacaaatcaccaagtaagcacacacaaactaggaactgaaagttccttttggacattgtgaataaagcactttttaaaaggtgttttccatgaatatgcttatgaaaacgtgcttaaaggtgggaaggccatgttagcagtctaagatctgttctgagtaaagatgttccatccagagaaacactgatggcgagtaaaccacatgtccttaacatgcagtccaagagaactaaatcttctcctgccctgtttgtttgtttgtttcatttttgccagaggatcagagagataatttgggttacaaatcatttaatctccagattatatccaagggctcacaatcagaggcaatccattgaccaactttagttttcaactaattaaaatgccagtgaggcaacagagagtaataccaaagcaagtatgttccctggaaggaaatcaccacatctccagctttaagttttcctataaggctgccatgtccatctacataaggaaaaatttttaaatgttaagtgttaaatttgccaacatcaacaattcctcattctcccttccttctcaccatcatatgcaccatctaaaaacacaaaaatgctttaacatcttaatcattctctgggagatcacctagcattgtctacagcatgtccaatggaaaaactgaggtacaggaatattaaatggttgcataagactgttctttcccttctgtaaattcccagactatttataatctacatgtcccaattaaagtatttgattatacagcctactgtcacattattctctatttttattactctctgttttatatcgtatccgtcataatatgactacatgaaatgaaatagtagctacagtcaggtatgtgctaaacacgatacttatgtcctttatttaatattcacaacagtcctatcagatagctattaatagttccattttacagaaaagtaaagagaggcttaaagacattaacttgcccaattcaacactggtaagtggcagatctagaaatgtttgactattaaacaatgacttaattatatattttattattctattccaaaagctcctattacagtgccagtcataagaaggcagtcaataaatactgcctgatgattaacatgacactagaaaagaacccatatctcccacacagactataagaccctcacctttctacacacaccctcatacacaccccactcaaggccactaagcaacttccaacaagccatgcagcattccttcagctcaactgctgcaaaggaatgacaagtaccaagcctccactttgctcacagccaaaaggacttggcaggcaggtggggtttccaatatccacattaggagctaactgaaactcagcctgccctatgacacacactcctgagtacagggagcaaaaggagaaaaacgcagtagcagagaaaagattctcaggctctgaatggcagtattatgtagggtaaagcagtaagttctcagacctgttctagatgtgtcaccaactagaagtgagagcataaaggaccagacaagagaggcagtaacaagtggtccagagaaatactaacaccaaaaacatttcacttaaattgtagatatagcattaaacaatgtaatccttctccaataccatttactgaagatatgtgaggaggggaattatagttttatctgtatggctctcactacctagttttgttttttgggttttgttttgtttt

SEQ ID NO: 10567 - RNA, 3074 nt, Homo sapiens
  source 1..3074: mol_type = other RNA
cggcccgggctgctgctgttcctctcactgctttcatagccagattccattcgctggattagtcgggggtgctgctctaaaaggtgagagcctggccgtgctgggccccagcgcttgtactgggggcttggtccaccaaatttaatgtcgtaagaaggtggcttgcttggttcatctggtataaattctttagctgaatcctcagaaaaggggctaagctgggtatagccacagtgcttccttttgtccttactaaagatactgtcaatattcagagattctcgtttgggtctccatgtgggacgatacttgctggaagaactggattttgactcactgctggtactctctatttcccagtcacgagagtgtaaaggcagggtcctaggaggttttttgtcaggctggtctcctcctctgcccctgcagtgagagcctacattggtctgagaagccagggatggtctgttatggatcatattgctgactgtctctttaaaatctctcagcctgttggtgctgctggatggtttggaggcatttctaggagcctgcttctctttcagtgtttctccttcactgtggtatcccgaggcctggggctcatcgcctttcctcctaacccgaccagagctcctcttgcgctctatcagtgaccctttcttggatgtgtgtttctgattacattcactatcagtcaggtgtcctgtgtcccgactgctctgagacatggaatcattttccacattatagatgactgtcccctgagaatcagaagagaagtgactgaccacagactcatggtgggaatgtttgtagggatagctctccgttgaggaatctgttcgagtgtcacttgagatggagggctccctccctgaatcttcactgtcgtagcatgtcctgctgtatgactggaactcagcttggggaggcaggtcctgggtggaaactggggtaccctggggatctgcataaagcagcagcaggggctgataatgccccttgatgcatttggtcaccacatccttccatttgggcccaatctccttgacatgagcatcatcaaaatacatccatttgcgaatctttgtttgaaaaaagaatgtagaataatgtttgccatagtaacagatcattccaactaagtacagttcagattgcttggcccggtcatccgtcactctgaaaaacagatcacccagcttaaggcaggttcccaggctgtggataacatcttctgctaagtctgagtggtctgagtcccataccagcccaatcgtgataatctgtggagcattcatcaacacacggcgaatcctgatcctctctccacagttgcttggacagttccgcagatcccccatggtgctggcattctgcagcagctcaccaaacatgcttggtgaaggtttctctcgtctttccagcatacaaatagcctgattgctgtccccagatccaaagctcatagaatccccactcctcctcccactttgctggccagtactgagccaaagggaagtggtggagatataatgtaccatctggatgaaaggcagcggatcagaagtggcaccacagctagtacatacacactgctcaaacaatgtcattgcaaatttctgatgggaaatgcagtgttgggcagtacatatatcctctttggtttcatcagcaatgtggaagtgaattctcatcaggaggttttcaaagcactctgcagcatcatccataattcccagctggaaacgttgttcatcctggaaagtctttgccagagcactgcggagagtgtcagatggaagcactttttcactactacactgaaactggttaaagattcccttgagagcgcaaaagatgcaggaatctcccatgcacttgtgagttgtaagctgcctaaagctacgtcggaagatatccaagtgccacaaaacctgcagggcactgttgaggaagcagctgttttgccctggctcattgctgaggcctttgctgggggctatggaggttgagcttcgaggtgcaaacatcccttgtacactaccacgaccccctgaaaaataatttctcttccaagacattattgttcacatttagcagctcctggcgccgcatacttaaccgccgcggctgctatagctacagggagccaaggcaaccagctctcgcgacactttccttggccatggcgagagcacacgagaagagactctcgcaagaaagtaaatgagtcaggctggaaacagcgaagtatatctcgcgatagcactgtttaaaatggcggcttcaaggcgtttcacgggtgtcccggacaggcgtggaggtggggcgcaggcgaggatgaagcttgagttggccaggagtcggaaaacgattgcaggcgggaccgcgtccgtcggggctgaggaaacttagcgtggcagaccctaaactgggataactttagggatatggccttcttttcccagttgcctcaaacttagagcagcgtcgtctttagccgaagattcattttcccagcattttccttctccaggcggagtagttggagacagagggcaagccagaaactgaccttcccatctcctcattcccttccatcaagaacttttcatcgttctttccccaccctggtttgtaaatggtatttggcttcataaaaacgtttgtccacaggtgccctgctccatcagttcgctccagcaatataggaagttaccaaaaaaaaaatttttttttattgaccttggatgcagaaaggaaccgcgttggtgtgtgatttgaattttggacttcttgtttcctgccttgtggccacgtcccccttacttggtgactctcagcacttagttgtggggctttttctctctgctctcagacaactataaaagcagactaattgaacagcatctagaacagaaggtggatgtaaagaacattggtcggccgggcgctgtggctcacgcctgtaatcccagcacttgagaggccgaggcgggcagatcacgaggtcaggagatcgagaccatcctgaccaacattgtgaaaccccgtctctactaaaaata

SEQ ID NO: 10568 - RNA, 2828 nt, Homo sapiens
  source 1..2828: mol_type = other RNA
cggcccgggctgctgctgttcctctcactgctttcatagccagattccattcgctggattagtcgggggtgctgctctaaaaggtgagagcctggccgtgctgggccccagcgcttgtactgggggcttggtccaccaaatttaatgtcgtaagaaggtggcttgcttggttcatctggtataaattctttagctgaatcctcagaaaaggggctaagctgggtatagccacagtgcttccttttgtccttactaaagatactgtcaatattcagagattctcgtttgggtctccatgtgggacgatacttgctggaagaactggattttgactcactgctggtactctctatttcccagtcacgagagtgtaaaggcagggtcctaggaggttttttgtcaggctggtctcctcctctgcccctgcagtgagagcctacattggtctgagaagccagggatggtctgttatggatcatattgctgactgtctctttaaaatctctcagcctgttggtgctgctggatggtttggaggcatttctaggagcctgcttctctttcagtgtttctccttcactgtggtatcccgaggcctggggctcatcgcctttcctcctaacccgaccagagctcctcttgcgctctatcagtgaccctttcttggatgtgtgtttctgattacattcactatcagtcaggtgtcctgtgtcccgactgctctgagacatggaatcattttccacattatagatgactgtcccctgagaatcagaagagaagtgactgaccacagactcatggtgggaatgtttgtagggatagctctccgttgaggaatctgttcgagtgtcacttgagatggagggctccctccctgaatcttcactgtcgtagcatgtcctgctgtatgactggaactcagcttggggaggcaggtcctgggtggaaactggggtaccctggggatctgcataaagcagcagcaggggctgataatgccccttgatgcatttggtcaccacatccttccatttgggcccaatctccttgacatgagcatcatcaaaatacatccatttgcgaatctttgtttgaaaaaagaatgtagaataatgtttgccatagtaacagatcattccaactaagtacagttcagattgcttggcccggtcatccgtcactctgaaaaacagatcacccagcttaaggcaggttcccaggctgtggataacatcttctgctaagtctgagtggtctgagtcccataccagcccaatcgtgataatctgtggagcattcatcaacacacggcgaatcctgatcctctctccacagttgcttggacagttccgcagatcccccatggtgctggcattctgcagcagctcaccaaacatgcttggtgaaggtttctctcgtctttccagcatacaaatagcctgattgctgtccccagatccaaagctcatagaatccccactcctcctcccactttgctggccagtactgagccaaagggaagtggtggagatataatgtaccatctggatgaaaggcagcggatcagaagtggcaccacagctagtacatacacactgctcaaacaatgtcattgcaaatttctgatgggaaatgcagtgttgggcagtacatatatcctctttggtttcatcagcaatgtggaagtgaattctcatcaggaggttttcaaagcactctgcagcatcatccataattcccagctggaaacgttgttcatcctggaaagtctttgccagagcactgcggagagtgtcagatggaagcactttttcactactacactgaaactggttaaagattcccttgagagcgcaaaagatgcaggaatctcccatgcacttgtgagttgtaagctgcctaaagctacgtcggaagatatccaagtgccacaaaacctgcagggcactgttgaggaagcagctgttttgccctggctcattgctgaggcctttgctgggggctatggaggttgagcttcgaggtgcaaacatcccttgtacactaccacgaccccctgaaaaataatttctcttccaagacattattgttcacatttagccaagtgcctgaagtgtcaatcatttcctgcttctcccagctgcaggacttggaactaggaaaacattcagtcagcgtctagagcaggtctggttagaaggatgagctcatccctttcagatgcacacctgatcctcaagaagctgcccctcctccagcaagcagatctttgtatgtttaaagtgacacccacaacctgtacaaccactttgccagagccaaagtaagtctttccttatacatgcctagtgccatggaatcatttcctggtctagccacctcacacagccactgaacgcaggtggcagtggcaacagctgctgctgctgctactatggctttgttagagaaggacttcattttcagctacaacggaggtcaagtccttcaccactgccctggaaacactgcactgtttgtttcaacagccccttgcccacagtcagatcttaccagaatcatgccttctttcaaaactcacaaccatttttctgaaccaacaatgtagcacctcaacatctgccttattccatttgccctgtctaaaagttaaattagccaaggcagctaaatgtactgtatgtatttagagctaaaatgttcccaactcaggtttgccctcagttttactacctctaagaaaacctttattctgccatagcagtctatttattggtaaagtatacagtaatcctaatacagagatatgtaaacttcacttcatg

SEQ ID NO: 10569 - RNA, 2169 nt, Homo sapiens
  source 1..2169: mol_type = other RNA
cggcccgggctgctgctgttcctctcactgctttcatagccagattccattcgctggattagtcgggggtgctgctctaaaaggtgagagcctggccgtgctgggccccagcgcttgtactgggggcttggtccaccaaatttaatgtcgtaagaaggtggcttgcttggttcatctggtataaattctttagctgaatcctcagaaaaggggctaagctgggtatagccacagtgcttccttttgtccttactaaagatactgtcaatattcagagattctcgtttgggtctccatgtgggacgatacttgctggaagaactggattttgactcactgctggtactctctatttcccagtcacgagagtgtaaaggcagggtcctaggaggttttttgtcaggctggtctcctcctctgcccctgcagtgagagcctacattggtctgagaagccagggatggtctgttatggatcatattgctgactgtctctttaaaatctctcagcctgttggtgctgctggatggtttggaggcatttctaggagcctgcttctctttcagtgtttctccttcactgtggtatcccgaggcctggggctcatcgcctttcctcctaacccgaccagagctcctcttgcgctctatcagtgaccctttcttggatgtgtgtttctgattacattcactatcagtcaggtgtcctgtgtcccgactgctctgagacatggaatcattttccacattatagatgactgtcccctgagaatcagaagagaagtgactgaccacagactcatggtgggaatgtttgtagggatagctctccgttgaggaatctgttcgagtgtcacttgagatggagggctccctccctgaatcttcactgtcgtagcatgtcctgctgtatgactggaactcagcttggggaggcaggtcctgggtggaaactggggtaccctggggatctgcataaagcagcagcaggggctgataatgccccttgatgcatttggtcaccacatccttccatttgggcccaatctccttgacatgagcatcatcaaaatacatccatttgcgaatctttgtttgaaaaaagaatgtagaataatgtttgccatagtaacagatcattccaactaagtacagttcagattgcttggcccggtcatccgtcactctgaaaaacagatcacccagcttaaggcaggttcccaggctgtggataacatcttctgctaagtctgagtggtctgagtcccataccagcccaatcgtgataatctgtggagcattcatcaacacacggcgaatcctgatcctctctccacagttgcttggacagttccgcagatcccccatggtgctggcattctgcagcagctcaccaaacatgcttggtgaaggtttctctcgtctttccagcatacaaatagcctgattgctgtccccagatccaaagctcatagaatccccactcctcctcccactttgctggccagtactgagccaaagggaagtggtggagatataatgtaccatctggatgaaaggcagcggatcagaagtggcaccacagctagtacatacacactgctcaaacaatgtcattgcaaatttctgatgggaaatgcagtgttgggcagtacatatatcctctttggtttcatcagcaatgtggaagtgaattctcatcaggaggttttcaaagcactctgcagcatcatccataattcccagctggaaacgttgttcatcctggaaagtctttgccagagcactgcggagagtgtcagatggaagcactttttcactactacactgaaactggttaaagattcccttgagagcgcaaaagatgcaggaatctcccatgcacttgtgagttgtaagctgcctaaagctacgtcggaagatatccaagtgccacaaaacctgcagggcactgttgaggaagcagctgttttgccctggctcattgctgaggcctttgctgggggctatggaggttgagcttcgaggtgcaaacatcccttgtacactaccacgaccccctgaaaaataatttctcttccaagacattattgttcacatttagccagacagcacagtcaacctccagcaaaagacctctaatcacgagggtatctgtggggcaagtgat

SEQ ID NO: 10570 - RNA, 2188 nt, Homo sapiens
  source 1..2188: mol_type = other RNA
cggcccgggctgctgctgttcctctcactgctttcatagccagattccattcgctggattagtcgggggtgctgctctaaaaggtgagagcctggccgtgctgggccccagcgcttgtactgggggcttggtccaccaaatttaatgtcgtaagaaggtggcttgcttggttcatctggtataaattctttagctgaatcctcagaaaaggggctaagctgggtatagccacagtgcttccttttgtccttactaaagatactgtcaatattcagagattctcgtttgggtctccatgtgggacgatacttgctggaagaactggattttgactcactgctggtactctctatttcccagtcacgagagtgtaaaggcagggtcctaggaggttttttgtcaggctggtctcctcctctgcccctgcagtgagagcctacattggtctgagaagccagggatggtctgttatggatcatattgctgactgtctctttaaaatctctcagcctgttggtgctgctggatggtttggaggcatttctaggagcctgcttctctttcagtgtttctccttcactgtggtatcccgaggcctggggctcatcgcctttcctcctaacccgaccagagctcctcttgcgctctatcagtgaccctttcttggatgtgtgtttctgattacattcactatcagtcaggtgtcctgtgtcccgactgctctgagacatggaatcattttccacattatagatgactgtcccctgagaatcagaagagaagtgactgaccacagactcatggtgggaatgtttgtagggatagctctccgttgaggaatctgttcgagtgtcacttgagatggagggctccctccctgaatcttcactgtcgtagcatgtcctgctgtatgactggaactcagcttggggaggcaggtcctgggtggaaactggggtaccctggggatctgcataaagcagcagcaggggctgataatgccccttgatgcatttggtcaccacatccttccatttgggcccaatctccttgacatgagcatcatcaaaatacatccatttgcgaatctttgtttgaaaaaagaatgtagaataatgtttgccatagtaacagatcattccaactaagtacagttcagattgcttggcccggtcatccgtcactctgaaaaacagatcacccagcttaaggcaggttcccaggctgtggataacatcttctgctaagtctgagtggtctgagtcccataccagcccaatcgtgataatctgtggagcattcatcaacacacggcgaatcctgatcctctctccacagttgcttggacagttccgcagatcccccatggtgctggcattctgcagcagctcaccaaacatgcttggtgaaggtttctctcgtctttccagcatacaaatagcctgattgctgtccccagatccaaagctcatagaatccccactcctcctcccactttgctggccagtactgagccaaagggaagtggtggagatataatgtaccatctggatgaaaggcagcggatcagaagtggcaccacagctagtacatacacactgctcaaacaatgtcattgcaaatttctgatgggaaatgcagtgttgggcagtacatatatcctctttggtttcatcagcaatgtggaagtgaattctcatcaggaggttttcaaagcactctgcagcatcatccataattcccagctggaaacgttgttcatcctggaaagtctttgccagagcactgcggagagtgtcagatggaagcactttttcactactacactgaaactggttaaagattcccttgagagcgcaaaagatgcaggaatctcccatgcacttgtgagttgtaagctgcctaaagctacgtcggaagatatccaagtgccacaaaacctgcagggcactgttgaggaagcagctgttttgccctggctcattgctgaggcctttgctgggggctatggaggttgagcttcgaggtgcaaacatcccttgtacactaccacgaccccctgaaaaataatttctcttccaagacattattgttcacatttagccctcctcgtcgctgtaccccatttcttcccacttctttcccaatgtagcctggtccctttatccagttccgagtctccgtaaac

SEQ ID NO: 10571 - RNA, 4388 nt, Homo sapiens
  source 1..4388: mol_type = other RNA
cggcccgggctgctgctgttcctctcactgctttcatagccagattccattcgctggattagtcgggggtgctgctctaaaaggtgagagcctggccgtgctgggccccagcgcttgtactgggggcttggtccaccaaatttaatgtcgtaagaaggtggcttgcttggttcatctggtataaattctttagctgaatcctcagaaaaggggctaagctgggtatagccacagtgcttccttttgtccttactaaagatactgtcaatattcagagattctcgtttgggtctccatgtgggacgatacttgctggaagaactggattttgactcactgctggtactctctatttcccagtcacgagagtgtaaaggcagggtcctaggaggttttttgtcaggctggtctcctcctctgcccctgcagtgagagcctacattggtctgagaagccagggatggtctgttatggatcatattgctgactgtctctttaaaatctctcagcctgttggtgctgctggatggtttggaggcatttctaggagcctgcttctctttcagtgtttctccttcactgtggtatcccgaggcctggggctcatcgcctttcctcctaacccgaccagagctcctcttgcgctctatcagtgaccctttcttggatgtgtgtttctgattacattcactatcagtcaggtgtcctgtgtcccgactgctctgagacatggaatcattttccacattatagatgactgtcccctgagaatcagaagagaagtgactgaccacagactcatggtgggaatgtttgtagggatagctctccgttgaggaatctgttcgagtgtcacttgagatggagggctccctccctgaatcttcactgtcgtagcatgtcctgctgtatgactggaactcagcttggggaggcaggtcctgggtggaaactggggtaccctggggatctgcataaagcagcagcaggggctgataatgccccttgatgcatttggtcaccacatccttccatttgggcccaatctccttgacatgagcatcatcaaaatacatccatttgcgaatctttgtttgaaaaaagaatgtagaataatgtttgccatagtaacagatcattccaactaagtacagttcagattgcttggcccggtcatccgtcactctgaaaaacagatcacccagcttaaggcaggttcccaggctgtggataacatcttctgctaagtctgagtggtctgagtcccataccagcccaatcgtgataatctgtggagcattcatcaacacacggcgaatcctgatcctctctccacagttgcttggacagttccgcagatcccccatggtgctggcattctgcagcagctcaccaaacatgcttggtgaaggtttctctcgtctttccagcatacaaatagcctgattgctgtccccagatccaaagctcatagaatccccactcctcctcccactttgctggccagtactgagccaaagggaagtggtggagatataatgtaccatctggatgaaaggcagcggatcagaagtggcaccacagctagtacatacacactgctcaaacaatgtcattgcaaatttctgatgggaaatgcagtgttgggcagtacatatatcctctttggtttcatcagcaatgtggaagtgaattctcatcaggaggttttcaaagcactctgcagcatcatccataattcccagctggaaacgttgttcatcctggaaagtctttgccagagcactgcggagagtgtcagatggaagcactttttcactactacactgaaactggttaaagattcccttgagagcgcaaaagatgcaggaatctcccatgcacttgtgagttgtaagctgcctaaagctacgtcggaagatatccaagtgccacaaaacctgcagggcactgttgaggaagcagctgttttgccctggctcattgctgaggcctttgctgggggctatggaggttgagcttcgaggtgcaaacatcccttgtacactaccacgaccccctgaaaaataatttctcttccaagacattattgttcacatttagccctctattgccttgtctcatcatcctctgaagcaaaaactcaaattctgagcaactgcaaaaggttccacaaagccaagaagaagcctgtttgaatcatctgaggtttttgttgatgttcttgctgcttctttttaatgtgccccaaacttctattgtcccatccagatcttcagcaagtctctcctctttcttctgggactagaatagccagctgtgtcagagagctttaacagaaataaaaaaaatcaaaagcttgcgtcacttaatgactctactggctttggactgttctgccaagatcaacgttgcctcacttctcactataaacttgaaaccttggcaaacaatgccaaaaaaaaagaaaaaaagaaaaaaaaaaaaaagagagagacacccaaactaaagagaaggaaaaaaaggtatgaacagctttactttcaggggaaaattctctgaaattttcttgaagcagaagaaagttgatctggatagaaataaaaacaaaatacaaactttccagtatcaggctaacacaaaacaaatcaccaagtaagcacacacaaactaggaactgaaagttccttttggacattgtgaataaagcactttttaaaaggtgttttccatgaatatgcttatgaaaacgtgcttaaaggtgggaaggccatgttagcagtctaagatctgttctgagtaaagatgttccatccagagaaacactgatggcgagtaaaccacatgtccttaacatgcagtccaagagaactaaatcttctcctgccctgtttgtttgtttgtttcatttttgccagaggatcagagagataatttgggttacaaatcatttaatctccagattatatccaagggctcacaatcagaggcaatccattgaccaactttagttttcaactaattaaaatgccagtgaggcaacagagagtaataccaaagcaagtatgttccctggaaggaaatcaccacatctccagctttaagttttcctataaggctgccatgtccatctacataaggaaaaatttttaaatgttaagtgttaaatttgccaacatcaacaattcctcattctcccttccttctcaccatcatatgcaccatctaaaaacacaaaaatgctttaacatcttaatcattctctgggagatcacctagcattgtctacagcatgtccaatggaaaaactgaggtacaggaatattaaatggttgcataagactgttctttcccttctgtaaattcccagactatttataatctacatgtcccaattaaagtatttgattatacagcctactgtcacattattctctatttttattactctctgttttatatcgtatccgtcataatatgactacatgaaatgaaatagtagctacagtcaggtatgtgctaaacacgatacttatgtcctttatttaatattcacaacagtcctatcagatagctattaatagttccattttacagaaaagtaaagagaggcttaaagacattaacttgcccaattcaacactggtaagtggcagatctagaaatgtttgactattaaacaatgacttaattatatattttattattctattccaaaagctcctattacagtgccagtcataagaaggcagtcaataaatactgcctgatgattaacatgacactagaaaagaacccatatctcccacacagactataagaccctcacctttctacacacaccctcatacacaccccactcaaggccactaagcaacttccaacaagccatgcagcattccttcagctcaactgctgcaaaggaatgacaagtaccaagcctccactttgctcacagccaaaaggacttggcaggcaggtggggtttccaatatccacattaggagctaactgaaactcagcctgccctatgacacacactcctgagtacagggagcaaaaggagaaaaacgcagtagcagagaaaagattctcaggctctgaatggcagtattatgtagggtaaagcagtaagttctcagacctgttctagatgtgtcaccaactagaagtgagagcataaaggaccagacaagagaggcagtaacaagtggtccagagaaatactaacaccaaaaacatttcacttaaattgtagatatagcattaaacaatgtaatccttctccaataccatttactgaagatatgtgaggaggggaattatagttttatctgtatggctctcactacctagttttgttttttgggttttgttttgttttgttt

SEQ ID NO: 10572 - RNA, 3760 nt, Homo sapiens
  source 1..3760: mol_type = other RNA
cggcccgggctgctgctgttcctctcactgctttcatagccagattccattcgctggattagtcgggggtgctgctctaaaaggtgagagcctggccgtgctgggccccagcgcttgtactgggggcttggtccaccaaatttaatgtcgtaagaaggtggcttgcttggttcatctggtataaattctttagctgaatcctcagaaaaggggctaagctgggtatagccacagtgcttccttttgtccttactaaagatactgtcaatattcagagattctcgtttgggtctccatgtgggacgatacttgctggaagaactggattttgactcactgctggtactctctatttcccagtcacgagagtgtaaaggcagggtcctaggaggttttttgtcaggctggtctcctcctctgcccctgcagtgagagcctacattggtctgagaagccagggatggtctgttatggatcatattgctgactgtctctttaaaatctctcagcctgttggtgctgctggatggtttggaggcatttctaggagcctgcttctctttcagtgtttctccttcactgtggtatcccgaggcctggggctcatcgcctttcctcctaacccgaccagagctcctcttgcgctctatcagtgaccctttcttggatgtgtgtttctgattacattcactatcagtcaggtgtcctgtgtcccgactgctctgagacatggaatcattttccacattatagatgactgtcccctgagaatcagaagagaagtgactgaccacagactcatggtgggaatgtttgtagggatagctctccgttgaggaatctgttcgagtgtcacttgagatggagggctccctccctgaatcttcactgtcgtagcatgtcctgctgtatgactggaactcagcttggggaggcaggtcctgggtggaaactggggtaccctggggatctgcataaagcagcagcaggggctgataatgccccttgatgcatttggtcaccacatccttccatttgggcccaatctccttgacatgagcatcatcaaaatacatccatttgcgaatctttgtttgaaaaaagaatgtagaataatgtttgccatagtaacagatcattccaactaagtacagttcagattgcttggcccggtcatccgtcactctgaaaaacagatcacccagcttaaggcaggttcccaggctgtggataacatcttctgctaagtctgagtggtctgagtcccataccagcccaatcgtgataatctgtggagcattcatcaacacacggcgaatcctgatcctctctccacagttgcttggacagttccgcagatcccccatggtgctggcattctgcagcagctcaccaaacatgcttggtgaaggtttctctcgtctttccagcatacaaatagcctgattgctgtccccagatccaaagctcatagaatccccactcctcctcccactttgctggccagtactgagccaaagggaagtggtggagatataatgtaccatctggatgaaaggcagcggatcagaagtggcaccacagctagtacatacacactgctcaaacaatgtcattgcaaatttctgatgggaaatgcagtgttgggcagtacatatatcctctttggtttcatcagcaatgtggaagtgaattctcatcaggaggttttcaaagcactctgcagcatcatccataattcccagctggaaacgttgttcatcctggaaagtctttgccagagcactgcggagagtgtcagatggaagcactttttcactactacactgaaactggttaaagattcccttgagagcgcaaaagatgcaggaatctcccatgcacttgtgagttgtaagctgcctaaagctacgtcggaagatatccaagtgccacaaaacctgcagggcactgttgaggaagcagctgttttgccctggctcattgctgaggcctttgctgggggctatggaggttgagcttcgaggtgcaaacatcccttgtacactaccacgaccccctgaaaaataatttctcttccaagacattattgttcacatttagcctgaaaaaaaaatggagaaggatttgtgcctttttggcaggaatttctgtctgctaaagttctaaaaggaaagggaatccagaatttagtgaatttattttggaagattttgactttaccaccttccaaatatcatctgtgtagtcaagggactcaggtatcctcctagatcaagatgacagagccctccctcacttgttccaaacaatctccaaaatgtaacatggcacaggactaatgcaaacagagaaatccttaagtattgcttccttctatttttcttgaacagcctccataaagtcctggtgaagtggatgtaattctcaactccaacagcatccaggatcagggtaagatgtgttcttcaggcttgttgataatgcttcttatggactgaagatttttccaactggaaggagaggcagacagagaagcaagaatccaacatgatcctcctcaccctctattgccttgtctcatcatcctctgaagcaaaaactcaaattctgagcaactgcaaaaggttccacaaagccaagaagaagcctgtttgaatcatctgaggtttttgttgatgttcttgctgcttctttttaatgtgccccaaacttctattgtcccatccagatcttcagcaagtctctcctctttcttctgggactagaatagccagctgtgtcagagagagctcctggcgccgcatacttaaccgccgcggctgctatagctacagggagccaaggcaaccagctctcgcgacactttccttggccatggcgagagcacacgagaagagactctcgcaagaaagtaaatgagtcaggctggaaacagcgaagtatatctcgcgatagcactgtttaaaatggcggcttcaaggcgtttcacgggtgtcccggacaggcgtggaggtggggcgcaggcgaggatgaagcttgagttggccaggagtcggaaaacgattgcaggcgggaccgcgtccgtcggggctgaggaaacttagcgtggcagaccctaaactgggataactttagggatatggccttcttttcccagttgcctcaaacttagagcagcgtcgtctttagccgaagattcattttcccagcattttccttctccaggcggagtagttggagacagagggcaagccagaaactgaccttcccatctcctcattcccttccatcaagaacttttcatcgttctttccccaccctggtttgtaaatggtatttggcttcataaaaacgtttgtccacaggtgccctgctccatcagttcgctccagcaatataggaagttaccaaaaaaaaaatttttttttattgaccttggatgcagaaaggaaccgcgttggtgtgtgatttgaattttggacttcttgtttcctgccttgtggccacgtcccccttacttggtgactctcagcacttagttgtggggctttttctctctgctctcagacaactataaaagcagactaattgaacagcatctagaacagaaggtggatgtaaagaacattggtcggccgggcgctgtggctcacgcctgtaatcccagcacttgagaggccgaggcgggcagatcacgaggtcaggagatcgagaccatcctgaccaacattgtgaaaccccgtctctactaaaaata

SEQ ID NO: 10573 - RNA, 2809 nt, Homo sapiens
  source 1..2809: mol_type = other RNA
cggcccgggctgctgctgttcctctcactgctttcatagccagattccattcgctggattagtcgggggtgctgctctaaaaggtgagagcctggccgtgctgggccccagcgcttgtactgggggcttggtccaccaaatttaatgtcgtaagaaggtggcttgcttggttcatctggtataaattctttagctgaatcctcagaaaaggggctaagctgggtatagccacagtgcttccttttgtccttactaaagatactgtcaatattcagagattctcgtttgggtctccatgtgggacgatacttgctggaagaactggattttgactcactgctggtactctctatttcccagtcacgagagtgtaaaggcagggtcctaggaggttttttgtcaggctggtctcctcctctgcccctgcagtgagagcctacattggtctgagaagccagggatggtctgttatggatcatattgctgactgtctctttaaaatctctcagcctgttggtgctgctggatggtttggaggcatttctaggagcctgcttctctttcagtgtttctccttcactgtggtatcccgaggcctggggctcatcgcctttcctcctaacccgaccagagctcctcttgcgctctatcagtgaccctttcttggatgtgtgtttctgattacattcactatcagtcaggtgtcctgtgtcccgactgctctgagacatggaatcattttccacattatagatgactgtcccctgagaatcagaagagaagtgactgaccacagactcatggtgggaatgtttgtagggatagctctccgttgaggaatctgttcgagtgtcacttgagatggagggctccctccctgaatcttcactgtcgtagcatgtcctgctgtatgactggaactcagcttggggaggcaggtcctgggtggaaactggggtaccctggggatctgcataaagcagcagcaggggctgataatgccccttgatgcatttggtcaccacatccttccatttgggcccaatctccttgacatgagcatcatcaaaatacatccatttgcgaatctttgtttgaaaaaagaatgtagaataatgtttgccatagtaacagatcattccaactaagtacagttcagattgcttggcccggtcatccgtcactctgaaaaacagatcacccagcttaaggcaggttcccaggctgtggataacatcttctgctaagtctgagtggtctgagtcccataccagcccaatcgtgataatctgtggagcattcatcaacacacggcgaatcctgatcctctctccacagttgcttggacagttccgcagatcccccatggtgctggcattctgcagcagctcaccaaacatgcttggtgaaggtttctctcgtctttccagcatacaaatagcctgattgctgtccccagatccaaagctcatagaatccccactcctcctcccactttgctggccagtactgagccaaagggaagtggtggagatataatgtaccatctggatgaaaggcagcggatcagaagtggcaccacagctagtacatacacactgctcaaacaatgtcattgcaaatttctgatgggaaatgcagtgttgggcagtacatatatcctctttggtttcatcagcaatgtggaagtgaattctcatcaggaggttttcaaagcactctgcagcatcatccataattcccagctggaaacgttgttcatcctggaaagtctttgccagagcactgcggagagtgtcagatggaagcactttttcactactacactgaaactggttaaagattcccttgagagcgcaaaagatgcaggaatctcccatgcacttgtgagttgtaagctgcctaaagctacgtcggaagatatccaagtgccacaaaacctgcagggcactgttgaggaagcagctgttttgccctggctcattgctgaggcctttgctgggggctatggaggttgagcttcgaggtgcaaacatcccttgtacactaccacgaccccctgaaaaataatttctcttccaagacattattgttcacatttagcctgaaaaaaaaatggagaaggatttgtgcctttttggcaggaatttctgtctgctaaagttctaaaaggaaagggaatccagaatttagtgaatttattttggaagattttgactttaccaccttccaaatatcatctgtgtagtcaagggactcaggtatcctcctagatcaagatgacagagccctccctcacttgttccaaacaatctccaaaatgtaacatggcacaggactaatgcaaacagagaaatccttaagtattgcttccttctatttttcttgaacagcctccataaagtcctggtgaagtggatgtaattctcaactccaacagcatccaggatcagggtaagatgtgttcttcaggcttgttgataatgcttcttatggactgaagatttttccaactggaaggagaggcagacagagaagcaagaatccaacatgatcctcctcaccctctattgccttgtctcatcatcctctgaagcaaaaactcaaattctgagcaactgcaaaaggttccacaaagccaagaagaagcctgtttgaatcatctgaggtttttgttgatgttcttgctgcttctttttaatgtgccccaaacttctattgtcccatccagatcttcagcaagtctctcctctttcttctgggactagaatagccagctgtgtcagagagattctgccttgcataagtt

SEQ ID NO: 10574 - RNA, 3514 nt, Homo sapiens
  source 1..3514: mol_type = other RNA
cggcccgggctgctgctgttcctctcactgctttcatagccagattccattcgctggattagtcgggggtgctgctctaaaaggtgagagcctggccgtgctgggccccagcgcttgtactgggggcttggtccaccaaatttaatgtcgtaagaaggtggcttgcttggttcatctggtataaattctttagctgaatcctcagaaaaggggctaagctgggtatagccacagtgcttccttttgtccttactaaagatactgtcaatattcagagattctcgtttgggtctccatgtgggacgatacttgctggaagaactggattttgactcactgctggtactctctatttcccagtcacgagagtgtaaaggcagggtcctaggaggttttttgtcaggctggtctcctcctctgcccctgcagtgagagcctacattggtctgagaagccagggatggtctgttatggatcatattgctgactgtctctttaaaatctctcagcctgttggtgctgctggatggtttggaggcatttctaggagcctgcttctctttcagtgtttctccttcactgtggtatcccgaggcctggggctcatcgcctttcctcctaacccgaccagagctcctcttgcgctctatcagtgaccctttcttggatgtgtgtttctgattacattcactatcagtcaggtgtcctgtgtcccgactgctctgagacatggaatcattttccacattatagatgactgtcccctgagaatcagaagagaagtgactgaccacagactcatggtgggaatgtttgtagggatagctctccgttgaggaatctgttcgagtgtcacttgagatggagggctccctccctgaatcttcactgtcgtagcatgtcctgctgtatgactggaactcagcttggggaggcaggtcctgggtggaaactggggtaccctggggatctgcataaagcagcagcaggggctgataatgccccttgatgcatttggtcaccacatccttccatttgggcccaatctccttgacatgagcatcatcaaaatacatccatttgcgaatctttgtttgaaaaaagaatgtagaataatgtttgccatagtaacagatcattccaactaagtacagttcagattgcttggcccggtcatccgtcactctgaaaaacagatcacccagcttaaggcaggttcccaggctgtggataacatcttctgctaagtctgagtggtctgagtcccataccagcccaatcgtgataatctgtggagcattcatcaacacacggcgaatcctgatcctctctccacagttgcttggacagttccgcagatcccccatggtgctggcattctgcagcagctcaccaaacatgcttggtgaaggtttctctcgtctttccagcatacaaatagcctgattgctgtccccagatccaaagctcatagaatccccactcctcctcccactttgctggccagtactgagccaaagggaagtggtggagatataatgtaccatctggatgaaaggcagcggatcagaagtggcaccacagctagtacatacacactgctcaaacaatgtcattgcaaatttctgatgggaaatgcagtgttgggcagtacatatatcctctttggtttcatcagcaatgtggaagtgaattctcatcaggaggttttcaaagcactctgcagcatcatccataattcccagctggaaacgttgttcatcctggaaagtctttgccagagcactgcggagagtgtcagatggaagcactttttcactactacactgaaactggttaaagattcccttgagagcgcaaaagatgcaggaatctcccatgcacttgtgagttgtaagctgcctaaagctacgtcggaagatatccaagtgccacaaaacctgcagggcactgttgaggaagcagctgttttgccctggctcattgctgaggcctttgctgggggctatggaggttgagcttcgaggtgcaaacatcccttgtacactaccacgaccccctgaaaaataatttctcttccaagacattattgttcacatttagcctgaaaaaaaaatggagaaggatttgtgcctttttggcaggaatttctgtctgctaaagttctaaaaggaaagggaatccagaatttagtgaatttattttggaagattttgactttaccaccttccaaatatcatctgtgtagtcaagggactcaggtatcctcctagatcaagatgacagagccctccctcacttgttccaaacaatctccaaaatgtaacatggcacaggactaatgcaaacagagaaatccttaagtattgcttccttctatttttcttgaacagcctccataaagtcctggtgaagtggatgtaattctcaactccaacagcatccaggatcagggtaagatgtgttcttcaggcttgttgataatgcttcttatggactgaagatttttccaactggaaggagaggcagacagagaagcaagaatccaacatgatcctcctcaccctctattgccttgtctcatcatcctctgaagcaaaaactcaaattctgagcaactgcaaaaggttccacaaagccaagaagaagcctgtttgaatcatctgaggtttttgttgatgttcttgctgcttctttttaatgtgccccaaacttctattgtcccatccagatcttcagcaagtctctcctctttcttctgggactagaatagccagctgtgtcagagagcaagtgcctgaagtgtcaatcatttcctgcttctcccagctgcaggacttggaactaggaaaacattcagtcagcgtctagagcaggtctggttagaaggatgagctcatccctttcagatgcacacctgatcctcaagaagctgcccctcctccagcaagcagatctttgtatgtttaaagtgacacccacaacctgtacaaccactttgccagagccaaagtaagtctttccttatacatgcctagtgccatggaatcatttcctggtctagccacctcacacagccactgaacgcaggtggcagtggcaacagctgctgctgctgctactatggctttgttagagaaggacttcattttcagctacaacggaggtcaagtccttcaccactgccctggaaacactgcactgtttgtttcaacagccccttgcccacagtcagatcttaccagaatcatgccttctttcaaaactcacaaccatttttctgaaccaacaatgtagcacctcaacatctgccttattccatttgccctgtctaaaagttaaattagccaaggcagctaaatgtactgtatgtatttagagctaaaatgttcccaactcaggtttgccctcagttttactacctctaagaaaacctttattctgccatagcagtctatttattggtaaagtatacagtaatcctaatacagagatatgtaaacttcacttcatg

SEQ ID NO: 10575 - RNA, 4345 nt, Homo sapiens
  source 1..4345: mol_type = other RNA
cggcccgggctgctgctgttcctctcactgctttcatagccagattccattcgctggattagtcgggggtgctgctctaaaaggtgagagcctggccgtgctgggccccagcgcttgtactgggggcttggtccaccaaatttaatgtcgtaagaaggtggcttgcttggttcatctggtataaattctttagctgaatcctcagaaaaggggctaagctgggtatagccacagtgcttccttttgtccttactaaagatactgtcaatattcagagattctcgtttgggtctccatgtgggacgatacttgctggaagaactggattttgactcactgctggtactctctatttcccagtcacgagagtgtaaaggcagggtcctaggaggttttttgtcaggctggtctcctcctctgcccctgcagtgagagcctacattggtctgagaagccagggatggtctgttatggatcatattgctgactgtctctttaaaatctctcagcctgttggtgctgctggatggtttggaggcatttctaggagcctgcttctctttcagtgtttctccttcactgtggtatcccgaggcctggggctcatcgcctttcctcctaacccgaccagagctcctcttgcgctctatcagtgaccctttcttggatgtgtgtttctgattacattcactatcagtcaggtgtcctgtgtcccgactgctctgagacatggaatcattttccacattatagatgactgtcccctgagaatcagaagagaagtgactgaccacagactcatggtgggaatgtttgtagggatagctctccgttgaggaatctgttcgagtgtcacttgagatggagggctccctccctgaatcttcactgtcgtagcatgtcctgctgtatgactggaactcagcttggggaggcaggtcctgggtggaaactggggtaccctggggatctgcataaagcagcagcaggggctgataatgccccttgatgcatttggtcaccacatccttccatttgggcccaatctccttgacatgagcatcatcaaaatacatccatttgcgaatctttgtttgaaaaaagaatgtagaataatgtttgccatagtaacagatcattccaactaagtacagttcagattgcttggcccggtcatccgtcactctgaaaaacagatcacccagcttaaggcaggttcccaggctgtggataacatcttctgctaagtctgagtggtctgagtcccataccagcccaatcgtgataatctgtggagcattcatcaacacacggcgaatcctgatcctctctccacagttgcttggacagttccgcagatcccccatggtgctggcattctgcagcagctcaccaaacatgcttggtgaaggtttctctcgtctttccagcatacaaatagcctgattgctgtccccagatccaaagctcatagaatccccactcctcctcccactttgctggccagtactgagccaaagggaagtggtggagatataatgtaccatctggatgaaaggcagcggatcagaagtggcaccacagctagtacatacacactgctcaaacaatgtcattgcaaatttctgatgggaaatgcagtgttgggcagtacatatatcctctttggtttcatcagcaatgtggaagtgaattctcatcaggaggttttcaaagcactctgcagcatcatccataattcccagctggaaacgttgttcatcctggaaagtctttgccagagcactgcggagagtgtcagatggaagcactttttcactactacactgaaactggttaaagattcccttgagagcgcaaaagatgcaggaatctcccatgcacttgtgagttgtaagctgcctaaagctacgtcggaagatatccaagtgccacaaaacctgcagggcactgttgaggaagcagctgttttgccctggctcattgctgaggcctttgctgggggctatggaggttgagcttcgaggtgcaaacatcccttgtacactaccacgaccccctgaaaaataatttctcttccaagacattattgttcacatttagcctgaaaaaaaaatggagaaggatttgtgcctttttggcaggaatttctgtctgctaaagttctaaaaggaaagggaatccagaatttagtgaatttattttggaagattttgactttaccaccttccaaatatcatctgtgtagtcaagggactcaggtatcctcctagatcaagatgacagagccctccctcacttgttccaaacaatctccaaaatgtaacatggcacaggactaatgcaaacagagaaatccttaagtattgcttccttctatttttcttgaacagcctccataaagtcctggtgaagtggatgtaattctcaactccaacagcatccaggatcagggtaagatgtgttcttcaggcttgttgataatgcttcttatggactgaagatttttccaactggaaggagaggcagacagagaagcaagaatccaacatgatcctcctcaccctctattgccttgtctcatcatcctctgaagcaaaaactcaaattctgagcaactgcaaaaggttccacaaagccaagaagaagcctgtttgaatcatctgaggtttttgttgatgttcttgctgcttctttttaatgtgccccaaacttctattgtcccatccagatcttcagcaagtctctcctctttcttctgggactagaatagccagctgtgtcagagagcagacagcacagtcaacctccagcaaaagacctctaatcacgagggtatctgtggggcaagtgatacaagaatggggagggatatgggaatagctagagctgtggggagggaaggctaggagggaggagacgactgtagctagcaacaatgagaaactgtgaatctaaaccacaaggacttcccgcagaacaggatatcagagagaaggcaattctttttaccaactaccaggaactcagcactgacaattcatgacaaagttaaaaaggtggagcttccaattaaaaacaaagtaaacttaagaaactaaccaaaagtaacttgaaaggacgttatcacaaacttcacctgaggcttaagaaaaacaattatgaagctgtttcctggggcattcctgatgacaaaggtcattaaacaataaggtttgcagggtggctgctgcttccaaagaagggccagtcccccacaaaaaaattcctttgcactgcagtcaaaaggagcacgagaagacaacatttttgtagttgtttacagaataatcaaaacaatgttattgttggaatccctaattcagaattccaagactgggcttaaattaaatcaaatcattttaataggcaaaactcctccaactgtcttaaacgagccacactattaaagaaaattattatttaaactgagccattggaatctactgagtcaattttaaaatgcttgggatctaagggttctcaaccccaaagtccacaacagggaaagatctccacccctctctcggggaagagacctagttacatcaccaagaacaaacagcaggcagagtcccacccccaaacatgtgatcagtcaaccgagaacttgcatttgcaggcagggcacaaaggccccagaggaccaacacacacccttctatgtattacctgaggttataaaacagttttattgaaagaagttgttttataagcatactgatgaaaaaaactcatcagcagaatccttgccaaatatgaaggtctgttgtgtttctataggttgagagaaaatatacgagttgactaaaaaaaagatgtaattaagatttattggtaaaatttaacaaacatgggcaatgtccaaaactaattaagctcttacattttaacaatacagtatattaaattgaagtagtcctttggccacaaggaaagtgccacaaaaaaaaaaaaaaaaaaaaagatactgttgcttttcttgttaaccattagcattctaactcaggtctcctagtggtgctaggtggaggaggaggtagtaatgccatttcaaagtgtgaaacacaaaatttctactgataagtgctgactgcaaataaagacatacaaacatcaagaccaagctcttcaatcaagtcattaaaatataggtatatattcattgtgaaactaatcaaataaaactagagtactgggacagagttacagagcttcaaccctgattacaactagacaacattacttttcatgtctcatccaggtaagggaagtgatccacagggaaatctcactctaatagatt

SEQ ID NO: 10576 - RNA, 2870 nt, Homo sapiens
  source 1..2870: mol_type = other RNA
cggcccgggctgctgctgttcctctcactgctttcatagccagattccattcgctggattagtcgggggtgctgctctaaaaggtgagagcctggccgtgctgggccccagcgcttgtactgggggcttggtccaccaaatttaatgtcgtaagaaggtggcttgcttggttcatctggtataaattctttagctgaatcctcagaaaaggggctaagctgggtatagccacagtgcttccttttgtccttactaaagatactgtcaatattcagagattctcgtttgggtctccatgtgggacgatacttgctggaagaactggattttgactcactgctggtactctctatttcccagtcacgagagtgtaaaggcagggtcctaggaggttttttgtcaggctggtctcctcctctgcccctgcagtgagagcctacattggtctgagaagccagggatggtctgttatggatcatattgctgactgtctctttaaaatctctcagcctgttggtgctgctggatggtttggaggcatttctaggagcctgcttctctttcagtgtttctccttcactgtggtatcccgaggcctggggctcatcgcctttcctcctaacccgaccagagctcctcttgcgctctatcagtgaccctttcttggatgtgtgtttctgattacattcactatcagtcaggtgtcctgtgtcccgactgctctgagacatggaatcattttccacattatagatgactgtcccctgagaatcagaagagaagtgactgaccacagactcatggtgggaatgtttgtagggatagctctccgttgaggaatctgttcgagtgtcacttgagatggagggctccctccctgaatcttcactgtcgtagcatgtcctgctgtatgactggaactcagcttggggaggcaggtcctgggtggaaactggggtaccctggggatctgcataaagcagcagcaggggctgataatgccccttgatgcatttggtcaccacatccttccatttgggcccaatctccttgacatgagcatcatcaaaatacatccatttgcgaatctttgtttgaaaaaagaatgtagaataatgtttgccatagtaacagatcattccaactaagtacagttcagattgcttggcccggtcatccgtcactctgaaaaacagatcacccagcttaaggcaggttcccaggctgtggataacatcttctgctaagtctgagtggtctgagtcccataccagcccaatcgtgataatctgtggagcattcatcaacacacggcgaatcctgatcctctctccacagttgcttggacagttccgcagatcccccatggtgctggcattctgcagcagctcaccaaacatgcttggtgaaggtttctctcgtctttccagcatacaaatagcctgattgctgtccccagatccaaagctcatagaatccccactcctcctcccactttgctggccagtactgagccaaagggaagtggtggagatataatgtaccatctggatgaaaggcagcggatcagaagtggcaccacagctagtacatacacactgctcaaacaatgtcattgcaaatttctgatgggaaatgcagtgttgggcagtacatatatcctctttggtttcatcagcaatgtggaagtgaattctcatcaggaggttttcaaagcactctgcagcatcatccataattcccagctggaaacgttgttcatcctggaaagtctttgccagagcactgcggagagtgtcagatggaagcactttttcactactacactgaaactggttaaagattcccttgagagcgcaaaagatgcaggaatctcccatgcacttgtgagttgtaagctgcctaaagctacgtcggaagatatccaagtgccacaaaacctgcagggcactgttgaggaagcagctgttttgccctggctcattgctgaggcctttgctgggggctatggaggttgagcttcgaggtgcaaacatcccttgtacactaccacgaccccctgaaaaataatttctcttccaagacattattgttcacatttagcctgaaaaaaaaatggagaaggatttgtgcctttttggcaggaatttctgtctgctaaagttctaaaaggaaagggaatccagaatttagtgaatttattttggaagattttgactttaccaccttccaaatatcatctgtgtagtcaagggactcaggtatcctcctagatcaagatgacagagccctccctcacttgttccaaacaatctccaaaatgtaacatggcacaggactaatgcaaacagagaaatccttaagtattgcttccttctatttttcttgaacagcctccataaagtcctggtgaagtggatgtaattctcaactccaacagcatccaggatcagggtaagatgtgttcttcaggcttgttgataatgcttcttatggactgaagatttttccaactggaaggagaggcagacagagaagcaagaatccaacatgatcctcctcaccctctattgccttgtctcatcatcctctgaagcaaaaactcaaattctgagcaactgcaaaaggttccacaaagccaagaagaagcctgtttgaatcatctgaggtttttgttgatgttcttgctgcttctttttaatgtgccccaaacttctattgtcccatccagatcttcagcaagtctctcctctttcttctgggactagaatagccagctgtgtcagagagcctcctcgtcgctgtaccccatttcttcccacttctttcccaatgtagcctggtccctttatccagttccgagtctccgt

SEQ ID NO: 10577 - RNA, 4020 nt, Homo sapiens
  source 1..4020: mol_type = other RNA
cggcccgggctgctgctgttcctctcactgctttcatagccagattccattcgctggattagtcgggggtgctgctctaaaaggtgagagcctggccgtgctgggccccagcgcttgtactgggggcttggtccaccaaatttaatgtcgtaagaaggtggcttgcttggttcatctggtataaattctttagctgaatcctcagaaaaggggctaagctgggtatagccacagtgcttccttttgtccttactaaagatactgtcaatattcagagattctcgtttgggtctccatgtgggacgatacttgctggaagaactggattttgactcactgctggtactctctatttcccagtcacgagagtgtaaaggcagggtcctaggaggttttttgtcaggctggtctcctcctctgcccctgcagtgagagcctacattggtctgagaagccagggatggtctgttatggatcatattgctgactgtctctttaaaatctctcagcctgttggtgctgctggatggtttggaggcatttctaggagcctgcttctctttcagtgtttctccttcactgtggtatcccgaggcctggggctcatcgcctttcctcctaacccgaccagagctcctcttgcgctctatcagtgaccctttcttggatgtgtgtttctgattacattcactatcagtcaggtgtcctgtgtcccgactgctctgagacatggaatcattttccacattatagatgactgtcccctgagaatcagaagagaagtgactgaccacagactcatggtgggaatgtttgtagggatagctctccgttgaggaatctgttcgagtgtcacttgagatggagggctccctccctgaatcttcactgtcgtagcatgtcctgctgtatgactggaactcagcttggggaggcaggtcctgggtggaaactggggtaccctggggatctgcataaagcagcagcaggggctgataatgccccttgatgcatttggtcaccacatccttccatttgggcccaatctccttgacatgagcatcatcaaaatacatccatttgcgaatctttgtttgaaaaaagaatgtagaataatgtttgccatagtaacagatcattccaactaagtacagttcagattgcttggcccggtcatccgtcactctgaaaaacagatcacccagcttaaggcaggttcccaggctgtggataacatcttctgctaagtctgagtggtctgagtcccataccagcccaatcgtgataatctgtggagcattcatcaacacacggcgaatcctgatcctctctccacagttgcttggacagttccgcagatcccccatggtgctggcattctgcagcagctcaccaaacatgcttggtgaaggtttctctcgtctttccagcatacaaatagcctgattgctgtccccagatccaaagctcatagaatccccactcctcctcccactttgctggccagtactgagccaaagggaagtggtggagatataatgtaccatctggatgaaaggcagcggatcagaagtggcaccacagctagtacatacacactgctcaaacaatgtcattgcaaatttctgatgggaaatgcagtgttgggcagtacatatatcctctttggtttcatcagcaatgtggaagtgaattctcatcaggaggttttcaaagcactctgcagcatcatccataattcccagctggaaacgttgttcatcctggaaagtctttgccagagcactgcggagagtgtcagatggaagcactttttcactactacactgaaactggttaaagattcccttgagagcgcaaaagatgcaggaatctcccatgcacttgtgagttgtaagctgcctaaagctacgtcggaagatatccaagtgccacaaaacctgcagggcactgttgaggaagcagctgttttgccctggctcattgctgaggcctttgctgggggctatggaggttgagcttcgaggtgcaaacatcccttgtacactaccacgaccccctgaaaaataatttctcttccaagacattattgttcacatttagcctgaaaaaaaaatggagaaggatttgtgcctttttggcaggaatttctgtctgctaaagttctaaaaggaaagggaatccagaatttagtgaatttattttggaagattttgactttaccaccttccaaatatcatctgtgtagtcaagggactcaggtatcctcctagatcaagatgacagagccctccctcacttgttccaaacaatctccaaaatgtaacatggcacaggactaatgcaaacagagaaatccttaagtattgcttccttctatttttcttgaacagcctccataaagtcctggtgaagtggatgtaattctcaactccaacagcatccaggatcagggtaagatgtgttcttcaggcttgttgataatgcttcttatggactgaagatttttccaactggaaggagaggcagacagagaagcaagaatccaacatgatcctcctcaccctctattgccttgtctcatcatcctctgaagcaaaaactcaaattctgagcaactgcaaaaggttccacaaagccaagaagaagcctgtttgaatcatctgaggtttttgttgatgttcttgctgcttctttttaatgtgccccaaacttctattgtcccatccagatcttcagcaagtctctcctctttcttctgggactagaatagccagctgtgtcagagagctttaacagaaataaaaaaaatcaaaagcttgcgtcacttaatgactctactggctttggactgttctgccaagatcaacgttgcctcacttctcactataaacttgaaaccttggcaaacaatgccaaaaaaaaagaaaaaaagaaaaaaaaaaaaaagagagagacacccaaactaaagagaaggaaaaaaaggtatgaacagctttactttcaggggaaaattctctgaaattttcttgaagcagaagaaagttgatagctcctggcgccgcatacttaaccgccgcggctgctatagctacagggagccaaggcaaccagctctcgcgacactttccttggccatggcgagagcacacgagaagagactctcgcaagaaagtaaatgagtcaggctggaaacagcgaagtatatctcgcgatagcactgtttaaaatggcggcttcaaggcgtttcacgggtgtcccggacaggcgtggaggtggggcgcaggcgaggatgaagcttgagttggccaggagtcggaaaacgattgcaggcgggaccgcgtccgtcggggctgaggaaacttagcgtggcagaccctaaactgggataactttagggatatggccttcttttcccagttgcctcaaacttagagcagcgtcgtctttagccgaagattcattttcccagcattttccttctccaggcggagtagttggagacagagggcaagccagaaactgaccttcccatctcctcattcccttccatcaagaacttttcatcgttctttccccaccctggtttgtaaatggtatttggcttcataaaaacgtttgtccacaggtgccctgctccatcagttcgctccagcaatataggaagttaccaaaaaaaaaatttttttttattgaccttggatgcagaaaggaaccgcgttggtgtgtgatttgaattttggacttcttgtttcctgccttgtggccacgtcccccttacttggtgactctcagcacttagttgtggggctttttctctctgctctcagacaactataaaagcagactaattgaacagcatctagaacagaaggtggatgtaaagaacattggtcggccgggcgctgtggctcacgcctgtaatcccagcacttgagaggccgaggcgggcagatcacgaggtcaggagatcgagaccatcctgaccaacattgtgaaaccccgtctctactaaaaata

SEQ ID NO: 10578 - RNA, 4605 nt, Homo sapiens
  source 1..4605: mol_type = other RNA
cggcccgggctgctgctgttcctctcactgctttcatagccagattccattcgctggattagtcgggggtgctgctctaaaaggtgagagcctggccgtgctgggccccagcgcttgtactgggggcttggtccaccaaatttaatgtcgtaagaaggtggcttgcttggttcatctggtataaattctttagctgaatcctcagaaaaggggctaagctgggtatagccacagtgcttccttttgtccttactaaagatactgtcaatattcagagattctcgtttgggtctccatgtgggacgatacttgctggaagaactggattttgactcactgctggtactctctatttcccagtcacgagagtgtaaaggcagggtcctaggaggttttttgtcaggctggtctcctcctctgcccctgcagtgagagcctacattggtctgagaagccagggatggtctgttatggatcatattgctgactgtctctttaaaatctctcagcctgttggtgctgctggatggtttggaggcatttctaggagcctgcttctctttcagtgtttctccttcactgtggtatcccgaggcctggggctcatcgcctttcctcctaacccgaccagagctcctcttgcgctctatcagtgaccctttcttggatgtgtgtttctgattacattcactatcagtcaggtgtcctgtgtcccgactgctctgagacatggaatcattttccacattatagatgactgtcccctgagaatcagaagagaagtgactgaccacagactcatggtgggaatgtttgtagggatagctctccgttgaggaatctgttcgagtgtcacttgagatggagggctccctccctgaatcttcactgtcgtagcatgtcctgctgtatgactggaactcagcttggggaggcaggtcctgggtggaaactggggtaccctggggatctgcataaagcagcagcaggggctgataatgccccttgatgcatttggtcaccacatccttccatttgggcccaatctccttgacatgagcatcatcaaaatacatccatttgcgaatctttgtttgaaaaaagaatgtagaataatgtttgccatagtaacagatcattccaactaagtacagttcagattgcttggcccggtcatccgtcactctgaaaaacagatcacccagcttaaggcaggttcccaggctgtggataacatcttctgctaagtctgagtggtctgagtcccataccagcccaatcgtgataatctgtggagcattcatcaacacacggcgaatcctgatcctctctccacagttgcttggacagttccgcagatcccccatggtgctggcattctgcagcagctcaccaaacatgcttggtgaaggtttctctcgtctttccagcatacaaatagcctgattgctgtccccagatccaaagctcatagaatccccactcctcctcccactttgctggccagtactgagccaaagggaagtggtggagatataatgtaccatctggatgaaaggcagcggatcagaagtggcaccacagctagtacatacacactgctcaaacaatgtcattgcaaatttctgatgggaaatgcagtgttgggcagtacatatatcctctttggtttcatcagcaatgtggaagtgaattctcatcaggaggttttcaaagcactctgcagcatcatccataattcccagctggaaacgttgttcatcctggaaagtctttgccagagcactgcggagagtgtcagatggaagcactttttcactactacactgaaactggttaaagattcccttgagagcgcaaaagatgcaggaatctcccatgcacttgtgagttgtaagctgcctaaagctacgtcggaagatatccaagtgccacaaaacctgcagggcactgttgaggaagcagctgttttgccctggctcattgctgaggcctttgctgggggctatggaggttgagcttcgaggtgcaaacatcccttgtacactaccacgaccccctgaaaaataatttctcttccaagacattattgttcacatttagcctgaaaaaaaaatggagaaggatttgtgcctttttggcaggaatttctgtctgctaaagttctaaaaggaaagggaatccagaatttagtgaatttattttggaagattttgactttaccaccttccaaatatcatctgtgtagtcaagggactcaggtatcctcctagatcaagatgacagagccctccctcacttgttccaaacaatctccaaaatgtaacatggcacaggactaatgcaaacagagaaatccttaagtattgcttccttctatttttcttgaacagcctccataaagtcctggtgaagtggatgtaattctcaactccaacagcatccaggatcagggtaagatgtgttcttcaggcttgttgataatgcttcttatggactgaagatttttccaactggaaggagaggcagacagagaagcaagaatccaacatgatcctcctcaccctctattgccttgtctcatcatcctctgaagcaaaaactcaaattctgagcaactgcaaaaggttccacaaagccaagaagaagcctgtttgaatcatctgaggtttttgttgatgttcttgctgcttctttttaatgtgccccaaacttctattgtcccatccagatcttcagcaagtctctcctctttcttctgggactagaatagccagctgtgtcagagagctttaacagaaataaaaaaaatcaaaagcttgcgtcacttaatgactctactggctttggactgttctgccaagatcaacgttgcctcacttctcactataaacttgaaaccttggcaaacaatgccaaaaaaaaagaaaaaaagaaaaaaaaaaaaaagagagagacacccaaactaaagagaaggaaaaaaaggtatgaacagctttactttcaggggaaaattctctgaaattttcttgaagcagaagaaagttgatcagacagcacagtcaacctccagcaaaagacctctaatcacgagggtatctgtggggcaagtgatacaagaatggggagggatatgggaatagctagagctgtggggagggaaggctaggagggaggagacgactgtagctagcaacaatgagaaactgtgaatctaaaccacaaggacttcccgcagaacaggatatcagagagaaggcaattctttttaccaactaccaggaactcagcactgacaattcatgacaaagttaaaaaggtggagcttccaattaaaaacaaagtaaacttaagaaactaaccaaaagtaacttgaaaggacgttatcacaaacttcacctgaggcttaagaaaaacaattatgaagctgtttcctggggcattcctgatgacaaaggtcattaaacaataaggtttgcagggtggctgctgcttccaaagaagggccagtcccccacaaaaaaattcctttgcactgcagtcaaaaggagcacgagaagacaacatttttgtagttgtttacagaataatcaaaacaatgttattgttggaatccctaattcagaattccaagactgggcttaaattaaatcaaatcattttaataggcaaaactcctccaactgtcttaaacgagccacactattaaagaaaattattatttaaactgagccattggaatctactgagtcaattttaaaatgcttgggatctaagggttctcaaccccaaagtccacaacagggaaagatctccacccctctctcggggaagagacctagttacatcaccaagaacaaacagcaggcagagtcccacccccaaacatgtgatcagtcaaccgagaacttgcatttgcaggcagggcacaaaggccccagaggaccaacacacacccttctatgtattacctgaggttataaaacagttttattgaaagaagttgttttataagcatactgatgaaaaaaactcatcagcagaatccttgccaaatatgaaggtctgttgtgtttctataggttgagagaaaatatacgagttgactaaaaaaaagatgtaattaagatttattggtaaaatttaacaaacatgggcaatgtccaaaactaattaagctcttacattttaacaatacagtatattaaattgaagtagtcctttggccacaaggaaagtgccacaaaaaaaaaaaaaaaaaaaaagatactgttgcttttcttgttaaccattagcattctaactcaggtctcctagtggtgctaggtggaggaggaggtagtaatgccatttcaaagtgtgaaacacaaaatttctactgataagtgctgactgcaaataaagacatacaaacatcaagaccaagctcttcaatcaagtcattaaaatataggtatatattcattgtgaaactaatcaaataaaactagagtactgggacagagttacagagcttcaaccctgattacaactagacaacattacttttcatgtctcatccaggtaagggaagtgatccacagggaaatctcactctaatagatt

SEQ ID NO: 10579 - RNA, 5353 nt, Homo sapiens
  source 1..5353: mol_type = other RNA
cggcccgggctgctgctgttcctctcactgctttcatagccagattccattcgctggattagtcgggggtgctgctctaaaaggtgagagcctggccgtgctgggccccagcgcttgtactgggggcttggtccaccaaatttaatgtcgtaagaaggtggcttgcttggttcatctggtataaattctttagctgaatcctcagaaaaggggctaagctgggtatagccacagtgcttccttttgtccttactaaagatactgtcaatattcagagattctcgtttgggtctccatgtgggacgatacttgctggaagaactggattttgactcactgctggtactctctatttcccagtcacgagagtgtaaaggcagggtcctaggaggttttttgtcaggctggtctcctcctctgcccctgcagtgagagcctacattggtctgagaagccagggatggtctgttatggatcatattgctgactgtctctttaaaatctctcagcctgttggtgctgctggatggtttggaggcatttctaggagcctgcttctctttcagtgtttctccttcactgtggtatcccgaggcctggggctcatcgcctttcctcctaacccgaccagagctcctcttgcgctctatcagtgaccctttcttggatgtgtgtttctgattacattcactatcagtcaggtgtcctgtgtcccgactgctctgagacatggaatcattttccacattatagatgactgtcccctgagaatcagaagagaagtgactgaccacagactcatggtgggaatgtttgtagggatagctctccgttgaggaatctgttcgagtgtcacttgagatggagggctccctccctgaatcttcactgtcgtagcatgtcctgctgtatgactggaactcagcttggggaggcaggtcctgggtggaaactggggtaccctggggatctgcataaagcagcagcaggggctgataatgccccttgatgcatttggtcaccacatccttccatttgggcccaatctccttgacatgagcatcatcaaaatacatccatttgcgaatctttgtttgaaaaaagaatgtagaataatgtttgccatagtaacagatcattccaactaagtacagttcagattgcttggcccggtcatccgtcactctgaaaaacagatcacccagcttaaggcaggttcccaggctgtggataacatcttctgctaagtctgagtggtctgagtcccataccagcccaatcgtgataatctgtggagcattcatcaacacacggcgaatcctgatcctctctccacagttgcttggacagttccgcagatcccccatggtgctggcattctgcagcagctcaccaaacatgcttggtgaaggtttctctcgtctttccagcatacaaatagcctgattgctgtccccagatccaaagctcatagaatccccactcctcctcccactttgctggccagtactgagccaaagggaagtggtggagatataatgtaccatctggatgaaaggcagcggatcagaagtggcaccacagctagtacatacacactgctcaaacaatgtcattgcaaatttctgatgggaaatgcagtgttgggcagtacatatatcctctttggtttcatcagcaatgtggaagtgaattctcatcaggaggttttcaaagcactctgcagcatcatccataattcccagctggaaacgttgttcatcctggaaagtctttgccagagcactgcggagagtgtcagatggaagcactttttcactactacactgaaactggttaaagattcccttgagagcgcaaaagatgcaggaatctcccatgcacttgtgagttgtaagctgcctaaagctacgtcggaagatatccaagtgccacaaaacctgcagggcactgttgaggaagcagctgttttgccctggctcattgctgaggcctttgctgggggctatggaggttgagcttcgaggtgcaaacatcccttgtacactaccacgaccccctgaaaaataatttctcttccaagacattattgttcacatttagcctgaaaaaaaaatggagaaggatttgtgcctttttggcaggaatttctgtctgctaaagttctaaaaggaaagggaatccagaatttagtgaatttattttggaagattttgactttaccaccttccaaatatcatctgtgtagtcaagggactcaggtatcctcctagatcaagatgacagagccctccctcacttgttccaaacaatctccaaaatgtaacatggcacaggactaatgcaaacagagaaatccttaagtattgcttccttctatttttcttgaacagcctccataaagtcctggtgaagtggatgtaattctcaactccaacagcatccaggatcagggtaagatgtgttcttcaggcttgttgataatgcttcttatggactgaagatttttccaactggaaggagaggcagacagagaagcaagaatccaacatgatcctcctcaccctctattgccttgtctcatcatcctctgaagcaaaaactcaaattctgagcaactgcaaaaggttccacaaagccaagaagaagcctgtttgaatcatctgaggtttttgttgatgttcttgctgcttctttttaatgtgccccaaacttctattgtcccatccagatcttcagcaagtctctcctctttcttctgggactagaatagccagctgtgtcagagagctttaacagaaataaaaaaaatcaaaagcttgcgtcacttaatgactctactggctttggactgttctgccaagatcaacgttgcctcacttctcactataaacttgaaaccttggcaaacaatgccaaaaaaaaagaaaaaaagaaaaaaaaaaaaaagagagagacacccaaactaaagagaaggaaaaaaaggtatgaacagctttactttcaggggaaaattctctgaaattttcttgaagcagaagaaagttgatctggatagaaataaaaacaaaatacaaactttccagtatcaggctaacacaaaacaaatcaccaagtaagcacacacaaactaggaactgaaagttccttttggacattgtgaataaagcactttttaaaaggtgttttccatgaatatgcttatgaaaacgtgcttaaaggtgggaaggccatgttagcagtctaagatctgttctgagtaaagatgttccatccagagaaacactgatggcgagtaaaccacatgtccttaacatgcagtccaagagaactaaatcttctcctgccctgtttgtttgtttgtttcatttttgccagaggatcagagagataatttgggttacaaatcatttaatctccagattatatccaagggctcacaatcagaggcaatccattgaccaactttagttttcaactaattaaaatgccagtgaggcaacagagagtaataccaaagcaagtatgttccctggaaggaaatcaccacatctccagctttaagttttcctataaggctgccatgtccatctacataaggaaaaatttttaaatgttaagtgttaaatttgccaacatcaacaattcctcattctcccttccttctcaccatcatatgcaccatctaaaaacacaaaaatgctttaacatcttaatcattctctgggagatcacctagcattgtctacagcatgtccaatggaaaaactgaggtacaggaatattaaatggttgcataagactgttctttcccttctgtaaattcccagactatttataatctacatgtcccaattaaagtatttgattatacagcctactgtcacattattctctatttttattactctctgttttatatcgtatccgtcataatatgactacatgaaatgaaatagtagctacagtcaggtatgtgctaaacacgatacttatgtcctttatttaatattcacaacagtcctatcagatagctattaatagttccattttacagaaaagtaaagagaggcttaaagacattaacttgcccaattcaacactggtaagtggcagatctagaaatgtttgactattaaacaatgacttaattatatattttattattctattccaaaagctcctattacagtgccagtcataagaaggcagtcaataaatactgcctgatgattaacatgacactagaaaagaacccatatctcccacacagactataagaccctcacctttctacacacaccctcatacacaccccactcaaggccactaagcaacttccaacaagccatgcagcattccttcagctcaactgctgcaaaggaatgacaagtaccaagcctccactttgctcacagccaaaaggacttggcaggcaggtggggtttccaatatccacattaggagctaactgaaactcagcctgccctatgacacacactcctgagtacagggagcaaaaggagaaaaacgcagtagcagagaaaagattctcaggctctgaatggcagtattatgtagggtaaagcagtaagttctcagacctgttctagatgtgtcaccaactagaagtgagagcataaaggaccagacaagagaggcagtaacaagtggtccagagaaatactaacaccaaaaacatttcacttaaattgtagatatagcattaaacaatgtaatccttctccaataccatttactgaagatatgtgaggaggggaattatagttttatctgtatggctctcactacctagttttgttttttgggttttgttttgttttgttttgttttgtttctgaggcagaatctcactgtcacccaggctggagtgcagtcgcgcaatattggctcactgcagcctccgcctcttaggttcaagcaatcctcctgcctcagcctcccgagtagctgggattacaggcatgtgccactatgcctggctaatttttgtatttttagtagagacgggatttcaccaggggctggtctcaaacccctgacttcaggtgatccacctgccttgacttcccaaatgctgggattacaggcatgagccaccgcacccagccagtcaattgatttttgatgaaagtaccaaggccatttaattgagaaatgacagtcttttcaacaaatgatgttggaacaattgggacacccatatgcaaaaaactgaacattgagtcataccttacatcttatacaaaaataattcaatacatcacagtcctaaacaaaaaacctaaaactataaattctaggagaagacaggagaaaattttataacctt

SEQ ID NO: 10580 - RNA, 3638 nt, Homo sapiens
  source 1..3638: mol_type = other RNA
cggcccgggctgctgctgttcctctcactgctttcatagccagattccattcgctggattagtcgggggtgctgctctaaaaggtgagagcctggccgtgctgggccccagcgcttgtactgggggcttggtccaccaaatttaatgtcgtaagaaggtggcttgcttggttcatctggtataaattctttagctgaatcctcagaaaaggggctaagctgggtatagccacagtgcttccttttgtccttactaaagatactgtcaatattcagagattctcgtttgggtctccatgtgggacgatacttgctggaagaactggattttgactcactgctggtactctctatttcccagtcacgagagtgtaaaggcagggtcctaggaggttttttgtcaggctggtctcctcctctgcccctgcagtgagagcctacattggtctgagaagccagggatggtctgttatggatcatattgctgactgtctctttaaaatctctcagcctgttggtgctgctggatggtttggaggcatttctaggagcctgcttctctttcagtgtttctccttcactgtggtatcccgaggcctggggctcatcgcctttcctcctaacccgaccagagctcctcttgcgctctatcagtgaccctttcttggatgtgtgtttctgattacattcactatcagtcaggtgtcctgtgtcccgactgctctgagacatggaatcattttccacattatagatgactgtcccctgagaatcagaagagaagtgactgaccacagactcatggtgggaatgtttgtagggatagctctccgttgaggaatctgttcgagtgtcacttgagatggagggctccctccctgaatcttcactgtcgtagcatgtcctgctgtatgactggaactcagcttggggaggcaggtcctgggtggaaactggggtaccctggggatctgcataaagcagcagcaggggctgataatgccccttgatgcatttggtcaccacatccttccatttgggcccaatctccttgacatgagcatcatcaaaatacatccatttgcgaatctttgtttgaaaaaagaatgtagaataatgtttgccatagtaacagatcattccaactaagtacagttcagattgcttggcccggtcatccgtcactctgaaaaacagatcacccagcttaaggcaggttcccaggctgtggataacatcttctgctaagtctgagtggtctgagtcccataccagcccaatcgtgataatctgtggagcattcatcaacacacggcgaatcctgatcctctctccacagttgcttggacagttccgcagatcccccatggtgctggcattctgcagcagctcaccaaacatgcttggtgaaggtttctctcgtctttccagcatacaaatagcctgattgctgtccccagatccaaagctcatagaatccccactcctcctcccactttgctggccagtactgagccaaagggaagtggtggagatataatgtaccatctggatgaaaggcagcggatcagaagtggcaccacagctagtacatacacactgctcaaacaatgtcattgcaaatttctgatgggaaatgcagtgttgggcagtacatatatcctctttggtttcatcagcaatgtggaagtgaattctcatcaggaggttttcaaagcactctgcagcatcatccataattcccagctggaaacgttgttcatcctggaaagtctttgccagagcactgcggagagtgtcagatggaagcactttttcactactacactgaaactggttaaagattcccttgagagcgcaaaagatgcaggaatctcccatgcacttgtgagttgtaagctgcctaaagctacgtcggaagatatccaagtgccacaaaacctgcagggcactgttgaggaagcagctgttttgccctggctcattgctgaggcctttgctgggggctatggaggttgagcttcgaggtgcaaacatcccttgtacactaccacgaccccctgaaaaataatttctcttccaagacattattgttcacatttagccttccaaatatcatctgtgtagtcaagggactcaggtatcctcctagatcaagatgacagagccctccctcacttgttccaaacaatctccaaaatgtaacatggcacaggactaatgcaaacagagaaatccttaagtattgcttccttctatttttcttgaacagcctccataaagtcctggtgaagtggatgtaattctcaactccaacagcatccaggatcagggtaagatgtgttcttcaggcttgttgataatgcttcttatggactgaagatttttccaactggaaggagaggcagacagagaagcaagaatccaacatgatcctcctcaccctctattgccttgtctcatcatcctctgaagcaaaaactcaaattctgagcaactgcaaaaggttccacaaagccaagaagaagcctgtttgaatcatctgaggtttttgttgatgttcttgctgcttctttttaatgtgccccaaacttctattgtcccatccagatcttcagcaagtctctcctctttcttctgggactagaatagccagctgtgtcagagagagctcctggcgccgcatacttaaccgccgcggctgctatagctacagggagccaaggcaaccagctctcgcgacactttccttggccatggcgagagcacacgagaagagactctcgcaagaaagtaaatgagtcaggctggaaacagcgaagtatatctcgcgatagcactgtttaaaatggcggcttcaaggcgtttcacgggtgtcccggacaggcgtggaggtggggcgcaggcgaggatgaagcttgagttggccaggagtcggaaaacgattgcaggcgggaccgcgtccgtcggggctgaggaaacttagcgtggcagaccctaaactgggataactttagggatatggccttcttttcccagttgcctcaaacttagagcagcgtcgtctttagccgaagattcattttcccagcattttccttctccaggcggagtagttggagacagagggcaagccagaaactgaccttcccatctcctcattcccttccatcaagaacttttcatcgttctttccccaccctggtttgtaaatggtatttggcttcataaaaacgtttgtccacaggtgccctgctccatcagttcgctccagcaatataggaagttaccaaaaaaaaaatttttttttattgaccttggatgcagaaaggaaccgcgttggtgtgtgatttgaattttggacttcttgtttcctgccttgtggccacgtcccccttacttggtgactctcagcacttagttgtggggctttttctctctgctctcagacaactataaaagcagactaattgaacagcatctagaacagaaggtggatgtaaagaacattggtcggccgggcgctgtggctcacgcctgtaatcccagcacttgagaggccgaggcgggcagatcacgaggtcaggagatcgagaccatcctgaccaacattgtgaaaccccgtctctactaaaaata

SEQ ID NO: 10581 - RNA, 2733 nt, Homo sapiens
  source 1..2733: mol_type = other RNA
cggcccgggctgctgctgttcctctcactgctttcatagccagattccattcgctggattagtcgggggtgctgctctaaaaggtgagagcctggccgtgctgggccccagcgcttgtactgggggcttggtccaccaaatttaatgtcgtaagaaggtggcttgcttggttcatctggtataaattctttagctgaatcctcagaaaaggggctaagctgggtatagccacagtgcttccttttgtccttactaaagatactgtcaatattcagagattctcgtttgggtctccatgtgggacgatacttgctggaagaactggattttgactcactgctggtactctctatttcccagtcacgagagtgtaaaggcagggtcctaggaggttttttgtcaggctggtctcctcctctgcccctgcagtgagagcctacattggtctgagaagccagggatggtctgttatggatcatattgctgactgtctctttaaaatctctcagcctgttggtgctgctggatggtttggaggcatttctaggagcctgcttctctttcagtgtttctccttcactgtggtatcccgaggcctggggctcatcgcctttcctcctaacccgaccagagctcctcttgcgctctatcagtgaccctttcttggatgtgtgtttctgattacattcactatcagtcaggtgtcctgtgtcccgactgctctgagacatggaatcattttccacattatagatgactgtcccctgagaatcagaagagaagtgactgaccacagactcatggtgggaatgtttgtagggatagctctccgttgaggaatctgttcgagtgtcacttgagatggagggctccctccctgaatcttcactgtcgtagcatgtcctgctgtatgactggaactcagcttggggaggcaggtcctgggtggaaactggggtaccctggggatctgcataaagcagcagcaggggctgataatgccccttgatgcatttggtcaccacatccttccatttgggcccaatctccttgacatgagcatcatcaaaatacatccatttgcgaatctttgtttgaaaaaagaatgtagaataatgtttgccatagtaacagatcattccaactaagtacagttcagattgcttggcccggtcatccgtcactctgaaaaacagatcacccagcttaaggcaggttcccaggctgtggataacatcttctgctaagtctgagtggtctgagtcccataccagcccaatcgtgataatctgtggagcattcatcaacacacggcgaatcctgatcctctctccacagttgcttggacagttccgcagatcccccatggtgctggcattctgcagcagctcaccaaacatgcttggtgaaggtttctctcgtctttccagcatacaaatagcctgattgctgtccccagatccaaagctcatagaatccccactcctcctcccactttgctggccagtactgagccaaagggaagtggtggagatataatgtaccatctggatgaaaggcagcggatcagaagtggcaccacagctagtacatacacactgctcaaacaatgtcattgcaaatttctgatgggaaatgcagtgttgggcagtacatatatcctctttggtttcatcagcaatgtggaagtgaattctcatcaggaggttttcaaagcactctgcagcatcatccataattcccagctggaaacgttgttcatcctggaaagtctttgccagagcactgcggagagtgtcagatggaagcactttttcactactacactgaaactggttaaagattcccttgagagcgcaaaagatgcaggaatctcccatgcacttgtgagttgtaagctgcctaaagctacgtcggaagatatccaagtgccacaaaacctgcagggcactgttgaggaagcagctgttttgccctggctcattgctgaggcctttgctgggggctatggaggttgagcttcgaggtgcaaacatcccttgtacactaccacgaccccctgaaaaataatttctcttccaagacattattgttcacatttagccttccaaatatcatctgtgtagtcaagggactcaggtatcctcctagatcaagatgacagagccctccctcacttgttccaaacaatctccaaaatgtaacatggcacaggactaatgcaaacagagaaatccttaagtattgcttccttctatttttcttgaacagcctccataaagtcctggtgaagtggatgtaattctcaactccaacagcatccaggatcagggtaagatgtgttcttcaggcttgttgataatgcttcttatggactgaagatttttccaactggaaggagaggcagacagagaagcaagaatccaacatgatcctcctcaccctctattgccttgtctcatcatcctctgaagcaaaaactcaaattctgagcaactgcaaaaggttccacaaagccaagaagaagcctgtttgaatcatctgaggtttttgttgatgttcttgctgcttctttttaatgtgccccaaacttctattgtcccatccagatcttcagcaagtctctcctctttcttctgggactagaatagccagctgtgtcagagagcagacagcacagtcaacctccagcaaaagacctctaatcacgagggtatctgtggggcaagtgat

SEQ ID NO: 10582 - RNA, 4726 nt, Homo sapiens
  source 1..4726: mol_type = other RNA
cggcccgggctgctgctgttcctctcactgctttcatagccagattccattcgctggattagtcgggggtgctgctctaaaaggtgagagcctggccgtgctgggccccagcgcttgtactgggggcttggtccaccaaatttaatgtcgtaagaaggtggcttgcttggttcatctggtataaattctttagctgaatcctcagaaaaggggctaagctgggtatagccacagtgcttccttttgtccttactaaagatactgtcaatattcagagattctcgtttgggtctccatgtgggacgatacttgctggaagaactggattttgactcactgctggtactctctatttcccagtcacgagagtgtaaaggcagggtcctaggaggttttttgtcaggctggtctcctcctctgcccctgcagtgagagcctacattggtctgagaagccagggatggtctgttatggatcatattgctgactgtctctttaaaatctctcagcctgttggtgctgctggatggtttggaggcatttctaggagcctgcttctctttcagtgtttctccttcactgtggtatcccgaggcctggggctcatcgcctttcctcctaacccgaccagagctcctcttgcgctctatcagtgaccctttcttggatgtgtgtttctgattacattcactatcagtcaggtgtcctgtgtcccgactgctctgagacatggaatcattttccacattatagatgactgtcccctgagaatcagaagagaagtgactgaccacagactcatggtgggaatgtttgtagggatagctctccgttgaggaatctgttcgagtgtcacttgagatggagggctccctccctgaatcttcactgtcgtagcatgtcctgctgtatgactggaactcagcttggggaggcaggtcctgggtggaaactggggtaccctggggatctgcataaagcagcagcaggggctgataatgccccttgatgcatttggtcaccacatccttccatttgggcccaatctccttgacatgagcatcatcaaaatacatccatttgcgaatctttgtttgaaaaaagaatgtagaataatgtttgccatagtaacagatcattccaactaagtacagttcagattgcttggcccggtcatccgtcactctgaaaaacagatcacccagcttaaggcaggttcccaggctgtggataacatcttctgctaagtctgagtggtctgagtcccataccagcccaatcgtgataatctgtggagcattcatcaacacacggcgaatcctgatcctctctccacagttgcttggacagttccgcagatcccccatggtgctggcattctgcagcagctcaccaaacatgcttggtgaaggtttctctcgtctttccagcatacaaatagcctgattgctgtccccagatccaaagctcatagaatccccactcctcctcccactttgctggccagtactgagccaaagggaagtggtggagatataatgtaccatctggatgaaaggcagcggatcagaagtggcaccacagctagtacatacacactgctcaaacaatgtcattgcaaatttctgatgggaaatgcagtgttgggcagtacatatatcctctttggtttcatcagcaatgtggaagtgaattctcatcaggaggttttcaaagcactctgcagcatcatccataattcccagctggaaacgttgttcatcctggaaagtctttgccagagcactgcggagagtgtcagatggaagcactttttcactactacactgaaactggttaaagattcccttgagagcgcaaaagatgcaggaatctcccatgcacttgtgagttgtaagctgcctaaagctacgtcggaagatatccaagtgccacaaaacctgcagggcactgttgaggaagcagctgttttgccctggctcattgctgaggcctttgctgggggctatggaggttgagcttcgaggtgcaaacatcccttgtacactaccacgaccccctgaaaaataatttctcttccaagacattattgttcacatttagccttccaaatatcatctgtgtagtcaagggactcaggtatcctcctagatcaagatgacagagccctccctcacttgttccaaacaatctccaaaatgtaacatggcacaggactaatgcaaacagagaaatccttaagtattgcttccttctatttttcttgaacagcctccataaagtcctggtgaagtggatgtaattctcaactccaacagcatccaggatcagggtaagatgtgttcttcaggcttgttgataatgcttcttatggactgaagatttttccaactggaaggagaggcagacagagaagcaagaatccaacatgatcctcctcaccctctattgccttgtctcatcatcctctgaagcaaaaactcaaattctgagcaactgcaaaaggttccacaaagccaagaagaagcctgtttgaatcatctgaggtttttgttgatgttcttgctgcttctttttaatgtgccccaaacttctattgtcccatccagatcttcagcaagtctctcctctttcttctgggactagaatagccagctgtgtcagagagctttaacagaaataaaaaaaatcaaaagcttgcgtcacttaatgactctactggctttggactgttctgccaagatcaacgttgcctcacttctcactataaacttgaaaccttggcaaacaatgccaaaaaaaaagaaaaaaagaaaaaaaaaaaaaagagagagacacccaaactaaagagaaggaaaaaaaggtatgaacagctttactttcaggggaaaattctctgaaattttcttgaagcagaagaaagttgatctggatagaaataaaaacaaaatacaaactttccagtatcaggctaacacaaaacaaatcaccaagtaagcacacacaaactaggaactgaaagttccttttggacattgtgaataaagcactttttaaaaggtgttttccatgaatatgcttatgaaaacgtgcttaaaggtgggaaggccatgttagcagtctaagatctgttctgagtaaagatgttccatccagagaaacactgatggcgagtaaaccacatgtccttaacatgcagtccaagagaactaaatcttctcctgccctgtttgtttgtttgtttcatttttgccagaggatcagagagataatttgggttacaaatcatttaatctccagattatatccaagggctcacaatcagaggcaatccattgaccaactttagttttcaactaattaaaatgccagtgaggcaacagagagtaataccaaagcaagtatgttccctggaaggaaatcaccacatctccagctttaagttttcctataaggctgccatgtccatctacataaggaaaaatttttaaatgttaagtgttaaatttgccaacatcaacaattcctcattctcccttccttctcaccatcatatgcaccatctaaaaacacaaaaatgctttaacatcttaatcattctctgggagatcacctagcattgtctacagcatgtccaatggaaaaactgaggtacaggaatattaaatggttgcataagactgttctttcccttctgtaaattcccagactatttataatctacatgtcccaattaaagtatttgattatacagcctactgtcacattattctctatttttattactctctgttttatatcgtatccgtcataatatgactacatgaaatgaaatagtagctacagtcaggtatgtgctaaacacgatacttatgtcctttatttaatattcacaacagtcctatcagatagctattaatagttccattttacagaaaagtaaagagaggcttaaagacattaacttgcccaattcaacactggtaagtggcagatctagaaatgtttgactattaaacaatgacttaattatatattttattattctattccaaaagctcctattacagtgccagtcataagaaggcagtcaataaatactgcctgatgattaacatgacactagaaaagaacccatatctcccacacagactataagaccctcacctttctacacacaccctcatacacaccccactcaaggccactaagcaacttccaacaagccatgcagcattccttcagctcaactgctgcaaaggaatgacaagtaccaagcctccactttgctcacagccaaaaggacttggcaggcaggtggggtttccaatatccacattaggagctaactgaaactcagcctgccctatgacacacactcctgagtacagggagcaaaaggagaaaaacgcagtagcagagaaaagattctcaggctctgaatggcagtattatgtagggtaaagcagtaagttctcagacctgttctagatgtgtcaccaactagaagtgagagcataaaggaccagacaagagaggcagtaacaagtggtccagagaaatactaacaccaaaaacatttcacttaaattgtagatatagcattaaacaatgtaatccttctccaataccatttactgaagatatgtgaggaggggaattatagttttatctgtatggctctcactacctagttttgttttttgggttttgttttgttttgttt

SEQ ID NO: 10583 - RNA, 1683 nt, Homo sapiens
  source 1..1683: mol_type = other RNA
cggcccgggctgctgctgttcctcttcaaagtccaccaggtcccattcatattccagtctggcttgtcgttgtttccaaaactccaaaaataaggtgacccaaattcccatgaatattgcaaagaacactgttgactcattatcaaacaaatgggagaactttgaagccaaacacgtactatttagtctccaataatcacacacttgatcacagagtgggcacatgatcatctgaccaccaatctcagggtcacagatttcagtgctgcttgtgttatgttccattgataataagccataaataaaacaagctaagccaactacagctgcaaagaatagcatttctgtgtaaaatccaagaaagacaaaatagataccaattttttctccataataattcttaatcaagtctaaaggctgctccttgtagaaataggaaaatcgagcccaattctggtgaagtgtgtatctttcattggtaggattgggaggttctgatggcttccaatattggccatcatggagtggataggcagatgagtaagtgttagagtttagcagtctttcaatcccaaaccttttcttcccatcttctatgccaaaaggacatcttgagagaatatagtacacaattctgtttcttgatgaggatggaaagaaggttgcctgatcttcgatgaggaagagctcctgccgatgtctgctgaattgtgcagtaaaatattcaggatggggatacttcacactcagtgggagtcttacaggtccaagcacatagcttataggagtgtgcttagggcggggaatatcactctccttaataggcattttgattcccaagacttcagcataggtaactaatacctcccaaggggcatggatcttgacaaaataagttcttccatcttccgagtcccttttgtcttctatttccaactcaagacctgtttttctgagattagtttcaaactcttttcttctttccgcctttaactctgcgtctttctttacatcatcaacgtaggaaagcacaaaatcaatttgcctaatcccatctcggaagaagatagaatctttgctttgctgatttttttgaaacataagccgccgcctcaggaacaaattgaatcgctttgcaggcattgtttcttcattgatgagaaagctggtctctctgctgctcaggctctcactcatttggaaagagtagtctatatgcttattgactttttccccttcctccgccaacacttccaggagatccgggtcgcccatcttcgccagctcgttaatggcactggtgcctgagaggcagcaggagaggggcagctgagacagacgtggagatctgaggcaggtgctgaatctgactgtgggccgccggagttgctgctgctggacttctaagggcctgctcttccttctgcaggcctccttctcctcctcctcggactccaccgtctctgggcgccacagccagccggccttcctctccggcgggtacttccactcgacccggtcccccacaacctgcttcgcgcgcttggccctgcgcttccccaccctcagccggtagcgctcctgggcgctctcccagtacttctccaggcacctgtccctgtgcctgctcggcagctgatcccgcagccgccactcctcccggtgctcgccaggatcctttcc

SEQ ID NO: 10584 - RNA, 1480 nt, Homo sapiens
  source 1..1480: mol_type = other RNA
cggcccgggctgctgctgttcctcttcaaagtccaccaggtcccattcatattccagtctggcttgtcgttgtttccaaaactccaaaaataaggtgacccaaattcccatgaatattgcaaagaacactgttgactcattatcaaacaaatgggagaactttgaagccaaacacgtactatttagtctccaataatcacacacttgatcacagagtgggcacatgatcatctgaccaccaatctcagggtcacagatttcagtgctgcttgtgttatgttccattgataataagccataaataaaacaagctaagccaactacagctgcaaagaatagcatttctgtgtaaaatccaagaaagacaaaatagataccaattttttctccataataattcttaatcaagtctaaaggctgctccttgtagaaataggaaaatcgagcccaattctggtgaagtgtgtatctttcattggtaggattgggaggttctgatggcttccaatattggccatcatggagtggataggcagatgagtaagtgttagagtttagcagtctttcaatcccaaaccttttcttcccatcttctatgccaaaaggacatcttgagagaatatagtacacaattctgtttcttgatgaggatggaaagaaggttgcctgatcttcgatgaggaagagctcctgccgatgtctgctgaattgtgcagtaaaatattcaggatggggatacttcacactcagtgggagtcttacaggtccaagcacatagcttataggagtgtgcttagggcggggaatatcactctccttaataggcattttgattcccaagacttcagcataggtaactaatacctcccaaggggcatggatcttgacaaaataagttcttccatcttccgagtcccttttgtcttctatttccaactcaagacctgtttttctgagattagtttcaaactcttttcttctttccgcctttaactctgcgtctttctttacatcatcaacgtaggaaagcacaaaatcaatttgcctaatcccatctcggaagaagatagaatctttgctttgctgatttttttgaaacataagccgccgcctcaggaacaaattgaatcgctttgcaggcattgtttcttcattgatgagaaagctggtctctctgctgctcaggctctgctcactcatttggaaagagtagtctatatgcttattgactttttcccctcctgtcggaatcctcctcctccgatccccaaagggggtcccgatgctccctcagccggttggccgggtcttcatcgatccgctcatgcgtgccactcggagagaacccctctcccagttgggagttacttttggtctcgtggggaaaagtccctctcccttaaaggaacccctcccttttaaggccggctcatggcccgagactccaaggtgccagcagccccttccccatagcgtctgg

SEQ ID NO: 10585 - RNA, 1686 nt, Homo sapiens
  source 1..1686: mol_type = other RNA
cggcccgggctgctgctgttcctcttcaaagtccaccaggtcccattcatattccagtctggcttgtcgttgtttccaaaactccaaaaataaggtgacccaaattcccatgaatattgcaaagaacactgttgactcattatcaaacaaatgggagaactttgaagccaaacacgtactatttagtctccaataatcacacacttgatcacagagtgggcacatgatcatctgaccaccaatctcagggtcacagatttcagtgctgcttgtgttatgttccattgataataagccataaataaaacaagctaagccaactacagctgcaaagaatagcatttctgtgtaaaatccaagaaagacaaaatagataccaattttttctccataataattcttaatcaagtctaaaggctgctccttgtagaaataggaaaatcgagcccaattctggtgaagtgtgtatctttcattggtaggattgggaggttctgatggcttccaatattggccatcatggagtggataggcagatgagtaagtgttagagtttagcagtctttcaatcccaaaccttttcttcccatcttctatgccaaaaggacatcttgagagaatatagtacacaattctgtttcttgatgaggatggaaagaaggttgcctgatcttcgatgaggaagagctcctgccgatgtctgctgaattgtgcagtaaaatattcaggatggggatacttcacactcagtgggagtcttacaggtccaagcacatagcttataggagtgtgcttagggcggggaatatcactctccttaataggcattttgattcccaagacttcagcataggtaactaatacctcccaaggggcatggatcttgacaaaataagttcttccatcttccgagtcccttttgtcttctatttccaactcaagacctgtttttctgagattagtttcaaactcttttcttctttccgcctttaactctgcgtctttctttacatcatcaacgtaggaaagcacaaaatcaatttgcctaatcccatctcggaagaagatagaatctttgctttgctgatttttttgaaacataagccgccgcctcaggaacaaattgaatcgctttgcaggcattgtttcttcattgatgagaaagctggtctctctgctgctcaggctctgctcactcatttggaaagagtagtctatatgcttattgactttttccccttcctccgccaacacttccaggagatccgggtcgcccatcttcgccagctcgttaatggcactggtgcctgagaggcagcaggagaggggcagctgagacagacgtggagatctgaggcaggtgctgaatctgactgtgggccgccggagttgctgctgctggacttctaagggcctgctcttccttctgcaggcctccttctcctcctcctcggactccaccgtctctgggcgccacagccagccggccttcctctccggcgggtacttccactcgacccggtcccccacaacctgcttcgcgcgcttggccctgcgcttccccaccctcagccggtagcgctcctgggcgctctcccagtacttctccaggcacctgtccctgtgcctgctcggcagctgatcccgcagccgccactcctcccggtgctcgccaggatcctttcc

SEQ ID NO: 10586 - RNA, 1696 nt, Homo sapiens
  source 1..1696: mol_type = other RNA
cggcccgggctgctgctgttcctcttcaaagtccaccaggtcccattcatattccagtctggcttgtcgttgtttccaaaactccaaaaataaggtgacccaaattcccatgaatattgcaaagaacactgttgactcattatcaaacaaatgggagaactttgaagccaaacacgtactatttagtctccaataatcacacacttgatcacagagtgggcacatgatcatctgaccaccaatctcagggtcacagatttcagtgctgcttgtgttatgttccattgataataagccataaataaaacaagctaagccaactacagctgcaaagaatagcatttctgtgtaaaatccaagaaagacaaaatagataccaattttttctccataataattcttaatcaagtctaaaggctgctccttgtagaaataggaaaatcgagcccaattctggtgaagtgtgtatctttcattggtaggattgggaggttctgatggcttccaatattggccatcatggagtggataggcagatgagtaagtgttagagtttagcagtctttcaatcccaaaccttttcttcccatcttctatgccaaaaggacatcttgagagaatatagtacacaattctgtttcttgatgaggatggaaagaaggttgcctgatcttcgatgaggaagagctcctgccgatgtctgctgaattgtgcagtaaaatattcaggatggggatacttcacactcagtgggagtcttacaggtccaagcacatagcttataggagtgtgcttagggcggggaatatcactctccttaataggcattttgattcccaagacttcagcataggtaactaatacctcccaaggggcatggatcttgacaaaataagttcttccatcttccgagtcccttttgtcttctatttccaactcaagacctgtttttctgagattagtttcaaactcttttcttctttccgcctttaactctgcgtctttctttacatcatcaacgtaggaaagcacaaaatcaatttgcctaatcccatctcggaagaagatagaatctttgctttgctgatttttttgaaacattgtttcttcattgatgagaaagctggtctctctgctgctcaggctctcactcatttggaaagagtagtctatatgcttattgactttttccccttcctccgccaacacttccaggagatccgggtcgcccatcttcgccagctcgttaatggcactggtgcctgagaggcagcaggagaggggcagctgagacagacgtggagatctgaggcaggtgctgaatctgactgtgggccgccggagttgctgctgctggacttctaagggcctgctcttccttctgcaggcctccttctcctcctcctcggactccaccgtctctgggcgccacagccagccggccttcctctccggcgggtacttccactcgacccggtcccccacaacctgcttcgcgcgcttggccctgcgcttccccaccctcagccggtagcgctcctgggcgctctcccagtacttctccaggcacctgtccctgtgcctgctcggcagctgatcccgcagccgccactcctcccggtgctcgccaggatcctttccactcctgccctctggcagctttcctttccccttcgctgcgtccctgtttccacgc

SEQ ID NO: 10587 - RNA, 1699 nt, Homo sapiens
  source 1..1699: mol_type = other RNA
cggcccgggctgctgctgttcctcttcaaagtccaccaggtcccattcatattccagtctggcttgtcgttgtttccaaaactccaaaaataaggtgacccaaattcccatgaatattgcaaagaacactgttgactcattatcaaacaaatgggagaactttgaagccaaacacgtactatttagtctccaataatcacacacttgatcacagagtgggcacatgatcatctgaccaccaatctcagggtcacagatttcagtgctgcttgtgttatgttccattgataataagccataaataaaacaagctaagccaactacagctgcaaagaatagcatttctgtgtaaaatccaagaaagacaaaatagataccaattttttctccataataattcttaatcaagtctaaaggctgctccttgtagaaataggaaaatcgagcccaattctggtgaagtgtgtatctttcattggtaggattgggaggttctgatggcttccaatattggccatcatggagtggataggcagatgagtaagtgttagagtttagcagtctttcaatcccaaaccttttcttcccatcttctatgccaaaaggacatcttgagagaatatagtacacaattctgtttcttgatgaggatggaaagaaggttgcctgatcttcgatgaggaagagctcctgccgatgtctgctgaattgtgcagtaaaatattcaggatggggatacttcacactcagtgggagtcttacaggtccaagcacatagcttataggagtgtgcttagggcggggaatatcactctccttaataggcattttgattcccaagacttcagcataggtaactaatacctcccaaggggcatggatcttgacaaaataagttcttccatcttccgagtcccttttgtcttctatttccaactcaagacctgtttttctgagattagtttcaaactcttttcttctttccgcctttaactctgcgtctttctttacatcatcaacgtaggaaagcacaaaatcaatttgcctaatcccatctcggaagaagatagaatctttgctttgctgatttttttgaaacattgtttcttcattgatgagaaagctggtctctctgctgctcaggctctgctcactcatttggaaagagtagtctatatgcttattgactttttccccttcctccgccaacacttccaggagatccgggtcgcccatcttcgccagctcgttaatggcactggtgcctgagaggcagcaggagaggggcagctgagacagacgtggagatctgaggcaggtgctgaatctgactgtgggccgccggagttgctgctgctggacttctaagggcctgctcttccttctgcaggcctccttctcctcctcctcggactccaccgtctctgggcgccacagccagccggccttcctctccggcgggtacttccactcgacccggtcccccacaacctgcttcgcgcgcttggccctgcgcttccccaccctcagccggtagcgctcctgggcgctctcccagtacttctccaggcacctgtccctgtgcctgctcggcagctgatcccgcagccgccactcctcccggtgctcgccaggatcctttccactcctgccctctggcagctttcctttccccttcgctgcgtccctgtttccacgc

SEQ ID NO: 10588 - RNA, 1648 nt, Homo sapiens
  source 1..1648: mol_type = other RNA
cggcccgggctgctgctgttcctcttcaaagtccaccaggtcccattcatattccagtctggcttgtcgttgtttccaaaactccaaaaataaggtgacccaaattcccatgaatattgcaaagaacactgttgactcattatcaaacaaatgggagaactttgaagccaaacacgtactatttagtctccaataatcacacacttgatcacagagtgggcacatgatcatctgaccaccaatctcagggtcacagatttcagtgctgcttgtgttatgttccattgataataagccataaataaaacaagctaagccaactacagctgcaaagaatagcatttctgtgtaaaatccaagaaagacaaaatagataccaattttttctccataataattcttaatcaagtctaaaggctgctccttgtagaaataggaaaatcgagcccaattctggtgaagtgtgtatctttcattggtaggattgggaggttctgatggcttccaatattggccatcatggagtggataggcagatgagtaagtgttagagtttagcagtctttcaatcccaaaccttttcttcccatcttctatgccaaaaggacatcttgagagaatatagtacacaattctgtttcttgatgaggatggaaagaaggttgcctgatcttcgatgaggaagagctcctgccgatgtctgctgaattgtgcagtaaaatattcaggatggggatacttcacactcagtgggagtcttacaggtccaagcacatagcttataggagtgtgcttagggcggggaatatcactctccttaataggcattttgattcccaagacttcagcataggtaactaatacctcccaaggggcatggatcttgacaaaataagttcttccatcttccgagtcccttttgtcttctatttccaactcaagacctgtttttctgagattagtttcaaactcttttcttctttccgcctttaactctgcgtctttctttacatcatcaacgtaggaaagcacaaaatcaatttgcctaatcccatctcggaagaagatagaatctttgctttgctgatttttttgaaactcactcatttggaaagagtagtctatatgcttattgactttttccccttcctccgccaacacttccaggagatccgggtcgcccatcttcgccagctcgttaatggcactggtgcctgagaggcagcaggagaggggcagctgagacagacgtggagatctgaggcaggtgctgaatctgactgtgggccgccggagttgctgctgctggacttctaagggcctgctcttccttctgcaggcctccttctcctcctcctcggactccaccgtctctgggcgccacagccagccggccttcctctccggcgggtacttccactcgacccggtcccccacaacctgcttcgcgcgcttggccctgcgcttccccaccctcagccggtagcgctcctgggcgctctcccagtacttctccaggcacctgtccctgtgcctgctcggcagctgatcccgcagccgccactcctcccggtgctcgccaggatcctttccactcctgccctctggcagctttcctttccccttcgctgcgtccctgtttccacgc

SEQ ID NO: 10589 - RNA, 649 nt, Homo sapiens
  source 1..649: mol_type = other RNA
cggcccgggctgctgctgttcctcttccacctcggggtgctccaggtcggcctccaccgactcgttcacctccccacctgccgcctcgtcggtcacctccacctccgcagacccctccaagtggttcatggtgggagtcggaacggctaggagagaagctgggcccggctcactgcgctctcattttgctccactgggattgacaaagtaattctcccactctcagataggcgtggatggtggattctaatcccagctctcctttccttctctccaacgtgcatgttttccaaacccaagcctagggtgggatgtcaagcagaaacacaacttttattatcaactgctcacactgtacactgcacaatgaaggaaaaaatgttacctgttgaatgaatgcatgacaagggttgaaaatctttaaaaaactaaattataaaaataaccacattagagaaaaggagaaattgcccataacctcagcattagtcatctgtttcctgtgccagttctacaccgctgtatcataaaagtctatccagtatttttgatcctggcctttttatccatttaaataattatttactctataaaaatagccattaaaatgtatgttttctgagaacatttaatatgcatagggaaatgc

SEQ ID NO: 10590 - RNA, 360 nt, Homo sapiens
  source 1..360: mol_type = other RNA
cggcccgggctgctgctgttcctcttccacctcggggtgctccaggtcggcctccaccgactcgttcacctccccacctgccgcctcgtcggtcacctccacctccgcagacccctccaagtggttcatggtgggagtcggaacggctaggagagaagctgggcccggctcactgcgctctcattttgctccactgggctctgcgcgaagcaacgggccacgctgcaggaccacgaagccaggcagccgcgtcgactcctgcagggtgttctctccggagtgactcccgagctttcccgcttcccaggccccttagatatcgcctgcgcttcaaattcggagattgacggcgtctccgga

SEQ ID NO: 10591 - RNA, 417 nt, Homo sapiens
  source 1..417: mol_type = other RNA
cggcccgggctgctgctgttcctcttccacctcggggtgctccaggtcggcctccaccgactcgttcacctccccacctgccgcctcgtcggtcacctccacctccgcagacccctccaagtggttcatggtgggagtcggaacggctaggagagaagctgggcccggctcactgcgctctcattttgctccactgggcttgcctgacagctgggtccgcgggcccgcgggagcaggcggcgctagtgacagcgctggtgccaagcctgggaataaagctccgctccagccgctgctgcctccagcgccaccatcttctcccgccgcagctgccgccgccgccgccgccgccgggaccgcagccgccctcgcccagctccggctccgcagccgctgctcggacccctccggtctcgc

SEQ ID NO: 10592 - RNA, 436 nt, Homo sapiens
  source 1..436: mol_type = other RNA
cggcccgggctgctgctgttcctcttccacctcggggtgctccaggtcggcctccaccgactcgttcacctccccacctgccgcctcgtcggtcacctccacctccgcagacccctccaagtggttcatggtgggagtcggaacggctaggagagaagctgggcccggctcactgcgctctcattttgctccactgggcttgcctgacagctgggtccgcgggcccgcgggagcaggcggcgctagtgacagcgctggtgccaagcctgggaataaagctccgctccagccgctgctgcctccagcgccaccatcttctcccgccgcagctgccgccgccgccgccgccgccgggaccgcagccgccctcgcccagctccggctccgcagccgctgctcggacccctccggtctcgcggccccaccccctttcccc

SEQ ID NO: 10593 - RNA, 1706 nt, Homo sapiens
  source 1..1706: mol_type = other RNA
cggcccgggctgctgctgttcctgctgccgtagtaagtgcccctgcagcctctgctggtgcaaagcttcctggtgttcccgcagctgctgggcctcctccacctgctgcactgccagtctctgctgttccaactgttcctcatagggtgattggaatttgatcattggcttggctgaagggtacacctcagcacgcgcgtgcccttccaggaggttggctgcttctcgttgctcatgctgctctttccactcccgatcctgctcctctggtgatggatcgtgttcctcctcaagatgttctgcttgcccgacctgctccatttcttcctcctccagggcctttctgtgctcctcttccacctgatgctcctcaggttctctgcgttccacttcttgttggattggctctgggggagcctgaaattctgcctccttatgggtgggagcatagagttttgtgtcttctgctcttccaggaactgcttcatggttctgccacacatcattatttcgagacacctcctgcacctctcgggttggcttctcccttgctgtgttgtaaccttgtggagaatgtgccacctgggtcacattttgctgttctgctggatcaggttttcgaaggcttggaatcctattcagagtatctttcagttgtttatattctgcaacttgagtctgtgcagcagctagtgcactcttgtggtcttccaaagtcactacaagttgttcatgctcggagagtaaattcttatgctgttgcttgacatcttgaagctgtgtatgtatgtcttggtgtgctttccttagttgtctattctcttctctcaaattgtatacagtctcttttagcttagaaagttcttgttctttttcttgctggagctgcaagtatttttgcttatggtcattaaatgttctactgaagtcttccccttgtttgcgatgttcctcttccaagtcactgtgctgtttctttagctcctcgtgttggcttttcaacatctgatgttggacattcagtgcactgtatctgctattggaatcttgccttcctttatttaatgtttcttgtgcttctaacttataaacaagaaaatcttcctttgcttttttatgttcaagtctttctttttgcaaggatttctctaatcttgatctgtgttcatatacaacttgtaactgggcggagagggactcctggtgctgctggtacttgagcgccaccgcctcggctttccgcagctgcgtctgcagctcgtagtagagcatcgcgccgtagagaaagccgaacacgacggtcagcagcagcagcgtctggaaaatccgcttctgctttcgggagcacatcccgtttcccatagtcccgcctggacccaaagccgcggccgcccccgccgtctcctccccttggtccgagcgagcgtctcagcagcggccgccgcagtaggtggccagacgcagcatgaggaggagatgccagacacaaaagccggcccggaggggaagtggcgcccgctcagcccccgcgcggcgcggggcgcgcagccatcgacgccgcccgggcagctgcagccaaacttctgcgaggctcgttctccgcgaatgcccggggccgggaggaggccctccgcatacttcagagccggctgccctcgcgcctgtccccagatgcctcctgccttttttccttcttcccacttttt

SEQ ID NO: 10594 - RNA, 2001 nt, Homo sapiens
  source 1..2001: mol_type = other RNA
cggcccgggctgctgctgttcctgctgccgtagtaagtgcccctgcagcctctgctggtgcaaagcttcctggtgttcccgcagctgctgggcctcctccacctgctgcactgccagtctctgctgttccaactgttcctcatagggtgattggaatttgatcattggcttggctgaagggtacacctcagcacgcgcgtgcccttccaggaggttggctgcttctcgttgctcatgctgctctttccactcccgatcctgctcctctggtgatggatcgtgttcctcctcaagatgttctgcttgcccgacctgctccatttcttcctcctccagggcctttctgtgctcctcttccacctgatgctcctcaggttctctgcgttccacttcttgttggattggctctgggggagcctgaaattctgcctccttatgggtgggagcatagagttttgtgtcttctgctcttccaggaactgcttcatggttctgccacacatcattatttcgagacacctcctgcacctctcgggttggcttctcccttgctgtgttgtaaccttgtggagaatgtgccacctgggtcacattttgctgttctgctggatcaggttttcgaaggcttggaatcctattcagagtatctttcagttgtttatattctgcaacttgagtctgtgcagcagctagtgcactcttgtggtcttccaaagtcactacaagttgttcatgctcggagagtaaattcttatgctgttgcttgacatcttgaagctgtgtatgtatgtcttggtgtgctttccttagttgtctattctcttctctcaaattgtatacagtctcttttagcttagaaagttcttgttctttttcttgctggagctgcaagtatttttgcttatggtcattaaatgttctactgaagtcttccccttgtttgcgatgttcctcttccaagtcactgtgctgtttctttagctcctcgtgttggcttttcaacatctgatgttggacattcagtgcactgtatctgctattggaatcttgccttcctttatttaatgtttcttgtgcttctaacttataaacaagaaaatcttcctttgcttttttatgttcaagtctttctttttgcaaggatttctctaatcttgatctgtgttcatatacaacttgtaactgggcggagagggactcctggtgctgctggtacttgagcgccaccgcctcggctttccgcagctgcgtctgcagctcgtagtagagcatcgcgccgtagagaaagccgaacacgacggtcagcagcagcagcgtctggaaaatccgcttctgctttcgggagcacatcccgtttcccatagtcccgcctggacccaaagccgcggccgcccccgccgtctcctccccttggtccgagcgagcgtctcagcagcggccgccgcagtaggtggccagacgcagcatgaggaggagatgccagacacaaaagccggcccggaggggaagtggcgcccgctcagcccccgcgcggcgcggggcgcgcagccatcgacgccgcccgggcagctgcagccaaacttctgcgaggctcgttctccgcgaatgcccggggccgggaggaggccctccgcatacttcagagccggctgccctcgcgcctgtccccagatgcctcctgccttttttccttcttcccactttttggccccgctgcccccgggcagttcttggagtcccgccctggccactccccgccctatcgcggcggctcccactgcacgactttgttgccacctaagggagggggtgcgcgcccaacaaagggaccaggactccgggccgcgcccccgtgcggcctgcccaatgggtggaagggtgggggccagctgtctcggctggttttggggacggcacagcggtgtcactgacgggtcggctggtgcctctgccgccccgccacctcctgcccaacttacgtgtcacccacggcccggctat

SEQ ID NO: 10595 - RNA, 1396 nt, Homo sapiens
  source 1..1396: mol_type = other RNA
cggcccgggctgctgctgttcctgctgccgtagtaagtgcccctgcagcctctgctggtgcaaagcttcctggtgttcccgcagctgctgggcctcctccacctgctgcactgccagtctctgctgttccaactgttcctcatagggtgattggaatttgatcattggcttggctgaagggtacacctcagcacgcgcgtgcccttccaggaggttggctgcttctcgttgctcatgctgctctttccactcccgatcctgctcctctggtgatggatcgtgttcctcctcaagatgttctgcttgcccgacctgctccatttcttcctcctccagggcctttctgtgctcctcttccacctgatgctcctcaggttctctgcgttccacttcttgttggattggctctgggggagcctgaaattctgcctccttatgggtgggagcatagagttttgtgtcttctgctcttccaggaactgcttcatggttctgccacacatcattatttcgagacacctcctgcacctctcgggttggcttctcccttgctgtgttgtaaccttgtggagaatgtgccacctgggtcacattttgctgttctgctggatcaggttttcgaaggcttggaatcctattcagagtatctttcagttgtttatattctgcaacttgagtcttgacatcttgaagctgtgtatgtatgtcttggtgtgctttccttagttgtctattctcttctctcaaattgtatacagtctcttttagcttagaaagttcttgttctttttcttgctggagctgcaagtatttttgcttatggtcattaaatgttctactgaagtcttccccttgtttgcgatgttcctcttccaagtcactgtgctgtttctttagctcctcgtgttggcttttcaacatctgatgttggacattcagtgcactgtatctgctattggaatcttgccttcctttatttaatgtttcttgtgcttctaacttataaacaagaaaatcttcctttgcttttttatgttcaagtctttctttttgcaaggatttctctaatcttgatctgtgttcatatacaactagaatccacggaacaatgctcctcagagcagggctggcagaagcggcggagggctaccagtttccctgccccgattgcagctgggcctttgacaagagctcgggtaaaggactatctgtgcacccgcccaccaaacgcccagcgggacgatgggctggtgctacgaagttctaaacctaaccgctgggaggaagaagcgggaggatgagaatgtcatctcccctgacactctggtgccggcagtcctgaaacgctcacctctgacgtccctgaaggtcagaggtggcaaccacagtgccaata

SEQ ID NO: 10596 - RNA, 1397 nt, Homo sapiens
  source 1..1397: mol_type = other RNA
cggcccgggctgctgctgttcctgctgccgtagtaagtgcccctgcagcctctgctggtgcaaagcttcctggtgttcccgcagctgctgggcctcctccacctgctgcactgccagtctctgctgttccaactgttcctcatagggtgattggaatttgatcattggcttggctgaagggtacacctcagcacgcgcgtgcccttccaggaggttggctgcttctcgttgctcatgctgctctttccactcccgatcctgctcctctggtgatggatcgtgttcctcctcaagatgttctgcttgcccgacctgctccatttcttcctcctccagggcctttctgtgctcctcttccacctgatgctcctcaggttctctgcgttccacttcttgttggattggctctgggggagcctgaaattctgcctccttatgggtgggagcatagagttttgtgtcttctgctcttccaggaactgcttcatggttctgccacacatcattatttcgagacacctcctgcacctctcgggttggcttctcccttgctgtgttgtaaccttgtggagaatgtgccacctgggtcacattttgctgttctgctggatcaggttttcgaaggcttggaatcctattcagagtatctttcagttgtttatattctgcaacttgagtcttgacatcttgaagctgtgtatgtatgtcttggtgtgctttccttagttgtctattctcttctctcaaattgtatacagtctcttttagcttagaaagttcttgttctttttcttgctggagctgcaagtatttttgcttatggtcattaaatgttctactgaagtcttccccttgtttgcgatgttcctcttccaagtcactgtgctgtttctttagctcctcgtgttggcttttcaacatctgatgttggacattcagtgcactgtatctgctattggaatcttgccttcctttatttaatgtttcttgtgcttctaacttataaacaagaaaatcttcctttgcttttttatgttcaagtctttctttttgcaaggatttctctaatcttgatctgtgttcatatacaactagaatccacggaacaatgctcctcagagcagggctggcagaagcggcggagggctaccagtttccctgccccgattgcagctgggcctttgacaagagctcgggtaaaggactatctgtgcacccgcccaccaaacgcccagcgggacgatgggctggtgctacgaagttctaaacctaaccgctgggaggaagaagcgggaggatgagaatgtcatctcccctgacactctggtgccggcagtcctgaaacgctcacctctgacgtccctgaaggtcagaggtggcaaccacagtgccaatag

SEQ ID NO: 10597 - RNA, 1622 nt, Homo sapiens
  source 1..1622: mol_type = other RNA
cggcccgggctgctgctgttcctgctgccgtagtaagtgcccctgcagcctctgctggtgcaaagcttcctggtgttcccgcagctgctgggcctcctccacctgctgcactgccagtctctgctgttccaactgttcctcatagggtgattggaatttgatcattggcttggctgaagggtacacctcagcacgcgcgtgcccttccaggaggttggctgcttctcgttgctcatgctgctctttccactcccgatcctgctcctctggtgatggatcgtgttcctcctcaagatgttctgcttgcccgacctgctccatttcttcctcctccagggcctttctgtgctcctcttccacctgatgctcctcaggttctctgcgttccacttcttgttggattggctctgggggagcctgaaattctgcctccttatgggtgggagcatagagttttgtgtcttctgctcttccaggaactgcttcatggttctgccacacatcattatttcgagacacctcctgcacctctcgggttggcttctcccttgctgtgttgtaaccttgtggagaatgtgccacctgggtcacattttgctgttctgctggatcaggttttcgaaggcttggaatcctattcagagtatctttcagttgtttatattctgcaacttgagtcttgacatcttgaagctgtgtatgtatgtcttggtgtgctttccttagttgtctattctcttctctcaaattgtatacagtctcttttagcttagaaagttcttgttctttttcttgctggagctgcaagtatttttgcttatggtcattaaatgttctactgaagtcttccccttgtttgcgatgttcctcttccaagtcactgtgctgtttctttagctcctcgtgttggcttttcaacatctgatgttggacattcagtgcactgtatctgctattggaatcttgccttcctttatttaatgtttcttgtgcttctaacttataaacaagaaaatcttcctttgcttttttatgttcaagtctttctttttgcaaggatttctctaatcttgatctgtgttcatatacaacttgtaactgggcggagagggactcctggtgctgctggtacttgagcgccaccgcctcggctttccgcagctgcgtctgcagctcgtagtagagcatcgcgccgtagagaaagccgaacacgacggtcagcagcagcagcgtctggaaaatccgcttctgctttcgggagcacatcccgtttcccatagtcccgcctggacccaaagccgcggccgcccccgccgtctcctccccttggtccgagcgagcgtctcagcagcggccgccgcagtaggtggccagacgcagcatgaggaggagatgccagacacaaaagccggcccggaggggaagtggcgcccgctcagcccccgcgcggcgcggggcgcgcagccatcgacgccgcccgggcagctgcagccaaacttctgcgaggctcgttctccgcgaatgcccggggccgggaggaggccctccgcatacttcagagccggctgccctcgcgcctgtccccagatgcctcctgccttttttccttcttcccacttttt

SEQ ID NO: 10598 - RNA, 1917 nt, Homo sapiens
  source 1..1917: mol_type = other RNA
cggcccgggctgctgctgttcctgctgccgtagtaagtgcccctgcagcctctgctggtgcaaagcttcctggtgttcccgcagctgctgggcctcctccacctgctgcactgccagtctctgctgttccaactgttcctcatagggtgattggaatttgatcattggcttggctgaagggtacacctcagcacgcgcgtgcccttccaggaggttggctgcttctcgttgctcatgctgctctttccactcccgatcctgctcctctggtgatggatcgtgttcctcctcaagatgttctgcttgcccgacctgctccatttcttcctcctccagggcctttctgtgctcctcttccacctgatgctcctcaggttctctgcgttccacttcttgttggattggctctgggggagcctgaaattctgcctccttatgggtgggagcatagagttttgtgtcttctgctcttccaggaactgcttcatggttctgccacacatcattatttcgagacacctcctgcacctctcgggttggcttctcccttgctgtgttgtaaccttgtggagaatgtgccacctgggtcacattttgctgttctgctggatcaggttttcgaaggcttggaatcctattcagagtatctttcagttgtttatattctgcaacttgagtcttgacatcttgaagctgtgtatgtatgtcttggtgtgctttccttagttgtctattctcttctctcaaattgtatacagtctcttttagcttagaaagttcttgttctttttcttgctggagctgcaagtatttttgcttatggtcattaaatgttctactgaagtcttccccttgtttgcgatgttcctcttccaagtcactgtgctgtttctttagctcctcgtgttggcttttcaacatctgatgttggacattcagtgcactgtatctgctattggaatcttgccttcctttatttaatgtttcttgtgcttctaacttataaacaagaaaatcttcctttgcttttttatgttcaagtctttctttttgcaaggatttctctaatcttgatctgtgttcatatacaacttgtaactgggcggagagggactcctggtgctgctggtacttgagcgccaccgcctcggctttccgcagctgcgtctgcagctcgtagtagagcatcgcgccgtagagaaagccgaacacgacggtcagcagcagcagcgtctggaaaatccgcttctgctttcgggagcacatcccgtttcccatagtcccgcctggacccaaagccgcggccgcccccgccgtctcctccccttggtccgagcgagcgtctcagcagcggccgccgcagtaggtggccagacgcagcatgaggaggagatgccagacacaaaagccggcccggaggggaagtggcgcccgctcagcccccgcgcggcgcggggcgcgcagccatcgacgccgcccgggcagctgcagccaaacttctgcgaggctcgttctccgcgaatgcccggggccgggaggaggccctccgcatacttcagagccggctgccctcgcgcctgtccccagatgcctcctgccttttttccttcttcccactttttggccccgctgcccccgggcagttcttggagtcccgccctggccactccccgccctatcgcggcggctcccactgcacgactttgttgccacctaagggagggggtgcgcgcccaacaaagggaccaggactccgggccgcgcccccgtgcggcctgcccaatgggtggaagggtgggggccagctgtctcggctggttttggggacggcacagcggtgtcactgacgggtcggctggtgcctctgccgccccgccacctcctgcccaacttacgtgtcacccacggcccggctat

SEQ ID NO: 10599 - RNA, 4826 nt, Homo sapiens
  source 1..4826: mol_type = other RNA
cggcccgggctgctgctgttcctgggatggagagttactctgcatggcaactattgagtgctgtgactggaacatggttccttgttggctttgaggcattggattaggtggaagggagcccagggccacctgaggctgaaataaaccctgctgcgggggttgtgcctgttcttgggaaagcataggagtctggatgtgtgatattggagcttgctgttggaaagcagcttgttgttcactgtttgatgttgactgaagtggagaaattgagttcggtgctgcaaaaaatgcttcttgggctactgtgttagtctgaagattattcatgggactctgggaaagaaatatgttggttgactgctggtcttgaggaactgaagagccctgtaacacagcaatggtactttgagagtgaaacattggaggctgcatttgttcagaggaggttgtagaagtctgactgtggacaataggatttggactatgaaagagagaaccttgagtttcctgggaaaggttctgagcatcggcaataggattttgaggatgaaaaagttgggcctgtgaatgagaagactgctgcaaaaaatttccagattgaagtgacatcatctcattcccttgctggaataaaccattaccttgttgttgggtaccactattctgaacactcatcatactttttgtggatgaaaaaaggttaacttgaggttgattgtccccactatgttgcatttggaccatggtctgaaagacactgttctgaatctgttttgcttgtgttccagtttcttctccatctcctgaacttgatgtctgaaacatggtagtgccaggggttgcaacctgctgtgtggtagttgtagaagtttcatttccagaaactgcaggaggagaagaaaacaattcacactgcatttgcatatcctcattggtagacaatgcactcatcatgtgagaagtctgctggtaaactggcgattgctgaaggtttccatttgctgaagcagttgaagggaataactctgactgaatctgggcagctgcctggcagatactctgttgcatctccatcaccattgcggctgaagattccatcacttgctgttgctgctgctgctgctgctgttgattagataacgtgttttcagactgtggatgaacactttcagctcttccaggtaataaattatctggtctggtatggactgttggctctgttgaggaaaacattccagggcttacaccactctgaatttgactgacttgttgaaaaatatctgcactaagctgctcttgaacattctcattaccatctggagcagaaaataaaactgaagataactgctgctgtgcctctaaaacttgttggaccaagtcaacacttccactgctgccactagcagtactgcctgtgaaactccctgcttgcagctgctgaatagtattctgaagctgactcacactatttggtgatggaaaaatatttgatgaaatctgctgctgtaaagtctgtgcttgttcttgtagtggtgactgctgctgttgttgtgatgcctcagtcagttgtgacaaattaaccactgtaccatctgactgtaatatctctctagactgagtttctcttgtctgaaactgtgtagcctgctgcaatagtgcatcgctgttgggcagctgactagaagcagaaactgctggaaaagtaccaggctgtgagatgtcctgggtttgaatagttgtcagggtctctgggttgtatgccttgggctgaatctgctgctgtttttcattttcagaaggtaggtgggaagatgatggtgatgaaaaagagccatttcctgctatgtttgagatgttttctaatgtttgctgagttgatccaacagactttgtagtcttaaaaatagtggaagatcttttttctgctgttacttccattggagtaacatcttcactcttaatcatactgcttggtatgagtggagtcatcagggcattagggataatatttaccttatctaaattacatccagtagttttcattgctttcatggcctcttcaaaagagcaaggtcttgctggactagatatttccttcttcacatttacattcaaagcaccagctgctgctgggtctggagtgtaagtgaatggttgaacatcatgagatcttccagcatttgtcactacatatattcccactgacacaggcaaagttatatgttggtcatgatagggaggaaccttcacaataagatgattctgatgaaatagttccatatcaatttcagcttctgacttccaagagttttcatcagaaacattttcttggaaaataactttagttcctttcagaaagttcttgccgattaaaaacacttcttcttctcctttcactgaacagctatgcaagcttttctttaagatttctggcactcctgctggctgagtacacaaaattggagaagagggtgtttgcagtgtcaaagtggagccatctttcctcatgatattaactcgaaaaaccaatctggcacgagtgcttttcttcttggaaccagcaattcctattctggcttcgacatcagcattcctcaatttcaatatccctacgcagtccaccgccagtgtcatgttgttgctaggatcaaggccgacttctataacagtagtgccttcaatgtccacttctttgcaaggagttgtatttcgtccagttactctgcaggcctgataaaatccatgtggtttcactcgtccagagtcgttgcccacaaacacttgcaacactacaggttcattatggccttccagctttactgtaggaaagccttgctgtgttctatctttcactgagccacggctgccctcagtcaggtaccgagctcggtgctgtgtctcaggttgtacaactatcttcagctcctttccctcacttttaacaggatattgtccacacaacatagggctcttctttactccagttcctttttggttttccaatgttccatttcccgcttttgagttgcctttgttgtccgtggtaagctgagaaagcacatagtgaggtgctttggcactgtcggcatcaaatatatccatattagattcttcacaatctcgtcgtttgacccccggcctctgctttggatttcgttttcgtgatttacgaggtacctcagtgttatcattgtaggaactggtgctcatgttactgaagttggagggggaatcctccatccacatactgcagctctgctcagattccaatccacacccctcatcctggcaggacatccgactgttatccagcaagtcctcaggtggtggtgagatgtacaagactgtgtgcctcttcggtgttgatggatgctgctgaactgtgttactggttaactgcttttcacttacccctctgttacttacccccacggctgaggagcagctctccacttgcatagccttgctgtcggtgactgaggtagaataaatggtagggctggaagaggtggtaaaggagctgcaagcaccgcccatggaggaagaggagggagctgaagaagcatcagcagcaacaacagctggaggaggcgagcctgcctcaccaccgcttgtctgactcattgatgctacagatgtttctctagatggaggtaactgtaactcctttgggagaagatcatagacagattcatgagtcttctcttggtcatataattacttgtttgacatcttatttgccacagtcacaggggctaagtatttttgtctatgccagctcctcttcactatcaccttcaacctgacaaagcagtaattaaacattcattcaacatttatttagcacctgcactgatctagggacacaatacaaaagaaagtcacccttattaagcagttcacagtctagagataataaaatgagtcaagtttaaaataatgcagtatgtgctttaataaagtatgaagtgttacacaactggagaagagggaacctttaatgttatctgtggaggatctgagaaggcagcacagaggatgtaacaccagaagtcaaccttgaatattgaaatggctatttagcagacagactggggaaaaggaaggagaaactataaaagcaaacctgaacaaaaagagtattttcatctcaggttattaggtaactcagttactcagaacacggaagttacaagcagtaacatgagatgaaactactaaaggcagggtgaggccagattatgacagggcttgtgtatcatgctaagcagtaagggttttatccctcagcacacagggagcctttgagggttttaagcaaagaaatgataaactcaaacatatatttgaggaagatcatcctaccaggaatacagagaatagattaggtcctagagatggcgatgagtaagaaggtttttacaataatagcctaagcaagaaataatgaaatcctgaaccaaggcagtggcagtgaaatagtcaataggctacgaatttaaagctgtttaaatggatgaactaaattggatcactggctacggtggggaagggagagggaaaaaaaggagagttccaagtagcacatagaactctggcttgggaaaattgataaaaagtggtgccatttcctgtgatagagaatataggagttaagaataaacctggaaagagaattcagttttaaatgatgaatttggatgcctatgggacttccaagtgaatacataaacaggagagaggtctagcaattgatgttactaaacaaatagcctgctttacttttgttttttatatcaaatctgtcctagaactacagttttgcc

SEQ ID NO: 10600 - RNA, 4101 nt, Homo sapiens
  source 1..4101: mol_type = other RNA
cggcccgggctgctgctgttcctgggatggagagttactctgcatggcaactattgagtgctgtgactggaacatggttccttgttggctttgaggcattggattaggtggaagggagcccagggccacctgaggctgaaataaaccctgctgcgggggttgtgcctgttcttgggaaagcataggagtctggatgtgtgatattggagcttgctgttggaaagcagcttgttgttcactgtttgatgttgactgaagtggagaaattgagttcggtgctgcaaaaaatgcttcttgggctactgtgttagtctgaagattattcatgggactctgggaaagaaatatgttggttgactgctggtcttgaggaactgaagagccctgtaacacagcaatggtactttgagagtgaaacattggaggctgcatttgttcagaggaggttgtagaagtctgactgtggacaataggatttggactatgaaagagagaaccttgagtttcctgggaaaggttctgagcatcggcaataggattttgaggatgaaaaagttgggcctgtgaatgagaagactgctgcaaaaaatttccagattgaagtgacatcatctcattcccttgctggaataaaccattaccttgttgttgggtaccactattctgaacactcatcatactttttgtggatgaaaaaaggttaacttgaggttgattgtccccactatgttgcatttggaccatggtctgaaagacactgttctgaatctgttttgcttgtgttccagtttcttctccatctcctgaacttgatgtctgaaacatggtagtgccaggggttgcaacctgctgtgtggtagttgtagaagtttcatttccagaaactgcaggaggagaagaaaacaattcacactgcatttgcatatcctcattggtagacaatgcactcatcatgtgagaagtctgctggtaaactggcgattgctgaaggtttccatttgctgaagcagttgaagggaataactctgactgaatctgggcagctgcctggcagatactctgttgcatctccatcaccattgcggctgaagattccatcacttgctgttgctgctgctgctgctgctgttgattagataacgtgttttcagactgtggatgaacactttcagctcttccaggtaataaattatctggtctggtatggactgttggctctgttgaggaaaacattccagggcttacaccactctgaatttgactgacttgttgaaaaatatctgcactaagctgctcttgaacattctcattaccatctggagcagaaaataaaactgaagataactgctgctgtgcctctaaaacttgttggaccaagtcaacacttccactgctgccactagcagtactgcctgtgaaactccctgcttgcagctgctgaatagtattctgaagctgactcacactatttggtgatggaaaaatatttgatgaaatctgctgctgtaaagtctgtgcttgttcttgtagtggtgactgctgctgttgttgtgatgcctcagtcagttgtgacaaattaaccactgtaccatctgactgtaatatctctctagactgagtttctcttgtctgaaactgtgtagcctgctgcaatagtgcatcgctgttgggcagctgactagaagcagaaactgctggaaaagtaccaggctgtgagatgtcctgggtttgaatagttgtcagggtctctgggttgtatgccttgggctgaatctgctgctgtttttcattttcagaaggtaggtgggaagatgatggtgatgaaaaagagccatttcctgctatgtttgagatgttttctaatgtttgctgagttgatccaacagactttgtagtcttaaaaatagtggaagatcttttttctgctgttacttccattggagtaacatcttcactcttaatcatactgcttggtatgagtggagtcatcagggcattagggataatatttaccttatctaaattacatccagtagttttcattgctttcatggcctcttcaaaagagcaaggtcttgctggactagatatttccttcttcacatttacattcaaagcaccagctgctgctgggtctggagtgtaagtgaatggttgaacatcatgagatcttccagcatttgtcactacatatattcccactgacacaggcaaagttatatgttggtcatgatagggaggaaccttcacaataagatgattctgatgaaatagttccatatcaatttcagcttctgacttccaagagttttcatcagaaacattttcttggaaaataactttagttcctttcagaaagttcttgccgattaaaaacacttcttcttctcctttcactgaacagctatgcaagcttttctttaagatttctggcactcctgctggctgagtacacaaaattggagaagagggtgtttgcagtgtcaaagtggagccatctttcctcatgatattaactcgaaaaaccaatctggcacgagtgcttttcttcttggaaccagcaattcctattctggcttcgacatcagcattcctcaatttcaatatccctacgcagtccaccgccagtgtcatgttgttgctaggatcaaggccgacttctataacagtagtgccttcaatgtccacttctttgcaaggagttgtatttcgtccagttactctgcaggcctgataaaatccatgtggtttcactcgtccagagtcgttgcccacaaacacttgcaacactacaggttcattatggccttccagctttactgtaggaaagccttgctgtgttctatctttcactgagccacggctgccctcagtcaggtaccgagctcggtgctgtgtctcaggttgtacaactatcttcagctcctttccctcacttttaacaggatattgtccacacaacatagggctcttctttactccagttcctttttggttttccaatgttccatttcccgcttttgagttgcctttgttgtccgtggtaagctgagaaagcacatagtgaggtgctttggcactgtcggcatcaaatatatccatattagattcttcacaatctcgtcgtttgacccccggcctctgctttggatttcgttttcgtgatttacgaggtacctcagtgttatcattgtaggaactggtgctcatgttactgaagttggagggggaatcctccatccacatactgcagctctgctcagattccaatccacacccctcatcctggcaggacatccgactgttatccagcaagtcctcaggtggtggtgagatgtacaagactgtgtgcctcttcggtgttgatggatgctgctgaactgtgttactggttaactgcttttcacttacccctctgttacttacccccacggctgaggagcagctctccacttgcatagccttgctgtcggtgactgaggtagaataaatggtagggctggaagaggtggtaaaggagctgcaagcaccgcccatggaggaagaggagggagctgaagaagcatcagcagcaacaacagctggaggaggcgagcctgcctcaccaccgcttgtctgactcattgatgctacagatgtttctctagatggaggtaactgtaactcctttgggagaagatcatagacagattctcgcgagtagagggacttgggcgattccaggtctaggtccgcgctgagcaatgagatgaagtccgagggcatcgcagctcgacccagcccggcccgagggcagcgggagggggggagcggcggtggcggcggcacctcctctccgggaccgcgggcaccgaaccgggggcggcgacgcgagggcggctgccgctgcctcctcctcgagggtagtgacttccactgggccgaggaccgaggaaacgatggcgaggtggagggggaactccacggggactgattctcggtgaccaggagaggggttcaggacggggaaggggaagggggagagccaaagggtccgtttcgtgtttctcctcagcgaaaactgacggtcgccgccaccgccgccgccgctgacaggaatct

SEQ ID NO: 10601 - RNA, 4155 nt, Homo sapiens
  source 1..4155: mol_type = other RNA
cggcccgggctgctgctgttcctgggatggagagttactctgcatggcaactattgagtgctgtgactggaacatggttccttgttggctttgaggcattggattaggtggaagggagcccagggccacctgaggctgaaataaaccctgctgcgggggttgtgcctgttcttgggaaagcataggagtctggatgtgtgatattggagcttgctgttggaaagcagcttgttgttcactgtttgatgttgactgaagtggagaaattgagttcggtgctgcaaaaaatgcttcttgggctactgtgttagtctgaagattattcatgggactctgggaaagaaatatgttggttgactgctggtcttgaggaactgaagagccctgtaacacagcaatggtactttgagagtgaaacattggaggctgcatttgttcagaggaggttgtagaagtctgactgtggacaataggatttggactatgaaagagagaaccttgagtttcctgggaaaggttctgagcatcggcaataggattttgaggatgaaaaagttgggcctgtgaatgagaagactgctgcaaaaaatttccagattgaagtgacatcatctcattcccttgctggaataaaccattaccttgttgttgggtaccactattctgaacactcatcatactttttgtggatgaaaaaaggttaacttgaggttgattgtccccactatgttgcatttggaccatggtctgaaagacactgttctgaatctgttttgcttgtgttccagtttcttctccatctcctgaacttgatgtctgaaacatggtagtgccaggggttgcaacctgctgtgtggtagttgtagaagtttcatttccagaaactgcaggaggagaagaaaacaattcacactgcatttgcatatcctcattggtagacaatgcactcatcatgtgagaagtctgctggtaaactggcgattgctgaaggtttccatttgctgaagcagttgaagggaataactctgactgaatctgggcagctgcctggcagatactctgttgcatctccatcaccattgcggctgaagattccatcacttgctgttgctgctgctgctgctgctgttgattagataacgtgttttcagactgtggatgaacactttcagctcttccaggtaataaattatctggtctggtatggactgttggctctgttgaggaaaacattccagggcttacaccactctgaatttgactgacttgttgaaaaatatctgcactaagctgctcttgaacattctcattaccatctggagcagaaaataaaactgaagataactgctgctgtgcctctaaaacttgttggaccaagtcaacacttccactgctgccactagcagtactgcctgtgaaactccctgcttgcagctgctgaatagtattctgaagctgactcacactatttggtgatggaaaaatatttgatgaaatctgctgctgtaaagtctgtgcttgttcttgtagtggtgactgctgctgttgttgtgatgcctcagtcagttgtgacaaattaaccactgtaccatctgactgtaatatctctctagactgagtttctcttgtctgaaactgtgtagcctgctgcaatagtgcatcgctgttgggcagctgactagaagcagaaactgctggaaaagtaccaggctgtgagatgtcctgggtttgaatagttgtcagggtctctgggttgtatgccttgggctgaatctgctgctgtttttcattttcagaaggtaggtgggaagatgatggtgatgaaaaagagccatttcctgctatgtttgagatgttttctaatgtttgctgagttgatccaacagactttgtagtcttaaaaatagtggaagatcttttttctgctgttacttccattggagtaacatcttcactcttaatcatactgcttggtatgagtggagtcatcagggcattagggataatatttaccttatctaaattacatccagtagttttcattgctttcatggcctcttcaaaagagcaaggtcttgctggactagatatttccttcttcacatttacattcaaagcaccagctgctgctgggtctggagtgtaagtgaatggttgaacatcatgagatcttccagcatttgtcactacatatattcccactgacacaggcaaagttatatgttggtcatgatagggaggaaccttcacaataagatgattctgatgaaatagttccatatcaatttcagcttctgacttccaagagttttcatcagaaacattttcttggaaaataactttagttcctttcagaaagttcttgccgattaaaaacacttcttcttctcctttcactgaacagctatgcaagcttttctttaagatttctggcactcctgctggctgagtacacaaaattggagaagagggtgtttgcagtgtcaaagtggagccatctttcctcatgatattaactcgaaaaaccaatctggcacgagtgcttttcttcttggaaccagcaattcctattctggcttcgacatcagcattcctcaatttcaatatccctacgcagtccaccgccagtgtcatgttgttgctaggatcaaggccgacttctataacagtagtgccttcaatgtccacttctttgcaaggagttgtatttcgtccagttactctgcaggcctgataaaatccatgtggtttcactcgtccagagtcgttgcccacaaacacttgcaacactacaggttcattatggccttccagctttactgtaggaaagccttgctgtgttctatctttcactgagccacggctgccctcagtcaggtaccgagctcggtgctgtgtctcaggttgtacaactatcttcagctcctttccctcacttttaacaggatattgtccacacaacatagggctcttctttactccagttcctttttggttttccaatgttccatttcccgcttttgagttgcctttgttgtccgtggtaagctgagaaagcacatagtgaggtgctttggcactgtcggcatcaaatatatccatattagattcttcacaatctcgtcgtttgacccccggcctctgctttggatttcgttttcgtgatttacgaggtacctcagtgttatcattgtaggaactggtgctcatgttactgaagttggagggggaatcctccatccacatactgcagctctgctcagattccaatccacacccctcatcctggcaggacatccgactgttatccagcaagtcctcaggtggtggtgagatgtacaagactgtgtgcctcttcggtgttgatggatgctgctgaactgtgttactggttaactgcttttcacttacccctctgttacttacccccacggctgaggagcagctctccacttgcatagccttgctgtcggtgactgaggtagaataaatggtagggctggaagaggtggtaaaggagctgcaagcaccgcccatggaggaagaggagggagctgaagaagcatcagcagcaacaacagctggaggaggcgagcctgcctcaccaccgcttgtctgactcattgatgctacagatgtttctctagatggaggtaactgtaactcctttgggagaagatcatagacagattcttccaatagtccagctctatgaaaattctgtgatgggtgtaacttcagagaatctcgcgagtagagggacttgggcgattccaggtctaggtccgcgctgagcaatgagatgaagtccgagggcatcgcagctcgacccagcccggcccgagggcagcgggagggggggagcggcggtggcggcggcacctcctctccgggaccgcgggcaccgaaccgggggcggcgacgcgagggcggctgccgctgcctcctcctcgagggtagtgacttccactgggccgaggaccgaggaaacgatggcgaggtggagggggaactccacggggactgattctcggtgaccaggagaggggttcaggacggggaaggggaagggggagagccaaagggtccgtttcgtgtttctcctcagcgaaaactgacggtcgccgccaccgccgccgccgctgacaggaatct

SEQ ID NO: 10602 - RNA, 4163 nt, Homo sapiens
  source 1..4163: mol_type = other RNA
cggcccgggctgctgctgttcctgggatggagagttactctgcatggcaactattgagtgctgtgactggaacatggttccttgttggctttgaggcattggattaggtggaagggagcccagggccacctgaggctgaaataaaccctgctgcgggggttgtgcctgttcttgggaaagcataggagtctggatgtgtgatattggagcttgctgttggaaagcagcttgttgttcactgtttgatgttgactgaagtggagaaattgagttcggtgctgcaaaaaatgcttcttgggctactgtgttagtctgaagattattcatgggactctgggaaagaaatatgttggttgactgctggtcttgaggaactgaagagccctgtaacacagcaatggtactttgagagtgaaacattggaggctgcatttgttcagaggaggttgtagaagtctgactgtggacaataggatttggactatgaaagagagaaccttgagtttcctgggaaaggttctgagcatcggcaataggattttgaggatgaaaaagttgggcctgtgaatgagaagactgctgcaaaaaatttccagattgaagtgacatcatctcattcccttgctggaataaaccattaccttgttgttgggtaccactattctgaacactcatcatactttttgtggatgaaaaaaggttaacttgaggttgattgtccccactatgttgcatttggaccatggtctgaaagacactgttctgaatctgttttgcttgtgttccagtttcttctccatctcctgaacttgatgtctgaaacatggtagtgccaggggttgcaacctgctgtgtggtagttgtagaagtttcatttccagaaactgcaggaggagaagaaaacaattcacactgcatttgcatatcctcattggtagacaatgcactcatcatgtgagaagtctgctggtaaactggcgattgctgaaggtttccatttgctgaagcagttgaagggaataactctgactgaatctgggcagctgcctggcagatactctgttgcatctccatcaccattgcggctgaagattccatcacttgctgttgctgctgctgctgctgctgttgattagataacgtgttttcagactgtggatgaacactttcagctcttccaggtaataaattatctggtctggtatggactgttggctctgttgaggaaaacattccagggcttacaccactctgaatttgactgacttgttgaaaaatatctgcactaagctgctcttgaacattctcattaccatctggagcagaaaataaaactgaagataactgctgctgtgcctctaaaacttgttggaccaagtcaacacttccactgctgccactagcagtactgcctgtgaaactccctgcttgcagctgctgaatagtattctgaagctgactcacactatttggtgatggaaaaatatttgatgaaatctgctgctgtaaagtctgtgcttgttcttgtagtggtgactgctgctgttgttgtgatgcctcagtcagttgtgacaaattaaccactgtaccatctgactgtaatatctctctagactgagtttctcttgtctgaaactgtgtagcctgctgcaatagtgcatcgctgttgggcagctgactagaagcagaaactgctggaaaagtaccaggctgtgagatgtcctgggtttgaatagttgtcagggtctctgggttgtatgccttgggctgaatctgctgctgtttttcattttcagaaggtaggtgggaagatgatggtgatgaaaaagagccatttcctgctatgtttgagatgttttctaatgtttgctgagttgatccaacagactttgtagtcttaaaaatagtggaagatcttttttctgctgttacttccattggagtaacatcttcactcttaatcatactgcttggtatgagtggagtcatcagggcattagggataatatttaccttatctaaattacatccagtagttttcattgctttcatggcctcttcaaaagagcaaggtcttgctggactagatatttccttcttcacatttacattcaaagcaccagctgctgctgggtctggagtgtaagtgaatggttgaacatcatgagatcttccagcatttgtcactacatatattcccactgacacaggcaaagttatatgttggtcatgatagggaggaaccttcacaataagatgattctgatgaaatagttccatatcaatttcagcttctgacttccaagagttttcatcagaaacattttcttggaaaataactttagttcctttcagaaagttcttgccgattaaaaacacttcttcttctcctttcactgaacagctatgcaagcttttctttaagatttctggcactcctgctggctgagtacacaaaattggagaagagggtgtttgcagtgtcaaagtggagccatctttcctcatgatattaactcgaaaaaccaatctggcacgagtgcttttcttcttggaaccagcaattcctattctggcttcgacatcagcattcctcaatttcaatatccctacgcagtccaccgccagtgtcatgttgttgctaggatcaaggccgacttctataacagtagtgccttcaatgtccacttctttgcaaggagttgtatttcgtccagttactctgcaggcctgataaaatccatgtggtttcactcgtccagagtcgttgcccacaaacacttgcaacactacaggttcattatggccttccagctttactgtaggaaagccttgctgtgttctatctttcactgagccacggctgccctcagtcaggtaccgagctcggtgctgtgtctcaggttgtacaactatcttcagctcctttccctcacttttaacaggatattgtccacacaacatagggctcttctttactccagttcctttttggttttccaatgttccatttcccgcttttgagttgcctttgttgtccgtggtaagctgagaaagcacatagtgaggtgctttggcactgtcggcatcaaatatatccatattagattcttcacaatctcgtcgtttgacccccggcctctgctttggatttcgttttcgtgatttacgaggtacctcagtgttatcattgtaggaactggtgctcatgttactgaagttggagggggaatcctccatccacatactgcagctctgctcagattccaatccacacccctcatcctggcaggacatccgactgttatccagcaagtcctcaggtggtggtgagatgtacaagactgtgtgcctcttcggtgttgatggatgctgctgaactgtgttactggttaactgcttttcacttacccctctgttacttacccccacggctgaggagcagctctccacttgcatagccttgctgtcggtgactgaggtagaataaatggtagggctggaagaggtggtaaaggagctgcaagcaccgcccatggaggaagaggagggagctgaagaagcatctatgaagcagagaactacaggtcatttttaatgcagacactccctgcttcagaggcaaatccagcagcaacaacagctggaggaggcgagcctgcctcaccaccgcttgtctgactcattgatgctacagatgtttctctagatggaggtaactgtaactcctttgggagaagatcatagacagattctcgcgagtagagggacttgggcgattccaggtctaggtccgcgctgagcaatgagatgaagtccgagggcatcgcagctcgacccagcccggcccgagggcagcgggagggggggagcggcggtggcggcggcacctcctctccgggaccgcgggcaccgaaccgggggcggcgacgcgagggcggctgccgctgcctcctcctcgagggtagtgacttccactgggccgaggaccgaggaaacgatggcgaggtggagggggaactccacggggactgattctcggtgaccaggagaggggttcaggacggggaaggggaagggggagagccaaagggtccgtttcgtgtttctcctcagcgaaaactgacggtcgccgccaccgccgccgccgctgacaggaatct

SEQ ID NO: 10603 - RNA, 4217 nt, Homo sapiens
  source 1..4217: mol_type = other RNA
cggcccgggctgctgctgttcctgggatggagagttactctgcatggcaactattgagtgctgtgactggaacatggttccttgttggctttgaggcattggattaggtggaagggagcccagggccacctgaggctgaaataaaccctgctgcgggggttgtgcctgttcttgggaaagcataggagtctggatgtgtgatattggagcttgctgttggaaagcagcttgttgttcactgtttgatgttgactgaagtggagaaattgagttcggtgctgcaaaaaatgcttcttgggctactgtgttagtctgaagattattcatgggactctgggaaagaaatatgttggttgactgctggtcttgaggaactgaagagccctgtaacacagcaatggtactttgagagtgaaacattggaggctgcatttgttcagaggaggttgtagaagtctgactgtggacaataggatttggactatgaaagagagaaccttgagtttcctgggaaaggttctgagcatcggcaataggattttgaggatgaaaaagttgggcctgtgaatgagaagactgctgcaaaaaatttccagattgaagtgacatcatctcattcccttgctggaataaaccattaccttgttgttgggtaccactattctgaacactcatcatactttttgtggatgaaaaaaggttaacttgaggttgattgtccccactatgttgcatttggaccatggtctgaaagacactgttctgaatctgttttgcttgtgttccagtttcttctccatctcctgaacttgatgtctgaaacatggtagtgccaggggttgcaacctgctgtgtggtagttgtagaagtttcatttccagaaactgcaggaggagaagaaaacaattcacactgcatttgcatatcctcattggtagacaatgcactcatcatgtgagaagtctgctggtaaactggcgattgctgaaggtttccatttgctgaagcagttgaagggaataactctgactgaatctgggcagctgcctggcagatactctgttgcatctccatcaccattgcggctgaagattccatcacttgctgttgctgctgctgctgctgctgttgattagataacgtgttttcagactgtggatgaacactttcagctcttccaggtaataaattatctggtctggtatggactgttggctctgttgaggaaaacattccagggcttacaccactctgaatttgactgacttgttgaaaaatatctgcactaagctgctcttgaacattctcattaccatctggagcagaaaataaaactgaagataactgctgctgtgcctctaaaacttgttggaccaagtcaacacttccactgctgccactagcagtactgcctgtgaaactccctgcttgcagctgctgaatagtattctgaagctgactcacactatttggtgatggaaaaatatttgatgaaatctgctgctgtaaagtctgtgcttgttcttgtagtggtgactgctgctgttgttgtgatgcctcagtcagttgtgacaaattaaccactgtaccatctgactgtaatatctctctagactgagtttctcttgtctgaaactgtgtagcctgctgcaatagtgcatcgctgttgggcagctgactagaagcagaaactgctggaaaagtaccaggctgtgagatgtcctgggtttgaatagttgtcagggtctctgggttgtatgccttgggctgaatctgctgctgtttttcattttcagaaggtaggtgggaagatgatggtgatgaaaaagagccatttcctgctatgtttgagatgttttctaatgtttgctgagttgatccaacagactttgtagtcttaaaaatagtggaagatcttttttctgctgttacttccattggagtaacatcttcactcttaatcatactgcttggtatgagtggagtcatcagggcattagggataatatttaccttatctaaattacatccagtagttttcattgctttcatggcctcttcaaaagagcaaggtcttgctggactagatatttccttcttcacatttacattcaaagcaccagctgctgctgggtctggagtgtaagtgaatggttgaacatcatgagatcttccagcatttgtcactacatatattcccactgacacaggcaaagttatatgttggtcatgatagggaggaaccttcacaataagatgattctgatgaaatagttccatatcaatttcagcttctgacttccaagagttttcatcagaaacattttcttggaaaataactttagttcctttcagaaagttcttgccgattaaaaacacttcttcttctcctttcactgaacagctatgcaagcttttctttaagatttctggcactcctgctggctgagtacacaaaattggagaagagggtgtttgcagtgtcaaagtggagccatctttcctcatgatattaactcgaaaaaccaatctggcacgagtgcttttcttcttggaaccagcaattcctattctggcttcgacatcagcattcctcaatttcaatatccctacgcagtccaccgccagtgtcatgttgttgctaggatcaaggccgacttctataacagtagtgccttcaatgtccacttctttgcaaggagttgtatttcgtccagttactctgcaggcctgataaaatccatgtggtttcactcgtccagagtcgttgcccacaaacacttgcaacactacaggttcattatggccttccagctttactgtaggaaagccttgctgtgttctatctttcactgagccacggctgccctcagtcaggtaccgagctcggtgctgtgtctcaggttgtacaactatcttcagctcctttccctcacttttaacaggatattgtccacacaacatagggctcttctttactccagttcctttttggttttccaatgttccatttcccgcttttgagttgcctttgttgtccgtggtaagctgagaaagcacatagtgaggtgctttggcactgtcggcatcaaatatatccatattagattcttcacaatctcgtcgtttgacccccggcctctgctttggatttcgttttcgtgatttacgaggtacctcagtgttatcattgtaggaactggtgctcatgttactgaagttggagggggaatcctccatccacatactgcagctctgctcagattccaatccacacccctcatcctggcaggacatccgactgttatccagcaagtcctcaggtggtggtgagatgtacaagactgtgtgcctcttcggtgttgatggatgctgctgaactgtgttactggttaactgcttttcacttacccctctgttacttacccccacggctgaggagcagctctccacttgcatagccttgctgtcggtgactgaggtagaataaatggtagggctggaagaggtggtaaaggagctgcaagcaccgcccatggaggaagaggagggagctgaagaagcatctatgaagcagagaactacaggtcatttttaatgcagacactccctgcttcagaggcaaatccagcagcaacaacagctggaggaggcgagcctgcctcaccaccgcttgtctgactcattgatgctacagatgtttctctagatggaggtaactgtaactcctttgggagaagatcatagacagattcttccaatagtccagctctatgaaaattctgtgatgggtgtaacttcagagaatctcgcgagtagagggacttgggcgattccaggtctaggtccgcgctgagcaatgagatgaagtccgagggcatcgcagctcgacccagcccggcccgagggcagcgggagggggggagcggcggtggcggcggcacctcctctccgggaccgcgggcaccgaaccgggggcggcgacgcgagggcggctgccgctgcctcctcctcgagggtagtgacttccactgggccgaggaccgaggaaacgatggcgaggtggagggggaactccacggggactgattctcggtgaccaggagaggggttcaggacggggaaggggaagggggagagccaaagggtccgtttcgtgtttctcctcagcgaaaactgacggtcgccgccaccgccgccgccgctgacaggaatct

SEQ ID NO: 10604 - RNA, 4290 nt, Homo sapiens
  source 1..4290: mol_type = other RNA
cggcccgggctgctgctgttcctgggatggagagttactctgcatggcaactattgagtgctgtgactggaacatggttccttgttggctttgaggcattggattaggtggaagggagcccagggccacctgaggctgaaataaaccctgctgcgggggttgtgcctgttcttgggaaagcataggagtctggatgtgtgatattggagcttgctgttggaaagcagcttgttgttcactgtttgatgttgactgaagtggagaaattgagttcggtgctgcaaaaaatgcttcttgggctactgtgttagtctgaagattattcatgggactctgggaaagaaatatgttggttgactgctggtcttgaggaactgaagagccctgtaacacagcaatggtactttgagagtgaaacattggaggctgcatttgttcagaggaggttgtagaagtctgactgtggacaataggatttggactatgaaagagagaaccttgagtttcctgggaaaggttctgagcatcggcaataggattttgaggatgaaaaagttgggcctgtgaatgagaagactgctgcaaaaaatttccagattgaagtgacatcatctcattcccttgctggaataaaccattaccttgttgttgggtaccactattctgaacactcatcatactttttgtggatgaaaaaaggttaacttgaggttgattgtccccactatgttgcatttggaccatggtctgaaagacactgttctgaatctgttttgcttgtgttccagtttcttctccatctcctgaacttgatgtctgaaacatggtagtgccaggggttgcaacctgctgtgtggtagttgtagaagtttcatttccagaaactgcaggaggagaagaaaacaattcacactgcatttgcatatcctcattggtagacaatgcactcatcatgtgagaagtctgctggtaaactggcgattgctgaaggtttccatttgctgaagcagttgaagggaataactctgactgaatctgggcagctgcctggcagatactctgttgcatctccatcaccattgcggctgaagattccatcacttgctgttgctgctgctgctgctgctgttgattagataacgtgttttcagactgtggatgaacactttcagctcttccaggtaataaattatctggtctggtatggactgttggctctgttgaggaaaacattccagggcttacaccactctgaatttgactgacttgttgaaaaatatctgcactaagctgctcttgaacattctcattaccatctggagcagaaaataaaactgaagataactgctgctgtgcctctaaaacttgttggaccaagtcaacacttccactgctgccactagcagtactgcctgtgaaactccctgcttgcagctgctgaatagtattctgaagctgactcacactatttggtgatggaaaaatatttgatgaaatctgctgctgtaaagtctgtgcttgttcttgtagtggtgactgctgctgttgttgtgatgcctcagtcagttgtgacaaattaaccactgtaccatctgactgtaatatctctctagactgagtttctcttgtctgaaactgtgtagcctgctgcaatagtgcatcgctgttgggcagctgactagaagcagaaactgctggaaaagtaccaggctgtgagatgtcctgggtttgaatagttgtcagggtctctgggttgtatgccttgggctgaatctgctgctgtttttcattttcagaaggtaggtgggaagatgatggtgatgaaaaagagccatttcctgctatgtttgagatgttttctaatgtttgctgagttgatccaacagactttgtagtcttaaaaatagtggaagatcttttttctgctgttacttccattggagtaacatcttcactcttaatcatactgcttggtatgagtggagtcatcagggcattagggataatatttaccttatctaaattacatccagtagttttcattgctttcatggcctcttcaaaagagcaaggtcttgctggactagatatttccttcttcacatttacattcaaagcaccagctgctgctgggtctggagtgtaagtgaatggttgaacatcatgagatcttccagcatttgtcactacatatattcccactgacacaggcaaagttatatgttggtcatgatagggaggaaccttcacaataagatgattctgatgaaatagttccatatcaatttcagcttctgacttccaagagttttcatcagaaacattttcttggaaaataactttagttcctttcagaaagttcttgccgattaaaaacacttcttcttctcctttcactgaacagctatgcaagcttttctttaagatttctggcactcctgctggctgagtacacaaaattggagaagagggtgtttgcagtgtcaaagtggagccatctttcctcatgatattaactcgaaaaaccaatctggcacgagtgcttttcttcttggaaccagcaattcctattctggcttcgacatcagcattcctcaatttcaatatccctacgcagtccaccgccagtgtcatgttgttgctaggatcaaggccgacttctataacagtagtgccttcaatgtccacttctttgcaaggagttgtatttcgtccagttactctgcaggcctgataaaatccatgtggtttcactcgtccagagtcgttgcccacaaacacttgcaacactacaggttcattatggccttccagctttactgtaggaaagccttgctgtgttctatctttcactgagccacggctgccctcagtcaggtaccgagctcggtgctgtgtctcaggttgtacaactatcttcagctcctttccctcacttttaacaggatattgtccacacaacatagggctcttctttactccagttcctttttggttttccaatgttccatttcccgcttttgagttgcctttgttgtccgtggtaagctgagaaagcacatagtgaggtgctttggcactgtcggcatcaaatatatccatattagattcttcacaatctcgtcgtttgacccccggcctctgctttggatttcgttttcgtgatttacgaggtacctcagtgttatcattgtaggaactggtgctcatgttactgaagttggagggggaatcctccatccacatactgcagctctgctcagattccaatccacacccctcatcctggcaggacatccgactgttatccagcaagtcctcaggtggtggtgagatgtacaagactgtgtgcctcttcggtgttgatggatgctgctgaactgtgttactggttaactgcttttcacttacccctctgttacttacccccacggctgaggagcagctctccacttgcatagccttgctgtcggtgactgaggtagaataaatggtagggctggaagaggtggtaaaggagctgcaagcaccgcccatggaggaagaggagggagctgaagaagcatctatgaagcagagaactacaggtcatttttaatgcagacactccctgcttcagaggcaaatccctttttaaatctaaggatcatgcacatgagaatgcagagtatgaacatctcagggatcccagcagcaacaacagctggaggaggcgagcctgcctcaccaccgcttgtctgactcattgatgctacagatgtttctctagatggaggtaactgtaactcctttgggagaagatcatagacagattcttccaatagtccagctctatgaaaattctgtgatgggtgtaacttcagagaatctcgcgagtagagggacttgggcgattccaggtctaggtccgcgctgagcaatgagatgaagtccgagggcatcgcagctcgacccagcccggcccgagggcagcgggagggggggagcggcggtggcggcggcacctcctctccgggaccgcgggcaccgaaccgggggcggcgacgcgagggcggctgccgctgcctcctcctcgagggtagtgacttccactgggccgaggaccgaggaaacgatggcgaggtggagggggaactccacggggactgattctcggtgaccaggagaggggttcaggacggggaaggggaagggggagagccaaagggtccgtttcgtgtttctcctcagcgaaaactgacggtcgccgccaccgccgccgccgctgacaggaatctgagccccgccccc

SEQ ID NO: 10605 - RNA, 4450 nt, Homo sapiens
  source 1..4450: mol_type = other RNA
cggcccgggctgctgctgttcctgggatggagagttactctgcatggcaactattgagtgctgtgactggaacatggttccttgttggctttgaggcattggattaggtggaagggagcccagggccacctgaggctgaaataaaccctgctgcgggggttgtgcctgttcttgggaaagcataggagtctggatgtgtgatattggagcttgctgttggaaagcagcttgttgttcactgtttgatgttgactgaagtggagaaattgagttcggtgctgcaaaaaatgcttcttgggctactgtgttagtctgaagattattcatgggactctgggaaagaaatatgttggttgactgctggtcttgaggaactgaagagccctgtaacacagcaatggtactttgagagtgaaacattggaggctgcatttgttcagaggaggttgtagaagtctgactgtggacaataggatttggactatgaaagagagaaccttgagtttcctgggaaaggttctgagcatcggcaataggattttgaggatgaaaaagttgggcctgtgaatgagaagactgctgcaaaaaatttccagattgaagtgacatcatctcattcccttgctggaataaaccattaccttgttgttgggtaccactattctgaacactcatcatactttttgtggatgaaaaaaggttaacttgaggttgattgtccccactatgttgcatttggaccatggtctgaaagacactgttctgaatctgttttgcttgtgttccagtttcttctccatctcctgaacttgatgtctgaaacatggtagtgccaggggttgcaacctgctgtgtggtagttgtagaagtttcatttccagaaactgcaggaggagaagaaaacaattcacactgcatttgcatatcctcattggtagacaatgcactcatcatgtgagaagtctgctggtaaactggcgattgctgaaggtttccatttgctgaagcagttgaagggaataactctgactgaatctgggcagctgcctggcagatactctgttgcatctccatcaccattgcggctgaagattccatcacttgctgttgctgctgctgctgctgctgttgattagataacgtgttttcagactgtggatgaacactttcagctcttccaggtaataaattatctggtctggtatggactgttggctctgttgaggaaaacattccagggcttacaccactctgaatttgactgacttgttgaaaaatatctgcactaagctgctcttgaacattctcattaccatctggagcagaaaataaaactgaagataactgctgctgtgcctctaaaacttgttggaccaagtcaacacttccactgctgccactagcagtactgcctgtgaaactccctgcttgcagctgctgaatagtattctgaagctgactcacactatttggtgatggaaaaatatttgatgaaatctgctgctgtaaagtctgtgcttgttcttgtagtggtgactgctgctgttgttgtgatgcctcagtcagttgtgacaaattaaccactgtaccatctgactgtaatatctctctagactgagtttctcttgtctgaaactgtgtagcctgctgcaatagtgcatcgctgttgggcagctgactagaagcagaaactgctggaaaagtaccaggctgtgagatgtcctgggtttgaatagttgtcagggtctctgggttgtatgccttgggctgaatctgctgctgtttttcattttcagaaggtaggtgggaagatgatggtgatgaaaaagagccatttcctgctatgtttgagatgttttctaatgtttgctgagttgatccaacagactttgtagtcttaaaaatagtggaagatcttttttctgctgttacttccattggagtaacatcttcactcttaatcatactgcttggtatgagtggagtcatcagggcattagggataatatttaccttatctaaattacatccagtagttttcattgctttcatggcctcttcaaaagagcaaggtcttgctggactagatatttccttcttcacatttacattcaaagcaccagctgctgctgggtctggagtgtaagtgaatggttgaacatcatgagatcttccagcatttgtcactacatatattcccactgacacaggcaaagttatatgttggtcatgatagggaggaaccttcacaataagatgattctgatgaaatagttccatatcaatttcagcttctgacttccaagagttttcatcagaaacattttcttggaaaataactttagttcctttcagaaagttcttgccgattaaaaacacttcttcttctcctttcactgaacagctatgcaagcttttctttaagatttctggcactcctgctggctgagtacacaaaattggagaagagggtgtttgcagtgtcaaagtggagccatctttcctcatgatattaactcgaaaaaccaatctggcacgagtgcttttcttcttggaaccagcaattcctattctggcttcgacatcagcattcctcaatttcaatatccctacgcagtccaccgccagtgtcatgttgttgctaggatcaaggccgacttctataacagtagtgccttcaatgtccacttctttgcaaggagttgtatttcgtccagttactctgcaggcctgataaaatccatgtggtttcactcgtccagagtcgttgcccacaaacacttgcaacactacaggttcattatggccttccagctttactgtaggaaagccttgctgtgttctatctttcactgagccacggctgccctcagtcaggtaccgagctcggtgctgtgtctcaggttgtacaactatcttcagctcctttccctcacttttaacaggatattgtccacacaacatagggctcttctttactccagttcctttttggttttccaatgttccatttcccgcttttgagttgcctttgttgtccgtggtaagctgagaaagcacatagtgaggtgctttggcactgtcggcatcaaatatatccatattagattcttcacaatctcgtcgtttgacccccggcctctgctttggatttcgttttcgtgatttacgaggtacctcagtgttatcattgtaggaactggtgctcatgttactgaagttggagggggaatcctccatccacatactgcagctctgctcagattccaatccacacccctcatcctggcaggacatccgactgttatccagcaagtcctcaggtggtggtgagatgtacaagactgtgtgcctcttcggtgttgatggatgctgctgaactgtgttactggttaactgcttttcacttacccctctgttacttacccccacggctgaggagcagctctccacttgcatagccttgctgtcggtgactgaggtagaataaatggtagggctggaagaggtggtaaaggagctgcaagcaccgcccatggaggaagaggagggagctgaagaagcatctatgaagcagagaactacaggtcatttttaatgcagacactccctgcttcagaggcaaatcctataccctgggtgagattggatgggttaagtgtctctggcactatttgtcttcactattgacagacactgtcacacaacccaccacacgatgcctgtctctgaatggcgaagctagaatgcaagttaagtgtattaatagaaaaaacaactagcatcccagcatataaaataagcattccagattattaaaaaaacaaaaattgtagggctgatcatttacatgattaaaacagtttcaatctcccatttgtacttttcccacccaacatacgtttacatgttaaaataagcaatgttttaaaatgaacttcaaaaaatttaattattaacctctgaatgcatgtggggaaatttcttagacaaaatttttgtgaactcttattcaccaatttgttctgtttatagatgctctctaatccataagccagaattctctctttcaggtgtttttcaggctgttcccttacccaaactcttttgaagcgtggaagaagatatgttctgagcaatgcacttacactgtaaaaaaacctatattttagcagcaaaataacctttccatttttcagaccacactgactcctacatacttctttatactccccttaaaaaggataccaatttatacttttaatgatacatgctactttgtataatatgtttgatcctagaggctctatttttttaaaaaaaataatgagcactactgctgaagctgaagggtttgtttctgatttattgcagacatctttttcttctccagttcatcaaattgccattcagggttctaatgttataaaacaattactctccagttttt

SEQ ID NO: 10606 - RNA, 3250 nt, Homo sapiens
  source 1..3250: mol_type = other RNA
cggcccgggctgctgctgttcctgggatggagagttactctgcatggcaactattgagtgctgtgactggaacatggttccttgttggctttgaggcattggattaggtggaagggagcccagggccacctgaggctgaaataaaccctgctgcgggggttgtgcctgttcttgggaaagcataggagtctggatgtgtgatattggagcttgctgttggaaagcagcttgttgttcactgtttgatgttgactgaagtggagaaattgagttcggtgctgcaaaaaatgcttcttgggctactgtgttagtctgaagattattcatgggactctgggaaagaaatatgttggttgactgctggtcttgaggaactgaagagccctgtaacacagcaatggtactttgagagtgaaacattggaggctgcatttgttcagaggaggttgtagaagtctgactgtggacaataggatttggactatgaaagagagaaccttgagtttcctgggaaaggttctgagcatcggcaataggattttgaggatgaaaaagttgggcctgtgaatgagaagactgctgcaaaaaatttccagattgaagtgacatcatctcattcccttgctggaataaaccattaccttgttgttgggtaccactattctgaacactcatcatactttttgtggatgaaaaaaggttaacttgaggttgattgtccccactatgttgcatttggaccatggtctgaaagacactgttctgaatctgttttgcttgtgttccagtttcttctccatctcctgaacttgatgtctgaaacatggtagtgccaggggttgcaacctgctgtgtggtagttgtagaagtttcatttccagaaactgcaggaggagaagaaaacaattcacactgcatttgcatatcctcattggtagacaatgcactcatcatgtgagaagtctgctggtaaactggcgattgctgaaggtttccatttgctgaagcagttgaagggaataactctgactgaatctgggcagctgcctggcagatactctgttgcatctccatcaccattgcggctgaagattccatcacttgctgttgctgctgctgctgctgctgttgattagataacgtgttttcagactgtggatgaacactttcagctcttccaggtaataaattatctggtctggtatggactgttggctctgttgaggaaaacattccagggcttacaccactctgaatttgactgacttgttgaaaaatatctgcactaagctgctcttgaacattctcattaccatctggagcagaaaataaaactgaagataactgctgctgtgcctctaaaacttgttggaccaagtcaacacttccactgctgccactagcagtactgcctgtgaaactccctgcttgcagctgctgaatagtattctgaagctgactcacactatttggtgatggaaaaatatttgatgaaatctgctgctgtaaagtctgtgcttgttcttgtagtggtgactgctgctgttgttgtgatgcctcagtcagttgtgacaaattaaccactgtaccatctgactgtaatatctctctagactgagtttctcttgtctgaaactgtgtagcctgctgcaatagtgcatcgctgttgggcagctgactagaagcagaaactgctggaaaagtaccaggctgtgagatgtcctgggtttgaatagttgtcagggtctctgggttgtatgccttgggctgaatctgctgctgtttttcattttcagaaggtaggtgggaagatgatggtgatgaaaaagagccatttcctgctatgtttgagatgttttctaatgtttgctgagttgatccaacagactttgtagtcttaaaaatagtggaagatcttttttctgctgttacttccattggagtaacatcttcactcttaatcatactgcttggtatgagtggagtcatcagggcattagggataatatttaccttatctaaattacatccagtagttttcattgctttcatggcctcttcaaaagagcaaggtcttgctggactagatatttccttcttcacatttacattcaaagcaccagctgctgctgggtctggagtgtaagtgaatggttgaacatcatgagatcttccagcatttgtcactacatatattcccactgacacaggcaaagttatatgttggtcatgatagggaggaaccttcacaataagatgattctgatgaaatagttccatatcaatttcagcttctgacttccaagagttttcatcagaaacattttcttggaaaataactttagttcctttcagaaagttcttgccgattaaaaacacttcttcttctcctttcactgaacagctatgcaagcttttctttaagatttctggcactcctgctggctgagtacacaaaattggagaagagggtgtttgcagtgtcaaagtggagccatctttcctcatgatattaactcgaaaaaccaatctggcacgagtgcttttcttcttggaaccagcaattcctattctggcttcgacatcagcattcctcaatttcaatatccctacgcagtccaccgccagtgtcatgttgttgctaggatcaaggccgacttctataacagtagtgccttcaatgtccacttctttgcaaggagttgtatttcgtccagttactctgcaggcctgataaaatccatgtggtttcactcgtccagagtcgttgcccacaaacacttgcaacactacaggttcattatggccttccagctttactgtaggaaagccttgctgtgttctatctttcactgagccacggctgccctcagtcaggtaccgagctcggtgctgtgtctcaggttgtacaactatcttcagctcctttccctcacttttaacaggatattgtccacacaacatagggctcttctttactccagttcctttttggttttccaatgttccccacggctgaggagcagctctccacttgcatagccttgctgtcggtgactgaggtagaataaatggtagggctggaagaggtggtaaaggagctgcaagcaccgcccatggaggaagaggagggagctgaagaagcatcagcagcaacaacagctggaggaggcgagcctgcctcaccaccgcttgtctgactcattgatgctacagatgtttctctagatggaggtaactgtaactcctt

SEQ ID NO: 10607 - RNA, 3302 nt, Homo sapiens
  source 1..3302: mol_type = other RNA
cggcccgggctgctgctgttcctgggatggagagttactctgcatggcaactattgagtgctgtgactggaacatggttccttgttggctttgaggcattggattaggtggaagggagcccagggccacctgaggctgaaataaaccctgctgcgggggttgtgcctgttcttgggaaagcataggagtctggatgtgtgatattggagcttgctgttggaaagcagcttgttgttcactgtttgatgttgactgaagtggagaaattgagttcggtgctgcaaaaaatgcttcttgggctactgtgttagtctgaagattattcatgggactctgggaaagaaatatgttggttgactgctggtcttgaggaactgaagagccctgtaacacagcaatggtactttgagagtgaaacattggaggctgcatttgttcagaggaggttgtagaagtctgactgtggacaataggatttggactatgaaagagagaaccttgagtttcctgggaaaggttctgagcatcggcaataggattttgaggatgaaaaagttgggcctgtgaatgagaagactgctgcaaaaaatttccagattgaagtgacatcatctcattcccttgctggaataaaccattaccttgttgttgggtaccactattctgaacactcatcatactttttgtggatgaaaaaaggttaacttgaggttgattgtccccactatgttgcatttggaccatggtctgaaagacactgttctgaatctgttttgcttgtgttccagtttcttctccatctcctgaacttgatgtctgaaacatggtagtgccaggggttgcaacctgctgtgtggtagttgtagaagtttcatttccagaaactgcaggaggagaagaaaacaattcacactgcatttgcatatcctcattggtagacaatgcactcatcatgtgagaagtctgctggtaaactggcgattgctgaaggtttccatttgctgaagcagttgaagggaataactctgactgaatctgggcagctgcctggcagatactctgttgcatctccatcaccattgcggctgaagattccatcacttgctgttgctgctgctgctgctgctgttgattagataacgtgttttcagactgtggatgaacactttcagctcttccaggtaataaattatctggtctggtatggactgttggctctgttgaggaaaacattccagggcttacaccactctgaatttgactgacttgttgaaaaatatctgcactaagctgctcttgaacattctcattaccatctggagcagaaaataaaactgaagataactgctgctgtgcctctaaaacttgttggaccaagtcaacacttccactgctgccactagcagtactgcctgtgaaactccctgcttgcagctgctgaatagtattctgaagctgactcacactatttggtgatggaaaaatatttgatgaaatctgctgctgtaaagtctgtgcttgttcttgtagtggtgactgctgctgttgttgtgatgcctcagtcagttgtgacaaattaaccactgtaccatctgactgtaatatctctctagactgagtttctcttgtctgaaactgtgtagcctgctgcaatagtgcatcgctgttgggcagctgactagaagcagaaactgctggaaaagtaccaggctgtgagatgtcctgggtttgaatagttgtcagggtctctgggttgtatgccttgggctgaatctgctgctgtttttcattttcagaaggtaggtgggaagatgatggtgatgaaaaagagccatttcctgctatgtttgagatgttttctaatgtttgctgagttgatccaacagactttgtagtcttaaaaatagtggaagatcttttttctgctgttacttccattggagtaacatcttcactcttaatcatactgcttggtatgagtggagtcatcagggcattagggataatatttaccttatctaaattacatccagtagttttcattgctttcatggcctcttcaaaagagcaaggtcttgctggactagatatttccttcttcacatttacattcaaagcaccagctgctgctgggtctggagtgtaagtgaatggttgaacatcatgagatcttccagcatttgtcactacatatattcccactgacacaggcaaagttatatgttggtcatgatagggaggaaccttcacaataagatgattctgatgaaatagttccatatcaatttcagcttctgacttccaagagttttcatcagaaacattttcttggaaaataactttagttcctttcagaaagttcttgccgattaaaaacacttcttcttctcctttcactgaacagctatgcaagcttttctttaagatttctggcactcctgctggctgagtacacaaaattggagaagagggtgtttgcagtgtcaaagtggagccatctttcctcatgatattaactcgaaaaaccaatctggcacgagtgcttttcttcttggaaccagcaattcctattctggcttcgacatcagcattcctcaatttcaatatccctacgcagtccaccgccagtgtcatgttgttgctaggatcaaggccgacttctataacagtagtgccttcaatgtccacttctttgcaaggagttgtatttcgtccagttactctgcaggcctgataaaatccatgtggtttcactcgtccagagtcgttgcccacaaacacttgcaacactacaggttcattatggccttccagctttactgtaggaaagccttgctgtgttctatctttcactgagccacggctgccctcagtcaggtaccgagctcggtgctgtgtctcaggttgtacaactatcttcagctcctttccctcacttttaacaggatattgtccacacaacatagggctcttctttactccagttcctttttggttttccaatgttccccacggctgaggagcagctctccacttgcatagccttgctgtcggtgactgaggtagaataaatggtagggctggaagaggtggtaaaggagctgcaagcaccgcccatggaggaagaggagggagctgaagaagcatctatgaagcagagaactacaggtcatttttaatgcagacactccctgcttcagaggcaaatccagcagcaacaacagctggaggaggcgagcctgcctcaccaccgcttgtctgactcattgatgctacagatgtttctctagatggaggtaact

SEQ ID NO: 10608 - RNA, 3872 nt, Homo sapiens
  source 1..3872: mol_type = other RNA
cggcccgggctgctgctgttcctgggatggagagttactctgcatggcaactattgagtgctgtgactggaacatggttccttgttggctttgaggcattggattaggtggaagggagcccagggccacctgaggctgaaataaaccctgctgcgggggttgtgcctgttcttgggaaagcataggagtctggatgtgtgatattggagcttgctgttggaaagcagcttgttgttcactgtttgatgttgactgaagtggagaaattgagttcggtgctgcaaaaaatgcttcttgggctactgtgttagtctgaagattattcatgggactctgggaaagaaatatgttggttgactgctggtcttgaggaactgaagagccctgtaacacagcaatggtactttgagagtgaaacattggaggctgcatttgttcagaggaggttgtagaagtctgactgtggacaataggatttggactatgaaagagagaaccttgagtttcctgggaaaggttctgagcatcggcaataggattttgaggatgaaaaagttgggcctgtgaatgagaagactgctgcaaaaaatttccagattgaagtgacatcatctcattcccttgctggaataaaccattaccttgttgttgggtaccactattctgaacactcatcatactttttgtggatgaaaaaaggttaacttgaggttgattgtccccactatgttgcatttggaccatggtctgaaagacactgttctgaatctgttttgcttgtgttccagtttcttctccatctcctgaacttgatgtctgaaacatggtagtgccaggggttgcaacctgctgtgtggtagttgtagaagtttcatttccagaaactgcaggaggagaagaaaacaattcacactgcatttgcatatcctcattggtagacaatgcactcatcatgtgagaagtctgctggtaaactggcgattgctgaaggtttccatttgctgaagcagttgaagggaataactctgactgaatctgggcagctgcctggcagatactctgttgcatctccatcaccattgcggctgaagattccatcacttgctgttgctgctgctgctgctgctgttgattagataacgtgttttcagactgtggatgaacactttcagctcttccaggtaataaattatctggtctggtatggactgttggctctgttgaggaaaacattccagggcttacaccactctgaatttgactgacttgttgaaaaatatctgcactaagctgctcttgaacattctcattaccatctggagcagaaaataaaactgaagataactgctgctgtgcctctaaaacttgttggaccaagtcaacacttccactgctgccactagcagtactgcctgtgaaactccctgcttgcagctgctgaatagtattctgaagctgactcacactatttggtgatggaaaaatatttgatgaaatctgctgctgtaaagtctgtgcttgttcttgtagtggtgactgctgctgttgttgtgatgcctcagtcagttgtgacaaattaaccactgtaccatctgactgtaatatctctctagactgagtttctcttgtctgaaactgtgtagcctgctgcaatagtgcatcgctgttgggcagctgactagaagcagaaactgctggaaaagtaccaggctgtgagatgtcctgggtttgaatagttgtcagggtctctgggttgtatgccttgggctgaatctgctgctgtttttcattttcagaaggtaggtgggaagatgatggtgatgaaaaagagccatttcctgctatgtttgagatgttttctaatgtttgctgagttgatccaacagactttgtagtcttaaaaatagtggaagatcttttttctgctgttacttccattggagtaacatcttcactcttaatcatactgcttggtatgagtggagtcatcagggcattagggataatatttaccttatctaaattacatccagtagttttcattgctttcatggcctcttcaaaagagcaaggtcttgctggactagatatttccttcttcacatttacattcaaagcaccagctgctgctgggtctggagtgtaagtgaatggttgaacatcatgagatcttccagcatttgtcactacatatattcccactgacacaggcaaagttatatgttggtcatgatagggaggaaccttcacaataagatgattctgatgaaatagttccatatcaatttcagcttctgacttccaagagttttcatcagaaacattttcttggaaaataactttagttcctttcagaaagttcttgccgattaaaaacacttcttcttctcctttcactgaacagctatgcaagcttttctttaagatttctggcactcctgctggctgagtacacaaaattggagaagagggtgtttgcagtgtcaaagtggagccatctttcctcatgatattaactcgaaaaaccaatctggcacgagtgcttttcttcttggaaccagcaattcctattctggcttcgacatcagcattcctcaatttcaatatccctacgcagtccaccgccagtgtcatgttgttgctaggatcaaggccgacttctataacagtagtgccttcaatgtccacttctttgcaaggagttgtatttcgtccagttactctgcaggcctgataaaatccatgtggtttcactcgtccagagtcgttgcccacaaacacttgcaacactacaggttcattatggccttccagctttactgtaggaaagccttgctgtgttctatctttcactgagccacggctgccctcagtcaggtaccgagctcggtgctgtgtctcaggttgtacaactatcttcagctcctttccctcacttttaacaggatattgtccacacaacatagggctcttctttactccagttcctttttggttttccaatgttccccacggctgaggagcagctctccacttgcatagccttgctgtcggtgactgaggtagaataaatggtagggctggaagaggtggtaaaggagctgcaagcaccgcccatggaggaagaggagggagctgaagaagcatctatgaagcagagaactacaggtcatttttaatgcagacactccctgcttcagaggcaaatccctttttaaatctaaggatcatgcacatgagaatgcagagtatgaacatctcagggatcccagcagcaacaacagctggaggaggcgagcctgcctcaccaccgcttgtctgactcattgatgctacagatgtttctctagatggaggtaactgtaactcctttgggagaagatcatagacagattcttccaatagtccagctctatgaaaattctgtgatgggtgtaacttcagagaatctcgcgagtagagggacttgggcgattccaggtctaggtccgcgctgagcaatgagatgaagtccgagggcatcgcagctcgacccagcccggcccgagggcagcgggagggggggagcggcggtggcggcggcacctcctctccgggaccgcgggcaccgaaccgggggcggcgacgcgagggcggctgccgctgcctcctcctcgagggtagtgacttccactgggccgaggaccgaggaaacgatggcgaggtggagggggaactccacggggactgattctcggtgaccaggagaggggttcaggacggggaaggggaagggggagagccaaagggtccgtttcgtgtttctcctcagcgaaaactgacggtcgccgccaccgccgccgccgctgacaggaatctgagccccgcccccg

SEQ ID NO: 10609 - RNA, 4031 nt, Homo sapiens
  source 1..4031: mol_type = other RNA
cggcccgggctgctgctgttcctgggatggagagttactctgcatggcaactattgagtgctgtgactggaacatggttccttgttggctttgaggcattggattaggtggaagggagcccagggccacctgaggctgaaataaaccctgctgcgggggttgtgcctgttcttgggaaagcataggagtctggatgtgtgatattggagcttgctgttggaaagcagcttgttgttcactgtttgatgttgactgaagtggagaaattgagttcggtgctgcaaaaaatgcttcttgggctactgtgttagtctgaagattattcatgggactctgggaaagaaatatgttggttgactgctggtcttgaggaactgaagagccctgtaacacagcaatggtactttgagagtgaaacattggaggctgcatttgttcagaggaggttgtagaagtctgactgtggacaataggatttggactatgaaagagagaaccttgagtttcctgggaaaggttctgagcatcggcaataggattttgaggatgaaaaagttgggcctgtgaatgagaagactgctgcaaaaaatttccagattgaagtgacatcatctcattcccttgctggaataaaccattaccttgttgttgggtaccactattctgaacactcatcatactttttgtggatgaaaaaaggttaacttgaggttgattgtccccactatgttgcatttggaccatggtctgaaagacactgttctgaatctgttttgcttgtgttccagtttcttctccatctcctgaacttgatgtctgaaacatggtagtgccaggggttgcaacctgctgtgtggtagttgtagaagtttcatttccagaaactgcaggaggagaagaaaacaattcacactgcatttgcatatcctcattggtagacaatgcactcatcatgtgagaagtctgctggtaaactggcgattgctgaaggtttccatttgctgaagcagttgaagggaataactctgactgaatctgggcagctgcctggcagatactctgttgcatctccatcaccattgcggctgaagattccatcacttgctgttgctgctgctgctgctgctgttgattagataacgtgttttcagactgtggatgaacactttcagctcttccaggtaataaattatctggtctggtatggactgttggctctgttgaggaaaacattccagggcttacaccactctgaatttgactgacttgttgaaaaatatctgcactaagctgctcttgaacattctcattaccatctggagcagaaaataaaactgaagataactgctgctgtgcctctaaaacttgttggaccaagtcaacacttccactgctgccactagcagtactgcctgtgaaactccctgcttgcagctgctgaatagtattctgaagctgactcacactatttggtgatggaaaaatatttgatgaaatctgctgctgtaaagtctgtgcttgttcttgtagtggtgactgctgctgttgttgtgatgcctcagtcagttgtgacaaattaaccactgtaccatctgactgtaatatctctctagactgagtttctcttgtctgaaactgtgtagcctgctgcaatagtgcatcgctgttgggcagctgactagaagcagaaactgctggaaaagtaccaggctgtgagatgtcctgggtttgaatagttgtcagggtctctgggttgtatgccttgggctgaatctgctgctgtttttcattttcagaaggtaggtgggaagatgatggtgatgaaaaagagccatttcctgctatgtttgagatgttttctaatgtttgctgagttgatccaacagactttgtagtcttaaaaatagtggaagatcttttttctgctgttacttccattggagtaacatcttcactcttaatcatactgcttggtatgagtggagtcatcagggcattagggataatatttaccttatctaaattacatccagtagttttcattgctttcatggcctcttcaaaagagcaaggtcttgctggactagatatttccttcttcacatttacattcaaagcaccagctgctgctgggtctggagtgtaagtgaatggttgaacatcatgagatcttccagcatttgtcactacatatattcccactgacacaggcaaagttatatgttggtcatgatagggaggaaccttcacaataagatgattctgatgaaatagttccatatcaatttcagcttctgacttccaagagttttcatcagaaacattttcttggaaaataactttagttcctttcagaaagttcttgccgattaaaaacacttcttcttctcctttcactgaacagctatgcaagcttttctttaagatttctggcactcctgctggctgagtacacaaaattggagaagagggtgtttgcagtgtcaaagtggagccatctttcctcatgatattaactcgaaaaaccaatctggcacgagtgcttttcttcttggaaccagcaattcctattctggcttcgacatcagcattcctcaatttcaatatccctacgcagtccaccgccagtgtcatgttgttgctaggatcaaggccgacttctataacagtagtgccttcaatgtccacttctttgcaaggagttgtatttcgtccagttactctgcaggcctgataaaatccatgtggtttcactcgtccagagtcgttgcccacaaacacttgcaacactacaggttcattatggccttccagctttactgtaggaaagccttgctgtgttctatctttcactgagccacggctgccctcagtcaggtaccgagctcggtgctgtgtctcaggttgtacaactatcttcagctcctttccctcacttttaacaggatattgtccacacaacatagggctcttctttactccagttcctttttggttttccaatgttccccacggctgaggagcagctctccacttgcatagccttgctgtcggtgactgaggtagaataaatggtagggctggaagaggtggtaaaggagctgcaagcaccgcccatggaggaagaggagggagctgaagaagcatctatgaagcagagaactacaggtcatttttaatgcagacactccctgcttcagaggcaaatcctataccctgggtgagattggatgggttaagtgtctctggcactatttgtcttcactattgacagacactgtcacacaacccaccacacgatgcctgtctctgaatggcgaagctagaatgcaagttaagtgtattaatagaaaaaacaactagcatcccagcatataaaataagcattccagattattaaaaaaacaaaaattgtagggctgatcatttacatgattaaaacagtttcaatctcccatttgtacttttcccacccaacatacgtttacatgttaaaataagcaatgttttaaaatgaacttcaaaaaatttaattattaacctctgaatgcatgtggggaaatttcttagacaaaatttttgtgaactcttattcaccaatttgttctgtttatagatgctctctaatccataagccagaattctctctttcaggtgtttttcaggctgttcccttacccaaactcttttgaagcgtggaagaagatatgttctgagcaatgcacttacactgtaaaaaaacctatattttagcagcaaaataacctttccatttttcagaccacactgactcctacatacttctttatactccccttaaaaaggataccaatttatacttttaatgatacatgctactttgtataatatgtttgatcctagaggctctatttttttaaaaaaaataatgagcactactgctgaagctgaagggtttgtttctgatttattgcagacatctttttcttctccagttcatcaaattgccattcagggttctaatgttataaaacaattactctccagttttt

SEQ ID NO: 10610 - RNA, 4098 nt, Homo sapiens
  source 1..4098: mol_type = other RNA
cggcccgggctgctgctgttcctgggatggagagttactctgcatggcaactattgagtgctgtgactggaacatggttccttgttggctttgaggcattggattaggtggaagggagcccagggccacctgaggctgaaataaaccctgctgcgggggttgtgcctgttcttgggaaagcataggagtctggatgtgtgatattggagcttgctgttggaaagcagcttgttgttcactgtttgatgttgactgaagtggagaaattgagttcggtgctgcaaaaaatgcttcttgggctactgtgttagtctgaagattattcatgggactctgggaaagaaatatgttggttgactgctggtcttgaggaactgaagagccctgtaacacagcaatggtactttgagagtgaaacattggaggctgcatttgttcagaggaggttgtagaagtctgactgtggacaataggatttggactatgaaagagagaaccttgagtttcctgggaaaggttctgagcatcggcaataggattttgaggatgaaaaagttgggcctgtgaatgagaagactgctgcaaaaaatttccagattgaagtgacatcatctcattcccttgctggaataaaccattaccttgttgttgggtaccactattctgaacactcatcatactttttgtggatgaaaaaaggttaacttgaggttgattgtccccactatgttgcatttggaccatggtctgaaagacactgttctgaatctgttttgcttgtgttccagtttcttctccatctcctgaacttgatgtctgaaacatggtagtgccaggggttgcaacctgctgtgtggtagttgtagaagtttcatttccagaaactgcaggaggagaagaaaacaattcacactgcatttgcatatcctcattggtagacaatgcactcatcatgtgagaagtctgctggtaaactggcgattgctgaaggtttccatttgctgaagcagttgaagggaataactctgactgaatctgggcagctgcctggcagatactctgttgcatctccatcaccattgcggctgaagattccatcacttgctgttgctgctgctgctgctgctgttgattagataacgtgttttcagactgtggatgaacactttcagctcttccaggtaataaattatctggtctggtatggactgttggctctgttgaggaaaacattccagggcttacaccactctgaatttgactgacttgttgaaaaatatctgcactaagctgctcttgaacattctcattaccatctggagcagaaaataaaactgaagataactgctgctgtgcctctaaaacttgttggaccaagtcaacacttccactgctgccactagcagtactgcctgtgaaactccctgcttgcagctgctgaatagtattctgaagctgactcacactatttggtgatggaaaaatatttgatgaaatctgctgctgtaaagtctgtgcttgttcttgtagtggtgactgctgctgttgttgtgatgcctcagtcagttgtgacaaattaaccactgtaccatctgactgtaatatctctctagactgagtttctcttgtctgaaactgtgtagcctgctgcaatagtgcatcgctgttgggcagctgactagaagcagaaactgctggaaaagtaccaggctgtgagatgtcctgggtttgaatagttgtcagggtctctgggttgtatgccttgggctgaatctgctgctgtttttcattttcagaaggtaggtgggaagatgatggtgatgaaaaagagccatttcctgctatgtttgagatgttttctaatgtttgctgagttgatccaacagactttgtagtcttaaaaatagtggaagatcttttttctgctgttacttccattggagtaacatcttcactcttaatcatactgcttggtatgagtggagtcatcagggcattagggataatatttaccttatctaaattacatccagtagttttcattgctttcatggcctcttcaaaagagcaaggtcttgctggactagatatttccttcttcacatttacattcaaagcaccagctgctgggtctggagtgtaagtgaatggttgaacatcatgagatcttccagcatttgtcactacatatattcccactgacacaggcaaagttatatgttggtcatgatagggaggaaccttcacaataagatgattctgatgaaatagttccatatcaatttcagcttctgacttccaagagttttcatcagaaacattttcttggaaaataactttagttcctttcagaaagttcttgccgattaaaaacacttcttcttctcctttcactgaacagctatgcaagcttttctttaagatttctggcactcctgctggctgagtacacaaaattggagaagagggtgtttgcagtgtcaaagtggagccatctttcctcatgatattaactcgaaaaaccaatctggcacgagtgcttttcttcttggaaccagcaattcctattctggcttcgacatcagcattcctcaatttcaatatccctacgcagtccaccgccagtgtcatgttgttgctaggatcaaggccgacttctataacagtagtgccttcaatgtccacttctttgcaaggagttgtatttcgtccagttactctgcaggcctgataaaatccatgtggtttcactcgtccagagtcgttgcccacaaacacttgcaacactacaggttcattatggccttccagctttactgtaggaaagccttgctgtgttctatctttcactgagccacggctgccctcagtcaggtaccgagctcggtgctgtgtctcaggttgtacaactatcttcagctcctttccctcacttttaacaggatattgtccacacaacatagggctcttctttactccagttcctttttggttttccaatgttccatttcccgcttttgagttgcctttgttgtccgtggtaagctgagaaagcacatagtgaggtgctttggcactgtcggcatcaaatatatccatattagattcttcacaatctcgtcgtttgacccccggcctctgctttggatttcgttttcgtgatttacgaggtacctcagtgttatcattgtaggaactggtgctcatgttactgaagttggagggggaatcctccatccacatactgcagctctgctcagattccaatccacacccctcatcctggcaggacatccgactgttatccagcaagtcctcaggtggtggtgagatgtacaagactgtgtgcctcttcggtgttgatggatgctgctgaactgtgttactggttaactgcttttcacttacccctctgttacttacccccacggctgaggagcagctctccacttgcatagccttgctgtcggtgactgaggtagaataaatggtagggctggaagaggtggtaaaggagctgcaagcaccgcccatggaggaagaggagggagctgaagaagcatcagcagcaacaacagctggaggaggcgagcctgcctcaccaccgcttgtctgactcattgatgctacagatgtttctctagatggaggtaactgtaactcctttgggagaagatcatagacagattctcgcgagtagagggacttgggcgattccaggtctaggtccgcgctgagcaatgagatgaagtccgagggcatcgcagctcgacccagcccggcccgagggcagcgggagggggggagcggcggtggcggcggcacctcctctccgggaccgcgggcaccgaaccgggggcggcgacgcgagggcggctgccgctgcctcctcctcgagggtagtgacttccactgggccgaggaccgaggaaacgatggcgaggtggagggggaactccacggggactgattctcggtgaccaggagaggggttcaggacggggaaggggaagggggagagccaaagggtccgtttcgtgtttctcctcagcgaaaactgacggtcgccgccaccgccgccgccgctgacaggaatct

SEQ ID NO: 10611 - RNA, 4152 nt, Homo sapiens
  source 1..4152: mol_type = other RNA
cggcccgggctgctgctgttcctgggatggagagttactctgcatggcaactattgagtgctgtgactggaacatggttccttgttggctttgaggcattggattaggtggaagggagcccagggccacctgaggctgaaataaaccctgctgcgggggttgtgcctgttcttgggaaagcataggagtctggatgtgtgatattggagcttgctgttggaaagcagcttgttgttcactgtttgatgttgactgaagtggagaaattgagttcggtgctgcaaaaaatgcttcttgggctactgtgttagtctgaagattattcatgggactctgggaaagaaatatgttggttgactgctggtcttgaggaactgaagagccctgtaacacagcaatggtactttgagagtgaaacattggaggctgcatttgttcagaggaggttgtagaagtctgactgtggacaataggatttggactatgaaagagagaaccttgagtttcctgggaaaggttctgagcatcggcaataggattttgaggatgaaaaagttgggcctgtgaatgagaagactgctgcaaaaaatttccagattgaagtgacatcatctcattcccttgctggaataaaccattaccttgttgttgggtaccactattctgaacactcatcatactttttgtggatgaaaaaaggttaacttgaggttgattgtccccactatgttgcatttggaccatggtctgaaagacactgttctgaatctgttttgcttgtgttccagtttcttctccatctcctgaacttgatgtctgaaacatggtagtgccaggggttgcaacctgctgtgtggtagttgtagaagtttcatttccagaaactgcaggaggagaagaaaacaattcacactgcatttgcatatcctcattggtagacaatgcactcatcatgtgagaagtctgctggtaaactggcgattgctgaaggtttccatttgctgaagcagttgaagggaataactctgactgaatctgggcagctgcctggcagatactctgttgcatctccatcaccattgcggctgaagattccatcacttgctgttgctgctgctgctgctgctgttgattagataacgtgttttcagactgtggatgaacactttcagctcttccaggtaataaattatctggtctggtatggactgttggctctgttgaggaaaacattccagggcttacaccactctgaatttgactgacttgttgaaaaatatctgcactaagctgctcttgaacattctcattaccatctggagcagaaaataaaactgaagataactgctgctgtgcctctaaaacttgttggaccaagtcaacacttccactgctgccactagcagtactgcctgtgaaactccctgcttgcagctgctgaatagtattctgaagctgactcacactatttggtgatggaaaaatatttgatgaaatctgctgctgtaaagtctgtgcttgttcttgtagtggtgactgctgctgttgttgtgatgcctcagtcagttgtgacaaattaaccactgtaccatctgactgtaatatctctctagactgagtttctcttgtctgaaactgtgtagcctgctgcaatagtgcatcgctgttgggcagctgactagaagcagaaactgctggaaaagtaccaggctgtgagatgtcctgggtttgaatagttgtcagggtctctgggttgtatgccttgggctgaatctgctgctgtttttcattttcagaaggtaggtgggaagatgatggtgatgaaaaagagccatttcctgctatgtttgagatgttttctaatgtttgctgagttgatccaacagactttgtagtcttaaaaatagtggaagatcttttttctgctgttacttccattggagtaacatcttcactcttaatcatactgcttggtatgagtggagtcatcagggcattagggataatatttaccttatctaaattacatccagtagttttcattgctttcatggcctcttcaaaagagcaaggtcttgctggactagatatttccttcttcacatttacattcaaagcaccagctgctgggtctggagtgtaagtgaatggttgaacatcatgagatcttccagcatttgtcactacatatattcccactgacacaggcaaagttatatgttggtcatgatagggaggaaccttcacaataagatgattctgatgaaatagttccatatcaatttcagcttctgacttccaagagttttcatcagaaacattttcttggaaaataactttagttcctttcagaaagttcttgccgattaaaaacacttcttcttctcctttcactgaacagctatgcaagcttttctttaagatttctggcactcctgctggctgagtacacaaaattggagaagagggtgtttgcagtgtcaaagtggagccatctttcctcatgatattaactcgaaaaaccaatctggcacgagtgcttttcttcttggaaccagcaattcctattctggcttcgacatcagcattcctcaatttcaatatccctacgcagtccaccgccagtgtcatgttgttgctaggatcaaggccgacttctataacagtagtgccttcaatgtccacttctttgcaaggagttgtatttcgtccagttactctgcaggcctgataaaatccatgtggtttcactcgtccagagtcgttgcccacaaacacttgcaacactacaggttcattatggccttccagctttactgtaggaaagccttgctgtgttctatctttcactgagccacggctgccctcagtcaggtaccgagctcggtgctgtgtctcaggttgtacaactatcttcagctcctttccctcacttttaacaggatattgtccacacaacatagggctcttctttactccagttcctttttggttttccaatgttccatttcccgcttttgagttgcctttgttgtccgtggtaagctgagaaagcacatagtgaggtgctttggcactgtcggcatcaaatatatccatattagattcttcacaatctcgtcgtttgacccccggcctctgctttggatttcgttttcgtgatttacgaggtacctcagtgttatcattgtaggaactggtgctcatgttactgaagttggagggggaatcctccatccacatactgcagctctgctcagattccaatccacacccctcatcctggcaggacatccgactgttatccagcaagtcctcaggtggtggtgagatgtacaagactgtgtgcctcttcggtgttgatggatgctgctgaactgtgttactggttaactgcttttcacttacccctctgttacttacccccacggctgaggagcagctctccacttgcatagccttgctgtcggtgactgaggtagaataaatggtagggctggaagaggtggtaaaggagctgcaagcaccgcccatggaggaagaggagggagctgaagaagcatcagcagcaacaacagctggaggaggcgagcctgcctcaccaccgcttgtctgactcattgatgctacagatgtttctctagatggaggtaactgtaactcctttgggagaagatcatagacagattcttccaatagtccagctctatgaaaattctgtgatgggtgtaacttcagagaatctcgcgagtagagggacttgggcgattccaggtctaggtccgcgctgagcaatgagatgaagtccgagggcatcgcagctcgacccagcccggcccgagggcagcgggagggggggagcggcggtggcggcggcacctcctctccgggaccgcgggcaccgaaccgggggcggcgacgcgagggcggctgccgctgcctcctcctcgagggtagtgacttccactgggccgaggaccgaggaaacgatggcgaggtggagggggaactccacggggactgattctcggtgaccaggagaggggttcaggacggggaaggggaagggggagagccaaagggtccgtttcgtgtttctcctcagcgaaaactgacggtcgccgccaccgccgccgccgctgacaggaatct

SEQ ID NO: 10612 - RNA, 4173 nt, Homo sapiens
  source 1..4173: mol_type = other RNA
cggcccgggctgctgctgttcctgggatggagagttactctgcatggcaactattgagtgctgtgactggaacatggttccttgttggctttgaggcattggattaggtggaagggagcccagggccacctgaggctgaaataaaccctgctgcgggggttgtgcctgttcttgggaaagcataggagtctggatgtgtgatattggagcttgctgttggaaagcagcttgttgttcactgtttgatgttgactgaagtggagaaattgagttcggtgctgcaaaaaatgcttcttgggctactgtgttagtctgaagattattcatgggactctgggaaagaaatatgttggttgactgctggtcttgaggaactgaagagccctgtaacacagcaatggtactttgagagtgaaacattggaggctgcatttgttcagaggaggttgtagaagtctgactgtggacaataggatttggactatgaaagagagaaccttgagtttcctgggaaaggttctgagcatcggcaataggattttgaggatgaaaaagttgggcctgtgaatgagaagactgctgcaaaaaatttccagattgaagtgacatcatctcattcccttgctggaataaaccattaccttgttgttgggtaccactattctgaacactcatcatactttttgtggatgaaaaaaggttaacttgaggttgattgtccccactatgttgcatttggaccatggtctgaaagacactgttctgaatctgttttgcttgtgttccagtttcttctccatctcctgaacttgatgtctgaaacatggtagtgccaggggttgcaacctgctgtgtggtagttgtagaagtttcatttccagaaactgcaggaggagaagaaaacaattcacactgcatttgcatatcctcattggtagacaatgcactcatcatgtgagaagtctgctggtaaactggcgattgctgaaggtttccatttgctgaagcagttgaagggaataactctgactgaatctgggcagctgcctggcagatactctgttgcatctccatcaccattgcggctgaagattccatcacttgctgttgctgctgctgctgctgctgttgattagataacgtgttttcagactgtggatgaacactttcagctcttccaggtaataaattatctggtctggtatggactgttggctctgttgaggaaaacattccagggcttacaccactctgaatttgactgacttgttgaaaaatatctgcactaagctgctcttgaacattctcattaccatctggagcagaaaataaaactgaagataactgctgctgtgcctctaaaacttgttggaccaagtcaacacttccactgctgccactagcagtactgcctgtgaaactccctgcttgcagctgctgaatagtattctgaagctgactcacactatttggtgatggaaaaatatttgatgaaatctgctgctgtaaagtctgtgcttgttcttgtagtggtgactgctgctgttgttgtgatgcctcagtcagttgtgacaaattaaccactgtaccatctgactgtaatatctctctagactgagtttctcttgtctgaaactgtgtagcctgctgcaatagtgcatcgctgttgggcagctgactagaagcagaaactgctggaaaagtaccaggctgtgagatgtcctgggtttgaatagttgtcagggtctctgggttgtatgccttgggctgaatctgctgctgtttttcattttcagaaggtaggtgggaagatgatggtgatgaaaaagagccatttcctgctatgtttgagatgttttctaatgtttgctgagttgatccaacagactttgtagtcttaaaaatagtggaagatcttttttctgctgttacttccattggagtaacatcttcactcttaatcatactgcttggtatgagtggagtcatcagggcattagggataatatttaccttatctaaattacatccagtagttttcattgctttcatggcctcttcaaaagagcaaggtcttgctggactagatatttccttcttcacatttacattcaaagcaccagctgctgggtctggagtgtaagtgaatggttgaacatcatgagatcttccagcatttgtcactacatatattcccactgacacaggcaaagttatatgttggtcatgatagggaggaaccttcacaataagatgattctgatgaaatagttccatatcaatttcagcttctgacttccaagagttttcatcagaaacattttcttggaaaataactttagttcctttcagaaagttcttgccgattaaaaacacttcttcttctcctttcactgaacagctatgcaagcttttctttaagatttctggcactcctgctggctgagtacacaaaattggagaagagggtgtttgcagtgtcaaagtggagccatctttcctcatgatattaactcgaaaaaccaatctggcacgagtgcttttcttcttggaaccagcaattcctattctggcttcgacatcagcattcctcaatttcaatatccctacgcagtccaccgccagtgtcatgttgttgctaggatcaaggccgacttctataacagtagtgccttcaatgtccacttctttgcaaggagttgtatttcgtccagttactctgcaggcctgataaaatccatgtggtttcactcgtccagagtcgttgcccacaaacacttgcaacactacaggttcattatggccttccagctttactgtaggaaagccttgctgtgttctatctttcactgagccacggctgccctcagtcaggtaccgagctcggtgctgtgtctcaggttgtacaactatcttcagctcctttccctcacttttaacaggatattgtccacacaacatagggctcttctttactccagttcctttttggttttccaatgttccatttcccgcttttgagttgcctttgttgtccgtggtaagctgagaaagcacatagtgaggtgctttggcactgtcggcatcaaatatatccatattagattcttcacaatctcgtcgtttgacccccggcctctgctttggatttcgttttcgtgatttacgaggtacctcagtgttatcattgtaggaactggtgctcatgttactgaagttggagggggaatcctccatccacatactgcagctctgctcagattccaatccacacccctcatcctggcaggacatccgactgttatccagcaagtcctcaggtggtggtgagatgtacaagactgtgtgcctcttcggtgttgatggatgctgctgaactgtgttactggttaactgcttttcacttacccctctgttacttacccccacggctgaggagcagctctccacttgcatagccttgctgtcggtgactgaggtagaataaatggtagggctggaagaggtggtaaaggagctgcaagcaccgcccatggaggaagaggagggagctgaagaagcatctatgaagcagagaactacaggtcatttttaatgcagacactccctgcttcagaggcaaatccagcagcaacaacagctggaggaggcgagcctgcctcaccaccgcttgtctgactcattgatgctacagatgtttctctagatggaggtaactgtaactcctttgggagaagatcatagacagattctcgcgagtagagggacttgggcgattccaggtctaggtccgcgctgagcaatgagatgaagtccgagggcatcgcagctcgacccagcccggcccgagggcagcgggagggggggagcggcggtggcggcggcacctcctctccgggaccgcgggcaccgaaccgggggcggcgacgcgagggcggctgccgctgcctcctcctcgagggtagtgacttccactgggccgaggaccgaggaaacgatggcgaggtggagggggaactccacggggactgattctcggtgaccaggagaggggttcaggacggggaaggggaagggggagagccaaagggtccgtttcgtgtttctcctcagcgaaaactgacggtcgccgccaccgccgccgccgctgacaggaatctgagccccgccccc

SEQ ID NO: 10613 - RNA, 3679 nt, Homo sapiens
  source 1..3679: mol_type = other RNA
cggcccgggctgctgctgttcctgggatggagagttactctgcatggcaactattgagtgctgtgactggaacatggttccttgttggctttgaggcattggattaggtggaagggagcccagggccacctgaggctgaaataaaccctgctgcgggggttgtgcctgttcttgggaaagcataggagtctggatgtgtgatattggagcttgctgttggaaagcagcttgttgttcactgtttgatgttgactgaagtggagaaattgagttcggtgctgcaaaaaatgcttcttgggctactgtgttagtctgaagattattcatgggactctgggaaagaaatatgttggttgactgctggtcttgaggaactgaagagccctgtaacacagcaatggtactttgagagtgaaacattggaggctgcatttgttcagaggaggttgtagaagtctgactgtggacaataggatttggactatgaaagagagaaccttgagtttcctgggaaaggttctgagcatcggcaataggattttgaggatgaaaaagttgggcctgtgaatgagaagactgctgcaaaaaatttccagattgaagtgacatcatctcattcccttgctggaataaaccattaccttgttgttgggtaccactattctgaacactcatcatactttttgtggatgaaaaaaggttaacttgaggttgattgtccccactatgttgcatttggaccatggtctgaaagacactgttctgaatctgttttgcttgtgttccagtttcttctccatctcctgaacttgatgtctgaaacatggtagtgccaggggttgcaacctgctgtgtggtagttgtagaagtttcatttccagaaactgcaggaggagaagaaaacaattcacactgcatttgcatatcctcattggtagacaatgcactcatcatgtgagaagtctgctggtaaactggcgattgctgaaggtttccatttgctgaagcagttgaagggaataactctgactgaatctgggcagctgcctggcagatactctgttgcatctccatcaccattgcggctgaagattccatcacttgctgttgctgctgctgctgctgctgttgattagataacgtgttttcagactgtggatgaacactttcagctcttccaggtaataaattatctggtctggtatggactgttggctctgttgaggaaaacattccagggcttacaccactctgaatttgactgacttgttgaaaaatatctgcactaagctgctcttgaacattctcattaccatctggagcagaaaataaaactgaagataactgctgctgtgcctctaaaacttgttggaccaagtcaacacttccactgctgccactagcagtactgcctgtgaaactccctgcttgcagctgctgaatagtattctgaagctgactcacactatttggtgatggaaaaatatttgatgaaatctgctgctgtaaagtctgtgcttgttcttgtagtggtgactgctgctgttgttgtgatgcctcagtcagttgtgacaaattaaccactgtaccatctgactgtaatatctctctagactgagtttctcttgtctgaaactgtgtagcctgctgcaatagtgcatcgctgttgggcagctgactagaagcagaaactgctggaaaagtaccaggctgtgagatgtcctgggtttgaatagttgtcagggtctctgggttgtatgccttgggctgaatctgctgctgtttttcattttcagaaggtaggtgggaagatgatggtgatgaaaaagagccatttcctgctatgtttgagatgttttctaatgtttgctgagttgatccaacagactttgtagtcttaaaaatagtggaagatcttttttctgctgttacttccattggagtaacatcttcactcttaatcatactgcttggtatgagtggagtcatcagggcattagggataatatttaccttatctaaattacatccagtagttttcattgctttcatggcctcttcaaaagagcaaggtcttgctggactagatatttccttcttcacatttacattcaaagcaccagctgctgggtctggagtgtaagtgaatggttgaacatcatgagatcttccagcatttgtcactacatatattcccactgacacaggcaaagttatatgttggtcatgatagggaggaaccttcacaataagatgattctgatgaaatagttccatatcaatttcagcttctgacttccaagagttttcatcagaaacattttcttggaaaataactttagttcctttcagaaagttcttgccgattaaaaacacttcttcttctcctttcactgaacagctatgcaagcttttctttaagatttctggcactcctgctggctgagtacacaaaattggagaagagggtgtttgcagtgtcaaagtggagccatctttcctcatgatattaactcgaaaaaccaatctggcacgagtgcttttcttcttggaaccagcaattcctattctggcttcgacatcagcattcctcaatttcaatatccctacgcagtccaccgccagtgtcatgttgttgctaggatcaaggccgacttctataacagtagtgccttcaatgtccacttctttgcaaggagttgtatttcgtccagttactctgcaggcctgataaaatccatgtggtttcactcgtccagagtcgttgcccacaaacacttgcaacactacaggttcattatggccttccagctttactgtaggaaagccttgctgtgttctatctttcactgagccacggctgccctcagtcaggtaccgagctcggtgctgtgtctcaggttgtacaactatcttcagctcctttccctcacttttaacaggatattgtccacacaacatagggctcttctttactccagttcctttttggttttccaatgttccccacggctgaggagcagctctccacttgcatagccttgctgtcggtgactgaggtagaataaatggtagggctggaagaggtggtaaaggagctgcaagcaccgcccatggaggaagaggagggagctgaagaagcatcagcagcaacaacagctggaggaggcgagcctgcctcaccaccgcttgtctgactcattgatgctacagatgtttctctagatggaggtaactgtaactcctttgggagaagatcatagacagattctcgcgagtagagggacttgggcgattccaggtctaggtccgcgctgagcaatgagatgaagtccgagggcatcgcagctcgacccagcccggcccgagggcagcgggagggggggagcggcggtggcggcggcacctcctctccgggaccgcgggcaccgaaccgggggcggcgacgcgagggcggctgccgctgcctcctcctcgagggtagtgacttccactgggccgaggaccgaggaaacgatggcgaggtggagggggaactccacggggactgattctcggtgaccaggagaggggttcaggacggggaaggggaagggggagagccaaagggtccgtttcgtgtttctcctcagcgaaaactgacggtcgccgccaccgccgccgccgctgacaggaatct

SEQ ID NO: 10614 - RNA, 317 nt, Homo sapiens
  source 1..317: mol_type = other RNA
cggcccgggctgctgctgttcctggtccgtcttactgtggagtgtattagactgcgggggcgtccacaaggggggtgtgggtgggcccggagacctttcttccgggaggccaagtttccaaacccagtccttcacgttcaaggatgccctctccctgcaggatcctggacttgtcatggggtctggattaggttatgctaatggcatccacacttggcctttcccctctttccttataaatcagccaacattgggaggccatgggcttcgccagaagcctctggagacagagctgctcctttccagcaggccaggct

SEQ ID NO: 10615 - RNA, 2052 nt, Homo sapiens
  source 1..2052: mol_type = other RNA
cggcgcccgtgtctcctccagggcgccaagcacccagcccacagtgccatcgccaccacacaccagcacccggaagcagggcacctgggagaacaggtggagcccgggaagaggacctccgttggtcaggtcgaagacctgatgagggttcagtagcttccggaagctgcagagcaggtctcggcccttgaggcctccactcttggggttcacgaacacaaggaggggacagctgtctgggggcagcttcgcgtgcagcaggtcggggagcaccagggcagtgagcagccggccccgcacagccatgtccttcagcagcatgtacagccgctcggcctccgcaaagcaggcaacgtccaacactaccgcgccttgggaggagtagatgtgactcacggacaccacggtggccgcaaaacagcaaaacagggcatcaggaacactcccaggaattaagtcaacaggaaaacgaggaaaggggccacagaggcttccttgctgtggacaacccctgtccgttcccctcgaggacctcggggagatctgcagctcgaggcctccctgccggatgtcctgtagccggtccagcaggggctgttcgtccatcagcatcgtccgctggacgtgcctgcagcccatcgccacctccaccagctggaagctctcgggactctcggcctggcggccgagcagcggcaggacctccagcaccacagagcgggccgtgctcttcggggtcactcgcacggacacgtaggccacgcccaccttgagccagccagggtagatcttcaggacctcctgggcccgcggcagagcccggatgacccaggcctctggcgtggcctcgccggacccggggcttctgccctcctccgagatcacagcactcccagccttgcccccagcccaggcgtcacaggcctgagaggaagggggcagccggcacagctccaggtggccagggtcctcggggatgtggtgggcccgcagtgcggcctccagcacctcctcggcaccggccaggcgggacaccgtgacgaggcggaactggcttcttctcaccgcgtcgtcgccatcaaagatcttcagcgtttgcttcccggactccggagttgcctgtgtctctctgcctggacccacggcagcgctcccgtcggcgccgtcgcccccctcgcccggctccgcggcctccacgatgcggaagctctgcgtcttgctgaagccgccgggcagaaggcgcacgcacgcgggaggcaggaccagggagcgcagacgcccgaagccacactcgggagccagcgccgcggagcagagggagtgcgcctggaccccgcaccactcgcagcgcacgccggccagcacgtcagaggagccgcacgtcttcctgcagacctcgcagcgcgctcccgagggcaggttcccctcccgccagtggtggtgatgggtgtcgtgatcctggtgcccatcctggtggcactggcggcagtcactgcaggcgaagggcacacagtctgggtggaggtgcagctcacacacttcgcagtggagcgccggtgcctccaggaccttgcggcagacagcacagaacttgcgcttgtggagcccccgggggccgaagcagtgggctacaggaacccggaccaggctgggtgccacactcgtgcacgggatcctcacgtgcttcaggcacttctcatgagacatgaaattgcagacgtcgcacaggaagccggccagcccccagatgaagtcggagcagaggtggcagaaggtgggcttggtgagcgtcaccttccggaagctgtgtcccggcgcggcagcggggcccggggctctgacgcccgcccgctcgggtcccggccccggccccggccccgggcgcgcgcggcctcctgagcccagcacggggctgcaggccgggctgccggggcgcggggagccgccgcccagccaggcgcgggccccgggctcggccgccgccgccattcccggcccgagcggcccgagcccctttaggtccgcgccgggggtacaggagccgccgctcca

SEQ ID NO: 10616 - RNA, 2076 nt, Homo sapiens
  source 1..2076: mol_type = other RNA
cggcgcccgtgtctcctccagggcgccaagcacccagcccacagtgccatcgccaccacacaccagcacccggaagcagggcacctgggagaacaggtggagcccgggaagaggacctccgttggtcaggtcgaagacctgatgagggttcagtagcttccggaagctgcagagcaggtctcggcccttgaggcctccactcttggggttcacgaacacaaggaggggacagctgtctgggggcagcttcgcgtgcagcaggtcggggagcaccagggcagtgagcagccggccccgcacagccatgtccttcagcagcatgtacagccgctcggcctccgcaaagcaggcaacgtccaacactaccgcgccttgggaggagtagatgtgactcacggacaccacggtggctttggtagccccggcctcatgcagcaggctgctgtactcctcgggagacaggccgggaggcaggccgccaacaaacagggagacgtgcggggctacatccctgctctctgccacgtagaaccgcgtctggctcacctgccgcacagacatctgccggatgtcctgtagccggtccagcaggggctgttcgtccatcagcatcgtccgctggacgtgcctgcagcccatcgccacctccaccagctggaagctctcgggactctcggcctggcggccgagcagcggcaggacctccagcaccacagagcgggccgtgctcttcggggtcactcgcacggacacgtaggccacgcccaccttgagccagccagggtagatcttcaggacctcctgggcccgcggcagagcccggatgacccaggcctctggcgtggcctcgccggacccggggcttctgccctcctccgagatcacagcactcccagccttgcccccagcccaggcgtcacaggcctgagaggaagggggcagccggcacagctccaggtggccagggtcctcggggatgtggtgggcccgcagtgcggcctccagcacctcctcggcaccggccaggcgggacaccgtgacgaggcggaactggcttcttctcaccgcgtcgtcgccatcaaagatcttcagcgtttgcttcccggactccggagttgcctgtgtctctctgcctggacccacggcagcgctcccgtcggcgccgtcgcccccctcgcccggctccgcggcctccacgatgcggaagctctgcgtcttgctgaagccgccgggcagaaggcgcacgcacgcgggaggcaggaccagggagcgcagacgcccgaagccacactcgggagccagcgccgcggagcagagggagtgcgcctggaccccgcaccactcgcagcgcacgccggccagcacgtcagaggagccgcacgtcttcctgcagacctcgcagcgcgctcccgagggcaggttcccctcccgccagtggtggtgatgggtgtcgtgatcctggtgcccatcctggtggcactggcggcagtcactgcaggcgaagggcacacagtctgggtggaggtgcagctcacacacttcgcagtggagcgccggtgcctccaggaccttgcggcagacagcacagaacttgcgcttgtggagcccccgggggccgaagcagtgggctacaggaacccggaccaggctgggtgccacactcgtgcacgggatcctcacgtgcttcaggcacttctcatgagacatgaaattgcagacgtcgcacaggaagccggccagcccccagatgaagtcggagcagaggtggcagaaggtgggcttggtgagcgtcaccttccggaagctgtgtcccggcgcggcagcggggcccggggctctgacgcccgcccgctcgggtcccggccccggccccggccccgggcgcgcgcggcctcctgagcccagcacggggctgcaggccgggctgccggggcgcggggagccgccgcccagccaggcgcgggccccgggctcggccgccgccgccattcccggcccgagcggcccgagcccctttaggtccgcgccgggggtacaggagccgccgctccacggcccggtacactgcttccgact

SEQ ID NO: 10617 - RNA, 1201 nt, Homo sapiens
  source 1..1201: mol_type = other RNA
cggcgcccgtgtctcctccagtgtcccctgcaacttcccccgcagtgtccctgcttctgtggaagcctctcggcctggacttccttgcgagcagcagtttaaaggccgccgctctgtacttctttgaaatgaggttgtagaggattgggttgatagatgcgctcagatagaaaagttgcagagcgacgatgttaaagtactgagagaagtacatcatccgcgaatcttccgtgtttatgtaaatgattctgccaacgtggaagggcaaccagcaaattataaatgccagaaccaccaccagcaggacgcggacggtctgccggtggcctctctcccgccccgaggcggccgggcctcgcagcggccgccggctgctccacagctcccgcccgatgagcccgtagaggatgctgaggcacagaaagggcaggaagaagtaggcggtggtgacccacagcatgacacgcagcgcgcccagctgcgcggggctcggccggcattcgcggctgaacagcgccgcggcctccgcggtctcgggccccgacggcggggacggcggtggcgcccgcgagagccagagaggcggcgacgaggcgagaggcgaggaggcgatccgcgcggtgccattgaggcccgggactacggagatgccggggtcctgctcgacgcccaccaggaacaagaagggaccggcagagagcagcgccacggcccagagcacagcgatgagcgcgcggacgcggcgccgggtgaccaagacgcgggcgcggagcgggcggcagatggccaggtagcgctcgacgctgagcgcggtcatgtgcagcagcgtggcgtaggtgcagccctcgcccacgtagagggacaggcggcagagcagcggcccgaacacccagggccgcgagcgccagaggcggtacaggtcgaacggcagcccgagcaggatgagtaggtcggacacggccatgctgcccaggtacaagttggtggtggtccgcatgtcccggtagcgcccgatcagcatcacggtcaccacgttgccgctcaccccgacgacgaacaggcacaggcacacagcggtcaccggcaccagcgcccccaggggaaagggcgagcagcggcgctcgtcgcaaggcggcagcgcgggccacggcggctcccgcgccccctcggggccgtcgctgccgttccaggggctgcccat

SEQ ID NO: 10618 - RNA, 31 nt, Homo sapiens
  source 1..31: mol_type = other RNA
cggcggcggcggctctgggcgcgcccgcctg

SEQ ID NO: 10619 - RNA, 42 nt, Homo sapiens
  source 1..42: mol_type = other RNA
cggcggcggcggctctgggcgcgcccgcctggggccggcctg

SEQ ID NO: 10620 - RNA, 134 nt, Homo sapiens
  source 1..134: mol_type = other RNA
cggcggcggcggctctgggcgcgcccgcctggggccggcctggccctgcgggggacccaggggcggggacgggacctgggcacgcggggcgcaccccgagggcgcgcagacgcacaggcgggctcgcgcccgag

SEQ ID NO: 10621 - RNA, 177 nt, Homo sapiens
  source 1..177: mol_type = other RNA
cggcggcggcggctctgggcgcgcccgcctggggccggcctggccctgcgggggacccaggggcggggacgggacctgggcacgcggggcgcaccccgagggcgcgcagacgcacaggcgggctcgcgcccgagcccccgcacgggcccccgccaaacacgcacacgcacacgcacg

SEQ ID NO: 10622 - RNA, 696 nt, Homo sapiens
  source 1..696: mol_type = other RNA
cggcggcggcggctctgggcgtccacacgctccagggcggggggcccggtcccagctggccgcagaatcggcaaactcagggacttggagtccttcatgccctgctccaccttgccctcatctccaggcttggctggggctttgacacgaaggtagtgtcccccgaacctgtaggcctcgaaggtgagggacaggggtgtgttggactggtccaggtagatgtccactttgcccagcgcaatgcccttcctttcaaatacaggcagcagcacctcccccagtgacttcttcttcatggctgggacgatctctgtctcaatgtccacattcaggtcaaatttcagagtgaagcattccttgcttgggtcatccgtgtgtctcctccttgctttcttcttggagagtttcaggcctgtgctcttccggtcccctttgccatccacagagctctcctcctcctcctcctccaagtccactgcggggctggtgcgcggcgggcatgaccgggtggacacgttccgggccagcacagagccttgtgggggaaggtcgaagcggacatgcccatcataatgcatggtgctgtggaacttgctgtcacaggcctcgcagaggttgaggggcccccggcggtgcagctgctggcagtcggcgtggtgacatacatcctgcccgtcccttctccatgggggcctc

SEQ ID NO: 10623 - RNA, 801 nt, Homo sapiens
  source 1..801: mol_type = other RNA
cggcggcggcggctctgggcgtccacacgctccagggcggggggcccggtcccagctggccgcagaatcggcaaactcagggacttggagtccttcatgccctgctccaccttgccctcatctccaggcttggctggggctttgacacgaaggtagtgtcccccgaacctgtaggcctcgaaggtgagggacaggggtgtgttggactggtccaggtagatgtccactttgcccagcgcaatgcccttcctttcaaatacaggcagcagcacctcccccagtgacttcttcttcatggctgggacgatctctgtctcaatgtccacattcaggtcaaatttcagagtgaagcattccttgcttgggtcatccgtgtgtctcctccttgctttcttcttggagagtttcaggcctgtgctcttccggtcccctttgccatccacagagctctcctcctcctcctcctccaagtccactgcggggctggtgcgcggcgggcatgaccgggtggacacgttccgggccagcacagagccttgtgggggaaggtcgaagcggacatgcccatcataatgcatggtgctgtggaacttgctgtcacaggcctcgcagaggttgaggggcccccggcggtgcagctgctggcagtcggcgtggtgacatacctaggaacaggaccagggtctcctccccggtgtctaaggctctaaggctcgggccgagactgccaaagcctcatggggcgcgcggggagagggggacgggagccgcgggacgggctcagtcgactcagcgcaaact

SEQ ID NO: 10624 - RNA, 784 nt, Homo sapiens
  source 1..784: mol_type = other RNA
cggcggcggcggctctgggcgtccacacgctccagggcggggggcccggtcccagctggccgcagaatcggcaaactcagggacttggagtccttcatgccctgctccaccttgccctcatctccaggcttggctggggctttgacacgaaggtagtgtcccccgaacctgtaggcctcgaaggtgagggacaggggtgtgttggactggtccaggtagatgtccactttgcccagcgcaatgcccttcctttcaaatacaggcagcagcacctcccccagtgacttcttcttcatggctgggacgatctctgtctcaatgtccacattcaggtcaaatttcagagtgaagcattccttgcttgggtcatccgtgtgtctcctccttgctttcttcttggagagtttcaggcctgtgctcttccggtcccctttgccatccacagagctctcctcctcctcctcctccaagtccactgcggggctggtgcgcggcgggcatgaccgggtggacacgttccgggccagcacagagccttgtgggggaaggtcgaagcggacatgcccatcataatgcatggtgctgtggaacttgctgtcacaggcctcgcagaggttgaggggcccccggcggtgcagctgctggcagtcggcgtggtgacatacctctgcgcctctgcgcggccccgggcccctctcttctctgactccctcctcaacaccaatgccgggctcagagggctcctcagaacttgctctttctcctggggagctccttgaatgct

SEQ ID NO: 10625 - RNA, 811 nt, Homo sapiens
  source 1..811: mol_type = other RNA
cggcggcggcggctctgggcgtccacacgctccagggcggggggcccggtcccagctggccgcagaatcggcaaactcagggacttggagtccttcatgccctgctccaccttgccctcatctccaggcttggctggggctttgacacgaaggtagtgtcccccgaacctgtaggcctcgaaggtgagggacaggggtgtgttggactggtccaggtagatgtccactttgcccagcgcaatgcccttcctttcaaatacaggcagcagcacctcccccagtgacttcttcttcatggctgggacgatctctgtctcaatgtccacattcaggtcaaatttcagagtgaagcattccttgcttgggtcatccgtgtgtctcctccttgctttcttcttggagagtttcaggcctgtgctcttccggtcccctttgccatccacagagctctcctcctcctcctcctccaagtccactgcggggctggtgcgcggcgggcatgaccgggtggacacgttccgggccagcacagagccttgtgggggaaggtcgaagcggacatgcccatcataatgcatggtgctgtggaacttgctgtcacaggcctcgcagaggttgaggggcccccggcggtgcagctgctggcagtcggcgtggtgacatacctggctatcaccgtcgcgggcacgacccccggcccaggagggctccgagtcccggaggggcagccccgggcccggcctggaggctgctaggcgtccggagacaccgggtcctgtccccatggcggccggaggaagccgcggtctgc

SEQ ID NO: 10626 - RNA, 835 nt, Homo sapiens
  source 1..835: mol_type = other RNA
cggcggcggcggctctgggcgtccacacgctccagggcggggggcccggtcccagctggccgcagaatcggcaaactcagggacttggagtccttcatgccctgctccaccttgccctcatctccaggcttggctggggctttgacacgaaggtagtgtcccccgaacctgtaggcctcgaaggtgagggacaggggtgtgttggactggtccaggtagatgtccactttgcccagcgcaatgcccttcctttcaaatacaggcagcagcacctcccccagtgacttcttcttcatggctgggacgatctctgtctcaatgtccacattcaggtcaaatttcagagtgaagcattccttgcttgggtcatccgtgtgtctcctccttgctttcttcttggagagtttcaggcctgtgctcttccggtcccctttgccatccacagagctctcctcctcctcctcctccaagtccactgcggggctggtgcgcggcgggcatgaccgggtggacacgttccgggccagcacagagccttgtgggggaaggtcgaagcggacatgcccatcataatgcatggtgctgtggaacttgctgtcacaggcctcgcagaggttgaggggcccccggcggtgcagctgctggcagtcggcgtggtgacataccttggccgcccgccccttgtccatgcaggcggggttctgacagcgcagtcccttcttttcagcggggctctggtcgtccatggagcaggccccgtgccgcgcggggggcgggcggcgggcgggggcgccggggacgccggggactgggaggccgcagagccgccgccgcc

SEQ ID NO: 10627 - RNA, 1390 nt, Homo sapiens
  source 1..1390: mol_type = other RNA
cggcggcggcggctctgggcgtccacacgctccagggcggggggcccggtcccagctggccgcagaatcggcaaactcagggacttggagtccttcatgccctgctccaccttgccctcatctccaggcttggctggggctttgacacgaaggtagtgtcccccgaacctgtaggcctcgaaggtgagggacaggggtgtgttggactggtccaggtagatgtccactttgcccagcgcaatgcccttcctttcaaatacaggcagcagcacctcccccagtgacttcttcttcatggctgggacgatctctgtctcaatgtccacattcaggtcaaatttcagagtgaagcattccttgcttgggtcatccgtgtgtctcctccttgctttcttcttggagagtttcaggcctgtgctcttccggtcccctttgccatccacagagctctcctcctcctcctcctccaagtccactgcggggctggtgcgcggcgggcatgaccgggtggacacgttccgggccagcacagagccttgtgggggaaggtcgaagcggacatgcccatcataatgcatggtgctgtggaacttgctgtcacaggcctcgcagaggttgaggggcccccggcggtgcagctgctggcagtcggcgtggtgacataccttggccgcccgccccttgtccatgcaggcggggttctgacagcgcagtcccttcttttcagcggggctctggtcgtcggttcctgaacaaaggctgagccagcttcgaggtggagacccatgttttgtcaggactgaattcatgcttgacctctgcggtggtggcaccctgcctggacctccagccacatgccaatgccacaggcctctctaatcagacacacaggtctccgtcctgctttgcccagttgccatctcaacatggaaggcttctccccgactcagccccagtcttaatttctgcagctggacctgtctgcacagaaaaccaaggcgctctcagccctgccaatttgctccccgtccaacacaggtcccctgggcgctgtatatttgaaggcacagacttcgcagccgccgctcacactgcatttccttgttggtggttggttccttcttggattttccattcctgagtgcccatttgcgccctggaatgggctcccacactgctggctgccctggaggtgccgtccctcctttccaggaaagcaacaccacagagaccccggcctctgcaatcccagcagccagcagcagcccctctgctgggctccttggctaccaggaaggccttagtttggtggctttcccctgccaggcagagaggggctggtcacagcgggagatcaagtgagcctcaaaacattagaaaaacccaagcc

SEQ ID NO: 10628 - RNA, 1015 nt, Homo sapiens
  source 1..1015: mol_type = other RNA
cggcggcggcggctctgggcgtccacacgctccagggcggggggcccggtcccagctggccgcagaatcggcaaactcagggacttggagtccttcatgccctgctccaccttgccctcatctccaggcttggctggggctttgacacgaaggtagtgtcccccgaacctgtaggcctcgaaggtgagggacaggggtgtgttggactggtccaggtagatgtccactttgcccagcgcaatgcccttcctttcaaatacaggcagcagcacctcccccagtgacttcttcttcatggctgggacgatctctgtctcaatgtccacattcaggtcaaatttcagagtgaagcattccttgcttgggtcatccgtgtgtctcctccttgctttcttcttggagagtttcaggcctgtgctcttccggtcccctttgccatccacagagctctcctcctcctcctcctccaagtccactgcggggctggtgcgcggcgggcatgaccgggtggacacgttccgggccagcacagagccttgtgggggaaggtcgaagcggacatgcccatcataatgcatggtgctgtggaacttgctgtcacaggcctcgcagaggttgaggggcccccggcggtgcagctgctggcagtcggcgtggtgacataccttggccgcccgccccttgtccatgcaggcggggttctgacagcgcagtcccttcttttcagcggggctctggtcgtgccctgcatcgctccctttagagacagaggagcccccgaaggtctggggcgacccccgttccccaagactcatctttgaccctgaatttggccccctccaagctgcctctcttcctgggggctggagtgcaccgcggtgggggcagagcggcgcaaccagcgagaggcggggggagggaggagaagcggggtgctgccgaggcaggccccgacttgggggccgagtttgggtacgagcggcccgaagcccggtcggcgcccacccccttgcct

SEQ ID NO: 10629 - RNA, 23 nt, Homo sapiens
  source 1..23: mol_type = other RNA
cggcggggctcggagccgggatt

SEQ ID NO: 10630 - RNA, 77 nt, Homo sapiens
  source 1..77: mol_type = other RNA
cggcggggctcggagccgggattccaggccggtcagctggaggcgggccgcaccactcggcctgcggagacggggag

SEQ ID NO: 10631 - RNA, 456 nt, Homo sapiens
  source 1..456: mol_type = other RNA
cggcggggctcggagccgggcgcctcggggaaggcgggcagcgggggcggcggcgcgggccccggcccgggggcggagaaggcgaaggcgcagggcgtctcggcggcggcggcgggggcgcgacggaaggcggctgagtgcaggcgcagagccgggtgcgcgtcgagcacgagcgcgcggggcgcgggccgcagcgcgcacagctcgagcaccaggcagccggccaactcgcgcgcctcgggccgcagctccaggcccagctgcaggtggcggaggcggaagagctgcgcgctggaggccgaggccacgtccagggcgggcggcggctcgggcggcgggcggacgggcgcggcctcggcgccgggcgcctggcggcagcagcactgcgcggccatggccgccggcactaggtgaaatccatgggcggcggccgcgccgggccgcgggcgaggggcg

SEQ ID NO: 10632 - RNA, 498 nt, Homo sapiens
  source 1..498: mol_type = other RNA
cggcggggctcggagccgggcgcctcggggaaggcgggcagcgggggcggcggcgcgggccccggcccgggggcggagaaggcgaaggcgcagggcgtctcggcggcggcggcgggggcgcgacggaaggcggctgagtgcaggcgcagagccgggtgcgcgtcgagcacgagcgcgcggggcgcgggccgcagcgcgcacagctcgagcaccaggcagccggccaactcgcgcgcctcgggccgcagctccaggcccagctgcaggtggcggaggcggaagagctgcgcgctggaggccgaggccacgtccagggcgggcggcggctcgggcggcgggcggacgggcgcggcctcggcgccgggcgcctggcggcagcagcactgcgcggccatggccgccggcactaggtgaaatccatgggcggcggccgcgccgggccgcgggcgaggggcgccgggcggcggcggcggcggggcgcgggcacaacaggaagtc

SEQ ID NO: 10633 - RNA, 1041 nt, Homo sapiens
  source 1..1041: mol_type = other RNA
cggcggggctcggagccgggcttcggccgggccccgggccctcgaccggaccggtgcgcgggcgctgcggccgcacggcgcgactgtccccgggccgggcaccgcggtccgcctctcgctcgccgcccggacgtcggggccgccccgcggggcgggcggagcgccgtccccgcctcgccgccgcccgcgggcgccggccgcgcgcgcgcgcgcgtggccgccggtccctcccggccgccgggcgcgggtcgggccgtccgcctcctcgcgggcgggcgcgacgaagaagcgtcgcgggtctgtggcgcggggccccggtggtcgtgtcgcgtggggggcgggtggttggggcgtccggttcgccgcgccccgccccggccccaccggtcccggccgccgcccccgcgcccgctcgctccctcccgtccgcccgtccgcggcccgtccgtccgtccgtcgtcctcctcgcttgcggggcgccgggcccgtcctcgcgaggccccccggccggccgtccggccgcgtcggggcctcgccgcgctctaccttacctacctggttgatcggttctcggcggcgtcgcggcgggtctgggggggtctcggtgccctcctccccgccggggcccgtcgtccggccccgccgcgccggctccccgtcttcggggccggccggattcccgtcgcctccgccgcgccgctccgcgccgccgggcacggccccgctcgctctccccggccttcccgctagggcgtctcgagggtcgggggccggacgccggtcccctcccccgcctcctcgtccgcccccccgccgtccaggtacccggcggccgtcgcgcgcctgccgcgcgtgtggcgtgcgccccgcgccgtgggggcgggaacccccgggcgcctgtggggtggtgtccgcgctcgcccccgcgtgggcggcgcgcgcctccccgtggtgtgaaaccttccgacccctctccggagtccggtcccgtttgctgtctcgtctggccggcctgaggcaaccccctctcctattgatcat

SEQ ID NO: 10634 - RNA, 728 nt, Homo sapiens
  source 1..728: mol_type = other RNA
cggctctgggtctgtggggagtgcccgtggttccacaattagctgaacccctgacctcgccgcttaacagcagttcatttggcttctaaatgccatccagccggccgatgtcagtttagatacagcatttttctgtagcctgggaacaaaggtcactgttttcctcattcttccggtgcctgggaatcccctgtcttttctcaccctttgtaggtgctgcaaatgtgtccatctctgcattgatctgcttctagggtaagcagccctcacagttggagcagataaagacagacaagaatggaatgaaagagttttacaccaggcttccctcttctgtttctcttctttgtagactcaggctgtgaacatgaaatttgaatcaaggtgataaacagcatcaaggtttcccataatctctggtgggcccaggcacatcattctttcccgtttcaagtgttgtcctcggaatagcccaggatagcatacagtccaaataatgtaatccactctggtatcatcaaaggtagatcaggagaagtgggcagtaatgggcaatgaaatctacaccctcattttccatttgggaaggtaacagccaagcctacccctgtggccagggaagcaggcagccttctggaactggtgaattaggagaggctttcgtggcagttggaggactttgctgcagtcttcacagctctggcactcaggttgcagtgagatccagg

SEQ ID NO: 10635 - RNA, 1395 nt, Homo sapiens
  source 1..1395: mol_type = other RNA
cggctctgggtctgtggggagtgcccgtggttccacaattagctgaacccctgacctcgccgcttaacagcagttcatttggcttctaaatgccatccagccggccgatgtcagtttagatacagcatttttctgtagcctgggaacaaaggtcactgttttcctcattcttccggtgcctgggaatcccctgtcttttctcaccctttgtaggtgctgcaaatgtgtccatctctgcattgatctgcttctagggtaagcagccctcacagttggagcagataaagacagacaagaatggaatgaaagagttttacaccaggcttccctcttctgtttctcttctttgtagactcaggctgtgaacatgaaatttgaatcaaggtgataaacagcatcaaggtttcccataatctctggtgggcccaggcacatcattctttcccgtttcaagtgttgtcctcggaatagcccaggatagcatacagtccaaataatgtaatccactctggtatcatcaaaggtagatcaggagaagtgggcagtaatgggcaatgaaatctacaccctcattttccatttgggaaggtaacagccaagcctacccctgtggccagggaagcaggcagccttctggaactggtgaattaggagaggctttctcaaaaagaatattgctctttcagtatagaacaataagagatcaaattcaaagccatagtaattctgaatctggcttcagggctcaggttagcctgtcactcaaaagcaactggaactgggaaagaggaagagggagaaggtttttccctaactgcaggaaagctcttccatcccacaccagcttaattgttgaaagagagccgcctttaaacgctttagacaaaatctggatggagaggcacttccaacgagttctttcatcctgagatgttttagggcaagacacacctgcattttttatcctacccagggcttactgagctctttgtcagttgaggattcttggccttaaaccagctccaccactagcatttgtgtgctttggaaaaaacctctctgctgaagaattgagaaagtagtccatggtctcaaagtaatgacacactgtggcgatacaggatcttgaaatgtgtgggtaagatgtggcaggggcctcgtgtgctgtgacgttggctgcccggccacattaaccctcagtgacttccctgagcccagggtctcattgcccatcccactgcaactgctatcttcatccttccttttagaacacctgctcccacagtccctgagaaagaactgttctatgttgacagttcaccccaaccccaaaccaccttgggctgtttacagtaaatactgcacactagtgaggtcttattgatctctttcttc

SEQ ID NO: 10636 - RNA, 1584 nt, Homo sapiens
  source 1..1584: mol_type = other RNA
cgggagctggggtctgcaggtctccggtccacttcatgcagacaggccctgtcccccactggggcccaaggcccaggctaaactacagcccagccatcccaccccaggccgtgaatgccttctccaggagggcaaccaaggatggtgccacatgtgagcacaagcaaaacccggagccaaggcgagtcctgctgggtgcacgtttatcccagccaccgcctccagggcggccgcacaggccctgggcatcaatccagcagggctcccgactcactccctggagaccagctccccaaccacccggccctgatggcatcccgctgcggccaggtgtcctctcagccgaggtccttgtcactgcctagctgcgtccgcctgccacaccagctcacccgagatgtaggtggcctggacgtgaagggagtcgtcgagcaccacgaagtctgcgtcagcaccaaagtccagggtccccttactcttctccagccccagcaactgggcggggtgcagggatgcagcctccagggccgactccatgctgcagcctgccacgtaggccgtcagaccgtccacttccacttcctgctgtcccagcgtgtgccggccgttgcccaggcccaaggcagggatggcatcggtgaccagcaccagcccctggggatgggcacggtgggcgatccgcagggcggcggggttggtgtgcgtgccatctgcaatcatcccatagaagatgcagcggcctgcgggcagccggtcgctggtcaggagccccacgatgcctgggtcgcggtggtggaaaggcagcatggcgttgaagaggtgggtgatgaaggtggctccgctccacacagcatcctctgccgcccgcaggtcagccactgagtgccctagggacacgcagatgccacgggccgtcagcgcccggatcacttcgtggctacggcccaactctggggccagcgtcacgatgcggacattgtccaggggcccgtaggtggccagcaagtcctggaaggcatcggcctcgaaggagcggaggtgggcctcggggtgcgcgccccgcttctcccggctgatgaaggggccctccaggtgcagcccgaggacccctgccccatggggaccaccactcttcacagggatctgaggaacaaccttgtgataaacctccggtggggaagtgaccagggtggggcagaaggaggtgacgccgtgcgacaggatcctccgggccacgagggcaacccccgaacccacgtcctccgtggcttgagagaagtcaacaccaaatccaccgttgatctgcacgtcgatgaatccgggagccaagatgcggcccccgcagtcccgccgctcgtcggccacgcgccgctcctcaaagaacagcttctctgggtccaagatgcggcctccgcgcacccacagatcctccctgagcagtttccctccgcgcaggatccggcagttagtgaactggagcacgcgggcccccgccgcgccctgctcgccgcgcatcgtgagccgtgtcgggagcgagcggctccggagccccgcggcggccaaatcccgcgcccagtgacgaac

SEQ ID NO: 10637 - RNA, 1672 nt, Homo sapiens
  source 1..1672: mol_type = other RNA
cgggagctggggtctgcaggtctccggtccacttcatgcagacaggccctgtcccccactggggcccaaggcccaggctaaactacagcccagccatcccaccccaggccgtgaatgccttctccaggagggcaaccaaggatggtgccacatgtgagcacaagcaaaacccggagccaaggcgagtcctgctgggtgcacgtttatcccagccaccgcctccagggcggccgcacaggccctgggcatcaatccagcagggctcccgactcactccctggagaccagctccccaaccacccggccctgatggcatcccgctgcggccaggtgtcctctcagccgaggtccttgtcactgcctagctgcgtccgcctgccacaccagctcacccgagatgtaggtggcctggacgtgaagggagtcgtcgagcaccacgaagtctgcgtcagcaccaaagtccagggtccccttactcttctccagccccagcaactgggcggggtgcagggatgcagcctccagggccgactccatgctgcagcctgtggcctgcaggaagtgccggacacagacgtccattggggctatgctgccactcagcgtcttggtgcctgccacgtaggccgtcagaccgtccacttccacttcctgctgtcccagcgtgtgccggccgttgcccaggcccaaggcagggatggcatcggtgaccagcaccagcccctggggatgggcacggtgggcgatccgcagggcggcggggttggtgtgcgtgccatctgcaatcatcccatagaagatgcagcggcctgcgggcagccggtcgctggtcaggagccccacgatgcctgggtcgcggtggtggaaaggcagcatggcgttgaagaggtgggtgatgaaggtggctccgctccacacagcatcctctgccgcccgcaggtcagccactgagtgccctagggacacgcagatgccacgggccgtcagcgcccggatcacttcgtggctacggcccaactctggggccagcgtcacgatgcggacattgtccaggggcccgtaggtggccagcaagtcctggaaggcatcggcctcgaaggagcggaggtgggcctcggggtgcgcgccccgcttctcccggctgatgaaggggccctccaggtgcagcccgaggacccctgccccatggggaccaccactcttcacagggatctgaggaacaaccttgtgataaacctccggtggggaagtgaccagggtggggcagaaggaggtgacgccgtgcgacaggatcctccgggccacgagggcaacccccgaacccacgtcctccgtggcttgagagaagtcaacaccaaatccaccgttgatctgcacgtcgatgaatccgggagccaagatgcggcccccgcagtcccgccgctcgtcggccacgcgccgctcctcaaagaacagcttctctgggtccaagatgcggcctccgcgcacccacagatcctccctgagcagtttccctccgcgcaggatccggcagttagtgaactggagcacgcgggcccccgccgcgccctgctcgccgcgcatcgtgagccgtgtcgggagcgagcggctccggagccccgcggcggccaaatcccgcgcccagtgacgaaccccagccgagagctgagac

SEQ ID NO: 10638 - RNA, 1631 nt, Homo sapiens
  source 1..1631: mol_type = other RNA
cgggagctggggtctgcaggtctccggtccacttcatgcagacaggccctgtcccccactggggcccaaggcccaggctaaactacagcccagccatcccaccccaggccgtgaatgccttctccaggagggcaaccaaggatggtgccacatgtgagcacaagcaaaacccggagccaaggcgagtcctgctgggtgcacgtttatcccagccaccgcctccagggcggccgcacaggccctgggcatcaatccagcagggctcccgactcactccctggagaccagctccccaaccacccggccctgatggcatcccgctgcggccaggtgtcctctcagccgaggtccttgtcactgcctagctgcgtccgcctgccacaccagctcacccgagatgtaggtggcctggacgtgaagggagtcgtcgagcaccacgaagtctgcgtcagcaccaaagtccagggtccccttactcttctccagccccagcaactgggcggggtgcagggatgcagcctccagggccgactccatgctgcagcctgtggcctgcaggaagtgccggacacagacgtccattggggctatgctgccactcagcgtcttggtgccttgagagcagagagggcaggctctgggggggtcgtgggccacctggcatgcgggctgggacctgggacccagtgggtcagggcgctcacctgccacgtaggccgtcagaccgtccacttccacttcctgctgtcccagcgtgtgccggccgttgcccaggcccaaggcagggatggcatcggtgaccagcaccagcccctggggatgggcacggtgggcgatccgcagggcggcggggttggtgtgcgtgccatctgcaatcatcccatagaagatgcagcggcctgcgggcagccggtcgctggtcaggagccccacgatgcctgggtcgcggtggtggaaaggcagcatggcgttgaagaggtgggtgatgaaggtggctccgctccacacagcatcctctgccgcccgcaggtcagccactgagtgccctagggacacgcagatgccacgggccgtcagcgcccggatcacttcgtggctacggcccaactctggggccagcgtcacgatgcggacattgtccaggggcccgtaggtggccagcaagtccgaggacccctgccccatggggaccaccactcttcacagggatctgaggaacaaccttgtgataaacctccggtggggaagtgaccagggtggggcagaaggaggtgacgccgtgcgacaggatcctccgggccacgagggcaacccccgaacccacgtcctccgtggcttgagagaagtcaacaccaaatccaccgttgatctgcacgtcgatgaatccgggagccaagatgcggcccccgcagtcccgccgctcgtcggccacgcgccgctcctcaaagaacagcttctctgggtccaagatgcggcctccgcgcacccacagatcctccctgagcagtttccctccgcgcaggatccggcagttagtgaactggagcacgcgggcccccgccgcgccctgctcgccgcgcatcgtgagccgtgtcgggagcgagcggctccggagccccgcggcggccaaa

SEQ ID NO: 10639 - RNA, 1762 nt, Homo sapiens
  source 1..1762: mol_type = other RNA
cgggagctggggtctgcaggtctccggtccacttcatgcagacaggccctgtcccccactggggcccaaggcccaggctaaactacagcccagccatcccaccccaggccgtgaatgccttctccaggagggcaaccaaggatggtgccacatgtgagcacaagcaaaacccggagccaaggcgagtcctgctgggtgcacgtttatcccagccaccgcctccagggcggccgcacaggccctgggcatcaatccagcagggctcccgactcactccctggagaccagctccccaaccacccggccctgatggcatcccgctgcggccaggtgtcctctcagccgaggtccttgtcactgcctagctgcgtccgcctgccacaccagctcacccgagatgtaggtggcctggacgtgaagggagtcgtcgagcaccacgaagtctgcgtcagcaccaaagtccagggtccccttactcttctccagccccagcaactgggcggggtgcagggatgcagcctccagggccgactccatgctgcagcctgtggcctgcaggaagtgccggacacagacgtccattggggctatgctgccactcagcgtcttggtgccttgagagcagagagggcaggctctgggggggtcgtgggccacctggcatgcgggctgggacctgggacccagtgggtcagggcgctcacctgccacgtaggccgtcagaccgtccacttccacttcctgctgtcccagcgtgtgccggccgttgcccaggcccaaggcagggatggcatcggtgaccagcaccagcccctggggatgggcacggtgggcgatccgcagggcggcggggttggtgtgcgtgccatctgcaatcatcccatagaagatgcagcggcctgcgggcagccggtcgctggtcaggagccccacgatgcctgggtcgcggtggtggaaaggcagcatggcgttgaagaggtgggtgatgaaggtggctccgctccacacagcatcctctgccgcccgcaggtcagccactgagtgccctagggacacgcagatgccacgggccgtcagcgcccggatcacttcgtggctacggcccaactctggggccagcgtcacgatgcggacattgtccaggggcccgtaggtggccagcaagtcctggaaggcatcggcctcgaaggagcggaggtgggcctcggggtgcgcgccccgcttctcccggctgatgaaggggccctccaggtgcagcccgaggacccctgccccatggggaccaccactcttcacagggatctgaggaacaaccttgtgataaacctccggtggggaagtgaccagggtggggcagaaggaggtgacgccgtgcgacaggatcctccgggccacgagggcaacccccgaacccacgtcctccgtggcttgagagaagtcaacaccaaatccaccgttgatctgcacgtcgatgaatccgggagccaagatgcggcccccgcagtcccgccgctcgtcggccacgcgccgctcctcaaagaacagcttctctgggtccaagatgcggcctccgcgcacccacagatcctccctgagcagtttccctccgcgcaggatccggcagttagtgaactggagcacgcgggcccccgccgcgccctgctcgccgcgcatcgtgagccgtgtcgggagcgagcggctccggagccccgcggcggccaaatcccgcgcccagtgacgaaccccagccgagagctgagac

SEQ ID NO: 10640 - RNA, 1634 nt, Homo sapiens
  source 1..1634: mol_type = other RNA
cgggagctggggtctgcaggtctccggtccacttcatgcagacaggccctgtcccccactggggcccaaggcccaggctaaactacagcccagccatcccaccccaggccgtgaatgccttctccaggagggcaaccaaggatggtgccacatgtgagcacaagcaaaacccggagccaaggcgagtcctgctgggtgcacgtttatcccagccaccgcctccagggcggccgcacaggccctgggcatcaatccagcagggctcccgactcactccctggagaccagctccccaaccacccggccctgatggcatcccgctgcggccaggtgtcctctcagccgaggtccttgtcactgcctagctgcgtccgcctgccacaccagctcacccgagatgtaggtggcctggacgtgaagggagtcgtcgagcaccacgaagtctgcgtcagcaccaaagtccagggtccccttactcttctccagccccagcaactgggcggggtgcagggatgcagcctccagggccgactccatgctgcagcctgtggcctgcaggaagtgccggacacagacgtccattggggctatgctgccactcagcgtcttggtgccttgagagcagagagggcaggctctgggggggtcgtgggccacctggcatgcgggctgggacctgggacccagtgggtcagggcgctcacctgccacgtaggccgtcagaccgtccacttccacttcctgctgtcccagcgtgtgccggccgttgcccaggcccaaggcagggatggcatcggtgaccagcaccagcccctggggatgggcacggtgggcgatccgcagggcggcggggttggtgtgcgtgccatctgcaatcatcccatagaagatgcagcggcctgcgggcagccggtcgctggtcaggagccccacgatgcctgggtcgcggtggtggaaaggcagcatggcgttgaagaggtgggtgatgaaggtggctccgctccacacagcatcctctgccgcccgcaggtcagccactgagtgccctagggacacgcagatgccacgggccgtcagcgcccggatcacttcgtggctacggcccaactctggggccagcgtcacgatgcggacattgtccaggggcccgtaggtggccagcaagtcctggaaggcatcggcctcgaaggagcggaggtgggcctcggggtgcgcgccccgcttctcccggctgatgaaggggccctccaggtgcagcccgaggacccctgccccatggggaccaccactcttcacagggatctgaggaacaaccttgtgataaacctccggtggggaagtgaccagggtggggcagaaggaggtgacgccgtgcgacaggatcctccgggccacgagggcaacccccgaacccacgtcctccgtggcttgagagaagtcaacaccaaatccacctgagcagtttccctccgcgcaggatccggcagttagtgaactggagcacgcgggcccccgccgcgccctgctcgccgcgcatcgtgagccgtgtcgggagcgagcggctccggagccccgcggcggccaaatcccgcgcccagtgacgaaccccagccgagagctgagaccgcgcccac

SEQ ID NO: 10641 - RNA, 1551 nt, Homo sapiens
  source 1..1551: mol_type = other RNA
cgggagctggggtctgcaggtctccggtccacttcatgcagacaggccctgtcccccactggggcccaaggcccaggctaaactacagcccagccatcccaccccaggccgtgaatgccttctccaggagggcaaccaaggatggtgccacatgtgagcacaagcaaaacccggagccaaggcgagtcctgctgggtgcacgtttatcccagccaccgcctccagggcggccgcacaggccctgggcatcaatccagcagggctcccgactcactccctggagaccagctccccaaccacccggccctgatggcatcccgctgcggccaggtgtcctctcagccgaggtccttgtcactgcctagctgcgtccgcctgccacaccagctcacccgagatgtaggtggcctggacgtgaagggagtcgtcgagcaccacgaagtctgtggcctgcaggaagtgccggacacagacgtccattggggctatgctgccactcagcgtcttggtgcctgccacgtaggccgtcagaccgtccacttccacttcctgctgtcccagcgtgtgccggccgttgcccaggcccaaggcagggatggcatcggtgaccagcaccagcccctggggatgggcacggtgggcgatccgcagggcggcggggttggtgtgcgtgccatctgcaatcatcccatagaagatgcagcggcctgcgggcagccggtcgctggtcaggagccccacgatgcctgggtcgcggtggtggaaaggcagcatggcgttgaagaggtgggtgatgaaggtggctccgctccacacagcatcctctgccgcccgcaggtcagccactgagtgccctagggacacgcagatgccacgggccgtcagcgcccggatcacttcgtggctacggcccaactctggggccagcgtcacgatgcggacattgtccaggggcccgtaggtggccagcaagtcctggaaggcatcggcctcgaaggagcggaggtgggcctcggggtgcgcgccccgcttctcccggctgatgaaggggccctccaggtgcagcccgaggacccctgccccatggggaccaccactcttcacagggatctgaggaacaaccttgtgataaacctccggtggggaagtgaccagggtggggcagaaggaggtgacgccgtgcgacaggatcctccgggccacgagggcaacccccgaacccacgtcctccgtggcttgagagaagtcaacaccaaatccaccgttgatctgcacgtcgatgaatccgggagccaagatgcggcccccgcagtcccgccgctcgtcggccacgcgccgctcctcaaagaacagcttctctgggtccaagatgcggcctccgcgcacccacagatcctccctgagcagtttccctccgcgcaggatccggcagttagtgaactggagcacgcgggcccccgccgcgccctgctcgccgcgcatcgtgagccgtgtcgggagcgagcggctccggagccccgcggcggccaaatcccgcgcccagtgacgaac

SEQ ID NO: 10642 - RNA, 1641 nt, Homo sapiens
  source 1..1641: mol_type = other RNA
cgggagctggggtctgcaggtctccggtccacttcatgcagacaggccctgtcccccactggggcccaaggcccaggctaaactacagcccagccatcccaccccaggccgtgaatgccttctccaggagggcaaccaaggatggtgccacatgtgagcacaagcaaaacccggagccaaggcgagtcctgctgggtgcacgtttatcccagccaccgcctccagggcggccgcacaggccctgggcatcaatccagcagggctcccgactcactccctggagaccagctccccaaccacccggccctgatggcatcccgctgcggccaggtgtcctctcagccgaggtccttgtcactgcctagctgcgtccgcctgccacaccagctcacccgagatgtaggtggcctggacgtgaagggagtcgtcgagcaccacgaagtctgtggcctgcaggaagtgccggacacagacgtccattggggctatgctgccactcagcgtcttggtgccttgagagcagagagggcaggctctgggggggtcgtgggccacctggcatgcgggctgggacctgggacccagtgggtcagggcgctcacctgccacgtaggccgtcagaccgtccacttccacttcctgctgtcccagcgtgtgccggccgttgcccaggcccaaggcagggatggcatcggtgaccagcaccagcccctggggatgggcacggtgggcgatccgcagggcggcggggttggtgtgcgtgccatctgcaatcatcccatagaagatgcagcggcctgcgggcagccggtcgctggtcaggagccccacgatgcctgggtcgcggtggtggaaaggcagcatggcgttgaagaggtgggtgatgaaggtggctccgctccacacagcatcctctgccgcccgcaggtcagccactgagtgccctagggacacgcagatgccacgggccgtcagcgcccggatcacttcgtggctacggcccaactctggggccagcgtcacgatgcggacattgtccaggggcccgtaggtggccagcaagtcctggaaggcatcggcctcgaaggagcggaggtgggcctcggggtgcgcgccccgcttctcccggctgatgaaggggccctccaggtgcagcccgaggacccctgccccatggggaccaccactcttcacagggatctgaggaacaaccttgtgataaacctccggtggggaagtgaccagggtggggcagaaggaggtgacgccgtgcgacaggatcctccgggccacgagggcaacccccgaacccacgtcctccgtggcttgagagaagtcaacaccaaatccaccgttgatctgcacgtcgatgaatccgggagccaagatgcggcccccgcagtcccgccgctcgtcggccacgcgccgctcctcaaagaacagcttctctgggtccaagatgcggcctccgcgcacccacagatcctccctgagcagtttccctccgcgcaggatccggcagttagtgaactggagcacgcgggcccccgccgcgccctgctcgccgcgcatcgtgagccgtgtcgggagcgagcggctccggagccccgcggcggccaaatcccgcgcccagtgacgaac

SEQ ID NO: 10643 - RNA, 2629 nt, Homo sapiens
  source 1..2629: mol_type = other RNA
cgggagctggggtctgcaggttccctctcaaacctgggcccaaagtgcttttcctttccaggacctggcccagagggaagagaggagtgaggcagagcctgagacccagaaaagaaagctcactcccgggacccctgggccgggggacctgccctcccaaaacctgccttcccaagatgcccttgaagggctgggctcggacccgcacctgggccaggagagagcagaacttcaaagaccaccaaggatggacacccctgagtctgagaggaggaccctcaggatcagaaagcggagacccctcagcgtaagagagccgaggcctcctggggcgagatcaaagatgctcctcagagtcagaaggtgaagacacacgggggccagagcccaagggctcctcagggtcagagggaggagtcgaagagaatttagtcctaagtgccagggaaaggcgagtccccagagtccagggaagaagatgctgcggtcttgggaaggcaatatctcacaagcctgggaggtggctcccggagaggccactgtgcagcccccagaggaaggcgacccccatagccatccgagggactcctgcgggtccctgaaagcacagactccaaagcctgtgggcagggagagcccaaacctccggagaaggactaccacgctgacgcagagcatgatcaaaggcgagccacaaaggtcggcaccggcggtggcaaagctgggggccgcccgggagggggcgtgggctgcgcttacccgcccgaagcccccggcccggcggcggctcccaggtcgcggagccggagccgagatgccagcgaccctgcgcgccgaggtatccgggcagcaggggctcctcggggctctccggggcccccaggcctggagcgcgatccgcacgggctgcagggccctggagtgggccccgcaccgggggagcaggaggtgggccaggcttggcttccgggtgccctccggggtcgggtggggcggccctgagcgtcccaaggccttgaaggccgcgtggccggcgcccctcagcaccgccaaggcgcctgcgggcttaagcgcggcgcagcaggtgacggctctgcagcggctgctggagctgcacagcgcggccaggcggcagcgccgccggcgggaccgtgagcagcagcggctccgggtgtgtccccacgccgggatcggggcctgcctggagcgggcggggcaccgaggggcggccggacgctgactgccgcctctgcaggtcctggaacgcctccacatcgccaggaaccgccactgccgggttcaccccgtggggctcccgcccagtccggctcaactcccgccacaggcaagacccctagaaggcggtggggccacaaggagcctgcgcggggcaggggccgagcttagcgcgcccgggtccctttgaagtgagcgcactgcactctggcagtgactcggcggggcgcgaggggcaggtgtgccaggtgctgccccgcccgccccactgagccgcggacgctcagcgctccgcaccgccaggaggacgcggctgggcggcggcgcgccctgcgggagcagctggagcaaatgcatcgggagaggacggagcggctgcgggccctcggggccaggtgaggggcgggcaaggaggggtgtggcggtggcaggaggcccctttccctggcctccgaaatgacaagccgctctctccccaggaacacccagaacttcctggaactactgtgttcccctggtgctgaggatcccgtgcctgcgaagtagtgctcgcccttcccagcaccctctggtcattgctgagtcctcaaagggatgattaaagtgatgagggttacggaaaaagcaagagggcaacttgcaggtctgatagtttcagaaaggcctgaatgcaacctcagggacagggagagcagaggggcacagacacacacagcagctttgccccaccaggaggcctgttatttcttcttccctcccctaagcccacacctggcccacggtcagagggccaggtctcggggatcaagcagtgcgaaggccccgttcttgcggaagaatgactcaatgcggcacatcttgcaggagaccagttcttgcttcactggggggcccagctgccagccatacgtgaagctggtggtgatggggaagaggtatcgcgtctctggcatgtccagttttcgagtgttgaggtagcggtaccgcccctggaagtcgtgggagatgccttcatacagcagggctcgggtgataggtggtaccgggtacatttccgactgaaaaggcgcctctgggacagggctgggcaccttggaaggggctgacttgggggcgggtgggggtgagagtggggctttggggtgcagggtgggcagtttgaggggcaggcgggctgcagccttagccttctgcttggccttcaccatcgacccatacttgcggtaccattcacagcgcaacatcttttccctcagatattcctccttccagaagttctgccgtaacgcgtctatgttgagctgccgtgacatggtggccagggaaggagtggcaccagggtggccacagctgaggggtgagcacagcaagcagagtgcttctgacggcgagt

SEQ ID NO: 10644 - RNA, 1188 nt, Homo sapiens
  source 1..1188: mol_type = other RNA
cgggccggaggtcaagggcgtactggtagctgactccgatctccgtgtggctctggaggaataactccttgttgtggcttatccagtcaaacatcttctcagcatcctgctcgaagagccgcagctgaaagcactggtccagcttgagcttgcgcacatgccacatctggtgcaggtgctgccgggtggagtgcagcttgtccaggagactggtgatcttgggcaccaggctctggaagtcagcactgcccgggatgcagttgcgtcctgagaagccgtcgctgcagcggatgcactgcagcagccgctgcccctcccggtccagctcctccacaggggccttcagcacctttttcttgagctgtgtgtgttcgtcaatgagccgccgagagccctccacatccacaggaaactccttccgggctagcatctcctggaggtcctcgaggcgcgagagcaggtgcacggcgctgttgaagaactcctccagggagagccgcagttcgatccactcctcatggttgtagtccagggagccatcaaactcctccgtcagctgggaggggtccaccagctttgtgaggccctccacagataccatgctcgtctcaaagatgaatttggagctgccaaagttggtcttctgtttctgccagaagttgtcgggtttaatgatgagggccacatggatctcagctggaaaggcttcctgcagcgttttgaggaggggcttgatgaggtcccacttggagccccgcatgtcgatgatgacagtgaagccacgtttgcacacgtcctcacttggcacgctggccaaatacgtcacgagtttccgcaggtcttcctgtcttattctgtcatgattgctgcgagcagggaaggtcaggatgggtccgcctcgcttatcacgacccccagacacgaaggccaccttttcctttaggataggaaggacatcagaagctttcaaaccatcattccgaaaagaccctcgatccagcagccggagcaagcggagataccagagataccactggtcccagaagcggtccgtcatcccaccctgaactcatccttcacagccagtcccctcggcagagcctcatcccaccaccgctgactcgaggaggccggaatcacttgacgctgggctcgcacacagcctgctctaagcaaatgcctgcctgc

SEQ ID NO: 10645 - RNA, 1214 nt, Homo sapiens
  source 1..1214: mol_type = other RNA
cgggccggaggtcaagggcgtactggtagctgactccgatctccgtgtggctctggaggaataactccttgttgtggcttatccagtcaaacatcttctcagcatcctgctcgaagagccgcagctgaaagcactggtccagcttgagcttgcgcacatgccacatctggtgcaggtgctgccgggtggagtgcagcttgtccaggagactggtgatcttgggcaccaggctctggaagtcagcactgcccgggatgcagttgcgtcctgagaagccgtcgctgcagcggatgcactgcagcagccgctgcccctcccggtccagctcctccacaggggccttcagcacctttttcttgagctgtgtgtgttcgtcaatgagccgccgagagccctccacatccacaggaaactccttccgggctagcatctcctggaggtcctcgaggcgcgagagcaggtgcacggcgctgttgaagaactcctccagggagagccgcagttcgatccactcctcatggttgtagtccagggagccatcaaactcctccgtcagctgggaggggtccaccagctttgtgaggccctccacagataccatgctcgtctcaaagatgaatttggagctgccaaagttggtcttctgtttctgccagaagttgtcgggtttaatgatgagggccacatggatctcagctggaaaggcttcctgcagcgttttgaggaggggcttgatgaggtcccacttggagccccgcatgtcgatgatgacagtgaagccacgtttgcacacgtcctcacttggcacgctggccaaatacgtcacgagtttccgcaggtcttcctgtcttattctgtcatgattgctgcgagcagggaaggtcaggatgggtccgcctcgcttatcacgacccccagacacgaaggccaccttttcctttaggataggaaggacatcagaagctttcaaaccatcattccgaaaagaccctcgatccagcagccggagcaagcggagataccagagataccactggtcccagaagcggtccgtcatcccaccctgaactcatccttcacagccagtcccctcggcagagcctcatcccaccaccgctgactcgaggaggccggaatcacttgacgctgggctcgcacacagcctgctctaagcaaatgcctgcctgcaaagacagccaccagtcctcccacac

SEQ ID NO: 10646 - RNA, 1435 nt, Homo sapiens
  source 1..1435: mol_type = other RNA
cgggccggaggtcaagggcgtactggtagctgactccgatctccgtgtggctctggaggaataactccttgttgtggcttatccagtcaaacatcttctcagcatcctgctcgaagagccgcagctgaaagcactggtccagcttgagcttgcgcacatgccacatctggtgcaggtgctgccgggtggagtgcagcttgtccaggagactggtgatcttgggcaccaggctctggaagtcagcactgcccgggatgcagttgcgtcctgagaagccgtcgctgcagcggatgcactgcagcagccgctgcccctcccggtccagctcctccacaggggccttcagcacctttttcttgagctgtgtgtgttcgtcaatgagccgccgagagccctccacatccacaggaaactccttccgggctagcatctcctggaggtcctcgaggcgcgagagcaggtgcacggcgctgttgaagaactcctccagggagagccgcagttcgatccactcctcatggttgtagtccagggagccatcaaactcctccgtcagctgggaggggtccaccagctttgtgaggccctccacagataccatgctcgtctcaaagatgaatttggagctgccaaagttggtcttctgtttctgccagaagttgtcgggtttaatgatgagggccacatggatctcagctggaaaggcttcctgcagcgttttgaggaggggcttgatgaggtcccacttggagccccgcatgtcgatgatgacagtgaagccacgtttgcacacgtcctcacttggcacgctggccaaatacgtcacgagtttccgcaggtcttcctgtcttattctgtcatgattgctgcgagcagggaaggtcaggatgggtccgcctcgcttatcacgacccccagacacgaaggccaccttttcctttaggataggaaggacatcagaagctttcaaaccatcattccgaaaagaccctgtccggaaaaaggcgtccacgtccgagtctgctgctcctccttcctccgctgctccctcaggggggttcatgactgtgggagggcgtccgcgggcagccgggagccgaagaagcctggggccgagggctgctcggcgcccggtgggcggagggcgcggggcgcagctgctgcggccgcagagctggcggccgcggagcttcgagggcgggcgttgggcggcggggctggggcagaggacgctgagcctccctcaggcggaggcgcgcggcgggctgggggtgcctgccgccagctcccccatggtaccccttccccagggcgctggccgcctgctgtctggctggggccggggcccggggccggggtgcgggctgcctgggcgcccgctgtcccccagcagcggcagctggctctcctgctcgcccgtctgcctgtctctatt

SEQ ID NO: 10647 - RNA, 1455 nt, Homo sapiens
  source 1..1455: mol_type = other RNA
cgggccggaggtcaagggcgtactggtagctgactccgatctccgtgtggctctggaggaataactccttgttgtggcttatccagtcaaacatcttctcagcatcctgctcgaagagccgcagctgaaagcactggtccagcttgagcttgcgcacatgccacatctggtgcaggtgctgccgggtggagtgcagcttgtccaggagactggtgatcttgggcaccaggctctggaagtcagcactgcccgggatgcagttgcgtcctgagaagccgtcgctgcagcggatgcactgcagcagccgctgcccctcccggtccagctcctccacaggggccttcagcacctttttcttgagctgtgtgtgttcgtcaatgagccgccgagagccctccacatccacaggaaactccttccgggctagcatctcctggaggtcctcgaggcgcgagagcaggtgcacggcgctgttgaagaactcctccagggagagccgcagttcgatccactcctcatggttgtagtccagggagccatcaaactcctccgtcagctgggaggggtccaccagctttgtgaggccctccacagataccatgctcgtctcaaagatgaatttggagctgccaaagttggtcttctgtttctgccagaagttgtcgggtttaatgatgagggccacatggatctcagctggaaaggcttcctgcagcgttttgaggaggggcttgatgaggtcccacttggagccccgcatgtcgatgatgacagtgaagccacgtttgcacacgtcctcacttggcacgctggccaaatacgtcacgagtttccgcaggtcttcctgtcttattctgtcatgattgctgcgagcagggaaggtcaggatgggtccgcctcgcttatcacgacccccagacacgaaggccaccttttcctttaggataggaaggacatcagaagctttcaaaccatcattccgaaaagaccctgtccggaaaaaggcgtccacgtccgagtctgctgctcctccttcctccgctgctccctcaggggggttcatgactgtgggagggcgtccgcgggcagccgggagccgaagaagcctggggccgagggctgctcggcgcccggtgggcggagggcgcggggcgcagctgctgcggccgcagagctggcggccgcggagcttcgagggcgggcgttgggcggcggggctggggcagaggacgctgagcctccctcaggcggaggcgcgcggcgggctgggggtgcctgccgccagctcccccatggtaccccttccccagggcgctggccgcctgctgtctggctggggccggggcccggggccggggtgcgggctgcctgggcgcccgctgtcccccagcagcggcagctggctctcctgctcgcccgtctgcctgtctctattgttcagccctgctccgctct

SEQ ID NO: 10648 - RNA, 1456 nt, Homo sapiens
  source 1..1456: mol_type = other RNA
cgggccggaggtcaagggcgtactggtagctgactccgatctccgtgtggctctggaggaataactccttgttgtggcttatccagtcaaacatcttctcagcatcctgctcgaagagccgcagctgaaagcactggtccagcttgagcttgcgcacatgccacatctggtgcaggtgctgccgggtggagtgcagcttgtccaggagactggtgatcttgggcaccaggctctggaagtcagcactgcccgggatgcagttgcgtcctgagaagccgtcgctgcagcggatgcactgcagcagccgctgcccctcccggtccagctcctccacaggggccttcagcacctttttcttgagctgtgtgtgttcgtcaatgagccgccgagagccctccacatccacaggaaactccttccgggctagcatctcctggaggtcctcgaggcgcgagagcaggtgcacggcgctgttgaagaactcctccagggagagccgcagttcgatccactcctcatggttgtagtccagggagccatcaaactcctccgtcagctgggaggggtccaccagctttgtgaggccctccacagataccatgctcgtctcaaagatgaatttggagctgccaaagttggtcttctgtttctgccagaagttgtcgggtttaatgatgagggccacatggatctcagctggaaaggcttcctgcagcgttttgaggaggggcttgatgaggtcccacttggagccccgcatgtcgatgatgacagtgaagccacgtttgcacacgtcctcacttggcacgctggccaaatacgtcacgagtttccgcaggtcttcctgtcttattctgtcatgattgctgcgagcagggaaggtcaggatgggtccgcctcgcttatcacgacccccagacacgaaggccaccttttcctttaggataggaaggacatcagaagctttcaaaccatcattccgaaaagaccctgtccggaaaaaggcgtccacgtccgagtctgctgctcctccttcctccgctgctccctcaggggggttcatgactgtgggagggcgtccgcgggcagccgggagccgaagaagcctggggccgagggctgctcggcgcccggtgggcggagggcgcggggcgcagctgctgcggccgcagagctggcggccgcggagcttcgagggcgggcgttgggcggcggggctggggcagaggacgctgagcctccctcaggcggaggcgcgcggcgggctgggggtgcctgccgccagctcccccatggtaccccttccccagggcgctggccgcctgctgtctggctggggccggggcccggggccggggtgcgggctgcctgggcgcccgctgtcccccagcagcggcagctggctctcctgctcgcccgtctgcctgtctctattgttcagccctgctccgctctc

SEQ ID NO: 10649 - RNA, 1459 nt, Homo sapiens
  source 1..1459: mol_type = other RNA
cgggccggaggtcaagggcgtactggtagctgactccgatctccgtgtggctctggaggaataactccttgttgtggcttatccagtcaaacatcttctcagcatcctgctcgaagagccgcagctgaaagcactggtccagcttgagcttgcgcacatgccacatctggtgcaggtgctgccgggtggagtgcagcttgtccaggagactggtgatcttgggcaccaggctctggaagtcagcactgcccgggatgcagttgcgtcctgagaagccgtcgctgcagcggatgcactgcagcagccgctgcccctcccggtccagctcctccacaggggccttcagcacctttttcttgagctgtgtgtgttcgtcaatgagccgccgagagccctccacatccacaggaaactccttccgggctagcatctcctggaggtcctcgaggcgcgagagcaggtgcacggcgctgttgaagaactcctccagggagagccgcagttcgatccactcctcatggttgtagtccagggagccatcaaactcctccgtcagctgggaggggtccaccagctttgtgaggccctccacagataccatgctcgtctcaaagatgaatttggagctgccaaagttggtcttctgtttctgccagaagttgtcgggtttaatgatgagggccacatggatctcagctggaaaggcttcctgcagcgttttgaggaggggcttgatgaggtcccacttggagccccgcatgtcgatgatgacagtgaagccacgtttgcacacgtcctcacttggcacgctggccaaatacgtcacgagtttccgcaggtcttcctgtcttattctgtcatgattgctgcgagcagggaaggtcaggatgggtccgcctcgcttatcacgacccccagacacgaaggccaccttttcctttaggataggaaggacatcagaagctttcaaaccatcattccgaaaagaccctgtccggaaaaaggcgtccacgtccgagtctgctgctcctccttcctccgctgctccctcaggggggttcatgactgtgggagggcgtccgcgggcagccgggagccgaagaagcctggggccgagggctgctcggcgcccggtgggcggagggcgcggggcgcagctgctgcggccgcagagctggcggccgcggagcttcgagggcgggcgttgggcggcggggctggggcagaggacgctgagcctccctcaggcggaggcgcgcggcgggctgggggtgcctgccgccagctcccccatggtaccccttccccagggcgctggccgcctgctgtctggctggggccggggcccggggccggggtgcgggctgcctgggcgcccgctgtcccccagcagcggcagctggctctcctgctcgcccgtctgcctgtctctattgttcagccctgctccgctctctcc

SEQ ID NO: 10650 - RNA, 1460 nt, Homo sapiens
  source 1..1460: mol_type = other RNA
cgggccggaggtcaagggcgtactggtagctgactccgatctccgtgtggctctggaggaataactccttgttgtggcttatccagtcaaacatcttctcagcatcctgctcgaagagccgcagctgaaagcactggtccagcttgagcttgcgcacatgccacatctggtgcaggtgctgccgggtggagtgcagcttgtccaggagactggtgatcttgggcaccaggctctggaagtcagcactgcccgggatgcagttgcgtcctgagaagccgtcgctgcagcggatgcactgcagcagccgctgcccctcccggtccagctcctccacaggggccttcagcacctttttcttgagctgtgtgtgttcgtcaatgagccgccgagagccctccacatccacaggaaactccttccgggctagcatctcctggaggtcctcgaggcgcgagagcaggtgcacggcgctgttgaagaactcctccagggagagccgcagttcgatccactcctcatggttgtagtccagggagccatcaaactcctccgtcagctgggaggggtccaccagctttgtgaggccctccacagataccatgctcgtctcaaagatgaatttggagctgccaaagttggtcttctgtttctgccagaagttgtcgggtttaatgatgagggccacatggatctcagctggaaaggcttcctgcagcgttttgaggaggggcttgatgaggtcccacttggagccccgcatgtcgatgatgacagtgaagccacgtttgcacacgtcctcacttggcacgctggccaaatacgtcacgagtttccgcaggtcttcctgtcttattctgtcatgattgctgcgagcagggaaggtcaggatgggtccgcctcgcttatcacgacccccagacacgaaggccaccttttcctttaggataggaaggacatcagaagctttcaaaccatcattccgaaaagaccctgtccggaaaaaggcgtccacgtccgagtctgctgctcctccttcctccgctgctccctcaggggggttcatgactgtgggagggcgtccgcgggcagccgggagccgaagaagcctggggccgagggctgctcggcgcccggtgggcggagggcgcggggcgcagctgctgcggccgcagagctggcggccgcggagcttcgagggcgggcgttgggcggcggggctggggcagaggacgctgagcctccctcaggcggaggcgcgcggcgggctgggggtgcctgccgccagctcccccatggtaccccttccccagggcgctggccgcctgctgtctggctggggccggggcccggggccggggtgcgggctgcctgggcgcccgctgtcccccagcagcggcagctggctctcctgctcgcccgtctgcctgtctctattgttcagccctgctccgctctctcct

SEQ ID NO: 10651 - RNA, 1462 nt, Homo sapiens
  source 1..1462: mol_type = other RNA
cgggccggaggtcaagggcgtactggtagctgactccgatctccgtgtggctctggaggaataactccttgttgtggcttatccagtcaaacatcttctcagcatcctgctcgaagagccgcagctgaaagcactggtccagcttgagcttgcgcacatgccacatctggtgcaggtgctgccgggtggagtgcagcttgtccaggagactggtgatcttgggcaccaggctctggaagtcagcactgcccgggatgcagttgcgtcctgagaagccgtcgctgcagcggatgcactgcagcagccgctgcccctcccggtccagctcctccacaggggccttcagcacctttttcttgagctgtgtgtgttcgtcaatgagccgccgagagccctccacatccacaggaaactccttccgggctagcatctcctggaggtcctcgaggcgcgagagcaggtgcacggcgctgttgaagaactcctccagggagagccgcagttcgatccactcctcatggttgtagtccagggagccatcaaactcctccgtcagctgggaggggtccaccagctttgtgaggccctccacagataccatgctcgtctcaaagatgaatttggagctgccaaagttggtcttctgtttctgccagaagttgtcgggtttaatgatgagggccacatggatctcagctggaaaggcttcctgcagcgttttgaggaggggcttgatgaggtcccacttggagccccgcatgtcgatgatgacagtgaagccacgtttgcacacgtcctcacttggcacgctggccaaatacgtcacgagtttccgcaggtcttcctgtcttattctgtcatgattgctgcgagcagggaaggtcaggatgggtccgcctcgcttatcacgacccccagacacgaaggccaccttttcctttaggataggaaggacatcagaagctttcaaaccatcattccgaaaagaccctgtccggaaaaaggcgtccacgtccgagtctgctgctcctccttcctccgctgctccctcaggggggttcatgactgtgggagggcgtccgcgggcagccgggagccgaagaagcctggggccgagggctgctcggcgcccggtgggcggagggcgcggggcgcagctgctgcggccgcagagctggcggccgcggagcttcgagggcgggcgttgggcggcggggctggggcagaggacgctgagcctccctcaggcggaggcgcgcggcgggctgggggtgcctgccgccagctcccccatggtaccccttccccagggcgctggccgcctgctgtctggctggggccggggcccggggccggggtgcgggctgcctgggcgcccgctgtcccccagcagcggcagctggctctcctgctcgcccgtctgcctgtctctattgttcagccctgctccgctctctcctct

SEQ ID NO: 10652 - RNA, 1463 nt, Homo sapiens
  source 1..1463: mol_type = other RNA
cgggccggaggtcaagggcgtactggtagctgactccgatctccgtgtggctctggaggaataactccttgttgtggcttatccagtcaaacatcttctcagcatcctgctcgaagagccgcagctgaaagcactggtccagcttgagcttgcgcacatgccacatctggtgcaggtgctgccgggtggagtgcagcttgtccaggagactggtgatcttgggcaccaggctctggaagtcagcactgcccgggatgcagttgcgtcctgagaagccgtcgctgcagcggatgcactgcagcagccgctgcccctcccggtccagctcctccacaggggccttcagcacctttttcttgagctgtgtgtgttcgtcaatgagccgccgagagccctccacatccacaggaaactccttccgggctagcatctcctggaggtcctcgaggcgcgagagcaggtgcacggcgctgttgaagaactcctccagggagagccgcagttcgatccactcctcatggttgtagtccagggagccatcaaactcctccgtcagctgggaggggtccaccagctttgtgaggccctccacagataccatgctcgtctcaaagatgaatttggagctgccaaagttggtcttctgtttctgccagaagttgtcgggtttaatgatgagggccacatggatctcagctggaaaggcttcctgcagcgttttgaggaggggcttgatgaggtcccacttggagccccgcatgtcgatgatgacagtgaagccacgtttgcacacgtcctcacttggcacgctggccaaatacgtcacgagtttccgcaggtcttcctgtcttattctgtcatgattgctgcgagcagggaaggtcaggatgggtccgcctcgcttatcacgacccccagacacgaaggccaccttttcctttaggataggaaggacatcagaagctttcaaaccatcattccgaaaagaccctgtccggaaaaaggcgtccacgtccgagtctgctgctcctccttcctccgctgctccctcaggggggttcatgactgtgggagggcgtccgcgggcagccgggagccgaagaagcctggggccgagggctgctcggcgcccggtgggcggagggcgcggggcgcagctgctgcggccgcagagctggcggccgcggagcttcgagggcgggcgttgggcggcggggctggggcagaggacgctgagcctccctcaggcggaggcgcgcggcgggctgggggtgcctgccgccagctcccccatggtaccccttccccagggcgctggccgcctgctgtctggctggggccggggcccggggccggggtgcgggctgcctgggcgcccgctgtcccccagcagcggcagctggctctcctgctcgcccgtctgcctgtctctattgttcagccctgctccgctctctcctctt

SEQ ID NO: 10653 - RNA, 22 nt, Homo sapiens
  source 1..22: mol_type = other RNA
cgggcgccgcgctcccgcccgc

SEQ ID NO: 10654 - RNA, 47 nt, Homo sapiens
  source 1..47: mol_type = other RNA
cgggcgccgcgctcccgcccgccgcctcccaccacctccgccgccaa

SEQ ID NO: 10655 - RNA, 99 nt, Homo sapiens
  source 1..99: mol_type = other RNA
cgggcgccgcgctcccgcccgccgcctcccaccacctccgccgccaagcgcccgatccgcccgcaaggcctccctccgcaccacccgcggccgccgttc

SEQ ID NO: 10656 - RNA, 670 nt, Homo sapiens
  source 1..670: mol_type = other RNA
cgggcgccgcgctcccgcccgcgctccgaggcccaggcccggtcgcgttcccgctcgaggccgccccccggcccgggtcccccagcagcagcagcagcagcagccccaggagcgggagctccggcccccgcgctgggcgggcagcggccatggccaaccccgccaactcagcaaaagccccggcgcccccgcctgctcctcggagccccccggccacacgcacgacctcggcggccgcggaggcggctcaggcgacctgtgcgcccagagaatccgggcccgggcccccccggacgctccgcgcgccccggcccctcggcgcccaacttcgcaaactttggaacccggggcccatgttgggctgcggaggcccggaacgggatgcacgactccccaagccctagcctcgcaatccaagttgtcttcagccctaggagacccctgggcccccaatccccagccccattccctctcccaccattaaagccacctccccgccccgcgagggaggccagacgcgggccgggggtgcgagtgcagctccggctccgcccccgcgccagcccgcggcccagcagccaccttcgccccagcgcgccgcagccccccgaactctccccgccggcgacccggctcctttgttgctctagctcgctgggctctctggaat

SEQ ID NO: 10657 - RNA, 94 nt, Homo sapiens
  source 1..94: mol_type = other RNA
cgggcgccgcgctcccgcccgctcgctccgcccctccccgcagcgcgtccaggccgtggcccgcctatggcgcagccgccacccgaagtctcct

SEQ ID NO: 10658 - RNA, 1226 nt, Homo sapiens
  source 1..1226: mol_type = other RNA
cgggcgtggtggtgggggcctgtaatcctagctattccggaggctgaggcaggagaatcgcttgaaccaaggaggcagaggttgcagtgagccgagatcatgctattgcactccagcctgggcaacagaatgagaatccatctaaacaaaaaacaaacaaacaaacaaaaccaaaaaaccttccaaagggttccctgcatggggcaaaatttgtttttcactgctatgcataggaaggattaagaaagtggaacaaattcctttgtaactatagcatctctcatatttgaatggcaagcatgttcaatctgttgctgcatgttaagaaaatattgaggatatatatgaataaagcaaaacaagaaaaaaggttaaattatgagctttaaaaattaaaataaaaatctgtttttaagccaagtaggtgtgattctgataattattacatatgacataacccatagaaagcaaggccaagaaaaaaaaacttcatatcggtcagttcttggacttgatattgtcctaggaaaaacagtgataattcaacaaatgcatcacacatacaactaaaaagtctccttctggtttcagataaatttaaacaacaatcttcctaggctattttttctcctgtgtctaataaaccttctacgtgcaaggccagtgtaaatccctccaccctttcaaacactagagctgaacatccaggaacattttgcaatgcaaagtgctttgagaaagagatggattctgtagtgccagtggcataactgatcaaggaagctgggaagagattaacgctgatgggagccagtcaggcaatggtggtttgtttctctccttgggtgttcctccatcagctgcatgatcagttcatagagggctctgcagatctttgcagagccctctccatccaggacaaatctgttgtgctgagatatccatctgtcgtctccttgaatatcttccactgcatgtggaatagctgctgtgtttgagtcggcttgattcattctacactcacgtagagagtccatggaggccttacagggttgcagcattgacgggtggtgcgtctgtcactcgctcagtccctgtggccctcctccggcgcggacctcctcgggccccagcaccagcagcaaccttgttttgtggtttagaaggagccttttctcagcagtttcatgatcaaaagcacatattgcaagagggaatcaaatata

SEQ ID NO: 10659 - RNA, 2755 nt, Homo sapiens
  source 1..2755: mol_type = other RNA
cgggcgtggtggtggggggccctggcctccactcccgactccgcgggcaggctttcggcctgcttctggccccgtcagctgtgcagtctcctccttagggggctccttcttgggtggtggagtttgtatcttggccacttcatcactgcctgggggccaggggagtggacggggccctggttcctccagaggaaagcgagagattgggggcccaggggctccattctcaggaaagcctggataactggccagatagggtggtgggggaggtactggaggagtctcgctcctcatccccttgtcatcctcatccgcagcctggcgcagaggtgaggtaagtgggcggggttcagcgggtgtggcggtgaagacatctcctacccaggccaactttggatccaccggtggagtgccccgttcccgtaacatagcaggtgcatgacggtcaaatggctctgagcttgagcccccactgtctgaacgctctcggggaactaggccagagggatgcacaccaggagggtagaagtctagagggggacgaccctggaggagccgggggtccacataaggaggaatcatcatccatcggggatcaaagttcattgggggcatgggtgggggccggcccagagcacctgggtacagggccttggggggcgggggtggagcctgtggagctggcacagcccccagggtcacaggctgtggtggtgatgggggcactggggtaggaggggcagagccctgttgatgctgctgccactggtgctgctgctgctgcttcaggagctgctcctgctgctgccgctggaaacgaggaggcaacgacttctgatatttggggtagcccaagccctgactagggggctggcgggtgggaccaatcccatcacccttgggttccacctttggaactgggggtgtggtaggaggaggaacctcttctggtggttcaggaccctcttttgagggcagttgtggttccactgggctggcttcgaagctgccactgctggtgctactggtactgccaccaccactcaccagagtgggagccgcagccacacctggagtaggagtagattgggcaggaggggcctgtgctggctcttcaggttctgtctctggtgttggggctgatgctggaggtggagctggaggtgcagggagttctttagggactgcaggtggtggagctggggtagaaggggcagcaggtggggcagcaggctctgctttgagccgcttgtcaggtgccccaaacttttcatcgagtcgcttgagcttctcagcacaggctgcccggcgctcttcttgcatgcgccgctcctcttcttctcgccgtcgccgggcccgctccactgccagggaaatctcagatgacgactgctttcgtcgctgccgccatgcctcatcctcatcttcaggtgctgggggcttgcagggaggacccccacgatctgggtagtccccaggggggccccagttcccggcggggccccggtgaggtgggggtaggggaggctttggggcaggaggtcccggctctgtctctggaggccgagaggtttctgcccaggccgtcttaggagtgggcggttcgctgttgggggagttgccctttttgccatctgcttcagggggccgttcctcaccagaagctgattgggaatccctgtggccctcagcaccctcctcatcagagtctcgcccatcttcctcatcgctgaacttgagcttttcagtgtagtcaacctcttcatgggcccctgcccaaccatcatcattctcctgatccaactgatcaaactctttgagattatcctctttgagaatagagggacgacccacaggctctactaagcgcattggtggccctgagcctcgggggcccgccacacggggaaaacggctgggcccatcaggagtggggtatcggtaaggcccctggggtccatagggcggagggaacgggagatatgggggatacatgaaaggcggcatcattccgcggtagggagggaactggggtgggcctgaaggctgtagcccaccccggggatcatgaccatgatgaagtttggagtccgggccctccagctcatcagggccacgcccacctccgtccctccaagttgtagaattttgggggcggaggcttggtccgggcccagacgactgttcggcagactccctttccttggcagccttgtcctggtcgccagccgcctgcagggtcggaaattcctctcgagagaatcgtgacagtaggcttgatgcccttccaccatctccatgtgctccatgggtgacgctggcttgtgcccaggactttaccccgcttggaaccaaaggagtgttctcgggggctgctgggggtcgtttcggctggttggaggcaggcgtctgtgaagccggcagtggctgcgattccggcggctgagcggttgaggcatcggaactcttggggtcggactgctcctgtttgcttgcccatcctgttccgtcttttggcactagtgagacattggggtcattgcctttgttctcggctttcaggcttggaaggttggctggaggtggcatacgccgggcaatggcaactttcccgagactctgcaggccatggcgaggggcaacagcgggtttctggatctctaaggacttgcccttatacgtatcaaacaggttgagcgaggaatacttctttccatcctttcccttggcagtcggccccgagcgatcggacatt

SEQ ID NO: 10660 - RNA, 2961 nt, Homo sapiens
  source 1..2961: mol_type = other RNA
cgggcgtggtggtggggggccctggcctccactcccgactccgcgggcaggctttcggcctgcttctggccccgtcagctgtgcagtctcctccttagggggctccttcttgggtggtggagtttgtatcttggccacttcatcactgcctgggggccaggggagtggacggggccctggttcctccagaggaaagcgagagattgggggcccaggggctccattctcaggaaagcctggataactggccagatagggtggtgggggaggtactggaggagtctcgctcctcatccccttgtcatcctcatccgcagcctggcgcagaggtgaggtaagtgggcggggttcagcgggtgtggcggtgaagacatctcctacccaggccaactttggatccaccggtggagtgccccgttcccgtaacatagcaggtgcatgacggtcaaatggctctgagcttgagcccccactgtctgaacgctctcggggaactaggccagagggatgcacaccaggagggtagaagtctagagggggacgaccctggaggagccgggggtccacataaggaggaatcatcatccatcggggatcaaagttcattgggggcatgggtgggggccggcccagagcacctgggtacagggccttggggggcgggggtggagcctgtggagctggcacagcccccagggtcacaggctgtggtggtgatgggggcactggggtaggaggggcagagccctgttgatgctgctgccactggtgctgctgctgctgcttcaggagctgctcctgctgctgccgctggaaacgaggaggcaacgacttctgatatttggggtagcccaagccctgactagggggctggcgggtgggaccaatcccatcacccttgggttccacctttggaactgggggtgtggtaggaggaggaacctcttctggtggttcaggaccctcttttgagggcagttgtggttccactgggctggcttcgaagctgccactgctggtgctactggtactgccaccaccactcaccagagtgggagccgcagccacacctggagtaggagtagattgggcaggaggggcctgtgctggctcttcaggttctgtctctggtgttggggctgatgctggaggtggagctggaggtgcagggagttctttagggactgcaggtggtggagctggggtagaaggggcagcaggtggggcagcaggctctgctttgagccgcttgtcaggtgccccaaacttttcatcgagtcgcttgagcttctcagcacaggctgcccggcgctcttcttgcatgcgccgctcctcttcttctcgccgtcgccgggcccgctccactgccagggaaatctcagatgacgactgctttcgtcgctgccgccatgcctcatcctcatcttcaggtgctgggggcttgcagggaggacccccacgatctgggtagtccccaggggggccccagttcccggcggggccccggtgaggtgggggtaggggaggctttggggcaggaggtcccggctctgtctctggaggccgagaggtttctgcccaggccgtcttaggagtgggcggttcgctgttgggggagttgccctttttgccatctgcttcagggggccgttcctcaccagaagctgattgggaatccctgtggccctcagcaccctcctcatcagagtctcgcccatcttcctcatcgctgaacttgagcttttcagtgtagtcaacctcttcatgggcccctgcccaaccatcatcattctcctgatccaactgatcaaactctttgagattatcctctttgagaatagagggacgacccacaggctctactaagcgcattggtggccctgagcctcgggggcccgccacacggggaaaacggctgggcccatcaggagtggggtatcggtaaggcccctggggtccatagggcggagggaacgggagatatgggggatacatgaaaggcggcatcattccgcggtagggagggaactggggtgggcctgaaggctgtagcccaccccggggatcatgaccatgatgaagtttggagtccgggccctccagctcatcagggccacgcccacctccgtccctccaagttgtagaattttgggggcggaggcttggtccgggcccagacgactgttcggcagactccctttccttggcagccttgtcctggtcgccagccgcctgcagggtcggaaattcctctcgagagaatcgtgacagtaggcttgatgcccttccaccatctccatgtgctccatgggtgacgctggcttgtgcccaggactttaccccgcttggaaccaaaggagtgttctcgggggctgctgggggtcgtttcggctggttggaggcaggcgtctgtgaagccggcagtggctgcgattccggcggctgagcggttgaggcatcggaactcttggggtcggactgctcctgtttgcttgcccatcctgttccgtcttttggcactagtgagacattggggtcattgcctttgttctcggctttcaggcttggaaggttggctggaggtggcatacgccgggcaatggcaactttcccgagactctgcaggccatggcgaggggcaacagcgggtttctggatctctaaggacttgcccttatacgtatcaaacaggttgagcgaggaatacttctttccatcctttcccttggcagtcggccccgagcgatcggacattgcgctggaagctcattgagtatgttgggtcctgcaggcacctcccccaaaacgtgccagagcctggccgggtgcgcggggatccgggacccgggcctaggggctccccgggacgggatggcggtggggcgggggaggatggcggcggatggcgccgggttcggctcctcccgtctccctcgctcactccgcggctgagccccgact

SEQ ID NO: 10661 - RNA, 2998 nt, Homo sapiens
  source 1..2998: mol_type = other RNA
cgggcgtggtggtggggggccctggcctccactcccgactccgcgggcaggctttcggcctgcttctggccccgtcagctgtgcagtctcctccttagggggctccttcttgggtggtggagtttgtatcttggccacttcatcactgcctgggggccaggggagtggacggggccctggttcctccagaggaaagcgagagattgggggcccaggggctccattctcaggaaagcctggataactggccagatagggtggtgggggaggtactggaggagtctcgctcctcatccccttgtcatcctcatccgcagcctggcgcagaggtgaggtaagtgggcggggttcagcgggtgtggcggtgaagacatctcctacccaggccaactttggatccaccggtggagtgccccgttcccgtaacatagcaggtgcatgacggtcaaatggctctgagcttgagcccccactgtctgaacgctctcggggaactaggccagagggatgcacaccaggagggtagaagtctagagggggacgaccctggaggagccgggggtccacataaggaggaatcatcatccatcggggatcaaagttcattgggggcatgggtgggggccggcccagagcacctgggtacagggccttggggggcgggggtggagcctgtggagctggcacagcccccagggtcacaggctgtggtggtgatgggggcactggggtaggaggggcagagccctgttgatgctgctgccactggtgctgctgctgctgcttcaggagctgctcctgctgctgccgctggaaacgaggaggcaacgacttctgatatttggggtagcccaagccctgactagggggctggcgggtgggaccaatcccatcacccttgggttccacctttggaactgggggtgtggtaggaggaggaacctcttctggtggttcaggaccctcttttgagggcagttgtggttccactgggctggcttcgaagctgccactgctggtgctactggtactgccaccaccactcaccagagtgggagccgcagccacacctggagtaggagtagattgggcaggaggggcctgtgctggctcttcaggttctgtctctggtgttggggctgatgctggaggtggagctggaggtgcagggagttctttagggactgcaggtggtggagctggggtagaaggggcagcaggtggggcagcaggctctgctttgagccgcttgtcaggtgccccaaacttttcatcgagtcgcttgagcttctcagcacaggctgcccggcgctcttcttgcatgcgccgctcctcttcttctcgccgtcgccgggcccgctccactgccagggaaatctcagatgacgactgctttcgtcgctgccgccatgcctcatcctcatcttcaggtgctgggggcttgcagggaggacccccacgatctgggtagtccccaggggggccccagttcccggcggggccccggtgaggtgggggtaggggaggctttggggcaggaggtcccggctctgtctctggaggccgagaggtttctgcccaggccgtcttaggagtgggcggttcgctgttgggggagttgccctttttgccatctgcttcagggggccgttcctcaccagaagctgattgggaatccctgtggccctcagcaccctcctcatcagagtctcgcccatcttcctcatcgctgaacttgagcttttcagtgtagtcaacctcttcatgggcccctgcccaaccatcatcattctcctgatccaactgatcaaactctttgagattatcctctttgagaatagagggacgacccacaggctctactaagcgcattggtggccctgagcctcgggggcccgccacacggggaaaacggctgggcccatcaggagtggggtatcggtaaggcccctggggtccatagggcggagggaacgggagatatgggggatacatgaaaggcggcatcattccgcggtagggagggaactggggtgggcctgaaggctgtagcccaccccggggatcatgaccatgatgaagtttggagtccgggccctccagctcatcagggccacgcccacctccgtccctccaagttgtagaattttgggggcggaggcttggtccgggcccagacgactgttcggcagactccctttccttggcagccttgtcctggtcgccagccgcctgcagggtcggaaattcctctcgagagaatcgtgacagtaggcttgatgcccttccaccatctccatgtgctccatgggtgacgctggcttgtgcccaggactttaccccgcttggaaccaaaggagtgttctcgggggctgctgggggtcgtttcggctggttggaggcaggcgtctgtgaagccggcagtggctgcgattccggcggctgagcggttgaggcatcggaactcttggggtcggactgctcctgtttgcttgcccatcctgttccgtcttttggcactagtgagacattggggtcattgcctttgttctcggctttcaggcttggaaggttggctggaggtggcatacgccgggcaatggcaactttcccgagactctgcaggccatggcgaggggcaacagcgggtttctggatctctaaggacttgcccttatacgtatcaaacaggttgagcgaggaatacttctttccatcctttcccttggcagtcggccccgagcgatcggacattgcgctggaagctcattgagtatgttgggtcctgcaggcacctcccccaaaacgtgccagagcctgtgggccagacagcaagtgtctcagtctctgtcccctggccgggtgcgcggggatccgggacccgggcctaggggctccccgggacgggatggcggtggggcgggggaggatggcggcggatggcgccgggttcggctcctcccgtctccctcgctcactccgcggctgagccccgact

SEQ ID NO: 10662 - RNA, 950 nt, Homo sapiens
  source 1..950: mol_type = other RNA
cgggcgtggtggtgggggtgaaggcaggcaagggcactgcacacaggtgggatggggaggaaaggagggtccccgctagaggcgatgggcttcaaggaacatgctggtgggcagaggctgtggtccttgagtcctttatgctgcctccagcttctgtacaggctcaccgagacatcattcgcacaaactcttcgaagtcgaccagaccgtccccattgaggtccacgtcctggaggatctcgtccacctcccgctggctgaggcgctcccccagcagggccttgagggccgcccggagctcgcccacgctgatgcggccgtccccattggtgtcgaactcccggaaggcgtcccgtagctcccggacaccgatcatgtctgccgtctctgccagcagcttggggcccatcagctccacgaagtcttcaaagtccacctttccgccactgatttgttgtgagatctcgatgagctccatctcggtgggcatgtagcccagggtccgcatgcaggcacccagctcccggcagccaatgtagccgtcccggtctcggtcaaactcctggaaggcgacctgcagctcttcaatctcctcgggccgcagctcccggtcatacgagttgggtggcggcaatgctgggccgcaggaagatgcaggcaggccccaccaggctgttgagcaccgagtagccctggacgcctggcgcggggtccccctgctccttggggctggagctggggctggggcaggagccccttggtggggagccgagccactgcaaggggtccttagggccccggcgccagggccgcttggcacagttccccatgggccctgaaccatgccaggcctggaaccccgggggtggcccgggtgggcctcggcggatgctgctgcctgaggactcctgccagcccccagctgctcccgatgagagcctgggagtact

SEQ ID NO: 10663 - RNA, 946 nt, Homo sapiens
  source 1..946: mol_type = other RNA
cgggcgtggtggtgggggtgaaggcaggcaagggcactgcacacaggtgggatggggaggaaaggagggtccccgctagaggcgatgggcttcaaggaacatgctggtgggcagaggctgtggtccttgagtcctttatgctgcctccagcttctgtacaggctcaccgagacatcattcgcacaaactcttcgaagtcgaccagaccgtccccattgaggtccacgtcctggaggatctcgtccacctcccgctggctgaggcgctcccccagcagggccttgagggccgcccggagctcgcccacgctgatgcggccgtccccattggtgtcgaactcccggaaggcgtcccgtagctcccggacaccgatcatgtctgccgtctctgccagcagcttggggcccatcagctccacgaagtcttcaaagtccacctttccgccactgatttgttgtgagatctcgatgagctccatctcggtgggcatgtagcccagggtccgcatgcaggcacccagctcccggcagccaatgtagccgtcccggtctcggtcaaactcctggaaggcgacctgcagctcttcaatctcctcgggccgcagctcccggtcgagttgggtggcggcaatgctgggccgcaggaagatgcaggcaggccccaccaggctgttgagcaccgagtagccctggacgcctggcgcggggtccccctgctccttggggctggagctggggctggggcaggagccccttggtggggagccgagccactgcaaggggtccttagggccccggcgccagggccgcttggcacagttccccatgggccctgaaccatgccaggcctggaaccccgggggtggcccgggtgggcctcggcggatgctgctgcctgaggactcctgccagcccccagctgctcccgatgagagcctgggagtact

SEQ ID NO: 10664 - RNA, 1443 nt, Homo sapiens
  source 1..1443: mol_type = other RNA
cgggcgtggtggtgggggtgatggtgggggtggtggtgggggtgggggggggtgggcctgatgggggtgtgggcatgatgatgatgggcgtgatgatgatggggggtgatgatgggcatgatgatgggggtgatggtgcccaggcccttcagcaccgcaatatgctgcggaagttcttccggaagttgtcatctagaaaggcgtagaggaaggggttcaggcacgagttggcgtagctgaggctggtgatgacgtaggacatactgatgaccagtggggtctggggcaggtccgtggtcagggccacgacagaggccaggtggaagggcgtccagcagaggaggcacacggccagcacgacgaggaccaggacggtcaccttccgcctggccttgcctagagccttggctccagagcggagccgcacggcccgcagcctgcgcaggaggtctgtgtagagcacacagatggtgcacacgggcagcacgaagcccaggaccaacgtgtagacacggctggccttgaaccagacctgctcgggccacgggaagctcagcccacagcttgggacctgcagctcgttgctgtagacgccagcgaaagagaagaagggcagaaccaggaccgtgacgcccagccagacacacaggctggcgaccttcgccccccggtaggtgcgccagggcatgtggcgggacctcacggtggccagcaccaccaggtatcggtccacgctcatcacggctaggaagtagatgctggagaagatgttgtagtggtcgacggccagcaccagcttgcagagcagctccccgaagggccagtactgcagcaggtgctccgcgatgttgacgggcagtaccagcgtgaagagcccgtcggcgacggccaggttcaggatgaacacgttggtcaccgtcttcatcttgggcgcccttaggattacaaggatgacggccgtgttgccagtcagccccacagcacagatcccggagtacacggcgggcaggagcacatagaggaacggcagtggctcggagaaggtggcattgtggccagtgccattgtcctgagagacgttggcacccatcgtggggagggagaaggagcccctgctgtcaaggggctctgggtgcccagcggcctgcattgtagctgggaccgttgacgatttgcgccctgggcaggtgggaggtgccttggagttgggtatctggttgggggcctccttgggctggattctgtccagtgcttcgagtccagaagttggtagccttggtgtgttcctggttttggccagtacaggcagtcgcagggatggagggcgaggtgtggtcctcactgacagacctccagctgaggtttcaggagtttcaagacctgccctgctggctgcctcagccccggctgcgaggttcccagcctggtgtcagtgctgatgct

SEQ ID NO: 10665 - RNA, 591 nt, Homo sapiens
  source 1..591: mol_type = other RNA
cgggcgtggtggtgggggtgccggcgggggagccggtggagacagaggcaggggtggcgcctccatgcggggttcctccacaggaagggtatgtgccagcctggccaggctattggccttcttctgttcctgctctcgctcctgctccaagcgaagccgctcctgctcctcacgtgctctctgttgttgctgcgcttgccattccaggaagcgggccgcctccagtagcgtctctatgctcatcgcgccgagagctgccgggggcgcgccggggccgaggctgcggcccgcgagccgggcacaggtcaggctggcgggcaggcaggagggagggatcacctccggggggcgacagggctgggcggcgcagcgcactccgcagggaagaacgggggagcacggggagaaaaatcaatgtctctcaaaatatttgcaaaatataaaattgcaaatttaaaaaaatgggatgcaaaaaaaaaaaaaaggcggcactgcctcccttcttcccctccctctctacctcccttccgatgcctcccgccccgcggcccccgggagtcccgccgacaagaaagggctttgcaacaagat

SEQ ID NO: 10666 - RNA, 432 nt, Homo sapiens
  source 1..432: mol_type = other RNA
cgggcgtggtggtgggggtgccggcgggggagccggtggagacagaggcaggggtggcgcctccatgcggggttcctccacaggaagggtatgtgccagcctggccaggctattggccttcttctgttcctgctctcgctcctgctccaagcgaagccgctcctgctccttcgaactgcaacgtgttgatggcggcagcaggtgacttaatctctccgaaccttgtgcacggtcttcccctgacccctgtgcccaaacgtaggacattcttggtcaccaggggcactctccactgccagaccctgctctggaccatcaaggcaacagccggggagtgtgggcgatgtccccgcccatcacttctgcaaaacccaggcatctgagcctcacatatctccagtgactcttgaccttgagaggccggtcgccccg

SEQ ID NO: 10667 - RNA, 1224 nt, Homo sapiens
  source 1..1224: mol_type = other RNA
cgggcgtggtggtgggggtgcctctttctttctttgcttcattgtttcccctacagcattatcatagtgctaggcacataccaaggaatcaaagaacatttgttgattcagagattgattgattctgaggcacttgagtacatttgtaaatatcctttgaggatcttgcatcccattggaataaaacacttcatgttttattcagttctttccccatatgcaaatgtgcaggtgccccgatggcatatagataacatcattacacacacacacacacacacacactcctgcacaccaaagaaatgactgctcacatagatgacacgattagaggaagtattggggtttaatgcaagaatgattggatatattccccagatgcttacgtcctgcatttgcagggcatcctttcctacaagctccatgaagcaagagttagttaagctagacaacctgggatagagcaataaaaactagacaaggagccaggatgtttttagttctaggtctacaattcgtagctatgtgaccttgagcaagtcacgtcagcaagccaaacttcagtttctgatctgtttatgtgattccctgcatggccttgctgcttctccttgggaccaaactgtactattggtgccagcctatgagctctggtcccactattgcctgtaggaatttagcttgctcctcaactgttttttgttaatctgtttgattttggcttgatcctcacaggcaataagagctggcataagtagcttgagatacgcctcagttgtatcttcagtaacatagcgataatattgcctacctcccaggctcctctctttagggtctgttgccagcctggcagatatttgtgggtttctgatcagcacctggatttcctgtccttcccccttgagtgctcctggaacagtagagagctttgtagaccatgttggacaatttgaaccttatctgaaggcccttctgttatgtcccttttttgagtggaagtgtttgttgtagtcgttttattcctcttcatcattgtatcttttgtgtttcggggacataacctgtctttatattcagaggctgtggattataagcagctgcatccagacatgatgtcaatcacaagatcttggtggaggtcctccagttctcttaacatagtcaaatgtatctcctcttgttagccaattatgattccttccctcatctgtgaacatccaaagg

SEQ ID NO: 10668 - RNA, 1452 nt, Homo sapiens
  source 1..1452: mol_type = other RNA
cgggcgtggtggtgggggtgcctgggtctgctgggccagcgactctgactctgctcctcctcactgttgctttgcacctcctccaagtcaaaagtgtcctgtggctgctggcttaaagaccgacgcagttctggtctgtctacactctgcttccatttctgctgggtgatggacaggtccaaggacttaaccttcctgcccatgagattcttctggaagaggctctttcttgctctgctctttcttttccagaaagtctcatccttggctggatgggtttccgtattggtggctggtagactacacagctctctccttatctgagctgggtctgtgctccactgtggatcttctatgggcagagaatgtgtgcaacagggtaccttggggttcgaatccagagtttgggatggtgctagcactgtggacatcctctgctgtgtttcctcttcacagcagaagacacatggatagggagaagtgggcaacttcttaccctcagcagggggcacaggatcttcctgtgagaattgccccaaatcagagtcttgctggaggaactgcttctcttctttcactttgtccatcacttccaacacaacttggtccaaactgttccttttgggggtgttgtggggtggtggtggccggtctcgggggcatgtgtacagacacatcttggagatggctttccgaaggcggtctctgggtgactggggttcaggctctcgggacagaatcctgatggatggcacatcagttggatggttgcaattccagaacatgtgggatggtgtgaacttttggacaggtgtcttagacacataggagtagagacagaagaaggcatcagcagtgacagccagtgtttgcacctgcttaaacctgcctgggacttcaggaagagctggaaatcaatgcccttggcctgagagggggtggtgaaaaatcgggcgggtatccgagaagtgtctttgtgatcctcttggccaaagcccagactgaagaggacatcttctgcatcttcttgcactttgtccagaatttctgagatgctggagaagagtttgccattggcggccagtagtgtggcctccgctcccagggtcaagtcatcttcaaagctggtcccatggctgcagaagccattgtagataaactgtcctgcttcctcagaaaatccttcttcagagtatccgcaatcctgcagccagtcttcaattttattgattggattccctagaaaagtcagacactagatcactgtgagaactgaacgaaatcagacctcctccctgcaactaattccattccacaagtttattcttacataagctgcgtcatgaatctttttttctacataaagcttttctttaagatatgagaggaatacaccgtatataaaaatagtagatatttcttctctctctctgcttcttttctcccttcctc

SEQ ID NO: 10669 - RNA, 1551 nt, Homo sapiens
  source 1..1551: mol_type = other RNA
cgggcgtggtggtgggggtgcctgggtctgctgggccagcgactctgactctgctcctcctcactgttgctttgcacctcctccaagtcaaaagtgtcctgtggctgctggcttaaagaccgacgcagttctggtctgtctacactctgcttccatttctgctgggtgatggacaggtccaaggacttaaccttcctgcccatgagattcttctggaagaggctctttcttgctctgctctttcttttccagaaagtctcatccttggctggatgggtttccgtattggtggctggtagactacacagctctctccttatctgagctgggtctgtgctccactgtggatcttctatgggcagagaatgtgtgcaacagggtaccttggggttcgaatccagagtttgggatggtgctagcactgtggacatcctctgctgtgtttcctcttcacagcagaagacacatggatagggagaagtgggcaacttcttaccctcagcagggggcacaggatcttcctgtgagaattgccccaaatcagagtcttgctggaggaactgcttctcttctttcactttgtccatcacttccaacacaacttggtccaaactgttccttttgggggtgttgtggggtggtggtggccggtctcgggggcatgtgtacagacacatcttggagatggctttccgaaggcggtctctgggtgactggggttcaggctctcgggacagaatcctgatggatggcacatcagttggatggttgcaattccagaacatgtgggatggtgtgaacttttggacaggtgtcttagacacataggagtagagacagaagaaggcatcagcagtgacagccagtgtttgcacctgcttaaacctgcctgggacttcaggaagagctggaaatcaatgcccttggcctgagagggggtggtgaaaaatcgggcgggtatccgagaagtgtctttgtgatcctcttggccaaagcccagactgaagaggacatcttctgcatcttcttgcactttgtccagaatttctgagatgcttgaactagtcttgttggtccccccagtcatgctgctggaagccaaactacagccaagatcaagtagctggcaaggcctggctgtctcgaggaaactcctggagaagagtttgccattggcggccagtagtgtggcctccgctcccagggtcaagtcatcttcaaagctggtcccatggctgcagaagccattgtagataaactgtcctgcttcctcagaaaatccttcttcagagtatccgcaatcctgcagccagtcttcaattttattgattggattccctagaaaagtcagacactagatcactgtgagaactgaacgaaatcagacctcctccctgcaactaattccattccacaagtttattcttacataagctgcgtcatgaatctttttttctacataaagcttttctttaagatatgagaggaatacaccgtatataaaaatagtagatatttcttctctctctctgcttcttttctcccttcctc

SEQ ID NO: 10670 - RNA, 1672 nt, Homo sapiens
  source 1..1672: mol_type = other RNA
cgggcgtggtggtgggggtgcctgggtctgctgggccagcgactctgactctgctcctcctcactgttgctttgcacctcctccaagtcaaaagtgtcctgtggctgctggcttaaagaccgacgcagttctggtctgtctacactctgcttccatttctgctgggtgatggacaggtccaaggacttaaccttcctgcccatgagattcttctggaagaggctctttcttgctctgctctttcttttccagaaagtctcatccttggctggatgggtttccgtattggtggctggtagactacacagctctctccttatctgagctgggtctgtgctccactgtggatcttctatgggcagagaatgtgtgcaacagggtaccttggggttcgaatccagagtttgggatggtgctagcactgtggacatcctctgctgtgtttcctcttcacagcagaagacacatggatagggagaagtgggcaacttcttaccctcagcagggggcacaggatcttcctgtgagaattgccccaaatcagagtcttgctggaggaactgcttctcttctttcactttgtccatcacttccaacacaacttggtccaaactgttccttttgggggtgttgtggggtggtggtggccggtctcgggggcatgtgtacagacacatcttggagatggctttccgaaggcggtctctgggtgactggggttcaggctctcgggacagaatcctgatggatggcacatcagttggatggttgcaattccagaacatgtgggatggtgtgaacttttggacaggtgtcttagacacataggagtagagacagaagaaggcatcagcagtgacagccagtgtttgcacctgcttaaacctgcctgggacttcaggaagagctggaaatcaatgcccttggcctgagagggggtggtgaaaaatcgggcgggtatccgagaagtgtctttgtgatcctcttggccaaagcccagactgaagaggacatcttctgcatcttcttgcactttgtccagaatttctgagatgcttgaactagtcttgttggtccccccagtcatgctgctggaagccaaactacagccaagatcaagtagctggcaaggcctggctgtctcgaggaaactcctggagaagagtttgccattggcggccagtagtgtggcctccgctcccagggtcaagtcatcttcaaagctggtcccatggctgcagaagccattgtagataaactgtcctgcttcctcagaaaatccttcttcagagtatctaaaccaaaaacagtcttataggttgaagtcacttactacattttccaaggagctttttcatggaaaaactcacacatattcatattcttttccagtgagagtcagtagtatttaatttgccgcaatcctgcagccagtcttcaattttattgattggattccctagaaaagtcagacactagatcactgtgagaactgaacgaaatcagacctcctccctgcaactaattccattccacaagtttattcttacataagctgcgtcatgaatctttttttctacataaagcttttctttaagatatgagaggaatacaccgtatataaaaatagtagatatttcttctctctctctgcttcttttctcccttcctc

SEQ ID NO: 10671 - RNA, 1495 nt, Homo sapiens
  source 1..1495: mol_type = other RNA
cgggcgtggtggtgggggtgcctgggtctgctgggccagcgactctgactctgctcctcctcactgttgctttgcacctcctccaagtcaaaagtgtcctgtggctgctggcttaaagaccgacgcagttctggtctgtctacactctgcttccatttctgctgggtgatggacaggtccaaggacttaaccttcctgcccatgagattcttctggaagaggctctttcttgctctgctctttcttttccagaaagtctcatccttggctggatgggtttccgtattggtggctggtagactacacagctctctccttatctgagctgggtctgtgctccactgtggatcttctatgggcagagaatgtgtgcaacagggtaccttggggttcgaatccagagtttgggatggtgctagcactgtggacatcctctgctgtgtttcctcttcacagcagaagacacatggatagggagaagtgggcaacttcttaccctcagcagggggcacaggatcttcctgtgagaattgccccaaatcagagtcttgctggaggaactgcttctcttctttcactttgtccatcacttccaacacaacttggtccaaactgttccttttgggggtgttgtggggtggtggtggccggtctcgggggcatgtgtacagacacatcttggagatggctttccgaaggcggtctctgggtgactggggttcaggctctcgggacagaatcctgatggatggcacatcagttggatggttgcaattccagaacatgtgggatggtgtgaacttttggacaggtgtcttagacacataggagtagagacagaagaaggcatcagcagtgacagccagtgtttgcacctgcttaaacctgctggccagcatgaggcaggggtcttccatttcaatcctccgcacctgggacttcaggaagagctggaaatcaatgcccttggcctgagagggggtggtgaaaaatcgggcgggtatccgagaagtgtctttgtgatcctcttggccaaagcccagactgaagaggacatcttctgcatcttcttgcactttgtccagaatttctgagatgctggagaagagtttgccattggcggccagtagtgtggcctccgctcccagggtcaagtcatcttcaaagctggtcccatggctgcagaagccattgtagataaactgtcctgcttcctcagaaaatccttcttcagagtatccgcaatcctgcagccagtcttcaattttattgattggattccctagaaaagtcagacactagatcactgtgagaactgaacgaaatcagacctcctccctgcaactaattccattccacaagtttattcttacataagctgcgtcatgaatctttttttctacataaagcttttctttaagatatgagaggaatacaccgtatataaaaatagtagatatttcttctctctctctgcttcttttctcccttcctc

SEQ ID NO: 10672 - RNA, 1733 nt, Homo sapiens
  source 1..1733: mol_type = other RNA
cgggcgtggtggtgggggtgcctgggtctgctgggccagcgactctgactctgctcctcctcactgttgctttgcacctcctccaagtcaaaagtgtcctgtggctgctggcttaaagaccgacgcagttctggtctgtctacactctgcttccatttctgctgggtgatggacaggtccaaggacttaaccttcctgcccatgagattcttctggaagaggctctttcttgctctgctctttcttttccagaaagtctcatccttggctggatgggtttccgtattggtggctggtagactacacagctctctccttatctgagctgggtctgtgctccactgtggatcttctatgggcagagaatgtgtgcaacagggtaccttggggttcgaatccagagtttgggatggtgctagcactgtggacatcctctgctgtgtttcctcttcacagcagaagacacatggatagggagaagtgggcaacttcttaccctcagcagggggcacaggatcttcctgtgagaattgccccaaatcagagtcttgctggaggaactgcttctcttctttcactttgtccatcacttccaacacaacttggtccaaactgttccttttgggggtgttgtggggtggtggtggccggtctcgggggcatgtgtacagacacatcttggagatggctttccgaaggcggtctctgggtgactggggttcaggctctcgggacagaatcctgatggatggcacatcagttggatggttgcaattccagaacatgtgggatggtgtgaacttttggacaggtgtcttagacacataggagtagagacagaagaaggcatcagcagtgacagccagtgtttgcacctgcttaaacctgctggccagcatgaggcaggggtcttccatttcaatcctccgcacctgggacttcaggaagagctggaaatcaatgcccttggcctgagagggggtggtgaaaaatcgggcgggtatccgagaagtgtctttgtgatcctcttggccaaagcccagactgaagaggacatcttctgcatcttcttgcactttgtccagaatttctgagatgcttgaactagtcttgttggtccccccagtcatgctgctggaagccaaactacagccaagatcaagtagctggcaaggcctggctgtctcgaggaaactcctgcagagatcaaagctgatgtcatacaaatcttgtttccagtctgcaccctggcttcgaggaatccctgctggacttattcaccccctgaacagtagtctatgcagtgcttgttcgttggaaagtctcactctctaatgtgaatctttagctctttattttaatctctttgacctaccccaattcactgattcttaaaggagacatcattcaccctggctgaacctaacacttacctggagaagagtttgccattggcggccagtagtgtggcctccgctcccagggtcaagtcatcttcaaagctggtcccatggctgcagaagccattgtagataaactgtcctgcttcctcagaaaatccttcttcagagtatctaaaccaaaaacagtcttataggttgaagtcacttactacattttccaaggagctttttcatggaaaaactcacacatattcatattcttttccagtgagagtcagtagtatttaatttgccgcaatcctgcagccagtcttcaattttattgattgg

SEQ ID NO: 10673 - RNA, 1503 nt, Homo sapiens
  source 1..1503: mol_type = other RNA
cgggcgtggtggtgggggtgcctgggtctgctgggccagcgactctgactctgctcctcctcactgttgctttgcacctcctccaagtcaaaagtgtcctgtggctgctggcttaaagaccgacgcagttctggtctgtctacactctgcttccatttctgctgggtgatggacaggtccaaggacttaaccttcctgcccatgagattcttctggaagaggctctttcttgctctgctctttcttttccagaaagtctcatccttggctggatgggtttccgtattggtggctggtagactacacagctctctccttatctgagctgggtctgtgctccactgtggatcttctatgggcagagaatgtgtgcaacagggtaccttggggttcgaatccagagtttgggatggtgctagcactgtggacatcctctgctgtgtttcctcttcacagcagaagacacatggatagggagaagtgggcaacttcttaccctcagcagggggcacaggatcttcctgtgagaattgccccaaatcagagtcttgctggaggaactgcttctcttctttcactttgtccatcacttccaacacaacttggtccaaactgttccttttgggggtgttgtggggtggtggtggccggtctcgggggcatgtgtacagacacatcttggagatggctttccgaaggcggtctctgggtgactggggttcaggctctcgggacagaatcctgatggatggcacatcagttggatggttgcaattccagaacatgtgggatggtgtgaacttttggacaggtgtcttagacacataggagtagagacagaagaaggcatcagcagtgacagccagtgtttgcacctgcttaaacctgctggccagcatgaggcaggggtcttccatttcaatcctccgcacctgggacttcaggaagagctggaaatcaatgcccttggcctgagagggggtggtgaaaaatcgggcgggtatccgagaagtgtctttgtgatcctcttggccaaagcccagactgaagaggacatcttctgcatcttcttgcactttgtccagaatttctgagatgcttgaactagtcttgttggtccccccagtcatgctgctggaagccaaactacagccaagatcaagtagctggcaaggcctggctgtctcgaggaaactcctggagaagagtttgccattggcggccagtagtgtggcctccgctcccagggtcaagtcatcttcaaagctggtcccatggctgcagaagccattgtagataaactgtcctgcttcctcagaaaatccttcttcagagtatccgcaatcctgcagccagtcttcaattttattgattggattccataagctgcgtcatgaatctttttttctacataaagcttttctttaagatatgagaggaatacaccgtatataaaaatagtagatatttcttctctctctctgcttcttttctcccttcctc

SEQ ID NO: 10674 - RNA, 1594 nt, Homo sapiens
  source 1..1594: mol_type = other RNA
cgggcgtggtggtgggggtgcctgggtctgctgggccagcgactctgactctgctcctcctcactgttgctttgcacctcctccaagtcaaaagtgtcctgtggctgctggcttaaagaccgacgcagttctggtctgtctacactctgcttccatttctgctgggtgatggacaggtccaaggacttaaccttcctgcccatgagattcttctggaagaggctctttcttgctctgctctttcttttccagaaagtctcatccttggctggatgggtttccgtattggtggctggtagactacacagctctctccttatctgagctgggtctgtgctccactgtggatcttctatgggcagagaatgtgtgcaacagggtaccttggggttcgaatccagagtttgggatggtgctagcactgtggacatcctctgctgtgtttcctcttcacagcagaagacacatggatagggagaagtgggcaacttcttaccctcagcagggggcacaggatcttcctgtgagaattgccccaaatcagagtcttgctggaggaactgcttctcttctttcactttgtccatcacttccaacacaacttggtccaaactgttccttttgggggtgttgtggggtggtggtggccggtctcgggggcatgtgtacagacacatcttggagatggctttccgaaggcggtctctgggtgactggggttcaggctctcgggacagaatcctgatggatggcacatcagttggatggttgcaattccagaacatgtgggatggtgtgaacttttggacaggtgtcttagacacataggagtagagacagaagaaggcatcagcagtgacagccagtgtttgcacctgcttaaacctgctggccagcatgaggcaggggtcttccatttcaatcctccgcacctgggacttcaggaagagctggaaatcaatgcccttggcctgagagggggtggtgaaaaatcgggcgggtatccgagaagtgtctttgtgatcctcttggccaaagcccagactgaagaggacatcttctgcatcttcttgcactttgtccagaatttctgagatgcttgaactagtcttgttggtccccccagtcatgctgctggaagccaaactacagccaagatcaagtagctggcaaggcctggctgtctcgaggaaactcctggagaagagtttgccattggcggccagtagtgtggcctccgctcccagggtcaagtcatcttcaaagctggtcccatggctgcagaagccattgtagataaactgtcctgcttcctcagaaaatccttcttcagagtatccgcaatcctgcagccagtcttcaattttattgattggattccctagaaaagtcagacactagatcactgtgagaactgaacgaaatcagacctcctccctgcaactaattccattccacaagtttattcttacataagctgcgtcatgaatctttttttctacataaagcttttctttaagatatgagaggaatacaccgtatataaaaatagtagatatttcttctctctctctgcttcttttctcccttcctc

SEQ ID NO: 10675 - RNA, 1747 nt, Homo sapiens
  source 1..1747: mol_type = other RNA
cgggcgtggtggtgggggtgcctgggtctgctgggccagcgactctgactctgctcctcctcactgttgctttgcacctcctccaagtcaaaagtgtcctgtggctgctggcttaaagaccgacgcagttctggtctgtctacactctgcttccatttctgctgggtgatggacaggtccaaggacttaaccttcctgcccatgagattcttctggaagaggctctttcttgctctgctctttcttttccagaaagtctcatccttggctggatgggtttccgtattggtggctggtagactacacagctctctccttatctgagctgggtctgtgctccactgtggatcttctatgggcagagaatgtgtgcaacagggtaccttggggttcgaatccagagtttgggatggtgctagcactgtggacatcctctgctgtgtttcctcttcacagcagaagacacatggatagggagaagtgggcaacttcttaccctcagcagggggcacaggatcttcctgtgagaattgccccaaatcagagtcttgctggaggaactgcttctcttctttcactttgtccatcacttccaacacaacttggtccaaactgttccttttgggggtgttgtggggtggtggtggccggtctcgggggcatgtgtacagacacatcttggagatggctttccgaaggcggtctctgggtgactggggttcaggctctcgggacagaatcctgatggatggcacatcagttggatggttgcaattccagaacatgtgggatggtgtgaacttttggacaggtgtcttagacacataggagtagagacagaagaaggcatcagcagtgacagccagtgtttgcacctgcttaaacctgctggccagcatgaggcaggggtcttccatttcaatcctccgcacctgggacttcaggaagagctggaaatcaatgcccttggcctgagagggggtggtgaaaaatcgggcgggtatccgagaagtgtctttgtgatcctcttggccaaagcccagactgaagaggacatcttctgcatcttcttgcactttgtccagaatttctgagatgcttgaactagtcttgttggtccccccagtcatgctgctggaagccaaactacagccaagatcaagtagctggcaaggcctggctgtctcgaggaaactcctggagaagagtttgccattggcggccagtagtgtggcctccgctcccagggtcaagtcatcttcaaagctggtcccatggctgcagaagccattgtagataaactgtcctgcttcctcagaaaatccttcttcagagtatccgcaatcctgcagccagtcttcaattttattgattggattcccttcttggaaaacgtcatccaggctggaaggctcaggatctgggacatcctgcagggcggcggcagcctcctcttctaggacctgggtctgccagttacggctctgacggagccaggcccgccgtttctcccaggatgtggggctcagcacagaggcctccatggccctggctcagacttcagggcctcccgtaacagtaatgccgtcaagttctgagttccagatgcatgctttcttcctttatatcatacagccttcctcctgccacacttggtttccaaggcccagtcccaggtttgcctttagtgctctaggggacatgtatgagacagacctctcttctcttctgtctgttttgtacctat

SEQ ID NO: 10676 - RNA, 2085 nt, Homo sapiens
  source 1..2085: mol_type = other RNA
cgggcgtggtggtgggggtgcctgggtctgctgggccagcgactctgactctgctcctcctcactgttgctttgcacctcctccaagtcaaaagtgtcctgtggctgctggcttaaagaccgacgcagttctggtctgtctacactctgcttccatttctgctgggtgatggacaggtccaaggacttaaccttcctgcccatgagattcttctggaagaggctctttcttgctctgctctttcttttccagaaagtctcatccttggctggatgggtttccgtattggtggctggtagactacacagctctctccttatctgagctgggtctgtgctccactgtggatcttctatgggcagagaatgtgtgcaacagggtaccttggggttcgaatccagagtttgggatggtgctagcactgtggacatcctctgctgtgtttcctcttcacagcagaagacacatggatagggagaagtgggcaacttcttaccctcagcagggggcacaggatcttcctgtgagaattgccccaaatcagagtcttgctggaggaactgcttctcttctttcactttgtccatcacttccaacacaacttggtccaaactgttccttttgggggtgttgtggggtggtggtggccggtctcgggggcatgtgtacagacacatcttggagatggctttccgaaggcggtctctgggtgactggggttcaggctctcgggacagaatcctgatggatggcacatcagttggatggttgcaattccagaacatgtgggatggtgtgaacttttggacaggtgtcttagacacataggagtagagacagaagaaggcatcagcagtgacagccagtgtttgcacctgcttaaacctgctggccagcatgaggcaggggtcttccatttcaatcctccgcacctgggacttcaggaagagctggaaatcaatgcccttggcctgagagggggtggtgaaaaatcgggcgggtatccgagaagtgtctttgtgatcctcttggccaaagcccagactgaagaggacatcttctgcatcttcttgcactttgtccagaatttctgagatgcttgaactagtcttgttggtccccccagtcatgctgctggaagccaaactacagccaagatcaagtagctggcaaggcctggctgtctcgaggaaactcctggagaagagtttgccattggcggccagtagtgtggcctccgctcccagggtcaagtcatcttcaaagctggtcccatggctgcagaagccattgtagataaactgtcctgcttcctcagaaaatccttcttcagagtatccgcaatcctgcagccagtcttcaattttattgattggattcccttcttggaaaacgtcatccaggctggaaggctcaggatctgggacatcctgcagggcggcggcagcctcctcttctaggacctgggtctgccagttacggctctgacggagccaggcccgccgtttctcccaggatgtggggctcagcacagaggcctccatggccctggctcagacttcagggcctcccgtaacagtaatgccgtcaagttctgagttccagatgcatgctttcttcctttatatcatacagccttcctcctgccacacttggtttccaaggcccagtcccaggtttgcctttagtgctctaggggacatgtatgagacagacctctcttctcttctgtctgttttgtacctatgccccaagcagtgcctcactcaagtgtgtacatcctccctcgtagctgacctcaatatatcttgctgcagtttatctcaacaagtttcttctacagcttctgaagaaagaggtcatacccacagaaagcaaagttgatttcagccaggtactctcaatggttggagctatggacactagagtagggcctgtctgctggtagaaagctgagtttgaggcaaagcagttgtcgaagctgggccgaggccttcacaggtgtgggcacagaggtgaagcaagtgagaaagtatcatgttgtagattatgcctttctccctgaactcattcaactgctgttgc

SEQ ID NO: 10677 - RNA, 2098 nt, Homo sapiens
  source 1..2098: mol_type = other RNA
cgggcgtggtggtgggggtgcctgggtctgctgggccagcgactctgactctgctcctcctcactgttgctttgcacctcctccaagtcaaaagtgtcctgtggctgctggcttaaagaccgacgcagttctggtctgtctacactctgcttccatttctgctgggtgatggacaggtccaaggacttaaccttcctgcccatgagattcttctggaagaggctctttcttgctctgctctttcttttccagaaagtctcatccttggctggatgggtttccgtattggtggctggtagactacacagctctctccttatctgagctgggtctgtgctccactgtggatcttctatgggcagagaatgtgtgcaacagggtaccttggggttcgaatccagagtttgggatggtgctagcactgtggacatcctctgctgtgtttcctcttcacagcagaagacacatggatagggagaagtgggcaacttcttaccctcagcagggggcacaggatcttcctgtgagaattgccccaaatcagagtcttgctggaggaactgcttctcttctttcactttgtccatcacttccaacacaacttggtccaaactgttccttttgggggtgttgtggggtggtggtggccggtctcgggggcatgtgtacagacacatcttggagatggctttccgaaggcggtctctgggtgactggggttcaggctctcgggacagaatcctgatggatggcacatcagttggatggttgcaattccagaacatgtgggatggtgtgaacttttggacaggtgtcttagacacataggagtagagacagaagaaggcatcagcagtgacagccagtgtttgcacctgcttaaacctgctggccagcatgaggcaggggtcttccatttcaatcctccgcacctgggacttcaggaagagctggaaatcaatgcccttggcctgagagggggtggtgaaaaatcgggcgggtatccgagaagtgtctttgtgatcctcttggccaaagcccagactgaagaggacatcttctgcatcttcttgcactttgtccagaatttctgagatgcttgaactagtcttgttggtccccccagtcatgctgctggaagccaaactacagccaagatcaagtagctggcaaggcctggctgtctcgaggaaactcctggagaagagtttgccattggcggccagtagtgtggcctccgctcccagggtcaagtcatcttcaaagctggtcccatggctgcagaagccattgtagataaactgtcctgcttcctcagaaaatccttcttcagagtatccgcaatcctgcagccagtcttcaattttattgattggattcccttcttggaaaacgtcatccaggctggaaggctcaggatctgggacatcctgcagggcggcggcagcctcctcttctaggacctgggtctgccagttacggctctgacggagccaggcccgccgtttctcccaggatgtggggctcagcacagaggcctccatggccctggctcagacttcagggcctcccgtaacagtaatgccgtcaagttctgagttccagatgcatgctttcttcctttatatcatacagccttcctcctgccacacttggtttccaaggcccagtcccaggtttgcctttagtgctctaggggacatgtatgagacagacctctcttctcttctgtctgttttgtacctatgccccaagcagtgcctgtgagttgagactcactcaagtgtgtacatcctccctcgtagctgacctcaatatatcttgctgcagtttatctcaacaagtttcttctacagcttctgaagaaagaggtcatacccacagaaagcaaagttgatttcagccaggtactctcaatggttggagctatggacactagagtagggcctgtctgctggtagaaagctgagtttgaggcaaagcagttgtcgaagctgggccgaggccttcacaggtgtgggcacagaggtgaagcaagtgagaaagtatcatgttgtagattatgcctttctccctgaactcattcaactgctgttgc

SEQ ID NO: 10678 - RNA, 3148 nt, Homo sapiens
  source 1..3148: mol_type = other RNA
cgggcgtggtggtgggggtgcctgggtctgctgggccagcgactctgactctgctcctcctcactgttgctttgcacctcctccaagtcaaaagtgtcctgtggctgctggcttaaagaccgacgcagttctggtctgtctacactctgcttccatttctgctgggtgatggacaggtccaaggacttaaccttcctgcccatgagattcttctggaagaggctctttcttgctctgctctttcttttccagaaagtctcatccttggctggatgggtttccgtattggtggctggtagactacacagctctctccttatctgagctgggtctgtgctccactgtggatcttctatgggcagagaatgtgtgcaacagggtaccttggggttcgaatccagagtttgggatggtgctagcactgtggacatcctctgctgtgtttcctcttcacagcagaagacacatggatagggagaagtgggcaacttcttaccctcagcagggggcacaggatcttcctgtgagaattgccccaaatcagagtcttgctggaggaactgcttctcttctttcactttgtccatcacttccaacacaacttggtccaaactgttccttttgggggtgttgtggggtggtggtggccggtctcgggggcatgtgtacagacacatcttggagatggctttccgaaggcggtctctgggtgactggggttcaggctctcgggacagaatcctgatggatggcacatcagttggatggttgcaattccagaacatgtgggatggtgtgaacttttggacaggtgtcttagacacataggagtagagacagaagaaggcatcagcagtgacagccagtgtttgcacctgcttaaacctgctggccagcatgaggcaggggtcttccatttcaatcctccgcacctgggacttcaggaagagctggaaatcaatgcccttggcctgagagggggtggtgaaaaatcgggcgggtatccgagaagtgtctttgtgatcctcttggccaaagcccagactgaagaggacatcttctgcatcttcttgcactttgtccagaatttctgagatgcttgaactagtcttgttggtccccccagtcatgctgctggaagccaaactacagccaagatcaagtagctggcaaggcctggctgtctcgaggaaactcctggagaagagtttgccattggcggccagtagtgtggcctccgctcccagggtcaagtcatcttcaaagctggtcccatggctgcagaagccattgtagataaactgtcctgcttcctcagaaaatccttcttcagagtatccgcaatcctgcagccagtcttcaattttattgattggattcccttcttggaaaacgtcatccaggctggaaggctcaggatctgggacatcctgcagggcggcggcagcctcctcttctaggacctgggtctgccagttacggctctgacggagccaggcccgccgtttctcccaggatgtggggctcagcacagaggcctccatggccctggctcagacttcagggcctcccgtaacagtaatgccgtcaagttctgagttccagatgcatgctttcttcctttatatcatacagccttcctcctgccacacttggtttccaaggcccagtcccaggtttgcctttagtgctctaggggacatgtatgagacagacctctcttctcttctgtctgttttgtacctatgccccaagcagtgcctgtgagttgagactgagagtgagaaccagtgtgggaggagagaagaaggaaatggggtttccatgatgtggcccataagaccttctgcatccacagccaagatatacatcattaccatcgcagagctgcgggaaatcccagagtagctaacatttctctgttcatgaactggacaaactccacctcaacccaggtggattgtcccccatttgacataccccaatctgcaacaaattctcacattccttcatagaactgtcttctagctcctaaccctcttccatgtcactcaggttggaagatcatcagaacaagaatttccctgagtataatatttgagcattctgagacttctattgtctaaggagcagttcaatctgttcggggaaaaggagagatgttacttggtaaataacagaaagaaaaaatgcccattagtcaatagaactcctattcccctcccttttcatactctttctcccacaaataagcgtagctgaataaatactgaaagaagaccatctaagacctttttcctctccttccctttcttccttacttccacttttaggatatgaattttaagaaaggcttgtataattgctacaggaaatattaaagttgtggatttggaaaaaaaattaatcgcttgttctcaatgtagggagacatcaaatatcttcatttgaatgggcaataaagacatcaagaataagaaacagcagtttatctgagctgatttatagatggcttcatcaagagaaagtagggagaatgagcagatttctcaaccattgtgttagctctgtgaattcgtatctttaattcttcagtttcatttccttggtaataagctctgtcctgcatatattcatttttcttctttcctgcttttctttttcaatatctacacactctcttctcctcgtccctctacttatttgactgaactcttttctcaatctgaaatctgtgtttaggccattctgcatcaggcctgggtgttgtaaggcacacagtactgtgggtactggaatatccactttggtcttgtgcctcactcaagtgtgtacatcctccctcgtagctgacctcaatatatcttgctgcagtttatctcaacaagtttcttctacagcttctgaagaaagaggtcatacccacagaaagcaaagttgatttcagccaggtactctcaatggttggagctatggacactagagtagggcctgtctgctggtagaaagctgagtttgaggcaaagcagttgtcgaagctgggccgaggccttcacaggtgtgggcacagaggtgaagcaagtgagaaagtatcatgttgtagattatgcctttctccctgaactcattcaactgctgttgcctgctc

SEQ ID NO: 10679 - RNA, 3054 nt, Homo sapiens
  source 1..3054: mol_type = other RNA
cgggcgtggtggtgggggtgcctgggtctgctgggccagcgactctgactctgctcctcctcactgttgctttgcacctcctccaagtcaaaagtgtcctgtggctgctggcttaaagaccgacgcagttctggtctgtctacactctgcttccatttctgctgggtgatggacaggtccaaggacttaaccttcctgcccatgagattcttctggaagaggctctttcttgctctgctctttcttttccagaaagtctcatccttggctggatgggtttccgtattggtggctggtagactacacagctctctccttatctgagctgggtctgtgctccactgtggatcttctatgggcagagaatgtgtgcaacagggtaccttggggttcgaatccagagtttgggatggtgctagcactgtggacatcctctgctgtgtttcctcttcacagcagaagacacatggatagggagaagtgggcaacttcttaccctcagcagggggcacaggatcttcctgtgagaattgccccaaatcagagtcttgctggaggaactgcttctcttctttcactttgtccatcacttccaacacaacttggtccaaactgttccttttgggggtgttgtggggtggtggtggccggtctcgggggcatgtgtacagacacatcttggagatggctttccgaaggcggtctctgggtgactggggttcaggctctcgggacagaatcctgatggatggcacatcagttggatggttgcaattccagaacatgtgggatggtgtgaacttttggacaggtgtcttagacacataggagtagagacagaagaaggcatcagcagtgacagccagtgtttgcacctgcttaaacctgctggccagcatgaggcaggggtcttccatttcaatcctccgcacctgggacttcaggaagagctggaaatcaatgcccttggcctgagagggggtggtgaaaaatcgggcgggtatccgagaagtgtctttgtgatcctcttggccaaagcccagactgaagaggacatcttctgcatcttcttgcactttgtccagaatttctgagatgcttgaactagtcttgttggtccccccagtcatgctgctggaagccaaactacagccaagatcaagtagctggcaaggcctggctgtctcgaggaaactcctggagaagagtttgccattggcggccagtagtgtggcctccgctcccagggtcaagtcatcttcaaagctggtcccatggctgcagaagccattgtagataaactgtcctgcttcctcagaaaatccttcttcagagtatccgcaatcctgcagccagtcttcaattttattgattggattcccttcttggaaaacgtcatccaggctggaaggctcaggatctgggacatcctgcagggcggcggcagcctcctcttctaggacctgggtctgccagttacggctctgacggagccaggcccgccgtttctcccaggatgtggggctcagcacagaggcctccatggccctggctcagacttcagggcctcccgtaacagtaatgccgtcaagttctgagttccagatgcatgctttcttcctttatatcatacagccttcctcctgccacacttggtttccaaggcccagtcccaggtttgcctttagtgctctaggggacatgtatgagacagacctctcttctcttctgtctgttttgtacctatgccccaagcagtgcctgtgagttgagactgagagtgagaaccagtgtgggaggagagaagaaggaaatggggtttccatgatgtggcccataagaccttctgcatccacagccaagatatacatcattaccatcgcagagctgcgggaaatcccagagtagctaacatttctctgttcatgaactggacaaactccacctcaacccaggtggattgtcccccatttgacataccccaatctgcaacaaattctcacattccttcatagaactgtcttctagctcctaaccctcttccatgtcactcaggttggaagatcatcagaacaagaatttccctgagtataatatttgagcattctgagacttctattgtctaaggagcagttcaatctgttcggggaaaaggagagatgttacttggtaaataacagaaagaaaaaatgcccattagtcaatagaactcctattcccctcccttttcatactctttctcccacaaataagcgtagctgaataaatactgaaagaagaccatctaagacctttttcctctccttccctttcttccttacttccacttttaggatatgaattttaagaaaggcttgtataattgctacaggaaatattaaagttgtggatttggaaaaaaaattaatcgcttgttctcaatgtagggagacatcaaatatcttcatttgaatgggcaataaagacatcaagaataagaaacagcagtttatctgagctgatttatagatggcttcatcaagagaaagtagggagaatgagcagatttctcaaccattgtgttagctctgtgaattcgtatctttaattcttcagtttcatttccttggtaataagctctgtcctgcatatattcatttttcttctttcctgcttttctttttcaatatctacacactctcttctcctcgtccctctacttatttgactgaactcttttctcaatctgaaatctgtgtttaggccattctgcatcaggcctgggtgttgtaaggcacacagtactgtgggtactggaatatccactttggtcttgtgcctcactcaagtgtgtacatcctccctcgtagctgacctcaatatatcttgctgcagtttatctcaacaagtttcttctacagcttctgtctgctggtagaaagctgagtttgaggcaaagcagttgtcgaagctgggccgaggccttcacaggtgtgggcacagaggtgaagcaagtgagaaagtatcatgttgtagattatgcctttctccctgaactcattcaactgctgttgc

SEQ ID NO: 10680 - RNA, 1940 nt, Homo sapiens
  source 1..1940: mol_type = other RNA
cgggcgtggtggtgggggtgcctgggtctgctgggccagcgactctgactctgctcctcctcactgttgctttgcacctcctccaagtcaaaagtgtcctgtggctgctggcttaaagaccgacgcagttctggtctgtctacactctgcttccatttctgctgggtgatggacaggtccaaggacttaaccttcctgcccatgagattcttctggaagaggctctttcttgctctgctctttcttttccagaaagtctcatccttggctggatgggtttccgtattggtggctggtagactacacagctctctccttatctgagctgggtctgtgctccactgtggatcttctatgggcagagaatgtgtgcaacagggtaccttggggttcgaatccagagtttgggatggtgctagcactgtggacatcctctgctgtgtttcctcttcacagcagaagacacatggatagggagaagtgggcaacttcttaccctcagcagggggcacaggatcttcctgtgagaattgccccaaatcagagtcttgctggaggaactgcttctcttctttcactttgtccatcacttccaacacaacttggtccaaactgttccttttgggggtgttgtggggtggtggtggccggtctcgggggcatgtgtacagacacatcttggagatggctttccgaaggcggtctctgggtgactggggttcaggctctcgggacagaatcctgatggatggcacatcagttggatggttgcaattccagaacatgtgggatggtgtgaacttttggacaggtgtcttagacacataggagtagagacagaagaaggcatcagcagtgacagccagtgtttgcacctgcttaaacctgctggccagcatgaggcaggggtcttccatttcaatcctccgcacctgggacttcaggaagagctggaaatcaatgcccttggcctgagagggggtggtgaaaaatcgggcgggtatccgagaagtgtctttgtgatcctcttggccaaagcccagactgaagaggacatcttctgcatcttcttgcactttgtccagaatttctgagatgcttgaactagtcttgttggtccccccagtcatgctgctggaagccaaactacagccaagatcaagtagctggcaaggcctggctgtctcgaggaaactcctggagaagagtttgccattggcggccagtagtgtggcctccgctcccagggtcaagtcatcttcaaagctggtcccatggctgcagaagccattgtagataaactgtcctgcttcctcagaaaatccttcttcagagtatccgcaatcctgcagccagtcttcaattttattgattggattcccttcttggaaaacgtcatccaggctggaaggctcaggatctgggacatcctgcagggcggcggcagcctcctcttctaggacctgggtctgccagttacggctctgacggagccaggcccgccgtttctcccaggatgtggggctcagcacagaggcctccatggccctggctcagacttcagggcctcccgtaacagtaatgccgtcctcactcaagtgtgtacatcctccctcgtagctgacctcaatatatcttgctgcagtttatctcaacaagtttcttctacagcttctgaagaaagaggtcatacccacagaaagcaaagttgatttcagccaggtactctcaatggttggagctatggacactagagtagggcctgtctgctggtagaaagctgagtttgaggcaaagcagttgtcgaagctgggccgaggccttcacaggtgtgggcacagaggtgaagcaagtgagaaagtatcatgttgtagattatgcctttctccctgaactcattcaactgctgttgcctgctcaaaaggggaagcggaaatgag

SEQ ID NO: 10681 - RNA, 1756 nt, Homo sapiens
  source 1..1756: mol_type = other RNA
cgggcgtggtggtgggggtgcctgggtctgctgggccagcgactctgactctgctcctcctcactgttgctttgcacctcctccaagtcaaaagtgtcctgtggctgctggcttaaagaccgacgcagttctggtctgtctacactctgcttccatttctgctgggtgatggacaggtccaaggacttaaccttcctgcccatgagattcttctggaagaggctctttcttgctctgctctttcttttccagaaagtctcatccttggctggatgggtttccgtattggtggctggtagactacacagctctctccttatctgagctgggtctgtgctccactgtggatcttctatgggcagagaatgtgtgcaacagggtaccttggggttcgaatccagagtttgggatggtgctagcactgtggacatcctctgctgtgtttcctcttcacagcagaagacacatggatagggagaagtgggcaacttcttaccctcagcagggggcacaggatcttcctgtgagaattgccccaaatcagagtcttgctggaggaactgcttctcttctttcactttgtccatcacttccaacacaacttggtccaaactgttccttttgggggtgttgtggggtggtggtggccggtctcgggggcatgtgtacagacacatcttggagatggctttccgaaggcggtctctgggtgactggggttcaggctctcgggacagaatcctgatggatggcacatcagttggatggttgcaattccagaacatgtgggatggtgtgaacttttggacaggtgtcttagacacataggagtagagacagaagaaggcatcagcagtgacagccagtgtttgcacctgcttaaacctgctggccagcatgaggcaggggtcttccatttcaatcctccgcacctgggacttcaggaagagctggaaatcaatgcccttggcctgagagggggtggtgaaaaatcgggcgggtatccgagaagtgtctttgtgatcctcttggccaaagcccagactgaagaggacatcttctgcatcttcttgcactttgtccagaatttctgagatgcttgaactagtcttgttggtccccccagtcatgctgctggaagccaaactacagccaagatcaagtagctggcaaggcctggctgtctcgaggaaactcctggagaagagtttgccattggcggccagtagtgtggcctccgctcccagggtcaagtcatcttcaaagctggtcccatggctgcagaagccattgtagataaactgtcctgcttcctcagaaaatccttcttcagagtatccgcaatcctgcagccagtcttcaattttattgattggattcccttcttggaaaacgtcatccaggctggaaggctcaggatctgggacatcctgcagggcggcggcagcctcctcttctaggacctgggtctgccagttacggctctgacggagccaggcccgccgtttctcccaggatgtggggctcagcacagaggcctccatggccctggctcagacttcagggcctcccgtaacagtaatgccgtcctctttttttaacctcggttttctcaaattctttccctccttctcttcatcttcctcagtctttgccacactcaccctgcagtgtccagctcttaaccagcgtcctccatggagccatgcctggcttccacagcctaccttaatcgctttcactgggctctttctct

SEQ ID NO: 10682 - RNA, 6203 nt, Homo sapiens
  source 1..6203: mol_type = other RNA
cgggcgtggtggtgggggtgcctgggtctgctgggccagcgactctgactctgctcctcctcactgttgctttgcacctcctccaagtcaaaagtgtcctgtggctgctggcttaaagaccgacgcagttctggtctgtctacactctgcttccatttctgctgggtgatggacaggtccaaggacttaaccttcctgcccatgagattcttctggaagaggctctttcttgctctgctctttcttttccagaaagtctcatccttggctggatgggtttccgtattggtggctggtagactacacagctctctccttatctgagctgggtctgtgctccactgtggatcttctatgggcagagaatgtgtgcaacagggtaccttggggttcgaatccagagtttgggatggtgctagcactgtggacatcctctgctgtgtttcctcttcacagcagaagacacatggatagggagaagtgggcaacttcttaccctcagcagggggcacaggatcttcctgtgagaattgccccaaatcagagtcttgctggaggaactgcttctcttctttcactttgtccatcacttccaacacaacttggtccaaactgttccttttgggggtgttgtggggtggtggtggccggtctcgggggcatgtgtacagacacatcttggagatggctttccgaaggcggtctctgggtgactggggttcaggctctcgggacagaatcctgatggatggcacatcagttggatggttgcaattccagaacatgtgggatggtgtgaacttttggacaggtgtcttagacacataggagtagagacagaagaaggcatcagcagtgacagccagtgtttgcacctgcttaaacctgctggccagcatgaggcaggggtcttccatttcaatcctccgcacctgggacttcaggaagagctggaaatcaatgcccttggcctgagagggggtggtgaaaaatcgggcgggtatccgagaagtgtctttgtgatcctcttggccaaagcccagactgaagaggacatcttctgcatcttcttgcactttgtccagaatttctgagatgcttgaactagtcttgttggtccccccagtcatgctgctggaagccaaactacagccaagatcaagtagctggcaaggcctggctgtctcgaggaaactcctggagaagagtttgccattggcggccagtagtgtggcctccgctcccagggtcaagtcatcttcaaagctggtcccatggctgcagaagccattgtagataaactgtcctgcttcctcagaaaatccttcttcagagtatccgcaatcctgcagccagtcttcaattttattgattggattcccttcttggaaaacgtcatccaggctggaaggctcaggatctgggacatcctgcagggcggcggcagcctcctcttctaggacctgggtctgccagttacggctctgacggagccaggcccgccgtttctcccaggatgtggggctcagcacagaggcctccatggccctggctcagacttcagggcctcccgtaacagtaatgccgtcctctttttttaacctcggttttctcaaattctttccctccttctcttcatcttcctcagtctttgccacactcaccctgcagtgtccagctcttaaccagcgtcctccatggagccatgcctggcttccacagcctaccttaatcgctttcactgggctctttctctgcttgatttttttcttcttaggtcttatcactaacataccttacattttatttatttacccaatttattgtttactcttctgattagaatacaagctccacgaggacagaaattttgggtcatttactgctgtgtttctaatgcctaaaacagaatctcacacattgtaaccacttaatgaatactcattgtctaaacgagtgaatgtttagaaggtgccctttcctcataggagcccagtgccttccagagtcatcagagacacatgcagggagatcggctgcaaaacagtaacaataagctggtaactatgtgcttactaagcatgtaaaaatgttgtgggttgaaagttggagaaaagagagatggttattctaagacttgtttttatcctagaagttcctacaattgagaacaaagattgcattttcttgactaatccctatttactccctgtctctatgtcctatgtacagaagttttacttaatgttaattcttaaaggaaaatgcctatgaaggcagaatccttaatgcttaagagttccaaagaaaggcttacaaataaatggcaattgcaggtatgacaataaaaagaccagacaggttaagtgttcactgagaatgacagacattttcctggcaatttgggtgagaatgtaataatttttctacttgaaaaagtaatagtgatctcaagtcttgaagaaaagacacaaggtagatctaagctaatcttcacaactctagcacacaggatagaggactgggaaattgcataaataatttttttcccaatctcagcaacacttgaattgtagagccctgtccatggagtgttatatgggaatactataagtacagcaatatcaagaggcaagaagaaatggtagtgtctggttagtggtaataggaggaagctgtactgctgggagacaagaaaccgttttttttttgtttttttttctgtggaaatctgcaggaagcggcaaatgattatcagacaagcacatcagccatgagagtgttagacagaattaaaaagcgagtgcacacagatgtcaagatagcagctttgtaggtcttggggccccttgtaatagagacaaagatatggagatgtttcctccaaataagtcattcgaaaacgtacactgataatacaatggagtttggtgcagtgaaaagaaaactgactagaaatcagaagacttggacatttttctgacttgtccaattaattgacttatggcatgtcagttaggcttttttattacggtttcagtttaatcctctaggaaagggattggctggactcaatgttgtgtaaatttacttccagtaccaatgtttattaatttatttaggtgagtttgaaatatgcataggaatagtacccataaaagaaagtgcatttatacagtttttcccattaaaaaatgcgaaatgcttcagtggtctctagagttacttcccatataccaaattccctttcaaattaacaccaacatatggagctcctgcacatgcgaccttcacattggatccaggaaagtggtgagcctgaacaggaaggccatacaggaacttatacagggagtcagtcaggtgctactcattgactctcaacattgcttgaacttttctgcttttttgctttagcttatagtttcatcccccttcctctctaatcaaacgaattctttctaccctttaagggcctacttaagtcatctcctttctctgtcctacctgtagcaacaaacacccatgcctgcgccatatgcaacaagacagtaagtggctacctctcttgtcatcattcaccactacttgtaacttctcccctaaacccatcatagaacatagcacagtactttgcaaaagaagggactccataagtgctgtacctgcagaggagcaagaatcaccctggcactgggaaattatccccaattagtattcgtcataggacgggtgctcctgactgtcctcatggccttggatcctaatgtacatttttgcacagttagtgaagaggaaaaaggcttggagcatagtctttccagtcctttgttgacataacataaggtcacccaagtctgacttaatttatgaagcttgaactaccaaattctcctatttaaaaaaaatattttccagagtctttcatttcaagtttttattcacttcttcatcaaaatttccttctggagttcatctatcatctctcttgatgctgcttatagtatgtgatcatatttagtcttctctatgaggatagaaatataaagcctgtagatatctgttctccaattttcccatgaaactaagaaattcccacagtggtactattgcttcttgcctgaatccgcccaaaccctcatgtcccccctctgctaccatttccagccttttgttctttcctcttttctacatttctctagacgttcattccataaatccttctccacaatctttcaagagttctggaatctgggttcagccaagtggagtaagatataattcttgttctgaggatgctatagttaaaagcagaaattgtagtagataggattgaggttagacaggagaaatatcctccactggtttaagatgagggagttaagagctgtgaaatgagtatcttccaacaaaaattattatcagaggcagtaactgtagcagcggcagaaaacctgtagaggtatgtcataattatgactcgaagaatatcgcctatttctagtctctgttttcccagggaagcaggtggggattcactacacattgacacgggcaagtcaaaggtaggtagtcataataactgaaatgtatagagtactgcatatttatccataaaactttcctgtaaactgcttaacttaatcctgacaaccactttagagctgattatggttacctgaccctcacagagatacgttatttgtccaaggccacatccctgtagtgctgagatttaaactcaagttggtctgactccatgttatatagtttttccactgacattagaataagaaaatggcccaatgtcaccatccaatgtaatttgggattaaaaaaaaaggagaagttattttagtaaattctccattttgcatctatgtaagctctccatcttatagtctagtagagaagaagcaccataaacacaatgtaatttatatttggttctgtgacagtcttagtgcaggaagtgttgctttgtttgtgttattagaataatttcctttctgactccagctaggtgattatgaagcagtttagccttcctcaggcttacagagtggtttttttggcaagggcccacctaacttctagttgggaggagagaatctgcctggaattccgcattactttcaggttgttgtggcattcagaatatttcataacggtttggggcaccacagagcaatgagagctgataccatcaccgccctgtggtggggccccgcccggtacatggctgatgtggccttgaatttctggggcctgtctggggagtcttgaggaaagagctgggatagctgggctggtcatgggcactcagagggcttgggaaagtggataattatcattagtagacatattttaatattttagcaactattagcctaccagtttgcacctgacaaatatcagctctgcttacagatacttcaccatggggcaattttcaaggggctcagtaaggatgaccaatgcttctttttctttaaagttcagagtgttatttagaaattaaagaaaaggaaaactgtagaaagagtttgggccttggaatcagagtaagcctaatttggaatcatagttctgtctgctttctgcatatttgtccttggtaacactatcttttcttctatacctaagtttcttctttttctttttcttttgtcttgctgtgttactcaggctggtcttgaacacctggcctcaagcaatcctcccaccttggcctcccaaagtgctgggattataggtgtgagccaccacacctagtctatacctaattttcttcataaaatagatactgtgccaaactagttgggtgattggcagttgtaatcaggtaacacatattaagtccctgatgtataaaggtggtgcttaataagtgatagatatgattatgattatgaatctcccctcagtctaagatgttcactaaagttgaaacatcttgaggaataaggaaggaaagaaggaaggaagaaggtgagaattgcagggtacagttgacagtataaaatcaagatggtgaaaaagattttttaaatctgtgttaagcagagataaaaagtaagcaatgaaaagtctttctttcctggggcctgtcctagggtggggggaggggggagagatagcattaggagatgtacctaatgtaactgacgagttaacgggtgcagcacaccaacatggcacat

SEQ ID NO: 10683 - RNA, 1767 nt, Homo sapiens
  source 1..1767: mol_type = other RNA
cgggcgtggtggtgggggtgcctgggtctgctgggccagcgactctgactctgctcctcctcactgttgctttgcacctcctccaagtcaaaagtgtcctgtggctgctggcttaaagaccgacgcagttctggtctgtctacactctgcttccatttctgctgggtgatggacaggtccaaggacttaaccttcctgcccatgagattcttctggaagaggctctttcttgctctgctctttcttttccagaaagtctcatccttggctggatgggtttccgtattggtggctggtagactacacagctctctccttatctgagctgggtctgtgctccactgtggatcttctatgggcagagaatgtgtgcaacagggtaccttggggttcgaatccagagtttgggatggtgctagcactgtggacatcctctgctgtgtttcctcttcacagcagaagacacatggatagggagaagtgggcaacttcttaccctcagcagggggcacaggatcttcctgtgagaattgccccaaatcagagtcttgctggaggaactgcttctcttctttcactttgtccatcacttccaacacaacttggtccaaactgttccttttgggggtgttgtggggtggtggtggccggtctcgggggcatgtgtacagacacatcttggagatggctttccgaaggcggtctctgggtgactggggttcaggctctcgggacagaatcctgatggatggcacatcagttggatggttgcaattccagaacatgtgggatggtgtgaacttttggacaggtgtcttagacacataggagtagagacagaagaaggcatcagcagtgacagccagtgtttgcacctgcttaaacctgctggccagcatgaggcaggggtcttccatttcaatcctccgcacctgggacttcaggaagagctggaaatcaatgcccttggcctgagagggggtggtgaaaaatcgggcgggtatccgagaagtgtctttgtgatcctcttggccaaagcccagactgaagaggacatcttctgcatcttcttgcactttgtccagaatttctgagatgcttgaactagtcttgttggtccccccagtcatgctgctggaagccaaactacagccaagatcaagtagctggcaaggcctggctgtctcgaggaaactcctggagaagagtttgccattggcggccagtagtgtggcctccgctcccagggtcaagtcatcttcaaagctggtcccatggctgcagaagccattgtagataaactgtcctgcttcctcagaaaatccttcttcagagtatccgcaatcctgcagccagtcttcaattttattgattggattcccttcttggaaaacgtcatccaggctggaaggctcaggatctgggacatcctgcagggcggcggcagcctcctcttctaggacctgggtctgccagttacggctctgacggagccaggcccgccgtttctcccaggatgtggggctcagcacagaggcctccatggccctggctcagacttcagggcctcccgtaacagtaatgccgtcctgtctgctggtagaaagctgagtttgaggcaaagcagttgtcgaagctgggccgaggccttcacaggtgtgggcacagaggtgaagcaagtgagaaagtatcatgttgtagattatgcctttctccctgaactcattcaactgctgttgcctgctcaaaaggggaagcggaaatgag

SEQ ID NO: 10684 - RNA, 1682 nt, Homo sapiens
  source 1..1682: mol_type = other RNA
cgggcgtggtggtgggggtgcctgggtctgctgggccagcgactctgactctgctcctcctcactgttgctttgcacctcctccaagtcaaaagtgtcctgtggctgctggcttaaagaccgacgcagttctggtctgtctacactctgcttccatttctgctgggtgatggacaggtccaaggacttaaccttcctgcccatgagattcttctggaagaggctctttcttgctctgctctttcttttccagaaagtctcatccttggctggatgggtttccgtattggtggctggtagactacacagctctctccttatctgagctgggtctgtgctccactgtggatcttctatgggcagagaatgtgtgcaacagggtaccttggggttcgaatccagagtttgggatggtgctagcactgtggacatcctctgctgtgtttcctcttcacagcagaagacacatggatagggagaagtgggcaacttcttaccctcagcagggggcacaggatcttcctgtgagaattgccccaaatcagagtcttgctggaggaactgcttctcttctttcactttgtccatcacttccaacacaacttggtccaaactgttccttttgggggtgttgtggggtggtggtggccggtctcgggggcatgtgtacagacacatcttggagatggctttccgaaggcggtctctgggtgactggggttcaggctctcgggacagaatcctgatggatggcacatcagttggatggttgcaattccagaacatgtgggatggtgtgaacttttggacaggtgtcttagacacataggagtagagacagaagaaggcatcagcagtgacagccagtgtttgcacctgcttaaacctgctggccagcatgaggcaggggtcttccatttcaatcctccgcacctgggacttcaggaagagctggaaatcaatgcccttggcctgagagggggtggtgaaaaatcgggcgggtatccgagaagtgtctttgtgatcctcttggccaaagcccagactgaagaggacatcttctgcatcttcttgcactttgtccagaatttctgagatgcttgaactagtcttgttggtccccccagtcatgctgctggaagccaaactacagccaagatcaagtagctggcaaggcctggctgtctcgaggaaactcctggagaagagtttgccattggcggccagtagtgtggcctccgctcccagggtcaagtcatcttcaaagctggtcccatggctgcagaagccattgtagataaactgtcctgcttcctcagaaaatccttcttcagagtatctaaaccaaaaacagtcttataggttgaagtcacttactacattttccaaggagctttttcatggaaaaactcacacatattcatattccgcaatcctgcagccagtcttcaattttattgattggattccctagaaaagtcagacactagatcactgtgagaactgaacgaaatcagacctcctccctgcaactaattccattccacaagtttattcttacataagctgcgtcatgaatctttttttctacataaagcttttctttaagatatgagaggaatacaccgtatataaaaatagtagatatttcttctctctctctgcttcttttctcccttcctc

SEQ ID NO: 10685 - RNA, 1715 nt, Homo sapiens
  source 1..1715: mol_type = other RNA
cgggcgtggtggtgggggtgcctgggtctgctgggccagcgactctgactctgctcctcctcactgttgctttgcacctcctccaagtcaaaagtgtcctgtggctgctggcttaaagaccgacgcagttctggtctgtctacactctgcttccatttctgctgggtgatggacaggtccaaggacttaaccttcctgcccatgagattcttctggaagaggctctttcttgctctgctctttcttttccagaaagtctcatccttggctggatgggtttccgtattggtggctggtagactacacagctctctccttatctgagctgggtctgtgctccactgtggatcttctatgggcagagaatgtgtgcaacagggtaccttggggttcgaatccagagtttgggatggtgctagcactgtggacatcctctgctgtgtttcctcttcacagcagaagacacatggatagggagaagtgggcaacttcttaccctcagcagggggcacaggatcttcctgtgagaattgccccaaatcagagtcttgctggaggaactgcttctcttctttcactttgtccatcacttccaacacaacttggtccaaactgttccttttgggggtgttgtggggtggtggtggccggtctcgggggcatgtgtacagacacatcttggagatggctttccgaaggcggtctctgggtgactggggttcaggctctcgggacagaatcctgatggatggcacatcagttggatggttgcaattccagaacatgtgggatggtgtgaacttttggacaggtgtcttagacacataggagtagagacagaagaaggcatcagcagtgacagccagtgtttgcacctgcttaaacctgctggccagcatgaggcaggggtcttccatttcaatcctccgcacctgggacttcaggaagagctggaaatcaatgcccttggcctgagagggggtggtgaaaaatcgggcgggtatccgagaagtgtctttgtgatcctcttggccaaagcccagactgaagaggacatcttctgcatcttcttgcactttgtccagaatttctgagatgcttgaactagtcttgttggtccccccagtcatgctgctggaagccaaactacagccaagatcaagtagctggcaaggcctggctgtctcgaggaaactcctggagaagagtttgccattggcggccagtagtgtggcctccgctcccagggtcaagtcatcttcaaagctggtcccatggctgcagaagccattgtagataaactgtcctgcttcctcagaaaatccttcttcagagtatctaaaccaaaaacagtcttataggttgaagtcacttactacattttccaaggagctttttcatggaaaaactcacacatattcatattcttttccagtgagagtcagtagtatttaatttgccgcaatcctgcagccagtcttcaattttattgattggattccctagaaaagtcagacactagatcactgtgagaactgaacgaaatcagacctcctccctgcaactaattccattccacaagtttattcttacataagctgcgtcatgaatctttttttctacataaagcttttctttaagatatgagaggaatacaccgtatataaaaatagtagatatttcttctctctctctgcttcttttctcccttcctc

SEQ ID NO: 10686 - RNA, 1543 nt, Homo sapiens
  source 1..1543: mol_type = other RNA
cgggcgtggtggtgggggtgcctgggtctgctgggccagcgactctgactctgctcctcctcactgttgctttgcacctcctccaagtcaaaagtgtcctgtggctgctggcttaaagaccgacgcagttctggtctgtctacactctgcttccatttctgctgggtgatggacaggtccaaggacttaaccttcctgcccatgagattcttctggaagaggctctttcttgctctgctctttcttttccagaaagtctcatccttggctggatgggtttccgtattggtggctggtagactacacagctctctccttatctgagctgggtctgtgctccactgtggatcttctatgggcagagaatgtgtgcaacagggtaccttggggttcgaatccagagtttgggatggtgctagcactgtggacatcctctgctgtgtttcctcttcacagcagaagacacatggatagggagaagtgggcaacttcttaccctcagcagggggcacaggatcttcctgtgagaattgccccaaatcagagtcttgctggaggaactgcttctcttctttcactttgtccatcacttccaacacaacttggtccaaactgttccttttgggggtgttgtggggtggtggtggccggtctcgggggcatgtgtacagacacatcttggagatggctttccgaaggcggtctctgggtgactggggttcaggctctcgggacagaatcctgatggatggcacatcagttggatggttgcaattccagaacatgtgggatggtgtgaacttttggacaggtgtcttagacacataggagtagagacagaagaaggcatcagcagtgacagccagtgtttgcacctgcttaaacctgctggccagcatgaggcaggggtcttccatttcaatcctccgcacctgggacttcaggaagagctggaaatcaatgcccttggcctgagagggggtggtgaaaaatcgggcgggtatccgagaagtgtctttgtgatcctcttggccaaagcccagactgaagaggacatcttctgcatcttcttgcactttgtccagaatttctgagatgcttgaactagtcttgttggtccccccagtcatgctgctggaagccaaactacagccaagatcaagtagctggcaaggcctggctgtctcgaggaaactcctggagaagagtttgccattggcggccagtagtgtggcctccgctcccagggtcaagtcatcttcaaagctggtcccatggctgcagaagccattgtagataaactgtcctgcttcctcagaaaatccttcttcagagtatctaaaccaaaaacagtcttataggttgaagtcacttactacattttccaaggagctttttcatggaaaaactcacacatattcatattcttttccagtgagagtcagtagtatttaatttgccgcaatcctgcagccagtcttcaattttattgattggattcccttcttggaaaacgtcatccaggctggaaggctcaggatct

SEQ ID NO: 10687 - RNA, 1577 nt, Homo sapiens
  source 1..1577: mol_type = other RNA
cgggcgtggtggtgggggtgcctgggtctgctgggccagcgactctgactctgctcctcctcactgttgctttgcacctcctccaagtcaaaagtgtcctgtggctgctggcttaaagaccgacgcagttctggtctgtctacactctgcttccatttctgctgggtgatggacaggtccaaggacttaaccttcctgcccatgagattcttctggaagaggctctttcttgctctgctctttcttttccagaaagtctcatccttggctggatgggtttccgtattggtggctggtagactacacagctctctccttatctgagctgggtctgtgctccactgtggatcttctatgggcagagaatgtgtgcaacagggtaccttggggttcgaatccagagtttgggatggtgctagcactgtggacatcctctgctgtgtttcctcttcacagcagaagacacatggatagggagaagtgggcaacttcttaccctcagcagggggcacaggatcttcctgtgagaattgccccaaatcagagtcttgctggaggaactgcttctcttctttcactttgtccatcacttccaacacaacttggtccaaactgttccttttgggggtgttgtggggtggtggtggccggtctcgggggcatgtgtacagacacatcttggagatggctttccgaaggcggtctctgggtgactggggttcaggctctcgggacagaatcctgatggatggcacatcagttggatggttgcaattccagaacatgtgggatggtgtgaacttttggacaggtgtcttagacacataggagtagagacagaagaaggcatcagcagtgacagccagtgtttgcacctgcttaaacctgctggccagcatgaggcaggggtcttccatttcaatcctccgcacctgggacttcaggaagagctggaaatcaatgcccttggcctgagagggggtggtgaaaaatcgggcgggtatccgagaagtgtctttgtgatcctcttggccaaagcccagactgaagaggacatcttctgcatcttcttgcactttgtccagaatttctgagatgcttgaactagtcttgttggtccccccagtcatgctgctggaagccaaactacagccaagatcaagtagctggcaaggcctggctgtctcgaggaaactcctggagaagagtttgccattggcggccagtagtgtggcctccgctcccagggtcaagtcatcttcaaagctggtcccatggctgcagaagccattgtagataaactgtcctgcttcctcagaaaatccttcttcagagtatctaaaccaaaaacagtcttataggttgaagtcacttactacattttccaaggagctttttcatggaaaaactcacacatattcatattcttttccagtgagagtcagtagtatttaatttgccgcaatcctgcagccagtcttcaattttattgattggattcccttcttggaaaacgtcatccaggctggaaggctcaggatctgggacatcctgcagggcggcggcagcctcctctt

SEQ ID NO: 10688 - RNA, 1547 nt, Homo sapiens
  source 1..1547: mol_type = other RNA
cgggcgtggtggtgggggtgcctgggtctgctgggccagcgactctgactctgctcctcctcactgttgctttgcacctcctccaagtcaaaagtgtcctgtggctgctggcttaaagaccgacgcagttctggtctgtctacactctgcttccatttctgctgggtgatggacaggtccaaggacttaaccttcctgcccatgagattcttctggaagaggctctttcttgctctgctctttcttttccagaaagtctcatccttggctggatgggtttccgtattggtggctggtagactacacagctctctccttatctgagctgggtctgtgctccactgtggatcttctatgggcagagaatgtgtgcaacagggtaccttggggttcgaatccagagtttgggatggtgctagcactgtggacatcctctgctgtgtttcctcttcacagcagaagacacatggatagggagaagtgggcaacttcttaccctcagcagggggcacaggatcttcctgtgagaattgccccaaatcagagtcttgctggaggaactgcttctcttctttcactttgtccatcacttccaacacaacttggtccaaactgttccttttgggggtgttgtggggtggtggtggccggtctcgggggcatgtgtacagacacatcttggagatggctttccgaaggcggtctctgggtgactggggttcaggctctcgggacagaatcctgatggatggcacatcagttggatggttgcaattccagaacatgtgggatggtgtgaacttttggacaggtgtcttagacacataggagtagagacagaagaaggcatcagcagtgacagccagtgtttgcacctgcttaaacctgggacttcaggaagagctggaaatcaatgcccttggcctgagagggggtggtgaaaaatcgggcgggtatccgagaagtgtctttgtgatcctcttggccaaagcccagactgaagaggacatcttctgcatcttcttgcactttgtccagaatttctgagatgcttgaactagtcttgttggtccccccagtcatgctgctggaagccaaactacagccaagatcaagtagctggcaaggcctggctgtctcgaggaaactcctggagaagagtttgccattggcggccagtagtgtggcctccgctcccagggtcaagtcatcttcaaagctggtcccatggctgcagaagccattgtagataaactgtcctgcttcctcagaaaatccttcttcagagtatccgcaatcctgcagccagtcttcaattttattgattggattccctagaaaagtcagacactagatcactgtgagaactgaacgaaatcagacctcctccctgcaactaattccattccacaagtttattcttacataagctgcgtcatgaatctttttttctacataaagcttttctttaagatatgagaggaatacaccgtatataaaaatagtagatatttcttctctctctctgcttcttttctcccttcctc

SEQ ID NO: 10689 - RNA, 1668 nt, Homo sapiens
  source 1..1668: mol_type = other RNA
cgggcgtggtggtgggggtgcctgggtctgctgggccagcgactctgactctgctcctcctcactgttgctttgcacctcctccaagtcaaaagtgtcctgtggctgctggcttaaagaccgacgcagttctggtctgtctacactctgcttccatttctgctgggtgatggacaggtccaaggacttaaccttcctgcccatgagattcttctggaagaggctctttcttgctctgctctttcttttccagaaagtctcatccttggctggatgggtttccgtattggtggctggtagactacacagctctctccttatctgagctgggtctgtgctccactgtggatcttctatgggcagagaatgtgtgcaacagggtaccttggggttcgaatccagagtttgggatggtgctagcactgtggacatcctctgctgtgtttcctcttcacagcagaagacacatggatagggagaagtgggcaacttcttaccctcagcagggggcacaggatcttcctgtgagaattgccccaaatcagagtcttgctggaggaactgcttctcttctttcactttgtccatcacttccaacacaacttggtccaaactgttccttttgggggtgttgtggggtggtggtggccggtctcgggggcatgtgtacagacacatcttggagatggctttccgaaggcggtctctgggtgactggggttcaggctctcgggacagaatcctgatggatggcacatcagttggatggttgcaattccagaacatgtgggatggtgtgaacttttggacaggtgtcttagacacataggagtagagacagaagaaggcatcagcagtgacagccagtgtttgcacctgcttaaacctgggacttcaggaagagctggaaatcaatgcccttggcctgagagggggtggtgaaaaatcgggcgggtatccgagaagtgtctttgtgatcctcttggccaaagcccagactgaagaggacatcttctgcatcttcttgcactttgtccagaatttctgagatgcttgaactagtcttgttggtccccccagtcatgctgctggaagccaaactacagccaagatcaagtagctggcaaggcctggctgtctcgaggaaactcctggagaagagtttgccattggcggccagtagtgtggcctccgctcccagggtcaagtcatcttcaaagctggtcccatggctgcagaagccattgtagataaactgtcctgcttcctcagaaaatccttcttcagagtatctaaaccaaaaacagtcttataggttgaagtcacttactacattttccaaggagctttttcatggaaaaactcacacatattcatattcttttccagtgagagtcagtagtatttaatttgccgcaatcctgcagccagtcttcaattttattgattggattccctagaaaagtcagacactagatcactgtgagaactgaacgaaatcagacctcctccctgcaactaattccattccacaagtttattcttacataagctgcgtcatgaatctttttttctacataaagcttttctttaagatatgagaggaatacaccgtatataaaaatagtagatatttcttctctctctctgcttcttttctcccttcctc

SEQ ID NO: 10690 - RNA, 1590 nt, Homo sapiens
  source 1..1590: mol_type = other RNA
cgggcgtggtggtgggggtgcctgggtctgctgggccagcgactctgactctgctcctcctcactgttgctttgcacctcctccaagtcaaaagtgtcctgtggctgctggcttaaagaccgacgcagttctggtctgtctacactctgcttccatttctgctgggtgatggacaggtccaaggacttaaccttcctgcccatgagattcttctggaagaggctctttcttgctctgctctttcttttccagaaagtctcatccttggctggatgggtttccgtattggtggctggtagactacacagctctctccttatctgagctgggtctgtgctccactgtggatcttctatgggcagagaatgtgtgcaacagggtaccttggggttcgaatccagagtttgggatggtgctagcactgtggacatcctctgctgtgtttcctcttcacagcagaagacacatggatagggagaagtgggcaacttcttaccctcagcagggggcacaggatcttcctgtgagaattgccccaaatcagagtcttgctggaggaactgcttctcttctttcactttgtccatcacttccaacacaacttggtccaaactgttccttttgggggtgttgtggggtggtggtggccggtctcgggggcatgtgtacagacacatcttggagatggctttccgaaggcggtctctgggtgactggggttcaggctctcgggacagaatcctgatggatggcacatcagttggatggttgcaattccagaacatgtgggatggtgtgaacttttggacaggtgtcttagacacataggagtagagacagaagaaggcatcagcagtgacagccagtgtttgcacctgcttaaactggccagcatgaggcaggggtcttccatttcaatcctccgcacctgggacttcaggaagagctggaaatcaatgcccttggcctgagagggggtggtgaaaaatcgggcgggtatccgagaagtgtctttgtgatcctcttggccaaagcccagactgaagaggacatcttctgcatcttcttgcactttgtccagaatttctgagatgcttgaactagtcttgttggtccccccagtcatgctgctggaagccaaactacagccaagatcaagtagctggcaaggcctggctgtctcgaggaaactcctggagaagagtttgccattggcggccagtagtgtggcctccgctcccagggtcaagtcatcttcaaagctggtcccatggctgcagaagccattgtagataaactgtcctgcttcctcagaaaatccttcttcagagtatccgcaatcctgcagccagtcttcaattttattgattggattccctagaaaagtcagacactagatcactgtgagaactgaacgaaatcagacctcctccctgcaactaattccattccacaagtttattcttacataagctgcgtcatgaatctttttttctacataaagcttttctttaagatatgagaggaatacaccgtatataaaaatagtagatatttcttctctctctctgcttcttttctcccttcctc

SEQ ID NO: 10691 - RNA, 1498 nt, Homo sapiens
  source 1..1498: mol_type = other RNA
cgggcgtggtggtgggggtggagggcggaggggaaaattatgcatgtcaaacactggaagaggaaaggggtattgtggcataatgggattattttgtctctgagaaggaaatcctgaagtctcctgagataccatatgttctgagttatagaaatgctgaggtggaggcctgccatggcaagatcgagggtatctggccctggaaaatcctcgtgtgaattctctgttacgatatccttttgcatgctctgaagcagagctatgagcattccaattctgatgtacttcagtaaaatcttcaccaggctcattaaattcagatttgagttttttccggccttgaatctgagattttttcctctgtttggcttccttctctttttcatcatcactaaaatctaaggcctctggtggtggttcctgatcattcttccatgatgcatctgatcccttatcctgttttagtttttctgtgaatatatattgagtgaaatctttcattgatggagcaaaatacatagtctcctttattttaatacctttactctcaatgtgatctgaagaattaaaccgtaacacataaaatggatgtgcaacaggtccaaatatctcgaatatctttcctgctgcttgtcgatcacttttaaaaattacagtctcctcattaactggaggtaggttagtcatagattcaattattactagttgttcaataatacttgaaaccatcccaagaggctttaactcaatatcttcaggcagaataatagtgagttcttcaacagaaggcagttcattaagaagtaattcatcttttgttttaagaggaaaattcttattttccttctcaatttgtaaatcatcatctccatctgacagcactggaggaagtgatatacaagaggaagaagacgacgatgaggaagatgaagaggaagacgatgaacttgaactatctgaatctgtttcactgtccgagtccgaatccgagtccgaggtctccaaggagtccggcgcccgcgcaggctctgcggctcctggggaggtgacgcagtctccgcaggccggcgattcagccggtggctgtggctgcggcgccggggtcccggccgcgacggcgttcagaacgggctgcagaggctgctccccggcaggcttaacctccacggtctgcccagcgtccggggacccctcaaacgactgtagcggcggctgtgtccctggcacaggggcagagcccggagacggagccgccggaccttccccaactccaaagtcggtgccattgaatttcagagtttccagctgagcggcggcggcctccactacctccatcgcaccgcgccagaaaccgggtcggcctcaggattggggcccctggacaagctcacggctctctccagaaatagaaaaacaacttaggcaaccgcagcaacactgcctgggcccaacttcccgcgtttctcaggtaactacacgcggaggagccaaaagacac

SEQ ID NO: 10692 - RNA, 1518 nt, Homo sapiens
  source 1..1518: mol_type = other RNA
cgggcgtggtggtgggggtggagggcggaggggaaaattatgcatgtcaaacactggaagaggaaaggggtattgtggcataatgggattattttgtctctgagaaggaaatcctgaagtctcctgagataccatatgttctgagttatagaaatgctgaggtggaggcctgccatggcaagatcgagggtatctggccctggaaaatcctcgtgtgaattctctgttacgatatccttttgcatgctctgaagcagagctatgagcattccaattctgatgtacttcagtaaaatcttcaccaggctcattaaattcagatttgagttttttccggccttgaatctgagattttttcctctgtttggcttccttctctttttcatcatcactaaaatctaaggcctctggtggtggttcctgatcattcttccatgatgcatctgatcccttatcctgttttagtttttctgtgaatatatattgagtgaaatctttcattgatggagcaaaatacatagtctcctttattttaatacctttactctcaatgtgatctgaagaattaaaccgtaacacataaaatggatgtgcaacaggtccaaatatctcgaatatctttcctgctgcttgtcgatcacttttaaaaattacagtctcctcattaactggaggtaggttagtcatagattcaattattactagttgttcaataatacttgaaaccatcccaagaggctttaactcaatatcttcaggcagaataatagtgagttcttcaacagaaggcagttcattaagaagtaattcatcttttgttttaagaggaaaattcttattttccttctcaatttgtaaatcatcatctccatctgacagcactggaggaagtgatatacaagaggaagaagacgacgatgaggaagatgaagaggaagacgatgaacttgaactatctgaatctgtttcactgtccgagtccgaatccgagtccgaggtctccaaggagtccggcgcccgcgcaggctctgcggctcctggggaggtgacgcagtctccgcaggccggcgattcagccggtggctgtggctgcggcgccggggtcccggccgcgacggcgttcagaacgggctgcagaggctgctccccggcaggcttaacctccacggtctgcccagcgtccggggacccctcaaacgactgtagcggcggctgtgtccctggcacaggggcagagcccggagacggagccgccggaccttccccaactccaaagtcggtgccattgaatttcagagtttccagctgagcggcggcggcctccactacctccatcgcaccgcgccagaaaccgggtcggcctcaggattggggcccctggacaagctcacggctctctccagaaatagaaaaacaacttaggcaaccgcagcaacactgcctgggcccaacttcccgcgtttctcaggtaactacacgcggaggagccaaaagacacgcccccgccatttacgcagc

SEQ ID NO: 10693 - RNA, 1542 nt, Homo sapiens
  source 1..1542: mol_type = other RNA
cgggcgtggtggtgggggtggagggcggaggggaaaattatgcatgtcaaacactggaagaggaaaggggtattgtggcataatgggattattttgtctctgagaaggaaatcctgaagtctcctgagataccatatgttctgagttatagaaatgctgaggtggaggcctgccatggcaagatcgagggtatctggccctggaaaatcctcgtgtgaattctctgttacgatatccttttgcatgctctgaagcagagctatgagcattccaattctgatgtacttcagtaaaatcttcaccaggctcattaaattcagatttgagttttttccggccttgaatctgagattttttcctctgtttggcttccttctctttttcatcatcactaaaatctaaggcctctggtggtggttcctgatcattcttccatgatgcatctgatcccttatcctgttttagtttttctgtgaatatatattgagtgaaatctttcattgatggagcaaaatacatagtctcctttattttaatacctttactctcaatgtgatctgaagaattaaaccgtaacacataaaatggatgtgcaacaggtccaaatatctcgaatatctttcctgctgcttgtcgatcacttttaaaaattacagtctcctcattaactggaggtaggttagtcatagattcaattattactagttgttcaataatacttgaaaccatcccaagaggctttaactcaatatcttcaggcagaataatagtgagttcttcaacagaaggcagttcctgatgctattaggtgagccttcacttttcagatatggttggaaagtaggatccaatccctggagtactgagagccatgactgaattttttttttctctatagattaagaagtaattcatcttttgttttaagaggaaaattcttattttccttctcaatttgtaaatcatcatctccatctgacagcactggaggaagtgatatacaagaggaagaagacgacgatgaggaagatgaagaggaagacgatgaacttgaactatctgaatctgtttcactgtccgagtccgaatccgagtccgaggtctccaaggagtccggcgcccgcgcaggctctgcggctcctggggaggtgacgcagtctccgcaggccggcgattcagccggtggctgtggctgcggcgccggggtcccggccgcgacggcgttcagaacgggctgcagaggctgctccccggcaggcttaacctccacggtctgcccagcgtccggggacccctcaaacgactgtagcggcggctgtgtccctggcacaggggcagagcccggagacggagccgccggaccttccccaactccaaagtcggtgccattgaatttcagagtttccagctgagcggcggcggcctccactacctccatcgcaccgcgccagaaaccgggtcggcctcaggattggggcccctggacaagctcacggctctctccagaaatagaaaaacaacttaggcaaccgcagcaacact

SEQ ID NO: 10694 - RNA, 239 nt, Homo sapiens
  source 1..239: mol_type = other RNA
cgggcgtggtggtgggggtggggggcaagcaagagagaaagagagagaaaaactccaatcattctttacatgaatagagaattacaaatagctctctaatttcaaattgtgccttgtcaacagatgcttcttctttcttgttctgagtttagtcccaaccttaaatcttcttttttattttgttttaacttttattttaagttcaggggtacgtgtacaggtttgctacataggttata

SEQ ID NO: 10695 - RNA, 1419 nt, Homo sapiens
  source 1..1419: mol_type = other RNA
cgggcgtggtggtgggggtgggggggggtgggcctgatgggggtgtgggcatgatgatgatgggcgtgatgatgatggggggtgatgatgggcatgatgatgggggtgatggtgcccaggcccttcagcaccgcaatatgctgcggaagttcttccggaagttgtcatctagaaaggcgtagaggaaggggttcaggcacgagttggcgtagctgaggctggtgatgacgtaggacatactgatgaccagtggggtctggggcaggtccgtggtcagggccacgacagaggccaggtggaagggcgtccagcagaggaggcacacggccagcacgacgaggaccaggacggtcaccttccgcctggccttgcctagagccttggctccagagcggagccgcacggcccgcagcctgcgcaggaggtctgtgtagagcacacagatggtgcacacgggcagcacgaagcccaggaccaacgtgtagacacggctggccttgaaccagacctgctcgggccacgggaagctcagcccacagcttgggacctgcagctcgttgctgtagacgccagcgaaagagaagaagggcagaaccaggaccgtgacgcccagccagacacacaggctggcgaccttcgccccccggtaggtgcgccagggcatgtggcgggacctcacggtggccagcaccaccaggtatcggtccacgctcatcacggctaggaagtagatgctggagaagatgttgtagtggtcgacggccagcaccagcttgcagagcagctccccgaagggccagtactgcagcaggtgctccgcgatgttgacgggcagtaccagcgtgaagagcccgtcggcgacggccaggttcaggatgaacacgttggtcaccgtcttcatcttgggcgcccttaggattacaaggatgacggccgtgttgccagtcagccccacagcacagatcccggagtacacggcgggcaggagcacatagaggaacggcagtggctcggagaaggtggcattgtggccagtgccattgtcctgagagacgttggcacccatcgtggggagggagaaggagcccctgctgtcaaggggctctgggtgcccagcggcctgcattgtagctgggaccgttgacgatttgcgccctgggcaggtgggaggtgccttggagttgggtatctggttgggggcctccttgggctggattctgtccagtgcttcgagtccagaagttggtagccttggtgtgttcctggttttggccagtacaggcagtcgcagggatggagggcgaggtgtggtcctcactgacagacctccagctgaggtttcaggagtttcaagacctgccctgctggctgcctcagccccggctgcgaggttcccagcctggtgtcagtgctgatgct

SEQ ID NO: 10696 - RNA, 915 nt, Homo sapiens
  source 1..915: mol_type = other RNA
cgggcgtggtggtgggggtggtgggagcagctgcagtttctgtttctggagtctaatcaagtgctccacgtggcttttattttccagtggagcacttgcttccaagatgctggaatctttacctgcgcagtactagaccagggacgctcgatttctctggtagtacaggtgacgtctgcctcagcctgctcggctcctccctcctggccccggcctccctgcgcgtcctgtcctgcagctgccgggccacagctctgaccatcttcttcacagaggccaccttccacctctcctgggcaaagtctgtggccatccactgcatctcctccagcagatagtcccagtgggacttgggtcgtgggcctcctgcagcttcagcagacgcctctgggaccacagacctgctttcctcagctccgcaatgcgctgatgcacctggttctcctgtgggcgccagtgttcactgcctcttagatgcttccatttttatggaattcacatctccaggtactggagtccccatatgtatttgctggagcggctgctgctgggctggaaaagccgcagaagtcctcggcggtagctgggttgctatggcaacaggagtcccaggctgcccgtgctttctggccacaacctttacctgtaattgctactcaggaggctgaggcgggagaatcgcttgaacctgggagacggaggttgtggtgatccaagattgcgccactacactccagcccagctcttgggcaagataagtgtctttattataaaaggcgtcaattcgcagcgtctttacgcggctgccgggcgacgcagccaagggctcccggcgcggatgagcgctgcgacagcggaccgggcggcgaggccactacaaccgaccaaaccgaccggccgacgcggagccagtgc

SEQ ID NO: 10697 - RNA, 2014 nt, Homo sapiens
  source 1..2014: mol_type = other RNA
cgggcgtggtggtgggggtggtggtggtatccccatcattccaggtaaaggaggtggtggaggaggaagaggagctcctccgggtagaggtggcgcgggtggtggtggaggcggccctacacctggcaatggaggtgctgcaggaggacctggaattcctgatgaacttgagagtacttgtgcctgggttcgaagttgctggatttctgcttcaagttctttgattttctcatctcttttttgaagctctgcttgagcttcctgtcgagctgtgaattcttcatcgaacttctttgaaaactctgcagctttttgttcactttcttcaactttcgccttgttcacacaagaatctatcagatgagttaaatcgatgtctaatctttgcctgtatttgaagtctggatccataccactgcagtgtagcactatctgtgaaacacattcctcaattattttataatattgtggcctgatataataatcatttctgataagcaaaaaatgttgtagaatagataagaagtaattttcagcagcagtgtccttcagcatattatatagaagatggtagacttcattcatatcatccatttctgctcgaatgtcattgagacggtgtgataattcagttaggtcatcttctttgttttcatcaaatactttcaactgaatatcaagctcatcattctctttttcttttagatctggtaacattgtttttagtcctgaacggaggaattcattccttaaatgtattcgaaaatcaagctcataaggagaagtgacaagggcatttataaactgcatgcaggccacctgtaattgcaaggcttcctgattttctaaaccttccacaattggtgaaaatcgttccctgttatttctttctgctgctgttgttatagcccctaaaagtttatctagaatgttctcttctccaacaatgcaaatagcagaaagtatttttactatttcagtcatcatgttgggttgtttggggtcaattgctcttgccaatagtaaaagacttctttcatctcctagaatcctttgtaatccaaacttattattcataaatgctttgaggcattgaataagtttatactgattcttcttgtcaatattttcttgctgttttttgtccagaagcttttccagctcatccaataagagtccaagaccttcatggccaaagttgttaacccagctgaccggattgctggttaaagaaaccctgagggattctaggcaattaagaagtttctcatctgatatacccgatcgtaattcatgaacatattcttgtgaagacagggtgcattcatgtttgctgtttttcagcccaccagatttggcagtggcagaaatatactggacaaccatctcacgtttggtggtaaagtctttgtttcgtaaaggagcttttttctcttcgttaaggttcatgtcctccatcattttttcaaagagatccaatacttccttttctgacaaattcaaagatcgttcatcatataatggctgagctgcaggaaactcactcatcgcgacttgagaatcaataggatgttgaataagaggtttttcttttttgacagtagattttctaaaacttgtaattcggtcacgcacatcatctgccaaagtttttatttgaatgttcaatttgggtttgtttttcgtttcctcttcattggcggcccggttccccgcgctccgcttgttgctccggcccccaccgggttcctcgctgccgcctcccgctcccgacgccgccgccccgggctgctccatctttctccggccctgtcacctgtgccctgtaaccccacctctcctcaactgagaaagcacctcggggcgctcacactgccccgcgctgactcggcggcacctcttcctgagggagagagtgtctgcccgggaagctgccgatttcaggcccccgggactccaggctcccaggcacccccgacgcaaccacgccgttgccactactcggcgctggggc

SEQ ID NO: 10698 - RNA, 446 nt, Homo sapiens
  source 1..446: mol_type = other RNA
cgggcgtggtggtgggggtggtggtggtgatgggggtgaaggtgccctcccggaccggcgcccggcgcgctcttggtgcttcccgcgtgcaagtgagtatggtcggcgcgcagcaccttgaagcgcttgcgacgccgcaggaagctgccgttctcgaacatgtccccgcagtcggggtgcagcgcccagaagctacccttgccaggctggtcgggcctccgcggaatcttgatgaagcagtcgttgaaggagaggttgtggcgcaggctgttctgccagcgctgtgtgtgctcgcggtagtaggggaagcgctccatgatgaacttgtagatgtcgctcagcggcagcatcttctcggccgagtgctggattgccatggcggtcagcgagatgtaagagtagggcggtttttggtcgctgtacgagctcttccccggccgcggcat

SEQ ID NO: 10699 - RNA, 2305 nt, Homo sapiens
  source 1..2305: mol_type = other RNA
cgggcgtggtggtgggggtgtgtgtgtatctgtggtacagcccgtggggttgggggacagggaagggtggagcagcagtggcctgggctctggggggccagcatctgtggtattagggctcagaaaatgatacccacaaagatggcactttgacatgctgaattgaagaagcagcctccaggtctctctgacctacctcccacaaaagcccctgtctctcccaaagcacaggatgaggctgtcttctgaagctcccatatcgaactggaaactggactcccaagcaggagcagaattgccttcgatccctctcctgaaatttcattaatcagaggagatgaaaactcctaccacagaggaagagactgatcacgaaacaccacatctagagcccaaactgtgtctcaaactattgtttgttctctggtcccattcagtttccaaaaagaatcattcacaagataatgcctgcctcctggctccattcatcccccaccataaaagtatttatgcctgtaacaccttgtctctttccactataaagaagggtttacaagcacctggacctctctgggttatcgggtaatcattctcccgccatacccctgtgctatgcatgttaaataacatccgtttacctcttttttctattgatctgctttttgtcagctcactttctgcaaaccttcagagggtgaagggggaagctttccttctttgcccctacactggcaactgggacttcactttccagctgctagctggggccttagagaggaccccacaactggaagccatcacagctcttcccccaccctgctggcctgtgggggatgctgttgcctcttcagctcccctctgactgtggtccctctgtttcgaagccctagcctcaagcctcatccccactctctttcctactaccaagagcagacaccaaaatatttctgcgtttcctctggaaaaatcctgggaggtctgtttatggctgtagcaaagcggcacacatctgtgcacagttgagctgggacagctggaaactcaggcactggagtttgctggaattcggagcacgttggtgtacacagtgcctgccccccacctacccacccaacgtgcctccccatctctgcacgagtgtcccaccagagtcagttcttgcttctatgaataacccttccctggcccctgcacaaacacacccacatacgcagacacactcctgcacacagccgatttcagtaggacacacagagacagagaaagggacacgtggcacacagatatgccagcacattctgagaacaaactcaagcatggttcctcaggtctagaggcccacagacacacacaggcaccctcccgcttcaccagggcacacccttgacctgtcacccaccagtaacacctacatacaccagcagacacgcaggacaacgcatgctgactcggcacacccacatataaacatgcaacccacacagaaggtgtgattcacctccagccacgtacagaaacccactcccagccagtcggggcccgccacctaacctcaggcgaggactaccctcccctgggagacctggggactcctgagcctgggaatgtccctgttctttcccattgcctgccctgtccctgaccctggctcccctctcaactctaccatgtgctgtctctgtcaggcaggccagggaacctgagttcccccagtcctgacctgcctcttccttcccttctgttcctgtaccccacatctttccagaggcctagaaagctctagggctaattatctcatggccctccctgctgccaggaactcctctgcccagtggctgacaccccttctgcctccctcaatccttcagggctgctcttggatctgaagtctcttcttcctcagccccaggccccccagattcccacaaggctccctgatggggaaagaaatgtactcttcaggacagattggggaggagcaggcagatgaagggagacaggaagaaggggagagagaaagtggaaagaaacaaaatgaacagatatttcctaaggcctaggaaggaaggaggggcagattgagtgcagctgtaggatgcccagggtagcaggtgtctgtggggagcagggacagagctgggccacctcagacccccttgctttgctgggcacccattttaagggcttacttggcccacatgaggacaaggcctctctagcaatttatcccaaactcctgatcttctcaggccagaccgggattctccagggctcttggagtggggagttctaggcctcctcttta

SEQ ID NO: 10700 - RNA, 23 nt, Homo sapiens
  source 1..23: mol_type = other RNA
cggggcagctcagtacaggatgc

SEQ ID NO: 10701 - RNA, 3996 nt, Homo sapiens
  source 1..3996: mol_type = other RNA
cggggccatggagcagcctgtgtcacacagactgcattccagtaccagctccatcacttcctggctgtgtgaccttggaccagccattttccctccaccttctcacccttatcactgggttgataaaaatttctcacatggctgttgtgagaatggcatgaatgtaaggcgcctggtgtatagaaagtggtcttcatatggtagctgtcattcttacttcattttaagggtgaggaaagggaaagatggagtgacaagtgactgatggagcagagaagcaggagagatgtcacagccacactctgagattctgaaggtcttcctccaataacagtggctcagagtttggttccgtgtaaaggctgttgtcttattgcattaccagcgcccccccccaccaccccaccccctgactcacccactgggcatctgatggaaggagaggttgttggcttccagtaatgttgaactggagtccctagagagctgaggccatagacaggcaagtggagatggctgacttccaaggcaggtttccttctgctaaagtgagtcttgtcctgtctgtatgtgtgcaggtacacacacacacacacacacgcgcgcgcgcacacctgggaggctggctaacacttactctctatgtggctggggaagtaagaactatgcattatgcaaagctcttggggtgttggagattgctgaggcagatctcaggtcccagagtccccccaactaccctgggccagtcagtgttgtctaactccttcaagtgtcaggttgtctgaagtgctgaaatcaactagaagcctgtgtacagcacccttggttgccggatgggtctgagtgttggtgatggtggggggagctgaagtcccctttccttacacttgcattcccatctcccaacccttgctctcctgctggaaagtgtcattgctaggaactcgcaaactctggtgccccctcccagaactgcctctggagaaggatattctgacctgggaatgtgctgccaggggtctggggaaatggtgtggaggcctcctgtctctctgctatgtctgaagacagcttcggagcagggcctctcatccttggcgctattgacattttgagccagataattctctttggtggggctttcctgtacactgtgggatgtctagcagcatccctggcctctacgcattagatgccaatcacattcacttccctattgtgagaacttagaatgtctccagacattgaccaatgtttcctttggaaagaattgcagtgtgaacaccgctttggagcaaactcctgaaattggagtcacctcgactgctctgggagatgctgctgcccctggatcctgatggtgcctgacacctagaccctcttctcagaggtttacccatggccatcagtccaacagcctagcttctggggcctgccaggagcatagatgagatgctcttcttaatgccaactctattcccatccttggcctgggttgacttagctgcttcccctcttccccactatccattcttgggctgagagggagacaccatggggaaggtgatgtggctgaaggcatttggatgtatcaggaaaggggaaggagagacaagagaacactgaggtggctgggatatcattcaagtagaggctgtatcccttctgctcaaatcctccctccagctgctcacacaatcaacgggacaaataacagaacgctcagcctgcaaatctccagacccatctcttcctttttccctaccaaacccacacatgcttcaacagaaaccatgtcctctacaccccaaacacaccatactagcccctccatcctgctaccatcttgaataaaaaagatgcaaggctctctgtattccgacctaaataattaatctgcatccttgtcttagtagctgacaaaccaggggctttctccattcttgagcaaaactttattttaatcaaaatgagtgggaattccaggatacagaaagacaaaggacagtcaaaatagttgtattgtcacctttgtcaaattcaacacttagacacatccagctgtcagcagccctgcatccgatactcctctgctagaaggtgagatttgtcagttgtctgaatggttctgggccctgagttggttctgctgtcttggagataaggagggttcaccaggggcagggcttgctcctggcagttgaagctgtcaccagagaggagtgtgttttgacccccactgttttccctcagaaatggtagttttgctgggaccatcagtcatagctgtttttaccactcttgggattccaagaggcaagtttctctcttctctatagagatagagtaagtaagccaatgcaataaaggcttttggcagggaattttctccattgatgacgtggggaagaggcacacagagagttctgtgagttggtgaagagtaacagaccaagttccagtctcctaactccctcagcctaccctgagatgagtgaatccttacatgggatactggatacctttcccagaaacctttcctcagccagtgtaggcttcccatggcctcttgactggcctggcttagcttgattctgcttctgagcctttgctattgctatgatttctgcctggaaaacccctttggacttccctggcaagtacagtttaagcatccttcaagaccctgtggggagggtctcatgaatgtggtttcacagttggagggcgggtatagaaggaactggagccattccctcccctctactttgaagccttcctgggtaccccagtccttggagcttctggggaatgccagttctctgtggtgcctctttttacaatcccaatagttaatttggaagctcacccctgctcttgtcccacacccaccaaatttggaaatcatatcaatcccctctggagcagttatgccaggcaaacctgtttccagacactgtctcccagtagggtgatagtgaacaatgtacttaacctctccgagcctcagttttcctcatctgtcaagtgggtgagggtgttgctgggattaaatgagataaagtacttagctatgggtagttatagctatggcaacttcctgtattccagccagaccccctgctgggtcctgctctggggaaggtctcatggatgtggtttcacagttggagatggagtatagaaggaaccagagccatctctgacctccgtgttgccttccttctcatatcactgctctgtggccactgttctcaaacacagaaaacctcagtgagccacagaatccattccttgaagaactgatgtcagatctgtgcggctgcagcctgtttggcaggagttacggcacagcacagttctgcttccttcccaccctgatggcacttgtgaactctctgtgtgcattcagtaggataaacctttgcattatctccattttatagatgagaaaacagaggtttagaaacctaatgtgacctacccaaggtctcacatgtgtcttacaggtagcaggggacacccaacccttgacaccccacccaactctgtatgctccaaagctcatgtgctgaacaacacctgcccccctaccctatatggccataacatgcccatgagctgaggctgcatagtgcccgagccaaggaaaagatcagctgtcagcctatggggaagatggtcttaacaatcacgatgaacacaccttgactcggggtttcaagacctctgttgaggttcttggaaaaattctttgagctcaagccctgagctgggcctttggggacagattttacaggctctgtggcatcagttgttttgggtggagagagaactggtggcagtggcagtagtaaaaagttggtggctgggagcattcagcagtcttcaggagcagtagccctgccagggatggagaggaagtgtgttgtgatagttccataccattctggggtgaggatggttacactgtaaagagagctttccacctct

SEQ ID NO: 10702 - RNA, 40 nt, Homo sapiens
  source 1..40: mol_type = other RNA
cggggcggcaggggcctcataggagctgcatgcgaccgct

SEQ ID NO: 10703 - RNA, 41 nt, Homo sapiens
  source 1..41: mol_type = other RNA
cggggcggcaggggcctcataggagctgcatgcgaccgctg

SEQ ID NO: 10704 - RNA, 44 nt, Homo sapiens
  source 1..44: mol_type = other RNA
cggggcggcaggggcctcataggagctgcatgcgaccgctgtcc

SEQ ID NO: 10705 - RNA, 30 nt, Homo sapiens
  source 1..30: mol_type = other RNA
cggggcggcaggggcctcgggagcggcggc

SEQ ID NO: 10706 - RNA, 116 nt, Homo sapiens
  source 1..116: mol_type = other RNA
cggggtcggcggcgacgtgctcagcttggcacccaagttctgccgctccgacgcccggcccgtggctctgcagcccgccttccctctgggcaacggcgacggcgccttcgtcagct

SEQ ID NO: 10707 - RNA, 405 nt, Homo sapiens
  source 1..405: mol_type = other RNA
cgggtagagagggcagtgggaggatggagcttctctgctctttccaacctcaccaccctcccagcacttcgatgtgttcaccaacctggaagctacctgaactccattgtttaggggtttttatgaaaatttcattatgtaggcatcattgattaaataacattggccgttagtgactgaaaatctccagtccctctcccctttccagaagttgatggtgggcgtaaaagttccaatgctggaatcacatggttagatcctctggtgaccaggccccatcctgaagctacccaggtgcctacagtgagttaccacattagaacaaacttaggtatggttaacaggggctcgctatgaataacaaaggacactcttatcaggaatggggctctgtgatgtgacatg

SEQ ID NO: 10708 - RNA, 4442 nt, Homo sapiens
  source 1..4442: mol_type = other RNA
cgggttgtaccttttttgctgacagaaaaggatcagatatgtataaaatagttgaacttgacagcatataacttaaagtgaaaatgtttttgccagaacatgtcttggtaccttgtgaaagcaggctgcccttgttcttgagatagactttaaaatgaaccagctctgaaaagtacttctgctgctctggtctatccctgaaaacagatgtcttgaaacacttttcatattcttaaaataatcttcacttctgttaagaagaacatgttggtgggtaattatgcgaatgtttccctgtccctgatttctcgattaggcgtatgggttttgaaaaagagatttttcagaagattgtcagcttcagtattcatgttccatcgtgtcatctgggtctgttagtgtagtgaccctcagtgcagtctgtcccagcgtttacgtccttgcttcctctgagcagaggcctccatcttagtatcaacatatttaaagaaattgatggtgttcatcaagctggggcctgtggcagttgttgcctgagcaccaagtaacccaagccacctatgtgacaacttctgggcccaggagtaatttctcagcattgagggtaaaataggatggagtgctctgttgatcatttgggagatgtaggttacctgatttgtgccttaggatgcagcgtgaagcagaagtccatattgcaattatgattttagaaggaactaagcattttactcacacccacagcagcaagaatgacctcctgcagcagatattccacctgtaatagcactttggaactgtgggcaaaaccaaaaggctagtgtttccatttattccatgttggtgtatggggttgaactggaaaattccctgaggcaaaactcactggccaaattttgagagggtatagaaaatgactttagagatgagtggttttgtgtatgtgtctgatgatattcagtctgatgttccgcaattttaaaagttataataaaataccatttttttaatctggaaggacattgatatatgaattcttagaatttgctattaaaaagggtagcccccattccacaagctggttttgagggtgatcttgctctaaaaaacctcattcatcataggctcagtctgacaggttctgtacggggctatcatctttctcctcctctgctaaatgcctctttcttccagctgctcactgggtcaaagggatgtcctttctcagatgtattcttgatacatctcagatgtattcgtagctgtgctccttccatacttccaaggagtccggcttctacagaattcctctgtacctcacactgcaacacatgtagatagcgcttttgaaaaatacatatatttttactatagtatgagaggtcctggggctcaaactttaaacatttcctaactcagcttacactggtttaaaatgtccaggtctctgctgaattctcttgttgaattcatagctctgtgttgattcctatgcccctaaccctgcagcctctttgttttatttttttccccatctctgttggtcccagggaaagcaaggaaattttcttttgaggacttataggttgattgcccacaggtcaaactgttggcattgaactcctctcatttcttgccattggattgtttcctaaacgttggataggagaattcgaaattgttgctatttttatgagctgtgcccttgatcaaatctgtgctgtgggtctgagtcactttgccaatgtcgtcttcagtttcaacactctgatcagcatgcaggcgaggggcatgtttaatttacttcactaactgctatattctatagctttagacttcatatttcttatccacctttgtctaggctcacgatctttgggcaagggagctttgtcaccgtggttgggctagaacaaatattgagaagtttaccaacacagatgttgagaagtttattgaaaggcactgacattagcagaataagtgatggacattagttgaaccccttcagtgtctatgtgttttattgtattgtctttaactcgttcttgaagcacagatttcagcgagcctttcagctattcagtgccagcggttttccccactcaggaaagatggtgtgagccatacacacagcaggattagacggggagagtttcagctgcagcttctagtttaagaccaaagcccttcctcccgctgctgcatctgtctgagaggggaagctcttgttttccaagctggaaccgtttatgaggaaaactgagcagggtggcaaaatggaaaaggaacaattttctagtttttcctacgcgtgatattgacgcgtgctttttctttgatttgaggtacagcatgtaaataacaaatttccatattcaaaatgatcatattagagtgactgagtgaccttttgattttgaagcagactaaaatctgaccagaccacaatgaaaagtataaaattagaaacttaaattccaagctaaatttcagctttgacccacctaactccagtgaataggtggcagctcagaaacaaggacagcactgctgctgccagagcaagctcacatccagctggcacttcgtgagagctccttcctgccgggcacgtgtgagttcagcgtgggcaagagacttttatgcacattctgtcattcaaaagggaaatgatgccaaccccagatgcagcatgtcctgaatgaatgatcacttctgctgctctccactccttcttgcagatccaagtttctgtttcctcgtaggatggtgacattgcgaaggatttctccatgctgtgtgtccactgccttcatctcctccacgatcatggagaggttccggacgttgaggtccagccgggcactgagcaggctgaagcgctcccggagcaggtctgtggtgcccagcatgatggagacagacttgttcaggtagtagagctcctcggcatgggtgtggaagcccagcgtgcaggagagccgcacgtcatccaggtacttgagcatgctgtgcacgtggttgtcggtggcattgatgttggtgaagatggtgccaatttcaatctcgtgagaagccatgcgtccttccagagactcaaacctctccacagtgcggttctgggcgtagtgggtatggtactgaagatcatgcatgttctcttcgtggtcatccaggaaggacgagatgttatccagctgcagctgcaagcccatgacctggagtaccaggtcgtgcatgctctctgagttctggctgatgcgctgtgaggaggcccccagggtggcctggatgttcttgaccgcctctccagtcttggtggaggtggtgcgcaggccgctgaagagccgtgtgtagttctgccagtcggtgacaatcttctggagggtcagggtctcctcgtctgtcttccgctggatcccgtggatccactcggaagtctgccccacggtgaagttgatctggtgcactgcagccttgacatcgtagcactcctgggtgaggtccttcagagagaggtccaggccagctgtggtggcctgccagcctctcacctgggccaggaagagccccagagactggttaacctggtggatggagaaggagcaactgcccatctcctgggagatttgtctgctggtggtggagagcacctcctgggcctgtaaggtctggtccagctgcacctcctgggccagaagcagcttctgaattccctccagctcctcctgcagttttcggatctctggccccagctgcccagcttcatggcagaaagagcagttgttcagggctttcggatccaggccctggagatttttctgcattaacacaagcttcttgtcataaatagactgggtcaaggagatgtcttcggagagagagtccacttttctgaaaaccagagaggccaacacagccacggccaccaggagcagggccaggaagaggtaaagaatccgcaccgatgtgtgcaaagataggttcttctggcagcggctgcagcggggccctggccggcccttctgggtgcatgggaaggtcggcatgtcctcgtcgtcacccgccaggtcctcttctgtaacgcacaaggcatctccatcgccgccggccgacctcactttcatggtctcttcctctggggcctcaggagggccccgctgcaggcggctggagctgtagtggagccgggcggccggcggatcctccagggcgcggatcgccgtcctaggcgccgcccgcggccgtggggctccggccgggactcatgctccggcgcgcgggctgcggaggcggcgggaggagtggagggtcccgcggggtcgcagcctggggaagccccgccgggcgcctagcgccgcgccccgccgcccagagcgcgcatcccgccgccgcccgcgcttcccgctggggccccgcgaggtctgccgccgcccctc

SEQ ID NO: 10709 - RNA, 79 nt, Homo sapiens
  source 1..79: mol_type = other RNA
cgtcccaccccccactcctgtttctggtgaaatattcaaacaggagtgggggtgggacataaggaggatagggaacaca

SEQ ID NO: 10710 - RNA, 4681 nt, Homo sapiens
  source 1..4681: mol_type = other RNA
cgtcttacccagcagtgtttggcatataattgcccagtacatagaaatgagatgcctggctagcttaatagaaataaaaaaattaattaaaaaaaagagagagaaacggcacaacaggtggcagtggtggtgactgatagggacaggaaggaaaggaggattaggaatataaacatggaatcagagtaaacaggatattgaggaaaacttctgtcatgctcattcctgtgaactaccctcctctactcctttatttacccaccttagaccacccagactagtcaagtatcttctttccttttccagtatcccagttcacccaactgaacttttgctataccatgctttccacaaacaattttaacttgccaacaaagaattacaaaaaaggtcattctttaatgattacacatttttctactatcagtgagcaaatatagtgtcccttctgttacatgaactataataggatatccgggtaactagtaatttttctctcttccatgaacgtggcccctacaaaaacaaaacaacaaaacaaacaaacaaaaaacagctggaatgtgtagaacacgttgaactaaacggtcttatgccccgtatgctgccatatctggaggtgagggtaggaggaactttgcaattccattagccaaaattaatttttatttatttcttatatccacttacttatttagccaagccagcatctggttctgtgctattcccttaggataggaccaagacagatcaagccagaaggggcatcatattagttcataagactggtctgttatctctaatcagggttttctgggttactttcccaagctggagccaagttggggcaattttgatgagatatctctgtgcccatgccacccattttgctctcaactgctgagtaatctcatgaaaatgttgctgccaagagaagcatattttcaagatcctacagaaagaatagaaagatggcagattccctacccttcccacccctacctcaagaaccactatatttaggctgaactactttaaaaagcaactaacctaatatattttcttgctattcttccaatataccaacttgtccccacctcagggcactgccctttctgctactgtaacatggaattctccccaaagctatttatatgattcagtcttgctttttctttgcttaaaaatcatctcctcaaagatgccttctagcagtgctattcttaccactatttccttgtcctgatttccctttgctacacttatcactactaccagggaatgttatattacacataaatttatttgctgtattttctgcaccacctaactcccccacccccacgcatattgtaagctctgtgcaagtaggacctttgcatttctcattcactgctatatccccagggcctaatatagtgcctactggttaatatatatttgttgaatggttgaacagactcagactgaatgccaaataatgttaacttaaaaaaaaagtatacacatcaaaatatttaaagaaacaattattgatttaaacataaaactgatattgggtaccttggttttacaaacactcctcacaatacttccccttggtgaagcctttcaggaactcttctgcaagaattattttcagagccagcttgtcaacgacatgattggtctttttacttcataagtcttattttgtttcaccaaaagcttcacagtgtaacaaaccaaactcagcacagaaaacatatgacaatatattttagattctctaagacaaggtctcataagtttagatgacaagtgacaacatcaatggactaagtatatcacctcccataacttaaaaggctaatactcataaacatgaaagttctggagtatgaaatttaaaacacaaattttggatataaattatctgagtacaaagctgtaggtaattcttatctttcacttcccctcataactccaaacataacgccattgtaggtgggttgctgctagactacatccaagattgttcagctgaggacttgcccactctcccagttacttggaattttcaaccttcccatactctagcccacatggcatttgcactcagcttctcctactgatccagccacacatcatcttcttcatgaatgtgggcagtctaaagacttcctgtctggcaaagtattatttcaaacaactaagaggaaaatctttggaagcagaagtggaaacacaggaaaagtggcagcaaaaccctcagcctcaggatagtagcttattcaaaagtatatttaaatgtcacagggtaaaatagaccagctgagtccgtatcttagaaaggaagcctactgctttctcctggtaggcaacaaagagaaccccacctaggactttaacccactcttttcccaatgtattccaatactattagccagctgaactaaaagagaatgggtgctggtaggcaactccattgatctccctttctttagcaataagtactggccagctgagggctaaagataatgaggattgaaagaaaagcagacataccaaaggtactgtgtcaagtaatacatgagatgtgttcataaacgaatgagttattccagagccatacaaacaaatcaatctctttactggacaggcatacctctcatatgtatattattcgaatatactaacacatgaaagatcacatcaccttgtttacggatacatttaatatcccttactcttcccgactttcaaaacataatagtatacaaaatataaaatatcttaaatatttataaaaatcacaagaaaaaaatagaacgtatgaaaatatttttatctgagttctccctcattgttgagaggcagcttagtttgccttgagttcataactgttgagtgggtaggagtatgccctgcctaatactattctgtcccggagaagtttaaataaaacatagtagttgcagaagaggatgagagccatggaaagtgtgtggttccacttctccgaccgcagcaaggaatagagctgatagaagacgacactgccctcaataaggatgagcagatttaacagccttaatggtcgatgaaataagaaataaaagcgggcatgagatacatctgaaggcactgccacgttgtaaggccccatggctctatataaacatctgctgtgccgcaccagcaccccttgaggccatattgtattttctgaccaaatgtgctgtggagcattgctgtaggacccatgttccaacttctgccacttgcccaggtgagcagctgatttatgtagcaaatcacagtatttggatggcaacagttgcgtggtgagcatgacaaaagcattgatccacaccataatgaggtgctcacatgaccagcgcatgtcatagtactgggtactcttcacaaaacacagggggagaaatgcaacatagtaggcactgaagagggagttgaagagaacctccttgattctgtggttgaaatctgctttcagacattctacttcattgcgaatgaggtctggagataggggacaactgtgggtggggatgggtgtggcattattaaactgttcttttagcgactccagcaacaaggagagaaagtctttggatttggccaagcctcccacagtcgaggcactttcctctactgcctcgtgctgaaccacatagttgtagtctgtgagaagaagatgtgctctactatcttgatgaaaacagcaaagaggaacataaacaccaaacgggtagccaaggaaaaggagattgaggactgaatggcttcgaaagagattgacgagggtccaacaaagtacccatccacacaaagtgagtagtaccaagcgagctgatatcagaaccatgtagtgaatcattgatgctgcacctgccttagtagcctctgagatgagagcccatacaagcctcctcgcaagcatcactgtgatgaatgctgccagatgataatcaatgagatgaaaattcagtgatgtacaagaagcaggatgattgtaaggataccaccacactgttttataaatgttgatgtactgaatgaaaagagcaaccaacaggtagatgaaaaaaaggaattcaaagagtaggctcccatccacaggcaagtcaggaatttggcaatgacgaacaggacctggggtgattaaggctgtgataggtgggactggaaggccaatagcactaccattcctgtttctcaagcctgttccattgccacagcctccaccaaccaaagtctgcaaagaaggtaaagctgaacggcttagctgttgccgactagggcccctccttccaccgggcatgtccaggaaccagtctgcttccagtgccacctgtagttgcaacccaggttaatggttgtcaaccagtttcaactgcatggaagagtcccagccggtggggcggggtccctagaaagcggcgacaactttacagactggaccccaggtaagggaactccctcccagcgttggaacgctgcaaaccagctgcttggacgcaggcagcccccgcctagagaatcaagaaaaggtgtccaggcttcgggctgccagactcagacccagactccgacgcagttccagtgccagagctaaagctagagccagagcctgatacttcagcacccatccctagcctccattaccgcggagctg

SEQ ID NO: 10711 - RNA, 4790 nt, Homo sapiens
  source 1..4790: mol_type = other RNA
cgtcttacccagcagtgtttggcatataattgcccagtacatagaaatgagatgcctggctagcttaatagaaataaaaaaattaattaaaaaaaagagagagaaacggcacaacaggtggcagtggtggtgactgatagggacaggaaggaaaggaggattaggaatataaacatggaatcagagtaaacaggatattgaggaaaacttctgtcatgctcattcctgtgaactaccctcctctactcctttatttacccaccttagaccacccagactagtcaagtatcttctttccttttccagtatcccagttcacccaactgaacttttgctataccatgctttccacaaacaattttaacttgccaacaaagaattacaaaaaaggtcattctttaatgattacacatttttctactatcagtgagcaaatatagtgtcccttctgttacatgaactataataggatatccgggtaactagtaatttttctctcttccatgaacgtggcccctacaaaaacaaaacaacaaaacaaacaaacaaaaaacagctggaatgtgtagaacacgttgaactaaacggtcttatgccccgtatgctgccatatctggaggtgagggtaggaggaactttgcaattccattagccaaaattaatttttatttatttcttatatccacttacttatttagccaagccagcatctggttctgtgctattcccttaggataggaccaagacagatcaagccagaaggggcatcatattagttcataagactggtctgttatctctaatcagggttttctgggttactttcccaagctggagccaagttggggcaattttgatgagatatctctgtgcccatgccacccattttgctctcaactgctgagtaatctcatgaaaatgttgctgccaagagaagcatattttcaagatcctacagaaagaatagaaagatggcagattccctacccttcccacccctacctcaagaaccactatatttaggctgaactactttaaaaagcaactaacctaatatattttcttgctattcttccaatataccaacttgtccccacctcagggcactgccctttctgctactgtaacatggaattctccccaaagctatttatatgattcagtcttgctttttctttgcttaaaaatcatctcctcaaagatgccttctagcagtgctattcttaccactatttccttgtcctgatttccctttgctacacttatcactactaccagggaatgttatattacacataaatttatttgctgtattttctgcaccacctaactcccccacccccacgcatattgtaagctctgtgcaagtaggacctttgcatttctcattcactgctatatccccagggcctaatatagtgcctactggttaatatatatttgttgaatggttgaacagactcagactgaatgccaaataatgttaacttaaaaaaaaagtatacacatcaaaatatttaaagaaacaattattgatttaaacataaaactgatattgggtaccttggttttacaaacactcctcacaatacttccccttggtgaagcctttcaggaactcttctgcaagaattattttcagagccagcttgtcaacgacatgattggtctttttacttcataagtcttattttgtttcaccaaaagcttcacagtgtaacaaaccaaactcagcacagaaaacatatgacaatatattttagattctctaagacaaggtctcataagtttagatgacaagtgacaacatcaatggactaagtatatcacctcccataacttaaaaggctaatactcataaacatgaaagttctggagtatgaaatttaaaacacaaattttggatataaattatctgagtacaaagctgtaggtaattcttatctttcacttcccctcataactccaaacataacgccattgtaggtgggttgctgctagactacatccaagattgttcagctgaggacttgcccactctcccagttacttggaattttcaaccttcccatactctagcccacatggcatttgcactcagcttctcctactgatccagccacacatcatcttcttcatgaatgtgggcagtctaaagacttcctgtctggcaaagtattatttcaaacaactaagaggaaaatctttggaagcagaagtggaaacacaggaaaagtggcagcaaaaccctcagcctcaggatagtagcttattcaaaagtatatttaaatgtcacagggtaaaatagaccagctgagtccgtatcttagaaaggaagcctactgctttctcctggtaggcaacaaagagaaccccacctaggactttaacccactcttttcccaatgtattccaatactattagccagctgaactaaaagagaatgggtgctggtaggcaactccattgatctccctttctttagcaataagtactggccagctgagggctaaagataatgaggattgaaagaaaagcagacataccaaaggtactgtgtcaagtaatacatgagatgtgttcataaacgaatgagttattccagagccatacaaacaaatcaatctctttactggacaggcatacctctcatatgtatattattcgaatatactaacacatgaaagatcacatcaccttgtttacggatacatttaatatcccttactcttcccgactttcaaaacataatagtatacaaaatataaaatatcttaaatatttataaaaatcacaagaaaaaaatagaacgtatgaaaatatttttatctgagttctccctcattgttgagaggcagcttagtttgccttgagttcataactgttgagtgggtaggagtatgccctgcctaatactattctgtcccggagaagtttaaataaaacatagtagttgcagaagaggatgagagccatggaaagtgtgtggttccacttctccgaccgcagcaaggaatagagctgatagaagacgacactgccctcaataaggatgagcagatttaacagccttaatggtcgatgaaataagaaataaaagcgggcatgagatacatctgaaggcactgccacgttgtaaggccccatggctctatataaacatctgctgtgccgcaccagcaccccttgaggccatattgtattttctgaccaaatgtgctgtggagcattgctgtaggacccatgttccaacttctgccacttgcccaggtgagcagctgatttatgtagcaaatcacagtatttggatggcaacagttgcgtggtgagcatgacaaaagcattgatccacaccataatgaggtgctcacatgaccagcgcatgtcatagtactgggtactcttcacaaaacacagggggagaaatgcaacatagtaggcactgaagagggagttgaagagaacctccttgattctgtggttgaaatctgctttcagacattctacttcattgcgaatgaggtctggagataggggacaactgtgggtggggatgggtgtggcattattaaactgttcttttagcgactccagcaacaaggagagaaagtctttggatttggccaagcctcccacagtcgaggcactttcctctactgcctcgtgctgaaccacatagttgtagtctgtgagaagaagatgtgctctactatcttgatgaaaacagcaaagaggaacataaacaccaaacgggtagccaaggaaaaggagattgaggactgaatggcttcgaaagagattgacgagggtccaacaaagtacccatccacacaaagtgagtagtaccaagcgagctgatatcagaaccatgtagtgaatcattgatgctgcacctgccttagtagcctgtgctttttggttaacttcaaatggttttcagatcttgacttagtatttccagttactctgcttccagaaatagggttcctgaaaatcagagcttacacacacagacctctgagatgagagcccatacaagcctcctcgcaagcatcactgtgatgaatgctgccagatgataatcaatgagatgaaaattcagtgatgtacaagaagcaggatgattgtaaggataccaccacactgttttataaatgttgatgtactgaatgaaaagagcaaccaacaggtagatgaaaaaaaggaattcaaagagtaggctcccatccacaggcaagtcaggaatttggcaatgacgaacaggacctggggtgattaaggctgtgataggtgggactggaaggccaatagcactaccattcctgtttctcaagcctgttccattgccacagcctccaccaaccaaagtctgcaaagaaggtaaagctgaacggcttagctgttgccgactagggcccctccttccaccgggcatgtccaggaaccagtctgcttccagtgccacctgtagttgcaacccaggttaatggttgtcaaccagtttcaactgcatggaagagtcccagccggtggggcggggtccctagaaagcggcgacaactttacagactggaccccaggtaagggaactccctcccagcgttggaacgctgcaaaccagctgcttggacgcaggcagcccccgcctagagaatcaagaaaaggtgtccaggcttcgggctgccagactcagacccagactccgacgcagttccagtgccagagctaaagctagagccagagcctgatacttcagcacccatccctagcctccattaccgcggagctg

SEQ ID NO: 10712 - RNA, 3911 nt, Homo sapiens
  source 1..3911: mol_type = other RNA
cgtcttacccagcagtgtttgggaacctcccccagtccactggtagcagctaaatcaagtatgatatatttgtacagtggaataaaatgcaacttgggggtgtggggggaaactgaggcaagtccttatacactgaaatggaatacatttccagataaattaagtagaaaaacatctgctttacaatgtgtagggtatgataccatttaggttaacatatgaaatataaatatttctataaactatcactggaagaattacaattgcctataagaatagcctctaaagaggcctatccgtttttatcacttgagtatttctgtgttaccaattcataaataaatttttgaaaatgagacatgtggaaggatttgtcacaatgtgtcaattgtgcaagttttaatggactgtaggccttcatcacatttaatttcgcaagaaaacttaagtgtaacttggcgtgaaaggatccacactttcacccatttttaaaattgctctctccagctcactttttttttcgggaacccttccttctttcctctgctgaggggacatctgaagccattatttccaaaataattgtcactacaaccccctgacatctggacctgagaaaggtaaaagttacttttggcttgaggaatgttgtataagccaagaaaatgtttcaaggagagtgggaaggactaggaatttgtccaaaagtgtgaaaagctaagggttgaggggctatttcctgtatactcatcaatatgtcatagtcttgtagtcagaatttatgtatcttgactccaacatcagcactctcataaatgacttcacattaacaaaatatataatatatgcaagtgtgtgtgtgtgtgtgtgtgtgtgtgtgtgtgtgtgtgtgtagagggagagataggagataaatgtgaataatgccagaaagtctaaagttacctcatctttatttatctgtttattcccaacgacatttgcctatccttaacatttttcactatataccaggttgacacctcaaaagtgaagagacagttaaatccaccagttaagaagcttatctgtttgtccaaccctgggcaaaatacatgtgaaacaaatgaaactgcataaacccatccctgggggagcttaaaatcttcaaacagcaaccacacttctcagggaattctggagtgctggatttacactcaatttccctaggaatagacactgttttctcttttattccatgcaaagaaattacaaaatatatttatctaaaagtggcacttatatactggattcttcttatgccttcgaatgttaaaaagcagtatttatgctgcatgtaaacccagctgtttcaagtaaatgcagtactacaggaaaatgtgctattcctgagagctgaacttcttgtcaaaccacagtgaatgctcctagttccagagattcatcattaagaagaatcattcctggaaagatggaaagtcttagaaaaccctaaaaacaggtacttactgaatttggaataactgatttaaaaatcccaatgtttcctaccataaaagaccagtctgcaattgttgacttctctctccctcttaaaacctgtgcccctcaagctcccttctccctaactgcccatatctcatagaattggctttgtaggagaaacaaaccatggtcaataatcaatacaggcttcagaaaggaaagcaaagacatggtaatatctctaggtccttgggtctagaggaataagaaactactttccttttggaaaaattatctggtattagtgaaggaatttgcatatcaagagttttaggaaaggtgtctgaccctaagcatgaaaaacataatcatgtattcccacccaccataacattttataattcagtattaaaccaatactgaactaccaaaaaaggaagaaaatacaatcaaattctaatttttatcatgatgactactacattgctagagttattattttccaaatgctttttgatgcccctgtttgctaagcacattcctggtatgttgggtaatctgataccagtttgcataatttctcccagtagcactatgaaaaatggtactaaggactcaaaagccaaagtttggccaagtctataataaaataaattgtaaatcttgcctttgattttcccatctaggataatgcttcggcagtgtgtcctgtaatgtgatttaaatacaacaatgttctaggtactgatcaataatattataaattgaggacatgagtagttttttaatctgaacaattaaaacagacattcacctaagaggcggtgataacaagtcctaggagcgtctgttagccaaagatatttatttcaaagtttcctattcttaaattcctatggagtttgacactgagattcttttccaaattttacaaatttatatactctttatagaactcagttgaaaggccaactgagtgaattctattaacaaaatgaatggtattaataaaattatttttacgtgatggccaaattttaaactaaaaacactgaacccttagctaattctcaaattagtaatacattggcatagattgtttctcttcaataaaaagccctttacaagttaatatttactaaaatgaaggctcttctgtagaaacaaataagtgatcactaagttatactgctttttgttttctcgatatgaattggtcactgaaagaatacagtaaaaaatcattgcaaatgttgtaattttctttcttgttcctcatttaactctggtttcatattacaaagtcttttatttcattgatgtttgtacaatgcctagaactaagccatattaagtaagtaaatctggaacttcaaaaatgtgttttaatttccattttattctcttagtgcttttgaggttatacaacatgaataatgagatatacagtcatcatgacatccagtaactgtgatgaagcaataccattctaatgatgctaccacacaagatattgaaattgactatattattattaaaaaaatcattaaatggggaaacaatcagcttatccattttatactcctatgtatactctggaacccaactatctgaaggttagcatattcacttgctaagactgtggttaagatgagatggatgtctcctaccctagaaataattcagttccctataataacaaactgactggaaaaagaactcacaggaaaaataagacaaacaagcaaacaaacaaaagactcataaagaataaaggaagatacagtcccttaaaagatgaaagatgataaatagaaatatcagtatacaaaataaagcacaaaaacattatttaccctatatgaggatcatattactatactcctgagaaaaaaatgaatgcctattactaggaagcttctacataaatctgattatattcccatttaactttctgcttgtctttttgtacctttaagatagctcacaactcttaggactcacccacttccacagaactccatgtatcagtccctaaagttccatagagctgctctaacatgaggaagcatggcttaatcggatcccttttgaacagaactcaacagaatatcaggcatgggttcgcctttaagtggttcatgagcacatattatgaacatagaaatccaatgagaaattacagtggaaagaaatgtaaagagaagtggagcttgtttctaaagcagcacgaaaagtaatcaataaccctaccctaccgttaaaatgattctctctcttcagtctttgtactcatttgcattcaccagatacataccattattttccagcttcagaagttaccatggaagctttgttgttgtttttgttattgttcatttttcgagacagtgtctcactctgtcacctaggctggagtgcactgg

SEQ ID NO: 10713 - RNA, 328 nt, Homo sapiens
  source 1..328: mol_type = other RNA
cgtgccacccttttccccagtgtgctgagagccaaccccaacccggaatagaggacgagggaggccagtgaggcagcccccatgggcccaccgcctccccgccggcagggcccagagtgggtcatggctcagatctggagggtcatgggattatgcatcagacctgaggctgcagtgacaacggtcctatgacctccaggcaagactgggatggtcaactctgccttgtcctccaaaaagcagtgtcagtgtgggtcaccagtgaatgccctgagtttaagggcacagtgctccaggtggctggccaagtctgcccaggccttctgat

SEQ ID NO: 10714 - RNA, 57 nt, Homo sapiens
  source 1..57: mol_type = other RNA
cgtggaggacgaggaggaggcacaggcgcctggtccgggctccggctagctgcgtgt

SEQ ID NO: 10715 - RNA, 2252 nt, Homo sapiens
  source 1..2252: mol_type = other RNA
cgtggaggacgaggaggaggcagatgaggaggaggaggacgaagaggatgatgaggggggaggctgagccacgggaggggccggggccttggggggcggccgtgaagagctgccagtgctgaggtccaggctgctgccatatggagaagtgcggaggccgaagggtgagacccgaagctgcagctggggctggggtgggggtggcagactgggagtggccggcaggggtgcagggggtgagacaggaggccgagggaccggtggaggcggtggttcctttggggggaaaggcactagcagcgggtcgggccccgggggctgttcttggctccgctccaggcccgacactttagggaccacggagagttttgcttcacagttcccattgaaggcgccgtgggggcccgaggctttgctggttgagacagtaaaggatgggtcgaggtcatcatcggagaccctctcgtccagatcactttccgcgtcacatatgtatccagcttccagagagtgacgggaggacgcctcttttcttctccgcttattgggccattttcgggcccgatccccagggggccggccaggctctcgatcagagctgtcccctggctccccggtggccccactggagcccccccttttccgcttcccagaatgcttcagccgatgttccagtcgctctgggggctgaagagatgcatccttctgcaaggcctcgagggtggcgaagctggcgatggcgaagccatcgatcaagtcctcctcctcctcttcctcctcctcaggctcctcctcggcttcgccgtcgtctgcgcccccctcctcctcctcctcctcctcttcctccccgcggctgcccgagccggcaggccgcttccgagctcggggtcgcgggggtcgaggtctcggacggggccgccggcgtctcgggcccccaggccgctctccagacgaagctgacgaccaaggcctggcgggcggcggcggcgacgacgaggacgaggagccgcgcggggcggccaacagggcccggggcgcgtcgccgcctggacctcggcggcgccgctgctcccggtctcggtctcggcgcgagcagcgccgccgtcggcgctccccctctgctgcccagcccggacccggggccgcggccgctgccgtctccatggcgaccgccctcagcgccgcatccggaggcggcggggcccgaagcggcctgtccgcaggcccggggtcgcaggcgcggcgctggcggctgcacagtgacgagagggccacggcttctcctttaaagccggatctgctggccccgagcttgccccaaggccacggcccggggagccggcgccgcccccggggcgacaagcccgagggccccccctgcgggctcggcggggccgcgacggcgaaaacggggcggccgtccctttaaggcgaggccccaagttgtccagctcccggcccctttaagacgacccgacagtgtccggcggcctagtgcggtggccaccccctgccaggggtcgatgcaagtctccccgaggaagaggaagggccacccctttaaaaggggccgaaagctcgccccgaaacgcagacctcccctttaaaagtgtctcaagtcctccggctcaaagaggccacccctttaaggagtccagggtccttctaacagcaggccgtccctttaagggctcggagttagtttctagtcctccacaagcggccacttcccctttaagttgaatttaaaagacttcttgtgtgtgggggaggaggacgtaaagaaaaaccccactcgccccagttctcccaacggcacagttctcaatttgtcagcgtctgctcggcggcttcccctttaaggctggcgttgcagtccgccgagttcagtggccacccctttaaggagatttaaaggggcctcctccgggcccagctcctccagcctccgcctccggtcgccatgaaaggcgcgaggcggggcggggcagcgaggccagccctccaaagccccggatgtgaggcaacggtgacgggtacagctcccctgtccgccgacataaaagtctcttcctcctttcctccgtctctgtccgacttgggccttaggggatccggaacggccgatgggcagcgggggagctccagcacaaactcctgttgtctcctttggagtcttagggcgcttctccgccaggacttccctacccctcctccctcttcctcctcagcctacgcctccttcctctctc

SEQ ID NO: 10716 - RNA, 2186 nt, Homo sapiens
  source 1..2186: mol_type = other RNA
cgtggaggacgaggaggaggcagatgaggaggaggaggacgaagaggatgatgaggggggaggctgagccacgggaggggccggggccttggggggcggccgtgaagagctgccagtgctgaggtccaggctgctgccatatggagaagtgcggaggccgaagggtgagacccgaagctgcagctggggctggggtgggggtggcagactgggagtggccggcaggggtgcagggggtgagacaggaggccgagggaccggtggaggcggtggttcctttggggggaaaggcactagcagcgggtcgggccccgggggctgttcttggctccgctccaggcccgacactttagggaccacggagagttttgcttcacagttcccattgaaggcgccgtgggggcccgaggctttgctggttgagacagtaaaggatgggtcgaggtcatcatcggagacctcttttcttctccgcttattgggccattttcgggcccgatccccagggggccggccaggctctcgatcagagctgtcccctggctccccggtggccccactggagcccccccttttccgcttcccagaatgcttcagccgatgttccagtcgctctgggggctgaagagatgcatccttctgcaaggcctcgagggtggcgaagctggcgatggcgaagccatcgatcaagtcctcctcctcctcttcctcctcctcaggctcctcctcggcttcgccgtcgtctgcgcccccctcctcctcctcctcctcctcttcctccccgcggctgcccgagccggcaggccgcttccgagctcggggtcgcgggggtcgaggtctcggacggggccgccggcgtctcgggcccccaggccgctctccagacgaagctgacgaccaaggcctggcgggcggcggcggcgacgacgaggacgaggagccgcgcggggcggccaacagggcccggggcgcgtcgccgcctggacctcggcggcgccgctgctcccggtctcggtctcggcgcgagcagcgccgccgtcggcgctccccctctgctgcccagcccggacccggggccgcggccgctgccgtctccatggcgaccgccctcagcgccgcatccggaggcggcggggcccgaagcggcctgtccgcaggcccggggtcgcaggcgcggcgctggcggctgcacagtgacgagagggccacggcttctcctttaaagccggatctgctggccccgagcttgccccaaggccacggcccggggagccggcgccgcccccggggcgacaagcccgagggccccccctgcgggctcggcggggccgcgacggcgaaaacggggcggccgtccctttaaggcgaggccccaagttgtccagctcccggcccctttaagacgacccgacagtgtccggcggcctagtgcggtggccaccccctgccaggggtcgatgcaagtctccccgaggaagaggaagggccacccctttaaaaggggccgaaagctcgccccgaaacgcagacctcccctttaaaagtgtctcaagtcctccggctcaaagaggccacccctttaaggagtccagggtccttctaacagcaggccgtccctttaagggctcggagttagtttctagtcctccacaagcggccacttcccctttaagttgaatttaaaagacttcttgtgtgtgggggaggaggacgtaaagaaaaaccccactcgccccagttctcccaacggcacagttctcaatttgtcagcgtctgctcggcggcttcccctttaaggctggcgttgcagtccgccgagttcagtggccacccctttaaggagatttaaaggggcctcctccgggcccagctcctccagcctccgcctccggtcgccatgaaaggcgcgaggcggggcggggcagcgaggccagccctccaaagccccggatgtgaggcaacggtgacgggtacagctcccctgtccgccgacataaaagtctcttcctcctttcctccgtctctgtccgacttgggccttaggggatccggaacggccgatgggcagcgggggagctccagcacaaactcctgttgtctcctttggagtcttagggcgcttctccgccaggacttccctacccctcctccctcttcctcctcagcctacgcctccttcctctctc

SEQ ID NO: 10717 - RNA, 2222 nt, Homo sapiens
  source 1..2222: mol_type = other RNA
cgtggaggacgaggaggaggcagatgaggaggaggaggacgaagaggatgatgaggggggaggctgagccacgggaggggccggggccttggggggcggccgtgaagagctgccagtgctgaggtccaggctgctgccatatggagaagtgcggaggccgaagggtgagacccgaagctgcagctggggctggggtgggggtggcagactgggagtggccggcaggggtgcagggggtgagacaggaggccgagggaccggtggaggcggtggttcctttggggggaaaggcactagcagcgggtcgggccccgggggctgttcttggctccgctccaggcccgacactttagggaccacggagagttttgcttcacagttcccattgaaggcgccgtgggggcccgaggctttgctggttgagacagtaaaggatgggtcgaggtcatcatcggagactatgtatccagcttccagagagtgacgggaggacgcctcttttcttctccgcttattgggccattttcgggcccgatccccagggggccggccaggctctcgatcagagctgtcccctggctccccggtggccccactggagcccccccttttccgcttcccagaatgcttcagccgatgttccagtcgctctgggggctgaagagatgcatccttctgcaaggcctcgagggtggcgaagctggcgatggcgaagccatcgatcaagtcctcctcctcctcttcctcctcctcaggctcctcctcggcttcgccgtcgtctgcgcccccctcctcctcctcctcctcctcttcctccccgcggctgcccgagccggcaggccgcttccgagctcggggtcgcgggggtcgaggtctcggacggggccgccggcgtctcgggcccccaggccgctctccagacgaagctgacgaccaaggcctggcgggcggcggcggcgacgacgaggacgaggagccgcgcggggcggccaacagggcccggggcgcgtcgccgcctggacctcggcggcgccgctgctcccggtctcggtctcggcgcgagcagcgccgccgtcggcgctccccctctgctgcccagcccggacccggggccgcggccgctgccgtctccatggcgaccgccctcagcgccgcatccggaggcggcggggcccgaagcggcctgtccgcaggcccggggtcgcaggcgcggcgctggcggctgcacagtgacgagagggccacggcttctcctttaaagccggatctgctggccccgagcttgccccaaggccacggcccggggagccggcgccgcccccggggcgacaagcccgagggccccccctgcgggctcggcggggccgcgacggcgaaaacggggcggccgtccctttaaggcgaggccccaagttgtccagctcccggcccctttaagacgacccgacagtgtccggcggcctagtgcggtggccaccccctgccaggggtcgatgcaagtctccccgaggaagaggaagggccacccctttaaaaggggccgaaagctcgccccgaaacgcagacctcccctttaaaagtgtctcaagtcctccggctcaaagaggccacccctttaaggagtccagggtccttctaacagcaggccgtccctttaagggctcggagttagtttctagtcctccacaagcggccacttcccctttaagttgaatttaaaagacttcttgtgtgtgggggaggaggacgtaaagaaaaaccccactcgccccagttctcccaacggcacagttctcaatttgtcagcgtctgctcggcggcttcccctttaaggctggcgttgcagtccgccgagttcagtggccacccctttaaggagatttaaaggggcctcctccgggcccagctcctccagcctccgcctccggtcgccatgaaaggcgcgaggcggggcggggcagcgaggccagccctccaaagccccggatgtgaggcaacggtgacgggtacagctcccctgtccgccgacataaaagtctcttcctcctttcctccgtctctgtccgacttgggccttaggggatccggaacggccgatgggcagcgggggagctccagcacaaactcctgttgtctcctttggagtcttagggcgcttctccgccaggacttccctacccctcctccctcttcctcctcagcctacgcctccttcctctctc

SEQ ID NO: 10718 - RNA, 424 nt, Homo sapiens
  source 1..424: mol_type = other RNA
cgtggaggacgaggaggaggcagccgccgccgaggtggacgaggacgacgaggtggcctgggccagcttggggggcgtcggctgctgcggcggctgctgctgctgctgctgcggcggcggctgctgaggggactgggcgaccccggatccccgctggccgctgccgcccccggcgcctccgggaccaccgcccgcccctccgcgttccgccatggcccggctaggcgggggttacggaggccgaggcgacgccgatctggctcccaggcttcccccgcggcggcggcggcgggggcgcggcagcctcctcagcccgcctgcccgagcgcgagcagccagcgagctgcacgcacgcgcggggcctctgggcgcgcgggcctcgcgctcgaccgccgctgcctgttgcggctcgcgaggccgacac

SEQ ID NO: 10719 - RNA, 428 nt, Homo sapiens
  source 1..428: mol_type = other RNA
cgtggaggacgaggaggaggcagccgccgccgaggtggacgaggacgacgaggtggcctgggccagcttggggggcgtcggctgctgcggcggctgctgctgctgctgctgcggcggcggctgctgaggggactgggcgaccccggatccccgctggccgctgccgcccccggcgcctccgggaccaccgcccgcccctccgcgttccgccatggcccggctaggcgggggttacggaggccgaggcgacgccgatctggctcccaggcttcccccgcggcggcggcggcgggggcgcggcagcctcctcagcccgcctgcccgagcgcgagcagccagcgagctgcacgcacgcgcggggcctctgggcgcgcgggcctcgcgctcgaccgccgctgcctgttgcggctcgcgaggccgacacgggt

SEQ ID NO: 10720 - RNA, 3435 nt, Homo sapiens
  source 1..3435: mol_type = other RNA
cgtggatattccttctatgtttgttcttctgagtttatcatgatctttcaaaggaattcagctacatactgtatttttgggggggccttaatttgacctttagaaaactgaggtggacctaactcaaaggagaggtaaagaagctgagaaaccacaatcataggaaaaaactaagattcccaggattactgtgggcatgaacaattacactatcatccctatcccaggaaaacttaaaaaaaaaaaaaaaaagtaaatccacatcaagaaaaagtatgtgtattgggtaaagacacatggtgaaacatttttttaaacaagcatctgaagtggacaatgtgtccaaacatatgtacatccttatctccttataaaagtgtttcataactcaagcctccatattttttataaagatgtatgcttctgcacctcgagagtggagaacgttgcaggactaagcaagttttcacaaaatgttttcaagccctcgtttgtataactgttctgacactgggcagcagtgaatgcatacacagaaaaataaaggggatgagatctttcgtttctgaaacatttccctctcccacataaaataacaaagggacgacaaaattgccataggcttgtcagacaagtctaaaagaagctgtggtttctttctcttccctatatttcctcttcctttgtttaaatatccctgagatggccgggcgcggtggctcacgcctgtaatcccagcactttgggaggctgaggcgggcggatcacgaggtcaggagatcgagaccatcccggctaaaacggtgaaaccccgtctctactaaaaatacaaaaaattagccaggcgtagtggcgggtgcctgtagtcccagctacttgggaggctgaggcaggagaatggcgtgaacccgggaggcggagcttgcagtgagccgagatcccgccactgcactccagcctgggcgacagagcgagactccgtctcaaaaaaaaaaaaaaaatatccctgagataatatttcactgtaaactaagaagaaagatgtggctgaaagttttcctaagtgcatagcaaccactgggtctctctcatgggtgaattctcaggtggagaataagactccaggctggttcaatttctaacttgattgtttagacgacaaatgatcatctattacacgttttctcaaagagaggatgcttatgaagtttctcttcagtgtgaatggccagatggtaagatgttccctttcaccacagattttcttcagtggtgatattcaaaaactctttccctaataaaagttcctggatgttgactgaagtctgtgcagtcataaaaggtcttcccacatctgttacaatggtagggtttctcccagtatgaatcctttgatgatgtgtgagggatgagccgcgattaaaagcctttccacactcactgcattcatacggcttctctccagtgtgaatgatggagtgtcgaataaggtttgcgctccggcaaaaggctttcccacactggatgcattcatagggtttctctccagtgtgaatctgttggtgcctcgtgaggtgtgagctgcggttgaaggcctttccacactccacgcactcatagggtttctctccagtgtggatgctgaagtggcgaatgaggtctgccctatcactaaaggcttttccacattctttgcattcatagggtttttctcctgtgtgggtccttttatgcaagacaaaagtggagcagtgggtgaaggcctttccacattcactgcattcataaggcttctccccagtgtgaatccgttgatgctgcttgaggtgtgacctacggttgaacgccttcccacactccatgcacttatagggcttctccccagtgtggataatgtagtgttgaatgaggtctgcactctcgcaaaaagcttttccacactcgttgcattcaaagggtttcactccagtgtgaatctgttggtgccacgtgaggtatgaccggcggttgaaggccttcccacactcaatgcactcatagggcttctctcccgtgtggatgatgtagtgtcgaatgaaacctggcctatctcgaaaggctttgccacactctttgcacacaaagggtttttctccagtgtggctcctgtgatgcaagacaaaagtggagcggtgggtgaaggcctttccacattcactgcacttataaggcttctctccactgtgaatccgctggtgccgtgtgaggtgtgacctgcggttaaaagccttcccacactccatgcacttatagggcttctccccagtgtggatgatgaggtgctgaagaagatgagtgctcttgctaaaggttttcccacactctgtgcattcatagggcttcacttgagtgtgaatccgttcatgctgaacaaggagggcattctttttaaacactttcccgcattcctcacatttataggaatttttctcttcgcgaatcaaggcatctgtaactggtccatgtgaatcacattcatagagatcaccttctgttgaaacttgtttctgtgtaatctttgtacatacaccatcatctgaccccaaaccatcacgttcagaactcattttctccagcagcttcccccgctgggggcctatccctattttcaagtggacttcttgcatttcagatggcccatcctgatccttggattgccctaattgggagttctttgaggctccttgtgtcagttgttcctggagtaagacttcctcaggcaaggccaggtgagaaaaggtaggctctgtggtcttgggttttgtgttgtcacctggataggagctttgggagaggtcttttgtagccatccatagctcctgtctgtgatccaactggtagatcagctctggtttgaacaaaggacagcccagagacatgagaagtccgcaggtctccagcatcacctcctgatacaaggttctctgggctgcatccaactgtccccactcctcctgggtgaatgtcacagccacatcctcaaaggtcacagacacctgcgccgaggctgccatcctgagaccctgcagccctagcggggcccgggaatgccgcggctcagccgacccccagcccttctctgtcctgggcggggcgacctcggctgactttcgcactcggagcctcagtttccccagagaaaaatgcgcacaaagcgggcgcagcgtcggggctgaggagacggagggcggctgcggaggcctaggcctcggcaggcgccggtggaacaccccgttagggaagaagcggggcgtcaggctcccgccaagatgcggagaaggcgcgtaacagcctcattaccctcccctgctcaggccgctggacgcgcctacccagcggtccaggccccacactgttccagggccaatcctgctcacggagatgacgtcacgcgac

SEQ ID NO: 10721 - RNA, 3568 nt, Homo sapiens
  source 1..3568: mol_type = other RNA
cgtgtgggaaggcgtggggtgcggaccccggcccgacctcgccgtcccgcccgccgccttctgcgtcgcggggcgggccggcggggtcctctgacgcggcagacagccctcgctgtcgcctccagtggttgtcgacttgcgggcggcccccctccgcggcggtgggggtgccgtcccgccggcccgtcgtgctgccctctcggggggtttgcgcgagcgtcggctccgcctgggcccttgcggtgctcctggagcgctccgggttgtccctcaggtgcccgaggccgaacggtggtgtgtcgttcccgcccccggcgccccctcctccggtcgccgccgcggtgtccgcgcgtgggtcctgagggagctcgtcggtgtggggttcgaggcggtttgagtgagacgagacgagacgcgcccctcccacgcggggaagggcgcccgcctgctctcggtgagcgcacgtcccgtgctcccctctggcgggtgcgcgcgggccgtgtgagcgatcgcggtgggttcgggccggtgtgacgcgtgcgccggccggccgccgaggggctgccgttctgcctccgaccggtcgtgtgtgggttgacttcggaggcgctctgcctcggaaggaaggaggtgggtggacgggggggcctggtggggttgcgcgcacgcgcgcaccggccgggcccccgccctgaacgcgaacgctcgaggtggccgcgcgcaggtgtttcctcgtaccgcagggccccctcccttccccaggcgtccctcggcgcctctgcgggcccgaggaggagcggctggcgggtggggggagtgtgacccaccctcggtgagaaaagccttctctagcgatctgagaggcgtgccttgggggtaccggatcccccgggccgccgcctctgtctctgcctccgttatggtagcgctgccgtagcgacccgctcgcagaggaccctcctccgcttccccctcgacggggttgggggggagaagcgagggttccgccggccaccgcggtggtggccgagtgcggctcgtcgcctactgtggcccgcgcctcccccttccgagtcgggggaggatcccgccgggccgggcccggcgttcccagcgggttgggacgcggcggccggcgggcggtgggtgtgcgcgcccggcgctctgtccggcgcgtgaccccctccgccgcgagtcggctctccgcccgctcccgtgccgagtcgtgaccggtgccgacgaccgcgtttgcgtggcacggggtcgggcccgcctggccctgggaaagcgtcccacggtgggggcgcgccggtctcccggagcgggaccgggtcggaggatggacgagaatcacgagcgacggtggtgcgggcgtgtcgggttcgtggctgcggtcgctccggggcccccggtggcggggccccggggctcgcgaggcggttctcggtgggggccgagggccgtccggcgtcccaggcggggcgccgcgggaccgccctcgtgtctgtggcggtgggatcccgcggccgtgttttcctggtggcccggccgtgcctgaggtttctccccgagccgccgcctctgcgggctcccgggtgcccttgccctcgcggtccccggccctcgcccgtctgtgccctcttccccgcccgccgcccgccgatcctcttcttccccccgagcggctcaccggcttcacgtccgttggtggccccgcctgggaccgaacccggcaccgcctcgtggggcgccgccgccggccactgatcggcccggcgtccgcgtcccccggcgcgcgccttggggaccgggtcggtggcgccccgcgtggggcccggtgggcttcccggagggttccgggggtcggcctgcggcgcgtgcgggggaggagacggttccgggggaccggccgcgactgcggcggcggtggtgggggcagccgcggggatcgccgagggccggtcggccgccccgggtgccgcgcggtgccgccggcggcggtgaggccccgcgcgtgtgtcccggccgcggtcggccgcgctcgaggggtccccgtggcgtccccttccccgccggccgcctttctcgcgccttccccgtcgccccggcctcgcccgtggtctctcgtcttctcccggcccgctcttccgaaccgggtcggcgcgtcccccgggtgcgcctcgcttcccgggcctgccgcggcccttccccgaggcgtccgtcccgggcgtcggcgtcggggagagcccgtcctccccgcgtggcgtcgccccgttcggcgcgcgcgtgcgcccgagcgcggcccggtggtccctgccggacaggcgttcgtgcgacgtgtggcgtgggtcgacctccgccttgccggtcgctcgccctttccccgggtcggggggtggggcccgggccggggcctcggccccggtcgcggtcccccgtcccgggcgggggcgggcgcgccggccggcctcggtcggccctcccttggccgtcgtgtggcgtgtgccacccctgcgcccgcgcccgccggcggggctcggagccgggcttcggccgggccccgggccctcgaccggaccggtgcgcgggcgctgcggccgcacggcgcgactgtccccgggccgggcaccgcggtccgcctctcgctcgccgcccggacgtcggggccgccccgcggggcgggcggagcgccgtccccgcctcgccgccgcccgcgggcgccggccgcgcgcgcgcgcgcgtggccgccggtccctcccggccgccgggcgcgggtcgggccgtccgcctcctcgcgggcgggcgcgacgaagaagcgtcgcgggtctgtggcgcggggccccggtggtcgtgtcgcgtggggggcgggtggttggggcgtccggttcgccgcgccccgccccggccccaccggtcccggccgccgcccccgcgcccgctcgctccctcccgtccgcccgtccgcggcccgtccgtccgtccgtcgtcctcctcgcttgcggggcgccgggcccgtcctcgcgaggccccccggccggccgtccggccgcgtcggggcctcgccgcgctctaccttacctacctggttgatcggttctcggcggcgtcgcggcgggtctgggggggtctcggtgccctcctccccgccggggcccgtcgtccggccccgccgcgccggctccccgtcttcggggccggccggattcccgtcgcctccgccgcgccgctccgcgccgccgggcacggccccgctcgctctccccggccttcccgctagggcgtctcgagggtcgggggccggacgccggtcccctcccccgcctcctcgtccgcccccccgccgtccaggtacccggcggccgtcgcgcgcctgccgcgcgtgtggcgtgcgccccgcgccgtgggggcgggaacccccgggcgcctgtggggtggtgtccgcgctcgcccccgcgtgggcggcgcgcgcctccccgtggtgtgaaaccttccgacccctctccggagtccggtcccgtttgctgtctcgtctggccggcctgaggcaaccccctctcctattgatcat

SEQ ID NO: 10722 - RNA, 206 nt, Homo sapiens
  source 1..206: mol_type = other RNA
ctaggaggccttggcctgtctgaaattgttctatgtttcatcagattccttgactgacacaacaagaatgacagctgtgatgtgatttagaaccacctatgttaatgctcatacagtaatgacttttcttcttcttggcatgcttgggcactctgacatttgcaccagtaactccctccagctggagtggtcttccctgattatcc

SEQ ID NO: 10723 - RNA, 287 nt, Homo sapiens
  source 1..287: mol_type = other RNA
ctaggaggccttggcctgtctgaaattgttctatgtttcatcagattccttgactgacacaacaagaatgacagctgtgatgtgatttagaaccacctatgttaatgctcatacagtaatgacttttcttcttcttggcatgcttgggcactctgacatttgcaccagtaactccctccagctggagtggtcttccctgattatcctgtagcctattttagagatgtagtagtcagagtcataaggtaatgagataaaaacaaaactcagagtgtgtacgtccaaat

SEQ ID NO: 10724 - RNA, 2191 nt, Homo sapiens
  source 1..2191: mol_type = other RNA
ctagtgagggacagaaccaggattcagattcaggtttttttactctaaaacaatgctaatttcccccttgtgcaggaagtaaaaaaaaagaaaatgggtcaggcgcggtggcttatgcctgtaaccccagcattttgggaggccgaggcaggcggatcacctgaggtcaggagtttgacaccagcctgaccaatatgatgaaaccccgtctctactaaaaaaataaaataaaatacaaaaattagccgggcatggtggcatacgcctgtaatcccagctactcaggaggctgagacaggagaatggcttgaacgcgggaggcagaggttgcagtgagctgagattgtgccattgcactccagcctgagcagcaagagcgaaactccatctcaaaaaaaaaaaaaagaaaaagagagagagaaaatacctaggttgctataggaggtagcaagctgataattatttatctagtagagaaacaattttaaataagtttattcacgtttgagatgcagttggtgtggaactctgaaagataattgatgttttaattttctacagtaagaaaattatcatttgctctgaaagatggcaaaaataagtggggggatagatgaaacaagattggtaaaatgttgataattgttgaagcaatgacgtctatgtctgttgtaaaaacttttttttttttttttgagacggagtttcactcttgttgcccaggctggagtgcaatggcacgatctcagctcaccacaacccccgcctcgcaggttcaagcaattctcctgcctcagcctcccgagtagccgggattacaggcatgtgccaccatgcccggctaatttttgtattttattttgtatttttagtagagacgaggtttctccatgttggtcaggctggtcttgaactcccgacctcaggtatctgcccgcccgggcctcccaaagtgctgggatgacaggtgtgagccaccacacccagcctgttgtaaaaacttcttaaactttaaaaaaaaaataacccatgaaaatggcttaataaaataacattacaataaaactcttctataatactttttacaagtaaaaactgaacaatgtaacaggattcaaaaaaaaaaacacaagaaaggcaagagtttattaactgagataatatctgtaaagcataaaatacaacatcctgtgacagaagggacccagtgttaatttttgtccctcttcacatcaggctaaccaaagccatttatgcaaaaaagggatgacttcattataaacggtgttttatataagcctttagaaaaaaataacactttatagctacataaacgagcaattaatctaatgtccttttaaaaagagaaaatatcattattagtatgattataaatgtaatctaaatattcatatataatgtatatattttttgtagatatgctcccaaaactctgctgtttgcagataacatgaaggtaatggtcatgattttaaaacttactagataggcacttttgcccagtcgtattggtctgaaagccacatcatatgtcaagaaaactctttgaatctccaagaatgtttcttcatctagccattgttatactgtacatattttttaataaattttttatcccaattatggaattttttttttcaatttaaaaataaatagccaatggaaaatgtgatgcagtactgcctatgtattctaactcataaatagaattttgatacattattttaaaaaactgtgctacaattacaagactggattttagtcctagctctaccattaaccagaaattgttcagagtactttaccttttctttccacctgaattctttcattctataattcatttccttcagctgtcaaatgaagaaaggaatgttcttcctatttcacatcaggaagcccagacagacgccaaagtggtgggaaactggttaaaatagtccatagaggtcagcttctggaccacagcacagagtagagaatgatgatgtgatctgagttgaagaagagacttattccttcatccattcatttttcttcttctcatatgactctggggttcagaatatcagacaaagatccttgctgaatgcccactcctgagcggtccggtcagggctccatgggaatgctgaccacacttcctctcaggggcagacctgcacggctg

SEQ ID NO: 10725 - RNA, 5115 nt, Homo sapiens
  source 1..5115: mol_type = other RNA
ctagtgagggacagaaccaggattcagattcaggtttttttactctaaaacaatgctaatttcccccttgtgcaggaagtaaaaaaaaagaaaatgggtcaggcgcggtggcttatgcctgtaaccccagcattttgggaggccgaggcaggcggatcacctgaggtcaggagtttgacaccagcctgaccaatatgatgaaaccccgtctctactaaaaaaataaaataaaatacaaaaattagccgggcatggtggcatacgcctgtaatcccagctactcaggaggctgagacaggagaatggcttgaacgcgggaggcagaggttgcagtgagctgagattgtgccattgcactccagcctgagcagcaagagcgaaactccatctcaaaaaaaaaaaaaagaaaaagagagagagaaaatacctaggttgctataggaggtagcaagctgataattatttatctagtagagaaacaattttaaataagtttattcacgtttgagatgcagttggtgtggaactctgaaagataattgatgttttaattttctacagtaagaaaattatcatttgctctgaaagatggcaaaaataagtggggggatagatgaaacaagattggtaaaatgttgataattgttgaagcaatgacgtctatgtctgttgtaaaaacttttttttttttttttgagacggagtttcactcttgttgcccaggctggagtgcaatggcacgatctcagctcaccacaacccccgcctcgcaggttcaagcaattctcctgcctcagcctcccgagtagccgggattacaggcatgtgccaccatgcccggctaatttttgtattttattttgtatttttagtagagacgaggtttctccatgttggtcaggctggtcttgaactcccgacctcaggtatctgcccgcccgggcctcccaaagtgctgggatgacaggtgtgagccaccacacccagcctgttgtaaaaacttcttaaactttaaaaaaaaaataacccatgaaaatggcttaataaaataacattacaataaaactcttctataatactttttacaagtaaaaactgaacaatgtaacaggattcaaaaaaaaaaacacaagaaaggcaagagtttattaactgagataatatctgtaaagcataaaatacaacatcctgtgacagaagggacccagtgttaatttttgtccctcttcacatcaggctaaccaaagccatttatgcaaaaaagggatgacttcattataaacggtgttttatataagcctttagaaaaaaataacactttatagctacataaacgagcaattaatctaatgtccttttaaaaagagaaaatatcattattagtatgattataaatgtaatctaaatattcatatataatgtatatattttttgtagatatgctcccaaaactctgctgtttgcagataacatgaaggtaatggtcatgattttaaaacttactagataggcacttttgcccagtcgtattggtctgaaagccacatcatatgtcaagaaaactctttgaatctccaagaatgtttcttcatctagccattgttatactgtacatattttttaataaattttttatcccaattatggaattttttttttcaatttaaaaataaatagccaatggaaaatgtgatgcagtactgcctatgtattctaactcataaatagaattttgatacattattttaaaaaactgtgctacaattacaagactggattttagtcctagctctaccattaaccagaaattgttcagagtactttaccttttctttccacctgaattctttcattctataattcatttccttcagctgtcaaatgaagaaaggaatgttcttcctatttcacatcaggaagcccagacagacgccaaagtggtgggaaactggttaaaatagtccatagaggtcagcttctggaccacagcacagagtagagaatgatgatgtgatctgagttgaagaagagacttattccttcatccattcatttttcttcttctcatatgactctggggttcagaatatcagacaaagatccttgctgcttcaataggtaaacaaaaatataagaacaatgatgattctcagcctttatcactatgtctggtacaagttttctgtctgtcacaggagcatgaagcacttcttcatgttcaaaaagaatgaaaagggctatttttaaaaacaattttttgcaagaaaaataaaacactttcattcatttagcaaatatataagcatctgctttccaaactctgcatcataaccttcaaggccctgcaactctggcttctgcctatctcttcaaactctgcttatacctctctcctactcattcactaccatccattgccttttcagttccatgcacgctttgccactttggaagctttcatttgtatgtcccttctctggaattctcttccctccacacttcacatgcttgaatccttcttatccttcaaggcttagctaatatatcactacctcttctagaatgacctttcctattccccacaccctcatcattttctatcccagcacctgcttatttccttcatcgcatgtaccacaaattataattattttatttgttggtttacttgtttttggctatttctctccagtaaaatgtaacaggatatctttgtgtcagggactatgtctttcttctgtaccatgaaatgcgtagcacatatggaattcctaatacataataggcactcagaaatgtttggtgcactaacaaatgaatgagtgaaaggtgtatgctattcattaaggattcattatatagatatagatatatatagatatatataaaagagaagtttcctgttctcaagaactttatagtttaacaaaggatacatatcagctatcaaagcagttgctctataacctaagtgcataatgttagaagcatttagtgctataggagcatataagaaagacctgaagatttctgcttctgctatgatagaatagcatatttggaccaattctcccaccaagaacatctataaaaactatgtaaaattttttaaagaaaagcaaaagcagatgtctgaagaaaataaccaagacagccaggattccgggcactaagatcccagagaaaaagtgaaccacagagaagtaaaactggaattcttcaccatatttttcctcaaagcatttactaattcctaagccaggagtgaggtggggtgagagctattaatactacaggaggcaaagaagccaagcataaaaaagagtagctaagaagctaatgaaataagcagaattttcatgagtcttatgagttcaggacctgttatagaggaggggccctggtaaatatctcaggctttcagcttgaagggctatgctttaggaataaagacaatctgcagataaactagccttcacacggactgaaattcagcatcaaactatctcaatccctgattagatcaagataatctgagttttccttaactgccagaagacctcaaattctttttggaggaatatatcattgtccaaagccttttcaattttttcatacctgatatttgggcttcaatctgaaaagttgccagacatgctagagatagagcaaaatgactaaaaattaagataggaaacaattgataaagtagacctaaaaatgatgctgatacttatattgtctcacatggactttaataaccattatatgtttaagaaaaagggatgacaaagtgggaaatttcactagaaaactggtatctattcataagaatcaaattgaaattttggaaaagggatagaaaatatagaaatgagcataaaagacaaatgggatgtggtgaaaggtcaaacatatatgtagatgaagtctaagaaggagaggggagacagagtgagcaaaacgatatttaaaatattggcggatagttttccaaaatcaataaaagacatcaagccagaaattctaggagctctactaatctcgagccggataaataaaagaaaccatacctaggtaatcagcaaaactactgaaaactaaagacggagaaaattttaccagaaggacacattgccttcaaaggagcaacaataaaactaacaaatgatttaaatggaaatgatggaacccagaaaacaatggactgggatttgtaaaatgcaggaaaaaaatactgccagtagggaactctatagtcatcaaaaatgtacttcaaaaatgaaggtggagtaaagacaatttcagccaaacaaaaactgtgcggacctagactaaatagagtttttaaggtggaaggattatggaagcatggaaatgcagaaaggactaaagagggttaacatgtcagcaaatgtaaatgagtgttgatcatgtaaaataataatgtcttgtgaggcttaaaatatgaatactatatagtgaatatataaatatcaagtatatattgtcaacatagtatatgtagaaaatatatacaataaataaaatacatatacttaaaatataaacatatacatgcacatacgtatatgcttaaaatgcatgtaaaatatatacacacaatagcatgaaaggtagaaaggcataaattgagttgatatgttttaaggttcttgtattgtctgggaagtgatttttaaaaacccagttatgagtagactgtaataagtcaaggatgcatattgtaaatctctaaaataattactaacataataatataagaatatgtaactaacaagctaatagaggggaaagaatattaaataaaaaatatttcatgaatcctaagggaggtatagaagaaggaaaaaggaaatcaaagcagaagtgacaaatggtacagtgatagttttaaacccaaatatagcagtaatcatactacatgtaggccaggtgcggtggctcatgcctataatcccagcactttaggaggctgaggtggactgatcatgtggggccaggagttcgagaccagcctaaccaacgtaatgaaacctcgtctctatacaaaaattagctgggtgtggtggcatgtgcctgtagtcccagcta

SEQ ID NO: 10726 - RNA, 133 nt, Homo sapiens
  source 1..133: mol_type = other RNA
ctatacgacctgctgcctttctcctcagcatcctttatctctttcctcctcactcactttccattcagcgactcccctctcctttcccacccaaatccccttcctcacacctagataacagataacagcccta

SEQ ID NO: 10727 - RNA, 619 nt, Homo sapiens
  source 1..619: mol_type = other RNA
ctatacggcctcctagctttccccaggctgcgccctgcacgggacggggcccggcggggacccccagccccactcagggacccttagccccactgggctgccccagggaccctgggaggaagagccgggctcttttctgtccttgtccctgcatcccctccttcccctgaaatctgttttccttccctgtctgtctccatctctgctgtgtctctgtggcttctgtgtctctttcacagtggatcctctgactccctcttattctggctttctaggtctctgcccctcccgatatctctctgtgtctctatttctgtcgtttttggtctttctgtctctggctctcagaatgtctctgtgcctatctccatctctgacccccaccccagggtctaccgggccaccgcacaccatgttgccagtctctaggtccctgagaccctttaacctgtgaggacatccagggtcacaggtgaggttcttgggagcctggcgtctggcccaaccacacacctggggaattgctggcctgacttctgacccctgactcctcatacccttcctccagagcatgacatttgaccaccaactgaaacctgacctctgaccccagaccact

SEQ ID NO: 10728 - RNA, 34 nt, Homo sapiens
  source 1..34: mol_type = other RNA
ctattaaggacatttgtgattcacgggaggaggt

SEQ ID NO: 10729 - RNA, 32 nt, Homo sapiens
  source 1..32: mol_type = other RNA
ctcaaaccggctgtgcctgtggacgcagccca

SEQ ID NO: 10730 - RNA, 866 nt, Homo sapiens
  source 1..866: mol_type = other RNA
ctcaagatggaagcagtttctgaagatcttttaccatcacatcttctatgatgtcactgtcccgggtgtgcttgacaaagcccatggcccagcctcctccagggacagcacaacaggctgccagccaaacaaactcagggactgccactttgtctttaactctgtagtctgagggcactgtgcctgtgaggatatataggtcttccccactgccacactgtggggtcaaagcccggtccattaggctgtggagattcacataccaccgttcctggaaggactgagtcattggggctgaatttgtgagagtaaatgtggccacctggacatcactgctaagggagaatgggtaaagctgtcctctttggtaatcagaatcaaggtaatctgtattcaaggcttgcttgcttcccaggctgttcacagaggtgatggcctctgcctcattaatcgcctcctcaaggttgctgttggggtcatcgatctgcggctccaccagccatcgctgctcggcgccgccgggcgcagggcgcggggcgcggaacgcggagtacacggggatgcggtcccgggtgctgtagagggtggcgaagcgctcagcaccctccgcgcgctgacagatcttcacgtgggaatcggccgccagccccgcaggcggggtcccggcgtagaagaacttgtcacattcgccaaagccggcttcctcctcgcccacgagccggccttccagcagcccagccagggcgaagaggctgcccagcgcgagccagcgcgcggtgcccatggcggcctctgcgagcgcggcggggccgagcggctgggctgccgcggcgcgagctctgcaggctgggcggggagcgcactac

SEQ ID NO: 10731 - RNA, 11264 nt, Homo sapiens
  source 1..11264: mol_type = other RNA
ctcatctgcaaagaagtaagtgggcaacgtcaaataaagttaaacggcatacacagggctgtagcttaaaccatatgtgtgtatatataagatatttgattgaaatttatgaatttattaatgtggccaaatcacggaaacaaatacatggatctatttgggatctagttggttatatggctgataaacatatggctgataaattataaataaccaaaacattgtggtaaaagagtcaaagaaaaaatgaagtaattgtgcaaggttaatatgaacagcagaaggaatgtaaaaatgtaaagtggtcttctaattcttatgtaagctttgtcatagttattaaaaagacggtatcatattagaaagcccccacccactttcccaatgctgtatacattatacaaatccgtgacaaatgtattaccatttccaaatacctctctgttcattaatttacacttgcatagaaagggaagaagaaaacaataatatatggttattataaaaacaaaatatccatttctctttggatagtcagtgttttactctttcagtagaacacacagtcagcactcaacatcgtgggccaaggagccatggagcttctgatttaatggaacttggaattggcatttgctgaaaagggcaacactgtacgtcaggaaacattggttggccggatgaatacttcacattgcctgtggcctgctgggaacatttgggcagcaagatggaaacgtgctgtgaatctgctccatgacctccgtgagatccgtgctggtgtcgtgcggtggggccagcaggtcctctcccgctgcctggtggaactgtgggccggaggcatctggatcaagcgagtagctcagtgcagaatgctgaggagaagcccatggggaaacaccattgattcgggaatcagattcaggctgctccagcagctgtcggaggcggtggagctgagactccagctgtttattgtgatcttctaaaatctgcatcctagcctccagccgacctttgtgctgcctgaggagttttgcttctgctataagttctgaatcctcagacgtgtgatggggagatataatcgactctggcggtgaaccgacagggagcccccttcggaggtgctggtccttcagctgctcatactccacctgtagatttctttgttcttcctccaggtcagcaatgatcctctccagttctccacgttcttccctctctactgacttcaggatctgagctgggctctgcggctggctcactggggactctcctccgagtgtttggcaatactgctggatgagggcgtgctcgtcttccacacttcctgtggtggagctgctatcagtgagaaaagacccattagtcctttccatctgggccagtcgtgtggcatattgttctattcttgaatgggtgtcatcatgaaacagttgaggagattgtgagggggtctctaagttgtcaccttcaagaactgtctggacaggcaggtaaccaagtcgagggtgtttggcaaagtacttcttcgacctgaacttgttcttaagtacctttgtgaagtctcgtacatcttccccagatgttgtaggtatacaatattccaccattgggtaatgtaatttgtgaccttttgctgttcgacccgaaaagaaacaactctggcagacatcatagttaaaatgcttaaggcttctatacctgaacccgacaattggacattctttacagatgttgcatttggcctgatgttttgcagtctccgctgctgccactcgatgtaaaactgggagccaaaccatggactgtggttccaaatgcatccaatctataaactctttcacacttatttctggtttattgttattctgttggaagcagctgcgaacactaggctcaatattactgcctccaaaagctgctacttcacctagctgccgggggatctggatggcatcatgaagtaacaggcccagctgcctctggtcacacatttctgttggccctgcaacttccttaaagagatatctgtatttttcttccaagagacctttggagagagacattaatccaatcttcagactctgcactctaatttttccagttcgacccgtgtcatagacattgagcaaccaattgagacacatatcaacacagagtggaacgttgaccaggtccttatgcatttgctcaagtccatcataagttgttgtcagacagttgatgacatctggaacactgaggagctggtcattttggttcaacttgtgctgtttgaaaatttcatttgttgtactcaactctaagagatccaaacatagtgctttttgtagtcttcggattttgattgctgtacggtaggcagaaaaacgtacattattcaggtcagcaagggattgaaagagttcggtcattttaggatggtcccaacaggtggtctgtgtttgatggttgatgtaatagggcactttattatgtgaaatggatctttgccacggcagctggactgacgtagagagaaaatgctgagaggatggtccaaaatctctgtgggcttcctgaagctgtttaaggcgatcatccacagaaacctgtaaaagtttccatcgcatattaaggtcatctagctggcgagacatctttagagagggatgcaggtcaagtggagacagctgactggataaatcattcaccgttttaactttaaagttgattggtgcaatttcttctctaaatgccatgattttttcaatgtgatcctgcagcgagtcaatgagtaagtctcccacgggcttccagccattccgcacggactctgcctccttcatgtcagcgtccaggtcatccatagctccctgcaggtctctgagtttctccaatgccttgtccacttgcttttgccaattgctagttacagcatttagactttcccatttttctttgacttcagaagactgtttgcgcatggctttggcaatcttttgggctctctcctcaggagttaattctgtttttgattgtaggtttcttcttggctcttcaggggcctcaattggctgatcagccaagaaaactcgggcctggtcgacagcattcaggacagaatattctttctcctttaactcccgtctcagggccttacaatggtcatactggagctgtaaggctggaacatctcctccaataggcatttgtttcttaagctcttcatctttcatattcagccatttgatcagttcttctaaggacatcagcaacctgttccacttctcagcgctggcctccaaatgggccctgatgctagcagattttgcttttaagtcattccatctttggttcatatcatccagtcgatgttgaagcatagtagcctcttcagaatttcccaaagcttttaccatcttctgcctgtttccgtcaatgcttttaaatatgtcattgtgggcatcaatttctgcctggatgtcctgcatctgctgtttgagttccctggccaagatactatcctgaagagcattctcccgatgagaggcatccacaagcacattcactgtggtctctgcttcttggatccacttcaggaagttttccagatctctgcgagaggcctgcaccgtcctccactcagcctccaaggcgttctgtctgtcagcaatactttgtttgagattgatccatgatgtttttaagtactctgtggtttctttcacattccttgtgtcatcactcccatattcctccaggagtttctgcaggacgttatcgaacgccatgacgataccatctccaggacccagttcttgaagcagtatttggttatcagaaatttgtttggtgagtggatcccgtcgggcttgctgaagaatatagagtcgagcctcatattttctcatcagttcttcagtctcctccctatggtcatcccactgaagactgtcaataatcatgtcctcaagctgctgctgtcttagctcaacgccatgctgggtgccatcccactggttcttgaccctttccaatttttctgtaattgctgttctcatatctgaactggaagctttatttttcaaattctgtgccaatgtaaaaacataatccagctgaggatggcgctgttctaagtcagcctttgtaattttcattcgggaaacggtcttattgatctcttctacatccccaacagtgacaatgttggacttcagcatctggtcgattaataccagccagtcggctagttctgttatagttttatcaagatcagcaggaattgaaatttccgaagtacgatgagactgaacaggaatatctgacgcagatgatactagcaccaccttttggacattaggatgagcagcaatccttgtctgtgaaacagaactgggctcctggatgcattccttcagggtggtaggcacctctctgcaaatcttattccatgtcatatttacagtccttaagctttctgaaattttatccctttcaggtaaactcagacttttatctgaaagcatctccaattcagttctattcagccatttgagtttttcagcatgtacttccatttcttgagttaagtctcttaattcttgcaggttttctcccaattcggtggttgatctcttttgcatagcatgctcagcctttgttaaccaacagataatctcatctagctgatgcctgtacttcatcacctgcttactttctccttttagccttggctgcctatccttcacttctgcaacaattgcatcccagcgttggtttaaacctgccagtttttctttcaagaagcttccatctgcctgggagagtttctgcacaatcccatccccagttcggtttagtgctgcaaaactgggctggtggctgctgatgcccacctcaagttcctgctgatgtatcctggctttctctaagtccaggctgccacctggagcacaggtatcaaccagtaattcttcagcctctgttatccactgtgtgaggtcattaaggtcacaatggaactgtctccattcttccattgccctgtcaaaacaacctttccgatcactgtacattctattaattctgtcccattttgcattcagctgagtaagtgtatctctgatctgaatggcttcaggtccagaggcttcaaggatgacatctggctgtttttcatgaatgactgcaatctgctctccaagtttgtccagttggtctttgatattcttcagagagtcttcctgaaaagagaagtcttcgtaaatagcagtgttgagctctggaacattaagcgataattcaacatcatccatgcaaagtaaaattttgttaatttcaaccagataatctgtaggaagaagtgatgatctaattccagaagcaagttgacccattttcctctgttgaatagggattgccttaattttgttgtatctagtatgcaaaagtaataattgcaaacggatcttttcttttttattatcttccataggttgatgtaacatttcttctcctctttgtagaacttcctcaatctgggcactctcctcatccatcttttcatcttcatcactggattccaagtgtttttccacaaattttaacatattttctatgtcattttctaatttttccaagtcagagaaaggcacaccagtttcaaatgtttcagtggtgaccaaacattggtataatggttcctgagcaattagcaatttggcacttttgatatgttgagacaccttttcaaagttcctattcagctcagctaactttggttctacaagctccctgcttgagcttccacgggcattcatcaaaataagggcttgatcgcggacattttcaacctggaggttggcatcatccagctcagatactaaacgcttcacaatttcttcctgtttacttgttggtttcttttcaatttcatccaatagagcttcagcttgataaagccaggtacttatgtgagccacgttcccatcaaatatttctagctggttctgatggttcatcaaggtattgcaccaatcttcagtccaggtacgaactcggctccacccagcgttaaggacgcagagcctctcttctaaaataggctcactgccctcaatcaagttttgcagggcagcactactctctgtgatggtatttaaatcagcttttctcttttccagatccttcagaacatttttagcccaggaaatttctgtatccaagtcaccaagcagaccttctgaagtggacttctgtaccaattcagtttcagtagcagaaagccattcagagagagaagcagcctctttcttcattttccgggccaactgtgatgctctttccagatcctgttttccttctgtcacctgtgcgcccaggtcattgtaaagaaccttcagggaagtcagctgctcatccatcccttttgggttgtccgtttgctgtttctggacaatatgtcttcctgttttaatcacagtttccacttcaagtttgacttcactcaaagttttatacagtttcatacacttgtccaggtgcgtctgtatgacgtcagggtctacgtccttcacatccagaacgtgaagttctgctttcacgccatccagcacacgcttgcagtccagcatgcgctgctcgaagttagctggcttctggaaaagctggaactttgtggacacctctcggagtttcctctgtagcacatccatctgacttcctcctctggcagtcctactctctggggaggtcaggggctgagaacgcatatttcttctcaactcctctagggttagctcatgggctgagatctctgcttggattttctgagcttcctgtggaacttggaaagcatctatcctgtcagtcaggtatgtggtgagctgtttgtccagctcccccaagctctcttgcaagacttgaagcatctggtcagtttcccgcagcacctggagttgcttttccaaagaaatctgcttgctctctgccaggtgacttagatcttcatatcggctgttgaaagcctccagtttctcactgattatatcatccaggatccccccatcaatcagagtctggccaagctctcgaatctgggtgcgattatctgccgggtggcgcagaacagattccagagactccagggcttcgttgacagcatccgtcttctcaggcaggacctctgtgctcttcatccgctcttccaaagtgtttaaccaggtagtttcaagatccaaatagtgaagcagttcaatccaacaagaccagacctcctctagcgtgtggcactttcctcgaattctattacaaagaagttggtaattctccagcacaacattcagctcagacgtcaactcctggccaccagagggcaccttggcagctaataacttgatgttgtccttgagaatcttcactctcacctccttctgcaacacatcctcttttgccctcttcatctcttccacagcactctcaagctcttctggtgacttgtactcaaaatcccgctccaaatattcttcctcggcctgggtcatccattcctgcatctctgccaagtctttcttcaggttcgcagctttttcttgactttcagacaacctacttttttgagtagcgatctccttgctaagtttctccagttgagtttggtagtcacctagtcttgtctgcacccaagtttttattccagcaactggaccacttcgaagattagtctctatttccttcatgtttttcagagatgattcaattgtttctatttcattaacaaatgcagagcactggtctaactgcctctgtagacctgcgtcgtctccttgggcagcctgctgtttcattaagaagtctttcacgccatccatccacttctcaatgactgttgaatcggcctcaaaagctctgagtgtgagagcaatttcctcaagcaaatgtagatctttggaaaccaagacctttagcttgttccactttccttgcacatcatcaaattcttgcttatataatttttctacatcaggatgaacatttttctccagagcctttgtttcttctgcaagtttatgtaatgcaggtttctgattctcaaggatttcatcaagggtctttttttcttgcagggccttctccaccttggcaagatcattaaggacattcagagacacctgggccttattttctgaatcatttagcacatctttcagtgttttcaatgtttccagatatgcatgtccaggttggcccttcagttcattctctagatgttgttgacgatcctctacagcctcttgtacagcttggtagcggcccagaaagctatcgaagccccgctggacaaaatctggggcagaaggctgagacatcagggccgagcagcttgcacgagccatttcaattttggggtgaaggccaagaagatttgtcaattcccgctgacaggaatccttcaagcttggcaaggactgccgggaagattcagaaatggaagtgtgttttacccactcctcctttgtcttgatgaccttttcaagctcatcaagctgcttgaaataagcatttatatcttcctgtagctgaatctttctttctagatcttccaaatgttgagatacattcttccattctgatgaaaccttctccagaacattttttatttcttcagtaggaaggccttcttttcccatttgctccacaaggatttgtccagtttggtttaattcatctgctctggggattctttctctctgttctttttctaatgccttcaacttctttttcatttcggaagtgtcttgcatcttcatatactcttttatctctgtggtctgaatggcagttttccatttcaaaatccagttcaacagctctgcacttatagcatcaaactttttcttagcttcaatatccacatggatctgtctcttctttgggggaggaggaggaggcagttcctgcttagatttttttgtaattgcttgttctcttacacgaacagtctccaaaaggtccttctgaggaatctgagacatccccagctttgctacagcctgagtcacctggttggaggaatcttctagtctctgaaccaaagaatcccatctttgagtcagttcctctgagtcactgttgatcttcttagatgccttggaattatcaagtaattgtcccacatcctggccaatctcactcagctgatccaatgtttgacgcttcatttccatgtcttccttcaaaatagccagacgtcgaacactgacacttagttccttttggtctttgaagttgcttgtctggactttatttaaagcctcttctttttcggttaaccaagctttcaacaagcactgttcttccaataattcctgccacaatatattgatttcttgtaacctattccagcgttcttcagtccaacggcatactgctgtccagcgctcaccaagtttctgtaactggtcttctaggatagctgtagcactctcaccactgttttcatcaacaatgaccaccatgtgagttagtgaatttactttcacctgttcagcctcaagatcactttgcaaacttttatgttcttctagcagcttttgtagagattttacatcatcatccagggggcaagtttccatcttctgaatgcgctcctctgtgagtgttaaccaggcggagagctgctgcagttgcttcttctgcagttccatcagcacatcgtgcagccgggactgtctgtccatactctccaccctaagagcctcccatctagcattcagcagggtcatctgttcctgaatctcaaattcttcttcgtctgacagagttccttgtgttatcagttggttgcctgcctgcaggacgctgcccacactgctctggtgtgcagtcagttccatcataaaagcttcatgggttgcaaactggtctttgacttcttcaacatcatcagaaatatcatcctgctcctggaaagtgtcctcagcagaaagcaaccaggtcagcacttcctccaacgcaatctgatagctgtccagatccatgtcaacctcagtgacagtgctgggagtttcagctcggggactctcatgctcctcctcaggcgctgtactctgtatattaattgcctcttcttcacattcttttttatatttccttgggagtgtctctacctcacggatggcgtctatggtgacttgctgaggtagcacctcaaacaaagatgttaaatacataattatggatttcttgtcaggaagctgaacggcaacatcttcaggatctaacagcttttcaattcccaaataagtttgagccttgctgaaggcatgttcaagtctctcaattggtgacattttgacaactttatcccagctgaagagatcaggtttatgtcggtggaggacagcattaaaggcgagtccatctgtccagctggtggtgaagttgaggacgttgacttggctgtagggcctggtggtctgacgcacccagctgagcaggatcttctcactgttcgtctgctgcaggtccgacatgacatccttcatgacatctttcacctgccagtgcaaaatgatgctccaaagtaaccccaaagtcagtttgtgatttccatccacaatgtcagttccccctatattcactaattccacattgttctgatgtaaaacctgcagcactctgttgacgttatttaaggcatgtacccttgtggaaccacgttcctttggcagtgatgttcctgtgaggccttctagaagatccaatagcttccttccatctttgaggtctgtgaacatatcattgatgggtggtttcccactctttgaaaatcgagcatttatccatttggtaaaggttttcttctgtacgtcattgtgttcatcaattaggttgagttggtgatgcaatccgatggcaggagattgcagctggggaatctggtctgaatgcggaatgaggagcaaagggccattatctctctctcctgtagtaggagagggcagatctggacttaatgatatcactgaattcgttctgcccattgtcaggactggcttcatgttctccatacttggccatcttgccagagtttcaagataatccaaaaactttaccaagtcctctttctaaggctttcaacttcctacgatggttcagcttgacatcaataccttgtcagttgcagcaagagatccccagagtccggaaaaggagagccggcgactgcgcgggactacacaccaatggggcgcccccctcctcctgtcccctca

SEQ ID NO: 10732 - RNA, 11762 nt, Homo sapiens
  source 1..11762: mol_type = other RNA
ctcatctgcaaagaagtaagtgggcaacgtcaaataaagttaaacggcatacacagggctgtagcttaaaccatatgtgtgtatatataagatatttgattgaaatttatgaatttattaatgtggccaaatcacggaaacaaatacatggatctatttgggatctagttggttatatggctgataaacatatggctgataaattataaataaccaaaacattgtggtaaaagagtcaaagaaaaaatgaagtaattgtgcaaggttaatatgaacagcagaaggaatgtaaaaatgtaaagtggtcttctaattcttatgtaagctttgtcatagttattaaaaagacggtatcatattagaaagcccccacccactttcccaatgctgtatacattatacaaatccgtgacaaatgtattaccatttccaaatacctctctgttcattaatttacacttgcatagaaagggaagaagaaaacaataatatatggttattataaaaacaaaatatccatttctctttggatagtcagtgttttactctttcagtagaacacacagtcagcactcaacatcgtgggccaaggagccatggagcttctgatttaatggaacttggaattggcatttgctgaaaagggcaacactgtacgtcaggaaacattggttggccggatgaatacttcacattgcctgtggcctgctgggaacatttgggcagcaagatggaaacgtgctgtgaatctgctccatgacctccgtgagatccgtgctggtgtcgtgcggtggggccagcaggtcctctcccgctgcctggtggaactgtgggccggaggcatctggatcaagcgagtagctcagtgcagaatgctgaggagaagcccatggggaaacaccattgattcgggaatcagattcaggctgctccagcagctgtcggaggcggtggagctgagactccagctgtttattgtgatcttctaaaatctgcatcctagcctccagccgacctttgtgctgcctgaggagttttgcttctgctataagttctgaatcctcagacgtgtgatggggagatataatcgactctggcggtgaaccgacagggagcccccttcggaggtgctggtccttcagctgctcatactccacctgtagatttctttgttcttcctccaggtcagcaatgatcctctccagttctccacgttcttccctctctactgacttcaggatctgagctgggctctgcggctggctcactggggactctcctccgagtgtttggcaatactgctggatgagggcgtgctcgtcttccacacttcctgtggtggagctgctatcagtgagaaaagacccattagtcctttccatctgggccagtcgtgtggcatattgttctattcttgaatgggtgtcatcatgaaacagttgaggagattgtgaggggtcatagtgctctggccacatactgatgagtgtgataggagtctctaagttgtcaccttcaagaactgtctggacaggcaggtaaccaagtcgagggtgtttggcaaagtacttcttcgacctgaacttgttcttaagtacctttgtgaagtctcgtacatcttccccagatgttgtaggtatacaatattccaccattgggtaatgtaatttgtgaccttttgctgttcgacccgaaaagaaacaactctggcagacatcatagttaaaatgcttaaggcttctatacctgaacccgacaattggacattctttacagatgttgcatttggcctgatgttttgcagtctccgctgctgccactcgatgtaaaactgggagccaaaccatggactgtggttccaaatgcatccaatctataaactctttcacacttatttctggtttattgttattctgttggaagcagctgcgaacactaggctcaatattactgcctccaaaagctgctacttcacctagctgccgggggatctggatggcatcatgaagtaacaggcccagctgcctctggtcacacatttctgttggccctgcaacttccttaaagagatatctgtatttttcttccaagagacctttggagagagacattaatccaatcttcagactctgcactctaatttttccagttcgacccgtgtcatagacattgagcaaccaattgagacacatatcaacacagagtggaacgttgaccaggtccttatgcatttgctcaagtccatcataagttgttgtcagacagttgatgacatctggaacactgaggagctggtcattttggttcaacttgtgctgtttgaaaatttcatttgttgtactcaactctaagagatccaaacatagtgctttttgtagtcttcggattttgattgctgtacggtaggcagaaaaacgtacattattcaggtcagcaagggattgaaagagttcggtcattttaggatggtcccaacaggtggtctgtgtttgatggttgatgtaatagggcactttattatgtgaaatggatctttgccacggcagctggactgacgtagagagaaaatgctgagaggatggtccaaaatctctgtgggcttcctgaagctgtttaaggcgatcatccacagaaacctgtaaaagtttccatcgcatattaaggtcatctagctggcgagacatctttagagagggatgcaggtcaagtggagacagctgactggataaatcattcaccgttttaactttaaagttgattggtgcaatttcttctctaaatgccatgattttttcaatgtgatcctgcagcgagtcaatgagtaagtctcccacgggcttccagccattccgcacggactctgcctccttcatgtcagcgtccaggtcatccatagctccctgcaggtctctgagtttctccaatgccttgtccacttgcttttgccaattgctagttacagcatttagactttcccatttttctttgacttcagaagactgtttgcgcatggctttggcaatcttttgggctctctcctcaggagttaattctgtttttgattgtaggtttcttcttggctcttcaggggcctcaattggctgatcagccaagaaaactcgggcctggtcgacagcattcaggacagaatattctttctcctttaactcccgtctcagggccttacaatggtcatactggagctgtaaggctggaacatctcctccaataggcatttgtttcttaagctcttcatctttcatattcagccatttgatcagttcttctaaggacatcagcaacctgttccacttctcagcgctggcctccaaatgggccctgatgctagcagattttgcttttaagtcattccatctttggttcatatcatccagtcgatgttgaagcatagtagcctcttcagaatttcccaaagcttttaccatcttctgcctgtttccgtcaatgcttttaaatatgtcattgtgggcatcaatttctgcctggatgtcctgcatctgctgtttgagttccctggccaagatactatcctgaagagcattctcccgatgagaggcatccacaagcacattcactgtggtctctgcttcttggatccacttcaggaagttttccagatctctgcgagaggcctgcaccgtcctccactcagcctccaaggcgttctgtctgtcagcaatactttgtttgagattgatccatgatgtttttaagtactctgtggtttctttcacattccttgtgtcatcactcccatattcctccaggagtttctgcaggacgttatcgaacgccatgacgataccatctccaggacccagttcttgaagcagtatttggttatcagaaatttgtttggtgagtggatcccgtcgggcttgctgaagaatatagagtcgagcctcatattttctcatcagttcttcagtctcctccctatggtcatcccactgaagactgtcaataatcatgtcctcaagctgctgctgtcttagctcaacgccatgctgggtgccatcccactggttcttgaccctttccaatttttctgtaattgctgttctcatatctgaactggaagctttatttttcaaattctgtgccaatgtaaaaacataatccagctgaggatggcgctgttctaagtcagcctttgtaattttcattcgggaaacggtcttattgatctcttctacatccccaacagtgacaatgttggacttcagcatctggtcgattaataccagccagtcggctagttctgttatagttttatcaagatcagcaggaattgaaatttccgaagtacgatgagactgaacaggaatatctgacgcagatgatactagcaccaccttttggacattaggatgagcagcaatccttgtctgtgaaacagaactgggctcctggatgcattccttcagggtggtaggcacctctctgcaaatcttattccatgtcatatttacagtccttaagctttctgaaattttatccctttcaggtaaactcagacttttatctgaaagcatctccaattcagttctattcagccatttgagtttttcagcatgtacttccatttcttgagttaagtctcttaattcttgcaggttttctcccaattcggtggttgatctcttttgcatagcatgctcagcctttgttaaccaacagataatctcatctagctgatgcctgtacttcatcacctgcttactttctccttttagccttggctgcctatccttcacttctgcaacaattgcatcccagcgttggtttaaacctgccagtttttctttcaagaagcttccatctgcctgggagagtttctgcacaatcccatccccagttcggtttagtgctgcaaaactgggctggtggctgctgatgcccacctcaagttcctgctgatgtatcctggctttctctaagtccaggctgccacctggagcacaggtatcaaccagtaattcttcagcctctgttatccactgtgtgaggtcattaaggtcacaatggaactgtctccattcttccattgccctgtcaaaacaacctttccgatcactgtacattctattaattctgtcccattttgcattcagctgagtaagtgtatctctgatctgaatggcttcaggtccagaggcttcaaggatgacatctggctgtttttcatgaatgactgcaatctgctctccaagtttgtccagttggtctttgatattcttcagagagtcttcctgaaaagagaagtcttcgtaaatagcagtgttgagctctggaacattaagcgataattcaacatcatccatgcaaagtaaaattttgttaatttcaaccagataatctgtaggaagaagtgatgatctaattccagaagcaagttgacccattttcctctgttgaatagggattgccttaattttgttgtatctagtatgcaaaagtaataattgcaaacggatcttttcttttttattatcttccataggttgatgtaacatttcttctcctctttgtagaacttcctcaatctgggcactctcctcatccatcttttcatcttcatcactggattccaagtgtttttccacaaattttaacatattttctatgtcattttctaatttttccaagtcagagaaaggcacaccagtttcaaatgtttcagtggtgaccaaacattggtataatggttcctgagcaattagcaatttggcacttttgatatgttgagacaccttttcaaagttcctattcagctcagctaactttggttctacaagctccctgcttgagcttccacgggcattcatcaaaataagggcttgatcgcggacattttcaacctggaggttggcatcatccagctcagatactaaacgcttcacaatttcttcctgtttacttgttggtttcttttcaatttcatccaatagagcttcagcttgataaagccaggtacttatgtgagccacgttcccatcaaatatttctagctggttctgatggttcatcaaggtattgcaccaatcttcagtccaggtacgaactcggctccacccagcgttaaggacgcagagcctctcttctaaaataggctcactgccctcaatcaagttttgcagggcagcactactctctgtgatggtatttaaatcagcttttctcttttccagatccttcagaacatttttagcccaggaaatttctgtatccaagtcaccaagcagaccttctgaagtggacttctgtaccaattcagtttcagtagcagaaagccattcagagagagaagcagcctctttcttcattttccgggccaactgtgatgctctttccagatcctgttttccttctgtcacctgtgcgcccaggtcattgtaaagaaccttcagggaagtcagctgctcatccatcccttttgggttgtccgtttgctgtttctggacaatatgtcttcctgttttaatcacagtttccacttcaagtttgacttcactcaaagttttatacagtttcatacacttgtccaggtgcgtctgtatgacgtcagggtctacgtccttcacatccagaacgtgaagttctgctttcacgccatccagcacacgcttgcagtccagcatgcgctgctcgaagttagctggcttctggaaaagctggaactttgtggacacctctcggagtttcctctgtagcacatccatctgacttcctcctctggcagtcctactctctggggaggtcaggggctgagaacgcatatttcttctcaactcctctagggttagctcatgggctgagatctctgcttggattttctgagcttcctgtggaacttggaaagcatctatcctgtcagtcaggtatgtggtgagctgtttgtccagctcccccaagctctcttgcaagacttgaagcatctggtcagtttcccgcagcacctggagttgcttttccaaagaaatctgcttgctctctgccaggtgacttagatcttcatatcggctgttgaaagcctccagtttctcactgattatatcatccaggatccccccatcaatcagagtctggccaagctctcgaatctgggtgcgattatctgccgggtggcgcagaacagattccagagactccagggcttcgttgacagcatccgtcttctcaggcaggacctctgtgctcttcatccgctcttccaaagtgtttaaccaggtagtttcaagatccaaatagtgaagcagttcaatccaacaagaccagacctcctctagcgtgtggcactttcctcgaattctattacaaagaagttggtaattctccagcacaacattcagctcagacgtcaactcctggccaccagagggcaccttggcagctaataacttgatgttgtccttgagaatcttcactctcacctccttctgcaacacatcctcttttgccctcttcatctcttccacagcactctcaagctcttctggtgacttgtactcaaaatcccgctccaaatattcttcctcggcctgggtcatccattcctgcatctctgccaagtctttcttcaggttcgcagctttttcttgactttcagacaacctacttttttgagtagcgatctccttgctaagtttctccagttgagtttggtagtcacctagtcttgtctgcacccaagtttttattccagcaactggaccacttcgaagattagtctctatttccttcatgtttttcagagatgattcaattgtttctatttcattaacaaatgcagagcactggtctaactgcctctgtagacctgcgtcgtctccttgggcagcctgctgtttcattaagaagtctttcacgccatccatccacttctcaatgactgttgaatcggcctcaaaagctctgagtgtgagagcaatttcctcaagcaaatgtagatctttggaaaccaagacctttagcttgttccactttccttgcacatcatcaaattcttgcttatataatttttctacatcaggatgaacatttttctccagagcctttgtttcttctgcaagtttatgtaatgcaggtttctgattctcaaggatttcatcaagggtctttttttcttgcagggccttctccaccttggcaagatcattaaggacattcagagacacctgggccttattttctgaatcatttagcacatctttcagtgttttcaatgtttccagatatgcatgtccaggttggcccttcagttcattctctagatgttgttgacgatcctctacagcctcttgtacagcttggtagcggcccagaaagctatcgaagccccgctggacaaaatctggggcagaaggctgagacatcagggccgagcagcttgcacgagccatttcaattttggggtgaaggccaagaagatttgtcaattcccgctgacaggaatccttcaagcttggcaaggactgccgggaagattcagaaatggaagtgtgttttacccactcctcctttgtcttgatgaccttttcaagctcatcaagctgcttgaaataagcatttatatcttcctgtagctgaatctttctttctagatcttccaaatgttgagatacattcttccattctgatgaaaccttctccagaacattttttatttcttcagtaggaaggccttcttttcccatttgctccacaaggatttgtccagtttggtttaattcatctgctctggggattctttctctctgttctttttctaatgccttcaacttctttttcatttcggaagtgtcttgcatcttcatatactcttttatctctgtggtctgaatggcagttttccatttcaaaatccagttcaacagctctgcacttatagcatcaaactttttcttagcttcaatatccacatggatctgtctcttctttgggggaggaggaggaggcagttcctgcttagatttttttgtaattgcttgttctcttacacgaacagtctccaaaaggtccttctgaggaatctgagacatccccagctttgctacagcctgagtcacctggttggaggaatcttctagtctctgaaccaaagaatcccatctttgagtcagttcctctgagtcactgttgatcttcttagatgccttggaattatcaagtaattgtcccacatcctggccaatctcactcagctgatccaatgtttgacgcttcatttccatgtcttccttcaaaatagccagacgtcgaacactgacacttagttccttttggtctttgaagttgcttgtctggactttatttaaagcctcttctttttcggttaaccaagctttcaacaagcactgttcttccaataattcctgccacaatatattgatttcttgtaacctattccagcgttcttcagtccaacggcatactgctgtccagcgctcaccaagtttctgtaactggtcttctaggatagctgtagcactctcaccactgttttcatcaacaatgaccaccatgtgagttagtgaatttactttcacctgttcagcctcaagatcactttgcaaacttttatgttcttctagcagcttttgtagagattttacatcatcatccagggggcaagtttccatcttctgaatgcgctcctctgtgagtgttaaccaggcggagagctgctgcagttgcttcttctgcagttccatcagcacatcgtgcagccgggactgtctgtccatactctccaccctaagagcctcccatctagcattcagcagggtcatctgttcctgaatctcaaattcttcttcgtctgacagagttccttgtgttatcagttggttgcctgcctgcaggacgctgcccacactgctctggtgtgcagtcagttccatcataaaagcttcatgggttgcaaactggtctttgacttcttcaacatcatcagaaatatcatcctgctcctggaaagtgtcctcagcagaaagcaaccaggtcagcacttcctccaacgcaatctgatagctgtccagatccatgtcaacctcagtgacagtgctgggagtttcagctcggggactctcatgctcctcctcaggcgctgtactctgtatattaattgcctcttcttcacattcttttttatatttccttgggagtgtctctacctcacggatggcgtctatggtgacttgctgaggtagcacctcaaacaaagatgttaaatacataattatggatttcttgtcaggaagctgaacggcaacatcttcaggatctaacagcttttcaattcccaaataagtttgagccttgctgaaggcatgttcaagtctctcaattggtgacattttgacaactttatcccagctgaagagatcaggtttatgtcggtggaggacagcattaaaggcgagtccatctgtccagctggtggtgaagttgaggacgttgacttggctgtagggcctggtggtctgacgcacccagctgagcaggatcttctcactgttcgtctgctgcaggtccgacatgacatccttcatgacatctttcacctgccagtgcaaaatgatgctccaaagtaaccccaaagtcagtttgtgatttccatccacaatgtcagttccccctatattcactaattccacattgttctgatgtaaaacctgcagcactctgttgacgttatttaaggcatgtacccttgtggaaccacgttcctttggcagtgatgttcctgtgaggccttctagaagatccaatagcttccttccatctttgaggtctgtgaacatatcattgatgggtggtttcccactctttgaaaatcgagcatttatccatttggtaaaggttttcttctgtacgtcattgtgttcatcaattaggttgagttggtgatgcaatccgatggcaggagattgcagctggggaatctggtctgaatgcggaatgaggagcaaagggccattatctctctctcctgtagtaggagagggcagatctggacttaatgatatcactgaattcgttctgcccattgtcaggactggcttcatgttctccatacttggccatcttgccagagtttcaagataatccaaaaactttaccaagtcctctttctaaggctttcaacttcctacgatggttcagcttgacatcaatacctgctgcccgcgggcctcctcgcctgccggtcgccaccgccgcaccccgagctggccaagggctcctctaggagtttgacacggagtaaccgcgggggtgtgtgcgagtgttagtttggtggtgcgatgtatttaaaaaaaaaaataaagcttggagaagcagacacgaaccgaaattttaaaaaaagaaagaaagaaagagaaattgacacccgactgaaaacgccccttacttgtgcaatcttcctgcctggtagttccgccaaaaacaaaacagtcaaagcgcaaacctggaaggggcgcgcaggcaccaactttgccaaacgctacagagttttccgtttgcagaaatgacccaaaagaaggggggcgccgctccccgtgattccccaatcggcttctggagccagaggctcctcctcgcccctcggcgggagaaagcccgcggccggctgctgctgcccgcttccctgctccgaggaaaaacgactccacaactttgtgcgcgagagaggctcgctccttcggcggctcctcctcctcctccccgctgcgggcctg

SEQ ID NO: 10733 - RNA, 11303 nt, Homo sapiens
  source 1..11303: mol_type = other RNA
ctcatctgcaaagaagtaagtgggcaacgtcaaataaagttaaacggcatacacagggctgtagcttaaaccatatgtgtgtatatataagatatttgattgaaatttatgaatttattaatgtggccaaatcacggaaacaaatacatggatctatttgggatctagttggttatatggctgataaacatatggctgataaattataaataaccaaaacattgtggtaaaagagtcaaagaaaaaatgaagtaattgtgcaaggttaatatgaacagcagaaggaatgtaaaaatgtaaagtggtcttctaattcttatgtaagctttgtcatagttattaaaaagacggtatcatattagaaagcccccacccactttcccaatgctgtatacattatacaaatccgtgacaaatgtattaccatttccaaatacctctctgttcattaatttacacttgcatagaaagggaagaagaaaacaataatatatggttattataaaaacaaaatatccatttctctttggatagtcagtgttttactctttcagtagaacacacagtcagcactcaacatcgtgggccaaggagccatggagcttctgatttaatggaacttggaattggcatttgctgaaaagggcaacactgtacgtcaggaaacattggttggccggatgaatacttcacattgcctgtggcctgctgggaacatttgggcagcaagatggaaacgtgctgtgaatctgctccatgacctccgtgagatccgtgctggtgtcgtgcggtggggccagcaggtcctctcccgctgcctggtggaactgtgggccggaggcatctggatcaagcgagtagctcagtgcagaatgctgaggagaagcccatggggaaacaccattgattcgggaatcagattcaggctgctccagcagctgtcggaggcggtggagctgagactccagctgtttattgtgatcttctaaaatctgcatcctagcctccagccgacctttgtgctgcctgaggagttttgcttctgctataagttctgaatcctcagacgtgtgatggggagatataatcgactctggcggtgaaccgacagggagcccccttcggaggtgctggtccttcagctgctcatactccacctgtagatttctttgttcttcctccaggtcagcaatgatcctctccagttctccacgttcttccctctctactgacttcaggatctgagctgggctctgcggctggctcactggggactctcctccgagtgtttggcaatactgctggatgagggcgtgctcgtcttccacacttcctgtggtggagctgctatcagtgagaaaagacccattagtcctttccatctgggccagtcgtgtggcatattgttctattcttgaatgggtgtcatcatgaaacagttgaggagattgtgaggggtcatagtgctctggccacatactgatgagtgtgataggagtctctaagttgtcaccttcaagaactgtctggacaggcaggtaaccaagtcgagggtgtttggcaaagtacttcttcgacctgaacttgttcttaagtacctttgtgaagtctcgtacatcttccccagatgttgtaggtatacaatattccaccattgggtaatgtaatttgtgaccttttgctgttcgacccgaaaagaaacaactctggcagacatcatagttaaaatgcttaaggcttctatacctgaacccgacaattggacattctttacagatgttgcatttggcctgatgttttgcagtctccgctgctgccactcgatgtaaaactgggagccaaaccatggactgtggttccaaatgcatccaatctataaactctttcacacttatttctggtttattgttattctgttggaagcagctgcgaacactaggctcaatattactgcctccaaaagctgctacttcacctagctgccgggggatctggatggcatcatgaagtaacaggcccagctgcctctggtcacacatttctgttggccctgcaacttccttaaagagatatctgtatttttcttccaagagacctttggagagagacattaatccaatcttcagactctgcactctaatttttccagttcgacccgtgtcatagacattgagcaaccaattgagacacatatcaacacagagtggaacgttgaccaggtccttatgcatttgctcaagtccatcataagttgttgtcagacagttgatgacatctggaacactgaggagctggtcattttggttcaacttgtgctgtttgaaaatttcatttgttgtactcaactctaagagatccaaacatagtgctttttgtagtcttcggattttgattgctgtacggtaggcagaaaaacgtacattattcaggtcagcaagggattgaaagagttcggtcattttaggatggtcccaacaggtggtctgtgtttgatggttgatgtaatagggcactttattatgtgaaatggatctttgccacggcagctggactgacgtagagagaaaatgctgagaggatggtccaaaatctctgtgggcttcctgaagctgtttaaggcgatcatccacagaaacctgtaaaagtttccatcgcatattaaggtcatctagctggcgagacatctttagagagggatgcaggtcaagtggagacagctgactggataaatcattcaccgttttaactttaaagttgattggtgcaatttcttctctaaatgccatgattttttcaatgtgatcctgcagcgagtcaatgagtaagtctcccacgggcttccagccattccgcacggactctgcctccttcatgtcagcgtccaggtcatccatagctccctgcaggtctctgagtttctccaatgccttgtccacttgcttttgccaattgctagttacagcatttagactttcccatttttctttgacttcagaagactgtttgcgcatggctttggcaatcttttgggctctctcctcaggagttaattctgtttttgattgtaggtttcttcttggctcttcaggggcctcaattggctgatcagccaagaaaactcgggcctggtcgacagcattcaggacagaatattctttctcctttaactcccgtctcagggccttacaatggtcatactggagctgtaaggctggaacatctcctccaataggcatttgtttcttaagctcttcatctttcatattcagccatttgatcagttcttctaaggacatcagcaacctgttccacttctcagcgctggcctccaaatgggccctgatgctagcagattttgcttttaagtcattccatctttggttcatatcatccagtcgatgttgaagcatagtagcctcttcagaatttcccaaagcttttaccatcttctgcctgtttccgtcaatgcttttaaatatgtcattgtgggcatcaatttctgcctggatgtcctgcatctgctgtttgagttccctggccaagatactatcctgaagagcattctcccgatgagaggcatccacaagcacattcactgtggtctctgcttcttggatccacttcaggaagttttccagatctctgcgagaggcctgcaccgtcctccactcagcctccaaggcgttctgtctgtcagcaatactttgtttgagattgatccatgatgtttttaagtactctgtggtttctttcacattccttgtgtcatcactcccatattcctccaggagtttctgcaggacgttatcgaacgccatgacgataccatctccaggacccagttcttgaagcagtatttggttatcagaaatttgtttggtgagtggatcccgtcgggcttgctgaagaatatagagtcgagcctcatattttctcatcagttcttcagtctcctccctatggtcatcccactgaagactgtcaataatcatgtcctcaagctgctgctgtcttagctcaacgccatgctgggtgccatcccactggttcttgaccctttccaatttttctgtaattgctgttctcatatctgaactggaagctttatttttcaaattctgtgccaatgtaaaaacataatccagctgaggatggcgctgttctaagtcagcctttgtaattttcattcgggaaacggtcttattgatctcttctacatccccaacagtgacaatgttggacttcagcatctggtcgattaataccagccagtcggctagttctgttatagttttatcaagatcagcaggaattgaaatttccgaagtacgatgagactgaacaggaatatctgacgcagatgatactagcaccaccttttggacattaggatgagcagcaatccttgtctgtgaaacagaactgggctcctggatgcattccttcagggtggtaggcacctctctgcaaatcttattccatgtcatatttacagtccttaagctttctgaaattttatccctttcaggtaaactcagacttttatctgaaagcatctccaattcagttctattcagccatttgagtttttcagcatgtacttccatttcttgagttaagtctcttaattcttgcaggttttctcccaattcggtggttgatctcttttgcatagcatgctcagcctttgttaaccaacagataatctcatctagctgatgcctgtacttcatcacctgcttactttctccttttagccttggctgcctatccttcacttctgcaacaattgcatcccagcgttggtttaaacctgccagtttttctttcaagaagcttccatctgcctgggagagtttctgcacaatcccatccccagttcggtttagtgctgcaaaactgggctggtggctgctgatgcccacctcaagttcctgctgatgtatcctggctttctctaagtccaggctgccacctggagcacaggtatcaaccagtaattcttcagcctctgttatccactgtgtgaggtcattaaggtcacaatggaactgtctccattcttccattgccctgtcaaaacaacctttccgatcactgtacattctattaattctgtcccattttgcattcagctgagtaagtgtatctctgatctgaatggcttcaggtccagaggcttcaaggatgacatctggctgtttttcatgaatgactgcaatctgctctccaagtttgtccagttggtctttgatattcttcagagagtcttcctgaaaagagaagtcttcgtaaatagcagtgttgagctctggaacattaagcgataattcaacatcatccatgcaaagtaaaattttgttaatttcaaccagataatctgtaggaagaagtgatgatctaattccagaagcaagttgacccattttcctctgttgaatagggattgccttaattttgttgtatctagtatgcaaaagtaataattgcaaacggatcttttcttttttattatcttccataggttgatgtaacatttcttctcctctttgtagaacttcctcaatctgggcactctcctcatccatcttttcatcttcatcactggattccaagtgtttttccacaaattttaacatattttctatgtcattttctaatttttccaagtcagagaaaggcacaccagtttcaaatgtttcagtggtgaccaaacattggtataatggttcctgagcaattagcaatttggcacttttgatatgttgagacaccttttcaaagttcctattcagctcagctaactttggttctacaagctccctgcttgagcttccacgggcattcatcaaaataagggcttgatcgcggacattttcaacctggaggttggcatcatccagctcagatactaaacgcttcacaatttcttcctgtttacttgttggtttcttttcaatttcatccaatagagcttcagcttgataaagccaggtacttatgtgagccacgttcccatcaaatatttctagctggttctgatggttcatcaaggtattgcaccaatcttcagtccaggtacgaactcggctccacccagcgttaaggacgcagagcctctcttctaaaataggctcactgccctcaatcaagttttgcagggcagcactactctctgtgatggtatttaaatcagcttttctcttttccagatccttcagaacatttttagcccaggaaatttctgtatccaagtcaccaagcagaccttctgaagtggacttctgtaccaattcagtttcagtagcagaaagccattcagagagagaagcagcctctttcttcattttccgggccaactgtgatgctctttccagatcctgttttccttctgtcacctgtgcgcccaggtcattgtaaagaaccttcagggaagtcagctgctcatccatcccttttgggttgtccgtttgctgtttctggacaatatgtcttcctgttttaatcacagtttccacttcaagtttgacttcactcaaagttttatacagtttcatacacttgtccaggtgcgtctgtatgacgtcagggtctacgtccttcacatccagaacgtgaagttctgctttcacgccatccagcacacgcttgcagtccagcatgcgctgctcgaagttagctggcttctggaaaagctggaactttgtggacacctctcggagtttcctctgtagcacatccatctgacttcctcctctggcagtcctactctctggggaggtcaggggctgagaacgcatatttcttctcaactcctctagggttagctcatgggctgagatctctgcttggattttctgagcttcctgtggaacttggaaagcatctatcctgtcagtcaggtatgtggtgagctgtttgtccagctcccccaagctctcttgcaagacttgaagcatctggtcagtttcccgcagcacctggagttgcttttccaaagaaatctgcttgctctctgccaggtgacttagatcttcatatcggctgttgaaagcctccagtttctcactgattatatcatccaggatccccccatcaatcagagtctggccaagctctcgaatctgggtgcgattatctgccgggtggcgcagaacagattccagagactccagggcttcgttgacagcatccgtcttctcaggcaggacctctgtgctcttcatccgctcttccaaagtgtttaaccaggtagtttcaagatccaaatagtgaagcagttcaatccaacaagaccagacctcctctagcgtgtggcactttcctcgaattctattacaaagaagttggtaattctccagcacaacattcagctcagacgtcaactcctggccaccagagggcaccttggcagctaataacttgatgttgtccttgagaatcttcactctcacctccttctgcaacacatcctcttttgccctcttcatctcttccacagcactctcaagctcttctggtgacttgtactcaaaatcccgctccaaatattcttcctcggcctgggtcatccattcctgcatctctgccaagtctttcttcaggttcgcagctttttcttgactttcagacaacctacttttttgagtagcgatctccttgctaagtttctccagttgagtttggtagtcacctagtcttgtctgcacccaagtttttattccagcaactggaccacttcgaagattagtctctatttccttcatgtttttcagagatgattcaattgtttctatttcattaacaaatgcagagcactggtctaactgcctctgtagacctgcgtcgtctccttgggcagcctgctgtttcattaagaagtctttcacgccatccatccacttctcaatgactgttgaatcggcctcaaaagctctgagtgtgagagcaatttcctcaagcaaatgtagatctttggaaaccaagacctttagcttgttccactttccttgcacatcatcaaattcttgcttatataatttttctacatcaggatgaacatttttctccagagcctttgtttcttctgcaagtttatgtaatgcaggtttctgattctcaaggatttcatcaagggtctttttttcttgcagggccttctccaccttggcaagatcattaaggacattcagagacacctgggccttattttctgaatcatttagcacatctttcagtgttttcaatgtttccagatatgcatgtccaggttggcccttcagttcattctctagatgttgttgacgatcctctacagcctcttgtacagcttggtagcggcccagaaagctatcgaagccccgctggacaaaatctggggcagaaggctgagacatcagggccgagcagcttgcacgagccatttcaattttggggtgaaggccaagaagatttgtcaattcccgctgacaggaatccttcaagcttggcaaggactgccgggaagattcagaaatggaagtgtgttttacccactcctcctttgtcttgatgaccttttcaagctcatcaagctgcttgaaataagcatttatatcttcctgtagctgaatctttctttctagatcttccaaatgttgagatacattcttccattctgatgaaaccttctccagaacattttttatttcttcagtaggaaggccttcttttcccatttgctccacaaggatttgtccagtttggtttaattcatctgctctggggattctttctctctgttctttttctaatgccttcaacttctttttcatttcggaagtgtcttgcatcttcatatactcttttatctctgtggtctgaatggcagttttccatttcaaaatccagttcaacagctctgcacttatagcatcaaactttttcttagcttcaatatccacatggatctgtctcttctttgggggaggaggaggaggcagttcctgcttagatttttttgtaattgcttgttctcttacacgaacagtctccaaaaggtccttctgaggaatctgagacatccccagctttgctacagcctgagtcacctggttggaggaatcttctagtctctgaaccaaagaatcccatctttgagtcagttcctctgagtcactgttgatcttcttagatgccttggaattatcaagtaattgtcccacatcctggccaatctcactcagctgatccaatgtttgacgcttcatttccatgtcttccttcaaaatagccagacgtcgaacactgacacttagttccttttggtctttgaagttgcttgtctggactttatttaaagcctcttctttttcggttaaccaagctttcaacaagcactgttcttccaataattcctgccacaatatattgatttcttgtaacctattccagcgttcttcagtccaacggcatactgctgtccagcgctcaccaagtttctgtaactggtcttctaggatagctgtagcactctcaccactgttttcatcaacaatgaccaccatgtgagttagtgaatttactttcacctgttcagcctcaagatcactttgcaaacttttatgttcttctagcagcttttgtagagattttacatcatcatccagggggcaagtttccatcttctgaatgcgctcctctgtgagtgttaaccaggcggagagctgctgcagttgcttcttctgcagttccatcagcacatcgtgcagccgggactgtctgtccatactctccaccctaagagcctcccatctagcattcagcagggtcatctgttcctgaatctcaaattcttcttcgtctgacagagttccttgtgttatcagttggttgcctgcctgcaggacgctgcccacactgctctggtgtgcagtcagttccatcataaaagcttcatgggttgcaaactggtctttgacttcttcaacatcatcagaaatatcatcctgctcctggaaagtgtcctcagcagaaagcaaccaggtcagcacttcctccaacgcaatctgatagctgtccagatccatgtcaacctcagtgacagtgctgggagtttcagctcggggactctcatgctcctcctcaggcgctgtactctgtatattaattgcctcttcttcacattcttttttatatttccttgggagtgtctctacctcacggatggcgtctatggtgacttgctgaggtagcacctcaaacaaagatgttaaatacataattatggatttcttgtcaggaagctgaacggcaacatcttcaggatctaacagcttttcaattcccaaataagtttgagccttgctgaaggcatgttcaagtctctcaattggtgacattttgacaactttatcccagctgaagagatcaggtttatgtcggtggaggacagcattaaaggcgagtccatctgtccagctggtggtgaagttgaggacgttgacttggctgtagggcctggtggtctgacgcacccagctgagcaggatcttctcactgttcgtctgctgcaggtccgacatgacatccttcatgacatctttcacctgccagtgcaaaatgatgctccaaagtaaccccaaagtcagtttgtgatttccatccacaatgtcagttccccctatattcactaattccacattgttctgatgtaaaacctgcagcactctgttgacgttatttaaggcatgtacccttgtggaaccacgttcctttggcagtgatgttcctgtgaggccttctagaagatccaatagcttccttccatctttgaggtctgtgaacatatcattgatgggtggtttcccactctttgaaaatcgagcatttatccatttggtaaaggttttcttctgtacgtcattgtgttcatcaattaggttgagttggtgatgcaatccgatggcaggagattgcagctggggaatctggtctgaatgcggaatgaggagcaaagggccattatctctctctcctgtagtaggagagggcagatctggacttaatgatatcactgaattcgttctgcccattgtcaggactggcttcatgttctccatacttggccatcttgccagagtttcaagataatccaaaaactttaccaagtcctctttctaaggctttcaacttcctacgatggttcagcttgacatcaataccttgtcagttgcagcaagagatccccagagtccggaaaaggagagccggcgactgcgcgggactacacaccaatggggcgcccccctcctcctgtcccctca

SEQ ID NO: 10734 - RNA, 11083 nt, Homo sapiens
  source 1..11083: mol_type = other RNA
ctcatctgcaaagaagtaagtgggcaacgtcaaataaagttaaacggcatacacagggctgtagcttaaaccatatgtgtgtatatataagatatttgattgaaatttatgaatttattaatgtggccaaatcacggaaacaaatacatggatctatttgggatctagttggttatatggctgataaacatatggctgataaattataaataaccaaaacattgtggtaaaagagtcaaagaaaaaatgaagtaattgtgcaaggttaatatgaacagcagaaggaatgtaaaaatgtaaagtggtcttctaattcttatgtaagctttgtcatagttattaaaaagacggtatcatattagaaagcccccacccactttcccaatgctgtatacattatacaaatccgtgacaaatgtattaccatttccaaatacctctctgttcattaatttacacttgcatagaaagggaagaagaaaacaataatatatggttattataaaaacaaaatatccatttctctttggatagtcagtgttttactctttcagtagaacacacagtcagcactcaacatcgtgggccaaggagccatggagcttctgatttaatggaacttggaattggcatttgctgaaaagggcaacactgtacgtcaggaaacattggttggccggatgaatacttcacattgcctgtggcctgctgggaacatttgggcagcaagatggaaacgtgctgtgaatctgctccatgacctccgtgagatccgtgctggtgtcgtgcggtggggccagcaggtcctctcccgctgcctggtggaactgtgggccggaggcatctggatcaagcgagtagctcagtgcagaatgctgaggagaagcccatggggaaacaccattgattcgggaatcagattcaggctgctccagcagctgtcggaggcggtggagctgagactccagctgtttattgtgatcttctaaaatctgcatcctagcctccagccgacctttgtgctgcctgaggagttttgcttctgctataagttctgaatcctcagacgtgtgatggggagatataatcgactctggcggtgaaccgacagggagcccccttcggaggtgctggtccttcagctgctcatactccacctgtagatttctttgttcttcctccaggtcagcaatgatcctctccagttctccacgttcttccctctctactgacttcaggatctgagctgggctctgcggctggctcactggggactctcctccgagtgtttggcaatactgctggatgagggcgtgctcgtcttccacacttcctgtggtggagctgctatcagtgagaaaagacccattagtcctttccatctgggccagtcgtgtggcatattgttctattcttgaatgggtgtcatcatgaaacagttgaggagattgtgaggggtcatagtgctctggccacatactgatgagtgtgataggagtctctaagttgtcaccttcaagaactgtctggacaggcaggtaaccaagtcgagggtgtttggcaaagtacttcttcgacctgaacttgttcttaagtacctttgtgaagtctcgtacatcttccccagatgttgtaggtatacaatattccaccattgggtaatgtaatttgtgaccttttgctgttcgacccgaaaagaaacaactctggcagacatcatagttaaaatgcttaaggcttctatacctgaacccgacaattggacattctttacagatgttgcatttggcctgatgttttgcagtctccgctgctgccactcgatgtaaaactgggagccaaaccatggactgtggttccaaatgcatccaatctataaactctttcacacttatttctggtttattgttattctgttggaagcagctgcgaacactaggctcaatattactgcctccaaaagctgctacttcacctagctgccgggggatctggatggcatcatgaagtaacaggcccagctgcctctggtcacacatttctgttggccctgcaacttccttaaagagatatctgtatttttcttccaagagacctttggagagagacattaatccaatcttcagactctgcactctaatttttccagttcgacccgtgtcatagacattgagcaaccaattgagacacatatcaacacagagtggaacgttgaccaggtccttatgcatttgctcaagtccatcataagttgttgtcagacagttgatgacatctggaacactgaggagctggtcattttggttcaacttgtgctgtttgaaaatttcatttgttgtactcaactctaagagatccaaacatagtgctttttgtagtcttcggattttgattgctgtacggtaggcagaaaaacgtacattattcaggtcagcaagggattgaaagagttcggtcattttaggatggtcccaacaggtggtctgtgtttgatggttgatgtaatagggcactttattatgtgaaatggatctttgccacggcagctggactgacgtagagagaaaatgctgagaggatggtccaaaatctctgtgggcttcctgaagctgtttaaggcgatcatccacagaaacctgtaaaagtttccatcgcatattaaggtcatctagctggcgagacatctttagagagggatgcaggtcaagtggagacagctgactggataaatcattcaccgttttaactttaaagttgattggtgcaatttcttctctaaatgccatgattttttcaatgtgatcctgcagcgagtcaatgagtaagtctcccacgggcttccagccattccgcacggactctgcctccttcatgtcagcgtccaggtcatccatagctccctgcaggtctctgagtttctccaatgccttgtccacttgcttttgccaattgctagttacagcatttagactttcccatttttctttgacttcagaagactgtttgcgcatggctttggcaatcttttgggctctctcctcaggagttaattctgtttttgattgtaggtttcttcttggctcttcaggggcctcaattggctgatcagccaagaaaactcgggcctggtcgacagcattcaggacagaatattctttctcctttaactcccgtctcagggccttacaatggtcatactggagctgtaaggctggaacatctcctccaataggcatttgtttcttaagctcttcatctttcatattcagccatttgatcagttcttctaaggacatcagcaacctgttccacttctcagcgctggcctccaaatgggccctgatgctagcagattttgcttttaagtcattccatctttggttcatatcatccagtcgatgttgaagcatagtagcctcttcagaatttcccaaagcttttaccatcttctgcctgtttccgtcaatgcttttaaatatgtcattgtgggcatcaatttctgcctggatgtcctgcatctgctgtttgagttccctggccaagatactatcctgaagagcattctcccgatgagaggcatccacaagcacattcactgtggtctctgcttcttggatccacttcaggaagttttccagatctctgcgagaggcctgcaccgtcctccactcagcctccaaggcgttctgtctgtcagcaatactttgtttgagattgatccatgatgtttttaagtactctgtggtttctttcacattccttgtgtcatcactcccatattcctccaggagtttctgcaggacgttatcgaacgccatgacgataccatctccaggacccagttcttgaagcagtatttggttatcagaaatttgtttggtgagtggatcccgtcgggcttgctgaagaatatagagtcgagcctcatattttctcatcagttcttcagtctcctccctatggtcatcccactgaagactgtcaataatcatgtcctcaagctgctgctgtcttagctcaacgccatgctgggtgccatcccactggttcttgaccctttccaatttttctgtaattgctgttctcatatctgaactggaagctttatttttcaaattctgtgccaatgtaaaaacataatccagctgaggatggcgctgttctaagtcagcctttgtaattttcattcgggaaacggtcttattgatctcttctacatccccaacagtgacaatgttggacttcagcatctggtcgattaataccagccagtcggctagttctgttatagttttatcaagatcagcaggaattgaaatttccgaagtacgatgagactgaacaggaatatctgacgcagatgatactagcaccaccttttggacattaggatgagcagcaatccttgtctgtgaaacagaactgggctcctggatgcattccttcagggtggtaggcacctctctgcaaatcttattccatgtcatatttacagtccttaagctttctgaaattttatccctttcaggtaaactcagacttttatctgaaagcatctccaattcagttctattcagccatttgagtttttcagcatgtacttccatttcttgagttaagtctcttaattcttgcaggttttctcccaattcggtggttgatctcttttgcatagcatgctcagcctttgttaaccaacagataatctcatctagctgatgcctgtacttcatcacctgcttactttctccttttagccttggctgcctatccttcacttctgcaacaattgcatcccagcgttggtttaaacctgccagtttttctttcaagaagcttccatctgcctgggagagtttctgcacaatcccatccccagttcggtttagtgctgcaaaactgggctggtggctgctgatgcccacctcaagttcctgctgatgtatcctggctttctctaagtccaggctgccacctggagcacaggtatcaaccagtaattcttcagcctctgttatccactgtgtgaggtcattaaggtcacaatggaactgtctccattcttccattgccctgtcaaaacaacctttccgatcactgtacattctattaattctgtcccattttgcattcagctgagtaagtgtatctctgatctgaatggcttcaggtccagaggcttcaaggatgacatctggctgtttttcatgaatgactgcaatctgctctccaagtttgtccagttggtctttgatattcttcagagagtcttcctgaaaagagaagtcttcgtaaatagcagtgttgagctctggaacattaagcgataattcaacatcatccatgcaaagtaaaattttgttaatttcaaccagataatctgtaggaagaagtgatgatctaattccagaagcaagttgacccattttcctctgttgaatagggattgccttaattttgttgtatctagtatgcaaaagtaataattgcaaacggatcttttcttttttattatcttccataggttgatgtaacatttcttctcctctttgtagaacttcctcaatctgggcactctcctcatccatcttttcatcttcatcactggattccaagtgtttttccacaaattttaacatattttctatgtcattttctaatttttccaagtcagagaaaggcacaccagtttcaaatgtttcagtggtgaccaaacattggtataatggttcctgagcaattagcaatttggcacttttgatatgttgagacaccttttcaaagttcctattcagctcagctaactttggttctacaagctccctgcttgagcttccacgggcattcatcaaaataagggcttgatcgcggacattttcaacctggaggttggcatcatccagctcagatactaaacgcttcacaatttcttcctgtttacttgttggtttcttttcaatttcatccaatagagcttcagcttgataaagccaggtacttatgtgagccacgttcccatcaaatatttctagctggttctgatggttcatcaaggtattgcaccaatcttcagtccaggtacgaactcggctccacccagcgttaaggacgcagagcctctcttctaaaataggctcactgccctcaatcaagttttgcagggcagcactactctctgtgatggtatttaaatcagcttttctcttttccagatccttcagaacatttttagcccaggaaatttctgtatccaagtcaccaagcagaccttctgaagtggacttctgtaccaattcagtttcagtagcagaaagccattcagagagagaagcagcctctttcttcattttccgggccaactgtgatgctctttccagatcctgttttccttctgtcacctgtgcgcccaggtcattgtaaagaaccttcagggaagtcagctgctcatccatcccttttgggttgtccgtttgctgtttctggacaatatgtcttcctgttttaatcacagtttccacttcaagtttgacttcactcaaagttttatacagtttcatacacttgtccaggtgcgtctgtatgacgtcagggtctacgtccttcacatccagaacgtgaagttctgctttcacgccatccagcacacgcttgcagtccagcatgcgctgctcgaagttagctggcttctggaaaagctggaactttgtggacacctctcggagtttcctctgtagcacatccatctgacttcctcctctggcagtcctactctctggggaggtcaggggctgagaacgcatatttcttctcaactcctctagggttagctcatgggctgagatctctgcttggattttctgagcttcctgtggaacttggaaagcatctatcctgtcagtcaggtatgtggtgagctgtttgtccagctcccccaagctctcttgcaagacttgaagcatctggtcagtttcccgcagcacctggagttgcttttccaaagaaatctgcttgctctctgccaggtgacttagatcttcatatcggctgttgaaagcctccagtttctcactgattatatcatccaggatccccccatcaatcagagtctggccaagctctcgaatctgggtgcgattatctgccgggtggcgcagaacagattccagagactccagggcttcgttgacagcatccgtcttctcaggcaggacctctgtgctcttcatccgctcttccaaagtgtttaaccaggtagtttcaagatccaaatagtgaagcagttcaatccaacaagaccagacctcctctagcgtgtggcactttcctcgaattctattacaaagaagttggtaattctccagcacaacattcagctcagacgtcaactcctggccaccagagggcaccttggcagctaataacttgatgttgtccttgagaatcttcactctcacctccttctgcaacacatcctcttttgccctcttcatctcttccacagcactctcaagctcttctggtgacttgtactcaaaatcccgctccaaatattcttcctcggcctgggtcatccattcctgcatctctgccaagtctttcttcaggttcgcagctttttcttgactttcagacaacctacttttttgagtagcgatctccttgctaagtttctccagttgagtttggtagtcacctagtcttgtctgcacccaagtttttattccagcaactggaccacttcgaagattagtctctatttccttcatgtttttcagagatgattcaattgtttctatttcattaacaaatgcagagcactggtctaactgcctctgtagacctgcgtcgtctccttgggcagcctgctgtttcattaagaagtctttcacgccatccatccacttctcaatgactgttgaatcggcctcaaaagctctgagtgtgagagcaatttcctcaagcaaatgtagatctttggaaaccaagacctttagcttgttccactttccttgcacatcatcaaattcttgcttatataatttttctacatcaggatgaacatttttctccagagcctttgtttcttctgcaagtttatgtaatgcaggtttctgattctcaaggatttcatcaagggtctttttttcttgcagggccttctccaccttggcaagatcattaaggacattcagagacacctgggccttattttctgaatcatttagcacatctttcagtgttttcaatgtttccagatatgcatgtccaggttggcccttcagttcattctctagatgttgttgacgatcctctacagcctcttgtacagcttggtagcggcccagaaagctatcgaagccccgctggacaaaatctggggcagaaggctgagacatcagggccgagcagcttgcacgagccatttcaattttggggtgaaggccaagaagatttgtcaattcccgctgacaggaatccttcaagcttggcaaggactgccgggaagattcagaaatggaagtgtgttttacccactcctcctttgtcttgatgaccttttcaagctcatcaagctgcttgaaataagcatttatatcttcctgtagctgaatctttctttctagatcttccaaatgttgagatacattcttccattctgatgaaaccttctccagaacattttttatttcttcagtaggaaggccttcttttcccatttgctccacaaggatttgtccagtttggtttaattcatctgctctggggattctttctctctgttctttttctaatgccttcaacttctttttcatttcggaagtgtcttgcatcttcatatactcttttatctctgtggtctgaatggcagttttccatttcaaaatccagttcaacagctctgcacttatagcatcaaactttttcttagcttcaatatccacatggatctgtctcttctttgggggaggaggaggaggcagttcctgcttagatttttttgtaattgcttgttctcttacacgaacagtctccaaaaggtccttctgaggaatctgagacatccccagctttgctacagcctgagtcacctggttggaggaatcttctagtctctgaaccaaagaatcccatctttgagtcagttcctctgagtcactgttgatcttcttagatgccttggaattatcaagtaattgtcccacatcctggccaatctcactcagctgatccaatgtttgacgcttcatttccatgtcttccttcaaaatagccagacgtcgaacactgacacttagttccttttggtctttgaagttgcttgtctggactttatttaaagcctcttctttttcggttaaccaagctttcaacaagcactgttcttccaataattcctgccacaatatattgatttcttgtaacctattccagcgttcttcagtccaacggcatactgctgtccagcgctcaccaagtttctgtaactggtcttctaggatagctgtagcactctcaccactgttttcatcaacaatgaccaccatgtgagttagtgaatttactttcacctgttcagcctcaagatcactttgcaaacttttatgttcttctagcagcttttgtagagattttacatcatcatccagggggcaagtttccatcttctgaatgcgctcctctgtgagtgttaaccaggcggagagctgctgcagttgcttcttctgcagttccatcagcacatcgtgcagccgggactgtctgtccatactctccaccctaagagcctcccatctagcattcagcagggtcatctgttcctgaatctcaaattcttcttcgtctgacagagttccttgtgttatcagttggttgcctgcctgcaggacgctgcccacactgctctggtgtgcagtcagttccatcataaaagcttcatgggttgcaaactggtctttgacttcttcaacatcatcagaaatatcatcctgctcctggaaagtgtcctcagcagaaagcaaccaggtcagcacttcctccaacgcaatctgatagctgtccagatccatgtcaacctcagtgacagtgctgggagtttcagctcggggactctcatgctcctcctcaggcgctgtactctgtatattaattgcctcttcttcacattcttttttatatttccttgggagtgtctctacctcacggatggcgtctatggtgacttgctgaggtagcacctcaaacaaagatgttaaatacataattatggatttcttgtcaggaagctgaacggcaacatcttcaggatctaacagcttttcaattcccaaataagtttgagccttgctgaaggcatgttcaagtctctcaattggtgacattttgacaactttatcccagctgaagagatcaggtttatgtcggtggaggacagcattaaaggcgagtccatctgtccagctggtggtgaagttgaggacgttgacttggctgtagggcctggtggtctgacgcacccagctgagcaggatcttctcactgttcgtctgctgcaggtccgacatgacatccttcatgacatctttcacctgccagtgcaaaatgatgctccaaagtaaccccaaagtcagtttgtgatttccatccacaatgtcagttccccctatattcactaattccacattgttctgatgtaaaacctgcagcactctgttgacgttatttaaggcatgtacccttgtggaaccacgttcctttggcagtgatgttcctgtgaggccttctagaagatccaatagcttccttccatctttgaggtctgtgaacatatcattgatgggtggtttcccactctttgaaaatcgagcatttatccatttggtaaaggttttcttctgtacgtcattgtgttcatcagatctggacttaatgatatcactgaattcgttctgcccattgtcaggactggcttcatgttctccatacttggccatcttgccagagtttcaagataatccaaaaactttaccaagtcctctttctaaggctttcaacttcctacgatggttcagcttgacatcaatac

SEQ ID NO: 10735 - RNA, 11950 nt, Homo sapiens
  source 1..11950: mol_type = other RNA
ctcatctgcaaagaagtaagtgggcaacgtcaaataaagttaaacggcatacacagggctgtagcttaaaccatatgtgtgtatatataagatatttgattgaaatttatgaatttattaatgtggccaaatcacggaaacaaatacatggatctatttgggatctagttggttatatggctgataaacatatggctgataaattataaataaccaaaacattgtggtaaaagagtcaaagaaaaaatgaagtaattgtgcaaggttaatatgaacagcagaaggaatgtaaaaatgtaaagtggtcttctaattcttatgtaagctttgtcatagttattaaaaagacggtatcatattagaaagcccccacccactttcccaatgctgtatacattatacaaatccgtgacaaatgtattaccatttccaaatacctctctgttcattaatttacacttgcatagaaagggaagaagaaaacaataatatatggttattataaaaacaaaatatccatttctctttggatagtcagtgttttactctttcagtagaacacacagtcagcactcaacatcgtgggccaaggagccatggagcttctgatttaatggaacttggaattggcatttgctgaaaagggcaacactgtacgtcaggaaacattggttggccggatgaatacttcacattgcctgtggcctgctgggaacatttgggcagcaagatggaaacgtgctgtgaatctgctccatgacctccgtgagatccgtgctggtgtcgtgcggtggggccagcaggtcctctcccgctgcctggtggaactgtgggccggaggcatctggatcaagcgagtagctcagtgcagaatgctgaggagaagcccatggggaaacaccattgattcgggaatcagattcaggctgctccagcagctgtcggaggcggtggagctgagactccagctgtttattgtgatcttctaaaatctgcatcctagcctccagccgacctttgtgctgcctgaggagttttgcttctgctataagttctgaatcctcagacgtgtgatggggagatataatcgactctggcggtgaaccgacagggagcccccttcggaggtgctggtccttcagctgctcatactccacctgtagatttctttgttcttcctccaggtcagcaatgatcctctccagttctccacgttcttccctctctactgacttcaggatctgagctgggctctgcggctggctcactggggactctcctccgagtgtttggcaatactgctggatgagggcgtgctcgtcttccacacttcctgtggtggagctgctatcagtgagaaaagacccattagtcctttccatctgggccagtcgtgtggcatattgttctattcttgaatgggtgtcatcatgaaacagttgaggagattgtgaggggtcatagtgctctggccacatactgatgagtgtgataggagtctctaagttgtcaccttcaagaactgtctggacaggcaggtaaccaagtcgagggtgtttggcaaagtacttcttcgacctgaacttgttcttaagtacctttgtgaagtctcgtacatcttccccagatgttgtaggtatacaatattccaccattgggtaatgtaatttgtgaccttttgctgttcgacccgaaaagaaacaactctggcagacatcatagttaaaatgcttaaggcttctatacctgaacccgacaattggacattctttacagatgttgcatttggcctgatgttttgcagtctccgctgctgccactcgatgtaaaactgggagccaaaccatggactgtggttccaaatgcatccaatctataaactctttcacacttatttctggtttattgttattctgttggaagcagctgcgaacactaggctcaatattactgcctccaaaagctgctacttcacctagctgccgggggatctggatggcatcatgaagtaacaggcccagctgcctctggtcacacatttctgttggccctgcaacttccttaaagagatatctgtatttttcttccaagagacctttggagagagacattaatccaatcttcagactctgcactctaatttttccagttcgacccgtgtcatagacattgagcaaccaattgagacacatatcaacacagagtggaacgttgaccaggtccttatgcatttgctcaagtccatcataagttgttgtcagacagttgatgacatctggaacactgaggagctggtcattttggttcaacttgtgctgtttgaaaatttcatttgttgtactcaactctaagagatccaaacatagtgctttttgtagtcttcggattttgattgctgtacggtaggcagaaaaacgtacattattcaggtcagcaagggattgaaagagttcggtcattttaggatggtcccaacaggtggtctgtgtttgatggttgatgtaatagggcactttattatgtgaaatggatctttgccacggcagctggactgacgtagagagaaaatgctgagaggatggtccaaaatctctgtgggcttcctgaagctgtttaaggcgatcatccacagaaacctgtaaaagtttccatcgcatattaaggtcatctagctggcgagacatctttagagagggatgcaggtcaagtggagacagctgactggataaatcattcaccgttttaactttaaagttgattggtgcaatttcttctctaaatgccatgattttttcaatgtgatcctgcagcgagtcaatgagtaagtctcccacgggcttccagccattccgcacggactctgcctccttcatgtcagcgtccaggtcatccatagctccctgcaggtctctgagtttctccaatgccttgtccacttgcttttgccaattgctagttacagcatttagactttcccatttttctttgacttcagaagactgtttgcgcatggctttggcaatcttttgggctctctcctcaggagttaattctgtttttgattgtaggtttcttcttggctcttcaggggcctcaattggctgatcagccaagaaaactcgggcctggtcgacagcattcaggacagaatattctttctcctttaactcccgtctcagggccttacaatggtcatactggagctgtaaggctggaacatctcctccaataggcatttgtttcttaagctcttcatctttcatattcagccatttgatcagttcttctaaggacatcagcaacctgttccacttctcagcgctggcctccaaatgggccctgatgctagcagattttgcttttaagtcattccatctttggttcatatcatccagtcgatgttgaagcatagtagcctcttcagaatttcccaaagcttttaccatcttctgcctgtttccgtcaatgcttttaaatatgtcattgtgggcatcaatttctgcctggatgtcctgcatctgctgtttgagttccctggccaagatactatcctgaagagcattctcccgatgagaggcatccacaagcacattcactgtggtctctgcttcttggatccacttcaggaagttttccagatctctgcgagaggcctgcaccgtcctccactcagcctccaaggcgttctgtctgtcagcaatactttgtttgagattgatccatgatgtttttaagtactctgtggtttctttcacattccttgtgtcatcactcccatattcctccaggagtttctgcaggacgttatcgaacgccatgacgataccatctccaggacccagttcttgaagcagtatttggttatcagaaatttgtttggtgagtggatcccgtcgggcttgctgaagaatatagagtcgagcctcatattttctcatcagttcttcagtctcctccctatggtcatcccactgaagactgtcaataatcatgtcctcaagctgctgctgtcttagctcaacgccatgctgggtgccatcccactggttcttgaccctttccaatttttctgtaattgctgttctcatatctgaactggaagctttatttttcaaattctgtgccaatgtaaaaacataatccagctgaggatggcgctgttctaagtcagcctttgtaattttcattcgggaaacggtcttattgatctcttctacatccccaacagtgacaatgttggacttcagcatctggtcgattaataccagccagtcggctagttctgttatagttttatcaagatcagcaggaattgaaatttccgaagtacgatgagactgaacaggaatatctgacgcagatgatactagcaccaccttttggacattaggatgagcagcaatccttgtctgtgaaacagaactgggctcctggatgcattccttcagggtggtaggcacctctctgcaaatcttattccatgtcatatttacagtccttaagctttctgaaattttatccctttcaggtaaactcagacttttatctgaaagcatctccaattcagttctattcagccatttgagtttttcagcatgtacttccatttcttgagttaagtctcttaattcttgcaggttttctcccaattcggtggttgatctcttttgcatagcatgctcagcctttgttaaccaacagataatctcatctagctgatgcctgtacttcatcacctgcttactttctccttttagccttggctgcctatccttcacttctgcaacaattgcatcccagcgttggtttaaacctgccagtttttctttcaagaagcttccatctgcctgggagagtttctgcacaatcccatccccagttcggtttagtgctgcaaaactgggctggtggctgctgatgcccacctcaagttcctgctgatgtatcctggctttctctaagtccaggctgccacctggagcacaggtatcaaccagtaattcttcagcctctgttatccactgtgtgaggtcattaaggtcacaatggaactgtctccattcttccattgccctgtcaaaacaacctttccgatcactgtacattctattaattctgtcccattttgcattcagctgagtaagtgtatctctgatctgaatggcttcaggtccagaggcttcaaggatgacatctggctgtttttcatgaatgactgcaatctgctctccaagtttgtccagttggtctttgatattcttcagagagtcttcctgaaaagagaagtcttcgtaaatagcagtgttgagctctggaacattaagcgataattcaacatcatccatgcaaagtaaaattttgttaatttcaaccagataatctgtaggaagaagtgatgatctaattccagaagcaagttgacccattttcctctgttgaatagggattgccttaattttgttgtatctagtatgcaaaagtaataattgcaaacggatcttttcttttttattatcttccataggttgatgtaacatttcttctcctctttgtagaacttcctcaatctgggcactctcctcatccatcttttcatcttcatcactggattccaagtgtttttccacaaattttaacatattttctatgtcattttctaatttttccaagtcagagaaaggcacaccagtttcaaatgtttcagtggtgaccaaacattggtataatggttcctgagcaattagcaatttggcacttttgatatgttgagacaccttttcaaagttcctattcagctcagctaactttggttctacaagctccctgcttgagcttccacgggcattcatcaaaataagggcttgatcgcggacattttcaacctggaggttggcatcatccagctcagatactaaacgcttcacaatttcttcctgtttacttgttggtttcttttcaatttcatccaatagagcttcagcttgataaagccaggtacttatgtgagccacgttcccatcaaatatttctagctggttctgatggttcatcaaggtattgcaccaatcttcagtccaggtacgaactcggctccacccagcgttaaggacgcagagcctctcttctaaaataggctcactgccctcaatcaagttttgcagggcagcactactctctgtgatggtatttaaatcagcttttctcttttccagatccttcagaacatttttagcccaggaaatttctgtatccaagtcaccaagcagaccttctgaagtggacttctgtaccaattcagtttcagtagcagaaagccattcagagagagaagcagcctctttcttcattttccgggccaactgtgatgctctttccagatcctgttttccttctgtcacctgtgcgcccaggtcattgtaaagaaccttcagggaagtcagctgctcatccatcccttttgggttgtccgtttgctgtttctggacaatatgtcttcctgttttaatcacagtttccacttcaagtttgacttcactcaaagttttatacagtttcatacacttgtccaggtgcgtctgtatgacgtcagggtctacgtccttcacatccagaacgtgaagttctgctttcacgccatccagcacacgcttgcagtccagcatgcgctgctcgaagttagctggcttctggaaaagctggaactttgtggacacctctcggagtttcctctgtagcacatccatctgacttcctcctctggcagtcctactctctggggaggtcaggggctgagaacgcatatttcttctcaactcctctagggttagctcatgggctgagatctctgcttggattttctgagcttcctgtggaacttggaaagcatctatcctgtcagtcaggtatgtggtgagctgtttgtccagctcccccaagctctcttgcaagacttgaagcatctggtcagtttcccgcagcacctggagttgcttttccaaagaaatctgcttgctctctgccaggtgacttagatcttcatatcggctgttgaaagcctccagtttctcactgattatatcatccaggatccccccatcaatcagagtctggccaagctctcgaatctgggtgcgattatctgccgggtggcgcagaacagattccagagactccagggcttcgttgacagcatccgtcttctcaggcaggacctctgtgctcttcatccgctcttccaaagtgtttaaccaggtagtttcaagatccaaatagtgaagcagttcaatccaacaagaccagacctcctctagcgtgtggcactttcctcgaattctattacaaagaagttggtaattctccagcacaacattcagctcagacgtcaactcctggccaccagagggcaccttggcagctaataacttgatgttgtccttgagaatcttcactctcacctccttctgcaacacatcctcttttgccctcttcatctcttccacagcactctcaagctcttctggtgacttgtactcaaaatcccgctccaaatattcttcctcggcctgggtcatccattcctgcatctctgccaagtctttcttcaggttcgcagctttttcttgactttcagacaacctacttttttgagtagcgatctccttgctaagtttctccagttgagtttggtagtcacctagtcttgtctgcacccaagtttttattccagcaactggaccacttcgaagattagtctctatttccttcatgtttttcagagatgattcaattgtttctatttcattaacaaatgcagagcactggtctaactgcctctgtagacctgcgtcgtctccttgggcagcctgctgtttcattaagaagtctttcacgccatccatccacttctcaatgactgttgaatcggcctcaaaagctctgagtgtgagagcaatttcctcaagcaaatgtagatctttggaaaccaagacctttagcttgttccactttccttgcacatcatcaaattcttgcttatataatttttctacatcaggatgaacatttttctccagagcctttgtttcttctgcaagtttatgtaatgcaggtttctgattctcaaggatttcatcaagggtctttttttcttgcagggccttctccaccttggcaagatcattaaggacattcagagacacctgggccttattttctgaatcatttagcacatctttcagtgttttcaatgtttccagatatgcatgtccaggttggcccttcagttcattctctagatgttgttgacgatcctctacagcctcttgtacagcttggtagcggcccagaaagctatcgaagccccgctggacaaaatctggggcagaaggctgagacatcagggccgagcagcttgcacgagccatttcaattttggggtgaaggccaagaagatttgtcaattcccgctgacaggaatccttcaagcttggcaaggactgccgggaagattcagaaatggaagtgtgttttacccactcctcctttgtcttgatgaccttttcaagctcatcaagctgcttgaaataagcatttatatcttcctgtagctgaatctttctttctagatcttccaaatgttgagatacattcttccattctgatgaaaccttctccagaacattttttatttcttcagtaggaaggccttcttttcccatttgctccacaaggatttgtccagtttggtttaattcatctgctctggggattctttctctctgttctttttctaatgccttcaacttctttttcatttcggaagtgtcttgcatcttcatatactcttttatctctgtggtctgaatggcagttttccatttcaaaatccagttcaacagctctgcacttatagcatcaaactttttcttagcttcaatatccacatggatctgtctcttctttgggggaggaggaggaggcagttcctgcttagatttttttgtaattgcttgttctcttacacgaacagtctccaaaaggtccttctgaggaatctgagacatccccagctttgctacagcctgagtcacctggttggaggaatcttctagtctctgaaccaaagaatcccatctttgagtcagttcctctgagtcactgttgatcttcttagatgccttggaattatcaagtaattgtcccacatcctggccaatctcactcagctgatccaatgtttgacgcttcatttccatgtcttccttcaaaatagccagacgtcgaacactgacacttagttccttttggtctttgaagttgcttgtctggactttatttaaagcctcttctttttcggttaaccaagctttcaacaagcactgttcttccaataattcctgccacaatatattgatttcttgtaacctattccagcgttcttcagtccaacggcatactgctgtccagcgctcaccaagtttctgtaactggtcttctaggatagctgtagcactctcaccactgttttcatcaacaatgaccaccatgtgagttagtgaatttactttcacctgttcagcctcaagatcactttgcaaacttttatgttcttctagcagcttttgtagagattttacatcatcatccagggggcaagtttccatcttctgaatgcgctcctctgtgagtgttaaccaggcggagagctgctgcagttgcttcttctgcagttccatcagcacatcgtgcagccgggactgtctgtccatactctccaccctaagagcctcccatctagcattcagcagggtcatctgttcctgaatctcaaattcttcttcgtctgacagagttccttgtgttatcagttggttgcctgcctgcaggacgctgcccacactgctctggtgtgcagtcagttccatcataaaagcttcatgggttgcaaactggtctttgacttcttcaacatcatcagaaatatcatcctgctcctggaaagtgtcctcagcagaaagcaaccaggtcagcacttcctccaacgcaatctgatagctgtccagatccatgtcaacctcagtgacagtgctgggagtttcagctcggggactctcatgctcctcctcaggcgctgtactctgtatattaattgcctcttcttcacattcttttttatatttccttgggagtgtctctacctcacggatggcgtctatggtgacttgctgaggtagcacctcaaacaaagatgttaaatacataattatggatttcttgtcaggaagctgaacggcaacatcttcaggatctaacagcttttcaattcccaaataagtttgagccttgctgaaggcatgttcaagtctctcaattggtgacattttgacaactttatcccagctgaagagatcaggtttatgtcggtggaggacagcattaaaggcgagtccatctgtccagctggtggtgaagttgaggacgttgacttggctgtagggcctggtggtctgacgcacccagctgagcaggatcttctcactgttcgtctgctgcaggtccgacatgacatccttcatgacatctttcacctgccagtgcaaaatgatgctccaaagtaaccccaaagtcagtttgtgatttccatccacaatgtcagttccccctatattcactaattccacattgttctgatgtaaaacctgcagcactctgttgacgttatttaaggcatgtacccttgtggaaccacgttcctttggcagtgatgttcctgtgaggccttctagaagatccaatagcttccttccatctttgaggtctgtgaacatatcattgatgggtggtttcccactctttgaaaatcgagcatttatccatttggtaaaggttttcttctgtacgtcattgtgttcatcagatctggacttaatgatatcactgaattcgttctgcccattgtcaggactggcttcatgttctccatacttggccatcttgccagagtttcaagataatccaaaaactttaccaagtcctctttctaaggctttcaacttcctacgatggttcagcttgacatcaatacctgctgcccgcgggcctcctcgcctgccggtcgccaccgccgcaccccgagctggccaagggctcctctaggagtttgacacggagtaaccgcgggggtgtgtgcgagtgttagtttggtggtgcgatgtatttaaaaaaaaaaataaagcttggagaagcagacacgaaccgaaattttaaaaaaagaaagaaagaaagagaaattgacacccgactgaaaacgccccttacttgtgcaatcttcctgcctggtagttccgccaaaaacaaaacagtcaaagcgcaaacctggaaggggcgcgcaggcaccaactttgccaaacgctacagagttttccgtttgcagaaatgacccaaaagaaggggggcgccgctccccgtgattccccaatcggcttctggagccagaggctcctcctcgcccctcggcgggagaaagcccgcggccggctgctgctgcccgcttccctgctccgaggaaaaacgactccacaactttgtgcgcgagagaggctcgctccttcggcggctcctcctcctcctccccgctgcgggcctgcccctttgttggagccgagcgctggaggcggaggagggagggtggggcgcaggaccgctgggtcgcgcgttgccgcccccaccccccgggaaggggctcgcctccgggcagccaggggtccgctctccagatgagaagggtgcagatcagcgccagccctccggcccgcgcctctgcagcgctccggctccccctcggcgctctcgccccgccgccgccggcccagcaactttgttccggaagatcagccccactacgttcccgggtcagcgtctgccgggcctcggcggtcaccgcggccaccgc
